European Patent Application EP 4 520 821 A1 - sequence listing, part 12

SEQ ID NO: 16867 - RNA, 5555 nt, Homo sapiens
  source 1..5555: mol_type = other RNA
tacgtagatatatatgtatttttttacacgtaaatacttgaccacttggaacttcccttagtataaaaaggagtctaatccaacttttctcttttcaaggtggcccaaacttctgagcatgggtagttgttgcaaagttccagttcctgatcacacacggcccctttgtgccacgccgagttcctgtgtatttggcttatttgtggactttcttgttccaggaatctttttaaagggccagcatcatgctgtttcaattacaatgttctaaaaacagcagaatttaaaacaatttgactagtctggcatatttgcttttctgttttaactttagaatccgcttgtgttttaaaggaaggttttacatcttaagatactgtatagcaaaatgtgagaatcaacagaactttcacttattcagggcctgtgttccttagtaatgttataatacctttcacataggtgtttccctatttgttactaggtattttatcttttttgggggttgctattgaaaaaatgacttctggtcaggtgcagtgtctcatgcctgtaatcccagcatttggggaggctgaggtaggaggttcgcttgaggccaggagtacaagaacagccttggcaacatagcaagacactgcctctataaaaaatacaataaaaattatctgggcgtggtgatgtacacctgtaggcccagctactcaggtggctgagaagagaggatcgcttgagcccagaaggtagaggctgccgtgaaacatgatcatgccactgcactccagtccaggtgacagttaagaccctgtctctaaataaaaataaaaaatgaccctccattatagcctatatttataggaaagctactgatgtttttgttaattttgtgtctggttaacttggtgaattctttcttcagtcacagattttcatttgctccttagatgacctgggtatgcaaccatctaacctgcaagtaatttcaccttctcctttccacttttacagcatttctgtctaagtgctgtttctttttcaatgatttcttctatactatttgttttaccacactgacctttaacaataaaacattaaatattgctaaataagagaatagatataaatagattttcctttcttttataaaacagaaacaggcaggccgggcatggtggctcacgcctgtaatcccagcactttgggaggccaaggcgggcagatcacctgaggttaggagttcaagaccagtctggccaacatagtgaaaccccgtctctacaaaaatacaaatattagctgggcatgatggcgggtgcctgtaatcccagctacttgggagactgaggtgggagaactgcttgaacccaggaggcggagggtgcagtgagctgagattgcaccactgcactccagcttgggcaacagagcaagactccacctcaattaaaaataaataaactaaaatggaaacaggatctccctatggtgctcaggatggtctggaactcaggctcaaacgatcctcccaccttgccctcccatagctgggactacaggcgtgagccactgtgctcaaatgaaacaaaggcacagcacaacgaatcgtccaagtaaaaaagacccacttgtcactacctggccccactggtattttgtggtagaggtggccaggaaagaataatcacttgagaggggacaggtgctccctgctctgacttctgtctagtgcactagtagtcaaagctgctaaagagttatgaagaatgtgtcatttgcatatcacaaagttttattaatgtaattttaaggccaattaaactaattttattcaaagtaagtctacattaaattacaatattaacaatctctagacacaacgaacttataagaaaaaaaaaatagaaatctgtttggtctttcttagaccacatatcatggaactcataaatgaaaattttcaaagatagaaatgacaattaaagagtgaggattttaatatggaaacccacaaggtgtcatatttcaaacccgcatgtttcaaaaagagactcttaataatttagcacaaaatcaaattatataaacttggtatattccagaaaatattgctttaaacacttatgccatgatcaaaattcctttggtagcttttaatcaaaatgaaacatgctattatgtaaaatataaagtacttttaaatgttatctcaaaagtatctttgtcatagttacccttctaacatcactactgaactttcctttcactgttcaacctcatgtatatatacacaacacaaaaccaggtaccaacaaaatccttttaatctttccacaaaataacctctgcttcacaacatcaagactttaagtctccataaactttttacagtttacagcagagaacaaggatcgtccctgcgcatgactgtaaaaaccaaaccaaactttattattgcaatcacacaaatactgcaattaaaaaaaatcaaagagcagttaccccaatgcaaaaaaacagggactgccagactcaatcttagaatggaaacacaaacacactagccccaaaccctaaaacagagattcacaaggaactcagctgacgaacagacgcagcagggcggacaccatggccttggcacctcagggagctcacttagaaacctgacttacgaaaaatcagccatcaaagtttacaacttttggaaatacatgaaacagagaggggccagtggctagggtgcgtcatccattcgccagctttgaaccctggctctttctaatgttcacccatgaagggcccttgttttcactctaaatgctgatcatctgagcgagctgtcttcagggatacctaaggaatcttcagagctaaaaaatgcagcatctagggtcttcttcattgtgcactcatgatcacacacgagaacaaaccaaacttgcagctttttgacacaagaacaagaccttttaaaggaacttctctttagtaacatcttcttgtccaatctcaaagttattttgcacagagtaacagaaacaatttaaatgcctaaaagaactagaggaaaaactggagggaaaaagatacatctgcaggttgaagtcttgagccttgtgaaagatgacccaggagccacctcccttccttcgccttccaatgtccacagctggatcaatcagagtcccagaaatggcacaggtgtgcttcctgctctgagggtacattctagtgtttcatgaaggggaaccgtctgcagatgcgtcaggccacgtagtggtactgattcggattgtctttgtctctctccatatagtctctgtctatcagagattcaattctctttttcaaatctccaggctttactggaaatttcagctgattatataattcagaaactagaagattatgaccaagagtctttctcatcttcattattctgacgatagcagcatcaatctgatattgtctatcctgaaacactctctcagtggtgctaacctgttcctcaacagtttccttcatctgaatttgattgatctttattctaaacaacttgtgcttgaactctccattaaaaatgaacttgtctccatcttccacttcctttcctttgggacttttaatcagcacacgtgctttgccacaggccagggactgcagcgttctgcgcaattcactatcctctatccccgtggccatttttatctcctcaaagctgaagccatctccctcgttgaacatgaggagcaccagtgtctggaagagggacacctggaattccttcttcccttctttaaactccgcttttaaaacagcatgtcccaaagtagtttgccactgaagttttcgaccactgtgctttccaagataaaatgccttaaatacttcctgaagtttaatcatttctggggttaagtgcacttccatgggcgtgtatgttggccagtagcccattgtgagtatgttcactgtgaggtctatagggcctgagtcactctgattctgcatatgctgcttgaaatgaaccatgatgtccttcgaaagctccatgtccttgaacatgccttccagcttgctggtgaaggctgcaccgcactcatgcttgagctttgacaacatagacttttcagcatcgactgaggcacttttcccaacaaggagtctttttgccaaatcttttttataaaatgcttcaaagacatctttaccgtggataaacctgaacaggatcatgatcttgtccaacgtccgctccagctcctcgtctgtggcttctttgttgcctgctcttaactttgaatccacatgctttgcgatcagttctgcaggcttgttgggtctcttgttgatgaacgtctcaaaggactccttcatcaggttgacgaaccgctcattcttctggaagcagacctcgatcacgtggtccaccttgtccttgaagtccaacaggtcttggaccatgtctttgtctttctcaggattgattacgatcgctgttccaaaagtcttgatgtactcgctccagtgctgcagcagcgcctgctgcccgcccctcacccggctgaacagctggtacatctgtgcgaggtccggcactctgttctcatccagtaagtggtcgagccctttctgcagaattgctgttaaatgttctcctaatagctgtttctccacacaagcaatcagtggtttctgtgtgctgtggtccaagtaagtgattactctgtctccctcttcctctaagcgtttacttacatggttaagatattctggaacctctctttcctgcattaacctttggccttcggcagcatataagcaattagtctcttccaaaaatttcagttcaaatgaatctttatacacctgcaggtcagacagcatgcccaggaggctccgcaacaggctccggtccacggcctcgccgctcctctcgcgctcgatcagcagtaggattccatcaatggttttactctgaaccattttatcactaataatatgggttctaaacagttctaatcccatatcccagatggagggcagcgtggagttctgcagcacataggtgcggtccaagaacaggaagatgcttctgatcatgatcatttgtctgcagtggtcctgccagcacgtgttaatcttctttaaaaataaaacactatctagtgatctctaaacggaaggatctgtgcctggacgtggtcttcacaggcctgacgcagttgcttgtagagcattggggagactttgtgagaacagagattttccacagcctggtagagctcctcgaggttgtacctgatggaggtgctgctctgcacggcccgcaccgcctcgtgcagcttccgccacgtgtcctgcgtgtagttgtcgggcagccgaggtctgtctcggaagttcttgatgaccagcttcttggagccgcccgcgccccccggcttggcgggcgcggcggccagggccgcgggcttggtgaggccgttggtgcggcccacgagcgccgagaagctgcccttccgcggggcctcgtccgccatggctgggccggaacc

SEQ ID NO: 16868 - RNA, 5479 nt, Homo sapiens
  source 1..5479: mol_type = other RNA
tacgtagatatatatgtatttttttacacgtaaatacttgaccacttggaacttcccttagtataaaaaggagtctaatccaacttttctcttttcaaggtggcccaaacttctgagcatgggtagttgttgcaaagttccagttcctgatcacacacggcccctttgtgccacgccgagttcctgtgtatttggcttatttgtggactttcttgttccaggaatctttttaaagggccagcatcatgctgtttcaattacaatgttctaaaaacagcagaatttaaaacaatttgactagtctggcatatttgcttttctgttttaactttagaatccgcttgtgttttaaaggaaggttttacatcttaagatactgtatagcaaaatgtgagaatcaacagaactttcacttattcagggcctgtgttccttagtaatgttataatacctttcacataggtgtttccctatttgttactaggtattttatcttttttgggggttgctattgaaaaaatgacttctggtcaggtgcagtgtctcatgcctgtaatcccagcatttggggaggctgaggtaggaggttcgcttgaggccaggagtacaagaacagccttggcaacatagcaagacactgcctctataaaaaatacaataaaaattatctgggcgtggtgatgtacacctgtaggcccagctactcaggtggctgagaagagaggatcgcttgagcccagaaggtagaggctgccgtgaaacatgatcatgccactgcactccagtccaggtgacagttaagaccctgtctctaaataaaaataaaaaatgaccctccattatagcctatatttataggaaagctactgatgtttttgttaattttgtgtctggttaacttggtgaattctttcttcagtcacagattttcatttgctccttagatgacctgggtatgcaaccatctaacctgcaagtaatttcaccttctcctttccacttttacagcatttctgtctaagtgctgtttctttttcaatgatttcttctatactatttgttttaccacactgacctttaacaataaaacattaaatattgctaaataagagaatagatataaatagattttcctttcttttataaaacagaaacaggcaggccgggcatggtggctcacgcctgtaatcccagcactttgggaggccaaggcgggcagatcacctgaggttaggagttcaagaccagtctggccaacatagtgaaaccccgtctctacaaaaatacaaatattagctgggcatgatggcgggtgcctgtaatcccagctacttgggagactgaggtgggagaactgcttgaacccaggaggcggagggtgcagtgagctgagattgcaccactgcactccagcttgggcaacagagcaagactccacctcaattaaaaataaataaactaaaatggaaacaggatctccctatggtgctcaggatggtctggaactcaggctcaaacgatcctcccaccttgccctcccatagctgggactacaggcgtgagccactgtgctcaaatgaaacaaaggcacagcacaacgaatcgtccaagtaaaaaagacccacttgtcactacctggccccactggtattttgtggtagaggtggccaggaaagaataatcacttgagaggggacaggtgctccctgctctgacttctgtctagtgcactagtagtcaaagctgctaaagagttatgaagaatgtgtcatttgcatatcacaaagttttattaatgtaattttaaggccaattaaactaattttattcaaagtaagtctacattaaattacaatattaacaatctctagacacaacgaacttataagaaaaaaaaaatagaaatctgtttggtctttcttagaccacatatcatggaactcataaatgaaaattttcaaagatagaaatgacaattaaagagtgaggattttaatatggaaacccacaaggtgtcatatttcaaacccgcatgtttcaaaaagagactcttaataatttagcacaaaatcaaattatataaacttggtatattccagaaaatattgctttaaacacttatgccatgatcaaaattcctttggtagcttttaatcaaaatgaaacatgctattatgtaaaatataaagtacttttaaatgttatctcaaaagtatctttgtcatagttacccttctaacatcactactgaactttcctttcactgttcaacctcatgtatatatacacaacacaaaaccaggtaccaacaaaatccttttaatctttccacaaaataacctctgcttcacaacatcaagactttaagtctccataaactttttacagtttacagcagagaacaaggatcgtccctgcgcatgactgtaaaaaccaaaccaaactttattattgcaatcacacaaatactgcaattaaaaaaaatcaaagagcagttaccccaatgcaaaaaaacagggactgccagactcaatcttagaatggaaacacaaacacactagccccaaaccctaaaacagagattcacaaggaactcagctgacgaacagacgcagcagggcggacaccatggccttggcacctcagggagctcacttagaaacctgacttacgaaaaatcagccatcaaagtttacaacttttggaaatacatgaaacagagaggggccagtggctagggtgcgtcatccattcgccagctttgaaccctggctctttctaatgttcacccatgaagggcccttgttttcactctaaatgctgatcatctgagcgagctgtcttcagggatacctaaggaatcttcagagctaaaaaatgcagcatctagggtcttcttcattgtgcactcatgatcacacacgagaacaaaccaaacttgcagctttttgacacaagaacaagaccttttaaaggaacttctctttagtaacatcttcttgtccaatctcaaagttattttgcacagagtaacagaaacaatttaaatgcctaaaagaactagaggaaaaactggagggaaaaagatacatctgcaggttgaagtcttgagccttgtgaaagatgacccaggagccacctcccttccttcgccttccaatgtccacagctggatcaatcagagtcccagaaatggcacaggtgtgcttcctgctctgagggtacattctagtgtttcatgaaggggaaccgtctgcagatgcgtcaggccacgtagtggtactgattcggattgtctttgtctctctccatatagtctctgtctatcagagattcaattctctttttcaaatctccaggctttactggaaatttcagctgattatataattcagaaactagaagattatgaccaagagtctttctcatcttcattattctgacgatagcagcatcaatctgatattgtctatcctgaaacactctctcagtggtgctaacctgttcctcaacagtttccttcatctgaatttgattgatctttattctaaacaacttgtgcttgaactctccattaaaaatgaacttgtctccatcttccacttcctttcctttgggacttttaatcagcacacgtgctttgccacaggccagggactgcagcgttctgcgcaattcactatcctctatccccgtggccatttttatctcctcaaagctgaagccatctccctcgttgaacatgaggagcaccagtgtctggaagagggacacctggaattccttcttcccttctttaaactccgcttttaaaacagcatgtcccaaagtagtttgccactgaagttttcgaccactgtgctttccaagataaaatgccttaaatacttcctgaagtttaatcatttctggggttaagtgcacttccatgggcgtgtatgttggccagtagcccattgtgagtatgttcactgtgaggtctatagggcctgagtcactctgattctgcatatgctgcttgaaatgaaccatgatgtccttcgaaagctccatgtccttgaacatgccttccagcttgctggtgaaggctgcaccgcactcatgcttgagctttgacaacatagacttttcagcatcgactgaggcacttttcccaacaaggagtctttttgccaaatcttttttataaaatgcttcaaagacatctttaccgtggataaacctgaacaggatcatgatcttgtccaacgtccgctccagctcctcgtctgtggcttctttgttgcctgctcttaactttgaatccacatgctttgcgatcagttctgcaggcttgttgggtctcttgttgatgaacgtctcaaaggactccttcatcaggttgacgaaccgctcattcttctggaagcagacctcgatcacgtggtccaccttgtccttgaagtccaacaggtcttggaccatgtctttgtctttctcaggattgattacgatcgctgttccaaaagtcttgatgtactcgctccagtgctgcagcagcgcctgctgcccgcccctcacccggctgaacagctggtacatctgtgcgaggtccggcactctgttctcatccagtaagtggtcgagccctttctgcagaattgctgttaaatgttctcctaatagctgtttctccacacaagcaatcagtggtttctgtgtgctgtggtccaagtaagtgattactctgtctccctcttcctctaagcgtttacttacatggttaagatattctggaacctctctttcctgcattaacctttggccttcggcagcatataagcaattagtctcttccaaaaatttcagttcaaatgaatctttatacacctgcaggtcagacagcatgcccaggaggctccgcaacaggctccggtccacggcctcgccgctcctctcgcgctcgatcagcagtaggattccatcaatggttttactctgaaccattttatcactaataatatgggttctaaacagttctaatcccatatccctgtatagacagtaagaaacaggacagatggagggcagcgtggagttctgcagcacataggtgcggtccaagaacaggaagatgcttctgatcatgatcatttgtctgcagtggtcctgccagcacgtgttaatcttctttaaaaataaaacactatctagtgagtcttctctaaacggaaggatctgtgcctggacgtggtcttcacaggcctgacgcagttgcttgtagagcattggggagactttgtgagaacagagattttccacagcctggtagagctcctcgaggttgtacctgatggaggtgctgctctgcacggcccgcaccgcctcgtgcagcttccgccacgtgtcctgcgtgtagttgtcgggcagccgaggtctgtctgcgcacccgcggcggggccgggggcgccaggacccagacggaccgagggccggaagt

SEQ ID NO: 16869 - RNA, 7174 nt, Homo sapiens
  source 1..7174: mol_type = other RNA
tacgtagatatatatgtatttttttttcttaaaaagggaaaacaactgttcaaaaccaactgggcagtatggtgggggtggggagcagtcctacagaagggggccgagaacttcccccccaggaacaaagaacaaacacaatacaaagaaaataaccaccaatgctcccgcatggctcaggagcctctagagaacagattgtcccatcctcaaactggctttttttttttccttttttttttaatcttttttttttccattttcttttttgttgttgttgttttagcacctgtacaataaaactgtaccatctccaaccagagccggccacggcgaggccctcctgcctttggatggtacatactctacaaggattgttcggaaaaatagcaattggtagaaaaataagagtgggagggacaatgccacagagggggcggggacagggaagcaacccaagctcctctctctctctcactcgacaaacccagcgctggaggcccagaggccagggggaggccaggtagggataccactcagccccaggcccccaggcatgagtggagcaagggctggagaccactttcctgcccttgcctaggaaacagctgacgcctggatttcacatccggcagtgagtcccagagccctctgcagattcccaaggagaatgaggggctgagggaggaggtgggaggagaggaaggaaaggggtgctgtgagtctcagaaggggcagggatgggggtggctgagggctgggaggtgagaggctcagtatcttgagacagggaggccagaacggggtgggagagtggaggcaggaacaaactcgtattgtgcactctgaggggggcagtgaagaaggcgtgaggaggggggccaccctcacccctcagatcccttctccacgctcctttattagagtaacttattaacccctcacctcacaatcctcccctccctgtcaacactaatctcaagatagcggggctgctgcaaagggcgggaatgggtgggtgggggagcaccaaagcctcaggatttacccccaagcccccagccctgggccagcagcaaccagcttcgttagtcacaagtccatgttcccccaccccattccacctcaccccctccccagtgggggaaaaaaacaccagggaatagctttgtcagagctcatcaacaaagaaaaagaaaaggaggtacagaaagtccctcaatacaacaagttgtctcaaatcgtcacagtgatacagacttatcagaaaccaatgaaacaatacaaattaaatactaataaaataaatactacagaagacagaagaacacaggggaatggagttggggggcgctcagagatctgggattttctcatttctcctcgggacaggccaaggccatccagggcccaggtttggtcttggtcatgaacaaggaggccagtccaagggaccccggcgccacctcccaccacccccgggacctcttgtcctcagacatggagttcaactttccacccccatcagcaaccacgataacaatgacgacgacagggagatgagaactaattgtaaccaaaaaaacaaaaacagtccagtcgctaatgctggcattgataaggcggcttcttgttggtccgtattattgcctcattctgcagtctggtgctcggtcggggaaagacaaggaggtgggggaagggcgaactcggaaggagaaagaagaggaggggctgttttcccggtcaactgttgcaagactggaattccacctcggaccctaggagccgaagtaggtctggctcgtaccgcaccagctccacagtctcagaggagcctgggggggatctgtcgtccaagcctccaggcctctcggcaggggtcagcagctgactggaggccacctgcctgtagaactcggccttgggcatggtggtgatttcaaagtgcgggaaccgggcctgaaagatcctcgaggaaagcttcagcctcttcaagacatcggaaaagaggaaccagttgcagggcccgcgggacactgacacttggaggttgtagcaagggagaagaggcttgtctgagagttcaaacatgaaatcatcctcctccatcggatcgtctccttcttgatctgagctcccaggaggattatgtaggaggtcacaggcaaacccgtctttttcctccaacacagaactgctgtaaaaatcccaggatacaccgggatcaccctctgcccggccctgaagatccgagaggtgatcactgagaaagcgcttcatggtgtcgctgctggccagcttcatggctgtctgacccgagtaggtagccagtgtgggatcggccccataggacagcaggagccagatggtctccaggttgtcattgaccaccgcatcatgaactggcctcgtgccgtcctgcgcactgcagttcacgttggccccgtgctccagcaggatgttcaggatgtcggtccagccccgggaacaagcctcatgcagggctgtgtagccagcattgtcacggtgattcacatcttcactgtctttctggaggcagtagagaacaacatccttatagccaagacgcgccgccctctgcaggagggtctcaccagcatttttgttcactatgagccgacgtgcctctggggggatctgccgggctgtaggtgactctgaggcctcctctgagctggcacttcgggacttagagggtgtacatggttctgtgggtttcactggggtgggagatttgggagatcgtgtcttctgctggctccaacgacctttgccctttgcctcttctgagacggttgccatgtgcttggtcttgcactttcgttttcctgatggcttttctgaattttcaaggcaggctggctcttccaggttatttgggaggaaaccgtttggtgaatccgagatcccctggactttgttgggcaagagaaggttcctgttcctgaggcggtgctccaaactttgggaggaggaagtcttctgcttacgggcctttaaatcagactgactgcgcgtgcgggtgctcagaaccacaggaataaagtcacggaaactgctctttgctttcttttccaaggaaccttcctcgtggctgtcggctcgttttcctggagactgggactccggctttgtcggcttccggtgcttgtgctttcccctgactccattgtgctcttttcctgaatctgaagcccccctggggcttttcttggtggattcctgggggtcactgggcagcttccggcacttgggtctgtgggaactccggaccacggccttggcttgtggctggagctgctgctcttcactgtccttctctttgccgcacttcatcttcttgggcggcagagattccgtcacatcatctggctgccacttgttcttgcaagcaaagacccctacgctttcctgtttcactcgagcctgcccggccttagcccgaacttcagcttggcccctctggggagccactgggaggccatcagcccggaagcaggtggctaaattgaagaccacatcaccatccaccttctccattttcactcgccccagatccacctggcttccaagctgtgggcgctctgtgctggagcccctcctgctgctcggaaccacgtccaatataagttccttggggtggctgtcgtgaggtagcaaaggcagctcaggcatcttaggcaggttctggggggtggccaggaccagctcatgggacatgtaggtggccagcacttggttcttaggcttcgtgtctcctgccagcttcaggccacaagccccctgggggccttccatcttaggagtgctgtcagagcagaggtggctctctgattcctcaggcccctgattcattcgaatgtccccaccgctaggctgaacagacagtgccagggtcccagtctgagggctgagggtcaagaggacaggattgacttgttcttcataaggcttggcagcaatccggcaagttttgttctttgtaacagggtcctgctctggaacgaaggagcccccaggccgtggttgcccctcaggaagtccgtgcacggcttcgctggagctgagagatggcacaccagaaaactccgaaacaacgctggtgggcctgatgggcgccccctgactgggggtcagctgcccggcactggaaatgccaatggaaagcagagacgcctggtggtacggggaccagccaacaggcaggacctgggtgctggtaggtttcccattgactgaacaccggggataaatatttgccggccccgtgggtttccacaaagagagttccttggtttggcaccctggcagcccaggggcaatgcgggctggagtatatcgtttcactgtgcttggctgtccctcagcaccagcctggctgccctttttgccacacgtggcaccagtgcccttaggctctccttgatcaatgatggagatgggctcctgcttggggagatggcgggggtcacggttgaggcccaggttggggtctttgttcagcagcagggatgcaggcactgggttggccactcccacgtaggtgccaggaatggtgctgatcagtgcagttgagttcttcacccaggtgctcgggtccccattcctcacgatctcgggaaagatgacaaagggcgaggaagtggagcccaggcaggaggtgacattgccaccggcagcctgggttgtgcgctgagacctagacaggactgtggagaggagggccttgctgctggtgtgcacgggggtcaacacaggcatggggggtgtcttgcgctggttcggcaatggaagcttctggcggttggacttggaggacagatcaaggggcatctcgctgcactcaggtggagaggccatctctcgttccagctgtggcggtgacttaagaggagagaaggtaacggaagtcccttctgtttgctgctcggtgccactgggcatcttggcggggtgcggtggggctgagctcccactgggggctggcagcagaggctgtggagttggaagcaccttggcagaagcagtaacaagggaggtatctgccaaaggcccagggaccccatcgggtgcaggctgggtggtggtgctaccggatggggaagtgcaggggagcctgttcacctccagagataccagcttggaatccgaagtcagaggccgggccacagaaaatgcatacgggtaagaacggagctcgggggaggctagcacgcctgggagacacctgtcctgcaggtaggacggcaggacagggagcgtaagagtggaggaaacccctagagtggttggcagtgtggccacactgagtggctgcccacagcttggaggcgggatatataccagcggctggctcggggtcagcactgtccctggctgaaaggacagggggactttttgcatagctggtgcctgagctgcaggaaagcacactctactcaaactgaaggaggccgggatgggtgcagaggtgggaatggcagctggcgtggcagcaggcatgggtgtaggggctggagtaaagatgggggctggggtgggtgcaggcaccggtgtaggagcaaaggcggggatgagggtgggggtagaaggtgggccggaagatggggttggagtgggcatgggcacagacggaggggcaggggccgctggaggcgtggatgctggcatgggagccagaaccggagtggggacgggagcgagaaccaaggtcggagctgaagggggcacaggagcctggatgagagccaagggaggagctgaaactgggactgaaagcggggcaggagctggagccgacaagggaaccgggcctgaagggggagcagaagctggcacaggcaccaagactgaggccgaaacagaaagggggttcgagtcagagatgagcgtgggcactgacggtggcgctggagccagagccgggacaggtgctaagggaggggaaggagctggaaccgaagtggcaacttggactggaacaagccctgaatgggggactggggcagggacggagaggggaacctggaatgcatctggaacagagtggggcacagaggccgaaccgggagcagggggacagataggggctggcagaggactgaagttagtggtaaccaggggcagggtcccctccacagggactccagttcccagagttgccaaaatgaaagtattcttctctccaacaccttgccgagagtccaaagcctttactccggcgggtgagcagtcaacctgtttgctcatttgggtgttgagtggagtccaggagcagtcggccctgctgttgctggcctcggcgctgtcagatgcgggaagcttgagcccgtctcctgggctgctcaggggcaccaagaggccctcagcctctgccacgttcccagcgtagtccatttttggctggggatcgtcaggcttgtcttctgacttgtgcccaagtttttctgtagcactgccatctgggtctgccccccgggcattgctgccacttccaactgccgtgagctccaccttggaaaaactgctgctgacacaaaactcctgagatccaaagtgctggcagtcgcctgtcgttgactcctcatcagaaagaggtgctcttctctcctcgttgatgccacacatgcgaatccggtcagaactggtccagttgtgcacgccgctgtagagcggtgctgtagagatcatgacagccactcaccaccagataggacctgctgtggccactcccccgaaataatggtgggggcgacccgagttggactggtggctactttccctccaaggctagccgtccttcgccacgccgaccccctaggagagtcagatggctgaagaagggggaaggcggtgggagtgctggagagtaaaaggactgtggcggggagggtccgcggcccccactacgagagcagaatccagatgctaagaggtgggtggggggtgcggcacaatcgcagactgtgtctttcctcgcttttcccggaatcgccgcccgatcaccgtctaacactcggagttgcttaccactcagtcccctagccccatttgtgcgcgtgaggcggccagagcccgggaagcccgggcacaaactccgcggaagctggccttcgctgccgccgcgccgccgcgggcctccctccctccg

SEQ ID NO: 16870 - RNA, 7595 nt, Homo sapiens
  source 1..7595: mol_type = other RNA
tacgtagatatatatgtatttttttttcttaaaaagggaaaacaactgttcaaaaccaactgggcagtatggtgggggtggggagcagtcctacagaagggggccgagaacttcccccccaggaacaaagaacaaacacaatacaaagaaaataaccaccaatgctcccgcatggctcaggagcctctagagaacagattgtcccatcctcaaactggctttttttttttccttttttttttaatcttttttttttccattttcttttttgttgttgttgttttagcacctgtacaataaaactgtaccatctccaaccagagccggccacggcgaggccctcctgcctttggatggtacatactctacaaggattgttcggaaaaatagcaattggtagaaaaataagagtgggagggacaatgccacagagggggcggggacagggaagcaacccaagctcctctctctctctcactcgacaaacccagcgctggaggcccagaggccagggggaggccaggtagggataccactcagccccaggcccccaggcatgagtggagcaagggctggagaccactttcctgcccttgcctaggaaacagctgacgcctggatttcacatccggcagtgagtcccagagccctctgcagattcccaaggagaatgaggggctgagggaggaggtgggaggagaggaaggaaaggggtgctgtgagtctcagaaggggcagggatgggggtggctgagggctgggaggtgagaggctcagtatcttgagacagggaggccagaacggggtgggagagtggaggcaggaacaaactcgtattgtgcactctgaggggggcagtgaagaaggcgtgaggaggggggccaccctcacccctcagatcccttctccacgctcctttattagagtaacttattaacccctcacctcacaatcctcccctccctgtcaacactaatctcaagatagcggggctgctgcaaagggcgggaatgggtgggtgggggagcaccaaagcctcaggatttacccccaagcccccagccctgggccagcagcaaccagcttcgttagtcacaagtccatgttcccccaccccattccacctcaccccctccccagtgggggaaaaaaacaccagggaatagctttgtcagagctcatcaacaaagaaaaagaaaaggaggtacagaaagtccctcaatacaacaagttgtctcaaatcgtcacagtgatacagacttatcagaaaccaatgaaacaatacaaattaaatactaataaaataaatactacagaagacagaagaacacaggggaatggagttggggggcgctcagagatctgggattttctcatttctcctcgggacaggccaaggccatccagggcccaggtttggtcttggtcatgaacaaggaggccagtccaagggaccccggcgccacctcccaccacccccgggacctcttgtcctcagacatggagttcaactttccacccccatcagcaaccacgataacaatgacgacgacagggagatgagaactaattgtaaccaaaaaaacaaaaacagtccagtcgctaatgctggcattgataaggcggcttcttgttggtccgtattattgcctcattctgcagtctggtgctcggtcggggaaagacaaggaggtgggggaagggcgaactcggaaggagaaagaagaggaggggctgttttcccggtcaactgttgcaagactggaattccacctcggaccctaggagccgaagtaggtctggctcgtaccgcaccagctccacagtctcagaggagcctgggggggatctgtcgtccaagcctccaggcctctcggcaggggtcagcagctgactggaggccacctgcctgtagaactcggccttgggcatggtggtgatttcaaagtgcgggaaccgggcctgaaagatcctcgaggaaagcttcagcctcttcaagacatcggaaaagaggaaccagttgcagggcccgcgggacactgacacttggaggttgtagcaagggagaagaggcttgtctgagagttcaaacatgaaatcatcctcctccatcggatcgtctccttcttgatctgagctcccaggaggattatgtaggaggtcacaggcaaacccgtctttttcctccaacacagaactgctgtaaaaatcccaggatacaccgggatcaccctctgcccggccctgaagatccgagaggtgatcactgagaaagcgcttcatggtgtcgctgctggccagcttcatggctgtctgacccgagtaggtagccagtgtgggatcggccccataggacagcaggagccagatggtctccaggttgtcattgaccaccgcatcatgaactggcctcgtgccgtcctgcgcactgcagttcacgttggccccgtgctccagcaggatgttcaggatgtcggtccagccccgggaacaagcctcatgcagggctgtgtagccagcattgtcacggtgattcacatcttcactgtctttctggaggcagtagagaacaacatccttatagccaagacgcgccgccctctgcaggagggtctcaccagcatttttgttcactatgagccgacgtgcctctggggggatctgccgggctgtaggtgactctgaggcctcctctgagctggcacttcgggacttagagggtgtacatggttctgtgggtttcactggggtgggagatttgggagatcgtgtcttctgctggctccaacgacctttgccctttgcctcttctgagacggttgccatgtgcttggtcttgcactttcgttttcctgatggcttttctgaattttcaaggcaggctggctcttccaggttatttgggaggaaaccgtttggtgaatccgagatcccctggactttgttgggcaagagaaggttcctgttcctgaggcggtgctccaaactttgggaggaggaagtcttctgcttacgggcctttaaatctgctctccctttccgccgctgctcgtcttcttgctctgtcaggtactccccagtctgatattttcggctcttctgccgtcttcgtttcttcctcttcagcaggccctcctcctcttcttcctcctcctcctcattggtgtcccacatttgccgggcagcctctgtcctccagggcatttctcgggctcgccacaggtgccttcggccctggctcagcagagacttgtcctgggcatggtggctgcgatactgggtgtcccgttgggtctttctcacctttcgacgcttagctggggtgggggttacctcctcttcttcttctgtggggaagacttcctggcttcccatgtcactgtctgccatgccagcaaaggagctacagatgcttccagactgactgcgcgtgcgggtgctcagaaccacaggaataaagtcacggaaactgctctttgctttcttttccaaggaaccttcctcgtggctgtcggctcgttttcctggagactgggactccggctttgtcggcttccggtgcttgtgctttcccctgactccattgtgctcttttcctgaatctgaagcccccctggggcttttcttggtggattcctgggggtcactgggcagcttccggcacttgggtctgtgggaactccggaccacggccttggcttgtggctggagctgctgctcttcactgtccttctctttgccgcacttcatcttcttgggcggcagagattccgtcacatcatctggctgccacttgttcttgcaagcaaagacccctacgctttcctgtttcactcgagcctgcccggccttagcccgaacttcagcttggcccctctggggagccactgggaggccatcagcccggaagcaggtggctaaattgaagaccacatcaccatccaccttctccattttcactcgccccagatccacctggcttccaagctgtgggcgctctgtgctggagcccctcctgctgctcggaaccacgtccaatataagttccttggggtggctgtcgtgaggtagcaaaggcagctcaggcatcttaggcaggttctggggggtggccaggaccagctcatgggacatgtaggtggccagcacttggttcttaggcttcgtgtctcctgccagcttcaggccacaagccccctgggggccttccatcttaggagtgctgtcagagcagaggtggctctctgattcctcaggcccctgattcattcgaatgtccccaccgctaggctgaacagacagtgccagggtcccagtctgagggctgagggtcaagaggacaggattgacttgttcttcataaggcttggcagcaatccggcaagttttgttctttgtaacagggtcctgctctggaacgaaggagcccccaggccgtggttgcccctcaggaagtccgtgcacggcttcgctggagctgagagatggcacaccagaaaactccgaaacaacgctggtgggcctgatgggcgccccctgactgggggtcagctgcccggcactggaaatgccaatggaaagcagagacgcctggtggtacggggaccagccaacaggcaggacctgggtgctggtaggtttcccattgactgaacaccggggataaatatttgccggccccgtgggtttccacaaagagagttccttggtttggcaccctggcagcccaggggcaatgcgggctggagtatatcgtttcactgtgcttggctgtccctcagcaccagcctggctgccctttttgccacacgtggcaccagtgcccttaggctctccttgatcaatgatggagatgggctcctgcttggggagatggcgggggtcacggttgaggcccaggttggggtctttgttcagcagcagggatgcaggcactgggttggccactcccacgtaggtgccaggaatggtgctgatcagtgcagttgagttcttcacccaggtgctcgggtccccattcctcacgatctcgggaaagatgacaaagggcgaggaagtggagcccaggcaggaggtgacattgccaccggcagcctgggttgtgcgctgagacctagacaggactgtggagaggagggccttgctgctggtgtgcacgggggtcaacacaggcatggggggtgtcttgcgctggttcggcaatggaagcttctggcggttggacttggaggacagatcaaggggcatctcgctgcactcaggtggagaggccatctctcgttccagctgtggcggtgacttaagaggagagaaggtaacggaagtcccttctgtttgctgctcggtgccactgggcatcttggcggggtgcggtggggctgagctcccactgggggctggcagcagaggctgtggagttggaagcaccttggcagaagcagtaacaagggaggtatctgccaaaggcccagggaccccatcgggtgcaggctgggtggtggtgctaccggatggggaagtgcaggggagcctgttcacctccagagataccagcttggaatccgaagtcagaggccgggccacagaaaatgcatacgggtaagaacggagctcgggggaggctagcacgcctgggagacacctgtcctgcaggtaggacggcaggacagggagcgtaagagtggaggaaacccctagagtggttggcagtgtggccacactgagtggctgcccacagcttggaggcgggatatataccagcggctggctcggggtcagcactgtccctggctgaaaggacagggggactttttgcatagctggtgcctgagctgcaggaaagcacactctactcaaactgaaggaggccgggatgggtgcagaggtgggaatggcagctggcgtggcagcaggcatgggtgtaggggctggagtaaagatgggggctggggtgggtgcaggcaccggtgtaggagcaaaggcggggatgagggtgggggtagaaggtgggccggaagatggggttggagtgggcatgggcacagacggaggggcaggggccgctggaggcgtggatgctggcatgggagccagaaccggagtggggacgggagcgagaaccaaggtcggagctgaagggggcacaggagcctggatgagagccaagggaggagctgaaactgggactgaaagcggggcaggagctggagccgacaagggaaccgggcctgaagggggagcagaagctggcacaggcaccaagactgaggccgaaacagaaagggggttcgagtcagagatgagcgtgggcactgacggtggcgctggagccagagccgggacaggtgctaagggaggggaaggagctggaaccgaagtggcaacttggactggaacaagccctgaatgggggactggggcagggacggagaggggaacctggaatgcatctggaacagagtggggcacagaggccgaaccgggagcagggggacagataggggctggcagaggactgaagttagtggtaaccaggggcagggtcccctccacagggactccagttcccagagttgccaaaatgaaagtattcttctctccaacaccttgccgagagtccaaagcctttactccggcgggtgagcagtcaacctgtttgctcatttgggtgttgagtggagtccaggagcagtcggccctgctgttgctggcctcggcgctgtcagatgcgggaagcttgagcccgtctcctgggctgctcaggggcaccaagaggccctcagcctctgccacgttcccagcgtagtccatttttggctggggatcgtcaggcttgtcttctgacttgtgcccaagtttttctgtagcactgccatctgggtctgccccccgggcattgctgccacttccaactgccgtgagctccaccttggaaaaactgctgctgacacaaaactcctgagatccaaagtgctggcagtcgcctgtcgttgactcctcatcagaaagaggtgctcttctctcctcgttgatgccacacatgcgaatccggtcagaactggtccagttgtgcacgccgctgtagagcggtgctgtagagatcatgacagccactcaccaccagataggacctgctgtggccactcccccagtatccccttcttagcgttgccccctcaccgaaataatggtgggggcgacccgagttggactggtggctactttccctccaaggctagccgtccttcgccacgccgaccccctaggagagtcagatggctgaagaagggggaaggcggtgggagtgctggagagtaaaaggactgtggcggggagggtccgcggcccccactacgagagcagaatccagatgctaagaggtgggtggggggtgcggcacaatcgcagactgtgtctttcctcgcttttcccggaatcgccgcccgatcaccgtctaacactcggagttgcttaccactcagtcccctagccccatttgtgcgcgtgaggcggccagagcccgggaagcccgggcacaaactccgcggaagctggccttcgctgccgccgcgccgccgcgggcctccctccctccg

SEQ ID NO: 16871 - RNA, 7649 nt, Homo sapiens
  source 1..7649: mol_type = other RNA
tacgtagatatatatgtatttttttttcttaaaaagggaaaacaactgttcaaaaccaactgggcagtatggtgggggtggggagcagtcctacagaagggggccgagaacttcccccccaggaacaaagaacaaacacaatacaaagaaaataaccaccaatgctcccgcatggctcaggagcctctagagaacagattgtcccatcctcaaactggctttttttttttccttttttttttaatcttttttttttccattttcttttttgttgttgttgttttagcacctgtacaataaaactgtaccatctccaaccagagccggccacggcgaggccctcctgcctttggatggtacatactctacaaggattgttcggaaaaatagcaattggtagaaaaataagagtgggagggacaatgccacagagggggcggggacagggaagcaacccaagctcctctctctctctcactcgacaaacccagcgctggaggcccagaggccagggggaggccaggtagggataccactcagccccaggcccccaggcatgagtggagcaagggctggagaccactttcctgcccttgcctaggaaacagctgacgcctggatttcacatccggcagtgagtcccagagccctctgcagattcccaaggagaatgaggggctgagggaggaggtgggaggagaggaaggaaaggggtgctgtgagtctcagaaggggcagggatgggggtggctgagggctgggaggtgagaggctcagtatcttgagacagggaggccagaacggggtgggagagtggaggcaggaacaaactcgtattgtgcactctgaggggggcagtgaagaaggcgtgaggaggggggccaccctcacccctcagatcccttctccacgctcctttattagagtaacttattaacccctcacctcacaatcctcccctccctgtcaacactaatctcaagatagcggggctgctgcaaagggcgggaatgggtgggtgggggagcaccaaagcctcaggatttacccccaagcccccagccctgggccagcagcaaccagcttcgttagtcacaagtccatgttcccccaccccattccacctcaccccctccccagtgggggaaaaaaacaccagggaatagctttgtcagagctcatcaacaaagaaaaagaaaaggaggtacagaaagtccctcaatacaacaagttgtctcaaatcgtcacagtgatacagacttatcagaaaccaatgaaacaatacaaattaaatactaataaaataaatactacagaagacagaagaacacaggggaatggagttggggggcgctcagagatctgggattttctcatttctcctcgggacaggccaaggccatccagggcccaggtttggtcttggtcatgaacaaggaggccagtccaagggaccccggcgccacctcccaccacccccgggacctcttgtcctcagacatggagttcaactttccacccccatcagcaaccacgataacaatgacgacgacagggagatgagaactaattgtaaccaaaaaaacaaaaacagtccagtcgctaatgctggcattgataaggcggcttcttgttggtccgtattattgcctcattctgcagtctggtgctcggtcggggaaagacaaggaggtgggggaagggcgaactcggaaggagaaagaagaggaggggctgttttcccggtcaactgttgcaagactggaattccacctcggaccctaggagccgaagtaggtctggctcgtaccgcaccagctccacagtctcagaggagcctgggggggatctgtcgtccaagcctccaggcctctcggcaggggtcagcagctgactggaggccacctgcctgtagaactcggccttgggcatggtggtgatttcaaagtgcgggaaccgggcctgaaagatcctcgaggaaagcttcagcctcttcaagacatcggaaaagaggaaccagttgcagggcccgcgggacactgacacttggaggttgtagcaagggagaagaggcttgtctgagagttcaaacatgaaatcatcctcctccatcggatcgtctccttcttgatctgagctcccaggaggattatgtaggaggtcacaggcaaacccgtctttttcctccaacacagaactgctgtaaaaatcccaggatacaccgggatcaccctctgcccggccctgaagatccgagaggtgatcactgagaaagcgcttcatggtgtcgctgctggccagcttcatggctgtctgacccgagtaggtagccagtgtgggatcggccccataggacagcaggagccagatggtctccaggttgtcattgaccaccgcatcatgaactggcctcgtgccgtcctgcgcactgcagttcacgttggccccgtgctccagcaggatgttcaggatgtcggtccagccccgggaacaagcctcatgcagggctgtgtagccagcattgtcacggtgattcacatcttcactgtctttctggaggcagtagagaacaacatccttatagccaagacgcgccgccctctgcaggagggtctcaccagcatttttgttcactatgagccgacgtgcctctggggggatctgccgggctgtaggtgactctgaggcctcctctgagctggcacttcgggacttagagggtgtacatggttctgtgggtttcactggggtgggagatttgggagatcgtgtcttctgctggctccaacgacctttgccctttgcctcttctgagacggttgccatgtgcttggtcttgcactttcgttttcctgatggcttttctgaattttcaaggcaggctggctcttccaggttatttgggaggaaaccgtttggtgaatccgagatcccctggactttgttgggcaagagaaggttcctgttcctgaggcggtgctccaaactttgggaggaggaagtcttctgcttacgggcctttaaatctgctctccctttccgccgctgctcgtcttcttgctctgtcaggtactccccagtctgatattttcggctcttctgccgtcttcgtttcttcctcttcagcaggccctcctcctcttcttcctcctcctcctcattggtgtcccacatttgccgggcagcctctgtcctccagggcatttctcgggctcgccacaggtgccttcggccctggctcagcagagacttgtcctgggcatggtggctgcgatactgggtgtcccgttgggtctttctcacctttcgacgcttagctggggtgggggttacctcctcttcttcttctgtggggaagacttcctggcttcccatgtcactgtctgccatgccagcaaaggagctacagatgcttccagactgactgcgcgtgcgggtgctcagaaccacaggaataaagtcacggaaactgctctttgctttcttttccaaggaaccttcctcgtggctgtcggctcgttttcctggagactgggactccggctttgtcggcttccggtgcttgtgctttcccctgactccattgtgctcttttcctgaatctgaagcccccctggggcttttcttggtggattcctgggggtcactgggcagcttccggcacttgggtctgtgggaactccggaccacggccttggcttgtggctggagctgctgctcttcactgtccttctctttgccgcacttcatcttcttgggcggcagagattccgtcacatcatctggctgccacttgttcttgcaagcaaagacccctacgctttcctgtttcactcgagcctgcccggccttagcccgaacttcagcttggcccctctggggagccactgggaggccatcagcccggaagcaggtggctaaattgaagaccacatcaccatccaccttctccattttcactcgccccagatccacctggcttccaagctgtgggcgctctgtgctggagcccctcctgctgctcggaaccacgtccaatataagttccttggggtggctgtcgtgaggtagcaaaggcagctcaggcatcttaggcaggttctggggggtggccaggaccagctcatgggacatgtaggtggccagcacttggttcttaggcttcgtgtctcctgccagcttcaggccacaagccccctgggggccttccatcttaggagtgctgtcagagcagaggtggctctctgattcctcaggcccctgattcattcgaatgtccccaccgctaggctgaacagacagtgccagggtcccagtctgagggctgagggtcaagaggacaggattgacttgttcttcataaggcttggcagcaatccggcaagttttgttctttgtaacagggtcctgctctggaacgaaggagcccccaggccgtggttgcccctcaggaagtccgtgcacggcttcgctggagctgagagatggcacaccagaaaactccgaaacaacgctggtgggcctgatgggcgccccctgactgggggtcagctgcccggcactggaaatgccaatggaaagcagagacgcctggtggtacggggaccagccaacaggcaggacctgggtgctggtaggtttcccattgactgaacaccggggataaatatttgccggccccgtgggtttccacaaagagagttccttggtttggcaccctggcagcccaggggcaatgcgggctggagtatatcgtttcactgtgcttggctgtccctcagcaccagcctggctgccctttttgccacacgtggcaccagtgcccttaggctctccttgatcaatgatggagatgggctcctgcttggggagatggcgggggtcacggttgaggcccaggttggggtctttgttcagcagcagggatgcaggcactgggttggccactcccacgtaggtgccaggaatggtgctgatcagtgcagttgagttcttcacccaggtgctcgggtccccattcctcacgatctcgggaaagatgacaaagggcgaggaagtggagcccaggcaggaggtgacattgccaccggcagcctgggttgtgcgctgagacctagacaggactgtggagaggagggccttgctgctggtgtgcacgggggtcaacacaggcatggggggtgtcttgcgctggttcggcaatggaagcttctggcggttggacttggaggacagatcaaggggcatctcgctgcactcaggtggagaggccatctctcgttccagctgtggcggtgacttaagaggagagaaggtaacggaagtcccttctgtttgctgctcggtgccactgggcatcttggcggggtgcggtggggctgagctcccactgggggctggcagcagaggctgtggagttggaagcaccttggcagaagcagtaacaagggaggtatctgccaaaggcccagggaccccatcgggtgcaggctgggtggtggtgctaccggatggggaagtgcaggggagcctgttcacctccagagataccagcttggaatccgaagtcagaggccgggccacagaaaatgcatacgggtaagaacggagctcgggggaggctagcacgcctgggagacacctgtcctgcaggtaggacggcaggacagggagcgtaagagtggaggaaacccctagagtggttggcagtgtggccacactgagtggctgcccacagcttggaggcgggatatataccagcggctggctcggggtcagcactgtccctggctgaaaggacagggggactttttgcatagctggtgcctgagctgcaggaaagcacactctactcaaactgaaggaggccgggatgggtgcagaggtgggaatggcagctggcgtggcagcaggcatgggtgtaggggctggagtaaagatgggggctggggtgggtgcaggcaccggtgtaggagcaaaggcggggatgagggtgggggtagaaggtgggccggaagatggggttggagtgggcatgggcacagacggaggggcaggggccgctggaggcgtggatgctggcatgggagccagaaccggagtggggacgggagcgagaaccaaggtcggagctgaagggggcacaggagcctggatgagagccaagggaggagctgaaactgggactgaaagcggggcaggagctggagccgacaagggaaccgggcctgaagggggagcagaagctggcacaggcaccaagactgaggccgaaacagaaagggggttcgagtcagagatgagcgtgggcactgacggtggcgctggagccagagccgggacaggtgctaagggaggggaaggagctggaaccgaagtggcaacttggactggaacaagccctgaatgggggactggggcagggacggagaggggaacctggaatgcatctggaacagagtggggcacagaggccgaaccgggagcagggggacagataggggctggcagaggactgaagttagtggtaaccaggggcagggtcccctccacagggactccagttcccagagttgccaaaatgaaagtattcttctctccaacaccttgccgagagtccaaagcctttactccggcgggtgagcagtcaacctgtttgctcatttgggtgttgagtggagtccaggagcagtcggccctgctgttgctggcctcggcgctgtcagatgcgggaagcttgagcccgtctcctgggctgctcaggggcaccaagaggccctcagcctctgccacgttcccagcgtagtccatttttggctggggatcgtcaggcttgtcttctgacttgtgcccaagtttttctgtagcactgccatctgggtctgccccccgggcattgctgccacttccaactgccgtgagctccaccttggaaaaactgctgctgacacaaaactcctgagatccaaagtgctggcagtcgcctgtcgttgactcctcatcagaaagaggtgctcttctctcctcgttgatgccacacatgcgaatccggtcagaactggtccagttgtgcacgccgctgtagagcggtgctgtagagatcatgacagccactcaccaccagataggacctgctgtggccactcccccccaaagtagtcgcctcaggaggctggacagtcatctcagccgagcggccagggcttgcaatctccctggagttcctctgtgagcgttagcatccagaccaatactacgtccttttcactctcctcattagtgctggaacccatcctttcagggtcgatctgatgtttaggaacatccaaaatccattcagaacaatctactcaaacagcagcaatattaaacagaaccatctaatcaagtaatgccttgaaaagtgatatactctagcacccatagcctacactgcggtgggaaaacttggagaacactcccagtccccacttctcagccatctcagactatctctctatgtccatttaccatgtcacctgcaaaatgggaataaactactagtccctactaaaaatttggaataacatgaaagcacttagaaaaggaccatagactggccggacatggtggctcacgcctgtaatcccagcactttgggaagccaaggc

SEQ ID NO: 16872 - RNA, 7349 nt, Homo sapiens
  source 1..7349: mol_type = other RNA
tacgtagatatatatgtatttttttttcttaaaaagggaaaacaactgttcaaaaccaactgggcagtatggtgggggtggggagcagtcctacagaagggggccgagaacttcccccccaggaacaaagaacaaacacaatacaaagaaaataaccaccaatgctcccgcatggctcaggagcctctagagaacagattgtcccatcctcaaactggctttttttttttccttttttttttaatcttttttttttccattttcttttttgttgttgttgttttagcacctgtacaataaaactgtaccatctccaaccagagccggccacggcgaggccctcctgcctttggatggtacatactctacaaggattgttcggaaaaatagcaattggtagaaaaataagagtgggagggacaatgccacagagggggcggggacagggaagcaacccaagctcctctctctctctcactcgacaaacccagcgctggaggcccagaggccagggggaggccaggtagggataccactcagccccaggcccccaggcatgagtggagcaagggctggagaccactttcctgcccttgcctaggaaacagctgacgcctggatttcacatccggcagtgagtcccagagccctctgcagattcccaaggagaatgaggggctgagggaggaggtgggaggagaggaaggaaaggggtgctgtgagtctcagaaggggcagggatgggggtggctgagggctgggaggtgagaggctcagtatcttgagacagggaggccagaacggggtgggagagtggaggcaggaacaaactcgtattgtgcactctgaggggggcagtgaagaaggcgtgaggaggggggccaccctcacccctcagatcccttctccacgctcctttattagagtaacttattaacccctcacctcacaatcctcccctccctgtcaacactaatctcaagatagcggggctgctgcaaagggcgggaatgggtgggtgggggagcaccaaagcctcaggatttacccccaagcccccagccctgggccagcagcaaccagcttcgttagtcacaagtccatgttcccccaccccattccacctcaccccctccccagtgggggaaaaaaacaccagggaatagctttgtcagagctcatcaacaaagaaaaagaaaaggaggtacagaaagtccctcaatacaacaagttgtctcaaatcgtcacagtgatacagacttatcagaaaccaatgaaacaatacaaattaaatactaataaaataaatactacagaagacagaagaacacaggggaatggagttggggggcgctcagagatctgggattttctcatttctcctcgggacaggccaaggccatccagggcccaggtttggtcttggtcatgaacaaggaggccagtccaagggaccccggcgccacctcccaccacccccgggacctcttgtcctcagacatggagttcaactttccacccccatcagcaaccacgataacaatgacgacgacagggagatgagaactaattgtaaccaaaaaaacaaaaacagtccagtcgctaatgctggcattgataaggcggcttcttgttggtccgtattattgcctcattctgcagtctggtgctcggtcggggaaagacaaggaggtgggggaagggcgaactcggaaggagaaagaagaggaggggctgttttcccggtcaactgttgcaagactggaattccacctcggaccctaggagccgaagtaggtctggctcgtaccgcaccagctccacagtctcagaggagcctgggggggatctgtcgtccaagcctccaggcctctcggcaggggtcagcagctgactggaggccacctgcctgtagaactcggccttgggcatggtggtgatttcaaagtgcgggaaccgggcctgaaagatcctcgaggaaagcttcagcctcttcaagacatcggaaaagaggaaccagttgcagggcccgcgggacactgacacttggaggttgtagcaagggagaagaggcttgtctgagagttcaaacatgaaatcatcctcctccatcggatcgtctccttcttgatctgagctcccaggaggattatgtaggaggtcacaggcaaacccgtctttttcctccaacacagaactgctgtaaaaatcccaggatacaccgggatcaccctctgcccggccctgaagatccgagaggtgatcactgagaaagcgcttcatggtgtcgctgctggccagcttcatggctgtctgacccgagtaggtagccagtgtgggatcggccccataggacagcaggagccagatggtctccaggttgtcattgaccaccgcatcatgaactggcctcgtgccgtcctgcgcactgcagttcacgttggccccgtgctccagcaggatgttcaggatgtcggtccagccccgggaacaagcctcatgcagggctgtgtagccagcattgtcacggtgattcacatcttcactgtctttctggaggcagtagagaacaacatccttatagccaagacgcgccgccctctgcaggagggtctcaccagcatttttgttcactatgagccgacgtgcctctggggggatctgccgggctgtaggtgactctgaggcctcctctgagctggcacttcgggacttagagggtgtacatggttctgtgggtttcactggggtgggagatttgggagatcgtgtcttctgctggctccaacgacctttgccctttgcctcttctgagacggttgccatgtgcttggtcttgcactttcgttttcctgatggcttttctgaattttcaaggcaggctggctcttccaggttatttgggaggaaaccgtttggtgaatccgagatcccctggactttgttgggcaagagaaggttcctgttcctgaggcggtgctccaaactttgggaggaggaagtcttctgcttacgggcctttaaatctgctctccctttccgccgctgctcgtcttcttgctctgtcaggtactccccagtctgatattttcggctcttctgccgtcttcgtttcttcctcttcagcaggccctcctcctcttcttcctcctcctcctcattggtgtcccacatttgccgggcagcctctgtcctccagggcatttctcgggctcgccacaggtgccttcggccctggctcagcagagacttgtcctgggcatggtggctgcgatactgggtgtcccgttgggtctttctcacctttcgacgcttagctggggtgggggttacctcctcttcttcttctgtggggaagacttcctggcttcccatgtcactgtctgccatgccagcaaaggagctacagatgcttccagactgactgcgcgtgcgggtgctcagaaccacaggaataaagtcacggaaactgctctttgctttcttttccaaggaaccttcctcgtggctgtcggctcgttttcctggagactgggactccggctttgtcggcttccggtgcttgtgctttcccctgactccattgtgctcttttcctgaatctgaagcccccctggggcttttcttggtggattcctgggggtcactgggcagcttccggcacttgggtctgtgggaactccggaccacggccttggcttgtggctggagctgctgctcttcactgtccttctctttgccgcacttcatcttcttgggcggcagagattccgtcacatcatctggctgccacttgttcttgcaagcaaagacccctacgctttcctgtttcactcgagcctgcccggccttagcccgaacttcagcttggcccctctggggagccactgggaggccatcagcccggaagcaggtggctaaattgaagaccacatcaccatccaccttctccattttcactcgccccagatccacctggcttccaagctgtgggcgctctgtgctggagcccctcctgctgctcggaaccacgtccaatataagttccttggggtggctgtcgtgaggtagcaaaggcagctcaggcatcttaggcaggttctggggggtggccaggaccagctcatgggacatgtaggtggccagcacttggttcttaggcttcgtgtctcctgccagcttcaggccacaagccccctgggggccttccatcttaggagtgctgtcagagcagaggtggctctctgattcctcaggcccctgattcattcgaatgtccccaccgctaggctgaacagacagtgccagggtcccagtctgagggctgagggtcaagaggacaggattgacttgttcttcataaggcttggcagcaatccggcaagttttgttctttgtaacagggtcctgctctggaacgaaggagcccccaggccgtggttgcccctcaggaagtccgtgcacggcttcgctggagctgagagatggcacaccagaaaactccgaaacaacgctggtgggcctgatgggcgccccctgactgggggtcagctgcccggcactggaaatgccaatggaaagcagagacgcctggtggtacggggaccagccaacaggcaggacctgggtgctggtaggtttcccattgactgaacaccggggataaatatttgccggccccgtgggtttccacaaagagagttccttggtttggcaccctggcagcccaggggcaatgcgggctggagtatatcgtttcactgtgcttggctgtccctcagcaccagcctggctgccctttttgccacacgtggcaccagtgcccttaggctctccttgatcaatgatggagatgggctcctgcttggggagatggcgggggtcacggttgaggcccaggttggggtctttgttcagcagcagggatgcaggcactgggttggccactcccacgtaggtgccaggaatggtgctgatcagtgcagttgagttcttcacccaggtgctcgggtccccattcctcacgatctcgggaaagatgacaaagggcgaggaagtggagcccaggcaggaggtgacattgccaccggcagcctgggttgtgcgctgagacctagacaggactgtggagaggagggccttgctgctggtgtgcacgggggtcaacacaggcatggggggtgtcttgcgctggttcggcaatggaagcttctggcggttggacttggaggacagatcaaggggcatctcgctgcactcaggtggagaggccatctctcgttccagctgtggcggtgacttaagaggagagaaggtaacggaagtcccttctgtttgctgctcggtgccactgggcatcttggcggggtgcggtggggctgagctcccactgggggctggcagcagaggctgtggagttggaagcaccttggcagaagcagtaacaagggaggtatctgccaaaggcccagggaccccatcgggtgcaggctgggtggtggtgctaccggatggggaagtgcaggggagcctgttcacctccagagataccagcttggaatccgaagtcagaggccgggccacagaaaatgcatacgggtaagaacggagctcgggggaggctagcacgcctgggagacacctgtcctgcaggtaggacggcaggacagggagcgtaagagtggaggaaacccctagagtggttggcagtgtggccacactgagtggctgcccacagcttggaggcgggatatataccagcggctggctcggggtcagcactgtccctggctgaaaggacagggggactttttgcatagctggtgcctgagctgcaggaaagcacactctactcaaactgaaggaggccgggatgggtgcagaggtgggaatggcagctggcgtggcagcaggcatgggtgtaggggctggagtaaagatgggggctggggtgggtgcaggcaccggtgtaggagcaaaggcggggatgagggtgggggtagaaggtgggccggaagatggggttggagtgggcatgggcacagacggaggggcaggggccgctggaggcgtggatgctggcatgggagccagaaccggagtggggacgggagcgagaaccaaggtcggagctgaagggggcacaggagcctggatgagagccaagggaggagctgaaactgggactgaaagcggggcaggagctggagccgacaagggaaccgggcctgaagggggagcagaagctggcacaggcaccaagactgaggccgaaacagaaagggggttcgagtcagagatgagcgtgggcactgacggtggcgctggagccagagccgggacaggtgctaagggaggggaaggagctggaaccgaagtggcaacttggactggaacaagccctgaatgggggactggggcagggacggagaggggaacctggaatgcatctggaacagagtggggcacagaggccgaaccgggagcagggggacagataggggctggcagaggactgaagttagtggtaaccaggggcagggtcccctccacagggactccagttcccagagttgccaaaatgaaagtattcttctctccaacaccttgccgagagtccaaagcctttactccggcgggtgagcagtcaacctgtttgctcatttgggtgttgagtggagtccaggagcagtcggccctgctgttgctggcctcggcgctgtcagatgcgggaagcttgagcccgtctcctgggctgctcaggggcaccaagaggccctcagcctctgccacgttcccagcgtagtccatttttggctggggatcgtcaggcttgtcttctgacttgtgcccaagtttttctgtagcactgccatctgggtctgccccccgggcattgctgccacttccaactgccgtgagctccaccttggaaaaactgctgctgacacaaaactcctgagatccaaagtgctggcagtcgcctgtcgttgactcctcatcagaaagaggtgctcttctctcctcgttgatgccacacatgcgaatccggtcagaactggtccagttgtgcacgccgctgtagagcggtgctgtagagatcatgacagccactcaccaccagataggacctgctgtggccactcccccgaaataatggtgggggcgacccgagttggactggtggctactttccctccaaggctagccgtccttcgccacgccgacccactcagtcccctagccccatttgtgcgcgtgaggcggccagagcccgggaagcccgggcacaaactccgcggaagctggccttcgctgccgccgcgccgccgcgggcctccctccctccg

SEQ ID NO: 16873 - RNA, 7583 nt, Homo sapiens
  source 1..7583: mol_type = other RNA
tacgtagatatatatgtatttttttttcttaaaaagggaaaacaactgttcaaaaccaactgggcagtatggtgggggtggggagcagtcctacagaagggggccgagaacttcccccccaggaacaaagaacaaacacaatacaaagaaaataaccaccaatgctcccgcatggctcaggagcctctagagaacagattgtcccatcctcaaactggctttttttttttccttttttttttaatcttttttttttccattttcttttttgttgttgttgttttagcacctgtacaataaaactgtaccatctccaaccagagccggccacggcgaggccctcctgcctttggatggtacatactctacaaggattgttcggaaaaatagcaattggtagaaaaataagagtgggagggacaatgccacagagggggcggggacagggaagcaacccaagctcctctctctctctcactcgacaaacccagcgctggaggcccagaggccagggggaggccaggtagggataccactcagccccaggcccccaggcatgagtggagcaagggctggagaccactttcctgcccttgcctaggaaacagctgacgcctggatttcacatccggcagtgagtcccagagccctctgcagattcccaaggagaatgaggggctgagggaggaggtgggaggagaggaaggaaaggggtgctgtgagtctcagaaggggcagggatgggggtggctgagggctgggaggtgagaggctcagtatcttgagacagggaggccagaacggggtgggagagtggaggcaggaacaaactcgtattgtgcactctgaggggggcagtgaagaaggcgtgaggaggggggccaccctcacccctcagatcccttctccacgctcctttattagagtaacttattaacccctcacctcacaatcctcccctccctgtcaacactaatctcaagatagcggggctgctgcaaagggcgggaatgggtgggtgggggagcaccaaagcctcaggatttacccccaagcccccagccctgggccagcagcaaccagcttcgttagtcacaagtccatgttcccccaccccattccacctcaccccctccccagtgggggaaaaaaacaccagggaatagctttgtcagagctcatcaacaaagaaaaagaaaaggaggtacagaaagtccctcaatacaacaagttgtctcaaatcgtcacagtgatacagacttatcagaaaccaatgaaacaatacaaattaaatactaataaaataaatactacagaagacagaagaacacaggggaatggagttggggggcgctcagagatctgggattttctcatttctcctcgggacaggccaaggccatccagggcccaggtttggtcttggtcatgaacaaggaggccagtccaagggaccccggcgccacctcccaccacccccgggacctcttgtcctcagacatggagttcaactttccacccccatcagcaaccacgataacaatgacgacgacagggagatgagaactaattgtaaccaaaaaaacaaaaacagtccagtcgctaatgctggcattgataaggcggcttcttgttggtccgtattattgcctcattctgcagtctggtgctcggtcggggaaagacaaggaggtgggggaagggcgaactcggaaggagaaagaagaggaggggctgttttcccggtcaactgttgcaagactggaattccacctcggaccctaggagccgaagtaggtctggctcgtaccgcaccagctccacagtctcagaggagcctgggggggatctgtcgtccaagcctccaggcctctcggcaggggtcagcagctgactggaggccacctgcctgtagaactcggccttgggcatggtggtgatttcaaagtgcgggaaccgggcctgaaagatcctcgaggaaagcttcagcctcttcaagacatcggaaaagaggaaccagttgcagggcccgcgggacactgacacttggaggttgtagcaagggagaagaggcttgtctgagagttcaaacatgaaatcatcctcctccatcggatcgtctccttcttgatctgagctcccaggaggattatgtaggaggtcacaggcaaacccgtctttttcctccaacacagaactgctgtaaaaatcccaggatacaccgggatcaccctctgcccggccctgaagatccgagaggtgatcactgagaaagcgcttcatggtgtcgctgctggccagcttcatggctgtctgacccgagtaggtagccagtgtgggatcggccccataggacagcaggagccagatggtctccaggttgtcattgaccaccgcatcatgaactggcctcgtgccgtcctgcgcactgcagttcacgttggccccgtgctccagcaggatgttcaggatgtcggtccagccccgggaacaagcctcatgcagggctgtgtagccagcattgtcacggtgattcacatcttcactgtctttctggaggcagtagagaacaacatccttatagccaagacgcgccgccctctgcaggagggtctcaccagcatttttgttcactatgagccgacgtgcctctggggggatctgccgggctgtaggtgactctgaggcctcctctgagctggcacttcgggacttagagggtgtacatggttctgtgggtttcactggggtgggagatttgggagatcgtgtcttctgctggctccaacgacctttgccctttgcctcttctgagacggttgccatgtgcttggtcttgcactttcgttttcctgatggcttttctgaattttcaaggcaggctggctcttccaggttatttgggaggaaaccgtttggtgaatccgagatcccctggactttgttgggcaagagaaggttcctgttcctgaggcggtgctccaaactttgggaggaggaagtcttctgcttacgggcctttaaatctgctctccctttccgccgctgctcgtcttcttgctctgtcaggtactccccagtctgatattttcggctcttctgccgtcttcgtttcttcctcttcagcaggccctcctcctcttcttcctcctcctcctcattggtgtcccacatttgccgggcagcctctgtcctccagggcatttctcgggctcgccacaggtgccttcggccctggctcagcagagacttgtcctgggcatggtggctgcgatactgggtgtcccgttgggtctttctcacctttcgacgcttagctggggtgggggttacctcctcttcttcttctgtggggaagacttcctggcttcccatgtcactgtctgccatgccagcaaaggagctacagatgcttccagactgactgcgcgtgcgggtgctcagaaccacaggaataaagtcacggaaactgctctttgctttcttttccaaggaaccttcctcgtggctgtcggctcgttttcctggagactgggactccggctttgtcggcttccggtgcttgtgctttcccctgactccattgtgctcttttcctgaatctgaagcccccctggggcttttcttggtggattcctgggggtcactgggcagcttccggcacttgggtctgtgggaactccggaccacggccttggcttgtggctggagctgctgctcttcactgtccttctctttgccgcacttcatcttcttgggcggcagagattccgtcacatcatctggctgccacttgttcttgcaagcaaagacccctacgctttcctgtttcactcgagcctgcccggccttagcccgaacttcagcttggcccctctggggagccactgggaggccatcagcccggaagcaggtggctaaattgaagaccacatcaccatccaccttctccattttcactcgccccagatccacctggcttccaagctgtgggcgctctgtgctggagcccctcctgctgctcggaaccacgtccaatataagttccttggggtggctgtcgtgaggtagcaaaggcagctcaggcatcttaggcaggttctggggggtggccaggaccagctcatgggacatgtaggtggccagcacttggttcttaggcttcgtgtctcctgccagcttcaggccacaagccccctgggggccttccatcttaggagtgctgtcagagcagaggtggctctctgattcctcaggcccctgattcattcgaatgtccccaccgctaggctgaacagacagtgccagggtcccagtctgagggctgagggtcaagaggacaggattgacttgttcttcataaggcttggcagcaatccggcaagttttgttctttgtaacagggtcctgctctggaacgaaggagcccccaggccgtggttgcccctcaggaagtccgtgcacggcttcgctggagctgagagatggcacaccagaaaactccgaaacaacgctggtgggcctgatgggcgccccctgactgggggtcagctgcccggcactggaaatgccaatggaaagcagagacgcctggtggtacggggaccagccaacaggcaggacctgggtgctggtaggtttcccattgactgaacaccggggataaatatttgccggccccgtgggtttccacaaagagagttccttggtttggcaccctggcagcccaggggcaatgcgggctggagtatatcgtttcactgtgcttggctgtccctcagcaccagcctggctgccctttttgccacacgtggcaccagtgcccttaggctctccttgatcaatgatggagatgggctcctgcttggggagatggcgggggtcacggttgaggcccaggttggggtctttgttcagcagcagggatgcaggcactgggttggccactcccacgtaggtgccaggaatggtgctgatcagtgcagttgagttcttcacccaggtgctcgggtccccattcctcacgatctcgggaaagatgacaaagggcgaggaagtggagcccaggcaggaggtgacattgccaccggcagcctgggttgtgcgctgagacctagacaggactgtggagaggagggccttgctgctggtgtgcacgggggtcaacacaggcatggggggtgtcttgcgctggttcggcaatggaagcttctggcggttggacttggaggacagatcaaggggcatctcgctgcactcaggtggagaggccatctctcgttccagctgtggcggtgacttaagaggagagaaggtaacggaagtcccttctgtttgctgctcggtgccactgggcatcttggcggggtgcggtggggctgagctcccactgggggctggcagcagaggctgtggagttggaagcaccttggcagaagcagtaacaagggaggtatctgccaaaggcccagggaccccatcgggtgcaggctgggtggtggtgctaccggatggggaagtgcaggggagcctgttcacctccagagataccagcttggaatccgaagtcagaggccgggccacagaaaatgcatacgggtaagaacggagctcgggggaggctagcacgcctgggagacacctgtcctgcaggtaggacggcaggacagggagcgtaagagtggaggaaacccctagagtggttggcagtgtggccacactgagtggctgcccacagcttggaggcgggatatataccagcggctggctcggggtcagcactgtccctggctgaaaggacagggggactttttgcatagctggtgcctgagctgcaggaaagcacactctactcaaactgaaggaggccgggatgggtgcagaggtgggaatggcagctggcgtggcagcaggcatgggtgtaggggctggagtaaagatgggggctggggtgggtgcaggcaccggtgtaggagcaaaggcggggatgagggtgggggtagaaggtgggccggaagatggggttggagtgggcatgggcacagacggaggggcaggggccgctggaggcgtggatgctggcatgggagccagaaccggagtggggacgggagcgagaaccaaggtcggagctgaagggggcacaggagcctggatgagagccaagggaggagctgaaactgggactgaaagcggggcaggagctggagccgacaagggaaccgggcctgaagggggagcagaagctggcacaggcaccaagactgaggccgaaacagaaagggggttcgagtcagagatgagcgtgggcactgacggtggcgctggagccagagccgggacaggtgctaagggaggggaaggagctggaaccgaagtggcaacttggactggaacaagccctgaatgggggactggggcagggacggagaggggaacctggaatgcatctggaacagagtggggcacagaggccgaaccgggagcagggggacagataggggctggcagaggactgaagttagtggtaaccaggggcagggtcccctccacagggactccagttcccagagttgccaaaatgaaagtattcttctctccaacaccttgccgagagtccaaagcctttactccggcgggtgagcagtcaacctgtttgctcatttgggtgttgagtggagtccaggagcagtcggccctgctgttgctggcctcggcgctgtcagatgcgggaagcttgagcccgtctcctgggctgctcaggggcaccaagaggccctcagcctctgccacgttcccagcgtagtccatttttggctggggatcgtcaggcttgtcttctgacttgtgcccaagtttttctgtagcactgccatctgggtctgccccccgggcattgctgccacttccaactgccgtgagctccaccttggaaaaactgctgctgacacaaaactcctgagatccaaagtgctggcagtcgcctgtcgttgactcctcatcagaaagaggtgctcttctctcctcgttgatgccacacatgcgaatccggtcagaactggtccagttgtgcacgccgctgtagagcggtgctgtagagatcatgacagccactcaccaccagataggacctgctgtggccactcccccgaaataatggtgggggcgacccgagttggactggtggctactttccctccaaggctagccgtccttcgccacgccgaccccctaggagagtcagatggctgaagaagggggaaggcggtgggagtgctggagagtaaaaggactgtggcggggagggtccgcggcccccactacgagagcagaatccagatgctaagaggtgggtggggggtgcggcacaatcgcagactgtgtctttcctcgcttttcccggaatcgccgcccgatcaccgtctaacactcggagttgcttaccactcagtcccctagccccatttgtgcgcgtgaggcggccagagcccgggaagcccgggcacaaactccgcggaagctggccttcgctgccgccgcgccgccgcgggcctccctccctccgctcgcggccccgccgatct

SEQ ID NO: 16874 - RNA, 7332 nt, Homo sapiens
  source 1..7332: mol_type = other RNA
tacgtagatatatatgtatttttttttcttaaaaagggaaaacaactgttcaaaaccaactgggcagtatggtgggggtggggagcagtcctacagaagggggccgagaacttcccccccaggaacaaagaacaaacacaatacaaagaaaataaccaccaatgctcccgcatggctcaggagcctctagagaacagattgtcccatcctcaaactggctttttttttttccttttttttttaatcttttttttttccattttcttttttgttgttgttgttttagcacctgtacaataaaactgtaccatctccaaccagagccggccacggcgaggccctcctgcctttggatggtacatactctacaaggattgttcggaaaaatagcaattggtagaaaaataagagtgggagggacaatgccacagagggggcggggacagggaagcaacccaagctcctctctctctctcactcgacaaacccagcgctggaggcccagaggccagggggaggccaggtagggataccactcagccccaggcccccaggcatgagtggagcaagggctggagaccactttcctgcccttgcctaggaaacagctgacgcctggatttcacatccggcagtgagtcccagagccctctgcagattcccaaggagaatgaggggctgagggaggaggtgggaggagaggaaggaaaggggtgctgtgagtctcagaaggggcagggatgggggtggctgagggctgggaggtgagaggctcagtatcttgagacagggaggccagaacggggtgggagagtggaggcaggaacaaactcgtattgtgcactctgaggggggcagtgaagaaggcgtgaggaggggggccaccctcacccctcagatcccttctccacgctcctttattagagtaacttattaacccctcacctcacaatcctcccctccctgtcaacactaatctcaagatagcggggctgctgcaaagggcgggaatgggtgggtgggggagcaccaaagcctcaggatttacccccaagcccccagccctgggccagcagcaaccagcttcgttagtcacaagtccatgttcccccaccccattccacctcaccccctccccagtgggggaaaaaaacaccagggaatagctttgtcagagctcatcaacaaagaaaaagaaaaggaggtacagaaagtccctcaatacaacaagttgtctcaaatcgtcacagtgatacagacttatcagaaaccaatgaaacaatacaaattaaatactaataaaataaatactacagaagacagaagaacacaggggaatggagttggggggcgctcagagatctgggattttctcatttctcctcgggacaggccaaggccatccagggcccaggtttggtcttggtcatgaacaaggaggccagtccaagggaccccggcgccacctcccaccacccccgggacctcttgtcctcagacatggagttcaactttccacccccatcagcaaccacgataacaatgacgacgacagggagatgagaactaattgtaaccaaaaaaacaaaaacagtccagtcgctaatgctggcattgataaggcggcttcttgttggtccgtattattgcctcattctgcagtctggtgctcggtcggggaaagacaaggaggtgggggaagggcgaactcggaaggagaaagaagaggaggggctgttttcccggtcaactgttgcaagactggaattccacctcggaccctaggagccgaagtaggtctggctcgtaccgcaccagctccacagtctcagaggagcctgggggggatctgtcgtccaagcctccaggcctctcggcaggggtcagcagctgactggaggccacctgcctgtagaactcggccttgggcatggtggtgatttcaaagtgcgggaaccgggcctgaaagatcctcgaggaaagcttcagcctcttcaagacatcggaaaagaggaaccagttgcagggcccgcgggacactgacacttggaggttgtagcaagggagaagaggcttgtctgagagttcaaacatgaaatcatcctcctccatcggatcgtctccttcttgatctgagctcccaggaggattatgtaggaggtcacaggcaaacccgtctttttcctccaacacagaactgctgtaaaaatcccaggatacaccgggatcaccctctgcccggccctgaagatccgagaggtgatcactgagaaagcgcttcatggtgtcgctgctggccagcttcatggctgtctgacccgagtaggtagccagtgtgggatcggccccataggacagcaggagccagatggtctccaggttgtcattgaccaccgcatcatgaactggcctcgtgccgtcctgcgcactgcagttcacgttggccccgtgctccagcaggatgttcaggatgtcggtccagccccgggaacaagcctcatgcagggctgtgtagccagcattgtcacggtgattcacatcttcactgtctttctggaggcagtagagaacaacatccttatagccaagacgcgccgccctctgcaggagggtctcaccagcatttttgttcactatgagccgacgtgcctctggggggatctgccgggctgtaggtgactctgaggcctcctctgagctggcacttcgggacttagagggtgtacatggttctgtgggtttcactggggtgggagatttgggagatcgtgtcttctgctggctccaacgacctttgccctttgcctcttctgagacggttgccatgtgcttggtcttgcactttcgttttcctgatggcttttctgaattttcaaggcaggctggctcttccaggttatttgggaggaaaccgtttggtgaatccgagatcccctggactttgttgggcaagagaaggttcctgttcctgaggcggtgctccaaactttgggaggaggaagtcttctgcttacgggcctttaaatctgctctccctttccgccgctgctcgtcttcttgctctgtcaggtactccccagtctgatattttcggctcttctgccgtcttcgtttcttcctcttcagcaggccctcctcctcttcttcctcctcctcctcattggtgtcccacatttgccgggcagcctctgtcctccagggcatttctcgggctcgccacaggtgccttcggccctggctcagcagagacttgtcctgggcatggtggctgcgatactgggtgtcccgttgggtctttctcacctttcgacgcttagctggggtgggggttacctcctcttcttcttctgtggggaagacttcctggcttcccatgtcactgtctgccatgccagcaaaggagctacagatgcttccagactgactgcgcgtgcgggtgctcagaaccacaggaataaagtcacggaaactgctctttgctttcttttccaaggaaccttcctcgtggctgtcggctcgttttcctggagactgggactccggctttgtcggcttccggtgcttgtgctttcccctgactccattgtgctcttttcctgaatctgaagcccccctggggcttttcttggtggattcctgggggtcactgggcagcttccggcacttgggtctgtgggaactccggaccacggccttggcttgtggctggagctgctgctcttcactgtccttctctttgccgcacttcatcttcttgggcggcagagattccgtcacatcatctggctgccacttgttcttgcaagcaaagacccctacgctttcctgtttcactcgagcctgcccggccttagcccgaacttcagcttggcccctctggggagccactgggaggccatcagcccggaagcaggtggctaaattgaagaccacatcaccatccaccttctccattttcactcgccccagatccacctggcttccaagctgtgggcgctctgtgctggagcccctcctgctgctcggaaccacgtccaatataagttccttggggtggctgtcgtgaggtagcaaaggcagctcaggcatcttaggcaggttctggggggtggccaggaccagctcatgggacatgtaggtggccagcacttggttcttaggcttcgtgtctcctgccagcttcaggccacaagccccctgggggccttccatcttaggagtgctgtcagagcagaggtggctctctgattcctcaggcccctgattcattcgaatgtccccaccgctaggctgaacagacagtgccagggtcccagtctgagggctgagggtcaagaggacaggattgacttgttcttcataaggcttggcagcaatccggcaagttttgttctttgtaacagggtcctgctctggaacgaaggagcccccaggccgtggttgcccctcaggaagtccgtgcacggcttcgctggagctgagagatggcacaccagaaaactccgaaacaacgctggtgggcctgatgggcgccccctgactgggggtcagctgcccggcactggaaatgccaatggaaagcagagacgcctggtggtacggggaccagccaacaggcaggacctgggtgctggtaggtttcccattgactgaacaccggggataaatatttgccggccccgtgggtttccacaaagagagttccttggtttggcaccctggcagcccaggggcaatgcgggctggagtatatcgtttcactgtgcttggctgtccctcagcaccagcctggctgccctttttgccacacgtggcaccagtgcccttaggctctccttgatcaatgatggagatgggctcctgcttggggagatggcgggggtcacggttgaggcccaggttggggtctttgttcagcagcagggatgcaggcactgggttggccactcccacgtaggtgccaggaatggtgctgatcagtgcagttgagttcttcacccaggtgctcgggtccccattcctcacgatctcgggaaagatgacaaagggcgaggaagtggagcccaggcaggaggtgacattgccaccggcagcctgggttgtgcgctgagacctagacaggactgtggagaggagggccttgctgctggtgtgcacgggggtcaacacaggcatggggggtgtcttgcgctggttcggcaatggaagcttctggcggttggacttggaggacagatcaaggggcatctcgctgcactcaggtggagaggccatctctcgttccagctgtggcggtgacttaagaggagagaaggtaacggaagtcccttctgtttgctgctcggtgccactgggcatcttggcggggtgcggtggggctgagctcccactgggggctggcagcagaggctgtggagttggaagcaccttggcagaagcagtaacaagggaggtatctgccaaaggcccagggaccccatcgggtgcaggctgggtggtggtgctaccggatggggaagtgcaggggagcctgttcacctccagagataccagcttggaatccgaagtcagaggccgggccacagaaaatgcatacgggtaagaacggagctcgggggaggctagcacgcctgggagacacctgtcctgcaggtaggacggcaggacagggagcgtaagagtggaggaaacccctagagtggttggcagtgtggccacactgagtggctgcccacagcttggaggcgggatatataccagcggctggctcggggtcagcactgtccctggctgaaaggacagggggactttttgcatagctggtgcctgagctgcaggaaagcacactctactcaaactgaaggaggccgggatgggtgcagaggtgggaatggcagctggcgtggcagcaggcatgggtgtaggggctggagtaaagatgggggctggggtgggtgcaggcaccggtgtaggagcaaaggcggggatgagggtgggggtagaaggtgggccggaagatggggttggagtgggcatgggcacagacggaggggcaggggccgctggaggcgtggatgctggcatgggagccagaaccggagtggggacgggagcgagaaccaaggtcggagctgaagggggcacaggagcctggatgagagccaagggaggagctgaaactgggactgaaagcggggcaggagctggagccgacaagggaaccgggcctgaagggggagcagaagctggcacaggcaccaagactgaggccgaaacagaaagggggttcgagtcagagatgagcgtgggcactgacggtggcgctggagccagagccgggacaggtgctaagggaggggaaggagctggaaccgaagtggcaacttggactggaacaagccctgaatgggggactggggcagggacggagaggggaacctggaatgcatctggaacagagtggggcacagaggccgaaccgggagcagggggacagataggggctggcagaggactgaagttagtggtaaccaggggcagggtcccctccacagggactccagttcccagagttgccaaaatgaaagtattcttctctccaacaccttgccgagagtccaaagcctttactccggcgggtgagcagtcaacctgtttgctcatttgggtgttgagtggagtccaggagcagtcggccctgctgttgctggcctcggcgctgtcagatgcgggaagcttgagcccgtctcctgggctgctcaggggcaccaagaggccctcagcctctgccacgttcccagcgtagtccatttttggctggggatcgtcaggcttgtcttctgacttgtgcccaagtttttctgtagcactgccatctgggtctgccccccgggcattgctgccacttccaactgccgtgagctccaccttggaaaaactgctgctgacacaaaactcctgagatccaaagtgctggcagtcgcctgtcgttgactcctcatcagaaagaggtgctcttctctcctcgttgatgccacacatgcgaatccggtcagaactggtccagttgtgcacgccgctgtagagcggtgctgtagagatcatgacagccactcaccaccagataggacctgctgtggccactcccccgaaataatggtgggggcgacccgagttggactggtggctactttccctccaaggctagccgtccttcgccacgccgaccctgggcagagcccccggccgctgtcgcaactttgctcttctccacgccgccggggaagcgggcgaagcgggaggagggaggtggcggggggtgctgggatcagg

SEQ ID NO: 16875 - RNA, 7276 nt, Homo sapiens
  source 1..7276: mol_type = other RNA
tacgtagatatatatgtatttttttttcttaaaaagggaaaacaactgttcaaaaccaactgggcagtatggtgggggtggggagcagtcctacagaagggggccgagaacttcccccccaggaacaaagaacaaacacaatacaaagaaaataaccaccaatgctcccgcatggctcaggagcctctagagaacagattgtcccatcctcaaactggctttttttttttccttttttttttaatcttttttttttccattttcttttttgttgttgttgttttagcacctgtacaataaaactgtaccatctccaaccagagccggccacggcgaggccctcctgcctttggatggtacatactctacaaggattgttcggaaaaatagcaattggtagaaaaataagagtgggagggacaatgccacagagggggcggggacagggaagcaacccaagctcctctctctctctcactcgacaaacccagcgctggaggcccagaggccagggggaggccaggtagggataccactcagccccaggcccccaggcatgagtggagcaagggctggagaccactttcctgcccttgcctaggaaacagctgacgcctggatttcacatccggcagtgagtcccagagccctctgcagattcccaaggagaatgaggggctgagggaggaggtgggaggagaggaaggaaaggggtgctgtgagtctcagaaggggcagggatgggggtggctgagggctgggaggtgagaggctcagtatcttgagacagggaggccagaacggggtgggagagtggaggcaggaacaaactcgtattgtgcactctgaggggggcagtgaagaaggcgtgaggaggggggccaccctcacccctcagatcccttctccacgctcctttattagagtaacttattaacccctcacctcacaatcctcccctccctgtcaacactaatctcaagatagcggggctgctgcaaagggcgggaatgggtgggtgggggagcaccaaagcctcaggatttacccccaagcccccagccctgggccagcagcaaccagcttcgttagtcacaagtccatgttcccccaccccattccacctcaccccctccccagtgggggaaaaaaacaccagggaatagctttgtcagagctcatcaacaaagaaaaagaaaaggaggtacagaaagtccctcaatacaacaagttgtctcaaatcgtcacagtgatacagacttatcagaaaccaatgaaacaatacaaattaaatactaataaaataaatactacagaagacagaagaacacaggggaatggagttggggggcgctcagagatctgggattttctcatttctcctcgggacaggccaaggccatccagggcccaggtttggtcttggtcatgaacaaggaggccagtccaagggaccccggcgccacctcccaccacccccgggacctcttgtcctcagacatggagttcaactttccacccccatcagcaaccacgataacaatgacgacgacagggagatgagaactaattgtaaccaaaaaaacaaaaacagtccagtcgctaatgctggcattgataaggcggcttcttgttggtccgtattattgcctcattctgcagtctggtgctcggtcggggaaagacaaggaggtgggggaagggcgaactcggaaggagaaagaagaggaggggctgttttcccggtcaactgttgcaagactggaattccacctcggaccctaggagccgaagtaggtctggctcgtaccgcaccagctccacagtctcagaggagcctgggggggatctgtcgtccaagcctccaggcctctcggcaggggtcagcagctgactggaggccacctgcctgtagaactcggccttgggcatggtggtgatttcaaagtgcgggaaccgggcctgaaagatcctcgaggaaagcttcagcctcttcaagacatcggaaaagaggaaccagttgcagggcccgcgggacactgacacttggaggttgtagcaagggagaagaggcttgtctgagagttcaaacatgaaatcatcctcctccatcggatcgtctccttcttgatctgagctcccaggaggattatgtaggaggtcacaggcaaacccgtctttttcctccaacacagaactgctgtaaaaatcccaggatacaccgggatcaccctctgcccggccctgaagatccgagaggtgatcactgagaaagcgcttcatggtgtcgctgctggccagcttcatggctgtctgacccgagtaggtagccagtgtgggatcggccccataggacagcaggagccagatggtctccaggttgtcattgaccaccgcatcatgaactggcctcgtgccgtcctgcgcactgcagttcacgttggccccgtgctccagcaggatgttcaggatgtcggtccagccccgggaacaagcctcatgcagggctgtgtagccagcattgtcacggtgattcacatcttcactgtctttctggaggcagtagagaacaacatccttatagccaagacgcgccgccctctgcaggagggtctcaccagcatttttgttcactatgagccgacgtgcctctggggggatctgccgggctgtaggtgactctgaggcctcctctgagctggcacttcgggacttagagggtgtacatggttctgtgggtttcactggggtgggagatttgggagatcgtgtcttctgctggctccaacgacctttgccctttgcctcttctgagacggttgccatgtgcttggtcttgcactttcgttttcctgatggcttttctgaattttcaaggcaggctggctcttccaggttatttgggaggaaaccgtttggtgaatccgagatcccctggactttgttgggcaagagaaggttcctgttcctgaggcggtgctccaaactttgggaggaggaagtcttctgcttacgggcctttaaatctgctctccctttccgccgctgctcgtcttcttgctctgtcaggtactccccagtctgatattttcggctcttctgccgtcttcgtttcttcctcttcagcaggccctcctcctcttcttcctcctcctcctcattggtgtcccacatttgccgggcagcctctgtcctccagggcatttctcgggctcgccacaggtgccttcggccctggctcagcagagacttgtcctgggcatggtggctgcgatactgggtgtcccgttgggtctttctcacctttcgacgcttagctggggtgggggttacctcctcttcttcttctgtggggaagacttcctggcttcccatgtcactgtctgccatgccagcaaaggagctacagatgcttccagactgactgcgcgtgcgggtgctcagaaccacaggaataaagtcacggaaactgctctttgctttcttttccaaggaaccttcctcgtggctgtcggctcgttttcctggagactgggactccggctttgtcggcttccggtgcttgtgctttcccctgactccattgtgctcttttcctgaatctgaagcccccctggggcttttcttggtggattcctgggggtcactgggcagcttccggcacttgggtctgtgggaactccggaccacggccttggcttgtggctggagctgctgctcttcactgtccttctctttgccgcacttcatcttcttgggcggcagagattccgtcacatcatctggctgccacttgttcttgcaagcaaagacccctacgctttcctgtttcactcgagcctgcccggccttagcccgaacttcagcttggcccctctggggagccactgggaggccatcagcccggaagcaggtggctaaattgaagaccacatcaccatccaccttctccattttcactcgccccagatccacctggcttccaagctgtgggcgctctgtgctggagcccctcctgctgctcggaaccacgtccaatataagttccttggggtggctgtcgtgaggtagcaaaggcagctcaggcatcttaggcaggttctggggggtggccaggaccagctcatgggacatgtaggtggccagcacttggttcttaggcttcgtgtctcctgccagcttcaggccacaagccccctgggggccttccatcttaggagtgctgtcagagcagaggtggctctctgattcctcaggcccctgattcattcgaatgtccccaccgctaggctgaacagacagtgccagggtcccagtctgagggctgagggtcaagaggacaggattgacttgttcttcataaggcttggcagcaatccggcaagttttgttctttgtaacagggtcctgctctggaacgaaggagcccccaggccgtggttgcccctcaggaagtccgtgcacggcttcgctggagctgagagatggcacaccagaaaactccgaaacaacgctggtgggcctgatgggcgccccctgactgggggtcagctgcccggcactggaaatgccaatggaaagcagagacgcctggtggtacggggaccagccaacaggcaggacctgggtgctggtaggtttcccattgactgaacaccggggataaatatttgccggccccgtgggtttccacaaagagagttccttggtttggcaccctggcagcccaggggcaatgcgggctggagtatatcgtttcactgtgcttggctgtccctcagcaccagcctggctgccctttttgccacacgtggcaccagtgcccttaggctctccttgatcaatgatggagatgggctcctgcttggggagatggcgggggtcacggttgaggcccaggttggggtctttgttcagcagcagggatgcaggcactgggttggccactcccacgtaggtgccaggaatggtgctgatcagtgcagttgagttcttcacccaggtgctcgggtccccattcctcacgatctcgggaaagatgacaaagggcgaggaagtggagcccaggcaggaggtgacattgccaccggcagcctgggttgtgcgctgagacctagacaggactgtggagaggagggccttgctgctggtgtgcacgggggtcaacacaggcatggggggtgtcttgcgctggttcggcaatggaagcttctggcggttggacttggaggacagatcaaggggcatctcgctgcactcaggtggagaggccatctctcgttccagctgtggcggtgacttaagaggagagaaggtaacggaagtcccttctgtttgctgctcggtgccactgggcatcttggcggggtgcggtggggctgagctcccactgggggctggcagcagaggctgtggagttggaagcaccttggcagaagcagtaacaagggaggtatctgccaaaggcccagggaccccatcgggtgcaggctgggtggtggtgctaccggatggggaagtgcaggggagcctgttcacctccagagataccagcttggaatccgaagtcagaggccgggccacagaaaatgcatacgggtaagaacggagctcgggggaggctagcacgcctgggagacacctgtcctgcaggtaggacggcaggacagggagcgtaagagtggaggaaacccctagagtggttggcagtgtggccacactgagtggctgcccacagcttggaggcgggatatataccagcggctggctcggggtcagcactgtccctggctgaaaggacagggggactttttgcatagctggtgcctgagctgcaggaaagcacactctactcaaactgaaggaggccgggatgggtgcagaggtgggaatggcagctggcgtggcagcaggcatgggtgtaggggctggagtaaagatgggggctggggtgggtgcaggcaccggtgtaggagcaaaggcggggatgagggtgggggtagaaggtgggccggaagatggggttggagtgggcatgggcacagacggaggggcaggggccgctggaggcgtggatgctggcatgggagccagaaccggagtggggacgggagcgagaaccaaggtcggagctgaagggggcacaggagcctggatgagagccaagggaggagctgaaactgggactgaaagcggggcaggagctggagccgacaagggaaccgggcctgaagggggagcagaagctggcacaggcaccaagactgaggccgaaacagaaagggggttcgagtcagagatgagcgtgggcactgacggtggcgctggagccagagccgggacaggtgctaagggaggggaaggagctggaaccgaagtggcaacttggactggaacaagccctgaatgggggactggggcagggacggagaggggaacctggaatgcatctggaacagagtggggcacagaggccgaaccgggagcagggggacagataggggctggcagaggactgaagttagtggtaaccaggggcagggtcccctccacagggactccagttcccagagttgccaaaatgaaagtattcttctctccaacaccttgccgagagtccaaagcctttactccggcgggtgagcagtcaacctgtttgctcatttgggtgttgagtggagtccaggagcagtcggccctgctgttgctggcctcggcgctgtcagatgcgggaagcttgagcccgtctcctgggctgctcaggggcaccaagaggccctcagcctctgccacgttcccagcgtagtccatttttggctggggatcgtcaggcttgtcttctgacttgtgcccaagtttttctgtagcactgccatctgggtctgccccccgggcattgctgccacttccaactgccgtgagctccaccttggaaaaactgctgctgacacaaaactcctgagatccaaagtgctggcagtcgcctgtcgttgactcctcatcagaaagaggtgctcttctctcctcgttgatgccacacatgcgaatccggtcagaactggtccagttgtgcacgccgctgtagagcggtgctgtagagatcatgacagccactcaccaccagataggacctgctgtggccactccccctccttctcctctctctcggcggcggcggcggtcggactctaggaactgagaggaagaagggagggctcagcaaagcggaggagagacagagccacacactggcagcagccgcggcgagcgaaagagt

SEQ ID NO: 16876 - RNA, 7219 nt, Homo sapiens
  source 1..7219: mol_type = other RNA
tacgtagatatatatgtatttttttttcttaaaaagggaaaacaactgttcaaaaccaactgggcagtatggtgggggtggggagcagtcctacagaagggggccgagaacttcccccccaggaacaaagaacaaacacaatacaaagaaaataaccaccaatgctcccgcatggctcaggagcctctagagaacagattgtcccatcctcaaactggctttttttttttccttttttttttaatcttttttttttccattttcttttttgttgttgttgttttagcacctgtacaataaaactgtaccatctccaaccagagccggccacggcgaggccctcctgcctttggatggtacatactctacaaggattgttcggaaaaatagcaattggtagaaaaataagagtgggagggacaatgccacagagggggcggggacagggaagcaacccaagctcctctctctctctcactcgacaaacccagcgctggaggcccagaggccagggggaggccaggtagggataccactcagccccaggcccccaggcatgagtggagcaagggctggagaccactttcctgcccttgcctaggaaacagctgacgcctggatttcacatccggcagtgagtcccagagccctctgcagattcccaaggagaatgaggggctgagggaggaggtgggaggagaggaaggaaaggggtgctgtgagtctcagaaggggcagggatgggggtggctgagggctgggaggtgagaggctcagtatcttgagacagggaggccagaacggggtgggagagtggaggcaggaacaaactcgtattgtgcactctgaggggggcagtgaagaaggcgtgaggaggggggccaccctcacccctcagatcccttctccacgctcctttattagagtaacttattaacccctcacctcacaatcctcccctccctgtcaacactaatctcaagatagcggggctgctgcaaagggcgggaatgggtgggtgggggagcaccaaagcctcaggatttacccccaagcccccagccctgggccagcagcaaccagcttcgttagtcacaagtccatgttcccccaccccattccacctcaccccctccccagtgggggaaaaaaacaccagggaatagctttgtcagagctcatcaacaaagaaaaagaaaaggaggtacagaaagtccctcaatacaacaagttgtctcaaatcgtcacagtgatacagacttatcagaaaccaatgaaacaatacaaattaaatactaataaaataaatactacagaagacagaagaacacaggggaatggagttggggggcgctcagagatctgggattttctcatttctcctcgggacaggccaaggccatccagggcccaggtttggtcttggtcatgaacaaggaggccagtccaagggaccccggcgccacctcccaccacccccgggacctcttgtcctcagacatggagttcaactttccacccccatcagcaaccacgataacaatgacgacgacagggagatgagaactaattgtaaccaaaaaaacaaaaacagtccagtcgctaatgctggcattgataaggcggcttcttgttggtccgtattattgcctcattctgcagtctggtgctcggtcggggaaagacaaggaggtgggggaagggcgaactcggaaggagaaagaagaggaggggctgttttcccggtcaactgttgcaagactggaattccacctcggaccctaggagccgaagtaggtctggctcgtaccgcaccagctccacagtctcagaggagcctgggggggatctgtcgtccaagcctccaggcctctcggcaggggtcagcagctgactggaggccacctgcctgtagaactcggccttgggcatggtggtgatttcaaagtgcgggaaccgggcctgaaagatcctcgaggaaagcttcagcctcttcaagacatcggaaaagaggaaccagttgcagggcccgcgggacactgacacttggaggttgtagcaagggagaagaggcttgtctgagagttcaaacatgaaatcatcctcctccatcggatcgtctccttcttgatctgagctcccaggaggattatgtaggaggtcacaggcaaacccgtctttttcctccaacacagaactgctgtaaaaatcccaggatacaccgggatcaccctctgcccggccctgaagatccgagaggtgatcactgagaaagcgcttcatggtgtcgctgctggccagcttcatggctgtctgacccgagtaggtagccagtgtgggatcggccccataggacagcaggagccagatggtctccaggttgtcattgaccaccgcatcatgaactggcctcgtgccgtcctgcgcactgcagttcacgttggccccgtgctccagcaggatgttcaggatgtcggtccagccccgggaacaagcctcatgcagggctgtgtagccagcattgtcacggtgattcacatcttcactgtctttctggaggcagtagagaacaacatccttatagccaagacgcgccgccctctgcaggagggtctcaccagcatttttgttcactatgagccgacgtgcctctggggggatctgccgggctgtaggtgactctgaggcctcctctgagctggcacttcgggacttagagggtgtacatggttctgtgggtttcactggggtgggagatttgggagatcgtgtcttctgctggctccaacgacctttgccctttgcctcttctgagacggttgccatgtgcttggtcttgcactttcgttttcctgatggcttttctgaattttcaaggcaggctggctcttccaggttatttgggaggaaaccgtttggtgaatccgagatcccctggactttgttgggcaagagaaggttcctgttcctgaggcggtgctccaaactttgggaggaggaagtcttctgcttacgggcctttaaatctgctctccctttccgccgctgctcgtcttcttgctctgtcaggtactccccagtctgatattttcggctcttctgccgtcttcgtttcttcctcttcagcaggccctcctcctcttcttcctcctcctcctcattggtgtcccacatttgccgggcagcctctgtcctccagggcatttctcgggctcgccacaggtgccttcggccctggctcagcagagacttgtcctgggcatggtggctgcgatactgggtgtcccgttgggtctttctcacctttcgacgcttagctggggtgggggttacctcctcttcttcttctgtggggaagacttcctggcttcccatgtcactgtctgccatgccagcaaaggagctacagatgcttccagactgactgcgcgtgcgggtgctcagaaccacaggaataaagtcacggaaactgctctttgctttcttttccaaggaaccttcctcgtggctgtcggctcgttttcctggagactgggactccggctttgtcggcttccggtgcttgtgctttcccctgactccattgtgctcttttcctgaatctgaagcccccctggggcttttcttggtggattcctgggggtcactgggcagcttccggcacttgggtctgtgggaactccggaccacggccttggcttgtggctggagctgctgctcttcactgtccttctctttgccgcacttcatcttcttgggcggcagagattccgtcacatcatctggctgccacttgttcttgcaagcaaagacccctacgctttcctgtttcactcgagcctgcccggccttagcccgaacttcagcttggcccctctggggagccactgggaggccatcagcccggaagcaggtggctaaattgaagaccacatcaccatccaccttctccattttcactcgccccagatccacctggcttccaagctgtgggcgctctgtgctggagcccctcctgctgctcggaaccacgtccaatataagttccttggggtggctgtcgtgaggtagcaaaggcagctcaggcatcttaggcaggttctggggggtggccaggaccagctcatgggacatgtaggtggccagcacttggttcttaggcttcgtgtctcctgccagcttcaggccacaagccccctgggggccttccatcttaggagtgctgtcagagcagaggtggctctctgattcctcaggcccctgattcattcgaatgtccccaccgctaggctgaacagacagtgccagggtcccagtctgagggctgagggtcaagaggacaggattgacttgttcttcataaggcttggcagcaatccggcaagttttgttctttgtaacagggtcctgctctggaacgaaggagcccccaggccgtggttgcccctcaggaagtccgtgcacggcttcgctggagctgagagatggcacaccagaaaactccgaaacaacgctggtgggcctgatgggcgccccctgactgggggtcagctgcccggcactggaaatgccaatggaaagcagagacgcctggtggtacggggaccagccaacaggcaggacctgggtgctggtaggtttcccattgactgaacaccggggataaatatttgccggccccgtgggtttccacaaagagagttccttggtttggcaccctggcagcccaggggcaatgcgggctggagtatatcgtttcactgtgcttggctgtccctcagcaccagcctggctgccctttttgccacacgtggcaccagtgcccttaggctctccttgatcaatgatggagatgggctcctgcttggggagatggcgggggtcacggttgaggcccaggttggggtctttgttcagcagcagggatgcaggcactgggttggccactcccacgtaggtgccaggaatggtgctgatcagtgcagttgagttcttcacccaggtgctcgggtccccattcctcacgatctcgggaaagatgacaaagggcgaggaagtggagcccaggcaggaggtgacattgccaccggcagcctgggttgtgcgctgagacctagacaggactgtggagaggagggccttgctgctggtgtgcacgggggtcaacacaggcatggggggtgtcttgcgctggttcggcaatggaagcttctggcggttggacttggaggacagatcaaggggcatctcgctgcactcaggtggagaggccatctctcgttccagctgtggcggtgacttaagaggagagaaggtaacggaagtcccttctgtttgctgctcggtgccactgggcatcttggcggggtgcggtggggctgagctcccactgggggctggcagcagaggctgtggagttggaagcaccttggcagaagcagtaacaagggaggtatctgccaaaggcccagggaccccatcgggtgcaggctgggtggtggtgctaccggatggggaagtgcaggggagcctgttcacctccagagataccagcttggaatccgaagtcagaggccgggccacagaaaatgcatacgggtaagaacggagctcgggggaggctagcacgcctgggagacacctgtcctgcaggtaggacggcaggacagggagcgtaagagtggaggaaacccctagagtggttggcagtgtggccacactgagtggctgcccacagcttggaggcgggatatataccagcggctggctcggggtcagcactgtccctggctgaaaggacagggggactttttgcatagctggtgcctgagctgcaggaaagcacactctactcaaactgaaggaggccgggatgggtgcagaggtgggaatggcagctggcgtggcagcaggcatgggtgtaggggctggagtaaagatgggggctggggtgggtgcaggcaccggtgtaggagcaaaggcggggatgagggtgggggtagaaggtgggccggaagatggggttggagtgggcatgggcacagacggaggggcaggggccgctggaggcgtggatgctggcatgggagccagaaccggagtggggacgggagcgagaaccaaggtcggagctgaagggggcacaggagcctggatgagagccaagggaggagctgaaactgggactgaaagcggggcaggagctggagccgacaagggaaccgggcctgaagggggagcagaagctggcacaggcaccaagactgaggccgaaacagaaagggggttcgagtcagagatgagcgtgggcactgacggtggcgctggagccagagccgggacaggtgctaagggaggggaaggagctggaaccgaagtggcaacttggactggaacaagccctgaatgggggactggggcagggacggagaggggaacctggaatgcatctggaacagagtggggcacagaggccgaaccgggagcagggggacagataggggctggcagaggactgaagttagtggtaaccaggggcagggtcccctccacagggactccagttcccagagttgccaaaatgaaagtattcttctctccaacaccttgccgagagtccaaagcctttactccggcgggtgagcagtcaacctgtttgctcatttgggtgttgagtggagtccaggagcagtcggccctgctgttgctggcctcggcgctgtcagatgcgggaagcttgagcccgtctcctgggctgctcaggggcaccaagaggccctcagcctctgccacgttcccagcgtagtccatttttggctggggatcgtcaggcttgtcttctgacttgtgcccaagtttttctgtagcactgccatctgggtctgccccccgggcattgctgccacttccaactgccgtgagctccaccttggaaaaactgctgctgacacaaaactcctgagatccaaagtgctggcagtcgcctgtcgttgactcctcatcagaaagaggtgctcttctctcctcgttgatgccacacatgcgaatccggtcagaactggtccagttgtgcacgccgctgtagagcggtgctgtagagatcatgacagccactcaccaccagataggacctgctgtggccactccccctcgtcctccatgcacccggcccccggggctcctcgtcgtcgtcgtcccggctcgtaccgccccccgtcgg

SEQ ID NO: 16877 - RNA, 7244 nt, Homo sapiens
  source 1..7244: mol_type = other RNA
tacgtagatatatatgtatttttttttcttaaaaagggaaaacaactgttcaaaaccaactgggcagtatggtgggggtggggagcagtcctacagaagggggccgagaacttcccccccaggaacaaagaacaaacacaatacaaagaaaataaccaccaatgctcccgcatggctcaggagcctctagagaacagattgtcccatcctcaaactggctttttttttttccttttttttttaatcttttttttttccattttcttttttgttgttgttgttttagcacctgtacaataaaactgtaccatctccaaccagagccggccacggcgaggccctcctgcctttggatggtacatactctacaaggattgttcggaaaaatagcaattggtagaaaaataagagtgggagggacaatgccacagagggggcggggacagggaagcaacccaagctcctctctctctctcactcgacaaacccagcgctggaggcccagaggccagggggaggccaggtagggataccactcagccccaggcccccaggcatgagtggagcaagggctggagaccactttcctgcccttgcctaggaaacagctgacgcctggatttcacatccggcagtgagtcccagagccctctgcagattcccaaggagaatgaggggctgagggaggaggtgggaggagaggaaggaaaggggtgctgtgagtctcagaaggggcagggatgggggtggctgagggctgggaggtgagaggctcagtatcttgagacagggaggccagaacggggtgggagagtggaggcaggaacaaactcgtattgtgcactctgaggggggcagtgaagaaggcgtgaggaggggggccaccctcacccctcagatcccttctccacgctcctttattagagtaacttattaacccctcacctcacaatcctcccctccctgtcaacactaatctcaagatagcggggctgctgcaaagggcgggaatgggtgggtgggggagcaccaaagcctcaggatttacccccaagcccccagccctgggccagcagcaaccagcttcgttagtcacaagtccatgttcccccaccccattccacctcaccccctccccagtgggggaaaaaaacaccagggaatagctttgtcagagctcatcaacaaagaaaaagaaaaggaggtacagaaagtccctcaatacaacaagttgtctcaaatcgtcacagtgatacagacttatcagaaaccaatgaaacaatacaaattaaatactaataaaataaatactacagaagacagaagaacacaggggaatggagttggggggcgctcagagatctgggattttctcatttctcctcgggacaggccaaggccatccagggcccaggtttggtcttggtcatgaacaaggaggccagtccaagggaccccggcgccacctcccaccacccccgggacctcttgtcctcagacatggagttcaactttccacccccatcagcaaccacgataacaatgacgacgacagggagatgagaactaattgtaaccaaaaaaacaaaaacagtccagtcgctaatgctggcattgataaggcggcttcttgttggtccgtattattgcctcattctgcagtctggtgctcggtcggggaaagacaaggaggtgggggaagggcgaactcggaaggagaaagaagaggaggggctgttttcccggtcaactgttgcaagactggaattccacctcggaccctaggagccgaagtaggtctggctcgtaccgcaccagctccacagtctcagaggagcctgggggggatctgtcgtccaagcctccaggcctctcggcaggggtcagcagctgactggaggccacctgcctgtagaactcggccttgggcatggtggtgatttcaaagtgcgggaaccgggcctgaaagatcctcgaggaaagcttcagcctcttcaagacatcggaaaagaggaaccagttgcagggcccgcgggacactgacacttggaggttgtagcaagggagaagaggcttgtctgagagttcaaacatgaaatcatcctcctccatcggatcgtctccttcttgatctgagctcccaggaggattatgtaggaggtcacaggcaaacccgtctttttcctccaacacagaactgctgtaaaaatcccaggatacaccgggatcaccctctgcccggccctgaagatccgagaggtgatcactgagaaagcgcttcatggtgtcgctgctggccagcttcatggctgtctgacccgagtaggtagccagtgtgggatcggccccataggacagcaggagccagatggtctccaggttgtcattgaccaccgcatcatgaactggcctcgtgccgtcctgcgcactgcagttcacgttggccccgtgctccagcaggatgttcaggatgtcggtccagccccgggaacaagcctcatgcagggctgtgtagccagcattgtcacggtgattcacatcttcactgtctttctggaggcagtagagaacaacatccttatagccaagacgcgccgccctctgcaggagggtctcaccagcatttttgttcactatgagccgacgtgcctctggggggatctgccgggctgtaggtgactctgaggcctcctctgagctggcacttcgggacttagagggtgtacatggttctgtgggtttcactggggtgggagatttgggagatcgtgtcttctgctggctccaacgacctttgccctttgcctcttctgagacggttgccatgtgcttggtcttgcactttcgttttcctgatggcttttctgaattttcaaggcaggctggctcttccaggttatttgggaggaaaccgtttggtgaatccgagatcccctggactttgttgggcaagagaaggttcctgttcctgaggcggtgctccaaactttgggaggaggaagtcttctgcttacgggcctttaaatctgctctccctttccgccgctgctcgtcttcttgctctgtcaggtactccccagtctgatattttcggctcttctgccgtcttcgtttcttcctcttcagcaggccctcctcctcttcttcctcctcctcctcattggtgtcccacatttgccgggcagcctctgtcctccagggcatttctcgggctcgccacaggtgccttcggccctggctcagcagagacttgtcctgggcatggtggctgcgatactgggtgtcccgttgggtctttctcacctttcgacgcttagctggggtgggggttacctcctcttcttcttctgtggggaagacttcctggcttcccatgtcactgtctgccatgccagcaaaggagctacagatgcttccagactgactgcgcgtgcgggtgctcagaaccacaggaataaagtcacggaaactgctctttgctttcttttccaaggaaccttcctcgtggctgtcggctcgttttcctggagactgggactccggctttgtcggcttccggtgcttgtgctttcccctgactccattgtgctcttttcctgaatctgaagcccccctggggcttttcttggtggattcctgggggtcactgggcagcttccggcacttgggtctgtgggaactccggaccacggccttggcttgtggctggagctgctgctcttcactgtccttctctttgccgcacttcatcttcttgggcggcagagattccgtcacatcatctggctgccacttgttcttgcaagcaaagacccctacgctttcctgtttcactcgagcctgcccggccttagcccgaacttcagcttggcccctctggggagccactgggaggccatcagcccggaagcaggtggctaaattgaagaccacatcaccatccaccttctccattttcactcgccccagatccacctggcttccaagctgtgggcgctctgtgctggagcccctcctgctgctcggaaccacgtccaatataagttccttggggtggctgtcgtgaggtagcaaaggcagctcaggcatcttaggcaggttctggggggtggccaggaccagctcatgggacatgtaggtggccagcacttggttcttaggcttcgtgtctcctgccagcttcaggccacaagccccctgggggccttccatcttaggagtgctgtcagagcagaggtggctctctgattcctcaggcccctgattcattcgaatgtccccaccgctaggctgaacagacagtgccagggtcccagtctgagggctgagggtcaagaggacaggattgacttgttcttcataaggcttggcagcaatccggcaagttttgttctttgtaacagggtcctgctctggaacgaaggagcccccaggccgtggttgcccctcaggaagtccgtgcacggcttcgctggagctgagagatggcacaccagaaaactccgaaacaacgctggtgggcctgatgggcgccccctgactgggggtcagctgcccggcactggaaatgccaatggaaagcagagacgcctggtggtacggggaccagccaacaggcaggacctgggtgctggtaggtttcccattgactgaacaccggggataaatatttgccggccccgtgggtttccacaaagagagttccttggtttggcaccctggcagcccaggggcaatgcgggctggagtatatcgtttcactgtgcttggctgtccctcagcaccagcctggctgccctttttgccacacgtggcaccagtgcccttaggctctccttgatcaatgatggagatgggctcctgcttggggagatggcgggggtcacggttgaggcccaggttggggtctttgttcagcagcagggatgcaggcactgggttggccactcccacgtaggtgccaggaatggtgctgatcagtgcagttgagttcttcacccaggtgctcgggtccccattcctcacgatctcgggaaagatgacaaagggcgaggaagtggagcccaggcaggaggtgacattgccaccggcagcctgggttgtgcgctgagacctagacaggactgtggagaggagggccttgctgctggtgtgcacgggggtcaacacaggcatggggggtgtcttgcgctggttcggcaatggaagcttctggcggttggacttggaggacagatcaaggggcatctcgctgcactcaggtggagaggccatctctcgttccagctgtggcggtgacttaagaggagagaaggtaacggaagtcccttctgtttgctgctcggtgccactgggcatcttggcggggtgcggtggggctgagctcccactgggggctggcagcagaggctgtggagttggaagcaccttggcagaagcagtaacaagggaggtatctgccaaaggcccagggaccccatcgggtgcaggctgggtggtggtgctaccggatggggaagtgcaggggagcctgttcacctccagagataccagcttggaatccgaagtcagaggccgggccacagaaaatgcatacgggtaagaacggagctcgggggaggctagcacgcctgggagacacctgtcctgcaggtaggacggcaggacagggagcgtaagagtggaggaaacccctagagtggttggcagtgtggccacactgagtggctgcccacagcttggaggcgggatatataccagcggctggctcggggtcagcactgtccctggctgaaaggacagggggactttttgcatagctggtgcctgagctgcaggaaagcacactctactcaaactgaaggaggccgggatgggtgcagaggtgggaatggcagctggcgtggcagcaggcatgggtgtaggggctggagtaaagatgggggctggggtgggtgcaggcaccggtgtaggagcaaaggcggggatgagggtgggggtagaaggtgggccggaagatggggttggagtgggcatgggcacagacggaggggcaggggccgctggaggcgtggatgctggcatgggagccagaaccggagtggggacgggagcgagaaccaaggtcggagctgaagggggcacaggagcctggatgagagccaagggaggagctgaaactgggactgaaagcggggcaggagctggagccgacaagggaaccgggcctgaagggggagcagaagctggcacaggcaccaagactgaggccgaaacagaaagggggttcgagtcagagatgagcgtgggcactgacggtggcgctggagccagagccgggacaggtgctaagggaggggaaggagctggaaccgaagtggcaacttggactggaacaagccctgaatgggggactggggcagggacggagaggggaacctggaatgcatctggaacagagtggggcacagaggccgaaccgggagcagggggacagataggggctggcagaggactgaagttagtggtaaccaggggcagggtcccctccacagggactccagttcccagagttgccaaaatgaaagtattcttctctccaacaccttgccgagagtccaaagcctttactccggcgggtgagcagtcaacctgtttgctcatttgggtgttgagtggagtccaggagcagtcggccctgctgttgctggcctcggcgctgtcagatgcgggaagcttgagcccgtctcctgggctgctcaggggcaccaagaggccctcagcctctgccacgttcccagcgtagtccatttttggctggggatcgtcaggcttgtcttctgacttgtgcccaagtttttctgtagcactgccatctgggtctgccccccgggcattgctgccacttccaactgccgtgagctccaccttggaaaaactgctgctgacacaaaactcctgagatccaaagtgctggcagtcgcctgtcgttgactcctcatcagaaagaggtgctcttctctcctcgttgatgccacacatgcgaatccggtcagaactggtccagttgtgcacgccgctgtagagcggtgctgtagagatcatgacagccactcaccaccagataggacctgctgtggccactccccctgggcagagcccccggccgctgtcgcaactttgctcttctccacgccgccggggaagcgggcgaagcgggaggagggaggtggcggggggtgctg

SEQ ID NO: 16878 - RNA, 7404 nt, Homo sapiens
  source 1..7404: mol_type = other RNA
tacgtagatatatatgtatttttttttcttaaaaagggaaaacaactgttcaaaaccaactgggcagtatggtgggggtggggagcagtcctacagaagggggccgagaacttcccccccaggaacaaagaacaaacacaatacaaagaaaataaccaccaatgctcccgcatggctcaggagcctctagagaacagattgtcccatcctcaaactggctttttttttttccttttttttttaatcttttttttttccattttcttttttgttgttgttgttttagcacctgtacaataaaactgtaccatctccaaccagagccggccacggcgaggccctcctgcctttggatggtacatactctacaaggattgttcggaaaaatagcaattggtagaaaaataagagtgggagggacaatgccacagagggggcggggacagggaagcaacccaagctcctctctctctctcactcgacaaacccagcgctggaggcccagaggccagggggaggccaggtagggataccactcagccccaggcccccaggcatgagtggagcaagggctggagaccactttcctgcccttgcctaggaaacagctgacgcctggatttcacatccggcagtgagtcccagagccctctgcagattcccaaggagaatgaggggctgagggaggaggtgggaggagaggaaggaaaggggtgctgtgagtctcagaaggggcagggatgggggtggctgagggctgggaggtgagaggctcagtatcttgagacagggaggccagaacggggtgggagagtggaggcaggaacaaactcgtattgtgcactctgaggggggcagtgaagaaggcgtgaggaggggggccaccctcacccctcagatcccttctccacgctcctttattagagtaacttattaacccctcacctcacaatcctcccctccctgtcaacactaatctcaagatagcggggctgctgcaaagggcgggaatgggtgggtgggggagcaccaaagcctcaggatttacccccaagcccccagccctgggccagcagcaaccagcttcgttagtcacaagtccatgttcccccaccccattccacctcaccccctccccagtgggggaaaaaaacaccagggaatagctttgtcagagctcatcaacaaagaaaaagaaaaggaggtacagaaagtccctcaatacaacaagttgtctcaaatcgtcacagtgatacagacttatcagaaaccaatgaaacaatacaaattaaatactaataaaataaatactacagaagacagaagaacacaggggaatggagttggggggcgctcagagatctgggattttctcatttctcctcgggacaggccaaggccatccagggcccaggtttggtcttggtcatgaacaaggaggccagtccaagggaccccggcgccacctcccaccacccccgggacctcttgtcctcagacatggagttcaactttccacccccatcagcaaccacgataacaatgacgacgacagggagatgagaactaattgtaaccaaaaaaacaaaaacagtccagtcgctaatgctggcattgataaggcggcttcttgttggtccgtattattgcctcattctgcagtctggtgctcggtcggggaaagacaaggaggtgggggaagggcgaactcggaaggagaaagaagaggaggggctgttttcccggtcaactgttgcaagactggaattccacctcggaccctaggagccgaagtaggtctggctcgtaccgcaccagctccacagtctcagaggagcctgggggggatctgtcgtccaagcctccaggcctctcggcaggggtcagcagctgactggaggccacctgcctgtagaactcggccttgggcatggtggtgatttcaaagtgcgggaaccgggcctgaaagatcctcgaggaaagcttcagcctcttcaagacatcggaaaagaggaaccagttgcagggcccgcgggacactgacacttggaggttgtagcaagggagaagaggcttgtctgagagttcaaacatgaaatcatcctcctccatcggatcgtctccttcttgatctgagctcccaggaggattatgtaggaggtcacaggcaaacccgtctttttcctccaacacagaactgctgtaaaaatcccaggatacaccgggatcaccctctgcccggccctgaagatccgagaggtgatcactgagaaagcgcttcatggtgtcgctgctggccagcttcatggctgtctgacccgagtaggtagccagtgtgggatcggccccataggacagcaggagccagatggtctccaggttgtcattgaccaccgcatcatgaactggcctcgtgccgtcctgcgcactgcagttcacgttggccccgtgctccagcaggatgttcaggatgtcggtccagccccgggaacaagcctcatgcagggctgtgtagccagcattgtcacggtgattcacatcttcactgtctttctggaggcagtagagaacaacatccttatagccaagacgcgccgccctctgcaggagggtctcaccagcatttttgttcactatgagccgacgtgcctctggggggatctgccgggctgtaggtgactctgaggcctcctctgagctggcacttcgggacttagagggtgtacatggttctgtgggtttcactggggtgggagatttgggagatcgtgtcttctgctggctccaacgacctttgccctttgcctcttctgagacggttgccatgtgcttggtcttgcactttcgttttcctgatggcttttctgaattttcaaggcaggctggctcttccaggttatttgggaggaaaccgtttggtgaatccgagatcccctggactttgttgggcaagagaaggttcctgttcctgaggcggtgctccaaactttgggaggaggaagtcttctgcttacgggcctttaaatctgctctccctttccgccgctgctcgtcttcttgctctgtcaggtactccccagtctgatattttcggctcttctgccgtcttcgtttcttcctcttcagcaggccctcctcctcttcttcctcctcctcctcattggtgtcccacatttgccgggcagcctctgtcctccagggcatttctcgggctcgccacaggtgccttcggccctggctcagcagagacttgtcctgggcatggtggctgcgatactgggtgtcccgttgggtctttctcacctttcgacgcttagctggggtgggggttacctcctcttcttcttctgtggggaagacttcctggcttcccatgtcactgtctgccatgccagcaaaggagctacagatgcttccagactgactgcgcgtgcgggtgctcagaaccacaggaataaagtcacggaaactgctctttgctttcttttccaaggaaccttcctcgtggctgtcggctcgttttcctggagactgggactccggctttgtcggcttccggtgcttgtgctttcccctgactccattgtgctcttttcctgaatctgaagcccccctggggcttttcttggtggattcctgggggtcactgggcagcttccggcacttgggtctgtgggaactccggaccacggccttggcttgtggctggagctgctgctcttcactgtccttctctttgccgcacttcatcttcttgggcggcagagattccgtcacatcatctggctgccacttgttcttgcaagcaaagacccctacgctttcctgtttcactcgagcctgcccggccttagcccgaacttcagcttggcccctctggggagccactgggaggccatcagcccggaagcaggtggctaaattgaagaccacatcaccatccaccttctccattttcactcgccccagatccacctggcttccaagctgtgggcgctctgtgctggagcccctcctgctgctcggaaccacgtccaatataagttccttggggtggctgtcgtgaggtagcaaaggcagctcaggcatcttaggcaggttctggggggtggccaggaccagctcatgggacatgtaggtggccagcacttggttcttaggcttcgtgtctcctgccagcttcaggccacaagccccctgggggccttccatcttaggagtgctgtcagagcagaggtggctctctgattcctcaggcccctgattcattcgaatgtccccaccgctaggctgaacagacagtgccagggtcccagtctgagggctgagggtcaagaggacaggattgacttgttcttcataaggcttggcagcaatccggcaagttttgttctttgtaacagggtcctgctctggaacgaaggagcccccaggccgtggttgcccctcaggaagtccgtgcacggcttcgctggagctgagagatggcacaccagaaaactccgaaacaacgctggtgggcctgatgggcgccccctgactgggggtcagctgcccggcactggaaatgccaatggaaagcagagacgcctggtggtacggggaccagccaacaggcaggacctgggtgctggtaggtttcccattgactgaacaccggggataaatatttgccggccccgtgggtttccacaaagagagttccttggtttggcaccctggcagcccaggggcaatgcgggctggagtatatcgtttcactgtgcttggctgtccctcagcaccagcctggctgccctttttgccacacgtggcaccagtgcccttaggctctccttgatcaatgatggagatgggctcctgcttggggagatggcgggggtcacggttgaggcccaggttggggtctttgttcagcagcagggatgcaggcactgggttggccactcccacgtaggtgccaggaatggtgctgatcagtgcagttgagttcttcacccaggtgctcgggtccccattcctcacgatctcgggaaagatgacaaagggcgaggaagtggagcccaggcaggaggtgacattgccaccggcagcctgggttgtgcgctgagacctagacaggactgtggagaggagggccttgctgctggtgtgcacgggggtcaacacaggcatggggggtgtcttgcgctggttcggcaatggaagcttctggcggttggacttggaggacagatcaaggggcatctcgctgcactcaggtggagaggccatctctcgttccagctgtggcggtgacttaagaggagagaaggtaacggaagtcccttctgtttgctgctcggtgccactgggcatcttggcggggtgcggtggggctgagctcccactgggggctggcagcagaggctgtggagttggaagcaccttggcagaagcagtaacaagggaggtatctgccaaaggcccagggaccccatcgggtgcaggctgggtggtggtgctaccggatggggaagtgcaggggagcctgttcacctccagagataccagcttggaatccgaagtcagaggccgggccacagaaaatgcatacgggtaagaacggagctcgggggaggctagcacgcctgggagacacctgtcctgcaggtaggacggcaggacagggagcgtaagagtggaggaaacccctagagtggttggcagtgtggccacactgagtggctgcccacagcttggaggcgggatatataccagcggctggctcggggtcagcactgtccctggctgaaaggacagggggactttttgcatagctggtgcctgagctgcaggaaagcacactctactcaaactgaaggaggccgggatgggtgcagaggtgggaatggcagctggcgtggcagcaggcatgggtgtaggggctggagtaaagatgggggctggggtgggtgcaggcaccggtgtaggagcaaaggcggggatgagggtgggggtagaaggtgggccggaagatggggttggagtgggcatgggcacagacggaggggcaggggccgctggaggcgtggatgctggcatgggagccagaaccggagtggggacgggagcgagaaccaaggtcggagctgaagggggcacaggagcctggatgagagccaagggaggagctgaaactgggactgaaagcggggcaggagctggagccgacaagggaaccgggcctgaagggggagcagaagctggcacaggcaccaagactgaggccgaaacagaaagggggttcgagtcagagatgagcgtgggcactgacggtggcgctggagccagagccgggacaggtgctaagggaggggaaggagctggaaccgaagtggcaacttggactggaacaagccctgaatgggggactggggcagggacggagaggggaacctggaatgcatctggaacagagtggggcacagaggccgaaccgggagcagggggacagataggggctggcagaggactgaagttagtggtaaccaggggcagggtcccctccacagggactccagttcccagagttgccaaaatgaaagtattcttctctccaacaccttgccgagagtccaaagcctttactccggcgggtgagcagtcaacctgtttgctcatttgggtgttgagtggagtccaggagcagtcggccctgctgttgctggcctcggcgctgtcagatgcgggaagcttgagcccgtctcctgggctgctcaggggcaccaagaggccctcagcctctgccacgttcccagcgtagtccatttttggctggggatcgtcaggcttgtcttctgacttgtgcccaagtttttctgtagcactgccatctgggtctgccccccgggcattgctgccacttccaactgccgtgagctccaccttggaaaaactgctgctgacacaaaactcctgagatccaaagtgctggcagtcgcctgtcgttgactcctcatcagaaagaggtgctcttctctcctcgttgatgccacacatgcgaatccggtcagaactggtccagttgtgcacgccgctgtagagcggtgctgtagagatcatgacagccactcaccaccagataggacctgctgtggccactccccctgttcccgggtcggctccgcggggaggctcaggccgccacccgggctccctcttactccctcttaaccgccacccgcctaatactgccccgatctgatgcccccctccgccccttatcgccaccgacctccttctcctctctctcggcggcggcggcggtcggactctaggaactgagaggaagaagggagggctcagcaaagcggaggagagacagagccacacactggcagcagccgcggcgagcgaaagagt

SEQ ID NO: 16879 - RNA, 7435 nt, Homo sapiens
  source 1..7435: mol_type = other RNA
tacgtagatatatatgtatttttttttcttaaaaagggaaaacaactgttcaaaaccaactgggcagtatggtgggggtggggagcagtcctacagaagggggccgagaacttcccccccaggaacaaagaacaaacacaatacaaagaaaataaccaccaatgctcccgcatggctcaggagcctctagagaacagattgtcccatcctcaaactggctttttttttttccttttttttttaatcttttttttttccattttcttttttgttgttgttgttttagcacctgtacaataaaactgtaccatctccaaccagagccggccacggcgaggccctcctgcctttggatggtacatactctacaaggattgttcggaaaaatagcaattggtagaaaaataagagtgggagggacaatgccacagagggggcggggacagggaagcaacccaagctcctctctctctctcactcgacaaacccagcgctggaggcccagaggccagggggaggccaggtagggataccactcagccccaggcccccaggcatgagtggagcaagggctggagaccactttcctgcccttgcctaggaaacagctgacgcctggatttcacatccggcagtgagtcccagagccctctgcagattcccaaggagaatgaggggctgagggaggaggtgggaggagaggaaggaaaggggtgctgtgagtctcagaaggggcagggatgggggtggctgagggctgggaggtgagaggctcagtatcttgagacagggaggccagaacggggtgggagagtggaggcaggaacaaactcgtattgtgcactctgaggggggcagtgaagaaggcgtgaggaggggggccaccctcacccctcagatcccttctccacgctcctttattagagtaacttattaacccctcacctcacaatcctcccctccctgtcaacactaatctcaagatagcggggctgctgcaaagggcgggaatgggtgggtgggggagcaccaaagcctcaggatttacccccaagcccccagccctgggccagcagcaaccagcttcgttagtcacaagtccatgttcccccaccccattccacctcaccccctccccagtgggggaaaaaaacaccagggaatagctttgtcagagctcatcaacaaagaaaaagaaaaggaggtacagaaagtccctcaatacaacaagttgtctcaaatcgtcacagtgatacagacttatcagaaaccaatgaaacaatacaaattaaatactaataaaataaatactacagaagacagaagaacacaggggaatggagttggggggcgctcagagatctgggattttctcatttctcctcgggacaggccaaggccatccagggcccaggtttggtcttggtcatgaacaaggaggccagtccaagggaccccggcgccacctcccaccacccccgggacctcttgtcctcagacatggagttcaactttccacccccatcagcaaccacgataacaatgacgacgacagggagatgagaactaattgtaaccaaaaaaacaaaaacagtccagtcgctaatgctggcattgataaggcggcttcttgttggtccgtattattgcctcattctgcagtctggtgctcggtcggggaaagacaaggaggtgggggaagggcgaactcggaaggagaaagaagaggaggggctgttttcccggtcaactgttgcaagactggaattccacctcggaccctaggagccgaagtaggtctggctcgtaccgcaccagctccacagtctcagaggagcctgggggggatctgtcgtccaagcctccaggcctctcggcaggggtcagcagctgactggaggccacctgcctgtagaactcggccttgggcatggtggtgatttcaaagtgcgggaaccgggcctgaaagatcctcgaggaaagcttcagcctcttcaagacatcggaaaagaggaaccagttgcagggcccgcgggacactgacacttggaggttgtagcaagggagaagaggcttgtctgagagttcaaacatgaaatcatcctcctccatcggatcgtctccttcttgatctgagctcccaggaggattatgtaggaggtcacaggcaaacccgtctttttcctccaacacagaactgctgtaaaaatcccaggatacaccgggatcaccctctgcccggccctgaagatccgagaggtgatcactgagaaagcgcttcatggtgtcgctgctggccagcttcatggctgtctgacccgagtaggtagccagtgtgggatcggccccataggacagcaggagccagatggtctccaggttgtcattgaccaccgcatcatgaactggcctcgtgccgtcctgcgcactgcagttcacgttggccccgtgctccagcaggatgttcaggatgtcggtccagccccgggaacaagcctcatgcagggctgtgtagccagcattgtcacggtgattcacatcttcactgtctttctggaggcagtagagaacaacatccttatagccaagacgcgccgccctctgcaggagggtctcaccagcatttttgttcactatgagccgacgtgcctctggggggatctgccgggctgtaggtgactctgaggcctcctctgagctggcacttcgggacttagagggtgtacatggttctgtgggtttcactggggtgggagatttgggagatcgtgtcttctgctggctccaacgacctttgccctttgcctcttctgagacggttgccatgtgcttggtcttgcactttcgttttcctgatggcttttctgaattttcaaggcaggctggctcttccaggttatttgggaggaaaccgtttggtgaatccgagatcccctggactttgttgggcaagagaaggttcctgttcctgaggcggtgctccaaactttgggaggaggaagtcttctgcttacgggcctttaaatctgctctccctttccgccgctgctcgtcttcttgctctgtcaggtactccccagtctgatattttcggctcttctgccgtcttcgtttcttcctcttcagcaggccctcctcctcttcttcctcctcctcctcattggtgtcccacatttgccgggcagcctctgtcctccagggcatttctcgggctcgccacaggtgccttcggccctggctcagcagagacttgtcctgggcatggtggctgcgatactgggtgtcccgttgggtctttctcacctttcgacgcttagctggggtgggggttacctcctcttcttcttctgtggggaagacttcctggcttcccatgtcactgtctgccatgccagcaaaggagctacagatgcttccagactgactgcgcgtgcgggtgctcagaaccacaggaataaagtcacggaaactgctctttgctttcttttccaaggaaccttcctcgtggctgtcggctcgttttcctggagactgggactccggctttgtcggcttccggtgcttgtgctttcccctgactccattgtgctcttttcctgaatctgaagcccccctggggcttttcttggtggattcctgggggtcactgggcagcttccggcacttgggtctgtgggaactccggaccacggccttggcttgtggctggagctgctgctcttcactgtccttctctttgccgcacttcatcttcttgggcggcagagattccgtcacatcatctggctgccacttgttcttgcaagcaaagacccctacgctttcctgtttcactcgagcctgcccggccttagcccgaacttcagcttggcccctctggggagccactgggaggccatcagcccggaagcaggtggctaaattgaagaccacatcaccatccaccttctccattttcactcgccccagatccacctggcttccaagctgtgggcgctctgtgctggagcccctcctgctgctcggaaccacgtccaatataagttccttggggtggctgtcgtgaggtagcaaaggcagctcaggcatcttaggcaggttctggggggtggccaggaccagctcatgggacatgtaggtggccagcacttggttcttaggcttcgtgtctcctgccagcttcaggccacaagccccctgggggccttccatcttaggagtgctgtcagagcagaggtggctctctgattcctcaggcccctgattcattcgaatgtccccaccgctaggctgaacagacagtgccagggtcccagtctgagggctgagggtcaagaggacaggattgacttgttcttcataaggcttggcagcaatccggcaagttttgttctttgtaacagggtcctgctctggaacgaaggagcccccaggccgtggttgcccctcaggaagtccgtgcacggcttcgctggagctgagagatggcacaccagaaaactccgaaacaacgctggtgggcctgatgggcgccccctgactgggggtcagctgcccggcactggaaatgccaatggaaagcagagacgcctggtggtacggggaccagccaacaggcaggacctgggtgctggtaggtttcccattgactgaacaccggggataaatatttgccggccccgtgggtttccacaaagagagttccttggtttggcaccctggcagcccaggggcaatgcgggctggagtatatcgtttcactgtgcttggctgtccctcagcaccagcctggctgccctttttgccacacgtggcaccagtgcccttaggctctccttgatcaatgatggagatgggctcctgcttggggagatggcgggggtcacggttgaggcccaggttggggtctttgttcagcagcagggatgcaggcactgggttggccactcccacgtaggtgccaggaatggtgctgatcagtgcagttgagttcttcacccaggtgctcgggtccccattcctcacgatctcgggaaagatgacaaagggcgaggaagtggagcccaggcaggaggtgacattgccaccggcagcctgggttgtgcgctgagacctagacaggactgtggagaggagggccttgctgctggtgtgcacgggggtcaacacaggcatggggggtgtcttgcgctggttcggcaatggaagcttctggcggttggacttggaggacagatcaaggggcatctcgctgcactcaggtggagaggccatctctcgttccagctgtggcggtgacttaagaggagagaaggtaacggaagtcccttctgtttgctgctcggtgccactgggcatcttggcggggtgcggtggggctgagctcccactgggggctggcagcagaggctgtggagttggaagcaccttggcagaagcagtaacaagggaggtatctgccaaaggcccagggaccccatcgggtgcaggctgggtggtggtgctaccggatggggaagtgcaggggagcctgttcacctccagagataccagcttggaatccgaagtcagaggccgggccacagaaaatgcatacgggtaagaacggagctcgggggaggctagcacgcctgggagacacctgtcctgcaggtaggacggcaggacagggagcgtaagagtggaggaaacccctagagtggttggcagtgtggccacactgagtggctgcccacagcttggaggcgggatatataccagcggctggctcggggtcagcactgtccctggctgaaaggacagggggactttttgcatagctggtgcctgagctgcaggaaagcacactctactcaaactgaaggaggccgggatgggtgcagaggtgggaatggcagctggcgtggcagcaggcatgggtgtaggggctggagtaaagatgggggctggggtgggtgcaggcaccggtgtaggagcaaaggcggggatgagggtgggggtagaaggtgggccggaagatggggttggagtgggcatgggcacagacggaggggcaggggccgctggaggcgtggatgctggcatgggagccagaaccggagtggggacgggagcgagaaccaaggtcggagctgaagggggcacaggagcctggatgagagccaagggaggagctgaaactgggactgaaagcggggcaggagctggagccgacaagggaaccgggcctgaagggggagcagaagctggcacaggcaccaagactgaggccgaaacagaaagggggttcgagtcagagatgagcgtgggcactgacggtggcgctggagccagagccgggacaggtgctaagggaggggaaggagctggaaccgaagtggcaacttggactggaacaagccctgaatgggggactggggcagggacggagaggggaacctggaatgcatctggaacagagtggggcacagaggccgaaccgggagcagggggacagataggggctggcagaggactgaagttagtggtaaccaggggcagggtcccctccacagggactccagttcccagagttgccaaaatgaaagtattcttctctccaacaccttgccgagagtccaaagcctttactccggcgggtgagcagtcaacctgtttgctcatttgggtgttgagtggagtccaggagcagtcggccctgctgttgctggcctcggcgctgtcagatgcgggaagcttgagcccgtctcctgggctgctcaggggcaccaagaggccctcagcctctgccacgttcccagcgtagtccatttttggctggggatcgtcaggcttgtcttctgacttgtgcccaagtttttctgtagcactgccatctgggtctgccccccgggcattgctgccacttccaactgccgtgagctccaccttggaaaaactgctgctgacacaaaactcctgagatccaaagtgctggcagtcgcctgtcgttgactcctcatcagaaagaggtgctcttctggggcaagagaagcaaaaaaggcaagggggatcaccacgggcctctccccatcttttcagggatccagaaggggctaaccgagggggaaaggcttgttccctttaaaaggcagttggactggcagaagtgggagggctccactgctggaagtgactctcctcgttgatgccacacatgcgaatccggtcagaactggtccagttgtgcacgccgctgtagagcggtgctgtagagatcatgacagccactcaccaccagataggacctgctgtggccactccccctccttctcctctctctcggcggcggcggcggtcggactctaggaactgagaggaagaagggagggctcagcaaagcggaggagagacagagccacacactggcagcagccgcggcgagcgaaagagtgag

SEQ ID NO: 16880 - RNA, 7054 nt, Homo sapiens
  source 1..7054: mol_type = other RNA
tacgtagatatatatgtatttttttttcttaaaaagggaaaacaactgttcaaaaccaactgggcagtatggtgggggtggggagcagtcctacagaagggggccgagaacttcccccccaggaacaaagaacaaacacaatacaaagaaaataaccaccaatgctcccgcatggctcaggagcctctagagaacagattgtcccatcctcaaactggctttttttttttccttttttttttaatcttttttttttccattttcttttttgttgttgttgttttagcacctgtacaataaaactgtaccatctccaaccagagccggccacggcgaggccctcctgcctttggatggtacatactctacaaggattgttcggaaaaatagcaattggtagaaaaataagagtgggagggacaatgccacagagggggcggggacagggaagcaacccaagctcctctctctctctcactcgacaaacccagcgctggaggcccagaggccagggggaggccaggtagggataccactcagccccaggcccccaggcatgagtggagcaagggctggagaccactttcctgcccttgcctaggaaacagctgacgcctggatttcacatccggcagtgagtcccagagccctctgcagattcccaaggagaatgaggggctgagggaggaggtgggaggagaggaaggaaaggggtgctgtgagtctcagaaggggcagggatgggggtggctgagggctgggaggtgagaggctcagtatcttgagacagggaggccagaacggggtgggagagtggaggcaggaacaaactcgtattgtgcactctgaggggggcagtgaagaaggcgtgaggaggggggccaccctcacccctcagatcccttctccacgctcctttattagagtaacttattaacccctcacctcacaatcctcccctccctgtcaacactaatctcaagatagcggggctgctgcaaagggcgggaatgggtgggtgggggagcaccaaagcctcaggatttacccccaagcccccagccctgggccagcagcaaccagcttcgttagtcacaagtccatgttcccccaccccattccacctcaccccctccccagtgggggaaaaaaacaccagggaatagctttgtcagagctcatcaacaaagaaaaagaaaaggaggtacagaaagtccctcaatacaacaagttgtctcaaatcgtcacagtgatacagacttatcagaaaccaatgaaacaatacaaattaaatactaataaaataaatactacagaagacagaagaacacaggggaatggagttggggggcgctcagagatctgggattttctcatttctcctcgggacaggccaaggccatccagggcccaggtttggtcttggtcatgaacaaggaggccagtccaagggaccccggcgccacctcccaccacccccgggacctcttgtcctcagacatggagttcaactttccacccccatcagcaaccacgataacaatgacgacgacagggagatgagaactaattgtaaccaaaaaaacaaaaacagtccagtcgctaatgctggcattgataaggcggcttcttgttggtccgtattattgcctcattctgcagtctggtgctcggtcggggaaagacaaggaggtgggggaagggcgaactcggaaggagaaagaagaggaggggctgttttcccggtcaactgttgcaagactggaattccacctcggaccctaggagccgaagtaggtctggctcgtaccgcaccagctccacagtctcagaggagcctgggggggatctgtcgtccaagcctccaggcctctcggcaggggtcagcagctgactggaggccacctgcctgtagaactcggccttgggcatggtggtgatttcaaagtgcgggaaccgggcctgaaagatcctcgaggaaagcttcagcctcttcaagacatcggaaaagaggaaccagttgcagggcccgcgggacactgacacttggaggttgtagcaagggagaagaggcttgtctgagagttcaaacatgaaatcatcctcctccatcggatcgtctccttcttgatctgagctcccaggaggattatgtaggaggtcacaggcaaacccgtctttttcctccaacacagaactgctgtaaaaatcccaggatacaccgggatcaccctctgcccggccctgaagatccgagaggtgatcactgagaaagcgcttcatggtgtcgctgctggccagcttcatggctgtctgacccgagtaggtagccagtgtgggatcggccccataggacagcaggagccagatggtctccaggttgtcattgaccaccgcatcatgaactggcctcgtgccgtcctgcgcactgcagttcacgttggccccgtgctccagcaggatgttcaggatgtcggtccagccccgggaacaagcctcatgcagggctgtgtagccagcattgtcacggtgattcacatcttcactgtctttctggaggcagtagagaacaacatcctttgcctcttctgagacggttgccatgtgcttggtcttgcactttcgttttcctgatggcttttctgaattttcaaggcaggctggctcttccaggttatttgggaggaaaccgtttggtgaatccgagatcccctggactttgttgggcaagagaaggttcctgttcctgaggcggtgctccaaactttgggaggaggaagtcttctgcttacgggcctttaaatctgctctccctttccgccgctgctcgtcttcttgctctgtcaggtactccccagtctgatattttcggctcttctgccgtcttcgtttcttcctcttcagcaggccctcctcctcttcttcctcctcctcctcattggtgtcccacatttgccgggcagcctctgtcctccagggcatttctcgggctcgccacaggtgccttcggccctggctcagcagagacttgtcctgggcatggtggctgcgatactgggtgtcccgttgggtctttctcacctttcgacgcttagctggggtgggggttacctcctcttcttcttctgtggggaagacttcctggcttcccatgtcactgtctgccatgccagcaaaggagctacagatgcttccagactgactgcgcgtgcgggtgctcagaaccacaggaataaagtcacggaaactgctctttgctttcttttccaaggaaccttcctcgtggctgtcggctcgttttcctggagactgggactccggctttgtcggcttccggtgcttgtgctttcccctgactccattgtgctcttttcctgaatctgaagcccccctggggcttttcttggtggattcctgggggtcactgggcagcttccggcacttgggtctgtgggaactccggaccacggccttggcttgtggctggagctgctgctcttcactgtccttctctttgccgcacttcatcttcttgggcggcagagattccgtcacatcatctggctgccacttgttcttgcaagcaaagacccctacgctttcctgtttcactcgagcctgcccggccttagcccgaacttcagcttggcccctctggggagccactgggaggccatcagcccggaagcaggtggctaaattgaagaccacatcaccatccaccttctccattttcactcgccccagatccacctggcttccaagctgtgggcgctctgtgctggagcccctcctgctgctcggaaccacgtccaatataagttccttggggtggctgtcgtgaggtagcaaaggcagctcaggcatcttaggcaggttctggggggtggccaggaccagctcatgggacatgtaggtggccagcacttggttcttaggcttcgtgtctcctgccagcttcaggccacaagccccctgggggccttccatcttaggagtgctgtcagagcagaggtggctctctgattcctcaggcccctgattcattcgaatgtccccaccgctaggctgaacagacagtgccagggtcccagtctgagggctgagggtcaagaggacaggattgacttgttcttcataaggcttggcagcaatccggcaagttttgttctttgtaacagggtcctgctctggaacgaaggagcccccaggccgtggttgcccctcaggaagtccgtgcacggcttcgctggagctgagagatggcacaccagaaaactccgaaacaacgctggtgggcctgatgggcgccccctgactgggggtcagctgcccggcactggaaatgccaatggaaagcagagacgcctggtggtacggggaccagccaacaggcaggacctgggtgctggtaggtttcccattgactgaacaccggggataaatatttgccggccccgtgggtttccacaaagagagttccttggtttggcaccctggcagcccaggggcaatgcgggctggagtatatcgtttcactgtgcttggctgtccctcagcaccagcctggctgccctttttgccacacgtggcaccagtgcccttaggctctccttgatcaatgatggagatgggctcctgcttggggagatggcgggggtcacggttgaggcccaggttggggtctttgttcagcagcagggatgcaggcactgggttggccactcccacgtaggtgccaggaatggtgctgatcagtgcagttgagttcttcacccaggtgctcgggtccccattcctcacgatctcgggaaagatgacaaagggcgaggaagtggagcccaggcaggaggtgacattgccaccggcagcctgggttgtgcgctgagacctagacaggactgtggagaggagggccttgctgctggtgtgcacgggggtcaacacaggcatggggggtgtcttgcgctggttcggcaatggaagcttctggcggttggacttggaggacagatcaaggggcatctcgctgcactcaggtggagaggccatctctcgttccagctgtggcggtgacttaagaggagagaaggtaacggaagtcccttctgtttgctgctcggtgccactgggcatcttggcggggtgcggtggggctgagctcccactgggggctggcagcagaggctgtggagttggaagcaccttggcagaagcagtaacaagggaggtatctgccaaaggcccagggaccccatcgggtgcaggctgggtggtggtgctaccggatggggaagtgcaggggagcctgttcacctccagagataccagcttggaatccgaagtcagaggccgggccacagaaaatgcatacgggtaagaacggagctcgggggaggctagcacgcctgggagacacctgtcctgcaggtaggacggcaggacagggagcgtaagagtggaggaaacccctagagtggttggcagtgtggccacactgagtggctgcccacagcttggaggcgggatatataccagcggctggctcggggtcagcactgtccctggctgaaaggacagggggactttttgcatagctggtgcctgagctgcaggaaagcacactctactcaaactgaaggaggccgggatgggtgcagaggtgggaatggcagctggcgtggcagcaggcatgggtgtaggggctggagtaaagatgggggctggggtgggtgcaggcaccggtgtaggagcaaaggcggggatgagggtgggggtagaaggtgggccggaagatggggttggagtgggcatgggcacagacggaggggcaggggccgctggaggcgtggatgctggcatgggagccagaaccggagtggggacgggagcgagaaccaaggtcggagctgaagggggcacaggagcctggatgagagccaagggaggagctgaaactgggactgaaagcggggcaggagctggagccgacaagggaaccgggcctgaagggggagcagaagctggcacaggcaccaagactgaggccgaaacagaaagggggttcgagtcagagatgagcgtgggcactgacggtggcgctggagccagagccgggacaggtgctaagggaggggaaggagctggaaccgaagtggcaacttggactggaacaagccctgaatgggggactggggcagggacggagaggggaacctggaatgcatctggaacagagtggggcacagaggccgaaccgggagcagggggacagataggggctggcagaggactgaagttagtggtaaccaggggcagggtcccctccacagggactccagttcccagagttgccaaaatgaaagtattcttctctccaacaccttgccgagagtccaaagcctttactccggcgggtgagcagtcaacctgtttgctcatttgggtgttgagtggagtccaggagcagtcggccctgctgttgctggcctcggcgctgtcagatgcgggaagcttgagcccgtctcctgggctgctcaggggcaccaagaggccctcagcctctgccacgttcccagcgtagtccatttttggctggggatcgtcaggcttgtcttctgacttgtgcccaagtttttctgtagcactgccatctgggtctgccccccgggcattgctgccacttccaactgccgtgagctccaccttggaaaaactgctgctgacacaaaactcctgagatccaaagtgctggcagtcgcctgtcgttgactcctcatcagaaagaggtgctcttctctcctcgttgatgccacacatgcgaatccggtcagaactggtccagttgtgcacgccgctgtagagcggtgctgtagagatcatgacagccactcaccaccagataggacctgctgtggccactccccctccttctcctctctctcggcggcggcggcggtcggactctaggaactgagaggaagaagggagggctcagcaaagcggaggagagacagagccacacactggcagcagccgcggcgagcgaaagagt

SEQ ID NO: 16881 - RNA, 4929 nt, Homo sapiens
  source 1..4929: mol_type = other RNA
tacgtagatatatatgtatttttttttttacagaaacaaaaataagatttcactaatgacactgaataccatatcatagatatgctgcaacagtccaaattcaagaagaaacatgtcaatgtaaatgtgcaaaaggctagcttactctaaactattcaaactttgttcactttatgttctacagacaggtaaatcctgactttaaacacagaaccttgaaaccctcctcagaacagtaagtgaaatggaacagatctttccctccccaagaaaacaaagccttgttgcaagctaatgaaaagatacattaaaacacacacacacacacacacacacacacacacacacacacaatgtatagtatgctttcaacagtataataaacattgaaaatttttatgggagtcaaaacaatgccccattatttaaaaactggctcttttagtctaaattcaagatgcagctctgtcaggcttctctaagcccgacgactgaaaagcagggaagacagacgcaggacttcgactggcagatacaacaatctgagagagagatggagagagtgaagaaaccttagatgctggagtatttatggtattcaaaatggctccttctgggctaaccaacaattttttgacaggtgggtccaaatgaaacactgaagtgctacttggcagtggaggattactggggcaaatggcagaaaccaaagatgtcttagccaaaagagtagctggagacttaattactgaagtcagtgatactgttggtacaggaggtggaacaggaaccttagcagttgtgtttatgagttgtggtgatgtatgtactgtgggtatagaacttgcattcccaaaagagtttataaattttgtagggcttcttagaggatgttgtagaggttggccacttaaggaattatttgatgctagtgtgatcttctgggcagagttatctattggtgtagattgaatgccttggccactgttaagaactaagggggctccatattttggattagtagatataaggagaacatggctgccagctccaagaccttgtggtggaacaataaaccgggttccgttaatcataatctgagtaccaggtgccaaaggtgtactggtattgatgactattttttgctgaatacaaggttcactgaactgactcccgactagactagttacattggatggtgccgaagccgtgtgaatggtagtgccacctggagcagaactgtaactgggggtttttactaaagcttgctgatttggcagagaagcaaaattggacgtattagttattttacctggacttgttgaaagggacgacaattcagtttgaggtttatttgtgtttacatttgttggcactgtagttgaaatccctggtgaatggaactggagtgaagtccgagattgtcttttagaaatagatacagaacgtgtggctcctggtactgctgccgaatgtggaactgtgtttattattttaggggatgtagtcgcaggtgtaggtaaggcaaccgtaacaggaatttgcaaagctgatgttaaacatttaggagacactactggttgtgtagttgaaatcagaacagatgatgcaaggtgtcctgttttcacagttgatatagccacagtgtttccgagacttgatgagcaaagtctatttgacaaaataggcataattcttgaagaggtatcatttccactgactaaaacaggaggttgtgccccagctgaagcagaggctgaggtcactggaaaggaacccaaagataaatttgctccggtaactgaaagcacatttactgctcttgctgaagaaaccactgattcattaacaggggtaatattctgactcacaaaatttgagcttactggaactgaattaccacttgttgacaatggcaaaatatagcccttgctacttttgtcttctccttttggggttacattttgtaatatgttaattgatggtatagctggcacagtgcctgaagtatttacaattgcttgacctatgtttagtccaattttcacatcctttatctgagacacagctggtgatgaatttatttttattggtgtgcccactgtagacggaatcagtactatttggggttgctctggagtcttaacatatgctttatgcaatggaggaggaagagtttgttttaatgattctgcaacaagagttggggttgatgtaccactaggaactggggcattaataaaaactaatttctgggcagaaacacctgtagatgtcagcgcaggtgtcatattaattgcagttccattgccagaagaaagaatagatggagctgataccagcataagtttctgaactggagtcccactgattacatctccatttgttgctgctgttgcttctgaccttgtaacagggtaactttttgtgatataatctacttgttgctgtttagttggagtatgaataatatttgcattgttttgtccaaaatttgctgctgatatgctaattacacttaccgaactacttgttgttgatggtagtagagtactagaacaaatagaggacttcaagggagaagagggcatgtgtgaagttttatctatcacgtggcccaaatcaccactgccagtggtgtggcctaatgtaagtttgagatttttccccatggatggggcaaagctagctggaatggaaacagaagttggtgtttggctaaaaggtgaaagactagatgtagtagttgttccagctacaggtgaaaaagcagaggaagaagttgttgattttggcaccagaaatgcctgcagctgaggagcaaaagtgaaaactgaacttgaagatacagtattgggtgaattttgatctgggttggtctgtacttttacaactccagtgttcccacctcgtgtcctaacaagaattgactgtgaatctcttatgcacacagttttcagctcttgctttgcttcagaagaatcagcagtctgttgtgcaaaacagttgaaggaactaccaggatttgtagacccatttagtgttgttgttgatgacagaggctgacctgtggaggaaatggtcggtgaagcactgggcaaggagaatgtggctgctgaaactgcattcttggcttttcctgcctcactctggctagtcttaactgatggtgttaataagttacttacagaggttacaggcgacaaaggctgtggtctagcactacttatatttgataaaggtgtaattgttttgttgaaagctgtatttggtagttgggtagaaacagttcctggtgagttgacaaaaactgatgctaaagaagaatttatatttgttgtctgtgggaaagatgaacaatgttgttctgtacctttctgttgaagtggtggcacttcttttgcaactgcttttccttctttatgctgaatcacaaaattcttaggcagaataagaacttgctgcatgattttttctcctgttttaggatccaccataggctgcacctgaatctttacagagctattttgaagatctattggcaaccactggccacagggcattttgtataccatttgtaaaggaccttttgtattggtgtggcaggtcaatgctggctttatcgggcttgcttccggaggagataaaactggtttttccacagcaagagcatttctacctgtggaaggaggcagttgatttgttaaggtcactttattcccaatattctttgcaagcaaagcctgaatgggtttggtccctttctggagagtagacactggtactgaatccaatgaggcaaatgactctggaaatgatggctctgtatgctttgattcactgaaacagtcaatctgcacatcactttctagattctcaactgttgtctcatttgtgcttaactttgccttcttccttggagaaagctcttttgtgctgtcatccacataatcagtttgtttggactgtcgtttaagtgttttaagcagtgtcttcggtaagtcttttgaaggcaattcctttttcaacagcttgcttctagccataggaaaatctatttctgacaacttcatatcatctgaatcaaagtgatctttctccaggatatccagaggttctgttgagtctatagacttactgatttctcccttaggagagtcttttccaagatctccttcaccttcatcagtggtccatagttctctattaaatgtatcatgatcaggttgtcttctgaaatcatcatagtctttcttcaggcggctcctgtttctttggaaagccttcattaactttggttcccatggcagcaattcatttaaaagacgtatcaatgtactatgtaattcttttacagcttgcctccgatgataccattttcccagatttgtgcttcttgtgttttgctttttttttgatgatcaataacttattctggatctcaggtttgtaagacttgaatgcaagagaatgaagaccttcacgctttctctgtaagttttcattcaaaacatctttcaatttcttttttttctttttcttcttttttgccctcattttagttagtttgagtttcttgtggctctgtagtgactgctctaatagaatatcccttacaactttgtggcagttaatttctggatgatcactgtgacttccatttacatgtatttggcaagattttagagtattttcttttaatggactgggttcaatctttattctggaagcttcaccgtatttttcctgattttctataaaccttatttcacctggactaagaggctctccaaagccagtaacttcccctggactccttggtttctctaaattttctttacaacaatcagtttttttaatttcacaaggcctgcgaattctaatttcatagttggattttactcccatttcaacagagatgtcatgatt

SEQ ID NO: 16882 - RNA, 4826 nt, Homo sapiens
  source 1..4826: mol_type = other RNA
tacgtagatatatatgtatttttttttttacagaaacaaaaataagatttcactaatgacactgaataccatatcatagatatgctgcaacagtccaaattcaagaagaaacatgtcaatgtaaatgtgcaaaaggctagcttactctaaactattcaaactttgttcactttatgttctacagacaggtaaatcctgactttaaacacagaaccttgaaaccctcctcagaacagtaagtgaaatggaacagatctttccctccccaagaaaacaaagccttgttgcaagctaatgaaaagatacattaaaacacacacacacacacacacacacacacacacacacacacaatgtatagtatgctttcaacagtataataaacattgaaaatttttatgggagtcaaaacaatgccccattatttaaaaactggctcttttagtctaaattcaagatgcagctctgtcaggcttctctaagcccgacgactgaaaagcagggaagacagacgcaggacttcgactggcagatacaacaatctgagagagagatggagagagtgaagaaaccttagatgctggagtatttatggtattcaaaatggctccttctgggctaaccaacaattttttgacaggtgggtccaaatgaaacactgaagtgctacttggcagtggaggattactggggcaaatggcagaaaccaaagatgtcttagccaaaagagtagctggagacttaattactgaagtcagtgatactgttggtacaggaggtggaacaggaaccttagcagttgtgtttatgagttgtggtgatgtatgtactgtgggtatagaacttgcattcccaaaagagtttataaattttgtagggcttcttagaggatgttgtagaggttggccacttaaggaattatttgatgctagtgtgatcttctgggcagagttatctattggtgtagattgaatgccttggccactgttaagaactaagggggctccatattttggattagtagatataaggagaacatggctgccagctccaagaccttgtggtggaacaataaaccgggttccgttaatcataatctgagtaccaggtgccaaaggtgtactggtattgatgactattttttgctgaatacaaggttcactgaactgactcccgactagactagttacattggatggtgccgaagccgtgtgaatggtagtgccacctggagcagaactgtaactgggggtttttactaaagcttgctgatttggcagagaagcaaaattggacgtattagttattttacctggacttgttgaaagggacgacaattcagtttgaggtttatttgtgtttacatttgttggcactgtagttgaaatccctggtgaatggaactggagtgaagtccgagattgtcttttagaaatagatacagaacgtgtggctcctggtactgctgccgaatgtggaactgtgtttattattttaggggatgtagtcgcaggtgtaggtaaggcaaccgtaacaggaatttgcaaagctgatgttaaacatttaggagacactactggttgtgtagttgaaatcagaacagatgatgcaaggtgtcctgttttcacagttgatatagccacagtgtttccgagacttgatgagcaaagtctatttgacaaaataggcataattcttgaagaggtatcatttccactgactaaaacaggaggttgtgccccagctgaagcagaggctgaggtcactggaaaggaacccaaagataaatttgctccggtaactgaaagcacatttactgctcttgctgaagaaaccactgattcattaacaggggtaatattctgactcacaaaatttgagcttactggaactgaattaccacttgttgacaatggcaaaatatagcccttgctacttttgtcttctccttttggggttacattttgtaatatgttaattgatggtatagctggcacagtgcctgaagtatttacaattgcttgacctatgtttagtccaattttcacatcctttatctgagacacagctggtgatgaatttatttttattggtgtgcccactgtagacggaatcagtactatttggggttgctctggagtcttaacatatgctttatgcaatggaggaggaagagtttgttttaatgattctgcaacaagagttggggttgatgtaccactaggaactggggcattaataaaaactaatttctgggcagaaacacctgtagatgtcagcgcaggtgtcatattaattgcagttccattgccagaagaaagaatagatggagctgataccagcataagtttctgaactggagtcccactgattacatctccatttgttgctgctgttgcttctgaccttgtaacagggtaactttttgtgatataatctacttgttgctgtttagttggagtatgaataatatttgcattgttttgtccaaaatttgctgctgatatgctaattacacttaccgaactacttgttgttgatggtagtagagtactagaacaaatagaggacttcaagggagaagagggcatgtgtgaagttttatctatcacgtggcccaaatcaccactgccagtggtgtggcctaatgtaagtttgagatttttccccatggatggggcaaagctagctggaatggaaacagaagttggtgtttggctaaaaggtgaaagactagatgtagtagttgttccagctacaggtgaaaaagcagaggaagaagttgttgattttggcaccagaaatgcctgcagctgaggagcaaaagtgaaaactgaacttgaagatacagtattgggtgaattttgatctgggttggtctgtacttttacaactccagtgttcccacctcgtgtcctaacaagaattgactgtgaatctcttatgcacacagttttcagctcttgctttgcttcagaagaatcagcagtctgttgtgcaaaacagttgaaggaactaccaggatttgtagacccatttagtgttgttgttgatgacagaggctgacctgtggaggaaatggtcggtgaagcactgggcaaggagaatgtggctgctgaaactgcattcttggcttttcctgcctcactctggctagtcttaactgatggtgttaataagttacttacagaggttacaggcgacaaaggctgtggtctagcactacttatatttgataaaggtgtaattgttttgttgaaagctgtatttggtagttgggtagaaacagttcctggtgagttgacaaaaactgatgctaaagaagaatttatatttgttgtctgtgggaaagatgaacaatgttgttctgtacctttctgttgaagtggtggcacttcttttgcaactgcttttccttctttatgctgaatcacaaaattcttaggcagaataagaacttgctgcatgattttttctcctgttttaggatccaccataggctgcacctgaatctttacagagctattttgaagatctattggcaaccactggccacagggcattttgtataccatttgtaaaggaccttttgtattggtgtggcaggtcaatgctggctttatcgggcttgcttccggaggagataaaactggtttttccacagcaagagcatttctacctgtggaaggaggcagttgatttgttaaggtcactttattcccaatattctttgcaagcaaagcctgaatgggtttggtccctttctggagagtagacactggtactgaatccaatgaggcaaatgactctggaaatgatggctctgtatgctttgattcactgaaacagtcaatctgcacatcactttctagattctcaactgttgtctcatttgtgcttaactttgccttcttccttggagaaagctcttttgtgctgtcatccacataatcagtttgtttggactgtcgtttaagtgttttaagcagtgtcttcggtaagtcttttgaaggcaattcctttttcaacagcttgcttctagccataggaaaatctatttctgacaacttcatatcatctgaatcaaagtgatctttctccaggatatccagaggttctgttgagtctatagacttactgatttctcccttaggagagtcttttccaagatctccttcaccttcatcagtggtccatagttctctattaaatgtatcatgatcaggttgtcttctgaaatcatcatagtctttcttcaggcggctcctgtttctttggaaagccttcattaactttggttcccatggcagcaattcatttaaaagacgtatcaatgtactatgtaattcttttacagcttgcctccgatgataccattttccccactaatctgttttgaaatgtctgttatcttttaacattatatgttttgtggccttcttctctttctttatgtattttcagtctggggtagtggtggtatagtacttcattcataatttgaaaatgcttattaaatcattctttcatgctttctcatccaatgtccacggcagctgcagattgccagctccctttccataagatggcccaactaccaaacactggaggttttataaccccatagggattgctacaacaaggaactggtctatggtcacaagattaagtccttcattatatcatgcagttttataagtctttgaatgtaacagattaataacttaaggaatcataaaggaaaataaaaaataacttacaaaactacacaatattgtaaaaagaaaagctgcatctctatgtatgtgaaatgagtcgggagggaa

SEQ ID NO: 16883 - RNA, 7459 nt, Homo sapiens
  source 1..7459: mol_type = other RNA
tacgtagatatatatgtatttttttttttacagaaacaaaaataagatttcactaatgacactgaataccatatcatagatatgctgcaacagtccaaattcaagaagaaacatgtcaatgtaaatgtgcaaaaggctagcttactctaaactattcaaactttgttcactttatgttctacagacaggtaaatcctgactttaaacacagaaccttgaaaccctcctcagaacagtaagtgaaatggaacagatctttccctccccaagaaaacaaagccttgttgcaagctaatgaaaagatacattaaaacacacacacacacacacacacacacacacacacacacacaatgtatagtatgctttcaacagtataataaacattgaaaatttttatgggagtcaaaacaatgccccattatttaaaaactggctcttttagtctaaattcaagatgcagctctgtcaggcttctctaagcccgacgactgaaaagcagggaagacagacgcaggacttcgactggcagatacaacaatctgagagagagatggagagagtgaagaaaccttagatgctggagtatttatggtattcaaaatggctccttctgggctaaccaacaattttttgacaggtgggtccaaatgaaacactgaagtgctacttggcagtggaggattactggggcaaatggcagaaaccaaagatgtcttagccaaaagagtagctggagacttaattactgaagtcagtgatactgttggtacaggaggtggaacaggaaccttagcagttgtgtttatgagttgtggtgatgtatgtactgtgggtatagaacttgcattcccaaaagagtttataaattttgtagggcttcttagaggatgttgtagaggttggccacttaaggaattatttgatgctagtgtgatcttctgggcagagttatctattggtgtagattgaatgccttggccactgttaagaactaagggggctccatattttggattagtagatataaggagaacatggctgccagctccaagaccttgtggtggaacaataaaccgggttccgttaatcataatctgagtaccaggtgccaaaggtgtactggtattgatgactattttttgctgaatacaaggttcactgaactgactcccgactagactagttacattggatggtgccgaagccgtgtgaatggtagtgccacctggagcagaactgtaactgggggtttttactaaagcttgctgatttggcagagaagcaaaattggacgtattagttattttacctggacttgttgaaagggacgacaattcagtttgaggtttatttgtgtttacatttgttggcactgtagttgaaatccctggtgaatggaactggagtgaagtccgagattgtcttttagaaatagatacagaacgtgtggctcctggtactgctgccgaatgtggaactgtgtttattattttaggggatgtagtcgcaggtgtaggtaaggcaaccgtaacaggaatttgcaaagctgatgttaaacatttaggagacactactggttgtgtagttgaaatcagaacagatgatgcaaggtgtcctgttttcacagttgatatagccacagtgtttccgagacttgatgagcaaagtctatttgacaaaataggcataattcttgaagaggtatcatttccactgactaaaacaggaggttgtgccccagctgaagcagaggctgaggtcactggaaaggaacccaaagataaatttgctccggtaactgaaagcacatttactgctcttgctgaagaaaccactgattcattaacaggggtaatattctgactcacaaaatttgagcttactggaactgaattaccacttgttgacaatggcaaaatatagcccttgctacttttgtcttctccttttggggttacattttgtaatatgttaattgatggtatagctggcacagtgcctgaagtatttacaattgcttgacctatgtttagtccaattttcacatcctttatctgagacacagctggtgatgaatttatttttattggtgtgcccactgtagacggaatcagtactatttggggttgctctggagtcttaacatatgctttatgcaatggaggaggaagagtttgttttaatgattctgcaacaagagttggggttgatgtaccactaggaactggggcattaataaaaactaatttctgggcagaaacacctgtagatgtcagcgcaggtgtcatattaattgcagttccattgccagaagaaagaatagatggagctgataccagcataagtttctgaactggagtcccactgattacatctccatttgttgctgctgttgcttctgaccttgtaacagggtaactttttgtgatataatctacttgttgctgtttagttggagtatgaataatatttgcattgttttgtccaaaatttgctgctgatatgctaattacacttaccgaactacttgttgttgatggtagtagagtactagaacaaatagaggacttcaagggagaagagggcatgtgtgaagttttatctatcacgtggcccaaatcaccactgccagtggtgtggcctaatgtaagtttgagatttttccccatggatggggcaaagctagctggaatggaaacagaagttggtgtttggctaaaaggtgaaagactagatgtagtagttgttccagctacaggtgaaaaagcagaggaagaagttgttgattttggcaccagaaatgcctgcagctgaggagcaaaagtgaaaactgaacttgaagatacagtattgggtgaattttgatctgggttggtctgtacttttacaactccagtgttcccacctcgtgtcctaacaagaattgactgtgaatctcttatgcacacagttttcagctcttgctttgcttcagaagaatcagcagtctgttgtgcaaaacagttgaaggaactaccaggatttgtagacccatttagtgttgttgttgatgacagaggctgacctgtggaggaaatggtcggtgaagcactgggcaaggagaatgtggctgctgaaactgcattcttggcttttcctgcctcactctggctagtcttaactgatggtgttaataagttacttacagaggttacaggcgacaaaggctgtggtctagcactacttatatttgataaaggtgtaattgttttgttgaaagctgtatttggtagttgggtagaaacagttcctggtgagttgacaaaaactgatgctaaagaagaatttatatttgttgtctgtgggaaagatgaacaatgttgttctgtacctttctgttgaagtggtggcacttcttttgcaactgcttttccttctttatgctgaatcacaaaattcttaggcagaataagaacttgctgcatgattttttctcctgttttaggatccaccataggctgcacctgaatctttacagagctattttgaagatctattggcaaccactggccacagggcattttgtataccatttgtaaaggaccttttgtattggtgtggcaggtcaatgctggctttatcgggcttgcttccggaggagataaaactggtttttccacagcaagagcatttctacctgtggaaggaggcagttgatttgttaaggtcactttattcccaatattctttgcaagcaaagcctgaatgggtttggtccctttctggagagtagacactggtactgaatccaatgaggcaaatgactctggaaatgatggctctgtatgctttgattcactgaaacagtcaatctgcacatcactttctagattctcaactgttgtctcatttgtgcttaactttgccttcttccttggagaaagctcttttgtgctgtcatccacataatcagtttgtttggactgtcgtttaagtgttttaagcagtgtcttcggtaagtcttttgaaggcaattcctttttcaacagcttgcttctagccataggaaaatctatttctgacaacttcatatcatctgaatcaaagtgatctttctccaggatatccagaggttctgttgagtctatagacttactgatttctcccttaggagagtcttttccaagatctccttcaccttcatcagtggtccatagttctctattaaatgtatcatgatcaggttgtcttctgaaatcatcatagtctttcttcaggcggctcctgtttctttggaaagccttcattaactttggttcccatggcagcaattcatttaaaagacgtatcaatgtactatgtaattcttttacagcttgcctccgatgataccattttcccgatttttttctactgttttccagatctttgagttcattctcgatttttgtgattaattccctgagttcatcaagattagtgcaaataagctgaaactctggtacagtaggtgactttatgacagttttcctcttctttgtgattgcttttttagagacggatttttttccagatttgtgcttcttgtgttttgctttttttttgatgatcaataacttattctggatctcaggtttgtaagacttgaatgcaagagaatgaagaccttcacgctttctctgtaagttttcattcaaaacatctttcaatttcttttttttctttttcttcttttttgccctcattttagttagtttgagtttcttgtggctctgtagtgactgctctaatagaatatcccttacaactttgtggcagttaatttctggatgatcactgtgacttccatttacatgtatttggcaagattttagagtattttcttttaatggactgggttcaatctttattctggaagcttcaccgtatttttcctgattttctataaaccttatttcacctggactaagaggctctccaaagccagtaacttcccctggactccttggtttctctaaattttctttacaacaatcagtttttttaatttcacaaggcctgcgaattctaatttcatagttggattttactcccatttcaacagagatgtcatgattatccaagatcattttagcaggacagcaagctggatcaaaattattttcctgctctttcttgaaggaagagggcaggctatctctgctacatctatgttctccattacttgtactaacatagtcacacttcaatttctccaatttaatccgaggtactctttgtattttaatgggtggaattggaaattctggggcctgaaagggtctctgtttataaatccgtacatctgcaccacagaactgtggaaaatgtacataagcattctccaaataatcataaccaagaataacttccctgcattcatggataggctgtccaagtacagcatcttgaacttccttttgtgtttcatacacaaagtcacaaagacccttaagtagccacactttttggtaaaaaggtagttcgtgaaaaggtttttcttccaatggattaacttctccaagaactttaaaaaactgaggacacaaccccagtttttcagcacagttatcaggattttcagtttgccctacagcagtgtaccactgttgtactttctgcctcagcgctgcttcccaggtcctataaggcaaagtaggtcttcgatgtaaggtaggtctgcgatggggaggacttaatagagaagtcattattttcgatagaaaagcattacactgaggcatcagaagacaacgttccaattcgtaaaagactatttctggcaaatttagaatttgctgagctaaacaaaggaaatgcccaatagctggaatttcccacatggtctccatacaagttggagctgcttgagctagaagttttctttcccattcttctatttccttttgactagcttcttctgcttcttttctttcctgctcccgaagccttttttcttcttttgctctcagctgttcttcctgtctcaaaacttgaaccattatagattcaaaaactccacttgtcaagcctgccaaacttcgcggtgttgaccgacgccttgttgaggtacatgcagttcccttctcatcctccaatccataatagcctctagatgtaactgctatcgttgtcttttctctcaagtgccgagagagaagcgctaacttctgctccagcatcatctccagcttctggccctgtttggagatccagtggtccactccgtgcaggcggtagcacgtctccagcatcaacctgaagtccgccacgaactcggtgatgcccccgtactggccgctggcgaacttctcttccatctgcagcagacacatgccctgtccgggctgctgcgggaaggcgcgaccgccccggcccccgctgcgcggcccttccgccacctcctcctccgcggtggcaacgccccccaagggctgcagaaagggggcggtgaggccccggtgcttctcctgcaggaactcgcccaggatgcggtagccctgctgtagctcgtaggtcagctcctgctccttgcagcaaccgcctccgatcaccatcgcctccatctcttcctcctgatcgtccgcgtcctccagcgaggaggcactccttccgtgggccggccctgaggtctgggccgccgctgccacctcctcctcgtcgtcctctccttcggccgccggtggcggccgctcttcctccccagccggctccatcgctcccggcgtcccgggcacactcatgccccggcaggcctaggctgggcggtgtggaacagccgctcgaggtgctgggggacgcgtgagcgcgagccgcttcctcacggctcggccgcggcgcgtagcccccgccacatcgggcctggctctcctcagccgccggctcggctcggtgcgcgcgggggtcttgagctcaccgccggcggggcggggttacatggcgcgcgaggaggggggagagaagaggagagcctaggtgccctcctctcccctcccccccggcggcggcgcgcgcacggccctcgccggcctcacccctccgcaccccgcccgcctgctcttcaccggccaggccctgccgggtcgccgcggcctcggcgccccaccccctcccgggccagcggggggctgggagggggcgaggaggaagggggttctcctctcccctccccggagggggccgcagcggcggctccggctcctcctctccctcacaccccctcccgcccccctctacctgcgggggacacgggcagaaggaggcggtgcacggacggggcccggcgacaactgtcagttagaagccccgctgggcggtgaggggggagaaaggggaggggcagggagagaagggggagggcactcagccccccggctgggaagagctgtggagagaagcaaagaaagaggccctgtcgccatccccggtgcgcatgcgt

SEQ ID NO: 16884 - RNA, 5004 nt, Homo sapiens
  source 1..5004: mol_type = other RNA
tacgtagatatatatgtatttttttttttacagaaacaaaaataagatttcactaatgacactgaataccatatcatagatatgctgcaacagtccaaattcaagaagaaacatgtcaatgtaaatgtgcaaaaggctagcttactctaaactattcaaactttgttcactttatgttctacagacaggtaaatcctgactttaaacacagaaccttgaaaccctcctcagaacagtaagtgaaatggaacagatctttccctccccaagaaaacaaagccttgttgcaagctaatgaaaagatacattaaaacacacacacacacacacacacacacacacacacacacacaatgtatagtatgctttcaacagtataataaacattgaaaatttttatgggagtcaaaacaatgccccattatttaaaaactggctcttttagtctaaattcaagatgcagctctgtcaggcttctctaagcccgacgactgaaaagcagggaagacagacgcaggacttcgactggcagatacaacaatctgagagagagatggagagagtgaagaaaccttagatgctggagtatttatggtattcaaaatggctccttctgggctaaccaacaattttttgacaggtgggtccaaatgaaacactgaagtgctacttggcagtggaggattactggggcaaatggcagaaaccaaagatgtcttagccaaaagagtagctggagacttaattactgaagtcagtgatactgttggtacaggaggtggaacaggaaccttagcagttgtgtttatgagttgtggtgatgtatgtactgtgggtatagaacttgcattcccaaaagagtttataaattttgtagggcttcttagaggatgttgtagaggttggccacttaaggaattatttgatgctagtgtgatcttctgggcagagttatctattggtgtagattgaatgccttggccactgttaagaactaagggggctccatattttggattagtagatataaggagaacatggctgccagctccaagaccttgtggtggaacaataaaccgggttccgttaatcataatctgagtaccaggtgccaaaggtgtactggtattgatgactattttttgctgaatacaaggttcactgaactgactcccgactagactagttacattggatggtgccgaagccgtgtgaatggtagtgccacctggagcagaactgtaactgggggtttttactaaagcttgctgatttggcagagaagcaaaattggacgtattagttattttacctggacttgttgaaagggacgacaattcagtttgaggtttatttgtgtttacatttgttggcactgtagttgaaatccctggtgaatggaactggagtgaagtccgagattgtcttttagaaatagatacagaacgtgtggctcctggtactgctgccgaatgtggaactgtgtttattattttaggggatgtagtcgcaggtgtaggtaaggcaaccgtaacaggaatttgcaaagctgatgttaaacatttaggagacactactggttgtgtagttgaaatcagaacagatgatgcaaggtgtcctgttttcacagttgatatagccacagtgtttccgagacttgatgagcaaagtctatttgacaaaataggcataattcttgaagaggtatcatttccactgactaaaacaggaggttgtgccccagctgaagcagaggctgaggtcactggaaaggaacccaaagataaatttgctccggtaactgaaagcacatttactgctcttgctgaagaaaccactgattcattaacaggggtaatattctgactcacaaaatttgagcttactggaactgaattaccacttgttgacaatggcaaaatatagcccttgctacttttgtcttctccttttggggttacattttgtaatatgttaattgatggtatagctggcacagtgcctgaagtatttacaattgcttgacctatgtttagtccaattttcacatcctttatctgagacacagctggtgatgaatttatttttattggtgtgcccactgtagacggaatcagtactatttggggttgctctggagtcttaacatatgctttatgcaatggaggaggaagagtttgttttaatgattctgcaacaagagttggggttgatgtaccactaggaactggggcattaataaaaactaatttctgggcagaaacacctgtagatgtcagcgcaggtgtcatattaattgcagttccattgccagaagaaagaatagatggagctgataccagcataagtttctgaactggagtcccactgattacatctccatttgttgctgctgttgcttctgaccttgtaacagggtaactttttgtgatataatctacttgttgctgtttagttggagtatgaataatatttgcattgttttgtccaaaatttgctgctgatatgctaattacacttaccgaactacttgttgttgatggtagtagagtactagaacaaatagaggacttcaagggagaagagggcatgtgtgaagttttatctatcacgtggcccaaatcaccactgccagtggtgtggcctaatgtaagtttgagatttttccccatggatggggcaaagctagctggaatggaaacagaagttggtgtttggctaaaaggtgaaagactagatgtagtagttgttccagctacaggtgaaaaagcagaggaagaagttgttgattttggcaccagaaatgcctgcagctgaggagcaaaagtgaaaactgaacttgaagatacagtattgggtgaattttgatctgggttggtctgtacttttacaactccagtgttcccacctcgtgtcctaacaagaattgactgtgaatctcttatgcacacagttttcagctcttgctttgcttcagaagaatcagcagtctgttgtgcaaaacagttgaaggaactaccaggatttgtagacccatttagtgttgttgttgatgacagaggctgacctgtggaggaaatggtcggtgaagcactgggcaaggagaatgtggctgctgaaactgcattcttggcttttcctgcctcactctggctagtcttaactgatggtgttaataagttacttacagaggttacaggcgacaaaggctgtggtctagcactacttatatttgataaaggtgtaattgttttgttgaaagctgtatttggtagttgggtagaaacagttcctggtgagttgacaaaaactgatgctaaagaagaatttatatttgttgtctgtgggaaagatgaacaatgttgttctgtacctttctgttgaagtggtggcacttcttttgcaactgcttttccttctttatgctgaatcacaaaattcttaggcagaataagaacttgctgcatgattttttctcctgttttaggatccaccataggctgcacctgaatctttacagagctattttgaagatctattggcaaccactggccacagggcattttgtataccatttgtaaaggaccttttgtattggtgtggcaggtcaatgctggctttatcgggcttgcttccggaggagataaaactggtttttccacagcaagagcatttctacctgtggaaggaggcagttgatttgttaaggtcactttattcccaatattctttgcaagcaaagcctgaatgggtttggtccctttctggagagtagacactggtactgaatccaatgaggcaaatgactctggaaatgatggctctgtatgctttgattcactgaaacagtcaatctgcacatcactttctagattctcaactgttgtctcatttgtgcttaactttgccttcttccttggagaaagctcttttgtgctgtcatccacataatcagtttgtttggactgtcgtttaagtgttttaagcagtgtcttcggtaagtcttttgaaggcaattcctttttcaacagcttgcttctagccataggaaaatctatttctgacaacttcatatcatctgaatcaaagtgatctttctccaggatatccagaggttctgttgagtctatagacttactgatttctcccttaggagagtcttttccaagatctccttcaccttcatcagtggtccatagttctctattaaatgtatcatgatcaggttgtcttctgaaatcatcatagtctttcttcaggcggctcctgtttctttggaaagccttcattaactttggttcccatggcagcaattcatttaaaagacgtatcaatgtactatgtaattcttttacagcttgcctccgatgataccattttccctcacaactaaagaacaactgcattctgctacagtaatctgggatgggtatgacagcaccagcataacactggctggagtgtggcaaggagagggagttggcaatctactgatgctggggacattggataccgatttttttctactgttttccagatctttgagttcattctcgatttttgtgattaattccctgagttcatcaagattagtgcaaataagctgaaactctggtacagtaggtgactttatgacagttttcctcttctttgtgattgcttttttagagacggatttttttccagatttgtgcttcttgtgttttgctttttttttgatgatcaataacttattctggatctcaggtttgtaagacttgaatgcaagagaatgaagaccttcacgctttctctgtaagttttcattcaaaacatctttcaatttcttttttttctttttcttcttttttgccctcattttagttagtttgagtttcttgtggctctgtagtgactgctctaatagaatatcccttacaactttgtggcagttaatttctggatgatcactgtgacttccatttacatgtatttggcaagattttagagtattttcttttaatg

SEQ ID NO: 16885 - RNA, 7597 nt, Homo sapiens
  source 1..7597: mol_type = other RNA
tacgtagatatatatgtatttttttttttacagaaacaaaaataagatttcactaatgacactgaataccatatcatagatatgctgcaacagtccaaattcaagaagaaacatgtcaatgtaaatgtgcaaaaggctagcttactctaaactattcaaactttgttcactttatgttctacagacaggtaaatcctgactttaaacacagaaccttgaaaccctcctcagaacagtaagtgaaatggaacagatctttccctccccaagaaaacaaagccttgttgcaagctaatgaaaagatacattaaaacacacacacacacacacacacacacacacacacacacacaatgtatagtatgctttcaacagtataataaacattgaaaatttttatgggagtcaaaacaatgccccattatttaaaaactggctcttttagtctaaattcaagatgcagctctgtcaggcttctctaagcccgacgactgaaaagcagggaagacagacgcaggacttcgactggcagatacaacaatctgagagagagatggagagagtgaagaaaccttagatgctggagtatttatggtattcaaaatggctccttctgggctaaccaacaattttttgacaggtgggtccaaatgaaacactgaagtgctacttggcagtggaggattactggggcaaatggcagaaaccaaagatgtcttagccaaaagagtagctggagacttaattactgaagtcagtgatactgttggtacaggaggtggaacaggaaccttagcagttgtgtttatgagttgtggtgatgtatgtactgtgggtatagaacttgcattcccaaaagagtttataaattttgtagggcttcttagaggatgttgtagaggttggccacttaaggaattatttgatgctagtgtgatcttctgggcagagttatctattggtgtagattgaatgccttggccactgttaagaactaagggggctccatattttggattagtagatataaggagaacatggctgccagctccaagaccttgtggtggaacaataaaccgggttccgttaatcataatctgagtaccaggtgccaaaggtgtactggtattgatgactattttttgctgaatacaaggttcactgaactgactcccgactagactagttacattggatggtgccgaagccgtgtgaatggtagtgccacctggagcagaactgtaactgggggtttttactaaagcttgctgatttggcagagaagcaaaattggacgtattagttattttacctggacttgttgaaagggacgacaattcagtttgaggtttatttgtgtttacatttgttggcactgtagttgaaatccctggtgaatggaactggagtgaagtccgagattgtcttttagaaatagatacagaacgtgtggctcctggtactgctgccgaatgtggaactgtgtttattattttaggggatgtagtcgcaggtgtaggtaaggcaaccgtaacaggaatttgcaaagctgatgttaaacatttaggagacactactggttgtgtagttgaaatcagaacagatgatgcaaggtgtcctgttttcacagttgatatagccacagtgtttccgagacttgatgagcaaagtctatttgacaaaataggcataattcttgaagaggtatcatttccactgactaaaacaggaggttgtgccccagctgaagcagaggctgaggtcactggaaaggaacccaaagataaatttgctccggtaactgaaagcacatttactgctcttgctgaagaaaccactgattcattaacaggggtaatattctgactcacaaaatttgagcttactggaactgaattaccacttgttgacaatggcaaaatatagcccttgctacttttgtcttctccttttggggttacattttgtaatatgttaattgatggtatagctggcacagtgcctgaagtatttacaattgcttgacctatgtttagtccaattttcacatcctttatctgagacacagctggtgatgaatttatttttattggtgtgcccactgtagacggaatcagtactatttggggttgctctggagtcttaacatatgctttatgcaatggaggaggaagagtttgttttaatgattctgcaacaagagttggggttgatgtaccactaggaactggggcattaataaaaactaatttctgggcagaaacacctgtagatgtcagcgcaggtgtcatattaattgcagttccattgccagaagaaagaatagatggagctgataccagcataagtttctgaactggagtcccactgattacatctccatttgttgctgctgttgcttctgaccttgtaacagggtaactttttgtgatataatctacttgttgctgtttagttggagtatgaataatatttgcattgttttgtccaaaatttgctgctgatatgctaattacacttaccgaactacttgttgttgatggtagtagagtactagaacaaatagaggacttcaagggagaagagggcatgtgtgaagttttatctatcacgtggcccaaatcaccactgccagtggtgtggcctaatgtaagtttgagatttttccccatggatggggcaaagctagctggaatggaaacagaagttggtgtttggctaaaaggtgaaagactagatgtagtagttgttccagctacaggtgaaaaagcagaggaagaagttgttgattttggcaccagaaatgcctgcagctgaggagcaaaagtgaaaactgaacttgaagatacagtattgggtgaattttgatctgggttggtctgtacttttacaactccagtgttcccacctcgtgtcctaacaagaattgactgtgaatctcttatgcacacagttttcagctcttgctttgcttcagaagaatcagcagtctgttgtgcaaaacagttgaaggaactaccaggatttgtagacccatttagtgttgttgttgatgacagaggctgacctgtggaggaaatggtcggtgaagcactgggcaaggagaatgtggctgctgaaactgcattcttggcttttcctgcctcactctggctagtcttaactgatggtgttaataagttacttacagaggttacaggcgacaaaggctgtggtctagcactacttatatttgataaaggtgtaattgttttgttgaaagctgtatttggtagttgggtagaaacagttcctggtgagttgacaaaaactgatgctaaagaagaatttatatttgttgtctgtgggaaagatgaacaatgttgttctgtacctttctgttgaagtggtggcacttcttttgcaactgcttttccttctttatgctgaatcacaaaattcttaggcagaataagaacttgctgcatgattttttctcctgttttaggatccaccataggctgcacctgaatctttacagagctattttgaagatctattggcaaccactggccacagggcattttgtataccatttgtaaaggaccttttgtattggtgtggcaggtcaatgctggctttatcgggcttgcttccggaggagataaaactggtttttccacagcaagagcatttctacctgtggaaggaggcagttgatttgttaaggtcactttattcccaatattctttgcaagcaaagcctgaatgggtttggtccctttctggagagtagacactggtactgaatccaatgaggcaaatgactctggaaatgatggctctgtatgctttgattcactgaaacagtcaatctgcacatcactttctagattctcaactgttgtctcatttgtgcttaactttgccttcttccttggagaaagctcttttgtgctgtcatccacataatcagtttgtttggactgtcgtttaagtgttttaagcagtgtcttcggtaagtcttttgaaggcaattcctttttcaacagcttgcttctagccataggaaaatctatttctgacaacttcatatcatctgaatcaaagtgatctttctccaggatatccagaggttctgttgagtctatagacttactgatttctcccttaggagagtcttttccaagatctccttcaccttcatcagtggtccatagttctctattaaatgtatcatgatcaggttgtcttctgaaatcatcatagtctttcttcaggcggctcctgtttctttggaaagccttcattaactttggttcccatggcagcaattcatttaaaagacgtatcaatgtactatgtaattcttttacagcttgcctccgatgataccattttccctcacaactaaagaacaactgcattctgctacagtaatctgggatgggtatgacagcaccagcataacactggctggagtgtggcaaggagagggagttggcaatctactgatgctggggacattggataccgatttttttctactgttttccagatctttgagttcattctcgatttttgtgattaattccctgagttcatcaagattagtgcaaataagctgaaactctggtacagtaggtgactttatgacagttttcctcttctttgtgattgcttttttagagacggatttttttccagatttgtgcttcttgtgttttgctttttttttgatgatcaataacttattctggatctcaggtttgtaagacttgaatgcaagagaatgaagaccttcacgctttctctgtaagttttcattcaaaacatctttcaatttcttttttttctttttcttcttttttgccctcattttagttagtttgagtttcttgtggctctgtagtgactgctctaatagaatatcccttacaactttgtggcagttaatttctggatgatcactgtgacttccatttacatgtatttggcaagattttagagtattttcttttaatggactgggttcaatctttattctggaagcttcaccgtatttttcctgattttctataaaccttatttcacctggactaagaggctctccaaagccagtaacttcccctggactccttggtttctctaaattttctttacaacaatcagtttttttaatttcacaaggcctgcgaattctaatttcatagttggattttactcccatttcaacagagatgtcatgattatccaagatcattttagcaggacagcaagctggatcaaaattattttcctgctctttcttgaaggaagagggcaggctatctctgctacatctatgttctccattacttgtactaacatagtcacacttcaatttctccaatttaatccgaggtactctttgtattttaatgggtggaattggaaattctggggcctgaaagggtctctgtttataaatccgtacatctgcaccacagaactgtggaaaatgtacataagcattctccaaataatcataaccaagaataacttccctgcattcatggataggctgtccaagtacagcatcttgaacttccttttgtgtttcatacacaaagtcacaaagacccttaagtagccacactttttggtaaaaaggtagttcgtgaaaaggtttttcttccaatggattaacttctccaagaactttaaaaaactgaggacacaaccccagtttttcagcacagttatcaggattttcagtttgccctacagcagtgtaccactgttgtactttctgcctcagcgctgcttcccaggtcctataaggcaaagtaggtcttcgatgtaaggtaggtctgcgatggggaggacttaatagagaagtcattattttcgatagaaaagcattacactgaggcatcagaagacaacgttccaattcgtaaaagactatttctggcaaatttagaatttgctgagctaaacaaaggaaatgcccaatagctggaatttcccacatggtctccatacaagttggagctgcttgagctagaagttttctttcccattcttctatttccttttgactagcttcttctgcttcttttctttcctgctcccgaagccttttttcttcttttgctctcagctgttcttcctgtctcaaaacttgaaccattatagattcaaaaactccacttgtcaagcctgccaaacttcgcggtgttgaccgacgccttgttgaggtacatgcagttcccttctcatcctccaatccataatagcctctagatgtaactgctatcgttgtcttttctctcaagtgccgagagagaagcgctaacttctgctccagcatcatctccagcttctggccctgtttggagatccagtggtccactccgtgcaggcggtagcacgtctccagcatcaacctgaagtccgccacgaactcggtgatgcccccgtactggccgctggcgaacttctcttccatctgcagcagacacatgccctgtccgggctgctgcgggaaggcgcgaccgccccggcccccgctgcgcggcccttccgccacctcctcctccgcggtggcaacgccccccaagggctgcagaaagggggcggtgaggccccggtgcttctcctgcaggaactcgcccaggatgcggtagccctgctgtagctcgtaggtcagctcctgctccttgcagcaaccgcctccgatcaccatcgcctccatctcttcctcctgatcgtccgcgtcctccagcgaggaggcactccttccgtgggccggccctgaggtctgggccgccgctgccacctcctcctcgtcgtcctctccttcggccgccggtggcggccgctcttcctccccagccggctccatcgctcccggcgtcccgggcacactcatgccccggcaggcctaggctgggcggtgtggaacagccgctcgaggtgctgggggacgcgtgagcgcgagccgcttcctcacggctcggccgcggcgcgtagcccccgccacatcgggcctggctctcctcagccgccggctcggctcggtgcgcgcgggggtcttgagctcaccgccggcggggcggggttacatggcgcgcgaggaggggggagagaagaggagagcctaggtgccctcctctcccctcccccccggcggcggcgcgcgcacggccctcgccggcctcacccctccgcaccccgcccgcctgctcttcaccggccaggccctgccgggtcgccgcggcctcggcgccccaccccctcccgggccagcggggggctgggagggggcgaggaggaagggggttctcctctcccctccccggagggggccgcagcggcggctccggctcctcctctccctcacaccccctcccgcccccctctacctgcgggggacacgggcagaaggaggcggtgcacggacggggcccggcgacaactgtcagttagaagccccgctgggcggtgaggggggagaaaggggaggggcagggagagaagggggagggcactcagccccccggctgggaagagctgtggagagaagcaaagaaagaggccctgtcgccatccccggtgcgcatgcgtagtagaa

SEQ ID NO: 16886 - RNA, 7375 nt, Homo sapiens
  source 1..7375: mol_type = other RNA
tacgtagatatatatgtatttttttttttacagaaacaaaaataagatttcactaatgacactgaataccatatcatagatatgctgcaacagtccaaattcaagaagaaacatgtcaatgtaaatgtgcaaaaggctagcttactctaaactattcaaactttgttcactttatgttctacagacaggtaaatcctgactttaaacacagaaccttgaaaccctcctcagaacagtaagtgaaatggaacagatctttccctccccaagaaaacaaagccttgttgcaagctaatgaaaagatacattaaaacacacacacacacacacacacacacacacacacacacacaatgtatagtatgctttcaacagtataataaacattgaaaatttttatgggagtcaaaacaatgccccattatttaaaaactggctcttttagtctaaattcaagatgcagctctgtcaggcttctctaagcccgacgactgaaaagcagggaagacagacgcaggacttcgactggcagatacaacaatctgagagagagatggagagagtgaagaaaccttagatgctggagtatttatggtattcaaaatggctccttctgggctaaccaacaattttttgacaggtgggtccaaatgaaacactgaagtgctacttggcagtggaggattactggggcaaatggcagaaaccaaagatgtcttagccaaaagagtagctggagacttaattactgaagtcagtgatactgttggtacaggaggtggaacaggaaccttagcagttgtgtttatgagttgtggtgatgtatgtactgtgggtatagaacttgcattcccaaaagagtttataaattttgtagggcttcttagaggatgttgtagaggttggccacttaaggaattatttgatgctagtgtgatcttctgggcagagttatctattggtgtagattgaatgccttggccactgttaagaactaagggggctccatattttggattagtagatataaggagaacatggctgccagctccaagaccttgtggtggaacaataaaccgggttccgttaatcataatctgagtaccaggtgccaaaggtgtactggtattgatgactattttttgctgaatacaaggttcactgaactgactcccgactagactagttacattggatggtgccgaagccgtgtgaatggtagtgccacctggagcagaactgtaactgggggtttttactaaagcttgctgatttggcagagaagcaaaattggacgtattagttattttacctggacttgttgaaagggacgacaattcagtttgaggtttatttgtgtttacatttgttggcactgtagttgaaatccctggtgaatggaactggagtgaagtccgagattgtcttttagaaatagatacagaacgtgtggctcctggtactgctgccgaatgtggaactgtgtttattattttaggggatgtagtcgcaggtgtaggtaaggcaaccgtaacaggaatttgcaaagctgatgttaaacatttaggagacactactggttgtgtagttgaaatcagaacagatgatgcaaggtgtcctgttttcacagttgatatagccacagtgtttccgagacttgatgagcaaagtctatttgacaaaataggcataattcttgaagaggtatcatttccactgactaaaacaggaggttgtgccccagctgaagcagaggctgaggtcactggaaaggaacccaaagataaatttgctccggtaactgaaagcacatttactgctcttgctgaagaaaccactgattcattaacaggggtaatattctgactcacaaaatttgagcttactggaactgaattaccacttgttgacaatggcaaaatatagcccttgctacttttgtcttctccttttggggttacattttgtaatatgttaattgatggtatagctggcacagtgcctgaagtatttacaattgcttgacctatgtttagtccaattttcacatcctttatctgagacacagctggtgatgaatttatttttattggtgtgcccactgtagacggaatcagtactatttggggttgctctggagtcttaacatatgctttatgcaatggaggaggaagagtttgttttaatgattctgcaacaagagttggggttgatgtaccactaggaactggggcattaataaaaactaatttctgggcagaaacacctgtagatgtcagcgcaggtgtcatattaattgcagttccattgccagaagaaagaatagatggagctgataccagcataagtttctgaactggagtcccactgattacatctccatttgttgctgctgttgcttctgaccttgtaacagggtaactttttgtgatataatctacttgttgctgtttagttggagtatgaataatatttgcattgttttgtccaaaatttgctgctgatatgctaattacacttaccgaactacttgttgttgatggtagtagagtactagaacaaatagaggacttcaagggagaagagggcatgtgtgaagttttatctatcacgtggcccaaatcaccactgccagtggtgtggcctaatgtaagtttgagatttttccccatggatggggcaaagctagctggaatggaaacagaagttggtgtttggctaaaaggtgaaagactagatgtagtagttgttccagctacaggtgaaaaagcagaggaagaagttgttgattttggcaccagaaatgcctgcagctgaggagcaaaagtgaaaactgaacttgaagatacagtattgggtgaattttgatctgggttggtctgtacttttacaactccagtgttcccacctcgtgtcctaacaagaattgactgtgaatctcttatgcacacagttttcagctcttgctttgcttcagaagaatcagcagtctgttgtgcaaaacagttgaaggaactaccaggatttgtagacccatttagtgttgttgttgatgacagaggctgacctgtggaggaaatggtcggtgaagcactgggcaaggagaatgtggctgctgaaactgcattcttggcttttcctgcctcactctggctagtcttaactgatggtgttaataagttacttacagaggttacaggcgacaaaggctgtggtctagcactacttatatttgataaaggtgtaattgttttgttgaaagctgtatttggtagttgggtagaaacagttcctggtgagttgacaaaaactgatgctaaagaagaatttatatttgttgtctgtgggaaagatgaacaatgttgttctgtacctttctgttgaagtggtggcacttcttttgcaactgcttttccttctttatgctgaatcacaaaattcttaggcagaataagaacttgctgcatgattttttctcctgttttaggatccaccataggctgcacctgaatctttacagagctattttgaagatctattggcaaccactggccacagggcattttgtataccatttgtaaaggaccttttgtattggtgtggcaggtcaatgctggctttatcgggcttgcttccggaggagataaaactggtttttccacagcaagagcatttctacctgtggaaggaggcagttgatttgttaaggtcactttattcccaatattctttgcaagcaaagcctgaatgggtttggtccctttctggagagtagacactggtactgaatccaatgaggcaaatgactctggaaatgatggctctgtatgctttgattcactgaaacagtcaatctgcacatcactttctagattctcaactgttgtctcatttgtgcttaactttgccttcttccttggagaaagctcttttgtgctgtcatccacataatcagtttgtttggactgtcgtttaagtgttttaagcagtgtcttcggtaagtcttttgaaggcaattcctttttcaacagcttgcttctagccataggaaaatctatttctgacaacttcatatcatctgaatcaaagtgatctttctccaggatatccagaggttctgttgagtctatagacttactgatttctcccttaggagagtcttttccaagatctccttcaccttcatcagtggtccatagttctctattaaatgtatcatgatcaggttgtcttctgaaatcatcatagtctttcttcaggcggctcctgtttctttggaaagccttcattaactttggttcccatggcagcaattcatttaaaagacgtatcaatgtactatgtaattcttttacagcttgcctccgatgataccattttccctgaaactctggtacagtaggtgactttatgacagttttcctcttctttgtgattgcttttttagagacggatttttttccagatttgtgcttcttgtgttttgctttttttttgatgatcaataacttattctggatctcaggtttgtaagacttgaatgcaagagaatgaagaccttcacgctttctctgtaagttttcattcaaaacatctttcaatttcttttttttctttttcttcttttttgccctcattttagttagtttgagtttcttgtggctctgtagtgactgctctaatagaatatcccttacaactttgtggcagttaatttctggatgatcactgtgacttccatttacatgtatttggcaagattttagagtattttcttttaatggactgggttcaatctttattctggaagcttcaccgtatttttcctgattttctataaaccttatttcacctggactaagaggctctccaaagccagtaacttcccctggactccttggtttctctaaattttctttacaacaatcagtttttttaatttcacaaggcctgcgaattctaatttcatagttggattttactcccatttcaacagagatgtcatgattatccaagatcattttagcaggacagcaagctggatcaaaattattttcctgctctttcttgaaggaagagggcaggctatctctgctacatctatgttctccattacttgtactaacatagtcacacttcaatttctccaatttaatccgaggtactctttgtattttaatgggtggaattggaaattctggggcctgaaagggtctctgtttataaatccgtacatctgcaccacagaactgtggaaaatgtacataagcattctccaaataatcataaccaagaataacttccctgcattcatggataggctgtccaagtacagcatcttgaacttccttttgtgtttcatacacaaagtcacaaagacccttaagtagccacactttttggtaaaaaggtagttcgtgaaaaggtttttcttccaatggattaacttctccaagaactttaaaaaactgaggacacaaccccagtttttcagcacagttatcaggattttcagtttgccctacagcagtgtaccactgttgtactttctgcctcagcgctgcttcccaggtcctataaggcaaagtaggtcttcgatgtaaggtaggtctgcgatggggaggacttaatagagaagtcattattttcgatagaaaagcattacactgaggcatcagaagacaacgttccaattcgtaaaagactatttctggcaaatttagaatttgctgagctaaacaaaggaaatgcccaatagctggaatttcccacatggtctccatacaagttggagctgcttgagctagaagttttctttcccattcttctatttccttttgactagcttcttctgcttcttttctttcctgctcccgaagccttttttcttcttttgctctcagctgttcttcctgtctcaaaacttgaaccattatagattcaaaaactccacttgtcaagcctgccaaacttcgcggtgttgaccgacgccttgttgaggtacatgcagttcccttctcatcctccaatccataatagcctctagatgtaactgctatcgttgtcttttctctcaagtgccgagagagaagcgctaacttctgctccagcatcatctccagcttctggccctgtttggagatccagtggtccactccgtgcaggcggtagcacgtctccagcatcaacctgaagtccgccacgaactcggtgatgcccccgtactggccgctggcgaacttctcttccatctgcagcagacacatgccctgtccgggctgctgcgggaaggcgcgaccgccccggcccccgctgcgcggcccttccgccacctcctcctccgcggtggcaacgccccccaagggctgcagaaagggggcggtgaggccccggtgcttctcctgcaggaactcgcccaggatgcggtagccctgctgtagctcgtaggtcagctcctgctccttgcagcaaccgcctccgatcaccatcgcctccatctcttcctcctgatcgtccgcgtcctccagcgaggaggcactccttccgtgggccggccctgaggtctgggccgccgctgccacctcctcctcgtcgtcctctccttcggccgccggtggcggccgctcttcctccccagccggctccatcgctcccggcgtcccgggcacactcatgccccggcaggcctaggctgggcggtgtggaacagccgctcgaggtgctgggggacgcgtgagcgcgagccgcttcctcacggctcggccgcggcgcgtagcccccgccacatcgggcctggctctcctcagccgccggctcggctcggtgcgcgcgggggtcttgagctcaccgccggcggggcggggttacatggcgcgcgaggaggggggagagaagaggagagcctaggtgccctcctctcccctcccccccggcggcggcgcgcgcacggccctcgccggcctcacccctccgcaccccgcccgcctgctcttcaccggccaggccctgccgggtcgccgcggcctcggcgccccaccccctcccgggccagcggggggctgggagggggcgaggaggaagggggttctcctctcccctccccggagggggccgcagcggcggctccggctcctcctctccctcacaccccctcccgcccccctctacctgcgggggacacgggcagaaggaggcggtgcacggacggggcccggcgacaactgtcagttagaagccccgctgggcggtgaggggggagaaaggggaggggcagggagagaagggggagggcactcagccccccggctgggaagagctgtggagagaagcaaagaaagaggccctgtcgccatccccggtgcgcatgcgtagtaga

SEQ ID NO: 16887 - RNA, 4578 nt, Homo sapiens
  source 1..4578: mol_type = other RNA
tacgtagatatatatgtatttttttttttacagaaacaaaaataagatttcactaatgacactgaataccatatcatagatatgctgcaacagtccaaattcaagaagaaacatgtcaatgtaaatgtgcaaaaggctagcttactctaaactattcaaactttgttcactttatgttctacagacaggtaaatcctgactttaaacacagaaccttgaaaccctcctcagaacagtaagtgaaatggaacagatctttccctccccaagaaaacaaagccttgttgcaagctaatgaaaagatacattaaaacacacacacacacacacacacacacacacacacacacacaatgtatagtatgctttcaacagtataataaacattgaaaatttttatgggagtcaaaacaatgccccattatttaaaaactggctcttttagtctaaattcaagatgcagctctgtcaggcttctctaagcccgacgactgaaaagcagggaagacagacgcaggacttcgactggcagatacaacaatctgagagagagatggagagagtgaagaaaccttagatgctggagtatttatggtattcaaaatggctccttctgggctaaccaacaattttttgacaggtgggtccaaatgaaacactgaagtgctacttggcagtggaggattactggggcaaatggcagaaaccaaagatgtcttagccaaaagagtagctggagacttaattactgaagtcagtgatactgttggtacaggaggtggaacaggaaccttagcagttgtgtttatgagttgtggtgatgtatgtactgtgggtatagaacttgcattcccaaaagagtttataaattttgtagggcttcttagaggatgttgtagaggttggccacttaaggaattatttgatgctagtgtgatcttctgggcagagttatctattggtgtagattgaatgccttggccactgttaagaactaagggggctccatattttggattagtagatataaggagaacatggctgccagctccaagaccttgtggtggaacaataaaccgggttccgttaatcataatctgagtaccaggtgccaaaggtgtactggtattgatgactattttttgctgaatacaaggttcactgaactgactcccgactagactagttacattggatggtgccgaagccgtgtgaatggtagtgccacctggagcagaactgtaactgggggtttttactaaagcttgctgatttggcagagaagcaaaattggacgtattagttattttacctggacttgttgaaagggacgacaattcagtttgaggtttatttgtgtttacatttgttggcactgtagttgaaatccctggtgaatggaactggagtgaagtccgagattgtcttttagaaatagatacagaacgtgtggctcctggtactgctgccgaatgtggaactgtgtttattattttaggggatgtagtcgcaggtgtaggtaaggcaaccgtaacaggaatttgcaaagctgatgttaaacatttaggagacactactggttgtgtagttgaaatcagaacagatgatgcaaggtgtcctgttttcacagttgatatagccacagtgtttccgagacttgatgagcaaagtctatttgacaaaataggcataattcttgaagaggtatcatttccactgactaaaacaggaggttgtgccccagctgaagcagaggctgaggtcactggaaaggaacccaaagataaatttgctccggtaactgaaagcacatttactgctcttgctgaagaaaccactgattcattaacaggggtaatattctgactcacaaaatttgagcttactggaactgaattaccacttgttgacaatggcaaaatatagcccttgctacttttgtcttctccttttggggttacattttgtaatatgttaattgatggtatagctggcacagtgcctgaagtatttacaattgcttgacctatgtttagtccaattttcacatcctttatctgagacacagctggtgatgaatttatttttattggtgtgcccactgtagacggaatcagtactatttggggttgctctggagtcttaacatatgctttatgcaatggaggaggaagagtttgttttaatgattctgcaacaagagttggggttgatgtaccactaggaactggggcattaataaaaactaatttctgggcagaaacacctgtagatgtcagcgcaggtgtcatattaattgcagttccattgccagaagaaagaatagatggagctgataccagcataagtttctgaactggagtcccactgattacatctccatttgttgctgctgttgcttctgaccttgtaacagggtaactttttgtgatataatctacttgttgctgtttagttggagtatgaataatatttgcattgttttgtccaaaatttgctgctgatatgctaattacacttaccgaactacttgttgttgatggtagtagagtactagaacaaatagaggacttcaagggagaagagggcatgtgtgaagttttatctatcacgtggcccaaatcaccactgccagtggtgtggcctaatgtaagtttgagatttttccccatggatggggcaaagctagctggaatggaaacagaagttggtgtttggctaaaaggtgaaagactagatgtagtagttgttccagctacaggtgaaaaagcagaggaagaagttgttgattttggcaccagaaatgcctgcagctgaggagcaaaagtgaaaactgaacttgaagatacagtattgggtgaattttgatctgggttggtctgtacttttacaactccagtgttcccacctcgtgtcctaacaagaattgactgtgaatctcttatgcacacagttttcagctcttgctttgcttcagaagaatcagcagtctgttgtgcaaaacagttgaaggaactaccaggatttgtagacccatttagtgttgttgttgatgacagaggctgacctgtggaggaaatggtcggtgaagcactgggcaaggagaatgtggctgctgaaactgcattcttggcttttcctgcctcactctggctagtcttaactgatggtgttaataagttacttacagaggttacaggcgacaaaggctgtggtctagcactacttatatttgataaaggtgtaattgttttgttgaaagctgtatttggtagttgggtagaaacagttcctggtgagttgacaaaaactgatgctaaagaagaatttatatttgttgtctgtgggaaagatgaacaatgttgttctgtacctttctgttgaagtggtggcacttcttttgcaactgcttttccttctttatgctgaatcacaaaattcttaggcagaataagaacttgctgcatgattttttctcctgttttaggatccaccataggctgcacctgaatctttacagagctattttgaagatctattggcaaccactggccacagggcattttgtataccatttgtaaaggaccttttgtattggtgtggcaggtcaatgctggctttatcgggcttgcttccggaggagataaaactggtttttccacagcaagagcatttctacctgtggaaggaggcagttgatttgttaaggtcactttattcccaatattctttgcaagcaaagcctgaatgggtttggtccctttctggagagtagacactggtactgaatccaatgaggcaaatgactctggaaatgatggctctgtatgctttgattcactgaaacagtcaatctgcacatcactttctagattctcaactgttgtctcatttgtgcttaactttgccttcttccttggagaaagctcttttgtgctgtcatccacataatcagtttgtttggactgtcgtttaagtgttttaagcagtgtcttcggtaagtcttttgaaggcaattcctttttcaacagcttgcttctagccataggaaaatctatttctgacaacttcatatcatctgaatcaaagtgatctttctccaggatatccagaggttctgttgagtctatagacttactgatttctcccttaggagagtcttttccaagatctccttcaccttcatcagtggtccatagttctctattaaatgtatcatgatcaggttgtcttctgaaatcatcatagtctttcttcaggcggctcctgtttctttggaaagccttcattaactttggttcccatggcagcaattcatttaaaagacgtatcaatgtactatgtaattcttttacagcttgcctccgatgataccattttccctgaaactctggtacagtaggtgactttatgacagttttcctcttctttgtgattgcttttttagagacggatttttttcctggttttcctgtcttcactcctcagacctctgggctactcatactcagacttccactttaagccaagtgtggtggtgcatgcctgtgatcccagctcgcctgtggtcccagctac

SEQ ID NO: 16888 - RNA, 4685 nt, Homo sapiens
  source 1..4685: mol_type = other RNA
tacgtagatatatatgtatttttttttttacagaaacaaaaataagatttcactaatgacactgaataccatatcatagatatgctgcaacagtccaaattcaagaagaaacatgtcaatgtaaatgtgcaaaaggctagcttactctaaactattcaaactttgttcactttatgttctacagacaggtaaatcctgactttaaacacagaaccttgaaaccctcctcagaacagtaagtgaaatggaacagatctttccctccccaagaaaacaaagccttgttgcaagctaatgaaaagatacattaaaacacacacacacacacacacacacacacacacacacacacaatgtatagtatgctttcaacagtataataaacattgaaaatttttatgggagtcaaaacaatgccccattatttaaaaactggctcttttagtctaaattcaagatgcagctctgtcaggcttctctaagcccgacgactgaaaagcagggaagacagacgcaggacttcgactggcagatacaacaatctgagagagagatggagagagtgaagaaaccttagatgctggagtatttatggtattcaaaatggctccttctgggctaaccaacaattttttgacaggtgggtccaaatgaaacactgaagtgctacttggcagtggaggattactggggcaaatggcagaaaccaaagatgtcttagccaaaagagtagctggagacttaattactgaagtcagtgatactgttggtacaggaggtggaacaggaaccttagcagttgtgtttatgagttgtggtgatgtatgtactgtgggtatagaacttgcattcccaaaagagtttataaattttgtagggcttcttagaggatgttgtagaggttggccacttaaggaattatttgatgctagtgtgatcttctgggcagagttatctattggtgtagattgaatgccttggccactgttaagaactaagggggctccatattttggattagtagatataaggagaacatggctgccagctccaagaccttgtggtggaacaataaaccgggttccgttaatcataatctgagtaccaggtgccaaaggtgtactggtattgatgactattttttgctgaatacaaggttcactgaactgactcccgactagactagttacattggatggtgccgaagccgtgtgaatggtagtgccacctggagcagaactgtaactgggggtttttactaaagcttgctgatttggcagagaagcaaaattggacgtattagttattttacctggacttgttgaaagggacgacaattcagtttgaggtttatttgtgtttacatttgttggcactgtagttgaaatccctggtgaatggaactggagtgaagtccgagattgtcttttagaaatagatacagaacgtgtggctcctggtactgctgccgaatgtggaactgtgtttattattttaggggatgtagtcgcaggtgtaggtaaggcaaccgtaacaggaatttgcaaagctgatgttaaacatttaggagacactactggttgtgtagttgaaatcagaacagatgatgcaaggtgtcctgttttcacagttgatatagccacagtgtttccgagacttgatgagcaaagtctatttgacaaaataggcataattcttgaagaggtatcatttccactgactaaaacaggaggttgtgccccagctgaagcagaggctgaggtcactggaaaggaacccaaagataaatttgctccggtaactgaaagcacatttactgctcttgctgaagaaaccactgattcattaacaggggtaatattctgactcacaaaatttgagcttactggaactgaattaccacttgttgacaatggcaaaatatagcccttgctacttttgtcttctccttttggggttacattttgtaatatgttaattgatggtatagctggcacagtgcctgaagtatttacaattgcttgacctatgtttagtccaattttcacatcctttatctgagacacagctggtgatgaatttatttttattggtgtgcccactgtagacggaatcagtactatttggggttgctctggagtcttaacatatgctttatgcaatggaggaggaagagtttgttttaatgattctgcaacaagagttggggttgatgtaccactaggaactggggcattaataaaaactaatttctgggcagaaacacctgtagatgtcagcgcaggtgtcatattaattgcagttccattgccagaagaaagaatagatggagctgataccagcataagtttctgaactggagtcccactgattacatctccatttgttgctgctgttgcttctgaccttgtaacagggtaactttttgtgatataatctacttgttgctgtttagttggagtatgaataatatttgcattgttttgtccaaaatttgctgctgatatgctaattacacttaccgaactacttgttgttgatggtagtagagtactagaacaaatagaggacttcaagggagaagagggcatgtgtgaagttttatctatcacgtggcccaaatcaccactgccagtggtgtggcctaatgtaagtttgagatttttccccatggatggggcaaagctagctggaatggaaacagaagttggtgtttggctaaaaggtgaaagactagatgtagtagttgttccagctacaggtgaaaaagcagaggaagaagttgttgattttggcaccagaaatgcctgcagctgaggagcaaaagtgaaaactgaacttgaagatacagtattgggtgaattttgatctgggttggtctgtacttttacaactccagtgttcccacctcgtgtcctaacaagaattgactgtgaatctcttatgcacacagttttcagctcttgctttgcttcagaagaatcagcagtctgttgtgcaaaacagttgaaggaactaccaggatttgtagacccatttagtgttgttgttgatgacagaggctgacctgtggaggaaatggtcggtgaagcactgggcaaggagaatgtggctgctgaaactgcattcttggcttttcctgcctcactctggctagtcttaactgatggtgttaataagttacttacagaggttacaggcgacaaaggctgtggtctagcactacttatatttgataaaggtgtaattgttttgttgaaagctgtatttggtagttgggtagaaacagttcctggtgagttgacaaaaactgatgctaaagaagaatttatatttgttgtctgtgggaaagatgaacaatgttgttctgtacctttctgttgaagtggtggcacttcttttgcaactgcttttccttctttatgctgaatcacaaaattcttaggcagaataagaacttgctgcatgattttttctcctgttttaggatccaccataggctgcacctgaatctttacagagctattttgaagatctattggcaaccactggccacagggcattttgtataccatttgtaaaggaccttttgtattggtgtggcaggtcaatgctggctttatcgggcttgcttccggaggagataaaactggtttttccacagcaagagcatttctacctgtggaaggaggcagttgatttgttaaggtcactttattcccaatattctttgcaagcaaagcctgaatgggtttggtccctttctggagagtagacactggtactgaatccaatgaggcaaatgactctggaaatgatggctctgtatgctttgattcactgaaacagtcaatctgcacatcactttctagattctcaactgttgtctcatttgtgcttaactttgccttcttccttggagaaagctcttttgtgctgtcatccacataatcagtttgtttggactgtcgtttaagtgttttaagcagtgtcttcggtaagtcttttgaaggcaattcctttttcaacagcttgcttctagccataggaaaatctatttctgacaacttcatatcatctgaatcaaagtgatctttctccaggatatccagaggttctgttgagtctatagacttactgatttctcccttaggagagtcttttccaagatctccttcaccttcatcagtggtccatagttctctattaaatgtatcatgatcaggttgtcttctgaaatcatcatagtctttcttcaggcggctcctgtttctttggaaagccttcattaactttggttcccatggcagcaattcatttaaaagacgtatcaatgtactatgtaattcttttacagcttgcctccgatgataccattttccctttcatgctttctcatccaatgtccacggcagctgcagattgccagctccctttccataagatggcccaactaccaaacactggaggttttataaccccatagggattgctacaacaaggaactggtctatggtcacaagattaagtccttcattatatcatgcagttttataagtctttgaatgtaacagattaataacttaaggaatcataaaggaaaataaaaaataacttacaaaactacacaatattgtaaaaagaaaagctgcatctctatgtatgtgaaatgagtcgggagggaa

SEQ ID NO: 16889 - RNA, 2414 nt, Homo sapiens
  source 1..2414: mol_type = other RNA
tactgcagacagtggcaatcagcatgtcctggagaggacacaggatggggagggacaggcagtggggctcaggtgcccttccttcaccccctctttgagggggtaccctaagttggcatggccattctcacatgtgcaaaagcagctggatccatccctgaaatgattttccgctcatgcaatttctatactcttgctttgttccctgaagggtaataatgcggacttctcaaggtcagggactaagttgtactcaggttggtaactccagcgcgtcacacagggcctggtgaacagatggtgccctctaaagattcctgaataaaaaggcaactgtgcagagtacatccaaaagtgggtgggtgtagcatggaaacgtgtggggcagaagagaaaaaacagcctggggctctttctggtcctataaaacagactcaggtcaccgtgggtcatggctaccttttcccactttgatttctgtgtggtagagagaggttttcggtcaaaccatttgaaaatccatccttgtcaatcaaaatgttcaaacatctacaatttaagtttcaatcaaatggtaggcagaggggttaaaaacacttatttcagatgcagaaatctgagtttgaattctgacctctctgcttagaacccatgtgacattgaacatgttactccacatttctcagcttccattcctttgtggacctgcgtagttgtcaagttgtaacaataacacattgcctgtttagctgctactataccttctccaaggttttagcactcagacctggttctattccttttttttcttttttcttttcttgtttttttttttttttttttttttttttgactgagtcttgctctgtcacccagactggagtgcaatggcgctttctcggttcactgcagcctccacctcccaggttccagcaattctcctgcctcagcctcccaggtagctgggattacaggcacgtgccaccatacctggctaatttttgtatttttagtagagacggggtttcaccatgttggtcaggctggtcctgaactcctgacctcaggtgatccatccgcctcagcctcccaaagtgctgggattacaggcgtgagccactgggcccagctggttctattccgttttatttgtcctctatagtcctaaaggtagatcatggccatattttgttagttactaccccactctgcagtgtactttctgcatgatgttagtcattatactgtttgtcattttaaaataagattgaactagaagcttaaaaacagtcattctgttggtttttctattaaaatcagaaattttaatacaggcggaaagtattttttggtatttaattattcaaactaatgggatttttaaaaaccattatgattgacaaagggctgaggcttacaatattttcttttacagatatatgctgctttaatgaaacccaatatgcaaaaatctaaacttaggtaaattggaagctttatctaggcttatattgtttacattacaaaagggctattctgcttcactaaagcatttatttcagtgttccttaaaaagtgagatctctgtggtgcatttagaatacaacttgaatgattaccaggttatttatacacaggtgttttgtgtaaagcaaggttcacctggggagagggttgggctgcactaggaatgactctgtattgtgtaatcagccaatgaagaggaattgagaaaagattttgagtgacatcctcgtagaaggtaagaaaggttcaacatgcgactttcagggccctatctcatcttgatgtgaaggcatctgtcaaatgtaccattatatctctttagcttaaacggagcagtgtttagcgattaaagtaatggaacatgattcaggagtcgtgttttctgtttctgtctcctgtagcttccaagtaggtagtcttgacgtgttcactttaatgccagttcactttaaagcaattatttccatcctaggtgaggcagtaaaatcttgttaatgtttttaatagcctgtgaactcttcagatgaaatatctggcctttgtgccctcctcagcttgtgaaccaattgccagcaagccctctattcaccatgtgtcctcacagttttcgtgagtcatgaatgtgggagccacttagctgggtggttctggcttagtctctcataagattgcagcaaagtcattgcccacggctgcagcatctgaaagcttgactggtgctgaagagtctgcttccagggaggcttgccacactcctggtaagggaatatcggttgtgaggggtgctcagtttttttccacatgggctcctccatacagctgcttgagcatctcacaacatggcagctggttccccccaagcaagtgatccaagggagacagcaaga

SEQ ID NO: 16890 - RNA, 4009 nt, Homo sapiens
  source 1..4009: mol_type = other RNA
tactgcatcaggaactgattggacataaacagtttcactcagaatgagctgttttctatgcacgacactattcaagttactacactccaaccacatttcctctgaacattatttacacaccaaatttcactctggtagcaactaaattttggcacagatgagattaaccactaaaggccacatttgctggtccagttccctagaaagcaatgacacaacaaatttgttaggaagacttggttcaaggggaaaaactgatagcaggagatactttggaaaaagagcacactgacagagtgtctctgccccaaagaactctgcagtctggtattgaaaagtaaattttcaatgaggctgggcgcggtggctcatgcctgtaatcccggcactttgggaggccaaggcggacagatcacttgaggtcagtgtgagaccagccgggctaacaccgtctctgctaaaaatacaaaaattagctgggcacggtggtgcgcacctgtcccagctcttcaggagactgaggtgggagaattgcttgaacctgggagatggagctgagatcacatcactgcactccagcctgggccaaagagcaagactccatctcaaaaagaaaaagaaattgaaccttgggagtttccatacaaattaaatcactagaacaattattgggataaatgtcaaacaaaacgactgatatgaaattctgaataagcctgtaaaacttgtgcttcaatgctaacaaaaaaaaaagttgaacaaatgaggtaaggaactcagtatttgaagataagctaggagcagcatttcctactcaaaagatttaccaagagataaacagttgaagagaattgagtataaatggtgacagcttgcttcccaactagtatgaaagctcaaaaccccttaatacagtaatatatgcaccttatttaatatattaatatataaatcaattttggaaaccagtttgaagttaagccattttgttaagtatgtattgtaaatggtgaaaatttcttcataaatatgcccagacaatgcaggagaccaagaatgcccaggttttaaggccaggctgtttccttttctttttggtaaacccctcagttttgatacattcttctaaaatacacagggctagactctaatagaataaaggaattcatgggggacaacgtgagggcaagtttccgcagactcggaacattttcccaagaggcaagtactgaattgagactaaaagaagctaattctgttctcaaatttctgtaactttaaaacatttgaaaaatgaagatctcctgtggcctttttaagagacttttatttgagtggttcttacaaagattgttgcaatatgaaagtcatttgtttgatagaaatatcaagctgtcttgtcaaacacactgaagtaacccaaaaatatatttcagagctcacagagcttaaaaagagcaaagattatatgcaaccagacaaaacctatttctgcatttcctatttctttctcagactgctttgcctaccagactctcacgtttaaacatcttcaggaaatgcagggatcattttgtttggaattttaagacacaccagaacacatagtatttacaaagaaacttttacagatacattaattgaaaagataccatcaagaaatataattttgaaatctccctttcttgccaattgatcagaatgcaagatgagatgctaaccaaacagccctttagctgtcttgtatttccatacactaaatgtgtatttcagaaactgctcaaccatcagccaaatatcaacattagtgaaatgtgaaatgtaaccactgtgtaaaaagttaggcttctgaaacattaaaaacattacatccctggtctgcctttttacagaaagcacatttgttctcctagagctattcctatagttcattaattttctacatgaacattttaaaaggcagaacaagagaacagttttgtatacagtgggatttactatttagggagaatgagcacactgcattcctgttaacatttttattttttcaaggtaacaggaaattgcatacaaatgacagtagatccttgcctctttatttttatctaaataaaagataactcaagatgaattctcaagaaagaaaaaaagctatatacataagggactatatcttccttcatcgtctacttggaaccagtagctgtgttgctgtcatagaatcaggaaacaggttgtggtaagttggaagaggtacatatgctgctgttatcattttaccagcaaaccacctgccatgcaatgcattgacagcagcaatagctgcagcaattgatgggcacttcacatacacattgccctgagctgaatttttgtcaacataaatatgaataactcctccatgtttattacattcttcaatcacatcatccttaatctcggtatcccatccaacttcttcttctgtttgagggttaaacatgttagagagttggaaacattgtgttgcaagtggctgaacagaggcagctgcagctaaagctgaagcttcagtctgctgggaaagtcttgtttgcaaatcctctgcaagtcttgccattaactgaagacgaccagttgttcccaaatcaattccagtcctttccagttcatcactgtccaaaaatgaactagcactcgaagcatcagtacgttcagtaacatgaccaactttcattggtcttcctgctagttcaaatccattaagttgttccaaagcctttttggcacattctgagtcagaaaatgtaataaatccatatcccttggatcgaccagtttcactgtccatcatcagctggatactttcaattcttccaaaaggctcaaagatcccacgaagcatatcttcagttatgttgaagtgtaatgagcccacataaagcctcataggtccagcacttcccttttgtaaattgtttgccattgctgcagctctgtttttttctgcctgtgatgcctgtactatgattggcacgcctaaaactcgttggccagttaatcctattgctagaggcactgagctaacatcgacgaactccacataagcaattcctttggaacgtcttgaatttctgtcagaaatcatcctcacatctcgaacctttcctactgtagagaaaaactcttccaaatcccttggtcgaattcttgccgccagctgcatacagaagactgtccttgcatctctttcctcaggagttaaattatcaataggttctctcacagggctcttgtcttttctgaatggacttttgcttcgggaacgtcgtctgcttaatttgatgctatgaggcaacccaatctttcctcggatggcactgttaaattttggtccggagtaaggacttctgtagcggcctctaaatcttcgatctcgacttcttgagcggctccgtcgcctctctttgcttctacttcgctttctttcacggcttttgctctttttcctttctctgtctctacttcgcttccgttccttacttttgcttctctttcgttcatgactacgacttctgctcttgctttttttcctctttttgctacgttcttcatggccgttggcactgctcaacttgttctcatccttcttgtaaggagcctcaagcattgcttcaatatcaatatcgtctgccattttctctaaacgcctgttccggccttcgggcgcctgtggtgctcgtgttcgggaagagattgctgctgctgctgctgctgctgccgccgccgccgcttctgttgctactgttaagcccctaggcccaggccgcggaaccgcccagcccgaatatcgggttccaaggacggctaggcccgagagaatctaaaaaaaacaatggaattagagaagcccacgcgggagagcaggacggcggcttcggcagctcaggatccacccctgcgacagcgtcgacaagctccctgaaatggcggccgctgcttccctgtactcacattcaccagcacacat

SEQ ID NO: 16891 - RNA, 4250 nt, Homo sapiens
  source 1..4250: mol_type = other RNA
tactgcatcaggaactgattggacataaacagtttcactcagaatgagctgttttctatgcacgacactattcaagttactacactccaaccacatttcctctgaacattatttacacaccaaatttcactctggtagcaactaaattttggcacagatgagattaaccactaaaggccacatttgctggtccagttccctagaaagcaatgacacaacaaatttgttaggaagacttggttcaaggggaaaaactgatagcaggagatactttggaaaaagagcacactgacagagtgtctctgccccaaagaactctgcagtctggtattgaaaagtaaattttcaatgaggctgggcgcggtggctcatgcctgtaatcccggcactttgggaggccaaggcggacagatcacttgaggtcagtgtgagaccagccgggctaacaccgtctctgctaaaaatacaaaaattagctgggcacggtggtgcgcacctgtcccagctcttcaggagactgaggtgggagaattgcttgaacctgggagatggagctgagatcacatcactgcactccagcctgggccaaagagcaagactccatctcaaaaagaaaaagaaattgaaccttgggagtttccatacaaattaaatcactagaacaattattgggataaatgtcaaacaaaacgactgatatgaaattctgaataagcctgtaaaacttgtgcttcaatgctaacaaaaaaaaaagttgaacaaatgaggtaaggaactcagtatttgaagataagctaggagcagcatttcctactcaaaagatttaccaagagataaacagttgaagagaattgagtataaatggtgacagcttgcttcccaactagtatgaaagctcaaaaccccttaatacagtaatatatgcaccttatttaatatattaatatataaatcaattttggaaaccagtttgaagttaagccattttgttaagtatgtattgtaaatggtgaaaatttcttcataaatatgcccagacaatgcaggagaccaagaatgcccaggttttaaggccaggctgtttccttttctttttggtaaacccctcagttttgatacattcttctaaaatacacagggctagactctaatagaataaaggaattcatgggggacaacgtgagggcaagtttccgcagactcggaacattttcccaagaggcaagtactgaattgagactaaaagaagctaattctgttctcaaatttctgtaactttaaaacatttgaaaaatgaagatctcctgtggcctttttaagagacttttatttgagtggttcttacaaagattgttgcaatatgaaagtcatttgtttgatagaaatatcaagctgtcttgtcaaacacactgaagtaacccaaaaatatatttcagagctcacagagcttaaaaagagcaaagattatatgcaaccagacaaaacctatttctgcatttcctatttctttctcagactgctttgcctaccagactctcacgtttaaacatcttcaggaaatgcagggatcattttgtttggaattttaagacacaccagaacacatagtatttacaaagaaacttttacagatacattaattgaaaagataccatcaagaaatataattttgaaatctccctttcttgccaattgatcagaatgcaagatgagatgctaaccaaacagccctttagctgtcttgtatttccatacactaaatgtgtatttcagaaactgctcaaccatcagccaaatatcaacattagtgaaatgtgaaatgtaaccactgtgtaaaaagttaggcttctgaaacattaaaaacattacatccctggtctgcctttttacagaaagcacatttgttctcctagagctattcctatagttcattaattttctacatgaacattttaaaaggcagaacaagagaacagttttgtatacagtgggatttactatttagggagaatgagcacactgcattcctgttaacatttttattttttcaaggtaacaggaaattgcatacaaatgacagtagatccttgcctctttatttttatctaaataaaagataactcaagatgaattctcaagaaagaaaaaaagctatatacataagggactatatcttccttcatcgtctacttggaaccagtagctgtgttgctgtcatagaatcaggaaacaggttgtggtaagttggaagaggtacatatgctgctgttatcattttaccagcaaaccacctgccatgcaatgcattgacagcagcaatagctgcagcaattgatgggcacttcacatacacattgccctgagctgaatttttgtcaacataaatatgaataactcctccatgtttattacattcttcaatcacatcatccttaatctcggtatcccatccaacttcttcttctgtttgagggttaaacatgttagagagttggaaacattgtgttgcaagtggctgaacagaggcagctgcagctaaagctgaagcttcagtctgctgggaaagtcttgtttgcaaatctataacaaaagagaattctgccacagcaccaaatgccaaagagccactcatctgtagagcttgctgtgctgctggcggaatctgcaaacctgtaccctctgcaagtcttgccattaactgaagacgaccagttgttcccaaatcaattccagtcctttccagttcatcactgtccaaaaatgaactagcactcgaagcatcagtacgttcagtaacatgaccaactttcattggtcttcctgctagttcaaatccattaagttgttccaaagcctttttggcacattctgagtcagaaaatgtaataaatccatatcccttggatcgaccagtttcactgtccatcatcagctggatactttcaattcttccaaaaggctcaaagatcccacgaagcatatcttcagttatgttgaagtgtaatgagcccacataaagcctcataggtccagcacttcccttttgtaaattgtttgccattgctgcagctctgtttttttctgcctgtgatgcctgtactatgattggcacgcctaaaactcgttggccagttaatcctattgctagaggcactgagctaacatcgacgaactccacataagcaattcctttggaacgtcttgaatttctgtcagaaatcatcctcacatctcgaacctttcctactgtagagaaaaactcttccaaatcccttggtcgaattcttgccgccagctgcatacagaagactgtccttgcatctctttcctcaggagttaaattatcaataggttctctcacagggctcttgtcttttctgaatggacttttgcttcgggaacgtcgtctgcttaatttgatgctatgaggcaacccaatctttcctcggatggcactgttaaattttggtccggagtaaggacttctgtagcggcctctaaatcttcgatctcgacttcttgagcggctccgtcgcctctctttgcttctacttcgctttctttcacggcttttgctctttttcctttctctgtctctacttcgcttccgttccttacttttgcttctctttcgttcatgactacgacttctgctcttgctttttttcctccttctggaatcttgaaacccacactccaatcacaaggagatgtagagctttccaaggaggcagaaagtttgttttttgctacgttcttcatggccgttggcactgctcaacttgttctcatccttatgattgacagttcacactggaatcaaaggtgaattcatgggagtagaggtgagatatcgttaggcaagtcttcttgtaaggagcctcaagcattgcttcaatatcaatatcgtctgccattttctctaaacgcctgttccggccttcgggcgcctgtggtgctcgtgttcgggaagagattgctgctgctgctgctgctgctgccgccgccgccgcttctgttgctactgttaagcccctaggcccaggccgcggaaccgcccagcccgaatatcgggttccaaggacggctaggcccgagagaatctaaaaaaaacaatggaattagagaagcccacgcgggagagcaggacggcggcttcggcagctcaggatccacccctgcgacagcgtcgacaagctccctgaaatggcggccgctgcttccctgtactcacattcaccagcacacat

SEQ ID NO: 16892 - RNA, 4177 nt, Homo sapiens
  source 1..4177: mol_type = other RNA
tactgcatcaggaactgattggacataaacagtttcactcagaatgagctgttttctatgcacgacactattcaagttactacactccaaccacatttcctctgaacattatttacacaccaaatttcactctggtagcaactaaattttggcacagatgagattaaccactaaaggccacatttgctggtccagttccctagaaagcaatgacacaacaaatttgttaggaagacttggttcaaggggaaaaactgatagcaggagatactttggaaaaagagcacactgacagagtgtctctgccccaaagaactctgcagtctggtattgaaaagtaaattttcaatgaggctgggcgcggtggctcatgcctgtaatcccggcactttgggaggccaaggcggacagatcacttgaggtcagtgtgagaccagccgggctaacaccgtctctgctaaaaatacaaaaattagctgggcacggtggtgcgcacctgtcccagctcttcaggagactgaggtgggagaattgcttgaacctgggagatggagctgagatcacatcactgcactccagcctgggccaaagagcaagactccatctcaaaaagaaaaagaaattgaaccttgggagtttccatacaaattaaatcactagaacaattattgggataaatgtcaaacaaaacgactgatatgaaattctgaataagcctgtaaaacttgtgcttcaatgctaacaaaaaaaaaagttgaacaaatgaggtaaggaactcagtatttgaagataagctaggagcagcatttcctactcaaaagatttaccaagagataaacagttgaagagaattgagtataaatggtgacagcttgcttcccaactagtatgaaagctcaaaaccccttaatacagtaatatatgcaccttatttaatatattaatatataaatcaattttggaaaccagtttgaagttaagccattttgttaagtatgtattgtaaatggtgaaaatttcttcataaatatgcccagacaatgcaggagaccaagaatgcccaggttttaaggccaggctgtttccttttctttttggtaaacccctcagttttgatacattcttctaaaatacacagggctagactctaatagaataaaggaattcatgggggacaacgtgagggcaagtttccgcagactcggaacattttcccaagaggcaagtactgaattgagactaaaagaagctaattctgttctcaaatttctgtaactttaaaacatttgaaaaatgaagatctcctgtggcctttttaagagacttttatttgagtggttcttacaaagattgttgcaatatgaaagtcatttgtttgatagaaatatcaagctgtcttgtcaaacacactgaagtaacccaaaaatatatttcagagctcacagagcttaaaaagagcaaagattatatgcaaccagacaaaacctatttctgcatttcctatttctttctcagactgctttgcctaccagactctcacgtttaaacatcttcaggaaatgcagggatcattttgtttggaattttaagacacaccagaacacatagtatttacaaagaaacttttacagatacattaattgaaaagataccatcaagaaatataattttgaaatctccctttcttgccaattgatcagaatgcaagatgagatgctaaccaaacagccctttagctgtcttgtatttccatacactaaatgtgtatttcagaaactgctcaaccatcagccaaatatcaacattagtgaaatgtgaaatgtaaccactgtgtaaaaagttaggcttctgaaacattaaaaacattacatccctggtctgcctttttacagaaagcacatttgttctcctagagctattcctatagttcattaattttctacatgaacattttaaaaggcagaacaagagaacagttttgtatacagtgggatttactatttagggagaatgagcacactgcattcctgttaacatttttattttttcaaggtaacaggaaattgcatacaaatgacagtagatccttgcctctttatttttatctaaataaaagataactcaagatgaattctcaagaaagaaaaaaagctatatacataagggactatatcttccttcatcgtctacttggaaccagtagctgtgttgctgtcatagaatcaggaaacaggttgtggtaagttggaagaggtacatatgctgctgttatcattttaccagcaaaccacctgccatgcaatgcattgacagcagcaatagctgcagcaattgatgggcacttcacatacacattgccctgagctgaatttttgtcaacataaatatgaataactcctccatgtttattacattcttcaatcacatcatccttaatctcggtatcccatccaacttcttcttctgtttgagggttaaacatgttagagagttggaaacattgtgttgcaagtggctgaacagaggcagctgcagctaaagctgaagcttcagtctgctgggaaagtcttgtttgcaaatctataacaaaagagaattctgccacagcaccaaatgccaaagagccactcatctgtagagcttgctgtgctgctggcggaatctgcaaacctgtaccctctgcaagtcttgccattaactgaagacgaccagttgttcccaaatcaattccagtcctttccagttcatcactgtccaaaaatgaactagcactcgaagcatcagtacgttcagtaacatgaccaactttcattggtcttcctgctagttcaaatccattaagttgttccaaagcctttttggcacattctgagtcagaaaatgtaataaatccatatcccttggatcgaccagtttcactgtccatcatcagctggatactttcaattcttccaaaaggctcaaagatcccacgaagcatatcttcagttatgttgaagtgtaatgagcccacataaagcctcataggtccagcacttcccttttgtaaattgtttgccattgctgcagctctgtttttttctgcctgtgatgcctgtactatgattggcacgcctaaaactcgttggccagttaatcctattgctagaggcactgagctaacatcgacgaactccacataagcaattcctttggaacgtcttgaatttctgtcagaaatcatcctcacatctcgaacctttcctactgtagagaaaaactcttccaaatcccttggtcgaattcttgccgccagctgcatacagaagactgtccttgcatctctttcctcaggagttaaattatcaataggttctctcacagggctcttgtcttttctgaatggacttttgcttcgggaacgtcgtctgcttaatttgatgctatgaggcaacccaatctttcctcggatggcactgttaaattttggtccggagtaaggacttctgtagcggcctctaaatcttcgatctcgacttcttgagcggctccgtcgcctctctttgcttctacttcgctttctttcacggcttttgctctttttcctttctctgtctctacttcgcttccgttccttacttttgcttctctttcgttcatgactacgacttctgctcttgctttttttcctccttctggaatcttgaaacccacactccaatcacaaggagatgtagagctttccaaggaggcagaaagtttgttttttgctacgttcttcatggccgttggcactgctcaacttgttctcatccttcttgtaaggagcctcaagcattgcttcaatatcaatatcgtctgccattttctctaaacgcctgttccggccttcgggcgcctgtggtgctcgtgttcgggaagagattgctgctgctgctgctgctgctgccgccgccgccgcttctgttgctactgttaagcccctaggcccaggccgcggaaccgcccagcccgaatatcgggttccaaggacggctaggcccgagagaatctaaaaaaaacaatggaattagagaagcccacgcgggagagcaggacggcggcttcggcagctcaggatccacccctgcgacagcgtcgacaagctccctgaaatggcggccgctgcttccctgtactcacattcaccagcacacat

SEQ ID NO: 16893 - RNA, 4178 nt, Homo sapiens
  source 1..4178: mol_type = other RNA
tactgcatcaggaactgattggacataaacagtttcactcagaatgagctgttttctatgcacgacactattcaagttactacactccaaccacatttcctctgaacattatttacacaccaaatttcactctggtagcaactaaattttggcacagatgagattaaccactaaaggccacatttgctggtccagttccctagaaagcaatgacacaacaaatttgttaggaagacttggttcaaggggaaaaactgatagcaggagatactttggaaaaagagcacactgacagagtgtctctgccccaaagaactctgcagtctggtattgaaaagtaaattttcaatgaggctgggcgcggtggctcatgcctgtaatcccggcactttgggaggccaaggcggacagatcacttgaggtcagtgtgagaccagccgggctaacaccgtctctgctaaaaatacaaaaattagctgggcacggtggtgcgcacctgtcccagctcttcaggagactgaggtgggagaattgcttgaacctgggagatggagctgagatcacatcactgcactccagcctgggccaaagagcaagactccatctcaaaaagaaaaagaaattgaaccttgggagtttccatacaaattaaatcactagaacaattattgggataaatgtcaaacaaaacgactgatatgaaattctgaataagcctgtaaaacttgtgcttcaatgctaacaaaaaaaaaagttgaacaaatgaggtaaggaactcagtatttgaagataagctaggagcagcatttcctactcaaaagatttaccaagagataaacagttgaagagaattgagtataaatggtgacagcttgcttcccaactagtatgaaagctcaaaaccccttaatacagtaatatatgcaccttatttaatatattaatatataaatcaattttggaaaccagtttgaagttaagccattttgttaagtatgtattgtaaatggtgaaaatttcttcataaatatgcccagacaatgcaggagaccaagaatgcccaggttttaaggccaggctgtttccttttctttttggtaaacccctcagttttgatacattcttctaaaatacacagggctagactctaatagaataaaggaattcatgggggacaacgtgagggcaagtttccgcagactcggaacattttcccaagaggcaagtactgaattgagactaaaagaagctaattctgttctcaaatttctgtaactttaaaacatttgaaaaatgaagatctcctgtggcctttttaagagacttttatttgagtggttcttacaaagattgttgcaatatgaaagtcatttgtttgatagaaatatcaagctgtcttgtcaaacacactgaagtaacccaaaaatatatttcagagctcacagagcttaaaaagagcaaagattatatgcaaccagacaaaacctatttctgcatttcctatttctttctcagactgctttgcctaccagactctcacgtttaaacatcttcaggaaatgcagggatcattttgtttggaattttaagacacaccagaacacatagtatttacaaagaaacttttacagatacattaattgaaaagataccatcaagaaatataattttgaaatctccctttcttgccaattgatcagaatgcaagatgagatgctaaccaaacagccctttagctgtcttgtatttccatacactaaatgtgtatttcagaaactgctcaaccatcagccaaatatcaacattagtgaaatgtgaaatgtaaccactgtgtaaaaagttaggcttctgaaacattaaaaacattacatccctggtctgcctttttacagaaagcacatttgttctcctagagctattcctatagttcattaattttctacatgaacattttaaaaggcagaacaagagaacagttttgtatacagtgggatttactatttagggagaatgagcacactgcattcctgttaacatttttattttttcaaggtaacaggaaattgcatacaaatgacagtagatccttgcctctttatttttatctaaataaaagataactcaagatgaattctcaagaaagaaaaaaagctatatacataagggactatatcttccttcatcgtctacttggaaccagtagctgtgttgctgtcatagaatcaggaaacaggttgtggtaagttggaagaggtacatatgctgctgttatcattttaccagcaaaccacctgccatgcaatgcattgacagcagcaatagctgcagcaattgatgggcacttcacatacacattgccctgagctgaatttttgtcaacataaatatgaataactcctccatgtttattacattcttcaatcacatcatccttaatctcggtatcccatccaacttcttcttctgtttgagggttaaacatgttagagagttggaaacattgtgttgcaagtggctgaacagaggcagctgcagctaaagctgaagcttcagtctgctgggaaagtcttgtttgcaaatctataacaaaagagaattctgccacagcaccaaatgccaaagagccactcatctgtagagcttgctgtgctgctggcggaatctgcaaacctgtaccctctgcaagtcttgccattaactgaagacgaccagttgttcccaaatcaattccagtcctttccagttcatcactgtccaaaaatgaactagcactcgaagcatcagtacgttcagtaacatgaccaactttcattggtcttcctgctagttcaaatccattaagttgttccaaagcctttttggcacattctgagtcagaaaatgtaataaatccatatcccttggatcgaccagtttcactgtccatcatcagctggatactttcaattcttccaaaaggctcaaagatcccacgaagcatatcttcagttatgttgaagtgtaatgagcccacataaagcctcataggtccagcacttcccttttgtaaattgtttgccattgctgcagctctgtttttttctgcctgtgatgcctgtactatgattggcacgcctaaaactcgttggccagttaatcctattgctagaggcactgagctaacatcgacgaactccacataagcaattcctttggaacgtcttgaatttctgtcagaaatcatcctcacatctcgaacctttcctactgtagagaaaaactcttccaaatcccttggtcgaattcttgccgccagctgcatacagaagactgtccttgcatctctttcctcaggagttaaattatcaataggttctctcacagggctcttgtcttttctgaatggacttttgcttcgggaacgtcgtctgcttaatttgatgctatgaggcaacccaatctttcctcggatggcactgttaaattttggtccggagtaaggacttctgtagcggcctctaaatcttcgatctcgacttcttgagcggctccgtcgcctctctttgcttctacttcgctttctttcacggcttttgctctttttcctttctctgtctctacttcgcttccgttccttacttttgcttctctttcgttcatgactacgacttctgctcttgctttttttcctctttttgctacgttcttcatggccgttggcactgctcaacttgttctcatccttatgattgacagttcacactggaatcaaaggtgaattcatgggagtagaggtgagatatcgttaggcaagtcttcttgtaaggagcctcaagcattgcttcaatatcaatatcgtctgccattttctctaaacgcctgttccggccttcgggcgcctgtggtgctcgtgttcgggaagagattgctgctgctgctgctgctgctgccgccgccgccgcttctgttgctactgttaagcccctaggcccaggccgcggaaccgcccagcccgaatatcgggttccaaggacggctaggcccgagagaatctaaaaaaaacaatggaattagagaagcccacgcgggagagcaggacggcggcttcggcagctcaggatccacccctgcgacagcgtcgacaagctccctgaaatggcggccgctgcttccctgtactcacattcaccagcacacat

SEQ ID NO: 16894 - RNA, 4105 nt, Homo sapiens
  source 1..4105: mol_type = other RNA
tactgcatcaggaactgattggacataaacagtttcactcagaatgagctgttttctatgcacgacactattcaagttactacactccaaccacatttcctctgaacattatttacacaccaaatttcactctggtagcaactaaattttggcacagatgagattaaccactaaaggccacatttgctggtccagttccctagaaagcaatgacacaacaaatttgttaggaagacttggttcaaggggaaaaactgatagcaggagatactttggaaaaagagcacactgacagagtgtctctgccccaaagaactctgcagtctggtattgaaaagtaaattttcaatgaggctgggcgcggtggctcatgcctgtaatcccggcactttgggaggccaaggcggacagatcacttgaggtcagtgtgagaccagccgggctaacaccgtctctgctaaaaatacaaaaattagctgggcacggtggtgcgcacctgtcccagctcttcaggagactgaggtgggagaattgcttgaacctgggagatggagctgagatcacatcactgcactccagcctgggccaaagagcaagactccatctcaaaaagaaaaagaaattgaaccttgggagtttccatacaaattaaatcactagaacaattattgggataaatgtcaaacaaaacgactgatatgaaattctgaataagcctgtaaaacttgtgcttcaatgctaacaaaaaaaaaagttgaacaaatgaggtaaggaactcagtatttgaagataagctaggagcagcatttcctactcaaaagatttaccaagagataaacagttgaagagaattgagtataaatggtgacagcttgcttcccaactagtatgaaagctcaaaaccccttaatacagtaatatatgcaccttatttaatatattaatatataaatcaattttggaaaccagtttgaagttaagccattttgttaagtatgtattgtaaatggtgaaaatttcttcataaatatgcccagacaatgcaggagaccaagaatgcccaggttttaaggccaggctgtttccttttctttttggtaaacccctcagttttgatacattcttctaaaatacacagggctagactctaatagaataaaggaattcatgggggacaacgtgagggcaagtttccgcagactcggaacattttcccaagaggcaagtactgaattgagactaaaagaagctaattctgttctcaaatttctgtaactttaaaacatttgaaaaatgaagatctcctgtggcctttttaagagacttttatttgagtggttcttacaaagattgttgcaatatgaaagtcatttgtttgatagaaatatcaagctgtcttgtcaaacacactgaagtaacccaaaaatatatttcagagctcacagagcttaaaaagagcaaagattatatgcaaccagacaaaacctatttctgcatttcctatttctttctcagactgctttgcctaccagactctcacgtttaaacatcttcaggaaatgcagggatcattttgtttggaattttaagacacaccagaacacatagtatttacaaagaaacttttacagatacattaattgaaaagataccatcaagaaatataattttgaaatctccctttcttgccaattgatcagaatgcaagatgagatgctaaccaaacagccctttagctgtcttgtatttccatacactaaatgtgtatttcagaaactgctcaaccatcagccaaatatcaacattagtgaaatgtgaaatgtaaccactgtgtaaaaagttaggcttctgaaacattaaaaacattacatccctggtctgcctttttacagaaagcacatttgttctcctagagctattcctatagttcattaattttctacatgaacattttaaaaggcagaacaagagaacagttttgtatacagtgggatttactatttagggagaatgagcacactgcattcctgttaacatttttattttttcaaggtaacaggaaattgcatacaaatgacagtagatccttgcctctttatttttatctaaataaaagataactcaagatgaattctcaagaaagaaaaaaagctatatacataagggactatatcttccttcatcgtctacttggaaccagtagctgtgttgctgtcatagaatcaggaaacaggttgtggtaagttggaagaggtacatatgctgctgttatcattttaccagcaaaccacctgccatgcaatgcattgacagcagcaatagctgcagcaattgatgggcacttcacatacacattgccctgagctgaatttttgtcaacataaatatgaataactcctccatgtttattacattcttcaatcacatcatccttaatctcggtatcccatccaacttcttcttctgtttgagggttaaacatgttagagagttggaaacattgtgttgcaagtggctgaacagaggcagctgcagctaaagctgaagcttcagtctgctgggaaagtcttgtttgcaaatctataacaaaagagaattctgccacagcaccaaatgccaaagagccactcatctgtagagcttgctgtgctgctggcggaatctgcaaacctgtaccctctgcaagtcttgccattaactgaagacgaccagttgttcccaaatcaattccagtcctttccagttcatcactgtccaaaaatgaactagcactcgaagcatcagtacgttcagtaacatgaccaactttcattggtcttcctgctagttcaaatccattaagttgttccaaagcctttttggcacattctgagtcagaaaatgtaataaatccatatcccttggatcgaccagtttcactgtccatcatcagctggatactttcaattcttccaaaaggctcaaagatcccacgaagcatatcttcagttatgttgaagtgtaatgagcccacataaagcctcataggtccagcacttcccttttgtaaattgtttgccattgctgcagctctgtttttttctgcctgtgatgcctgtactatgattggcacgcctaaaactcgttggccagttaatcctattgctagaggcactgagctaacatcgacgaactccacataagcaattcctttggaacgtcttgaatttctgtcagaaatcatcctcacatctcgaacctttcctactgtagagaaaaactcttccaaatcccttggtcgaattcttgccgccagctgcatacagaagactgtccttgcatctctttcctcaggagttaaattatcaataggttctctcacagggctcttgtcttttctgaatggacttttgcttcgggaacgtcgtctgcttaatttgatgctatgaggcaacccaatctttcctcggatggcactgttaaattttggtccggagtaaggacttctgtagcggcctctaaatcttcgatctcgacttcttgagcggctccgtcgcctctctttgcttctacttcgctttctttcacggcttttgctctttttcctttctctgtctctacttcgcttccgttccttacttttgcttctctttcgttcatgactacgacttctgctcttgctttttttcctctttttgctacgttcttcatggccgttggcactgctcaacttgttctcatccttcttgtaaggagcctcaagcattgcttcaatatcaatatcgtctgccattttctctaaacgcctgttccggccttcgggcgcctgtggtgctcgtgttcgggaagagattgctgctgctgctgctgctgctgccgccgccgccgcttctgttgctactgttaagcccctaggcccaggccgcggaaccgcccagcccgaatatcgggttccaaggacggctaggcccgagagaatctaaaaaaaacaatggaattagagaagcccacgcgggagagcaggacggcggcttcggcagctcaggatccacccctgcgacagcgtcgacaagctccctgaaatggcggccgctgcttccctgtactcacattcaccagcacacat

SEQ ID NO: 16895 - RNA, 4039 nt, Homo sapiens
  source 1..4039: mol_type = other RNA
tactgcatcaggaactgattggacataaacagtttcactcagaatgagctgttttctatgcacgacactattcaagttactacactccaaccacatttcctctgaacattatttacacaccaaatttcactctggtagcaactaaattttggcacagatgagattaaccactaaaggccacatttgctggtccagttccctagaaagcaatgacacaacaaatttgttaggaagacttggttcaaggggaaaaactgatagcaggagatactttggaaaaagagcacactgacagagtgtctctgccccaaagaactctgcagtctggtattgaaaagtaaattttcaatgaggctgggcgcggtggctcatgcctgtaatcccggcactttgggaggccaaggcggacagatcacttgaggtcagtgtgagaccagccgggctaacaccgtctctgctaaaaatacaaaaattagctgggcacggtggtgcgcacctgtcccagctcttcaggagactgaggtgggagaattgcttgaacctgggagatggagctgagatcacatcactgcactccagcctgggccaaagagcaagactccatctcaaaaagaaaaagaaattgaaccttgggagtttccatacaaattaaatcactagaacaattattgggataaatgtcaaacaaaacgactgatatgaaattctgaataagcctgtaaaacttgtgcttcaatgctaacaaaaaaaaaagttgaacaaatgaggtaaggaactcagtatttgaagataagctaggagcagcatttcctactcaaaagatttaccaagagataaacagttgaagagaattgagtataaatggtgacagcttgcttcccaactagtatgaaagctcaaaaccccttaatacagtaatatatgcaccttatttaatatattaatatataaatcaattttggaaaccagtttgaagttaagccattttgttaagtatgtattgtaaatggtgaaaatttcttcataaatatgcccagacaatgcaggagaccaagaatgcccaggttttaaggccaggctgtttccttttctttttggtaaacccctcagttttgatacattcttctaaaatacacagggctagactctaatagaataaaggaattcatgggggacaacgtgagggcaagtttccgcagactcggaacattttcccaagaggcaagtactgaattgagactaaaagaagctaattctgttctcaaatttctgtaactttaaaacatttgaaaaatgaagatctcctgtggcctttttaagagacttttatttgagtggttcttacaaagattgttgcaatatgaaagtcatttgtttgatagaaatatcaagctgtcttgtcaaacacactgaagtaacccaaaaatatatttcagagctcacagagcttaaaaagagcaaagattatatgcaaccagacaaaacctatttctgcatttcctatttctttctcagactgctttgcctaccagactctcacgtttaaacatcttcaggaaatgcagggatcattttgtttggaattttaagacacaccagaacacatagtatttacaaagaaacttttacagatacattaattgaaaagataccatcaagaaatataattttgaaatctccctttcttgccaattgatcagaatgcaagatgagatgctaaccaaacagccctttagctgtcttgtatttccatacactaaatgtgtatttcagaaactgctcaaccatcagccaaatatcaacattagtgaaatgtgaaatgtaaccactgtgtaaaaagttaggcttctgaaacattaaaaacattacatccctggtctgcctttttacagaaagcacatttgttctcctagagctattcctatagttcattaattttctacatgaacattttaaaaggcagaacaagagaacagttttgtatacagtgggatttactatttagggagaatgagcacactgcattcctgttaacatttttattttttcaaggtaacaggaaattgcatacaaatgacagtagatccttgcctctttatttttatctaaataaaagataactcaagatgaattctcaagaaagaaaaaaagctatatacataagggactatatcttccttcatcgtctacttggaaccagtagctgtgttgctgtcatagaatcaggaaacaggttgtggtaagttggaagaggtacatatgctgctgttatcattttaccagcaaaccacctgccatgcaatgcattgacagcagcaatagctgcagcaattgatgggcacttcacatacacattgccctgagctgaatttttgtcaacataaatatgaataactcctccatgtttattacattcttcaatcacatcatccttaatctcggtatcccatccaacttcttcttctgtttgagggttaaacatgttagagagttggaaacattgtgttgcaagtggctgaacagaggcagctgcagctaaagctgaagcttcagtctgctgggaaagtcttgtttgcaaatctataacaaaagagaattctgccacagcaccaaatgccaaagagccactcatctgtagagcttgctgtgctgctggcggaatctgcaaacctgtaccctctgcaagtcttgccattaactgaagacgaccagttgttcccaaatcaattccagtcctttccagttcatcactgtccaaaaatgaactagcactcgaagcatcagtacgttcagtaacatgaccaactttcattggtcttcctgctagttcaaatccattaagttgttccaaagcctttttggcacattctgagtcagaaaatgtaataaatccatatcccttggatcgaccagtttcactgtccatcatcagctggatactttcaattcttccaaaaggctcaaagatcccacgaagcatatcttcagttatgttgaagtgtaatgagcccacataaagcctcataggtccagcacttcccttttgtaaattgtttgccattgctgcagctctgtttttttctgcctgtgatgcctgtactatgattggcacgcctaaaactcgttggccagttaatcctattgctagaggcactgagctaacatcgacgaactccacataagcaattcctttggaacgtcttgaatttctgtcagaaatcatcctcacatctcgaacctttcctactgtagagaaaaactcttccaaatcccttggtcgaattcttgccgccagctgcatacagaagactgtccttgcatctctttcctcaggagttaaattatcaataggttctctcacagggctcttgtcttttctgaatggacttttgcttcgggaacgtcgtctgtaaggacttctgtagcggcctctaaatcttcgatctcgacttcttgagcggctccgtcgcctctctttgcttctacttcgctttctttcacggcttttgctctttttcctttctctgtctctacttcgcttccgttccttacttttgcttctctttcgttcatgactacgacttctgctcttgctttttttcctctttttgctacgttcttcatggccgttggcactgctcaacttgttctcatccttcttgtaaggagcctcaagcattgcttcaatatcaatatcgtctgccattttctctaaacgcctgttccggccttcgggcgcctgtggtgctcgtgttcgggaagagattgctgctgctgctgctgctgctgccgccgccgccgcttctgttgctactgttaagcccctaggcccaggccgcggaaccgcccagcccgaatatcgggttccaaggacggctaggcccgagagaatctaaaaaaaacaatggaattagagaagcccacgcgggagagcaggacggcggcttcggcagctcaggatccacccctgcgacagcgtcgacaagctccctgaaatggcggccgctgcttccctgtactcacattcaccagcacacat

SEQ ID NO: 16896 - RNA, 4102 nt, Homo sapiens
  source 1..4102: mol_type = other RNA
tactgcatcaggaactgattggacataaacagtttcactcagaatgagctgttttctatgcacgacactattcaagttactacactccaaccacatttcctctgaacattatttacacaccaaatttcactctggtagcaactaaattttggcacagatgagattaaccactaaaggccacatttgctggtccagttccctagaaagcaatgacacaacaaatttgttaggaagacttggttcaaggggaaaaactgatagcaggagatactttggaaaaagagcacactgacagagtgtctctgccccaaagaactctgcagtctggtattgaaaagtaaattttcaatgaggctgggcgcggtggctcatgcctgtaatcccggcactttgggaggccaaggcggacagatcacttgaggtcagtgtgagaccagccgggctaacaccgtctctgctaaaaatacaaaaattagctgggcacggtggtgcgcacctgtcccagctcttcaggagactgaggtgggagaattgcttgaacctgggagatggagctgagatcacatcactgcactccagcctgggccaaagagcaagactccatctcaaaaagaaaaagaaattgaaccttgggagtttccatacaaattaaatcactagaacaattattgggataaatgtcaaacaaaacgactgatatgaaattctgaataagcctgtaaaacttgtgcttcaatgctaacaaaaaaaaaagttgaacaaatgaggtaaggaactcagtatttgaagataagctaggagcagcatttcctactcaaaagatttaccaagagataaacagttgaagagaattgagtataaatggtgacagcttgcttcccaactagtatgaaagctcaaaaccccttaatacagtaatatatgcaccttatttaatatattaatatataaatcaattttggaaaccagtttgaagttaagccattttgttaagtatgtattgtaaatggtgaaaatttcttcataaatatgcccagacaatgcaggagaccaagaatgcccaggttttaaggccaggctgtttccttttctttttggtaaacccctcagttttgatacattcttctaaaatacacagggctagactctaatagaataaaggaattcatgggggacaacgtgagggcaagtttccgcagactcggaacattttcccaagaggcaagtactgaattgagactaaaagaagctaattctgttctcaaatttctgtaactttaaaacatttgaaaaatgaagatctcctgtggcctttttaagagacttttatttgagtggttcttacaaagattgttgcaatatgaaagtcatttgtttgatagaaatatcaagctgtcttgtcaaacacactgaagtaacccaaaaatatatttcagagctcacagagcttaaaaagagcaaagattatatgcaaccagacaaaacctatttctgcatttcctatttctttctcagactgctttgcctaccagactctcacgtttaaacatcttcaggaaatgcagggatcattttgtttggaattttaagacacaccagaacacatagtatttacaaagaaacttttacagatacattaattgaaaagataccatcaagaaatataattttgaaatctccctttcttgccaattgatcagaatgcaagatgagatgctaaccaaacagccctttagctgtcttgtatttccatacactaaatgtgtatttcagaaactgctcaaccatcagccaaatatcaacattagtgaaatgtgaaatgtaaccactgtgtaaaaagttaggcttctgaaacattaaaaacattacatccctggtctgcctttttacagaaagcacatttgttctcctagagctattcctatagttcattaattttctacatgaacattttaaaaggcagaacaagagaacagttttgtatacagtgggatttactatttagggagaatgagcacactgcattcctgttaacatttttattttttcaaggtaacaggaaattgcatacaaatgacagtagatccttgcctctttatttttatctaaataaaagataactcaagatgaattctcaagaaagaaaaaaagctatatacataagggactatatcttccttcatcgtctacttggaaccagtagctgtgttgctgtcatagaatcaggaaacaggttgtggtaagttggaagaggtacatatgctgctgttatcattttaccagcaaaccacctgccatgcaatgcattgacagcagcaatagctgcagcaattgatgggcacttcacatacacattgccctgagctgaatttttgtcaacataaatatgaataactcctccatgtttattacattcttcaatcacatcatccttaatctcggtatcccatccaacttcttcttctgtttgagggttaaacatgttagagagttggaaacattgtgttgcaagtggctgaacagaggcagctgcagctaaagctgaagcttcagtctgctgggaaagtcttgtttgcaaatctataacaaaagagaattctgccacagcaccaaatgccaaagagccactcatctgtagagcttgctgtgctgctggcggaatctgcaaacctgtaccctctgcaagtcttgccattaactgaagacgaccagttgttcccaaatcaattccagtcctttccagttcatcactgtccaaaaatgaactagcactcgaagcatcagtacgttcagtaacatgaccaactttcattggtcttcctgctagttcaaatccattaagttgttccaaagcctttttggcacattctgagtcagaaaatgtaataaatccatatcccttggatcgaccagtttcactgtccatcatcagctggatactttcaattcttccaaaaggctcaaagatcccacgaagcatatcttcagttatgttgaagtgtaatgagcccacataaagcctcataggtccagcacttcccttttgtaaattgtttgccattgctgcagctctgtttttttctgcctgtgatgcctgtactatgattggcacgcctaaaactcgttggccagttaatcctattgctagaggcactgagctaacatcgacgaactccacataagcaattcctttggaacgtcttgaatttctgtcagaaatcatcctcacatctcgaacctttcctactgtagagaaaaactcttccaaatcccttggtcgaattcttgccgccagctgcatacagaagactgtccttgcatctctttcctcaggagttaaattatcaataggttctctcacagggctcttgtcttttctgaatggacttttgcttcgggaacgtcgtcttaatttgatgctatgaggcaacccaatctttcctcggatggcactgttaaattttggtccggagtaaggacttctgtagcggcctctaaatcttcgatctcgacttcttgagcggctccgtcgcctctctttgcttctacttcgctttctttcacggcttttgctctttttcctttctctgtctctacttcgcttccgttccttacttttgcttctctttcgttcatgactacgacttctgctcttgctttttttcctctttttgctacgttcttcatggccgttggcactgctcaacttgttctcatccttcttgtaaggagcctcaagcattgcttcaatatcaatatcgtctgccattttctctaaacgcctgttccggccttcgggcgcctgtggtgctcgtgttcgggaagagattgctgctgctgctgctgctgctgccgccgccgccgcttctgttgctactgttaagcccctaggcccaggccgcggaaccgcccagcccgaatatcgggttccaaggacggctaggcccgagagaatctaaaaaaaacaatggaattagagaagcccacgcgggagagcaggacggcggcttcggcagctcaggatccacccctgcgacagcgtcgacaagctccctgaaatggcggccgctgcttccctgtactcacattcaccagcacacat

SEQ ID NO: 16897 - RNA, 4160 nt, Homo sapiens
  source 1..4160: mol_type = other RNA
tactgcatcaggaactgattggacataaacagtttcactcagaatgagctgttttctatgcacgacactattcaagttactacactccaaccacatttcctctgaacattatttacacaccaaatttcactctggtagcaactaaattttggcacagatgagattaaccactaaaggccacatttgctggtccagttccctagaaagcaatgacacaacaaatttgttaggaagacttggttcaaggggaaaaactgatagcaggagatactttggaaaaagagcacactgacagagtgtctctgccccaaagaactctgcagtctggtattgaaaagtaaattttcaatgaggctgggcgcggtggctcatgcctgtaatcccggcactttgggaggccaaggcggacagatcacttgaggtcagtgtgagaccagccgggctaacaccgtctctgctaaaaatacaaaaattagctgggcacggtggtgcgcacctgtcccagctcttcaggagactgaggtgggagaattgcttgaacctgggagatggagctgagatcacatcactgcactccagcctgggccaaagagcaagactccatctcaaaaagaaaaagaaattgaaccttgggagtttccatacaaattaaatcactagaacaattattgggataaatgtcaaacaaaacgactgatatgaaattctgaataagcctgtaaaacttgtgcttcaatgctaacaaaaaaaaaagttgaacaaatgaggtaaggaactcagtatttgaagataagctaggagcagcatttcctactcaaaagatttaccaagagataaacagttgaagagaattgagtataaatggtgacagcttgcttcccaactagtatgaaagctcaaaaccccttaatacagtaatatatgcaccttatttaatatattaatatataaatcaattttggaaaccagtttgaagttaagccattttgttaagtatgtattgtaaatggtgaaaatttcttcataaatatgcccagacaatgcaggagaccaagaatgcccaggttttaaggccaggctgtttccttttctttttggtaaacccctcagttttgatacattcttctaaaatacacagggctagactctaatagaataaaggaattcatgggggacaacgtgagggcaagtttccgcagactcggaacattttcccaagaggcaagtactgaattgagactaaaagaagctaattctgttctcaaatttctgtaactttaaaacatttgaaaaatgaagatctcctgtggcctttttaagagacttttatttgagtggttcttacaaagattgttgcaatatgaaagtcatttgtttgatagaaatatcaagctgtcttgtcaaacacactgaagtaacccaaaaatatatttcagagctcacagagcttaaaaagagcaaagattatatgcaaccagacaaaacctatttctgcatttcctatttctttctcagactgctttgcctaccagactctcacgtttaaacatcttcaggaaatgcagggatcattttgtttggaattttaagacacaccagaacacatagtatttacaaagaaacttttacagatacattaattgaaaagataccatcaagaaatataattttgaaatctccctttcttgccaattgatcagaatgcaagatgagatgctaaccaaacagccctttagctgtcttgtatttccatacactaaatgtgtatttcagaaactgctcaaccatcagccaaatatcaacattagtgaaatgtgaaatgtaaccactgtgtaaaaagttaggcttctgaaacattaaaaacattacatccctggtctgcctttttacagaaagcacatttgttctcctagagctattcctatagttcattaattttctacatgaacattttaaaaggcagaacaagagaacagttttgtatacagtgggatttactatttagggagaatgagcacactgcattcctgttaacatttttattttttcaaggtaacaggaaattgcatacaaatgacagtagatccttgcctctttatttttatctaaataaaagataactcaagatgaattctcaagaaagaaaaaaagctatatacataagggactatatcttccttcatcgtctacttggaaccagtagctgtgttgctgtcatagaatcaggaaacaggttgtggtaagttggaagaggtacatatgctgctgttatcattttaccagcaaaccacctgccatgcaatgcattgacagcagcaatagctgcagcaattgatgggcacttcacatacacattgccctgagctgaatttttgtcaacataaatatgaataactcctccatgtttattacattcttcaatcacatcatccttaatctcggtatcccatccaacttcttcttctgtttgagggttaaacatgttagagagttggaaacattgtgttgcaagtggctgaacagaggcagctgcagctaaagctgaagcttcagtctgctgggaaagtcttgtttgcaaatctgccacagcaccaaatgccaaagagccactcatctgtagagcttgctgtgctgctggcggaatctgcaaacctgtaccctctgcaagtcttgccattaactgaagacgaccagttgttcccaaatcaattccagtcctttccagttcatcactgtccaaaaatgaactagcactcgaagcatcagtacgttcagtaacatgaccaactttcattggtcttcctgctagttcaaatccattaagttgttccaaagcctttttggcacattctgagtcagaaaatgtaataaatccatatcccttggatcgaccagtttcactgtccatcatcagctggatactttcaattcttccaaaaggctcaaagatcccacgaagcatatcttcagttatgttgaagtgtaatgagcccacataaagcctcataggtccagcacttcccttttgtaaattgtttgccattgctgcagctctgtttttttctgcctgtgatgcctgtactatgattggcacgcctaaaactcgttggccagttaatcctattgctagaggcactgagctaacatcgacgaactccacataagcaattcctttggaacgtcttgaatttctgtcagaaatcatcctcacatctcgaacctttcctactgtagagaaaaactcttccaaatcccttggtcgaattcttgccgccagctgcatacagaagactgtccttgcatctctttcctcaggagttaaattatcaataggttctctcacagggctcttgtcttttctgaatggacttttgcttcgggaacgtcgtctgcttaatttgatgctatgaggcaacccaatctttcctcggatggcactgttaaattttggtccggagtaaggacttctgtagcggcctctaaatcttcgatctcgacttcttgagcggctccgtcgcctctctttgcttctacttcgctttctttcacggcttttgctctttttcctttctctgtctctacttcgcttccgttccttacttttgcttctctttcgttcatgactacgacttctgctcttgctttttttcctctttttgctacgttcttcatggccgttggcactgctcaacttgttctcatccttatgattgacagttcacactggaatcaaaggtgaattcatgggagtagaggtgagatatcgttaggcaagtcttcttgtaaggagcctcaagcattgcttcaatatcaatatcgtctgccattttctctaaacgcctgttccggccttcgggcgcctgtggtgctcgtgttcgggaagagattgctgctgctgctgctgctgctgccgccgccgccgcttctgttgctactgttaagcccctaggcccaggccgcggaaccgcccagcccgaatatcgggttccaaggacggctaggcccgagagaatctaaaaaaaacaatggaattagagaagcccacgcgggagagcaggacggcggcttcggcagctcaggatccacccctgcgacagcgtcgacaagctccctgaaatggcggccgctgcttccctgtactcacattcaccagcacacat

SEQ ID NO: 16898 - RNA, 4087 nt, Homo sapiens
  source 1..4087: mol_type = other RNA
tactgcatcaggaactgattggacataaacagtttcactcagaatgagctgttttctatgcacgacactattcaagttactacactccaaccacatttcctctgaacattatttacacaccaaatttcactctggtagcaactaaattttggcacagatgagattaaccactaaaggccacatttgctggtccagttccctagaaagcaatgacacaacaaatttgttaggaagacttggttcaaggggaaaaactgatagcaggagatactttggaaaaagagcacactgacagagtgtctctgccccaaagaactctgcagtctggtattgaaaagtaaattttcaatgaggctgggcgcggtggctcatgcctgtaatcccggcactttgggaggccaaggcggacagatcacttgaggtcagtgtgagaccagccgggctaacaccgtctctgctaaaaatacaaaaattagctgggcacggtggtgcgcacctgtcccagctcttcaggagactgaggtgggagaattgcttgaacctgggagatggagctgagatcacatcactgcactccagcctgggccaaagagcaagactccatctcaaaaagaaaaagaaattgaaccttgggagtttccatacaaattaaatcactagaacaattattgggataaatgtcaaacaaaacgactgatatgaaattctgaataagcctgtaaaacttgtgcttcaatgctaacaaaaaaaaaagttgaacaaatgaggtaaggaactcagtatttgaagataagctaggagcagcatttcctactcaaaagatttaccaagagataaacagttgaagagaattgagtataaatggtgacagcttgcttcccaactagtatgaaagctcaaaaccccttaatacagtaatatatgcaccttatttaatatattaatatataaatcaattttggaaaccagtttgaagttaagccattttgttaagtatgtattgtaaatggtgaaaatttcttcataaatatgcccagacaatgcaggagaccaagaatgcccaggttttaaggccaggctgtttccttttctttttggtaaacccctcagttttgatacattcttctaaaatacacagggctagactctaatagaataaaggaattcatgggggacaacgtgagggcaagtttccgcagactcggaacattttcccaagaggcaagtactgaattgagactaaaagaagctaattctgttctcaaatttctgtaactttaaaacatttgaaaaatgaagatctcctgtggcctttttaagagacttttatttgagtggttcttacaaagattgttgcaatatgaaagtcatttgtttgatagaaatatcaagctgtcttgtcaaacacactgaagtaacccaaaaatatatttcagagctcacagagcttaaaaagagcaaagattatatgcaaccagacaaaacctatttctgcatttcctatttctttctcagactgctttgcctaccagactctcacgtttaaacatcttcaggaaatgcagggatcattttgtttggaattttaagacacaccagaacacatagtatttacaaagaaacttttacagatacattaattgaaaagataccatcaagaaatataattttgaaatctccctttcttgccaattgatcagaatgcaagatgagatgctaaccaaacagccctttagctgtcttgtatttccatacactaaatgtgtatttcagaaactgctcaaccatcagccaaatatcaacattagtgaaatgtgaaatgtaaccactgtgtaaaaagttaggcttctgaaacattaaaaacattacatccctggtctgcctttttacagaaagcacatttgttctcctagagctattcctatagttcattaattttctacatgaacattttaaaaggcagaacaagagaacagttttgtatacagtgggatttactatttagggagaatgagcacactgcattcctgttaacatttttattttttcaaggtaacaggaaattgcatacaaatgacagtagatccttgcctctttatttttatctaaataaaagataactcaagatgaattctcaagaaagaaaaaaagctatatacataagggactatatcttccttcatcgtctacttggaaccagtagctgtgttgctgtcatagaatcaggaaacaggttgtggtaagttggaagaggtacatatgctgctgttatcattttaccagcaaaccacctgccatgcaatgcattgacagcagcaatagctgcagcaattgatgggcacttcacatacacattgccctgagctgaatttttgtcaacataaatatgaataactcctccatgtttattacattcttcaatcacatcatccttaatctcggtatcccatccaacttcttcttctgtttgagggttaaacatgttagagagttggaaacattgtgttgcaagtggctgaacagaggcagctgcagctaaagctgaagcttcagtctgctgggaaagtcttgtttgcaaatctgccacagcaccaaatgccaaagagccactcatctgtagagcttgctgtgctgctggcggaatctgcaaacctgtaccctctgcaagtcttgccattaactgaagacgaccagttgttcccaaatcaattccagtcctttccagttcatcactgtccaaaaatgaactagcactcgaagcatcagtacgttcagtaacatgaccaactttcattggtcttcctgctagttcaaatccattaagttgttccaaagcctttttggcacattctgagtcagaaaatgtaataaatccatatcccttggatcgaccagtttcactgtccatcatcagctggatactttcaattcttccaaaaggctcaaagatcccacgaagcatatcttcagttatgttgaagtgtaatgagcccacataaagcctcataggtccagcacttcccttttgtaaattgtttgccattgctgcagctctgtttttttctgcctgtgatgcctgtactatgattggcacgcctaaaactcgttggccagttaatcctattgctagaggcactgagctaacatcgacgaactccacataagcaattcctttggaacgtcttgaatttctgtcagaaatcatcctcacatctcgaacctttcctactgtagagaaaaactcttccaaatcccttggtcgaattcttgccgccagctgcatacagaagactgtccttgcatctctttcctcaggagttaaattatcaataggttctctcacagggctcttgtcttttctgaatggacttttgcttcgggaacgtcgtctgcttaatttgatgctatgaggcaacccaatctttcctcggatggcactgttaaattttggtccggagtaaggacttctgtagcggcctctaaatcttcgatctcgacttcttgagcggctccgtcgcctctctttgcttctacttcgctttctttcacggcttttgctctttttcctttctctgtctctacttcgcttccgttccttacttttgcttctctttcgttcatgactacgacttctgctcttgctttttttcctctttttgctacgttcttcatggccgttggcactgctcaacttgttctcatccttcttgtaaggagcctcaagcattgcttcaatatcaatatcgtctgccattttctctaaacgcctgttccggccttcgggcgcctgtggtgctcgtgttcgggaagagattgctgctgctgctgctgctgctgccgccgccgccgcttctgttgctactgttaagcccctaggcccaggccgcggaaccgcccagcccgaatatcgggttccaaggacggctaggcccgagagaatctaaaaaaaacaatggaattagagaagcccacgcgggagagcaggacggcggcttcggcagctcaggatccacccctgcgacagcgtcgacaagctccctgaaatggcggccgctgcttccctgtactcacattcaccagcacacat

SEQ ID NO: 16899 - RNA, 4021 nt, Homo sapiens
  source 1..4021: mol_type = other RNA
tactgcatcaggaactgattggacataaacagtttcactcagaatgagctgttttctatgcacgacactattcaagttactacactccaaccacatttcctctgaacattatttacacaccaaatttcactctggtagcaactaaattttggcacagatgagattaaccactaaaggccacatttgctggtccagttccctagaaagcaatgacacaacaaatttgttaggaagacttggttcaaggggaaaaactgatagcaggagatactttggaaaaagagcacactgacagagtgtctctgccccaaagaactctgcagtctggtattgaaaagtaaattttcaatgaggctgggcgcggtggctcatgcctgtaatcccggcactttgggaggccaaggcggacagatcacttgaggtcagtgtgagaccagccgggctaacaccgtctctgctaaaaatacaaaaattagctgggcacggtggtgcgcacctgtcccagctcttcaggagactgaggtgggagaattgcttgaacctgggagatggagctgagatcacatcactgcactccagcctgggccaaagagcaagactccatctcaaaaagaaaaagaaattgaaccttgggagtttccatacaaattaaatcactagaacaattattgggataaatgtcaaacaaaacgactgatatgaaattctgaataagcctgtaaaacttgtgcttcaatgctaacaaaaaaaaaagttgaacaaatgaggtaaggaactcagtatttgaagataagctaggagcagcatttcctactcaaaagatttaccaagagataaacagttgaagagaattgagtataaatggtgacagcttgcttcccaactagtatgaaagctcaaaaccccttaatacagtaatatatgcaccttatttaatatattaatatataaatcaattttggaaaccagtttgaagttaagccattttgttaagtatgtattgtaaatggtgaaaatttcttcataaatatgcccagacaatgcaggagaccaagaatgcccaggttttaaggccaggctgtttccttttctttttggtaaacccctcagttttgatacattcttctaaaatacacagggctagactctaatagaataaaggaattcatgggggacaacgtgagggcaagtttccgcagactcggaacattttcccaagaggcaagtactgaattgagactaaaagaagctaattctgttctcaaatttctgtaactttaaaacatttgaaaaatgaagatctcctgtggcctttttaagagacttttatttgagtggttcttacaaagattgttgcaatatgaaagtcatttgtttgatagaaatatcaagctgtcttgtcaaacacactgaagtaacccaaaaatatatttcagagctcacagagcttaaaaagagcaaagattatatgcaaccagacaaaacctatttctgcatttcctatttctttctcagactgctttgcctaccagactctcacgtttaaacatcttcaggaaatgcagggatcattttgtttggaattttaagacacaccagaacacatagtatttacaaagaaacttttacagatacattaattgaaaagataccatcaagaaatataattttgaaatctccctttcttgccaattgatcagaatgcaagatgagatgctaaccaaacagccctttagctgtcttgtatttccatacactaaatgtgtatttcagaaactgctcaaccatcagccaaatatcaacattagtgaaatgtgaaatgtaaccactgtgtaaaaagttaggcttctgaaacattaaaaacattacatccctggtctgcctttttacagaaagcacatttgttctcctagagctattcctatagttcattaattttctacatgaacattttaaaaggcagaacaagagaacagttttgtatacagtgggatttactatttagggagaatgagcacactgcattcctgttaacatttttattttttcaaggtaacaggaaattgcatacaaatgacagtagatccttgcctctttatttttatctaaataaaagataactcaagatgaattctcaagaaagaaaaaaagctatatacataagggactatatcttccttcatcgtctacttggaaccagtagctgtgttgctgtcatagaatcaggaaacaggttgtggtaagttggaagaggtacatatgctgctgttatcattttaccagcaaaccacctgccatgcaatgcattgacagcagcaatagctgcagcaattgatgggcacttcacatacacattgccctgagctgaatttttgtcaacataaatatgaataactcctccatgtttattacattcttcaatcacatcatccttaatctcggtatcccatccaacttcttcttctgtttgagggttaaacatgttagagagttggaaacattgtgttgcaagtggctgaacagaggcagctgcagctaaagctgaagcttcagtctgctgggaaagtcttgtttgcaaatctgccacagcaccaaatgccaaagagccactcatctgtagagcttgctgtgctgctggcggaatctgcaaacctgtaccctctgcaagtcttgccattaactgaagacgaccagttgttcccaaatcaattccagtcctttccagttcatcactgtccaaaaatgaactagcactcgaagcatcagtacgttcagtaacatgaccaactttcattggtcttcctgctagttcaaatccattaagttgttccaaagcctttttggcacattctgagtcagaaaatgtaataaatccatatcccttggatcgaccagtttcactgtccatcatcagctggatactttcaattcttccaaaaggctcaaagatcccacgaagcatatcttcagttatgttgaagtgtaatgagcccacataaagcctcataggtccagcacttcccttttgtaaattgtttgccattgctgcagctctgtttttttctgcctgtgatgcctgtactatgattggcacgcctaaaactcgttggccagttaatcctattgctagaggcactgagctaacatcgacgaactccacataagcaattcctttggaacgtcttgaatttctgtcagaaatcatcctcacatctcgaacctttcctactgtagagaaaaactcttccaaatcccttggtcgaattcttgccgccagctgcatacagaagactgtccttgcatctctttcctcaggagttaaattatcaataggttctctcacagggctcttgtcttttctgaatggacttttgcttcgggaacgtcgtctgtaaggacttctgtagcggcctctaaatcttcgatctcgacttcttgagcggctccgtcgcctctctttgcttctacttcgctttctttcacggcttttgctctttttcctttctctgtctctacttcgcttccgttccttacttttgcttctctttcgttcatgactacgacttctgctcttgctttttttcctctttttgctacgttcttcatggccgttggcactgctcaacttgttctcatccttcttgtaaggagcctcaagcattgcttcaatatcaatatcgtctgccattttctctaaacgcctgttccggccttcgggcgcctgtggtgctcgtgttcgggaagagattgctgctgctgctgctgctgctgccgccgccgccgcttctgttgctactgttaagcccctaggcccaggccgcggaaccgcccagcccgaatatcgggttccaaggacggctaggcccgagagaatctaaaaaaaacaatggaattagagaagcccacgcgggagagcaggacggcggcttcggcagctcaggatccacccctgcgacagcgtcgacaagctccctgaaatggcggccgctgcttccctgtactcacattcaccagcacacat

SEQ ID NO: 16900 - RNA, 797 nt, Homo sapiens
  source 1..797: mol_type = other RNA
tacttttctaggttgttggggagagtgatagacaaagttctggattctgggcatcgtcggcgcatgcttgtaatcctacttgggaggttgagacaggaggatcacttgaggctaggagttggaggctgcagtgtactatgttcgcatctgtgaatagccactgcactctagcctggacaatatagtgagaacccatctcaaaaaaaaaaaaaaaaaaaaaaaggcaaagttctagatcctaactggaagagttaggccaagaaggaagaagaggttctgggagctgctggctactcctcatcctcctcactatcgagatacttgtgggtggcgtagcccatcagggcaccaatattacctatgacgacgctgctgccaccagccccgaggctctgcagcgtggccactagccccccggcgggcacgccgcccccattcaggatcgcagaccagctcatcagcgaggcagccaccgagttggccgcgatgccggcgccggtgaagcccagcgcgggcagcccggcgactgcgagtcctcctccgacggccatgaaggtcagggccttccagaacccggagccgctgtccgagctctccgagcactttttcttacccgcattctcacctgcctccaccccactgcaagtgaagagcagcaggtagcacaagaaaagcgataccgccttctgccgcatggtggcgccgcgcgcgggctccgtcactagaccttggaggagagaagagaagcaatcttcagcccggagcctgctgatagatgggcacagcagcgagtaaac

SEQ ID NO: 16901 - RNA, 809 nt, Homo sapiens
  source 1..809: mol_type = other RNA
tacttttctaggttgttggggagagtgatagacaaagttctggattctgggcatcgtcggcgcatgcttgtaatcctacttgggaggttgagacaggaggatcacttgaggctaggagttggaggctgcagtgtactatgttcgcatctgtgaatagccactgcactctagcctggacaatatagtgagaacccatctcaaaaaaaaaaaaaaaaaaaaaaaggcaaagttctagatcctaactggaagagttaggccaagaaggaagaagaggttctgggagctgctggctactcctcatcctcctcactatcgagatacttgtgggtggcgtagcccatcagggcaccaatattacctatgacgacgctgctgccaccagccccgaggctctgcagcgtggccactagccccccggcgggcacgccgcccccattcaggatcgcagaccagctcatcagcgaggcagccaccgagttggccgcgatgccggcgccggtgaagcccagcgcgggcagcccggcgactgcgagtcctcctccgacggccatgaaggtcagggccttccagaacccggagccgctgtccgagctctccgagcactttttcttacctgcatccttacccgcattctcacctgcctccaccccactgcaagtgaagagcagcaggtagcacaagaaaagcgataccgccttctgccgcatggtggcgccgcgcgcgggctccgtcactagaccttggaggagagaagagaagcaatcttcagcccggagcctgctgatagatgggcacagcagcgagtaaac

SEQ ID NO: 16902 - RNA, 785 nt, Homo sapiens
  source 1..785: mol_type = other RNA
tacttttctaggttgttggggagagtgatagacaaagttctggattctgggcatcgtcggcgcatgcttgtaatcctacttgggaggttgagacaggaggatcacttgaggctaggagttggaggctgcagtgtactatgttcgcatctgtgaatagccactgcactctagcctggacaatatagtgagaacccatctcaaaaaaaaaaaaaaaaaaaaaaaggcaaagttctagatcctaactggaagagttaggccaagaaggaagaagaggttctgggagctgctggctactcctcatcctcctcactatcgagatacttgtgggtggcgtagcccatcagggcaccaatattacctatgacgacgctgctgccaccagccccgaggctctgcagcgtggccactagccccccggcgggcacgccgcccccattcaggatcgcagaccagctcatcagcgaggcagccaccgagttggccgcgatgccggcgccggtgaagcccagcgcgggcagcccggcgactgcgagtcctcctccgacggccatgaaggtcagggccttccagaacccggagccgctgtccgagctctccgagcactttttcttacctgcctccaccccactgcaagtgaagagcagcaggtagcacaagaaaagcgataccgccttctgccgcatggtggcgccgcgcgcgggctccgtcactagaccttggaggagagaagagaagcaatcttcagcccggagcctgctgatagatgggcacagcagcgagtaaac

SEQ ID NO: 16903 - RNA, 904 nt, Homo sapiens
  source 1..904: mol_type = other RNA
tacttttctaggttgttggggagagtgatagacaaagttctggattctgggcatcgtcggcgcatgcttgtaatcctacttgggaggttgagacaggaggatcacttgaggctaggagttggaggctgcagtgtactatgttcgcatctgtgaatagccactgcactctagcctggacaatatagtgagaacccatctcaaaaaaaaaaaaaaaaaaaaaaaggcaaagttctagatcctaactggaagagttaggccaagaaggaagaagaggttctgggagctgctggctactcctcatcctcctcactatcgagatacttgtgggtggcgtagcccatcagggcaccaatattacctatgacgacgctgctgccaccagccccgaggctctgcagcgtggccactagccccccggcgggcacgccgcccccattcaggatcgcagaccagctcatcagcgaggcagccaccgagttggccgcgatgccggcgccggtgaagcccagcgcgggcagcccggcgactgcgagtcctggaggaacaggagcaggtgagggagcgtccgcggcagaggcccgccccgcctgcccgagatcctcgccctccagacccacctcctccgacggccatgaaggtcagggccttccagaacccggagccgctgtccgagctctccgagcactttttcttacctgcctccaccccactgcaagtgaagagcagcaggtagcacaagaaaagcgataccgccttctgccgcatggtggcgccgcgcgcgggctccgtcactagaccttggaggagagaagagaagcaatcttcagcccggagcctgctgatagatgggcacagcagcgagtaaacggttctccggctgaaggctggctttttatcatcactt

SEQ ID NO: 16904 - RNA, 1300 nt, Homo sapiens
  source 1..1300: mol_type = other RNA
tagaccatctttctagagtatgctatagatcccattctccccttgtttaaatcttctcaaggtctccccctcccaggacacaatccatgctctgtggtctggggtctgagccctgccttgtgcagcccctgcccctctctgggctctattcccaccatcccttcggtcccaggtgtagtcaactacagatgcctgctctctttccactgagccactgagcctggtgcatgctgttccctttgcatggaaccactcccatgttacaaggctcctgctttattaagaaataaatcaccaaacaggtcacctgtgtgttttaaatattcacattgaagacattaatgcctttggtgcatcaaaaagacattgcattataattgcgcttgtcaaatgataatttcagggcttagaacagagttctcaacctcggtgctgttgacatttggggctggatgattctttgtggtggaggctgtcctgtgcactagacagggatgttcagcagcagccctgcctggcctccacccaggagatgccagtagcaactcctccagtcattgccaaatgtcccctggggagggaggactgtccctgttgagaaccactgatttaggagatgaactcctcatgcccccaggacagggtggtctgcaatgggtacatgatcatagccatgtgatgaacaccttcttcccaccttgaaatgttccatgactgaatgaactacctccctggggaaggatgtccagtgtcgacatccaagacccttcatgtgtgtgaggccgaccctgctggaacctccctctccaagccctgccaaggcgtcacctcttctgaccagccttcccagacgccccagacagtgtcacctctccttccagcgagtgttgcagctgcattcgcacattggtgtgtgtctgctccttccccagagcctggggttgggagttcccagaattgagtggaacacttctttggatttgctgtccgctgcagccttggccctggtttcacatcccctccctcactgactcgctgtgtgaccttgagcactgtgtgtctctgagcctggttcatccaagagtttaccgacggccctcgtgtgccagccactgtcctagacagggacagactttcccgcctttgtggagcttaccccggaagaccaaggctggaatcccgtggctgatcctgcctctgccctttggctcccgggactcagcccacaccacctgggtcacagagcatcccattcccacacaccgttgtggccacctcaccagcaggggcaggcccatat

SEQ ID NO: 16905 - RNA, 3648 nt, Homo sapiens
  source 1..3648: mol_type = other RNA
tagaggaagctgtggagagaagggtgttaacattggctaatcagaaccaggcccacaattgggcagctcacacataccgttttgcttgttgacataccaacccaatgacaatagccttgaccatacagatgagaatgctaaggaccagaatgttaagaacttgaccaagctcacactgtaagtcactgagcccaaattcaaacctaattctgacttcaaatatcttgttctcttcacattgaatctctatctccaagtaatttctttttcatcagaatttgagtctaatgctcctattccaggccagagggaagagagacatggaaggaaggctctactaccatgtatacagacgctagagaactaggcacttaggaatgtgtctgttgcctgggaaaccacacctggcacagagacagtcctgagatccctggcactcactaaccagccccttccaagggaggaagtaacttcagccaactcccgaagggcctagaggagtggcattgcctcctaccccaaagactgcttccacttcaaccatcagccaccaacaccaaatttatccagaggcttcttacttgtccagcactagaaaaaaaaactacacagcagtgggatcagaaatcctacagtccagcagacacctccaatatcttcggcaacctctcctcacaacagaaagggcagcatctaagggatccagaaagccaatgtgccaggacttgccaggactcagagaaggtaatcgacattgggcattgcttcaggggtgctgggaaagctctccaccctgcagacccacaccaggtggatggtatttgagataccaattcagaactgcttctctgtggcttagggctctagtgcaggttaaaatgcaggggacacttacaactgtggcagccattgcaaacttagcatgaattgctttccagtctaattacgaaaacaggttctgaaagggaggtaaaaagacaaaaataggatgactctggatgtttactgtggaggcctcaaatagaaaagtcaaagtgactttgtatacattccccattcacagcttgacaggacgggaaagttcaccacttaacgtttttaagagttgatggaagccaccaatccaataaggtgtcccctggagcccatccagaatccatcctttagtccatgagagttgagctccagcttccctctcctgactccatatcccagctgtggttctgtggtttggtgtacattgtgcaggttggaagtggcctgttttcctggaaagaatgaaatgtgcccaaatggaaagacaaaccaggtcccaatcttggatttgggaatatgggttcctggttccccagaatccagctgaggaattttctgacttcagttagacagagaaaatgacatgggaacagatgtgcaactccaaacatgcttgacagcataggctacgaacctgggcagcccctataccaggcccctctcccaagagcaagctggctctgagaatctgagaagtgaagaattcaagcttttcctacaggcttatgacagaaattatgccatttgggtatgtatccaaattatataattgtgattctgggtcatagctttcataatctttcaatgtttgcaaaatgaacagatattaatatcagaagaaagggggaacacatcgttcaagtcattgctattgttaatgtggaaactacttcatagtgctatcttcacttctgcctgaactccaagaggtctttaaatatattttatatatatgtatgttttggagacatggtctcactctgtcgcccaggctggaatgcagtggcacaatcagggctcactgcaaccttcacctcctgggctcaagcgatcctcccacctcagcctaccaagcagccgcacgtgtcaccatgcccagctaatttttgtagtttgtgtagagatgaggtttcaccatgttgcccaggctggtctcaaactcctgggctcaagcaatccacccaccttagcctcccaaagtgcgaggattacaggtgtgagccaccgcgcccagcctaaatatctcattttgaggcatacacagaaatcatcctcaggattcttaggctctctccttccatctaagtatgtcccacaatacaccatgcatatgaatttgactcaataactacacacttgagggaaacataagtataaatttactatccacctagtggtagctaggtaaaattgcaggcataaagataaaaaagaaatcatcaactttgtagttcctcagcttcaaacccaaacctgcaagggagaggagagacccagacgcctcagggaccaggcagataatacaaataaatgaaacaggccaggtgagagagtacaagtcttgccaaaagaagaaacccctacttagtttcaattgattgtcctcttctgaaaatgcagatcagaattgccacacattctgaccgatcgagagaggccagaaattctaattttaatgtgaaacctcttgatttcttagacggtggctcaattttcttgaaaacactaggtgagctaaataaagctgacagtccaccagttttcaatactcctcttgcagagagtgaatggcatctcccctaactgtagtattagactgccactcaccagccacagtttgcaactgcaaaagaggcataaactgacggggatctcctgctttactatgcacacacagctgaactctccagccgtggagaacaactaactctataggaaaaagtagaaggctaagctgagccatccagggatggcggcaggggccttcatggctagctgctggcctgtaggcactaaattgcagactgctcctgcaggaagccttcagggcctgggaggcctttatctggctcagaagctagggctgcttctcgaaggacttccaaatgctcctcagcagccgacagagactggtcaatccagtccaggcctcccgtcagatggcaggcattccttgtcaccagcaccaggtgactgacagacaggagcagggcagtcgtccgtgcgtccaggagtttggggtccaacggagggtacatcgacttcacaacatcatccaccctggggctgatccgcttggccaccacaatgatgtcgctgacactggctgaagtcttcatcttggccccagagcccattgtcatggcaacaagcttctctgtcagagtgtgacaaatcttcaagatggcaatgcagtgggacatgagacccgaggcatcttcgatccagtcttcattctccagaatggcctcaatgtgggggttggtgataacgacatcgtccagttctaactcagagggctcagactgggtctccatggcaccaatgaggtccacaatgggcttagaatcatagcgctgcagcaggtctcgcggccggcagtagcgctgcctgcaaaccagcaccaaggctgcaaacgaagccagaaagatggtggccagcacacctatggcaacaatcaccacagtctccatgcttccagagggctcctgactcagtcccggtcacatcctcctcatgggctaaagctcaggctgtggctcccgggcgcatcccgcgactgccccgccgatggcaaagtccgggcgcgggcgcgggcctgcagcggagcat

SEQ ID NO: 16906 - RNA, 3724 nt, Homo sapiens
  source 1..3724: mol_type = other RNA
tagaggaagctgtggagagaagggtgttaacattggctaatcagaaccaggcccacaattgggcagctcacacataccgttttgcttgttgacataccaacccaatgacaatagccttgaccatacagatgagaatgctaaggaccagaatgttaagaacttgaccaagctcacactgtaagtcactgagcccaaattcaaacctaattctgacttcaaatatcttgttctcttcacattgaatctctatctccaagtaatttctttttcatcagaatttgagtctaatgctcctattccaggccagagggaagagagacatggaaggaaggctctactaccatgtatacagacgctagagaactaggcacttaggaatgtgtctgttgcctgggaaaccacacctggcacagagacagtcctgagatccctggcactcactaaccagccccttccaagggaggaagtaacttcagccaactcccgaagggcctagaggagtggcattgcctcctaccccaaagactgcttccacttcaaccatcagccaccaacaccaaatttatccagaggcttcttacttgtccagcactagaaaaaaaaactacacagcagtgggatcagaaatcctacagtccagcagacacctccaatatcttcggcaacctctcctcacaacagaaagggcagcatctaagggatccagaaagccaatgtgccaggacttgccaggactcagagaaggtaatcgacattgggcattgcttcaggggtgctgggaaagctctccaccctgcagacccacaccaggtggatggtatttgagataccaattcagaactgcttctctgtggcttagggctctagtgcaggttaaaatgcaggggacacttacaactgtggcagccattgcaaacttagcatgaattgctttccagtctaattacgaaaacaggttctgaaagggaggtaaaaagacaaaaataggatgactctggatgtttactgtggaggcctcaaatagaaaagtcaaagtgactttgtatacattccccattcacagcttgacaggacgggaaagttcaccacttaacgtttttaagagttgatggaagccaccaatccaataaggtgtcccctggagcccatccagaatccatcctttagtccatgagagttgagctccagcttccctctcctgactccatatcccagctgtggttctgtggtttggtgtacattgtgcaggttggaagtggcctgttttcctggaaagaatgaaatgtgcccaaatggaaagacaaaccaggtcccaatcttggatttgggaatatgggttcctggttccccagaatccagctgaggaattttctgacttcagttagacagagaaaatgacatgggaacagatgtgcaactccaaacatgcttgacagcataggctacgaacctgggcagcccctataccaggcccctctcccaagagcaagctggctctgagaatctgagaagtgaagaattcaagcttttcctacaggcttatgacagaaattatgccatttgggtatgtatccaaattatataattgtgattctgggtcatagctttcataatctttcaatgtttgcaaaatgaacagatattaatatcagaagaaagggggaacacatcgttcaagtcattgctattgttaatgtggaaactacttcatagtgctatcttcacttctgcctgaactccaagaggtctttaaatatattttatatatatgtatgttttggagacatggtctcactctgtcgcccaggctggaatgcagtggcacaatcagggctcactgcaaccttcacctcctgggctcaagcgatcctcccacctcagcctaccaagcagccgcacgtgtcaccatgcccagctaatttttgtagtttgtgtagagatgaggtttcaccatgttgcccaggctggtctcaaactcctgggctcaagcaatccacccaccttagcctcccaaagtgcgaggattacaggtgtgagccaccgcgcccagcctaaatatctcattttgaggcatacacagaaatcatcctcaggattcttaggctctctccttccatctaagtatgtcccacaatacaccatgcatatgaatttgactcaataactacacacttgagggaaacataagtataaatttactatccacctagtggtagctaggtaaaattgcaggcataaagataaaaaagaaatcatcaactttgtagttcctcagcttcaaacccaaacctgcaagggagaggagagacccagacgcctcagggaccaggcagataatacaaataaatgaaacaggccaggtgagagagtacaagtcttgccaaaagaagaaacccctacttagtttcaattgattgtcctcttctgaaaatgcagatcagaattgccacacattctgaccgatcgagagaggccagaaattctaattttaatgtgaaacctcttgatttcttagacggtggctcaattttcttgaaaacactaggtgagctaaataaagctgacagtccaccagttttcaatactcctcttgcagagagtgaatggcatctcccctaactgtagtattagactgccactcaccagccacagtttgcaactgcaaaagaggcataaactgacggggatctcctgctttactatgcacacacagctgaactctccagccgtggagaacaactaactctataggaaaaagtagaaggctaagctgagccatccagggatggcggcaggggccttcatggctagctgctggcctgtaggcactaaattgcagactgctcctgcaggaagccttcagggcctgggaggcctttatctggctcagaagctagggctgcttctcgaaggacttccaaatgctcctcagcagccgacagagactggtcaatccagtccaggcctcccgtcagatggcaggcattccttgtcaccagcaccaggtgactgacagacaggagcagggcagtcgtccgtgcgtccaggagtttggggtccaacggagggtacatcgacttcacaacatcatccaccctggggctgatccgcttggccaccacaatgatgtcgctgacactggctgaagtcttcatcttggccccagagcccattgtcatggcaacaagcttctctgtcagagtgtgacaaatcttcaagatggcaatgcagtgggacatgagacccgaggcatcttcgatccagtcttcattctccagaatggcctcaatgtgggggttggtgataacgacatcgtccagttctaactcagagggctcagactgggtctccatggcaccaatgaggtccacaatgggcttagaatcatagcgctgcagcaggtctcgcggccggcagtagcgctgcctgcaaaccagcaccaaggctgcaaacgaagccagaaagatggtggccagcacacctatggcaacaatcaccacagtctccatgcttccagagggctcctgactcagtcccggtcacatcctcctcatgggctaaagctgctggaagtggcaaattggggaagaggatggcaggtgctaggttcctccacgacacctgcagagacctgagggcctcaggctgtggctcccgggcgcatcccgcgactgccccgccgatggcaaagtccgggcgcgggcgcgggcctgcagcggagcat

SEQ ID NO: 16907 - RNA, 3796 nt, Homo sapiens
  source 1..3796: mol_type = other RNA
tagaggaagctgtggagagaagggtgttaacattggctaatcagaaccaggcccacaattgggcagctcacacataccgttttgcttgttgacataccaacccaatgacaatagccttgaccatacagatgagaatgctaaggaccagaatgttaagaacttgaccaagctcacactgtaagtcactgagcccaaattcaaacctaattctgacttcaaatatcttgttctcttcacattgaatctctatctccaagtaatttctttttcatcagaatttgagtctaatgctcctattccaggccagagggaagagagacatggaaggaaggctctactaccatgtatacagacgctagagaactaggcacttaggaatgtgtctgttgcctgggaaaccacacctggcacagagacagtcctgagatccctggcactcactaaccagccccttccaagggaggaagtaacttcagccaactcccgaagggcctagaggagtggcattgcctcctaccccaaagactgcttccacttcaaccatcagccaccaacaccaaatttatccagaggcttcttacttgtccagcactagaaaaaaaaactacacagcagtgggatcagaaatcctacagtccagcagacacctccaatatcttcggcaacctctcctcacaacagaaagggcagcatctaagggatccagaaagccaatgtgccaggacttgccaggactcagagaaggtaatcgacattgggcattgcttcaggggtgctgggaaagctctccaccctgcagacccacaccaggtggatggtatttgagataccaattcagaactgcttctctgtggcttagggctctagtgcaggttaaaatgcaggggacacttacaactgtggcagccattgcaaacttagcatgaattgctttccagtctaattacgaaaacaggttctgaaagggaggtaaaaagacaaaaataggatgactctggatgtttactgtggaggcctcaaatagaaaagtcaaagtgactttgtatacattccccattcacagcttgacaggacgggaaagttcaccacttaacgtttttaagagttgatggaagccaccaatccaataaggtgtcccctggagcccatccagaatccatcctttagtccatgagagttgagctccagcttccctctcctgactccatatcccagctgtggttctgtggtttggtgtacattgtgcaggttggaagtggcctgttttcctggaaagaatgaaatgtgcccaaatggaaagacaaaccaggtcccaatcttggatttgggaatatgggttcctggttccccagaatccagctgaggaattttctgacttcagttagacagagaaaatgacatgggaacagatgtgcaactccaaacatgcttgacagcataggctacgaacctgggcagcccctataccaggcccctctcccaagagcaagctggctctgagaatctgagaagtgaagaattcaagcttttcctacaggcttatgacagaaattatgccatttgggtatgtatccaaattatataattgtgattctgggtcatagctttcataatctttcaatgtttgcaaaatgaacagatattaatatcagaagaaagggggaacacatcgttcaagtcattgctattgttaatgtggaaactacttcatagtgctatcttcacttctgcctgaactccaagaggtctttaaatatattttatatatatgtatgttttggagacatggtctcactctgtcgcccaggctggaatgcagtggcacaatcagggctcactgcaaccttcacctcctgggctcaagcgatcctcccacctcagcctaccaagcagccgcacgtgtcaccatgcccagctaatttttgtagtttgtgtagagatgaggtttcaccatgttgcccaggctggtctcaaactcctgggctcaagcaatccacccaccttagcctcccaaagtgcgaggattacaggtgtgagccaccgcgcccagcctaaatatctcattttgaggcatacacagaaatcatcctcaggattcttaggctctctccttccatctaagtatgtcccacaatacaccatgcatatgaatttgactcaataactacacacttgagggaaacataagtataaatttactatccacctagtggtagctaggtaaaattgcaggcataaagataaaaaagaaatcatcaactttgtagttcctcagcttcaaacccaaacctgcaagggagaggagagacccagacgcctcagggaccaggcagataatacaaataaatgaaacaggccaggtgagagagtacaagtcttgccaaaagaagaaacccctacttagtttcaattgattgtcctcttctgaaaatgcagatcagaattgccacacattctgaccgatcgagagaggccagaaattctaattttaatgtgaaacctcttgatttcttagacggtggctcaattttcttgaaaacactaggtgagctaaataaagctgacagtccaccagttttcaatactcctcttgcagagagtgaatggcatctcccctaactgtagtattagactgccactcaccagccacagtttgcaactgcaaaagaggcataaactgacggggatctcctgctttactatgcacacacagctgaactctccagccgtggagaacaactaactctataggaaaaagtagaaggctaagctgagccatccagggatggcggcaggggccttcatggctagctgctggcctgtaggcactaaattgcagactgctcctgcaggaagccttcagggcctgggaggcctttatctggctcagaagctagggctgcttctcgaaggacttccaaatgctcctcagcagccgacagagactggtcaatccagtccaggcctcccgtcagatggcaggcattccttgtcaccagcaccaggtgactgacagacaggagcagggcagtcgtccgtgcgtccaggagtttggggtccaacggagggtacatcgacttcacaacatcatccaccctggggctgatccgcttggccaccacaatgatgtcgctgacactggctgaagtcttcatcttggccccagagcccattgtcatggcaacaagcttctctgtcagagtgtgacaaatcttcaagatggcaatgcagtgggacatgagacccgaggcatcttcgatccagtcttcattctccagaatggcctcaatgtgggggttggtgataacgacatcgtccagttctaactcagagggctcagactgggtctccatggcaccaatgaggtccacaatgggcttagaatcatagcgctgcagcaggtctcgcggccggcagtagcgctgcctgcaaaccagcaccaaggctgcaaacgaagccagaaagatggtggccagcacacctatggcaacaatcaccacagtctccatgcttccagagggctcctgactcagtcccggtcacatcctcctcatgggctaaagctgctggaagtggcaaattggggaagaggatggcaggtgctaggttcctccacgacacctgcagagacctgagggcctcgggcctcccaaagtgctgggattacacgcgtgagacaccgagcccggccttaaaatagctttttaaaccctcaggctgtggctcccgggcgcatcccgcgactgccccgccgatggcaaagtccgggcgcgggcgcgggcctgcagcggagcat

SEQ ID NO: 16908 - RNA, 388 nt, Homo sapiens
  source 1..388: mol_type = other RNA
tagataaaatattggtacctgctgttggttaccaagaatgctttgcaattaacaactcattaacagaatgtacgaattctgccagtgctaaaatatcacgctgtgaatttaataaagaacatgtgaggtaagtttttttttttttttaagatagtatggcctctactatcagagagagagaaaagaaagtgacaaagaaaaaggaggagagagagaagtgggggtaagcatgaataagcagtatcttatttgctggtggattcattgccacatcccctggtcacagtatcctccccggtacgatgatgacaatggccctctgcctggagtccgctctcaacagcaggagggtcaccatgccctggaagaagccatgctgctcccacaa

SEQ ID NO: 16909 - RNA, 470 nt, Homo sapiens
  source 1..470: mol_type = other RNA
tagatctttgactctggcagtctccaggagaggccaatttatgtggttgacctgagccacagacaacaaaaacaaacagtgccaacagccatggtcccacaggatatttctcctcttgcggcctcagggttttggctacgttccccctctgggtgatgtttttgctgtgcttctcgttagccatccggatccgctgtttggccaccatggcttgtgcgctctgaaatgctcccaccccgcgcggccaccgaggcaggcgcgaccgcacgtcctcccgcgccgagcggccggagcgcagcgcgcagagccggggccctgcagtgtcgcggtcctgtagccgaatgctgcggggccgaaggttcgggcgaccacggcgtttgtgagcgcgtcggggacggggacgcggcccctcctgtgtttgtcggccggtgacccaccccagccccggggaagggatgagggcggccgcg

SEQ ID NO: 16910 - RNA, 410 nt, Homo sapiens
  source 1..410: mol_type = other RNA
tagatctttgactctggcagtctccaggagaggccaatttatgtggttgacctgagccacagacaacaaaaacaaacagtgccaacagccatggtcccacaggatatttctcctcttgcggcctcagggttttggctacgttccccctctgggtgatgtttttgctgtgcttctcgttagccatccggatccgctgtttggccaccatggcttgtgcgctctgaaatgctcccacctgcaaggattccccctgcgttagctcctgcgacagggccgagcgcgtcccgccgaggcccccgcggcccacccgggcgctgcaggtggcaaggcgtggccccgagccctgcgcaccccgctccccgagccccggctagccgactccagagagaggccgcagcccggacggaagt

SEQ ID NO: 16911 - RNA, 458 nt, Homo sapiens
  source 1..458: mol_type = other RNA
tagatctttgactctggcagtctccaggagaggccaatttatgtggttgacctgagccacagacaacaaaaacaaacagtgccaacagccatggtcccacaggatatttctcctcttgcggcctcagggttttggctacgttccccctctgggtgatgtttttgctgtgcttctcgttagccatccggatccgctgtttggccaccatggcttgtgcgctctgaaatgctcccacctgcaaggattccccctgcgttagctcctgcgacagggccgagcgcgtcccgccgaggcccccgcggcccacccgggcgctgcaggtggcaaggcgtggccccgagccctgcgcaccccgctccccgagccccggctagccgactccagagagaggccgcagcccggacggaagtaatctctcatctcaggaaaccctttccgacttcctcgccatccttccg

SEQ ID NO: 16912 - RNA, 2749 nt, Homo sapiens
  source 1..2749: mol_type = other RNA
tagatctttgactctggcagtctccagggctctgagggtcccctccgatgggagcaccttccattcccagatcccaagttagaccaggggcttccgaagctggaatctgctctctggaggcaaggctgcccaaacagcctctgtacagagtggggcgcacctcagacactcctcgggatgtagaaccagcattcttgctgctgagccactgccttgcattaggcagcagtggaggaaggggacggaggagagagaattgggaggcagaagggctgggtgtgggcctgggtcctcaggggacgtcttgacccccagctgctggcacttctccatcctcctgccatcactggagcagacatcagggacgagacaagatgccacctcctgccaccacagggcctgctctctcccccaccccccgccagaatacttgtccccctgcttggcagttgccctgggctctctgagtccaggaggtgggccctgctttgcaggggggcagttcctcaggtcaccacttgctggatccagctgatcacacctgtgatgcgggtgtagacgccgaagtagttaggccggccacagcccaggccccagctgaccagccccgccaggaaccagcggccactgagtgccttgcacaccagcggaccacctgagtcaccctgacaggcatccttcttgcccttgcggtagccggcacacagcatgcgtggcgtcacctggtagcgatagacctcgctgcacaggtcctgtgggatcaactgcacatccactttctgcagagcgttgctgatggggcagcaacatgtctctgagccttggtttctccatccataaaatagggccacagcatccgcccgtagggcgccctcgcgcaaggcgccccagcccgtaatccagcagtgcaggccgggctcgaagaagtgggagcgcgcgggcaggcagacggggcgcacggcggccgagcgcaccaccgggtggtcgagctgcagcagcgccacgtcgtagtcatggctgtcctcttcgtggtacgggtgcaggagcaggcggctcaccttgaaggacacctctccaggccagcgcgagttctgccacaccttgcccaggaacacggtccacagcaccgtggaggccatgctgtcctcctggaagcagtgggcagctgttatcacccagcggtcagcgatgagggcccccccacagatgtgtcgaccccgaacctggaggctggcctgccatggccactcaccctcggaggacacagctccaccaacaatgcggctggaggggccctggaggccacagtcacagtgctcctcatccgagccgtccctgcagtcgggccgcccatcacactgcgggttgggcttcttcacgcagctccggtcctcacactggaaggtgaatgtcccacatggcaccccttcctggcactgctcttcgtcgctgccgttgagacaatcaggctgcccatcacagaccttgggcagtgagatgcatgtgctgtcctctttgcactggaatgtggctctgcaaacgcagtttctctcatccaggccgttggggcagtccttgaccccatcacaggcagggacacagagtccattcacagaacagaggaactctccagggcaggggtccgactggttgtacaagccatagtgcacccgcacaccgggcccggtgagggagatctgggaggtgaagttgatggtgatcccggccgtggccaccacggggatcctctcggcgtagggctgcaggatgcgcaagccacacagcctcctgttctggatcgtccactggccctgggtgcacggcaaatcatacttctgcctcctcagtgcataggcatcaaaccagagggccaagccgtagtccagagagggcaccgtgaggtgccaggagcagtgggtttggggcgagtagtagctggggaagtacggggtgctgaggacgccctgggagtcgagcctgttgtccagcgtcaggttcacttcacaggcctggaagaccaccggctgcacggagagcacgaaggggtcgtagtagctgtgcaggcccttcttccagacgaccgccatgatggcccccgacgccagaacctccaccacgggctcctggcggctgcagccgtacaccccaaaggaatagacggagctggagttgtagtaagttcccaggcgggtgctggtgatgagctccttgagcatcttctgggctttggcggtttcactgcggaaggcactagattcccggcgggtaagatcctgggagaagtggcgattgagtacacgcagactgcctgagtacacctggctgaccatcacctccgccttgtaccctaggaaataccagagtagcacccccgccgaagccagcacgagcagggccagcagcacaaacaggggcaccaggcggaggtagccccgggcttttctcttggagtcctcacaggccttgaacatcccctccggctccgcttcctcgccatcacctccgtccccctgcccgccagccacctggggggcctcggccacgggcatcctttgggagcggcagataggtgccgggcctgcacacaggcctcaggagcctctgtttgtccaggccaaggcctccccacccccacccagccagcccaggctggatcaatggcctagagccatgaccagggtgtctggcccttgtcccctgtggcctgtggcctcaggctccatggaactcctcctgctgggtcctggac

SEQ ID NO: 16913 - RNA, 3055 nt, Homo sapiens
  source 1..3055: mol_type = other RNA
tagatctttgactctggcagtctccagggctctgagggtcccctccgatgggagcaccttccattcccagatcccaagttagaccaggggcttccgaagctggaatctgctctctggaggcaaggctgcccaaacagcctctgtacagagtggggcgcacctcagacactcctcgggatgtagaaccagcattcttgctgctgagccactgccttgcattaggcagcagtggaggaaggggacggaggagagagaattgggaggcagaagggctgggtgtgggcctgggtcctcaggggacgtcttgacccccagctgctggcacttctccatcctcctgccatcactggagcagacatcagggacgagacaagatgccacctcctgccaccacagggcctgctctctcccccaccccccgccagaatacttgtccccctgcttggcagttgccctgggctctctgagtccaggaggtgggccctgctttgcaggggggcagttcctcaggtcaccacttgctggatccagctgatcacacctgtgatgcgggtgtagacgccgaagtagttaggccggccacagcccaggccccagctgaccagccccgccaggaaccagcggccactgagtgccttgcacaccagcggaccacctgagtcaccctgacaggcatccttcttgcccttgcggtagccggcacacagcatgcgtggcgtcacctggtagcgatagacctcgctgcacaggtcctgtgggatcaactgcacatccactttctgcagagcgttgctgatggggcagcaacatgtctctgagccttggtttctccatccataaaatagggccacagcatccgcccgtagggcgccctcgcgcaaggcgccccagcccgtaatccagcagtgcaggccgggctcgaagaagtgggagcgcgcgggcaggcagacggggcgcacggcggccgagcgcaccaccgggtggtcgagctgcagcagcgccacgtcgtagtcatggctgtcctcttcgtggtacgggtgcaggagcaggcggctcaccttgaaggacacctctccaggccagcgcgagttctgccacaccttgcccaggaacacggtccacagcaccgtggaggccatgctgtcctcctggaagcagtgggcagctgttatcacccagcggtcagcgatgagggcccccccacagatgtgtcgaccccgaacctggaggctggcctgccatggccactcaccctcggaggacacagctccaccaacaatgcggctggaggggccctggaggccacagtcacagtgctcctcatccgagccgtccctgcagtcgggccgcccatcacactgcgggttgggcttcttcacgcagctccggtcctcacactggaaggtgaatgtcccacatggcaccccttcctggcactgctcttcgtcgctgccgttgagacaatcaggctgcccatcacagaccttgggcagtgagatgcatgtgctgtcctctttgcactggaatgtggctctgcaaacgcagtttctctcatccaggccgttggggcagtccttgaccccatcacaggcagggacacagagtccattcacagaacagaggaactctccagggcaggggtccgactggttgtacaagccatagtgcacccgcacaccgggcccggtgagggagatctgggaggtgaagttgatggtgatcccggccgtggccaccacggggatcctctcggcgtagggctgcaggatgcgcaagccacacagcctcctgttctggatcgtccactggccctgggtgcacggcaaatcatacttctgcctcctcagtgcataggcatcaaaccagagggccaagccgtagtccagagagggcaccgtgaggtgccaggagcagtgggtttggggcgagtagtagctggggaagtacggggtgctgaggacgccctgggagtcgagcctgttgtccagcgtcaggttcacttcacaggcctggaagaccaccggctgcacggagagcacgaaggggtcgtagtagctgtgcaggcccttcttccagacgaccgccatgatggcccccgacgccagaacctccaccacgggctcctggcggctgcagccgtacaccgaggtgatgagcctcttctccaggggcccggccacgtcatacatggccagtcggtcccggcactctgccagcgtccactccagccggagtttgagcatgaggtccttggggccctgcaggtgccacaggcagctggaggccaggtggtcaggccccttcagccggaggacctggccctggcccacgtagctgtagcggtaacaacccagcgtggaattcaatgcagctatgtctttcacactggcttccaggatcactaggccctcggggtccacttcgtactcggccctgtaggggacggcagccgagctgttgactgtggacagcagctcctccaccagcagtgcctgcaccacctcggggctcagcatcagccggcggtgctcggggatttggagaatgaaccagaagaagcaggtgaggggtccctccccaaaggaatagacggagctggagttgtagtaagttcccaggcgggtgctggtgatgagctccttgagcatcttctgggctttggcggtttcactgcggaaggcactagattcccggcgggtaagatcctgggagaagtggcgattgagtacacgcagactgcctgagtacacctggctgaccatcacctccgccttgtaccctaggaaataccagagtagcacccccgccgaagccagcacgagcagggccagcagcacaaacaggggcaccaggcggaggtagccccgggcttttctcttggagtcctcacaggccttgaacatcccctccggctccgcttcctcgccatcacctccgtccccctgcccgccagccacctggggggcctcggccacgggcatcctggacaggcgagactaaaggagctgctggcctgagagagagaaaaggaggctgggcccatatactctgggga

SEQ ID NO: 16914 - RNA, 3153 nt, Homo sapiens
  source 1..3153: mol_type = other RNA
tagatctttgactctggcagtctccagggctctgagggtcccctccgatgggagcaccttccattcccagatcccaagttagaccaggggcttccgaagctggaatctgctctctggaggcaaggctgcccaaacagcctctgtacagagtggggcgcacctcagacactcctcgggatgtagaaccagcattcttgctgctgagccactgccttgcattaggcagcagtggaggaaggggacggaggagagagaattgggaggcagaagggctgggtgtgggcctgggtcctcaggggacgtcttgacccccagctgctggcacttctccatcctcctgccatcactggagcagacatcagggacgagacaagatgccacctcctgccaccacagggcctgctctctcccccaccccccgccagaatacttgtccccctgcttggcagttgccctgggctctctgagtccaggaggtgggccctgctttgcaggggggcagttcctcaggtcaccacttgctggatccagctgatcacacctgtgatgcgggtgtagacgccgaagtagttaggccggccacagcccaggccccagctgaccagccccgccaggaaccagcggccactgagtgccttgcacaccagcggaccacctgagtcaccctgacaggcatccttcttgcccttgcggtagccggcacacagcatgcgtggcgtcacctggtagcgatagacctcgctgcacaggtcctgtgggatcaactgcacatccactttctgcagagcgttgctgatggggcagcaacatgtctctgagccttggtttctccatccataaaatagggccacagcatccgcccgtagggcgccctcgcgcaaggcgccccagcccgtaatccagcagtgcaggccgggctcgaagaagtgggagcgcgcgggcaggcagacggggcgcacggcggccgagcgcaccaccgggtggtcgagctgcagcagcgccacgtcgtagtcatggctgtcctcttcgtggtacgggtgcaggagcaggcggctcaccttgaaggacacctctccaggccagcgcgagttctgccacaccttgcccaggaacacggtccacagcaccgtggaggccatgctgtcctcctggaagcagtgggcagctgttatcacccagcggtcagcgatgagggcccccccacagatgtgtcgaccccgaacctggaggctggcctgccatggccactcaccctcggaggacacagctccaccaacaatgcggctggaggggccctggaggccacagtcacagtgctcctcatccgagccgtccctgcagtcgggccgcccatcacactgcgggttgggcttcttcacgcagctccggtcctcacactggaaggtgaatgtcccacatggcaccccttcctggcactgctcttcgtcgctgccgttgagacaatcaggctgcccatcacagaccttgggcagtgagatgcatgtgctgtcctctttgcactggaatgtggctctgcaaacgcagtttctctcatccaggccgttggggcagtccttgaccccatcacaggcagggacacagagtccattcacagaacagaggaactctccagggcaggggtccgactggttgtacaagccatagtgcacccgcacaccgggcccggtgagggagatctgggaggtgaagttgatggtgatcccggccgtggccaccacggggatcctctcggcgtagggctgcaggatgcgcaagccacacagcctcctgttctggatcgtccactggccctgggtgcacggcaaatcatacttctgcctcctcagtgcataggcatcaaaccagagggccaagccgtagtccagagagggcaccgtgaggtgccaggagcagtgggtttggggcgagtagtagctggggaagtacggggtgctgaggacgccctgggagtcgagcctgttgtccagcgtcaggttcacttcacaggcctggaagaccaccggctgcacggagagcacgaaggggtcgtagtagctgtgcaggcccttcttccagacgaccgccatgatggcccccgacgccagaacctccaccacgggctcctggcggctgcagccgtacaccgaggtgatgagcctcttctccaggggcccggccacgtcatacatggccagtcggtcccggcactctgccagcgtccactccagccggagtttgagcatgaggtccttggggccctgcaggtgccacaggcagctggaggccaggtggtcaggccccttcagccggaggacctggccctggcccacgtagctgtagcggtaacaacccagcgtggaattcaatgcagctatgtctttcacactggcttccaggatcactaggccctcggggtccacttcgtactcggccctgtaggggacggcagccgagctgttgactgtggacagcagctcctccaccagcagtgcctgcaccacctcggggctcagcatcagccggcggtgctcggggatttggagaatgaaccagaagaagcaggtgaggggtccctccccaaaggaatagacggagctggagttgtagtaagttcccaggcgggtgctggtgatgagctccttgagcatcttctgggctttggcggtttcactgcggaaggcactagattcccggcgggtaagatcctgggagaagtggcgattgagtacacgcagactgcctgagtacacctggctgaccatcacctccgccttgtaccctaggaaataccagagtagcacccccgccgaagccagcacgagcagggccagcagcacaaacaggggcaccaggcggaggtagccccgggcttttctcttggagtcctcacaggccttgaacatcccctccggctccgcttcctcgccatcacctccgtccccctgcccgccagccacctggggggcctcggccacgggcatcctggttccgtagcgctgtgctgtccatgacggtagccgctggtcacccgtggctcttgagtcagtctgaactgagaaaagctgcacgggggagacgcacaccaggtttccaaggccaagtgcaaacaggatgtcaaccaacgcgataacaatttttatattgattttatgt

SEQ ID NO: 16915 - RNA, 3117 nt, Homo sapiens
  source 1..3117: mol_type = other RNA
tagatctttgactctggcagtctccagggctctgagggtcccctccgatgggagcaccttccattcccagatcccaagttagaccaggggcttccgaagctggaatctgctctctggaggcaaggctgcccaaacagcctctgtacagagtggggcgcacctcagacactcctcgggatgtagaaccagcattcttgctgctgagccactgccttgcattaggcagcagtggaggaaggggacggaggagagagaattgggaggcagaagggctgggtgtgggcctgggtcctcaggggacgtcttgacccccagctgctggcacttctccatcctcctgccatcactggagcagacatcagggacgagacaagatgccacctcctgccaccacagggcctgctctctcccccaccccccgccagaatacttgtccccctgcttggcagttgccctgggctctctgagtccaggaggtgggccctgctttgcaggggggcagttcctcaggtcaccacttgctggatccagctgatcacacctgtgatgcgggtgtagacgccgaagtagttaggccggccacagcccaggccccagctgaccagccccgccaggaaccagcggccactgagtgccttgcacaccagcggaccacctgagtcaccctgacaggcatccttcttgcccttgcggtagccggcacacagcatgcgtggcgtcacctggtagcgatagacctcgctgcacaggtcctgtgggatcaactgcacatccactttctgcagagcgttgctgatggggcagcaacatgtctctgagccttggtttctccatccataaaatagggccacagcatccgcccgtagggcgccctcgcgcaaggcgccccagcccgtaatccagcagtgcaggccgggctcgaagaagtgggagcgcgcgggcaggcagacggggcgcacggcggccgagcgcaccaccgggtggtcgagctgcagcagcgccacgtcgtagtcatggctgtcctcttcgtggtacgggtgcaggagcaggcggctcaccttgaaggacacctctccaggccagcgcgagttctgccacaccttgcccaggaacacggtccacagcaccgtggaggccatgctgtcctcctggaagcagtgggcagctgttatcacccagcggtcagcgatgagggcccccccacagatgtgtcgaccccgaacctggaggctggcctgccatggccactcaccctcggaggacacagctccaccaacaatgcggctggaggggccctggaggccacagtcacagtgctcctcatccgagccgtccctgcagtcgggccgcccatcacactgcgggttgggcttcttcacgcagctccggtcctcacactggaaggtgaatgtcccacatggcaccccttcctggcactgctcttcgtcgctgccgttgagacaatcaggctgcccatcacagaccttgggcagtgagatgcatgtgctgtcctctttgcactggaatgtggctctgcaaacgcagtttctctcatccaggccgttggggcagtccttgaccccatcacaggcagggacacagagtccattcacagaacagaggaactctccagggcaggggtccgactggttgtacaagccatagtgcacccgcacaccgggcccggtgagggagatctgggaggtgaagttgatggtgatcccggccgtggccaccacggggatcctctcggcgtagggctgcaggatgcgcaagccacacagcctcctgttctggatcgtccactggccctgggtgcacggcaaatcatacttctgcctcctcagtgcataggcatcaaaccagagggccaagccgtagtccagagagggcaccgtgaggtgccaggagcagtgggtttggggcgagtagtagctggggaagtacggggtgctgaggacgccctgggagtcgagcctgttgtccagcgtcaggttcacttcacaggcctggaagaccaccggctgcacggagagcacgaaggggtcgtagtagctgtgcaggcccttcttccagacgaccgccatgatggcccccgacgccagaacctccaccacgggctcctggcggctgcagccgtacaccgaggtgatgagcctcttctccaggggcccggccacgtcatacatggccagtcggtcccggcactctgccagcgtccactccagccggagtttgagcatgaggtccttggggccctgcaggtgccacaggcagctggaggccaggtggtcaggccccttcagccggaggacctggccctggcccacgtagctgtagcggtaacaacccagcgtggaattcaatgcagctatgtctttcacactggcttccaggatcactaggccctcggggtccacttcgtactcggccctgtaggggacggcagccgagctgttgactgtggacagcagctcctccaccagcagtgcctgcaccacctcggggctcagcatcagccggcggtgctcggggatttggagaatgaaccagaagaagcaggtgaggggtccctccccaaaggaatagacggagctggagttgtagtaagttcccaggcgggtgctggtgatgagctccttgagcatcttctgggctttggcggtttcactgcggaaggcactagattcccggcgggtaagatcctgggagaagtggcgattgagtacacgcagactgcctgagtacacctggctgaccatcacctccgccttgtaccctaggaaataccagagtagcacccccgccgaagccagcacgagcagggccagcagcacaaacaggggcaccaggcggaggtagccccgggcttttctcttggagtcctcacaggccttgaacatcccctccggctccgcttcctcgccatcacctccgtccccctgcccgccagccacctggggggcctcggccacgggcatccttctgctcactgatcaccctctggccgatgaggccctgcaggcctggcctcggagcagggtaggtggctcaggctgcagggagccaggcccagctcttagggtggacactgtcactaggtcatttatagatccc

SEQ ID NO: 16916 - RNA, 3193 nt, Homo sapiens
  source 1..3193: mol_type = other RNA
tagatctttgactctggcagtctccagggctctgagggtcccctccgatgggagcaccttccattcccagatcccaagttagaccaggggcttccgaagctggaatctgctctctggaggcaaggctgcccaaacagcctctgtacagagtggggcgcacctcagacactcctcgggatgtagaaccagcattcttgctgctgagccactgccttgcattaggcagcagtggaggaaggggacggaggagagagaattgggaggcagaagggctgggtgtgggcctgggtcctcaggggacgtcttgacccccagctgctggcacttctccatcctcctgccatcactggagcagacatcagggacgagacaagatgccacctcctgccaccacagggcctgctctctcccccaccccccgccagaatacttgtccccctgcttggcagttgccctgggctctctgagtccaggaggtgggccctgctttgcaggggggcagttcctcaggtcaccacttgctggatccagctgatcacacctgtgatgcgggtgtagacgccgaagtagttaggccggccacagcccaggccccagctgaccagccccgccaggaaccagcggccactgagtgccttgcacaccagcggaccacctgagtcaccctgacaggcatccttcttgcccttgcggtagccggcacacagcatgcgtggcgtcacctggtagcgatagacctcgctgcacaggtcctgtgggatcaactgcacatccactttctgcagagcgttgctgatggggcagcaacatgtctctgagccttggtttctccatccataaaatagggccacagcatccgcccgtagggcgccctcgcgcaaggcgccccagcccgtaatccagcagtgcaggccgggctcgaagaagtgggagcgcgcgggcaggcagacggggcgcacggcggccgagcgcaccaccgggtggtcgagctgcagcagcgccacgtcgtagtcatggctgtcctcttcgtggtacgggtgcaggagcaggcggctcaccttgaaggacacctctccaggccagcgcgagttctgccacaccttgcccaggaacacggtccacagcaccgtggaggccatgctgtcctcctggaagcagtgggcagctgttatcacccagcggtcagcgatgagggcccccccacagatgtgtcgaccccgaacctggaggctggcctgccatggccactcaccctcggaggacacagctccaccaacaatgcggctggaggggccctggaggccacagtcacagtgctcctcatccgagccgtccctgcagtcgggccgcccatcacactgcgggttgggcttcttcacgcagctccggtcctcacactggaaggtgaatgtcccacatggcaccccttcctggcactgctcttcgtcgctgccgttgagacaatcaggctgcccatcacagaccttgggcagtgagatgcatgtgctgtcctctttgcactggaatgtggctctgcaaacgcagtttctctcatccaggccgttggggcagtccttgaccccatcacaggcagggacacagagtccattcacagaacagaggaactctccagggcaggggtccgactggttgtacaagccatagtgcacccgcacaccgggcccggtgagggagatctgggaggtgaagttgatggtgatcccggccgtggccaccacggggatcctctcggcgtagggctgcaggatgcgcaagccacacagcctcctgttctggatcgtccactggccctgggtgcacggcaaatcatacttctgcctcctcagtgcataggcatcaaaccagagggccaagccgtagtccagagagggcaccgtgaggtgccaggagcagtgggtttggggcgagtagtagctggggaagtacggggtgctgaggacgccctgggagtcgagcctgttgtccagcgtcaggttcacttcacaggcctggaagaccaccggctgcacggagagcacgaaggggtcgtagtagctgtgcaggcccttcttccagacgaccgccatgatggcccccgacgccagaacctccaccacgggctcctggcggctgcagccgtacaccgaggtgatgagcctcttctccaggggcccggccacgtcatacatggccagtcggtcccggcactctgccagcgtccactccagccggagtttgagcatgaggtccttggggccctgcaggtgccacaggcagctggaggccaggtggtcaggccccttcagccggaggacctggccctggcccacgtagctgtagcggtaacaacccagcgtggaattcaatgcagctatgtctttcacactggcttccaggatcactaggccctcggggtccacttcgtactcggccctgtaggggacggcagccgagctgttgactgtggacagcagctcctccaccagcagtgcctgcaccacctcggggctcagcatcagccggcggtgctcggggatttggagaatgaaccagaagaagcaggtgaggggtccctccccaaaggaatagacggagctggagttgtagtaagttcccaggcgggtgctggtgatgagctccttgagcatcttctgggctttggcggtttcactgcggaaggcactagattcccggcgggtaagatcctgggagaagtggcgattgagtacacgcagactgcctgagtacacctggctgaccatcacctccgccttgtaccctaggaaataccagagtagcacccccgccgaagccagcacgagcagggccagcagcacaaacaggggcaccaggcggaggtagccccgggcttttctcttggagtcctcacaggccttgaacatcccctccggctccgcttcctcgccatcacctccgtccccctgcccgccagccacctggggggcctcggccacgggcatcctttgggagcggcagataggtgccgggcctgcacacaggcctcaggagcctctgtttgtccaggccaaggcctccccacccccacccagccagcccaggctggatcaatggcctagagccatgaccagggtgtctggcccttgtcccctgtggcctgtggcctcaggctccatggaactcctcctgctgggtcctggacagcactgtgact

SEQ ID NO: 16917 - RNA, 2919 nt, Homo sapiens
  source 1..2919: mol_type = other RNA
tagatctttgactctggcagtctccagggctctgagggtcccctccgatgggagcaccttccattcccagatcccaagttagaccaggggcttccgaagctggaatctgctctctggaggcaaggctgcccaaacagcctctgtacagagtggggcgcacctcagacactcctcgggatgtagaaccagcattcttgctgctgagccactgccttgcattaggcagcagtggaggaaggggacggaggagagagaattgggaggcagaagggctgggtgtgggcctgggtcctcaggggacgtcttgacccccagctgctggcacttctccatcctcctgccatcactggagcagacatcagggacgagacaagatgccacctcctgccaccacagggcctgctctctcccccaccccccgccagaatacttgtccccctgcttggcagttgccctgggctctctgagtccaggaggtgggccctgctttgcaggggggcagttcctcaggtcaccacttgctggatccagctgatcacacctgtgatgcgggtgtagacgccgaagtagttaggccggccacagcccaggccccagctgaccagccccgccaggaaccagcggccactgagtgccttgcacaccagcggaccacctgagtcaccctgacaggcatccttcttgcccttgcggtagccggcacacagcatgcgtggcgtcacctggtagcgatagacctcgctgcacaggtcctgtgggatcaactgcacatccactttctgcagagcgttgctgatggggccgccctcgcgcaaggcgccccagcccgtaatccagcagtgcaggccgggctcgaagaagtgggagcgcgcgggcaggcagacggggcgcacggcggccgagcgcaccaccgggtggtcgagctgcagcagcgccacgtcgtagtcatggctgtcctcttcgtggtacgggtgcaggagcaggcggctcaccttgaaggacacctctccaggccagcgcgagttctgccacaccttgcccaggaacacggtccacagcaccgtggaggccatgctgtcctcctggaagcagtgggcagctgttatcacccagcggtcagcgatgagggcccccccacagatgtgtcgaccccgaacctggaggctggcctgccatggccactcaccctcggaggacacagctccaccaacaatgcggctggaggggccctggaggccacagtcacagtgctcctcatccgagccgtccctgcagtcgggccgcccatcacactgcgggttgggcttcttcacgcagctccggtcctcacactggaaggtgaatgtcccacatggcaccccttcctggcactgctcttcgtcgctgccgttgagacaatcaggctgcccatcacagaccttgggcagtgagatgcatgtgctgtcctctttgcactggaatgtggctctgcaaacgcagtttctctcatccaggccgttggggcagtccttgaccccatcacaggcagggacacagagtccattcacagaacagaggaactctccagggcaggggtccgactggttgtacaagccatagtgcacccgcacaccgggcccggtgagggagatctgggaggtgaagttgatggtgatcccggccgtggccaccacggggatcctctcggcgtagggctgcaggatgcgcaagccacacagcctcctgttctggatcgtccactggccctgggtgcacggcaaatcatacttctgcctcctcagtgcataggcatcaaaccagagggccaagccgtagtccagagagggcaccgtgaggtgccaggagcagtgggtttggggcgagtagtagctggggaagtacggggtgctgaggacgccctgggagtcgagcctgttgtccagcgtcaggttcacttcacaggcctggaagaccaccggctgcacggagagcacgaaggggtcgtagtagctgtgcaggcccttcttccagacgaccgccatgatggcccccgacgccagaacctccaccacgggctcctggcggctgcagccgtacaccgaggtgatgagcctcttctccaggggcccggccacgtcatacatggccagtcggtcccggcactctgccagcgtccactccagccggagtttgagcatgaggtccttggggccctgcaggtgccacaggcagctggaggccaggtggtcaggccccttcagccggaggacctggccctggcccacgtagctgtagcggtaacaacccagcgtggaattcaatgcagctatgtctttcacactggcttccaggatcactaggccctcggggtccacttcgtactcggccctgtaggggacggcagccgagctgttgactgtggacagcagctcctccaccagcagtgcctgcaccacctcggggctcagcatcagccggcggtgctcggggatttggagaatgaaccagaagaagcaggtgaggggtccctccccaaaggaatagacggagctggagttgtagtaagttcccaggcgggtgctggtgatgagctccttgagcatcttctgggctttggcggtttcactgcggaaggcactagattcccggcgggtaagatcctgggagaagtggcgattgagtacacgcagactgcctgagtacacctggctgaccatcacctccgccttgtaccctaggaaataccagagtagcacccccgccgaagccagcacgagcagggccagcagcacaaacaggggcaccaggcggaggtagccccgggcttttctcttggagtcctcacaggccttgaacatcccctccggctccgcttcctcgccatcacctccgtccccctgcccgccagccacctggggggcctcggccacgggcatcctg

SEQ ID NO: 16918 - RNA, 3015 nt, Homo sapiens
  source 1..3015: mol_type = other RNA
tagatctttgactctggcagtctccagggctctgagggtcccctccgatgggagcaccttccattcccagatcccaagttagaccaggggcttccgaagctggaatctgctctctggaggcaaggctgcccaaacagcctctgtacagagtggggcgcacctcagacactcctcgggatgtagaaccagcattcttgctgctgagccactgccttgcattaggcagcagtggaggaaggggacggaggagagagaattgggaggcagaagggctgggtgtgggcctgggtcctcaggggacgtcttgacccccagctgctggcacttctccatcctcctgccatcactggagcagacatcagggacgagacaagatgccacctcctgccaccacagggcctgctctctcccccaccccccgccagaatacttgtccccctgcttggcagttgccctgggctctctgagtccaggaggtgggccctgctttgcaggggggcagttcctcaggtcaccacttgctggatccagctgatcacacctgtgatgcgggtgtagacgccgaagtagttaggccggccacagcccaggccccagctgaccagccccgccaggaaccagcggccactgagtgccttgcacaccagcggaccacctgagtcaccctgacaggcatccttcttgcccttgcggtagccggcacacagcatgcgtggcgtcacctggtagcgatagacctcgctgcacaggtcctgtgggatcaactgcacatccactttctgcagagcgttgctgatggggccgccctcgcgcaaggcgccccagcccgtaatccagcagtgcaggccgggctcgaagaagtgggagcgcgcgggcaggcagacggggcgcacggcggccgagcgcaccaccgggtggtcgagctgcagcagcgccacgtcgtagtcatggctgtcctcttcgtggtacgggtgcaggagcaggcggctcaccttgaaggacacctctccaggccagcgcgagttctgccacaccttgcccaggaacacggtccacagcaccgtggaggccatgctgtcctcctggaagcagtgggcagctgttatcacccagcggtcagcgatgagggcccccccacagatgtgtcgaccccgaacctggaggctggcctgccatggccactcaccctcggaggacacagctccaccaacaatgcggctggaggggccctggaggccacagtcacagtgctcctcatccgagccgtccctgcagtcgggccgcccatcacactgcgggttgggcttcttcacgcagctccggtcctcacactggaaggtgaatgtcccacatggcaccccttcctggcactgctcttcgtcgctgccgttgagacaatcaggctgcccatcacagaccttgggcagtgagatgcatgtgctgtcctctttgcactggaatgtggctctgcaaacgcagtttctctcatccaggccgttggggcagtccttgaccccatcacaggcagggacacagagtccattcacagaacagaggaactctccagggcaggggtccgactggttgtacaagccatagtgcacccgcacaccgggcccggtgagggagatctgggaggtgaagttgatggtgatcccggccgtggccaccacggggatcctctcggcgtagggctgcaggatgcgcaagccacacagcctcctgttctggatcgtccactggccctgggtgcacggcaaatcatacttctgcctcctcagtgcataggcatcaaaccagagggccaagccgtagtccagagagggcaccgtgaggtgccaggagcagtgggtttggggcgagtagtagctggggaagtacggggtgctgaggacgccctgggagtcgagcctgttgtccagcgtcaggttcacttcacaggcctggaagaccaccggctgcacggagagcacgaaggggtcgtagtagctgtgcaggcccttcttccagacgaccgccatgatggcccccgacgccagaacctccaccacgggctcctggcggctgcagccgtacaccgaggtgatgagcctcttctccaggggcccggccacgtcatacatggccagtcggtcccggcactctgccagcgtccactccagccggagtttgagcatgaggtccttggggccctgcaggtgccacaggcagctggaggccaggtggtcaggccccttcagccggaggacctggccctggcccacgtagctgtagcggtaacaacccagcgtggaattcaatgcagctatgtctttcacactggcttccaggatcactaggccctcggggtccacttcgtactcggccctgtaggggacggcagccgagctgttgactgtggacagcagctcctccaccagcagtgcctgcaccacctcggggctcagcatcagccggcggtgctcggggatttggagaatgaaccagaagaagcaggtgaggggtccctccccaaaggaatagacggagctggagttgtagtaagttcccaggcgggtgctggtgatgagctccttgagcatcttctgggctttggcggtttcactgcggaaggcactagattcccggcgggtaagatcctgggagaagtggcgattgagtacacgcagactgcctgagtacacctggctgaccatcacctccgccttgtaccctaggaaataccagagtagcacccccgccgaagccagcacgagcagggccagcagcacaaacaggggcaccaggcggaggtagccccgggcttttctcttggagtcctcacaggccttgaacatcccctccggctccgcttcctcgccatcacctccgtccccctgcccgccagccacctggggggcctcggccacgggcatccttctgctcactgatcaccctctggccgatgaggccctgcaggcctggcctcggagcagggtaggtggctcaggctgcagggagccaggcccagctctt

SEQ ID NO: 16919 - RNA, 3127 nt, Homo sapiens
  source 1..3127: mol_type = other RNA
tagatctttgactctggcagtctccagggctctgagggtcccctccgatgggagcaccttccattcccagatcccaagttagaccaggggcttccgaagctggaatctgctctctggaggcaaggctgcccaaacagcctctgtacagagtggggcgcacctcagacactcctcgggatgtagaaccagcattcttgctgctgagccactgccttgcattaggcagcagtggaggaaggggacggaggagagagaattgggaggcagaagggctgggtgtgggcctgggtcctcaggggacgtcttgacccccagctgctggcacttctccatcctcctgccatcactggagcagacatcagggacgagacaagatgccacctcctgccaccacagggcctgctctctcccccaccccccgccagaatacttgtccccctgcttggcagttgccctgggctctctgagtccaggaggtgggccctgctttgcaggggggcagttcctcaggtcaccacttgctggatccagctgatcacacctgtgatgcgggtgtagacgccgaagtagttaggccggccacagcccaggccccagctgaccagccccgccaggaaccagcggccactgagtgccttgcacaccagcggaccacctgagtcaccctgacaggcatccttcttgcccttgcggtagccggcacacagcatgcgtggcgtcacctggtagcgatagacctcgctgcacaggtcctgtgggatcaactgcacatccactttctgcagagcgttgctgatggggccgccctcgcgcaaggcgccccagcccgtaatccagcagtgcaggccgggctcgaagaagtgggagcgcgcgggcaggcagacggggcgcacggcggccgagcgcaccaccgggtggtcgagctgcagcagcgccacgtcgtagtcatggctgtcctcttcgtggtacgggtgcaggagcaggcggctcaccttgaaggacacctctccaggccagcgcgagttctgccacaccttgcccaggaacacggtccacagcaccgtggaggccatgctgtcctcctggaagcagtgggcagctgttatcacccagcggtcagcgatgagggcccccccacagatgtgtcgaccccgaacctggaggctggcctgccatggccactcaccctcggaggacacagctccaccaacaatgcggctggaggggccctggaggccacagtcacagtgctcctcatccgagccgtccctgcagtcgggccgcccatcacactgcgggttgggcttcttcacgcagctccggtcctcacactggaaggtgaatgtcccacatggcaccccttcctggcactgctcttcgtcgctgccgttgagacaatcaggctgcccatcacagaccttgggcagtgagatgcatgtgctgtcctctttgcactggaatgtggctctgcaaacgcagtttctctcatccaggccgttggggcagtccttgaccccatcacaggcagggacacagagtccattcacagaacagaggaactctccagggcaggggtccgactggttgtacaagccatagtgcacccgcacaccgggcccggtgagggagatctgggaggtgaagttgatggtgatcccggccgtggccaccacggggatcctctcggcgtagggctgcaggatgcgcaagccacacagcctcctgttctggatcgtccactggccctgggtgcacggcaaatcatacttctgcctcctcagtgcataggcatcaaaccagagggccaagccgtagtccagagagggcaccgtgaggtgccaggagcagtgggtttggggcgagtagtagctggggaagtacggggtgctgaggacgccctgggagtcgagcctgttgtccagcgtcaggttcacttcacaggcctggaagaccaccggctgcacggagagcacgaaggggtcgtagtagctgtgcaggcccttcttccagacgaccgccatgatggcccccgacgccagaacctccaccacgggctcctggcggctgcagccgtacaccgaggtgatgagcctcttctccaggggcccggccacgtcatacatggccagtcggtcccggcactctgccagcgtccactccagccggagtttgagcatgaggtccttggggccctgcaggtgccacaggcagctggaggccaggtggtcaggccccttcagccggaggacctggccctggcccacgtagctgtagcggtaacaacccagcgtggaattcaatgcagctatgtctttcacactggcttccaggatcactaggccctcggggtccacttcgtactcggccctgtaggggacggcagccgagctgttgactgtggacagcagctcctccaccagcagtgcctgcaccacctcggggctcagcatcagccggcggtgctcggggatttggagaatgaaccagaagaagcaggtgaggggtccctccccaaaggaatagacggagctggagttgtagtaagttcccaggcgggtgctggtgatgagctccttgagcatcttctgggctttggcggtttcactgcggaaggcactagattcccggcgggtaagatcctgggagaagtggcgattgagtacacgcagactgcctgagtacacctggctgaccatcacctccgccttgtaccctaggaaataccagagtagcacccccgccgaagccagcacgagcagggccagcagcacaaacaggggcaccaggcggaggtagccccgggcttttctcttggagtcctcacaggccttgaacatcccctccggctccgcttcctcgccatcacctccgtccccctgcccgccagccacctggggggcctcggccacgggcatcctttgggagcggcagataggtgccgggcctgcacacaggcctcaggagcctctgtttgtccaggccaaggcctccccacccccacccagccagcccaggctggatcaatggcctagagccatgaccagggtgtctggcccttgtcccctgtggcctgtggcctcaggctccatggaactcctcctgctgggtcctggacagcactgtgact

SEQ ID NO: 16920 - RNA, 3059 nt, Homo sapiens
  source 1..3059: mol_type = other RNA
tagatctttgactctggcagtctccagggctctgagggtcccctccgatgggagcaccttccattcccagatcccaagttagaccaggggcttccgaagctggaatctgctctctggaggcaaggctgcccaaacagcctctgtacagagtggggcgcacctcagacactcctcgggatgtagaaccagcattcttgctgctgagccactgccttgcattaggcagcagtggaggaaggggacggaggagagagaattgggaggcagaagggctgggtgtgggcctgggtcctcaggggacgtcttgacccccagctgctggcacttctccatcctcctgccatcactggagcagacatcagggacgagacaagatgccacctcctgccaccacagggcctgctctctcccccaccccccgccagaatacttgtccccctgcttggcagttgccctgggctctctgagtccaggaggtgggccctgctttgcaggggggcagttcctcaggtcaccacttgctggatccagctgatcacacctgtgatgcgggtgtagacgccgaagtagttaggccggccacagcccaggccccagctgaccagccccgccaggaaccagcggccactgagtgccttgcacaccagcggaccacctgagtcaccctgacaggcatccttcttgcccttgcggtagccggcacacagcatgcgtggcgtcacctggtagcgatagacctcgctgcacaggtcctgtgggatcaactgcacatccactttctgcagagcgttgctgatggggccgccctcgcgcaaggcgccccagcccgtaatccagcagtgcaggccgggctcgaagaagtgggagcgcgcgggcaggcagacggggcgcacggcggccgagcgcaccaccgggtggtcgagctgcagcagcgccacgtcgtagtcatggctgtcctcttcgtggtacgggtgcaggagcaggcggctcaccttgaaggacacctctccaggccagcgcgagttctgccacaccttgcccaggaacacggtccacagcaccgtggaggccatgctgtcctcctggaagcagtgggcagctgttatcacccagcggtcagcgatgagggcccccccacagatgtgtcgaccccgaacctggaggctggcctgccatggccactcaccctcggaggacacagctccaccaacaatgcggctggaggggccctggaggccacagtcacagtgctcctcatccgagccgtccctgcagtcgggccgcccatcacactgcgggttgggcttcttcacgcagctccggtcctcacactggaaggtgaatgtcccacatggcaccccttcctggcactgctcttcgtcgctgccgttgagacaatcaggctgcccatcacagaccttgggcagtgagatgcatgtgctgtcctctttgcactggaatgtggctctgcaaacgcagtttctctcatccaggccgttggggcagtccttgaccccatcacaggcagggacacagagtccattcacagaacagaggaactctccagggcaggggtccgactggttgtacaagccatagtgcacccgcacaccgggcccggtgagggagatctgggaggtgaagttgatggtgatcccggccgtggccaccacggggatcctctcggcgtagggctgcaggatgcgcaagccacacagcctcctgttctggatcgtccactggccctgggtgcacggcaaatcatacttctgcctcctcagtgcataggcatcaaaccagagggccaagccgtagtccagagagggcaccgtgaggtgccaggagcagtgggtttggggcgagtagtagctggggaagtacggggtgctgaggacgccctgggagtcgagcctgttgtccagcgtcaggttcacttcacaggcctggaagaccaccggctgcacggagagcacgaaggggtcgtagtagctgtgcaggcccttcttccagacgaccgccatgatggcccccgacgccagaacctccaccacgggctcctggcggctgcagccgtacaccgaggtgatgagcctcttctccaggggcccggccacgtcatacatggccagtcggtcccggcactctgccagcgtccactccagccggagtttgagcatgaggtccttggggccctgcaggtgccacaggcagctggaggccaggtggtcaggccccttcagccggaggacctggccctggcccacgtagctgtagcggtaacaacccagcgtggaattcaatgcagctatgtctttcacactggcttccaggatcactaggccctcggggtccacttcgtactcggccctgtaggggacggcagccgagctgttgactgtggacagcagctcctccaccagcagtgcctgcaccacctcggggctcagcatcagccggcggtgctcggggatttggagaatgaaccagaagaagcaggtgaggggtccctccccaaaggaatagacggagctggagttgtagtaagttcccaggcgggtgctggtgatgagctccttgagcatcttctgggctttggcggtttcactgcggaaggcactagattcccggcgggtaagatcctgggagaagtggcgattgagtacacgcagactgcctgagtacacctggctgaccatcacctccgccttgtaccctaggaaataccagagtagcacccccgccgaagccagcacgagcagggccagcagcacaaacaggggcaccaggcggaggtagccccgggcttttctcttggagtcctcacaggccttgaacatcccctccggctccgcttcctcgccatcacctccgtccccctgcccgccagccacctggggggcctcggccacgggcatccttttggagtggaagagtaacaacatcaggcggcagtgactgcaagtgggtgccgagacagctcacagaggagggaagtgcatctcaggtcagctcgcaccagagggcaggcaccagagctggactgggtctggctcaagaac

SEQ ID NO: 16921 - RNA, 64 nt, Homo sapiens
  source 1..64: mol_type = other RNA
tagcaagagaaccattaccattactaaactcagtaatggtaacggtttccttgccattcccaag

SEQ ID NO: 16922 - RNA, 3177 nt, Homo sapiens
  source 1..3177: mol_type = other RNA
tagcaatacagtacaaatatagtccttctttcctgagggggctaggagagaaagacaatgaatggcaccctgcctgatcttcagggaaagctgaaatactggtccacagattggagccactgcccaatataacttctcaagtccctggctgaagacagacttgagggctggcatcacctacttccctagccccagtgtgatgtggcataggtcttgatacccaaggagtcccatcttcaaggaagcaactccagcctagtcacagcttcatcctagagttagctgtctccttttctcattagccagtgatttacaacttcctgctctcctttgctttccaccatctaagctataccctgtccctaagtcctgagccaccctctcctgctgttttcctggtttggtaagtcaggaggaaaggtttgatggttctttccccacttctttttggaggagtaaggaagtgaggttcttatccttcacatatgagtgccctggattttggttcttagttgatgaatactcaacacccagttctttgttttggctgcagccacgcagtgcagctaatgtgtggcttaagaatgaccctcttcctaggcctcgcccaccttgggacggtgggcaggaaccccagtagaactggtaaattacttgttccgtctttaaagggcctcctacgagctactcttgggccatatggggttaaagaaacttcctgaacatagcactctggaggaaggagtcctcttccctccacctgtagccacagtgtggttggcaaaccctcaagcctatcaggaggtagagggcaagatgagcgctttgtcttaaaggccaaagagaacagcaccaagcgtttctacccagggccttccttctctcttcccatgaagtctttgcccttctcccataaactttgggtcccaggagaaccttggttgctgaaggctaggctcagtcctccgcctgggagtctgaggaaatgctcttcttacctaagaaatggaagatggggcctaggaggccctgctgttgctacattcccctctgctgtgcaaactgctgtccctggccagctctcccttgctcttaacctgatacataggagctagtccttcatttccaaatgctcccctttgtggagtgcatggttggcctgacagtgtcactgaccccagggctctccttgcccctggagtacccacaggccttggtccacatctttaaatttgggagccaggtggagagaaattgtgttcatgctgcatgggaggtagagaatggaggtgactttttatccctgccacccctcattttgtttccttctctgaagcacctgcctctgagctcagttccccaaagaggcaggcgggcagccaagcaagggcaaagctctggtcggggaatgggtagaggtagggcagccccaggctcgaggactccctggttgccgtttccctcctacctcgatgctccactttcgcaggtcactggggaggcaggcccatggcacatgagggacagtgggggtgggggaagaggaagaagcaccctgtagcctttggcccacccacgaggcagggtggagggttcttcctggatccaagggtggaacctccccacgagcctgggtccatccccttggatagcttaggaaggaaggaaagagcgagctgcacacagcaggacacacgggggacggggtttgaggagctttgatacgaaacgcaccggaggggaggggtcagagaaagagaagtgggggaagagagaaaaagcagagaagagacacgatgcacggagaaaggagcagctgaaagtggcctggactccagccctggctgttgtctggtgggtgcgggatggtgagacagtgcttgcggcacatcgtgggggtcgtagcaggcctgtggctggggaaacaggctgaagaagaccactccagggtggacgggctggggacaggggctgcttgagatgacagcagagccgctctcagggccaggcagggggagtagtggctactgatactcaatagggtcatcacacgagaggacagcagcagggcaaagccccggctcccctgtctgcccacgggcctcctgagggaagaggggtgtcgtgtggggtgccccacacaggactcagcaccagcaggttttcgaagagttcgctgggccctcgggtttgccctcctcctcctccagctctgccagtgccaactcattgctggcacgcatccggaggccttccagctccttcctatgggcctgcagcaccagctctgtcagacgcgtgaatgactctttaatgttgaggttggtgcaggcacttgtttcatagaagtccatgccatactccttcgccagctgctgcccttgctctcttcccacctgccgtttctgctcctcatcagccttattcccaataaggatcttctggacgccttctggtgcgtaccagaggtcttcatccagggctgtggaaggcaaagcttcctggaagcatttgccttcccatctggccctcgccttgccttccccggtgaggcaccctctccacaccccggcagtgaggtggcatctcctacctcatccacgtcactgacccacttcatgatgtgctggtaagagcgctcgctgctaatgtcatagaccaaaaatatcccctgggcccgccgatagtactgctttgtgatggtctggtatctctcctgccctgcagtgtcccagatctgtatccgcactttgatgccgtctacctctatggtcttcatcttaaagtcaacaccgatggtggagatgtgcgaggagtggaactcgttgtcggtgaagcggcacagcaggcaggtcttgcccaccccggagtccccgatcagcagcagccggaacagcacatcgtactgcttcgccatgactggggccagcggggccgggaactgcgggcgggcagcgggctcagccctgctccgccgctgccatcgcggcccgcgcccgcccggggacgctgcgggcggcgaggaggacgccgggcccggcccccgcggctgcctcgcccgcccgcctgcccactcgctcgctgggtgccgggaagcgcggctgcggcgggagcccggcgcggcgcccgctcggctcggctcggctcggctgggctggcgcgaggcggtgggaggag

SEQ ID NO: 16923 - RNA, 2830 nt, Homo sapiens
  source 1..2830: mol_type = other RNA
tagcaatacagtacaaatatagtccttctttcctgagggggctaggagagaaagacaatgaatggcaccctgcctgatcttcagggaaagctgaaatactggtccacagattggagccactgcccaatataacttctcaagtccctggctgaagacagacttgagggctggcatcacctacttccctagccccagtgtgatgtggcataggtcttgatacccaaggagtcccatcttcaaggaagcaactccagcctagtcacagcttcatcctagagttagctgtctccttttctcattagccagtgatttacaacttcctgctctcctttgctttccaccatctaagctataccctgtccctaagtcctgagccaccctctcctgctgttttcctggtttggtaagtcaggaggaaaggtttgatggttctttccccacttctttttggaggagtaaggaagtgaggttcttatccttcacatatgagtgccctggattttggttcttagttgatgaatactcaacacccagttctttgttttggctgcagccacgcagtgcagctaatgtgtggcttaagaatgaccctcttcctaggcctcgcccaccttgggacggtgggcaggaaccccagtagaactggtaaattacttgttccgtctttaaagggcctcctacgagctactcttgggccatatggggttaaagaaacttcctgaacatagcactctggaggaaggagtcctcttccctccacctgtagccacagtgtggttggcaaaccctcaagcctatcaggaggtagagggcaagatgagcgctttgtcttaaaggccaaagagaacagcaccaagcgtttctacccagggccttccttctctcttcccatgaagtctttgcccttctcccataaactttgggtcccaggagaaccttggttgctgaaggctaggctcagtcctccgcctgggagtctgaggaaatgctcttcttacctaagaaatggaagatggggcctaggaggccctgctgttgctacattcccctctgctgtgcaaactgctgtccctggccagctctcccttgctcttaacctgatacataggagctagtccttcatttccaaatgctcccctttgtggagtgcatggttggcctgacagtgtcactgaccccagggctctccttgcccctggagtacccacaggccttggtccacatctttaaatttgggagccaggtggagagaaattgtgttcatgctgcatgggaggtagagaatggaggtgactttttatccctgccacccctcattttgtttccttctctgaagcacctgcctctgagctcagttccccaaagaggcaggcgggcagccaagcaagggcaaagctctggtcggggaatgggtagaggtagggcagccccaggctcgaggactccctggttgccgtttccctcctacctcgatgctccactttcgcaggtcactggggaggcaggcccatggcacatgagggacagtgggggtgggggaagaggaagaagcaccctgtagcctttggcccacccacgaggcagggtggagggttcttcctggatccaagggtggaacctccccacgagcctgggtccatccccttggatagcttaggaaggaaggaaagagcgagctgcacacagcaggacacacgggggacggggtttgaggagctttgatacgaaacgcaccggaggggaggggtcagagaaagagaagtgggggaagagagaaaaagcagagaagagacacgatgcacggagaaaggagcagctgaaagtggcctggactccagccctggctgttgtctggtgggtgcgggatggtgagacagtgcttgcggcacatcgtgggggtcgtagcaggcctgtggctggggaaacaggctgaagaagaccactccagggtggacgggctggggacaggggctgcttgagatgacagcagagccgctctcagggccaggcagggggagtagtggctactgatactcaatagggtcatcacacgagaggacagcagcagggcaaagccccggctcccctgtctgcccacgggcctcctgagggaagaggggtgtcgtgtggggtgccccacacaggactcagcaccagcaggttttcgaagagttcgctgggccctcgggtttgccctcctcctcctccagctctgccagtgccaactcattgctggcacgcatccggaggccttccagctccttcctatgggcctgcagcaccagctctgtcagacgcgtgaatgactctttaatgttgaggttggtgcaggcacttgtttcatagaagtccatgccatactccttcgccagctgctgcccttgctctcttcccacctgccgtttctgctcctcatcagccttattcccaataaggatcttctggacgccttctggtgcgtaccagaggtcttcatccagggctgtggaaggcaaagcttcctggaagcatttgccttcccatctggccctcgccttgccttccccggtgaggcaccctctccacaccccggcagtgaggtggcatctcctacctcatccacgtcactgacccacttcatgatgtgctggtaagagcgctcgctgctaatgtcatagaccaaaaatatcccctgggcccgccgatagtactgctttgtgatggtctggtatctctcctgccctgcagtgtcccagatctgtatccgcactttgatgccgtctacctctatggtcttcatcttaaagtcaacacctgatgccttttctcttttttcttgacggagtcttcc

SEQ ID NO: 16924 - RNA, 3046 nt, Homo sapiens
  source 1..3046: mol_type = other RNA
tagcaatacagtacaaatatagtccttctttcctgagggggctaggagagaaagacaatgaatggcaccctgcctgatcttcagggaaagctgaaatactggtccacagattggagccactgcccaatataacttctcaagtccctggctgaagacagacttgagggctggcatcacctacttccctagccccagtgtgatgtggcataggtcttgatacccaaggagtcccatcttcaaggaagcaactccagcctagtcacagcttcatcctagagttagctgtctccttttctcattagccagtgatttacaacttcctgctctcctttgctttccaccatctaagctataccctgtccctaagtcctgagccaccctctcctgctgttttcctggtttggtaagtcaggaggaaaggtttgatggttctttccccacttctttttggaggagtaaggaagtgaggttcttatccttcacatatgagtgccctggattttggttcttagttgatgaatactcaacacccagttctttgttttggctgcagccacgcagtgcagctaatgtgtggcttaagaatgaccctcttcctaggcctcgcccaccttgggacggtgggcaggaaccccagtagaactggtaaattacttgttccgtctttaaagggcctcctacgagctactcttgggccatatggggttaaagaaacttcctgaacatagcactctggaggaaggagtcctcttccctccacctgtagccacagtgtggttggcaaaccctcaagcctatcaggaggtagagggcaagatgagcgctttgtcttaaaggccaaagagaacagcaccaagcgtttctacccagggccttccttctctcttcccatgaagtctttgcccttctcccataaactttgggtcccaggagaaccttggttgctgaaggctaggctcagtcctccgcctgggagtctgaggaaatgctcttcttacctaagaaatggaagatggggcctaggaggccctgctgttgctacattcccctctgctgtgcaaactgctgtccctggccagctctcccttgctcttaacctgatacataggagctagtccttcatttccaaatgctcccctttgtggagtgcatggttggcctgacagtgtcactgaccccagggctctccttgcccctggagtacccacaggccttggtccacatctttaaatttgggagccaggtggagagaaattgtgttcatgctgcatgggaggtagagaatggaggtgactttttatccctgccacccctcattttgtttccttctctgaagcacctgcctctgagctcagttccccaaagaggcaggcgggcagccaagcaagggcaaagctctggtcggggaatgggtagaggtagggcagccccaggctcgaggactccctggttgccgtttccctcctacctcgatgctccactttcgcaggtcactggggaggcaggcccatggcacatgagggacagtgggggtgggggaagaggaagaagcaccctgtagcctttggcccacccacgaggcagggtggagggttcttcctggatccaagggtggaacctccccacgagcctgggtccatccccttggatagcttaggaaggaaggaaagagcgagctgcacacagcaggacacacgggggacggggtttgaggagctttgatacgaaacgcaccggaggggaggggtcagagaaagagaagtgggggaagagagaaaaagcagagaagagacacgatgcacggagaaaggagcagctgaaagtggcctggactccagccctggctgttgtctggtgggtgcgggatggtgagacagtgcttgcggcacatcgtgggggtcgtagcaggcctgtggctggggaaacaggctgaagaagaccactccagggtggacgggctggggacaggggctgcttgagatgacagcagagccgctctcagggccaggcagggggagtagtggctactgatactcaatagggtcatcacacgagaggacagcagcagggcaaagccccggctcccctgtctgcccacgggcctcctgagggaagaggggtgtcgtgtggggtgccccacacaggactcagcaccagcaggttttcgaagagttcgctgggccctcgggtttgccctcctcctcctccagctctgccagtgccaactcattgctggcacgcatccggaggccttccagctccttcctatgggcctgcagcaccagctctgtcagacgcgtgaatgactctttaatgttgaggttggtgcaggcacttgtttcatagaagtccatgccatactccttcgccagctgctgcccttgctctcttcccacctgccgtttctgctcctcatcagccttattcccaataaggatcttctggacgccttctggtgcgtactcatccacgtcactgacccacttcatgatgtgctggtaagagcgctcgctgctaatgtcatagaccaaaaatatcccctgggcccgccgatagtactgctttgtgatggtctggtatctctcctgccctgcagtgtcccagatctgtatccgcactttgatgccgtctacctctatggtcttcatcttaaagtcaacaccgatggtggagatgtgcgaggagtggaactcgttgtcggtgaagcggcacagcaggcaggtcttgcccaccccggagtccccgatcagcagcagccggaacagcacatcgtactgcttcgccatgactggggccagcggggccgggaactgcgggcgggcagcgggctcagccctgctccgccgctgccatcgcggcccgcgcccgcccggggacgctgcgggcggcgaggaggacgccgggcccggcccccgcggctgcctcgcccgcccgcctgcccactcgctcgctgggtgccgggaagcgcggctgcggcgggagcccggcgcggcgcccgctcggctcggctcggctcggctgggctggcgcgaggcggtgggaggag

SEQ ID NO: 16925 - RNA, 3266 nt, Homo sapiens
  source 1..3266: mol_type = other RNA
tagcaatacagtacaaatatagtccttctttcctgagggggctaggagagaaagacaatgaatggcaccctgcctgatcttcagggaaagctgaaatactggtccacagattggagccactgcccaatataacttctcaagtccctggctgaagacagacttgagggctggcatcacctacttccctagccccagtgtgatgtggcataggtcttgatacccaaggagtcccatcttcaaggaagcaactccagcctagtcacagcttcatcctagagttagctgtctccttttctcattagccagtgatttacaacttcctgctctcctttgctttccaccatctaagctataccctgtccctaagtcctgagccaccctctcctgctgttttcctggtttggtaagtcaggaggaaaggtttgatggttctttccccacttctttttggaggagtaaggaagtgaggttcttatccttcacatatgagtgccctggattttggttcttagttgatgaatactcaacacccagttctttgttttggctgcagccacgcagtgcagctaatgtgtggcttaagaatgaccctcttcctaggcctcgcccaccttgggacggtgggcaggaaccccagtagaactggtaaattacttgttccgtctttaaagggcctcctacgagctactcttgggccatatggggttaaagaaacttcctgaacatagcactctggaggaaggagtcctcttccctccacctgtagccacagtgtggttggcaaaccctcaagcctatcaggaggtagagggcaagatgagcgctttgtcttaaaggccaaagagaacagcaccaagcgtttctacccagggccttccttctctcttcccatgaagtctttgcccttctcccataaactttgggtcccaggagaaccttggttgctgaaggctaggctcagtcctccgcctgggagtctgaggaaatgctcttcttacctaagaaatggaagatggggcctaggaggccctgctgttgctacattcccctctgctgtgcaaactgctgtccctggccagctctcccttgctcttaacctgatacataggagctagtccttcatttccaaatgctcccctttgtggagtgcatggttggcctgacagtgtcactgaccccagggctctccttgcccctggagtacccacaggccttggtccacatctttaaatttgggagccaggtggagagaaattgtgttcatgctgcatgggaggtagagaatggaggtgactttttatccctgccacccctcattttgtttccttctctgaagcacctgcctctgagctcagttccccaaagaggcaggcgggcagccaagcaagggcaaagctctggtcggggaatgggtagaggtagggcagccccaggctcgaggactccctggttgccgtttccctcctacctcgatgctccactttcgcaggtcactggggaggcaggcccatggcacatgagggacagtgggggtgggggaagaggaagaagcaccctgtagcctttggcccacccacgaggcagggtggagggttcttcctggatccaagggtggaacctccccacgagcctgggtccatccccttggatagcttaggaaggaaggaaagagcgagctgcacacagcaggacacacgggggacggggtttgaggagctttgatacgaaacgcaccggaggggaggggtcagagaaagagaagtgggggaagagagaaaaagcagagaagagacacgatgcacggagaaaggagcagctgaaagtggcctggactccagccctggctgttgtctggtgggtgcgggatggtgagacagtgcttgcggcacatcgtgggggtcgtagcaggcctgtggctggggaaacaggctgaagaagaccactccagggtggacgggctggggacaggggctgcttgagatgacagcagagccgctctcagggccaggcagggggagtagtggctactgatactcaatagggtcatcacacgagaggacagcagcagggcaaagccccggctcccctgtctgcccacgggcctcctgagggaagaggggtgtcgtgtggggtgccccacacaggactcagcaccagcaggttttcgaagagttcgctgggccctcgggtttgccctcctcctcctccagctctgccagtgccaactcattgctggcacgcatccggaggccttccagctccttcctatgggcctgcagcaccagctctgtcagacgcgtgaatgactctttaatgttgaggttggtgcaggcacttgtttcatagaagtccatgccatactccttcgccagctgctgcccttgctctcttcccacctgccgtttctgctcctcatcagccttattcccaataaggatcttctggacgccttctggtgcgtactcatccacgtcactgacccacttcatgatgtgctggtaagagcgctcgctgctaatgtcatagaccaaaaatatcccctgggcccgccgatagtactgctttgtgatggtctggtatctctcctgccctgcagtgtcccagatctgtatccgcactttgatgccgtctacctctatggtcttcatcttaaagtcaacacctgatgccttttctcttttttcttgacggagtcttcctctgtcgcccaggctggagtgcagtggcacgatctcaggtcactgcaacctctgcctcctgggttcaagcgattctcctgcctcagcctcccaagtagctgggattacaggcacgtgccaccacacccagctaattttttgtatttttagtagagacggggtttcactgacattatgcggcatcgatggtggagatgtgcgaggagtggaactcgttgtcggtgaagcggcacagcaggcaggtcttgcccaccccggagtccccgatcagcagcagccggaacagcacatcgtactgcttcgccatgactggggccagcggggccgggaactgcgggcgggcagcgggctcagccctgctccgccgctgccatcgcggcccgcgcccgcccggggacgctgcgggcggcgaggaggacgccgggcccggcccccgcggctgcctcgcccgcccgcctgcccactcgctcgctgggtgccgggaagcgcggctgcggcgggagcccggcgcggcgcccgctcggctcggctcggctcggctgggctggcgcgaggcggtgggaggag

SEQ ID NO: 16926 - RNA, 672 nt, Homo sapiens
  source 1..672: mol_type = other RNA
tagcaccatttgaaatcagtgttttccttttcttgatgacatcctgaagtacttgttacctggcaagcaaatgacgcagctcagctggaagtttcaggtacccagaaattgatttacttgaatattatcatcgaagcactacctttaagcacctagttattagagaaggaagaggaatatgtctgtgagccggcggctaggaggaatcctaagaaaacacaagtttttatgacgctgtggtgtgtcaggacagagtccggcagacctgggagacgggagataagagtcctggttcccagcccgtcgccagcagccttaagactccttaagtacagtgcatactcatgggcgaaacaaagcgagaagcagcaccgaggagcagcctgcgactctgctatttttaaactgccaattagaacgcctaaaattacgtggctagaaccaccacatccgctcagagttaatcatacacttctgagctgaagttttaaattttctgttttccaagtccctgatcagaatatttaaaaagattatttcttggctgcctcaggcccacagttgagttgtggttcgggatgatttctactgggaatggcttttcttggccagagttaaaatctgtcatatatacacacacacacacacacacacatacacatacacacacac

SEQ ID NO: 16927 - RNA, 512 nt, Homo sapiens
  source 1..512: mol_type = other RNA
tagcagcacagaaatattggctgactgcgctgccttcaggattgcgtcaaacctctgaaaactctcctctatggaacaattgatgttcttcttggtgaagagctctgaggcagctccaaagatgactacttccttggctccagcagcaaccgctgcctcgaagcctttcaaatttggggtcaggactgggtagttgatgccaggaaacttctgaatgcccttcaagacttcagtgtggtcacccatctggggaacccacttaggagacacaaagctggtggtttctataacagagagtcctgcttcagaaagcatgtctatcagcttgattttcactggagtagatacgatattcttttcattttgtagtccatctcggggaccaacttccacaattttcacccgctttggtaaagtgcccatagatgaggtgctgacagcccggagggacgccaagcccaccagtcgccgcggaagcgccttcctcattgctgccatcttggcccagaatc

SEQ ID NO: 16928 - RNA, 37 nt, Homo sapiens
  source 1..37: mol_type = other RNA
tagcccccaggcttcacttggcgctgtccgctgcggt

SEQ ID NO: 16929 - RNA, 79 nt, Homo sapiens
  source 1..79: mol_type = other RNA
taggactagatgttggaattagacacaattttttgtgtctaacttttttctgtctaattccaacatctagtcctaaatg

SEQ ID NO: 16930 - RNA, 16604 nt, Homo sapiens
  source 1..16604: mol_type = other RNA
taggactgtgcttggcacatagaaaatatttaactcagccaggcgtggtggctcatgcctgtaatgccaacagtttgggagaccgaggcgggtggatcacctgaggtcaggagttcaagaccagcctggccaacatggcgaaaccccggctgtactaaaaatacaaaaaaattagctgggtgtggttgtgcgcacttgtagtcccagctgctctggaggctgaggcaggagaatcgcttgaaaccgggaggcagaggttgcggtgagccgaggtcgtggtgagccgaggtcgcgccactgcactccagcctgggagacggagcgggactacgtctcaaaaaaaacaaagcaaacaaacaaacataaaaaatatttaacaagcctgaacttgtttattttttaatatatttatttatttatttattttgagacggagtcccactctatcacccaagctggagtgccgtggcgtgaccttggctcactgcaacctccacctccctggttcaagcaattctcctgcctcagcctcccgaacagctgggactataggcgggcgccaccacacccggctaatttttttgtatttttagtagagatggggtttcgccatgttggccaggctggtctcaaactcctgacctcaggtgatccgcctgtctcggcctcccaaagtgctggcattacaggcgtgagccaccgtgcccggccttaacaagcaacatggtgaaaccccgtctctacaaaaaaatacaaaaactagctgggcatggttgcatgcacctgtaatccctcgtacttgggaggctgaggtgggaggatcacttgagcctgggaggcagaggttgcggtgagccaagatcatgccactgcactccagcctgggtgacagagtgagactctgtctcaaaaaaaagaaaaagaaaaagaaaaaaatatatatatttaacaaatgttaactatttttattatcatatttatgttaacaaatgcacactagaaatggcaatcatttcttccctgggtactgatcacattacatgctcctcctggttttcctcctccgccctggctgctccttctgtctcctctgccagctcctcactccacccaagctctcccaagctgggcttcccagggcttggttatgtgctctgtaccttcctttctctttctctttccgggagtcccatagctttaaatatcaaatttacaccttctggccagaaatcctcccctgagcttcaagtccatctgcctcctagacttctccacttggaagtctaatacctatcttaaattaaataaattcaaacgtgaatacttggttgtacatcctggccaacttcttcctttccccagtcattctttttaagtatatatcaatatattccacccatttgctcaaacaaatactaggagccactcttgattcttttctttctttattcccatatttaatttattagcaaatcttgattttgactctgaaacgaacccccggttcatcccttcctctccttctacctggctatctagtccaagccaccctcatctcctgtgttgctccttaattgtggtctctcacttccctcatgccattccttcccaagctcctccccacccgtggaccccaaacacaactacaacatctacagtgatgtttaaaattgtggttaaaaaattacatagtataaaatttactatcttaaccatgtttaatatgatgttatctgcatgcatattgttggacaacagatctttagaactttttatcttgcaaaactgaaaccctgtaaacactgaacaacaatttccattttcttcctcatcccgatccctggcaatcaccattctgctttctgtttataagagtttgactactttagatatctcatagaagtaaaatcatgcaatgtttgtcctttattgattggctcatttcacttagcttagtatccttaagtttcatccatattgtggcatatgacaggaattccttcttttttaaggctgcataatattctattttatgtgtatggcacattttctttacccattcatccattcatgggttgcttctctcttgtggctattgtgaattaagctgcgtgaacatgagtgtgcaaatatctcttctgttttcaattcttttggatatgtacccagaagtgggcttggtggatcatatgagggttttatttttaattttttgaggaacttccacactgttttccttagtggctctaccattttacattcccaccaacagtgcacaagggtgtcagtttctctacaccctggccaatacttgttattttctggagtttgatcatttgagagtggccatcctaatgggtatgaggtgatatctcattgtggttttgagggtcatcttctaaaaatatagatgctgtcatgttcctttttggaaacttccaatggctttccttgaacttagaatgacatctaagtaccttacttttttttttttttttgagatggagtctcactgtgccgcccaggctgtagtgcagtggcacaatctcgggtcactgcaacctccgtctcatgggttcaagcaattcccctgcttcagcctcccgagtaggtgggattacagttgtgcaccaccaagcccggctaattttaagtaccttactttggcctccaaaatctgatctctgtccacattctggcctttattttcatctccagggcttcttgcttatggtggtacagtcacagtgaatgtgtttgactctttaaccacgtgagcatggtcctgttttcccatgtgcagttccttctgcttgggtctttctcttccttttcacatggctggttccttctcattattcaggtcttagctcaaatgctaccacatccaaggtggcattcaagctgtcccatctaaaatgcttctcctagacactctaaattctatcaccctgtttatttcacttttgctttttgtagcagttatcaacacctgaaattattttgccggtttagctgttggcttatgtagtggtttttttttttttttttttttttttaaatcataccaggaagtacactccatgagaccaggagccctgtgtgtctcattcacagctagatccccggaagggagcctgatttaatgaaaacaaaatgtaacagaacaattaatgccagctgggaggtttggggaacccttcatgaaggatgtaaccattttgttgggtttggaatgatgaatataatttcaacaggcagttgtcaggatgaagtaggggacattttaggctgaggaatgacatgaagtatatgcggagggagcacacagcatcacattttcaaagaaaggtagcttgctatggctgaaactaaaggttccgaagaggaggtggtgagcaggaaggctgaaatggcaggctgaggtcaaagcggcagacattgaattcatttcagttccgccgatttgctatttagttagtgatgcattaggcttgaagatacaaagatgaataagacacagtagtatgccgtcctgcagcagtggggacccacgtgtggcttttgagcagggtaatgacatgagcatgttacagaggtcagaatgcagcagtggttatgagcatagcctccagcaccagatggcgtggaatcaaatcctgctctgtcactatctagctgtgtgaccagggcaagtgtttaactcctgcggcttaattttcttacggataaagatgatgataataactgtggctctcttggctttcttatgagggttaacatttgtagcatggagtctggtactcaatacatgttggctattgacatgcaacgtgttgaggaaaacgatgtcagtacatggtacattttcaatgattgtttgttaggtttctcattttgtttttgagaaagatgatttattggcagcagtgtagataatcatttcaaggaggagacagtgggcacagccacaccaccgtggaagctacggcaatcgttgtggcaaggggaatggtgcacagaattagcttagagcagagataggcagcggaacagattggaggatgtagaggggctgcagaatattttttggaatgaaacaaagtgggtttaatttttgggtctgttgagcttaaggtgcctgaggaaaatctctgtttgctgatgtttagctgaaacaataaagagtcatctgaagtttaggacacagaggtgagtgaaatagagatttgtactctggaaatgtgggtgtgcacattaacaaactgctaagaatttgcattgagcctatcactcacctagtacactggtaaagaaacatgaccatgttttatactcgtgtactgttatgcattactggcagggatgtaaatttgtacaactttgctggaaaacaggtcggcaatatttgtcatgagccttacagataattgcatcctctgacccagtgatttcactttttggagtcaatgctaactttatgatccaaacacagacaattaattattatatacagagctgctcaccacaacataacattcaattgaaaaaaaaacaaaaccttcaaacaggctcactcagtgacaggaaaatggttaaataatgatgtgttcatacgctagaatattatacagccattaaaaaatcatgttgactgagactcctagtgtgaattgctataagggagaaaaacccaatgtatatacaattatatacagaatatgagtttgactctgcttaaaaataacataatgtaaggattagaagacaatatactaagatgttcatattattatttctgtttgggaaatggaggcatgggttggtatttgttgaagtctagtaactgagtttgacttatgactatataatagatttttggcttacttaaaatttcttttccttcttttcctaatgcatctcgtaatatttagttactaacacagtaacaatctttgggcttacagaccaaaattcaaatggcaatttctattacaaatcttgaccatgttttttttttttttttttttttttttgagatagcttctcactcttccacccaggttggagtgcagtggtgcaatcatagcttattgcagcctcaaacatctgggctcaagcaatcttcctgcctcagcctcccaagtacctagtactataggcatgtactactatgtctggctaatttttgtattttttttttttttggtagagatgggatctcacaaaaaaatataaaaattcgcattttttgatcctcctgccttggcctctcaaagtgctgggattacaggcatgagacaccactttttgtttttaatagatgcagtccatcaaaggcccagaacctcaaacttcatttttgagttaatgtcatgtcattgtacaattttgaatgtgccactggaccactgaagatgtttccttctctcctggcttattggcacaatcatccacttgcatttagagggacatgatttttacacaaggggttccttgggtatgtcagagacagaagattagaacaatacaccatcattgagagggtaattcatcaaaagtcctaacttcagctgcacagccaagcagctaaaagaaacccagtgaccctcggaagcacccctgatagacagctgttgggtgtgaaggatccatccataagtcgccagaattggatcgcaaatatcctagagctgacgatctcctggatcatgctgccataactgccttcaagatgttaatactgaacaaggcatgttgtttcagcactgcgggaggagcaatctctcttcccaacccctccgcaccctcccacccacacacgtgcacatgcacacaagcacatgtgttgatatccagcccagtcccatttctcttgctgagactgaccttgatagaaaaactattttgtttttattatagaaggcaagttttctatttactatgtagaaacagataaaaggctactgaagaggtgatgaacctcaccgtgattattaagtgagcaaaaatatttatactaaagtttaaatacttatttgcttatactatagtataagtaagccaaaaattgattatctggtcctaattaattcaaattcgtttactaaacttcaataaattaccaacccatgcctcagtttcccaatattttccagggctatatggcctgtggatagaatttaccatcattctgtgcttttaggacctttttgacattctaggtcaaacttggggaattttcctttttaggagtcccaactactcaaggcagaagccagcaaacacccttgctctgcctttctaagattcttacagggtgcaggcatatgaactgtgggaactgacgaccagttacaccccgttgggactctggttcgggagtgagagatggggaggcaggcgcaattttctcaacaggagatggtcgtggcaggctgaggagcttaagatttgagggtagcaggatggtggagtctttcctggaacaactctacagactgatttgggcatttgttcctggtgggctagcctctaaatccaactctgtggtcctaaagtaggcattgaagaaaaagcatccagcatcgggtaagagaacatgacttgataagcatcaagtaaagcttcaactagtttcagtgtcatctatgaatatttccagtctccatatcagacagtgcttttttggaaagaaagaaaagtatccttgcctttgagtaggccttccggtcaacaggttagttcaacattattccgtcatagtttgggaaaacaattcctttgacaggtgggtccctcaccccccattcatttctccatgtttaaagatatctgcatatactacccaaagtttaatcaggaaatactaaaataaatataatattgagcatattcatgtaatggaattctatatagcagtaaaaatggaaaaaccactattttactaacaatgacgactcttacaaacatacatttcaacaaaaggagccagacacaaaatctacatactgtatgaacccatttatagaaagctaagatgacaggcaaaactacaccatggtgtgattagtcaggatactgatacattcacagaggcatgagcacagtagcttctgggatgctgataatgtgctattgcttaaactgggtggtggatacatcagtgtgtcagctcgtgagaactgttacactaatgatttgcacacttttgttagtattctgcactttaataaaaagtgtttttccttgatttgcctgtcattttttaaactttatatcttatcaatattcaatcttgcacaacttacattgttttacaaagctatctactacatattgctagacctcaagttatcttttttttatatttaaagaaaaatacctggccagatgcaatggctcacacctgtaatcccagcacttgggaggctgaggcaggtagatagatcactttaggtcaggagtttgagaccagcctggccaacatggtgaaaccccgtttccactaaaaatacgaaaagtagctgggtgtggtggcgggtgcctgtaattacagctacttaggaggctgaggcaggagaatcgcttgaatccaggagggggaggttgcagtgagctgagattgcaccactgcactacagcctgggtgacacagagagattcgtctcaaaaaaaaaaaaaaaaaagtaaagaaaaataccaatacacggggagttctaagcacagaaaaataacctaaggattatttttcaatttattcaaatgaaaccaaagatgggcttgccgtggttaactagagtctttctcaaaagaaagatttcaatctggtgtatgtttaggaggcttgtacactctcagcttctcagttaagtgtctgccaagactcttttctctgactacacattgagcctccaaaccatgactgaaaaaccacagcttcatgggcagggccctgtgcaggacaccctatttccaaatgaacaagaaatgaaagtgagataaaaaaatattttaaaggtaaaagtttcacattatttaatgcaagctagctgtcaaggagaaagtagtgatgaatgaaaggaaaggaacaaagacaccacagagatgcacatcaaactggaagcagacaaaggcagccagaactatcttatttattataaagatacaccgtgaagaacaaacctgactgtatactgaagcctgtaatggtacatgccaaaaatgtacagtactatacataaaagtgcattgtcacaacagattaacaaaacattttttttctttccagactgtaaaagcatccccctttattttcacctcagagaggagggaatgaaatggtgagaggcagtacagagcacgggcgaatgcgatgctgtcagcagcacatgagcgggggactgatgcggtgggatgggaggacacaggggtgagaaaggcacaatcacgtctacaaggaaaacgagacagtctgaggaccgacagggaggtgagatgggacattactgagcaccgaggcacaggaaggcggggatggggaaggtgggggacagggaggaagcttcgaaacactcgagtgggcagcaggaattgggaggaggaggtgggggtggggcacagagcggggcaacggtacaagagcaaggctaaaactcctctaaaatagaaaggcactttcacatgtacatactacagatgtacattgacacaattaggtaacagtcacaagcaggaagctaccggtaccgcaattgatcaaaccgacaggaaaggacaatactgatttaattacgcgggcagcagttacccttcagtacgtaggtaaacagcagtctctcctgttacacagccacttactatactttaaatatctataataaccatcacactacacactgaacttggatgaatgctctaaggggggcattcacaaatgcacggttcatatattttcttttactaaagtttctaagataagcattatggaacccagtacaattatttaaacatacaaaattccctacgtaatttaaagacacaggtatccatctcgattataccacatagacttttttttttttttaagaacgtatactagggtaagtgaaagctcaaattccagtttgctttatggatctgacaaaacttcgccaaagtcaccctgcaccaagcctgactctccagcccagctggagcttgtgttctcaacttgggaggtgggtggcaggtggtctggagtagggagctctatttacgcctgggtagagacttctaagctgctctgtgtctcagggtttctgtggtggataatcgaaaacaagactgagtcctaagcacatttcctgcacaaaaaatggcctctcactgctatggtcaggaatcaatgagcatcatcccaaatttgaatcctctaacccccgcctcaagagacacataggctctttaactttggatttccaaggctgatcagatgaaagtttcttcagtttgtagactccagaggctatgtcattcctaaatgttaaggacacaactaccaacccacgcctcttttccttttctttaaattataaaccccccctttttttggtcgcgggggggatagcaaaagttagaaaacccttaacggatacaatttgactcttggagcactatatccactgataactgttcacgatcattgcagtagattgtgggaccctgctataaattattctacaggtggctcaaggggcaccaaagccagattatgttgtacgaagatgtgcaaagctgttgaatggtgttgacactgaacgtgaacatggagctctacaaagcgccactcagcaggttcaaacagttcacgtaacgcccattagaaaatgtgtactaagtacacctttctctctatccccaaatccactccccaaaccccaacccagtccaaaaggctgacttgatgaatctccttcagtgagttctatggatgggatgtgaacacacagttatatcagctgagaatacatattcttgtgtcagtggagtcaggtaatctttgtagagccattatttacccaccatcaaaaagctcccctccccaaattgcacatgaagcctgataagctccttgaaattgggggcagaacacctcaaggcctcattatccttcttctctcgtttccctgtgtcttcccacctcccctgtgtgctgcctctgtggctataaagaagggctgtgaaccttctcagctgcagtggcttttaatgagctttactgagcatgattctggattctttgtgaagtggccaccttgtcttatctctggaatctgaagacatttaataaaccaagtaaggagaggtgagtctttactgagtcctcactcactctgaggtcatacccttcatttggaattgaaaaaaaaaaaaagtctcaagctgacaataggagtatagggaaataagatggagacaggtaaagtgagtgatgggagagtattaggagctgtttcctgaaacaaggcacagcctgtgaggctctgcagcagcacgactcctgccggccaagacagcaaagtcctgatggggagcacagaaaggcaatcctcgttccaccgtaggtggacacatcagagagaggagccgctggggaggatgaccagatagaaggctgaataaatgaacaggtaggaggaagatctgaaaagctaaggctgaagctcagaaaagacattgaaaaaaaataaattcaaagacacctctggccctttgatgccctctgttaacatcttactcttccatcaaacaaggaatatggtttttaagaattcttactattttaaagaagtggtggaatggccgggcatggtggctcacatctgtaatcccagcactttgggaggctgaggctggtgggtcacctgaggtcaggagtttgagaccagcctggccaacatggtgacaccccatctctactaaaaatacaaaaattagctgggcgtggtggtggcgcctgtaatcccagctactcaggagaattgcttgaacccgggagatggaggttgcagggagccgagattgcaccactgtactctggcctgggcgacagagcaagactccaactcaaaaaaaaaaaaaaaaaaaaaaaaaagtgggggattattttggaaagtttaaattcctaaggaatttgtgaggattgtttaaaagggctagtgctattcaaagctcagtcttggctggatctccacggtgtccaagggtgctgaaggaccccaaaagctcaggagaaatggggaggggctagacaaggtgctgtcctgggcttctttttcaaaatgggcaaaaagtatggctctgaaaatttggaggtttaaaagtttaccatacctagaaatacatgggaaaaaagtcactattcatttgtgaaattaggccccaggcaagcaatcagcagtgtgactctgaaagtaacaatatctcatcaatttaatctcttcctgcaatagaatgactacactggcaaactgaggtagagatcaaagtaatgatcttgattttagtacagatcccagttcttttctgcacgatgcattcaccaatgggctgatgaagtaaaatctacactgtgtagctcttagatgggcgtgcaattggctgccagtttgaaatgaaaccaagaaggaaattaatggtgggccagagggattagttgtgggaaatccatttctcccaacaacaacaacaacaacaaaaatctttatcagtaacttcaatgatagaatagataaaatgctcataggtctacaggtgatatcagctgctgctagtaggagaatggaaatcaaagcaaattttcttaagatgggggaaaatgtagcataaatataggcttaaaaaattgcctgtgtgctaggatgccagagaaagagggtctccaattgagagttcagctgactatgggagttacatagagcccacatacaaaaccaaaaccaaaaaggggaaaagggacaaagaaaaagaagttgtggttgtgaggtacacaactgggtgagaaccacaaggccatgttctgctgatggccctgcatggctcttactcaggtaccagggccagttcagggttggctcaaagacaaatggagaggacagttgggatttcaaatttaggatcatcaggactttgtagcattttttttttttttaagagacagggtctcacactatgctgcccaggctggactcgaactactaggcccaaagccatcctcctgtgtaaaccacccgagtagctgggagtacaggtgtgcaccaccatgcctgggctttgtagcatgtttaaaggaacctaggtgatttagtcaaaagagaacactgcatgaaccaaggcctcaggtgcttcttgctgccttcatttccacagaggagaacacagggatttagaggagatggaaacattttctaggcagttattgaataacggatctttggaggagttcgtggagtagtgtaaccagaaagtctttaaaattaaacccttctaatcgtttgtaagtgtagatggggggacttggaaatctccggggcctaatcatgctcgcaaaaggagtgacattaatagctttggagatggtgtcttcctctcctttcccaggttaagttcaagcagtaacagcagaggttctacctccttccatcgagtctttaagctggacccggggaaataactgttaggaaagaggcaagcatccaacccactcgagctgtgggctgacagtcccactgggatcgtcccatggagacaattgcaagtcttttgcatgagctaaaccccgctccacatggaaccgaaggtgctcattgtcagctaccacgcaatgccattatcacctttcagcccaagtgccacagaccaacactggctatactccaatgaggtgtggcattcgggttcttctgccttcaggtcacaacctttctgactcagctgggctacattaaacctgaagctctgtacaatgtggagagcggtgttgccttcattacaagtggtgcagcattggattttcaagtaagtctaagtgtttctattgtccttaaaatgacatatgtccagttatttaaaaaaattacaaaatacaaatgcccgtgttaatttagctagtctcagacattacattcgacaacatagaaaagccaaaagatctccagttataagcacaaaactaaggaaagttatggatcagtgacttttgtcactaatccattttcttttttaagtcacctccctttatggccttgcttggctggtttttacattgtgcatgacttgtctgttggaccctggggaggtggggcaggtcctatggtaggatttgtttttggaagaacagcaggttttggcctaagggctggaggcttcagctgcacgcccattctgggtgccaccataggcttgaaagtactcattgtgtcactggaggagctcgtgctacgtcgaatctgaggctcggagctcctgagggcaacgttgtgcaaagggctgagagattccgtggaagtggcaggggtgggagagtttttcacttgctccagggtatccagcaccacatcaggggcatgctttgctgtgctctgtctctccagttctcggagttcattcaaagctgtgttcatcgtttcttcaatatcctgagcaattgtctctgggtccagtggcttgtggtcattgaagcccgtgtattgccctgatgacgtggaccttctaatgggagggctgtcgatcttcttgagggagtcgtgccggctgatgttggtcaggctgccatggccaggcctgcgcctccgctcaggactgtcattgttgaggccacggttctgcagcaggccccgggggtgactggcaaggcttggggaccctaggtcaactgaggagttagaaagggcatgtggagggtggagcgggcaatggccatcactggtcctgccaggacgccttactggagggggtggctctcctctttttcgttgcctggctaaatagccgtcaggatgacggtctgtcggggagttcatgtccttggatgaggacttgtcttccgtgactggcccactgctggcctcactgtcggctttttggctcagagtgtctgaaaacgtatcatccatatcctgcaccactatatactggtgaggcaccagcccgtcaatcccgttgtgcctgccttcccaccagtcctcagatgcacggtgatacagcagcagggaggcacccttcttgaaggatagttctctggcagaccgcccaacatagtcaaacttggctattgcttctattggctcacattcatcttcacttgtgtggggctctgtaccagcatcttggtccacttcctccaatgtaccgtgctcactgtatgggctgtcgcaatagtcatctccagccatacatttctcataaacagggccatccagctctttagcatctgggaaaatagtctcatggtggatgatgatggttttgataatttcattcacatgtgcctggcaagacacttgatcctgtatttctgggacaggcatcaatgttgggccaaagcaaatggccaggttataagggtccatcatattctcatcgctgtactgtgatagatgattgaggaaggcaaagaggtacctcatcactataaggaccgacctgggcaaagtcaggaggagtttgcggatgtgaagcgccctctcatagagattatctattctgatacaagaaatcagatcgttaaatctttccttaggaaagagggggttttccagcccacggaaatagagcttcagaacgccagcaactgagttaatatcatggttactctggtcatcagccaaaggattttcacctctctcaaatgaatttttaatatcattgacttccacctgggaaccagacactctgaaaatcccctgatgctgaagaccatagagattgatgaaccgaatacagctttccacaatgaggggaataacctgtcctgagtcctgatgtcttgtgtgcgagtttcttcgtcctcggcttgtagtcatatattcagctctatgaccttctcccagggtcctctgcagcaagtcatgtttggcttgaagttttgtgatgagattactgccttccaaatattctctgagtttcatgaagtagaactgttcagtttcctgctggttggctcttctcttggcgatgctgggtttactcaggtaggtttcagagacagtggacttcactgattctgtggaacgactgtgctggaagcattcagaaacatcatagtcctcgatggtgaccatatcttgtatcgtctgcaaggtggcttcagtcgttttcttaacctcttcattctcgattttgagcgtggcaaggcgggactgcaactgttggtacctgagcatgagctctgcctggactggctgctgggcactgacctggcacacctcatcacccatgtgagactgaaactcaaacttcattggtggacagaacgcagcagggtacatctccatgaatctctgcttatcgctcctgggctctaaattatcaactgcattctcaataatgtctaagccctcatgtctggaggtttcaaggttgtactccgcagacagatatgttcttagggctctgttcagacttgcatggtagccaagatcacagcaatcaattaaatcagaaagatcatgaatatagtacttgaaaactgaggcattggtggcttcaagtgttaggagatattcgttccgtgccttaattgattttagcttattttctgaatattttgcttgtcttttttctttcattttttcaattttctttacagagcttcgccgttgatgtctctcctctagtcgaatatggaagactggatcaccagatctcccaatttgcttttcctcttgtttttcggcctctttcagcttgctctctgcactgatgctctctgcatgatacatatggtatgttttcatcaccgtataaagctcattaagaaccttcattaaatcctcatgaagttggaatgcaatctctttgctctttttaaacatcctggtagaatcctcacttatctgcatgaaccgcataatcacattgttcagatagatgtcactcaaggttgcatggtctttgctttctctccttacttggttcaggagcaaataccagcagttcactggagacaacaggttctggtctttcttgtattgttgatgatccttagtgcttcttgtttttgccatgaacctttctgctaacttctctagattccgggaatattccgtctcaatttcagctttttttcggaagaaatcttgcagatcctggagaagctgaactcgcatctccgtttgctgctccaggcatttttgttgttctaccagttgagctcgaatttctttgacttgactttcatactcggctatgatctctttgtccttcttgaatcggctcggggtggacattatccagctgttccgggtttgctttcaatgggcaagttttgttcagtggtcacaacccgttctccttggagaggcagagttgtactcccacacgcaggcaatccagaggcagcgccg

SEQ ID NO: 16931 - RNA, 16673 nt, Homo sapiens
  source 1..16673: mol_type = other RNA
taggactgtgcttggcacatagaaaatatttaactcagccaggcgtggtggctcatgcctgtaatgccaacagtttgggagaccgaggcgggtggatcacctgaggtcaggagttcaagaccagcctggccaacatggcgaaaccccggctgtactaaaaatacaaaaaaattagctgggtgtggttgtgcgcacttgtagtcccagctgctctggaggctgaggcaggagaatcgcttgaaaccgggaggcagaggttgcggtgagccgaggtcgtggtgagccgaggtcgcgccactgcactccagcctgggagacggagcgggactacgtctcaaaaaaaacaaagcaaacaaacaaacataaaaaatatttaacaagcctgaacttgtttattttttaatatatttatttatttatttattttgagacggagtcccactctatcacccaagctggagtgccgtggcgtgaccttggctcactgcaacctccacctccctggttcaagcaattctcctgcctcagcctcccgaacagctgggactataggcgggcgccaccacacccggctaatttttttgtatttttagtagagatggggtttcgccatgttggccaggctggtctcaaactcctgacctcaggtgatccgcctgtctcggcctcccaaagtgctggcattacaggcgtgagccaccgtgcccggccttaacaagcaacatggtgaaaccccgtctctacaaaaaaatacaaaaactagctgggcatggttgcatgcacctgtaatccctcgtacttgggaggctgaggtgggaggatcacttgagcctgggaggcagaggttgcggtgagccaagatcatgccactgcactccagcctgggtgacagagtgagactctgtctcaaaaaaaagaaaaagaaaaagaaaaaaatatatatatttaacaaatgttaactatttttattatcatatttatgttaacaaatgcacactagaaatggcaatcatttcttccctgggtactgatcacattacatgctcctcctggttttcctcctccgccctggctgctccttctgtctcctctgccagctcctcactccacccaagctctcccaagctgggcttcccagggcttggttatgtgctctgtaccttcctttctctttctctttccgggagtcccatagctttaaatatcaaatttacaccttctggccagaaatcctcccctgagcttcaagtccatctgcctcctagacttctccacttggaagtctaatacctatcttaaattaaataaattcaaacgtgaatacttggttgtacatcctggccaacttcttcctttccccagtcattctttttaagtatatatcaatatattccacccatttgctcaaacaaatactaggagccactcttgattcttttctttctttattcccatatttaatttattagcaaatcttgattttgactctgaaacgaacccccggttcatcccttcctctccttctacctggctatctagtccaagccaccctcatctcctgtgttgctccttaattgtggtctctcacttccctcatgccattccttcccaagctcctccccacccgtggaccccaaacacaactacaacatctacagtgatgtttaaaattgtggttaaaaaattacatagtataaaatttactatcttaaccatgtttaatatgatgttatctgcatgcatattgttggacaacagatctttagaactttttatcttgcaaaactgaaaccctgtaaacactgaacaacaatttccattttcttcctcatcccgatccctggcaatcaccattctgctttctgtttataagagtttgactactttagatatctcatagaagtaaaatcatgcaatgtttgtcctttattgattggctcatttcacttagcttagtatccttaagtttcatccatattgtggcatatgacaggaattccttcttttttaaggctgcataatattctattttatgtgtatggcacattttctttacccattcatccattcatgggttgcttctctcttgtggctattgtgaattaagctgcgtgaacatgagtgtgcaaatatctcttctgttttcaattcttttggatatgtacccagaagtgggcttggtggatcatatgagggttttatttttaattttttgaggaacttccacactgttttccttagtggctctaccattttacattcccaccaacagtgcacaagggtgtcagtttctctacaccctggccaatacttgttattttctggagtttgatcatttgagagtggccatcctaatgggtatgaggtgatatctcattgtggttttgagggtcatcttctaaaaatatagatgctgtcatgttcctttttggaaacttccaatggctttccttgaacttagaatgacatctaagtaccttacttttttttttttttttgagatggagtctcactgtgccgcccaggctgtagtgcagtggcacaatctcgggtcactgcaacctccgtctcatgggttcaagcaattcccctgcttcagcctcccgagtaggtgggattacagttgtgcaccaccaagcccggctaattttaagtaccttactttggcctccaaaatctgatctctgtccacattctggcctttattttcatctccagggcttcttgcttatggtggtacagtcacagtgaatgtgtttgactctttaaccacgtgagcatggtcctgttttcccatgtgcagttccttctgcttgggtctttctcttccttttcacatggctggttccttctcattattcaggtcttagctcaaatgctaccacatccaaggtggcattcaagctgtcccatctaaaatgcttctcctagacactctaaattctatcaccctgtttatttcacttttgctttttgtagcagttatcaacacctgaaattattttgccggtttagctgttggcttatgtagtggtttttttttttttttttttttttttaaatcataccaggaagtacactccatgagaccaggagccctgtgtgtctcattcacagctagatccccggaagggagcctgatttaatgaaaacaaaatgtaacagaacaattaatgccagctgggaggtttggggaacccttcatgaaggatgtaaccattttgttgggtttggaatgatgaatataatttcaacaggcagttgtcaggatgaagtaggggacattttaggctgaggaatgacatgaagtatatgcggagggagcacacagcatcacattttcaaagaaaggtagcttgctatggctgaaactaaaggttccgaagaggaggtggtgagcaggaaggctgaaatggcaggctgaggtcaaagcggcagacattgaattcatttcagttccgccgatttgctatttagttagtgatgcattaggcttgaagatacaaagatgaataagacacagtagtatgccgtcctgcagcagtggggacccacgtgtggcttttgagcagggtaatgacatgagcatgttacagaggtcagaatgcagcagtggttatgagcatagcctccagcaccagatggcgtggaatcaaatcctgctctgtcactatctagctgtgtgaccagggcaagtgtttaactcctgcggcttaattttcttacggataaagatgatgataataactgtggctctcttggctttcttatgagggttaacatttgtagcatggagtctggtactcaatacatgttggctattgacatgcaacgtgttgaggaaaacgatgtcagtacatggtacattttcaatgattgtttgttaggtttctcattttgtttttgagaaagatgatttattggcagcagtgtagataatcatttcaaggaggagacagtgggcacagccacaccaccgtggaagctacggcaatcgttgtggcaaggggaatggtgcacagaattagcttagagcagagataggcagcggaacagattggaggatgtagaggggctgcagaatattttttggaatgaaacaaagtgggtttaatttttgggtctgttgagcttaaggtgcctgaggaaaatctctgtttgctgatgtttagctgaaacaataaagagtcatctgaagtttaggacacagaggtgagtgaaatagagatttgtactctggaaatgtgggtgtgcacattaacaaactgctaagaatttgcattgagcctatcactcacctagtacactggtaaagaaacatgaccatgttttatactcgtgtactgttatgcattactggcagggatgtaaatttgtacaactttgctggaaaacaggtcggcaatatttgtcatgagccttacagataattgcatcctctgacccagtgatttcactttttggagtcaatgctaactttatgatccaaacacagacaattaattattatatacagagctgctcaccacaacataacattcaattgaaaaaaaaacaaaaccttcaaacaggctcactcagtgacaggaaaatggttaaataatgatgtgttcatacgctagaatattatacagccattaaaaaatcatgttgactgagactcctagtgtgaattgctataagggagaaaaacccaatgtatatacaattatatacagaatatgagtttgactctgcttaaaaataacataatgtaaggattagaagacaatatactaagatgttcatattattatttctgtttgggaaatggaggcatgggttggtatttgttgaagtctagtaactgagtttgacttatgactatataatagatttttggcttacttaaaatttcttttccttcttttcctaatgcatctcgtaatatttagttactaacacagtaacaatctttgggcttacagaccaaaattcaaatggcaatttctattacaaatcttgaccatgttttttttttttttttttttttttttgagatagcttctcactcttccacccaggttggagtgcagtggtgcaatcatagcttattgcagcctcaaacatctgggctcaagcaatcttcctgcctcagcctcccaagtacctagtactataggcatgtactactatgtctggctaatttttgtattttttttttttttggtagagatgggatctcacaaaaaaatataaaaattcgcattttttgatcctcctgccttggcctctcaaagtgctgggattacaggcatgagacaccactttttgtttttaatagatgcagtccatcaaaggcccagaacctcaaacttcatttttgagttaatgtcatgtcattgtacaattttgaatgtgccactggaccactgaagatgtttccttctctcctggcttattggcacaatcatccacttgcatttagagggacatgatttttacacaaggggttccttgggtatgtcagagacagaagattagaacaatacaccatcattgagagggtaattcatcaaaagtcctaacttcagctgcacagccaagcagctaaaagaaacccagtgaccctcggaagcacccctgatagacagctgttgggtgtgaaggatccatccataagtcgccagaattggatcgcaaatatcctagagctgacgatctcctggatcatgctgccataactgccttcaagatgttaatactgaacaaggcatgttgtttcagcactgcgggaggagcaatctctcttcccaacccctccgcaccctcccacccacacacgtgcacatgcacacaagcacatgtgttgatatccagcccagtcccatttctcttgctgagactgaccttgatagaaaaactattttgtttttattatagaaggcaagttttctatttactatgtagaaacagataaaaggctactgaagaggtgatgaacctcaccgtgattattaagtgagcaaaaatatttatactaaagtttaaatacttatttgcttatactatagtataagtaagccaaaaattgattatctggtcctaattaattcaaattcgtttactaaacttcaataaattaccaacccatgcctcagtttcccaatattttccagggctatatggcctgtggatagaatttaccatcattctgtgcttttaggacctttttgacattctaggtcaaacttggggaattttcctttttaggagtcccaactactcaaggcagaagccagcaaacacccttgctctgcctttctaagattcttacagggtgcaggcatatgaactgtgggaactgacgaccagttacaccccgttgggactctggttcgggagtgagagatggggaggcaggcgcaattttctcaacaggagatggtcgtggcaggctgaggagcttaagatttgagggtagcaggatggtggagtctttcctggaacaactctacagactgatttgggcatttgttcctggtgggctagcctctaaatccaactctgtggtcctaaagtaggcattgaagaaaaagcatccagcatcgggtaagagaacatgacttgataagcatcaagtaaagcttcaactagtttcagtgtcatctatgaatatttccagtctccatatcagacagtgcttttttggaaagaaagaaaagtatccttgcctttgagtaggccttccggtcaacaggttagttcaacattattccgtcatagtttgggaaaacaattcctttgacaggtgggtccctcaccccccattcatttctccatgtttaaagatatctgcatatactacccaaagtttaatcaggaaatactaaaataaatataatattgagcatattcatgtaatggaattctatatagcagtaaaaatggaaaaaccactattttactaacaatgacgactcttacaaacatacatttcaacaaaaggagccagacacaaaatctacatactgtatgaacccatttatagaaagctaagatgacaggcaaaactacaccatggtgtgattagtcaggatactgatacattcacagaggcatgagcacagtagcttctgggatgctgataatgtgctattgcttaaactgggtggtggatacatcagtgtgtcagctcgtgagaactgttacactaatgatttgcacacttttgttagtattctgcactttaataaaaagtgtttttccttgatttgcctgtcattttttaaactttatatcttatcaatattcaatcttgcacaacttacattgttttacaaagctatctactacatattgctagacctcaagttatcttttttttatatttaaagaaaaatacctggccagatgcaatggctcacacctgtaatcccagcacttgggaggctgaggcaggtagatagatcactttaggtcaggagtttgagaccagcctggccaacatggtgaaaccccgtttccactaaaaatacgaaaagtagctgggtgtggtggcgggtgcctgtaattacagctacttaggaggctgaggcaggagaatcgcttgaatccaggagggggaggttgcagtgagctgagattgcaccactgcactacagcctgggtgacacagagagattcgtctcaaaaaaaaaaaaaaaaaagtaaagaaaaataccaatacacggggagttctaagcacagaaaaataacctaaggattatttttcaatttattcaaatgaaaccaaagatgggcttgccgtggttaactagagtctttctcaaaagaaagatttcaatctggtgtatgtttaggaggcttgtacactctcagcttctcagttaagtgtctgccaagactcttttctctgactacacattgagcctccaaaccatgactgaaaaaccacagcttcatgggcagggccctgtgcaggacaccctatttccaaatgaacaagaaatgaaagtgagataaaaaaatattttaaaggtaaaagtttcacattatttaatgcaagctagctgtcaaggagaaagtagtgatgaatgaaaggaaaggaacaaagacaccacagagatgcacatcaaactggaagcagacaaaggcagccagaactatcttatttattataaagatacaccgtgaagaacaaacctgactgtatactgaagcctgtaatggtacatgccaaaaatgtacagtactatacataaaagtgcattgtcacaacagattaacaaaacattttttttctttccagactgtaaaagcatccccctttattttcacctcagagaggagggaatgaaatggtgagaggcagtacagagcacgggcgaatgcgatgctgtcagcagcacatgagcgggggactgatgcggtgggatgggaggacacaggggtgagaaaggcacaatcacgtctacaaggaaaacgagacagtctgaggaccgacagggaggtgagatgggacattactgagcaccgaggcacaggaaggcggggatggggaaggtgggggacagggaggaagcttcgaaacactcgagtgggcagcaggaattgggaggaggaggtgggggtggggcacagagcggggcaacggtacaagagcaaggctaaaactcctctaaaatagaaaggcactttcacatgtacatactacagatgtacattgacacaattaggtaacagtcacaagcaggaagctaccggtaccgcaattgatcaaaccgacaggaaaggacaatactgatttaattacgcgggcagcagttacccttcagtacgtaggtaaacagcagtctctcctgttacacagccacttactatactttaaatatctataataaccatcacactacacactgaacttggatgaatgctctaaggggggcattcacaaatgcacggttcatatattttcttttactaaagtttctaagataagcattatggaacccagtacaattatttaaacatacaaaattccctacgtaatttaaagacacaggtatccatctcgattataccacatagacttttttttttttttaagaacgtatactagggtaagtgaaagctcaaattccagtttgctttatggatctgacaaaacttcgccaaagtcaccctgcaccaagcctgactctccagcccagctggagcttgtgttctcaacttgggaggtgggtggcaggtggtctggagtagggagctctatttacgcctgggtagagacttctaagctgctctgtgtctcagggtttctgtggtggataatcgaaaacaagactgagtcctaagcacatttcctgcacaaaaaatggcctctcactgctatggtcaggaatcaatgagcatcatcccaaatttgaatcctctaacccccgcctcaagagacacataggctctttaactttggatttccaaggctgatcagatgaaagtttcttcagtttgtagactccagaggctatgtcattcctaaatgttaaggacacaactaccaacccacgcctcttttccttttctttaaattataaaccccccctttttttggtcgcgggggggatagcaaaagttagaaaacccttaacggatacaatttgactcttggagcactatatccactgataactgttcacgatcattgcagtagattgtgggaccctgctataaattattctacaggtggctcaaggggcaccaaagccagattatgttgtacgaagatgtgcaaagctgttgaatggtgttgacactgaacgtgaacatggagctctacaaagcgccactcagcaggttcaaacagttcacgtaacgcccattagaaaatgtgtactaagtacacctttctctctatccccaaatccactccccaaaccccaacccagtccaaaaggctgacttgatgaatctccttcagtgagttctatggatgggatgtgaacacacagttatatcagctgagaatacatattcttgtgtcagtggagtcaggtaatctttgtagagccattatttacccaccatcaaaaagctcccctccccaaattgcacatgaagcctgataagctccttgaaattgggggcagaacacctcaaggcctcattatccttcttctctcgtttccctgtgtcttcccacctcccctgtgtgctgcctctgtggctataaagaagggctgtgaaccttctcagctgcagtggcttttaatgagctttactgagcatgattctggattctttgtgaagtggccaccttgtcttatctctggaatctgaagacatttaataaaccaagtaaggagaggtgagtctttactgagtcctcactcactctgaggtcatacccttcatttggaattgaaaaaaaaaaaaagtctcaagctgacaataggagtatagggaaataagatggagacaggtaaagtgagtgatgggagagtattaggagctgtttcctgaaacaaggcacagcctgtgaggctctgcagcagcacgactcctgccggccaagacagcaaagtcctgatggggagcacagaaaggcaatcctcgttccaccgtaggtggacacatcagagagaggagccgctggggaggatgaccagatagaaggctgaataaatgaacaggtaggaggaagatctgaaaagctaaggctgaagctcagaaaagacattgaaaaaaaataaattcaaagacacctctggccctttgatgccctctgttaacatcttactcttccatcaaacaaggaatatggtttttaagaattcttactattttaaagaagtggtggaatggccgggcatggtggctcacatctgtaatcccagcactttgggaggctgaggctggtgggtcacctgaggtcaggagtttgagaccagcctggccaacatggtgacaccccatctctactaaaaatacaaaaattagctgggcgtggtggtggcgcctgtaatcccagctactcaggagaattgcttgaacccgggagatggaggttgcagggagccgagattgcaccactgtactctggcctgggcgacagagcaagactccaactcaaaaaaaaaaaaaaaaaaaaaaaaaagtgggggattattttggaaagtttaaattcctaaggaatttgtgaggattgtttaaaagggctagtgctattcaaagctcagtcttggctggatctccacggtgtccaagggtgctgaaggaccccaaaagctcaggagaaatggggaggggctagacaaggtgctgtcctgggcttctttttcaaaatgggcaaaaagtatggctctgaaaatttggaggtttaaaagtttaccatacctagaaatacatgggaaaaaagtcactattcatttgtgaaattaggccccaggcaagcaatcagcagtgtgactctgaaagtaacaatatctcatcaatttaatctcttcctgcaatagaatgactacactggcaaactgaggtagagatcaaagtaatgatcttgattttagtacagatcccagttcttttctgcacgatgcattcaccaatgggctgatgaagtaaaatctacactgtgtagctcttagatgggcgtgcaattggctgccagtttgaaatgaaaccaagaaggaaattaatggtgggccagagggattagttgtgggaaatccatttctcccaacaacaacaacaacaacaaaaatctttatcagtaacttcaatgatagaatagataaaatgctcataggtctacaggtgatatcagctgctgctagtaggagaatggaaatcaaagcaaattttcttaagatgggggaaaatgtagcataaatataggcttaaaaaattgcctgtgtgctaggatgccagagaaagagggtctccaattgagagttcagctgactatgggagttacatagagcccacatacaaaaccaaaaccaaaaaggggaaaagggacaaagaaaaagaagttgtggttgtgaggtacacaactgggtgagaaccacaaggccatgttctgctgatggccctgcatggctcttactcaggtaccagggccagttcagggttggctcaaagacaaatggagaggacagttgggatttcaaatttaggatcatcaggactttgtagcattttttttttttttaagagacagggtctcacactatgctgcccaggctggactcgaactactaggcccaaagccatcctcctgtgtaaaccacccgagtagctgggagtacaggtgtgcaccaccatgcctgggctttgtagcatgtttaaaggaacctaggtgatttagtcaaaagagaacactgcatgaaccaaggcctcaggtgcttcttgctgccttcatttccacagaggagaacacagggatttagaggagatggaaacattttctaggcagttattgaataacggatctttggaggagttcgtggagtagtgtaaccagaaagtctttaaaattaaacccttctaatcgtttgtaagtgtagatggggggacttggaaatctccggggcctaatcatgctcgcaaaaggagtgacattaatagctttggagatggtgtcttcctctcctttcccaggttaagttcaagcagtaacagcagaggttctacctccttccatcgagtctttaagctggacccggggaaataactgttaggaaagaggcaagcatccaacccactcgagctgtgggctgacagtcccactgggatcgtcccatggagacaattgcaagtcttttgcatgagctaaaccccgctccacatggaaccgaaggtgctcattgtcagctaccacgcaatgccattatcacctttcagcccaagtgccacagaccaacactggctatactccaatgaggtgtggcattcgggttcttctgccttcaggtcacaacctttctgactcagctgggctacattaaacctgaagctctgtacaatgtggagagcggtgttgccttcattacaagtggtgcagcattggattttcaagtaagtctaagtgtttctattgtccttaaaatgacatatgtccagttatttaaaaaaattacaaaatacaaatgcccgtgttaatttagctagtctcagacattacattcgacaacatagaaaagccaaaagatctccagttataagcacaaaactaaggaaagttatggatcagtgacttttgtcactaatccattttcttttttaagtcacctccctttatggccttgcttggctggtttttacattgtgcatgacttgtctgttggaccctggggaggtggggcaggtcctatggtaggatttgtttttggaagaacagcaggttttggcctaagggctggaggcttcagctgcacgcccattctgggtgccaccataggcttgaaagtactcattgtgtcactggaggagctcgtgctacgtcgaatctgaggctcggagctcctgagggcaacgttgtgcaaagggctgagagattccgtggaagtggcaggggtgggagagtttttcacttgctccagggtatccagcaccacatcaggggcatgctttgctgtgctctgtctctccagttctcggagttcattcaaagctgtgttcatcgtttcttcaatatcctgagcaattgtctctgggtccagtggcttgtggtcattgaagcccgtgtattgccctgatgacgtggaccttctaatgggagggctgtcgatcttcttgagggagtcgtgccggctgatgttggtcaggctgccatggccaggcctgcgcctccgctcaggactgtcattgttgaggccacggttctgcagcaggccccgggggtgactggcaaggcttggggaccctaggtcaactgaggagttagaaagggcatgtggagggtggagcgggcaatggccatcactggtcctgccaggacgccttactggagggggtggctctcctctttttcgttgcctggctaaatagccgtcaggatgacggtctgtcggggagttcatgtccttggatgaggacttgtcttccgtgactggcccactgctggcctcactgtcggctttttggctcagagtgtctgaaaacgtatcatccatatcctgcaccactatatactggtgaggcaccagcccgtcaatcccgttgtgcctgccttcccaccagtcctcagatgcacggtgatacagcagcagggaggcacccttcttgaaggatagttctctggcagaccgcccaacatagtcaaacttggctattgcttctattggctcacattcatcttcacttgtgtggggctctgtaccagcatcttggtccacttcctccaatgtaccgtgctcactgtatgggctgtcgcaatagtcatctccagccatacatttctcataaacagggccatccagctctttagcatctgggaaaatagtctcatggtggatgatgatggttttgataatttcattcacatgtgcctggcaagacacttgatcctgtatttctgggacaggcatcaatgttgggccaaagcaaatggccaggttataagggtccatcatattctcatcgctgtactgtgatagatgattgaggaaggcaaagaggtacctcatcactataaggaccgacctgggcaaagtcaggaggagtttgcggatgtgaagcgccctctcatagagattatctattctgatacaagaaatcagatcgttaaatctttccttaggaaagagggggttttccagcccacggaaatagagcttcagaacgccagcaactgagttaatatcatggttactctggtcatcagccaaaggattttcacctctctcaaatgaatttttaatatcattgacttccacctgggaaccagacactctgaaaatcccctgatgctgaagaccatagagattgatgaaccgaatacagctttccacaatgaggggaataacctgtcctgagtccttgacgaatgtttccaaatccccattaaacaacttagtattatactgtgagcggggcctggacttcctgtgtttctggggcttagggggaacatttggaggccttgtagtcatatattcagctctatgaccttctcccagggtcctctgcagcaagtcatgtttggcttgaagttttgtgatgagattactgccttccaaatattctctgagtttcatgaagtagaactgttcagtttcctgctggttggctcttctcttggcgatgctgggtttactcaggtaggtttcagagacagtggacttcactgattctgtggaacgactgtgctggaagcattcagaaacatcatagtcctcgatggtgaccatatcttgtatcgtctgcaaggtggcttcagtcgttttcttaacctcttcattctcgattttgagcgtggcaaggcgggactgcaactgttggtacctgagcatgagctctgcctggactggctgctgggcactgacctggcacacctcatcacccatgtgagactgaaactcaaacttcattggtggacagaacgcagcagggtacatctccatgaatctctgcttatcgctcctgggctctaaattatcaactgcattctcaataatgtctaagccctcatgtctggaggtttcaaggttgtactccgcagacagatatgttcttagggctctgttcagacttgcatggtagccaagatcacagcaatcaattaaatcagaaagatcatgaatatagtacttgaaaactgaggcattggtggcttcaagtgttaggagatattcgttccgtgccttaattgattttagcttattttctgaatattttgcttgtcttttttctttcattttttcaattttctttacagagcttcgccgttgatgtctctcctctagtcgaatatggaagactggatcaccagatctcccaatttgcttttcctcttgtttttcggcctctttcagcttgctctctgcactgatgctctctgcatgatacatatggtatgttttcatcaccgtataaagctcattaagaaccttcattaaatcctcatgaagttggaatgcaatctctttgctctttttaaacatcctggtagaatcctcacttatctgcatgaaccgcataatcacattgttcagatagatgtcactcaaggttgcatggtctttgctttctctccttacttggttcaggagcaaataccagcagttcactggagacaacaggttctggtctttcttgtattgttgatgatccttagtgcttcttgtttttgccatgaacctttctgctaacttctctagattccgggaatattccgtctcaatttcagctttttttcggaagaaatcttgcagatcctggagaagctgaactcgcatctccgtttgctgctccaggcatttttgttgttctaccagttgagctcgaatttctttgacttgactttcatactcggctatgatctctttgtccttcttgaatcggctcggggtggacattatccagctgttccgggtttgctttcaatgggcaagttttgttcagtggtcacaacccgttctccttggagaggcagagttgtactcccacacgcaggcaatccagaggcagcgccg

SEQ ID NO: 16932 - RNA, 4846 nt, Homo sapiens
  source 1..4846: mol_type = other RNA
taggactgtgcttggcacatagaactcaacaagtggtagcaattattattataaaagcaaaacaacctcttaaataaaaatcataaaatattagtgtcatcaaaattcagttattaaacatattttatgattaaaaagaagactgccaaaatcgtgaagcagttggaaaataaaaacattacacttgaaatttcaataacagtaagtttgagctagttgtatgtttgttttagaattttttggttatcatgagatttgacatcttaagtaaaaggtctgtttgttataccatgttctggtgtactctagtggttttgacaaggtatatacacacagatgttagaaaaaaaaaaacctttggttgttgcaattttctccttattgcatctaattgaaaacatagaggaaagtgtagaacacatctgtgggtacttttcataccagtgatagtaccatggaagccatggaagtctttaagagaactcctataggcttagaatgtagtgaaaatgttaggggactctataacatttgtattaccacccttacccttactccttacccacccacctgcaaaaaaacaaaaaagaaaaaaagaaactatcatagtaatcagctgcttcactgtgctaaaacgtatttctgttttggaaatatttgccaatgaaccaaaaagaatttggcatttggaaatatcttccattggcatagcttgtaatacaattcacagaaacttttaaaaacaacttgaatatagtatctgtaaactttcctatttaccacactttggggacaggatcttaaatcttcctatcttattcatcttcacttttgaagttctttcagaaatgttcatgctgattaatagttaaatgatttaagtattaacttacccatttctagcatatataatatagtagtagccttttagttgttttcttgcttctgaagcagccagcatccttacacattttttcattactcgttattgtcctcaaaaattgctcttcaagcaaaatgtggtttcctgtatttcctgtgtcattcaattaatgtatttctccaagtctaaccataagaactagataccacacactgtttcctaacagatggaaaatccttatgttttcacttaacatccctctattaagcagctctctctgggagctgtctcccttgccccattagtatgttaaagcagccagatccctgaaatataaatgataaaagtagatttcatatctgacattttaagttaccaggcatttttcctttatggcttaatcattgagatttttgaagattatatgtacaggaggggaaagatttttatttcagagactggaaaaaagcaacatagcattttagtagatttcataaaaatggagtaatagttaatttttataatttttttaaattttataattttttacttataaaattttactctagctattaaagacttctttttttataactacattttaacagcttttaatctaaccttaataataaatattagttcctttgcccagggcttggaaataatcagaaagagttctcaggcaaatctggctttttaaaatattttatcctgttgtattttgttgagatttcttgggaactggtacagggaaaagaagaataaaaaataagattcatttatttcttatttgctagaaaaaaagctgctattcataccaaacacacttttggactacagggcaattaaaaagaattcagtactaagaaaaaaaagctgctattgttttcttcactggcagaagcagcgagtaagtggcaactcatgactctaatgatgcatcatccctaggcagattatttataatgcatatgtaaagtcagtatcactagtgaaatctatatgtatttaaccctgaatcttcaatctcttttatcttttactttgaggaaacctattcttggtttacttgatacccgaactagtttggtatagaactgaacaattaacttctacatcaatttgtctgcactgtgactattttaactagctcagtttcaagccttgtttaaaaatggtaattcctctttctaaatttaattttatgtccaaatgtttttgttacagcctggccaaattcaggtccccatctaacttactatcatatttattcaaagactgaaagaaggccacaaggatgaagcatgaatgaagggtggattggtatgagatgagacaggatgtgggggtagagggatcaaatcatatatagctatatgaaggccatcataaggaggtcaaattttattctcagggaagccatttaaattagaatggcatgatgtgatatttcatttttaaaagatcactctaggtgctaaaaactacatggggcaggactagatgggagaccagagaggaggctcttagcataatctagaagattagaccagagtaatcaaggtgatggagagaaggggaaagattcaggacatgttttgcagataaaaggttccaggatctggtgacagatggtatgaaggctctaagcaaaagaagcatcaaagataggcctaggcctgatatttagttcatgccactgccttggctacctaggtctttgtgtgagtcttgttatgaagggccaatacttttctgtatctgatgagccaaagttttgggcttgaaatggggaaaaatcatggatgaacaagtttaaagaggagacaatctaagttctgtccagctacatgttttaacattcccagattgatgagatttactttaaaagtaccttcatgaaatttttctgaaactttattctacagcagttccaaaaacattccagacaaaagtgtgtcttattgtttcatataacagacatgaatctgatttcttccacaacttctgacatcttatccactagtgaattagcaaagttttgttagcctgcaggggtttctatgagggtttctcaccctcagcactactgacatttagatggggtactttggtttagggggctgttcagtacattatgggatgtttagcaccatctctggtccacaagatgccagccgcaactctcagttatgaaaaccaaaactgtttccagatatcaccaaatgtcctttgggagcaaaatcatccccagtttagaacccaactcatggtgctaatagtaacaaaactaacacttataaagcacttgttatagcccttttataatactaccagagccagtaggtaatgtttaaaatcttataaatcataaaaatagataaatgcctttaatttctattttaaatgtaattgtaaatccactcaacaattgatgttggaccacagccttttgagtatgaatccactggctggatttccaaattgccatggtacatgaagcattttctaccatttttagtttcaagtattttagtgggggaaaaactggattctgctttcatccttgctttctacatttgtccagtcttttagtttttttacccatacccaatttaaccactttttgactggggatgggttgaggggagcaactagctttttttttaaagtatttctaatgcattcaacctagctttcaaataaaaccagaagtcttttacactcacagtttatggactgctgaatatttaactaaattacataattaccctaagtaaaacaaacaggttcaatgaccactgccactagccttttgtaagcatgcagctgatcatctgttgggacaaaagcataaggttggttagagaatagcctcctagccagtcttctaccatgtgataagtaagtatgcctatcggctagttttactaggtaaaaattggttaagaggtattgtatgtgcgaaacaccatgtaaattactctacttgcattatctcttttaatcttcacaacaaccctaatacataattatgttaatgtttgtgttttgcctttgagaaaacaaacataaagataagtgttttacataaagttacatagctaataaaaggaccaggatgggaacctcaggcattctaatatgtgctttaccatttcatcacaagtccaaggccataaaggttaatttgctacagagcactaagctccagtttggtccatgatcacaaactgtaccttggaatcttgacctgtcatcttcaaactaagtgctacggcaataaaatatgggatattaatataaatctactacttggaacaattcaaaggattgataagaaagctcagtgattccaaatcatcaagtctatacatttaaagataacccaaatatacctgtattagtttcctatttatttgataacaaatcaacaaaagcttaatgccctaaaacaacaaaaatatattatctataggttagaagtttgacacaggtctcacagggccaaaaccaaggtgtcagcaggactgtgttcctttctggaggttccagggaagaatccatttccttaccttttctggcttctggagggcactcaattccttgacttgtgacccttcttccccctatcttcaaagccagtagttgcatctccctgaccattcatctgtagccacatcgccccgactctgaattttcctgcttccttcttccacttttcaaaacccttgtgatcacattgagctcacatggataatacaggctgatctccctacctcaataaaatgagccttagagccttggcacagctttgagccacagtcagttcctgttcagctacattaactgttttgtttttagtaggcgttttcaaaaggtgatgtgactcaaaggttgatttgtatgagaaatcagtcatgattgaattgcataactatctgtcctcaaagtccatgtaaa

SEQ ID NO: 16933 - RNA, 457 nt, Homo sapiens
  source 1..457: mol_type = other RNA
taggactgtgcttggcacatagcaggcacttccctcagttaggacgcgttgggcaacatgtaacagacaacctaacaacagtgctcaagcgatgagaaagtagaatgctctggcatcgccacacgtctggagagaagtggttgcagcttagtcagatgcgcagggatgttgacaaagacccaagcactttccctcttccatctttaccatccttggctatgtgggctttttgtccttagcttgttgcctcatggttgcaagatgactgctgcagctccaaacatcatgtctcacgctacagccggagcaggaagagcagggacccggaagcagtttgcctgggtttaaagtctggctccgtcacttctgagctgtgagatcttggaaaattcctaatcatctctgaactttggtatcttcattttcccaggccaggcgtggtggctcacgcctgtaa

SEQ ID NO: 16934 - RNA, 3221 nt, Homo sapiens
  source 1..3221: mol_type = other RNA
taggactgtgcttggcacatagtagagatttaataaatatttgttgaatgaataaatgaatgaagccccagtgcttagggcaggcgcctgtcatgtgataaatatttgttgaattaaacaaagctttaatgaatgagctagagaaaggtctgtgattcattcaaggttatgcagacagtgataacttgctttatctagatgcgaatccccgctaattctttctccaagccttcttcatttgtatacctcgtagcaaatccagcctgttgtaatgtcagaatgtctttgttcatcctttttggtacctgtaatcccagcactttcggaggtggaggcaggtagatcacaaggccaagatggtgcaaccctgtccctcaagcatctggagaagcttatactgctcagatctcaggaaccagggaggtcacgggggaaaagaccaaggacagtcgcaggcagcttcagcaaaagtagacccaacaataaaaatgatgtaagaagtgtattaagtatgtctttttattctgattcttcaacatcttggagtctagctgacgttgaaaggaactgcccctcccagggttatgaaattcctagagatagcaacttgcctgggagcctatctttcatacgcaaaccagccaatccaaagcccacacttctaccacctcctttatctggctcttatatgcagacccactatcccactgtcctaatcaccctaggccatgacaggataccagatgactagagacagcccctatgccccagatcctgctggaattattcaaactagccaatcctaaacctgcttactctgcctttcccttctcaataaaggttcttgtccacgatcccccctcactccttctttctcttgactcacccttctccatgttgccctacctagggtgctcctgttattaggtatctgtaagtataaaaacttattccttcatgactgtcttttctgcatgtcttaccatacctgattaaaacaaatcccaggtactcttatattaataaaaaggagccatcagggtttctaggatcatctcctctatccagatgacagccctctcttctctttttggacatgtttttcattttggtttggaaaggataatgtcttctgtgttctgagaagttactttttgcatttctctcctctctttctcatttattttatgtaaagccttattagctcccacaactttgtttgctctcttacttgataatggagaacataagagctaaagtcaagtggaggaaacaagttggtggtttctacatcctgcttcttataggacccggaagaggagcacctcttctatagcctgagctatctcaacagtgttctctatggctcatgctggtgactcagatttcttgtttagtttttaagttttactccccactcctgacaaacttttaatatttttaaaagcggttaaacaacgaggtactattatacacctataaggatggctaaaatccaaaaataactgacaataccatttgctgacaaggatcaacggaactttgtggaacaacaggagtctcattcattgctggtgtgaatttaaaacggttacagccactttggaagacagtttggcagtttcttagagttaaacatagcctcatcataggacccagcaatcatgttcgtaagtatttacttaaatgagttgagaacttatgtctacacaaaaatcagcatgagaattttatagcagttttatttacaactaccaaaaactagaagtaaactttagtaggtgaatggctaaataaactgtggcacatccacacaatggaatgagctgtcaaaccacaggaagacatagatgaatcttaaatgcatgttgctaagtgaaaaaagccagtcttaaaaggctacataaggtataattccatttaagtaatatcctggaaaaggcaaaactcttatggagatggcaaatagaccagtggtttcagaaactcttggtgaaaggaattgaataggtcaaccactagggattttttaaagggtggtaaaactatctttttatgatattgtgataatactagatacatgacactatgcacttgtcaaagcccatagaacttcatggcatagagaaacttaattatacaaaatttaaaaaatatttagaaggttggaggattccaggatgaaatgtaaaatatggcaaaataatctaactgtattacaaatgcatgaaataagcgtactgaaggggatgtgagagaaaatgcttacgtaagtaagtttggaaatgaatcgagtctgtaagattaaaggcaaaaagagctctgtataagcactcaaacttataaagttatttctatgtgggtatggcttaacaattatggaagtactctacaggagactggaattgaacaatgaaataaacgaatggctgatggcagaagccaggttcttcattgtaggagggagaggaaacaagcaagggggagaaggttagaattatctatgtgctactgggttgggattggagacatcagtatcaactcatatttagcttaatatagatacagatagttacaaagagaaggatttgtagatatatgtgtatagacatgggttaatttacacacatatatgttatttctctgtcagctgagcctagaagcaataacacctttgcaacaaggagcatgtccaggtcttggtttctaatacattctccaataaaagaaccaagctccttggagacatggactctaggatggagcaggaaatatacaagacgaacctagagcattttgtagctcctgaaagtaagaaagtgctcaaccaaatccaataatgacagggctatgttacagggacacaggagccaactgaatgtattctccatggccagggctggaacaacttgagcaacaaaataaaatagtattgaaagtgcaaaatagatatccatgagaccataatgatacaaacaaatgattgaataaataaatcaatgggggacaatagataaatctcccgggcagaagaagttcaaataatttctgtagatattttgccatcaaagagtggagtataaatcgctgcttcttaattgtgtgctatgccttgtggcttccttccagagtataatataaaaatgtggggaggtgcagtgggggagaagggctgtaatcctagcgcttgtggaagtcgaggtgggaggatcacttgaacc

SEQ ID NO: 16935 - RNA, 284 nt, Homo sapiens
  source 1..284: mol_type = other RNA
taggactgtgcttggcacatagtaggcattcaataaatatgctccttatctccatactacttcctgcttctaataccatcaggaaactatacagaaaatattaaaaaattaatctgggtagatgcctttagactttagatctaaagaatacttttaaataacttaatatccccatgctttctaaggaaaagctaaagtcactgccagagcatgaacatgttccagccagtacatgaacgcatactaaagtatctgttatctttcattgtcctccactgtttgga

SEQ ID NO: 16936 - RNA, 3741 nt, Homo sapiens
  source 1..3741: mol_type = other RNA
taggactgtgcttggcacatagtaggggcacagtgaactatatcagtgaatagatggatgcacagctggatggttgagtaatgaggatgtgtgacacatggaaggaggatggatggaagtctgatacaaggaaggatgacaagcaatcaatagaagatggatagatggatggatgaatggatggataattgatggatgatggatagatgaaggaatggatggatgatagataggtgtaaggataatggatggatagatgatgaatagatgaagaaatggataaagaataaatggataatgcagaaatggataatggatggatggatggttgatggataatgggcagatggagggatgaatggatgtgtggatgacggataatggatggatggatggttgatggataatgggcagatggagggatgaatggatgagtggatgatggataatggatagatggagggatgatggctgatgaatgatggataaaggatggatggatgatggatagatggatgaatggatagatagtggatggaaagatgatggatgatggatggaaggataaataatggataaatgaagaaatgcataatggttgaatggataagggatgaatggatgatggatagatggaggaatggataatggataaatagctaacgaatgggtggatggatgatgaatggatggatgaaagcatagacaatgaatggatagatgatggatggatggatggatggatggatgatggatggatggatgatggatagatagctgatgaataggtgggtggatgatgaatggatggatgaatggatagataatggatggacagatgatggatggatggatgggtggatggatggatgaaggatggatggatggatgatgaaggatggatggttgatggactatagatggataatagatgatgagtgggtggataatggattaatgatgatggagggatgaatgaaaaatggatgaatggacaatggacaatagctggatgagtgatagatgctggatggatggatggatggatagatgatggatagctgatgaatgagtggatggatggcaaatggatggatgaatggatagatgatggatggatggaaggatggatgaatgaatgaatgatggatggatgagtggaaagatgaattatgaatgatggatggatgatgaatgatggatggataatagatgatgaatgggtggataatagatggacgaatgatgaatggatggatggataatggataatggctggatgagtgatggatgatggatggaaggatggaaggataaaggagaagaatatattctacgtggggaaaagctctagaaattcttctgggaaggaataaggcctcttgggaaatgactgaacttggagtcaggagtcctgattcaaaccccatctctgccatttgctagctctgtaatcacaggcaagttacttcattcatctctgtgaccctaattttcctcctctttataataagaatctgtttctccaggcatctaagccctgggattttctgtaaaggtggtgctaggcacagggtaaagcctcctcagggtcagggtggtgtgatgttgctgagctctgaagagaaatgtggcttcttcaccctccctgcttagggcttgggtttgggggcccacttcttgctcgccccacatctcttgcttgcctggcccctgccttgcccactctctggaatacaaggcagccctgccagcctgtgtccagcctgggctctgtgctccctccctgccaccctgcagtgtctggccctggcctctgcacagtctctgctgtcaccttcagcctccttgaggagtaatggggtggggcaatgacagggcagccacagcccacagagcaactggcctccatacaccgcaagaaaacaagttcaacaagcatttattgagcccctgctgtgtgcctgctgtgtgacacccctgcagtgcctgcgccactgccccctccttcaggaagccactctctgccccccaaagggctctgcccctctgggcacctgactggcttgtgggtgccagccattcagtggccagtggccatgtgtctcctggcatcgcagctgtgcccagcagggctcatgtgatgatggcaagagtccggggctgctgtcccaaagtcactctgtgcagccctgtgcattcccttgggcctgccctggccccatttccaaggccatgggacccaggcagcgatgggcaggacaggcctggcatctcccacgcaggctgactgagttcacggcacacaggccagggttctgggggcaccactctggtggtcttgcagcaggggctggtgccagcgatggcctgaggtccgcgggccaggttgaggtcttggtcacacccagtgccccaagacccagcactgtcggttcagctctggtgcttcctgtgcggagctccggggccaggaatccgccatgtgtggctggtgtcgggcagggtatctctcgtggcggcagtctaagtgaaagtcctcctcgctcccgtccctcttctccatccagctgtgtgacctggggcaagtcgccctccctctctgtgcctcgatttgccacctctcccggaagtacttgatggcctcagggtctatgaaggtcggctcttcccggtagccctgctcaaagaccttgcgcttgtgccggaactcaatgaccgtcttggtgtaggagttgagcgtggtgacagaggctgccatgcagcaggtaaaggagccccacgccaggcagaaggaccacccgtagtcccaggaatggggtctccagtcctcaggaccgaggctcacggtgacctggaacacctgcgtgtacatcatgtgggcgaccattcccaggaggcctgagagcaccgtgaagacagccgcgaaggcattgagcttgagcccgtcgatgacattgctggagtggaagagctcgagacacatgaggctgaagccaaccaccagcagcagaatgtacagcacctcggagaccacagacagccacaggacccctttctccgatgccggggccaggtcaatgaagctgcgacatttttcaccaagcccgctgagctcctcctcgcacgagtaccagatgccggtgtggaaattcctgaagaggaagcggtcgtcgccggtctcccagctgtagagcgcgccgccaggggggccgttccccgaggcggtggcggcggcggcggcggcggcgggggcggcggtgccgttggccgtggcgttggcgcccgagttggggcagttggcgcgcccgccctggccgcagcccggcttggggacccgctgcgtgccctggcaccagtgcgtggtgaggaaagcggtggtggcgaacagcagcgccagcaggttcagggccacggccaggagcgctcggccgcggcggctagtcttcatgccgcccgcgccgccgggacgggactgcaccgccggggagctccgcgcgcgaagttggcagctggcgccccgcgtcagcggccgctgcccgccgcgccccggggctcgggtgcctgagatcggcggcggcggacgcggcgcgggcccatgccccccccaaccccggggtgggggcgcggcgcggggggcgtgcggggcgggctggcggggcgggcggcggtggaggagcggctacggcgcgcccggagcccggagcgcgagtgcacctcggctaggagccgctggcgcct

SEQ ID NO: 16937 - RNA, 3098 nt, Homo sapiens
  source 1..3098: mol_type = other RNA
taggactgtgcttggcacatagtaggggcacagtgaactatatcagtgaatagatggatgcacagctggatggttgagtaatgaggatgtgtgacacatggaaggaggatggatggaagtctgatacaaggaaggatgacaagcaatcaatagaagatggatagatggatggatgaatggatggataattgatggatgatggatagatgaaggaatggatggatgatagataggtgtaaggataatggatggatagatgatgaatagatgaagaaatggataaagaataaatggataatgcagaaatggataatggatggatggatggttgatggataatgggcagatggagggatgaatggatgtgtggatgacggataatggatggatggatggttgatggataatgggcagatggagggatgaatggatgagtggatgatggataatggatagatggagggatgatggctgatgaatgatggataaaggatggatggatgatggatagatggatgaatggatagatagtggatggaaagatgatggatgatggatggaaggataaataatggataaatgaagaaatgcataatggttgaatggataagggatgaatggatgatggatagatggaggaatggataatggataaatagctaacgaatgggtggatggatgatgaatggatggatgaaagcatagacaatgaatggatagatgatggatggatggatggatggatggatgatggatggatggatgatggatagatagctgatgaataggtgggtggatgatgaatggatggatgaatggatagataatggatggacagatgatggatggatggatgggtggatggatggatgaaggatggatggatggatgatgaaggatggatggttgatggactatagatggataatagatgatgagtgggtggataatggattaatgatgatggagggatgaatgaaaaatggatgaatggacaatggacaatagctggatgagtgatagatgctggatggatggatggatggatagatgatggatagctgatgaatgagtggatggatggcaaatggatggatgaatggatagatgatggatggatggaaggatggatgaatgaatgaatgatggatggatgagtggaaagatgaattatgaatgatggatggatgatgaatgatggatggataatagatgatgaatgggtggataatagatggacgaatgatgaatggatggatggataatggataatggctggatgagtgatggatgatggatggaaggatggaaggataaaggagaagaatatattctacgtggggaaaagctctagaaattcttctgggaaggaataaggcctcttgggaaatgactgaacttggagtcaggagtcctgattcaaaccccatctctgccatttgctagctctgtaatcacaggcaagttacttcattcatctctgtgaccctaattttcctcctctttataataagaatctgtttctccaggcatctaagccctgggattttctgtaaaggtggtgctaggcacagggtaaagcctcctcagggtcagggtggtgtgatgttgctgagctctgaagagaaatgtggcttcttcaccctccctgcttagggcttgggtttgggggcccacttcttgctcgccccacatctcttgcttgcctggcccctgccttgcccactctctggaatacaaggcagccctgccagcctgtgtccagcctgggctctgtgctccctccctgccaccctgcagtgtctggccctggcctctgcacagtctctgctgtcaccttcagcctccttgaggagtaatggggtggggcaatgacagggcagccacagcccacagagcaactggcctccatacaccgcaagaaaacaagttcaacaagcatttattgagcccctgctgtgtgcctgctgtgtgacacccctgcagtgcctgcgccactgccccctccttcaggaagccactctctgccccccaaagggctctgcccctctgggcacctgactggcttgtgggtgccagccattcagtggccagtggccatgtgtctcctggcatcgcagctgtgcccagcagggctcatgtgatgatggcaagagtccggggctgctgtcccaaagtcactctgtgcagccctgtgcattcccttgggcctgccctggccccatttccaaggccatgggacccaggcagcgatgggcaggacaggcctggcatctcccacgcaggctgactgagttcacggcacacaggccagggttctgggggcaccactctggtggtcttgcagcaggggctggtgccagcgatggcctgaggtccgcgggccaggttgaggtcttggtcacacccagtgccccaagacccagcactgtcggttcagctctggtgcttcctgtgcggagctccggggccaggaatccgccatgtgtggctggtgtcgggcagggtatctctcgtggcggcagtctaagtgaaagtcctcctcgctcccgtccctcttctccatcctctcccggaagtacttgatggcctcagggtctatgaaggtcggctcttcccggtagccctgctcaaagaccttgcgcttgtgccggaactcaatgaccgtcttggtgtaggagttgagcgtggtgacagaggctgccatgcagcaggtaaaggagccccacgccaggcagaaggaccacccgtagtcccaggaatggggtctccagtcctcaggaccgaggctcacggtgacctggaacacctgcgtgtacatcatgtgggcgaccattcccaggaggcctgagagcaccgtgaagacagccgcgaaggcattgagcttgagcccgtcgatgacattgctggagtggaagagctcgagacacatgaggctgaagccaaccaccagcagcagaatgtacagcacctcggagaccacagacagccacaggacccctcggagatgctgatgctcctatcgctgggtttccagcccctgttggtgctggcagggactgcccctcatcatggcgctgctcactgactcagctgcc

SEQ ID NO: 16938 - RNA, 3687 nt, Homo sapiens
  source 1..3687: mol_type = other RNA
taggactgtgcttggcacatagtaggggcacagtgaactatatcagtgaatagatggatgcacagctggatggttgagtaatgaggatgtgtgacacatggaaggaggatggatggaagtctgatacaaggaaggatgacaagcaatcaatagaagatggatagatggatggatgaatggatggataattgatggatgatggatagatgaaggaatggatggatgatagataggtgtaaggataatggatggatagatgatgaatagatgaagaaatggataaagaataaatggataatgcagaaatggataatggatggatggatggttgatggataatgggcagatggagggatgaatggatgtgtggatgacggataatggatggatggatggttgatggataatgggcagatggagggatgaatggatgagtggatgatggataatggatagatggagggatgatggctgatgaatgatggataaaggatggatggatgatggatagatggatgaatggatagatagtggatggaaagatgatggatgatggatggaaggataaataatggataaatgaagaaatgcataatggttgaatggataagggatgaatggatgatggatagatggaggaatggataatggataaatagctaacgaatgggtggatggatgatgaatggatggatgaaagcatagacaatgaatggatagatgatggatggatggatggatggatggatgatggatggatggatgatggatagatagctgatgaataggtgggtggatgatgaatggatggatgaatggatagataatggatggacagatgatggatggatggatgggtggatggatggatgaaggatggatggatggatgatgaaggatggatggttgatggactatagatggataatagatgatgagtgggtggataatggattaatgatgatggagggatgaatgaaaaatggatgaatggacaatggacaatagctggatgagtgatagatgctggatggatggatggatggatagatgatggatagctgatgaatgagtggatggatggcaaatggatggatgaatggatagatgatggatggatggaaggatggatgaatgaatgaatgatggatggatgagtggaaagatgaattatgaatgatggatggatgatgaatgatggatggataatagatgatgaatgggtggataatagatggacgaatgatgaatggatggatggataatggataatggctggatgagtgatggatgatggatggaaggatggaaggataaaggagaagaatatattctacgtggggaaaagctctagaaattcttctgggaaggaataaggcctcttgggaaatgactgaacttggagtcaggagtcctgattcaaaccccatctctgccatttgctagctctgtaatcacaggcaagttacttcattcatctctgtgaccctaattttcctcctctttataataagaatctgtttctccaggcatctaagccctgggattttctgtaaaggtggtgctaggcacagggtaaagcctcctcagggtcagggtggtgtgatgttgctgagctctgaagagaaatgtggcttcttcaccctccctgcttagggcttgggtttgggggcccacttcttgctcgccccacatctcttgcttgcctggcccctgccttgcccactctctggaatacaaggcagccctgccagcctgtgtccagcctgggctctgtgctccctccctgccaccctgcagtgtctggccctggcctctgcacagtctctgctgtcaccttcagcctccttgaggagtaatggggtggggcaatgacagggcagccacagcccacagagcaactggcctccatacaccgcaagaaaacaagttcaacaagcatttattgagcccctgctgtgtgcctgctgtgtgacacccctgcagtgcctgcgccactgccccctccttcaggaagccactctctgccccccaaagggctctgcccctctgggcacctgactggcttgtgggtgccagccattcagtggccagtggccatgtgtctcctggcatcgcagctgtgcccagcagggctcatgtgatgatggcaagagtccggggctgctgtcccaaagtcactctgtgcagccctgtgcattcccttgggcctgccctggccccatttccaaggccatgggacccaggcagcgatgggcaggacaggcctggcatctcccacgcaggctgactgagttcacggcacacaggccagggttctgggggcaccactctggtggtcttgcagcaggggctggtgccagcgatggcctgaggtccgcgggccaggttgaggtcttggtcacacccagtgccccaagacccagcactgtcggttcagctctggtgcttcctgtgcggagctccggggccaggaatccgccatgtgtggctggtgtcgggcagggtatctctcgtggcggcagtctaagtgaaagtcctcctcgctcccgtccctcttctccatcctctcccggaagtacttgatggcctcagggtctatgaaggtcggctcttcccggtagccctgctcaaagaccttgcgcttgtgccggaactcaatgaccgtcttggtgtaggagttgagcgtggtgacagaggctgccatgcagcaggtaaaggagccccacgccaggcagaaggaccacccgtagtcccaggaatggggtctccagtcctcaggaccgaggctcacggtgacctggaacacctgcgtgtacatcatgtgggcgaccattcccaggaggcctgagagcaccgtgaagacagccgcgaaggcattgagcttgagcccgtcgatgacattgctggagtggaagagctcgagacacatgaggctgaagccaaccaccagcagcagaatgtacagcacctcggagaccacagacagccacaggacccctttctccgatgccggggccaggtcaatgaagctgcgacatttttcaccaagcccgctgagctcctcctcgcacgagtaccagatgccggtgtggaaattcctgaagaggaagcggtcgtcgccggtctcccagctgtagagcgcgccgccaggggggccgttccccgaggcggtggcggcggcggcggcggcggcgggggcggcggtgccgttggccgtggcgttggcgcccgagttggggcagttggcgcgcccgccctggccgcagcccggcttggggacccgctgcgtgccctggcaccagtgcgtggtgaggaaagcggtggtggcgaacagcagcgccagcaggttcagggccacggccaggagcgctcggccgcggcggctagtcttcatgccgcccgcgccgccgggacgggactgcaccgccggggagctccgcgcgcgaagttggcagctggcgccccgcgtcagcggccgctgcccgccgcgccccggggctcgggtgcctgagatcggcggcggcggacgcggcgcgggcccatgccccccccaaccccggggtgggggcgcggcgcggggggcgtgcggggcgggctggcggggcgggcggcggtggaggagcggctacggcgcgcccggagcccggagcgcgagtgcacctcggctaggagccgctggcgcct

SEQ ID NO: 16939 - RNA, 3534 nt, Homo sapiens
  source 1..3534: mol_type = other RNA
taggactgtgcttggcacatagtaggggcacagtgaactatatcagtgaatagatggatgcacagctggatggttgagtaatgaggatgtgtgacacatggaaggaggatggatggaagtctgatacaaggaaggatgacaagcaatcaatagaagatggatagatggatggatgaatggatggataattgatggatgatggatagatgaaggaatggatggatgatagataggtgtaaggataatggatggatagatgatgaatagatgaagaaatggataaagaataaatggataatgcagaaatggataatggatggatggatggttgatggataatgggcagatggagggatgaatggatgtgtggatgacggataatggatggatggatggttgatggataatgggcagatggagggatgaatggatgagtggatgatggataatggatagatggagggatgatggctgatgaatgatggataaaggatggatggatgatggatagatggatgaatggatagatagtggatggaaagatgatggatgatggatggaaggataaataatggataaatgaagaaatgcataatggttgaatggataagggatgaatggatgatggatagatggaggaatggataatggataaatagctaacgaatgggtggatggatgatgaatggatggatgaaagcatagacaatgaatggatagatgatggatggatggatggatggatggatgatggatggatggatgatggatagatagctgatgaataggtgggtggatgatgaatggatggatgaatggatagataatggatggacagatgatggatggatggatgggtggatggatggatgaaggatggatggatggatgatgaaggatggatggttgatggactatagatggataatagatgatgagtgggtggataatggattaatgatgatggagggatgaatgaaaaatggatgaatggacaatggacaatagctggatgagtgatagatgctggatggatggatggatggatagatgatggatagctgatgaatgagtggatggatggcaaatggatggatgaatggatagatgatggatggatggaaggatggatgaatgaatgaatgatggatggatgagtggaaagatgaattatgaatgatggatggatgatgaatgatggatggataatagatgatgaatgggtggataatagatggacgaatgatgaatggatggatggataatggataatggctggatgagtgatggatgatggatggaaggatggaaggataaaggagaagaatatattctacgtggggaaaagctctagaaattcttctgggaaggaataaggcctcttgggaaatgactgaacttggagtcaggagtcctgattcaaaccccatctctgccatttgctagctctgtaatcacaggcaagttacttcattcatctctgtgaccctaattttcctcctctttataataagaatctgtttctccaggcatctaagccctgggattttctgtaaaggtggtgctaggcacagggtaaagcctcctcagggtcagggtggtgtgatgttgctgagctctgaagagaaatgtggcttcttcaccctccctgcttagggcttgggtttgggggcccacttcttgctcgccccacatctcttgcttgcctggcccctgccttgcccactctctggaatacaaggcagccctgccagcctgtgtccagcctgggctctgtgctccctccctgccaccctgcagtgtctggccctggcctctgcacagtctctgctgtcaccttcagcctccttgaggagtaatggggtggggcaatgacagggcagccacagcccacagagcaactggcctccatacaccgcaagaaaacaagttcaacaagcatttattgagcccctgctgtgtgcctgctgtgtgacacccctgcagtgcctgcgccactgccccctccttcaggaagccactctctgccccccaaagggctctgcccctctgggcacctgactggcttgtgggtgccagccattcagtggccagtggccatgtgtctcctggcatcgcagctgtgcccagcagggctcatgtgatgatggcaagagtccggggctgctgtcccaaagtcactctgtgcagccctgtgcattcccttgggcctgccctggccccatttccaaggccatgggacccaggcagcgatgggcaggacaggcctggcatctcccacgcaggctgactgagttcacggcacacaggccagggttctgggggcaccactctggtggtcttgcagcaggggctggtgccagcgatggcctgaggtccgcgggccaggttgaggtcttggtcacacccagtgccccaagacccagcactgtcggttcagctctggtgcttcctgtgcggagctccggggccaggaatccgccatgtgtggctggtgtcgggcagggtatctctcgtggcggcagtctaagtgaaagtcctcctcgctcccgtccctcttctccatcctctcccggaagtacttgatggcctcagggtctatgaaggtcggctcttcccggtagccctgctcaaagaccttgcgcttgtgccggaactcaatgaccgtcttggtgtaggagttgagcgtggtgacagaggctgccatgcagcaggtaaaggagccccacgccaggcagaaggaccacccgtagtcccaggaatggggtctccagtcctcaggaccgaggctcacggtgacctggaacacctgcgtgtacatcatgtgggcgaccattcccaggaggcctttctccgatgccggggccaggtcaatgaagctgcgacatttttcaccaagcccgctgagctcctcctcgcacgagtaccagatgccggtgtggaaattcctgaagaggaagcggtcgtcgccggtctcccagctgtagagcgcgccgccaggggggccgttccccgaggcggtggcggcggcggcggcggcggcgggggcggcggtgccgttggccgtggcgttggcgcccgagttggggcagttggcgcgcccgccctggccgcagcccggcttggggacccgctgcgtgccctggcaccagtgcgtggtgaggaaagcggtggtggcgaacagcagcgccagcaggttcagggccacggccaggagcgctcggccgcggcggctagtcttcatgccgcccgcgccgccgggacgggactgcaccgccggggagctccgcgcgcgaagttggcagctggcgccccgcgtcagcggccgctgcccgccgcgccccggggctcgggtgcctgagatcggcggcggcggacgcggcgcgggcccatgccccccccaaccccggggtgggggcgcggcgcggggggcgtgcggggcgggctggcggggcgggcggcggtggaggagcggctacggcgcgcccggagcccggagcgcgagtgcacctcggctaggagccgctggcgcct

SEQ ID NO: 16940 - RNA, 903 nt, Homo sapiens
  source 1..903: mol_type = other RNA
taggactgtgcttggcacatagtaggtagagcatttgttaaataagagaaaattttctttatttcactctcattacaatgctgtgaggactgtacagttatgctcctctgtagaggggaaactgaggctcacggaggtaaagtgtcttttctgaagatgcctcagagctgaatgtgggccttctgactctctatcccagttctcaccttgcgtctgcatccctctcccgcctgtgtaggtggcccttctcctcttccctgtgctgctgctctcttctgctaggagtgaatgccagaaagcagtcgccttgggtttctgataaggcttttgtgattgaggctgggatcccatgacccgccccccacttcttgtcattaggaagagcccagttccttaatccatgtacaggtagggtcagcacctgtgcatggtccacactgaaaaataaggatcagcatcagagaccttcttctccgctctctgcctcatcctctcttcctttttgttcctttcccttcgctgtcatttccattccccacccccaattgtacactaaacatgtacatgaatggtgcctagcttcctatgagtttatgacttatggttattcatcttaataactaagtggctttgccaggtaaaatattaaggcaccattgccattatgaccttgtcttccatgatctcattggcagctggtgttgccatgacaacttggctagaggaactggtatgagcttcagtggaaggcgatatgaacactggttgtgtgtgtgtgtgtgtgtgtatatgtgtgtaagagaatacagacttctcatcatgtgtatctgttgtgcagaaagccatgggtttccacaccttctgcttctccttccattttggtcaaaattagcctcagggatc

SEQ ID NO: 16941 - RNA, 1402 nt, Homo sapiens
  source 1..1402: mol_type = other RNA
taggactgtgcttggcacatagtgggcactcagtaaacctcggtgtcactgagaagacagaatgagaatgagcatgctgtggagtctttcacctgcctctcctctgggacaggttactctttcattctgtagactgtaatgacatggaaattccaagataccaagagacaatgatgaatcaaagatgagttcccaaaagacaaatcacatcccttattccccatcaaatctaaagcctaataaagtccatatagcactcatgaggcctctaaccttctgcctaaaagtgatcatcatcacagcaaacctgagcctcagaaaggacctagcttacttggtgacagaggagggcaacagaaggacttggcccatggcacccagctgaccatgtcagcaaatagagaggccttcaaagcctttgcattcctgttccctggagaaactgaggattgcagtaaagtgtaattacaacctctttttgccttgtttgaaatacaaagggacaatgtagccctaatatatttatagaaggaagtagagatcaaataaaggaagagggggaccaaaagaagggcatatccatgtttctcatcttctttcactgcagatcttaaaaaggaaccagaagcctcagcagtccctgctaaagaatcattgtcacattctattagttccctctgatcccgtgaagaggggggaaaaatcattgcatggcaatgccatgtgtctcaagcttcattaaagtgatttctcccaagagtctcgtataacagcatgtaaagcacttacaacagtacctgaatcatcgtaagtaatcaataaatgtaaacgagtagcagcagcagcaagagagacttgctgagatcattcatttagctacttggaaccctgcttagcatagaattcaagtcttttcacaatcaaatgagtgtttctcacaggaactcacactccttataccttcagagcctgagactctgccttctgtctccagtcttccaagctcttcagcagactgaaaaagttcttcaggatctactctctccaggtcctcaagcccacgatgacagagatatcccagctgaagaactgaatttcagaggtctgacactgacacaacccatggaattcagttctcaaagctgaggatacacatcggcttttcagagatggtgcaaagacccctccttgcagtccaggcctgtcccagccagcgagctcctaaaatttcattttattttatcatttccaattcagccgctgttctccccctcctcgttgtgctactgtctcctgtccatcctgtccaccctttggcatgccttccggcccagggtttaccactccaatcggccctgctggtgccatccaggaaaggaagagcggtcaagcgtcttggaga

SEQ ID NO: 16942 - RNA, 10205 nt, Homo sapiens
  source 1..10205: mol_type = other RNA
taggactgtgcttggcacatagtggtcctcaataaaaactgattgagttcatgaggggctgggatatttcatatgatgcttccctattttacttgtaaaatacattttgcattgaagaggtattataaatgaatgtggaagtgggtataaggaaaacaaacttatcttagcgctgggtagtatatacaggcactgcaattccagggtgtaatcctaagatccaagtgatctttgtttacaatgacacatgtactaagtgtggattcaaactggaggctctacattagccaggaatccatgcaaaatgtagacatttgatggccattggggaaaaaggtaatgtcccttggtgtggaggaaagtagccaattttggtaagtatgaaataatgttgttctagaaatatggagagaattctgtgataaaacctccaaagatgtttaaccacagttaccagtgattcaataagcattagaagagccgtctgtctttttctggttaagttctgccattctccttggtccttcatgtctccctagatctctggctatgagaagtcctaagacccagagtttaaaatcgtgcacagatagaagctgaggacaaagctactgtggtatagacttggacctcagtgtgagtgctcttgaccaggacatctaggcaagaagtccactgcatagaagcatccttctaaggctaatgggctggcgcaggcaagatccatgacctgtggctgaaagcagcagtcctgtcgttactcttctatgagtggattacagcaaggatttctgtgtgtcacaatctggtgaggtcagcttccttgaactggataggagtttttaatttaggagataatacattagctcaccagttttgaatacaggatctaatgggtcctgaaatcaataaggtggaaaacagatcagcagttcttgtgctggtagaggttatgggtcatccaggggtcctcccatttgtgatgattggtgcaggctatgactggatgcctggcttctccaggtattgctgccaagtttcaaacatggccttaatggccaagcattccttctttcagatattgtagtttcattctgcagggatgaagcctcttttgatggaacccgggagcctttcctcttgttccaccacgtctccagcatggctatgaagcaggagaggacaattccagcagccaggatacaaaagacccctgcaaagctctttatgtccagggcgcctcctttctgctttgtgtccactgacgagtacaggtcacactggccattcttaggccaccatttgtgcttcaggatgtccatgtcaccattctgctgaagctccaggatcctttgtgaaaaaacatctcggtaaggactgccatgttgtaatgcaattccatatccccgatcagcaacagtatttccaatggtgtaaaaggaacaatctgggtcattgatagccacatattccaatacagctgcatcccatacgaaagcataatttccatattttaccttttgaatgcctgcctgggactccagaacattgttctccgatccattgcttcggttgatcatccgccacatttgggaatacatgctgtccctctcaaaaggattcagtcctttcatgcggacatgctcatataccgcagagtctaggactgtgccataagggatttctgtttgcttggaaaggtcctggagagactggatggaactttcaatgcgtgtaatagtgaggaaagcagcgaggtttgccgtgtaagatgagataacaatcaaagcaaatagccaccaagcccccatcatcattcgggtagccagagtcgtgtacgggacttccccgccttgttgtacaaaagatccatacacaaaccacatggagttgtagagagtagtagacgtcattgatcccatttgtaatcgtgggggattaagccagttcaagaggtagaccagtagacccaccagaaggactgtgccagcaatgcaagcccatagagagagatcaaatggtgcaagacaggcaaacatatccactgtcttttcagcccttcgaagtagtacccccactgagtagtccatgtaacgtgtcgtaaagtccaccacattttcacgatctggagtgatggttaaagcagaaatccctatgtcggctctcttaaagacaagttctcctaccaagccattccatgtcccatcttcttgtgggcttccgtatttgtgatccggtgctacgtaaatttcgtagttaaaacccaggtagttagataaggcatccaaaacatcaatggagaagccctggtatttcttcggcttacccaagacattttcagagaccatcacaaaaggttcttccagaacagttactacacgtagaaccactccacgcatgttattctccaatttcttgtcagtcagtgacccattcagacctgtgacaggattccagcaaccaagctggggccagattttcccagtagagccctgtggtctgattctttcattttttcgaacacctctgccaagctcttctccatagttggttccaaggatttcaaagtggacattgggattgcctccattttctccaaattctagctctccagtcaacccactaactccacccttcttgatggtctccaacatggagcgcccaccctgccagggctttgagttctttctgatacatgacagacttgccatgctgtgccactttcggtcctccagcttcttatgaaaagcattagcaagcagaagcaccgtgtcatatatgtaaaggttggaaatctccatattctgagcaaatggatcctttggatcacacaatgttgaagatattcgatggttgccacggaaacaccgctgacttatgttctggggaactggaaatgtctgccgaataatcgttaaccttccaattgaccttcttacaagttcctgtacgtccacatcgtttatttcctcatttataatgatccagtgacagtcaaaagcaaccaaattagtctccacaacctcagtaatgaaggatttggctgtagcaggattcataacaaggatcgctcgcctaagagtgtctcgatagcgattcagttcttctattctcatggtgtcaaagagagtggtaatcattttattgatgttgttttctaccttctgaagtgcaacatccattccctgctgagagactttgtccaagaactcctgtattccacggatatcgtattcactatcatagaatataatgaatttctgccaggcatactctgtgaccactcttaggataacatcatgcaagtagacaggtgggcgaactgagagagtgtagtcatcattcctgttgctccgggtgagtccacagccactccttggggtcccagctgttgagcgctgaatgaagaggtgggggatatgcatggcgtctgccaaagactggagggatcctgctgacgtgcagccaatggagctgaccagggccaagatgccttgattcataagttcacaggttttttgtggcagggctgtggcaggactggctgtggtgtttgtccctctggtctctctgagtggcatcctcgttgctgcagtgacacctgacctcaccaccaccatgacagagcagaagaccctttgtgacactcttgaaggccacaatacctgagtaaccagatcgctactgccctggacatgatacagtccacctcttgagacaaaatcatcatcatgtggacattgaacagggacgaaaccaactatggcatcccacagcatgccctggagggtcatttccactttgtctatgacaaaatcatctcttcaggtggccactttttcctctcagcctcctgagatggaaacctgtgcttctgggatctgacaaagggcaccactatgagatgatctgtaggccataccaaggacgtgttgagtgtggccttctccattgacaacctgtagattgtctctagatcctgagataaaaccgtctagttatggttataaccctgagtatatacaaatacactgtccaggtggagagccactcagagtaggtgtcttatgtccacttctcacctaacggcagcaacactatcacctctgtagctgggacaagctggtcaaggtacggaatctggctaactgcaagctgaagatgaaccactttggccacacagtccatctgaacactgtgactgtctctccagatggatccctctgtgcttctggaggcaatgctggccatgccatgccatgccatgcgatctcaacaaaggcaagcaccttgatatgctatgtggtgggaatatcatcaatgccctgtgctttagcctcaactgctactggttctgcgctaccacaggcctcagcatcaagatctgggacttagaaggcaagaccaccatagaaattaagcaagaagttatcggaatctgcagcaaggcagagactccccattgcacctctctggtctgctgatggccagactgctggctacatagacaatctggtgcaagtgtggcaggtggccatcagcacctgctagatatttatggcagaactttaggtttctttcaactgactttctgatttaaaacaaaaaatcttcctactttaatcattattaacttccccagcagtgaaacataaagagatggggagaaagtatttaagtggctgttcatattatgaaacacagtttttgcttgagttgccggactgcttagcttgaggacaagttggaaatggaaaaaggaatcactgccttttggtcttgctatgtgtgttttattatgattgagagaatattacttaaaatagcttttatggtgccttattgagggggtgggctatatgcaggcagattccaacacaatttgtaagttgatcacagtagaatgatctggttttcttgtattacattaatgaatgtggaatgcttgtagaatcaaaaatattattttaaatttctgtttatgtaactccagggtattaactgaaatcaagatcaattacctagtaatatggtcaaatttaaatcttaaacacttttgagaaacttaaaaaaaacaaacagctacaaaaatactgtaacaaattcttacatagaatccatgattatcaatagaaacatttcatcattttaactttatctatgaaataaattaagcatgacagataaggttgtcaaccattttgttctctcttctaatcccattccctcattgccagaggcgctgaccatcctaattttggtgtgcttcttaatgtcgcattttgctccacatatttttgtattggaattatttacaagaagcactcattactttagaaataaacacaattttatgaaatatctggcctaaattatgttgaattaagccagttaaacatatcaattcaaaatatctacttttggagtatacctaaatttcaaattggctatatatatggttatttaaatgtatcaatttctttatcactgtgttaagtaaaaatcacaatatttatgcatacttccatgtataagttgtttataattagctgttttatcttaagtatatatattagagaagatgattatagtattgcttctaggttattttgttaatttgaaaatcagattagatttttagacatctaatttgatattatacagatacaagagaataggaattttgtacaatttaagattattaattataacatgataattttaatagatattgatttcagtaaaaattgaacctgaaattaatagaatgttgaagatacttgtatatacatcactgttgcctgaaatatcaaccgtagtacaaaaaatgcattctaaatagaactgaagaagtttatctgctgaaacgagactgcagaagacattatgccacccgctatttccagggtatttataggattctgacattctctaagctaaacactttctataaagttcattgcagccaagactactcacttctagtaagtaccataagcaaaccagaggttgcatagtgctgttttctttctttgttttcatttgctgctaacagtgttttgagtcattctgactttggtagagttaactctgcctgtttgatattttgagaatttttaggtttctgctatcttaactgtttctctgactttcagcttaaatctaaaggcattagagtgccctttagaatccctaagatctactcacatcgagttcacagcattgcactggtccttttgcctacatattaattcttagtttctagactttcaacatattccaaataagtatgtgtgtcataaaagaagcattacattcaaagttagaagggaaggattcttgtcatagccctctcccctaaaaaccaataaactttataaaactcattaattcccatgtctcagggctgtgggcagaaccaaatgagaagtgaatgtgaaagtctttaatatgcaaagcagagtatcttatgttgtcatttgtcagttctagattgtttcaagacagtgtctttcaaaaatgagattgtaaatggtactacgcaattggtagttaactcatcgaaattctattcatctgaaaaatatctgatgcttagtaaaagaaagcacattataattctcactattattcatatattatcaaaacaagacagacttttatcatttctcttcattatggagtactaataatttataagcttattgcaattaaaactgcttaataccaaagattacttaactgcaaacaagatatgaaaagaaaaaaaatattttaagcatctgagcaaaaaatatatctctaatttgtttttgtcacctatgctgtcgtagtaatatcctttcctgcagttggtagtcaaatatttccacaacatagtcctattatcatttttcaaatttattttttttaaatagtaagaatgaccattaattaaactgactccaaatactaagtattttacatgctttagtttatccccatcttacaggaaaatagagatttcaagaagtttagtaactagcccaagatcacatagttactgagtgaggctgtttgggttttatcctgcccatgtgattctaatattcctttttaaaccctattcactcttcatgccgcccccatacatgtgcccttcattttagtccagtggttctcagtactggctgcacattggaatcactcaggagcttaaaaacttctgatgccaggacccctctctcagcaattggggttgaatttgtctgtggtggagatttgtgatgatgtctgagcctaagttttaaaacctcccatgggtgattgtgatgtataaacagcactgagaatctcagatttggccaaaattatccactttctagataattctttgaatgatactatgctttcctattgccgtaacatttgctcatgctcatgctcatgctgggagtaaagttgcctagtttataaaacaagggctttggtgtaggacagaaataaatagttctgattcagtgcccattactaacctatcacagcattcaggtatatacagtgagaatgaagctcttgcaacataagcttcttcataaatatttaaaaatgagaaaaattatatgctatagaattattgtgaagggtatatcaagcagataaattacagatacaattatataatttgggcttcaagatattattcatgtagaaaacatgcttcaagtaagtattgcaaaagggtagttgtccataggcagaaattcattgagtatattcatatgtgtctgatataaacttcatgtttgcctcacacacccagaagagacatgaagtatgaaagagcacttccagaggggctgctctgggtgaggtaagagatttcaatggtatagcgactcatcaagttaatataagaaaggttcttctgacttcctcatatatttgccacttgcccatttacttaaaactaaattgaacagctaataagtttgcgagcaagatcatttccaagcaatacaccaaatcagactgttaactgtccattagtataggcaaaatagctcttattaagttgggccttcgttggtaatgccttttctcattctacctccacctgtcaaaattctccatcattatctttcaacacccatctcaaatgccatttttcttttttaatgtttcctgaatacaaagataatagctaatgacacttttagtctctcttgtatgggtgaagttgaatacaaaaaaaagaaggaatctgtattattcattcattcattcaaatgtaatttattgagaaatatacactgggcaagaggttatgatttttaaaatactgttattctgcttatcagtttataattaagtgggaataacagacataaagttcacagttgaagtttagtgtgacacctgagataatgtgacacctgagataacagaaacagttgtggatatagtgataacataaaagacaacatgatcatcaatatctcatatgtagatgtgtcacaaaaggtttcacacacatgaatatgattgaggtcagttttgcagcatcttttggataacatagtttttagcggcaaacatagcattggcctgactctaccacttataattctgtaaacttggacatgaaataaaactcctctgtatctgtttcctcactaaattgccatagaacttacattaaataatatgtgtaaaaaaattggcaaggctggacgcaagggctcacacctataatctcaacactttgagaggccaagggagaggatcacttgggccaaggagtttgagactagcatgggcaatatagtgagacaccatctctccaaaaaaaaaaagccaaatatctaacaacataaggcaagaagccatcaacaaatcccagtagttttgatacaaatcaattaaacattattataatggcattccagataaaatataagatttgaaaaaataaggaagcataaaaacaatctcaaggaattgtcagcaattctcataaaattaagcattagatatttatgaggagatatggccttatgagagatatggctagacaggtaggttaagactagaacttaaaggttttggtaaggtcatcctatggataaagtaatgtcatctaggataagtacaaactttatcctgaagaaaataggagtaaggtgtatggagagaatggtattaaaagttttgtagagaggaataatatgatccaattataattttttaaacccacagcaatgtagctgataaaagcggggataaaatgcagtgaaaaactaaatgaattaagccaaataagaaaaaaatatatagaattgctggtatttacagttaaagaaaattttaagggtgaatatgaggaaggaaacatactaaattgaattttaaaagacagattgaacatgacttagtggccagctggatgtgaatgtgagtagtgtagggttaatggtgactcctgggtccctgaattgtgtaactaggtgaaggtcattgaaggttttaaccatccaagatggttaaaacatgggactagattttaaagatagtagatgaagttctaagttacatgaagggcagctaggtagttatgtacaaagtaaaccttagaagagagagaagaattgcagatacatgcacactatatccctgtttttaaatttaacagtttttatttattgtaaagttatttctcctcaattttcaatacagcagagctttgtaagttgttaatgagtttaatcttttactaaatccacaaaaactctttcataaactagtactattagaatccccattttccagaagagttatgtaaactttaaacagtgaatgaaaaggtagaatttgaatctagaccacatgaatcaaatgccagaactcttttagtagcaaatatttacgcatcatttcttagaaaatacttaagatatttgtaatttttgtaattttagcatatttaaccttcatttgcaaacactcctcccttctccttgtggaaacctttaccaaactctgacatttattttgcctggctatataacagacaatcagtatacataaacctgaaaacaaggaaacatgcattaatgtatgagcaataataaggttttaatgtgaataaatttgaagacaaatgggttaaagtacattcggcataaatgggttaaggtacatctttagtaaaatgtactttttttttt

SEQ ID NO: 16943 - RNA, 1835 nt, Homo sapiens
  source 1..1835: mol_type = other RNA
taggatgggggtgagaggtggggagatgtggccgttcgctctgaagttgcgatgacttttgtgaacaagcaggttttcttgatgcaggtacagaagtgacggtggtggggtgatgacatgggagaattccagcaaaatccacctgggagaaccagcagctccactccacggacagagtggatctctgcggcacagcaacgcagcgaccccagcctggtccctcagcctgggaggcaggaaggagggattcttactggggcaggacggagggcgccccagatctgtggaagtggacgatctgccatttgccatcccggcggtgccagacacgggtctcctccgactgggcggtgcgtgggatgccgccagcgtccaggtactgcgtgatgcggatgtaggcgatgcaggctgactcgtcgcccatcaggtggatgtggggattcaggatggtggtgtgcacgggcttgctgttccgggaccacaggttttcaaaatagaatcgatggaagtccaggccctcaaccaggttccccagggcctcaggttcgaaggctgtcatgccagggtcgcacatcttcgtgtaggactcaaaatctccattgcttatggcttcaatcagctgctctgtcacttttataatttcctgtttccgcactttggtgtcttcatcctcgatggtggtgttggtgctctctgaggattccttcacaccatcgctcttcttgtttcccccactcttccctccggagaagttcctggtggccagcatcgtggtgagaatggctcccttcagtttcctcctggcattgaacttcttcaggcagtccacggtctcctgtctgtgcatgcaggatgccacggtggagcggtgcgagatccaggggtgcttaagggcttcggcagctgtgatgcgtttggatgggttaatggtcagcatcttattgatcagatccttggcttccggggtgacagtgtcccattccggcgatgggaaatcataggcgccggctttgatctgctggtacaggcggtgctggtcctcatcccagaacggggggtacccaaccagcaggatgtacaggatgaccccacaagcccacaggtccacaggcttcccgtacgggtccttccgcagcacttctggggagagatatccaggagtccctgcaaacccaaaccatgcctgctgctccccctccacctctatggccaggccaaagtctgccagcttcactgcggcacccttgagcttggaggccagcaacagattctcaggcttcaggtcccggtgcaccacccccatctggtggcagtgcagcacagcctccaggatctgctggatacagtgactggcatccgcctcactgtaatactcccgggccacgatatcttcaaacagttccccaccagtgaccaggtcgaagatcaggtagtggtgtccctcctctgagatgctgtcatgtagtcggacgatgttggggtgcttcagcaggcggcagatgcgggcttcacgctccagcttctgatggtctctggctgacagcttctttgtgttgatgatcttggcagcatactcctggccagccagcaccttcacacaccttcgcaccaccgagaaggctcccttgcccaattcctcgaagagctggtactcttccgtgaagcgggtgcaggtgatggtggccatcctggcgctgggcaggcaggtgaggcttgggactgggggaccaggactgaggcgctgctgctctgctcccgaacctagggaccacttgcctgcccgtgctgccgagtgcaaacagagaaccggtttgactgacgagcccggggcttct

SEQ ID NO: 16944 - RNA, 1839 nt, Homo sapiens
  source 1..1839: mol_type = other RNA
taggatgggggtgagaggtggggagatgtggccgttcgctctgaagttgcgatgacttttgtgaacaagcaggttttcttgatgcaggtacagaagtgacggtggtggggtgatgacatgggagaattccagcaaaatccacctgggagaaccagcagctccactccacggacagagtggatctctgcggcacagcaacgcagcgaccccagcctggtccctcagtggggcaggacggagggcgccccagatctgtggaagtggacgatctgccatttgccatcccggcggtgccagacacgggtctcctccgactgggcggtgcgtgggatgccgccagcgtccaggtactgcgtgatgcggatgtaggcgatgcaggctgactcgtcgcccatcaggtggatgtggggattcaggatggtggtgtgcacgggcttgctgttccgggaccacaggttttcaaaatagaatcgatggaagtccaggccctcaaccaggttccccagggcctcaggttcgaaggctgtcatgccagggtcgcacatcttcgtgtaggactcaaaatctccattgcttatggcttcaatcagctgctctgtcacttttataatttcctgtttccgcactttggtgtcttcatcctcgatggtggtgttggtgctctctgaggattccattaactgaacgctggaactggactttcttttcttcacaccatcgctcttcttgtttcccccactcttccctccggagaagttcctggtggccagcatcgtggtgagaatggctcccttcagtttcctcctggcattgaacttcttcaggcagtccacggtctcctgtctgtgcatgcaggatgccacggtggagcggtgcgagatccaggggtgcttaagggcttcggcagctgtgatgcgtttggatgggttaatggtcagcatcttattgatcagatccttggcttccggggtgacagtgtcccattccggcgatgggaaatcataggcgccggctttgatctgctggtacaggcggtgctggtcctcatcccagaacggggggtacccaaccagcaggatgtacaggatgaccccacaagcccacaggtccacaggcttcccgtacgggtccttccgcagcacttctggggagagatatccaggagtccctgcaaacccaaaccatgcctgctgctccccctccacctctatggccaggccaaagtctgccagcttcactgcggcacccttgagcttggaggccagcaacagattctcaggcttcaggtcccggtgcaccacccccatctggtggcagtgcagcacagcctccaggatctgctggatacagtgactggcatccgcctcactgtaatactcccgggccacgatatcttcaaacagttccccaccagtgaccaggtcgaagatcaggtagtggtgtccctcctctgagatgctgtcatgtagtcggacgatgttggggtgcttcagcaggcggcagatgcgggcttcacgctccagcttctgatggtctctggctgacagcttctttgtgttgatgatcttggcagcatactcctggccagccagcaccttcacacaccttcgcaccaccgagaaggctcccttgcccaattcctcgaagagctggtactcttccgtgaagcgggtgcaggtgatggtggccatcctggcgctgggcaggcaggtgaggcttgggactgggggaccaggactgaggcgctgctgctctgctcccgaacctagggaccacttgcctgcccgtgctgccgagtgcaaacagagaaccggtttgactgacgagcccggggcttct

SEQ ID NO: 16945 - RNA, 2025 nt, Homo sapiens
  source 1..2025: mol_type = other RNA
taggatgggggtgagaggtggggagatgtggccgttcgctctgaagttgcgatgacttttgtgaacaagcaggttttcttgatgcaggtacagaagtgacggtggtggggtgatgacatgggagaattccagcaaaatccacctgggagaaccagcagctccactccacggacagagtggatctctgcggcacagcaacgcagcgaccccagcctggtccctcagtggggcaggacggagggcgccccagatctgtggaagtggacgatctgccatttgccatcccggcggtgccagacacgggtctcctccgactgggcggtgcgtgggatgccgccagcgtccaggtactgcgtgatgcggatgtaggcgatgcaggctgactcgtcgcccatcaggtggatgtggggattcaggatggtggtgtgcacgggcttgctgttccgggaccacaggttttcaaaatagaatcgatggaagtccaggccctcaaccaggttccccagggcctcaggttcgaaggctgtcatgccagggtcgcacatcttcgtgtaggactcaaaatctccattgcttatggcttcaatcagctgctctgtcacttttataatttcctgtttccgcactttggtgtcttcatcctcgatggtggtgttggtgctctctgaggattccattaactgaacgctggaactggactttcttttcttcacaccatcgctcttcttgtttcccccactcttccctccggagaagttcctggtggccagcatcgtggtgagaatggctcccttcagtttcctcctggcattgaacttcttcaggcagtccacggtctcctgtctgtgcatgcaggatgccacggtggagcggtgcgagatccaggggtgcttaagggcttcggcagctgtgatgcgtttggatgggttaatggtcagcatcttattgatcagatccttggcttccggggtgacagtgtcccattccggcgatgggaaatcataggcgccggctttgatctgctggtacaggcggtgctggtcctcatcccagaacggggggtacccaaccagcaggatgtacaggatgaccccacaagcccacaggtccacaggcttcccgtacgggtccttccgcagcacttctggggagagatatccaggagtccctgcaaacccaaaccatgcctgctgctccccctccacctctatggccaggccaaagtctgccagcttcactgcggcacccttgagcttggaggccagcaacagattctcaggcttcaggtcccggtgcaccacccccatctggtggcagtgcagcacagcctccaggatctgctggatacagtgactggcatccgcctcactgtaatactcccgggccacgatatcttcaaacagttccccaccagtgaccaggtcgaagatcaggtagtggtgtccctcctctgagatgctgtcatgtagtcggacgatgttggggtgcttcagcaggcggcagatgcgggcttcacgctccagcttctgatggtctctggctgacagcttctttgtgttgatgatcttggcagcatactcctggccagccagcaccttcacacaccttcgcaccaccgagaaggctcccttgcccaattcctcgaagagctggtactcttccgtgaagcgggtgcaggtgatggtggccatcctggcgctgggcaggcaggtgaggcttgggactgggggaccaggactgaggcgctgctgctctgctcccgaacctagggaccacttgcctgcccgtgctgccttccactgcgaaacctgctctcggacgccctgaccataccgcacacaatactgcaagcctgtgtgggcctgggggtgggatggacccagcacccctggggtgatggacccaaggagggcctggaggaggtggaatagagcaaactttgtccacaagtgatcttttctcttcccacctcccccacctccaactgtggggcccttgtagcagacgggatgggattaagtgggg

SEQ ID NO: 16946 - RNA, 1806 nt, Homo sapiens
  source 1..1806: mol_type = other RNA
taggatgggggtgagaggtggggagatgtggccgttcgctctgaagttgcgatgacttttgtgaacaagcaggttttcttgatgcaggtacagaagtgacggtggtggggtgatgacatgggagaattccagcaaaatccacctgggagaaccagcagctccactccacggacagagtggatctctgcggcacagcaacgcagcgaccccagcctggtccctcagtggggcaggacggagggcgccccagatctgtggaagtggacgatctgccatttgccatcccggcggtgccagacacgggtctcctccgactgggcggtgcgtgggatgccgccagcgtccaggtactgcgtgatgcggatgtaggcgatgcaggctgactcgtcgcccatcaggtggatgtggggattcaggatggtggtgtgcacgggcttgctgttccgggaccacaggttttcaaaatagaatcgatggaagtccaggccctcaaccaggttccccagggcctcaggttcgaaggctgtcatgccagggtcgcacatcttcgtgtaggactcaaaatctccattgcttatggcttcaatcagctgctctgtcacttttataatttcctgtttccgcactttggtgtcttcatcctcgatggtggtgttggtgctctctgaggattccttcacaccatcgctcttcttgtttcccccactcttccctccggagaagttcctggtggccagcatcgtggtgagaatggctcccttcagtttcctcctggcattgaacttcttcaggcagtccacggtctcctgtctgtgcatgcaggatgccacggtggagcggtgcgagatccaggggtgcttaagggcttcggcagctgtgatgcgtttggatgggttaatggtcagcatcttattgatcagatccttggcttccggggtgacagtgtcccattccggcgatgggaaatcataggcgccggctttgatctgctggtacaggcggtgctggtcctcatcccagaacggggggtacccaaccagcaggatgtacaggatgaccccacaagcccacaggtccacaggcttcccgtacgggtccttccgcagcacttctggggagagatatccaggagtccctgcaaacccaaaccatgcctgctgctccccctccacctctatggccaggccaaagtctgccagcttcactgcggcacccttgagcttggaggccagcaacagattctcaggcttcaggtcccggtgcaccacccccatctggtggcagtgcagcacagcctccaggatctgctggatacagtgactggcatccgcctcactgtaatactcccgggccacgatatcttcaaacagttccccaccagtgaccaggtcgaagatcaggtagtggtgtccctcctctgagatgctgtcatgtagtcggacgatgttggggtgcttcagcaggcggcagatgcgggcttcacgctccagcttctgatggtctctggctgacagcttctttgtgttgatgatcttggcagcatactcctggccagccagcaccttcacacaccttcgcaccaccgagaaggctcccttgcccaattcctcgaagagctggtactcttccgtgaagcgggtgcaggtgatggtggccatcctggcgctgggcaggcaggtgaggcttgggactgggggaccaggactgaggcgctgctgctctgctcccgaacctagggaccacttgcctgcccgtgctgccgagtgcaaacagagaaccggtttgactgacgagcccggggcttct

SEQ ID NO: 16947 - RNA, 1992 nt, Homo sapiens
  source 1..1992: mol_type = other RNA
taggatgggggtgagaggtggggagatgtggccgttcgctctgaagttgcgatgacttttgtgaacaagcaggttttcttgatgcaggtacagaagtgacggtggtggggtgatgacatgggagaattccagcaaaatccacctgggagaaccagcagctccactccacggacagagtggatctctgcggcacagcaacgcagcgaccccagcctggtccctcagtggggcaggacggagggcgccccagatctgtggaagtggacgatctgccatttgccatcccggcggtgccagacacgggtctcctccgactgggcggtgcgtgggatgccgccagcgtccaggtactgcgtgatgcggatgtaggcgatgcaggctgactcgtcgcccatcaggtggatgtggggattcaggatggtggtgtgcacgggcttgctgttccgggaccacaggttttcaaaatagaatcgatggaagtccaggccctcaaccaggttccccagggcctcaggttcgaaggctgtcatgccagggtcgcacatcttcgtgtaggactcaaaatctccattgcttatggcttcaatcagctgctctgtcacttttataatttcctgtttccgcactttggtgtcttcatcctcgatggtggtgttggtgctctctgaggattccttcacaccatcgctcttcttgtttcccccactcttccctccggagaagttcctggtggccagcatcgtggtgagaatggctcccttcagtttcctcctggcattgaacttcttcaggcagtccacggtctcctgtctgtgcatgcaggatgccacggtggagcggtgcgagatccaggggtgcttaagggcttcggcagctgtgatgcgtttggatgggttaatggtcagcatcttattgatcagatccttggcttccggggtgacagtgtcccattccggcgatgggaaatcataggcgccggctttgatctgctggtacaggcggtgctggtcctcatcccagaacggggggtacccaaccagcaggatgtacaggatgaccccacaagcccacaggtccacaggcttcccgtacgggtccttccgcagcacttctggggagagatatccaggagtccctgcaaacccaaaccatgcctgctgctccccctccacctctatggccaggccaaagtctgccagcttcactgcggcacccttgagcttggaggccagcaacagattctcaggcttcaggtcccggtgcaccacccccatctggtggcagtgcagcacagcctccaggatctgctggatacagtgactggcatccgcctcactgtaatactcccgggccacgatatcttcaaacagttccccaccagtgaccaggtcgaagatcaggtagtggtgtccctcctctgagatgctgtcatgtagtcggacgatgttggggtgcttcagcaggcggcagatgcgggcttcacgctccagcttctgatggtctctggctgacagcttctttgtgttgatgatcttggcagcatactcctggccagccagcaccttcacacaccttcgcaccaccgagaaggctcccttgcccaattcctcgaagagctggtactcttccgtgaagcgggtgcaggtgatggtggccatcctggcgctgggcaggcaggtgaggcttgggactgggggaccaggactgaggcgctgctgctctgctcccgaacctagggaccacttgcctgcccgtgctgccttccactgcgaaacctgctctcggacgccctgaccataccgcacacaatactgcaagcctgtgtgggcctgggggtgggatggacccagcacccctggggtgatggacccaaggagggcctggaggaggtggaatagagcaaactttgtccacaagtgatcttttctcttcccacctcccccacctccaactgtggggcccttgtagcagacgggatgggattaagtgggg

SEQ ID NO: 16948 - RNA, 63 nt, Homo sapiens
  source 1..63: mol_type = other RNA
taggccacagccacccatgtgtagccacccctacacatgggtggctgtggcctaaacactgcc

SEQ ID NO: 16949 - RNA, 58 nt, Homo sapiens
  source 1..58: mol_type = other RNA
taggccacagccacccatgtgtgtaccatcctaccctggccgaggcccttgggaacac

SEQ ID NO: 16950 - RNA, 244 nt, Homo sapiens
  source 1..244: mol_type = other RNA
taggccacagccacccatgtgttcttgcactgatgtgctcctctcgacgtccaacctcctgtgtgtctgcctgtctcccgtaggtctcagtccaggttctgctatgcctttctcctggtgagccacctatttaagagtcgctgtgtcctgtaggtctcagtccaagatctgctctgactcccttgtggtgagttagccctttagaagtcacttggggtggggcatatgttaattccactaacat

SEQ ID NO: 16951 - RNA, 6953 nt, Homo sapiens
  source 1..6953: mol_type = other RNA
taggcctttagatcacttaaactacagataaaattagatgtgtagcacatatttctaaaatattgtccatattttttccattttaaataaaggtattaaggaattcgtgacaatgtaaaaaactactctatgcacttagaaaaattgtgaattcgaaaagttggagaataatttttgctaaataaataatcatttggcagtaagttctattctacctaaaataatttgcttgaaatgctgtaacagctacttcttatcaaggaataaagacaggcatcacatcctggtcaaacatgcaaaaccactcccaccccaccccatcctaaaactaaagaaaccttaggctgtcacacgtgaaagtgttatgacatatatatatacacacacgtatatatatgaagagtcttgatttggtagtgagcaatttcatttaaacctatcgtttgcttttggcacactaaaaaattcagatccttatgtagtgtttagaaaaccataaccagacaccgattgtgtgtacgtatgcacatcctggttttatgggcagggtgccttcgtgacctcttacacctggagctactgcactggtgcgtatgggagtaactactttcatgttaagttttccctgacattttgcctaaaggaaaagtttaaggacattaatttcaccaacttcttgactgaaagctcagctttcaactgttttgtcaaatagtttcaatcaatcaactgactctagaattttactattcttggaatttggtagtttcatgtttaatattgtaacctgtataaaaatgaaatctgtaatgttattttcgccttttaaaacttttttacatttcctacataaaaggcagcaatgacataattatacataaagtacccttaactgaaaatgagatgaggctgcattcataggcttcagagaatagtaaattgcatagaaattcatcaatttaagttacatggtaccatgacaacttgtatattagcagcttgacagacagcttcgaattttcacagactactacatgaactgttatggcaacggaaacttttacaaatagtagcatgttaaaagacctgtccacctaacagtacactacccaccgctcccatcagagacatgacacggtttgtttacatgatccaaatgaccatctcaatggtgattcgctgttatcactcacatcagctaacactactctgtgtatttatatgtgtgtatacatatttatgaaatgagaatacctggacagtctgattggttaacagcgtattggtacagttttgtcttctattacatgtcattcatttcagccctcaattttagaactctaaataaataaaatgtaatttacaaagataaattgttatttacaaatgcaaaaattcatcctgaggattttggtatctaggagaactgtttcacagaaaaaagcaagtatcaatctgtgaaataaaaatgcaccttgagttaaactaaataattcataattacaggttaatttacccaagttccagccaagaaaagcatgaagatatttaagaaatcttaaattgatttgcatgcaagaaattaatcacatacaacttttcaaatcccaatgttattcccccttaaacttcttgtttaatgttttagtctgactgtatttgtaaagtaggtgacagagaaaaaaatacctgaggaaagctcagtaacgtgctgagggttcttttcctcactggaaagcagcggggcttcaggccaccatgagaaacagccagtgggcctttgactttacccaagttaagctcccctaataggagtagttagctaaacaagttcaacgctttccaaaggaaaaaggtcaagttaaaacaaaaatctaaataaaggtaaaatatcaacagtttctctgctttacaatgtgaccataaaattacttatttacagaaattaaaagaaatggttcaacaaagaatcaaactggtttctccaggtatataccatgacaatgtatctttttactcgatgctgtgagcagacagtgattattttggagaaggaaaaataaggtgtggaattagtaatgcagatgctgaaaggcaagtggcaagagaagaatgcctcaaacaaaggctactttgttcccatctctactgcacctacacccacacccgccccggcccccaagctaaaagaccagaataaccaaagccattttaacagtagtgtgcaaaactgtcagctgacaaacaacataaaaacaagtcacactatgttatctgtggtcacgttcttcagggttagtccagtaactcaagactttacattcttttgtctttatttgtttattttaattaaacatataaaggttaataaacagacaaagtccagagttagtaggttggtattataacatttattaaaataatgctgtgggttaatagaaacagcaaagaaccaaagaattaaaatgcaagctatgtaaaatcccaactaaaacccaaaagtgtctaatgtattcattcattagctaactaaaagcccaaaaaagacaagacacccaatataataaagtactgcaaaacaattggcaattttcagttatcaaaattgtggattttgcattttgtatccttttctcaatcaagaaaaaaattctttttgaatgttatataacatacatataaaacaagatagaaaaatacattataaacttgtaacaatggctgtaaatacattatcttacatgtttctcataggcaataggttggttatggtacatacatagcatgaaactaagataataaagaatagacaaaaatacatgtcagctgtacgataacatacaagcgacactcccatctacccacgctaaaaaattacataatactgtcagaaaaaaagtcttaaaaactacatattttaataagaaataaattcaataaagaatgataatactgagaaccaaggcattcagagatttcaaaagtcatgcttttttcagttgatccaaaattttgtcaaccaagttttcaaaagtttgttcagagccaacattccctataaatgtcacacatttattatttcatacatttactttcttccccataaaagacctttgataaacatctaaaatgtccaggtataacatagttgagatgaaactggatcaaatactggtattgtttttaacaactatcacctcaagtgtttgagtgtcgcaaatttattcaaccaaccaaacaatataaaaatcaaaatggcacagcatatattgtaaataaatcaaaactgtatgtgtaacagaaagacaaagcagtggcatattaaaccaaagctagctggatacaaaacaatgaatgtctattgcatagtaaataaactgacaacggtttccaagtgagacaagatggtgggggaggtcaccaagaaggtaatgactcagcttcctgctgacctctgactgtgatgctgggaaggtgtggaagaggggacgagttgataagctgggcgggggggggggtccactgtcacttgagatttgccacgtctggtactgagcagttaatgattattcactcaagtgtttagatgtaggctttgcacacaaattgcttcaactacataactaactgtttcaacttcttgagaaattagaagcttaagctgaaatgtggttgagtatttatatgcactatgatgctagtttttcacattcttttaaagttaaggggtgggggaggcagaggttattgaaacagtaaaaggatacactacaccagttatctggtatgatataaagacatgtgattaaatttgggtgatttaaaacattgttttctagaatgaaaatcacaaagattcacttttgtgaaaacatttgctaggtatcctattatattcaattaattaaaaacaaaaaacaaaatcaaatgaatgcatcccccttctccaaataaaacaaagctctaattttgtctgtaaactgaagtttagatgacacataatttttatctcagaatcctttgggttaacattgaagattggaataaccaaaagtattaaactattcttttaaagaatgatgttttaaaacttactagtcaggcattagaaaagttatcaaatcttttcacagtatcagatttggcaaatttgcatcaaggtaacgtggcaaaaatcctataattcaaactatcaactcatttgtctccctcatatcttctttcacatactgggcgactgagtaacatgcattaacttgtattctgagggaggagctgatctttatgagacacttgactgaatgaccatgaaggaaaataaggcactttcttttctttagacttattccaatacttaaaaaataaaaaagaaagacaaaaaggctcttttggtcttttgtttcttgacaaccaccagaaaaaatcatttaatgaaataaagggtttctttgttctttttctttttttttataacacttgaaagtataaaatgctacatttccaaaaatatatatatttttttctgcaccagcacccttgtatagtaaaagtatctactttttgttcatttgtttcaatgcactacactttatctacaatttcattacatgtatacagcaaataggcaagcatggcttttacatccttaatgatttttttctatacagggaggtttaaaaaaaaatacttgaacagtttgcccagtaatgtgacacataatgcatgtaccttgttctcatatttttttaggtgtaaaataaagattcagtaattttaactcagatatttatctttttaaaaatagtgttgcagttttgttatttgcattacttttcaaaactccttaagtttttctctcatggcacactttcttctaatacttcaaattttggcaggcaatataaaaaaggctgcaacttctgccctttgagggcactgtagtgactaaacagcatatcaaattttgaatactttttgaaatcacttcaccaatgatatccctgaccgaaggttcatgcatgatgcatcatcacacagtacattcagagagagctttgacttcgctatgagaagaaaaagattcctagaagtctctcacagtaactgcctctgtcattgagtagttaaggaccatctgtctccccttcttaagagaggccttcttaccgttcgcttagggtgggatattaaaagatgatcagtgctgtgggatgaattgggccttattgctttactactattcagtgcagtttctagaaccactttcacccaaacaggaaaaaaaaaaaaaaaaagctgagttggaggacaacaatttctttgtcttttgtttggttagatggtaagacgaacggacaagtgcctcagctcgctgcactgacgacaggcaagcaaaggcgattaccagttaactgatcagcaggcaggcatggtcaggtcatcattgggtgaagagttcagaggtcagaaggtcataggttagttgccggtggcggctcggtctgcggtcacaatcctttggtaaggatggacacgcatatcgtgccttcgaactttagtagccaccgcacctaatacaccactaggttcaataggatactcaaggattgatgtagctggtgccaatgtgtaggggtactcatagggtgtatagattaaaccagcttcgggccctggaggaactattgcagcagttgggtgaggagttccgtttggcatgacagcggtctgtatttgtctgatcaaaggcattatggtagggccagctggcgtaggagtacgcagggcagctggtgggagaaccggcgcaggcccagtaatgatccttggagcagcctgggctgttgctgcaagagaaaaggcaagggctggtgatttaatgttggcatctctgtaggtgccattcagaatcgcaagctccatcagctgcatcttcttcaggctgtcttctccttctgccttttttttatccctcattgagcctttgcctcggaccatgattttacatccggtttctgcttcaagttgtttggctgtaagtcctctaggtccaaggattctcccaacaaaattaaaatctgggtattcttttacaggcacataaagtttctcttgtaactgaacaataggtcccacagcatcaggcaattctgcactccttttctctgtactgccatttaatgtgtcattgtacatgtctttccgtactctgctaatttcttcgtccagcagccgctcgaggtggttgaagatcccgcagaagttgggcaggctgctcatgagcttcttgtcgttcatcagctgcatcaggtaatctggggtgggcttcggcttctccttcgtttccatttccccgaccatattccaggctccgcagctcactccgcccgccgccgccgccgccgccgccggagaggagggaggggcgggggcgagccccggccgcgggccgctcgggacccggcgtcccgctccgcgccggctcccgctctggctcccgcgccgagccccggggcggccggcaccgcgcgctcgcccgccccccgcaggcactttccgcccgggcccgacgcgctcccagccgccgccgctctcggccgcccggctcggcgcgtccctcacgaggccggcgggcgggcgggaggcgggtctcggctggccgagtgcgggcgcggggcgcgggctgctggcgccggacgaggaggagccggggccgccgctcgctcggctggtcgagcccgctcagcgccgccgccgcctgtgccgcgggctcggggggtctctctgggctggtccccgccgcggcgcctctgccgctgccgccgcgctccgactgcgctcctcctcttcctcctcctccttctcctcctcctcctcctcactcacttggcggcggagttcgcctcagttcaggcggcgctgccagcggcggcggcagcagcggcggcggcggg

SEQ ID NO: 16952 - RNA, 6980 nt, Homo sapiens
  source 1..6980: mol_type = other RNA
taggcctttagatcacttaaactacagataaaattagatgtgtagcacatatttctaaaatattgtccatattttttccattttaaataaaggtattaaggaattcgtgacaatgtaaaaaactactctatgcacttagaaaaattgtgaattcgaaaagttggagaataatttttgctaaataaataatcatttggcagtaagttctattctacctaaaataatttgcttgaaatgctgtaacagctacttcttatcaaggaataaagacaggcatcacatcctggtcaaacatgcaaaaccactcccaccccaccccatcctaaaactaaagaaaccttaggctgtcacacgtgaaagtgttatgacatatatatatacacacacgtatatatatgaagagtcttgatttggtagtgagcaatttcatttaaacctatcgtttgcttttggcacactaaaaaattcagatccttatgtagtgtttagaaaaccataaccagacaccgattgtgtgtacgtatgcacatcctggttttatgggcagggtgccttcgtgacctcttacacctggagctactgcactggtgcgtatgggagtaactactttcatgttaagttttccctgacattttgcctaaaggaaaagtttaaggacattaatttcaccaacttcttgactgaaagctcagctttcaactgttttgtcaaatagtttcaatcaatcaactgactctagaattttactattcttggaatttggtagtttcatgtttaatattgtaacctgtataaaaatgaaatctgtaatgttattttcgccttttaaaacttttttacatttcctacataaaaggcagcaatgacataattatacataaagtacccttaactgaaaatgagatgaggctgcattcataggcttcagagaatagtaaattgcatagaaattcatcaatttaagttacatggtaccatgacaacttgtatattagcagcttgacagacagcttcgaattttcacagactactacatgaactgttatggcaacggaaacttttacaaatagtagcatgttaaaagacctgtccacctaacagtacactacccaccgctcccatcagagacatgacacggtttgtttacatgatccaaatgaccatctcaatggtgattcgctgttatcactcacatcagctaacactactctgtgtatttatatgtgtgtatacatatttatgaaatgagaatacctggacagtctgattggttaacagcgtattggtacagttttgtcttctattacatgtcattcatttcagccctcaattttagaactctaaataaataaaatgtaatttacaaagataaattgttatttacaaatgcaaaaattcatcctgaggattttggtatctaggagaactgtttcacagaaaaaagcaagtatcaatctgtgaaataaaaatgcaccttgagttaaactaaataattcataattacaggttaatttacccaagttccagccaagaaaagcatgaagatatttaagaaatcttaaattgatttgcatgcaagaaattaatcacatacaacttttcaaatcccaatgttattcccccttaaacttcttgtttaatgttttagtctgactgtatttgtaaagtaggtgacagagaaaaaaatacctgaggaaagctcagtaacgtgctgagggttcttttcctcactggaaagcagcggggcttcaggccaccatgagaaacagccagtgggcctttgactttacccaagttaagctcccctaataggagtagttagctaaacaagttcaacgctttccaaaggaaaaaggtcaagttaaaacaaaaatctaaataaaggtaaaatatcaacagtttctctgctttacaatgtgaccataaaattacttatttacagaaattaaaagaaatggttcaacaaagaatcaaactggtttctccaggtatataccatgacaatgtatctttttactcgatgctgtgagcagacagtgattattttggagaaggaaaaataaggtgtggaattagtaatgcagatgctgaaaggcaagtggcaagagaagaatgcctcaaacaaaggctactttgttcccatctctactgcacctacacccacacccgccccggcccccaagctaaaagaccagaataaccaaagccattttaacagtagtgtgcaaaactgtcagctgacaaacaacataaaaacaagtcacactatgttatctgtggtcacgttcttcagggttagtccagtaactcaagactttacattcttttgtctttatttgtttattttaattaaacatataaaggttaataaacagacaaagtccagagttagtaggttggtattataacatttattaaaataatgctgtgggttaatagaaacagcaaagaaccaaagaattaaaatgcaagctatgtaaaatcccaactaaaacccaaaagtgtctaatgtattcattcattagctaactaaaagcccaaaaaagacaagacacccaatataataaagtactgcaaaacaattggcaattttcagttatcaaaattgtggattttgcattttgtatccttttctcaatcaagaaaaaaattctttttgaatgttatataacatacatataaaacaagatagaaaaatacattataaacttgtaacaatggctgtaaatacattatcttacatgtttctcataggcaataggttggttatggtacatacatagcatgaaactaagataataaagaatagacaaaaatacatgtcagctgtacgataacatacaagcgacactcccatctacccacgctaaaaaattacataatactgtcagaaaaaaagtcttaaaaactacatattttaataagaaataaattcaataaagaatgataatactgagaaccaaggcattcagagatttcaaaagtcatgcttttttcagttgatccaaaattttgtcaaccaagttttcaaaagtttgttcagagccaacattccctataaatgtcacacatttattatttcatacatttactttcttccccataaaagacctttgataaacatctaaaatgtccaggtataacatagttgagatgaaactggatcaaatactggtattgtttttaacaactatcacctcaagtgtttgagtgtcgcaaatttattcaaccaaccaaacaatataaaaatcaaaatggcacagcatatattgtaaataaatcaaaactgtatgtgtaacagaaagacaaagcagtggcatattaaaccaaagctagctggatacaaaacaatgaatgtctattgcatagtaaataaactgacaacggtttccaagtgagacaagatggtgggggaggtcaccaagaaggtaatgactcagcttcctgctgacctctgactgtgatgctgggaaggtgtggaagaggggacgagttgataagctgggcgggggggggggtccactgtcacttgagatttgccacgtctggtactgagcagttaatgattattcactcaagtgtttagatgtaggctttgcacacaaattgcttcaactacataactaactgtttcaacttcttgagaaattagaagcttaagctgaaatgtggttgagtatttatatgcactatgatgctagtttttcacattcttttaaagttaaggggtgggggaggcagaggttattgaaacagtaaaaggatacactacaccagttatctggtatgatataaagacatgtgattaaatttgggtgatttaaaacattgttttctagaatgaaaatcacaaagattcacttttgtgaaaacatttgctaggtatcctattatattcaattaattaaaaacaaaaaacaaaatcaaatgaatgcatcccccttctccaaataaaacaaagctctaattttgtctgtaaactgaagtttagatgacacataatttttatctcagaatcctttgggttaacattgaagattggaataaccaaaagtattaaactattcttttaaagaatgatgttttaaaacttactagtcaggcattagaaaagttatcaaatcttttcacagtatcagatttggcaaatttgcatcaaggtaacgtggcaaaaatcctataattcaaactatcaactcatttgtctccctcatatcttctttcacatactgggcgactgagtaacatgcattaacttgtattctgagggaggagctgatctttatgagacacttgactgaatgaccatgaaggaaaataaggcactttcttttctttagacttattccaatacttaaaaaataaaaaagaaagacaaaaaggctcttttggtcttttgtttcttgacaaccaccagaaaaaatcatttaatgaaataaagggtttctttgttctttttctttttttttataacacttgaaagtataaaatgctacatttccaaaaatatatatatttttttctgcaccagcacccttgtatagtaaaagtatctactttttgttcatttgtttcaatgcactacactttatctacaatttcattacatgtatacagcaaataggcaagcatggcttttacatccttaatgatttttttctatacagggaggtttaaaaaaaaatacttgaacagtttgcccagtaatgtgacacataatgcatgtaccttgttctcatatttttttaggtgtaaaataaagattcagtaattttaactcagatatttatctttttaaaaatagtgttgcagttttgttatttgcattacttttcaaaactccttaagtttttctctcatggcacactttcttctaatacttcaaattttggcaggcaatataaaaaaggctgcaacttctgccctttgagggcactgtagtgactaaacagcatatcaaattttgaatactttttgaaatcacttcaccaatgatatccctgaccgaaggttcatgcatgatgcatcatcacacagtacattcagagagagctttgacttcgctatgagaagaaaaagattcctagaagtctctcacagtaactgcctctgtcattgagtagttaaggaccatctgtctccccttcttaagagaggccttcttaccgttcgcttagggtgggatattaaaagatgatcagtgctgtgggatgaattgggccttattgctttactactattcagtgcagtttctagaaccactttcacccaaacaggaaaaaaaaaaaaaaaaagctgagttggaggacaacaatttctttgtcttttgtttggttagatggtaagacgaacggacaagtgcctcagctcgctgcactgacgacaggcaagcaaaggcgattaccagttaactgatcagcaggcaggcatggtcaggtcatcattgggtgaagagttcagaggtcagaaggtcataggttagttgccggtggcggctcggtctgcggtcacaatcctttggtaaggatggacacgcatatcgtgccttcgaactttagtagccaccgcacctaatacaccactaggttcaataggatactcaaggattgatgtagctggtgccaatgtgtaggggtactcatagggtgtatagattaaaccagcttcgggccctggaggaactattgcagcagttgggtgaggagttccgtttggcatgacagcggtctgtatttgtctgatcaaaggcattatggtagggccagctggcgtaggagtacgcagggcagctggtgggagaaccggcgcaggcccagtaatgatccttggagcagcctgggctgttgctgcaagagaaaaggcaagggctggtgatttaatgttggcatctctgtaggtgccattcagaatcgcaagctccatcagctgcatcttcttcaggctgtcttctccttctgctgcaggtaccaataatttcttcacttcttcaactgctctcttcaatttgatttctgctctgttctgagcatcttccacagtgattagtacatgtaaatcttcatttagatgctcccaattgggcttgcctctattttgctcctccttttttttatccctcattgagcctttgcctcggaccatgattttacatccggtttctgcttcaagttgtttggctgtaagtcctctaggtccaaggattctcccaacaaaattaaaatctgggtattcttttacaggcacataaagtttctcttgtaactgaacaataggtcccacagcatcaggcaattctgcactccttttctctgtactgccatttaatgtgtcattgtacatgtctttccgtactctgctaatttcttcgtccagcagccgctcgaggtggttgaagatcccgcagaagttgggcaggctgctcatgagcttcttgtcgttcatcagctgcatcaggtaatctggggtgggcttcggcttctccttcgtttccatttccccgaccatattccaggctccgcagctcactccgcccgccgccgccgccgccgccgccggagaggagggaggggcgggggcgagccccggccgcgggccgctcgggacccggcgtcccgctccgcgccggctcccgctctggctcccgcgccgagccccggggcggccggcaccgcgcgctcgcccgccccccgcaggcactttccgcccgggcccgacgcgctcccagccgccgccgctctcggccgcccggctcggcgcgtccctcacgaggccggcgggcgggcgggaggcgggtctcggctggccgagtgcgggcgcggggcgcgggctgctggcgccggacgaggaggagccggggccgccgctcgctcggctggtcgagcccgctcagcgccgccgccgcctgtgccgcgggctcggggggtctctctgggctggtccccgccgcggcgcctctgccgctgccgccgcgctccgactgc

SEQ ID NO: 16953 - RNA, 6559 nt, Homo sapiens
  source 1..6559: mol_type = other RNA
taggcctttagatcacttaaactacagataaaattagatgtgtagcacatatttctaaaatattgtccatattttttccattttaaataaaggtattaaggaattcgtgacaatgtaaaaaactactctatgcacttagaaaaattgtgaattcgaaaagttggagaataatttttgctaaataaataatcatttggcagtaagttctattctacctaaaataatttgcttgaaatgctgtaacagctacttcttatcaaggaataaagacaggcatcacatcctggtcaaacatgcaaaaccactcccaccccaccccatcctaaaactaaagaaaccttaggctgtcacacgtgaaagtgttatgacatatatatatacacacacgtatatatatgaagagtcttgatttggtagtgagcaatttcatttaaacctatcgtttgcttttggcacactaaaaaattcagatccttatgtagtgtttagaaaaccataaccagacaccgattgtgtgtacgtatgcacatcctggttttatgggcagggtgccttcgtgacctcttacacctggagctactgcactggtgcgtatgggagtaactactttcatgttaagttttccctgacattttgcctaaaggaaaagtttaaggacattaatttcaccaacttcttgactgaaagctcagctttcaactgttttgtcaaatagtttcaatcaatcaactgactctagaattttactattcttggaatttggtagtttcatgtttaatattgtaacctgtataaaaatgaaatctgtaatgttattttcgccttttaaaacttttttacatttcctacataaaaggcagcaatgacataattatacataaagtacccttaactgaaaatgagatgaggctgcattcataggcttcagagaatagtaaattgcatagaaattcatcaatttaagttacatggtaccatgacaacttgtatattagcagcttgacagacagcttcgaattttcacagactactacatgaactgttatggcaacggaaacttttacaaatagtagcatgttaaaagacctgtccacctaacagtacactacccaccgctcccatcagagacatgacacggtttgtttacatgatccaaatgaccatctcaatggtgattcgctgttatcactcacatcagctaacactactctgtgtatttatatgtgtgtatacatatttatgaaatgagaatacctggacagtctgattggttaacagcgtattggtacagttttgtcttctattacatgtcattcatttcagccctcaattttagaactctaaataaataaaatgtaatttacaaagataaattgttatttacaaatgcaaaaattcatcctgaggattttggtatctaggagaactgtttcacagaaaaaagcaagtatcaatctgtgaaataaaaatgcaccttgagttaaactaaataattcataattacaggttaatttacccaagttccagccaagaaaagcatgaagatatttaagaaatcttaaattgatttgcatgcaagaaattaatcacatacaacttttcaaatcccaatgttattcccccttaaacttcttgtttaatgttttagtctgactgtatttgtaaagtaggtgacagagaaaaaaatacctgaggaaagctcagtaacgtgctgagggttcttttcctcactggaaagcagcggggcttcaggccaccatgagaaacagccagtgggcctttgactttacccaagttaagctcccctaataggagtagttagctaaacaagttcaacgctttccaaaggaaaaaggtcaagttaaaacaaaaatctaaataaaggtaaaatatcaacagtttctctgctttacaatgtgaccataaaattacttatttacagaaattaaaagaaatggttcaacaaagaatcaaactggtttctccaggtatataccatgacaatgtatctttttactcgatgctgtgagcagacagtgattattttggagaaggaaaaataaggtgtggaattagtaatgcagatgctgaaaggcaagtggcaagagaagaatgcctcaaacaaaggctactttgttcccatctctactgcacctacacccacacccgccccggcccccaagctaaaagaccagaataaccaaagccattttaacagtagtgtgcaaaactgtcagctgacaaacaacataaaaacaagtcacactatgttatctgtggtcacgttcttcagggttagtccagtaactcaagactttacattcttttgtctttatttgtttattttaattaaacatataaaggttaataaacagacaaagtccagagttagtaggttggtattataacatttattaaaataatgctgtgggttaatagaaacagcaaagaaccaaagaattaaaatgcaagctatgtaaaatcccaactaaaacccaaaagtgtctaatgtattcattcattagctaactaaaagcccaaaaaagacaagacacccaatataataaagtactgcaaaacaattggcaattttcagttatcaaaattgtggattttgcattttgtatccttttctcaatcaagaaaaaaattctttttgaatgttatataacatacatataaaacaagatagaaaaatacattataaacttgtaacaatggctgtaaatacattatcttacatgtttctcataggcaataggttggttatggtacatacatagcatgaaactaagataataaagaatagacaaaaatacatgtcagctgtacgataacatacaagcgacactcccatctacccacgctaaaaaattacataatactgtcagaaaaaaagtcttaaaaactacatattttaataagaaataaattcaataaagaatgataatactgagaaccaaggcattcagagatttcaaaagtcatgcttttttcagttgatccaaaattttgtcaaccaagttttcaaaagtttgttcagagccaacattccctataaatgtcacacatttattatttcatacatttactttcttccccataaaagacctttgataaacatctaaaatgtccaggtataacatagttgagatgaaactggatcaaatactggtattgtttttaacaactatcacctcaagtgtttgagtgtcgcaaatttattcaaccaaccaaacaatataaaaatcaaaatggcacagcatatattgtaaataaatcaaaactgtatgtgtaacagaaagacaaagcagtggcatattaaaccaaagctagctggatacaaaacaatgaatgtctattgcatagtaaataaactgacaacggtttccaagtgagacaagatggtgggggaggtcaccaagaaggtaatgactcagcttcctgctgacctctgactgtgatgctgggaaggtgtggaagaggggacgagttgataagctgggcgggggggggggtccactgtcacttgagatttgccacgtctggtactgagcagttaatgattattcactcaagtgtttagatgtaggctttgcacacaaattgcttcaactacataactaactgtttcaacttcttgagaaattagaagcttaagctgaaatgtggttgagtatttatatgcactatgatgctagtttttcacattcttttaaagttaaggggtgggggaggcagaggttattgaaacagtaaaaggatacactacaccagttatctggtatgatataaagacatgtgattaaatttgggtgatttaaaacattgttttctagaatgaaaatcacaaagattcacttttgtgaaaacatttgctaggtatcctattatattcaattaattaaaaacaaaaaacaaaatcaaatgaatgcatcccccttctccaaataaaacaaagctctaattttgtctgtaaactgaagtttagatgacacataatttttatctcagaatcctttgggttaacattgaagattggaataaccaaaagtattaaactattcttttaaagaatgatgttttaaaacttactagtcaggcattagaaaagttatcaaatcttttcacagtatcagatttggcaaatttgcatcaaggtaacgtggcaaaaatcctataattcaaactatcaactcatttgtctccctcatatcttctttcacatactgggcgactgagtaacatgcattaacttgtattctgagggaggagctgatctttatgagacacttgactgaatgaccatgaaggaaaataaggcactttcttttctttagacttattccaatacttaaaaaataaaaaagaaagacaaaaaggctcttttggtcttttgtttcttgacaaccaccagaaaaaatcatttaatgaaataaagggtttctttgttctttttctttttttttataacacttgaaagtataaaatgctacatttccaaaaatatatatatttttttctgcaccagcacccttgtatagtaaaagtatctactttttgttcatttgtttcaatgcactacactttatctacaatttcattacatgtatacagcaaataggcaagcatggcttttacatccttaatgatttttttctatacagggaggtttaaaaaaaaatacttgaacagtttgcccagtaatgtgacacataatgcatgtaccttgttctcatatttttttaggtgtaaaataaagattcagtaattttaactcagatatttatctttttaaaaatagtgttgcagttttgttatttgcattacttttcaaaactccttaagtttttctctcatggcacactttcttctaatacttcaaattttggcaggcaatataaaaaaggctgcaacttctgccctttgagggcactgtagtgactaaacagcatatcaaattttgaatactttttgaaatcacttcaccaatgatatccctgaccgaaggttcatgcatgatgcatcatcacacagtacattcagagagagctttgacttcgctatgagaagaaaaagattcctagaagtctctcacagtaactgcctctgtcattgagtagttaaggaccatctgtctccccttcttaagagaggccttcttaccgttcgcttagggtgggatattaaaagatgatcagtgctgtgggatgaattgggccttattgctttactactattcagtgcagtttctagaaccactttcacccaaacaggaaaaaaaaaaaaaaaaagctgagttggaggacaacaatttctttgtcttttgtttggttagatggtaagacgaacggacaagtgcctcagctcgctgcactgacgacaggcaagcaaaggcgattaccagttaactgatcagcaggcaggcatggtcaggtcatcattgggtgaagagttcagaggtcagaaggtcataggttagttgccggtggcggctcggtctgcggtcacaatcctttggtaaggatggacacgcatatcgtgccttcgaactttagtagccaccgcacctaatacaccactaggttcaataggatactcaaggattgatgtagctggtgccaatgtgtaggggtactcatagggtgtatagattaaaccagcttcgggccctggaggaactattgcagcagttgggtgaggagttccgtttggcatgacagcggtctgtatttgtctgatcaaaggcattatggtagggccagctggcgtaggagtacgcagggcagctggtgggagaaccggcgcaggcccagtaatgatccttggagcagcctgggctgttgctgcaagagaaaaggcaaggggtgatttaatgttggcatctctgtaggtgccattcagaatcgcaagctccatcagctgcatcttcttcaggctgtcttctccttctgctgcaggtaccaataatttcttcacttcttcaactgctctcttcaatttgatttctgctctgttctgagcatcttccacagtgattagtacatgtaaatcttcatttagatgctcccaattgggcttgcctctattttgctcctccttttttttatccctcattgagcctttgcctcggaccatgattttacatccggtttctgcttcaagttgtttggctgtaagtcctctaggtccaaggattctcccaacaaaattaaaatctgggtattcttttacaggcacataaagtttctcttgtaactgaacaataggtcccacagcatcaggcaattctgcactccttttctctgtactgccatttaatgtgtcattgtacatgtctttccgtactctgctaatttcttcgtccagcagccgctcgaggtggttgaagatcccgcagaagttgggcaggctgctcatgagcttcttgtcgttcatcagctgcatcaggtaatctggggtgggcttcggcttctccttcgtttccatttccccgaccatattccaggctccgcagctcactccgcccgccgccgccgccgccgccgccggagaggag

SEQ ID NO: 16954 - RNA, 6956 nt, Homo sapiens
  source 1..6956: mol_type = other RNA
taggcctttagatcacttaaactacagataaaattagatgtgtagcacatatttctaaaatattgtccatattttttccattttaaataaaggtattaaggaattcgtgacaatgtaaaaaactactctatgcacttagaaaaattgtgaattcgaaaagttggagaataatttttgctaaataaataatcatttggcagtaagttctattctacctaaaataatttgcttgaaatgctgtaacagctacttcttatcaaggaataaagacaggcatcacatcctggtcaaacatgcaaaaccactcccaccccaccccatcctaaaactaaagaaaccttaggctgtcacacgtgaaagtgttatgacatatatatatacacacacgtatatatatgaagagtcttgatttggtagtgagcaatttcatttaaacctatcgtttgcttttggcacactaaaaaattcagatccttatgtagtgtttagaaaaccataaccagacaccgattgtgtgtacgtatgcacatcctggttttatgggcagggtgccttcgtgacctcttacacctggagctactgcactggtgcgtatgggagtaactactttcatgttaagttttccctgacattttgcctaaaggaaaagtttaaggacattaatttcaccaacttcttgactgaaagctcagctttcaactgttttgtcaaatagtttcaatcaatcaactgactctagaattttactattcttggaatttggtagtttcatgtttaatattgtaacctgtataaaaatgaaatctgtaatgttattttcgccttttaaaacttttttacatttcctacataaaaggcagcaatgacataattatacataaagtacccttaactgaaaatgagatgaggctgcattcataggcttcagagaatagtaaattgcatagaaattcatcaatttaagttacatggtaccatgacaacttgtatattagcagcttgacagacagcttcgaattttcacagactactacatgaactgttatggcaacggaaacttttacaaatagtagcatgttaaaagacctgtccacctaacagtacactacccaccgctcccatcagagacatgacacggtttgtttacatgatccaaatgaccatctcaatggtgattcgctgttatcactcacatcagctaacactactctgtgtatttatatgtgtgtatacatatttatgaaatgagaatacctggacagtctgattggttaacagcgtattggtacagttttgtcttctattacatgtcattcatttcagccctcaattttagaactctaaataaataaaatgtaatttacaaagataaattgttatttacaaatgcaaaaattcatcctgaggattttggtatctaggagaactgtttcacagaaaaaagcaagtatcaatctgtgaaataaaaatgcaccttgagttaaactaaataattcataattacaggttaatttacccaagttccagccaagaaaagcatgaagatatttaagaaatcttaaattgatttgcatgcaagaaattaatcacatacaacttttcaaatcccaatgttattcccccttaaacttcttgtttaatgttttagtctgactgtatttgtaaagtaggtgacagagaaaaaaatacctgaggaaagctcagtaacgtgctgagggttcttttcctcactggaaagcagcggggcttcaggccaccatgagaaacagccagtgggcctttgactttacccaagttaagctcccctaataggagtagttagctaaacaagttcaacgctttccaaaggaaaaaggtcaagttaaaacaaaaatctaaataaaggtaaaatatcaacagtttctctgctttacaatgtgaccataaaattacttatttacagaaattaaaagaaatggttcaacaaagaatcaaactggtttctccaggtatataccatgacaatgtatctttttactcgatgctgtgagcagacagtgattattttggagaaggaaaaataaggtgtggaattagtaatgcagatgctgaaaggcaagtggcaagagaagaatgcctcaaacaaaggctactttgttcccatctctactgcacctacacccacacccgccccggcccccaagctaaaagaccagaataaccaaagccattttaacagtagtgtgcaaaactgtcagctgacaaacaacataaaaacaagtcacactatgttatctgtggtcacgttcttcagggttagtccagtaactcaagactttacattcttttgtctttatttgtttattttaattaaacatataaaggttaataaacagacaaagtccagagttagtaggttggtattataacatttattaaaataatgctgtgggttaatagaaacagcaaagaaccaaagaattaaaatgcaagctatgtaaaatcccaactaaaacccaaaagtgtctaatgtattcattcattagctaactaaaagcccaaaaaagacaagacacccaatataataaagtactgcaaaacaattggcaattttcagttatcaaaattgtggattttgcattttgtatccttttctcaatcaagaaaaaaattctttttgaatgttatataacatacatataaaacaagatagaaaaatacattataaacttgtaacaatggctgtaaatacattatcttacatgtttctcataggcaataggttggttatggtacatacatagcatgaaactaagataataaagaatagacaaaaatacatgtcagctgtacgataacatacaagcgacactcccatctacccacgctaaaaaattacataatactgtcagaaaaaaagtcttaaaaactacatattttaataagaaataaattcaataaagaatgataatactgagaaccaaggcattcagagatttcaaaagtcatgcttttttcagttgatccaaaattttgtcaaccaagttttcaaaagtttgttcagagccaacattccctataaatgtcacacatttattatttcatacatttactttcttccccataaaagacctttgataaacatctaaaatgtccaggtataacatagttgagatgaaactggatcaaatactggtattgtttttaacaactatcacctcaagtgtttgagtgtcgcaaatttattcaaccaaccaaacaatataaaaatcaaaatggcacagcatatattgtaaataaatcaaaactgtatgtgtaacagaaagacaaagcagtggcatattaaaccaaagctagctggatacaaaacaatgaatgtctattgcatagtaaataaactgacaacggtttccaagtgagacaagatggtgggggaggtcaccaagaaggtaatgactcagcttcctgctgacctctgactgtgatgctgggaaggtgtggaagaggggacgagttgataagctgggcgggggggggggtccactgtcacttgagatttgccacgtctggtactgagcagttaatgattattcactcaagtgtttagatgtaggctttgcacacaaattgcttcaactacataactaactgtttcaacttcttgagaaattagaagcttaagctgaaatgtggttgagtatttatatgcactatgatgctagtttttcacattcttttaaagttaaggggtgggggaggcagaggttattgaaacagtaaaaggatacactacaccagttatctggtatgatataaagacatgtgattaaatttgggtgatttaaaacattgttttctagaatgaaaatcacaaagattcacttttgtgaaaacatttgctaggtatcctattatattcaattaattaaaaacaaaaaacaaaatcaaatgaatgcatcccccttctccaaataaaacaaagctctaattttgtctgtaaactgaagtttagatgacacataatttttatctcagaatcctttgggttaacattgaagattggaataaccaaaagtattaaactattcttttaaagaatgatgttttaaaacttactagtcaggcattagaaaagttatcaaatcttttcacagtatcagatttggcaaatttgcatcaaggtaacgtggcaaaaatcctataattcaaactatcaactcatttgtctccctcatatcttctttcacatactgggcgactgagtaacatgcattaacttgtattctgagggaggagctgatctttatgagacacttgactgaatgaccatgaaggaaaataaggcactttcttttctttagacttattccaatacttaaaaaataaaaaagaaagacaaaaaggctcttttggtcttttgtttcttgacaaccaccagaaaaaatcatttaatgaaataaagggtttctttgttctttttctttttttttataacacttgaaagtataaaatgctacatttccaaaaatatatatatttttttctgcaccagcacccttgtatagtaaaagtatctactttttgttcatttgtttcaatgcactacactttatctacaatttcattacatgtatacagcaaataggcaagcatggcttttacatccttaatgatttttttctatacagggaggtttaaaaaaaaatacttgaacagtttgcccagtaatgtgacacataatgcatgtaccttgttctcatatttttttaggtgtaaaataaagattcagtaattttaactcagatatttatctttttaaaaatagtgttgcagttttgttatttgcattacttttcaaaactccttaagtttttctctcatggcacactttcttctaatacttcaaattttggcaggcaatataaaaaaggctgcaacttctgccctttgagggcactgtagtgactaaacagcatatcaaattttgaatactttttgaaatcacttcaccaatgatatccctgaccgaaggttcatgcatgatgcatcatcacacagtacattcagagagagctttgacttcgctatgagaagaaaaagattcctagaagtctctcacagtaactgcctctgtcattgagtagttaaggaccatctgtctccccttcttaagagaggccttcttaccgttcgcttagggtgggatattaaaagatgatcagtgctgtgggatgaattgggccttattgctttactactattcagtgcagtttctagaaccactttcacccaaacaggaaaaaaaaaaaaaaaaagctgagttggaggacaacaatttctttgtcttttgtttggttagatggtaagacgaacggacaagtgcctcagctcgctgcactgacgacaggcaagcaaaggcgattaccagttaactgatcagcaggcaggcatggtcaggtcatcattgggtgaagagttcagaggtcagaaggtcataggttagttgccggtggcggctcggtctgcggtcacaatcctttggtaaggatggacacgcatatcgtgccttcgaactttagtagccaccgcacctaatacaccactaggttcaataggatactcaaggattgatgtagctggtgccaatgtgtaggggtactcatagggtgtatagattaaaccagcttcgggccctggaggaactattgcagcagttgggtgaggagttccgtttggcatgacagcggtctgtatttgtctgatcaaaggcattatggtagggccagctggcgtaggagtacgcagggcagctggtgggagaaccggcgcaggcccagtaatgatccttggagcagcctgggctgttggtgatttaatgttggcatctctgtaggtgccattcagaatcgcaagctccatcagctgcatcttcttcaggctgtcttctccttctgctgcaggtaccaataatttcttcacttcttcaactgctctcttcaatttgatttctgctctgttctgagcatcttccacagtgattagtacatgtaaatcttcatttagatgctcccaattgggcttgcctctattttgctcctccttttttttatccctcattgagcctttgcctcggaccatgattttacatccggtttctgcttcaagttgtttggctgtaagtcctctaggtccaaggattctcccaacaaaattaaaatctgggtattcttttacaggcacataaagtttctcttgtaactgaacaataggtcccacagcatcaggcaattctgcactccttttctctgtactgccatttaatgtgtcattgtacatgtctttccgtactctgctaatttcttcgtccagcagccgctcgaggtggttgaagatcccgcagaagttgggcaggctgctcatgagcttcttgtcgttcatcagctgcatcaggtaatctggggtgggcttcggcttctccttcgtttccatttccccgaccatattccaggctccgcagctcactccgcccgccgccgccgccgccgccgccggagaggagggaggggcgggggcgagccccggccgcgggccgctcgggacccggcgtcccgctccgcgccggctcccgctctggctcccgcgccgagccccggggcggccggcaccgcgcgctcgcccgccccccgcaggcactttccgcccgggcccgacgcgctcccagccgccgccgctctcggccgcccggctcggcgcgtccctcacgaggccggcgggcgggcgggaggcgggtctcggctggccgagtgcgggcgcggggcgcgggctgctggcgccggacgaggaggagccggggccgccgctcgctcggctggtcgagcccgctcagcgccgccgccgcctgtgccgcgggctcggggggtctctctgggctggtccccgccgcggcgcctctgccgctgccgccgcgctccgactgc

SEQ ID NO: 16955 - RNA, 9266 nt, Homo sapiens
  source 1..9266: mol_type = other RNA
taggcctttagatcacttaaactacagataaaattagatgtgtagcacatatttctaaaatattgtccatattttttccattttaaataaaggtattaaggaattcgtgacaatgtaaaaaactactctatgcacttagaaaaattgtgaattcgaaaagttggagaataatttttgctaaataaataatcatttggcagtaagttctattctacctaaaataatttgcttgaaatgctgtaacagctacttcttatcaaggaataaagacaggcatcacatcctggtcaaacatgcaaaaccactcccaccccaccccatcctaaaactaaagaaaccttaggctgtcacacgtgaaagtgttatgacatatatatatacacacacgtatatatatgaagagtcttgatttggtagtgagcaatttcatttaaacctatcgtttgcttttggcacactaaaaaattcagatccttatgtagtgtttagaaaaccataaccagacaccgattgtgtgtacgtatgcacatcctggttttatgggcagggtgccttcgtgacctcttacacctggagctactgcactggtgcgtatgggagtaactactttcatgttaagttttccctgacattttgcctaaaggaaaagtttaaggacattaatttcaccaacttcttgactgaaagctcagctttcaactgttttgtcaaatagtttcaatcaatcaactgactctagaattttactattcttggaatttggtagtttcatgtttaatattgtaacctgtataaaaatgaaatctgtaatgttattttcgccttttaaaacttttttacatttcctacataaaaggcagcaatgacataattatacataaagtacccttaactgaaaatgagatgaggctgcattcataggcttcagagaatagtaaattgcatagaaattcatcaatttaagttacatggtaccatgacaacttgtatattagcagcttgacagacagcttcgaattttcacagactactacatgaactgttatggcaacggaaacttttacaaatagtagcatgttaaaagacctgtccacctaacagtacactacccaccgctcccatcagagacatgacacggtttgtttacatgatccaaatgaccatctcaatggtgattcgctgttatcactcacatcagctaacactactctgtgtatttatatgtgtgtatacatatttatgaaatgagaatacctggacagtctgattggttaacagcgtattggtacagttttgtcttctattacatgtcattcatttcagccctcaattttagaactctaaataaataaaatgtaatttacaaagataaattgttatttacaaatgcaaaaattcatcctgaggattttggtatctaggagaactgtttcacagaaaaaagcaagtatcaatctgtgaaataaaaatgcaccttgagttaaactaaataattcataattacaggttaatttacccaagttccagccaagaaaagcatgaagatatttaagaaatcttaaattgatttgcatgcaagaaattaatcacatacaacttttcaaatcccaatgttattcccccttaaacttcttgtttaatgttttagtctgactgtatttgtaaagtaggtgacagagaaaaaaatacctgaggaaagctcagtaacgtgctgagggttcttttcctcactggaaagcagcggggcttcaggccaccatgagaaacagccagtgggcctttgactttacccaagttaagctcccctaataggagtagttagctaaacaagttcaacgctttccaaaggaaaaaggtcaagttaaaacaaaaatctaaataaaggtaaaatatcaacagtttctctgctttacaatgtgaccataaaattacttatttacagaaattaaaagaaatggttcaacaaagaatcaaactggtttctccaggtatataccatgacaatgtatctttttactcgatgctgtgagcagacagtgattattttggagaaggaaaaataaggtgtggaattagtaatgcagatgctgaaaggcaagtggcaagagaagaatgcctcaaacaaaggctactttgttcccatctctactgcacctacacccacacccgccccggcccccaagctaaaagaccagaataaccaaagccattttaacagtagtgtgcaaaactgtcagctgacaaacaacataaaaacaagtcacactatgttatctgtggtcacgttcttcagggttagtccagtaactcaagactttacattcttttgtctttatttgtttattttaattaaacatataaaggttaataaacagacaaagtccagagttagtaggttggtattataacatttattaaaataatgctgtgggttaatagaaacagcaaagaaccaaagaattaaaatgcaagctatgtaaaatcccaactaaaacccaaaagtgtctaatgtattcattcattagctaactaaaagcccaaaaaagacaagacacccaatataataaagtactgcaaaacaattggcaattttcagttatcaaaattgtggattttgcattttgtatccttttctcaatcaagaaaaaaattctttttgaatgttatataacatacatataaaacaagatagaaaaatacattataaacttgtaacaatggctgtaaatacattatcttacatgtttctcataggcaataggttggttatggtacatacatagcatgaaactaagataataaagaatagacaaaaatacatgtcagctgtacgataacatacaagcgacactcccatctacccacgctaaaaaattacataatactgtcagaaaaaaagtcttaaaaactacatattttaataagaaataaattcaataaagaatgataatactgagaaccaaggcattcagagatttcaaaagtcatgcttttttcagttgatccaaaattttgtcaaccaagttttcaaaagtttgttcagagccaacattccctataaatgtcacacatttattatttcatacatttactttcttccccataaaagacctttgataaacatctaaaatgtccaggtataacatagttgagatgaaactggatcaaatactggtattgtttttaacaactatcacctcaagtgtttgagtgtcgcaaatttattcaaccaaccaaacaatataaaaatcaaaatggcacagcatatattgtaaataaatcaaaactgtatgtgtaacagaaagacaaagcagtggcatattaaaccaaagctagctggatacaaaacaatgaatgtctattgcatagtaaataaactgacaacggtttccaagtgagacaagatggtgggggaggtcaccaagaaggtaatgactcagcttcctgctgacctctgactgtgatgctgggaaggtgtggaagaggggacgagttgataagctgggcgggggggggggtccactgtcacttgagatttgccacgtctggtactgagcagttaatgattattcactcaagtgtttagatgtaggctttgcacacaaattgcttcaactacataactaactgtttcaacttcttgagaaattagaagcttaagctgaaatgtggttgagtatttatatgcactatgatgctagtttttcacattcttttaaagttaaggggtgggggaggcagaggttattgaaacagtaaaaggatacactacaccagttatctggtatgatataaagacatgtgattaaatttgggtgatttaaaacattgttttctagaatgaaaatcacaaagattcacttttgtgaaaacatttgctaggtatcctattatattcaattaattaaaaacaaaaaacaaaatcaaatgaatgcatcccccttctccaaataaaacaaagctctaattttgtctgtaaactgaagtttagatgacacataatttttatctcagaatcctttgggttaacattgaagattggaataaccaaaagtattaaactattcttttaaagaatgatgttttaaaacttactagtcaggcattagaaaagttatcaaatcttttcacagtatcagatttggcaaatttgcatcaaggtaacgtggcaaaaatcctataattcaaactatcaactcatttgtctccctcatatcttctttcacatactgggcgactgagtaacatgcattaacttgtattctgagggaggagctgatctttatgagacacttgactgaatgaccatgaaggaaaataaggcactttcttttctttagacttattccaatacttaaaaaataaaaaagaaagacaaaaaggctcttttggtcttttgtttcttgacaaccaccagaaaaaatcatttaatgaaataaagggtttctttgttctttttctttttttttataacacttgaaagtataaaatgctacatttccaaaaatatatatatttttttctgcaccagcacccttgtatagtaaaagtatctactttttgttcatttgtttcaatgcactacactttatctacaatttcattacatgtatacagcaaataggcaagcatggcttttacatccttaatgatttttttctatacagggaggtttaaaaaaaaatacttgaacagtttgcccagtaatgtgacacataatgcatgtaccttgttctcatatttttttaggtgtaaaataaagattcagtaattttaactcagatatttatctttttaaaaatagtgttgcagttttgttatttgcattacttttcaaaactccttaagtttttctctcatggcacactttcttctaatacttcaaattttggcaggcaatataaaaaaggctgcaacttctgccctttgagggcactgtagtgactaaacagcatatcaaattttgaatactttttgaaatcacttcaccaatgatatccctgaccgaaggttcatgcatgatgcatcatcacacagtacattcagagagagctttgacttcgctatgagaagaaaaagattcctagaagtctctcacagtaactgcctctgtcattgagtagttaaggaccatctgtctccccttcttaagagaggccttcttaccgttcgcttagggtgggatattaaaagatgatcagtgctgtgggatgaattgggccttattgctttactactattcagtgcagtttctagaaccactttcacccaaacaggaaaaaaaaaaaaaaaaagctgagttggaggacaacaatttctttgtcttttgtttggttagatggtaagacgaacggacaagtgcctcagctcgctgcactgacgacaggcaagcaaaggcgattaccagttaactgatcagcaggcaggcatggtcaggtcatcattgggtgaagagttcagaggtcagaaggtcataggttagttgccggtggcggctcggtctgcggtcacaatcctttggtaaggatggacacgcatatcgtgccttcgaactttagtagccaccgcacctagttaaattgcaattaccaagacaaagttagaaaacattcacaaggggggaaaaaacattaacagcaggtttatcaaaatggatttcaaatgttcatttactacaaaagtttaagaaacacgttaaggcacagtagttttaaaattaaccacaatatgtcatgtatatatgcatctattaatattgcattcatttcaaacatcttgggccttaacctattgtatccattcatttacaatccccaagttacagtatttcatgagctctattagatccaaacatatttaagctttactagtcacatattcactgaagtgcctttcttgcagcaggactacttaaataacgccatgtttaatacagacaattatttgctaaccttaagaccacttcaagagtttatcacttaaaaaggtttaaaagcaattcttaaagcctacagattgtggttttaaactctgagtcaataagtatgaactgcaatgaattaggtgattagtaaagcaaacagtatagtacacttagcagtcagtatactactatacactcctttataaattaccattactgtgtaatattacagactaaaccaaattaataacataattttactttatatctatgtgcaaaaagtgcaagtaagtcactgactgctaggctaagcttttttcccccggaggctgctgagactaagcatttgttaaattcagatctgatgagggttcagttaagaccgttcttgaattcttagcctttcgttgggaaagccatacctaaagataaaaggaagggaattaaaaattagtcatcaatgaagacttgatgctaataccaatctcctcactactaccaacacacatgtctgcatctgttttgaagggcactgcttattttaaaataatttaatgtgagatgtgacataaatagcatgcatgttatctgtgtgcaaatttattataacttagaaatttaaaataattttctgagttctccaagtggtcaatatcatgttttactgcttaggtggcaaagcaagaaatgaaattaaccataatagattttttcattgggcacttattattattcaccttatgaatgccaattagaaatctgcatattttggtctttattttaccagtctaataattaagtttctataagtaaaaattttccaacaaacaaaagacatgaagctttacaatgagaaacaagttttactgcagtgcctcttgctatttctaagcagtaaactggtccatcacctcttattcattttagataaggtaatcatatacaagtacaattccacgtggcaaaatcagggagatcttgcgctgaaagtgctggaacagcagctggtggctaagagccccagccctgcaggaagtcaagagtcataactcctcgggaacagatgctgtgggtgcagcagagaggagttctgggaaaaggagcatgcacgggaccacaggacagagtattaatagaaaagaaaacttaaacaacaaggttacaggttacatgttattttaaaaatgcttcaagaaatgtgcaacagacacaagcctctcataaacagttctgtggtataattctgacctgcaattactttatacaatgatttaaacagaaaacatgtacaatgaaatgtatttgttcatgaaacaaagggcacctgagtgcatgcacacacacagataacatacagagcatcatggctttctttacttgaacaacgaattttcgagtttaaatcttagtgttctccagttcattaaagattttcaaatctttataaatcaatattaatgctggggaaaaaaaaccttaaaagatcaaagtcctaaaagtcaacagcatgcatgcagcaccaaggtcatatacaattcaggaaaaaaagtattcaaattttgtctggtaaaacaaaggggttgcacagaaacagtttgttccacattgactggtcgtgttataacagctgctgtattctagtccttcatccagcaagtcaatgggctgaaatatcaggcatgactggcatttcaatccactctaatacaccactaggttcaataggatactcaaggattgatgtagctggtgccaatgtgtaggggtactcatagggtgtatagattaaaccagcttcgggccctggaggaactattgcagcagttgggtgaggagttccgtttggcatgacagcggtctgtatttgtctgatcaaaggcattatggtagggccagctggcgtaggagtacgcagggcagctggtgggagaaccggcgcaggcccagtaatgatccttggagcagcctgggctgttgctgcaagagaaaaggcaagggctggtgatttaatgttggcatctctgtaggtgccattcagaatcgcaagctccatcagctgcatcttcttcaggctgtcttctccttctgctgcaggtaccaataatttcttcacttcttcaactgctctcttcaatttgatttctgctctgttctgagcatcttccacagtgattagtacatgtaaatcttcatttagatgctcccaattgggcttgcctctattttgctcctccttttttttatccctcattgagcctttgcctcggaccatgattttacatccggtttctgcttcaagttgtttggctgtaagtcctctaggtccaaggattctcccaacaaaattaaaatctgggtattcttttacaggcacataaagtttctcttgtaactgaacaataggtcccacagcatcaggcaattctgcactccttttctctgtactgccatttaatgtgtcattgtacatgtctttccgtactctgctaatttcttcgtccagcagccgctcgaggtggttgaagatcccgcagaagttgggcaggctgctcatgagcttcttgtcgttcatcagctgcatcaggtaatctggggtgggcttcggcttctccttcgtttccatttccccgaccatattccaggctccgcagctcactccgcccgccgccgccgccgccgccgccggagaggagggaggggcgggggcgagccccggccgcgggccgctcgggacccggcgtcccgctccgcgccggctcccgctctggctcccgcgccgagccccggggcggccggcaccgcgcgctcgcccgccccccgcaggcactttccgcccgggcccgacgcgctcccagccgccgccgctctcggccgcccggctcggcgcgtccctcacgaggccggcgggcgggcgggaggcgggtctcggctggccgagtgcgggcgcggggcgcgggctgctggcgccggacgaggaggagccggggccgccgctcgctcggctggtcgagcccgctcagcgccgccgccgcctgtgccgcgggctcggggggtctctctgggctggtccccgccgcggcgcctctgccgctgccgccgcgctccgactgcgctcctcctcttcctcctcctccttctcctcctcctcctcctcactcacttggcggcggagttcgcctcagttcaggcggcgctgccagcggcggcggcagcagcggcggcggcggggggaggggcagcggcgcggggagggccgggggcgggcggcgggcggggccgcgcagggcggccgttagcgggtcccggccggcgcgctcccgctgcctgctgcccgccgccccgc

SEQ ID NO: 16956 - RNA, 8592 nt, Homo sapiens
  source 1..8592: mol_type = other RNA
taggcctttagatcacttaaactacagataaaattagatgtgtagcacatatttctaaaatattgtccatattttttccattttaaataaaggtattaaggaattcgtgacaatgtaaaaaactactctatgcacttagaaaaattgtgaattcgaaaagttggagaataatttttgctaaataaataatcatttggcagtaagttctattctacctaaaataatttgcttgaaatgctgtaacagctacttcttatcaaggaataaagacaggcatcacatcctggtcaaacatgcaaaaccactcccaccccaccccatcctaaaactaaagaaaccttaggctgtcacacgtgaaagtgttatgacatatatatatacacacacgtatatatatgaagagtcttgatttggtagtgagcaatttcatttaaacctatcgtttgcttttggcacactaaaaaattcagatccttatgtagtgtttagaaaaccataaccagacaccgattgtgtgtacgtatgcacatcctggttttatgggcagggtgccttcgtgacctcttacacctggagctactgcactggtgcgtatgggagtaactactttcatgttaagttttccctgacattttgcctaaaggaaaagtttaaggacattaatttcaccaacttcttgactgaaagctcagctttcaactgttttgtcaaatagtttcaatcaatcaactgactctagaattttactattcttggaatttggtagtttcatgtttaatattgtaacctgtataaaaatgaaatctgtaatgttattttcgccttttaaaacttttttacatttcctacataaaaggcagcaatgacataattatacataaagtacccttaactgaaaatgagatgaggctgcattcataggcttcagagaatagtaaattgcatagaaattcatcaatttaagttacatggtaccatgacaacttgtatattagcagcttgacagacagcttcgaattttcacagactactacatgaactgttatggcaacggaaacttttacaaatagtagcatgttaaaagacctgtccacctaacagtacactacccaccgctcccatcagagacatgacacggtttgtttacatgatccaaatgaccatctcaatggtgattcgctgttatcactcacatcagctaacactactctgtgtatttatatgtgtgtatacatatttatgaaatgagaatacctggacagtctgattggttaacagcgtattggtacagttttgtcttctattacatgtcattcatttcagccctcaattttagaactctaaataaataaaatgtaatttacaaagataaattgttatttacaaatgcaaaaattcatcctgaggattttggtatctaggagaactgtttcacagaaaaaagcaagtatcaatctgtgaaataaaaatgcaccttgagttaaactaaataattcataattacaggttaatttacccaagttccagccaagaaaagcatgaagatatttaagaaatcttaaattgatttgcatgcaagaaattaatcacatacaacttttcaaatcccaatgttattcccccttaaacttcttgtttaatgttttagtctgactgtatttgtaaagtaggtgacagagaaaaaaatacctgaggaaagctcagtaacgtgctgagggttcttttcctcactggaaagcagcggggcttcaggccaccatgagaaacagccagtgggcctttgactttacccaagttaagctcccctaataggagtagttagctaaacaagttcaacgctttccaaaggaaaaaggtcaagttaaaacaaaaatctaaataaaggtaaaatatcaacagtttctctgctttacaatgtgaccataaaattacttatttacagaaattaaaagaaatggttcaacaaagaatcaaactggtttctccaggtatataccatgacaatgtatctttttactcgatgctgtgagcagacagtgattattttggagaaggaaaaataaggtgtggaattagtaatgcagatgctgaaaggcaagtggcaagagaagaatgcctcaaacaaaggctactttgttcccatctctactgcacctacacccacacccgccccggcccccaagctaaaagaccagaataaccaaagccattttaacagtagtgtgcaaaactgtcagctgacaaacaacataaaaacaagtcacactatgttatctgtggtcacgttcttcagggttagtccagtaactcaagactttacattcttttgtctttatttgtttattttaattaaacatataaaggttaataaacagacaaagtccagagttagtaggttggtattataacatttattaaaataatgctgtgggttaatagaaacagcaaagaaccaaagaattaaaatgcaagctatgtaaaatcccaactaaaacccaaaagtgtctaatgtattcattcattagctaactaaaagcccaaaaaagacaagacacccaatataataaagtactgcaaaacaattggcaattttcagttatcaaaattgtggattttgcattttgtatccttttctcaatcaagaaaaaaattctttttgaatgttatataacatacatataaaacaagatagaaaaatacattataaacttgtaacaatggctgtaaatacattatcttacatgtttctcataggcaataggttggttatggtacatacatagcatgaaactaagataataaagaatagacaaaaatacatgtcagctgtacgataacatacaagcgacactcccatctacccacgctaaaaaattacataatactgtcagaaaaaaagtcttaaaaactacatattttaataagaaataaattcaataaagaatgataatactgagaaccaaggcattcagagatttcaaaagtcatgcttttttcagttgatccaaaattttgtcaaccaagttttcaaaagtttgttcagagccaacattccctataaatgtcacacatttattatttcatacatttactttcttccccataaaagacctttgataaacatctaaaatgtccaggtataacatagttgagatgaaactggatcaaatactggtattgtttttaacaactatcacctcaagtgtttgagtgtcgcaaatttattcaaccaaccaaacaatataaaaatcaaaatggcacagcatatattgtaaataaatcaaaactgtatgtgtaacagaaagacaaagcagtggcatattaaaccaaagctagctggatacaaaacaatgaatgtctattgcatagtaaataaactgacaacggtttccaagtgagacaagatggtgggggaggtcaccaagaaggtaatgactcagcttcctgctgacctctgactgtgatgctgggaaggtgtggaagaggggacgagttgataagctgggcgggggggggggtccactgtcacttgagatttgccacgtctggtactgagcagttaatgattattcactcaagtgtttagatgtaggctttgcacacaaattgcttcaactacataactaactgtttcaacttcttgagaaattagaagcttaagctgaaatgtggttgagtatttatatgcactatgatgctagtttttcacattcttttaaagttaaggggtgggggaggcagaggttattgaaacagtaaaaggatacactacaccagttatctggtatgatataaagacatgtgattaaatttgggtgatttaaaacattgttttctagaatgaaaatcacaaagattcacttttgtgaaaacatttgctaggtatcctattatattcaattaattaaaaacaaaaaacaaaatcaaatgaatgcatcccccttctccaaataaaacaaagctctaattttgtctgtaaactgaagtttagatgacacataatttttatctcagaatcctttgggttaacattgaagattggaataaccaaaagtattaaactattcttttaaagaatgatgttttaaaacttactagtcaggcattagaaaagttatcaaatcttttcacagtatcagatttggcaaatttgcatcaaggtaacgtggcaaaaatcctataattcaaactatcaactcatttgtctccctcatatcttctttcacatactgggcgactgagtaacatgcattaacttgtattctgagggaggagctgatctttatgagacacttgactgaatgaccatgaaggaaaataaggcactttcttttctttagacttattccaatacttaaaaaataaaaaagaaagacaaaaaggctcttttggtcttttgtttcttgacaaccaccagaaaaaatcatttaatgaaataaagggtttctttgttctttttctttttttttataacacttgaaagtataaaatgctacatttccaaaaatatatatatttttttctgcaccagcacccttgtatagtaaaagtatctactttttgttcatttgtttcaatgcactacactttatctacaatttcattacatgtatacagcaaataggcaagcatggcttttacatccttaatgatttttttctatacagggaggtttaaaaaaaaatacttgaacagtttgcccagtaatgtgacacataatgcatgtaccttgttctcatatttttttaggtgtaaaataaagattcagtaattttaactcagatatttatctttttaaaaatagtgttgcagttttgttatttgcattacttttcaaaactccttaagtttttctctcatggcacactttcttctaatacttcaaattttggcaggcaatataaaaaaggctgcaacttctgccctttgagggcactgtagtgactaaacagcatatcaaattttgaatactttttgaaatcacttcaccaatgatatccctgaccgaaggttcatgcatgatgcatcatcacacagtacattcagagagagctttgacttcgctatgagaagaaaaagattcctagaagtctctcacagtaactgcctctgtcattgagtagttaaggaccatctgtctccccttcttaagagaggccttcttaccgttcgcttagggtgggatattaaaagatgatcagtgctgtgggatgaattgggccttattgctttactactattcagtgcagtttctagaaccactttcacccaaacaggaaaaaaaaaaaaaaaaagctgagttggaggacaacaatttctttgtcttttgtttggttagatggtaagacgaacggacaagtgcctcagctcgctgcactgacgacaggcaagcaaaggcgattaccagttaactgatcagcaggcaggcatggtcaggtcatcattgggtgaagagttcagaggtcagaaggtcataggttagttgccggtggcggctcggtctgcggtcacaatcctttggtaaggatggacacgcatatcgtgccttcgaactttagtagccaccgcacctagttaaattgcaattaccaagacaaagttagaaaacattcacaaggggggaaaaaacattaacagcaggtttatcaaaatggatttcaaatgttcatttactacaaaagtttaagaaacacgttaaggcacagtagttttaaaattaaccacaatatgtcatgtatatatgcatctattaatattgcattcatttcaaacatcttgggccttaacctattgtatccattcatttacaatccccaagttacagtatttcatgagctctattagatccaaacatatttaagctttactagtcacatattcactgaagtgcctttcttgcagcaggactacttaaataacgccatgtttaatacagacaattatttgctaaccttaagaccacttcaagagtttatcacttaaaaaggtttaaaagcaattcttaaagcctacagattgtggttttaaactctgagtcaataagtatgaactgcaatgaattaggtgattagtaaagcaaacagtatagtacacttagcagtcagtatactactatacactcctttataaattaccattactgtgtaatattacagactaaaccaaattaataacataattttactttatatctatgtgcaaaaagtgcaagtaagtcactgactgctaggctaagcttttttcccccggaggctgctgagactaagcatttgttaaattcagatctgatgagggttcagttaagaccgttcttgaattcttagcctttcgttgggaaagccatacctaaagataaaaggaagggaattaaaaattagtcatcaatgaagacttgatgctaataccaatctcctcactactaccaacacacatgtctgcatctgttttgaagggcactgcttattttaaaataatttaatgtgagatgtgacataaatagcatgcatgttatctgtgtgcaaatttattataacttagaaatttaaaataattttctgagttctccaagtggtcaatatcatgttttactgcttaggtggcaaagcaagaaatgaaattaaccataatagattttttcattgggcacttattattattcaccttatgaatgccaattagaaatctgcatattttggtctttattttaccagtctaataattaagtttctataagtaaaaattttccaacaaacaaaagacatgaagctttacaatgagaaacaagttttactgcagtgcctcttgctatttctaagcagtaaactggtccatcacctcttattcattttagataaggtaatcatatacaagtacaattccacgtggcaaaatcagggagatcttgcgctgaaagtgctggaacagcagctggtggctaagagccccagccctgcaggaagtcaagagtcataactcctcgggaacagatgctgtgggtgcagcagagaggagttctgggaaaaggagcatgcacgggaccacaggacagagtattaatagaaaagaaaacttaaacaacaaggttacaggttacatgttattttaaaaatgcttcaagaaatgtgcaacagacacaagcctctcataaacagttctgtggtataattctgacctgcaattactttatacaatgatttaaacagaaaacatgtacaatgaaatgtatttgttcatgaaacaaagggcacctgagtgcatgcacacacacagataacatacagagcatcatggctttctttacttgaacaacgaattttcgagtttaaatcttagtgttctccagttcattaaagattttcaaatctttataaatcaatattaatgctggggaaaaaaaaccttaaaagatcaaagtcctaaaagtcaacagcatgcatgcagcaccaaggtcatatacaattcaggaaaaaaagtattcaaattttgtctggtaaaacaaaggggttgcacagaaacagtttgttccacattgactggtcgtgttataacagctgctgtattctagtccttcatccagcaagtcaatgggctgaaatatcaggcatgactggcatttcaatccactctaatacaccactaggttcaataggatactcaaggattgatgtagctggtgccaatgtgtaggggtactcatagggtgtatagattaaaccagcttcgggccctggaggaactattgcagcagttgggtgaggagttccgtttggcatgacagcggtctgtatttgtctgatcaaaggcattatggtagggccagctggcgtaggagtacgcagggcagctggtgggagaaccggcgcaggcccagtaatgatccttggagcagcctgggctgttggtgatttaatgttggcatctctgtaggtgccattcagaatcgcaagctccatcagctgcatcttcttcaggctgtcttctccttctgctgcaggtaccaataatttcttcacttcttcaactgctctcttcaatttgatttctgctctgttctgagcatcttccacagtgattagtacatgtaaatcttcatttagatgctcccaattgggcttgcctctattttgctcctccttttttttatccctcattgagcctttgcctcggaccatgattttacatccggtttctgcttcaagttgtttggctgtaagtcctctaggtccaaggattctcccaacaaaattaaaatctgggtattcttttacaggcacataaagtttctcttgtaactgaacaataggtcccacagcatcaggcaattctgcactccttttctctgtactgccatttaatgtgtcattgtacatgtctttccgtactctgctaatttcttcgtccagcagccgctcgaggtggttgaagatcccgcagaagttgggcaggctgctcatgagcttcttgtcgttcatcagctgcatcaggtaatctggggtgggcttcggcttctccttcgtttccatttccccgaccatattccaggctccgcagctcactccgcccgccgccgccgccgccgccgccggagaggag

SEQ ID NO: 16957 - RNA, 7337 nt, Homo sapiens
  source 1..7337: mol_type = other RNA
taggcctttagatcacttaaactacagataaaattagatgtgtagcacatatttctaaaatattgtccatattttttccattttaaataaaggtattaaggaattcgtgacaatgtaaaaaactactctatgcacttagaaaaattgtgaattcgaaaagttggagaataatttttgctaaataaataatcatttggcagtaagttctattctacctaaaataatttgcttgaaatgctgtaacagctacttcttatcaaggaataaagacaggcatcacatcctggtcaaacatgcaaaaccactcccaccccaccccatcctaaaactaaagaaaccttaggctgtcacacgtgaaagtgttatgacatatatatatacacacacgtatatatatgaagagtcttgatttggtagtgagcaatttcatttaaacctatcgtttgcttttggcacactaaaaaattcagatccttatgtagtgtttagaaaaccataaccagacaccgattgtgtgtacgtatgcacatcctggttttatgggcagggtgccttcgtgacctcttacacctggagctactgcactggtgcgtatgggagtaactactttcatgttaagttttccctgacattttgcctaaaggaaaagtttaaggacattaatttcaccaacttcttgactgaaagctcagctttcaactgttttgtcaaatagtttcaatcaatcaactgactctagaattttactattcttggaatttggtagtttcatgtttaatattgtaacctgtataaaaatgaaatctgtaatgttattttcgccttttaaaacttttttacatttcctacataaaaggcagcaatgacataattatacataaagtacccttaactgaaaatgagatgaggctgcattcataggcttcagagaatagtaaattgcatagaaattcatcaatttaagttacatggtaccatgacaacttgtatattagcagcttgacagacagcttcgaattttcacagactactacatgaactgttatggcaacggaaacttttacaaatagtagcatgttaaaagacctgtccacctaacagtacactacccaccgctcccatcagagacatgacacggtttgtttacatgatccaaatgaccatctcaatggtgattcgctgttatcactcacatcagctaacactactctgtgtatttatatgtgtgtatacatatttatgaaatgagaatacctggacagtctgattggttaacagcgtattggtacagttttgtcttctattacatgtcattcatttcagccctcaattttagaactctaaataaataaaatgtaatttacaaagataaattgttatttacaaatgcaaaaattcatcctgaggattttggtatctaggagaactgtttcacagaaaaaagcaagtatcaatctgtgaaataaaaatgcaccttgagttaaactaaataattcataattacaggttaatttacccaagttccagccaagaaaagcatgaagatatttaagaaatcttaaattgatttgcatgcaagaaattaatcacatacaacttttcaaatcccaatgttattcccccttaaacttcttgtttaatgttttagtctgactgtatttgtaaagtaggtgacagagaaaaaaatacctgaggaaagctcagtaacgtgctgagggttcttttcctcactggaaagcagcggggcttcaggccaccatgagaaacagccagtgggcctttgactttacccaagttaagctcccctaataggagtagttagctaaacaagttcaacgctttccaaaggaaaaaggtcaagttaaaacaaaaatctaaataaaggtaaaatatcaacagtttctctgctttacaatgtgaccataaaattacttatttacagaaattaaaagaaatggttcaacaaagaatcaaactggtttctccaggtatataccatgacaatgtatctttttactcgatgctgtgagcagacagtgattattttggagaaggaaaaataaggtgtggaattagtaatgcagatgctgaaaggcaagtggcaagagaagaatgcctcaaacaaaggctactttgttcccatctctactgcacctacacccacacccgccccggcccccaagctaaaagaccagaataaccaaagccattttaacagtagtgtgcaaaactgtcagctgacaaacaacataaaaacaagtcacactatgttatctgtggtcacgttcttcagggttagtccagtaactcaagactttacattcttttgtctttatttgtttattttaattaaacatataaaggttaataaacagacaaagtccagagttagtaggttggtattataacatttattaaaataatgctgtgggttaatagaaacagcaaagaaccaaagaattaaaatgcaagctatgtaaaatcccaactaaaacccaaaagtgtctaatgtattcattcattagctaactaaaagcccaaaaaagacaagacacccaatataataaagtactgcaaaacaattggcaattttcagttatcaaaattgtggattttgcattttgtatccttttctcaatcaagaaaaaaattctttttgaatgttatataacatacatataaaacaagatagaaaaatacattataaacttgtaacaatggctgtaaatacattatcttacatgtttctcataggcaataggttggttatggtacatacatagcatgaaactaagataataaagaatagacaaaaatacatgtcagctgtacgataacatacaagcgacactcccatctacccacgctaaaaaattacataatactgtcagaaaaaaagtcttaaaaactacatattttaataagaaataaattcaataaagaatgataatactgagaaccaaggcattcagagatttcaaaagtcatgcttttttcagttgatccaaaattttgtcaaccaagttttcaaaagtttgttcagagccaacattccctataaatgtcacacatttattatttcatacatttactttcttccccataaaagacctttgataaacatctaaaatgtccaggtataacatagttgagatgaaactggatcaaatactggtattgtttttaacaactatcacctcaagtgtttgagtgtcgcaaatttattcaaccaaccaaacaatataaaaatcaaaatggcacagcatatattgtaaataaatcaaaactgtatgtgtaacagaaagacaaagcagtggcatattaaaccaaagctagctggatacaaaacaatgaatgtctattgcatagtaaataaactgacaacggtttccaagtgagacaagatggtgggggaggtcaccaagaaggtaatgactcagcttcctgctgacctctgactgtgatgctgggaaggtgtggaagaggggacgagttgataagctgggcgggggggggggtccactgtcacttgagatttgccacgtctggtactgagcagttaatgattattcactcaagtgtttagatgtaggctttgcacacaaattgcttcaactacataactaactgtttcaacttcttgagaaattagaagcttaagctgaaatgtggttgagtatttatatgcactatgatgctagtttttcacattcttttaaagttaaggggtgggggaggcagaggttattgaaacagtaaaaggatacactacaccagttatctggtatgatataaagacatgtgattaaatttgggtgatttaaaacattgttttctagaatgaaaatcacaaagattcacttttgtgaaaacatttgctaggtatcctattatattcaattaattaaaaacaaaaaacaaaatcaaatgaatgcatcccccttctccaaataaaacaaagctctaattttgtctgtaaactgaagtttagatgacacataatttttatctcagaatcctttgggttaacattgaagattggaataaccaaaagtattaaactattcttttaaagaatgatgttttaaaacttactagtcaggcattagaaaagttatcaaatcttttcacagtatcagatttggcaaatttgcatcaaggtaacgtggcaaaaatcctataattcaaactatcaactcatttgtctccctcatatcttctttcacatactgggcgactgagtaacatgcattaacttgtattctgagggaggagctgatctttatgagacacttgactgaatgaccatgaaggaaaataaggcactttcttttctttagacttattccaatacttaaaaaataaaaaagaaagacaaaaaggctcttttggtcttttgtttcttgacaaccaccagaaaaaatcatttaatgaaataaagggtttctttgttctttttctttttttttataacacttgaaagtataaaatgctacatttccaaaaatatatatatttttttctgcaccagcacccttgtatagtaaaagtatctactttttgttcatttgtttcaatgcactacactttatctacaatttcattacatgtatacagcaaataggcaagcatggcttttacatccttaatgatttttttctatacagggaggtttaaaaaaaaatacttgaacagtttgcccagtaatgtgacacataatgcatgtaccttgttctcatatttttttaggtgtaaaataaagattcagtaattttaactcagatatttatctttttaaaaatagtgttgcagttttgttatttgcattacttttcaaaactccttaagtttttctctcatggcacactttcttctaatacttcaaattttggcaggcaatataaaaaaggctgcaacttctgccctttgagggcactgtagtgactaaacagcatatcaaattttgaatactttttgaaatcacttcaccaatgatatccctgaccgaaggttcatgcatgatgcatcatcacacagtacattcagagagagctttgacttcgctatgagaagaaaaagattcctagaagtctctcacagtaactgcctctgtcattgagtagttaaggaccatctgtctccccttcttaagagaggccttcttaccgttcgcttagggtgggatattaaaagatgatcagtgctgtgggatgaattgggccttattgctttactactattcagtgcagtttctagaaccactttcacccaaacaggaaaaaaaaaaaaaaaaagctgagttggaggacaacaatttctttgtcttttgtttggttagatggtaagacgaacggacaagtgcctcagctcgctgcactgacgacaggcaagcaaaggcgattaccagttaactgatcagcaggcaggcatggtcaggtcatcattgggtgaagagttcagaggtcagaaggtcataggttagttgccggtggcggctcggtctgcggtcacaatcctttggtaaggatggacacgcatatcgtgccttcgaactttagtagccaccgcacctagttaaattgcaattaccaagacaaagttagaaaacattcacaaggggggaaaaaacattaacagcaggtttatcaaaatggatttcaaatgttcatttactacaaaagtttaagaaacacgttaaggcacagtagttttaaaattaaccacaatatgtcatgtatatatgcatctattaatattgcattcatttcaaacatcttgggccttaacctattgtatccattcatttacaatccccaagttacagtatttcatgagctctattagatccaaacatatttaagctttactagtcacatattcactgaagtgcctttcttgcagcaggactacttaaataacgccatgtttaatacagacaattatttgctaaccttaagaccacttcaagagtttatcacttaaaaaggtttaaaagcaattcttaaagcctacagattgtggttttaaactctgagtcaataagtatgaactgcaatgaattaggtgattagtaaagcaaacagtatagtacacttagcagtcagtatactactatacactcctttataaattaccattactgtgtaatattacagactaaaccaaattaataacataattttactttatatctatgtgcaaaaagtgcaagtaagtcactgactgctaggctaagcttttttcccccggaggctgctgagactaagcatttgttaaattcagatctgatgagggttcagttaagaccgttcttgaattcttagcctttcgttgggaaagccatacctaatacaccactaggttcaataggatactcaaggattgatgtagctggtgccaatgtgtaggggtactcatagggtgtatagattaaaccagcttcgggccctggaggaactattgcagcagttgggtgaggagttccgtttggcatgacagcggtctgtatttgtctgatcaaaggcattatggtagggccagctggcgtaggagtacgcagggcagctggtgggagaaccggcgcaggcccagtaatgatccttggagcagcctgggctgttgctgcaagagaaaaggcaagggctggtgatttaatgttggcatctctgtaggtgccattcagaatcgcaagctccatcagctgcatcttcttcaggctgtcttctccttctgctgcaggtaccaataatttcttcacttcttcaactgctctcttcaatttgatttctgctctgttctgagcatcttccacagtgattagtacatgtaaatcttcatttagatgctcccaattgggcttgcctctattttgctcctccttttttttatccctcattgagcctttgcctcggaccatgattttacatccggtttctgcttcaagttgtttggctgtaagtcctctaggtccaaggattctcccaacaaaattaaaatctgggtattcttttacaggcacataaagtttctcttgtaactgaacaataggtcccacagcatcaggcaattctgcactccttttctctgtactgccatttaatgtgtcattgtacatgtctttccgtactctgctaatttcttcgtccagcagccgctcgaggtggttgaagatcccgcagaagttgggcaggctgctcatgagcttcttgtcgttcatcagctgcatcaggtaatctggggtgggcttcggcttctccttcgtttccatttccccgaccatattccaggctccgcagctcactccgcccgccgccgccgccgccgccgccggagaggag

SEQ ID NO: 16958 - RNA, 7334 nt, Homo sapiens
  source 1..7334: mol_type = other RNA
taggcctttagatcacttaaactacagataaaattagatgtgtagcacatatttctaaaatattgtccatattttttccattttaaataaaggtattaaggaattcgtgacaatgtaaaaaactactctatgcacttagaaaaattgtgaattcgaaaagttggagaataatttttgctaaataaataatcatttggcagtaagttctattctacctaaaataatttgcttgaaatgctgtaacagctacttcttatcaaggaataaagacaggcatcacatcctggtcaaacatgcaaaaccactcccaccccaccccatcctaaaactaaagaaaccttaggctgtcacacgtgaaagtgttatgacatatatatatacacacacgtatatatatgaagagtcttgatttggtagtgagcaatttcatttaaacctatcgtttgcttttggcacactaaaaaattcagatccttatgtagtgtttagaaaaccataaccagacaccgattgtgtgtacgtatgcacatcctggttttatgggcagggtgccttcgtgacctcttacacctggagctactgcactggtgcgtatgggagtaactactttcatgttaagttttccctgacattttgcctaaaggaaaagtttaaggacattaatttcaccaacttcttgactgaaagctcagctttcaactgttttgtcaaatagtttcaatcaatcaactgactctagaattttactattcttggaatttggtagtttcatgtttaatattgtaacctgtataaaaatgaaatctgtaatgttattttcgccttttaaaacttttttacatttcctacataaaaggcagcaatgacataattatacataaagtacccttaactgaaaatgagatgaggctgcattcataggcttcagagaatagtaaattgcatagaaattcatcaatttaagttacatggtaccatgacaacttgtatattagcagcttgacagacagcttcgaattttcacagactactacatgaactgttatggcaacggaaacttttacaaatagtagcatgttaaaagacctgtccacctaacagtacactacccaccgctcccatcagagacatgacacggtttgtttacatgatccaaatgaccatctcaatggtgattcgctgttatcactcacatcagctaacactactctgtgtatttatatgtgtgtatacatatttatgaaatgagaatacctggacagtctgattggttaacagcgtattggtacagttttgtcttctattacatgtcattcatttcagccctcaattttagaactctaaataaataaaatgtaatttacaaagataaattgttatttacaaatgcaaaaattcatcctgaggattttggtatctaggagaactgtttcacagaaaaaagcaagtatcaatctgtgaaataaaaatgcaccttgagttaaactaaataattcataattacaggttaatttacccaagttccagccaagaaaagcatgaagatatttaagaaatcttaaattgatttgcatgcaagaaattaatcacatacaacttttcaaatcccaatgttattcccccttaaacttcttgtttaatgttttagtctgactgtatttgtaaagtaggtgacagagaaaaaaatacctgaggaaagctcagtaacgtgctgagggttcttttcctcactggaaagcagcggggcttcaggccaccatgagaaacagccagtgggcctttgactttacccaagttaagctcccctaataggagtagttagctaaacaagttcaacgctttccaaaggaaaaaggtcaagttaaaacaaaaatctaaataaaggtaaaatatcaacagtttctctgctttacaatgtgaccataaaattacttatttacagaaattaaaagaaatggttcaacaaagaatcaaactggtttctccaggtatataccatgacaatgtatctttttactcgatgctgtgagcagacagtgattattttggagaaggaaaaataaggtgtggaattagtaatgcagatgctgaaaggcaagtggcaagagaagaatgcctcaaacaaaggctactttgttcccatctctactgcacctacacccacacccgccccggcccccaagctaaaagaccagaataaccaaagccattttaacagtagtgtgcaaaactgtcagctgacaaacaacataaaaacaagtcacactatgttatctgtggtcacgttcttcagggttagtccagtaactcaagactttacattcttttgtctttatttgtttattttaattaaacatataaaggttaataaacagacaaagtccagagttagtaggttggtattataacatttattaaaataatgctgtgggttaatagaaacagcaaagaaccaaagaattaaaatgcaagctatgtaaaatcccaactaaaacccaaaagtgtctaatgtattcattcattagctaactaaaagcccaaaaaagacaagacacccaatataataaagtactgcaaaacaattggcaattttcagttatcaaaattgtggattttgcattttgtatccttttctcaatcaagaaaaaaattctttttgaatgttatataacatacatataaaacaagatagaaaaatacattataaacttgtaacaatggctgtaaatacattatcttacatgtttctcataggcaataggttggttatggtacatacatagcatgaaactaagataataaagaatagacaaaaatacatgtcagctgtacgataacatacaagcgacactcccatctacccacgctaaaaaattacataatactgtcagaaaaaaagtcttaaaaactacatattttaataagaaataaattcaataaagaatgataatactgagaaccaaggcattcagagatttcaaaagtcatgcttttttcagttgatccaaaattttgtcaaccaagttttcaaaagtttgttcagagccaacattccctataaatgtcacacatttattatttcatacatttactttcttccccataaaagacctttgataaacatctaaaatgtccaggtataacatagttgagatgaaactggatcaaatactggtattgtttttaacaactatcacctcaagtgtttgagtgtcgcaaatttattcaaccaaccaaacaatataaaaatcaaaatggcacagcatatattgtaaataaatcaaaactgtatgtgtaacagaaagacaaagcagtggcatattaaaccaaagctagctggatacaaaacaatgaatgtctattgcatagtaaataaactgacaacggtttccaagtgagacaagatggtgggggaggtcaccaagaaggtaatgactcagcttcctgctgacctctgactgtgatgctgggaaggtgtggaagaggggacgagttgataagctgggcgggggggggggtccactgtcacttgagatttgccacgtctggtactgagcagttaatgattattcactcaagtgtttagatgtaggctttgcacacaaattgcttcaactacataactaactgtttcaacttcttgagaaattagaagcttaagctgaaatgtggttgagtatttatatgcactatgatgctagtttttcacattcttttaaagttaaggggtgggggaggcagaggttattgaaacagtaaaaggatacactacaccagttatctggtatgatataaagacatgtgattaaatttgggtgatttaaaacattgttttctagaatgaaaatcacaaagattcacttttgtgaaaacatttgctaggtatcctattatattcaattaattaaaaacaaaaaacaaaatcaaatgaatgcatcccccttctccaaataaaacaaagctctaattttgtctgtaaactgaagtttagatgacacataatttttatctcagaatcctttgggttaacattgaagattggaataaccaaaagtattaaactattcttttaaagaatgatgttttaaaacttactagtcaggcattagaaaagttatcaaatcttttcacagtatcagatttggcaaatttgcatcaaggtaacgtggcaaaaatcctataattcaaactatcaactcatttgtctccctcatatcttctttcacatactgggcgactgagtaacatgcattaacttgtattctgagggaggagctgatctttatgagacacttgactgaatgaccatgaaggaaaataaggcactttcttttctttagacttattccaatacttaaaaaataaaaaagaaagacaaaaaggctcttttggtcttttgtttcttgacaaccaccagaaaaaatcatttaatgaaataaagggtttctttgttctttttctttttttttataacacttgaaagtataaaatgctacatttccaaaaatatatatatttttttctgcaccagcacccttgtatagtaaaagtatctactttttgttcatttgtttcaatgcactacactttatctacaatttcattacatgtatacagcaaataggcaagcatggcttttacatccttaatgatttttttctatacagggaggtttaaaaaaaaatacttgaacagtttgcccagtaatgtgacacataatgcatgtaccttgttctcatatttttttaggtgtaaaataaagattcagtaattttaactcagatatttatctttttaaaaatagtgttgcagttttgttatttgcattacttttcaaaactccttaagtttttctctcatggcacactttcttctaatacttcaaattttggcaggcaatataaaaaaggctgcaacttctgccctttgagggcactgtagtgactaaacagcatatcaaattttgaatactttttgaaatcacttcaccaatgatatccctgaccgaaggttcatgcatgatgcatcatcacacagtacattcagagagagctttgacttcgctatgagaagaaaaagattcctagaagtctctcacagtaactgcctctgtcattgagtagttaaggaccatctgtctccccttcttaagagaggccttcttaccgttcgcttagggtgggatattaaaagatgatcagtgctgtgggatgaattgggccttattgctttactactattcagtgcagtttctagaaccactttcacccaaacaggaaaaaaaaaaaaaaaaagctgagttggaggacaacaatttctttgtcttttgtttggttagatggtaagacgaacggacaagtgcctcagctcgctgcactgacgacaggcaagcaaaggcgattaccagttaactgatcagcaggcaggcatggtcaggtcatcattgggtgaagagttcagaggtcagaaggtcataggttagttgccggtggcggctcggtctgcggtcacaatcctttggtaaggatggacacgcatatcgtgccttcgaactttagtagccaccgcacctagttaaattgcaattaccaagacaaagttagaaaacattcacaaggggggaaaaaacattaacagcaggtttatcaaaatggatttcaaatgttcatttactacaaaagtttaagaaacacgttaaggcacagtagttttaaaattaaccacaatatgtcatgtatatatgcatctattaatattgcattcatttcaaacatcttgggccttaacctattgtatccattcatttacaatccccaagttacagtatttcatgagctctattagatccaaacatatttaagctttactagtcacatattcactgaagtgcctttcttgcagcaggactacttaaataacgccatgtttaatacagacaattatttgctaaccttaagaccacttcaagagtttatcacttaaaaaggtttaaaagcaattcttaaagcctacagattgtggttttaaactctgagtcaataagtatgaactgcaatgaattaggtgattagtaaagcaaacagtatagtacacttagcagtcagtatactactatacactcctttataaattaccattactgtgtaatattacagactaaaccaaattaataacataattttactttatatctatgtgcaaaaagtgcaagtaagtcactgactgctaggctaagcttttttcccccggaggctgctgagactaagcatttgttaaattcagatctgatgagggttcagttaagaccgttcttgaattcttagcctttcgttgggaaagccatacctaatacaccactaggttcaataggatactcaaggattgatgtagctggtgccaatgtgtaggggtactcatagggtgtatagattaaaccagcttcgggccctggaggaactattgcagcagttgggtgaggagttccgtttggcatgacagcggtctgtatttgtctgatcaaaggcattatggtagggccagctggcgtaggagtacgcagggcagctggtgggagaaccggcgcaggcccagtaatgatccttggagcagcctgggctgttgctgcaagagaaaaggcaaggggtgatttaatgttggcatctctgtaggtgccattcagaatcgcaagctccatcagctgcatcttcttcaggctgtcttctccttctgctgcaggtaccaataatttcttcacttcttcaactgctctcttcaatttgatttctgctctgttctgagcatcttccacagtgattagtacatgtaaatcttcatttagatgctcccaattgggcttgcctctattttgctcctccttttttttatccctcattgagcctttgcctcggaccatgattttacatccggtttctgcttcaagttgtttggctgtaagtcctctaggtccaaggattctcccaacaaaattaaaatctgggtattcttttacaggcacataaagtttctcttgtaactgaacaataggtcccacagcatcaggcaattctgcactccttttctctgtactgccatttaatgtgtcattgtacatgtctttccgtactctgctaatttcttcgtccagcagccgctcgaggtggttgaagatcccgcagaagttgggcaggctgctcatgagcttcttgtcgttcatcagctgcatcaggtaatctggggtgggcttcggcttctccttcgtttccatttccccgaccatattccaggctccgcagctcactccgcccgccgccgccgccgccgccgccggagaggag

SEQ ID NO: 16959 - RNA, 12932 nt, Homo sapiens
  source 1..12932: mol_type = other RNA
taggcctttagatcacttaaactacagataaaattagatgtgtagcacatatttctaaaatattgtccatattttttccattttaaataaaggtattaaggaattcgtgacaatgtaaaaaactactctatgcacttagaaaaattgtgaattcgaaaagttggagaataatttttgctaaataaataatcatttggcagtaagttctattctacctaaaataatttgcttgaaatgctgtaacagctacttcttatcaaggaataaagacaggcatcacatcctggtcaaacatgcaaaaccactcccaccccaccccatcctaaaactaaagaaaccttaggctgtcacacgtgaaagtgttatgacatatatatatacacacacgtatatatatgaagagtcttgatttggtagtgagcaatttcatttaaacctatcgtttgcttttggcacactaaaaaattcagatccttatgtagtgtttagaaaaccataaccagacaccgattgtgtgtacgtatgcacatcctggttttatgggcagggtgccttcgtgacctcttacacctggagctactgcactggtgcgtatgggagtaactactttcatgttaagttttccctgacattttgcctaaaggaaaagtttaaggacattaatttcaccaacttcttgactgaaagctcagctttcaactgttttgtcaaatagtttcaatcaatcaactgactctagaattttactattcttggaatttggtagtttcatgtttaatattgtaacctgtataaaaatgaaatctgtaatgttattttcgccttttaaaacttttttacatttcctacataaaaggcagcaatgacataattatacataaagtacccttaactgaaaatgagatgaggctgcattcataggcttcagagaatagtaaattgcatagaaattcatcaatttaagttacatggtaccatgacaacttgtatattagcagcttgacagacagcttcgaattttcacagactactacatgaactgttatggcaacggaaacttttacaaatagtagcatgttaaaagacctgtccacctaacagtacactacccaccgctcccatcagagacatgacacggtttgtttacatgatccaaatgaccatctcaatggtgattcgctgttatcactcacatcagctaacactactctgtgtatttatatgtgtgtatacatatttatgaaatgagaatacctggacagtctgattggttaacagcgtattggtacagttttgtcttctattacatgtcattcatttcagccctcaattttagaactctaaataaataaaatgtaatttacaaagataaattgttatttacaaatgcaaaaattcatcctgaggattttggtatctaggagaactgtttcacagaaaaaagcaagtatcaatctgtgaaataaaaatgcaccttgagttaaactaaataattcataattacaggttaatttacccaagttccagccaagaaaagcatgaagatatttaagaaatcttaaattgatttgcatgcaagaaattaatcacatacaacttttcaaatcccaatgttattcccccttaaacttcttgtttaatgttttagtctgactgtatttgtaaagtaggtgacagagaaaaaaatacctgaggaaagctcagtaacgtgctgagggttcttttcctcactggaaagcagcggggcttcaggccaccatgagaaacagccagtgggcctttgactttacccaagttaagctcccctaataggagtagttagctaaacaagttcaacgctttccaaaggaaaaaggtcaagttaaaacaaaaatctaaataaaggtaaaatatcaacagtttctctgctttacaatgtgaccataaaattacttatttacagaaattaaaagaaatggttcaacaaagaatcaaactggtttctccaggtatataccatgacaatgtatctttttactcgatgctgtgagcagacagtgattattttggagaaggaaaaataaggtgtggaattagtaatgcagatgctgaaaggcaagtggcaagagaagaatgcctcaaacaaaggctactttgttcccatctctactgcacctacacccacacccgccccggcccccaagctaaaagaccagaataaccaaagccattttaacagtagtgtgcaaaactgtcagctgacaaacaacataaaaacaagtcacactatgttatctgtggtcacgttcttcagggttagtccagtaactcaagactttacattcttttgtctttatttgtttattttaattaaacatataaaggttaataaacagacaaagtccagagttagtaggttggtattataacatttattaaaataatgctgtgggttaatagaaacagcaaagaaccaaagaattaaaatgcaagctatgtaaaatcccaactaaaacccaaaagtgtctaatgtattcattcattagctaactaaaagcccaaaaaagacaagacacccaatataataaagtactgcaaaacaattggcaattttcagttatcaaaattgtggattttgcattttgtatccttttctcaatcaagaaaaaaattctttttgaatgttatataacatacatataaaacaagatagaaaaatacattataaacttgtaacaatggctgtaaatacattatcttacatgtttctcataggcaataggttggttatggtacatacatagcatgaaactaagataataaagaatagacaaaaatacatgtcagctgtacgataacatacaagcgacactcccatctacccacgctaaaaaattacataatactgtcagaaaaaaagtcttaaaaactacatattttaataagaaataaattcaataaagaatgataatactgagaaccaaggcattcagagatttcaaaagtcatgcttttttcagttgatccaaaattttgtcaaccaagttttcaaaagtttgttcagagccaacattccctataaatgtcacacatttattatttcatacatttactttcttccccataaaagacctttgataaacatctaaaatgtccaggtataacatagttgagatgaaactggatcaaatactggtattgtttttaacaactatcacctcaagtgtttgagtgtcgcaaatttattcaaccaaccaaacaatataaaaatcaaaatggcacagcatatattgtaaataaatcaaaactgtatgtgtaacagaaagacaaagcagtggcatattaaaccaaagctagctggatacaaaacaatgaatgtctattgcatagtaaataaactgacaacggtttccaagtgagacaagatggtgggggaggtcaccaagaaggtaatgactcagcttcctgctgacctctgactgtgatgctgggaaggtgtggaagaggggacgagttgataagctgggcgggggggggggtccactgtcacttgagatttgccacgtctggtactgagcagttaatgattattcactcaagtgtttagatgtaggctttgcacacaaattgcttcaactacataactaactgtttcaacttcttgagaaattagaagcttaagctgaaatgtggttgagtatttatatgcactatgatgctagtttttcacattcttttaaagttaaggggtgggggaggcagaggttattgaaacagtaaaaggatacactacaccagttatctggtatgatataaagacatgtgattaaatttgggtgatttaaaacattgttttctagaatgaaaatcacaaagattcacttttgtgaaaacatttgctaggtatcctattatattcaattaattaaaaacaaaaaacaaaatcaaatgaatgcatcccccttctccaaataaaacaaagctctaattttgtctgtaaactgaagtttagatgacacataatttttatctcagaatcctttgggttaacattgaagattggaataaccaaaagtattaaactattcttttaaagaatgatgttttaaaacttactagtcaggcattagaaaagttatcaaatcttttcacagtatcagatttggcaaatttgcatcaaggtaacgtggcaaaaatcctataattcaaactatcaactcatttgtctccctcatatcttctttcacatactgggcgactgagtaacatgcattaacttgtattctgagggaggagctgatctttatgagacacttgactgaatgaccatgaaggaaaataaggcactttcttttctttagacttattccaatacttaaaaaataaaaaagaaagacaaaaaggctcttttggtcttttgtttcttgacaaccaccagaaaaaatcatttaatgaaataaagggtttctttgttctttttctttttttttataacacttgaaagtataaaatgctacatttccaaaaatatatatatttttttctgcaccagcacccttgtatagtaaaagtatctactttttgttcatttgtttcaatgcactacactttatctacaatttcattacatgtatacagcaaataggcaagcatggcttttacatccttaatgatttttttctatacagggaggtttaaaaaaaaatacttgaacagtttgcccagtaatgtgacacataatgcatgtaccttgttctcatatttttttaggtgtaaaataaagattcagtaattttaactcagatatttatctttttaaaaatagtgttgcagttttgttatttgcattacttttcaaaactccttaagtttttctctcatggcacactttcttctaatacttcaaattttggcaggcaatataaaaaaggctgcaacttctgccctttgagggcactgtagtgactaaacagcatatcaaattttgaatactttttgaaatcacttcaccaatgatatccctgaccgaaggttcatgcatgatgcatcatcacacagtacattcagagagagctttgacttcgctatgagaagaaaaagattcctagaagtctctcacagtaactgcctctgtcattgagtagttaaggaccatctgtctccccttcttaagagaggccttcttaccgttcgcttagggtgggatattaaaagatgatcagtgctgtgggatgaattgggccttattgctttactactattcagtgcagtttctagaaccactttcacccaaacaggaaaaaaaaaaaaaaaaagctgagttggaggacaacaatttctttgtcttttgtttggttagatggtaagacgaacggacaagtgcctcagctcgctgcactgacgacaggcaagcaaaggcgattaccagttaactgatcagcaggcaggcatggtcaggtcatcattgggtgaagagttcagaggtcagaaggtcataggttagttgccggtggcggctgggtggttagaaacaaaaaaaaacaaaacaaaaaaaagaaaagaaaagatagagaagagattagtttcagctagtgacggcttaatgacaacatgaaaaactaatcacaactaataaaaaaaaaagcatgtttaattctgacaaactgattgacaccatctacagaatacaattaaaatcatgacaatttcgtatcatgatttgaacaaatgaagaagagcccactcccacaaaaaaaaaaaaaaaactggttaacaagaaaaaatagaaataaaatacaactaacaactaatagttagtagcagtcaatgaaggaaattgaaaaacaacaatgaataggtttggtatacagaatttttaaacagtcagtgcagttatcagtatctgactgctattaagcattagtattctctaagatgcaagcattaaagcaactattaatgatggatgtgattattaataactgatgattaacagaaatgaatctaaagaaattcaaaattctatgaaccatttggttcaacataaactctgggccaaacaaggtttcttttgttcaataaatgtttattgctttttcaattattctatttacaaacaacatggaatttcttggcctcatgatacaaagcgatactaaactgtagtctagcagtgtaggcaacatcatgggaaccagaaaatggccaggccttttgcactagccaacactttccagttgaaaatactattttacacatatagaacacttataaaatgcacttgcatgtaaacactgtaaaatcctgccatttaaaattctacactcaaaaagctctaagtacatcaaaaaatagaagaaatttctaattgataccaataaggcattttaaaactacaaacagctttctttattcaatttcaaagctaatactctgcaaatacaataaaatctgacatttcatatacattcctgctttatatttttatattttaaaagaagccacctgtaaatactattttcttttgcaaaataacaaaaaggacaaaaaaactttaaaaattacagtaaaacataaagtagttctcaagtggaaaagttatcattcccaatgtccttgagttgttccttccttaatcaacctttgtcacattctgcttcaccaaacttggtccacttaacagtagtataatttttaagactcattcaacagcttaattatttctactatattctgaggtttgatagaattttctgtactgttgccattgtgactaaggcagaggagatgtgaatgaaaagatattcagtgcaaagttagattctgtgccacttcataaatcaaagcccagaaggtgtaatgttcagtttaaatgatccaaaataatggactgatttaccttcatatgacaaaaatgttttctatagtctatcatttagaacagtttataaatactacaaaaatactgtatcttcaatgtgaccaaatcttccctgaatttcttaaaagtggaattttatttaaaataaaaattgctgctccaaaatcatagaagaaaataaatatttaacatgatgtagtcatactacttcacaggtattccaaaatatagaatcttaaagcatttttgatgttactcatagttttgattaaaactgtttaaagtttcttatacaaattatgtaagtgatggtttttgtattactcagaaaaaactctgacttcttttctgagtgtggaatatataaacgaagtgagtgaccatttatatataccaggacacctagactacatcctctgccaagtcttggcctcctacacaggtgtgtcaccatgcaagaccatacagttcattacaactaaaaggtcagttggtctctaataggcttcaaattcagttttgaaatatatataaagaggtgagtttacttttagtaaagaactagatattggtcaaccatgtagtactctaaacgttcatatagaattacatggttatatgtccaagggctgagtttttttgcattaaatgaatgcttatactaataaacttctcttcaaaatatttttttaaaataattttaacctcaaaaatagagaaaacagtagtatcataaaataatttaagtgaaggacttcagacatctcccttagacccaatgagtgcatacagtgataagtatacgagtactctgttactaaaaaagaaatgagcatttcggtttgctgacactgcattttaaataaaaacagtgacaggactaatcaaaacacgtaactacaaaagatccatgcatggaatgtgtcgtaattttccaaatacaataaaatcttcctaaaatatgtccaactatctcaaggcactggagtattaagtaggccaataattattgtgttaaagcaaaatggtgagaaatctcctaaaagggggcatacatagggaaagattagctgggggaaaaaaactactttaaaatactctttagaacaattgtagacattagcaatatgaataaaacctcaaattattcatggaattgtccagtttctttaaaactcaagtgactttccaaaaaacttccccatccctatgagacgtgctcatacagaacacttacaaggaataccatcctcatagacgaccacggagctggggtctattttgttcactgaacaatcactgttagtgatgaatacattagtttaaaagtcttcaacgttctttatggattatgctaaacaaatattaacaatgtctttgggaaaggcatgttatttctgatgtggacaacagctgtgtctagtatttatcatcagtactcaaggtaatcacataaagcaggtaggtccttcataaattcatagaagatgtacaattgaagtacaaatccagcactttttcctccactaatatttgagactttgatcaatttaatttgtaggaaacaaatgtgccataatagaaacttgtaaaaaatccttttttactaccatgcttgatattcctatcttgtgatggaaaaacttagaaaacaattcaatgtcaataaaccgaaaataccattcctcaataagcaaaaataatttataaaagggtccaagggcatatacaggacacaaattataaaagttgtaaaggagaaaaatgaagacttattttccagtcacaggttagtcaaaaattatattcacacagctggatctcataccaccacagaacttcaagagacagtttaccttcagataatatattttagcagcaaatgacaaaaatcaaaggatccattttggcaagagaatgtaagaataaaagggaattgacgctctaatttatataaaaaaatccaactacatgaaagttatcttcacagtcctcactttgttgattttagctaagtacttgacatgtgcaccctcatgtttatacagtggctcaaatattttattataaagaaaaatggaaactaaatcttcagttttctccaaaagtacacaggaggcatatattcctttacttctctcattaaagcaccatccgttcaattcattttgcaataccaaccccaaatttcagaacttttaaaaggtaaattttagcaaaagttattaatgaaaataactgaggcaacatcaaaatttaatagctccccaaattgactaatttatgttttagtaggaataaatcatagtacataataatagaagatttaataagttaaaatatgaagggagaaaaaaccaaaccaaaacaaaaaacccaacccttaaatctgtcaatgatcacaaacaaatttagaaaaggaaaaaaaactgtgtgcaggtaagcaattacatttttccatcaggtgtggtgttgcaaattttatggacacccaacgcatttcttatagacaagaactgcagaactaaactaacctcggtctgcggtcacaatcctttggtaaggatggacacgcatatcgtgccttcgaactttagtagccaccgcacctagttaaattgcaattaccaagacaaagttagaaaacattcacaaggggggaaaaaacattaacagcaggtttatcaaaatggatttcaaatgttcatttactacaaaagtttaagaaacacgttaaggcacagtagttttaaaattaaccacaatatgtcatgtatatatgcatctattaatattgcattcatttcaaacatcttgggccttaacctattgtatccattcatttacaatccccaagttacagtatttcatgagctctattagatccaaacatatttaagctttactagtcacatattcactgaagtgcctttcttgcagcaggactacttaaataacgccatgtttaatacagacaattatttgctaaccttaagaccacttcaagagtttatcacttaaaaaggtttaaaagcaattcttaaagcctacagattgtggttttaaactctgagtcaataagtatgaactgcaatgaattaggtgattagtaaagcaaacagtatagtacacttagcagtcagtatactactatacactcctttataaattaccattactgtgtaatattacagactaaaccaaattaataacataattttactttatatctatgtgcaaaaagtgcaagtaagtcactgactgctaggctaagcttttttcccccggaggctgctgagactaagcatttgttaaattcagatctgatgagggttcagttaagaccgttcttgaattcttagcctttcgttgggaaagccatacctaaagataaaaggaagggaattaaaaattagtcatcaatgaagacttgatgctaataccaatctcctcactactaccaacacacatgtctgcatctgttttgaagggcactgcttattttaaaataatttaatgtgagatgtgacataaatagcatgcatgttatctgtgtgcaaatttattataacttagaaatttaaaataattttctgagttctccaagtggtcaatatcatgttttactgcttaggtggcaaagcaagaaatgaaattaaccataatagattttttcattgggcacttattattattcaccttatgaatgccaattagaaatctgcatattttggtctttattttaccagtctaataattaagtttctataagtaaaaattttccaacaaacaaaagacatgaagctttacaatgagaaacaagttttactgcagtgcctcttgctatttctaagcagtaaactggtccatcacctcttattcattttagataaggtaatcatatacaagtacaattccacgtggcaaaatcagggagatcttgcgctgaaagtgctggaacagcagctggtggctaagagccccagccctgcaggaagtcaagagtcataactcctcgggaacagatgctgtgggtgcagcagagaggagttctgggaaaaggagcatgcacgggaccacaggacagagtattaatagaaaagaaaacttaaacaacaaggttacaggttacatgttattttaaaaatgcttcaagaaatgtgcaacagacacaagcctctcataaacagttctgtggtataattctgacctgcaattactttatacaatgatttaaacagaaaacatgtacaatgaaatgtatttgttcatgaaacaaagggcacctgagtgcatgcacacacacagataacatacagagcatcatggctttctttacttgaacaacgaattttcgagtttaaatcttagtgttctccagttcattaaagattttcaaatctttataaatcaatattaatgctggggaaaaaaaaccttaaaagatcaaagtcctaaaagtcaacagcatgcatgcagcaccaaggtcatatacaattcaggaaaaaaagtattcaaattttgtctggtaaaacaaaggggttgcacagaaacagtttgttccacattgactggtcgtgttataacagctgctgtattctagtccttcatccagcaagtcaatgggctgaaatatcaggcatgactggcatttcaatccactctaatacaccactaggttcaataggatactcaaggattgatgtagctggtgccaatgtgtaggggtactcatagggtgtatagattaaaccagcttcgggccctggaggaactattgcagcagttgggtgaggagttccgtttggcatgacagcggtctgtatttgtctgatcaaaggcattatggtagggccagctggcgtaggagtacgcagggcagctggtgggagaaccggcgcaggcccagtaatgatccttggagcagcctgggctgttgctgcaagagaaaaggcaagggctggtgatttaatgttggcatctctgtaggtgccattcagaatcgcaagctccatcagctgcatcttcttcaggctgtcttctccttctgctgcaggtaccaataatttcttcacttcttcaactgctctcttcaatttgatttctgctctgttctgagcatcttccacagtgattagtacatgtaaatcttcatttagatgctcccaattgggcttgcctctattttgctcctccttttttttatccctcattgagcctttgcctcggaccatgattttacatccggtttctgcttcaagttgtttggctgtaagtcctctaggtccaaggattctcccaacaaaattaaaatctgggtattcttttacaggcacataaagtttctcttgtaactgaacaataggtcccacagcatcaggcaattctgcactccttttctctgtactgccatttaatgtgtcattgtacatgtctttccgtactctgctaatttcttcgtccagcagccgctcgaggtggttgaagatcccgcagaagttgggcaggctgctcatgagcttcttgtcgttcatcagctgcatcaggtaatctggggtgggcttcggcttctccttcgtttccatttccccgaccatattccaggctccgcagctcactccgcccgccgccgccgccgccgccgccggagaggagggaggggcgggggcgagccccggccgcgggccgctcgggacccggcgtcccgctccgcgccggctcccgctctggctcccgcgccgagccccggggcggccggcaccgcgcgctcgcccgccccccgcaggcactttccgcccgggcccgacgcgctcccagccgccgccgctctcggccgcccggctcggcgcgtccctcacgaggccggcgggcgggcgggaggcgggtctcggctggccgagtgcgggcgcggggcgcgggctgctggcgccggacgaggaggagccggggccgccgctcgctcggctggtcgagcccgctcagcgccgccgccgcctgtgccgcgggctcggggggtctctctgggctggtccccgccgcggcgcctctgccgctgccgccgcgctccgactgc

SEQ ID NO: 16960 - RNA, 13879 nt, Homo sapiens
  source 1..13879: mol_type = other RNA
taggcctttagatcacttaaactacagataaaattagatgtgtagcacatatttctaaaatattgtccatattttttccattttaaataaaggtattaaggaattcgtgacaatgtaaaaaactactctatgcacttagaaaaattgtgaattcgaaaagttggagaataatttttgctaaataaataatcatttggcagtaagttctattctacctaaaataatttgcttgaaatgctgtaacagctacttcttatcaaggaataaagacaggcatcacatcctggtcaaacatgcaaaaccactcccaccccaccccatcctaaaactaaagaaaccttaggctgtcacacgtgaaagtgttatgacatatatatatacacacacgtatatatatgaagagtcttgatttggtagtgagcaatttcatttaaacctatcgtttgcttttggcacactaaaaaattcagatccttatgtagtgtttagaaaaccataaccagacaccgattgtgtgtacgtatgcacatcctggttttatgggcagggtgccttcgtgacctcttacacctggagctactgcactggtgcgtatgggagtaactactttcatgttaagttttccctgacattttgcctaaaggaaaagtttaaggacattaatttcaccaacttcttgactgaaagctcagctttcaactgttttgtcaaatagtttcaatcaatcaactgactctagaattttactattcttggaatttggtagtttcatgtttaatattgtaacctgtataaaaatgaaatctgtaatgttattttcgccttttaaaacttttttacatttcctacataaaaggcagcaatgacataattatacataaagtacccttaactgaaaatgagatgaggctgcattcataggcttcagagaatagtaaattgcatagaaattcatcaatttaagttacatggtaccatgacaacttgtatattagcagcttgacagacagcttcgaattttcacagactactacatgaactgttatggcaacggaaacttttacaaatagtagcatgttaaaagacctgtccacctaacagtacactacccaccgctcccatcagagacatgacacggtttgtttacatgatccaaatgaccatctcaatggtgattcgctgttatcactcacatcagctaacactactctgtgtatttatatgtgtgtatacatatttatgaaatgagaatacctggacagtctgattggttaacagcgtattggtacagttttgtcttctattacatgtcattcatttcagccctcaattttagaactctaaataaataaaatgtaatttacaaagataaattgttatttacaaatgcaaaaattcatcctgaggattttggtatctaggagaactgtttcacagaaaaaagcaagtatcaatctgtgaaataaaaatgcaccttgagttaaactaaataattcataattacaggttaatttacccaagttccagccaagaaaagcatgaagatatttaagaaatcttaaattgatttgcatgcaagaaattaatcacatacaacttttcaaatcccaatgttattcccccttaaacttcttgtttaatgttttagtctgactgtatttgtaaagtaggtgacagagaaaaaaatacctgaggaaagctcagtaacgtgctgagggttcttttcctcactggaaagcagcggggcttcaggccaccatgagaaacagccagtgggcctttgactttacccaagttaagctcccctaataggagtagttagctaaacaagttcaacgctttccaaaggaaaaaggtcaagttaaaacaaaaatctaaataaaggtaaaatatcaacagtttctctgctttacaatgtgaccataaaattacttatttacagaaattaaaagaaatggttcaacaaagaatcaaactggtttctccaggtatataccatgacaatgtatctttttactcgatgctgtgagcagacagtgattattttggagaaggaaaaataaggtgtggaattagtaatgcagatgctgaaaggcaagtggcaagagaagaatgcctcaaacaaaggctactttgttcccatctctactgcacctacacccacacccgccccggcccccaagctaaaagaccagaataaccaaagccattttaacagtagtgtgcaaaactgtcagctgacaaacaacataaaaacaagtcacactatgttatctgtggtcacgttcttcagggttagtccagtaactcaagactttacattcttttgtctttatttgtttattttaattaaacatataaaggttaataaacagacaaagtccagagttagtaggttggtattataacatttattaaaataatgctgtgggttaatagaaacagcaaagaaccaaagaattaaaatgcaagctatgtaaaatcccaactaaaacccaaaagtgtctaatgtattcattcattagctaactaaaagcccaaaaaagacaagacacccaatataataaagtactgcaaaacaattggcaattttcagttatcaaaattgtggattttgcattttgtatccttttctcaatcaagaaaaaaattctttttgaatgttatataacatacatataaaacaagatagaaaaatacattataaacttgtaacaatggctgtaaatacattatcttacatgtttctcataggcaataggttggttatggtacatacatagcatgaaactaagataataaagaatagacaaaaatacatgtcagctgtacgataacatacaagcgacactcccatctacccacgctaaaaaattacataatactgtcagaaaaaaagtcttaaaaactacatattttaataagaaataaattcaataaagaatgataatactgagaaccaaggcattcagagatttcaaaagtcatgcttttttcagttgatccaaaattttgtcaaccaagttttcaaaagtttgttcagagccaacattccctataaatgtcacacatttattatttcatacatttactttcttccccataaaagacctttgataaacatctaaaatgtccaggtataacatagttgagatgaaactggatcaaatactggtattgtttttaacaactatcacctcaagtgtttgagtgtcgcaaatttattcaaccaaccaaacaatataaaaatcaaaatggcacagcatatattgtaaataaatcaaaactgtatgtgtaacagaaagacaaagcagtggcatattaaaccaaagctagctggatacaaaacaatgaatgtctattgcatagtaaataaactgacaacggtttccaagtgagacaagatggtgggggaggtcaccaagaaggtaatgactcagcttcctgctgacctctgactgtgatgctgggaaggtgtggaagaggggacgagttgataagctgggcgggggggggggtccactgtcacttgagatttgccacgtctggtactgagcagttaatgattattcactcaagtgtttagatgtaggctttgcacacaaattgcttcaactacataactaactgtttcaacttcttgagaaattagaagcttaagctgaaatgtggttgagtatttatatgcactatgatgctagtttttcacattcttttaaagttaaggggtgggggaggcagaggttattgaaacagtaaaaggatacactacaccagttatctggtatgatataaagacatgtgattaaatttgggtgatttaaaacattgttttctagaatgaaaatcacaaagattcacttttgtgaaaacatttgctaggtatcctattatattcaattaattaaaaacaaaaaacaaaatcaaatgaatgcatcccccttctccaaataaaacaaagctctaattttgtctgtaaactgaagtttagatgacacataatttttatctcagaatcctttgggttaacattgaagattggaataaccaaaagtattaaactattcttttaaagaatgatgttttaaaacttactagtcaggcattagaaaagttatcaaatcttttcacagtatcagatttggcaaatttgcatcaaggtaacgtggcaaaaatcctataattcaaactatcaactcatttgtctccctcatatcttctttcacatactgggcgactgagtaacatgcattaacttgtattctgagggaggagctgatctttatgagacacttgactgaatgaccatgaaggaaaataaggcactttcttttctttagacttattccaatacttaaaaaataaaaaagaaagacaaaaaggctcttttggtcttttgtttcttgacaaccaccagaaaaaatcatttaatgaaataaagggtttctttgttctttttctttttttttataacacttgaaagtataaaatgctacatttccaaaaatatatatatttttttctgcaccagcacccttgtatagtaaaagtatctactttttgttcatttgtttcaatgcactacactttatctacaatttcattacatgtatacagcaaataggcaagcatggcttttacatccttaatgatttttttctatacagggaggtttaaaaaaaaatacttgaacagtttgcccagtaatgtgacacataatgcatgtaccttgttctcatatttttttaggtgtaaaataaagattcagtaattttaactcagatatttatctttttaaaaatagtgttgcagttttgttatttgcattacttttcaaaactccttaagtttttctctcatggcacactttcttctaatacttcaaattttggcaggcaatataaaaaaggctgcaacttctgccctttgagggcactgtagtgactaaacagcatatcaaattttgaatactttttgaaatcacttcaccaatgatatccctgaccgaaggttcatgcatgatgcatcatcacacagtacattcagagagagctttgacttcgctatgagaagaaaaagattcctagaagtctctcacagtaactgcctctgtcattgagtagttaaggaccatctgtctccccttcttaagagaggccttcttaccgttcgcttagggtgggatattaaaagatgatcagtgctgtgggatgaattgggccttattgctttactactattcagtgcagtttctagaaccactttcacccaaacaggaaaaaaaaaaaaaaaaagctgagttggaggacaacaatttctttgtcttttgtttggttagatggtaagacgaacggacaagtgcctcagctcgctgcactgacgacaggcaagcaaaggcgattaccagttaactgatcagcaggcaggcatggtcaggtcatcattgggtgaagagttcagaggtcagaaggtcataggttagttgccggtggcggctgggtggttagaaacaaaaaaaaacaaaacaaaaaaaagaaaagaaaagatagagaagagattagtttcagctagtgacggcttaatgacaacatgaaaaactaatcacaactaataaaaaaaaaagcatgtttaattctgacaaactgattgacaccatctacagaatacaattaaaatcatgacaatttcgtatcatgatttgaacaaatgaagaagagcccactcccacaaaaaaaaaaaaaaaactggttaacaagaaaaaatagaaataaaatacaactaacaactaatagttagtagcagtcaatgaaggaaattgaaaaacaacaatgaataggtttggtatacagaatttttaaacagtcagtgcagttatcagtatctgactgctattaagcattagtattctctaagatgcaagcattaaagcaactattaatgatggatgtgattattaataactgatgattaacagaaatgaatctaaagaaattcaaaattctatgaaccatttggttcaacataaactctgggccaaacaaggtttcttttgttcaataaatgtttattgctttttcaattattctatttacaaacaacatggaatttcttggcctcatgatacaaagcgatactaaactgtagtctagcagtgtaggcaacatcatgggaaccagaaaatggccaggccttttgcactagccaacactttccagttgaaaatactattttacacatatagaacacttataaaatgcacttgcatgtaaacactgtaaaatcctgccatttaaaattctacactcaaaaagctctaagtacatcaaaaaatagaagaaatttctaattgataccaataaggcattttaaaactacaaacagctttctttattcaatttcaaagctaatactctgcaaatacaataaaatctgacatttcatatacattcctgctttatatttttatattttaaaagaagccacctgtaaatactattttcttttgcaaaataacaaaaaggacaaaaaaactttaaaaattacagtaaaacataaagtagttctcaagtggaaaagttatcattcccaatgtccttgagttgttccttccttaatcaacctttgtcacattctgcttcaccaaacttggtccacttaacagtagtataatttttaagactcattcaacagcttaattatttctactatattctgaggtttgatagaattttctgtactgttgccattgtgactaaggcagaggagatgtgaatgaaaagatattcagtgcaaagttagattctgtgccacttcataaatcaaagcccagaaggtgtaatgttcagtttaaatgatccaaaataatggactgatttaccttcatatgacaaaaatgttttctatagtctatcatttagaacagtttataaatactacaaaaatactgtatcttcaatgtgaccaaatcttccctgaatttcttaaaagtggaattttatttaaaataaaaattgctgctccaaaatcatagaagaaaataaatatttaacatgatgtagtcatactacttcacaggtattccaaaatatagaatcttaaagcatttttgatgttactcatagttttgattaaaactgtttaaagtttcttatacaaattatgtaagtgatggtttttgtattactcagaaaaaactctgacttcttttctgagtgtggaatatataaacgaagtgagtgaccatttatatataccaggacacctagactacatcctctgccaagtcttggcctcctacacaggtgtgtcaccatgcaagaccatacagttcattacaactaaaaggtcagttggtctctaataggcttcaaattcagttttgaaatatatataaagaggtgagtttacttttagtaaagaactagatattggtcaaccatgtagtactctaaacgttcatatagaattacatggttatatgtccaagggctgagtttttttgcattaaatgaatgcttatactaataaacttctcttcaaaatatttttttaaaataattttaacctcaaaaatagagaaaacagtagtatcataaaataatttaagtgaaggacttcagacatctcccttagacccaatgagtgcatacagtgataagtatacgagtactctgttactaaaaaagaaatgagcatttcggtttgctgacactgcattttaaataaaaacagtgacaggactaatcaaaacacgtaactacaaaagatccatgcatggaatgtgtcgtaattttccaaatacaataaaatcttcctaaaatatgtccaactatctcaaggcactggagtattaagtaggccaataattattgtgttaaagcaaaatggtgagaaatctcctaaaagggggcatacatagggaaagattagctgggggaaaaaaactactttaaaatactctttagaacaattgtagacattagcaatatgaataaaacctcaaattattcatggaattgtccagtttctttaaaactcaagtgactttccaaaaaacttccccatccctatgagacgtgctcatacagaacacttacaaggaataccatcctcatagacgaccacggagctggggtctattttgttcactgaacaatcactgttagtgatgaatacattagtttaaaagtcttcaacgttctttatggattatgctaaacaaatattaacaatgtctttgggaaaggcatgttatttctgatgtggacaacagctgtgtctagtatttatcatcagtactcaaggtaatcacataaagcaggtaggtccttcataaattcatagaagatgtacaattgaagtacaaatccagcactttttcctccactaatatttgagactttgatcaatttaatttgtaggaaacaaatgtgccataatagaaacttgtaaaaaatccttttttactaccatgcttgatattcctatcttgtgatggaaaaacttagaaaacaattcaatgtcaataaaccgaaaataccattcctcaataagcaaaaataatttataaaagggtccaagggcatatacaggacacaaattataaaagttgtaaaggagaaaaatgaagacttattttccagtcacaggttagtcaaaaattatattcacacagctggatctcataccaccacagaacttcaagagacagtttaccttcagataatatattttagcagcaaatgacaaaaatcaaaggatccattttggcaagagaatgtaagaataaaagggaattgacgctctaatttatataaaaaaatccaactacatgaaagttatcttcacagtcctcactttgttgattttagctaagtacttgacatgtgcaccctcatgtttatacagtggctcaaatattttattataaagaaaaatggaaactaaatcttcagttttctccaaaagtacacaggaggcatatattcctttacttctctcattaaagcaccatccgttcaattcattttgcaataccaaccccaaatttcagaacttttaaaaggtaaattttagcaaaagttattaatgaaaataactgaggcaacatcaaaatttaatagctccccaaattgactaatttatgttttagtaggaataaatcatagtacataataatagaagatttaataagttaaaatatgaagggagaaaaaaccaaaccaaaacaaaaaacccaacccttaaatctgtcaatgatcacaaacaaatttagaaaaggaaaaaaaactgtgtgcaggtaagcaattacatttttccatcaggtgtggtgttgcaaattttatggacacccaacgcatttcttatagacaagaactgcagaactaaactaacctcggtctgcggtcacaatcctttggtaaggatggacacgcatatcgtgccttcgaactttagtagccaccgcacctagttaaattgcaattaccaagacaaagttagaaaacattcacaaggggggaaaaaacattaacagcaggtttatcaaaatggatttcaaatgttcatttactacaaaagtttaagaaacacgttaaggcacagtagttttaaaattaaccacaatatgtcatgtatatatgcatctattaatattgcattcatttcaaacatcttgggccttaacctattgtatccattcatttacaatccccaagttacagtatttcatgagctctattagatccaaacatatttaagctttactagtcacatattcactgaagtgcctttcttgcagcaggactacttaaataacgccatgtttaatacagacaattatttgctaaccttaagaccacttcaagagtttatcacttaaaaaggtttaaaagcaattcttaaagcctacagattgtggttttaaactctgagtcaataagtatgaactgcaatgaattaggtgattagtaaagcaaacagtatagtacacttagcagtcagtatactactatacactcctttataaattaccattactgtgtaatattacagactaaaccaaattaataacataattttactttatatctatgtgcaaaaagtgcaagtaagtcactgactgctaggctaagcttttttcccccggaggctgctgagactaagcatttgttaaattcagatctgatgagggttcagttaagaccgttcttgaattcttagcctttcgttgggaaagccatacctaaagataaaaggaagggaattaaaaattagtcatcaatgaagacttgatgctaataccaatctcctcactactaccaacacacatgtctgcatctgttttgaagggcactgcttattttaaaataatttaatgtgagatgtgacataaatagcatgcatgttatctgtgtgcaaatttattataacttagaaatttaaaataattttctgagttctccaagtggtcaatatcatgttttactgcttaggtggcaaagcaagaaatgaaattaaccataatagattttttcattgggcacttattattattcaccttatgaatgccaattagaaatctgcatattttggtctttattttaccagtctaataattaagtttctataagtaaaaattttccaacaaacaaaagacatgaagctttacaatgagaaacaagttttactgcagtgcctcttgctatttctaagcagtaaactggtccatcacctcttattcattttagataaggtaatcatatacaagtacaattccacgtggcaaaatcagggagatcttgcgctgaaagtgctggaacagcagctggtggctaagagccccagccctgcaggaagtcaagagtcataactcctcgggaacagatgctgtgggtgcagcagagaggagttctgggaaaaggagcatgcacgggaccacaggacagagtattaatagaaaagaaaacttaaacaacaaggttacaggttacatgttattttaaaaatgcttcaagaaatgtgcaacagacacaagcctctcataaacagttctgtggtataattctgacctgcaattactttatacaatgatttaaacagaaaacatgtacaatgaaatgtatttgttcatgaaacaaagggcacctgagtgcatgcacacacacagataacatacagagcatcatggctttctttacttgaacaacgaattttcgagtttaaatcttagtgttctccagttcattaaagattttcaaatctttataaatcaatattaatgctggggaaaaaaaaccttaaaagatcaaagtcctaaaagtcaacagcatgcatgcagcaccaaggtcatatacaattcaggaaaaaaagtattcaaattttgtctggtaaaacaaaggggttgcacagaaacagtttgttccacattgactggtcgtgttataacagctgctgtattctagtccttcatccagcaagtcaatgggctgaaatatcaggcatgactggcatttcaatccactctataaaaaaaaggcatcagtaatgtctttttcgagcacaccactttttgttcatgtaaaaccaagcgtttatattatgattttaatttctgccttaagtgagattctgaattcagtgatttgctatttatttaactattccatactgtactactgaaattaagagtatctctcatgtttaatatgactaggactccaaaacacaagaactgaaaaatcttaagaatacaactacagtcatgcctgcataacaacattttggtcaacaacggaccacttatactatgtggtcccataagattataatggctataccacacagcctaggtgtgtagtaaacgatatcatctatgtctgtgtaagtacactctatgatgtacaccaaatgatgaaactgccagacaaggcaattcttagactgtatccccgttgttaagcgatgcatgactgtatttatctgatattttaagtgatcgcaaatattacaaaacacacacaataatatgaattttataaagcgctcagactactttcacttagaagtttaaaaattttccaacaattacacaaacctgtgagataaaataaatctcaaataaagtttgagaagtggagctgatggaggtgacgggccaatggggtgggacctaaaactcagaatgacctcagtaatgtcaaatgtaaaagtatttgttgaaatgtacacaacagatttacccaaccaaactgaacctcagttaccaaagtggatctgaataaatttaaggtgcaattatttcaaaggggaacccttatgagaggctgaaataaaacaaaatttagttttcggtcttccctaatgcaaacttgtcttgcctctctaaaactgataaaatcatttcaaaatctgagggagcaaaaatatttataaagagaatgttgttaaccccatggggagaagaacttacctaatacaccactaggttcaataggatactcaaggattgatgtagctggtgccaatgtgtaggggtactcatagggtgtatagattaaaccagcttcgggccctggaggaactattgcagcagttgggtgaggagttccgtttggcatgacagcggtctgtatttgtctgatcaaaggcattatggtagggccagctggcgtaggagtacgcagggcagctggtgggagaaccggcgcaggcccagtaatgatccttggagcagcctgggctgttgctgcaagagaaaaggcaagggctggtgatttaatgttggcatctctgtaggtgccattcagaatcgcaagctccatcagctgcatcttcttcaggctgtcttctccttctgctgcaggtaccaataatttcttcacttcttcaactgctctcttcaatttgatttctgctctgttctgagcatcttccacagtgattagtacatgtaaatcttcatttagatgctcccaattgggcttgcctctattttgctcctccttttttttatccctcattgagcctttgcctcggaccatgattttacatccggtttctgcttcaagttgtttggctgtaagtcctctaggtccaaggattctcccaacaaaattaaaatctgggtattcttttacaggcacataaagtttctcttgtaactgaacaataggtcccacagcatcaggcaattctgcactccttttctctgtactgccatttaatgtgtcattgtacatgtctttccgtactctgctaatttcttcgtccagcagccgctcgaggtggttgaagatcccgcagaagttgggcaggctgctcatgagcttcttgtcgttcatcagctgcatcaggtaatctggggtgggcttcggcttctccttcgtttccatttccccgaccatattccaggctccgcagctcactccgcccgccgccgccgccgccgccgccggagaggagggaggggcgggggcgagccccggccgcgggccgctcgggacccggcgtcccgctccgcgccggctcccgctctggctcccgcgccgagccccggggcggccggcaccgcgcgctcgcccgccccccgcaggcactttccgcccgggcccgacgcgctcccagccgccgccgctctcggccgcccggctcggcgcgtccctcacgaggccggcgggcgggcgggaggcgggtctcggctggccgagtgcgggcgcggggcgcgggctgctggcgccggacgaggaggagccggggccgccgctcgctcggctggtcgagcccgctcagcgccgccgccgcctgtgccgcgggctcggggggtctctctgggctggtccccgccgcggcgcctctgccgctgccgccgcgctccgactgc

SEQ ID NO: 16961 - RNA, 11653 nt, Homo sapiens
  source 1..11653: mol_type = other RNA
taggcctttagatcacttaaactacagataaaattagatgtgtagcacatatttctaaaatattgtccatattttttccattttaaataaaggtattaaggaattcgtgacaatgtaaaaaactactctatgcacttagaaaaattgtgaattcgaaaagttggagaataatttttgctaaataaataatcatttggcagtaagttctattctacctaaaataatttgcttgaaatgctgtaacagctacttcttatcaaggaataaagacaggcatcacatcctggtcaaacatgcaaaaccactcccaccccaccccatcctaaaactaaagaaaccttaggctgtcacacgtgaaagtgttatgacatatatatatacacacacgtatatatatgaagagtcttgatttggtagtgagcaatttcatttaaacctatcgtttgcttttggcacactaaaaaattcagatccttatgtagtgtttagaaaaccataaccagacaccgattgtgtgtacgtatgcacatcctggttttatgggcagggtgccttcgtgacctcttacacctggagctactgcactggtgcgtatgggagtaactactttcatgttaagttttccctgacattttgcctaaaggaaaagtttaaggacattaatttcaccaacttcttgactgaaagctcagctttcaactgttttgtcaaatagtttcaatcaatcaactgactctagaattttactattcttggaatttggtagtttcatgtttaatattgtaacctgtataaaaatgaaatctgtaatgttattttcgccttttaaaacttttttacatttcctacataaaaggcagcaatgacataattatacataaagtacccttaactgaaaatgagatgaggctgcattcataggcttcagagaatagtaaattgcatagaaattcatcaatttaagttacatggtaccatgacaacttgtatattagcagcttgacagacagcttcgaattttcacagactactacatgaactgttatggcaacggaaacttttacaaatagtagcatgttaaaagacctgtccacctaacagtacactacccaccgctcccatcagagacatgacacggtttgtttacatgatccaaatgaccatctcaatggtgattcgctgttatcactcacatcagctaacactactctgtgtatttatatgtgtgtatacatatttatgaaatgagaatacctggacagtctgattggttaacagcgtattggtacagttttgtcttctattacatgtcattcatttcagccctcaattttagaactctaaataaataaaatgtaatttacaaagataaattgttatttacaaatgcaaaaattcatcctgaggattttggtatctaggagaactgtttcacagaaaaaagcaagtatcaatctgtgaaataaaaatgcaccttgagttaaactaaataattcataattacaggttaatttacccaagttccagccaagaaaagcatgaagatatttaagaaatcttaaattgatttgcatgcaagaaattaatcacatacaacttttcaaatcccaatgttattcccccttaaacttcttgtttaatgttttagtctgactgtatttgtaaagtaggtgacagagaaaaaaatacctgaggaaagctcagtaacgtgctgagggttcttttcctcactggaaagcagcggggcttcaggccaccatgagaaacagccagtgggcctttgactttacccaagttaagctcccctaataggagtagttagctaaacaagttcaacgctttccaaaggaaaaaggtcaagttaaaacaaaaatctaaataaaggtaaaatatcaacagtttctctgctttacaatgtgaccataaaattacttatttacagaaattaaaagaaatggttcaacaaagaatcaaactggtttctccaggtatataccatgacaatgtatctttttactcgatgctgtgagcagacagtgattattttggagaaggaaaaataaggtgtggaattagtaatgcagatgctgaaaggcaagtggcaagagaagaatgcctcaaacaaaggctactttgttcccatctctactgcacctacacccacacccgccccggcccccaagctaaaagaccagaataaccaaagccattttaacagtagtgtgcaaaactgtcagctgacaaacaacataaaaacaagtcacactatgttatctgtggtcacgttcttcagggttagtccagtaactcaagactttacattcttttgtctttatttgtttattttaattaaacatataaaggttaataaacagacaaagtccagagttagtaggttggtattataacatttattaaaataatgctgtgggttaatagaaacagcaaagaaccaaagaattaaaatgcaagctatgtaaaatcccaactaaaacccaaaagtgtctaatgtattcattcattagctaactaaaagcccaaaaaagacaagacacccaatataataaagtactgcaaaacaattggcaattttcagttatcaaaattgtggattttgcattttgtatccttttctcaatcaagaaaaaaattctttttgaatgttatataacatacatataaaacaagatagaaaaatacattataaacttgtaacaatggctgtaaatacattatcttacatgtttctcataggcaataggttggttatggtacatacatagcatgaaactaagataataaagaatagacaaaaatacatgtcagctgtacgataacatacaagcgacactcccatctacccacgctaaaaaattacataatactgtcagaaaaaaagtcttaaaaactacatattttaataagaaataaattcaataaagaatgataatactgagaaccaaggcattcagagatttcaaaagtcatgcttttttcagttgatccaaaattttgtcaaccaagttttcaaaagtttgttcagagccaacattccctataaatgtcacacatttattatttcatacatttactttcttccccataaaagacctttgataaacatctaaaatgtccaggtataacatagttgagatgaaactggatcaaatactggtattgtttttaacaactatcacctcaagtgtttgagtgtcgcaaatttattcaaccaaccaaacaatataaaaatcaaaatggcacagcatatattgtaaataaatcaaaactgtatgtgtaacagaaagacaaagcagtggcatattaaaccaaagctagctggatacaaaacaatgaatgtctattgcatagtaaataaactgacaacggtttccaagtgagacaagatggtgggggaggtcaccaagaaggtaatgactcagcttcctgctgacctctgactgtgatgctgggaaggtgtggaagaggggacgagttgataagctgggcgggggggggggtccactgtcacttgagatttgccacgtctggtactgagcagttaatgattattcactcaagtgtttagatgtaggctttgcacacaaattgcttcaactacataactaactgtttcaacttcttgagaaattagaagcttaagctgaaatgtggttgagtatttatatgcactatgatgctagtttttcacattcttttaaagttaaggggtgggggaggcagaggttattgaaacagtaaaaggatacactacaccagttatctggtatgatataaagacatgtgattaaatttgggtgatttaaaacattgttttctagaatgaaaatcacaaagattcacttttgtgaaaacatttgctaggtatcctattatattcaattaattaaaaacaaaaaacaaaatcaaatgaatgcatcccccttctccaaataaaacaaagctctaattttgtctgtaaactgaagtttagatgacacataatttttatctcagaatcctttgggttaacattgaagattggaataaccaaaagtattaaactattcttttaaagaatgatgttttaaaacttactagtcaggcattagaaaagttatcaaatcttttcacagtatcagatttggcaaatttgcatcaaggtaacgtggcaaaaatcctataattcaaactatcaactcatttgtctccctcatatcttctttcacatactgggcgactgagtaacatgcattaacttgtattctgagggaggagctgatctttatgagacacttgactgaatgaccatgaaggaaaataaggcactttcttttctttagacttattccaatacttaaaaaataaaaaagaaagacaaaaaggctcttttggtcttttgtttcttgacaaccaccagaaaaaatcatttaatgaaataaagggtttctttgttctttttctttttttttataacacttgaaagtataaaatgctacatttccaaaaatatatatatttttttctgcaccagcacccttgtatagtaaaagtatctactttttgttcatttgtttcaatgcactacactttatctacaatttcattacatgtatacagcaaataggcaagcatggcttttacatccttaatgatttttttctatacagggaggtttaaaaaaaaatacttgaacagtttgcccagtaatgtgacacataatgcatgtaccttgttctcatatttttttaggtgtaaaataaagattcagtaattttaactcagatatttatctttttaaaaatagtgttgcagttttgttatttgcattacttttcaaaactccttaagtttttctctcatggcacactttcttctaatacttcaaattttggcaggcaatataaaaaaggctgcaacttctgccctttgagggcactgtagtgactaaacagcatatcaaattttgaatactttttgaaatcacttcaccaatgatatccctgaccgaaggttcatgcatgatgcatcatcacacagtacattcagagagagctttgacttcgctatgagaagaaaaagattcctagaagtctctcacagtaactgcctctgtcattgagtagttaaggaccatctgtctccccttcttaagagaggccttcttaccgttcgcttagggtgggatattaaaagatgatcagtgctgtgggatgaattgggccttattgctttactactattcagtgcagtttctagaaccactttcacccaaacaggaaaaaaaaaaaaaaaaagctgagttggaggacaacaatttctttgtcttttgtttggttagatggtaagacgaacggacaagtgcctcagctcgctgcactgacgacaggcaagcaaaggcgattaccagttaactgatcagcaggcaggcatggtcaggtcatcattgggtgaagagttcagaggtcagaaggtcataggttagttgccggtggcggctgggtggttagaaacaaaaaaaaacaaaacaaaaaaaagaaaagaaaagatagagaagagattagtttcagctagtgacggcttaatgacaacatgaaaaactaatcacaactaataaaaaaaaaagcatgtttaattctgacaaactgattgacaccatctacagaatacaattaaaatcatgacaatttcgtatcatgatttgaacaaatgaagaagagcccactcccacaaaaaaaaaaaaaaaactggttaacaagaaaaaatagaaataaaatacaactaacaactaatagttagtagcagtcaatgaaggaaattgaaaaacaacaatgaataggtttggtatacagaatttttaaacagtcagtgcagttatcagtatctgactgctattaagcattagtattctctaagatgcaagcattaaagcaactattaatgatggatgtgattattaataactgatgattaacagaaatgaatctaaagaaattcaaaattctatgaaccatttggttcaacataaactctgggccaaacaaggtttcttttgttcaataaatgtttattgctttttcaattattctatttacaaacaacatggaatttcttggcctcatgatacaaagcgatactaaactgtagtctagcagtgtaggcaacatcatgggaaccagaaaatggccaggccttttgcactagccaacactttccagttgaaaatactattttacacatatagaacacttataaaatgcacttgcatgtaaacactgtaaaatcctgccatttaaaattctacactcaaaaagctctaagtacatcaaaaaatagaagaaatttctaattgataccaataaggcattttaaaactacaaacagctttctttattcaatttcaaagctaatactctgcaaatacaataaaatctgacatttcatatacattcctgctttatatttttatattttaaaagaagccacctgtaaatactattttcttttgcaaaataacaaaaaggacaaaaaaactttaaaaattacagtaaaacataaagtagttctcaagtggaaaagttatcattcccaatgtccttgagttgttccttccttaatcaacctttgtcacattctgcttcaccaaacttggtccacttaacagtagtataatttttaagactcattcaacagcttaattatttctactatattctgaggtttgatagaattttctgtactgttgccattgtgactaaggcagaggagatgtgaatgaaaagatattcagtgcaaagttagattctgtgccacttcataaatcaaagcccagaaggtgtaatgttcagtttaaatgatccaaaataatggactgatttaccttcatatgacaaaaatgttttctatagtctatcatttagaacagtttataaatactacaaaaatactgtatcttcaatgtgaccaaatcttccctgaatttcttaaaagtggaattttatttaaaataaaaattgctgctccaaaatcatagaagaaaataaatatttaacatgatgtagtcatactacttcacaggtattccaaaatatagaatcttaaagcatttttgatgttactcatagttttgattaaaactgtttaaagtttcttatacaaattatgtaagtgatggtttttgtattactcagaaaaaactctgacttcttttctgagtgtggaatatataaacgaagtgagtgaccatttatatataccaggacacctagactacatcctctgccaagtcttggcctcctacacaggtgtgtcaccatgcaagaccatacagttcattacaactaaaaggtcagttggtctctaataggcttcaaattcagttttgaaatatatataaagaggtgagtttacttttagtaaagaactagatattggtcaaccatgtagtactctaaacgttcatatagaattacatggttatatgtccaagggctgagtttttttgcattaaatgaatgcttatactaataaacttctcttcaaaatatttttttaaaataattttaacctcaaaaatagagaaaacagtagtatcataaaataatttaagtgaaggacttcagacatctcccttagacccaatgagtgcatacagtgataagtatacgagtactctgttactaaaaaagaaatgagcatttcggtttgctgacactgcattttaaataaaaacagtgacaggactaatcaaaacacgtaactacaaaagatccatgcatggaatgtgtcgtaattttccaaatacaataaaatcttcctaaaatatgtccaactatctcaaggcactggagtattaagtaggccaataattattgtgttaaagcaaaatggtgagaaatctcctaaaagggggcatacatagggaaagattagctgggggaaaaaaactactttaaaatactctttagaacaattgtagacattagcaatatgaataaaacctcaaattattcatggaattgtccagtttctttaaaactcaagtgactttccaaaaaacttccccatccctatgagacgtgctcatacagaacacttacaaggaataccatcctcatagacgaccacggagctggggtctattttgttcactgaacaatcactgttagtgatgaatacattagtttaaaagtcttcaacgttctttatggattatgctaaacaaatattaacaatgtctttgggaaaggcatgttatttctgatgtggacaacagctgtgtctagtatttatcatcagtactcaaggtaatcacataaagcaggtaggtccttcataaattcatagaagatgtacaattgaagtacaaatccagcactttttcctccactaatatttgagactttgatcaatttaatttgtaggaaacaaatgtgccataatagaaacttgtaaaaaatccttttttactaccatgcttgatattcctatcttgtgatggaaaaacttagaaaacaattcaatgtcaataaaccgaaaataccattcctcaataagcaaaaataatttataaaagggtccaagggcatatacaggacacaaattataaaagttgtaaaggagaaaaatgaagacttattttccagtcacaggttagtcaaaaattatattcacacagctggatctcataccaccacagaacttcaagagacagtttaccttcagataatatattttagcagcaaatgacaaaaatcaaaggatccattttggcaagagaatgtaagaataaaagggaattgacgctctaatttatataaaaaaatccaactacatgaaagttatcttcacagtcctcactttgttgattttagctaagtacttgacatgtgcaccctcatgtttatacagtggctcaaatattttattataaagaaaaatggaaactaaatcttcagttttctccaaaagtacacaggaggcatatattcctttacttctctcattaaagcaccatccgttcaattcattttgcaataccaaccccaaatttcagaacttttaaaaggtaaattttagcaaaagttattaatgaaaataactgaggcaacatcaaaatttaatagctccccaaattgactaatttatgttttagtaggaataaatcatagtacataataatagaagatttaataagttaaaatatgaagggagaaaaaaccaaaccaaaacaaaaaacccaacccttaaatctgtcaatgatcacaaacaaatttagaaaaggaaaaaaaactgtgtgcaggtaagcaattacatttttccatcaggtgtggtgttgcaaattttatggacacccaacgcatttcttatagacaagaactgcagaactaaactaacctcggtctgcggtcacaatcctttggtaaggatggacacgcatatcgtgccttcgaactttagtagccaccgcacctagttaaattgcaattaccaagacaaagttagaaaacattcacaaggggggaaaaaacattaacagcaggtttatcaaaatggatttcaaatgttcatttactacaaaagtttaagaaacacgttaaggcacagtagttttaaaattaaccacaatatgtcatgtatatatgcatctattaatattgcattcatttcaaacatcttgggccttaacctattgtatccattcatttacaatccccaagttacagtatttcatgagctctattagatccaaacatatttaagctttactagtcacatattcactgaagtgcctttcttgcagcaggactacttaaataacgccatgtttaatacagacaattatttgctaaccttaagaccacttcaagagtttatcacttaaaaaggtttaaaagcaattcttaaagcctacagattgtggttttaaactctgagtcaataagtatgaactgcaatgaattaggtgattagtaaagcaaacagtatagtacacttagcagtcagtatactactatacactcctttataaattaccattactgtgtaatattacagactaaaccaaattaataacataattttactttatatctatgtgcaaaaagtgcaagtaagtcactgactgctaggctaagcttttttcccccggaggctgctgagactaagcatttgttaaattcagatctgatgagggttcagttaagaccgttcttgaattcttagcctttcgttgggaaagccatacctaatacaccactaggttcaataggatactcaaggattgatgtagctggtgccaatgtgtaggggtactcatagggtgtatagattaaaccagcttcgggccctggaggaactattgcagcagttgggtgaggagttccgtttggcatgacagcggtctgtatttgtctgatcaaaggcattatggtagggccagctggcgtaggagtacgcagggcagctggtgggagaaccggcgcaggcccagtaatgatccttggagcagcctgggctgttgctgcaagagaaaaggcaagggctggtgatttaatgttggcatctctgtaggtgccattcagaatcgcaagctccatcagctgcatcttcttcaggctgtcttctccttctgctgcaggtaccaataatttcttcacttcttcaactgctctcttcaatttgatttctgctctgttctgagcatcttccacagtgattagtacatgtaaatcttcatttagatgctcccaattgggcttgcctctattttgctcctccttttttttatccctcattgagcctttgcctcggaccatgattttacatccggtttctgcttcaagttgtttggctgtaagtcctctaggtccaaggattctcccaacaaaattaaaatctgggtattcttttacaggcacataaagtttctcttgtaactgaacaataggtcccacagcatcaggcaattctgcactccttttctctgtactgccatttaatgtgtcattgtacatgtctttccgtactctgctaatttcttcgtccagcagccgctcgaggtggttgaagatcccgcagaagttgggcaggctgctcatgagcttcttgtcgttcatcagctgcatcaggtaatctggggtgggcttcggcttctccttcgtttccatttccccgaccatattccaggctccgcagctcactccgcccgccgccgccgccgccgccgccggagaggagggaggggcgggggcgagccccggccgcgggccgctcgggacccggcgtcccgctccgcgccggctcccgctctggctcccgcgccgagccccggggcggccggcaccgcgcgctcgcccgccccccgcaggcactttccgcccgggcccgacgcgctcccagccgccgccgctctcggccgcccggctcggcgcgtccctcacgaggccggcgggcgggcgggaggcgggtctcggctggccgagtgcgggcgcggggcgcgggctgctggcgccggacgaggaggagccggggccgccgctcgctcggctggtcgagcccgctcagcgccgccgccgcctgtgccgcgggctcggggggtctctctgggctggtccccgccgcggcgcctctgccgctgccgccgcgctccgactgc

SEQ ID NO: 16962 - RNA, 62 nt, Homo sapiens
  source 1..62: mol_type = other RNA
taggcctttagatcacttaaagagtattcaacatcagatgatctaaaggcctatacataaat

SEQ ID NO: 16963 - RNA, 2814 nt, Homo sapiens
  source 1..2814: mol_type = other RNA
taggcctttagatcacttaaatgtggttacaggtttattaaattaaaaatgtctgaaacatttcagcattcatatttttatacaagaagtttgtgtggtatccatcttccagttctcttggtagtatcagccatttgcttgcttatttttaagttttgagaacaaatcgcagtaagttgaagcaaatagtgctaacagaacttgtaaattcagcttggggggtggttcctgaaaagagtcaaagtaacaaccacctacaggtacagtcatgaaccaggaaagtgcaatccaaatgaaaaaattcatgctttgcaaaagccaaaaatgaggccactggtgttttcagaataacaccggtgctttgatgctgacttgcagtaaaatcctccctctgggtcccgcagcttggtggctcaggccggccacagtctccacattagcacccacattgtatatgtacagggacatatatattatatatattcatatttataaaaaagaaaacaaaaacaaacacctgtcctgattggtttttgttaaaacatgaaaaaaaattttattgttttagacaaagaggccacttttggaaaataatacttttttttttttagttgaatcaggtgaagacagagttaaaatcacataggatttgcatttttaaaaaaggaaagcactaggattgttggcactggagtaactatttacactgaacagaggtttggccttttacataacatcgatacaatgcattttccaaagtctgagaaataacaaggttctgtctcgaatgcttcacagaggaggttcggatttggggacaagtgtcattaatgagggccatggaagttcgtcagcttcagagtcacatgcaatctgatcctgggcggttccgctgctggggagcagctggctacggaattgaaagctaatggggaggggtggggcagcctctgggacaaggcctctctccgcagacccgggccttacaggttttcaccaggttggtactggggctctgtcgcggtaaagtagtcttccaggaagctctgcaagtactcaaaagtggggcgttcttcagggtcctttttccagcagtggatcatgagctcatgcagagagatggggcagtcctgcgggcagggcatcctgtagcctcgctccacctgctccagcacctcccggttgttcatgcctgggtatggcactcttcctttggtgaccagctctgtgagtaagattccaaaagaccacacgtcagacttgattgtgaacctcccgtacagggctgcctcgggggccgtccacttgatggggaactttgcaccttgtcttgctgtgtactcattgtcttctatcaatcgggccaatccgaagtcagcaatcttgcatatgagtccattccccactagaatgtttgctgatcgcagatctctatggatataattcatgcgctcgatgtaagccattcctgcagccacctgtgctgccatgtccacaagatttggtaatttcagagctcttccttctccatcttttaagaaatccagtaaacttcctttgttcatatactcggtgacgatgtagatgggctcctcagacaccactgcatagagctggaccagcttgtcgtgcttcagcttcttcatgatctgcgcttcctcaaggaatgattcgggggacattgtgcctggtttaagagtctttatggctacttttgtgtttccattccaggtaccaagccacacttcagcgaaacacccctgacccagcttcttctccagacacaacgaacgacgtgcaacttcccaagcatctttagccaatccagaagtttgtggggtacaactcgatgcaatcacagttaagttaaaacacaaaccatcagctttctctgagtaatgttgtacaagctgctgaagtgtttcaaactgggcccgggtggtaatgtagtatccaccattgtcaagtttgcgaattttataatgtttgacatggtctcctttcatatcatcccaatcacggatagaaagtgaataggcacctttggtggtttcactctcgcggataagaaaggtacctcttgggtttccaaaggacaatagctgtcgctcagcatcttttcggccaagttttccaaagtaccactcttctgcctggatagagtcaactggagccacataattgctgggaatgtaacctgtctctccagttgtcaaggagcgggcttcccaccaatctccttccgagctgttcaatatttgaaatttttctcctttgtgaaaactcaggtcatcttctgtccgtgcttcatagtcataaagggccacaaagagtgtcactcctgttcctcctctcgtacgcaaggtccccgtatgagacgaagagttcacacctccaaagacggtgagtccttggcccccggctgcgtggaagttgttgtagttggggatggaggtcacaccgaagctggggtagtgctgaggggtggggtctgtgccatagcggtacccagagctctggttcaggctgccgtccctctcctccgtcagttttgttgcttctttatccttacattgcacacagcccattatctaaattccaaaatgtccgccaacgatcacaaactttatatacaccacatgtcttctacaacagaggcaggactggtctttttccacgtttagatcagcatcctgcttcttcaaaaaaactgcgcggcgctgaggctccggagcccactcacatggtcctctccccgccctcctccggcgcggccgaggcggctccggggggtccccggcgggcccgggagcc

SEQ ID NO: 16964 - RNA, 2846 nt, Homo sapiens
  source 1..2846: mol_type = other RNA
taggcctttagatcacttaaatgtggttacaggtttattaaattaaaaatgtctgaaacatttcagcattcatatttttatacaagaagtttgtgtggtatccatcttccagttctcttggtagtatcagccatttgcttgcttatttttaagttttgagaacaaatcgcagtaagttgaagcaaatagtgctaacagaacttgtaaattcagcttggggggtggttcctgaaaagagtcaaagtaacaaccacctacaggtacagtcatgaaccaggaaagtgcaatccaaatgaaaaaattcatgctttgcaaaagccaaaaatgaggccactggtgttttcagaataacaccggtgctttgatgctgacttgcagtaaaatcctccctctgggtcccgcagcttggtggctcaggccggccacagtctccacattagcacccacattgtatatgtacagggacatatatattatatatattcatatttataaaaaagaaaacaaaaacaaacacctgtcctgattggtttttgttaaaacatgaaaaaaaattttattgttttagacaaagaggccacttttggaaaataatacttttttttttttagttgaatcaggtgaagacagagttaaaatcacataggatttgcatttttaaaaaaggaaagcactaggattgttggcactggagtaactatttacactgaacagaggtttggccttttacataacatcgatacaatgcattttccaaagtctgagaaataacaaggttctgtctcgaatgcttcacagaggaggttcggatttggggacaagtgtcattaatgagggccatggaagttcgtcagcttcagagtcacatgcaatctgatcctgggcggttccgctgctggggagcagctggctacggaattgaaagctaatggggaggggtggggcagcctctgggacaaggcctctctccgcagacccgggccttacaggttttcaccaggttggtactggggctctgtcgcggtaaagtagtcttccaggaagctctgcaagtactcaaaagtggggcgttcttcagggtcctttttccagcagtggatcatgagctcatgcagagagatggggcagtcctgcgggcagggcatcctgtagcctcgctccacctgctccagcacctcccggttgttcatgcctgggtatggcactcttcctttggtgaccagctctgtgagtaagattccaaaagaccacacgtcagacttgattgtgaacctcccgtacagggctgcctcgggggccgtccacttgatggggaactttgcaccttgtcttgctgtgtactcattgtcttctatcaatcgggccaatccgaagtcagcaatcttgcatatgagtccattccccactagaatgtttgctgatcgcagatctctatggatataattcatgcgctcgatgtaagccattcctgcagccacctgtgctgccatgtccacaagatttggtaatttcagagctcttccttctccatcttttaagaaatccagtaaacttcctttgttcatatactcggtgacgatgtagatgggctcctcagacaccactgcatagagctggaccagcttgtcgtgcttcagcttcttcatgatctgcgcttcctcaaggaatgattcgggggacattgtgcctggtttaagagtctttatggctacttttgtgtttccattccaggtacccatccatacttccccaaactgcccatttcccagtctcttgatcaactgcagggattctcgagggatttcccagacatctttggttttgacagacagatcggtaagccttggcatccctttgtgacagggaactactaggcggcagcagagacctgcagctctctctgagtaatgttgtacaagctgctgaagtgtttcaaactgggcccgggtggtaatgtagtatccaccattgtcaagtttgcgaattttataatgtttgacatggtctcctttcatatcatcccaatcacggatagaaagtgaataggcacctttggtggtttcactctcgcggataagaaaggtacctcttgggtttccaaaggacaatagctgtcgctcagcatcttttcggccaagttttccaaagtaccactcttctgcctggatagagtcaactggagccacataattgctgggaatgtaacctgtctctccagttgtcaaggagcgggcttcccaccaatctccttccgagctgttcaatatttgaaatttttctcctttgtgaaaactcaggtcatcttctgtccgtgcttcatagtcataaagggccacaaagagtgtcactcctgttcctcctctcgtacgcaaggtccccgtatgagacgaagagttcacacctccaaagacggtgagtccttggcccccggctgcgtggaagttgttgtagttggggatggaggtcacaccgaagctggggtagtgctgaggggtggggtctgtgccatagcggtacccagagctctggttcaggctgccgtccctctcctccgtcagttttgttgcttctttatccttacattgcacacagcccattatctaaattccaaaatgtccgccaacgatcacaaactttatatacaccacatgtcttctacaacagaggcaggactggtcctggcattctttagactggtggccaacagccctttttccattttaattcaagacccaagtcagaaaacaaaaacaaaaacaaaatgtatttggtttgtgtttttcaatttaaaagcgagtaattttacttggtcctgtgaaagggaccactttactgataagaaaaat

SEQ ID NO: 16965 - RNA, 2942 nt, Homo sapiens
  source 1..2942: mol_type = other RNA
taggcctttagatcacttaaatgtggttacaggtttattaaattaaaaatgtctgaaacatttcagcattcatatttttatacaagaagtttgtgtggtatccatcttccagttctcttggtagtatcagccatttgcttgcttatttttaagttttgagaacaaatcgcagtaagttgaagcaaatagtgctaacagaacttgtaaattcagcttggggggtggttcctgaaaagagtcaaagtaacaaccacctacaggtacagtcatgaaccaggaaagtgcaatccaaatgaaaaaattcatgctttgcaaaagccaaaaatgaggccactggtgttttcagaataacaccggtgctttgatgctgacttgcagtaaaatcctccctctgggtcccgcagcttggtggctcaggccggccacagtctccacattagcacccacattgtatatgtacagggacatatatattatatatattcatatttataaaaaagaaaacaaaaacaaacacctgtcctgattggtttttgttaaaacatgaaaaaaaattttattgttttagacaaagaggccacttttggaaaataatacttttttttttttagttgaatcaggtgaagacagagttaaaatcacataggatttgcatttttaaaaaaggaaagcactaggattgttggcactggagtaactatttacactgaacagaggtttggccttttacataacatcgatacaatgcattttccaaagtctgagaaataacaaggttctgtctcgaatgcttcacagaggaggttcggatttggggacaagtgtcattaatgagggccatggaagttcgtcagcttcagagtcacatgcaatctgatcctgggcggttccgctgctggggagcagctggctacggaattgaaagctaatggggaggggtggggcagcctctgggacaaggcctctctccgcagacccgggccttacaggttttcaccaggttggtactggggctctgtcgcggtaaagtagtcttccaggaagctctgcaagtactcaaaagtggggcgttcttcagggtcctttttccagcagtggatcatgagctcatgcagagagatggggcagtcctgcgggcagggcatcctgtagcctcgctccacctgctccagcacctcccggttgttcatgcctgggtatggcactcttcctttggtgaccagctctgtgagtaagattccaaaagaccacacgtcagacttgattgtgaacctcccgtacagggctgcctcgggggccgtccacttgatggggaactttgcaccttgtcttgctgtgtactcattgtcttctatcaatcgggccaatccgaagtcagcaatcttgcatatgagtccattccccactagaatgtttgctgatcgcagatctctatggatataattcatgcgctcgatgtaagccattcctgcagccacctgtgctgccatgtccacaagatttggtaatttcagagctcttccttctccatcttttaagaaatccagtaaacttcctttgttcatatactcggtgacgatgtagatgggctcctcagacaccactgcatagagctggaccagcttgtcgtgcttcagcttcttcatgatctgcgcttcctcaaggaatgattcgggggacattgtgcctggtttaagagtctttatggctacttttgtgtttccattccaggtacccatccatacttccccaaactgcccatttcccagtctcttgatcaactgcagggattctcgagggatttcccagacatctttggttttgacagacagatcggtaagccttggcatccctttgtgacagggaactactaggcggcagcagagacctgcagctctctctgagtaatgttgtacaagctgctgaagtgtttcaaactgggcccgggtggtaatgtagtatccaccattgtcaagtttgcgaattttataatgtttgacatggtctcctttcatatcatcccaatcacggatagaaagtgaataggcacctttggtggtttcactctcgcggataagaaaggtacctcttgggtttccaaaggacaatagctgtcgctcagcatcttttcggccaagttttccaaagtaccactcttctgcctggatagagtcaactggagccacataattgctgggaatgtaacctgtctctccagttgtcaaggagcgggcttcccaccaatctccttccgagctgttcaatatttgaaatttttctcctttgtgaaaactcaggtcatcttctgtccgtgcttcatagtcataaagggccacaaagagtgtcactcctgttcctcctctcgtacgcaaggtccccgtatgagacgaagagttcacacctccaaagacggtgagtccttggcccccggctgcgtggaagttgttgtagttggggatggaggtcacaccgaagctggggtagtgctgaggggtggggtctgtgccatagcggtacccagagctctggttcaggctgccgtccctctcctccgtcagttttgttgcttctttatccttacattgcacacagcccattatctaaattccaaaatgtccgccaacgatcacaaactttatatacaccacatgtcttctacaacagaggcaggactggtcctttgtgaatttctggggctctttagatccccctctggaatatacatggtcatgaggtccagagtcttcacccaggctgtcccccagtcttggggcagcttgacctccggcttctgctaggtcctctcctgcttctggtcagtcaatccattatcattagccatgtgctccacagagctgctccacctaccactgaaataaatcccttggagcatagaaaccgcgtggtcacactctggctttctcagacacttttgttctctt

SEQ ID NO: 16966 - RNA, 3204 nt, Homo sapiens
  source 1..3204: mol_type = other RNA
taggcctttagatcacttaaatgtggttacaggtttattaaattaaaaatgtctgaaacatttcagcattcatatttttatacaagaagtttgtgtggtatccatcttccagttctcttggtagtatcagccatttgcttgcttatttttaagttttgagaacaaatcgcagtaagttgaagcaaatagtgctaacagaacttgtaaattcagcttggggggtggttcctgaaaagagtcaaagtaacaaccacctacaggtacagtcatgaaccaggaaagtgcaatccaaatgaaaaaattcatgctttgcaaaagccaaaaatgaggccactggtgttttcagaataacaccggtgctttgatgctgacttgcagtaaaatcctccctctgggtcccgcagcttggtggctcaggccggccacagtctccacattagcacccacattgtatatgtacagggacatatatattatatatattcatatttataaaaaagaaaacaaaaacaaacacctgtcctgattggtttttgttaaaacatgaaaaaaaattttattgttttagacaaagaggccacttttggaaaataatacttttttttttttagttgaatcaggtgaagacagagttaaaatcacataggatttgcatttttaaaaaaggaaagcactaggattgttggcactggagtaactatttacactgaacagaggtttggccttttacataacatcgatacaatgcattttccaaagtctgagaaataacaaggttctgtctcgaatgcttcacagaggaggttcggatttggggacaagtgtcattaatgagggccatggaagttcgtcagcttcagagtcacatgcaatctgatcctgggcggttccgctgctggggagcagctggctacggaattgaaagctaatggggaggggtggggcagcctctgggacaaggcctctctccgcagacccgggccttacaggttttcaccaggttggtactggggctctgtcgcggtaaagtagtcttccaggaagctctgcaagtactcaaaagtggggcgttcttcagggtcctttttccagcagtggatcatgagctcatgcagagagatggggcagtcctgcgggcagggcatcctgtagcctcgctccacctgctccagcacctcccggttgttcatgcctgggtatggcactcttcctttggtgaccagctctgtgagtaagattccaaaagaccacacgtcagacttgattgtgaacctcccgtacagggctgcctcgggggccgtccacttgatggggaactttgcaccttgtcttgctgtgtactcattgtcttctatcaatcgggccaatccgaagtcagcaatcttgcatatgagtccattccccactagaatgtttgctgatcgcagatctctatggatataattcatgcgctcgatgtaagccattcctgcagccacctgtgctgccatgtccacaagatttggtaatttcagagctcttccttctccatcttttaagaaatccagtaaacttcctttgttcatatactcggtgacgatgtagatgggctcctcagacaccactgcatagagctggaccagcttgtcgtgcttcagcttcttcatgatctgcgcttcctcaaggaatgattcgggggacattgtgcctggtttaagagtctttatggctacttttgtgtttccattccaggtacccatccatacttccccaaactgcccatttcccagtctcttgatcaactgcagggattctcgagggatttcccagacatctttggttttgacagacagatcggtaagccttggcatccctttgtgacagggaactactaggcggcagcagagacctgcagctctctctgagtaatgttgtacaagctgctgaagtgtttcaaactgggcccgggtggtaatgtagtatccaccattgtcaagtttgcgaattttataatgtttgacatggtctcctttcatatcatcccaatcacggatagaaagtgaataggcacctttggtggtttcactctcgcggataagaaaggtacctcttgggtttccaaaggacaatagctgtcgctcagcatcttttcggccaagttttccaaagtaccactcttctgcctggatagagtcaactggagccacataattgctgggaatgtaacctgtctctccagttgtcaaggagcgggcttcccaccaatctccttccgagctgttcaatatttgaaatttttctcctttgtgaaaactcaggtcatcttctgtccgtgcttcatagtcataaagggccacaaagagtgtcactcctgttcctcctctcgtacgcaaggtccccgtatgagacgaagagttcacacctccaaagacggtgagtccttggcccccggctgcgtggaagttgttgtagttggggatggaggtcacaccgaagctggggtagtgctgaggggtggggtctgtgccatagcggtacccagagctctggttcaggctgccgtccctctcctccgtcagttttgttgcttctttatccttacattgcacacagcccattatctaaattccaaaatgtccgccaacgatcacaaactttatatacaccacatgtcttctacaacagaggcaggactggtctttttccacgtttagatcagcatcctgcttcttcaaaaaaactgcgcggcgctgaggctccggagcccactcacatggtcctctccccgccctcctccggcgcggccgaggcggctccggggggtccccggcgggcccgggagccggtgggccttccgagagcaccgagggggcggcgccggggtgtccccggcccggcggccgaatccctccctggcgcgggcggcggccgccgggcggtgcggcgcgggcggcggctttgtgtgcgcccgggcggtcctcggtgcgctgggagaagcgcggcgcgcccgggcgggagaggacgcgccgctcgcacaacaacctcgcctctactctcgccgccgggcggcgggcgggtctcgaaggccttcggctcgcggcgacccctcctcctcgcccgcggcagccccctcctcgccggctccgctcctgacagatggcgcaactgcaacgacgcgccgccgccaccagcgcggctgctcgctgctactcttgctgatgctct

SEQ ID NO: 16967 - RNA, 2856 nt, Homo sapiens
  source 1..2856: mol_type = other RNA
taggcctttagatcacttaaatgtggttacaggtttattaaattaaaaatgtctgaaacatttcagcattcatatttttatacaagaagtttgtgtggtatccatcttccagttctcttggtagtatcagccatttgcttgcttatttttaagttttgagaacaaatcgcagtaagttgaagcaaatagtgctaacagaacttgtaaattcagcttggggggtggttcctgaaaagagtcaaagtaacaaccacctacaggtacagtcatgaaccaggaaagtgcaatccaaatgaaaaaattcatgctttgcaaaagccaaaaatgaggccactggtgttttcagaataacaccggtgctttgatgctgacttgcagtaaaatcctccctctgggtcccgcagcttggtggctcaggccggccacagtctccacattagcacccacattgtatatgtacagggacatatatattatatatattcatatttataaaaaagaaaacaaaaacaaacacctgtcctgattggtttttgttaaaacatgaaaaaaaattttattgttttagacaaagaggccacttttggaaaataatacttttttttttttagttgaatcaggtgaagacagagttaaaatcacataggatttgcatttttaaaaaaggaaagcactaggattgttggcactggagtaactatttacactgaacagaggtttggccttttacataacatcgatacaatgcattttccaaagtctgagaaataacaaggttctgtctcgaatgcttcacagaggaggttcggatttggggacaagtgtcattaatgagggccatggaagttcgtcagcttcagagtcacatgcaatctgatcctgggcggttccgctgctggggagcagctggctacggaattgaaagctaatggggaggggtggggcagcctctgggacaaggcctctctccgcagacccgggccttacaggttttcaccaggttggtactggggctctgtcgcggtaaagtagtcttccaggaagctctgcaagtactcaaaagtggggcgttcttcagggtcctttttccagcagtggatcatgagctcatgcagagagatggggcagtcctgcgggcagggcatcctgtagcctcgctccacctgctccagcacctcccggttgttcatgcctgggtatggcactcttcctttggtgaccagctctgtgagtaagattccaaaagaccacacgtcagacttgattgtgaacctcccgtacagggctgcctcgggggccgtccacttgatggggaactttgcaccttgtcttgctgtgtactcattgtcttctatcaatcgggccaatccgaagtcagcaatcttgcatatgagtccattccccactagaatgtttgctgatcgcagatctctatggatataattcatgcgctcgatgtaagccattcctgcagccacctgtgctgccatgtccacaagatttggtaatttcagagctcttccttctccatcttttaagaaatccagtaaacttcctttgttcatatactcggtgacgatgtagatgggctcctcagacaccactgcatagagctggaccagcttgtcgtgcttcagcttcttcatgatctgcgcttcctcaaggaatgattcgggggacattgtgcctggtttaagagtctttatggctacttttgtgtttccattccaggtacccatccatacttccccaaactgcccatttcccagtctcttgatcaactgcagggattctcgagggatttcccagacatctttggttttgacagacagatcggtaagccttggcatccctttgtgacagggaactactaggcggcagcagagacctgcagctctctctgagtaatgttgtacaagctgctgaagtgtttcaaactgggcccgggtggtaatgtagtatccaccattgtcaagtttgcgaattttataatgtttgacatggtctcctttcatatcatcccaatcacggatagaaagtgaataggcacctttggtggtttcactctcgcggataagaaaggtacctcttgggtttccaaaggacaatagctgtcgctcagcatcttttcggccaagttttccaaagtaccactcttctgcctggatagagtcaactggagccacataattgctgggaatgtaacctgtctctccagttgtcaaggagcgggcttcccaccaatctccttccgagctgttcaatatttgaaatttttctcctttgtgaaaactcaggtcatcttctgtccgtgcttcatagtcataaagggccacaaagagtgtcactcctgttcctcctctcgtacgcaaggtccccgtatgagacgaagagttcacacctccaaagacggtgagtccttggcccccggctgcgtggaagttgttgtagttggggatggaggtcacaccgaagctggggtagtgctgaggggtggggtctgtgccatagcggtacccagagctctggttcaggctgccgtccctctcctccgtcagttttgttgcttctttatccttacattgcacacagcccattatctaaattccacctccagaacgccgcttctctgattagcaactttctccgatctgaagcgtggcttcccagccttccacaccagtggcctatatcttttccaccaatctcccactgcccctcacacactctccagccaggatggaatgcacctccacataactgtccatgcagttcccacatcttgtccaccggccaggcccatgcgagtcttacccttcacgtaagcctcccttctcagctcctcagacctgcgct

SEQ ID NO: 16968 - RNA, 2700 nt, Homo sapiens
  source 1..2700: mol_type = other RNA
taggcctttagatcacttaaatgtggttacaggtttattaaattaaaaatgtctgaaacatttcagcattcatatttttatacaagaagtttgtgtggtatccatcttccagttctcttggtagtatcagccatttgcttgcttatttttaagttttgagaacaaatcgcagtaagttgaagcaaatagtgctaacagaacttgtaaattcagcttggggggtggttcctgaaaagagtcaaagtaacaaccacctacaggtacagtcatgaaccaggaaagtgcaatccaaatgaaaaaattcatgctttgcaaaagccaaaaatgaggccactggtgttttcagaataacaccggtgctttgatgctgacttgcagtaaaatcctccctctgggtcccgcagcttggtggctcaggccggccacagtctccacattagcacccacattgtatatgtacagggacatatatattatatatattcatatttataaaaaagaaaacaaaaacaaacacctgtcctgattggtttttgttaaaacatgaaaaaaaattttattgttttagacaaagaggccacttttggaaaataatacttttttttttttagttgaatcaggtgaagacagagttaaaatcacataggatttgcatttttaaaaaaggaaagcactaggattgttggcactggagtaactatttacactgaacagaggtttggccttttacataacatcgatacaatgcattttccaaagtctgagaaataacaaggttctgtctcgaatgcttcacagaggaggttcggatttggggacaagtgtcattaatgagggccatggaagttcgtcagcttcagagtcacatgcaatctgatcctgggcggttccgctgctggggagcagctggctacggaattgaaagctaatggggaggggtggggcagcctctgggacaaggcctctctccgcagacccgggccttacaggttttcaccaggttggtactggggctctgtcgcggtaaagtagtcttccaggaagctctgcaagtactcaaaagtggggcgttcttcagggtcctttttccagcagtggatcatgagctcatgcagagagatggggcagtcctgcgggcagggcatcctgtagcctcgctccacctgctccagcacctcccggttgttcatgcctgggtatggcactcttcctttggtgaccagctctgtgagtaagattccaaaagaccacacgtcagacttgattgtgaacctcccgtacagggctgcctcgggggccgtccacttgatggggaactttgcaccttgtcttgctgtgtactcattgtcttctatcaatcgggccaatccgaagtcagcaatcttgcatatgagtccattccccactagaatgtttgctgatcgcagatctctatggatataattcatgcgctcgatgtaagccattcctgcagccacctgtgctgccatgtccacaagatttggtaatttcagagctcttccttctccatcttttaagaaatccagtaaacttcctttgttcatatactcggtgacgatgtagatgggctcctcagacaccactgcatagagctggaccagcttgtcgtgcttcagcttcttcatgatctgcgcttcctcaaggaatgattcgggggacattgtgcctggtttaagagtctttatggctacttttgtgtttccattccaggtacccatccatacttccccaaactgcccatttcccagtctcttgatcaactgcagggattctcgagggatttcccagacatctttggttttgacagacagatcggtaagccttggcatccctttgtgacagggaactactaggcggcagcagagacctgcagctctctctgagtaatgttgtacaagctgctgaagtgtttcaaactgggcccgggtggtaatgtagtatccaccattgtcaagtttgcgaattttataatgtttgacatggtctcctttcatatcatcccaatcacggatagaaagtgaataggcacctttggtggtttcactctcgcggataagaaaggtacctcttgggtttccaaaggacaatagctgtcgctcagcatcttttcggccaagttttccaaagtaccactcttctgcctggatagagtcaactggagccacataattgctgggaatgtaacctgtctctccagttgtcaaggagcgggcttcccaccaatctccttccgagctgttcaatatttgaaatttttctcctttgtgaaaactcaggtcatcttctgtccgtgcttcatagtcataaagggccacaaagagtgtcactcctgttcctcctctcgtacgcaaggtccccgtatgagacgaagagttcacacctccaaagacggtgagtccttggcccccggctgcgtggaagttgttgtagttggggatggaggtcacaccgaagctggggtagtgctgaggggtggggtctgtgccatagcggtacccagagctctggttcaggctgccgtccctctcctccgtcagttttgttgcttctttatccttacattgcacacagcccattatctaaattcccttcacgtaagcctcccttctcagctcctcagacctgcgctggtctccccctctctcagctccttggcttatacccaacacttgatcattt

SEQ ID NO: 16969 - RNA, 2681 nt, Homo sapiens
  source 1..2681: mol_type = other RNA
taggcctttagatcacttaaatgtggttacaggtttattaaattaaaaatgtctgaaacatttcagcattcatatttttatacaagaagtttgtgtggtatccatcttccagttctcttggtagtatcagccatttgcttgcttatttttaagttttgagaacaaatcgcagtaagttgaagcaaatagtgctaacagaacttgtaaattcagcttggggggtggttcctgaaaagagtcaaagtaacaaccacctacaggtacagtcatgaaccaggaaagtgcaatccaaatgaaaaaattcatgctttgcaaaagccaaaaatgaggccactggtgttttcagaataacaccggtgctttgatgctgacttgcagtaaaatcctccctctgggtcccgcagcttggtggctcaggccggccacagtctccacattagcacccacattgtatatgtacagggacatatatattatatatattcatatttataaaaaagaaaacaaaaacaaacacctgtcctgattggtttttgttaaaacatgaaaaaaaattttattgttttagacaaagaggccacttttggaaaataatacttttttttttttagttgaatcaggtgaagacagagttaaaatcacataggatttgcatttttaaaaaaggaaagcactaggattgttggcactggagtaactatttacactgaacagaggtttggccttttacataacatcgatacaatgcattttccaaagtctgagaaataacaaggttctgtctcgaatgcttcacagaggaggttcggatttggggacaagtgtcattaatgagggccatggaagttcgtcagcttcagagtcacatgcaatctgatcctgggcggttccgctgctggggagcagctggctacggaattgaaagctaatggggaggggtggggcagcctctgggacaaggcctctctccgcagacccgggccttacaggttttcaccaggttggtactggggctctgtcgcggtaaagtagtcttccaggaagctctgcaagtactcaaaagtggggcgttcttcagggtcctttttccagcagtggatcatgagctcatgcagagagatggggcagtcctgcgggcagggcatcctgtagcctcgctccacctgctccagcacctcccggttgttcatgcctgggtatggcactcttcctttggtgaccagctctgtgagtaagattccaaaagaccacacgtcagacttgattgtgaacctcccgtacagggctgcctcgggggccgtccacttgatggggaactttgcaccttgtcttgctgtgtactcattgtcttctatcaatcgggccaatccgaagtcagcaatcttgcatatgagtccattccccactagaatgtttgctgatcgcagatctctatggatataattcatgcgctcgatgtaagccattcctgcagccacctgtgctgccatgtccacaagatttggtaatttcagagctcttccttctccatcttttaagaaatccagtaaacttcctttgttcatatactcggtgacgatgtagatgggctcctcagacaccactgcatagagctggaccagcttgtcgtgcttcagcttcttcatgatctgcgcttcctcaaggaatgattcgggggacattgtgcctggtttaagagtctttatggctacttttgtgtttccattccaggtacccatccatacttccccaaactgcccatttcccagtctcttgatcaactgcagggattctcgagggatttcccagacatctttggttttgacagacagatcggtaagccttggcatccctttgtgacagggaactactaggcggcagcagagacctgcagctctctctgagtaatgttgtacaagctgctgaagtgtttcaaactgggcccgggtggtaatgtagtatccaccattgtcaagtttgcgaattttataatgtttgacatggtctcctttcatatcatcccaatcacggatagaaagtgaataggcacctttggtggtttcactctcgcggataagaaaggtacctcttgggtttccaaaggacaatagctgtcgctcagcatcttttcggccaagttttccaaagtaccactcttctgcctggatagagtcaactggagccacataattgctgggaatgtaacctgtctctccagttgtcaaggagcgggcttcccaccaatctccttccgagctgttcaatatttgaaatttttctcctttgtgaaaactcaggtcatcttctgtccgtgcttcatagtcataaagggccacaaagagtgtcactcctgttcctcctctcgtacgcaaggtccccgtatgagacgaagagttcacacctccaaagacggtgagtccttggcccccggctgcgtggaagttgttgtagttggggatggaggtcacaccgaagctggggtagtgctgaggggtggggtctgtgccatagcggtacccagagctctggttcaggctgccgtccctctcctccgtcagttttgttgcttctttatccttacattgcacacagcccattatctaaattcctgactgaaaggagaaggagaaaaggaataaagcagaaagcttcagttttcattcgattattctctccgctgt

SEQ ID NO: 16970 - RNA, 2658 nt, Homo sapiens
  source 1..2658: mol_type = other RNA
taggcctttagatcacttaaatgtggttacaggtttattaaattaaaaatgtctgaaacatttcagcattcatatttttatacaagaagtttgtgtggtatccatcttccagttctcttggtagtatcagccatttgcttgcttatttttaagttttgagaacaaatcgcagtaagttgaagcaaatagtgctaacagaacttgtaaattcagcttggggggtggttcctgaaaagagtcaaagtaacaaccacctacaggtacagtcatgaaccaggaaagtgcaatccaaatgaaaaaattcatgctttgcaaaagccaaaaatgaggccactggtgttttcagaataacaccggtgctttgatgctgacttgcagtaaaatcctccctctgggtcccgcagcttggtggctcaggccggccacagtctccacattagcacccacattgtatatgtacagggacatatatattatatatattcatatttataaaaaagaaaacaaaaacaaacacctgtcctgattggtttttgttaaaacatgaaaaaaaattttattgttttagacaaagaggccacttttggaaaataatacttttttttttttagttgaatcaggtgaagacagagttaaaatcacataggatttgcatttttaaaaaaggaaagcactaggattgttggcactggagtaactatttacactgaacagaggtttggccttttacataacatcgatacaatgcattttccaaagtctgagaaataacaaggttctgtctcgaatgcttcacagaggaggttcggatttggggacaagtgtcattaatgagggccatggaagttcgtcagcttcagagtcacatgcaatctgatcctgggcggttccgctgctggggagcagctggctacggaattgaaagctaatggggaggggtggggcagcctctgggacaaggcctctctccgcagacccgggccttacaggttttcaccaggttggtactggggctctgtcgcggtaaagtagtcttccaggaagctctgcaagtactcaaaagtggggcgttcttcagggtcctttttccagcagtggatcatgagctcatgcagagagatggggcagtcctgcgggcagggcatcctgtagcctcgctccacctgctccagcacctcccggttgttcatgcctgggtatggcactcttcctttggtgaccagctctgtgagtaagattccaaaagaccacacgtcagacttgattgtgaacctcccgtacagggctgcctcgggggccgtccacttgatggggaactttgcaccttgtcttgctgtgtactcattgtcttctatcaatcgggccaatccgaagtcagcaatcttgcatatgagtccattccccactagaatgtttgctgatcgcagatctctatggatataattcatgcgctcgatgtaagccattcctgcagccacctgtgctgccatgtccacaagatttggtaatttcagagctcttccttctccatcttttaagaaatccagtaaacttcctttgttcatatactcggtgacgatgtagatgggctcctcagacaccactgcatagagctggaccagcttgtcgtgcttcagcttcttcatgatctgcgcttcctcaaggaatgattcgggggacattgtgcctggtttaagagtctttatggctacttttgtgtttccattccaggtacctgagtaatgttgtacaagctgctgaagtgtttcaaactgggcccgggtggtaatgtagtatccaccattgtcaagtttgcgaattttataatgtttgacatggtctcctttcatatcatcccaatcacggatagaaagtgaataggcacctttggtggtttcactctcgcggataagaaaggtacctcttgggtttccaaaggacaatagctgtcgctcagcatcttttcggccaagttttccaaagtaccactcttctgcctggatagagtcaactggagccacataattgctgggaatgtaacctgtctctccagttgtcaaggagcgggcttcccaccaatctccttccgagctgttcaatatttgaaatttttctcctttgtgaaaactcaggtcatcttctgtccgtgcttcatagtcataaagggccacaaagagtgtcactcctgttcctcctctcgtacgcaaggtccccgtatgagacgaagagttcacacctccaaagacggtgagtccttggcccccggctgcgtggaagttgttgtagttggggatggaggtcacaccgaagctggggtagtgctgaggggtggggtctgtgccatagcggtacccagagctctggttcaggctgccgtccctctcctccgtcagttttgttgcttctttatccttacattgcacacagcccattatctaaattccaaaatgtccgccaacgatcacaaactttatatacaccacatgtcttctacaacagaggcaggactggtctttttccacgtttagatcagcatcctgcttcttcaaaaaaactgcgcggcgctgaggctccggagcccactcacatggtcctctccccgccctcctccggcgcggccgaggcggctccggggggtccccggcgggcccgggagcc

SEQ ID NO: 16971 - RNA, 2485 nt, Homo sapiens
  source 1..2485: mol_type = other RNA
taggcctttagatcacttaaatgtggttacaggtttattaaattaaaaatgtctgaaacatttcagcattcatatttttatacaagaagtttgtgtggtatccatcttccagttctcttggtagtatcagccatttgcttgcttatttttaagttttgagaacaaatcgcagtaagttgaagcaaatagtgctaacagaacttgtaaattcagcttggggggtggttcctgaaaagagtcaaagtaacaaccacctacaggtacagtcatgaaccaggaaagtgcaatccaaatgaaaaaattcatgctttgcaaaagccaaaaatgaggccactggtgttttcagaataacaccggtgctttgatgctgacttgcagtaaaatcctccctctgggtcccgcagcttggtggctcaggccggccacagtctccacattagcacccacattgtatatgtacagggacatatatattatatatattcatatttataaaaaagaaaacaaaaacaaacacctgtcctgattggtttttgttaaaacatgaaaaaaaattttattgttttagacaaagaggccacttttggaaaataatacttttttttttttagttgaatcaggtgaagacagagttaaaatcacataggatttgcatttttaaaaaaggaaagcactaggattgttggcactggagtaactatttacactgaacagaggtttggccttttacataacatcgatacaatgcattttccaaagtctgagaaataacaaggttctgtctcgaatgcttcacagaggaggttcggatttggggacaagtgtcattaatgagggccatggaagttcgtcagcttcagagtcacatgcaatctgatcctgggcggttccgctgctggggagcagctggctacggaattgaaagctaatggggaggggtggggcagcctctgggacaaggcctctctccgcagacccgggccttacaggttttcaccaggttggtactggggctctgtcgcggtaaagtagtcttccaggaagctctgcaagtactcaaaagtggggcgttcttcagggtcctttttccagcagtggatcatgagctcatgcagagagatggggcagtcctgcgggcagggcatcctgtagcctcgctccacctgctccagcacctcccggttgttcatgcctgggtatggcactcttcctttggtgaccagctctgtgagtaagattccaaaagaccacacgtcagacttgattgtgaacctcccgtacagggctgcctcgggggccgtccacttgatggggaactttgcaccttgtcttgctgtgtactcattgtcttctatcaatcgggccaatccgaagtcagcaatcttgcatatgagtccattccccactagaatgtttgctgatcgcagatctctatggatataattcatgcgctcgatgtaagccattcctgcagccacctgtgctgccatgtccacaagatttggtaatttcagagctcttccttctccatcttttaagaaatccagtaaacttcctttgttcatatactcggtgacgatgtagatgggctcctcagacaccactgcatagagctggaccagcttgtcgtgcttcagcttcttcatgatctgcgcttcctcaaggaatgattcgggggacattgtgcctggtttaagagtctttatggctacttttgtgtttccattccaggtacctgagtaatgttgtacaagctgctgaagtgtttcaaactgggcccgggtggtaatgtagtatccaccattgtcaagtttgcgaattttataatgtttgacatggtctcctttcatatcatcccaatcacggatagaaagtgaataggcacctttggtggtttcactctcgcggataagaaaggtacctcttgggtttccaaaggacaatagctgtcgctcagcatcttttcggccaagttttccaaagtaccactcttctgcctggatagagtcaactggagccacataattgctgggaatgtaacctgtctctccagttgtcaaggagcgggcttcccaccaatctccttccgagctgttcaatatttgaaatttttctcctttgtgaaaactcaggtcatcttctgtccgtgcttcatagtcataaagggccacaaagagtgtcactcctgttcctcctctcgtacgcaaggtccccgtatgagacgaagagttcacacctccaaagacggtgagtccttggcccccggctgcgtggaagttgttgtagttggggatggaggtcacaccgaagctggggtagtgctgaggggtggggtctgtgccatagcggtacccagagctctggttcaggctgccgtccctctcctccgtcagttttgttgcttctttatccttacattgcacacagcccattatctaaattcccttcacgtaagcctcccttctcagctcctcagacctgcgct

SEQ ID NO: 16972 - RNA, 2603 nt, Homo sapiens
  source 1..2603: mol_type = other RNA
taggggcagcagaggacctgggctctaaagtcccggctttgtccctggctggctgcatgacccaggcatgtatgacccttgccttctctcagcctgtctccatatctgtcacgtggccttccaggtttcttctagttgtcagagtctccagttgatggctaagtgggctttcctggtgtccctggcagcacgctgctttgcccgtttaaacacacacctccataacaaacgggcaaacaaaaggggcggggcagacagtaaacaccgcagattccaagcggtggcttcagtgagactgcttagtgtgagaagtacgcgtgagccgggtctggaaatggggcaggagtcagggagggcacacaccaggtgggcagaaacagaatacgcccaaatgaggacagaacccttccctgccgggagtcgggcgccagctccagtgctgctctgttcctatttgtgggactgcagggaaggtcccttttatgtcataatgaagaggtcacagaccaggtgtcctaaaattccacccagcaggagcatgctgtgcctcttaagtgtggtcacagtgtccagcgactcagctccagagaggagctgatgggtgtgggagatgccggcttttcagccgatgacaggcccggccggcaggagcagagagcccaaggcagaagcacctgccacccagtgtgggccacgggcaccgtctccaaggcgtgctgagcctttgccaaatccacacatcaaacgacaatttgattctcacacttggatccctgaatgctagctggcactgactgtctgagctacagcccttaaatctgtctcctcaccactgaggaaaggagtctgtgctctattaaaagcattttttaaaaaccagagaatgctaaatgtgtttgaaaaataaaaaccgaccaaaaaatacattttatccctctttagagttgttatcttcccatatattcgtggtgctgggcaccagctgggaatgcaagtctgaagactgtgtgagcaaggccccctctgcagaagcagagaccgcattggagccagccagagactcttccccagtccacgcatccccagacactgaagtgaatggttgagggccttttccctgtttctgtctctcaggttgaccctttacaatccatagtacatgcagttcccagatggggaaataatctctcagatccagtttgtggcctggcacccatctcactgccagagaaccacggcttgtctgtgccctccgtgtcccaagtatgcacttccctccgcctgggttgccattccccgacttgacccagcttacactgattcagtgcgatccaggcacgatctactccaagacgcccttgggcacagtccaggcatgatctactccaagaagccctctgccaagggtaggagctcagagctccacttttggttaatattacacctcccttaacatatcccggatacacggccatctgccgggaaagcttcttgaggccagggccatgtctctctcactttccttggcatcaggaacttagcacagaagcagtgctccgtgaagcctgatggctgggagcattcccagagtctgacggatccagccttgccttgtcatgtcagctgtgtccagctgcctccactggctatgcacttggaaggccctctctggcccagccacactgctcactctgagaccttgacctgcacttctaacgttcgcttccctaactgctatggaccgtttggccccttggaaagccttccccgttatctgtaggtgctgccaatccatgtccaccacatgccttgggctggtttaaaaacgcaatctcctgggggctgccatgaatgaatcccagctcactgccatcctggacacaactaggcctcagtttttaccaaggaccttaggggggggtcaccagatctggcagacaggctgtttttcaatgggtgatggctgcctccatcctgcgtctccatcacgcccggactctgcagaggaagagaaggccggaccgttccttagcccacagaaggcgtgactggcatatcttcactcccatcatgagacgggatgcagaaacgcatatcttttttccttagaagtgtgccagcagttagagccttgaattcggaaagagtgatgattccctgtagtggtatatcggtttgcatttgctaactgctttcaagttttctttcctgagtagatatttctagtccaagtaggctgtgagcagagtctgtgcctcattcatccctctgttcccatactgtgcattcgttcctaacaggtaatccataaatgcttgttacctaactaaaggcaaattaaatgctaaacagcactaatgacaagctgttgcaagatcccggctctcaggaaagaattacttgtggttgtcaggggcctgcctgttgcccaggtgtaggaaacatgaaacacttctttcccaactgcttctctattccagaggtggtgcattcttctaagattgctgcaatataatgtttgggaggcaggtttcattaaaattattttttgagacagagtcccactctgtcacccaggctggagtgcagtagtgcgatctcag

SEQ ID NO: 16973 - RNA, 1637 nt, Homo sapiens
  source 1..1637: mol_type = other RNA
tagggggtggcaggctggcctgggccgcgtggaggctgcgggtcccacccgccaggaccccggtgggcgcgagccgcgtctgtgaagctgccgtgacatggggggtccttgtctcgggaaaagcgggtctgtcctgtctctctcctaccaggcacaagtgcacggctctggttcggggggagtgttggggcgtggtgacgggtgggggcccctgtccctctttccagcgaaagaaaactcggaaggaacatgtaacaacacgccaagtcctggacccgtgaggctgtgggtggagggtgggcaggcgccgggaggggccgggctggtgggtgtctgtggtgtggggtgggggccggggtctcgggggccggctcacatgatggagcagcatttacaacggtgcttcttcatgtcgaggtcctgggggtcgctggtggtggcctcgggccccgcctgattctcttccctggaggcggcctccgtgggaggctcggcagcactgccgttgggtggtgcaggctccttgggctcagccgcgtcttcgatgaccaccagctccgccgtgatggtatcttgaaggcccagcaccttcttggtctcggcctcatcctccacgttctggtaacccatgaagatcattgtgaccgggggctcctggccgggctggatccccggcgggccggacgtggcctcgcctggctgtgcctgcacaccggtgatctcccgccgggagggcgtggtccgggctgccccctccacagccccccgggtctctgccgccccggccgtggaccctgcctcgctcagcgtgacctcgtccgctttgtggatgagttcgtccacctcggaggagctcagggggtggatcccgttctcggcggtgccgtccacagcatggaccactgccttcatcatgggggagccgtcaaccgtcctcaggggcgtgttggagactcgcttgtctttgggcgtgcccaccggcgtctgctgtgaattcatcaccacctctgtcttgcgctcctccttggctggactcggggctggggcccggactgggctcggggccgccgcgttctccttggcagtggctggggcggagtctccacgctccagcacctcaatttccttctccaacctggacaccgagtcctccagcagccgtgtcttctgctcgtcgtcctgcatctgcctcctcaggtcctcatccccctctgaggccgaggacggcgtcccctccagcagccagcgctcccgcagtgccttggacttcaggtgctgcagctgcctccgctcgtcctccagctgccggcgcttgttctcgatctccgcctgccgcttccgcttctctgcgatggcctgcagccgctcctgctgggacgtggtctctgccgccaggacccttggcagcatcggccctgtggttagcaacccgctagttctccttaaatcctcacattaacaaaaaataacctgttcttgaatgacatttaaaattctttaaattcttaaattcatttgtgaaactttccagcgagacgggcaccaccacaaaccacagccagctcccgtgtcttcgactggaaaatctgtggaaacgggaggaggcaagcgatcacgttctagcggacggggccttc

SEQ ID NO: 16974 - RNA, 1616 nt, Homo sapiens
  source 1..1616: mol_type = other RNA
tagggggtggcaggctggcctgggccgcgtggaggctgcgggtcccacccgccaggaccccggtgggcgcgagccgcgtctgtgaagctgccgtgacatggggggtccttgtctcgggaaaagcgggtctgtcctgtctctctcctaccaggcacaagtgcacggctctggttcggggggagtgttggggcgtggtgacgggtgggggcccctgtccctctttccagcgaaagaaaactcggaaggaacatgtaacaacacgccaagtcctggacccgtgaggctgtgggtggagggtgggcaggcgccgggaggggccgggctggtgggtgtctgtggtgtggggtgggggccggggtctcgggggccggctcacatgatggagcagcatttacaacggtgcttcttcatgtcgaggtcctgggggtcgctggtggtggcctcgggccccgcctgattctcttccctggaggcggcctccgtgggaggctcggcagcactgccgttgggtggtgcaggctccttgggctcagccgcgtcttcgatgaccaccagctccgccgtgatggtatcttgaaggcccagcaccttcttggtctcggcctcatcctccacgttctggtaacccatgaagatcattgtgaccgggggctcctggccgggctggatccccggcgggccggacgtggcctcgcctggctgtgcctgcacaccggtgatctcccgccgggagggcgtggtccgggctgccccctccacagccccccgggtctctgccgccccggccgtggaccctgcctcgctcagcgtgacctcgtccgctttgtggatgagttcgtccacctcggaggagctcagggggtggatcccgttctcggcggtgccgtccacagcatggaccactgccttcatcatgggggagccgtcaaccgtcctcaggggcgtgttggagactcgcttgtctttgggcgtgcccaccggcgtctgctgtgaattcatcaccacctctgtcttgcgctcctccttggctggactcggggctggggcccggactgggctcggggccgccgcgttctccttggcagtggctggggcggagtctccacgctccagcacctcaatttccttctccaacctggacaccgagtcctccagcagccgtgtcttctgctcgtcgtcctgcatctgcctcctcaggtcctcatccccctctgaggccgaggacggcgtcccctccagcagccagcgctcccgcagtgccttggacttcaggtgctgcagctgcctccgctcgtcctccagctgccggcgcttgttctcgatctccgcctgccgcttccgcttctctgcgatggcctgcagccgctcctgctgggacgtggtctctgccgccaggacctccatctccccgccgaggtccgggtgggtccgcggtgccgggcgggggcgggcgcgggtggcgcgcgggggaggggaggggagggggacgcggcctggcgggggccggggcgggctaaggcctggcggccggggctgcgcggcgcgggggcggcggcaccggctcgggcatcgccccgcgcaaagctgctgtttattgtccgggcggcggcgggcgc

SEQ ID NO: 16975 - RNA, 2089 nt, Homo sapiens
  source 1..2089: mol_type = other RNA
tagggggtggcaggctggcctgggccgcgtggaggctgcgggtcccacccgccaggaccccggtgggcgcgagccgcgtctgtgaagctgccgtgacatggggggtccttgtctcgggaaaagcgggtctgtcctgtctctctcctaccaggcacaagtgcacggctctggttcggggggagtgttggggcgtggtgacgggtgggggcccctgtccctctttccagcgaaagaaaactcggaaggaacatgtaacaacacgccaagtcctggacccgtgaggctgtgggtggagggtgggcaggcgccgggaggggccgggctggtgggtgtctgtggtgtggggtgggggccggggtctcgggggccggctcacatgatggagcagcatttacaacggtgcttcttcatgtcgaggtcctgggggtcgctggtggtggcctcgggccccgcctgattctcttccctggaggcggcctccgtgggaggctcggcagcactgccgttgggtggtgcaggctccttgggctcagccgcgtcttcgatgaccaccagctccgccgtgatggtatcttgaaggcccagcaccttcttggtctcggcctcatcctccacgttctggtaacccatgaagatcattgtgaccgggggctcctggccgggctggatccccggcgggccggacgtggcctcgcctggctgtgcctgcacaccggtgatctcccgccgggagggcgtggtccgggctgccccctccacagccccccgggtctctgccgccccggccgtggaccctgcctcgctcagcgtgacctcgtccgctttgtggatgagttcgtccacctcggaggagctcagggggtggatcccgttctcggcggtgccgtccacagcatggaccactttggtctcgtcctcgtagactttgatgcccagagggagcggctgccgagggagcagcgtggtgctggacagcaccctggtctcccctgtcaccttgtccttctccacagtgatctcaaccgagtacatggctgccttcatcatgggggagccgtcaaccgtcctcaggggcgtgttggagactcgcttgtctttgggcgtgcccaccggcgtctgctgtgaattcatcaccacctctgtcttgcgctcctccttggctggactcggggctggggcccggactgggctcggggccgccgcgttctccttggcagtggctggggcggagtctccacgctccagcacctcaatttccttctccaacctggacaccgagtcctccagcagccgtgtcttctgctcgtcgtcctgcatctgcctcctcaggtcctcatccccctctgaggccgaggacggcgtcccctccagcagccagcgctcccgcagtgccttggacttcaggtgctgcagctgcctccgctcgtcctccagctgccggcgcttgttctcgatctccgcctgccgcttccgcttctctgcgatggcctgcagccgctcctgctgggacgtggtctctgccgccaggaccatgctgggcggaggagctgagtcccgggcaaaggcgtggaaaagctcagggcggcggcggtcctggtgctgctgggggtcccagggcaggtgctgggggtcccggggcaggtgctgggtctccgagcctccctggctcccggcagccgcgcagagcccctggagcgccacgccccccgcccgacgcccaccccggcgcgcacaggcctcccgtccccgcgatgctttttacggcgtgtggcggtgtgggcggctcggggcccggcgagggcgtcgtctggagcgcgtgagatagtcctgctccaggagatgagttcatgaggcccaaacccgacgggagccccgcagaggcctccgcggtgcggggcgttggtgttggaagggcccagagaggttacgcaacggccaaggtcacccagcgagcagggcgggccctgtccgaggcgggaggggcgtgtgtgggatgggggcgtcgcactcgtccttccagaacccacgcccgggcagctccagccagaacgagggggtccctgcccgggcaggcgccgagcccagcgcc

SEQ ID NO: 16976 - RNA, 1746 nt, Homo sapiens
  source 1..1746: mol_type = other RNA
tagggggtggcaggctggcctgggccgcgtggaggctgcgggtcccacccgccaggaccccggtgggcgcgagccgcgtctgtgaagctgccgtgacatggggggtccttgtctcgggaaaagcgggtctgtcctgtctctctcctaccaggcacaagtgcacggctctggttcggggggagtgttggggcgtggtgacgggtgggggcccctgtccctctttccagcgaaagaaaactcggaaggaacatgtaacaacacgccaagtcctggacccgtgaggctgtgggtggagggtgggcaggcgccgggaggggccgggctggtgggtgtctgtggtgtggggtgggggccggggtctcgggggccggctcacatgatggagcagcatttacaacggtgcttcttcatgtcgaggtcctgggggtcgctggtggtggcctcgggccccgcctgattctcttccctggaggcggcctccgtgggaggctcggcagcactgccgttgggtggtgcaggctccttgggctcagccgcgtcttcgatgaccaccagctccgccgtgatggtatcttgaaggcccagcaccttcttggtctcggcctcatcctccacgttctggtaacccatgaagatcattgtgaccgggggctcctggccgggctggatccccggcgggccggacgtggcctcgcctggctgtgcctgcacaccggtgatctcccgccgggagggcgtggtccgggctgccccctccacagccccccgggtctctgccgccccggccgtggaccctgcctcgctcagcgtgacctcgtccgctttgtggatgagttcgtccacctcggaggagctcagggggtggatcccgttctcggcggtgccgtccacagcatggaccactttggtctcgtcctcgtagactttgatgcccagagggagcggctgccgagggagcagcgtggtgctggacagcaccctggtctcccctgtcaccttgtccttctccacagtgatctcaaccgagtacatggctgccttcatcatgggggagccgtcaaccgtcctcaggggcgtgttggagactcgcttgtctttgggcgtgcccaccggcgtctgctgtgaattcatcaccacctctgtcttgcgctcctccttggctggactcggggctggggcccggactgggctcggggccgccgcgttctccttggcagtggctggggcggagtctccacgctccagcacctcaatttccttctccaacctggacaccgagtcctccagcagccgtgtcttctgctcgtcgtcctgcatctgcctcctcaggtcctcatccccctctgaggccgaggacggcgtcccctccagcagccagcgctcccgcagtgccttggacttcaggtgctgcagctgcctccgctcgtcctccagctgccggcgcttgttctcgatctccgcctgccgcttccgcttctctgcgatggcctgcagccgctcctgctgggacgtggtctctgccgccaggacccttggcagcatcggccctgtggttagcaacccgctagttctccttaaatcctcacattaacaaaaaataacctgttcttgaatgacatttaaaattctttaaattcttaaattcatttgtgaaactttccagcgagacgggcaccaccacaaaccacagccagctcccgtgtcttcgactggaaaatctgtggaaacgggaggaggcaagcgatc

SEQ ID NO: 16977 - RNA, 1748 nt, Homo sapiens
  source 1..1748: mol_type = other RNA
tagggggtggcaggctggcctgggccgcgtggaggctgcgggtcccacccgccaggaccccggtgggcgcgagccgcgtctgtgaagctgccgtgacatggggggtccttgtctcgggaaaagcgggtctgtcctgtctctctcctaccaggcacaagtgcacggctctggttcggggggagtgttggggcgtggtgacgggtgggggcccctgtccctctttccagcgaaagaaaactcggaaggaacatgtaacaacacgccaagtcctggacccgtgaggctgtgggtggagggtgggcaggcgccgggaggggccgggctggtgggtgtctgtggtgtggggtgggggccggggtctcgggggccggctcacatgatggagcagcatttacaacggtgcttcttcatgtcgaggtcctgggggtcgctggtggtggcctcgggccccgcctgattctcttccctggaggcggcctccgtgggaggctcggcagcactgccgttgggtggtgcaggctccttgggctcagccgcgtcttcgatgaccaccagctccgccgtgatggtatcttgaaggcccagcaccttcttggtctcggcctcatcctccacgttctggtaacccatgaagatcattgtgaccgggggctcctggccgggctggatccccggcgggccggacgtggcctcgcctggctgtgcctgcacaccggtgatctcccgccgggagggcgtggtccgggctgccccctccacagccccccgggtctctgccgccccggccgtggaccctgcctcgctcagcgtgacctcgtccgctttgtggatgagttcgtccacctcggaggagctcagggggtggatcccgttctcggcggtgccgtccacagcatggaccactttggtctcgtcctcgtagactttgatgcccagagggagcggctgccgagggagcagcgtggtgctggacagcaccctggtctcccctgtcaccttgtccttctccacagtgatctcaaccgagtacatggctgccttcatcatgggggagccgtcaaccgtcctcaggggcgtgttggagactcgcttgtctttgggcgtgcccaccggcgtctgctgtgaattcatcaccacctctgtcttgcgctcctccttggctggactcggggctggggcccggactgggctcggggccgccgcgttctccttggcagtggctggggcggagtctccacgctccagcacctcaatttccttctccaacctggacaccgagtcctccagcagccgtgtcttctgctcgtcgtcctgcatctgcctcctcaggtcctcatccccctctgaggccgaggacggcgtcccctccagcagccagcgctcccgcagtgccttggacttcaggtgctgcagctgcctccgctcgtcctccagctgccggcgcttgttctcgatctccgcctgccgcttccgcttctctgcgatggcctgcagccgctcctgctgggacgtggtctctgccgccaggacctccatctccccgccgaggtccgggtgggtccgcggtgccgggcgggggcgggcgcgggtggcgcgcgggggaggggaggggagggggacgcggcctggcgggggccggggcgggctaaggcctggcggccggggctgcgcggcgcgggggcggcggcaccggctcgggcatcgccccgcgcaaagctgctgtttattgtccgggcggcggcgggcgc

SEQ ID NO: 16978 - RNA, 686 nt, Homo sapiens
  source 1..686: mol_type = other RNA
taggggtgggggaattcaggggtgttgctaccaggattgagctccctcaggcctagatcaactagtttcactcttcaaaaattttcccgtgagataaataggctccagagatctcatcagacactgtgaggctagtataattaccatcgccattttatggatatggaaactgaggctcactggggtcaagtgacgtacccagggctacttaaagaggctgtcatgttttctgcttcttaaacctcacggtaccagcccgcatccctcgccaaagggtacgcgccctttccgagccaggattatgacccaggtcacccaaacgcctagcccagtacttccatgccgcagcctgcccttgctaggtatgcttagggtagttgggccctatctgagaatctgggacatcctgttgaacggcagctctggaccctctgggtaagactaacaccccctgcgcaggctggagaagtcgctctgacccagggtcctcagagccaaaggcctcgtgggggctgccttctgtcagcccagccgtgtccgcaacccgtttctggccggctccttttggacacagtcccttctgggtactaatcatccacgctcaccccagaggggccacggcccaaggaccactcccgagggagcctgcagagccccaccaggccacagggccggaagcagacgag

SEQ ID NO: 16979 - RNA, 261 nt, Homo sapiens
  source 1..261: mol_type = other RNA
taggggtgggggaattcaggggtgttgctaccaggattgagctccctcaggcctccagggtcctcagagccaaaggcctcgtgggggctgccttctgtcagcccagccgtgtccgcaacccgtttctggccggctccttttggacacagtcccttctgggtactaatcatccacgctcaccccagaggggccacggcccaaggaccactcccgagggagcctgcagagccccaccaggccacagggccggaagcagacgag

SEQ ID NO: 16980 - RNA, 373 nt, Homo sapiens
  source 1..373: mol_type = other RNA
taggggtgggggaattcaggggtgttgctaccaggattgagctccctcaggcctcccagaggggccacggcccaaggaccactcccgagggagcctgcagagccccaccaggccacagggccggaagcagacgagggcgggaggctggaaaggaagaggcggcgcccgaggctgctatggcggaggggcggggctccccgcttctccgggcgtctgtctcatttctaccggcttccatttgacagcttccctcccgccagaactccagggctcccaagctggcgcggggtcctcagcccctgcccgtcccgacctccccggcggggaccgaacctcagctcctccatccggggcccacgcggcccgcgcctgc

SEQ ID NO: 16981 - RNA, 219 nt, Homo sapiens
  source 1..219: mol_type = other RNA
taggggtgggggaattcaggggtgttgctaccaggattgagctccctcaggcctccttgtaacggaaactgttagaacaactttgcaccctccttaaaggaaacagatgataaatccttctccgttggtggatttcttgtttctcaggattccaaagccttatgtggtttcagttatctgccctccaaacgaagccaggggccgggttagcctctggcc

SEQ ID NO: 16982 - RNA, 495 nt, Homo sapiens
  source 1..495: mol_type = other RNA
taggggtgggggaattcaggggtgttgctaccaggattgagctccctcaggcctctcagctcctccatccggggcccacgcggcccgcgcctgcgcgctggctccgccgacggcgtccccgccccgctcctgcccggacttggagcagccccgcctccctgcgcggcggccatgttgactccgggcgagcgggatgggggtcgccgctcggcgcctcgcctcgtagcaccttcccaccttggtgacacctgaagagttctctcgcacttcgctctccttcaaggccccccgccaccccgccttcaaatagtgagcggaggctgctgtctcagagtcagtgctcttgccccagctcccgctgacgttcactgagttcccggtgtgggccgaggctcttgtagtcggaggctgacccgcagcctcttcacagaaaccagagccgcgctcttcctgctgtcaggcaacaacagctcagcacagggcctgacacacaat

SEQ ID NO: 16983 - RNA, 312 nt, Homo sapiens
  source 1..312: mol_type = other RNA
taggggtgggggaattcaggggtgttgctaccaggattgagctccctcaggcctcttggtgacacctgaagagttctctcgcacttcgctctccttcaaggccccccgccaccccgccttcaaatagtgagcggaggctgctgtctcagagtcagtgctcttgccccagctcccgctgacgttcactgagttcccggtgtgggccgaggctcttgtagtcggaggctgacccgcagcctcttcacagaaaccagagccgcgctcttcctgctgtcaggcaacaacagctcagcacagggcctgacacacaat

SEQ ID NO: 16984 - RNA, 817 nt, Homo sapiens
  source 1..817: mol_type = other RNA
taggtagagtgtgaggaggaggtcgtgaacagtctctttctcgcggtctaggggctgttccaacaccagctccggatacttttgtccatcagttccgcttaccacatccagagagaagtgcagattggagctgagctggtaactccggagagagttcacacccacatccgcatcccgcgcgaagggaagcactaaccgtgtccctgcagccgcattttcattaacttttacttttaactcttcatcccggaaacgcgggaagttatcattaatatcgattatttctacttctactccataaattttcattttgttctcaaccaagatgttaaagttcaccacacacagtgggctctgagcgcagagctcctcccggtctatcctgcccgcggtgaccaagctgccgcttcgcgggttcagggcaaaaagctgcgtcctacctctggagacgatgcggactccgcgctccgccagctcctggggctccagcccaaggtccttggctatgttgccgacgaaggagcctttgtccagctcctccggcatcgagtagcggatctgcccggatcctggctcgcacagcgtccccaggagcatgaagggcagcagcagctctccgcagccccagcccctaggtggactcgccattgccttctctctgcccaattttctcttagttctggttcagcctgctgtttccttatttatctaaagccgatgggtacatattccctgacgaaaatgggcgtggagcgttggcttttcgtaggagcttgtctggtctgtgtgtttagtatggagggagcagagtcgggtc

SEQ ID NO: 16985 - RNA, 711 nt, Homo sapiens
  source 1..711: mol_type = other RNA
taggtagagtgtgaggaggaggtctcctccgcagggggagtgtactccccggagcagtcctccccttcagggttctcaaattccttgaagccgacatcgccccgtttgcagcacagacaggtgaggaggaggaagatgaaggccagcaggccggagcaggaaatgaggaccacagcgtagggaggagccagaggagcccggcccagggcgaatccatcggggtgggccggggacgccaggcagccggaggcggagacggccgcaaggaggatgagggcgccgggggcaggcatcttgtcgaggatggcagggaggtggaggtggtggcggccggaagcgcggactcccaccctgggcgcggacctctccatcgtccgtgagcacctgcgaggcgttcccctgggtgaggctgggccggagctgcgcacccaagacgcagcctcagcaacactcggcgcaggcgacccagcccccaaccccaacccccagcaggggcccagggctttccaccaaaacgcgcagccgtggcgcacaccggccgggcagtgcacactccccgcagagcgcagccgtcctcatcggggggctcaggggaaggggctgccctcagggtgtctcattggagaaactgaggcaggttcatcgcgggagggagggggcgcacggcctaggctgcagggtggaggggatgcaatcggggggcggggagtg

SEQ ID NO: 16986 - RNA, 678 nt, Homo sapiens
  source 1..678: mol_type = other RNA
taggtagagtgtgaggaggaggtctcctccgcagggggagtgtactccccggagcagtcctccccttcagggttctcaaattccttgaagccgacatcgccccgtttgcagcacagacaggtgaggaggaggaagatgaaggccagcaggccggagcaggaaatgaggaccacagcgtagggaggagccagaggagcccggcccagggcgaatccatcggggtgggccggggacgccaggcagccggaggcggagacggccgcaaggaggatgagggcgccgggggcaggcatcttgtcgaggatggcagggaggtggaggtggtggcggctctccatcgtccgtgagcacctgcgaggcgttcccctgggtgaggctgggccggagctgcgcacccaagacgcagcctcagcaacactcggcgcaggcgacccagcccccaaccccaacccccagcaggggcccagggctttccaccaaaacgcgcagccgtggcgcacaccggccgggcagtgcacactccccgcagagcgcagccgtcctcatcggggggctcaggggaaggggctgccctcagggtgtctcattggagaaactgaggcaggttcatcgcgggagggagggggcgcacggcctaggctgcagggtggaggggatgcaatcggggggcggggagtg

SEQ ID NO: 16987 - RNA, 552 nt, Homo sapiens
  source 1..552: mol_type = other RNA
taggtagagtgtgaggaggaggtctcctccgcagggggagtgtactccccggagcagtcctccccttcagggttctcaaattccttgaagccgacatcgccccgtttgcagcacagacaggtgaggaggaggaagatgaaggccagcaggccggagcaggaaatgaggaccacagcgtagggaggagccagaggagcccggcccagggcgaatccatcggggtgggccggggacgccaggcagccggaggcggagacggccgcaaggaggatgagggcgccgggggcaggcatcttgtcgaggatggcagggaggtggaggtggtggcggctggggaggaggggggggcgggccctcagcccccagccatggggacccgcgcgaccctggcctcctcccggcccaggagaggggcaggagacgcaggacagggggagggaggggctgcttgctggctcaggtacccccctccccctctttgaagggacagacggatgaagggatggagaggcggacagaggagagatgctggggagccggggttgctggggt

SEQ ID NO: 16988 - RNA, 353 nt, Homo sapiens
  source 1..353: mol_type = other RNA
taggtagagtgtgaggaggaggtctcctccgcagggggagtgtactccccggagcagtcctccccttcagggttctcaaattccttgaagccgacatcgccccgtttgcagcacagacaggtgaggaggaggaagatgaaggccagcaggccggagcaggaaatgaggaccacagcgtagggaggagccagaggagcccggcccagggcgaatccatcggggtgggccggggacgccaggcagccggaggcggagacggccgcaaggaggatgagggcgccgggggcaggcatcttgtcgaggatggcagggaggtggaggtggtggcgggtttcccgtgcggttacgcagac

SEQ ID NO: 16989 - RNA, 3393 nt, Homo sapiens
  source 1..3393: mol_type = other RNA
taggtagtttcatgttgttgggagaacttagcagaaatcggtaccttggtcattacaaagaagcacgttcaaaggaaaaaaaagacaattgcacaaggaggctttttacacggggaggggaggggcatggggggctcagccgggcctttgccgctcgccctcacagggcgagggagcctttgcttaaatccttttctttccccccggcccccaagagaagggaaggagatccacggtagctcacacacagaagctattacgagatactaccactagcggggactggcgcggcgggggacgctgcggtgggaggcccggctcctggccccgctagcggggccagagctctctcgggcaggggcgcgcggcggcggcgcggccgggacccgcggacgtgcgggcggccgcggccctggcagtcccagctgaagcctacttcttgtcgcccttctgcgcgtcgccctcgtccgccgcctctggggcccgctccagcttctgtttctccagctcctcctgctcgcatttgctgctggggaacttgtctttgttgttctcttttttccacttcatcctccggttctggaaccagattttgacctgtctctctgtcagtcccagggcgtgcgatacctcgattcgccgcttacgagtcagatagggattaaataggaactccttctccagctccagggtctggtagcggctgtaggtctgtcggcctcgcctgcgtccggcggctgcttgcgggcgcatccaggggaagagctgtgtgggcgacgggctctgctcggagccctcggcctcctcgcccaggccgctggcggcggcaagcttgcagtctgcgtactgcaccaggtctggatcctgcgcaccgaataggctctggcgttgcagcgggtcgtagccgtagaaattgccggggtccccgtggcacgccacggcgcacgggttctgctggtagggagccgtggacagcgacgacggcccgtggtagaactcctggatttgcgacgggtgctggaagctgccgccgctgctgggaccgtacaccacggtgggtcggccgcccaggtcctgggcgaagccgcagtcataataattggggcgcagggactccccggttttgtatttggagaacagtgagttgacgaaataagagctcattttattgaattttgaggcggcggcggcggcggaggctatagttgggggcaccacttaaagaggtcctcgctttacatttcgaagaagggatgccagttcataaacagttttcggtgatttacttccctgcaaatgagttgtttcatattttgcactgtcttttcatgatcatttgcatccattagagaccccgcatcctattggcttcttcgtactcctcccggacagaacgcagagcgagggtgagagcgagagagagcgagcgagagagagagcggcgaggtacaaattcaatggcttgttctaaatcatctctacaccgtgccagaaattcctccttgcactaagtcctggtgggggagaggagaggctgcagctggggtgattttgagggggtgggagtatctattgctggcgcaggtttgtcggatggaaggcagggatccggcggggccgggaggacacaggagatttggaatgcaaggggctgtgaacaaccagggtgcgggtctcagaacgaaagtgcccggagtccagacctccagctgctcaatgaggaaaggaccggcgcccccaggtttgcctgcggccagggccaaggcgcactgaagccgcacctctcacctggaagcccaggaacccagggagaacagagctcctgcgtcctgacgccgcgcccgccttcgcgcccatgggaaaacgcgcattctttgggagcgcgcaaagcatccagagaccacatccgagccttcccgcaccctgctgccctggggagcccctgccccgtgcctaggtcgccctgcgcgagcccagcccagccctggactcatacaaaggctccagagcttgcgcccgtgcgaagccgccctgccggctttgggcatctccgaatccccacaaaagctatggctccattcccccacacacacaaactggggggtctcgggctggcttacgtgattttctctccagccgatgggcagcttcctctccatcctaccttcttttgccggctagcccctctcacctgacctgctgacccgcatccagggacattcctttcgcctcctttcacggaaaatctcgttgtttcgaatcaattctccttttggatttggacccattattcctattattactattattccccgttttcacgcatttgttgccccaccgaacacagcaactgggtgagaatcactgagccctcctcttggggaaaattcagaaaattgaccatttgaggagatgggggaacactactataactgaaatctataaaatgggggtaaggccataacgagccctattttttttattaggtacaaattattcatgacttttggtagcactcagttcctggattcagggccgaccaaggcgcggtgccgggagcagacatccgcagctgccgctccagggagtttcacatggagcaagggtgccatctagcggctgctctgcgaaaaggcgccgcagccaccggctccaccagttttctgggagagcagccgcagaggtggccagcaggagaaactttcataactagcagtaaaaggggagggatagggagtgggcatcggaatcaggaaacggttcatgaaattgtgtagataagctaaaaaatagaaaaaaaacacaacagaggggaggaaaaaaaagaagccctaagcttttttctttctacgtacacctcccacccctgcccctaatttctagcggagaccgcaaagcagtgcgccctttatggcctgtaaaaagggggaccgagcagttttcaaactccacgcgattgtttcaaattctgaggagaaacagttgggctttttgtcgggggagaggaggcctgagaggataggatgagactgtaaaagaatcaagaggctgcccgcgcccagacgtctggccccgccggacctgagtgtgtgtgtgtgtgtgtgtgtgtgtgtgtgtgtgtgtgtgtgtgtgcgcgcgcgcgcaggaggctcctcgtttccgacgcctgattctggagggggtgtgaagaacaaagacaagagccccagttgcaatttctgaagcatttgcgacaacaaagtgttctttcccggcttctctcttctccctctctgccccctgccaccccccgccccggaagcccggagccccgtgttctgtgcgggtgagggtgaaggctgccggagcggggcccacccattcccccgccaggccgggagccccggcccagct

SEQ ID NO: 16990 - RNA, 1752 nt, Homo sapiens
  source 1..1752: mol_type = other RNA
taggtagtttcatgttgttgggagaacttagcagaaatcggtaccttggtcattacaaagaagcacgttcaaaggaaaaaaaagacaattgcacaaggaggctttttacacggggaggggaggggcatggggggctcagccgggcctttgccgctcgccctcacagggcgagggagcctttgcttaaatccttttctttccccccggcccccaagagaagggaaggagatccacggtagctcacacacagaagctattacgagatactaccactagcggggactggcgcggcgggggacgctgcggtgggaggcccggctcctggccccgctagcggggccagagctctctcgggcaggggcgcgcggcggcggcgcggccgggacccgcggacgtgcgggcggccgcggccctggcagtcccagctgaagcctacttcttgtcgcccttctgcgcgtcgccctcgtccgccgcctctggggcccgctccagcttctgtttctccagctcctcctgctcgcatttgctgctggggaacttgtctttgttgttctcttttttccacttcatcctccggttctggaaccagattttgacctgtctctctgtcagtcccagggcgtgcgatacctcgattcgccgcttacgagtcagatagggattaaataggaactccttctccagctccagggtctggtagcggctgtaggtctgtcggcctcgcctgcgtccggcggctgcttgcgggcgcatccaggggaagagctgtgtgggcgacgggctctgctcggagccctcggcctcctcgcccaggccgctggcggcggcaagcttgcagtctgcgtactgcaccaggtctggatcctgcgcaccgaataggctctggcgttgcagcgggtcgtagccgtagaaattgccggggtccccgtggcacgccacggcgcacgggttctgctggtagggagccgtggacagcgacgacggcccgtggtagaactcctggatttgcgacgggtgctggaagctgccgccgctgctgggaccgtacaccacggtgggtcggccgcccaggtcctgggcgaagccgcagtcataataattggggcgcagggactccccggttttgtatttggagaacagtgagttgacgaaataagagctcattttattgaattttgaggcggcggcggcggcggaggctatagttgggggctgttggggagggggtggggagggggaaagggagggagagagagaaaaaaacgcggattcgccggctcctagtcaccctcgccaggaaaggagagggaaagagaggagggaaaaaaagaaaagaaagaaaaggcgaagaagatctcgaagccgacacactttttgtggtttccaggaatagaaaaggacagagaagcctccaaaagtctaagcttgcatggcagccgcggctcgctcgccctccccccaccccccaccccccaaacaaaaatataccaccacttaaagaggtcctcgctttacatttcgaagaagggatgccagttcataaacagttttcggtgatttacttccctgcaaatgagttgtttcatattttgcactgtcttttcatgatcatttgcatccattagagaccccgcatcctattggcttcttcgtactcctcccggacagaacgcagagcgagggtgagagcgagagagagcgagcgagagagagagctagagcgagagagcgccagggagtgaggagagagcg

SEQ ID NO: 16991 - RNA, 3666 nt, Homo sapiens
  source 1..3666: mol_type = other RNA
taggtagtttcatgttgttgggagaacttagcagaaatcggtaccttggtcattacaaagaagcacgttcaaaggaaaaaaaagacaattgcacaaggaggctttttacacggggaggggaggggcatggggggctcagccgggcctttgccgctcgccctcacagggcgagggagcctttgcttaaatccttttctttccccccggcccccaagagaagggaaggagatccacggtagctcacacacagaagctattacgagatactaccactagcggggactggcgcggcgggggacgctgcggtgggaggcccggctcctggccccgctagcggggccagagctctctcgggcaggggcgcgcggcggcggcgcggccgggacccgcggacgtgcgggcggccgcggccctggcagtcccagctgaagcctacttcttgtcgcccttctgcgcgtcgccctcgtccgccgcctctggggcccgctccagcttctgtttctccagctcctcctgctcgcatttgctgctggggaacttgtctttgttgttctcttttttccacttcatcctccggttctggaaccagattttgacctgtctctctgtcagtcccagggcgtgcgatacctcgattcgccgcttacgagtcagatagggattaaataggaactccttctccagctccagggtctggtagcggctgtaggtctgtcggcctcgcctgcgtccggcggcttgcgggcgcatccaggggaagagctgtgtgggcgacgggctctgctcggagccctcggcctcctcgcccaggccgctggcggcggcaagcttgcagtctgcgtactgcaccaggtctggatcctgcgcaccgaataggctctggcgttgcagcgggtcgtagccgtagaaattgccggggtccccgtggcacgccacggcgcacgggttctgctggtagggagccgtggacagcgacgacggcccgtggtagaactcctggatttgcgacgggtgctggaagctgccgccgctgctgggaccgtacaccacggtgggtcggccgcccaggtcctgggcgaagccgcagtcataataattggggcgcagggactccccggttttgtatttggagaacagtgagttgacgaaataagagctcattttattgaattttgaggcggcggcggcggcggaggctatagttgggggctgttggggagggggtggggagggggaaagggagggagagagagaaaaaaacgcggattcgccggctcctagtcaccctcgccaggaaaggagagggaaagagaggagggaaaaaaagaaaagaaagaaaaggcgaagaagatctcgaagccgacacactttttgtggtttccaggaatagaaaaggacagagaagcctccaaaagtctaagcttgcatggcagccgcggctcgctcgccctccccccaccccccaccccccaaacaaaaatataccaccacttaaagaggtcctcgctttacatttcgaagaagggatgccagttcataaacagttttcggtgatttacttccctgcaaatgagttgtttcatattttgcactgtcttttcatgatcatttgcatccattagagaccccgcatcctattggcttcttcgtactcctcccggacagaacgcagagcgagggtgagagcgagagagagcgagcgagagagagagcggcgaggtacaaattcaatggcttgttctaaatcatctctacaccgtgccagaaattcctccttgcactaagtcctggtgggggagaggagaggctgcagctggggtgattttgagggggtgggagtatctattgctggcgcaggtttgtcggatggaaggcagggatccggcggggccgggaggacacaggagatttggaatgcaaggggctgtgaacaaccagggtgcgggtctcagaacgaaagtgcccggagtccagacctccagctgctcaatgaggaaaggaccggcgcccccaggtttgcctgcggccagggccaaggcgcactgaagccgcacctctcacctggaagcccaggaacccagggagaacagagctcctgcgtcctgacgccgcgcccgccttcgcgcccatgggaaaacgcgcattctttgggagcgcgcaaagcatccagagaccacatccgagccttcccgcaccctgctgccctggggagcccctgccccgtgcctaggtcgccctgcgcgagcccagcccagccctggactcatacaaaggctccagagcttgcgcccgtgcgaagccgccctgccggctttgggcatctccgaatccccacaaaagctatggctccattcccccacacacacaaactggggggtctcgggctggcttacgtgattttctctccagccgatgggcagcttcctctccatcctaccttcttttgccggctagcccctctcacctgacctgctgacccgcatccagggacattcctttcgcctcctttcacggaaaatctcgttgtttcgaatcaattctccttttggatttggacccattattcctattattactattattccccgttttcacgcatttgttgccccaccgaacacagcaactgggtgagaatcactgagccctcctcttggggaaaattcagaaaattgaccatttgaggagatgggggaacactactataactgaaatctataaaatgggggtaaggccataacgagccctattttttttattaggtacaaattattcatgacttttggtagcactcagttcctggattcagggccgaccaaggcgcggtgccgggagcagacatccgcagctgccgctccagggagtttcacatggagcaagggtgccatctagcggctgctctgcgaaaaggcgccgcagccaccggctccaccagttttctgggagagcagccgcagaggtggccagcaggagaaactttcataactagcagtaaaaggggagggatagggagtgggcatcggaatcaggaaacggttcatgaaattgtgtagataagctaaaaaatagaaaaaaaacacaacagaggggaggaaaaaaaagaagccctaagcttttttctttctacgtacacctcccacccctgcccctaatttctagcggagaccgcaaagcagtgcgccctttatggcctgtaaaaagggggaccgagcagttttcaaactccacgcgattgtttcaaattctgaggagaaacagttgggctttttgtcgggggagaggaggcctgagaggataggatgagactgtaaaagaatcaagaggctgcccgcgcccagacgtctggccccgccggacctgagtgtgtgtgtgtgtgtgtgtgtgtgtgtgtgtgtgtgtgtgtgtgtgcgcgcgcgcgcaggaggctcctcgtttccgacgcctgattctggagggggtgtgaagaacaaagacaagagccccagttgcaatttctgaagcatttgcgacaacaaagtgttctttcccggcttctctcttctccctctctgccccctgccaccccccgccccggaagcccggagccccgtgttctgtgcgggtgagggtgaaggctgccggagcggggcccacccattcccccgccaggccgggagccccggcccagct

SEQ ID NO: 16992 - RNA, 9501 nt, Homo sapiens
  source 1..9501: mol_type = other RNA
taggtagtttcatgttgttgggaggtgttatctggctggagtgcctcttaattctttttaaggtaatttaattatttcttgccaattgttctttcttgaatgaatgattacatccttaacagaaaacctgggtgtataaataatacagctgaaagaaacagaagtgtacaccttccaacaacatacactcccaaccacttgtgttgtttttggcaacaaccaaaatgccattgcttgcacaaaaagtaaataaatgatcatatgatggcaacattcatcataagagagccagtaggcagtgactgtaagcatcacagccaccaattatgtcattttagaattgtgagcaaattcacaagaacacacagtgcaatttttagctgcatacatttcttctgagctccaactcagcaatatgcaatcttgacatcaaagcattagccaaatatttgaggaaattttcttactaaaataccaagtatctgataaatcaattttaccaaaatatataaacatatagaaggataagtgcatttagtagaaatacttacaataaaaaaatctcttaaaatctatgagccattcaatgtatacacaacgcaagaagtggcaataaggctatgattacagctccaggtcctgactgacctcgccaagttccatacacaatatattttttaatgccatgtgattgcagtgtgtgtgcgtgtgtaaggtgggagtgatattcacacatatgtagttctgaacatctacacaaacggcatgcacattgttgagaagttatctgttctcttattgcatacatcttactcactgttgaatccctagcagttttggggttgggttagggtcaagcataggaaatcatcatatttctttccttctccactcttgaggatctggaatcaggtcacagactgtgctgggtccacacgcttacatatgtgaaccttcaagtaactaccattccctcaataggcccacatagacaccacggacaagcaaataaggaccctctgtctaccataaatagaacttgatgctttcactttccaggagaagctgattctgtcggctttctctttgcccctccaacttcttagttgggcctattctatgctgctacttcaagttactcaaatgtgttttgtctggtgttatttttttctccagtgttttggaccaagactagatttcctgagactttaaatacgcaagacaaatgcaaacaaaatctgccaacatacccaggctgcttttcaggagtgaatcactgaagcgcatttggatttcctataacactactttcttttgggaatgtacagccctcccccagctccccatcccccatcataatgtaaaccattctaatagaaaatatggatgttttggctgggggtggtggcacatgcctgtagtcccagctacttgggaagctgaagcaggaggaccacttgagcccaggagtttgaggctgcagtaagacatgatggcaccactgcagtccagtctgggtgacagatgacagaaaaaaaaaaaaaaaaagaaaagaaaagaaaatatggacattttatttctggactttatccttaaatgcttagctttagaatagtgcacaggtacatccttaataaaaagtaaatttgaaaagacaggaaaggactgtgcttttctcttccattttaccttttcattctgagaccactaaggtctttgcattaagtaggtgacgtgaaccctagtgaccactgcccaccaaaatgcccctcatctccagctctgtcaggagtacctttagttactcaaatggaaatatctcagtgtaatgatggggctacaacatatccaaagtatagatggttctctcagggctgctggggcagcttcctttagaatcctctagaacactattgttaaacactggatctcctcttgaagtttagtctgcataacctttaacacttaaacatgaatcagagtatctatataaatgcaaattttcatttcccttttataaaatgcaattttcaagcacatgctaattctggtgcacaatgaacccagacaaatttgtcttcagcacaaactctaacggccgaggtgctagatcaaaccacctgtgaccatttttgtagcttgggactgggatattttaagatttcaggctagtgatgattacagggtcacagatagtggcaaaggtaaatctggttcctcattttccctcttgccactttgtttccaacaacaatggagcaaaaggtgacagtcccattttgtgccagttgaaagctgagtttggctttagtacctatcatactgcaatcatgaactgctgtgggttaaaaaaagcttgtgatgttgagggtgtgaaatcaattgtcaatcccagctaaaggatgatagccacagaacagctttattgtcatgaaactaaagggggacttcatcaggagtgttagaatggatgaaatgaggtttcttccctaacttaacattctgcagaaaattcctgattcaggtaaaaaaagaatgagattagtattacataaactgtgagttacttgaagggagatggtcttaaacaaagtaatctgttataaaactaacatcctttaatgggaaaccctgacccagatacagctcatacaatgctttctgtctgcagcttggcctcctcaccacacattccctcccaacaaagcataacctataccccaaaacacttttggctattgttagaatcatactgagctctcctttagggaatcagttcatagcaaccagatattccctttttgttcattttctgataataaaaactgcagtttttaaggttgatgaaataacaattctgtgttaaattgtaaggacactgaaaaccactagcattaaagtaggaattgtgcaagacattggagccttgattaggtatcatgcactacagtcaataaaagaaataataggaaaacaaaatgtgcacaagatctgaggtctttcactttgctttcatacccttaatcagtttacatcttatgctttgtggggcaatcaaaccaaatgacttttacaatttcatccgttttaagtggtaatgttaaaataactcacttcggcctaaaattactataatttaacttaaaaaatcaaaatacttataatactaaatgattttaggaataagaatttgatttataacattgtcagttggacatttatctaaacattcaatatacaaagttataaagaaaaatacttctaagatatttaagaaaatgcaatataatagatcataaattaggtgcaaaaacaagacacttacagacatttccagtatatacatccattttcaaatattaccaaagtgtaaacataacttaagataatcatccttctatttctactcttgaatacagtgaaacttccagtgtgatccaggtcacttttttcccaaagataagcaaaaatggcaaaaatttacaatagcaagcactaatattaccagatttttactaatttagtgttttagtatttgaaaagttttgccaaattgtatcactcattaatagtggcttcttatttctcatgatgtgaaaaaataacaaagcaccagacatctcaagacattaatagagtatccaatacggcagtttcattatcatacccctaatgaagacagacagaaaaacataatggtgactttgataactgtaaaacacaatgttacttcatgtcaacgtttctgaggattgaatgaagggtctgtacctaatgacaaaagagctgacgcataaccgacaatactctggcaatgaaaagaaaacaggccttgggggtaaaacagaattaaaaatgtccagtttagataatttctgaattcagattttcagataaaaaaaaatcacactgttattaaaatacaagatggggctacaagggagttcccttaatctgttacactcaaaagccttgccgaggctctaaatatggaatacttctagtggaagatacgagatgctgggaacagagcagagattcccataaagtaaaagaagtaaaatactgtccaagaattcatgtggcctcaagtcttattctgaaacttgtcctttggaaagtggataacctcatttttagagtcaacgcagcaaagagaaccagatacatgagcataaaaaacaaaaaaccctcatcacatgaaatttctcaaaacgagtttattttctccttcttctgccccagtctcctgcacttgacttagtttggtgaaacatggaaatccttaatgctggcttaaaattagtataagttcctccactactaaagtatacctatgcactgccttaaacaaactttttctgtaaaattgagaatctttgaagtatggaaaggaatggttcggaaaaaccattcaaaatctctctaaaatgttaactgacagtttcctctaactggtatttctatttttcttaaaagtacatttgttaaaatactaactgagcccacctgggaaatcttgagtagaaaatatgtgatgagttcctgattgtgacataggcaggctgaagaccagccagaatgttccccaggagaggaaacctgaaaatggtggtttccttaaaaatcaatttcctgttcaatttcttgggttaggtagggggaagaggaactgtgttgtgtttgccagtgttgctgaaatgctgaacacacagcagtagcaaggtcaacagatcccaatatcccatggctgcattaatgtctgatttttttctttcttgttcagccgtatctagaggataaatattaccctcagaaccccaaggtaatacccacatccacattcttaaggcttttgcttttttcagtggttaacaaatagctataatttattttctttctttttgatgcctagcaagcagaatgacttgcttgccttttcccttagtaggtaactacagagcagagcacccatgtttccacagcggggtggtctcactgtccagactgagaattaagagcaaatctttcccacacattggagtaggtgttgcagtcctagaagttaagtactggtctcagatctcatggcagggtgctctctgccatgcagacatgtgcaattgccatttcaggatcccacactgaaaattcacggcgctccattaacaacaccagggtgtgtcatgctcttgggtggggtcacactagttctccaagtgacaaaacacacccaacacaacacaagatgttggtaagttagagaagagcaaaacacagctacttaaatgaaatctctggtttgttaatgaaccaaaggtggcttgggattattttagtagttaaaattaagagtgcattctattgcagaaaatgcagttattcaacacacagttcctcagccggcctagagccgcattacccttatcatttagtttctttttcatcctctggaggagagcagggcaggaagaggtggggacttctcttggagcatctccatcatctgtaagagggtatgtgttactgctcaccagcaccctcggctgtagttgacgtcatcttttctgtctttttggacttcctctgcatttgctcttgctcctttctccttagcttttctctttgtttttccattttctcttgggccttccgagccttctctagagacatcttcatttccttgagtttctttttgaccactgctcggtcctgggatgctgtcattccaagagcctcatctgatgacagtgctaaggactgagagagccctggtgttttaggttctgctcctaagccgctgaggtctgctgaactggtactgctgggactgaagtcatcattgaaggtaaaattcttggacccctttttatctgaaattagagtctcaggagaaggctgaagggaacttgtaggcgcaggcaggttcctgaaggaataggatcctttccggctgtcattaaaccatgagaaaggcatgcaaggggaacgagtggaggtctgagctgttgaacatggcttgggtgtccagttttccagtctgcctctgaagatcctgctacctgcagaaaacctactggcttctttttctttttctttccacttctttcccttgctggaattccttcgcaaaggcgcccccagatccacaaacttccgcttaatttttcctccttgcaccgccaatgaactggatgcccttagtgatttgggatctttggcatcatctttttctcgtaatattttcttgttggtggtttggtgatggcaaggagattcttccacatcatgatcagactttgaagtagaaaacagtgaagtgtctccccacatagaggagagaggccccatttctgggtccagtggttcttcttgaaattcagctatgtggtcagacgagaagggcacattgctatccaccggggtgaggggtggaacaccagaatctgattctggagaagacgttctcaaacccttaggtggaagtaatttggtaatatgcatgtggttatagaaactgtttgatggctttctctctagactgtcctccccatctgtggaactaacactatcatacagtcttgtcctagagggtctctggcgtctgttcttcacagagagctgggctcgagttttcagtgcttttgaatccaggcgctctgtctctgggactgcttcattcaagtcttgacttaggccatcttggcaagatgtctgcttgccatccaagttctccatggtatcccctttagagacttcaccaagagatgttcttctctcaaagatgttgttattattgttaacttgagtcccattttgcttcagtagcctgaatacctcagcttccaaatctctaatccgcacttggaggccttgcacttccacaagatgagctttttccaaatcttctattttctttctttctgcttcctgtcttttgatgaaatcaagctctttttgttgaaaatccttgatcaacttctttgccttgttgtatttcttttccaaggcctgatactggctttgagtctctttgagatgctcattcactgtgtggcataatgtttgggcctcaatccagtagctttccaacttcaacattctttccttattctcttctatgttttgttggagttgggttttttctagttcccacctcactttctcattttctgctgcctgcagcttggtcttcaatttttgaatctctgcttctgtaactgcatgtttgatttgcaactctttgaacttgtgactgagcttgcttgtgtccagttctgatggggaaaacatgtcctcattctcaggcagctcaaagacttcaatggccatgtcgctgccaggaaggacaggtcctacctcatcttcttcttcatctgtggcatattctcctgtctcgtcatcgtcggcatcatactgggcatagtgctgttccagcagctctctctggcgcctctcctgttccagtgtctggcttatcaactgggcaacctcgctcacttgtcctggtttttcccgcccaataacaaatctgacgttgcccttggtgtttctgagaactgttgctgcaaaattctgtgtcacacccaccaagctgattccatccacttccacaatctggtcattgacttgtattctgccatcccgttgagcagcaccaccttctgttactgtcttgacgaatattcccagcttttcaagtccagcatctgctccaacacccattccaataatacttataccaagaccatcctcatctttctctagctccactgggaaaagttccagcttttctacacgtttttcaagttcatactcagctgaagcagccacagggtcaacttcgtcatttctcctgtcatagtcttcattggagtatgtgttgaaaaccttaataggagcactactaaacttaattttcctatttgctgggatttcttcttcttctggcaatccaacaatttccgagtactccatatcaggctgatagtaactgttctcatcactatcttcctcctcatcctgctcagtgcctgtctctccccagtctgaattatacctggatctcaccctatacacattatagtcactgtgcatgtacacatgggaaccatcaaaattatttgaatcttcaggtacttcttttccacaactggatgcagaagcatcaggagaggtgaaatcaccacctgcaagttctttcctctgttgctttgctgcctcccttccaaccaaattagcttcagcatcttctaacagttggctttgtggtgaagggatttcggactttggcattgccttactttcagcacaaggttcttcaggaccatctttgtcaatgctgtcgggagtctgttgattagatgtggagtcctcgggttccttgctctgctggatctcttcaccaggtatcgaagctagagaggtacttttagaagccacttctggtactggagttgcattactcttgtgagcatcctctgtatcaacacctcgcttgtttgaaggaggccaggaattagaatccttcaggtgaccaaatgtgtcaagatttgtaacagtaacagatggtaaattcaagggataatgcccagtcactgagtattcattgttttcagccttctcagaaatgatggcactgggagaatcagtgttctcaaatactgcactcagttgactcacagttggggagacagcctcagttcgggagctaaggctgtccaaggaatcagtactgcctctgttggacttggaacctccccattcatcctgaggttcactccctccagctttctctttctttggggaatagcggttgttctgtcctgattcatgcacacttctctcaaacatctttcgagtctcagtgaacttggaatatgaagggccatcgtacatagtgtcaaatctactaattcgttcagaaacagaagactccaacttaacaactgagccatctgttttttccagaaattctttgggcttcattcttctctgaggagatgaatgtccacctttcccccttgttttggcaatgactgcagcattctcgttgggttccatacccatctgcataaataggtttttaattctgttgacattggagccatatttcctccccctgctctgctgggagccctcaccttcttttgttttttgttccccatctgacttgggtttgtcaaaggtacttttcagtgcctgaaactcagttcgatatgcattcctgtgaggagaggcacttctgagagtggttcgttcacctgaagactcagttttcaacattttcacttcaggggtgaaaagccaatgttcataatgatcaaagaaaaaaaccaaaaaccaagatacctctcttctctaatcaccagtattgggtcaagaaaagtacctctcaaatggtatacggtgtcagtgatcgtcccaacaggtgtattaggaacttagtcacagtcaagagttacacagaatgattttttcaaagcaagactagaggttcat

SEQ ID NO: 16993 - RNA, 9876 nt, Homo sapiens
  source 1..9876: mol_type = other RNA
taggtagtttcatgttgttgggaggtgttatctggctggagtgcctcttaattctttttaaggtaatttaattatttcttgccaattgttctttcttgaatgaatgattacatccttaacagaaaacctgggtgtataaataatacagctgaaagaaacagaagtgtacaccttccaacaacatacactcccaaccacttgtgttgtttttggcaacaaccaaaatgccattgcttgcacaaaaagtaaataaatgatcatatgatggcaacattcatcataagagagccagtaggcagtgactgtaagcatcacagccaccaattatgtcattttagaattgtgagcaaattcacaagaacacacagtgcaatttttagctgcatacatttcttctgagctccaactcagcaatatgcaatcttgacatcaaagcattagccaaatatttgaggaaattttcttactaaaataccaagtatctgataaatcaattttaccaaaatatataaacatatagaaggataagtgcatttagtagaaatacttacaataaaaaaatctcttaaaatctatgagccattcaatgtatacacaacgcaagaagtggcaataaggctatgattacagctccaggtcctgactgacctcgccaagttccatacacaatatattttttaatgccatgtgattgcagtgtgtgtgcgtgtgtaaggtgggagtgatattcacacatatgtagttctgaacatctacacaaacggcatgcacattgttgagaagttatctgttctcttattgcatacatcttactcactgttgaatccctagcagttttggggttgggttagggtcaagcataggaaatcatcatatttctttccttctccactcttgaggatctggaatcaggtcacagactgtgctgggtccacacgcttacatatgtgaaccttcaagtaactaccattccctcaataggcccacatagacaccacggacaagcaaataaggaccctctgtctaccataaatagaacttgatgctttcactttccaggagaagctgattctgtcggctttctctttgcccctccaacttcttagttgggcctattctatgctgctacttcaagttactcaaatgtgttttgtctggtgttatttttttctccagtgttttggaccaagactagatttcctgagactttaaatacgcaagacaaatgcaaacaaaatctgccaacatacccaggctgcttttcaggagtgaatcactgaagcgcatttggatttcctataacactactttcttttgggaatgtacagccctcccccagctccccatcccccatcataatgtaaaccattctaatagaaaatatggatgttttggctgggggtggtggcacatgcctgtagtcccagctacttgggaagctgaagcaggaggaccacttgagcccaggagtttgaggctgcagtaagacatgatggcaccactgcagtccagtctgggtgacagatgacagaaaaaaaaaaaaaaaaagaaaagaaaagaaaatatggacattttatttctggactttatccttaaatgcttagctttagaatagtgcacaggtacatccttaataaaaagtaaatttgaaaagacaggaaaggactgtgcttttctcttccattttaccttttcattctgagaccactaaggtctttgcattaagtaggtgacgtgaaccctagtgaccactgcccaccaaaatgcccctcatctccagctctgtcaggagtacctttagttactcaaatggaaatatctcagtgtaatgatggggctacaacatatccaaagtatagatggttctctcagggctgctggggcagcttcctttagaatcctctagaacactattgttaaacactggatctcctcttgaagtttagtctgcataacctttaacacttaaacatgaatcagagtatctatataaatgcaaattttcatttcccttttataaaatgcaattttcaagcacatgctaattctggtgcacaatgaacccagacaaatttgtcttcagcacaaactctaacggccgaggtgctagatcaaaccacctgtgaccatttttgtagcttgggactgggatattttaagatttcaggctagtgatgattacagggtcacagatagtggcaaaggtaaatctggttcctcattttccctcttgccactttgtttccaacaacaatggagcaaaaggtgacagtcccattttgtgccagttgaaagctgagtttggctttagtacctatcatactgcaatcatgaactgctgtgggttaaaaaaagcttgtgatgttgagggtgtgaaatcaattgtcaatcccagctaaaggatgatagccacagaacagctttattgtcatgaaactaaagggggacttcatcaggagtgttagaatggatgaaatgaggtttcttccctaacttaacattctgcagaaaattcctgattcaggtaaaaaaagaatgagattagtattacataaactgtgagttacttgaagggagatggtcttaaacaaagtaatctgttataaaactaacatcctttaatgggaaaccctgacccagatacagctcatacaatgctttctgtctgcagcttggcctcctcaccacacattccctcccaacaaagcataacctataccccaaaacacttttggctattgttagaatcatactgagctctcctttagggaatcagttcatagcaaccagatattccctttttgttcattttctgataataaaaactgcagtttttaaggttgatgaaataacaattctgtgttaaattgtaaggacactgaaaaccactagcattaaagtaggaattgtgcaagacattggagccttgattaggtatcatgcactacagtcaataaaagaaataataggaaaacaaaatgtgcacaagatctgaggtctttcactttgctttcatacccttaatcagtttacatcttatgctttgtggggcaatcaaaccaaatgacttttacaatttcatccgttttaagtggtaatgttaaaataactcacttcggcctaaaattactataatttaacttaaaaaatcaaaatacttataatactaaatgattttaggaataagaatttgatttataacattgtcagttggacatttatctaaacattcaatatacaaagttataaagaaaaatacttctaagatatttaagaaaatgcaatataatagatcataaattaggtgcaaaaacaagacacttacagacatttccagtatatacatccattttcaaatattaccaaagtgtaaacataacttaagataatcatccttctatttctactcttgaatacagtgaaacttccagtgtgatccaggtcacttttttcccaaagataagcaaaaatggcaaaaatttacaatagcaagcactaatattaccagatttttactaatttagtgttttagtatttgaaaagttttgccaaattgtatcactcattaatagtggcttcttatttctcatgatgtgaaaaaataacaaagcaccagacatctcaagacattaatagagtatccaatacggcagtttcattatcatacccctaatgaagacagacagaaaaacataatggtgactttgataactgtaaaacacaatgttacttcatgtcaacgtttctgaggattgaatgaagggtctgtacctaatgacaaaagagctgacgcataaccgacaatactctggcaatgaaaagaaaacaggccttgggggtaaaacagaattaaaaatgtccagtttagataatttctgaattcagattttcagataaaaaaaaatcacactgttattaaaatacaagatggggctacaagggagttcccttaatctgttacactcaaaagccttgccgaggctctaaatatggaatacttctagtggaagatacgagatgctgggaacagagcagagattcccataaagtaaaagaagtaaaatactgtccaagaattcatgtggcctcaagtcttattctgaaacttgtcctttggaaagtggataacctcatttttagagtcaacgcagcaaagagaaccagatacatgagcataaaaaacaaaaaaccctcatcacatgaaatttctcaaaacgagtttattttctccttcttctgccccagtctcctgcacttgacttagtttggtgaaacatggaaatccttaatgctggcttaaaattagtataagttcctccactactaaagtatacctatgcactgccttaaacaaactttttctgtaaaattgagaatctttgaagtatggaaaggaatggttcggaaaaaccattcaaaatctctctaaaatgttaactgacagtttcctctaactggtatttctatttttcttaaaagtacatttgttaaaatactaactgagcccacctgggaaatcttgagtagaaaatatgtgatgagttcctgattgtgacataggcaggctgaagaccagccagaatgttccccaggagaggaaacctgaaaatggtggtttccttaaaaatcaatttcctgttcaatttcttgggttaggtagggggaagaggaactgtgttgtgtttgccagtgttgctgaaatgctgaacacacagcagtagcaaggtcaacagatcccaatatcccatggctgcattaatgtctgatttttttctttcttgttcagccgtatctagaggataaatattaccctcagaaccccaaggtaatacccacatccacattcttaaggcttttgcttttttcagtggttaacaaatagctataatttattttctttctttttgatgcctagcaagcagaatgacttgcttgccttttcccttagtaggtaactacagagcagagcacccatgtttccacagcggggtggtctcactgtccagactgagaattaagagcaaatctttcccacacattggagtaggtgttgcagtcctagaagttaagtactggtctcagatctcatggcagggtgctctctgccatgcagacatgtgcaattgccatttcaggatcccacactgaaaattcacggcgctccattaacaacaccagggtgtgtcatgctcttgggtggggtcacactagttctccaagtgacaaaacacacccaacacaacacaagatgttggtaagttagagaagagcaaaacacagctacttaaatgaaatctctggtttgttaatgaaccaaaggtggcttgggattattttagtagttaaaattaagagtgcattctattgcagaaaatgcagttattcaacacacagttcctcagccggcctagagccgcattacccttatcatttagtttctttttcatcctctggaggagagcagggcaggaagaggtggggacttctcttggagcatctccatcatctgtaagagggtatgtgttactgctcaccagcaccctcggctgtagttgacgtcatcttttctgtctttttggacttcctctgcatttgctcttgctcctttctccttagcttttctctttgtttttccattttctcttgggccttccgagccttctctagagacatcttcatttccttgagtttctttttgaccactgctcggtcctgggatgctgtcattccaagagccttaagtttatttccatccaactgcaggagctgttctccagtgatgttttgggcactgaattcagatacatactgctccagatttaggctcattaaccagtgagaaacctgctgcacactccattcctgaacggcccgattctgacactgactgtgtttgggagactgtccatcatcaaggatctcatctgatgacagtgctaaggactgagagagccctggtgttttaggttctgctcctaagccgctgaggtctgctgaactggtactgctgggactgaagtcatcattgaaggtaaaattattggtttcttggatccagactacagacataagttgagaatgccttccaaagattgaagaagaggagggatttgggtttctcttgtttgcttttgtaatccatgtgttttctaccttggacccctttttatctgaaattagagtctcaggagaaggctgaagggaacttgtaggcgcaggcaggttcctgaaggaataggatcctttccggctgtcattaaaccatgagaaaggcatgcaaggggaacgagtggaggtctgagctgttgaacatggcttgggtgtccagttttccagtctgcctctgaagatcctgctacctgcagaaaacctactggcttctttttctttttctttccacttctttcccttgctggaattccttcgcaaaggcgcccccagatccacaaacttccgcttaatttttcctccttgcaccgccaatgaactggatgcccttagtgatttgggatctttggcatcatctttttctcgtaatattttcttgttggtggtttggtgatggcaaggagattcttccacatcatgatcagactttgaagtagaaaacagtgaagtgtctccccacatagaggagagaggccccatttctgggtccagtggttcttcttgaaattcagctatgtggtcagacgagaagggcacattgctatccaccggggtgaggggtggaacaccagaatctgattctggagaagacgttctcaaacccttaggtggaagtaatttggtaatatgcatgtggttatagaaactgtttgatggctttctctctagactgtcctccccatctgtggaactaacactatcatacagtcttgtcctagagggtctctggcgtctgttcttcacagagagctgggctcgagttttcagtgcttttgaatccaggcgctctgtctctgggactgcttcattcaagtcttgacttaggccatcttggcaagatgtctgcttgccatccaagttctccatggtatcccctttagagacttcaccaagagatgttcttctctcaaagatgttgttattattgttaacttgagtcccattttgcttcagtagcctgaatacctcagcttccaaatctctaatccgcacttggaggccttgcacttccacaagatgagctttttccaaatcttctattttctttctttctgcttcctgtcttttgatgaaatcaagctctttttgttgaaaatccttgatcaacttctttgccttgttgtatttcttttccaaggcctgatactggctttgagtctctttgagatgctcattcactgtgtggcataatgtttgggcctcaatccagtagctttccaacttcaacattctttccttattctcttctatgttttgttggagttgggttttttctagttcccacctcactttctcattttctgctgcctgcagcttggtcttcaatttttgaatctctgcttctgtaactgcatgtttgatttgcaactctttgaacttgtgactgagcttgcttgtgtccagttctgatggggaaaacatgtcctcattctcaggcagctcaaagacttcaatggccatgtcgctgccaggaaggacaggtcctacctcatcttcttcttcatctgtggcatattctcctgtctcgtcatcgtcggcatcatactgggcatagtgctgttccagcagctctctctggcgcctctcctgttccagtgtctggcttatcaactgggcaacctcgctcacttgtcctggtttttcccgcccaataacaaatctgacgttgcccttggtgtttctgagaactgttgctgcaaaattctgtgtcacacccaccaagctgattccatccacttccacaatctggtcattgacttgtattctgccatcccgttgagcagcaccaccttctgttactgtcttgacgaatattcccagcttttcaagtccagcatctgctccaacacccattccaataatacttataccaagaccatcctcatctttctctagctccactgggaaaagttccagcttttctacacgtttttcaagttcatactcagctgaagcagccacagggtcaacttcgtcatttctcctgtcatagtcttcattggagtatgtgttgaaaaccttaataggagcactactaaacttaattttcctatttgctgggatttcttcttcttctggcaatccaacaatttccgagtactccatatcaggctgatagtaactgttctcatcactatcttcctcctcatcctgctcagtgcctgtctctccccagtctgaattatacctggatctcaccctatacacattatagtcactgtgcatgtacacatgggaaccatcaaaattatttgaatcttcaggtacttcttttccacaactggatgcagaagcatcaggagaggtgaaatcaccacctgcaagttctttcctctgttgctttgctgcctcccttccaaccaaattagcttcagcatcttctaacagttggctttgtggtgaagggatttcggactttggcattgccttactttcagcacaaggttcttcaggaccatctttgtcaatgctgtcgggagtctgttgattagatgtggagtcctcgggttccttgctctgctggatctcttcaccaggtatcgaagctagagaggtacttttagaagccacttctggtactggagttgcattactcttgtgagcatcctctgtatcaacacctcgcttgtttgaaggaggccaggaattagaatccttcaggtgaccaaatgtgtcaagatttgtaacagtaacagatggtaaattcaagggataatgcccagtcactgagtattcattgttttcagccttctcagaaatgatggcactgggagaatcagtgttctcaaatactgcactcagttgactcacagttggggagacagcctcagttcgggagctaaggctgtccaaggaatcagtactgcctctgttggacttggaacctccccattcatcctgaggttcactccctccagctttctctttctttggggaatagcggttgttctgtcctgattcatgcacacttctctcaaacatctttcgagtctcagtgaacttggaatatgaagggccatcgtacatagtgtcaaatctactaattcgttcagaaacagaagactccaacttaacaactgagccatctgttttttccagaaattctttgggcttcattcttctctgaggagatgaatgtccacctttcccccttgttttggcaatgactgcagcattctcgttgggttccatacccatctgcataaataggtttttaattctgttgacattggagccatatttcctccccctgctctgctgggagccctcaccttcttttgttttttgttccccatctgacttgggtttgtcaaaggtacttttcagtgcctgaaactcagttcgatatgcattcctgtgaggagaggcacttctgagagtggttcgttcacctgaagactcagttttcaacattttcacttcaggggtgaaaagccaatgttcataatgatcaaagaaaaaaaccaaaaaccaagatacctctcttctctaatcaccagtattgggtcaagaaaagtacctctcaaatggtatacggtgtcagtgatcgtcccaacaggtgtattaggaacttagtcacagtcaagagttacacagaatgattttttcaaagcaagactagaggttcatccgagcgggagcgccgcgggcggggagggtcgggccgccgcggctcccaccccctcctcgcaggcgccccccgcccca

SEQ ID NO: 16994 - RNA, 9864 nt, Homo sapiens
  source 1..9864: mol_type = other RNA
taggtagtttcatgttgttgggaggtgttatctggctggagtgcctcttaattctttttaaggtaatttaattatttcttgccaattgttctttcttgaatgaatgattacatccttaacagaaaacctgggtgtataaataatacagctgaaagaaacagaagtgtacaccttccaacaacatacactcccaaccacttgtgttgtttttggcaacaaccaaaatgccattgcttgcacaaaaagtaaataaatgatcatatgatggcaacattcatcataagagagccagtaggcagtgactgtaagcatcacagccaccaattatgtcattttagaattgtgagcaaattcacaagaacacacagtgcaatttttagctgcatacatttcttctgagctccaactcagcaatatgcaatcttgacatcaaagcattagccaaatatttgaggaaattttcttactaaaataccaagtatctgataaatcaattttaccaaaatatataaacatatagaaggataagtgcatttagtagaaatacttacaataaaaaaatctcttaaaatctatgagccattcaatgtatacacaacgcaagaagtggcaataaggctatgattacagctccaggtcctgactgacctcgccaagttccatacacaatatattttttaatgccatgtgattgcagtgtgtgtgcgtgtgtaaggtgggagtgatattcacacatatgtagttctgaacatctacacaaacggcatgcacattgttgagaagttatctgttctcttattgcatacatcttactcactgttgaatccctagcagttttggggttgggttagggtcaagcataggaaatcatcatatttctttccttctccactcttgaggatctggaatcaggtcacagactgtgctgggtccacacgcttacatatgtgaaccttcaagtaactaccattccctcaataggcccacatagacaccacggacaagcaaataaggaccctctgtctaccataaatagaacttgatgctttcactttccaggagaagctgattctgtcggctttctctttgcccctccaacttcttagttgggcctattctatgctgctacttcaagttactcaaatgtgttttgtctggtgttatttttttctccagtgttttggaccaagactagatttcctgagactttaaatacgcaagacaaatgcaaacaaaatctgccaacatacccaggctgcttttcaggagtgaatcactgaagcgcatttggatttcctataacactactttcttttgggaatgtacagccctcccccagctccccatcccccatcataatgtaaaccattctaatagaaaatatggatgttttggctgggggtggtggcacatgcctgtagtcccagctacttgggaagctgaagcaggaggaccacttgagcccaggagtttgaggctgcagtaagacatgatggcaccactgcagtccagtctgggtgacagatgacagaaaaaaaaaaaaaaaaagaaaagaaaagaaaatatggacattttatttctggactttatccttaaatgcttagctttagaatagtgcacaggtacatccttaataaaaagtaaatttgaaaagacaggaaaggactgtgcttttctcttccattttaccttttcattctgagaccactaaggtctttgcattaagtaggtgacgtgaaccctagtgaccactgcccaccaaaatgcccctcatctccagctctgtcaggagtacctttagttactcaaatggaaatatctcagtgtaatgatggggctacaacatatccaaagtatagatggttctctcagggctgctggggcagcttcctttagaatcctctagaacactattgttaaacactggatctcctcttgaagtttagtctgcataacctttaacacttaaacatgaatcagagtatctatataaatgcaaattttcatttcccttttataaaatgcaattttcaagcacatgctaattctggtgcacaatgaacccagacaaatttgtcttcagcacaaactctaacggccgaggtgctagatcaaaccacctgtgaccatttttgtagcttgggactgggatattttaagatttcaggctagtgatgattacagggtcacagatagtggcaaaggtaaatctggttcctcattttccctcttgccactttgtttccaacaacaatggagcaaaaggtgacagtcccattttgtgccagttgaaagctgagtttggctttagtacctatcatactgcaatcatgaactgctgtgggttaaaaaaagcttgtgatgttgagggtgtgaaatcaattgtcaatcccagctaaaggatgatagccacagaacagctttattgtcatgaaactaaagggggacttcatcaggagtgttagaatggatgaaatgaggtttcttccctaacttaacattctgcagaaaattcctgattcaggtaaaaaaagaatgagattagtattacataaactgtgagttacttgaagggagatggtcttaaacaaagtaatctgttataaaactaacatcctttaatgggaaaccctgacccagatacagctcatacaatgctttctgtctgcagcttggcctcctcaccacacattccctcccaacaaagcataacctataccccaaaacacttttggctattgttagaatcatactgagctctcctttagggaatcagttcatagcaaccagatattccctttttgttcattttctgataataaaaactgcagtttttaaggttgatgaaataacaattctgtgttaaattgtaaggacactgaaaaccactagcattaaagtaggaattgtgcaagacattggagccttgattaggtatcatgcactacagtcaataaaagaaataataggaaaacaaaatgtgcacaagatctgaggtctttcactttgctttcatacccttaatcagtttacatcttatgctttgtggggcaatcaaaccaaatgacttttacaatttcatccgttttaagtggtaatgttaaaataactcacttcggcctaaaattactataatttaacttaaaaaatcaaaatacttataatactaaatgattttaggaataagaatttgatttataacattgtcagttggacatttatctaaacattcaatatacaaagttataaagaaaaatacttctaagatatttaagaaaatgcaatataatagatcataaattaggtgcaaaaacaagacacttacagacatttccagtatatacatccattttcaaatattaccaaagtgtaaacataacttaagataatcatccttctatttctactcttgaatacagtgaaacttccagtgtgatccaggtcacttttttcccaaagataagcaaaaatggcaaaaatttacaatagcaagcactaatattaccagatttttactaatttagtgttttagtatttgaaaagttttgccaaattgtatcactcattaatagtggcttcttatttctcatgatgtgaaaaaataacaaagcaccagacatctcaagacattaatagagtatccaatacggcagtttcattatcatacccctaatgaagacagacagaaaaacataatggtgactttgataactgtaaaacacaatgttacttcatgtcaacgtttctgaggattgaatgaagggtctgtacctaatgacaaaagagctgacgcataaccgacaatactctggcaatgaaaagaaaacaggccttgggggtaaaacagaattaaaaatgtccagtttagataatttctgaattcagattttcagataaaaaaaaatcacactgttattaaaatacaagatggggctacaagggagttcccttaatctgttacactcaaaagccttgccgaggctctaaatatggaatacttctagtggaagatacgagatgctgggaacagagcagagattcccataaagtaaaagaagtaaaatactgtccaagaattcatgtggcctcaagtcttattctgaaacttgtcctttggaaagtggataacctcatttttagagtcaacgcagcaaagagaaccagatacatgagcataaaaaacaaaaaaccctcatcacatgaaatttctcaaaacgagtttattttctccttcttctgccccagtctcctgcacttgacttagtttggtgaaacatggaaatccttaatgctggcttaaaattagtataagttcctccactactaaagtatacctatgcactgccttaaacaaactttttctgtaaaattgagaatctttgaagtatggaaaggaatggttcggaaaaaccattcaaaatctctctaaaatgttaactgacagtttcctctaactggtatttctatttttcttaaaagtacatttgttaaaatactaactgagcccacctgggaaatcttgagtagaaaatatgtgatgagttcctgattgtgacataggcaggctgaagaccagccagaatgttccccaggagaggaaacctgaaaatggtggtttccttaaaaatcaatttcctgttcaatttcttgggttaggtagggggaagaggaactgtgttgtgtttgccagtgttgctgaaatgctgaacacacagcagtagcaaggtcaacagatcccaatatcccatggctgcattaatgtctgatttttttctttcttgttcagccgtatctagaggataaatattaccctcagaaccccaaggtaatacccacatccacattcttaaggcttttgcttttttcagtggttaacaaatagctataatttattttctttctttttgatgcctagcaagcagaatgacttgcttgccttttcccttagtaggtaactacagagcagagcacccatgtttccacagcggggtggtctcactgtccagactgagaattaagagcaaatctttcccacacattggagtaggtgttgcagtcctagaagttaagtactggtctcagatctcatggcagggtgctctctgccatgcagacatgtgcaattgccatttcaggatcccacactgaaaattcacggcgctccattaacaacaccagggtgtgtcatgctcttgggtggggtcacactagttctccaagtgacaaaacacacccaacacaacacaagatgttggtaagttagagaagagcaaaacacagctacttaaatgaaatctctggtttgttaatgaaccaaaggtggcttgggattattttagtagttaaaattaagagtgcattctattgcagaaaatgcagttattcaacacacagttcctcagccggcctagagccgcattacccttatcatttagtttctttttcatcctctggaggagagcagggcaggaagaggtggggacttctcttggagcatctccatcatctgtaagagggtatgtgttactgctcaccagcaccctcggctgtagttgacgtcatcttttctgtctttttggacttcctctgcatttgctcttgctcctttctccttagcttttctctttgtttttccattttctcttgggccttccgagccttctctagagacatcttcatttccttgagtttctttttgaccactgctcggtcctgggatgctgtcattccaagagccttaagtttatttccatccaactgcaggagctgttctccagtgatgttttgggcactgaattcagatacatactgctccagatttaggctcattaaccagtgagaaacctgctgcacactccattcctgaacggcccgattctgacactgactgtgtttgggagactgtccatcatcaaggatctcatctgatgacagtgctaaggactgagagagccctggtgttttaggttctgctcctaagccgctgaggtctgctgaactggtactgctgggactgaagtcatcattgaaggtaaaattattggtttcttggatccagactacagacataagttgagaatgccttccaaagattgaagaagaggagggatttgggtttctcttgtttgcttttgtaatccatgtgttttctaccttggacccctttttatctgaaattagagtctcaggagaaggctgaagggaacttgtaggcgcaggcaggttcctgaaggaataggatcctttccggctgtcattaaaccatgagaaaggcatgcaaggggaacgagtggaggtctgagctgttgaacatggcttgggtgtccagttttccagtctgcctctgaagatcctgctacctgcagaaaacctactggcttctttttctttttctttccacttctttcccttgctggaattccttcgcaaaggcgcccccagatccacaaacttccgcttaatttttcctccttgcaccgccaatgaactggatgcccttagtgatttgggatctttggcatcatctttttctcgtaatattttcttgttggtggtttggtgatggcaaggagattcttccacatcatgatcagactttgaagtagaaaacagtgaagtgtctccccacatagaggagagaggccccatttctgggtccagtggttcttcttgaaattcagctatgtggtcagacgagaagggcacattgctatccaccggggtgaggggtggaacaccagaatctgattctggagaagacgttctcaaacccttaggtggaagtaatttggtaatatgcatgtggttatagaaactgtttgatggctttctctctagactgtcctccccatctgtggaactaacactatcatacagtcttgtcctagagggtctctggcgtctgttcttcacagagagctgggctcgagttttcagtgcttttgaatccaggcgctctgtctctgggactgcttcattcaagtcttgacttaggccatcttggcaagatgtctgcttgccatccaagttctccatggtatcccctttagagacttcaccaagagatgttcttctctcaaagatgttgttattattgttaacttgagtcccattttgcttcagtagcctgaatacctcagcttccaaatctctaatccgcacttggaggccttgcacttccacaagatgagctttttccaaatcttctattttctttctttctgcttcctgtcttttgatgaaatcaagctctttttgttgaaaatccttgatcaacttctttgccttgttgtatttcttttccaaggcctgatactggctttgagtctctttgagatgctcattcactgtgtggcataatgtttgggcctcaatccagtagctttccaacttcaacattctttccttattctcttctatgttttgttggagttgggttttttctagttcccacctcactttctcattttctgctgcctgcagcttggtcttcaatttttgaatctctgcttctgtaactgcatgtttgatttgcaactctttgaacttgtgactgagcttgcttgtgtccagttctgatggggaaaacatgtcctcattctcaggcagctcaaagacttcaatggccatgtcgctgccaggaaggacaggtcctacctcatcttcttcttcatctgtggcatattctcctgtctcgtcatcgtcggcatcatactgggcatagtgctgttccagcagctctctctggcgcctctcctgttccagtgtctggcttatcaactgggcaacctcgctcacttgtcctggtttttcccgcccaataacaaatctgacgttgcccttggtgtttctgagaactgttgctgcaaaattctgtgtcacacccaccaagctgattccatccacttccacaatctggtcattgacttgtattctgccatcccgttgagcagcaccaccttctgttactgtcttgacgaatattcccagcttttcaagtccagcatctgctccaacacccattccaataatacttataccaagaccatcctcatctttctctagctccactgggaaaagttccagcttttctacacgtttttcaagttcatactcagctgaagcagccacagggtcaacttcgtcatttctcctgtcatagtcttcattggagtatgtgttgaaaaccttaataggagcactactaaacttaattttcctatttgctgggatttcttcttcttctggcaatccaacaatttccgagtactccatatcaggctgatagtaactgttctcatcactatcttcctcctcatcctgctcagtgcctgtctctccccagtctgaattatacctggatctcaccctatacacattatagtcactgtgcatgtacacatgggaaccatcaaaattatttgaatcttcaggtacttcttttccacaactggatgcagaagcatcaggagaggtgaaatcaccacctgcaagttctttcctctgttgctttgctgcctcccttccaaccaaattagcttcagcatcttctaacagttggctttgtggtgaagggatttcggactttggcattgccttactttcagcacaaggttcttcaggaccatctttgtcaatgctgtcgggagtctgttgattagatgtggagtcctcgggttccttgctctgctggatctcttcaccaggtatcgaagctagagaggtacttttagaagccacttctggtactggagttgcattactcttgtgagcatcctctgtatcaacacctcgcttgtttgaaggaggccaggaattagaatccttcaggtgaccaaatgtgtcaagatttgtaacagtaacagatggtaaattcaagggataatgcccagtcactgagtattcattgttttcagccttctcagaaatgatggcactgggagaatcagtgttctcaaatactgcactcagttgactcacagttggggagacagcctcagttcgggagctaaggctgtccaaggaatcagtactgcctctgttggacttggaacctccccattcatcctgaggttcactccctccagctttctctttctttggggaatagcggttgttctgtcctgattcatgcacacttctctcaaacatctttcgagtctcagtgaacttggaatatgaagggccatcgtacatagtgtcaaatctactaattcgttcagaaacagaagactccaacttaacaactgagccatctgttttttccagaaattctttgggcttcattcttctctgaggagatgaatgtccacctttcccccttgttttggcaatgactgcagcattctcgttgggttccatacccatctgcataaataggtttttaattctgttgacattggagccatatttcctccccctgctctgctgggagccctcaccttcttttgttttttgttccccatctgacttgggtttgtcaaaggtacttttcagtgcctgaaactcagttcgatatgcattcctgtgaggagaggcacttctgagagtggttcgttcacctgaagactcagttttcaacattttcacttcaggggtgaaaagccaatgttcataatgatcaaagaaaaaaaccaaaaaccaagatacctctcttctctaatcaccagtattgggtcaagaaaagtacctctcaaatggtatacggtgtcagtgatcgtcccaacaggtgtattaggaacttagtcacagtcaagagttacacagaatgattttttcaaagcaagactagaggttcatctcggctgatgggattaactctagggccgcagagagagggagcccggcagcaaaatcccgggagag

SEQ ID NO: 16995 - RNA, 10006 nt, Homo sapiens
  source 1..10006: mol_type = other RNA
taggtagtttcatgttgttgggaggtgttatctggctggagtgcctcttaattctttttaaggtaatttaattatttcttgccaattgttctttcttgaatgaatgattacatccttaacagaaaacctgggtgtataaataatacagctgaaagaaacagaagtgtacaccttccaacaacatacactcccaaccacttgtgttgtttttggcaacaaccaaaatgccattgcttgcacaaaaagtaaataaatgatcatatgatggcaacattcatcataagagagccagtaggcagtgactgtaagcatcacagccaccaattatgtcattttagaattgtgagcaaattcacaagaacacacagtgcaatttttagctgcatacatttcttctgagctccaactcagcaatatgcaatcttgacatcaaagcattagccaaatatttgaggaaattttcttactaaaataccaagtatctgataaatcaattttaccaaaatatataaacatatagaaggataagtgcatttagtagaaatacttacaataaaaaaatctcttaaaatctatgagccattcaatgtatacacaacgcaagaagtggcaataaggctatgattacagctccaggtcctgactgacctcgccaagttccatacacaatatattttttaatgccatgtgattgcagtgtgtgtgcgtgtgtaaggtgggagtgatattcacacatatgtagttctgaacatctacacaaacggcatgcacattgttgagaagttatctgttctcttattgcatacatcttactcactgttgaatccctagcagttttggggttgggttagggtcaagcataggaaatcatcatatttctttccttctccactcttgaggatctggaatcaggtcacagactgtgctgggtccacacgcttacatatgtgaaccttcaagtaactaccattccctcaataggcccacatagacaccacggacaagcaaataaggaccctctgtctaccataaatagaacttgatgctttcactttccaggagaagctgattctgtcggctttctctttgcccctccaacttcttagttgggcctattctatgctgctacttcaagttactcaaatgtgttttgtctggtgttatttttttctccagtgttttggaccaagactagatttcctgagactttaaatacgcaagacaaatgcaaacaaaatctgccaacatacccaggctgcttttcaggagtgaatcactgaagcgcatttggatttcctataacactactttcttttgggaatgtacagccctcccccagctccccatcccccatcataatgtaaaccattctaatagaaaatatggatgttttggctgggggtggtggcacatgcctgtagtcccagctacttgggaagctgaagcaggaggaccacttgagcccaggagtttgaggctgcagtaagacatgatggcaccactgcagtccagtctgggtgacagatgacagaaaaaaaaaaaaaaaaagaaaagaaaagaaaatatggacattttatttctggactttatccttaaatgcttagctttagaatagtgcacaggtacatccttaataaaaagtaaatttgaaaagacaggaaaggactgtgcttttctcttccattttaccttttcattctgagaccactaaggtctttgcattaagtaggtgacgtgaaccctagtgaccactgcccaccaaaatgcccctcatctccagctctgtcaggagtacctttagttactcaaatggaaatatctcagtgtaatgatggggctacaacatatccaaagtatagatggttctctcagggctgctggggcagcttcctttagaatcctctagaacactattgttaaacactggatctcctcttgaagtttagtctgcataacctttaacacttaaacatgaatcagagtatctatataaatgcaaattttcatttcccttttataaaatgcaattttcaagcacatgctaattctggtgcacaatgaacccagacaaatttgtcttcagcacaaactctaacggccgaggtgctagatcaaaccacctgtgaccatttttgtagcttgggactgggatattttaagatttcaggctagtgatgattacagggtcacagatagtggcaaaggtaaatctggttcctcattttccctcttgccactttgtttccaacaacaatggagcaaaaggtgacagtcccattttgtgccagttgaaagctgagtttggctttagtacctatcatactgcaatcatgaactgctgtgggttaaaaaaagcttgtgatgttgagggtgtgaaatcaattgtcaatcccagctaaaggatgatagccacagaacagctttattgtcatgaaactaaagggggacttcatcaggagtgttagaatggatgaaatgaggtttcttccctaacttaacattctgcagaaaattcctgattcaggtaaaaaaagaatgagattagtattacataaactgtgagttacttgaagggagatggtcttaaacaaagtaatctgttataaaactaacatcctttaatgggaaaccctgacccagatacagctcatacaatgctttctgtctgcagcttggcctcctcaccacacattccctcccaacaaagcataacctataccccaaaacacttttggctattgttagaatcatactgagctctcctttagggaatcagttcatagcaaccagatattccctttttgttcattttctgataataaaaactgcagtttttaaggttgatgaaataacaattctgtgttaaattgtaaggacactgaaaaccactagcattaaagtaggaattgtgcaagacattggagccttgattaggtatcatgcactacagtcaataaaagaaataataggaaaacaaaatgtgcacaagatctgaggtctttcactttgctttcatacccttaatcagtttacatcttatgctttgtggggcaatcaaaccaaatgacttttacaatttcatccgttttaagtggtaatgttaaaataactcacttcggcctaaaattactataatttaacttaaaaaatcaaaatacttataatactaaatgattttaggaataagaatttgatttataacattgtcagttggacatttatctaaacattcaatatacaaagttataaagaaaaatacttctaagatatttaagaaaatgcaatataatagatcataaattaggtgcaaaaacaagacacttacagacatttccagtatatacatccattttcaaatattaccaaagtgtaaacataacttaagataatcatccttctatttctactcttgaatacagtgaaacttccagtgtgatccaggtcacttttttcccaaagataagcaaaaatggcaaaaatttacaatagcaagcactaatattaccagatttttactaatttagtgttttagtatttgaaaagttttgccaaattgtatcactcattaatagtggcttcttatttctcatgatgtgaaaaaataacaaagcaccagacatctcaagacattaatagagtatccaatacggcagtttcattatcatacccctaatgaagacagacagaaaaacataatggtgactttgataactgtaaaacacaatgttacttcatgtcaacgtttctgaggattgaatgaagggtctgtacctaatgacaaaagagctgacgcataaccgacaatactctggcaatgaaaagaaaacaggccttgggggtaaaacagaattaaaaatgtccagtttagataatttctgaattcagattttcagataaaaaaaaatcacactgttattaaaatacaagatggggctacaagggagttcccttaatctgttacactcaaaagccttgccgaggctctaaatatggaatacttctagtggaagatacgagatgctgggaacagagcagagattcccataaagtaaaagaagtaaaatactgtccaagaattcatgtggcctcaagtcttattctgaaacttgtcctttggaaagtggataacctcatttttagagtcaacgcagcaaagagaaccagatacatgagcataaaaaacaaaaaaccctcatcacatgaaatttctcaaaacgagtttattttctccttcttctgccccagtctcctgcacttgacttagtttggtgaaacatggaaatccttaatgctggcttaaaattagtataagttcctccactactaaagtatacctatgcactgccttaaacaaactttttctgtaaaattgagaatctttgaagtatggaaaggaatggttcggaaaaaccattcaaaatctctctaaaatgttaactgacagtttcctctaactggtatttctatttttcttaaaagtacatttgttaaaatactaactgagcccacctgggaaatcttgagtagaaaatatgtgatgagttcctgattgtgacataggcaggctgaagaccagccagaatgttccccaggagaggaaacctgaaaatggtggtttccttaaaaatcaatttcctgttcaatttcttgggttaggtagggggaagaggaactgtgttgtgtttgccagtgttgctgaaatgctgaacacacagcagtagcaaggtcaacagatcccaatatcccatggctgcattaatgtctgatttttttctttcttgttcagccgtatctagaggataaatattaccctcagaaccccaaggtaatacccacatccacattcttaaggcttttgcttttttcagtggttaacaaatagctataatttattttctttctttttgatgcctagcaagcagaatgacttgcttgccttttcccttagtaggtaactacagagcagagcacccatgtttccacagcggggtggtctcactgtccagactgagaattaagagcaaatctttcccacacattggagtaggtgttgcagtcctagaagttaagtactggtctcagatctcatggcagggtgctctctgccatgcagacatgtgcaattgccatttcaggatcccacactgaaaattcacggcgctccattaacaacaccagggtgtgtcatgctcttgggtggggtcacactagttctccaagtgacaaaacacacccaacacaacacaagatgttggtaagttagagaagagcaaaacacagctacttaaatgaaatctctggtttgttaatgaaccaaaggtggcttgggattattttagtagttaaaattaagagtgcattctattgcagaaaatgcagttattcaacacacagttcctcagccggcctagagccgcattacccttatcatttagtttctttttcatcctctggaggagagcagggcaggaagaggtggggacttctcttggagcatctccatcatctgtaagagggtatgtgttactgctcaccagcaccctcggctgtagttgacgtcatcttttctgtctttttggacttcctctgcatttgctcttgctcctttctccttagcttttctctttgtttttccattttctcttgggccttccgagccttctctagagacatcttcatttccttgagtttctttttgaccactgctcggtcctgggatgctgtcattccaagagccttaagtttatttccatccaactgcaggagctgttctccagtgatgttttgggcactgaattcagatacatactgctccagatttaggctcattaaccagtgagaaacctgctgcacactccattcctgaacggcccgattctgacactgactgtgtttgggagactgtccatcatcaaggatctcatctgatgacagtgctaaggactgagagagccctggtgttttaggttctgctcctaagccgctgaggtctgctgaactggtactgctgggactgaagtcatcattgaaggtaaaattattggtttcttggatccagactacagacataagttgagaatgccttccaaagattgaagaagaggagggatttgggtttctcttgtttgcttttgtaatccatgtgttttctaccttggacccctttttatctgaaattagagtctcaggagaaggctgaagggaacttgtaggcgcaggcaggttcctgaaggaataggatcctttccggctgtcattaaaccatgagaaaggcatgcaaggggaacgagtggaggtctgagctgttgaacatggcttgggtgtccagttttccagtctgcctctgaagatcctgctacctgcagaaaacctactggcttctttttctttttctttccacttctttcccttgctggaattccttcgcaaaggcgcccccagatccacaaacttccgcttaatttttcctccttgcaccgccaatgaactggatgcccttagtgatttgggatctttggcatcatctttttctcgtaatattttcttgttggtggtttggtgatggcaaggagattcttccacatcatgatcagactttgaagtagaaaacagtgaagtgtctccccacatagaggagagaggccccatttctgggtccagtggttcttcttgaaattcagctatgtggtcagacgagaagggcacattgctatccaccggggtgaggggtggaacaccagaatctgattctggagaagacgttctcaaacccttaggtggaagtaatttggtaatatgcatgtggttatagaaactgtttgatggctttctctctagactgtcctccccatctgtggaactaacactatcatacagtcttgtcctagagggtctctggcgtctgttcttcacagagagctgggctcgagttttcagtgcttttgaatccaggcgctctgtctctgggactgcttcattcaagtcttgacttaggccatcttggcaagatgtctgcttgccatccaagttctccatggtatcccctttagagacttcaccaagagatgttcttctctcaaagatgttgttattattgttaacttgagtcccattttgcttcagtagcctgaatacctcagcttccaaatctctaatccgcacttggaggccttgcacttccacaagatgagctttttccaaatcttctattttctttctttctgcttcctgtcttttgatgaaatcaagctctttttgttgaaaatccttgatcaacttctttgccttgttgtatttcttttccaaggcctgatactggctttgagtctctttgagatgctcattcactgtgtggcataatgtttgggcctcaatccagtagctttccaacttcaacattctttccttattctcttctatgttttgttggagttgggttttttctagttcccacctcactttctcattttctgctgcctgcagcttggtcttcaatttttgaatctctgcttctgtaactgcatgtttgatttgcaactctttgaacttgtgactgagcttgcttgtgtccagttctgatggggaaaacatgtcctcattctcaggcagctcaaagacttcaatggccatgtcgctgccaggaaggacaggtcctacctcatcttcttcttcatctgtggcatattctcctgtcttaagaaaatagttgttattgttattgcagttgccagacattccttgcaattcagccacagtgttcccccgagtgtcatgaaatagtgctgattgtctgagagatttattgaaatcctccatggcaacctcgtcatcgtcggcatcatactgggcatagtgctgttccagcagctctctctggcgcctctcctgttccagtgtctggcttatcaactgggcaacctcgctcacttgtcctggtttttcccgcccaataacaaatctgacgttgcccttggtgtttctgagaactgttgctgcaaaattctgtgtcacacccaccaagctgattccatccacttccacaatctggtcattgacttgtattctgccatcccgttgagcagcaccaccttctgttactgtcttgacgaatattcccagcttttcaagtccagcatctgctccaacacccattccaataatacttataccaagaccatcctcatctttctctagctccactgggaaaagttccagcttttctacacgtttttcaagttcatactcagctgaagcagccacagggtcaacttcgtcatttctcctgtcatagtcttcattggagtatgtgttgaaaaccttaataggagcactactaaacttaattttcctatttgctgggatttcttcttcttctggcaatccaacaatttccgagtactccatatcaggctgatagtaactgttctcatcactatcttcctcctcatcctgctcagtgcctgtctctccccagtctgaattatacctggatctcaccctatacacattatagtcactgtgcatgtacacatgggaaccatcaaaattatttgaatcttcaggtacttcttttccacaactggatgcagaagcatcaggagaggtgaaatcaccacctgcaagttctttcctctgttgctttgctgcctcccttccaaccaaattagcttcagcatcttctaacagttggctttgtggtgaagggatttcggactttggcattgccttactttcagcacaaggttcttcaggaccatctttgtcaatgctgtcgggagtctgttgattagatgtggagtcctcgggttccttgctctgctggatctcttcaccaggtatcgaagctagagaggtacttttagaagccacttctggtactggagttgcattactcttgtgagcatcctctgtatcaacacctcgcttgtttgaaggaggccaggaattagaatccttcaggtgaccaaatgtgtcaagatttgtaacagtaacagatggtaaattcaagggataatgcccagtcactgagtattcattgttttcagccttctcagaaatgatggcactgggagaatcagtgttctcaaatactgcactcagttgactcacagttggggagacagcctcagttcgggagctaaggctgtccaaggaatcagtactgcctctgttggacttggaacctccccattcatcctgaggttcactccctccagctttctctttctttggggaatagcggttgttctgtcctgattcatgcacacttctctcaaacatctttcgagtctcagtgaacttggaatatgaagggccatcgtacatagtgtcaaatctactaattcgttcagaaacagaagactccaacttaacaactgagccatctgttttttccagaaattctttgggcttcattcttctctgaggagatgaatgtccacctttcccccttgttttggcaatgactgcagcattctcgttgggttccatacccatctgcataaataggtttttaattctgttgacattggagccatatttcctccccctgctctgctgggagccctcaccttcttttgttttttgttccccatctgacttgggtttgtcaaaggtacttttcagtgcctgaaactcagttcgatatgcattcctgtgaggagaggcacttctgagagtggttcgttcacctgaagactcagttttcaacattttcacttcaggggtgaaaagccaatgttcataatgatcaaagaaaaaaaccaaaaaccaagatacctctcttctctaatcaccagtattgggtcaagaaaagtacctctcaaatggtatacggtgtcagtgatcgtcccaacaggtgtattaggaacttagtcacagtcaagagttacacagaatgattttttcaaagcaagactagaggttcatccgagcgggagcgccgcgggcggggagggtcgggccgccgcggctcccaccccctcctcgcaggcgccccccgccccac

SEQ ID NO: 16996 - RNA, 9993 nt, Homo sapiens
  source 1..9993: mol_type = other RNA
taggtagtttcatgttgttgggaggtgttatctggctggagtgcctcttaattctttttaaggtaatttaattatttcttgccaattgttctttcttgaatgaatgattacatccttaacagaaaacctgggtgtataaataatacagctgaaagaaacagaagtgtacaccttccaacaacatacactcccaaccacttgtgttgtttttggcaacaaccaaaatgccattgcttgcacaaaaagtaaataaatgatcatatgatggcaacattcatcataagagagccagtaggcagtgactgtaagcatcacagccaccaattatgtcattttagaattgtgagcaaattcacaagaacacacagtgcaatttttagctgcatacatttcttctgagctccaactcagcaatatgcaatcttgacatcaaagcattagccaaatatttgaggaaattttcttactaaaataccaagtatctgataaatcaattttaccaaaatatataaacatatagaaggataagtgcatttagtagaaatacttacaataaaaaaatctcttaaaatctatgagccattcaatgtatacacaacgcaagaagtggcaataaggctatgattacagctccaggtcctgactgacctcgccaagttccatacacaatatattttttaatgccatgtgattgcagtgtgtgtgcgtgtgtaaggtgggagtgatattcacacatatgtagttctgaacatctacacaaacggcatgcacattgttgagaagttatctgttctcttattgcatacatcttactcactgttgaatccctagcagttttggggttgggttagggtcaagcataggaaatcatcatatttctttccttctccactcttgaggatctggaatcaggtcacagactgtgctgggtccacacgcttacatatgtgaaccttcaagtaactaccattccctcaataggcccacatagacaccacggacaagcaaataaggaccctctgtctaccataaatagaacttgatgctttcactttccaggagaagctgattctgtcggctttctctttgcccctccaacttcttagttgggcctattctatgctgctacttcaagttactcaaatgtgttttgtctggtgttatttttttctccagtgttttggaccaagactagatttcctgagactttaaatacgcaagacaaatgcaaacaaaatctgccaacatacccaggctgcttttcaggagtgaatcactgaagcgcatttggatttcctataacactactttcttttgggaatgtacagccctcccccagctccccatcccccatcataatgtaaaccattctaatagaaaatatggatgttttggctgggggtggtggcacatgcctgtagtcccagctacttgggaagctgaagcaggaggaccacttgagcccaggagtttgaggctgcagtaagacatgatggcaccactgcagtccagtctgggtgacagatgacagaaaaaaaaaaaaaaaaagaaaagaaaagaaaatatggacattttatttctggactttatccttaaatgcttagctttagaatagtgcacaggtacatccttaataaaaagtaaatttgaaaagacaggaaaggactgtgcttttctcttccattttaccttttcattctgagaccactaaggtctttgcattaagtaggtgacgtgaaccctagtgaccactgcccaccaaaatgcccctcatctccagctctgtcaggagtacctttagttactcaaatggaaatatctcagtgtaatgatggggctacaacatatccaaagtatagatggttctctcagggctgctggggcagcttcctttagaatcctctagaacactattgttaaacactggatctcctcttgaagtttagtctgcataacctttaacacttaaacatgaatcagagtatctatataaatgcaaattttcatttcccttttataaaatgcaattttcaagcacatgctaattctggtgcacaatgaacccagacaaatttgtcttcagcacaaactctaacggccgaggtgctagatcaaaccacctgtgaccatttttgtagcttgggactgggatattttaagatttcaggctagtgatgattacagggtcacagatagtggcaaaggtaaatctggttcctcattttccctcttgccactttgtttccaacaacaatggagcaaaaggtgacagtcccattttgtgccagttgaaagctgagtttggctttagtacctatcatactgcaatcatgaactgctgtgggttaaaaaaagcttgtgatgttgagggtgtgaaatcaattgtcaatcccagctaaaggatgatagccacagaacagctttattgtcatgaaactaaagggggacttcatcaggagtgttagaatggatgaaatgaggtttcttccctaacttaacattctgcagaaaattcctgattcaggtaaaaaaagaatgagattagtattacataaactgtgagttacttgaagggagatggtcttaaacaaagtaatctgttataaaactaacatcctttaatgggaaaccctgacccagatacagctcatacaatgctttctgtctgcagcttggcctcctcaccacacattccctcccaacaaagcataacctataccccaaaacacttttggctattgttagaatcatactgagctctcctttagggaatcagttcatagcaaccagatattccctttttgttcattttctgataataaaaactgcagtttttaaggttgatgaaataacaattctgtgttaaattgtaaggacactgaaaaccactagcattaaagtaggaattgtgcaagacattggagccttgattaggtatcatgcactacagtcaataaaagaaataataggaaaacaaaatgtgcacaagatctgaggtctttcactttgctttcatacccttaatcagtttacatcttatgctttgtggggcaatcaaaccaaatgacttttacaatttcatccgttttaagtggtaatgttaaaataactcacttcggcctaaaattactataatttaacttaaaaaatcaaaatacttataatactaaatgattttaggaataagaatttgatttataacattgtcagttggacatttatctaaacattcaatatacaaagttataaagaaaaatacttctaagatatttaagaaaatgcaatataatagatcataaattaggtgcaaaaacaagacacttacagacatttccagtatatacatccattttcaaatattaccaaagtgtaaacataacttaagataatcatccttctatttctactcttgaatacagtgaaacttccagtgtgatccaggtcacttttttcccaaagataagcaaaaatggcaaaaatttacaatagcaagcactaatattaccagatttttactaatttagtgttttagtatttgaaaagttttgccaaattgtatcactcattaatagtggcttcttatttctcatgatgtgaaaaaataacaaagcaccagacatctcaagacattaatagagtatccaatacggcagtttcattatcatacccctaatgaagacagacagaaaaacataatggtgactttgataactgtaaaacacaatgttacttcatgtcaacgtttctgaggattgaatgaagggtctgtacctaatgacaaaagagctgacgcataaccgacaatactctggcaatgaaaagaaaacaggccttgggggtaaaacagaattaaaaatgtccagtttagataatttctgaattcagattttcagataaaaaaaaatcacactgttattaaaatacaagatggggctacaagggagttcccttaatctgttacactcaaaagccttgccgaggctctaaatatggaatacttctagtggaagatacgagatgctgggaacagagcagagattcccataaagtaaaagaagtaaaatactgtccaagaattcatgtggcctcaagtcttattctgaaacttgtcctttggaaagtggataacctcatttttagagtcaacgcagcaaagagaaccagatacatgagcataaaaaacaaaaaaccctcatcacatgaaatttctcaaaacgagtttattttctccttcttctgccccagtctcctgcacttgacttagtttggtgaaacatggaaatccttaatgctggcttaaaattagtataagttcctccactactaaagtatacctatgcactgccttaaacaaactttttctgtaaaattgagaatctttgaagtatggaaaggaatggttcggaaaaaccattcaaaatctctctaaaatgttaactgacagtttcctctaactggtatttctatttttcttaaaagtacatttgttaaaatactaactgagcccacctgggaaatcttgagtagaaaatatgtgatgagttcctgattgtgacataggcaggctgaagaccagccagaatgttccccaggagaggaaacctgaaaatggtggtttccttaaaaatcaatttcctgttcaatttcttgggttaggtagggggaagaggaactgtgttgtgtttgccagtgttgctgaaatgctgaacacacagcagtagcaaggtcaacagatcccaatatcccatggctgcattaatgtctgatttttttctttcttgttcagccgtatctagaggataaatattaccctcagaaccccaaggtaatacccacatccacattcttaaggcttttgcttttttcagtggttaacaaatagctataatttattttctttctttttgatgcctagcaagcagaatgacttgcttgccttttcccttagtaggtaactacagagcagagcacccatgtttccacagcggggtggtctcactgtccagactgagaattaagagcaaatctttcccacacattggagtaggtgttgcagtcctagaagttaagtactggtctcagatctcatggcagggtgctctctgccatgcagacatgtgcaattgccatttcaggatcccacactgaaaattcacggcgctccattaacaacaccagggtgtgtcatgctcttgggtggggtcacactagttctccaagtgacaaaacacacccaacacaacacaagatgttggtaagttagagaagagcaaaacacagctacttaaatgaaatctctggtttgttaatgaaccaaaggtggcttgggattattttagtagttaaaattaagagtgcattctattgcagaaaatgcagttattcaacacacagttcctcagccggcctagagccgcattacccttatcatttagtttctttttcatcctctggaggagagcagggcaggaagaggtggggacttctcttggagcatctccatcatctgtaagagggtatgtgttactgctcaccagcaccctcggctgtagttgacgtcatcttttctgtctttttggacttcctctgcatttgctcttgctcctttctccttagcttttctctttgtttttccattttctcttgggccttccgagccttctctagagacatcttcatttccttgagtttctttttgaccactgctcggtcctgggatgctgtcattccaagagccttaagtttatttccatccaactgcaggagctgttctccagtgatgttttgggcactgaattcagatacatactgctccagatttaggctcattaaccagtgagaaacctgctgcacactccattcctgaacggcccgattctgacactgactgtgtttgggagactgtccatcatcaaggatctcatctgatgacagtgctaaggactgagagagccctggtgttttaggttctgctcctaagccgctgaggtctgctgaactggtactgctgggactgaagtcatcattgaaggtaaaattattggtttcttggatccagactacagacataagttgagaatgccttccaaagattgaagaagaggagggatttgggtttctcttgtttgcttttgtaatccatgtgttttctaccttggacccctttttatctgaaattagagtctcaggagaaggctgaagggaacttgtaggcgcaggcaggttcctgaaggaataggatcctttccggctgtcattaaaccatgagaaaggcatgcaaggggaacgagtggaggtctgagctgttgaacatggcttgggtgtccagttttccagtctgcctctgaagatcctgctacctgcagaaaacctactggcttctttttctttttctttccacttctttcccttgctggaattccttcgcaaaggcgcccccagatccacaaacttccgcttaatttttcctccttgcaccgccaatgaactggatgcccttagtgatttgggatctttggcatcatctttttctcgtaatattttcttgttggtggtttggtgatggcaaggagattcttccacatcatgatcagactttgaagtagaaaacagtgaagtgtctccccacatagaggagagaggccccatttctgggtccagtggttcttcttgaaattcagctatgtggtcagacgagaagggcacattgctatccaccggggtgaggggtggaacaccagaatctgattctggagaagacgttctcaaacccttaggtggaagtaatttggtaatatgcatgtggttatagaaactgtttgatggctttctctctagactgtcctccccatctgtggaactaacactatcatacagtcttgtcctagagggtctctggcgtctgttcttcacagagagctgggctcgagttttcagtgcttttgaatccaggcgctctgtctctgggactgcttcattcaagtcttgacttaggccatcttggcaagatgtctgcttgccatccaagttctccatggtatcccctttagagacttcaccaagagatgttcttctctcaaagatgttgttattattgttaacttgagtcccattttgcttcagtagcctgaatacctcagcttccaaatctctaatccgcacttggaggccttgcacttccacaagatgagctttttccaaatcttctattttctttctttctgcttcctgtcttttgatgaaatcaagctctttttgttgaaaatccttgatcaacttctttgccttgttgtatttcttttccaaggcctgatactggctttgagtctctttgagatgctcattcactgtgtggcataatgtttgggcctcaatccagtagctttccaacttcaacattctttccttattctcttctatgttttgttggagttgggttttttctagttcccacctcactttctcattttctgctgcctgcagcttggtcttcaatttttgaatctctgcttctgtaactgcatgtttgatttgcaactctttgaacttgtgactgagcttgcttgtgtccagttctgatggggaaaacatgtcctcattctcaggcagctcaaagacttcaatggccatgtcgctgccaggaaggacaggtcctacctcatcttcttcttcatctgtggcatattctcctgtcttaagaaaatagttgttattgttattgcagttgccagacattccttgcaattcagccacagtgttcccccgagtgtcatgaaatagtgctgattgtctgagagatttattgaaatcctccatggcaacctcgtcatcgtcggcatcatactgggcatagtgctgttccagcagctctctctggcgcctctcctgttccagtgtctggcttatcaactgggcaacctcgctcacttgtcctggtttttcccgcccaataacaaatctgacgttgcccttggtgtttctgagaactgttgctgcaaaattctgtgtcacacccaccaagctgattccatccacttccacaatctggtcattgacttgtattctgccatcccgttgagcagcaccaccttctgttactgtcttgacgaatattcccagcttttcaagtccagcatctgctccaacacccattccaataatacttataccaagaccatcctcatctttctctagctccactgggaaaagttccagcttttctacacgtttttcaagttcatactcagctgaagcagccacagggtcaacttcgtcatttctcctgtcatagtcttcattggagtatgtgttgaaaaccttaataggagcactactaaacttaattttcctatttgctgggatttcttcttcttctggcaatccaacaatttccgagtactccatatcaggctgatagtaactgttctcatcactatcttcctcctcatcctgctcagtgcctgtctctccccagtctgaattatacctggatctcaccctatacacattatagtcactgtgcatgtacacatgggaaccatcaaaattatttgaatcttcaggtacttcttttccacaactggatgcagaagcatcaggagaggtgaaatcaccacctgcaagttctttcctctgttgctttgctgcctcccttccaaccaaattagcttcagcatcttctaacagttggctttgtggtgaagggatttcggactttggcattgccttactttcagcacaaggttcttcaggaccatctttgtcaatgctgtcgggagtctgttgattagatgtggagtcctcgggttccttgctctgctggatctcttcaccaggtatcgaagctagagaggtacttttagaagccacttctggtactggagttgcattactcttgtgagcatcctctgtatcaacacctcgcttgtttgaaggaggccaggaattagaatccttcaggtgaccaaatgtgtcaagatttgtaacagtaacagatggtaaattcaagggataatgcccagtcactgagtattcattgttttcagccttctcagaaatgatggcactgggagaatcagtgttctcaaatactgcactcagttgactcacagttggggagacagcctcagttcgggagctaaggctgtccaaggaatcagtactgcctctgttggacttggaacctccccattcatcctgaggttcactccctccagctttctctttctttggggaatagcggttgttctgtcctgattcatgcacacttctctcaaacatctttcgagtctcagtgaacttggaatatgaagggccatcgtacatagtgtcaaatctactaattcgttcagaaacagaagactccaacttaacaactgagccatctgttttttccagaaattctttgggcttcattcttctctgaggagatgaatgtccacctttcccccttgttttggcaatgactgcagcattctcgttgggttccatacccatctgcataaataggtttttaattctgttgacattggagccatatttcctccccctgctctgctgggagccctcaccttcttttgttttttgttccccatctgacttgggtttgtcaaaggtacttttcagtgcctgaaactcagttcgatatgcattcctgtgaggagaggcacttctgagagtggttcgttcacctgaagactcagttttcaacattttcacttcaggggtgaaaagccaatgttcataatgatcaaagaaaaaaaccaaaaaccaagatacctctcttctctaatcaccagtattgggtcaagaaaagtacctctcaaatggtatacggtgtcagtgatcgtcccaacaggtgtattaggaacttagtcacagtcaagagttacacagaatgattttttcaaagcaagactagaggttcatctcggctgatgggattaactctagggccgcagagagagggagcccggcagcaaaatcccgggagag

SEQ ID NO: 16997 - RNA, 10047 nt, Homo sapiens
  source 1..10047: mol_type = other RNA
taggtagtttcatgttgttgggaggtgttatctggctggagtgcctcttaattctttttaaggtaatttaattatttcttgccaattgttctttcttgaatgaatgattacatccttaacagaaaacctgggtgtataaataatacagctgaaagaaacagaagtgtacaccttccaacaacatacactcccaaccacttgtgttgtttttggcaacaaccaaaatgccattgcttgcacaaaaagtaaataaatgatcatatgatggcaacattcatcataagagagccagtaggcagtgactgtaagcatcacagccaccaattatgtcattttagaattgtgagcaaattcacaagaacacacagtgcaatttttagctgcatacatttcttctgagctccaactcagcaatatgcaatcttgacatcaaagcattagccaaatatttgaggaaattttcttactaaaataccaagtatctgataaatcaattttaccaaaatatataaacatatagaaggataagtgcatttagtagaaatacttacaataaaaaaatctcttaaaatctatgagccattcaatgtatacacaacgcaagaagtggcaataaggctatgattacagctccaggtcctgactgacctcgccaagttccatacacaatatattttttaatgccatgtgattgcagtgtgtgtgcgtgtgtaaggtgggagtgatattcacacatatgtagttctgaacatctacacaaacggcatgcacattgttgagaagttatctgttctcttattgcatacatcttactcactgttgaatccctagcagttttggggttgggttagggtcaagcataggaaatcatcatatttctttccttctccactcttgaggatctggaatcaggtcacagactgtgctgggtccacacgcttacatatgtgaaccttcaagtaactaccattccctcaataggcccacatagacaccacggacaagcaaataaggaccctctgtctaccataaatagaacttgatgctttcactttccaggagaagctgattctgtcggctttctctttgcccctccaacttcttagttgggcctattctatgctgctacttcaagttactcaaatgtgttttgtctggtgttatttttttctccagtgttttggaccaagactagatttcctgagactttaaatacgcaagacaaatgcaaacaaaatctgccaacatacccaggctgcttttcaggagtgaatcactgaagcgcatttggatttcctataacactactttcttttgggaatgtacagccctcccccagctccccatcccccatcataatgtaaaccattctaatagaaaatatggatgttttggctgggggtggtggcacatgcctgtagtcccagctacttgggaagctgaagcaggaggaccacttgagcccaggagtttgaggctgcagtaagacatgatggcaccactgcagtccagtctgggtgacagatgacagaaaaaaaaaaaaaaaaagaaaagaaaagaaaatatggacattttatttctggactttatccttaaatgcttagctttagaatagtgcacaggtacatccttaataaaaagtaaatttgaaaagacaggaaaggactgtgcttttctcttccattttaccttttcattctgagaccactaaggtctttgcattaagtaggtgacgtgaaccctagtgaccactgcccaccaaaatgcccctcatctccagctctgtcaggagtacctttagttactcaaatggaaatatctcagtgtaatgatggggctacaacatatccaaagtatagatggttctctcagggctgctggggcagcttcctttagaatcctctagaacactattgttaaacactggatctcctcttgaagtttagtctgcataacctttaacacttaaacatgaatcagagtatctatataaatgcaaattttcatttcccttttataaaatgcaattttcaagcacatgctaattctggtgcacaatgaacccagacaaatttgtcttcagcacaaactctaacggccgaggtgctagatcaaaccacctgtgaccatttttgtagcttgggactgggatattttaagatttcaggctagtgatgattacagggtcacagatagtggcaaaggtaaatctggttcctcattttccctcttgccactttgtttccaacaacaatggagcaaaaggtgacagtcccattttgtgccagttgaaagctgagtttggctttagtacctatcatactgcaatcatgaactgctgtgggttaaaaaaagcttgtgatgttgagggtgtgaaatcaattgtcaatcccagctaaaggatgatagccacagaacagctttattgtcatgaaactaaagggggacttcatcaggagtgttagaatggatgaaatgaggtttcttccctaacttaacattctgcagaaaattcctgattcaggtaaaaaaagaatgagattagtattacataaactgtgagttacttgaagggagatggtcttaaacaaagtaatctgttataaaactaacatcctttaatgggaaaccctgacccagatacagctcatacaatgctttctgtctgcagcttggcctcctcaccacacattccctcccaacaaagcataacctataccccaaaacacttttggctattgttagaatcatactgagctctcctttagggaatcagttcatagcaaccagatattccctttttgttcattttctgataataaaaactgcagtttttaaggttgatgaaataacaattctgtgttaaattgtaaggacactgaaaaccactagcattaaagtaggaattgtgcaagacattggagccttgattaggtatcatgcactacagtcaataaaagaaataataggaaaacaaaatgtgcacaagatctgaggtctttcactttgctttcatacccttaatcagtttacatcttatgctttgtggggcaatcaaaccaaatgacttttacaatttcatccgttttaagtggtaatgttaaaataactcacttcggcctaaaattactataatttaacttaaaaaatcaaaatacttataatactaaatgattttaggaataagaatttgatttataacattgtcagttggacatttatctaaacattcaatatacaaagttataaagaaaaatacttctaagatatttaagaaaatgcaatataatagatcataaattaggtgcaaaaacaagacacttacagacatttccagtatatacatccattttcaaatattaccaaagtgtaaacataacttaagataatcatccttctatttctactcttgaatacagtgaaacttccagtgtgatccaggtcacttttttcccaaagataagcaaaaatggcaaaaatttacaatagcaagcactaatattaccagatttttactaatttagtgttttagtatttgaaaagttttgccaaattgtatcactcattaatagtggcttcttatttctcatgatgtgaaaaaataacaaagcaccagacatctcaagacattaatagagtatccaatacggcagtttcattatcatacccctaatgaagacagacagaaaaacataatggtgactttgataactgtaaaacacaatgttacttcatgtcaacgtttctgaggattgaatgaagggtctgtacctaatgacaaaagagctgacgcataaccgacaatactctggcaatgaaaagaaaacaggccttgggggtaaaacagaattaaaaatgtccagtttagataatttctgaattcagattttcagataaaaaaaaatcacactgttattaaaatacaagatggggctacaagggagttcccttaatctgttacactcaaaagccttgccgaggctctaaatatggaatacttctagtggaagatacgagatgctgggaacagagcagagattcccataaagtaaaagaagtaaaatactgtccaagaattcatgtggcctcaagtcttattctgaaacttgtcctttggaaagtggataacctcatttttagagtcaacgcagcaaagagaaccagatacatgagcataaaaaacaaaaaaccctcatcacatgaaatttctcaaaacgagtttattttctccttcttctgccccagtctcctgcacttgacttagtttggtgaaacatggaaatccttaatgctggcttaaaattagtataagttcctccactactaaagtatacctatgcactgccttaaacaaactttttctgtaaaattgagaatctttgaagtatggaaaggaatggttcggaaaaaccattcaaaatctctctaaaatgttaactgacagtttcctctaactggtatttctatttttcttaaaagtacatttgttaaaatactaactgagcccacctgggaaatcttgagtagaaaatatgtgatgagttcctgattgtgacataggcaggctgaagaccagccagaatgttccccaggagaggaaacctgaaaatggtggtttccttaaaaatcaatttcctgttcaatttcttgggttaggtagggggaagaggaactgtgttgtgtttgccagtgttgctgaaatgctgaacacacagcagtagcaaggtcaacagatcccaatatcccatggctgcattaatgtctgatttttttctttcttgttcagccgtatctagaggataaatattaccctcagaaccccaaggtaatacccacatccacattcttaaggcttttgcttttttcagtggttaacaaatagctataatttattttctttctttttgatgcctagcaagcagaatgacttgcttgccttttcccttagtaggtaactacagagcagagcacccatgtttccacagcggggtggtctcactgtccagactgagaattaagagcaaatctttcccacacattggagtaggtgttgcagtcctagaagttaagtactggtctcagatctcatggcagggtgctctctgccatgcagacatgtgcaattgccatttcaggatcccacactgaaaattcacggcgctccattaacaacaccagggtgtgtcatgctcttgggtggggtcacactagttctccaagtgacaaaacacacccaacacaacacaagatgttggtaagttagagaagagcaaaacacagctacttaaatgaaatctctggtttgttaatgaaccaaaggtggcttgggattattttagtagttaaaattaagagtgcattctattgcagaaaatgcagttattcaacacacagttcctcagccggcctagagccgcattacccttatcatttagtttctttttcatcctctggaggagagcagggcaggaagaggtggggacttctcttggagcatctccatcatctgtaagagggtatgtgttactgctcaccagcaccctcggctgtagttgacgtcatcttttctgtctttttggacttcctctgcatttgctcttgctcctttctccttagcttttctctttgtttttccattttctcttgggccttccgagccttctctagagacatcttcatttccttgagtttctttttgaccactgctcggtcctgggatgctgtcattccaagagccttaagtttatttccatccaactgcaggagctgttctccagtgatgttttgggcactgaattcagatacatactgctccagatttaggctcattaaccagtgagaaacctgctgcacactccattcctgaacggcccgattctgacactgactgtgtttgggagactgtccatcatcaaggatctcatctgatgacagtgctaaggactgagagagccctggtgttttaggttctgctcctaagccgctgaggtctgctgaactggtactgctgggactgaagtcatcattgaaggtaaaattattggtttcttggatccagactacagacataagttgagaatgccttccaaagattgaagaagaggagggatttgggtttctcttgtttgcttttgtaatccatgtgttttctaccttggacccctttttatctgaaattagagtctcaggagaaggctgaagggaacttgtaggcgcaggcaggttcctgaaggaataggatcctttccggctgtcattaaaccatgagaaaggcatgcaaggggaacgagtggaggtctgagctgttgaacatggcttgggtgtccagttttccagtctgcctctgaagatcctgctacctgcagaaaacctactggcttctttttctttttctttccacttctttcccttgctggaattccttcgcaaaggcgcccccagatccacaaacttccgcttaatttttcctccttgcaccgccaatgaactggatgcccttagtgatttgggatctttggcatcatctttttctcgtaatattttcttgttggtggtttggtgatggcaaggagattcttccacatcatgatcagactttgaagtagaaaacagtgaagtgtctccccacatagaggagagaggccccatttctgggtccagtggttcttcttgaaattcagctatgtggtcagacgagaagggcacattgctatccaccggggtgaggggtggaacaccagaatctgattctggagaagacgttctcaaacccttaggtggaagtaatttggtaatatgcatgtggttatagaaactgtttgatggctttctctctagactgtcctccccatctgtggaactaacactatcatacagtcttgtcctagagggtctctggcgtctgttcttcacagagagctgggctcgagttttcagtgcttttgaatccaggcgctctgtctctgggactgcttcattcaagtcttgacttaggccatcttggcaagatgtctgcttgccatccaagttctccatggtatcccctttagagacttcaccaagagatgttcttctctcaaagatgttgttattattgttaacttgagtcccattttgcttcagtagcctgaatacctcagcttccaaatctctaatccgcacttggaggccttgcacttccacaagatgagctttttccaaatcttctattttctttctttctgcttcctgtcttttgatgaaatcaagctctttttgttgaaaatccttgatcaacttctttgccttgttgtatttcttttccaaggcctgatactggctttgagtctctttgagatgctcattcactgtgtggcataatgtttgggcctcaatccagtagctttccaacttcaacattctttccttattctcttctatgttttgttggagttgggttttttctagttcccacctcactttctcattttctgctgcctgcagcttggtcttcaatttttgaatctctgcttctgtaactgcatgtttgatttgcaactctttgaacttgtgactgagcttgcttgtgtccagttctgatggggaaaacatgtcctcattctcaggcagctcaaagacttcaatggccatgtcgctgccaggaaggacaggtcctacctcatcttcttcttcatctgtggcatattctcctgtcttaagaaaatagttgttattgttattgcagttgccagacattccttgcaattcagccacagtgttcccccgagtgtcatgaaatagtgctgattgtctgagagatttattgaaatcctccatggcaacctcgtcatcgtcggcatcatactgggcatagtgctgttccagcagctctctctggcgcctctcctgttccagtgtctggcttatcaactgggcaacctcgctcacttgtcctggtttttcccgcccaataacaaatctgacgttgcccttggtgtttctgagaactgttgctgcaaaattctgtgtcacacccaccaagctgattccatccacttccacaatctggtcattgacttgtattctgccatcccgttgagcagcaccaccttctgttactgtcttgacgaatattcccagcttttcaagtccagcatctgctccaacacccattccaataatacttataccaagaccatcctcatctttctctagctccactgggaaaagttccagcttttctacacgtttttcaagttcatactcagctgaagcagccacagggtcaacttcgtcatttctcctgtcatagtcttcattggagtatgtgttgaaaaccttaataggagcactactaaacttaattttcctatttgctgggatttcttcttcttctggcaatccaacaatttccgagtactccatatcaggctgatagtaactgttctcatcactatcttcctcctcatcctgctcagtgcctgtctctccccagtctgaattatacctggatctcaccctatacacattatagtcactgtgcatgtacacatgggaaccatcaaaattatttgaatcttcaggtacttcttttccacaactggatgcagaagcatcaggagaggtgaaatcaccacctgcaagttctttcctctgttgctttgctgcctcccttccaaccaaattagcttcagcatcttctaacagttggctttgtggtgaagggatttcggactttggcattgccttactttcagcacaaggttcttcaggaccatctttgtcaatgctgtcgggagtctgttgattagatgtggagtcctcgggttccttgctctgctggatctcttcaccaggtatcgaagctagagaggtacttttagaagccacttctggtactggagttgcattactcttgtgagcatcctctgtatcaacacctcgcttgtttgaaggaggccaggaattagaatccttcaggtgaccaaatgtgtcaagatttgtaacagtaacagatggtaaattcaagggataatgcccagtcactgagtattcattgttttcagccttctcagaaatgatggcactgggagaatcagtgttctcaaatactgcactcagttgactcacagttggggagacagcctcagttcgggagctaaggctgtccaaggaatcagtactgcctctgttggacttggaacctccccattcatcctgaggttcactccctccagctttctctttctttggggaatagcggttgttctgtcctgattcatgcacacttctctcaaacatctttcgagtctcagtgaacttggaatatgaagggccatcgtacatagtgtcaaatctactaattcgttcagaaacagaagactccaacttaacaactgagccatctgttttttccagaaattctttgggcttcattcttctctgaggagatgaatgtccacctttcccccttgttttggcaatgactgcagcattctcgttgggttccatacccatctgcataaataggtttttaattctgttgacattggagccatatttcctccccctgctctgctgggagccctcaccttcttttgttttttgttccccatctgacttgggtttgtcaaaggtacttttcagtgcctgaaactcagttcgatatgcattcctgtgaggagaggcacttctgagagtggttcgttcacctgaagactcagttttcaacattttcacttcaggggtgaaaagccaatgttcataatgatcaaagaaaaaaaccaaaaaccaagatacctctcttctctaatcaccagtattgggtcaagaaaagtacctctcaaatggtatacggtgtcagtgatcgtcccaacaggtgtattaggaacttagtcacagtcaagagttacacagaatgattttttcaaagcaagactagaggttcatcttgaccttaagatctcactgccaaagagaaagggatgaggaggtcttctacctttcctgtctagggagagtttttcagctcactcccccccgaaccccgcccttttctaaaggctcagt

SEQ ID NO: 16998 - RNA, 10117 nt, Homo sapiens
  source 1..10117: mol_type = other RNA
taggtagtttcatgttgttgggaggtgttatctggctggagtgcctcttaattctttttaaggtaatttaattatttcttgccaattgttctttcttgaatgaatgattacatccttaacagaaaacctgggtgtataaataatacagctgaaagaaacagaagtgtacaccttccaacaacatacactcccaaccacttgtgttgtttttggcaacaaccaaaatgccattgcttgcacaaaaagtaaataaatgatcatatgatggcaacattcatcataagagagccagtaggcagtgactgtaagcatcacagccaccaattatgtcattttagaattgtgagcaaattcacaagaacacacagtgcaatttttagctgcatacatttcttctgagctccaactcagcaatatgcaatcttgacatcaaagcattagccaaatatttgaggaaattttcttactaaaataccaagtatctgataaatcaattttaccaaaatatataaacatatagaaggataagtgcatttagtagaaatacttacaataaaaaaatctcttaaaatctatgagccattcaatgtatacacaacgcaagaagtggcaataaggctatgattacagctccaggtcctgactgacctcgccaagttccatacacaatatattttttaatgccatgtgattgcagtgtgtgtgcgtgtgtaaggtgggagtgatattcacacatatgtagttctgaacatctacacaaacggcatgcacattgttgagaagttatctgttctcttattgcatacatcttactcactgttgaatccctagcagttttggggttgggttagggtcaagcataggaaatcatcatatttctttccttctccactcttgaggatctggaatcaggtcacagactgtgctgggtccacacgcttacatatgtgaaccttcaagtaactaccattccctcaataggcccacatagacaccacggacaagcaaataaggaccctctgtctaccataaatagaacttgatgctttcactttccaggagaagctgattctgtcggctttctctttgcccctccaacttcttagttgggcctattctatgctgctacttcaagttactcaaatgtgttttgtctggtgttatttttttctccagtgttttggaccaagactagatttcctgagactttaaatacgcaagacaaatgcaaacaaaatctgccaacatacccaggctgcttttcaggagtgaatcactgaagcgcatttggatttcctataacactactttcttttgggaatgtacagccctcccccagctccccatcccccatcataatgtaaaccattctaatagaaaatatggatgttttggctgggggtggtggcacatgcctgtagtcccagctacttgggaagctgaagcaggaggaccacttgagcccaggagtttgaggctgcagtaagacatgatggcaccactgcagtccagtctgggtgacagatgacagaaaaaaaaaaaaaaaaagaaaagaaaagaaaatatggacattttatttctggactttatccttaaatgcttagctttagaatagtgcacaggtacatccttaataaaaagtaaatttgaaaagacaggaaaggactgtgcttttctcttccattttaccttttcattctgagaccactaaggtctttgcattaagtaggtgacgtgaaccctagtgaccactgcccaccaaaatgcccctcatctccagctctgtcaggagtacctttagttactcaaatggaaatatctcagtgtaatgatggggctacaacatatccaaagtatagatggttctctcagggctgctggggcagcttcctttagaatcctctagaacactattgttaaacactggatctcctcttgaagtttagtctgcataacctttaacacttaaacatgaatcagagtatctatataaatgcaaattttcatttcccttttataaaatgcaattttcaagcacatgctaattctggtgcacaatgaacccagacaaatttgtcttcagcacaaactctaacggccgaggtgctagatcaaaccacctgtgaccatttttgtagcttgggactgggatattttaagatttcaggctagtgatgattacagggtcacagatagtggcaaaggtaaatctggttcctcattttccctcttgccactttgtttccaacaacaatggagcaaaaggtgacagtcccattttgtgccagttgaaagctgagtttggctttagtacctatcatactgcaatcatgaactgctgtgggttaaaaaaagcttgtgatgttgagggtgtgaaatcaattgtcaatcccagctaaaggatgatagccacagaacagctttattgtcatgaaactaaagggggacttcatcaggagtgttagaatggatgaaatgaggtttcttccctaacttaacattctgcagaaaattcctgattcaggtaaaaaaagaatgagattagtattacataaactgtgagttacttgaagggagatggtcttaaacaaagtaatctgttataaaactaacatcctttaatgggaaaccctgacccagatacagctcatacaatgctttctgtctgcagcttggcctcctcaccacacattccctcccaacaaagcataacctataccccaaaacacttttggctattgttagaatcatactgagctctcctttagggaatcagttcatagcaaccagatattccctttttgttcattttctgataataaaaactgcagtttttaaggttgatgaaataacaattctgtgttaaattgtaaggacactgaaaaccactagcattaaagtaggaattgtgcaagacattggagccttgattaggtatcatgcactacagtcaataaaagaaataataggaaaacaaaatgtgcacaagatctgaggtctttcactttgctttcatacccttaatcagtttacatcttatgctttgtggggcaatcaaaccaaatgacttttacaatttcatccgttttaagtggtaatgttaaaataactcacttcggcctaaaattactataatttaacttaaaaaatcaaaatacttataatactaaatgattttaggaataagaatttgatttataacattgtcagttggacatttatctaaacattcaatatacaaagttataaagaaaaatacttctaagatatttaagaaaatgcaatataatagatcataaattaggtgcaaaaacaagacacttacagacatttccagtatatacatccattttcaaatattaccaaagtgtaaacataacttaagataatcatccttctatttctactcttgaatacagtgaaacttccagtgtgatccaggtcacttttttcccaaagataagcaaaaatggcaaaaatttacaatagcaagcactaatattaccagatttttactaatttagtgttttagtatttgaaaagttttgccaaattgtatcactcattaatagtggcttcttatttctcatgatgtgaaaaaataacaaagcaccagacatctcaagacattaatagagtatccaatacggcagtttcattatcatacccctaatgaagacagacagaaaaacataatggtgactttgataactgtaaaacacaatgttacttcatgtcaacgtttctgaggattgaatgaagggtctgtacctaatgacaaaagagctgacgcataaccgacaatactctggcaatgaaaagaaaacaggccttgggggtaaaacagaattaaaaatgtccagtttagataatttctgaattcagattttcagataaaaaaaaatcacactgttattaaaatacaagatggggctacaagggagttcccttaatctgttacactcaaaagccttgccgaggctctaaatatggaatacttctagtggaagatacgagatgctgggaacagagcagagattcccataaagtaaaagaagtaaaatactgtccaagaattcatgtggcctcaagtcttattctgaaacttgtcctttggaaagtggataacctcatttttagagtcaacgcagcaaagagaaccagatacatgagcataaaaaacaaaaaaccctcatcacatgaaatttctcaaaacgagtttattttctccttcttctgccccagtctcctgcacttgacttagtttggtgaaacatggaaatccttaatgctggcttaaaattagtataagttcctccactactaaagtatacctatgcactgccttaaacaaactttttctgtaaaattgagaatctttgaagtatggaaaggaatggttcggaaaaaccattcaaaatctctctaaaatgttaactgacagtttcctctaactggtatttctatttttcttaaaagtacatttgttaaaatactaactgagcccacctgggaaatcttgagtagaaaatatgtgatgagttcctgattgtgacataggcaggctgaagaccagccagaatgttccccaggagaggaaacctgaaaatggtggtttccttaaaaatcaatttcctgttcaatttcttgggttaggtagggggaagaggaactgtgttgtgtttgccagtgttgctgaaatgctgaacacacagcagtagcaaggtcaacagatcccaatatcccatggctgcattaatgtctgatttttttctttcttgttcagccgtatctagaggataaatattaccctcagaaccccaaggtaatacccacatccacattcttaaggcttttgcttttttcagtggttaacaaatagctataatttattttctttctttttgatgcctagcaagcagaatgacttgcttgccttttcccttagtaggtaactacagagcagagcacccatgtttccacagcggggtggtctcactgtccagactgagaattaagagcaaatctttcccacacattggagtaggtgttgcagtcctagaagttaagtactggtctcagatctcatggcagggtgctctctgccatgcagacatgtgcaattgccatttcaggatcccacactgaaaattcacggcgctccattaacaacaccagggtgtgtcatgctcttgggtggggtcacactagttctccaagtgacaaaacacacccaacacaacacaagatgttggtaagttagagaagagcaaaacacagctacttaaatgaaatctctggtttgttaatgaaccaaaggtggcttgggattattttagtagttaaaattaagagtgcattctattgcagaaaatgcagttattcaacacacagttcctcagccggcctagagccgcattacccttatcatttagtttctttttcatcctctggaggagagcagggcaggaagaggtggggacttctcttggagcatctccatcatctgtaagagggtatgtgttactgctcaccagcaccctcggctgtagttgacgtcatcttttctgtctttttggacttcctctgcatttgctcttgctcctttctccttagcttttctctttgtttttccattttctcttgggccttccgagccttctctagagacatcttcatttccttgagtttctttttgaccactgctcggtcctgggatgctgtcattccaagagccttaagtttatttccatccaactgcaggagctgttctccagtgatgttttgggcactgaattcagatacatactgctccagatttaggctcattaaccagtgagaaacctgctgcacactccattcctgaacggcccgattctgacactgactgtgtttgggagactgtccatcatcaaggatctcatctgatgacagtgctaaggactgagagagccctggtgttttaggttctgctcctaagccgctgaggtctgctgaactggtactgctgggactgaagtcatcattgaaggtaaaattattggtttcttggatccagactacagacataagttgagaatgccttccaaagattgaagaagaggagggatttgggtttctcttgtttgcttttgtaatccatgtgttttctaccttggacccctttttatctgaaattagagtctcaggagaaggctgaagggaacttgtaggcgcaggcaggttcctgaaggaataggatcctttccggctgtcattaaaccatgagaaaggcatgcaaggggaacgagtggaggtctgagctgttgaacatggcttgggtgtccagttttccagtctgcctctgaagatcctgctacctgcagaaaacctactggcttctttttctttttctttccacttctttcccttgctggaattccttcgcaaaggcgcccccagatccacaaacttccgcttaatttttcctccttgcaccgccaatgaactggatgcccttagtgatttgggatctttggcatcatctttttctcgtaatattttcttgttggtggtttggtgatggcaaggagattcttccacatcatgatcagactttgaagtagaaaacagtgaagtgtctccccacatagaggagagaggccccatttctgggtccagtggttcttcttgaaattcagctatgtggtcagacgagaagggcacattgctatccaccggggtgaggggtggaacaccagaatctgattctggagaagacgttctcaaacccttaggtggaagtaatttggtaatatgcatgtggttatagaaactgtttgatggctttctctctagactgtcctccccatctgtggaactaacactatcatacagtcttgtcctagagggtctctggcgtctgttcttcacagagagctgggctcgagttttcagtgcttttgaatccaggcgctctgtctctgggactgcttcattcaagtcttgacttaggccatcttggcaagatgtctgcttgccatccaagttctccatggtatcccctttagagacttcaccaagagatgttcttctctcaaagatgttgttattattgttaacttgagtcccattttgcttcagtagcctgaatacctcagcttccaaatctctaatccgcacttggaggccttgcacttccacaagatgagctttttccaaatcttctattttctttctttctgcttcctgtcttttgatgaaatcaagctctttttgttgaaaatccttgatcaacttctttgccttgttgtatttcttttccaaggcctgatactggctttgagtctctttgagatgctcattcactgtgtggcataatgtttgggcctcaatccagtagctttccaacttcaacattctttccttattctcttctatgttttgttggagttgggttttttctagttcccacctcactttctcattttctgctgcctgcagcttggtcttcaatttttgaatctctgcttctgtaactgcatgtttgatttgcaactctttgaacttgtgactgagcttgcttgtgtccagttctgatggggaaaacatgtcctcattctcaggcagctcaaagacttcaatggccatgtcgctgccaggaaggacaggtcctacctcatcttcttcttcatctgtggcatattctcctgtcttaagaaaatagttgttattgttattgcagttgccagacattccttgcaattcagccacagtgttcccccgagtgtcatgaaatagtgctgattgtctgagagatttattgaaatcctccatggcaacctcgtcatcgtcggcatcatactgggcatagtgctgttccagcagctctctctggcgcctctcctgttccagtgtctggcttatcaactgggcaacctcgctcacttgtcctggtttttcccgcccaataacaaatctgacgttgcccttggtgtttctgagaactgttgctgcaaaattctgtgtcacacccaccaagctgattccatccacttccacaatctggtcattgacttgtattctgccatcccgttgagcagcaccaccttctgttactgtcttgacgaatattcccagcttttcaagtccagcatctgctccaacacccattccaataatacttataccaagaccatcctcatctttctctagctccactgggaaaagttccagcttttctacacgtttttcaagttcatactcagctgaagcagccacagggtcaacttcgtcatttctcctgtcatagtcttcattggagtatgtgttgaaaaccttaataggagcactactaaacttaattttcctatttgctgggatttcttcttcttctggcaatccaacaatttccgagtactccatatcaggctgatagtaactgttctcatcactatcttcctcctcatcctgctcagtgcctgtctctccccagtctgaattatacctggatctcaccctatacacattatagtcactgtgcatgtacacatgggaaccatcaaaattatttgaatcttcaggtacttcttttccacaactggatgcagaagcatcaggagaggtgaaatcaccacctgcaagttctttcctctgttgctttgctgcctcccttccaaccaaattagcttcagcatcttctaacagttggctttgtggtgaagggatttcggactttggcattgccttactttcagcacaaggttcttcaggaccatctttgtcaatgctgtcgggagtctgttgattagatgtggagtcctcgggttccttgctctgctggatctcttcaccaggtatcgaagctagagaggtacttttagaagccacttctggtactggagttgcattactcttgtgagcatcctctgtatcaacacctcgcttgtttgaaggaggccaggaattagaatccttcaggtgaccaaatgtgtcaagatttgtaacagtaacagatggtaaattcaagggataatgcccagtcactgagtattcattgttttcagccttctcagaaatgatggcactgggagaatcagtgttctcaaatactgcactcagttgactcacagttggggagacagcctcagttcgggagctaaggctgtccaaggaatcagtactgcctctgttggacttggaacctccccattcatcctgaggttcactccctccagctttctctttctttggggaatagcggttgttctgtcctgattcatgcacacttctctcaaacatctttcgagtctcagtgaacttggaatatgaagggccatcgtacatagtgtcaaatctactaattcgttcagaaacagaagactccaacttaacaactgagccatctgttttttccagaaattctttgggcttcattcttctctgaggagatgaatgtccacctttcccccttgttttggcaatgactgcagcattctcgttgggttccatacccatctgcataaataggtttttaattctgttgacattggagccatatttcctccccctgctctgctgggagccctcaccttcttttgttttttgttccccatctgacttgggtttgtcaaaggtacttttcagtgcctgaaactcagttcgatatgcattcctgtgaggagaggcacttctgagagtggttcgttcacctgaagactcagttttcaacattttcacttcaggggtgaaaagccaatgttcataatgatcaaagaaaaaaaccaaaaaccaagatacctctcttctctaatcaccagtattgggtcaagaaaagtacctctcaaatggtatacggtgtcagtgatcgtcccaacaggtgtattaggaacttagtcacagtcaagagttacacagaatgattttttcaaagcaagactagaggttcatttgagaggcagccgattcccaagcccggttcgggacgcaatccctcggccctggggcaggaccgggagagcaggtgacgccaagcgctatggtaggaggtcgcagtctagctttgtgccaagaagcacctgaagtcctaacacattggctgcagctcccggcggctgccaggcggatcccactgtgacac

SEQ ID NO: 16999 - RNA, 8208 nt, Homo sapiens
  source 1..8208: mol_type = other RNA
taggtagtttcatgttgttgggaggtgttatctggctggagtgcctcttaattctttttaaggtaatttaattatttcttgccaattgttctttcttgaatgaatgattacatccttaacagaaaacctgggtgtataaataatacagctgaaagaaacagaagtgtacaccttccaacaacatacactcccaaccacttgtgttgtttttggcaacaaccaaaatgccattgcttgcacaaaaagtaaataaatgatcatatgatggcaacattcatcataagagagccagtaggcagtgactgtaagcatcacagccaccaattatgtcattttagaattgtgagcaaattcacaagaacacacagtgcaatttttagctgcatacatttcttctgagctccaactcagcaatatgcaatcttgacatcaaagcattagccaaatatttgaggaaattttcttactaaaataccaagtatctgataaatcaattttaccaaaatatataaacatatagaaggataagtgcatttagtagaaatacttacaataaaaaaatctcttaaaatctatgagccattcaatgtatacacaacgcaagaagtggcaataaggctatgattacagctccaggtcctgactgacctcgccaagttccatacacaatatattttttaatgccatgtgattgcagtgtgtgtgcgtgtgtaaggtgggagtgatattcacacatatgtagttctgaacatctacacaaacggcatgcacattgttgagaagttatctgttctcttattgcatacatcttactcactgttgaatccctagcagttttggggttgggttagggtcaagcataggaaatcatcatatttctttccttctccactcttgaggatctggaatcaggtcacagactgtgctgggtccacacgcttacatatgtgaaccttcaagtaactaccattccctcaataggcccacatagacaccacggacaagcaaataaggaccctctgtctaccataaatagaacttgatgctttcactttccaggagaagctgattctgtcggctttctctttgcccctccaacttcttagttgggcctattctatgctgctacttcaagttactcaaatgtgttttgtctggtgttatttttttctccagtgttttggaccaagactagatttcctgagactttaaatacgcaagacaaatgcaaacaaaatctgccaacatacccaggctgcttttcaggagtgaatcactgaagcgcatttggatttcctataacactactttcttttgggaatgtacagccctcccccagctccccatcccccatcataatgtaaaccattctaatagaaaatatggatgttttggctgggggtggtggcacatgcctgtagtcccagctacttgggaagctgaagcaggaggaccacttgagcccaggagtttgaggctgcagtaagacatgatggcaccactgcagtccagtctgggtgacagatgacagaaaaaaaaaaaaaaaaagaaaagaaaagaaaatatggacattttatttctggactttatccttaaatgcttagctttagaatagtgcacaggtacatccttaataaaaagtaaatttgaaaagacaggaaaggactgtgcttttctcttccattttaccttttcattctgagaccactaaggtctttgcattaagtaggtgacgtgaaccctagtgaccactgcccaccaaaatgcccctcatctccagctctgtcaggagtacctttagttactcaaatggaaatatctcagtgtaatgatggggctacaacatatccaaagtatagatggttctctcagggctgctggggcagcttcctttagaatcctctagaacactattgttaaacactggatctcctcttgaagtttagtctgcataacctttaacacttaaacatgaatcagagtatctatataaatgcaaattttcatttcccttttataaaatgcaattttcaagcacatgctaattctggtgcacaatgaacccagacaaatttgtcttcagcacaaactctaacggccgaggtgctagatcaaaccacctgtgaccatttttgtagcttgggactgggatattttaagatttcaggctagtgatgattacagggtcacagatagtggcaaaggtaaatctggttcctcattttccctcttgccactttgtttccaacaacaatggagcaaaaggtgacagtcccattttgtgccagttgaaagctgagtttggctttagtacctatcatactgcaatcatgaactgctgtgggttaaaaaaagcttgtgatgttgagggtgtgaaatcaattgtcaatcccagctaaaggatgatagccacagaacagctttattgtcatgaaactaaagggggacttcatcaggagtgttagaatggatgaaatgaggtttcttccctaacttaacattctgcagaaaattcctgattcaggtaaaaaaagaatgagattagtattacataaactgtgagttacttgaagggagatggtcttaaacaaagtaatctgttataaaactaacatcctttaatgggaaaccctgacccagatacagctcatacaatgctttctgtctgcagcttggcctcctcaccacacattccctcccaacaaagcataacctataccccaaaacacttttggctattgttagaatcatactgagctctcctttagggaatcagttcatagcaaccagatattccctttttgttcattttctgataataaaaactgcagtttttaaggttgatgaaataacaattctgtgttaaattgtaaggacactgaaaaccactagcattaaagtaggaattgtgcaagacattggagccttgattaggtatcatgcactacagtcaataaaagaaataataggaaaacaaaatgtgcacaagatctgaggtctttcactttgctttcatacccttaatcagtttacatcttatgctttgtggggcaatcaaaccaaatgacttttacaatttcatccgttttaagtggtaatgttaaaataactcacttcggcctaaaattactataatttaacttaaaaaatcaaaatacttataatactaaatgattttaggaataagaatttgatttataacattgtcagttggacatttatctaaacattcaatatacaaagttataaagaaaaatacttctaagatatttaagaaaatgcaatataatagatcataaattaggtgcaaaaacaagacacttacagacatttccagtatatacatccattttcaaatattaccaaagtgtaaacataacttaagataatcatccttctatttctactcttgaatacagtgaaacttccagtgtgatccaggtcacttttttcccaaagataagcaaaaatggcaaaaatttacaatagcaagcactaatattaccagatttttactaatttagtgttttagtatttgaaaagttttgccaaattgtatcactcattaatagtggcttcttatttctcatgatgtgaaaaaataacaaagcaccagacatctcaagacattaatagagtatccaatacggcagtttcattatcatacccctaatgaagacagacagaaaaacataatggtgactttgataactgtaaaacacaatgttacttcatgtcaacgtttctgaggattgaatgaagggtctgtacctaatgacaaaagagctgacgcataaccgacaatactctggcaatgaaaagaaaacaggccttgggggtaaaacagaattaaaaatgtccagtttagataatttctgaattcagattttcagataaaaaaaaatcacactgttattaaaatacaagatggggctacaagggagttcccttaatctgttacactcaaaagccttgccgaggctctaaatatggaatacttctagtggaagatacgagatgctgggaacagagcagagattcccataaagtaaaagaagtaaaatactgtccaagaattcatgtggcctcaagtcttattctgaaacttgtcctttggaaagtggataacctcatttttagagtcaacgcagcaaagagaaccagatacatgagcataaaaaacaaaaaaccctcatcacatgaaatttctcaaaacgagtttattttctccttcttctgccccagtctcctgcacttgacttagtttggtgaaacatggaaatccttaatgctggcttaaaattagtataagttcctccactactaaagtatacctatgcactgccttaaacaaactttttctgtaaaattgagaatctttgaagtatggaaaggaatggttcggaaaaaccattcaaaatctctctaaaatgttaactgacagtttcctctaactggtatttctatttttcttaaaagtacatttgttaaaatactaactgagcccacctgggaaatcttgagtagaaaatatgtgatgagttcctgattgtgacataggcaggctgaagaccagccagaatgttccccaggagaggaaacctgaaaatggtggtttccttaaaaatcaatttcctgttcaatttcttgggttaggtagggggaagaggaactgtgttgtgtttgccagtgttgctgaaatgctgaacacacagcagtagcaaggtcaacagatcccaatatcccatggctgcattaatgtctgatttttttctttcttgttcagccgtatctagaggataaatattaccctcagaaccccaaggtaatacccacatccacattcttaaggcttttgcttttttcagtggttaacaaatagctataatttattttctttctttttgatgcctagcaagcagaatgacttgcttgccttttcccttagtaggtaactacagagcagagcacccatgtttccacagcggggtggtctcactgtccagactgagaattaagagcaaatctttcccacacattggagtaggtgttgcagtcctagaagttaagtactggtctcagatctcatggcagggtgctctctgccatgcagacatgtgcaattgccatttcaggatcccacactgaaaattcacggcgctccattaacaacaccagggtgtgtcatgctcttgggtggggtcacactagttctccaagtgacaaaacacacccaacacaacacaagatgttggtaagttagagaagagcaaaacacagctacttaaatgaaatctctggtttgttaatgaaccaaaggtggcttgggattattttagtagttaaaattaagagtgcattctattgcagaaaatgcagttattcaacacacagttcctcagccggcctagagccgcattacccttatcatttagtttctttttcatcctctggaggagagcagggcaggaagaggtggggacttctcttggagcatctccatcatctgtaagagggtatgtgttactgctcaccagcaccctcggctgtagttgacgtcatcttttctgtctttttggacttcctctgcatttgctcttgctcctttctccttagcttttctctttgtttttccattttctcttgggccttccgagccttctctagagacatcttcatttccttgagtttctttttgaccactgctcggtcctgggatgctgtcattccaagagccttaagtttatttccatccaactgcaggagctgttctccagtgatgttttgggcactgaattcagatacatactgctccagatttaggctcattaaccagtgagaaacctgctgcacactccattcctgaacggcccgattctgacactgactgtgtttgggagactgtccatcatcaaggatctcatctgatgacagtgctaaggactgagagagccctggtgttttaggttctgctcctaagccgctgaggtctgctgaactggtactgctgggactgaagtcatcattgaaggtaaaattattggtttcttggatccagactacagacataagttgagaatgccttccaaagattgaagaagaggagggatttgggtttctcttgtttgcttttgtaatccatgtgttttctaccttggacccctttttatctgaaattagagtctcaggagaaggctgaagggaacttgtaggcgcaggcaggttcctgaaggaataggatcctttccggctgtcattaaaccatgagaaaggcatgcaaggggaacgagtggaggtctgagctgttgaacatggcttgggtgtccagttttccagtctgcctctgaagatcctgctacctgcagaaaacctactggcttctttttctttttctttccacttctttcccttgctggaattccttcgcaaaggcgcccccagatccacaaacttccgcttaatttttcctccttgcaccgccaatgaactggatgcccttagtgatttgggatctttggcatcatctttttctcgtaatattttcttgttggtggtttggtgatggcaaggagattcttccacatcatgatcagactttgaagtagaaaacagtgaagtgtctccccacatagaggagagaggccccatttctgggtccagtggttcttcttgaaattcagctatgtggtcagacgagaagggcacattgctatccaccggggtgaggggtggaacaccagaatctgattctggagaagacgttctcaaacccttaggtggaagtaatttggtaatatgcatgtggttatagaaactgtttgatggctttctctctagactgtcctccccatctgtggaactaacactatcatacagtcttgtcctagagggtctctggcgtctgttcttcacagagagctgggctcgagttttcagtgcttttgaatccaggcgctctgtctctgggactgcttcattcaagtcttgacttaggccatcttggcaagatgtctgcttgccatccaagttctccatggtatcccctttagagacttcaccaagagatgttcttctctcaaagatgttgttattattgttaacttgagtcccattttgcttcagtagcctgaatacctcagcttccaaatctctaatccgcacttggaggccttgcacttccacaagatgagctttttccaaatcttctattttctttctttctgcttcctgtcttttgatgaaatcaagctctttttgttgaaaatccttgatcaacttctttgccttgttgtatttcttttccaaggcctgatactggctttgagtctctttgagatgctcattcactgtgtggcataatgtttgggcctcaatccagtagctttccaacttcaacattctttccttattctcttctatgttttgttggagttgggttttttctagttcccacctcactttctcattttctgctgcctgcagcttggtcttcaatttttgaatctctgcttctgtaactgcatgtttgatttgcaactctttgaacttgtgactgagcttgcttgtgtccagttctgatggggaaaacatgtcctcattctcaggcagctcaaagacttcaatggccatgtcgctgccaggaaggacaggtcctacctcatcttcttcttcatctgtggcatattctcctgtcttaagaaaatagttgttattgttattgcagttgccagacattccttgcaattcagccacagtgttcccccgagtgtcatgaaatagtgctgattgtctgagagatttattgaaatcctccatggcaacctcgtcatcgtcggcatcatactgggcatagtgctgttccagcagctctctctggcgcctctcctgttccagtgtctggcttatcaactgggcaacctcgctcacttgtcctggtttttcccgcccaataacaaatctgacgttgcccttggtgtttctgagaactgttgctgcaaaattctgtgtcacacccaccaagctgattccatccacttccacaatctggtcattgacttgtattcttactggataagatagtctagggcactggttcccaaactgcctcactgccatcccgttgagcagcaccaccttctgttactgtcttgacgaatattcccagcttttcaagtccagcatctgctccaacacccattccaataatac

SEQ ID NO: 17000 - RNA, 9973 nt, Homo sapiens
  source 1..9973: mol_type = other RNA
taggtagtttcatgttgttgggaggtgttatctggctggagtgcctcttaattctttttaaggtaatttaattatttcttgccaattgttctttcttgaatgaatgattacatccttaacagaaaacctgggtgtataaataatacagctgaaagaaacagaagtgtacaccttccaacaacatacactcccaaccacttgtgttgtttttggcaacaaccaaaatgccattgcttgcacaaaaagtaaataaatgatcatatgatggcaacattcatcataagagagccagtaggcagtgactgtaagcatcacagccaccaattatgtcattttagaattgtgagcaaattcacaagaacacacagtgcaatttttagctgcatacatttcttctgagctccaactcagcaatatgcaatcttgacatcaaagcattagccaaatatttgaggaaattttcttactaaaataccaagtatctgataaatcaattttaccaaaatatataaacatatagaaggataagtgcatttagtagaaatacttacaataaaaaaatctcttaaaatctatgagccattcaatgtatacacaacgcaagaagtggcaataaggctatgattacagctccaggtcctgactgacctcgccaagttccatacacaatatattttttaatgccatgtgattgcagtgtgtgtgcgtgtgtaaggtgggagtgatattcacacatatgtagttctgaacatctacacaaacggcatgcacattgttgagaagttatctgttctcttattgcatacatcttactcactgttgaatccctagcagttttggggttgggttagggtcaagcataggaaatcatcatatttctttccttctccactcttgaggatctggaatcaggtcacagactgtgctgggtccacacgcttacatatgtgaaccttcaagtaactaccattccctcaataggcccacatagacaccacggacaagcaaataaggaccctctgtctaccataaatagaacttgatgctttcactttccaggagaagctgattctgtcggctttctctttgcccctccaacttcttagttgggcctattctatgctgctacttcaagttactcaaatgtgttttgtctggtgttatttttttctccagtgttttggaccaagactagatttcctgagactttaaatacgcaagacaaatgcaaacaaaatctgccaacatacccaggctgcttttcaggagtgaatcactgaagcgcatttggatttcctataacactactttcttttgggaatgtacagccctcccccagctccccatcccccatcataatgtaaaccattctaatagaaaatatggatgttttggctgggggtggtggcacatgcctgtagtcccagctacttgggaagctgaagcaggaggaccacttgagcccaggagtttgaggctgcagtaagacatgatggcaccactgcagtccagtctgggtgacagatgacagaaaaaaaaaaaaaaaaagaaaagaaaagaaaatatggacattttatttctggactttatccttaaatgcttagctttagaatagtgcacaggtacatccttaataaaaagtaaatttgaaaagacaggaaaggactgtgcttttctcttccattttaccttttcattctgagaccactaaggtctttgcattaagtaggtgacgtgaaccctagtgaccactgcccaccaaaatgcccctcatctccagctctgtcaggagtacctttagttactcaaatggaaatatctcagtgtaatgatggggctacaacatatccaaagtatagatggttctctcagggctgctggggcagcttcctttagaatcctctagaacactattgttaaacactggatctcctcttgaagtttagtctgcataacctttaacacttaaacatgaatcagagtatctatataaatgcaaattttcatttcccttttataaaatgcaattttcaagcacatgctaattctggtgcacaatgaacccagacaaatttgtcttcagcacaaactctaacggccgaggtgctagatcaaaccacctgtgaccatttttgtagcttgggactgggatattttaagatttcaggctagtgatgattacagggtcacagatagtggcaaaggtaaatctggttcctcattttccctcttgccactttgtttccaacaacaatggagcaaaaggtgacagtcccattttgtgccagttgaaagctgagtttggctttagtacctatcatactgcaatcatgaactgctgtgggttaaaaaaagcttgtgatgttgagggtgtgaaatcaattgtcaatcccagctaaaggatgatagccacagaacagctttattgtcatgaaactaaagggggacttcatcaggagtgttagaatggatgaaatgaggtttcttccctaacttaacattctgcagaaaattcctgattcaggtaaaaaaagaatgagattagtattacataaactgtgagttacttgaagggagatggtcttaaacaaagtaatctgttataaaactaacatcctttaatgggaaaccctgacccagatacagctcatacaatgctttctgtctgcagcttggcctcctcaccacacattccctcccaacaaagcataacctataccccaaaacacttttggctattgttagaatcatactgagctctcctttagggaatcagttcatagcaaccagatattccctttttgttcattttctgataataaaaactgcagtttttaaggttgatgaaataacaattctgtgttaaattgtaaggacactgaaaaccactagcattaaagtaggaattgtgcaagacattggagccttgattaggtatcatgcactacagtcaataaaagaaataataggaaaacaaaatgtgcacaagatctgaggtctttcactttgctttcatacccttaatcagtttacatcttatgctttgtggggcaatcaaaccaaatgacttttacaatttcatccgttttaagtggtaatgttaaaataactcacttcggcctaaaattactataatttaacttaaaaaatcaaaatacttataatactaaatgattttaggaataagaatttgatttataacattgtcagttggacatttatctaaacattcaatatacaaagttataaagaaaaatacttctaagatatttaagaaaatgcaatataatagatcataaattaggtgcaaaaacaagacacttacagacatttccagtatatacatccattttcaaatattaccaaagtgtaaacataacttaagataatcatccttctatttctactcttgaatacagtgaaacttccagtgtgatccaggtcacttttttcccaaagataagcaaaaatggcaaaaatttacaatagcaagcactaatattaccagatttttactaatttagtgttttagtatttgaaaagttttgccaaattgtatcactcattaatagtggcttcttatttctcatgatgtgaaaaaataacaaagcaccagacatctcaagacattaatagagtatccaatacggcagtttcattatcatacccctaatgaagacagacagaaaaacataatggtgactttgataactgtaaaacacaatgttacttcatgtcaacgtttctgaggattgaatgaagggtctgtacctaatgacaaaagagctgacgcataaccgacaatactctggcaatgaaaagaaaacaggccttgggggtaaaacagaattaaaaatgtccagtttagataatttctgaattcagattttcagataaaaaaaaatcacactgttattaaaatacaagatggggctacaagggagttcccttaatctgttacactcaaaagccttgccgaggctctaaatatggaatacttctagtggaagatacgagatgctgggaacagagcagagattcccataaagtaaaagaagtaaaatactgtccaagaattcatgtggcctcaagtcttattctgaaacttgtcctttggaaagtggataacctcatttttagagtcaacgcagcaaagagaaccagatacatgagcataaaaaacaaaaaaccctcatcacatgaaatttctcaaaacgagtttattttctccttcttctgccccagtctcctgcacttgacttagtttggtgaaacatggaaatccttaatgctggcttaaaattagtataagttcctccactactaaagtatacctatgcactgccttaaacaaactttttctgtaaaattgagaatctttgaagtatggaaaggaatggttcggaaaaaccattcaaaatctctctaaaatgttaactgacagtttcctctaactggtatttctatttttcttaaaagtacatttgttaaaatactaactgagcccacctgggaaatcttgagtagaaaatatgtgatgagttcctgattgtgacataggcaggctgaagaccagccagaatgttccccaggagaggaaacctgaaaatggtggtttccttaaaaatcaatttcctgttcaatttcttgggttaggtagggggaagaggaactgtgttgtgtttgccagtgttgctgaaatgctgaacacacagcagtagcaaggtcaacagatcccaatatcccatggctgcattaatgtctgatttttttctttcttgttcagccgtatctagaggataaatattaccctcagaaccccaaggtaatacccacatccacattcttaaggcttttgcttttttcagtggttaacaaatagctataatttattttctttctttttgatgcctagcaagcagaatgacttgcttgccttttcccttagtaggtaactacagagcagagcacccatgtttccacagcggggtggtctcactgtccagactgagaattaagagcaaatctttcccacacattggagtaggtgttgcagtcctagaagttaagtactggtctcagatctcatggcagggtgctctctgccatgcagacatgtgcaattgccatttcaggatcccacactgaaaattcacggcgctccattaacaacaccagggtgtgtcatgctcttgggtggggtcacactagttctccaagtgacaaaacacacccaacacaacacaagatgttggtaagttagagaagagcaaaacacagctacttaaatgaaatctctggtttgttaatgaaccaaaggtggcttgggattattttagtagttaaaattaagagtgcattctattgcagaaaatgcagttattcaacacacagttcctcagccggcctagagccgcattacccttatcatttagtttctttttcatcctctggaggagagcagggcaggaagaggtggggacttctcttggagcatctccatcatctgtaagagggtatgtgttactgctcaccagcaccctcggctgtagttgacgtcatcttttctgtctttttggacttcctctgcatttgctcttgctcctttctccttagcttttctctttgtttttccattttctcttgggccttccgagccttctctagagacatcttcatttccttgagtttctttttgaccactgctcggtcctgggatgctgtcattccaagagccttaagtttatttccatccaactgcaggagctgttctccagtgatgttttgggcactgaattcagatacatactgctccagatttaggctcattaaccagtgagaaacctgctgcacactccattcctgaacggcccgattctgacactgactgtgtttgggagactgtccatcatcaaggatctcatctgatgacagtgctaaggactgagagagccctggtgttttaggttctgctcctaagccgctgaggtctgctgaactggtactgctgggactgaagtcatcattgaaggtaaaattattggtttcttggatccagactacagacataagttgagaatgccttccaaagattgaagaagaggagggatttgggtttctcttgtttgcttttgtaatccatgtgttttctaccttggacccctttttatctgaaattagagtctcaggagaaggctgaagggaacttgtaggcgcaggcaggttcctgaaggaataggatcctttccggctgtcattaaaccatgagaaaggcatgcaaggggaacgagtggaggtctgagctgttgaacatggcttgggtgtccagttttccagtctgcctctgaagatcctgctacctgcagaaaacctactggcttctttttctttttctttccacttctttcccttgctggaattccttcgcaaaggcgcccccagatccacaaacttccgcttaatttttcctccttgcaccgccaatgaactggatgcccttagtgatttgggatctttggcatcatctttttctcgtaatattttcttgttggtggtttggtgatggcaaggagattcttccacatcatgatcagactttgaagtagaaaacagtgaagtgtctccccacatagaggagagaggccccatttctgggtccagtggttcttcttgaaattcagctatgtggtcagacgagaagggcacattgctatccaccggggtgaggggtggaacaccagaatctgattctggagaagacgttctcaaacccttaggtggaagtaatttggtaatatgcatgtggttatagaaactgtttgatggctttctctctagactgtcctccccatctgtggaactaacactatcatacagtcttgtcctagagggtctctggcgtctgttcttcacagagagctgggctcgagttttcagtgcttttgaatccaggcgctctgtctctgggactgcttcattcaagtcttgacttaggccatcttggcaagatgtctgcttgccatccaagttctccatggtatcccctttagagacttcaccaagagatgttcttctctcaaagatgttgttattattgttaacttgagtcccattttgcttcagtagcctgaatacctcagcttccaaatctctaatccgcacttggaggccttgcacttccacaagatgagctttttccaaatcttctattttctttctttctgcttcctgtcttttgatgaaatcaagctctttttgttgaaaatccttgatcaacttctttgccttgttgtatttcttttccaaggcctgatactggctttgagtctctttgagatgctcattcactgtgtggcataatgtttgggcctcaatccagtagctttccaacttcaacattctttccttattctcttctatgttttgttggagttgggttttttctagttcccacctcactttctcattttctgctgcctgcagcttggtcttcaatttttgaatctctgcttctgtaactgcatgtttgatttgcaactctttgaacttgtgactgagcttgcttgtgtccagttctgatggggaaaacatgtcctcattctcaggcagctcaaagacttcaatggccatgtcgctgccaggaaggacaggtcctacctcatcttcttcttcatctgtggcatattctcctgtcttaagaaaatagttgttattgttattgcagttgccagacattccttgcaattcagccacagtgttctcgtcatcgtcggcatcatactgggcatagtgctgttccagcagctctctctggcgcctctcctgttccagtgtctggcttatcaactgggcaacctcgctcacttgtcctggtttttcccgcccaataacaaatctgacgttgcccttggtgtttctgagaactgttgctgcaaaattctgtgtcacacccaccaagctgattccatccacttccacaatctggtcattgacttgtattctgccatcccgttgagcagcaccaccttctgttactgtcttgacgaatattcccagcttttcaagtccagcatctgctccaacacccattccaataatacttataccaagaccatcctcatctttctctagctccactgggaaaagttccagcttttctacacgtttttcaagttcatactcagctgaagcagccacagggtcaacttcgtcatttctcctgtcatagtcttcattggagtatgtgttgaaaaccttaataggagcactactaaacttaattttcctatttgctgggatttcttcttcttctggcaatccaacaatttccgagtactccatatcaggctgatagtaactgttctcatcactatcttcctcctcatcctgctcagtgcctgtctctccccagtctgaattatacctggatctcaccctatacacattatagtcactgtgcatgtacacatgggaaccatcaaaattatttgaatcttcaggtacttcttttccacaactggatgcagaagcatcaggagaggtgaaatcaccacctgcaagttctttcctctgttgctttgctgcctcccttccaaccaaattagcttcagcatcttctaacagttggctttgtggtgaagggatttcggactttggcattgccttactttcagcacaaggttcttcaggaccatctttgtcaatgctgtcgggagtctgttgattagatgtggagtcctcgggttccttgctctgctggatctcttcaccaggtatcgaagctagagaggtacttttagaagccacttctggtactggagttgcattactcttgtgagcatcctctgtatcaacacctcgcttgtttgaaggaggccaggaattagaatccttcaggtgaccaaatgtgtcaagatttgtaacagtaacagatggtaaattcaagggataatgcccagtcactgagtattcattgttttcagccttctcagaaatgatggcactgggagaatcagtgttctcaaatactgcactcagttgactcacagttggggagacagcctcagttcgggagctaaggctgtccaaggaatcagtactgcctctgttggacttggaacctccccattcatcctgaggttcactccctccagctttctctttctttggggaatagcggttgttctgtcctgattcatgcacacttctctcaaacatctttcgagtctcagtgaacttggaatatgaagggccatcgtacatagtgtcaaatctactaattcgttcagaaacagaagactccaacttaacaactgagccatctgttttttccagaaattctttgggcttcattcttctctgaggagatgaatgtccacctttcccccttgttttggcaatgactgcagcattctcgttgggttccatacccatctgcataaataggtttttaattctgttgacattggagccatatttcctccccctgctctgctgggagccctcaccttcttttgttttttgttccccatctgacttgggtttgtcaaaggtacttttcagtgcctgaaactcagttcgatatgcattcctgtgaggagaggcacttctgagagtggttcgttcacctgaagactcagttttcaacattttcacttcaggggtgaaaagccaatgttcataatgatcaaagaaaaaaaccaaaaaccaagatacctctcttctctaatcaccagtattgggtcaagaaaagtacctctcaaatggtatacggtgtcagtgatcgtcccaacaggtgtattaggaacttagtcacagtcaagagttacacagaatgattttttcaaagcaagactagaggttcatctcggctgatgggattaactctagggccgcagagagagggagcccggcagcaaaatcccgggagagggagagagagggagcctctggcggccaaggaagggcgaaaagc

SEQ ID NO: 17001 - RNA, 12813 nt, Homo sapiens
  source 1..12813: mol_type = other RNA
taggtagtttcatgttgttgggaggtgttatctggctggagtgcctcttaattctttttaaggtaatttaattatttcttgccaattgttctttcttgaatgaatgattacatccttaacagaaaacctgggtgtataaataatacagctgaaagaaacagaagtgtacaccttccaacaacatacactcccaaccacttgtgttgtttttggcaacaaccaaaatgccattgcttgcacaaaaagtaaataaatgatcatatgatggcaacattcatcataagagagccagtaggcagtgactgtaagcatcacagccaccaattatgtcattttagaattgtgagcaaattcacaagaacacacagtgcaatttttagctgcatacatttcttctgagctccaactcagcaatatgcaatcttgacatcaaagcattagccaaatatttgaggaaattttcttactaaaataccaagtatctgataaatcaattttaccaaaatatataaacatatagaaggataagtgcatttagtagaaatacttacaataaaaaaatctcttaaaatctatgagccattcaatgtatacacaacgcaagaagtggcaataaggctatgattacagctccaggtcctgactgacctcgccaagttccatacacaatatattttttaatgccatgtgattgcagtgtgtgtgcgtgtgtaaggtgggagtgatattcacacatatgtagttctgaacatctacacaaacggcatgcacattgttgagaagttatctgttctcttattgcatacatcttactcactgttgaatccctagcagttttggggttgggttagggtcaagcataggaaatcatcatatttctttccttctccactcttgaggatctggaatcaggtcacagactgtgctgggtccacacgcttacatatgtgaaccttcaagtaactaccattccctcaataggcccacatagacaccacggacaagcaaataaggaccctctgtctaccataaatagaacttgatgctttcactttccaggagaagctgattctgtcggctttctctttgcccctccaacttcttagttgggcctattctatgctgctacttcaagttactcaaatgtgttttgtctggtgttatttttttctccagtgttttggaccaagactagatttcctgagactttaaatacgcaagacaaatgcaaacaaaatctgccaacatacccaggctgcttttcaggagtgaatcactgaagcgcatttggatttcctataacactactttcttttgggaatgtacagccctcccccagctccccatcccccatcataatgtaaaccattctaatagaaaatatggatgttttggctgggggtggtggcacatgcctgtagtcccagctacttgggaagctgaagcaggaggaccacttgagcccaggagtttgaggctgcagtaagacatgatggcaccactgcagtccagtctgggtgacagatgacagaaaaaaaaaaaaaaaaagaaaagaaaagaaaatatggacattttatttctggactttatccttaaatgcttagctttagaatagtgcacaggtacatccttaataaaaagtaaatttgaaaagacaggaaaggactgtgcttttctcttccattttaccttttcattctgagaccactaaggtctttgcattaagtaggtgacgtgaaccctagtgaccactgcccaccaaaatgcccctcatctccagctctgtcaggagtacctttagttactcaaatggaaatatctcagtgtaatgatggggctacaacatatccaaagtatagatggttctctcagggctgctggggcagcttcctttagaatcctctagaacactattgttaaacactggatctcctcttgaagtttagtctgcataacctttaacacttaaacatgaatcagagtatctatataaatgcaaattttcatttcccttttataaaatgcaattttcaagcacatgctaattctggtgcacaatgaacccagacaaatttgtcttcagcacaaactctaacggccgaggtgctagatcaaaccacctgtgaccatttttgtagcttgggactgggatattttaagatttcaggctagtgatgattacagggtcacagatagtggcaaaggtaaatctggttcctcattttccctcttgccactttgtttccaacaacaatggagcaaaaggtgacagtcccattttgtgccagttgaaagctgagtttggctttagtacctatcatactgcaatcatgaactgctgtgggttaaaaaaagcttgtgatgttgagggtgtgaaatcaattgtcaatcccagctaaaggatgatagccacagaacagctttattgtcatgaaactaaagggggacttcatcaggagtgttagaatggatgaaatgaggtttcttccctaacttaacattctgcagaaaattcctgattcaggtaaaaaaagaatgagattagtattacataaactgtgagttacttgaagggagatggtcttaaacaaagtaatctgttataaaactaacatcctttaatgggaaaccctgacccagatacagctcatacaatgctttctgtctgcagcttggcctcctcaccacacattccctcccaacaaagcataacctataccccaaaacacttttggctattgttagaatcatactgagctctcctttagggaatcagttcatagcaaccagatattccctttttgttcattttctgataataaaaactgcagtttttaaggttgatgaaataacaattctgtgttaaattgtaaggacactgaaaaccactagcattaaagtaggaattgtgcaagacattggagccttgattaggtatcatgcactacagtcaataaaagaaataataggaaaacaaaatgtgcacaagatctgaggtctttcactttgctttcatacccttaatcagtttacatcttatgctttgtggggcaatcaaaccaaatgacttttacaatttcatccgttttaagtggtaatgttaaaataactcacttcggcctaaaattactataatttaacttaaaaaatcaaaatacttataatactaaatgattttaggaataagaatttgatttataacattgtcagttggacatttatctaaacattcaatatacaaagttataaagaaaaatacttctaagatatttaagaaaatgcaatataatagatcataaattaggtgcaaaaacaagacacttacagacatttccagtatatacatccattttcaaatattaccaaagtgtaaacataacttaagataatcatccttctatttctactcttgaatacagtgaaacttccagtgtgatccaggtcacttttttcccaaagataagcaaaaatggcaaaaatttacaatagcaagcactaatattaccagatttttactaatttagtgttttagtatttgaaaagttttgccaaattgtatcactcattaatagtggcttcttatttctcatgatgtgaaaaaataacaaagcaccagacatctcaagacattaatagagtatccaatacggcagtttcattatcatacccctaatgaagacagacagaaaaacataatggtgactttgataactgtaaaacacaatgttacttcatgtcaacgtttctgaggattgaatgaagggtctgtacctaatgacaaaagagctgacgcataaccgacaatactctggcaatgaaaagaaaacaggccttgggggtaaaacagaattaaaaatgtccagtttagataatttctgaattcagattttcagataaaaaaaaatcacactgttattaaaatacaagatggggctacaagggagttcccttaatctgttacactcaaaagccttgccgaggctctaaatatggaatacttctagtggaagatacgagatgctgggaacagagcagagattcccataaagtaaaagaagtaaaatactgtccaagaattcatgtggcctcaagtcttattctgaaacttgtcctttggaaagtggataacctcatttttagagtcaacgcagcaaagagaaccagatacatgagcataaaaaacaaaaaaccctcatcacatgaaatttctcaaaacgagtttattttctccttcttctgccccagtctcctgcacttgacttagtttggtgaaacatggaaatccttaatgctggcttaaaattagtataagttcctccactactaaagtatacctatgcactgccttaaacaaactttttctgtaaaattgagaatctttgaagtatggaaaggaatggttcggaaaaaccattcaaaatctctctaaaatgttaactgacagtttcctctaactggtatttctatttttcttaaaagtacatttgttaaaatactaactgagcccacctgggaaatcttgagtagaaaatatgtgatgagttcctgattgtgacataggcaggctgaagaccagccagaatgttccccaggagaggaaacctgaaaatggtggtttccttaaaaatcaatttcctgttcaatttcttgggttaggtagggggaagaggaactgtgttgtgtttgccagtgttgctgaaatgctgaacacacagcagtagcaaggtcaacagatcccaatatcccatggctgcattaatgtctgatttttttctttcttgttcagccgtatctagaggataaatattaccctcagaaccccaaggtaatacccacatccacattcttaaggcttttgcttttttcagtggttaacaaatagctataatttattttctttctttttgatgcctagcaagcagaatgacttgcttgccttttcccttagtaggtaactacagagcagagcacccatgtttccacagcggggtggtctcactgtccagactgagaattaagagcaaatctttcccacacattggagtaggtgttgcagtcctagaagttaagtactggtctcagatctcatggcagggtgctctctgccatgcagacatgtgcaattgccatttcaggatcccacactgaaaattcacggcgctccattaacaacaccagggtgtgtcatgctcttgggtggggtcacactagttctccaagtgacaaaacacacccaacacaacacaagatgttggtaagttagagaagagcaaaacacagctacttaaatgaaatctctggtttgttaatgaaccaaaggtggcttgggattattttagtagttaaaattaagagtgcattctattgcagaaaatgcagttattcaacacacagttcctcagccggcctagagccgcattacccttatcatttagtttctttttcatcctctggaggagagcagggcaggaagaggtggggacttctcttggagcatctccatcatctgtaagagggtatgtgttactgctcaccagcaccctcggctgtagttgacgtcatcttttctgtctttttggacttcctctgcatttgctcttgctcctttctccttagcttttctctttgtttttccattttctcttgggccttccgagccttctctagagacatcttcatttccttgagtttctttttgaccactgctcggtcctgggatgctgtcattccaagagccttaagtttatttccatccaactgcaggagctgttctccagtgatgttttgggcactgaattcagatacatactgctccagatttaggctcattaaccagtgagaaacctgctgcacactccattcctgaacggcccgattctgacactgactgtgtttgggagactgtccatcatcaaggatctcatctgatgacagtgctaaggactgagagagccctggtgttttaggttctgctcctaagccgctgaggtctgctgaactggtactgctgggactgaagtcatcattgaaggtaaaattattggtttcttggatccagactacagacataagttgagaatgccttccaaagattgaagaagaggagggatttgggtttctcttgtttgcttttgtaatccatgtgttttctaccttggacccctttttatctgaaattagagtctcaggagaaggctgaagggaacttgtaggcgcaggcaggttcctgaaggaataggatcctttccggctgtcattaaaccatgagaaaggcatgcaaggggaacgagtggaggtctgagctgttgaacatggcttgggtgtccagttttccagtctgcctctgaagatcctgctacctgcagaaaacctactggcttctttttctttttctttccacttctttcccttgctggaattccttcgcaaaggcgcccccagatccacaaacttccgcttaatttttcctccttgcaccgccaatgaactggatgcccttagtgatttgggatctttggcatcatctttttctcgtaatattttcttgttggtggtttggtgatggcaaggagattcttccacatcatgatcagactttgaagtagaaaacagtgaagtgtctccccacatagaggagagaggccccatttctgggtccagtggttcttcttgaaattcagctatgtggtcagacgagaagggcacattgctatccaccggggtgaggggtggaacaccagaatctgattctggagaagacgttctcaaacccttaggtggaagtaatttggtaatatgcatgtggttatagaaactgtttgatggctttctctctagactgtcctccccatctgtggaactaacactatcatacagtcttgtcctagagggtctctggcgtctgttcttcacagagagctgggctcgagttttcagtgcttttgaatccaggcgctctgtctctgggactgcttcattcaagtcttgacttaggccatcttggcaagatgtctgcttgccatccaagttctccatggtatcccctttagagacttcaccaagagatgttcttctctcaaagatgttgttattattgttaacttgagtcccattttgcttcagtagcctgaatacctcagcttccaaatctctaatccgcacttggaggccttgcacttccacaagatgagctttttccaaatcttctattttctttctttctgcttcctgtcttttgatgaaatcaagctctttttgttgaaaatccttgatcaacttctttgccttgttgtatttcttttccaaggcctgatactggctttgagtctctttgagatgctcattcactgtgtggcataatgtttgggcctcaatccagtagctttccaacttcaacattctttccttattctcttctatgttttgttggagttgggttttttctagttcccacctcactttctcattttctgctgcctgcagcttggtcttcaatttttgaatctctgcttctgtaactgcatgtttgatttgcaactggacgtgtgaagatttattccaaatctgcaagaaaggtggcgctatggtcctgtgagttgcaagcacattctgatcagcagctccaattcttcctgacctggtcactctggccatcttgctggtgtggctattgctccttgcaccctcaccggctcctaggggcttctatgcttgaacagtttctagagtaggaccctatgtggaaatgttatttttataagacacaaaatctggctcttttagtttcttaccacagcacaagtggtacaattcttacttacctgcctttagcagatgctcagagtattagtgcacctggcaaggaacctaatcacaagttttctcaatgactagattggaagaaggtgtaaagacacaacagtgctgctcagaaatccctgcaattcctaccccttcactgatgaggtctatactcatcctaagtcctagtctggatggatcttttggaatcctgacacaccaggctagccagtcagataggcttgaatgcccagtggacgctccaactgtaggctcttctgaactcattttagacacgggaagactaaagattggagaagacagccaacctggtcttttcctcacagtgaatcaccattaaaaccagaactaaaacctggatcttctcgttctgatccattgccactttccttagaaaataaggatgaattcaataggcattcgttgaagagttgctatgtgcaggatgctgtaaaaatgactttttctccctctaataaatattagggctaatctcccccaccagtataaactaataacgtaaaaaagggcaaaagtacttagacattagacacattatttatatataaatctacaaaaacaaataatgtatatgcacacaaacatacatggctatgtgctaaggcatccagaaaatccatacacttaggtgattttataggatttgcaatcgctattgacaagatatacttcttgttctttcaaccatgtgccaagcatgaagagtagttaacttagactgcttgaattcatctctggtctaccatgtactctatggagcattagaaaattacttaacctctttcatttcactttccttgcctgtaaaattcagttccttataagtcataaccttccttattggatgattaagtgataaaacccatataaagcacttagcacagtggctagcatatagtatgtcctcaataaactcagctaggaccaagaaagaatgatctgaataactcaaatatgattaccccagcttcacctctcagttaaatgtgctaactgctgtaaaatgtcacacctgaagtaaaatgaacacctctgattcaatttaaagagaaacaagaaatcaaaagggcagattccacagtgaacactgcactatgggcaagtgacagattttattaactcctcgtagggtaaccaaatacgtggcatgcagcttgttggcattttggactttcttttctcagatcactgtgtcttctataagttgcttctctgggcctcagtttcccatatgaaaaatgctagatgtgaggaactccaagggccctttcacatacaacaggtgtgacatttatgaaacaaagaacctgaaggtagttgtcaaggttgcagagcttagaaattcttgtcctgagccaatattttccttcttgtgaataaatacactagattaatccacaaattgtgggacaaacccaggtaaaactgtgaaacagcccatgttgatctattctaccctttccatctcaccaaaaatggataacaggagggaactgaactaattagcagtgaggtgagaacaactgcgcaaagtttggagtgttactaagtatagctaaattctttacatataggaaagcagaatgaattgtgtaaattcacattattcagaatggacaagattttcttagtacacatgaggcctaaaattaaaaatatgcgattattttaattctgtatgtacattaagagaatttctacaaatccatcacttttgacaagaaaagcatcaaaatacactaactgaaccctttttgttttatatagtatggacctgtgtctagtgagcttaccttggaaggctattaggtgccaaagccaggttttagaaatcccagcccatggttctttccactaatactaaatttcttacatttgtaggcccctttatttttaatcatctccctttatcattgcaaatgactgggggaggcagggcaggtgttgtgaacctcatggttcagatgaggaaagaggctcagggaagtcacacaccttttcaagttcccactagaaacaggtgatggagcggaaacaaaaccagatttgactcttcctacctctgttcctcccttaaccatgtatctaactgaaccagttgctttgggatatatttttcatttaatcttcccccaaaccccaagccatatgtcatcatcataacctctcagatgagaagttattactccaactggaaaccatggatcacttctggtagtctctgagcattctgacagtgaatgcaaaatggtgctcaatcagctgctgttattattaatgaagcttagaaagcagacctccacctcccttaataatcaattggcctttagtgactgagactacgtgctaggtactatgctaatcactgaggatacatgaacatgacatagaatctactttcaagatacttcagggagattaataaaaacaccttgtaagaattctccagatcaccctgtgagaaaggtcagaggcaacctgctgctggatggcttgtttagtcttttgttcctatagccagatcagatgtcatgtgtctttggcctgtttgtccagacgtggaccctactttccaagcaaagtgagcaagatggacccaagttatctccatttcatgaggaaaagaaaattgcttttcacaggggtgaaggacctcgacaaatgaagcatagttggtaaaaggttgagttttcttattctagagcagttccctttccacatgtttaagagatttatgtcaagaatcaataaccttttcaaagtacaggtccaagagtttgcaagaatggtcaggcacgctgactgcagggatagaaggttaacagggctggttaatagaaatagagcctgagatgcctgttggagtttttgggcttcagagaagctaggtttggagaaaagagttgggattaggagggcataaataaaaagaaaaggttaaggactgcaggtaaaagtcttttaacttacaagaccatcattttcatctcttcagtcatctttaatatgaaagccatagatatgcacctcaggatttcagcacaaataaacatacacattcctatgagaacaggagctttcatttaacattctgaaggtgtacctgctgtgtataatttttttttcaaaaagatgaatacagaacatgcactcatattaccggatcgatataatccaaatataactgtgctagaaatagaaacatcctttacacagaaacttaaatagtgagactgaacttttgccctctctctacttatcctgtgagagcatggaaacatttttctttaaaaagtgaaaaatatctttgcaggaaatgttttaagagagctctagttctagaaatattacaatcagataagggcaacattttctgctgttgctttacaaaagcaaatcaataactaatatttgcatagaactttataaagtgctttctagattgggatctaaatttttagttatctttgtgagtatttgagtgatgtatgtcttacctacaacaatatagcttcacaaaagaaatcaaagctgtttttaactacattttggtgttaagatgaagctttgccatatttctttgtaatttctgctgaaaagtttacatatggtatctatccagtattaacgaaagtgttttacttagggaatcatgtatgcaaaatgaactaaaactggctgactgaacaatatcacaatctaatctgaatggtaacactaatggcagcatatgtagcattgggtgagattctctaacaaggtcactccctaagtaggtactcataaacttgttattaatgatgctgctgctggatgtagttgatggcctgtaattacagctcttttttaaataagtaactgtttgctattaagtaggcagcaatttatagcttccctacatggtagtggaaacttccataaagataacttaatgttattatcccatgcattttataacttttctagattctttttcatagaattaaataaataaaataaaccaacttttagactccattttttcttcaagagaaatgtcgaatttttttaattgttgcaattgctgtgactcctgaggaggaatggcaagggagaaattggacagtcactttaaatggtacctggctaacagttcctgagccagcctcgccgtaccttccattaaactgccagtgtaatcacattaaaaacaaaaaaactcacaatcaaaaatgaacaccacaactaaaaacaacagttcatagaatataaaagagtcatgaagttgaattaagaaaaatctatccaagatcccctctgacatcagggagacactttgtaccaccctcactgatggcttgagatccattctgtcccaagcaaaaagtggacaacccctactgtcttgcccaggaatggggcctcaaactgggctctctaacttcctcagtattccatatttgctcagaaagcaactgttagggggaaatgcaggaaggtggctgatgcatggcacactgcatactttcagctgcagacctatatagacatgggtggcttcagtaagtgccttgctagcagtgaagactggaaattaccttttttatctctttaacttagagaactgtgtggcaatacttgggagtatctgaccttagtacagagaattgccctagatgtcagactgctagaaaatagcaactgggctggacacgaggcacctaaatatccctcctgatctaagtctagaaatgagattcataatcaaaaagtgaataattactgactaacctactaaaagatttttgtttcatttcaagataaggaaagaaaaaacaggtcaccttaggtctattaacaaatactgcaaatcaaggtaaagaaaatatcaacttgaacacacaaataagtaaacttgtgaaaatgatgtatcccataagtaaaaaaatattttaagatcactttttgaaattctaggctgaagagaaagta

SEQ ID NO: 17002 - RNA, 9914 nt, Homo sapiens
  source 1..9914: mol_type = other RNA
taggtagtttcatgttgttgggaggtgttatctggctggagtgcctcttaattctttttaaggtaatttaattatttcttgccaattgttctttcttgaatgaatgattacatccttaacagaaaacctgggtgtataaataatacagctgaaagaaacagaagtgtacaccttccaacaacatacactcccaaccacttgtgttgtttttggcaacaaccaaaatgccattgcttgcacaaaaagtaaataaatgatcatatgatggcaacattcatcataagagagccagtaggcagtgactgtaagcatcacagccaccaattatgtcattttagaattgtgagcaaattcacaagaacacacagtgcaatttttagctgcatacatttcttctgagctccaactcagcaatatgcaatcttgacatcaaagcattagccaaatatttgaggaaattttcttactaaaataccaagtatctgataaatcaattttaccaaaatatataaacatatagaaggataagtgcatttagtagaaatacttacaataaaaaaatctcttaaaatctatgagccattcaatgtatacacaacgcaagaagtggcaataaggctatgattacagctccaggtcctgactgacctcgccaagttccatacacaatatattttttaatgccatgtgattgcagtgtgtgtgcgtgtgtaaggtgggagtgatattcacacatatgtagttctgaacatctacacaaacggcatgcacattgttgagaagttatctgttctcttattgcatacatcttactcactgttgaatccctagcagttttggggttgggttagggtcaagcataggaaatcatcatatttctttccttctccactcttgaggatctggaatcaggtcacagactgtgctgggtccacacgcttacatatgtgaaccttcaagtaactaccattccctcaataggcccacatagacaccacggacaagcaaataaggaccctctgtctaccataaatagaacttgatgctttcactttccaggagaagctgattctgtcggctttctctttgcccctccaacttcttagttgggcctattctatgctgctacttcaagttactcaaatgtgttttgtctggtgttatttttttctccagtgttttggaccaagactagatttcctgagactttaaatacgcaagacaaatgcaaacaaaatctgccaacatacccaggctgcttttcaggagtgaatcactgaagcgcatttggatttcctataacactactttcttttgggaatgtacagccctcccccagctccccatcccccatcataatgtaaaccattctaatagaaaatatggatgttttggctgggggtggtggcacatgcctgtagtcccagctacttgggaagctgaagcaggaggaccacttgagcccaggagtttgaggctgcagtaagacatgatggcaccactgcagtccagtctgggtgacagatgacagaaaaaaaaaaaaaaaaagaaaagaaaagaaaatatggacattttatttctggactttatccttaaatgcttagctttagaatagtgcacaggtacatccttaataaaaagtaaatttgaaaagacaggaaaggactgtgcttttctcttccattttaccttttcattctgagaccactaaggtctttgcattaagtaggtgacgtgaaccctagtgaccactgcccaccaaaatgcccctcatctccagctctgtcaggagtacctttagttactcaaatggaaatatctcagtgtaatgatggggctacaacatatccaaagtatagatggttctctcagggctgctggggcagcttcctttagaatcctctagaacactattgttaaacactggatctcctcttgaagtttagtctgcataacctttaacacttaaacatgaatcagagtatctatataaatgcaaattttcatttcccttttataaaatgcaattttcaagcacatgctaattctggtgcacaatgaacccagacaaatttgtcttcagcacaaactctaacggccgaggtgctagatcaaaccacctgtgaccatttttgtagcttgggactgggatattttaagatttcaggctagtgatgattacagggtcacagatagtggcaaaggtaaatctggttcctcattttccctcttgccactttgtttccaacaacaatggagcaaaaggtgacagtcccattttgtgccagttgaaagctgagtttggctttagtacctatcatactgcaatcatgaactgctgtgggttaaaaaaagcttgtgatgttgagggtgtgaaatcaattgtcaatcccagctaaaggatgatagccacagaacagctttattgtcatgaaactaaagggggacttcatcaggagtgttagaatggatgaaatgaggtttcttccctaacttaacattctgcagaaaattcctgattcaggtaaaaaaagaatgagattagtattacataaactgtgagttacttgaagggagatggtcttaaacaaagtaatctgttataaaactaacatcctttaatgggaaaccctgacccagatacagctcatacaatgctttctgtctgcagcttggcctcctcaccacacattccctcccaacaaagcataacctataccccaaaacacttttggctattgttagaatcatactgagctctcctttagggaatcagttcatagcaaccagatattccctttttgttcattttctgataataaaaactgcagtttttaaggttgatgaaataacaattctgtgttaaattgtaaggacactgaaaaccactagcattaaagtaggaattgtgcaagacattggagccttgattaggtatcatgcactacagtcaataaaagaaataataggaaaacaaaatgtgcacaagatctgaggtctttcactttgctttcatacccttaatcagtttacatcttatgctttgtggggcaatcaaaccaaatgacttttacaatttcatccgttttaagtggtaatgttaaaataactcacttcggcctaaaattactataatttaacttaaaaaatcaaaatacttataatactaaatgattttaggaataagaatttgatttataacattgtcagttggacatttatctaaacattcaatatacaaagttataaagaaaaatacttctaagatatttaagaaaatgcaatataatagatcataaattaggtgcaaaaacaagacacttacagacatttccagtatatacatccattttcaaatattaccaaagtgtaaacataacttaagataatcatccttctatttctactcttgaatacagtgaaacttccagtgtgatccaggtcacttttttcccaaagataagcaaaaatggcaaaaatttacaatagcaagcactaatattaccagatttttactaatttagtgttttagtatttgaaaagttttgccaaattgtatcactcattaatagtggcttcttatttctcatgatgtgaaaaaataacaaagcaccagacatctcaagacattaatagagtatccaatacggcagtttcattatcatacccctaatgaagacagacagaaaaacataatggtgactttgataactgtaaaacacaatgttacttcatgtcaacgtttctgaggattgaatgaagggtctgtacctaatgacaaaagagctgacgcataaccgacaatactctggcaatgaaaagaaaacaggccttgggggtaaaacagaattaaaaatgtccagtttagataatttctgaattcagattttcagataaaaaaaaatcacactgttattaaaatacaagatggggctacaagggagttcccttaatctgttacactcaaaagccttgccgaggctctaaatatggaatacttctagtggaagatacgagatgctgggaacagagcagagattcccataaagtaaaagaagtaaaatactgtccaagaattcatgtggcctcaagtcttattctgaaacttgtcctttggaaagtggataacctcatttttagagtcaacgcagcaaagagaaccagatacatgagcataaaaaacaaaaaaccctcatcacatgaaatttctcaaaacgagtttattttctccttcttctgccccagtctcctgcacttgacttagtttggtgaaacatggaaatccttaatgctggcttaaaattagtataagttcctccactactaaagtatacctatgcactgccttaaacaaactttttctgtaaaattgagaatctttgaagtatggaaaggaatggttcggaaaaaccattcaaaatctctctaaaatgttaactgacagtttcctctaactggtatttctatttttcttaaaagtacatttgttaaaatactaactgagcccacctgggaaatcttgagtagaaaatatgtgatgagttcctgattgtgacataggcaggctgaagaccagccagaatgttccccaggagaggaaacctgaaaatggtggtttccttaaaaatcaatttcctgttcaatttcttgggttaggtagggggaagaggaactgtgttgtgtttgccagtgttgctgaaatgctgaacacacagcagtagcaaggtcaacagatcccaatatcccatggctgcattaatgtctgatttttttctttcttgttcagccgtatctagaggataaatattaccctcagaaccccaaggtaatacccacatccacattcttaaggcttttgcttttttcagtggttaacaaatagctataatttattttctttctttttgatgcctagcaagcagaatgacttgcttgccttttcccttagtaggtaactacagagcagagcacccatgtttccacagcggggtggtctcactgtccagactgagaattaagagcaaatctttcccacacattggagtaggtgttgcagtcctagaagttaagtactggtctcagatctcatggcagggtgctctctgccatgcagacatgtgcaattgccatttcaggatcccacactgaaaattcacggcgctccattaacaacaccagggtgtgtcatgctcttgggtggggtcacactagttctccaagtgacaaaacacacccaacacaacacaagatgttggtaagttagagaagagcaaaacacagctacttaaatgaaatctctggtttgttaatgaaccaaaggtggcttgggattattttagtagttaaaattaagagtgcattctattgcagaaaatgcagttattcaacacacagttcctcagccggcctagagccgcattacccttatcatttagtttctttttcatcctctggaggagagcagggcaggaagaggtggggacttctcttggagcatctccatcatctgtaagagggtatgtgttactgctcaccagcaccctcggctgtagttgacgtcatcttttctgtctttttggacttcctctgcatttgctcttgctcctttctccttagcttttctctttgtttttccattttctcttgggccttccgagccttctctagagacatcttcatttccttgagtttctttttgaccactgctcggtcctgggatgctgtcattccaagagccttaagtttatttccatccaactgcaggagctgttctccagtgatgttttgggcactgaattcagatacatactgctccagatttaggctcattaaccagtgagaaacctgctgcacactccattcctgaacggcccgattctgacactgactgtgtttgggagactgtccatcatcaaggatctcatctgatgacagtgctaaggactgagagagccctggtgttttaggttctgctcctaagccgctgaggtctgctgaactggtactgctgggactgaagtcatcattgaaggtaaaattattggtttcttggatccagactacagacataagttgagaatgccttccaaagattgaagaagaggagggatttgggtttctcttgtttgcttttgtaatccatgtgttttctaccttggacccctttttatctgaaattagagtctcaggagaaggctgaagggaacttgtaggcgcaggcaggttcctgaaggaataggatcctttccggctgtcattaaaccatgagaaaggcatgcaaggggaacgagtggaggtctgagctgttgaacatggcttgggtgtccagttttccagtctgcctctgaagatcctgctacctgcagaaaacctactggcttctttttctttttctttccacttctttcccttgctggaattccttcgcaaaggcgcccccagatccacaaacttccgcttaatttttcctccttgcaccgccaatgaactggatgcccttagtgatttgggatctttggcatcatctttttctcgtaatattttcttgttggtggtttggtgatggcaaggagattcttccacatcatgatcagactttgaagtagaaaacagtgaagtgtctccccacatagaggagagaggccccatttctgggtccagtggttcttcttgaaattcagctatgtggtcagacgagaagggcacattgctatccaccggggtgaggggtggaacaccagaatctgattctggagaagacgttctcaaacccttaggtggaagtaatttggtaatatgcatgtggttatagaaactgtttgatggctttctctctagactgtcctccccatctgtggaactaacactatcatacagtcttgtcctagagggtctctggcgtctgttcttcacagagagctgggctcgagttttcagtgcttttgaatccaggcgctctgtctctgggactgcttcattcaagtcttgacttaggccatcttggcaagatgtctgcttgccatccaagttctccatggtatcccctttagagacttcaccaagagatgttcttctctcaaagatgttgttattattgttaacttgagtcccattttgcttcagtagcctgaatacctcagcttccaaatctctaatccgcacttggaggccttgcacttccacaagatgagctttttccaaatcttctattttctttctttctgcttcctgtcttttgatgaaatcaagctctttttgttgaaaatccttgatcaacttctttgccttgttgtatttcttttccaaggcctgatactggctttgagtctctttgagatgctcattcactgtgtggcataatgtttgggcctcaatccagtagctttccaacttcaacattctttccttattctcttctatgttttgttggagttgggttttttctagttcccacctcactttctcattttctgctgcctgcagcttggtcttcaatttttgaatctctgcttctgtaactgcatgtttgatttgcaactggacgtgtgaagatttattccaaatctgcaagaaaggtggcgctatggtcctgtgagttgcaagcacattctgatcagcagctccactctttgaacttgtgactgagcttgcttgtgtccagttctgatggggaaaacatgtcctcattctcaggcagctcaaagacttcaatggccatgtcgctgccaggaaggacaggtcctacctcatcttcttcttcatctgtggcatattctcctgtctcgtcatcgtcggcatcatactgggcatagtgctgttccagcagctctctctggcgcctctcctgttccagtgtctggcttatcaactgggcaacctcgctcacttgtcctggtttttcccgcccaataacaaatctgacgttgcccttggtgtttctgagaactgttgctgcaaaattctgtgtcacacccaccaagctgattccatccacttccacaatctggtcattgacttgtattctgccatcccgttgagcagcaccaccttctgttactgtcttgacgaatattcccagcttttcaagtccagcatctgctccaacacccattccaataatacttataccaagaccatcctcatctttctctagctccactgggaaaagttccagcttttctacacgtttttcaagttcatactcagctgaagcagccacagggtcaacttcgtcatttctcctgtcatagtcttcattggagtatgtgttgaaaaccttaataggagcactactaaacttaattttcctatttgctgggatttcttcttcttctggcaatccaacaatttccgagtactccatatcaggctgatagtaactgttctcatcactatcttcctcctcatcctgctcagtgcctgtctctccccagtctgaattatacctggatctcaccctatacacattatagtcactgtgcatgtacacatgggaaccatcaaaattatttgaatcttcaggtacttcttttccacaactggatgcagaagcatcaggagaggtgaaatcaccacctgcaagttctttcctctgttgctttgctgcctcccttccaaccaaattagcttcagcatcttctaacagttggctttgtggtgaagggatttcggactttggcattgccttactttcagcacaaggttcttcaggaccatctttgtcaatgctgtcgggagtctgttgattagatgtggagtcctcgggttccttgctctgctggatctcttcaccaggtatcgaagctagagaggtacttttagaagccacttctggtactggagttgcattactcttgtgagcatcctctgtatcaacacctcgcttgtttgaaggaggccaggaattagaatccttcaggtgaccaaatgtgtcaagatttgtaacagtaacagatggtaaattcaagggataatgcccagtcactgagtattcattgttttcagccttctcagaaatgatggcactgggagaatcagtgttctcaaatactgcactcagttgactcacagttggggagacagcctcagttcgggagctaaggctgtccaaggaatcagtactgcctctgttggacttggaacctccccattcatcctgaggttcactccctccagctttctctttctttggggaatagcggttgttctgtcctgattcatgcacacttctctcaaacatctttcgagtctcagtgaacttggaatatgaagggccatcgtacatagtgtcaaatctactaattcgttcagaaacagaagactccaacttaacaactgagccatctgttttttccagaaattctttgggcttcattcttctctgaggagatgaatgtccacctttcccccttgttttggcaatgactgcagcattctcgttgggttccatacccatctgcataaataggtttttaattctgttgacattggagccatatttcctccccctgctctgctgggagccctcaccttcttttgttttttgttccccatctgacttgggtttgtcaaaggtacttttcagtgcctgaaactcagttcgatatgcattcctgtgaggagaggcacttctgagagtggttcgttcacctgaagactcagttttcaacattttcacttcaggggtgaaaagccaatgttcataatgatcaaagaaaaaaaccaaaaaccaagatacctctcttctctaatcaccagtattgggtcaagaaaagtacctctcaaatggtatacggtgtcagtgatcgtcccaacaggtgtattaggaacttagtcacagtcaagagttacacagaatgattttttcaaagcaagactagaggttcatctcggctgatgggattaactctagggcc

SEQ ID NO: 17003 - RNA, 9939 nt, Homo sapiens
  source 1..9939: mol_type = other RNA
taggtagtttcatgttgttgggaggtgttatctggctggagtgcctcttaattctttttaaggtaatttaattatttcttgccaattgttctttcttgaatgaatgattacatccttaacagaaaacctgggtgtataaataatacagctgaaagaaacagaagtgtacaccttccaacaacatacactcccaaccacttgtgttgtttttggcaacaaccaaaatgccattgcttgcacaaaaagtaaataaatgatcatatgatggcaacattcatcataagagagccagtaggcagtgactgtaagcatcacagccaccaattatgtcattttagaattgtgagcaaattcacaagaacacacagtgcaatttttagctgcatacatttcttctgagctccaactcagcaatatgcaatcttgacatcaaagcattagccaaatatttgaggaaattttcttactaaaataccaagtatctgataaatcaattttaccaaaatatataaacatatagaaggataagtgcatttagtagaaatacttacaataaaaaaatctcttaaaatctatgagccattcaatgtatacacaacgcaagaagtggcaataaggctatgattacagctccaggtcctgactgacctcgccaagttccatacacaatatattttttaatgccatgtgattgcagtgtgtgtgcgtgtgtaaggtgggagtgatattcacacatatgtagttctgaacatctacacaaacggcatgcacattgttgagaagttatctgttctcttattgcatacatcttactcactgttgaatccctagcagttttggggttgggttagggtcaagcataggaaatcatcatatttctttccttctccactcttgaggatctggaatcaggtcacagactgtgctgggtccacacgcttacatatgtgaaccttcaagtaactaccattccctcaataggcccacatagacaccacggacaagcaaataaggaccctctgtctaccataaatagaacttgatgctttcactttccaggagaagctgattctgtcggctttctctttgcccctccaacttcttagttgggcctattctatgctgctacttcaagttactcaaatgtgttttgtctggtgttatttttttctccagtgttttggaccaagactagatttcctgagactttaaatacgcaagacaaatgcaaacaaaatctgccaacatacccaggctgcttttcaggagtgaatcactgaagcgcatttggatttcctataacactactttcttttgggaatgtacagccctcccccagctccccatcccccatcataatgtaaaccattctaatagaaaatatggatgttttggctgggggtggtggcacatgcctgtagtcccagctacttgggaagctgaagcaggaggaccacttgagcccaggagtttgaggctgcagtaagacatgatggcaccactgcagtccagtctgggtgacagatgacagaaaaaaaaaaaaaaaaagaaaagaaaagaaaatatggacattttatttctggactttatccttaaatgcttagctttagaatagtgcacaggtacatccttaataaaaagtaaatttgaaaagacaggaaaggactgtgcttttctcttccattttaccttttcattctgagaccactaaggtctttgcattaagtaggtgacgtgaaccctagtgaccactgcccaccaaaatgcccctcatctccagctctgtcaggagtacctttagttactcaaatggaaatatctcagtgtaatgatggggctacaacatatccaaagtatagatggttctctcagggctgctggggcagcttcctttagaatcctctagaacactattgttaaacactggatctcctcttgaagtttagtctgcataacctttaacacttaaacatgaatcagagtatctatataaatgcaaattttcatttcccttttataaaatgcaattttcaagcacatgctaattctggtgcacaatgaacccagacaaatttgtcttcagcacaaactctaacggccgaggtgctagatcaaaccacctgtgaccatttttgtagcttgggactgggatattttaagatttcaggctagtgatgattacagggtcacagatagtggcaaaggtaaatctggttcctcattttccctcttgccactttgtttccaacaacaatggagcaaaaggtgacagtcccattttgtgccagttgaaagctgagtttggctttagtacctatcatactgcaatcatgaactgctgtgggttaaaaaaagcttgtgatgttgagggtgtgaaatcaattgtcaatcccagctaaaggatgatagccacagaacagctttattgtcatgaaactaaagggggacttcatcaggagtgttagaatggatgaaatgaggtttcttccctaacttaacattctgcagaaaattcctgattcaggtaaaaaaagaatgagattagtattacataaactgtgagttacttgaagggagatggtcttaaacaaagtaatctgttataaaactaacatcctttaatgggaaaccctgacccagatacagctcatacaatgctttctgtctgcagcttggcctcctcaccacacattccctcccaacaaagcataacctataccccaaaacacttttggctattgttagaatcatactgagctctcctttagggaatcagttcatagcaaccagatattccctttttgttcattttctgataataaaaactgcagtttttaaggttgatgaaataacaattctgtgttaaattgtaaggacactgaaaaccactagcattaaagtaggaattgtgcaagacattggagccttgattaggtatcatgcactacagtcaataaaagaaataataggaaaacaaaatgtgcacaagatctgaggtctttcactttgctttcatacccttaatcagtttacatcttatgctttgtggggcaatcaaaccaaatgacttttacaatttcatccgttttaagtggtaatgttaaaataactcacttcggcctaaaattactataatttaacttaaaaaatcaaaatacttataatactaaatgattttaggaataagaatttgatttataacattgtcagttggacatttatctaaacattcaatatacaaagttataaagaaaaatacttctaagatatttaagaaaatgcaatataatagatcataaattaggtgcaaaaacaagacacttacagacatttccagtatatacatccattttcaaatattaccaaagtgtaaacataacttaagataatcatccttctatttctactcttgaatacagtgaaacttccagtgtgatccaggtcacttttttcccaaagataagcaaaaatggcaaaaatttacaatagcaagcactaatattaccagatttttactaatttagtgttttagtatttgaaaagttttgccaaattgtatcactcattaatagtggcttcttatttctcatgatgtgaaaaaataacaaagcaccagacatctcaagacattaatagagtatccaatacggcagtttcattatcatacccctaatgaagacagacagaaaaacataatggtgactttgataactgtaaaacacaatgttacttcatgtcaacgtttctgaggattgaatgaagggtctgtacctaatgacaaaagagctgacgcataaccgacaatactctggcaatgaaaagaaaacaggccttgggggtaaaacagaattaaaaatgtccagtttagataatttctgaattcagattttcagataaaaaaaaatcacactgttattaaaatacaagatggggctacaagggagttcccttaatctgttacactcaaaagccttgccgaggctctaaatatggaatacttctagtggaagatacgagatgctgggaacagagcagagattcccataaagtaaaagaagtaaaatactgtccaagaattcatgtggcctcaagtcttattctgaaacttgtcctttggaaagtggataacctcatttttagagtcaacgcagcaaagagaaccagatacatgagcataaaaaacaaaaaaccctcatcacatgaaatttctcaaaacgagtttattttctccttcttctgccccagtctcctgcacttgacttagtttggtgaaacatggaaatccttaatgctggcttaaaattagtataagttcctccactactaaagtatacctatgcactgccttaaacaaactttttctgtaaaattgagaatctttgaagtatggaaaggaatggttcggaaaaaccattcaaaatctctctaaaatgttaactgacagtttcctctaactggtatttctatttttcttaaaagtacatttgttaaaatactaactgagcccacctgggaaatcttgagtagaaaatatgtgatgagttcctgattgtgacataggcaggctgaagaccagccagaatgttccccaggagaggaaacctgaaaatggtggtttccttaaaaatcaatttcctgttcaatttcttgggttaggtagggggaagaggaactgtgttgtgtttgccagtgttgctgaaatgctgaacacacagcagtagcaaggtcaacagatcccaatatcccatggctgcattaatgtctgatttttttctttcttgttcagccgtatctagaggataaatattaccctcagaaccccaaggtaatacccacatccacattcttaaggcttttgcttttttcagtggttaacaaatagctataatttattttctttctttttgatgcctagcaagcagaatgacttgcttgccttttcccttagtaggtaactacagagcagagcacccatgtttccacagcggggtggtctcactgtccagactgagaattaagagcaaatctttcccacacattggagtaggtgttgcagtcctagaagttaagtactggtctcagatctcatggcagggtgctctctgccatgcagacatgtgcaattgccatttcaggatcccacactgaaaattcacggcgctccattaacaacaccagggtgtgtcatgctcttgggtggggtcacactagttctccaagtgacaaaacacacccaacacaacacaagatgttggtaagttagagaagagcaaaacacagctacttaaatgaaatctctggtttgttaatgaaccaaaggtggcttgggattattttagtagttaaaattaagagtgcattctattgcagaaaatgcagttattcaacacacagttcctcagccggcctagagccgcattacccttatcatttagtttctttttcatcctctggaggagagcagggcaggaagaggtggggacttctcttggagcatctccatcatctgtaagagggtatgtgttactgctcaccagcaccctcggctgtagttgacgtcatcttttctgtctttttggacttcctctgcatttgctcttgctcctttctccttagcttttctctttgtttttccattttctcttgggccttccgagccttctctagagacatcttcatttccttgagtttctttttgaccactgctcggtcctgggatgctgtcattccaagagccttaagtttatttccatccaactgcaggagctgttctccagtgatgttttgggcactgaattcagatacatactgctccagatttaggctcattaaccagtgagaaacctgctgcacactccattcctgaacggcccgattctgacactgactgtgtttgggagactgtccatcatcaaggatctcatctgatgacagtgctaaggactgagagagccctggtgttttaggttctgctcctaagccgctgaggtctgctgaactggtactgctgggactgaagtcatcattgaaggtaaaattattggtttcttggatccagactacagacataagttgagaatgccttccaaagattgaagaagaggagggatttgggtttctcttgtttgcttttgtaatccatgtgttttctaccttggacccctttttatctgaaattagagtctcaggagaaggctgaagggaacttgtaggcgcaggcaggttcctgaaggaataggatcctttccggctgtcattaaaccatgagaaaggcatgcaaggggaacgagtggaggtctgagctgttgaacatggcttgggtgtccagttttccagtctgcctctgaagatcctgctacctgcagaaaacctactggcttctttttctttttctttccacttctttcccttgctggaattccttcgcaaaggcgcccccagatccacaaacttccgcttaatttttcctccttgcaccgccaatgaactggatgcccttagtgatttgggatctttggcatcatctttttctcgtaatattttcttgttggtggtttggtgatggcaaggagattcttccacatcatgatcagactttgaagtagaaaacagtgaagtgtctccccacatagaggagagaggccccatttctgggtccagtggttcttcttgaaattcagctatgtggtcagacgagaagggcacattgctatccaccggggtgaggggtggaacaccagaatctgattctggagaagacgttctcaaaccctttctctctagactgtcctccccatctgtggaactaacactatcatacagtcttgtcctagagggtctctggcgtctgttcttcacagagagctgggctcgagttttcagtgcttttgaatccaggcgctctgtctctgggactgcttcattcaagtcttgacttaggccatcttggcaagatgtctgcttgccatccaagttctccatggtatcccctttagagacttcaccaagagatgttcttctctcaaagatgttgttattattgttaacttgagtcccattttgcttcagtagcctgaatacctcagcttccaaatctctaatccgcacttggaggccttgcacttccacaagatgagctttttccaaatcttctattttctttctttctgcttcctgtcttttgatgaaatcaagctctttttgttgaaaatccttgatcaacttctttgccttgttgtatttcttttccaaggcctgatactggctttgagtctctttgagatgctcattcactgtgtggcataatgtttgggcctcaatccagtagctttccaacttcaacattctttccttattctcttctatgttttgttggagttgggttttttctagttcccacctcactttctcattttctgctgcctgcagcttggtcttcaatttttgaatctctgcttctgtaactgcatgtttgatttgcaactctttgaacttgtgactgagcttgcttgtgtccagttctgatggggaaaacatgtcctcattctcaggcagctcaaagacttcaatggccatgtcgctgccaggaaggacaggtcctacctcatcttcttcttcatctgtggcatattctcctgtcttaagaaaatagttgttattgttattgcagttgccagacattccttgcaattcagccacagtgttcccccgagtgtcatgaaatagtgctgattgtctgagagatttattgaaatcctccatggcaacctcgtcatcgtcggcatcatactgggcatagtgctgttccagcagctctctctggcgcctctcctgttccagtgtctggcttatcaactgggcaacctcgctcacttgtcctggtttttcccgcccaataacaaatctgacgttgcccttggtgtttctgagaactgttgctgcaaaattctgtgtcacacccaccaagctgattccatccacttccacaatctggtcattgacttgtattctgccatcccgttgagcagcaccaccttctgttactgtcttgacgaatattcccagcttttcaagtccagcatctgctccaacacccattccaataatacttataccaagaccatcctcatctttctctagctccactgggaaaagttccagcttttctacacgtttttcaagttcatactcagctgaagcagccacagggtcaacttcgtcatttctcctgtcatagtcttcattggagtatgtgttgaaaaccttaataggagcactactaaacttaattttcctatttgctgggatttcttcttcttctggcaatccaacaatttccgagtactccatatcaggctgatagtaactgttctcatcactatcttcctcctcatcctgctcagtgcctgtctctccccagtctgaattatacctggatctcaccctatacacattatagtcactgtgcatgtacacatgggaaccatcaaaattatttgaatcttcaggtacttcttttccacaactggatgcagaagcatcaggagaggtgaaatcaccacctgcaagttctttcctctgttgctttgctgcctcccttccaaccaaattagcttcagcatcttctaacagttggctttgtggtgaagggatttcggactttggcattgccttactttcagcacaaggttcttcaggaccatctttgtcaatgctgtcgggagtctgttgattagatgtggagtcctcgggttccttgctctgctggatctcttcaccaggtatcgaagctagagaggtacttttagaagccacttctggtactggagttgcattactcttgtgagcatcctctgtatcaacacctcgcttgtttgaaggaggccaggaattagaatccttcaggtgaccaaatgtgtcaagatttgtaacagtaacagatggtaaattcaagggataatgcccagtcactgagtattcattgttttcagccttctcagaaatgatggcactgggagaatcagtgttctcaaatactgcactcagttgactcacagttggggagacagcctcagttcgggagctaaggctgtccaaggaatcagtactgcctctgttggacttggaacctccccattcatcctgaggttcactccctccagctttctctttctttggggaatagcggttgttctgtcctgattcatgcacacttctctcaaacatctttcgagtctcagtgaacttggaatatgaagggccatcgtacatagtgtcaaatctactaattcgttcagaaacagaagactccaacttaacaactgagccatctgttttttccagaaattctttgggcttcattcttctctgaggagatgaatgtccacctttcccccttgttttggcaatgactgcagcattctcgttgggttccatacccatctgcataaataggtttttaattctgttgacattggagccatatttcctccccctgctctgctgggagccctcaccttcttttgttttttgttccccatctgacttgggtttgtcaaaggtacttttcagtgcctgaaactcagttcgatatgcattcctgtgaggagaggcacttctgagagtggttcgttcacctgaagactcagttttcaacattttcacttcaggggtgaaaagccaatgttcataatgatcaaagaaaaaaaccaaaaaccaagatacctctcttctctaatcaccagtattgggtcaagaaaagtacctctcaaatggtatacggtgtcagtgatcgtcccaacaggtgtattaggaacttagtcacagtcaagagttacacagaatgattttttcaaagcaagactagaggttcatctcggctgatgggattaactctagggccgcagagagagggagcccggcagcaaaatcccgggagag

SEQ ID NO: 17004 - RNA, 9879 nt, Homo sapiens
  source 1..9879: mol_type = other RNA
taggtagtttcatgttgttgggaggtgttatctggctggagtgcctcttaattctttttaaggtaatttaattatttcttgccaattgttctttcttgaatgaatgattacatccttaacagaaaacctgggtgtataaataatacagctgaaagaaacagaagtgtacaccttccaacaacatacactcccaaccacttgtgttgtttttggcaacaaccaaaatgccattgcttgcacaaaaagtaaataaatgatcatatgatggcaacattcatcataagagagccagtaggcagtgactgtaagcatcacagccaccaattatgtcattttagaattgtgagcaaattcacaagaacacacagtgcaatttttagctgcatacatttcttctgagctccaactcagcaatatgcaatcttgacatcaaagcattagccaaatatttgaggaaattttcttactaaaataccaagtatctgataaatcaattttaccaaaatatataaacatatagaaggataagtgcatttagtagaaatacttacaataaaaaaatctcttaaaatctatgagccattcaatgtatacacaacgcaagaagtggcaataaggctatgattacagctccaggtcctgactgacctcgccaagttccatacacaatatattttttaatgccatgtgattgcagtgtgtgtgcgtgtgtaaggtgggagtgatattcacacatatgtagttctgaacatctacacaaacggcatgcacattgttgagaagttatctgttctcttattgcatacatcttactcactgttgaatccctagcagttttggggttgggttagggtcaagcataggaaatcatcatatttctttccttctccactcttgaggatctggaatcaggtcacagactgtgctgggtccacacgcttacatatgtgaaccttcaagtaactaccattccctcaataggcccacatagacaccacggacaagcaaataaggaccctctgtctaccataaatagaacttgatgctttcactttccaggagaagctgattctgtcggctttctctttgcccctccaacttcttagttgggcctattctatgctgctacttcaagttactcaaatgtgttttgtctggtgttatttttttctccagtgttttggaccaagactagatttcctgagactttaaatacgcaagacaaatgcaaacaaaatctgccaacatacccaggctgcttttcaggagtgaatcactgaagcgcatttggatttcctataacactactttcttttgggaatgtacagccctcccccagctccccatcccccatcataatgtaaaccattctaatagaaaatatggatgttttggctgggggtggtggcacatgcctgtagtcccagctacttgggaagctgaagcaggaggaccacttgagcccaggagtttgaggctgcagtaagacatgatggcaccactgcagtccagtctgggtgacagatgacagaaaaaaaaaaaaaaaaagaaaagaaaagaaaatatggacattttatttctggactttatccttaaatgcttagctttagaatagtgcacaggtacatccttaataaaaagtaaatttgaaaagacaggaaaggactgtgcttttctcttccattttaccttttcattctgagaccactaaggtctttgcattaagtaggtgacgtgaaccctagtgaccactgcccaccaaaatgcccctcatctccagctctgtcaggagtacctttagttactcaaatggaaatatctcagtgtaatgatggggctacaacatatccaaagtatagatggttctctcagggctgctggggcagcttcctttagaatcctctagaacactattgttaaacactggatctcctcttgaagtttagtctgcataacctttaacacttaaacatgaatcagagtatctatataaatgcaaattttcatttcccttttataaaatgcaattttcaagcacatgctaattctggtgcacaatgaacccagacaaatttgtcttcagcacaaactctaacggccgaggtgctagatcaaaccacctgtgaccatttttgtagcttgggactgggatattttaagatttcaggctagtgatgattacagggtcacagatagtggcaaaggtaaatctggttcctcattttccctcttgccactttgtttccaacaacaatggagcaaaaggtgacagtcccattttgtgccagttgaaagctgagtttggctttagtacctatcatactgcaatcatgaactgctgtgggttaaaaaaagcttgtgatgttgagggtgtgaaatcaattgtcaatcccagctaaaggatgatagccacagaacagctttattgtcatgaaactaaagggggacttcatcaggagtgttagaatggatgaaatgaggtttcttccctaacttaacattctgcagaaaattcctgattcaggtaaaaaaagaatgagattagtattacataaactgtgagttacttgaagggagatggtcttaaacaaagtaatctgttataaaactaacatcctttaatgggaaaccctgacccagatacagctcatacaatgctttctgtctgcagcttggcctcctcaccacacattccctcccaacaaagcataacctataccccaaaacacttttggctattgttagaatcatactgagctctcctttagggaatcagttcatagcaaccagatattccctttttgttcattttctgataataaaaactgcagtttttaaggttgatgaaataacaattctgtgttaaattgtaaggacactgaaaaccactagcattaaagtaggaattgtgcaagacattggagccttgattaggtatcatgcactacagtcaataaaagaaataataggaaaacaaaatgtgcacaagatctgaggtctttcactttgctttcatacccttaatcagtttacatcttatgctttgtggggcaatcaaaccaaatgacttttacaatttcatccgttttaagtggtaatgttaaaataactcacttcggcctaaaattactataatttaacttaaaaaatcaaaatacttataatactaaatgattttaggaataagaatttgatttataacattgtcagttggacatttatctaaacattcaatatacaaagttataaagaaaaatacttctaagatatttaagaaaatgcaatataatagatcataaattaggtgcaaaaacaagacacttacagacatttccagtatatacatccattttcaaatattaccaaagtgtaaacataacttaagataatcatccttctatttctactcttgaatacagtgaaacttccagtgtgatccaggtcacttttttcccaaagataagcaaaaatggcaaaaatttacaatagcaagcactaatattaccagatttttactaatttagtgttttagtatttgaaaagttttgccaaattgtatcactcattaatagtggcttcttatttctcatgatgtgaaaaaataacaaagcaccagacatctcaagacattaatagagtatccaatacggcagtttcattatcatacccctaatgaagacagacagaaaaacataatggtgactttgataactgtaaaacacaatgttacttcatgtcaacgtttctgaggattgaatgaagggtctgtacctaatgacaaaagagctgacgcataaccgacaatactctggcaatgaaaagaaaacaggccttgggggtaaaacagaattaaaaatgtccagtttagataatttctgaattcagattttcagataaaaaaaaatcacactgttattaaaatacaagatggggctacaagggagttcccttaatctgttacactcaaaagccttgccgaggctctaaatatggaatacttctagtggaagatacgagatgctgggaacagagcagagattcccataaagtaaaagaagtaaaatactgtccaagaattcatgtggcctcaagtcttattctgaaacttgtcctttggaaagtggataacctcatttttagagtcaacgcagcaaagagaaccagatacatgagcataaaaaacaaaaaaccctcatcacatgaaatttctcaaaacgagtttattttctccttcttctgccccagtctcctgcacttgacttagtttggtgaaacatggaaatccttaatgctggcttaaaattagtataagttcctccactactaaagtatacctatgcactgccttaaacaaactttttctgtaaaattgagaatctttgaagtatggaaaggaatggttcggaaaaaccattcaaaatctctctaaaatgttaactgacagtttcctctaactggtatttctatttttcttaaaagtacatttgttaaaatactaactgagcccacctgggaaatcttgagtagaaaatatgtgatgagttcctgattgtgacataggcaggctgaagaccagccagaatgttccccaggagaggaaacctgaaaatggtggtttccttaaaaatcaatttcctgttcaatttcttgggttaggtagggggaagaggaactgtgttgtgtttgccagtgttgctgaaatgctgaacacacagcagtagcaaggtcaacagatcccaatatcccatggctgcattaatgtctgatttttttctttcttgttcagccgtatctagaggataaatattaccctcagaaccccaaggtaatacccacatccacattcttaaggcttttgcttttttcagtggttaacaaatagctataatttattttctttctttttgatgcctagcaagcagaatgacttgcttgccttttcccttagtaggtaactacagagcagagcacccatgtttccacagcggggtggtctcactgtccagactgagaattaagagcaaatctttcccacacattggagtaggtgttgcagtcctagaagttaagtactggtctcagatctcatggcagggtgctctctgccatgcagacatgtgcaattgccatttcaggatcccacactgaaaattcacggcgctccattaacaacaccagggtgtgtcatgctcttgggtggggtcacactagttctccaagtgacaaaacacacccaacacaacacaagatgttggtaagttagagaagagcaaaacacagctacttaaatgaaatctctggtttgttaatgaaccaaaggtggcttgggattattttagtagttaaaattaagagtgcattctattgcagaaaatgcagttattcaacacacagttcctcagccggcctagagccgcattacccttatcatttagtttctttttcatcctctggaggagagcagggcaggaagaggtggggacttctcttggagcatctccatcatctgtaagagggtatgtgttactgctcaccagcaccctcggctgtagttgacgtcatcttttctgtctttttggacttcctctgcatttgctcttgctcctttctccttagcttttctctttgtttttccattttctcttgggccttccgagccttctctagagacatcttcatttccttgagtttctttttgaccactgctcggtcctgggatgctgtcattccaagagccttaagtttatttccatccaactgcaggagctgttctccagtgatgttttgggcactgaattcagatacatactgctccagatttaggctcattaaccagtgagaaacctgctgcacactccattcctgaacggcccgattctgacactgactgtgtttgggagactgtccatcatcaaggatctcatctgatgacagtgctaaggactgagagagccctggtgttttaggttctgctcctaagccgctgaggtctgctgaactggtactgctgggactgaagtcatcattgaaggtaaaattcttggacccctttttatctgaaattagagtctcaggagaaggctgaagggaacttgtaggcgcaggcaggttcctgaaggaataggatcctttccggctgtcattaaaccatgagaaaggcatgcaaggggaacgagtggaggtctgagctgttgaacatggcttgggtgtccagttttccagtctgcctctgaagatcctgctacctgcagaaaacctactggcttctttttctttttctttccacttctttcccttgctggaattccttcgcaaaggcgcccccagatccacaaacttccgcttaatttttcctccttgcaccgccaatgaactggatgcccttagtgatttgggatctttggcatcatctttttctcgtaatattttcttgttggtggtttggtgatggcaaggagattcttccacatcatgatcagactttgaagtagaaaacagtgaagtgtctccccacatagaggagagaggccccatttctgggtccagtggttcttcttgaaattcagctatgtggtcagacgagaagggcacattgctatccaccggggtgaggggtggaacaccagaatctgattctggagaagacgttctcaaacccttaggtggaagtaatttggtaatatgcatgtggttatagaaactgtttgatggctttctctctagactgtcctccccatctgtggaactaacactatcatacagtcttgtcctagagggtctctggcgtctgttcttcacagagagctgggctcgagttttcagtgcttttgaatccaggcgctctgtctctgggactgcttcattcaagtcttgacttaggccatcttggcaagatgtctgcttgccatccaagttctccatggtatcccctttagagacttcaccaagagatgttcttctctcaaagatgttgttattattgttaacttgagtcccattttgcttcagtagcctgaatacctcagcttccaaatctctaatccgcacttggaggccttgcacttccacaagatgagctttttccaaatcttctattttctttctttctgcttcctgtcttttgatgaaatcaagctctttttgttgaaaatccttgatcaacttctttgccttgttgtatttcttttccaaggcctgatactggctttgagtctctttgagatgctcattcactgtgtggcataatgtttgggcctcaatccagtagctttccaacttcaacattctttccttattctcttctatgttttgttggagttgggttttttctagttcccacctcactttctcattttctgctgcctgcagcttggtcttcaatttttgaatctctgcttctgtaactgcatgtttgatttgcaactctttgaacttgtgactgagcttgcttgtgtccagttctgatggggaaaacatgtcctcattctcaggcagctcaaagacttcaatggccatgtcgctgccaggaaggacaggtcctacctcatcttcttcttcatctgtggcatattctcctgtcttaagaaaatagttgttattgttattgcagttgccagacattccttgcaattcagccacagtgttcccccgagtgtcatgaaatagtgctgattgtctgagagatttattgaaatcctccatggcaacctcgtcatcgtcggcatcatactgggcatagtgctgttccagcagctctctctggcgcctctcctgttccagtgtctggcttatcaactgggcaacctcgctcacttgtcctggtttttcccgcccaataacaaatctgacgttgcccttggtgtttctgagaactgttgctgcaaaattctgtgtcacacccaccaagctgattccatccacttccacaatctggtcattgacttgtattctgccatcccgttgagcagcaccaccttctgttactgtcttgacgaatattcccagcttttcaagtccagcatctgctccaacacccattccaataatacttataccaagaccatcctcatctttctctagctccactgggaaaagttccagcttttctacacgtttttcaagttcatactcagctgaagcagccacagggtcaacttcgtcatttctcctgtcatagtcttcattggagtatgtgttgaaaaccttaataggagcactactaaacttaattttcctatttgctgggatttcttcttcttctggcaatccaacaatttccgagtactccatatcaggctgatagtaactgttctcatcactatcttcctcctcatcctgctcagtgcctgtctctccccagtctgaattatacctggatctcaccctatacacattatagtcactgtgcatgtacacatgggaaccatcaaaattatttgaatcttcaggtacttcttttccacaactggatgcagaagcatcaggagaggtgaaatcaccacctgcaagttctttcctctgttgctttgctgcctcccttccaaccaaattagcttcagcatcttctaacagttggctttgtggtgaagggatttcggactttggcattgccttactttcagcacaaggttcttcaggaccatctttgtcaatgctgtcgggagtctgttgattagatgtggagtcctcgggttccttgctctgctggatctcttcaccaggtatcgaagctagagaggtacttttagaagccacttctggtactggagttgcattactcttgtgagcatcctctgtatcaacacctcgcttgtttgaaggaggccaggaattagaatccttcaggtgaccaaatgtgtcaagatttgtaacagtaacagatggtaaattcaagggataatgcccagtcactgagtattcattgttttcagccttctcagaaatgatggcactgggagaatcagtgttctcaaatactgcactcagttgactcacagttggggagacagcctcagttcgggagctaaggctgtccaaggaatcagtactgcctctgttggacttggaacctccccattcatcctgaggttcactccctccagctttctctttctttggggaatagcggttgttctgtcctgattcatgcacacttctctcaaacatctttcgagtctcagtgaacttggaatatgaagggccatcgtacatagtgtcaaatctactaattcgttcagaaacagaagactccaacttaacaactgagccatctgttttttccagaaattctttgggcttcattcttctctgaggagatgaatgtccacctttcccccttgttttggcaatgactgcagcattctcgttgggttccatacccatctgcataaataggtttttaattctgttgacattggagccatatttcctccccctgctctgctgggagccctcaccttcttttgttttttgttccccatctgacttgggtttgtcaaaggtacttttcagtgcctgaaactcagttcgatatgcattcctgtgaggagaggcacttctgagagtggttcgttcacctgaagactcagttttcaacattttcacttcaggggtgaaaagccaatgttcataatgatcaaagaaaaaaaccaaaaaccaagatacctctcttctctaatcaccagtattgggtcaagaaaagtacctctcaaatggtatacggtgtcagtgatcgtcccaacaggtgtattaggaacttagtcacagtcaagagttacacagaatgattttttcaaagcaagactagaggttcatctcggctgatgggattaactctagggccgcagagagagggagcccggcagcaaaatcccgggagag

SEQ ID NO: 17005 - RNA, 9630 nt, Homo sapiens
  source 1..9630: mol_type = other RNA
taggtagtttcatgttgttgggaggtgttatctggctggagtgcctcttaattctttttaaggtaatttaattatttcttgccaattgttctttcttgaatgaatgattacatccttaacagaaaacctgggtgtataaataatacagctgaaagaaacagaagtgtacaccttccaacaacatacactcccaaccacttgtgttgtttttggcaacaaccaaaatgccattgcttgcacaaaaagtaaataaatgatcatatgatggcaacattcatcataagagagccagtaggcagtgactgtaagcatcacagccaccaattatgtcattttagaattgtgagcaaattcacaagaacacacagtgcaatttttagctgcatacatttcttctgagctccaactcagcaatatgcaatcttgacatcaaagcattagccaaatatttgaggaaattttcttactaaaataccaagtatctgataaatcaattttaccaaaatatataaacatatagaaggataagtgcatttagtagaaatacttacaataaaaaaatctcttaaaatctatgagccattcaatgtatacacaacgcaagaagtggcaataaggctatgattacagctccaggtcctgactgacctcgccaagttccatacacaatatattttttaatgccatgtgattgcagtgtgtgtgcgtgtgtaaggtgggagtgatattcacacatatgtagttctgaacatctacacaaacggcatgcacattgttgagaagttatctgttctcttattgcatacatcttactcactgttgaatccctagcagttttggggttgggttagggtcaagcataggaaatcatcatatttctttccttctccactcttgaggatctggaatcaggtcacagactgtgctgggtccacacgcttacatatgtgaaccttcaagtaactaccattccctcaataggcccacatagacaccacggacaagcaaataaggaccctctgtctaccataaatagaacttgatgctttcactttccaggagaagctgattctgtcggctttctctttgcccctccaacttcttagttgggcctattctatgctgctacttcaagttactcaaatgtgttttgtctggtgttatttttttctccagtgttttggaccaagactagatttcctgagactttaaatacgcaagacaaatgcaaacaaaatctgccaacatacccaggctgcttttcaggagtgaatcactgaagcgcatttggatttcctataacactactttcttttgggaatgtacagccctcccccagctccccatcccccatcataatgtaaaccattctaatagaaaatatggatgttttggctgggggtggtggcacatgcctgtagtcccagctacttgggaagctgaagcaggaggaccacttgagcccaggagtttgaggctgcagtaagacatgatggcaccactgcagtccagtctgggtgacagatgacagaaaaaaaaaaaaaaaaagaaaagaaaagaaaatatggacattttatttctggactttatccttaaatgcttagctttagaatagtgcacaggtacatccttaataaaaagtaaatttgaaaagacaggaaaggactgtgcttttctcttccattttaccttttcattctgagaccactaaggtctttgcattaagtaggtgacgtgaaccctagtgaccactgcccaccaaaatgcccctcatctccagctctgtcaggagtacctttagttactcaaatggaaatatctcagtgtaatgatggggctacaacatatccaaagtatagatggttctctcagggctgctggggcagcttcctttagaatcctctagaacactattgttaaacactggatctcctcttgaagtttagtctgcataacctttaacacttaaacatgaatcagagtatctatataaatgcaaattttcatttcccttttataaaatgcaattttcaagcacatgctaattctggtgcacaatgaacccagacaaatttgtcttcagcacaaactctaacggccgaggtgctagatcaaaccacctgtgaccatttttgtagcttgggactgggatattttaagatttcaggctagtgatgattacagggtcacagatagtggcaaaggtaaatctggttcctcattttccctcttgccactttgtttccaacaacaatggagcaaaaggtgacagtcccattttgtgccagttgaaagctgagtttggctttagtacctatcatactgcaatcatgaactgctgtgggttaaaaaaagcttgtgatgttgagggtgtgaaatcaattgtcaatcccagctaaaggatgatagccacagaacagctttattgtcatgaaactaaagggggacttcatcaggagtgttagaatggatgaaatgaggtttcttccctaacttaacattctgcagaaaattcctgattcaggtaaaaaaagaatgagattagtattacataaactgtgagttacttgaagggagatggtcttaaacaaagtaatctgttataaaactaacatcctttaatgggaaaccctgacccagatacagctcatacaatgctttctgtctgcagcttggcctcctcaccacacattccctcccaacaaagcataacctataccccaaaacacttttggctattgttagaatcatactgagctctcctttagggaatcagttcatagcaaccagatattccctttttgttcattttctgataataaaaactgcagtttttaaggttgatgaaataacaattctgtgttaaattgtaaggacactgaaaaccactagcattaaagtaggaattgtgcaagacattggagccttgattaggtatcatgcactacagtcaataaaagaaataataggaaaacaaaatgtgcacaagatctgaggtctttcactttgctttcatacccttaatcagtttacatcttatgctttgtggggcaatcaaaccaaatgacttttacaatttcatccgttttaagtggtaatgttaaaataactcacttcggcctaaaattactataatttaacttaaaaaatcaaaatacttataatactaaatgattttaggaataagaatttgatttataacattgtcagttggacatttatctaaacattcaatatacaaagttataaagaaaaatacttctaagatatttaagaaaatgcaatataatagatcataaattaggtgcaaaaacaagacacttacagacatttccagtatatacatccattttcaaatattaccaaagtgtaaacataacttaagataatcatccttctatttctactcttgaatacagtgaaacttccagtgtgatccaggtcacttttttcccaaagataagcaaaaatggcaaaaatttacaatagcaagcactaatattaccagatttttactaatttagtgttttagtatttgaaaagttttgccaaattgtatcactcattaatagtggcttcttatttctcatgatgtgaaaaaataacaaagcaccagacatctcaagacattaatagagtatccaatacggcagtttcattatcatacccctaatgaagacagacagaaaaacataatggtgactttgataactgtaaaacacaatgttacttcatgtcaacgtttctgaggattgaatgaagggtctgtacctaatgacaaaagagctgacgcataaccgacaatactctggcaatgaaaagaaaacaggccttgggggtaaaacagaattaaaaatgtccagtttagataatttctgaattcagattttcagataaaaaaaaatcacactgttattaaaatacaagatggggctacaagggagttcccttaatctgttacactcaaaagccttgccgaggctctaaatatggaatacttctagtggaagatacgagatgctgggaacagagcagagattcccataaagtaaaagaagtaaaatactgtccaagaattcatgtggcctcaagtcttattctgaaacttgtcctttggaaagtggataacctcatttttagagtcaacgcagcaaagagaaccagatacatgagcataaaaaacaaaaaaccctcatcacatgaaatttctcaaaacgagtttattttctccttcttctgccccagtctcctgcacttgacttagtttggtgaaacatggaaatccttaatgctggcttaaaattagtataagttcctccactactaaagtatacctatgcactgccttaaacaaactttttctgtaaaattgagaatctttgaagtatggaaaggaatggttcggaaaaaccattcaaaatctctctaaaatgttaactgacagtttcctctaactggtatttctatttttcttaaaagtacatttgttaaaatactaactgagcccacctgggaaatcttgagtagaaaatatgtgatgagttcctgattgtgacataggcaggctgaagaccagccagaatgttccccaggagaggaaacctgaaaatggtggtttccttaaaaatcaatttcctgttcaatttcttgggttaggtagggggaagaggaactgtgttgtgtttgccagtgttgctgaaatgctgaacacacagcagtagcaaggtcaacagatcccaatatcccatggctgcattaatgtctgatttttttctttcttgttcagccgtatctagaggataaatattaccctcagaaccccaaggtaatacccacatccacattcttaaggcttttgcttttttcagtggttaacaaatagctataatttattttctttctttttgatgcctagcaagcagaatgacttgcttgccttttcccttagtaggtaactacagagcagagcacccatgtttccacagcggggtggtctcactgtccagactgagaattaagagcaaatctttcccacacattggagtaggtgttgcagtcctagaagttaagtactggtctcagatctcatggcagggtgctctctgccatgcagacatgtgcaattgccatttcaggatcccacactgaaaattcacggcgctccattaacaacaccagggtgtgtcatgctcttgggtggggtcacactagttctccaagtgacaaaacacacccaacacaacacaagatgttggtaagttagagaagagcaaaacacagctacttaaatgaaatctctggtttgttaatgaaccaaaggtggcttgggattattttagtagttaaaattaagagtgcattctattgcagaaaatgcagttattcaacacacagttcctcagccggcctagagccgcattacccttatcatttagtttctttttcatcctctggaggagagcagggcaggaagaggtggggacttctcttggagcatctccatcatctgtaagagggtatgtgttactgctcaccagcaccctcggctgtagttgacgtcatcttttctgtctttttggacttcctctgcatttgctcttgctcctttctccttagcttttctctttgtttttccattttctcttgggccttccgagccttctctagagacatcttcatttccttgagtttctttttgaccactgctcggtcctgggatgctgtcattccaagagccttaagtttatttccatccaactgcaggagctgttctccagtgatgttttgggcactgaattcagatacatactgctccagatttaggctcattaaccagtgagaaacctgctgcacactccattcctgaacggcccgattctgacactgactgtgtttgggagactgtccatcatcaaggatctcatctgatgacagtgctaaggactgagagagccctggtgttttaggttctgctcctaagccgctgaggtctgctgaactggtactgctgggactgaagtcatcattgaaggtaaaattcttggacccctttttatctgaaattagagtctcaggagaaggctgaagggaacttgtaggcgcaggcaggttcctgaaggaataggatcctttccggctgtcattaaaccatgagaaaggcatgcaaggggaacgagtggaggtctgagctgttgaacatggcttgggtgtccagttttccagtctgcctctgaagatcctgctacctgcagaaaacctactggcttctttttctttttctttccacttctttcccttgctggaattccttcgcaaaggcgcccccagatccacaaacttccgcttaatttttcctccttgcaccgccaatgaactggatgcccttagtgatttgggatctttggcatcatctttttctcgtaatattttcttgttggtggtttggtgatggcaaggagattcttccacatcatgatcagactttgaagtagaaaacagtgaagtgtctccccacatagaggagagaggccccatttctgggtccagtggttcttcttgaaattcagctatgtggtcagacgagaagggcacattgctatccaccggggtgaggggtggaacaccagaatctgattctggagaagacgttctcaaaccctttctctctagactgtcctccccatctgtggaactaacactatcatacagtcttgtcctagagggtctctggcgtctgttcttcacagagagctgggctcgagttttcagtgcttttgaatccaggcgctctgtctctgggactgcttcattcaagtcttgacttaggccatcttggcaagatgtctgcttgccatccaagttctccatggtatcccctttagagacttcaccaagagatgttcttctctcaaagatgttgttattattgttaacttgagtcccattttgcttcagtagcctgaatacctcagcttccaaatctctaatccgcacttggaggccttgcacttccacaagatgagctttttccaaatcttctattttctttctttctgcttcctgtcttttgatgaaatcaagctctttttgttgaaaatccttgatcaacttctttgccttgttgtatttcttttccaaggcctgatactggctttgagtctctttgagatgctcattcactgtgtggcataatgtttgggcctcaatccagtagctttccaacttcaacattctttccttattctcttctatgttttgttggagttgggttttttctagttcccacctcactttctcattttctgctgcctgcagcttggtcttcaatttttgaatctctgcttctgtaactgcatgtttgatttgcaactctttgaacttgtgactgagcttgcttgtgtccagttctgatggggaaaacatgtcctcattctcaggcagctcaaagacttcaatggccatgtcgctgccaggaaggacaggtcctacctcatcttcttcttcatctgtggcatattctcctgtctcgtcatcgtcggcatcatactgggcatagtgctgttccagcagctctctctggcgcctctcctgttccagtgtctggcttatcaactgggcaacctcgctcacttgtcctggtttttcccgcccaataacaaatctgacgttgcccttggtgtttctgagaactgttgctgcaaaattctgtgtcacacccaccaagctgattccatccacttccacaatctggtcattgacttgtattctgccatcccgttgagcagcaccaccttctgttactgtcttgacgaatattcccagcttttcaagtccagcatctgctccaacacccattccaataatacttataccaagaccatcctcatctttctctagctccactgggaaaagttccagcttttctacacgtttttcaagttcatactcagctgaagcagccacagggtcaacttcgtcatttctcctgtcatagtcttcattggagtatgtgttgaaaaccttaataggagcactactaaacttaattttcctatttgctgggatttcttcttcttctggcaatccaacaatttccgagtactccatatcaggctgatagtaactgttctcatcactatcttcctcctcatcctgctcagtgcctgtctctccccagtctgaattatacctggatctcaccctatacacattatagtcactgtgcatgtacacatgggaaccatcaaaattatttgaatcttcaggtacttcttttccacaactggatgcagaagcatcaggagaggtgaaatcaccacctgcaagttctttcctctgttgctttgctgcctcccttccaaccaaattagcttcagcatcttctaacagttggctttgtggtgaagggatttcggactttggcattgccttactttcagcacaaggttcttcaggaccatctttgtcaatgctgtcgggagtctgttgattagatgtggagtcctcgggttccttgctctgctggatctcttcaccaggtatcgaagctagagaggtacttttagaagccacttctggtactggagttgcattactcttgtgagcatcctctgtatcaacacctcgcttgtttgaaggaggccaggaattagaatccttcaggtgaccaaatgtgtcaagatttgtaacagtaacagatggtaaattcaagggataatgcccagtcactgagtattcattgttttcagccttctcagaaatgatggcactgggagaatcagtgttctcaaatactgcactcagttgactcacagttggggagacagcctcagttcgggagctaaggctgtccaaggaatcagtactgcctctgttggacttggaacctccccattcatcctgaggttcactccctccagctttctctttctttggggaatagcggttgttctgtcctgattcatgcacacttctctcaaacatctttcgagtctcagtgaacttggaatatgaagggccatcgtacatagtgtcaaatctactaattcgttcagaaacagaagactccaacttaacaactgagccatctgttttttccagaaattctttgggcttcattcttctctgaggagatgaatgtccacctttcccccttgttttggcaatgactgcagcattctcgttgggttccatacccatctgcataaataggtttttaattctgttgacattggagccatatttcctccccctgctctgctgggagccctcaccttcttttgttttttgttccccatctgacttgggtttgtcaaaggtacttttcagtgcctgaaactcagttcgatatgcattcctgtgaggagaggcacttctgagagtggttcgttcacctgaagactcagttttcaacattttcacttcaggggtgaaaagccaatgttcataatgatcaaagaaaaaaaccaaaaaccaagatacctctcttctctaatcaccagtattgggtcaagaaaagtacctctcaaatggtatacggtgtcagtgatcgtcccaacaggtgtattaggaacttagtcacagtcaagagttacacagaatgattttttcaaagcaagactagaggttcat

SEQ ID NO: 17006 - RNA, 9696 nt, Homo sapiens
  source 1..9696: mol_type = other RNA
taggtagtttcatgttgttgggaggtgttatctggctggagtgcctcttaattctttttaaggtaatttaattatttcttgccaattgttctttcttgaatgaatgattacatccttaacagaaaacctgggtgtataaataatacagctgaaagaaacagaagtgtacaccttccaacaacatacactcccaaccacttgtgttgtttttggcaacaaccaaaatgccattgcttgcacaaaaagtaaataaatgatcatatgatggcaacattcatcataagagagccagtaggcagtgactgtaagcatcacagccaccaattatgtcattttagaattgtgagcaaattcacaagaacacacagtgcaatttttagctgcatacatttcttctgagctccaactcagcaatatgcaatcttgacatcaaagcattagccaaatatttgaggaaattttcttactaaaataccaagtatctgataaatcaattttaccaaaatatataaacatatagaaggataagtgcatttagtagaaatacttacaataaaaaaatctcttaaaatctatgagccattcaatgtatacacaacgcaagaagtggcaataaggctatgattacagctccaggtcctgactgacctcgccaagttccatacacaatatattttttaatgccatgtgattgcagtgtgtgtgcgtgtgtaaggtgggagtgatattcacacatatgtagttctgaacatctacacaaacggcatgcacattgttgagaagttatctgttctcttattgcatacatcttactcactgttgaatccctagcagttttggggttgggttagggtcaagcataggaaatcatcatatttctttccttctccactcttgaggatctggaatcaggtcacagactgtgctgggtccacacgcttacatatgtgaaccttcaagtaactaccattccctcaataggcccacatagacaccacggacaagcaaataaggaccctctgtctaccataaatagaacttgatgctttcactttccaggagaagctgattctgtcggctttctctttgcccctccaacttcttagttgggcctattctatgctgctacttcaagttactcaaatgtgttttgtctggtgttatttttttctccagtgttttggaccaagactagatttcctgagactttaaatacgcaagacaaatgcaaacaaaatctgccaacatacccaggctgcttttcaggagtgaatcactgaagcgcatttggatttcctataacactactttcttttgggaatgtacagccctcccccagctccccatcccccatcataatgtaaaccattctaatagaaaatatggatgttttggctgggggtggtggcacatgcctgtagtcccagctacttgggaagctgaagcaggaggaccacttgagcccaggagtttgaggctgcagtaagacatgatggcaccactgcagtccagtctgggtgacagatgacagaaaaaaaaaaaaaaaaagaaaagaaaagaaaatatggacattttatttctggactttatccttaaatgcttagctttagaatagtgcacaggtacatccttaataaaaagtaaatttgaaaagacaggaaaggactgtgcttttctcttccattttaccttttcattctgagaccactaaggtctttgcattaagtaggtgacgtgaaccctagtgaccactgcccaccaaaatgcccctcatctccagctctgtcaggagtacctttagttactcaaatggaaatatctcagtgtaatgatggggctacaacatatccaaagtatagatggttctctcagggctgctggggcagcttcctttagaatcctctagaacactattgttaaacactggatctcctcttgaagtttagtctgcataacctttaacacttaaacatgaatcagagtatctatataaatgcaaattttcatttcccttttataaaatgcaattttcaagcacatgctaattctggtgcacaatgaacccagacaaatttgtcttcagcacaaactctaacggccgaggtgctagatcaaaccacctgtgaccatttttgtagcttgggactgggatattttaagatttcaggctagtgatgattacagggtcacagatagtggcaaaggtaaatctggttcctcattttccctcttgccactttgtttccaacaacaatggagcaaaaggtgacagtcccattttgtgccagttgaaagctgagtttggctttagtacctatcatactgcaatcatgaactgctgtgggttaaaaaaagcttgtgatgttgagggtgtgaaatcaattgtcaatcccagctaaaggatgatagccacagaacagctttattgtcatgaaactaaagggggacttcatcaggagtgttagaatggatgaaatgaggtttcttccctaacttaacattctgcagaaaattcctgattcaggtaaaaaaagaatgagattagtattacataaactgtgagttacttgaagggagatggtcttaaacaaagtaatctgttataaaactaacatcctttaatgggaaaccctgacccagatacagctcatacaatgctttctgtctgcagcttggcctcctcaccacacattccctcccaacaaagcataacctataccccaaaacacttttggctattgttagaatcatactgagctctcctttagggaatcagttcatagcaaccagatattccctttttgttcattttctgataataaaaactgcagtttttaaggttgatgaaataacaattctgtgttaaattgtaaggacactgaaaaccactagcattaaagtaggaattgtgcaagacattggagccttgattaggtatcatgcactacagtcaataaaagaaataataggaaaacaaaatgtgcacaagatctgaggtctttcactttgctttcatacccttaatcagtttacatcttatgctttgtggggcaatcaaaccaaatgacttttacaatttcatccgttttaagtggtaatgttaaaataactcacttcggcctaaaattactataatttaacttaaaaaatcaaaatacttataatactaaatgattttaggaataagaatttgatttataacattgtcagttggacatttatctaaacattcaatatacaaagttataaagaaaaatacttctaagatatttaagaaaatgcaatataatagatcataaattaggtgcaaaaacaagacacttacagacatttccagtatatacatccattttcaaatattaccaaagtgtaaacataacttaagataatcatccttctatttctactcttgaatacagtgaaacttccagtgtgatccaggtcacttttttcccaaagataagcaaaaatggcaaaaatttacaatagcaagcactaatattaccagatttttactaatttagtgttttagtatttgaaaagttttgccaaattgtatcactcattaatagtggcttcttatttctcatgatgtgaaaaaataacaaagcaccagacatctcaagacattaatagagtatccaatacggcagtttcattatcatacccctaatgaagacagacagaaaaacataatggtgactttgataactgtaaaacacaatgttacttcatgtcaacgtttctgaggattgaatgaagggtctgtacctaatgacaaaagagctgacgcataaccgacaatactctggcaatgaaaagaaaacaggccttgggggtaaaacagaattaaaaatgtccagtttagataatttctgaattcagattttcagataaaaaaaaatcacactgttattaaaatacaagatggggctacaagggagttcccttaatctgttacactcaaaagccttgccgaggctctaaatatggaatacttctagtggaagatacgagatgctgggaacagagcagagattcccataaagtaaaagaagtaaaatactgtccaagaattcatgtggcctcaagtcttattctgaaacttgtcctttggaaagtggataacctcatttttagagtcaacgcagcaaagagaaccagatacatgagcataaaaaacaaaaaaccctcatcacatgaaatttctcaaaacgagtttattttctccttcttctgccccagtctcctgcacttgacttagtttggtgaaacatggaaatccttaatgctggcttaaaattagtataagttcctccactactaaagtatacctatgcactgccttaaacaaactttttctgtaaaattgagaatctttgaagtatggaaaggaatggttcggaaaaaccattcaaaatctctctaaaatgttaactgacagtttcctctaactggtatttctatttttcttaaaagtacatttgttaaaatactaactgagcccacctgggaaatcttgagtagaaaatatgtgatgagttcctgattgtgacataggcaggctgaagaccagccagaatgttccccaggagaggaaacctgaaaatggtggtttccttaaaaatcaatttcctgttcaatttcttgggttaggtagggggaagaggaactgtgttgtgtttgccagtgttgctgaaatgctgaacacacagcagtagcaaggtcaacagatcccaatatcccatggctgcattaatgtctgatttttttctttcttgttcagccgtatctagaggataaatattaccctcagaaccccaaggtaatacccacatccacattcttaaggcttttgcttttttcagtggttaacaaatagctataatttattttctttctttttgatgcctagcaagcagaatgacttgcttgccttttcccttagtaggtaactacagagcagagcacccatgtttccacagcggggtggtctcactgtccagactgagaattaagagcaaatctttcccacacattggagtaggtgttgcagtcctagaagttaagtactggtctcagatctcatggcagggtgctctctgccatgcagacatgtgcaattgccatttcaggatcccacactgaaaattcacggcgctccattaacaacaccagggtgtgtcatgctcttgggtggggtcacactagttctccaagtgacaaaacacacccaacacaacacaagatgttggtaagttagagaagagcaaaacacagctacttaaatgaaatctctggtttgttaatgaaccaaaggtggcttgggattattttagtagttaaaattaagagtgcattctattgcagaaaatgcagttattcaacacacagttcctcagccggcctagagccgcattacccttatcatttagtttctttttcatcctctggaggagagcagggcaggaagaggtggggacttctcttggagcatctccatcatctgtaagagggtatgtgttactgctcaccagcaccctcggctgtagttgacgtcatcttttctgtctttttggacttcctctgcatttgctcttgctcctttctccttagcttttctctttgtttttccattttctcttgggccttccgagccttctctagagacatcttcatttccttgagtttctttttgaccactgctcggtcctgggatgctgtcattccaagagccttaagtttatttccatccaactgcaggagctgttctccagtgatgttttgggcactgaattcagatacatactgctccagatttaggctcattaaccagtgagaaacctgctgcacactccattcctgaacggcccgattctgacactgactgtgtttgggagactgtccatcatcaaggatctcatctgatgacagtgctaaggactgagagagccctggtgttttaggttctgctcctaagccgctgaggtctgctgaactggtactgctgggactgaagtcatcattgaaggtaaaattcttggacccctttttatctgaaattagagtctcaggagaaggctgaagggaacttgtaggcgcaggcaggttcctgaaggaataggatcctttccggctgtcattaaaccatgagaaaggcatgcaaggggaacgagtggaggtctgagctgttgaacatggcttgggtgtccagttttccagtctgcctctgaagatcctgctacctgcagaaaacctactggcttctttttctttttctttccacttctttcccttgctggaattccttcgcaaaggcgcccccagatccacaaacttccgcttaatttttcctccttgcaccgccaatgaactggatgcccttagtgatttgggatctttggcatcatctttttctcgtaatattttcttgttggtggtttggtgatggcaaggagattcttccacatcatgatcagactttgaagtagaaaacagtgaagtgtctccccacatagaggagagaggccccatttctgggtccagtggttcttcttgaaattcagctatgtggtcagacgagaagggcacattgctatccaccggggtgaggggtggaacaccagaatctgattctggagaagacgttctcaaaccctttctctctagactgtcctccccatctgtggaactaacactatcatacagtcttgtcctagagggtctctggcgtctgttcttcacagagagctgggctcgagttttcagtgcttttgaatccaggcgctctgtctctgggactgcttcattcaagtcttgacttaggccatcttggcaagatgtctgcttgccatccaagttctccatggtatcccctttagagacttcaccaagagatgttcttctctcaaagatgttgttattattgttaacttgagtcccattttgcttcagtagcctgaatacctcagcttccaaatctctaatccgcacttggaggccttgcacttccacaagatgagctttttccaaatcttctattttctttctttctgcttcctgtcttttgatgaaatcaagctctttttgttgaaaatccttgatcaacttctttgccttgttgtatttcttttccaaggcctgatactggctttgagtctctttgagatgctcattcactgtgtggcataatgtttgggcctcaatccagtagctttccaacttcaacattctttccttattctcttctatgttttgttggagttgggttttttctagttcccacctcactttctcattttctgctgcctgcagcttggtcttcaatttttgaatctctgcttctgtaactgcatgtttgatttgcaactctttgaacttgtgactgagcttgcttgtgtccagttctgatggggaaaacatgtcctcattctcaggcagctcaaagacttcaatggccatgtcgctgccaggaaggacaggtcctacctcatcttcttcttcatctgtggcatattctcctgtctcgtcatcgtcggcatcatactgggcatagtgctgttccagcagctctctctggcgcctctcctgttccagtgtctggcttatcaactgggcaacctcgctcacttgtcctggtttttcccgcccaataacaaatctgacgttgcccttggtgtttctgagaactgttgctgcaaaattctgtgtcacacccaccaagctgattccatccacttccacaatctggtcattgacttgtattctgccatcccgttgagcagcaccaccttctgttactgtcttgacgaatattcccagcttttcaagtccagcatctgctccaacacccattccaataatacttataccaagaccatcctcatctttctctagctccactgggaaaagttccagcttttctacacgtttttcaagttcatactcagctgaagcagccacagggtcaacttcgtcatttctcctgtcatagtcttcattggagtatgtgttgaaaaccttaataggagcactactaaacttaattttcctatttgctgggatttcttcttcttctggcaatccaacaatttccgagtactccatatcaggctgatagtaactgttctcatcactatcttcctcctcatcctgctcagtgcctgtctctccccagtctgaattatacctggatctcaccctatacacattatagtcactgtgcatgtacacatgggaaccatcaaaattatttgaatcttcaggtacttcttttccacaactggatgcagaagcatcaggagaggtgaaatcaccacctgcaagttctttcctctgttgctttgctgcctcccttccaaccaaattagcttcagcatcttctaacagttggctttgtggtgaagggatttcggactttggcattgccttactttcagcacaaggttcttcaggaccatctttgtcaatgctgtcgggagtctgttgattagatgtggagtcctcgggttccttgctctgctggatctcttcaccaggtatcgaagctagagaggtacttttagaagccacttctggtactggagttgcattactcttgtgagcatcctctgtatcaacacctcgcttgtttgaaggaggccaggaattagaatccttcaggtgaccaaatgtgtcaagatttgtaacagtaacagatggtaaattcaagggataatgcccagtcactgagtattcattgttttcagccttctcagaaatgatggcactgggagaatcagtgttctcaaatactgcactcagttgactcacagttggggagacagcctcagttcgggagctaaggctgtccaaggaatcagtactgcctctgttggacttggaacctccccattcatcctgaggttcactccctccagctttctctttctttggggaatagcggttgttctgtcctgattcatgcacacttctctcaaacatctttcgagtctcagtgaacttggaatatgaagggccatcgtacatagtgtcaaatctactaattcgttcagaaacagaagactccaacttaacaactgagccatctgttttttccagaaattctttgggcttcattcttctctgaggagatgaatgtccacctttcccccttgttttggcaatgactgcagcattctcgttgggttccatacccatctgcataaataggtttttaattctgttgacattggagccatatttcctccccctgctctgctgggagccctcaccttcttttgttttttgttccccatctgacttgggtttgtcaaaggtacttttcagtgcctgaaactcagttcgatatgcattcctgtgaggagaggcacttctgagagtggttcgttcacctgaagactcagttttcaacattttcacttcaggggtgaaaagccaatgttcataatgatcaaagaaaaaaaccaaaaaccaagatacctctcttctctaatcaccagtattgggtcaagaaaagtacctctcaaatggtatacggtgtcagtgatcgtcccaacaggtgtattaggaacttagtcacagtcaagagttacacagaatgattttttcaaagcaagactagaggttcatctcggctgatgggattaactctagggccgcagagagagggagcccggcagcaaaatcccgggagag

SEQ ID NO: 17007 - RNA, 9762 nt, Homo sapiens
  source 1..9762: mol_type = other RNA
taggtagtttcatgttgttgggaggtgttatctggctggagtgcctcttaattctttttaaggtaatttaattatttcttgccaattgttctttcttgaatgaatgattacatccttaacagaaaacctgggtgtataaataatacagctgaaagaaacagaagtgtacaccttccaacaacatacactcccaaccacttgtgttgtttttggcaacaaccaaaatgccattgcttgcacaaaaagtaaataaatgatcatatgatggcaacattcatcataagagagccagtaggcagtgactgtaagcatcacagccaccaattatgtcattttagaattgtgagcaaattcacaagaacacacagtgcaatttttagctgcatacatttcttctgagctccaactcagcaatatgcaatcttgacatcaaagcattagccaaatatttgaggaaattttcttactaaaataccaagtatctgataaatcaattttaccaaaatatataaacatatagaaggataagtgcatttagtagaaatacttacaataaaaaaatctcttaaaatctatgagccattcaatgtatacacaacgcaagaagtggcaataaggctatgattacagctccaggtcctgactgacctcgccaagttccatacacaatatattttttaatgccatgtgattgcagtgtgtgtgcgtgtgtaaggtgggagtgatattcacacatatgtagttctgaacatctacacaaacggcatgcacattgttgagaagttatctgttctcttattgcatacatcttactcactgttgaatccctagcagttttggggttgggttagggtcaagcataggaaatcatcatatttctttccttctccactcttgaggatctggaatcaggtcacagactgtgctgggtccacacgcttacatatgtgaaccttcaagtaactaccattccctcaataggcccacatagacaccacggacaagcaaataaggaccctctgtctaccataaatagaacttgatgctttcactttccaggagaagctgattctgtcggctttctctttgcccctccaacttcttagttgggcctattctatgctgctacttcaagttactcaaatgtgttttgtctggtgttatttttttctccagtgttttggaccaagactagatttcctgagactttaaatacgcaagacaaatgcaaacaaaatctgccaacatacccaggctgcttttcaggagtgaatcactgaagcgcatttggatttcctataacactactttcttttgggaatgtacagccctcccccagctccccatcccccatcataatgtaaaccattctaatagaaaatatggatgttttggctgggggtggtggcacatgcctgtagtcccagctacttgggaagctgaagcaggaggaccacttgagcccaggagtttgaggctgcagtaagacatgatggcaccactgcagtccagtctgggtgacagatgacagaaaaaaaaaaaaaaaaagaaaagaaaagaaaatatggacattttatttctggactttatccttaaatgcttagctttagaatagtgcacaggtacatccttaataaaaagtaaatttgaaaagacaggaaaggactgtgcttttctcttccattttaccttttcattctgagaccactaaggtctttgcattaagtaggtgacgtgaaccctagtgaccactgcccaccaaaatgcccctcatctccagctctgtcaggagtacctttagttactcaaatggaaatatctcagtgtaatgatggggctacaacatatccaaagtatagatggttctctcagggctgctggggcagcttcctttagaatcctctagaacactattgttaaacactggatctcctcttgaagtttagtctgcataacctttaacacttaaacatgaatcagagtatctatataaatgcaaattttcatttcccttttataaaatgcaattttcaagcacatgctaattctggtgcacaatgaacccagacaaatttgtcttcagcacaaactctaacggccgaggtgctagatcaaaccacctgtgaccatttttgtagcttgggactgggatattttaagatttcaggctagtgatgattacagggtcacagatagtggcaaaggtaaatctggttcctcattttccctcttgccactttgtttccaacaacaatggagcaaaaggtgacagtcccattttgtgccagttgaaagctgagtttggctttagtacctatcatactgcaatcatgaactgctgtgggttaaaaaaagcttgtgatgttgagggtgtgaaatcaattgtcaatcccagctaaaggatgatagccacagaacagctttattgtcatgaaactaaagggggacttcatcaggagtgttagaatggatgaaatgaggtttcttccctaacttaacattctgcagaaaattcctgattcaggtaaaaaaagaatgagattagtattacataaactgtgagttacttgaagggagatggtcttaaacaaagtaatctgttataaaactaacatcctttaatgggaaaccctgacccagatacagctcatacaatgctttctgtctgcagcttggcctcctcaccacacattccctcccaacaaagcataacctataccccaaaacacttttggctattgttagaatcatactgagctctcctttagggaatcagttcatagcaaccagatattccctttttgttcattttctgataataaaaactgcagtttttaaggttgatgaaataacaattctgtgttaaattgtaaggacactgaaaaccactagcattaaagtaggaattgtgcaagacattggagccttgattaggtatcatgcactacagtcaataaaagaaataataggaaaacaaaatgtgcacaagatctgaggtctttcactttgctttcatacccttaatcagtttacatcttatgctttgtggggcaatcaaaccaaatgacttttacaatttcatccgttttaagtggtaatgttaaaataactcacttcggcctaaaattactataatttaacttaaaaaatcaaaatacttataatactaaatgattttaggaataagaatttgatttataacattgtcagttggacatttatctaaacattcaatatacaaagttataaagaaaaatacttctaagatatttaagaaaatgcaatataatagatcataaattaggtgcaaaaacaagacacttacagacatttccagtatatacatccattttcaaatattaccaaagtgtaaacataacttaagataatcatccttctatttctactcttgaatacagtgaaacttccagtgtgatccaggtcacttttttcccaaagataagcaaaaatggcaaaaatttacaatagcaagcactaatattaccagatttttactaatttagtgttttagtatttgaaaagttttgccaaattgtatcactcattaatagtggcttcttatttctcatgatgtgaaaaaataacaaagcaccagacatctcaagacattaatagagtatccaatacggcagtttcattatcatacccctaatgaagacagacagaaaaacataatggtgactttgataactgtaaaacacaatgttacttcatgtcaacgtttctgaggattgaatgaagggtctgtacctaatgacaaaagagctgacgcataaccgacaatactctggcaatgaaaagaaaacaggccttgggggtaaaacagaattaaaaatgtccagtttagataatttctgaattcagattttcagataaaaaaaaatcacactgttattaaaatacaagatggggctacaagggagttcccttaatctgttacactcaaaagccttgccgaggctctaaatatggaatacttctagtggaagatacgagatgctgggaacagagcagagattcccataaagtaaaagaagtaaaatactgtccaagaattcatgtggcctcaagtcttattctgaaacttgtcctttggaaagtggataacctcatttttagagtcaacgcagcaaagagaaccagatacatgagcataaaaaacaaaaaaccctcatcacatgaaatttctcaaaacgagtttattttctccttcttctgccccagtctcctgcacttgacttagtttggtgaaacatggaaatccttaatgctggcttaaaattagtataagttcctccactactaaagtatacctatgcactgccttaaacaaactttttctgtaaaattgagaatctttgaagtatggaaaggaatggttcggaaaaaccattcaaaatctctctaaaatgttaactgacagtttcctctaactggtatttctatttttcttaaaagtacatttgttaaaatactaactgagcccacctgggaaatcttgagtagaaaatatgtgatgagttcctgattgtgacataggcaggctgaagaccagccagaatgttccccaggagaggaaacctgaaaatggtggtttccttaaaaatcaatttcctgttcaatttcttgggttaggtagggggaagaggaactgtgttgtgtttgccagtgttgctgaaatgctgaacacacagcagtagcaaggtcaacagatcccaatatcccatggctgcattaatgtctgatttttttctttcttgttcagccgtatctagaggataaatattaccctcagaaccccaaggtaatacccacatccacattcttaaggcttttgcttttttcagtggttaacaaatagctataatttattttctttctttttgatgcctagcaagcagaatgacttgcttgccttttcccttagtaggtaactacagagcagagcacccatgtttccacagcggggtggtctcactgtccagactgagaattaagagcaaatctttcccacacattggagtaggtgttgcagtcctagaagttaagtactggtctcagatctcatggcagggtgctctctgccatgcagacatgtgcaattgccatttcaggatcccacactgaaaattcacggcgctccattaacaacaccagggtgtgtcatgctcttgggtggggtcacactagttctccaagtgacaaaacacacccaacacaacacaagatgttggtaagttagagaagagcaaaacacagctacttaaatgaaatctctggtttgttaatgaaccaaaggtggcttgggattattttagtagttaaaattaagagtgcattctattgcagaaaatgcagttattcaacacacagttcctcagccggcctagagccgcattacccttatcatttagtttctttttcatcctctggaggagagcagggcaggaagaggtggggacttctcttggagcatctccatcatctgtaagagggtatgtgttactgctcaccagcaccctcggctgtagttgacgtcatcttttctgtctttttggacttcctctgcatttgctcttgctcctttctccttagcttttctctttgtttttccattttctcttgggccttccgagccttctctagagacatcttcatttccttgagtttctttttgaccactgctcggtcctgggatgctgtcattccaagagccttaagtttatttccatccaactgcaggagctgttctccagtgatgttttgggcactgaattcagatacatactgctccagatttaggctcattaaccagtgagaaacctgctgcacactccattcctgaacggcccgattctgacactgactgtgtttgggagactgtccatcatcaaggatctcatctgatgacagtgctaaggactgagagagccctggtgttttaggttctgctcctaagccgctgaggtctgctgaactggtactgctgggactgaagtcatcattgaaggtaaaattcttggacccctttttatctgaaattagagtctcaggagaaggctgaagggaacttgtaggcgcaggcaggttcctgaaggaataggatcctttccggctgtcattaaaccatgagaaaggcatgcaaggggaacgagtggaggtctgagctgttgaacatggcttgggtgtccagttttccagtctgcctctgaagatcctgctacctgcagaaaacctactggcttctttttctttttctttccacttctttcccttgctggaattccttcgcaaaggcgcccccagatccacaaacttccgcttaatttttcctccttgcaccgccaatgaactggatgcccttagtgatttgggatctttggcatcatctttttctcgtaatattttcttgttggtggtttggtgatggcaaggagattcttccacatcatgatcagactttgaagtagaaaacagtgaagtgtctccccacatagaggagagaggccccatttctgggtccagtggttcttcttgaaattcagctatgtggtcagacgagaagggcacattgctatccaccggggtgaggggtggaacaccagaatctgattctggagaagacgttctcaaaccctttctctctagactgtcctccccatctgtggaactaacactatcatacagtcttgtcctagagggtctctggcgtctgttcttcacagagagctgggctcgagttttcagtgcttttgaatccaggcgctctgtctctgggactgcttcattcaagtcttgacttaggccatcttggcaagatgtctgcttgccatccaagttctccatggtatcccctttagagacttcaccaagagatgttcttctctcaaagatgttgttattattgttaacttgagtcccattttgcttcagtagcctgaatacctcagcttccaaatctctaatccgcacttggaggccttgcacttccacaagatgagctttttccaaatcttctattttctttctttctgcttcctgtcttttgatgaaatcaagctctttttgttgaaaatccttgatcaacttctttgccttgttgtatttcttttccaaggcctgatactggctttgagtctctttgagatgctcattcactgtgtggcataatgtttgggcctcaatccagtagctttccaacttcaacattctttccttattctcttctatgttttgttggagttgggttttttctagttcccacctcactttctcattttctgctgcctgcagcttggtcttcaatttttgaatctctgcttctgtaactgcatgtttgatttgcaactctttgaacttgtgactgagcttgcttgtgtccagttctgatggggaaaacatgtcctcattctcaggcagctcaaagacttcaatggccatgtcgctgccaggaaggacaggtcctacctcatcttcttcttcatctgtggcatattctcctgtcttaagaaaatagttgttattgttattgcagttgccagacattccttgcaattcagccacagtgttctcgtcatcgtcggcatcatactgggcatagtgctgttccagcagctctctctggcgcctctcctgttccagtgtctggcttatcaactgggcaacctcgctcacttgtcctggtttttcccgcccaataacaaatctgacgttgcccttggtgtttctgagaactgttgctgcaaaattctgtgtcacacccaccaagctgattccatccacttccacaatctggtcattgacttgtattctgccatcccgttgagcagcaccaccttctgttactgtcttgacgaatattcccagcttttcaagtccagcatctgctccaacacccattccaataatacttataccaagaccatcctcatctttctctagctccactgggaaaagttccagcttttctacacgtttttcaagttcatactcagctgaagcagccacagggtcaacttcgtcatttctcctgtcatagtcttcattggagtatgtgttgaaaaccttaataggagcactactaaacttaattttcctatttgctgggatttcttcttcttctggcaatccaacaatttccgagtactccatatcaggctgatagtaactgttctcatcactatcttcctcctcatcctgctcagtgcctgtctctccccagtctgaattatacctggatctcaccctatacacattatagtcactgtgcatgtacacatgggaaccatcaaaattatttgaatcttcaggtacttcttttccacaactggatgcagaagcatcaggagaggtgaaatcaccacctgcaagttctttcctctgttgctttgctgcctcccttccaaccaaattagcttcagcatcttctaacagttggctttgtggtgaagggatttcggactttggcattgccttactttcagcacaaggttcttcaggaccatctttgtcaatgctgtcgggagtctgttgattagatgtggagtcctcgggttccttgctctgctggatctcttcaccaggtatcgaagctagagaggtacttttagaagccacttctggtactggagttgcattactcttgtgagcatcctctgtatcaacacctcgcttgtttgaaggaggccaggaattagaatccttcaggtgaccaaatgtgtcaagatttgtaacagtaacagatggtaaattcaagggataatgcccagtcactgagtattcattgttttcagccttctcagaaatgatggcactgggagaatcagtgttctcaaatactgcactcagttgactcacagttggggagacagcctcagttcgggagctaaggctgtccaaggaatcagtactgcctctgttggacttggaacctccccattcatcctgaggttcactccctccagctttctctttctttggggaatagcggttgttctgtcctgattcatgcacacttctctcaaacatctttcgagtctcagtgaacttggaatatgaagggccatcgtacatagtgtcaaatctactaattcgttcagaaacagaagactccaacttaacaactgagccatctgttttttccagaaattctttgggcttcattcttctctgaggagatgaatgtccacctttcccccttgttttggcaatgactgcagcattctcgttgggttccatacccatctgcataaataggtttttaattctgttgacattggagccatatttcctccccctgctctgctgggagccctcaccttcttttgttttttgttccccatctgacttgggtttgtcaaaggtacttttcagtgcctgaaactcagttcgatatgcattcctgtgaggagaggcacttctgagagtggttcgttcacctgaagactcagttttcaacattttcacttcaggggtgaaaagccaatgttcataatgatcaaagaaaaaaaccaaaaaccaagatacctctcttctctaatcaccagtattgggtcaagaaaagtacctctcaaatggtatacggtgtcagtgatcgtcccaacaggtgtattaggaacttagtcacagtcaagagttacacagaatgattttttcaaagcaagactagaggttcatctcggctgatgggattaactctagggccgcagagagagggagcccggcagcaaaatcccgggagag

SEQ ID NO: 17008 - RNA, 9012 nt, Homo sapiens
  source 1..9012: mol_type = other RNA
taggtagtttcatgttgttgggaggtgttatctggctggagtgcctcttaattctttttaaggtaatttaattatttcttgccaattgttctttcttgaatgaatgattacatccttaacagaaaacctgggtgtataaataatacagctgaaagaaacagaagtgtacaccttccaacaacatacactcccaaccacttgtgttgtttttggcaacaaccaaaatgccattgcttgcacaaaaagtaaataaatgatcatatgatggcaacattcatcataagagagccagtaggcagtgactgtaagcatcacagccaccaattatgtcattttagaattgtgagcaaattcacaagaacacacagtgcaatttttagctgcatacatttcttctgagctccaactcagcaatatgcaatcttgacatcaaagcattagccaaatatttgaggaaattttcttactaaaataccaagtatctgataaatcaattttaccaaaatatataaacatatagaaggataagtgcatttagtagaaatacttacaataaaaaaatctcttaaaatctatgagccattcaatgtatacacaacgcaagaagtggcaataaggctatgattacagctccaggtcctgactgacctcgccaagttccatacacaatatattttttaatgccatgtgattgcagtgtgtgtgcgtgtgtaaggtgggagtgatattcacacatatgtagttctgaacatctacacaaacggcatgcacattgttgagaagttatctgttctcttattgcatacatcttactcactgttgaatccctagcagttttggggttgggttagggtcaagcataggaaatcatcatatttctttccttctccactcttgaggatctggaatcaggtcacagactgtgctgggtccacacgcttacatatgtgaaccttcaagtaactaccattccctcaataggcccacatagacaccacggacaagcaaataaggaccctctgtctaccataaatagaacttgatgctttcactttccaggagaagctgattctgtcggctttctctttgcccctccaacttcttagttgggcctattctatgctgctacttcaagttactcaaatgtgttttgtctggtgttatttttttctccagtgttttggaccaagactagatttcctgagactttaaatacgcaagacaaatgcaaacaaaatctgccaacatacccaggctgcttttcaggagtgaatcactgaagcgcatttggatttcctataacactactttcttttgggaatgtacagccctcccccagctccccatcccccatcataatgtaaaccattctaatagaaaatatggatgttttggctgggggtggtggcacatgcctgtagtcccagctacttgggaagctgaagcaggaggaccacttgagcccaggagtttgaggctgcagtaagacatgatggcaccactgcagtccagtctgggtgacagatgacagaaaaaaaaaaaaaaaaagaaaagaaaagaaaatatggacattttatttctggactttatccttaaatgcttagctttagaatagtgcacaggtacatccttaataaaaagtaaatttgaaaagacaggaaaggactgtgcttttctcttccattttaccttttcattctgagaccactaaggtctttgcattaagtaggtgacgtgaaccctagtgaccactgcccaccaaaatgcccctcatctccagctctgtcaggagtacctttagttactcaaatggaaatatctcagtgtaatgatggggctacaacatatccaaagtatagatggttctctcagggctgctggggcagcttcctttagaatcctctagaacactattgttaaacactggatctcctcttgaagtttagtctgcataacctttaacacttaaacatgaatcagagtatctatataaatgcaaattttcatttcccttttataaaatgcaattttcaagcacatgctaattctggtgcacaatgaacccagacaaatttgtcttcagcacaaactctaacggccgaggtgctagatcaaaccacctgtgaccatttttgtagcttgggactgggatattttaagatttcaggctagtgatgattacagggtcacagatagtggcaaaggtaaatctggttcctcattttccctcttgccactttgtttccaacaacaatggagcaaaaggtgacagtcccattttgtgccagttgaaagctgagtttggctttagtacctatcatactgcaatcatgaactgctgtgggttaaaaaaagcttgtgatgttgagggtgtgaaatcaattgtcaatcccagctaaaggatgatagccacagaacagctttattgtcatgaaactaaagggggacttcatcaggagtgttagaatggatgaaatgaggtttcttccctaacttaacattctgcagaaaattcctgattcaggtaaaaaaagaatgagattagtattacataaactgtgagttacttgaagggagatggtcttaaacaaagtaatctgttataaaactaacatcctttaatgggaaaccctgacccagatacagctcatacaatgctttctgtctgcagcttggcctcctcaccacacattccctcccaacaaagcataacctataccccaaaacacttttggctattgttagaatcatactgagctctcctttagggaatcagttcatagcaaccagatattccctttttgttcattttctgataataaaaactgcagtttttaaggttgatgaaataacaattctgtgttaaattgtaaggacactgaaaaccactagcattaaagtaggaattgtgcaagacattggagccttgattaggtatcatgcactacagtcaataaaagaaataataggaaaacaaaatgtgcacaagatctgaggtctttcactttgctttcatacccttaatcagtttacatcttatgctttgtggggcaatcaaaccaaatgacttttacaatttcatccgttttaagtggtaatgttaaaataactcacttcggcctaaaattactataatttaacttaaaaaatcaaaatacttataatactaaatgattttaggaataagaatttgatttataacattgtcagttggacatttatctaaacattcaatatacaaagttataaagaaaaatacttctaagatatttaagaaaatgcaatataatagatcataaattaggtgcaaaaacaagacacttacagacatttccagtatatacatccattttcaaatattaccaaagtgtaaacataacttaagataatcatccttctatttctactcttgaatacagtgaaacttccagtgtgatccaggtcacttttttcccaaagataagcaaaaatggcaaaaatttacaatagcaagcactaatattaccagatttttactaatttagtgttttagtatttgaaaagttttgccaaattgtatcactcattaatagtggcttcttatttctcatgatgtgaaaaaataacaaagcaccagacatctcaagacattaatagagtatccaatacggcagtttcattatcatacccctaatgaagacagacagaaaaacataatggtgactttgataactgtaaaacacaatgttacttcatgtcaacgtttctgaggattgaatgaagggtctgtacctaatgacaaaagagctgacgcataaccgacaatactctggcaatgaaaagaaaacaggccttgggggtaaaacagaattaaaaatgtccagtttagataatttctgaattcagattttcagataaaaaaaaatcacactgttattaaaatacaagatggggctacaagggagttcccttaatctgttacactcaaaagccttgccgaggctctaaatatggaatacttctagtggaagatacgagatgctgggaacagagcagagattcccataaagtaaaagaagtaaaatactgtccaagaattcatgtggcctcaagtcttattctgaaacttgtcctttggaaagtggataacctcatttttagagtcaacgcagcaaagagaaccagatacatgagcataaaaaacaaaaaaccctcatcacatgaaatttctcaaaacgagtttattttctccttcttctgccccagtctcctgcacttgacttagtttggtgaaacatggaaatccttaatgctggcttaaaattagtataagttcctccactactaaagtatacctatgcactgccttaaacaaactttttctgtaaaattgagaatctttgaagtatggaaaggaatggttcggaaaaaccattcaaaatctctctaaaatgttaactgacagtttcctctaactggtatttctatttttcttaaaagtacatttgttaaaatactaactgagcccacctgggaaatcttgagtagaaaatatgtgatgagttcctgattgtgacataggcaggctgaagaccagccagaatgttccccaggagaggaaacctgaaaatggtggtttccttaaaaatcaatttcctgttcaatttcttgggttaggtagggggaagaggaactgtgttgtgtttgccagtgttgctgaaatgctgaacacacagcagtagcaaggtcaacagatcccaatatcccatggctgcattaatgtctgatttttttctttcttgttcagccgtatctagaggataaatattaccctcagaaccccaaggtaatacccacatccacattcttaaggcttttgcttttttcagtggttaacaaatagctataatttattttctttctttttgatgcctagcaagcagaatgacttgcttgccttttcccttagtaggtaactacagagcagagcacccatgtttccacagcggggtggtctcactgtccagactgagaattaagagcaaatctttcccacacattggagtaggtgttgcagtcctagaagttaagtactggtctcagatctcatggcagggtgctctctgccatgcagacatgtgcaattgccatttcaggatcccacactgaaaattcacggcgctccattaacaacaccagggtgtgtcatgctcttgggtggggtcacactagttctccaagtgacaaaacacacccaacacaacacaagatgttggtaagttagagaagagcaaaacacagctacttaaatgaaatctctggtttgttaatgaaccaaaggtggcttgggattattttagtagttaaaattaagagtgcattctattgcagaaaatgcagttattcaacacacagttcctcagccggcctagagccgcattacccttatcatttagtttctttttcatcctctggaggagagcagggcaggaagaggtggggacttctcttggagcatctccatcatctgtaagagggtatgtgttactgctcaccagcaccctcggctgtagttgacgtcatcttttctgtctttttggacttcctctgcatttgctcttgctcctttctccttagcttttctctttgtttttccattttctcttgggccttccgagccttctctagagacatcttcatttccttgagtttctttttgaccactgctcggtcctgggatgctgtcattccaagagccttaagtttatttccatccaactgcaggagctgttctccagtgatgttttgggcactgaattcagatacatactgctccagatttaggctcattaaccagtgagaaacctgctgcacactccattcctgaacggcccgattctgacactgactgtgtttgggagactgtccatcatcaaggatctcatctgatgacagtgctaaggactgagagagccctggtgttttaggttctgctcctaagccgctgaggtctgctgaactggtactgctgggactgaagtcatcattgaaggtaaaattctttctctctagactgtcctccccatctgtggaactaacactatcatacagtcttgtcctagagggtctctggcgtctgttcttcacagagagctgggctcgagttttcagtgcttttgaatccaggcgctctgtctctgggactgcttcattcaagtcttgacttaggccatcttggcaagatgtctgcttgccatccaagttctccatggtatcccctttagagacttcaccaagagatgttcttctctcaaagatgttgttattattgttaacttgagtcccattttgcttcagtagcctgaatacctcagcttccaaatctctaatccgcacttggaggccttgcacttccacaagatgagctttttccaaatcttctattttctttctttctgcttcctgtcttttgatgaaatcaagctctttttgttgaaaatccttgatcaacttctttgccttgttgtatttcttttccaaggcctgatactggctttgagtctctttgagatgctcattcactgtgtggcataatgtttgggcctcaatccagtagctttccaacttcaacattctttccttattctcttctatgttttgttggagttgggttttttctagttcccacctcactttctcattttctgctgcctgcagcttggtcttcaatttttgaatctctgcttctgtaactgcatgtttgatttgcaactctttgaacttgtgactgagcttgcttgtgtccagttctgatggggaaaacatgtcctcattctcaggcagctcaaagacttcaatggccatgtcgctgccaggaaggacaggtcctacctcatcttcttcttcatctgtggcatattctcctgtctcgtcatcgtcggcatcatactgggcatagtgctgttccagcagctctctctggcgcctctcctgttccagtgtctggcttatcaactgggcaacctcgctcacttgtcctggtttttcccgcccaataacaaatctgacgttgcccttggtgtttctgagaactgttgctgcaaaattctgtgtcacacccaccaagctgattccatccacttccacaatctggtcattgacttgtattctgccatcccgttgagcagcaccaccttctgttactgtcttgacgaatattcccagcttttcaagtccagcatctgctccaacacccattccaataatacttataccaagaccatcctcatctttctctagctccactgggaaaagttccagcttttctacacgtttttcaagttcatactcagctgaagcagccacagggtcaacttcgtcatttctcctgtcatagtcttcattggagtatgtgttgaaaaccttaataggagcactactaaacttaattttcctatttgctgggatttcttcttcttctggcaatccaacaatttccgagtactccatatcaggctgatagtaactgttctcatcactatcttcctcctcatcctgctcagtgcctgtctctccccagtctgaattatacctggatctcaccctatacacattatagtcactgtgcatgtacacatgggaaccatcaaaattatttgaatcttcaggtacttcttttccacaactggatgcagaagcatcaggagaggtgaaatcaccacctgcaagttctttcctctgttgctttgctgcctcccttccaaccaaattagcttcagcatcttctaacagttggctttgtggtgaagggatttcggactttggcattgccttactttcagcacaaggttcttcaggaccatctttgtcaatgctgtcgggagtctgttgattagatgtggagtcctcgggttccttgctctgctggatctcttcaccaggtatcgaagctagagaggtacttttagaagccacttctggtactggagttgcattactcttgtgagcatcctctgtatcaacacctcgcttgtttgaaggaggccaggaattagaatccttcaggtgaccaaatgtgtcaagatttgtaacagtaacagatggtaaattcaagggataatgcccagtcactgagtattcattgttttcagccttctcagaaatgatggcactgggagaatcagtgttctcaaatactgcactcagttgactcacagttggggagacagcctcagttcgggagctaaggctgtccaaggaatcagtactgcctctgttggacttggaacctccccattcatcctgaggttcactccctccagctttctctttctttggggaatagcggttgttctgtcctgattcatgcacacttctctcaaacatctttcgagtctcagtgaacttggaatatgaagggccatcgtacatagtgtcaaatctactaattcgttcagaaacagaagactccaacttaacaactgagccatctgttttttccagaaattctttgggcttcattcttctctgaggagatgaatgtccacctttcccccttgttttggcaatgactgcagcattctcgttgggttccatacccatctgcataaataggtttttaattctgttgacattggagccatatttcctccccctgctctgctgggagccctcaccttcttttgttttttgttccccatctgacttgggtttgtcaaaggtacttttcagtgcctgaaactcagttcgatatgcattcctgtgaggagaggcacttctgagagtggttcgttcacctgaagactcagttttcaacattttcacttcaggggtgaaaagccaatgttcataatgatcaaagaaaaaaaccaaaaaccaagatacctctcttctctaatcaccagtattgggtcaagaaaagtacctctcaaatggtatacggtgtcagtgatcgtcccaacaggtgtattaggaacttagtcacagtcaagagttacacagaatgattttttcaaagcaagactagaggttcat

SEQ ID NO: 17009 - RNA, 9078 nt, Homo sapiens
  source 1..9078: mol_type = other RNA
taggtagtttcatgttgttgggaggtgttatctggctggagtgcctcttaattctttttaaggtaatttaattatttcttgccaattgttctttcttgaatgaatgattacatccttaacagaaaacctgggtgtataaataatacagctgaaagaaacagaagtgtacaccttccaacaacatacactcccaaccacttgtgttgtttttggcaacaaccaaaatgccattgcttgcacaaaaagtaaataaatgatcatatgatggcaacattcatcataagagagccagtaggcagtgactgtaagcatcacagccaccaattatgtcattttagaattgtgagcaaattcacaagaacacacagtgcaatttttagctgcatacatttcttctgagctccaactcagcaatatgcaatcttgacatcaaagcattagccaaatatttgaggaaattttcttactaaaataccaagtatctgataaatcaattttaccaaaatatataaacatatagaaggataagtgcatttagtagaaatacttacaataaaaaaatctcttaaaatctatgagccattcaatgtatacacaacgcaagaagtggcaataaggctatgattacagctccaggtcctgactgacctcgccaagttccatacacaatatattttttaatgccatgtgattgcagtgtgtgtgcgtgtgtaaggtgggagtgatattcacacatatgtagttctgaacatctacacaaacggcatgcacattgttgagaagttatctgttctcttattgcatacatcttactcactgttgaatccctagcagttttggggttgggttagggtcaagcataggaaatcatcatatttctttccttctccactcttgaggatctggaatcaggtcacagactgtgctgggtccacacgcttacatatgtgaaccttcaagtaactaccattccctcaataggcccacatagacaccacggacaagcaaataaggaccctctgtctaccataaatagaacttgatgctttcactttccaggagaagctgattctgtcggctttctctttgcccctccaacttcttagttgggcctattctatgctgctacttcaagttactcaaatgtgttttgtctggtgttatttttttctccagtgttttggaccaagactagatttcctgagactttaaatacgcaagacaaatgcaaacaaaatctgccaacatacccaggctgcttttcaggagtgaatcactgaagcgcatttggatttcctataacactactttcttttgggaatgtacagccctcccccagctccccatcccccatcataatgtaaaccattctaatagaaaatatggatgttttggctgggggtggtggcacatgcctgtagtcccagctacttgggaagctgaagcaggaggaccacttgagcccaggagtttgaggctgcagtaagacatgatggcaccactgcagtccagtctgggtgacagatgacagaaaaaaaaaaaaaaaaagaaaagaaaagaaaatatggacattttatttctggactttatccttaaatgcttagctttagaatagtgcacaggtacatccttaataaaaagtaaatttgaaaagacaggaaaggactgtgcttttctcttccattttaccttttcattctgagaccactaaggtctttgcattaagtaggtgacgtgaaccctagtgaccactgcccaccaaaatgcccctcatctccagctctgtcaggagtacctttagttactcaaatggaaatatctcagtgtaatgatggggctacaacatatccaaagtatagatggttctctcagggctgctggggcagcttcctttagaatcctctagaacactattgttaaacactggatctcctcttgaagtttagtctgcataacctttaacacttaaacatgaatcagagtatctatataaatgcaaattttcatttcccttttataaaatgcaattttcaagcacatgctaattctggtgcacaatgaacccagacaaatttgtcttcagcacaaactctaacggccgaggtgctagatcaaaccacctgtgaccatttttgtagcttgggactgggatattttaagatttcaggctagtgatgattacagggtcacagatagtggcaaaggtaaatctggttcctcattttccctcttgccactttgtttccaacaacaatggagcaaaaggtgacagtcccattttgtgccagttgaaagctgagtttggctttagtacctatcatactgcaatcatgaactgctgtgggttaaaaaaagcttgtgatgttgagggtgtgaaatcaattgtcaatcccagctaaaggatgatagccacagaacagctttattgtcatgaaactaaagggggacttcatcaggagtgttagaatggatgaaatgaggtttcttccctaacttaacattctgcagaaaattcctgattcaggtaaaaaaagaatgagattagtattacataaactgtgagttacttgaagggagatggtcttaaacaaagtaatctgttataaaactaacatcctttaatgggaaaccctgacccagatacagctcatacaatgctttctgtctgcagcttggcctcctcaccacacattccctcccaacaaagcataacctataccccaaaacacttttggctattgttagaatcatactgagctctcctttagggaatcagttcatagcaaccagatattccctttttgttcattttctgataataaaaactgcagtttttaaggttgatgaaataacaattctgtgttaaattgtaaggacactgaaaaccactagcattaaagtaggaattgtgcaagacattggagccttgattaggtatcatgcactacagtcaataaaagaaataataggaaaacaaaatgtgcacaagatctgaggtctttcactttgctttcatacccttaatcagtttacatcttatgctttgtggggcaatcaaaccaaatgacttttacaatttcatccgttttaagtggtaatgttaaaataactcacttcggcctaaaattactataatttaacttaaaaaatcaaaatacttataatactaaatgattttaggaataagaatttgatttataacattgtcagttggacatttatctaaacattcaatatacaaagttataaagaaaaatacttctaagatatttaagaaaatgcaatataatagatcataaattaggtgcaaaaacaagacacttacagacatttccagtatatacatccattttcaaatattaccaaagtgtaaacataacttaagataatcatccttctatttctactcttgaatacagtgaaacttccagtgtgatccaggtcacttttttcccaaagataagcaaaaatggcaaaaatttacaatagcaagcactaatattaccagatttttactaatttagtgttttagtatttgaaaagttttgccaaattgtatcactcattaatagtggcttcttatttctcatgatgtgaaaaaataacaaagcaccagacatctcaagacattaatagagtatccaatacggcagtttcattatcatacccctaatgaagacagacagaaaaacataatggtgactttgataactgtaaaacacaatgttacttcatgtcaacgtttctgaggattgaatgaagggtctgtacctaatgacaaaagagctgacgcataaccgacaatactctggcaatgaaaagaaaacaggccttgggggtaaaacagaattaaaaatgtccagtttagataatttctgaattcagattttcagataaaaaaaaatcacactgttattaaaatacaagatggggctacaagggagttcccttaatctgttacactcaaaagccttgccgaggctctaaatatggaatacttctagtggaagatacgagatgctgggaacagagcagagattcccataaagtaaaagaagtaaaatactgtccaagaattcatgtggcctcaagtcttattctgaaacttgtcctttggaaagtggataacctcatttttagagtcaacgcagcaaagagaaccagatacatgagcataaaaaacaaaaaaccctcatcacatgaaatttctcaaaacgagtttattttctccttcttctgccccagtctcctgcacttgacttagtttggtgaaacatggaaatccttaatgctggcttaaaattagtataagttcctccactactaaagtatacctatgcactgccttaaacaaactttttctgtaaaattgagaatctttgaagtatggaaaggaatggttcggaaaaaccattcaaaatctctctaaaatgttaactgacagtttcctctaactggtatttctatttttcttaaaagtacatttgttaaaatactaactgagcccacctgggaaatcttgagtagaaaatatgtgatgagttcctgattgtgacataggcaggctgaagaccagccagaatgttccccaggagaggaaacctgaaaatggtggtttccttaaaaatcaatttcctgttcaatttcttgggttaggtagggggaagaggaactgtgttgtgtttgccagtgttgctgaaatgctgaacacacagcagtagcaaggtcaacagatcccaatatcccatggctgcattaatgtctgatttttttctttcttgttcagccgtatctagaggataaatattaccctcagaaccccaaggtaatacccacatccacattcttaaggcttttgcttttttcagtggttaacaaatagctataatttattttctttctttttgatgcctagcaagcagaatgacttgcttgccttttcccttagtaggtaactacagagcagagcacccatgtttccacagcggggtggtctcactgtccagactgagaattaagagcaaatctttcccacacattggagtaggtgttgcagtcctagaagttaagtactggtctcagatctcatggcagggtgctctctgccatgcagacatgtgcaattgccatttcaggatcccacactgaaaattcacggcgctccattaacaacaccagggtgtgtcatgctcttgggtggggtcacactagttctccaagtgacaaaacacacccaacacaacacaagatgttggtaagttagagaagagcaaaacacagctacttaaatgaaatctctggtttgttaatgaaccaaaggtggcttgggattattttagtagttaaaattaagagtgcattctattgcagaaaatgcagttattcaacacacagttcctcagccggcctagagccgcattacccttatcatttagtttctttttcatcctctggaggagagcagggcaggaagaggtggggacttctcttggagcatctccatcatctgtaagagggtatgtgttactgctcaccagcaccctcggctgtagttgacgtcatcttttctgtctttttggacttcctctgcatttgctcttgctcctttctccttagcttttctctttgtttttccattttctcttgggccttccgagccttctctagagacatcttcatttccttgagtttctttttgaccactgctcggtcctgggatgctgtcattccaagagccttaagtttatttccatccaactgcaggagctgttctccagtgatgttttgggcactgaattcagatacatactgctccagatttaggctcattaaccagtgagaaacctgctgcacactccattcctgaacggcccgattctgacactgactgtgtttgggagactgtccatcatcaaggatctcatctgatgacagtgctaaggactgagagagccctggtgttttaggttctgctcctaagccgctgaggtctgctgaactggtactgctgggactgaagtcatcattgaaggtaaaattctttctctctagactgtcctccccatctgtggaactaacactatcatacagtcttgtcctagagggtctctggcgtctgttcttcacagagagctgggctcgagttttcagtgcttttgaatccaggcgctctgtctctgggactgcttcattcaagtcttgacttaggccatcttggcaagatgtctgcttgccatccaagttctccatggtatcccctttagagacttcaccaagagatgttcttctctcaaagatgttgttattattgttaacttgagtcccattttgcttcagtagcctgaatacctcagcttccaaatctctaatccgcacttggaggccttgcacttccacaagatgagctttttccaaatcttctattttctttctttctgcttcctgtcttttgatgaaatcaagctctttttgttgaaaatccttgatcaacttctttgccttgttgtatttcttttccaaggcctgatactggctttgagtctctttgagatgctcattcactgtgtggcataatgtttgggcctcaatccagtagctttccaacttcaacattctttccttattctcttctatgttttgttggagttgggttttttctagttcccacctcactttctcattttctgctgcctgcagcttggtcttcaatttttgaatctctgcttctgtaactgcatgtttgatttgcaactctttgaacttgtgactgagcttgcttgtgtccagttctgatggggaaaacatgtcctcattctcaggcagctcaaagacttcaatggccatgtcgctgccaggaaggacaggtcctacctcatcttcttcttcatctgtggcatattctcctgtctcgtcatcgtcggcatcatactgggcatagtgctgttccagcagctctctctggcgcctctcctgttccagtgtctggcttatcaactgggcaacctcgctcacttgtcctggtttttcccgcccaataacaaatctgacgttgcccttggtgtttctgagaactgttgctgcaaaattctgtgtcacacccaccaagctgattccatccacttccacaatctggtcattgacttgtattctgccatcccgttgagcagcaccaccttctgttactgtcttgacgaatattcccagcttttcaagtccagcatctgctccaacacccattccaataatacttataccaagaccatcctcatctttctctagctccactgggaaaagttccagcttttctacacgtttttcaagttcatactcagctgaagcagccacagggtcaacttcgtcatttctcctgtcatagtcttcattggagtatgtgttgaaaaccttaataggagcactactaaacttaattttcctatttgctgggatttcttcttcttctggcaatccaacaatttccgagtactccatatcaggctgatagtaactgttctcatcactatcttcctcctcatcctgctcagtgcctgtctctccccagtctgaattatacctggatctcaccctatacacattatagtcactgtgcatgtacacatgggaaccatcaaaattatttgaatcttcaggtacttcttttccacaactggatgcagaagcatcaggagaggtgaaatcaccacctgcaagttctttcctctgttgctttgctgcctcccttccaaccaaattagcttcagcatcttctaacagttggctttgtggtgaagggatttcggactttggcattgccttactttcagcacaaggttcttcaggaccatctttgtcaatgctgtcgggagtctgttgattagatgtggagtcctcgggttccttgctctgctggatctcttcaccaggtatcgaagctagagaggtacttttagaagccacttctggtactggagttgcattactcttgtgagcatcctctgtatcaacacctcgcttgtttgaaggaggccaggaattagaatccttcaggtgaccaaatgtgtcaagatttgtaacagtaacagatggtaaattcaagggataatgcccagtcactgagtattcattgttttcagccttctcagaaatgatggcactgggagaatcagtgttctcaaatactgcactcagttgactcacagttggggagacagcctcagttcgggagctaaggctgtccaaggaatcagtactgcctctgttggacttggaacctccccattcatcctgaggttcactccctccagctttctctttctttggggaatagcggttgttctgtcctgattcatgcacacttctctcaaacatctttcgagtctcagtgaacttggaatatgaagggccatcgtacatagtgtcaaatctactaattcgttcagaaacagaagactccaacttaacaactgagccatctgttttttccagaaattctttgggcttcattcttctctgaggagatgaatgtccacctttcccccttgttttggcaatgactgcagcattctcgttgggttccatacccatctgcataaataggtttttaattctgttgacattggagccatatttcctccccctgctctgctgggagccctcaccttcttttgttttttgttccccatctgacttgggtttgtcaaaggtacttttcagtgcctgaaactcagttcgatatgcattcctgtgaggagaggcacttctgagagtggttcgttcacctgaagactcagttttcaacattttcacttcaggggtgaaaagccaatgttcataatgatcaaagaaaaaaaccaaaaaccaagatacctctcttctctaatcaccagtattgggtcaagaaaagtacctctcaaatggtatacggtgtcagtgatcgtcccaacaggtgtattaggaacttagtcacagtcaagagttacacagaatgattttttcaaagcaagactagaggttcatctcggctgatgggattaactctagggccgcagagagagggagcccggcagcaaaatcccgggagag

SEQ ID NO: 17010 - RNA, 9207 nt, Homo sapiens
  source 1..9207: mol_type = other RNA
taggtagtttcatgttgttgggaggtgttatctggctggagtgcctcttaattctttttaaggtaatttaattatttcttgccaattgttctttcttgaatgaatgattacatccttaacagaaaacctgggtgtataaataatacagctgaaagaaacagaagtgtacaccttccaacaacatacactcccaaccacttgtgttgtttttggcaacaaccaaaatgccattgcttgcacaaaaagtaaataaatgatcatatgatggcaacattcatcataagagagccagtaggcagtgactgtaagcatcacagccaccaattatgtcattttagaattgtgagcaaattcacaagaacacacagtgcaatttttagctgcatacatttcttctgagctccaactcagcaatatgcaatcttgacatcaaagcattagccaaatatttgaggaaattttcttactaaaataccaagtatctgataaatcaattttaccaaaatatataaacatatagaaggataagtgcatttagtagaaatacttacaataaaaaaatctcttaaaatctatgagccattcaatgtatacacaacgcaagaagtggcaataaggctatgattacagctccaggtcctgactgacctcgccaagttccatacacaatatattttttaatgccatgtgattgcagtgtgtgtgcgtgtgtaaggtgggagtgatattcacacatatgtagttctgaacatctacacaaacggcatgcacattgttgagaagttatctgttctcttattgcatacatcttactcactgttgaatccctagcagttttggggttgggttagggtcaagcataggaaatcatcatatttctttccttctccactcttgaggatctggaatcaggtcacagactgtgctgggtccacacgcttacatatgtgaaccttcaagtaactaccattccctcaataggcccacatagacaccacggacaagcaaataaggaccctctgtctaccataaatagaacttgatgctttcactttccaggagaagctgattctgtcggctttctctttgcccctccaacttcttagttgggcctattctatgctgctacttcaagttactcaaatgtgttttgtctggtgttatttttttctccagtgttttggaccaagactagatttcctgagactttaaatacgcaagacaaatgcaaacaaaatctgccaacatacccaggctgcttttcaggagtgaatcactgaagcgcatttggatttcctataacactactttcttttgggaatgtacagccctcccccagctccccatcccccatcataatgtaaaccattctaatagaaaatatggatgttttggctgggggtggtggcacatgcctgtagtcccagctacttgggaagctgaagcaggaggaccacttgagcccaggagtttgaggctgcagtaagacatgatggcaccactgcagtccagtctgggtgacagatgacagaaaaaaaaaaaaaaaaagaaaagaaaagaaaatatggacattttatttctggactttatccttaaatgcttagctttagaatagtgcacaggtacatccttaataaaaagtaaatttgaaaagacaggaaaggactgtgcttttctcttccattttaccttttcattctgagaccactaaggtctttgcattaagtaggtgacgtgaaccctagtgaccactgcccaccaaaatgcccctcatctccagctctgtcaggagtacctttagttactcaaatggaaatatctcagtgtaatgatggggctacaacatatccaaagtatagatggttctctcagggctgctggggcagcttcctttagaatcctctagaacactattgttaaacactggatctcctcttgaagtttagtctgcataacctttaacacttaaacatgaatcagagtatctatataaatgcaaattttcatttcccttttataaaatgcaattttcaagcacatgctaattctggtgcacaatgaacccagacaaatttgtcttcagcacaaactctaacggccgaggtgctagatcaaaccacctgtgaccatttttgtagcttgggactgggatattttaagatttcaggctagtgatgattacagggtcacagatagtggcaaaggtaaatctggttcctcattttccctcttgccactttgtttccaacaacaatggagcaaaaggtgacagtcccattttgtgccagttgaaagctgagtttggctttagtacctatcatactgcaatcatgaactgctgtgggttaaaaaaagcttgtgatgttgagggtgtgaaatcaattgtcaatcccagctaaaggatgatagccacagaacagctttattgtcatgaaactaaagggggacttcatcaggagtgttagaatggatgaaatgaggtttcttccctaacttaacattctgcagaaaattcctgattcaggtaaaaaaagaatgagattagtattacataaactgtgagttacttgaagggagatggtcttaaacaaagtaatctgttataaaactaacatcctttaatgggaaaccctgacccagatacagctcatacaatgctttctgtctgcagcttggcctcctcaccacacattccctcccaacaaagcataacctataccccaaaacacttttggctattgttagaatcatactgagctctcctttagggaatcagttcatagcaaccagatattccctttttgttcattttctgataataaaaactgcagtttttaaggttgatgaaataacaattctgtgttaaattgtaaggacactgaaaaccactagcattaaagtaggaattgtgcaagacattggagccttgattaggtatcatgcactacagtcaataaaagaaataataggaaaacaaaatgtgcacaagatctgaggtctttcactttgctttcatacccttaatcagtttacatcttatgctttgtggggcaatcaaaccaaatgacttttacaatttcatccgttttaagtggtaatgttaaaataactcacttcggcctaaaattactataatttaacttaaaaaatcaaaatacttataatactaaatgattttaggaataagaatttgatttataacattgtcagttggacatttatctaaacattcaatatacaaagttataaagaaaaatacttctaagatatttaagaaaatgcaatataatagatcataaattaggtgcaaaaacaagacacttacagacatttccagtatatacatccattttcaaatattaccaaagtgtaaacataacttaagataatcatccttctatttctactcttgaatacagtgaaacttccagtgtgatccaggtcacttttttcccaaagataagcaaaaatggcaaaaatttacaatagcaagcactaatattaccagatttttactaatttagtgttttagtatttgaaaagttttgccaaattgtatcactcattaatagtggcttcttatttctcatgatgtgaaaaaataacaaagcaccagacatctcaagacattaatagagtatccaatacggcagtttcattatcatacccctaatgaagacagacagaaaaacataatggtgactttgataactgtaaaacacaatgttacttcatgtcaacgtttctgaggattgaatgaagggtctgtacctaatgacaaaagagctgacgcataaccgacaatactctggcaatgaaaagaaaacaggccttgggggtaaaacagaattaaaaatgtccagtttagataatttctgaattcagattttcagataaaaaaaaatcacactgttattaaaatacaagatggggctacaagggagttcccttaatctgttacactcaaaagccttgccgaggctctaaatatggaatacttctagtggaagatacgagatgctgggaacagagcagagattcccataaagtaaaagaagtaaaatactgtccaagaattcatgtggcctcaagtcttattctgaaacttgtcctttggaaagtggataacctcatttttagagtcaacgcagcaaagagaaccagatacatgagcataaaaaacaaaaaaccctcatcacatgaaatttctcaaaacgagtttattttctccttcttctgccccagtctcctgcacttgacttagtttggtgaaacatggaaatccttaatgctggcttaaaattagtataagttcctccactactaaagtatacctatgcactgccttaaacaaactttttctgtaaaattgagaatctttgaagtatggaaaggaatggttcggaaaaaccattcaaaatctctctaaaatgttaactgacagtttcctctaactggtatttctatttttcttaaaagtacatttgttaaaatactaactgagcccacctgggaaatcttgagtagaaaatatgtgatgagttcctgattgtgacataggcaggctgaagaccagccagaatgttccccaggagaggaaacctgaaaatggtggtttccttaaaaatcaatttcctgttcaatttcttgggttaggtagggggaagaggaactgtgttgtgtttgccagtgttgctgaaatgctgaacacacagcagtagcaaggtcaacagatcccaatatcccatggctgcattaatgtctgatttttttctttcttgttcagccgtatctagaggataaatattaccctcagaaccccaaggtaatacccacatccacattcttaaggcttttgcttttttcagtggttaacaaatagctataatttattttctttctttttgatgcctagcaagcagaatgacttgcttgccttttcccttagtaggtaactacagagcagagcacccatgtttccacagcggggtggtctcactgtccagactgagaattaagagcaaatctttcccacacattggagtaggtgttgcagtcctagaagttaagtactggtctcagatctcatggcagggtgctctctgccatgcagacatgtgcaattgccatttcaggatcccacactgaaaattcacggcgctccattaacaacaccagggtgtgtcatgctcttgggtggggtcacactagttctccaagtgacaaaacacacccaacacaacacaagatgttggtaagttagagaagagcaaaacacagctacttaaatgaaatctctggtttgttaatgaaccaaaggtggcttgggattattttagtagttaaaattaagagtgcattctattgcagaaaatgcagttattcaacacacagttcctcagccggcctagagccgcattacccttatcatttagtttctttttcatcctctggaggagagcagggcaggaagaggtggggacttctcttggagcatctccatcatctgtaagagggtatgtgttactgctcaccagcaccctcggctgtagttgacgtcatcttttctgtctttttggacttcctctgcatttgctcttgctcctttctccttagcttttctctttgtttttccattttctcttgggccttccgagccttctctagagacatcttcatttccttgagtttctttttgaccactgctcggtcctgggatgctgtcattccaagagccttaagtttatttccatccaactgcaggagctgttctccagtgatgttttgggcactgaattcagatacatactgctccagatttaggctcattaaccagtgagaaacctgctgcacactccattcctgaacggcccgattctgacactgactgtgtttgggagactgtccatcatcaaggatctcatctgatgacagtgctaaggactgagagagccctggtgttttaggttctgctcctaagccgctgaggtctgctgaactggtactgctgggactgaagtcatcattgaaggtaaaattctttctctctagactgtcctccccatctgtggaactaacactatcatacagtcttgtcctagagggtctctggcgtctgttcttcacagagagctgggctcgagttttcagtgcttttgaatccaggcgctctgtctctgggactgcttcattcaagtcttgacttaggccatcttggcaagatgtctgcttgccatccaagttctccatggtatcccctttagagacttcaccaagagatgttcttctctcaaagatgttgttattattgttaacttgagtcccattttgcttcagtagcctgaatacctcagcttccaaatctctaatccgcacttggaggccttgcacttccacaagatgagctttttccaaatcttctattttctttctttctgcttcctgtcttttgatgaaatcaagctctttttgttgaaaatccttgatcaacttctttgccttgttgtatttcttttccaaggcctgatactggctttgagtctctttgagatgctcattcactgtgtggcataatgtttgggcctcaatccagtagctttccaacttcaacattctttccttattctcttctatgttttgttggagttgggttttttctagttcccacctcactttctcattttctgctgcctgcagcttggtcttcaatttttgaatctctgcttctgtaactgcatgtttgatttgcaactctttgaacttgtgactgagcttgcttgtgtccagttctgatggggaaaacatgtcctcattctcaggcagctcaaagacttcaatggccatgtcgctgccaggaaggacaggtcctacctcatcttcttcttcatctgtggcatattctcctgtcttaagaaaatagttgttattgttattgcagttgccagacattccttgcaattcagccacagtgttcccccgagtgtcatgaaatagtgctgattgtctgagagatttattgaaatcctccatggcaacctcgtcatcgtcggcatcatactgggcatagtgctgttccagcagctctctctggcgcctctcctgttccagtgtctggcttatcaactgggcaacctcgctcacttgtcctggtttttcccgcccaataacaaatctgacgttgcccttggtgtttctgagaactgttgctgcaaaattctgtgtcacacccaccaagctgattccatccacttccacaatctggtcattgacttgtattctgccatcccgttgagcagcaccaccttctgttactgtcttgacgaatattcccagcttttcaagtccagcatctgctccaacacccattccaataatacttataccaagaccatcctcatctttctctagctccactgggaaaagttccagcttttctacacgtttttcaagttcatactcagctgaagcagccacagggtcaacttcgtcatttctcctgtcatagtcttcattggagtatgtgttgaaaaccttaataggagcactactaaacttaattttcctatttgctgggatttcttcttcttctggcaatccaacaatttccgagtactccatatcaggctgatagtaactgttctcatcactatcttcctcctcatcctgctcagtgcctgtctctccccagtctgaattatacctggatctcaccctatacacattatagtcactgtgcatgtacacatgggaaccatcaaaattatttgaatcttcaggtacttcttttccacaactggatgcagaagcatcaggagaggtgaaatcaccacctgcaagttctttcctctgttgctttgctgcctcccttccaaccaaattagcttcagcatcttctaacagttggctttgtggtgaagggatttcggactttggcattgccttactttcagcacaaggttcttcaggaccatctttgtcaatgctgtcgggagtctgttgattagatgtggagtcctcgggttccttgctctgctggatctcttcaccaggtatcgaagctagagaggtacttttagaagccacttctggtactggagttgcattactcttgtgagcatcctctgtatcaacacctcgcttgtttgaaggaggccaggaattagaatccttcaggtgaccaaatgtgtcaagatttgtaacagtaacagatggtaaattcaagggataatgcccagtcactgagtattcattgttttcagccttctcagaaatgatggcactgggagaatcagtgttctcaaatactgcactcagttgactcacagttggggagacagcctcagttcgggagctaaggctgtccaaggaatcagtactgcctctgttggacttggaacctccccattcatcctgaggttcactccctccagctttctctttctttggggaatagcggttgttctgtcctgattcatgcacacttctctcaaacatctttcgagtctcagtgaacttggaatatgaagggccatcgtacatagtgtcaaatctactaattcgttcagaaacagaagactccaacttaacaactgagccatctgttttttccagaaattctttgggcttcattcttctctgaggagatgaatgtccacctttcccccttgttttggcaatgactgcagcattctcgttgggttccatacccatctgcataaataggtttttaattctgttgacattggagccatatttcctccccctgctctgctgggagccctcaccttcttttgttttttgttccccatctgacttgggtttgtcaaaggtacttttcagtgcctgaaactcagttcgatatgcattcctgtgaggagaggcacttctgagagtggttcgttcacctgaagactcagttttcaacattttcacttcaggggtgaaaagccaatgttcataatgatcaaagaaaaaaaccaaaaaccaagatacctctcttctctaatcaccagtattgggtcaagaaaagtacctctcaaatggtatacggtgtcagtgatcgtcccaacaggtgtattaggaacttagtcacagtcaagagttacacagaatgattttttcaaagcaagactagaggttcatctcggctgatgggattaactctagggccgcagagagagggagcccggcagcaaaatcccgggagag

SEQ ID NO: 17011 - RNA, 9834 nt, Homo sapiens
  source 1..9834: mol_type = other RNA
taggtagtttcatgttgttgggaggtgttatctggctggagtgcctcttaattctttttaaggtaatttaattatttcttgccaattgttctttcttgaatgaatgattacatccttaacagaaaacctgggtgtataaataatacagctgaaagaaacagaagtgtacaccttccaacaacatacactcccaaccacttgtgttgtttttggcaacaaccaaaatgccattgcttgcacaaaaagtaaataaatgatcatatgatggcaacattcatcataagagagccagtaggcagtgactgtaagcatcacagccaccaattatgtcattttagaattgtgagcaaattcacaagaacacacagtgcaatttttagctgcatacatttcttctgagctccaactcagcaatatgcaatcttgacatcaaagcattagccaaatatttgaggaaattttcttactaaaataccaagtatctgataaatcaattttaccaaaatatataaacatatagaaggataagtgcatttagtagaaatacttacaataaaaaaatctcttaaaatctatgagccattcaatgtatacacaacgcaagaagtggcaataaggctatgattacagctccaggtcctgactgacctcgccaagttccatacacaatatattttttaatgccatgtgattgcagtgtgtgtgcgtgtgtaaggtgggagtgatattcacacatatgtagttctgaacatctacacaaacggcatgcacattgttgagaagttatctgttctcttattgcatacatcttactcactgttgaatccctagcagttttggggttgggttagggtcaagcataggaaatcatcatatttctttccttctccactcttgaggatctggaatcaggtcacagactgtgctgggtccacacgcttacatatgtgaaccttcaagtaactaccattccctcaataggcccacatagacaccacggacaagcaaataaggaccctctgtctaccataaatagaacttgatgctttcactttccaggagaagctgattctgtcggctttctctttgcccctccaacttcttagttgggcctattctatgctgctacttcaagttactcaaatgtgttttgtctggtgttatttttttctccagtgttttggaccaagactagatttcctgagactttaaatacgcaagacaaatgcaaacaaaatctgccaacatacccaggctgcttttcaggagtgaatcactgaagcgcatttggatttcctataacactactttcttttgggaatgtacagccctcccccagctccccatcccccatcataatgtaaaccattctaatagaaaatatggatgttttggctgggggtggtggcacatgcctgtagtcccagctacttgggaagctgaagcaggaggaccacttgagcccaggagtttgaggctgcagtaagacatgatggcaccactgcagtccagtctgggtgacagatgacagaaaaaaaaaaaaaaaaagaaaagaaaagaaaatatggacattttatttctggactttatccttaaatgcttagctttagaatagtgcacaggtacatccttaataaaaagtaaatttgaaaagacaggaaaggactgtgcttttctcttccattttaccttttcattctgagaccactaaggtctttgcattaagtaggtgacgtgaaccctagtgaccactgcccaccaaaatgcccctcatctccagctctgtcaggagtacctttagttactcaaatggaaatatctcagtgtaatgatggggctacaacatatccaaagtatagatggttctctcagggctgctggggcagcttcctttagaatcctctagaacactattgttaaacactggatctcctcttgaagtttagtctgcataacctttaacacttaaacatgaatcagagtatctatataaatgcaaattttcatttcccttttataaaatgcaattttcaagcacatgctaattctggtgcacaatgaacccagacaaatttgtcttcagcacaaactctaacggccgaggtgctagatcaaaccacctgtgaccatttttgtagcttgggactgggatattttaagatttcaggctagtgatgattacagggtcacagatagtggcaaaggtaaatctggttcctcattttccctcttgccactttgtttccaacaacaatggagcaaaaggtgacagtcccattttgtgccagttgaaagctgagtttggctttagtacctatcatactgcaatcatgaactgctgtgggttaaaaaaagcttgtgatgttgagggtgtgaaatcaattgtcaatcccagctaaaggatgatagccacagaacagctttattgtcatgaaactaaagggggacttcatcaggagtgttagaatggatgaaatgaggtttcttccctaacttaacattctgcagaaaattcctgattcaggtaaaaaaagaatgagattagtattacataaactgtgagttacttgaagggagatggtcttaaacaaagtaatctgttataaaactaacatcctttaatgggaaaccctgacccagatacagctcatacaatgctttctgtctgcagcttggcctcctcaccacacattccctcccaacaaagcataacctataccccaaaacacttttggctattgttagaatcatactgagctctcctttagggaatcagttcatagcaaccagatattccctttttgttcattttctgataataaaaactgcagtttttaaggttgatgaaataacaattctgtgttaaattgtaaggacactgaaaaccactagcattaaagtaggaattgtgcaagacattggagccttgattaggtatcatgcactacagtcaataaaagaaataataggaaaacaaaatgtgcacaagatctgaggtctttcactttgctttcatacccttaatcagtttacatcttatgctttgtggggcaatcaaaccaaatgacttttacaatttcatccgttttaagtggtaatgttaaaataactcacttcggcctaaaattactataatttaacttaaaaaatcaaaatacttataatactaaatgattttaggaataagaatttgatttataacattgtcagttggacatttatctaaacattcaatatacaaagttataaagaaaaatacttctaagatatttaagaaaatgcaatataatagatcataaattaggtgcaaaaacaagacacttacagacatttccagtatatacatccattttcaaatattaccaaagtgtaaacataacttaagataatcatccttctatttctactcttgaatacagtgaaacttccagtgtgatccaggtcacttttttcccaaagataagcaaaaatggcaaaaatttacaatagcaagcactaatattaccagatttttactaatttagtgttttagtatttgaaaagttttgccaaattgtatcactcattaatagtggcttcttatttctcatgatgtgaaaaaataacaaagcaccagacatctcaagacattaatagagtatccaatacggcagtttcattatcatacccctaatgaagacagacagaaaaacataatggtgactttgataactgtaaaacacaatgttacttcatgtcaacgtttctgaggattgaatgaagggtctgtacctaatgacaaaagagctgacgcataaccgacaatactctggcaatgaaaagaaaacaggccttgggggtaaaacagaattaaaaatgtccagtttagataatttctgaattcagattttcagataaaaaaaaatcacactgttattaaaatacaagatggggctacaagggagttcccttaatctgttacactcaaaagccttgccgaggctctaaatatggaatacttctagtggaagatacgagatgctgggaacagagcagagattcccataaagtaaaagaagtaaaatactgtccaagaattcatgtggcctcaagtcttattctgaaacttgtcctttggaaagtggataacctcatttttagagtcaacgcagcaaagagaaccagatacatgagcataaaaaacaaaaaaccctcatcacatgaaatttctcaaaacgagtttattttctccttcttctgccccagtctcctgcacttgacttagtttggtgaaacatggaaatccttaatgctggcttaaaattagtataagttcctccactactaaagtatacctatgcactgccttaaacaaactttttctgtaaaattgagaatctttgaagtatggaaaggaatggttcggaaaaaccattcaaaatctctctaaaatgttaactgacagtttcctctaactggtatttctatttttcttaaaagtacatttgttaaaatactaactgagcccacctgggaaatcttgagtagaaaatatgtgatgagttcctgattgtgacataggcaggctgaagaccagccagaatgttccccaggagaggaaacctgaaaatggtggtttccttaaaaatcaatttcctgttcaatttcttgggttaggtagggggaagaggaactgtgttgtgtttgccagtgttgctgaaatgctgaacacacagcagtagcaaggtcaacagatcccaatatcccatggctgcattaatgtctgatttttttctttcttgttcagccgtatctagaggataaatattaccctcagaaccccaaggtaatacccacatccacattcttaaggcttttgcttttttcagtggttaacaaatagctataatttattttctttctttttgatgcctagcaagcagaatgacttgcttgccttttcccttagtaggtaactacagagcagagcacccatgtttccacagcggggtggtctcactgtccagactgagaattaagagcaaatctttcccacacattggagtaggtgttgcagtcctagaagttaagtactggtctcagatctcatggcagggtgctctctgccatgcagacatgtgcaattgccatttcaggatcccacactgaaaattcacggcgctccattaacaacaccagggtgtgtcatgctcttgggtggggtcacactagttctccaagtgacaaaacacacccaacacaacacaagatgttggtaagttagagaagagcaaaacacagctacttaaatgaaatctctggtttgttaatgaaccaaaggtggcttgggattattttagtagttaaaattaagagtgcattctattgcagaaaatgcagttattcaacacacagttcctcagccggcctagagccgcattacccttatcatttagtttctttttcatcctctggaggagagcagggcaggaagaggtggggacttctcttggagcatctccatcatctgtaagagggtatgtgttactgctcaccagcaccctcggctgtagttgacgtcatcttttctgtctttttggacttcctctgcatttgctcttgctcctttctccttagcttttctctttgtttttccattttctcttgggccttccgagccttctctagagacatcttcatttccttgagtttctttttgaccactgctcggtcctgggatgctgtcattccaagagccttaagtttatttccatccaactgcaggagctgttctccagtgatgttttgggcactgaattcagatacatactgctccagatttaggctcattaaccagtgagaaacctgctgcacactccattcctgaacggcccgattctgacactgactgtgtttgggagactgtccatcatcaaggatctcgtcatctatcatatccaggctctcatctgatgacagtgctaaggactgagagagccctggtgttttaggttctgctcctaagccgctgaggtctgctgaactggtactgctgggactgaagtcatcattgaaggtaaaattattggtttcttggatccagactacagacataagttgagaatgccttccaaagattgaagaagaggagggatttgggtttctcttgtttgcttttgtaatccatgtgttttctaccttggacccctttttatctgaaattagagtctcaggagaaggctgaagggaacttgtaggcgcaggcaggttcctgaaggaataggatcctttccggctgtcattaaaccatgagaaaggcatgcaaggggaacgagtggaggtctgagctgttgaacatggcttgggtgtccagttttccagtctgcctctgaagatcctgctacctgcagaaaacctactggcttctttttctttttctttccacttctttcccttgctggaattccttcgcaaaggcgcccccagatccacaaacttccgcttaatttttcctccttgcaccgccaatgaactggatgcccttagtgatttgggatctttggcatcatctttttctcgtaatattttcttgttggtggtttggtgatggcaaggagattcttccacatcatgatcagactttgaagtagaaaacagtgaagtgtctccccacatagaggagagaggccccatttctgggtccagtggttcttcttgaaattcagctatgtggtcagacgagaagggcacattgctatccaccggggtgaggggtggaacaccagaatctgattctggagaagacgttctcaaaccctttctctctagactgtcctccccatctgtggaactaacactatcatacagtcttgtcctagagggtctctggcgtctgttcttcacagagagctgggctcgagttttcagtgcttttgaatccaggcgctctgtctctgggactgcttcattcaagtcttgacttaggccatcttggcaagatgtctgcttgccatccaagttctccatggtatcccctttagagacttcaccaagagatgttcttctctcaaagatgttgttattattgttaacttgagtcccattttgcttcagtagcctgaatacctcagcttccaaatctctaatccgcacttggaggccttgcacttccacaagatgagctttttccaaatcttctattttctttctttctgcttcctgtcttttgatgaaatcaagctctttttgttgaaaatccttgatcaacttctttgccttgttgtatttcttttccaaggcctgatactggctttgagtctctttgagatgctcattcactgtgtggcataatgtttgggcctcaatccagtagctttccaacttcaacattctttccttattctcttctatgttttgttggagttgggttttttctagttcccacctcactttctcattttctgctgcctgcagcttggtcttcaatttttgaatctctgcttctgtaactgcatgtttgatttgcaactctttgaacttgtgactgagcttgcttgtgtccagttctgatggggaaaacatgtcctcattctcaggcagctcaaagacttcaatggccatgtcgctgccaggaaggacaggtcctacctcatcttcttcttcatctgtggcatattctcctgtctcgtcatcgtcggcatcatactgggcatagtgctgttccagcagctctctctggcgcctctcctgttccagtgtctggcttatcaactgggcaacctcgctcacttgtcctggtttttcccgcccaataacaaatctgacgttgcccttggtgtttctgagaactgttgctgcaaaattctgtgtcacacccaccaagctgattccatccacttccacaatctggtcattgacttgtattctgccatcccgttgagcagcaccaccttctgttactgtcttgacgaatattcccagcttttcaagtccagcatctgctccaacacccattccaataatacttataccaagaccatcctcatctttctctagctccactgggaaaagttccagcttttctacacgtttttcaagttcatactcagctgaagcagccacagggtcaacttcgtcatttctcctgtcatagtcttcattggagtatgtgttgaaaaccttaataggagcactactaaacttaattttcctatttgctgggatttcttcttcttctggcaatccaacaatttccgagtactccatatcaggctgatagtaactgttctcatcactatcttcctcctcatcctgctcagtgcctgtctctccccagtctgaattatacctggatctcaccctatacacattatagtcactgtgcatgtacacatgggaaccatcaaaattatttgaatcttcaggtacttcttttccacaactggatgcagaagcatcaggagaggtgaaatcaccacctgcaagttctttcctctgttgctttgctgcctcccttccaaccaaattagcttcagcatcttctaacagttggctttgtggtgaagggatttcggactttggcattgccttactttcagcacaaggttcttcaggaccatctttgtcaatgctgtcgggagtctgttgattagatgtggagtcctcgggttccttgctctgctggatctcttcaccaggtatcgaagctagagaggtacttttagaagccacttctggtactggagttgcattactcttgtgagcatcctctgtatcaacacctcgcttgtttgaaggaggccaggaattagaatccttcaggtgaccaaatgtgtcaagatttgtaacagtaacagatggtaaattcaagggataatgcccagtcactgagtattcattgttttcagccttctcagaaatgatggcactgggagaatcagtgttctcaaatactgcactcagttgactcacagttggggagacagcctcagttcgggagctaaggctgtccaaggaatcagtactgcctctgttggacttggaacctccccattcatcctgaggttcactccctccagctttctctttctttggggaatagcggttgttctgtcctgattcatgcacacttctctcaaacatctttcgagtctcagtgaacttggaatatgaagggccatcgtacatagtgtcaaatctactaattcgttcagaaacagaagactccaacttaacaactgagccatctgttttttccagaaattctttgggcttcattcttctctgaggagatgaatgtccacctttcccccttgttttggcaatgactgcagcattctcgttgggttccatacccatctgcataaataggtttttaattctgttgacattggagccatatttcctccccctgctctgctgggagccctcaccttcttttgttttttgttccccatctgacttgggtttgtcaaaggtacttttcagtgcctgaaactcagttcgatatgcattcctgtgaggagaggcacttctgagagtggttcgttcacctgaagactcagttttcaacattttcacttcaggggtgaaaagccaatgttcataatgatcaaagaaaaaaaccaaaaaccaagatacctctcttctctaatcaccagtattgggtcaagaaaagtacctctcaaatggtatacggtgtcagtgatcgtcccaacaggtgtattaggaacttagtcacagtcaagagttacacagaatgattttttcaaagcaagactagaggttcatctcggctgatgggattaactctagggccgcagagagagggagcccggcagcaaaatcccgggagag

SEQ ID NO: 17012 - RNA, 9774 nt, Homo sapiens
  source 1..9774: mol_type = other RNA
taggtagtttcatgttgttgggaggtgttatctggctggagtgcctcttaattctttttaaggtaatttaattatttcttgccaattgttctttcttgaatgaatgattacatccttaacagaaaacctgggtgtataaataatacagctgaaagaaacagaagtgtacaccttccaacaacatacactcccaaccacttgtgttgtttttggcaacaaccaaaatgccattgcttgcacaaaaagtaaataaatgatcatatgatggcaacattcatcataagagagccagtaggcagtgactgtaagcatcacagccaccaattatgtcattttagaattgtgagcaaattcacaagaacacacagtgcaatttttagctgcatacatttcttctgagctccaactcagcaatatgcaatcttgacatcaaagcattagccaaatatttgaggaaattttcttactaaaataccaagtatctgataaatcaattttaccaaaatatataaacatatagaaggataagtgcatttagtagaaatacttacaataaaaaaatctcttaaaatctatgagccattcaatgtatacacaacgcaagaagtggcaataaggctatgattacagctccaggtcctgactgacctcgccaagttccatacacaatatattttttaatgccatgtgattgcagtgtgtgtgcgtgtgtaaggtgggagtgatattcacacatatgtagttctgaacatctacacaaacggcatgcacattgttgagaagttatctgttctcttattgcatacatcttactcactgttgaatccctagcagttttggggttgggttagggtcaagcataggaaatcatcatatttctttccttctccactcttgaggatctggaatcaggtcacagactgtgctgggtccacacgcttacatatgtgaaccttcaagtaactaccattccctcaataggcccacatagacaccacggacaagcaaataaggaccctctgtctaccataaatagaacttgatgctttcactttccaggagaagctgattctgtcggctttctctttgcccctccaacttcttagttgggcctattctatgctgctacttcaagttactcaaatgtgttttgtctggtgttatttttttctccagtgttttggaccaagactagatttcctgagactttaaatacgcaagacaaatgcaaacaaaatctgccaacatacccaggctgcttttcaggagtgaatcactgaagcgcatttggatttcctataacactactttcttttgggaatgtacagccctcccccagctccccatcccccatcataatgtaaaccattctaatagaaaatatggatgttttggctgggggtggtggcacatgcctgtagtcccagctacttgggaagctgaagcaggaggaccacttgagcccaggagtttgaggctgcagtaagacatgatggcaccactgcagtccagtctgggtgacagatgacagaaaaaaaaaaaaaaaaagaaaagaaaagaaaatatggacattttatttctggactttatccttaaatgcttagctttagaatagtgcacaggtacatccttaataaaaagtaaatttgaaaagacaggaaaggactgtgcttttctcttccattttaccttttcattctgagaccactaaggtctttgcattaagtaggtgacgtgaaccctagtgaccactgcccaccaaaatgcccctcatctccagctctgtcaggagtacctttagttactcaaatggaaatatctcagtgtaatgatggggctacaacatatccaaagtatagatggttctctcagggctgctggggcagcttcctttagaatcctctagaacactattgttaaacactggatctcctcttgaagtttagtctgcataacctttaacacttaaacatgaatcagagtatctatataaatgcaaattttcatttcccttttataaaatgcaattttcaagcacatgctaattctggtgcacaatgaacccagacaaatttgtcttcagcacaaactctaacggccgaggtgctagatcaaaccacctgtgaccatttttgtagcttgggactgggatattttaagatttcaggctagtgatgattacagggtcacagatagtggcaaaggtaaatctggttcctcattttccctcttgccactttgtttccaacaacaatggagcaaaaggtgacagtcccattttgtgccagttgaaagctgagtttggctttagtacctatcatactgcaatcatgaactgctgtgggttaaaaaaagcttgtgatgttgagggtgtgaaatcaattgtcaatcccagctaaaggatgatagccacagaacagctttattgtcatgaaactaaagggggacttcatcaggagtgttagaatggatgaaatgaggtttcttccctaacttaacattctgcagaaaattcctgattcaggtaaaaaaagaatgagattagtattacataaactgtgagttacttgaagggagatggtcttaaacaaagtaatctgttataaaactaacatcctttaatgggaaaccctgacccagatacagctcatacaatgctttctgtctgcagcttggcctcctcaccacacattccctcccaacaaagcataacctataccccaaaacacttttggctattgttagaatcatactgagctctcctttagggaatcagttcatagcaaccagatattccctttttgttcattttctgataataaaaactgcagtttttaaggttgatgaaataacaattctgtgttaaattgtaaggacactgaaaaccactagcattaaagtaggaattgtgcaagacattggagccttgattaggtatcatgcactacagtcaataaaagaaataataggaaaacaaaatgtgcacaagatctgaggtctttcactttgctttcatacccttaatcagtttacatcttatgctttgtggggcaatcaaaccaaatgacttttacaatttcatccgttttaagtggtaatgttaaaataactcacttcggcctaaaattactataatttaacttaaaaaatcaaaatacttataatactaaatgattttaggaataagaatttgatttataacattgtcagttggacatttatctaaacattcaatatacaaagttataaagaaaaatacttctaagatatttaagaaaatgcaatataatagatcataaattaggtgcaaaaacaagacacttacagacatttccagtatatacatccattttcaaatattaccaaagtgtaaacataacttaagataatcatccttctatttctactcttgaatacagtgaaacttccagtgtgatccaggtcacttttttcccaaagataagcaaaaatggcaaaaatttacaatagcaagcactaatattaccagatttttactaatttagtgttttagtatttgaaaagttttgccaaattgtatcactcattaatagtggcttcttatttctcatgatgtgaaaaaataacaaagcaccagacatctcaagacattaatagagtatccaatacggcagtttcattatcatacccctaatgaagacagacagaaaaacataatggtgactttgataactgtaaaacacaatgttacttcatgtcaacgtttctgaggattgaatgaagggtctgtacctaatgacaaaagagctgacgcataaccgacaatactctggcaatgaaaagaaaacaggccttgggggtaaaacagaattaaaaatgtccagtttagataatttctgaattcagattttcagataaaaaaaaatcacactgttattaaaatacaagatggggctacaagggagttcccttaatctgttacactcaaaagccttgccgaggctctaaatatggaatacttctagtggaagatacgagatgctgggaacagagcagagattcccataaagtaaaagaagtaaaatactgtccaagaattcatgtggcctcaagtcttattctgaaacttgtcctttggaaagtggataacctcatttttagagtcaacgcagcaaagagaaccagatacatgagcataaaaaacaaaaaaccctcatcacatgaaatttctcaaaacgagtttattttctccttcttctgccccagtctcctgcacttgacttagtttggtgaaacatggaaatccttaatgctggcttaaaattagtataagttcctccactactaaagtatacctatgcactgccttaaacaaactttttctgtaaaattgagaatctttgaagtatggaaaggaatggttcggaaaaaccattcaaaatctctctaaaatgttaactgacagtttcctctaactggtatttctatttttcttaaaagtacatttgttaaaatactaactgagcccacctgggaaatcttgagtagaaaatatgtgatgagttcctgattgtgacataggcaggctgaagaccagccagaatgttccccaggagaggaaacctgaaaatggtggtttccttaaaaatcaatttcctgttcaatttcttgggttaggtagggggaagaggaactgtgttgtgtttgccagtgttgctgaaatgctgaacacacagcagtagcaaggtcaacagatcccaatatcccatggctgcattaatgtctgatttttttctttcttgttcagccgtatctagaggataaatattaccctcagaaccccaaggtaatacccacatccacattcttaaggcttttgcttttttcagtggttaacaaatagctataatttattttctttctttttgatgcctagcaagcagaatgacttgcttgccttttcccttagtaggtaactacagagcagagcacccatgtttccacagcggggtggtctcactgtccagactgagaattaagagcaaatctttcccacacattggagtaggtgttgcagtcctagaagttaagtactggtctcagatctcatggcagggtgctctctgccatgcagacatgtgcaattgccatttcaggatcccacactgaaaattcacggcgctccattaacaacaccagggtgtgtcatgctcttgggtggggtcacactagttctccaagtgacaaaacacacccaacacaacacaagatgttggtaagttagagaagagcaaaacacagctacttaaatgaaatctctggtttgttaatgaaccaaaggtggcttgggattattttagtagttaaaattaagagtgcattctattgcagaaaatgcagttattcaacacacagttcctcagccggcctagagccgcattacccttatcatttagtttctttttcatcctctggaggagagcagggcaggaagaggtggggacttctcttggagcatctccatcatctgtaagagggtatgtgttactgctcaccagcaccctcggctgtagttgacgtcatcttttctgtctttttggacttcctctgcatttgctcttgctcctttctccttagcttttctctttgtttttccattttctcttgggccttccgagccttctctagagacatcttcatttccttgagtttctttttgaccactgctcggtcctgggatgctgtcattccaagagccttaagtttatttccatccaactgcaggagctgttctccagtgatgttttgggcactgaattcagatacatactgctccagatttaggctcattaaccagtgagaaacctgctgcacactccattcctgaacggcccgattctgacactgactgtgtttgggagactgtccatcatcaaggatctcgtcatctatcatatccaggctctcatctgatgacagtgctaaggactgagagagccctggtgttttaggttctgctcctaagccgctgaggtctgctgaactggtactgctgggactgaagtcatcattgaaggtaaaattcttggacccctttttatctgaaattagagtctcaggagaaggctgaagggaacttgtaggcgcaggcaggttcctgaaggaataggatcctttccggctgtcattaaaccatgagaaaggcatgcaaggggaacgagtggaggtctgagctgttgaacatggcttgggtgtccagttttccagtctgcctctgaagatcctgctacctgcagaaaacctactggcttctttttctttttctttccacttctttcccttgctggaattccttcgcaaaggcgcccccagatccacaaacttccgcttaatttttcctccttgcaccgccaatgaactggatgcccttagtgatttgggatctttggcatcatctttttctcgtaatattttcttgttggtggtttggtgatggcaaggagattcttccacatcatgatcagactttgaagtagaaaacagtgaagtgtctccccacatagaggagagaggccccatttctgggtccagtggttcttcttgaaattcagctatgtggtcagacgagaagggcacattgctatccaccggggtgaggggtggaacaccagaatctgattctggagaagacgttctcaaacccttaggtggaagtaatttggtaatatgcatgtggttatagaaactgtttgatggctttctctctagactgtcctccccatctgtggaactaacactatcatacagtcttgtcctagagggtctctggcgtctgttcttcacagagagctgggctcgagttttcagtgcttttgaatccaggcgctctgtctctgggactgcttcattcaagtcttgacttaggccatcttggcaagatgtctgcttgccatccaagttctccatggtatcccctttagagacttcaccaagagatgttcttctctcaaagatgttgttattattgttaacttgagtcccattttgcttcagtagcctgaatacctcagcttccaaatctctaatccgcacttggaggccttgcacttccacaagatgagctttttccaaatcttctattttctttctttctgcttcctgtcttttgatgaaatcaagctctttttgttgaaaatccttgatcaacttctttgccttgttgtatttcttttccaaggcctgatactggctttgagtctctttgagatgctcattcactgtgtggcataatgtttgggcctcaatccagtagctttccaacttcaacattctttccttattctcttctatgttttgttggagttgggttttttctagttcccacctcactttctcattttctgctgcctgcagcttggtcttcaatttttgaatctctgcttctgtaactgcatgtttgatttgcaactctttgaacttgtgactgagcttgcttgtgtccagttctgatggggaaaacatgtcctcattctcaggcagctcaaagacttcaatggccatgtcgctgccaggaaggacaggtcctacctcatcttcttcttcatctgtggcatattctcctgtctcgtcatcgtcggcatcatactgggcatagtgctgttccagcagctctctctggcgcctctcctgttccagtgtctggcttatcaactgggcaacctcgctcacttgtcctggtttttcccgcccaataacaaatctgacgttgcccttggtgtttctgagaactgttgctgcaaaattctgtgtcacacccaccaagctgattccatccacttccacaatctggtcattgacttgtattctgccatcccgttgagcagcaccaccttctgttactgtcttgacgaatattcccagcttttcaagtccagcatctgctccaacacccattccaataatacttataccaagaccatcctcatctttctctagctccactgggaaaagttccagcttttctacacgtttttcaagttcatactcagctgaagcagccacagggtcaacttcgtcatttctcctgtcatagtcttcattggagtatgtgttgaaaaccttaataggagcactactaaacttaattttcctatttgctgggatttcttcttcttctggcaatccaacaatttccgagtactccatatcaggctgatagtaactgttctcatcactatcttcctcctcatcctgctcagtgcctgtctctccccagtctgaattatacctggatctcaccctatacacattatagtcactgtgcatgtacacatgggaaccatcaaaattatttgaatcttcaggtacttcttttccacaactggatgcagaagcatcaggagaggtgaaatcaccacctgcaagttctttcctctgttgctttgctgcctcccttccaaccaaattagcttcagcatcttctaacagttggctttgtggtgaagggatttcggactttggcattgccttactttcagcacaaggttcttcaggaccatctttgtcaatgctgtcgggagtctgttgattagatgtggagtcctcgggttccttgctctgctggatctcttcaccaggtatcgaagctagagaggtacttttagaagccacttctggtactggagttgcattactcttgtgagcatcctctgtatcaacacctcgcttgtttgaaggaggccaggaattagaatccttcaggtgaccaaatgtgtcaagatttgtaacagtaacagatggtaaattcaagggataatgcccagtcactgagtattcattgttttcagccttctcagaaatgatggcactgggagaatcagtgttctcaaatactgcactcagttgactcacagttggggagacagcctcagttcgggagctaaggctgtccaaggaatcagtactgcctctgttggacttggaacctccccattcatcctgaggttcactccctccagctttctctttctttggggaatagcggttgttctgtcctgattcatgcacacttctctcaaacatctttcgagtctcagtgaacttggaatatgaagggccatcgtacatagtgtcaaatctactaattcgttcagaaacagaagactccaacttaacaactgagccatctgttttttccagaaattctttgggcttcattcttctctgaggagatgaatgtccacctttcccccttgttttggcaatgactgcagcattctcgttgggttccatacccatctgcataaataggtttttaattctgttgacattggagccatatttcctccccctgctctgctgggagccctcaccttcttttgttttttgttccccatctgacttgggtttgtcaaaggtacttttcagtgcctgaaactcagttcgatatgcattcctgtgaggagaggcacttctgagagtggttcgttcacctgaagactcagttttcaacattttcacttcaggggtgaaaagccaatgttcataatgatcaaagaaaaaaaccaaaaaccaagatacctctcttctctaatcaccagtattgggtcaagaaaagtacctctcaaatggtatacggtgtcagtgatcgtcccaacaggtgtattaggaacttagtcacagtcaagagttacacagaatgattttttcaaagcaagactagaggttcatctcggctgatgggattaactctagggccgcagagagagggagcccggcagcaaaatcccgggagag

SEQ ID NO: 17013 - RNA, 9903 nt, Homo sapiens
  source 1..9903: mol_type = other RNA
taggtagtttcatgttgttgggaggtgttatctggctggagtgcctcttaattctttttaaggtaatttaattatttcttgccaattgttctttcttgaatgaatgattacatccttaacagaaaacctgggtgtataaataatacagctgaaagaaacagaagtgtacaccttccaacaacatacactcccaaccacttgtgttgtttttggcaacaaccaaaatgccattgcttgcacaaaaagtaaataaatgatcatatgatggcaacattcatcataagagagccagtaggcagtgactgtaagcatcacagccaccaattatgtcattttagaattgtgagcaaattcacaagaacacacagtgcaatttttagctgcatacatttcttctgagctccaactcagcaatatgcaatcttgacatcaaagcattagccaaatatttgaggaaattttcttactaaaataccaagtatctgataaatcaattttaccaaaatatataaacatatagaaggataagtgcatttagtagaaatacttacaataaaaaaatctcttaaaatctatgagccattcaatgtatacacaacgcaagaagtggcaataaggctatgattacagctccaggtcctgactgacctcgccaagttccatacacaatatattttttaatgccatgtgattgcagtgtgtgtgcgtgtgtaaggtgggagtgatattcacacatatgtagttctgaacatctacacaaacggcatgcacattgttgagaagttatctgttctcttattgcatacatcttactcactgttgaatccctagcagttttggggttgggttagggtcaagcataggaaatcatcatatttctttccttctccactcttgaggatctggaatcaggtcacagactgtgctgggtccacacgcttacatatgtgaaccttcaagtaactaccattccctcaataggcccacatagacaccacggacaagcaaataaggaccctctgtctaccataaatagaacttgatgctttcactttccaggagaagctgattctgtcggctttctctttgcccctccaacttcttagttgggcctattctatgctgctacttcaagttactcaaatgtgttttgtctggtgttatttttttctccagtgttttggaccaagactagatttcctgagactttaaatacgcaagacaaatgcaaacaaaatctgccaacatacccaggctgcttttcaggagtgaatcactgaagcgcatttggatttcctataacactactttcttttgggaatgtacagccctcccccagctccccatcccccatcataatgtaaaccattctaatagaaaatatggatgttttggctgggggtggtggcacatgcctgtagtcccagctacttgggaagctgaagcaggaggaccacttgagcccaggagtttgaggctgcagtaagacatgatggcaccactgcagtccagtctgggtgacagatgacagaaaaaaaaaaaaaaaaagaaaagaaaagaaaatatggacattttatttctggactttatccttaaatgcttagctttagaatagtgcacaggtacatccttaataaaaagtaaatttgaaaagacaggaaaggactgtgcttttctcttccattttaccttttcattctgagaccactaaggtctttgcattaagtaggtgacgtgaaccctagtgaccactgcccaccaaaatgcccctcatctccagctctgtcaggagtacctttagttactcaaatggaaatatctcagtgtaatgatggggctacaacatatccaaagtatagatggttctctcagggctgctggggcagcttcctttagaatcctctagaacactattgttaaacactggatctcctcttgaagtttagtctgcataacctttaacacttaaacatgaatcagagtatctatataaatgcaaattttcatttcccttttataaaatgcaattttcaagcacatgctaattctggtgcacaatgaacccagacaaatttgtcttcagcacaaactctaacggccgaggtgctagatcaaaccacctgtgaccatttttgtagcttgggactgggatattttaagatttcaggctagtgatgattacagggtcacagatagtggcaaaggtaaatctggttcctcattttccctcttgccactttgtttccaacaacaatggagcaaaaggtgacagtcccattttgtgccagttgaaagctgagtttggctttagtacctatcatactgcaatcatgaactgctgtgggttaaaaaaagcttgtgatgttgagggtgtgaaatcaattgtcaatcccagctaaaggatgatagccacagaacagctttattgtcatgaaactaaagggggacttcatcaggagtgttagaatggatgaaatgaggtttcttccctaacttaacattctgcagaaaattcctgattcaggtaaaaaaagaatgagattagtattacataaactgtgagttacttgaagggagatggtcttaaacaaagtaatctgttataaaactaacatcctttaatgggaaaccctgacccagatacagctcatacaatgctttctgtctgcagcttggcctcctcaccacacattccctcccaacaaagcataacctataccccaaaacacttttggctattgttagaatcatactgagctctcctttagggaatcagttcatagcaaccagatattccctttttgttcattttctgataataaaaactgcagtttttaaggttgatgaaataacaattctgtgttaaattgtaaggacactgaaaaccactagcattaaagtaggaattgtgcaagacattggagccttgattaggtatcatgcactacagtcaataaaagaaataataggaaaacaaaatgtgcacaagatctgaggtctttcactttgctttcatacccttaatcagtttacatcttatgctttgtggggcaatcaaaccaaatgacttttacaatttcatccgttttaagtggtaatgttaaaataactcacttcggcctaaaattactataatttaacttaaaaaatcaaaatacttataatactaaatgattttaggaataagaatttgatttataacattgtcagttggacatttatctaaacattcaatatacaaagttataaagaaaaatacttctaagatatttaagaaaatgcaatataatagatcataaattaggtgcaaaaacaagacacttacagacatttccagtatatacatccattttcaaatattaccaaagtgtaaacataacttaagataatcatccttctatttctactcttgaatacagtgaaacttccagtgtgatccaggtcacttttttcccaaagataagcaaaaatggcaaaaatttacaatagcaagcactaatattaccagatttttactaatttagtgttttagtatttgaaaagttttgccaaattgtatcactcattaatagtggcttcttatttctcatgatgtgaaaaaataacaaagcaccagacatctcaagacattaatagagtatccaatacggcagtttcattatcatacccctaatgaagacagacagaaaaacataatggtgactttgataactgtaaaacacaatgttacttcatgtcaacgtttctgaggattgaatgaagggtctgtacctaatgacaaaagagctgacgcataaccgacaatactctggcaatgaaaagaaaacaggccttgggggtaaaacagaattaaaaatgtccagtttagataatttctgaattcagattttcagataaaaaaaaatcacactgttattaaaatacaagatggggctacaagggagttcccttaatctgttacactcaaaagccttgccgaggctctaaatatggaatacttctagtggaagatacgagatgctgggaacagagcagagattcccataaagtaaaagaagtaaaatactgtccaagaattcatgtggcctcaagtcttattctgaaacttgtcctttggaaagtggataacctcatttttagagtcaacgcagcaaagagaaccagatacatgagcataaaaaacaaaaaaccctcatcacatgaaatttctcaaaacgagtttattttctccttcttctgccccagtctcctgcacttgacttagtttggtgaaacatggaaatccttaatgctggcttaaaattagtataagttcctccactactaaagtatacctatgcactgccttaaacaaactttttctgtaaaattgagaatctttgaagtatggaaaggaatggttcggaaaaaccattcaaaatctctctaaaatgttaactgacagtttcctctaactggtatttctatttttcttaaaagtacatttgttaaaatactaactgagcccacctgggaaatcttgagtagaaaatatgtgatgagttcctgattgtgacataggcaggctgaagaccagccagaatgttccccaggagaggaaacctgaaaatggtggtttccttaaaaatcaatttcctgttcaatttcttgggttaggtagggggaagaggaactgtgttgtgtttgccagtgttgctgaaatgctgaacacacagcagtagcaaggtcaacagatcccaatatcccatggctgcattaatgtctgatttttttctttcttgttcagccgtatctagaggataaatattaccctcagaaccccaaggtaatacccacatccacattcttaaggcttttgcttttttcagtggttaacaaatagctataatttattttctttctttttgatgcctagcaagcagaatgacttgcttgccttttcccttagtaggtaactacagagcagagcacccatgtttccacagcggggtggtctcactgtccagactgagaattaagagcaaatctttcccacacattggagtaggtgttgcagtcctagaagttaagtactggtctcagatctcatggcagggtgctctctgccatgcagacatgtgcaattgccatttcaggatcccacactgaaaattcacggcgctccattaacaacaccagggtgtgtcatgctcttgggtggggtcacactagttctccaagtgacaaaacacacccaacacaacacaagatgttggtaagttagagaagagcaaaacacagctacttaaatgaaatctctggtttgttaatgaaccaaaggtggcttgggattattttagtagttaaaattaagagtgcattctattgcagaaaatgcagttattcaacacacagttcctcagccggcctagagccgcattacccttatcatttagtttctttttcatcctctggaggagagcagggcaggaagaggtggggacttctcttggagcatctccatcatctgtaagagggtatgtgttactgctcaccagcaccctcggctgtagttgacgtcatcttttctgtctttttggacttcctctgcatttgctcttgctcctttctccttagcttttctctttgtttttccattttctcttgggccttccgagccttctctagagacatcttcatttccttgagtttctttttgaccactgctcggtcctgggatgctgtcattccaagagccttaagtttatttccatccaactgcaggagctgttctccagtgatgttttgggcactgaattcagatacatactgctccagatttaggctcattaaccagtgagaaacctgctgcacactccattcctgaacggcccgattctgacactgactgtgtttgggagactgtccatcatcaaggatctcgtcatctatcatatccaggctctcatctgatgacagtgctaaggactgagagagccctggtgttttaggttctgctcctaagccgctgaggtctgctgaactggtactgctgggactgaagtcatcattgaaggtaaaattcttggacccctttttatctgaaattagagtctcaggagaaggctgaagggaacttgtaggcgcaggcaggttcctgaaggaataggatcctttccggctgtcattaaaccatgagaaaggcatgcaaggggaacgagtggaggtctgagctgttgaacatggcttgggtgtccagttttccagtctgcctctgaagatcctgctacctgcagaaaacctactggcttctttttctttttctttccacttctttcccttgctggaattccttcgcaaaggcgcccccagatccacaaacttccgcttaatttttcctccttgcaccgccaatgaactggatgcccttagtgatttgggatctttggcatcatctttttctcgtaatattttcttgttggtggtttggtgatggcaaggagattcttccacatcatgatcagactttgaagtagaaaacagtgaagtgtctccccacatagaggagagaggccccatttctgggtccagtggttcttcttgaaattcagctatgtggtcagacgagaagggcacattgctatccaccggggtgaggggtggaacaccagaatctgattctggagaagacgttctcaaacccttaggtggaagtaatttggtaatatgcatgtggttatagaaactgtttgatggctttctctctagactgtcctccccatctgtggaactaacactatcatacagtcttgtcctagagggtctctggcgtctgttcttcacagagagctgggctcgagttttcagtgcttttgaatccaggcgctctgtctctgggactgcttcattcaagtcttgacttaggccatcttggcaagatgtctgcttgccatccaagttctccatggtatcccctttagagacttcaccaagagatgttcttctctcaaagatgttgttattattgttaacttgagtcccattttgcttcagtagcctgaatacctcagcttccaaatctctaatccgcacttggaggccttgcacttccacaagatgagctttttccaaatcttctattttctttctttctgcttcctgtcttttgatgaaatcaagctctttttgttgaaaatccttgatcaacttctttgccttgttgtatttcttttccaaggcctgatactggctttgagtctctttgagatgctcattcactgtgtggcataatgtttgggcctcaatccagtagctttccaacttcaacattctttccttattctcttctatgttttgttggagttgggttttttctagttcccacctcactttctcattttctgctgcctgcagcttggtcttcaatttttgaatctctgcttctgtaactgcatgtttgatttgcaactctttgaacttgtgactgagcttgcttgtgtccagttctgatggggaaaacatgtcctcattctcaggcagctcaaagacttcaatggccatgtcgctgccaggaaggacaggtcctacctcatcttcttcttcatctgtggcatattctcctgtcttaagaaaatagttgttattgttattgcagttgccagacattccttgcaattcagccacagtgttcccccgagtgtcatgaaatagtgctgattgtctgagagatttattgaaatcctccatggcaacctcgtcatcgtcggcatcatactgggcatagtgctgttccagcagctctctctggcgcctctcctgttccagtgtctggcttatcaactgggcaacctcgctcacttgtcctggtttttcccgcccaataacaaatctgacgttgcccttggtgtttctgagaactgttgctgcaaaattctgtgtcacacccaccaagctgattccatccacttccacaatctggtcattgacttgtattctgccatcccgttgagcagcaccaccttctgttactgtcttgacgaatattcccagcttttcaagtccagcatctgctccaacacccattccaataatacttataccaagaccatcctcatctttctctagctccactgggaaaagttccagcttttctacacgtttttcaagttcatactcagctgaagcagccacagggtcaacttcgtcatttctcctgtcatagtcttcattggagtatgtgttgaaaaccttaataggagcactactaaacttaattttcctatttgctgggatttcttcttcttctggcaatccaacaatttccgagtactccatatcaggctgatagtaactgttctcatcactatcttcctcctcatcctgctcagtgcctgtctctccccagtctgaattatacctggatctcaccctatacacattatagtcactgtgcatgtacacatgggaaccatcaaaattatttgaatcttcaggtacttcttttccacaactggatgcagaagcatcaggagaggtgaaatcaccacctgcaagttctttcctctgttgctttgctgcctcccttccaaccaaattagcttcagcatcttctaacagttggctttgtggtgaagggatttcggactttggcattgccttactttcagcacaaggttcttcaggaccatctttgtcaatgctgtcgggagtctgttgattagatgtggagtcctcgggttccttgctctgctggatctcttcaccaggtatcgaagctagagaggtacttttagaagccacttctggtactggagttgcattactcttgtgagcatcctctgtatcaacacctcgcttgtttgaaggaggccaggaattagaatccttcaggtgaccaaatgtgtcaagatttgtaacagtaacagatggtaaattcaagggataatgcccagtcactgagtattcattgttttcagccttctcagaaatgatggcactgggagaatcagtgttctcaaatactgcactcagttgactcacagttggggagacagcctcagttcgggagctaaggctgtccaaggaatcagtactgcctctgttggacttggaacctccccattcatcctgaggttcactccctccagctttctctttctttggggaatagcggttgttctgtcctgattcatgcacacttctctcaaacatctttcgagtctcagtgaacttggaatatgaagggccatcgtacatagtgtcaaatctactaattcgttcagaaacagaagactccaacttaacaactgagccatctgttttttccagaaattctttgggcttcattcttctctgaggagatgaatgtccacctttcccccttgttttggcaatgactgcagcattctcgttgggttccatacccatctgcataaataggtttttaattctgttgacattggagccatatttcctccccctgctctgctgggagccctcaccttcttttgttttttgttccccatctgacttgggtttgtcaaaggtacttttcagtgcctgaaactcagttcgatatgcattcctgtgaggagaggcacttctgagagtggttcgttcacctgaagactcagttttcaacattttcacttcaggggtgaaaagccaatgttcataatgatcaaagaaaaaaaccaaaaaccaagatacctctcttctctaatcaccagtattgggtcaagaaaagtacctctcaaatggtatacggtgtcagtgatcgtcccaacaggtgtattaggaacttagtcacagtcaagagttacacagaatgattttttcaaagcaagactagaggttcatctcggctgatgggattaactctagggccgcagagagagggagcccggcagcaaaatcccgggagag

SEQ ID NO: 17014 - RNA, 9157 nt, Homo sapiens
  source 1..9157: mol_type = other RNA
taggtagtttcatgttgttgggaggtgttatctggctggagtgcctcttaattctttttaaggtaatttaattatttcttgccaattgttctttcttgaatgaatgattacatccttaacagaaaacctgggtgtataaataatacagctgaaagaaacagaagtgtacaccttccaacaacatacactcccaaccacttgtgttgtttttggcaacaaccaaaatgccattgcttgcacaaaaagtaaataaatgatcatatgatggcaacattcatcataagagagccagtaggcagtgactgtaagcatcacagccaccaattatgtcattttagaattgtgagcaaattcacaagaacacacagtgcaatttttagctgcatacatttcttctgagctccaactcagcaatatgcaatcttgacatcaaagcattagccaaatatttgaggaaattttcttactaaaataccaagtatctgataaatcaattttaccaaaatatataaacatatagaaggataagtgcatttagtagaaatacttacaataaaaaaatctcttaaaatctatgagccattcaatgtatacacaacgcaagaagtggcaataaggctatgattacagctccaggtcctgactgacctcgccaagttccatacacaatatattttttaatgccatgtgattgcagtgtgtgtgcgtgtgtaaggtgggagtgatattcacacatatgtagttctgaacatctacacaaacggcatgcacattgttgagaagttatctgttctcttattgcatacatcttactcactgttgaatccctagcagttttggggttgggttagggtcaagcataggaaatcatcatatttctttccttctccactcttgaggatctggaatcaggtcacagactgtgctgggtccacacgcttacatatgtgaaccttcaagtaactaccattccctcaataggcccacatagacaccacggacaagcaaataaggaccctctgtctaccataaatagaacttgatgctttcactttccaggagaagctgattctgtcggctttctctttgcccctccaacttcttagttgggcctattctatgctgctacttcaagttactcaaatgtgttttgtctggtgttatttttttctccagtgttttggaccaagactagatttcctgagactttaaatacgcaagacaaatgcaaacaaaatctgccaacatacccaggctgcttttcaggagtgaatcactgaagcgcatttggatttcctataacactactttcttttgggaatgtacagccctcccccagctccccatcccccatcataatgtaaaccattctaatagaaaatatggatgttttggctgggggtggtggcacatgcctgtagtcccagctacttgggaagctgaagcaggaggaccacttgagcccaggagtttgaggctgcagtaagacatgatggcaccactgcagtccagtctgggtgacagatgacagaaaaaaaaaaaaaaaaagaaaagaaaagaaaatatggacattttatttctggactttatccttaaatgcttagctttagaatagtgcacaggtacatccttaataaaaagtaaatttgaaaagacaggaaaggactgtgcttttctcttccattttaccttttcattctgagaccactaaggtctttgcattaagtaggtgacgtgaaccctagtgaccactgcccaccaaaatgcccctcatctccagctctgtcaggagtacctttagttactcaaatggaaatatctcagtgtaatgatggggctacaacatatccaaagtatagatggttctctcagggctgctggggcagcttcctttagaatcctctagaacactattgttaaacactggatctcctcttgaagtttagtctgcataacctttaacacttaaacatgaatcagagtatctatataaatgcaaattttcatttcccttttataaaatgcaattttcaagcacatgctaattctggtgcacaatgaacccagacaaatttgtcttcagcacaaactctaacggccgaggtgctagatcaaaccacctgtgaccatttttgtagcttgggactgggatattttaagatttcaggctagtgatgattacagggtcacagatagtggcaaaggtaaatctggttcctcattttccctcttgccactttgtttccaacaacaatggagcaaaaggtgacagtcccattttgtgccagttgaaagctgagtttggctttagtacctatcatactgcaatcatgaactgctgtgggttaaaaaaagcttgtgatgttgagggtgtgaaatcaattgtcaatcccagctaaaggatgatagccacagaacagctttattgtcatgaaactaaagggggacttcatcaggagtgttagaatggatgaaatgaggtttcttccctaacttaacattctgcagaaaattcctgattcaggtaaaaaaagaatgagattagtattacataaactgtgagttacttgaagggagatggtcttaaacaaagtaatctgttataaaactaacatcctttaatgggaaaccctgacccagatacagctcatacaatgctttctgtctgcagcttggcctcctcaccacacattccctcccaacaaagcataacctataccccaaaacacttttggctattgttagaatcatactgagctctcctttagggaatcagttcatagcaaccagatattccctttttgttcattttctgataataaaaactgcagtttttaaggttgatgaaataacaattctgtgttaaattgtaaggacactgaaaaccactagcattaaagtaggaattgtgcaagacattggagccttgattaggtatcatgcactacagtcaataaaagaaataataggaaaacaaaatgtgcacaagatctgaggtctttcactttgctttcatacccttaatcagtttacatcttatgctttgtggggcaatcaaaccaaatgacttttacaatttcatccgttttaagtggtaatgttaaaataactcacttcggcctaaaattactataatttaacttaaaaaatcaaaatacttataatactaaatgattttaggaataagaatttgatttataacattgtcagttggacatttatctaaacattcaatatacaaagttataaagaaaaatacttctaagatatttaagaaaatgcaatataatagatcataaattaggtgcaaaaacaagacacttacagacatttccagtatatacatccattttcaaatattaccaaagtgtaaacataacttaagataatcatccttctatttctactcttgaatacagtgaaacttccagtgtgatccaggtcacttttttcccaaagataagcaaaaatggcaaaaatttacaatagcaagcactaatattaccagatttttactaatttagtgttttagtatttgaaaagttttgccaaattgtatcactcattaatagtggcttcttatttctcatgatgtgaaaaaataacaaagcaccagacatctcaagacattaatagagtatccaatacggcagtttcattatcatacccctaatgaagacagacagaaaaacataatggtgactttgataactgtaaaacacaatgttacttcatgtcaacgtttctgaggattgaatgaagggtctgtacctaatgacaaaagagctgacgcataaccgacaatactctggcaatgaaaagaaaacaggccttgggggtaaaacagaattaaaaatgtccagtttagataatttctgaattcagattttcagataaaaaaaaatcacactgttattaaaatacaagatggggctacaagggagttcccttaatctgttacactcaaaagccttgccgaggctctaaatatggaatacttctagtggaagatacgagatgctgggaacagagcagagattcccataaagtaaaagaagtaaaatactgtccaagaattcatgtggcctcaagtcttattctgaaacttgtcctttggaaagtggataacctcatttttagagtcaacgcagcaaagagaaccagatacatgagcataaaaaacaaaaaaccctcatcacatgaaatttctcaaaacgagtttattttctccttcttctgccccagtctcctgcacttgacttagtttggtgaaacatggaaatccttaatgctggcttaaaattagtataagttcctccactactaaagtatacctatgcactgccttaaacaaactttttctgtaaaattgagaatctttgaagtatggaaaggaatggttcggaaaaaccattcaaaatctctctaaaatgttaactgacagtttcctctaactggtatttctatttttcttaaaagtacatttgttaaaatactaactgagcccacctgggaaatcttgagtagaaaatatgtgatgagttcctgattgtgacataggcaggctgaagaccagccagaatgttccccaggagaggaaacctgaaaatggtggtttccttaaaaatcaatttcctgttcaatttcttgggttaggtagggggaagaggaactgtgttgtgtttgccagtgttgctgaaatgctgaacacacagcagtagcaaggtcaacagatcccaatatcccatggctgcattaatgtctgatttttttctttcttgttcagccgtatctagaggataaatattaccctcagaaccccaaggtaatacccacatccacattcttaaggcttttgcttttttcagtggttaacaaatagctataatttattttctttctttttgatgcctagcaagcagaatgacttgcttgccttttcccttagtaggtaactacagagcagagcacccatgtttccacagcggggtggtctcactgtccagactgagaattaagagcaaatctttcccacacattggagtaggtgttgcagtcctagaagttaagtactggtctcagatctcatggcagggtgctctctgccatgcagacatgtgcaattgccatttcaggatcccacactgaaaattcacggcgctccattaacaacaccagggtgtgtcatgctcttgggtggggtcacactagttctccaagtgacaaaacacacccaacacaacacaagatgttggtaagttagagaagagcaaaacacagctacttaaatgaaatctctggtttgttaatgaaccaaaggtggcttgggattattttagtagttaaaattaagagtgcattctattgcagaaaatgcagttattcaacacacagttcctcagccggcctagagccgcattacccttatcatttagtttctttttcatcctctggaggagagcagggcaggaagaggtggggacttctcttggagcatctccatcatctgtaagagggtatgtgttactgctcaccagcaccctcggctgtagttgacgtcatcttttctgtctttttggacttcctctgcatttgctcttgctcctttctccttagcttttctctttgtttttccattttctcttgggccttccgagccttctctagagacatcttcatttccttgagtttctttttgaccactgctcggtcctgggatgctgtcattccaagagccttaagtttatttccatccaactgcaggagctgttctccagtgatgttttgggcactgaattcagatacatactgctccagatttaggctcattaaccagtgagaaacctgctgcacactccattcctgaacggcccgattctgacactgactgtgtttgggagactgtccatcatcaaggatctcgtcatctatcatatccaggctctcatctgatgacagtgctaaggactgagagagccctggtgttttaggttctgctcctaagccgctgaggtctgctgaactggtactgctgggactgaagtcatcattgaaggtaaaattctttctctctagactgtcctccccatctgtggaactaacactatcatacagtcttgtcctagagggtctctggcgtctgttcttcacagagagctgggctcgagttttcagtgcttttgaatccaggcgctctgtctctgggactgcttcattcaagtcttgacttaggccatcttggcaagatgtctgcttgccatccaagttctccatggtatcccctttagagacttcaccaagagatgttcttctctcaaagatgttgttattattgttaacttgagtcccattttgcttcagtagcctgaatacctcagcttccaaatctctaatccgcacttggaggccttgcacttccacaagatgagctttttccaaatcttctattttctttctttctgcttcctgtcttttgatgaaatcaagctctttttgttgaaaatccttgatcaacttctttgccttgttgtatttcttttccaaggcctgatactggctttgagtctctttgagatgctcattcactgtgtggcataatgtttgggcctcaatccagtagctttccaacttcaacattctttccttattctcttctatgttttgttggagttgggttttttctagttcccacctcactttctcattttctgctgcctgcagcttggtcttcaatttttgaatctctgcttctgtaactgcatgtttgatttgcaactctttgaacttgtgactgagcttgcttgtgtccagttctgatggggaaaacatgtcctcattctcaggcagctcaaagacttcaatggccatgtcgctgccaggaaggacaggtcctacctcatcttcttcttcatctgtggcatattctcctgtctcgtcatcgtcggcatcatactgggcatagtgctgttccagcagctctctctggcgcctctcctgttccagtgtctggcttatcaactgggcaacctcgctcacttgtcctggtttttcccgcccaataacaaatctgacgttgcccttggtgtttctgagaactgttgctgcaaaattctgtgtcacacccaccaagctgattccatccacttccacaatctggtcattgacttgtattctgccatcccgttgagcagcaccaccttctgttactgtcttgacgaatattcccagcttttcaagtccagcatctgctccaacacccattccaataatacttataccaagaccatcctcatctttctctagctccactgggaaaagttccagcttttctacacgtttttcaagttcatactcagctgaagcagccacagggtcaacttcgtcatttctcctgtcatagtcttcattggagtatgtgttgaaaaccttaataggagcactactaaacttaattttcctatttgctgggatttcttcttcttctggcaatccaacaatttccgagtactccatatcaggctgatagtaactgttctcatcactatcttcctcctcatcctgctcagtgcctgtctctccccagtctgaattatacctggatctcaccctatacacattatagtcactgtgcatgtacacatgggaaccatcaaaattatttgaatcttcaggtacttcttttccacaactggatgcagaagcatcaggagaggtgaaatcaccacctgcaagttctttcctctgttgctttgctgcctcccttccaaccaaattagcttcagcatcttctaacagttggctttgtggtgaagggatttcggactttggcattgccttactttcagcacaaggttcttcaggaccatctttgtcaatgctgtcgggagtctgttgattagatgtggagtcctcgggttccttgctctgctggatctcttcaccaggtatcgaagctagagaggtacttttagaagccacttctggtactggagttgcattactcttgtgagcatcctctgtatcaacacctcgcttgtttgaaggaggccaggaattagaatccttcaggtgaccaaatgtgtcaagatttgtaacagtaacagatggtaaattcaagggataatgcccagtcactgagtattcattgttttcagccttctcagaaatgatggcactgggagaatcagtgttctcaaatactgcactcagttgactcacagttggggagacagcctcagttcgggagctaaggctgtccaaggaatcagtactgcctctgttggacttggaacctccccattcatcctgaggttcactccctccagctttctctttctttggggaatagcggttgttctgtcctgattcatgcacacttctctcaaacatctttcgagtctcagtgaacttggaatatgaagggccatcgtacatagtgtcaaatctactaattcgttcagaaacagaagactccaacttaacaactgagccatctgttttttccagaaattctttgggcttcattcttctctgaggagatgaatgtccacctttcccccttgttttggcaatgactgcagcattctcgttgggttccatacccatctgcataaataggtttttaattctgttgacattggagccatatttcctccccctgctctgctgggagccctcaccttcttttgttttttgttccccatctgacttgggtttgtcaaaggtacttttcagtgcctgaaactcagttcgatatgcattcctgtgaggagaggcacttctgagagtggttcgttcacctgaagactcagttttcaacattttcacttcaggggtgaaaagccaatgttcataatgatcaaagaaaaaaaccaaaaaccaagatacctctcttctctaatcaccagtattgggtcaagaaaagtacctctcaaatggtatacggtgtcagtgatcgtcccaacaggtgtattaggaacttagtcacagtcaagagttacacagaatgattttttcaaagcaagactagaggttcatccgagcgggagcgccgcgggcggggagggtcgggccgccgcggctcccaccccctcctcgcaggcgccccccgccccacggtggacgcggcggctcggctcggcgccggcccgctgggtac

SEQ ID NO: 17015 - RNA, 9145 nt, Homo sapiens
  source 1..9145: mol_type = other RNA
taggtagtttcatgttgttgggaggtgttatctggctggagtgcctcttaattctttttaaggtaatttaattatttcttgccaattgttctttcttgaatgaatgattacatccttaacagaaaacctgggtgtataaataatacagctgaaagaaacagaagtgtacaccttccaacaacatacactcccaaccacttgtgttgtttttggcaacaaccaaaatgccattgcttgcacaaaaagtaaataaatgatcatatgatggcaacattcatcataagagagccagtaggcagtgactgtaagcatcacagccaccaattatgtcattttagaattgtgagcaaattcacaagaacacacagtgcaatttttagctgcatacatttcttctgagctccaactcagcaatatgcaatcttgacatcaaagcattagccaaatatttgaggaaattttcttactaaaataccaagtatctgataaatcaattttaccaaaatatataaacatatagaaggataagtgcatttagtagaaatacttacaataaaaaaatctcttaaaatctatgagccattcaatgtatacacaacgcaagaagtggcaataaggctatgattacagctccaggtcctgactgacctcgccaagttccatacacaatatattttttaatgccatgtgattgcagtgtgtgtgcgtgtgtaaggtgggagtgatattcacacatatgtagttctgaacatctacacaaacggcatgcacattgttgagaagttatctgttctcttattgcatacatcttactcactgttgaatccctagcagttttggggttgggttagggtcaagcataggaaatcatcatatttctttccttctccactcttgaggatctggaatcaggtcacagactgtgctgggtccacacgcttacatatgtgaaccttcaagtaactaccattccctcaataggcccacatagacaccacggacaagcaaataaggaccctctgtctaccataaatagaacttgatgctttcactttccaggagaagctgattctgtcggctttctctttgcccctccaacttcttagttgggcctattctatgctgctacttcaagttactcaaatgtgttttgtctggtgttatttttttctccagtgttttggaccaagactagatttcctgagactttaaatacgcaagacaaatgcaaacaaaatctgccaacatacccaggctgcttttcaggagtgaatcactgaagcgcatttggatttcctataacactactttcttttgggaatgtacagccctcccccagctccccatcccccatcataatgtaaaccattctaatagaaaatatggatgttttggctgggggtggtggcacatgcctgtagtcccagctacttgggaagctgaagcaggaggaccacttgagcccaggagtttgaggctgcagtaagacatgatggcaccactgcagtccagtctgggtgacagatgacagaaaaaaaaaaaaaaaaagaaaagaaaagaaaatatggacattttatttctggactttatccttaaatgcttagctttagaatagtgcacaggtacatccttaataaaaagtaaatttgaaaagacaggaaaggactgtgcttttctcttccattttaccttttcattctgagaccactaaggtctttgcattaagtaggtgacgtgaaccctagtgaccactgcccaccaaaatgcccctcatctccagctctgtcaggagtacctttagttactcaaatggaaatatctcagtgtaatgatggggctacaacatatccaaagtatagatggttctctcagggctgctggggcagcttcctttagaatcctctagaacactattgttaaacactggatctcctcttgaagtttagtctgcataacctttaacacttaaacatgaatcagagtatctatataaatgcaaattttcatttcccttttataaaatgcaattttcaagcacatgctaattctggtgcacaatgaacccagacaaatttgtcttcagcacaaactctaacggccgaggtgctagatcaaaccacctgtgaccatttttgtagcttgggactgggatattttaagatttcaggctagtgatgattacagggtcacagatagtggcaaaggtaaatctggttcctcattttccctcttgccactttgtttccaacaacaatggagcaaaaggtgacagtcccattttgtgccagttgaaagctgagtttggctttagtacctatcatactgcaatcatgaactgctgtgggttaaaaaaagcttgtgatgttgagggtgtgaaatcaattgtcaatcccagctaaaggatgatagccacagaacagctttattgtcatgaaactaaagggggacttcatcaggagtgttagaatggatgaaatgaggtttcttccctaacttaacattctgcagaaaattcctgattcaggtaaaaaaagaatgagattagtattacataaactgtgagttacttgaagggagatggtcttaaacaaagtaatctgttataaaactaacatcctttaatgggaaaccctgacccagatacagctcatacaatgctttctgtctgcagcttggcctcctcaccacacattccctcccaacaaagcataacctataccccaaaacacttttggctattgttagaatcatactgagctctcctttagggaatcagttcatagcaaccagatattccctttttgttcattttctgataataaaaactgcagtttttaaggttgatgaaataacaattctgtgttaaattgtaaggacactgaaaaccactagcattaaagtaggaattgtgcaagacattggagccttgattaggtatcatgcactacagtcaataaaagaaataataggaaaacaaaatgtgcacaagatctgaggtctttcactttgctttcatacccttaatcagtttacatcttatgctttgtggggcaatcaaaccaaatgacttttacaatttcatccgttttaagtggtaatgttaaaataactcacttcggcctaaaattactataatttaacttaaaaaatcaaaatacttataatactaaatgattttaggaataagaatttgatttataacattgtcagttggacatttatctaaacattcaatatacaaagttataaagaaaaatacttctaagatatttaagaaaatgcaatataatagatcataaattaggtgcaaaaacaagacacttacagacatttccagtatatacatccattttcaaatattaccaaagtgtaaacataacttaagataatcatccttctatttctactcttgaatacagtgaaacttccagtgtgatccaggtcacttttttcccaaagataagcaaaaatggcaaaaatttacaatagcaagcactaatattaccagatttttactaatttagtgttttagtatttgaaaagttttgccaaattgtatcactcattaatagtggcttcttatttctcatgatgtgaaaaaataacaaagcaccagacatctcaagacattaatagagtatccaatacggcagtttcattatcatacccctaatgaagacagacagaaaaacataatggtgactttgataactgtaaaacacaatgttacttcatgtcaacgtttctgaggattgaatgaagggtctgtacctaatgacaaaagagctgacgcataaccgacaatactctggcaatgaaaagaaaacaggccttgggggtaaaacagaattaaaaatgtccagtttagataatttctgaattcagattttcagataaaaaaaaatcacactgttattaaaatacaagatggggctacaagggagttcccttaatctgttacactcaaaagccttgccgaggctctaaatatggaatacttctagtggaagatacgagatgctgggaacagagcagagattcccataaagtaaaagaagtaaaatactgtccaagaattcatgtggcctcaagtcttattctgaaacttgtcctttggaaagtggataacctcatttttagagtcaacgcagcaaagagaaccagatacatgagcataaaaaacaaaaaaccctcatcacatgaaatttctcaaaacgagtttattttctccttcttctgccccagtctcctgcacttgacttagtttggtgaaacatggaaatccttaatgctggcttaaaattagtataagttcctccactactaaagtatacctatgcactgccttaaacaaactttttctgtaaaattgagaatctttgaagtatggaaaggaatggttcggaaaaaccattcaaaatctctctaaaatgttaactgacagtttcctctaactggtatttctatttttcttaaaagtacatttgttaaaatactaactgagcccacctgggaaatcttgagtagaaaatatgtgatgagttcctgattgtgacataggcaggctgaagaccagccagaatgttccccaggagaggaaacctgaaaatggtggtttccttaaaaatcaatttcctgttcaatttcttgggttaggtagggggaagaggaactgtgttgtgtttgccagtgttgctgaaatgctgaacacacagcagtagcaaggtcaacagatcccaatatcccatggctgcattaatgtctgatttttttctttcttgttcagccgtatctagaggataaatattaccctcagaaccccaaggtaatacccacatccacattcttaaggcttttgcttttttcagtggttaacaaatagctataatttattttctttctttttgatgcctagcaagcagaatgacttgcttgccttttcccttagtaggtaactacagagcagagcacccatgtttccacagcggggtggtctcactgtccagactgagaattaagagcaaatctttcccacacattggagtaggtgttgcagtcctagaagttaagtactggtctcagatctcatggcagggtgctctctgccatgcagacatgtgcaattgccatttcaggatcccacactgaaaattcacggcgctccattaacaacaccagggtgtgtcatgctcttgggtggggtcacactagttctccaagtgacaaaacacacccaacacaacacaagatgttggtaagttagagaagagcaaaacacagctacttaaatgaaatctctggtttgttaatgaaccaaaggtggcttgggattattttagtagttaaaattaagagtgcattctattgcagaaaatgcagttattcaacacacagttcctcagccggcctagagccgcattacccttatcatttagtttctttttcatcctctggaggagagcagggcaggaagaggtggggacttctcttggagcatctccatcatctgtaagagggtatgtgttactgctcaccagcaccctcggctgtagttgacgtcatcttttctgtctttttggacttcctctgcatttgctcttgctcctttctccttagcttttctctttgtttttccattttctcttgggccttccgagccttctctagagacatcttcatttccttgagtttctttttgaccactgctcggtcctgggatgctgtcattccaagagccttaagtttatttccatccaactgcaggagctgttctccagtgatgttttgggcactgaattcagatacatactgctccagatttaggctcattaaccagtgagaaacctgctgcacactccattcctgaacggcccgattctgacactgactgtgtttgggagactgtccatcatcaaggatctcgtcatctatcatatccaggctctcatctgatgacagtgctaaggactgagagagccctggtgttttaggttctgctcctaagccgctgaggtctgctgaactggtactgctgggactgaagtcatcattgaaggtaaaattctttctctctagactgtcctccccatctgtggaactaacactatcatacagtcttgtcctagagggtctctggcgtctgttcttcacagagagctgggctcgagttttcagtgcttttgaatccaggcgctctgtctctgggactgcttcattcaagtcttgacttaggccatcttggcaagatgtctgcttgccatccaagttctccatggtatcccctttagagacttcaccaagagatgttcttctctcaaagatgttgttattattgttaacttgagtcccattttgcttcagtagcctgaatacctcagcttccaaatctctaatccgcacttggaggccttgcacttccacaagatgagctttttccaaatcttctattttctttctttctgcttcctgtcttttgatgaaatcaagctctttttgttgaaaatccttgatcaacttctttgccttgttgtatttcttttccaaggcctgatactggctttgagtctctttgagatgctcattcactgtgtggcataatgtttgggcctcaatccagtagctttccaacttcaacattctttccttattctcttctatgttttgttggagttgggttttttctagttcccacctcactttctcattttctgctgcctgcagcttggtcttcaatttttgaatctctgcttctgtaactgcatgtttgatttgcaactctttgaacttgtgactgagcttgcttgtgtccagttctgatggggaaaacatgtcctcattctcaggcagctcaaagacttcaatggccatgtcgctgccaggaaggacaggtcctacctcatcttcttcttcatctgtggcatattctcctgtctcgtcatcgtcggcatcatactgggcatagtgctgttccagcagctctctctggcgcctctcctgttccagtgtctggcttatcaactgggcaacctcgctcacttgtcctggtttttcccgcccaataacaaatctgacgttgcccttggtgtttctgagaactgttgctgcaaaattctgtgtcacacccaccaagctgattccatccacttccacaatctggtcattgacttgtattctgccatcccgttgagcagcaccaccttctgttactgtcttgacgaatattcccagcttttcaagtccagcatctgctccaacacccattccaataatacttataccaagaccatcctcatctttctctagctccactgggaaaagttccagcttttctacacgtttttcaagttcatactcagctgaagcagccacagggtcaacttcgtcatttctcctgtcatagtcttcattggagtatgtgttgaaaaccttaataggagcactactaaacttaattttcctatttgctgggatttcttcttcttctggcaatccaacaatttccgagtactccatatcaggctgatagtaactgttctcatcactatcttcctcctcatcctgctcagtgcctgtctctccccagtctgaattatacctggatctcaccctatacacattatagtcactgtgcatgtacacatgggaaccatcaaaattatttgaatcttcaggtacttcttttccacaactggatgcagaagcatcaggagaggtgaaatcaccacctgcaagttctttcctctgttgctttgctgcctcccttccaaccaaattagcttcagcatcttctaacagttggctttgtggtgaagggatttcggactttggcattgccttactttcagcacaaggttcttcaggaccatctttgtcaatgctgtcgggagtctgttgattagatgtggagtcctcgggttccttgctctgctggatctcttcaccaggtatcgaagctagagaggtacttttagaagccacttctggtactggagttgcattactcttgtgagcatcctctgtatcaacacctcgcttgtttgaaggaggccaggaattagaatccttcaggtgaccaaatgtgtcaagatttgtaacagtaacagatggtaaattcaagggataatgcccagtcactgagtattcattgttttcagccttctcagaaatgatggcactgggagaatcagtgttctcaaatactgcactcagttgactcacagttggggagacagcctcagttcgggagctaaggctgtccaaggaatcagtactgcctctgttggacttggaacctccccattcatcctgaggttcactccctccagctttctctttctttggggaatagcggttgttctgtcctgattcatgcacacttctctcaaacatctttcgagtctcagtgaacttggaatatgaagggccatcgtacatagtgtcaaatctactaattcgttcagaaacagaagactccaacttaacaactgagccatctgttttttccagaaattctttgggcttcattcttctctgaggagatgaatgtccacctttcccccttgttttggcaatgactgcagcattctcgttgggttccatacccatctgcataaataggtttttaattctgttgacattggagccatatttcctccccctgctctgctgggagccctcaccttcttttgttttttgttccccatctgacttgggtttgtcaaaggtacttttcagtgcctgaaactcagttcgatatgcattcctgtgaggagaggcacttctgagagtggttcgttcacctgaagactcagttttcaacattttcacttcaggggtgaaaagccaatgttcataatgatcaaagaaaaaaaccaaaaaccaagatacctctcttctctaatcaccagtattgggtcaagaaaagtacctctcaaatggtatacggtgtcagtgatcgtcccaacaggtgtattaggaacttagtcacagtcaagagttacacagaatgattttttcaaagcaagactagaggttcatctcggctgatgggattaactctagggccgcagagagagggagcccggcagcaaaatcccgggagagggagagagagggagcctctggcggccaaggaagggcgaaaagc

SEQ ID NO: 17016 - RNA, 9226 nt, Homo sapiens
  source 1..9226: mol_type = other RNA
taggtagtttcatgttgttgggaggtgttatctggctggagtgcctcttaattctttttaaggtaatttaattatttcttgccaattgttctttcttgaatgaatgattacatccttaacagaaaacctgggtgtataaataatacagctgaaagaaacagaagtgtacaccttccaacaacatacactcccaaccacttgtgttgtttttggcaacaaccaaaatgccattgcttgcacaaaaagtaaataaatgatcatatgatggcaacattcatcataagagagccagtaggcagtgactgtaagcatcacagccaccaattatgtcattttagaattgtgagcaaattcacaagaacacacagtgcaatttttagctgcatacatttcttctgagctccaactcagcaatatgcaatcttgacatcaaagcattagccaaatatttgaggaaattttcttactaaaataccaagtatctgataaatcaattttaccaaaatatataaacatatagaaggataagtgcatttagtagaaatacttacaataaaaaaatctcttaaaatctatgagccattcaatgtatacacaacgcaagaagtggcaataaggctatgattacagctccaggtcctgactgacctcgccaagttccatacacaatatattttttaatgccatgtgattgcagtgtgtgtgcgtgtgtaaggtgggagtgatattcacacatatgtagttctgaacatctacacaaacggcatgcacattgttgagaagttatctgttctcttattgcatacatcttactcactgttgaatccctagcagttttggggttgggttagggtcaagcataggaaatcatcatatttctttccttctccactcttgaggatctggaatcaggtcacagactgtgctgggtccacacgcttacatatgtgaaccttcaagtaactaccattccctcaataggcccacatagacaccacggacaagcaaataaggaccctctgtctaccataaatagaacttgatgctttcactttccaggagaagctgattctgtcggctttctctttgcccctccaacttcttagttgggcctattctatgctgctacttcaagttactcaaatgtgttttgtctggtgttatttttttctccagtgttttggaccaagactagatttcctgagactttaaatacgcaagacaaatgcaaacaaaatctgccaacatacccaggctgcttttcaggagtgaatcactgaagcgcatttggatttcctataacactactttcttttgggaatgtacagccctcccccagctccccatcccccatcataatgtaaaccattctaatagaaaatatggatgttttggctgggggtggtggcacatgcctgtagtcccagctacttgggaagctgaagcaggaggaccacttgagcccaggagtttgaggctgcagtaagacatgatggcaccactgcagtccagtctgggtgacagatgacagaaaaaaaaaaaaaaaaagaaaagaaaagaaaatatggacattttatttctggactttatccttaaatgcttagctttagaatagtgcacaggtacatccttaataaaaagtaaatttgaaaagacaggaaaggactgtgcttttctcttccattttaccttttcattctgagaccactaaggtctttgcattaagtaggtgacgtgaaccctagtgaccactgcccaccaaaatgcccctcatctccagctctgtcaggagtacctttagttactcaaatggaaatatctcagtgtaatgatggggctacaacatatccaaagtatagatggttctctcagggctgctggggcagcttcctttagaatcctctagaacactattgttaaacactggatctcctcttgaagtttagtctgcataacctttaacacttaaacatgaatcagagtatctatataaatgcaaattttcatttcccttttataaaatgcaattttcaagcacatgctaattctggtgcacaatgaacccagacaaatttgtcttcagcacaaactctaacggccgaggtgctagatcaaaccacctgtgaccatttttgtagcttgggactgggatattttaagatttcaggctagtgatgattacagggtcacagatagtggcaaaggtaaatctggttcctcattttccctcttgccactttgtttccaacaacaatggagcaaaaggtgacagtcccattttgtgccagttgaaagctgagtttggctttagtacctatcatactgcaatcatgaactgctgtgggttaaaaaaagcttgtgatgttgagggtgtgaaatcaattgtcaatcccagctaaaggatgatagccacagaacagctttattgtcatgaaactaaagggggacttcatcaggagtgttagaatggatgaaatgaggtttcttccctaacttaacattctgcagaaaattcctgattcaggtaaaaaaagaatgagattagtattacataaactgtgagttacttgaagggagatggtcttaaacaaagtaatctgttataaaactaacatcctttaatgggaaaccctgacccagatacagctcatacaatgctttctgtctgcagcttggcctcctcaccacacattccctcccaacaaagcataacctataccccaaaacacttttggctattgttagaatcatactgagctctcctttagggaatcagttcatagcaaccagatattccctttttgttcattttctgataataaaaactgcagtttttaaggttgatgaaataacaattctgtgttaaattgtaaggacactgaaaaccactagcattaaagtaggaattgtgcaagacattggagccttgattaggtatcatgcactacagtcaataaaagaaataataggaaaacaaaatgtgcacaagatctgaggtctttcactttgctttcatacccttaatcagtttacatcttatgctttgtggggcaatcaaaccaaatgacttttacaatttcatccgttttaagtggtaatgttaaaataactcacttcggcctaaaattactataatttaacttaaaaaatcaaaatacttataatactaaatgattttaggaataagaatttgatttataacattgtcagttggacatttatctaaacattcaatatacaaagttataaagaaaaatacttctaagatatttaagaaaatgcaatataatagatcataaattaggtgcaaaaacaagacacttacagacatttccagtatatacatccattttcaaatattaccaaagtgtaaacataacttaagataatcatccttctatttctactcttgaatacagtgaaacttccagtgtgatccaggtcacttttttcccaaagataagcaaaaatggcaaaaatttacaatagcaagcactaatattaccagatttttactaatttagtgttttagtatttgaaaagttttgccaaattgtatcactcattaatagtggcttcttatttctcatgatgtgaaaaaataacaaagcaccagacatctcaagacattaatagagtatccaatacggcagtttcattatcatacccctaatgaagacagacagaaaaacataatggtgactttgataactgtaaaacacaatgttacttcatgtcaacgtttctgaggattgaatgaagggtctgtacctaatgacaaaagagctgacgcataaccgacaatactctggcaatgaaaagaaaacaggccttgggggtaaaacagaattaaaaatgtccagtttagataatttctgaattcagattttcagataaaaaaaaatcacactgttattaaaatacaagatggggctacaagggagttcccttaatctgttacactcaaaagccttgccgaggctctaaatatggaatacttctagtggaagatacgagatgctgggaacagagcagagattcccataaagtaaaagaagtaaaatactgtccaagaattcatgtggcctcaagtcttattctgaaacttgtcctttggaaagtggataacctcatttttagagtcaacgcagcaaagagaaccagatacatgagcataaaaaacaaaaaaccctcatcacatgaaatttctcaaaacgagtttattttctccttcttctgccccagtctcctgcacttgacttagtttggtgaaacatggaaatccttaatgctggcttaaaattagtataagttcctccactactaaagtatacctatgcactgccttaaacaaactttttctgtaaaattgagaatctttgaagtatggaaaggaatggttcggaaaaaccattcaaaatctctctaaaatgttaactgacagtttcctctaactggtatttctatttttcttaaaagtacatttgttaaaatactaactgagcccacctgggaaatcttgagtagaaaatatgtgatgagttcctgattgtgacataggcaggctgaagaccagccagaatgttccccaggagaggaaacctgaaaatggtggtttccttaaaaatcaatttcctgttcaatttcttgggttaggtagggggaagaggaactgtgttgtgtttgccagtgttgctgaaatgctgaacacacagcagtagcaaggtcaacagatcccaatatcccatggctgcattaatgtctgatttttttctttcttgttcagccgtatctagaggataaatattaccctcagaaccccaaggtaatacccacatccacattcttaaggcttttgcttttttcagtggttaacaaatagctataatttattttctttctttttgatgcctagcaagcagaatgacttgcttgccttttcccttagtaggtaactacagagcagagcacccatgtttccacagcggggtggtctcactgtccagactgagaattaagagcaaatctttcccacacattggagtaggtgttgcagtcctagaagttaagtactggtctcagatctcatggcagggtgctctctgccatgcagacatgtgcaattgccatttcaggatcccacactgaaaattcacggcgctccattaacaacaccagggtgtgtcatgctcttgggtggggtcacactagttctccaagtgacaaaacacacccaacacaacacaagatgttggtaagttagagaagagcaaaacacagctacttaaatgaaatctctggtttgttaatgaaccaaaggtggcttgggattattttagtagttaaaattaagagtgcattctattgcagaaaatgcagttattcaacacacagttcctcagccggcctagagccgcattacccttatcatttagtttctttttcatcctctggaggagagcagggcaggaagaggtggggacttctcttggagcatctccatcatctgtaagagggtatgtgttactgctcaccagcaccctcggctgtagttgacgtcatcttttctgtctttttggacttcctctgcatttgctcttgctcctttctccttagcttttctctttgtttttccattttctcttgggccttccgagccttctctagagacatcttcatttccttgagtttctttttgaccactgctcggtcctgggatgctgtcattccaagagccttaagtttatttccatccaactgcaggagctgttctccagtgatgttttgggcactgaattcagatacatactgctccagatttaggctcattaaccagtgagaaacctgctgcacactccattcctgaacggcccgattctgacactgactgtgtttgggagactgtccatcatcaaggatctcgtcatctatcatatccaggctctcatctgatgacagtgctaaggactgagagagccctggtgttttaggttctgctcctaagccgctgaggtctgctgaactggtactgctgggactgaagtcatcattgaaggtaaaattctttctctctagactgtcctccccatctgtggaactaacactatcatacagtcttgtcctagagggtctctggcgtctgttcttcacagagagctgggctcgagttttcagtgcttttgaatccaggcgctctgtctctgggactgcttcattcaagtcttgacttaggccatcttggcaagatgtctgcttgccatccaagttctccatggtatcccctttagagacttcaccaagagatgttcttctctcaaagatgttgttattattgttaacttgagtcccattttgcttcagtagcctgaatacctcagcttccaaatctctaatccgcacttggaggccttgcacttccacaagatgagctttttccaaatcttctattttctttctttctgcttcctgtcttttgatgaaatcaagctctttttgttgaaaatccttgatcaacttctttgccttgttgtatttcttttccaaggcctgatactggctttgagtctctttgagatgctcattcactgtgtggcataatgtttgggcctcaatccagtagctttccaacttcaacattctttccttattctcttctatgttttgttggagttgggttttttctagttcccacctcactttctcattttctgctgcctgcagcttggtcttcaatttttgaatctctgcttctgtaactgcatgtttgatttgcaactctttgaacttgtgactgagcttgcttgtgtccagttctgatggggaaaacatgtcctcattctcaggcagctcaaagacttcaatggccatgtcgctgccaggaaggacaggtcctacctcatcttcttcttcatctgtggcatattctcctgtctcgtcatcgtcggcatcatactgggcatagtgctgttccagcagctctctctggcgcctctcctgttccagtgtctggcttatcaactgggcaacctcgctcacttgtcctggtttttcccgcccaataacaaatctgacgttgcccttggtgtttctgagaactgttgctgcaaaattctgtgtcacacccaccaagctgattccatccacttccacaatctggtcattgacttgtattctgccatcccgttgagcagcaccaccttctgttactgtcttgacgaatattcccagcttttcaagtccagcatctgctccaacacccattccaataatacttataccaagaccatcctcatctttctctagctccactgggaaaagttccagcttttctacacgtttttcaagttcatactcagctgaagcagccacagggtcaacttcgtcatttctcctgtcatagtcttcattggagtatgtgttgaaaaccttaataggagcactactaaacttaattttcctatttgctgggatttcttcttcttctggcaatccaacaatttccgagtactccatatcaggctgatagtaactgttctcatcactatcttcctcctcatcctgctcagtgcctgtctctccccagtctgaattatacctggatctcaccctatacacattatagtcactgtgcatgtacacatgggaaccatcaaaattatttgaatcttcaggtacttcttttccacaactggatgcagaagcatcaggagaggtgaaatcaccacctgcaagttctttcctctgttgctttgctgcctcccttccaaccaaattagcttcagcatcttctaacagttggctttgtggtgaagggatttcggactttggcattgccttactttcagcacaaggttcttcaggaccatctttgtcaatgctgtcgggagtctgttgattagatgtggagtcctcgggttccttgctctgctggatctcttcaccaggtatcgaagctagagaggtacttttagaagccacttctggtactggagttgcattactcttgtgagcatcctctgtatcaacacctcgcttgtttgaaggaggccaggaattagaatccttcaggtgaccaaatgtgtcaagatttgtaacagtaacagatggtaaattcaagggataatgcccagtcactgagtattcattgttttcagccttctcagaaatgatggcactgggagaatcagtgttctcaaatactgcactcagttgactcacagttggggagacagcctcagttcgggagctaaggctgtccaaggaatcagtactgcctctgttggacttggaacctccccattcatcctgaggttcactccctccagctttctctttctttggggaatagcggttgttctgtcctgattcatgcacacttctctcaaacatctttcgagtctcagtgaacttggaatatgaagggccatcgtacatagtgtcaaatctactaattcgttcagaaacagaagactccaacttaacaactgagccatctgttttttccagaaattctttgggcttcattcttctctgaggagatgaatgtccacctttcccccttgttttggcaatgactgcagcattctcgttgggttccatacccatctgcataaataggtttttaattctgttgacattggagccatatttcctccccctgctctgctgggagccctcaccttcttttgttttttgttccccatctgacttgggtttgtcaaaggtacttttcagtgcctgaaactcagttcgatatgcattcctgtgaggagaggcacttctgagagtggttcgttcacctgaagactcagttttcaacattttcacttcaggggtgaaaagccaatgttcataatgatcaaagaaaaaaaccaaaaaccaagatacctctcttctctaatcaccagtattgggtcaagaaaagtacctctcaaatggtatacggtgtcagtgatcgtcccaacaggtgtattaggaacttagtcacagtcaagagttacacagaatgattttttcaaagcaagactagaggttcatttgagaggcagccgattcccaagcccggttcgggacgcaatccctcggccctggggcaggaccgggagagcaggtgacgccaagcgctatggtaggaggtcgcagtctagctttgtgccaagaagcacctgaagtcctaacacattggctgcagctcccggcggctgccaggcggatcccactgtgacac

SEQ ID NO: 17017 - RNA, 9231 nt, Homo sapiens
  source 1..9231: mol_type = other RNA
taggtagtttcatgttgttgggaggtgttatctggctggagtgcctcttaattctttttaaggtaatttaattatttcttgccaattgttctttcttgaatgaatgattacatccttaacagaaaacctgggtgtataaataatacagctgaaagaaacagaagtgtacaccttccaacaacatacactcccaaccacttgtgttgtttttggcaacaaccaaaatgccattgcttgcacaaaaagtaaataaatgatcatatgatggcaacattcatcataagagagccagtaggcagtgactgtaagcatcacagccaccaattatgtcattttagaattgtgagcaaattcacaagaacacacagtgcaatttttagctgcatacatttcttctgagctccaactcagcaatatgcaatcttgacatcaaagcattagccaaatatttgaggaaattttcttactaaaataccaagtatctgataaatcaattttaccaaaatatataaacatatagaaggataagtgcatttagtagaaatacttacaataaaaaaatctcttaaaatctatgagccattcaatgtatacacaacgcaagaagtggcaataaggctatgattacagctccaggtcctgactgacctcgccaagttccatacacaatatattttttaatgccatgtgattgcagtgtgtgtgcgtgtgtaaggtgggagtgatattcacacatatgtagttctgaacatctacacaaacggcatgcacattgttgagaagttatctgttctcttattgcatacatcttactcactgttgaatccctagcagttttggggttgggttagggtcaagcataggaaatcatcatatttctttccttctccactcttgaggatctggaatcaggtcacagactgtgctgggtccacacgcttacatatgtgaaccttcaagtaactaccattccctcaataggcccacatagacaccacggacaagcaaataaggaccctctgtctaccataaatagaacttgatgctttcactttccaggagaagctgattctgtcggctttctctttgcccctccaacttcttagttgggcctattctatgctgctacttcaagttactcaaatgtgttttgtctggtgttatttttttctccagtgttttggaccaagactagatttcctgagactttaaatacgcaagacaaatgcaaacaaaatctgccaacatacccaggctgcttttcaggagtgaatcactgaagcgcatttggatttcctataacactactttcttttgggaatgtacagccctcccccagctccccatcccccatcataatgtaaaccattctaatagaaaatatggatgttttggctgggggtggtggcacatgcctgtagtcccagctacttgggaagctgaagcaggaggaccacttgagcccaggagtttgaggctgcagtaagacatgatggcaccactgcagtccagtctgggtgacagatgacagaaaaaaaaaaaaaaaaagaaaagaaaagaaaatatggacattttatttctggactttatccttaaatgcttagctttagaatagtgcacaggtacatccttaataaaaagtaaatttgaaaagacaggaaaggactgtgcttttctcttccattttaccttttcattctgagaccactaaggtctttgcattaagtaggtgacgtgaaccctagtgaccactgcccaccaaaatgcccctcatctccagctctgtcaggagtacctttagttactcaaatggaaatatctcagtgtaatgatggggctacaacatatccaaagtatagatggttctctcagggctgctggggcagcttcctttagaatcctctagaacactattgttaaacactggatctcctcttgaagtttagtctgcataacctttaacacttaaacatgaatcagagtatctatataaatgcaaattttcatttcccttttataaaatgcaattttcaagcacatgctaattctggtgcacaatgaacccagacaaatttgtcttcagcacaaactctaacggccgaggtgctagatcaaaccacctgtgaccatttttgtagcttgggactgggatattttaagatttcaggctagtgatgattacagggtcacagatagtggcaaaggtaaatctggttcctcattttccctcttgccactttgtttccaacaacaatggagcaaaaggtgacagtcccattttgtgccagttgaaagctgagtttggctttagtacctatcatactgcaatcatgaactgctgtgggttaaaaaaagcttgtgatgttgagggtgtgaaatcaattgtcaatcccagctaaaggatgatagccacagaacagctttattgtcatgaaactaaagggggacttcatcaggagtgttagaatggatgaaatgaggtttcttccctaacttaacattctgcagaaaattcctgattcaggtaaaaaaagaatgagattagtattacataaactgtgagttacttgaagggagatggtcttaaacaaagtaatctgttataaaactaacatcctttaatgggaaaccctgacccagatacagctcatacaatgctttctgtctgcagcttggcctcctcaccacacattccctcccaacaaagcataacctataccccaaaacacttttggctattgttagaatcatactgagctctcctttagggaatcagttcatagcaaccagatattccctttttgttcattttctgataataaaaactgcagtttttaaggttgatgaaataacaattctgtgttaaattgtaaggacactgaaaaccactagcattaaagtaggaattgtgcaagacattggagccttgattaggtatcatgcactacagtcaataaaagaaataataggaaaacaaaatgtgcacaagatctgaggtctttcactttgctttcatacccttaatcagtttacatcttatgctttgtggggcaatcaaaccaaatgacttttacaatttcatccgttttaagtggtaatgttaaaataactcacttcggcctaaaattactataatttaacttaaaaaatcaaaatacttataatactaaatgattttaggaataagaatttgatttataacattgtcagttggacatttatctaaacattcaatatacaaagttataaagaaaaatacttctaagatatttaagaaaatgcaatataatagatcataaattaggtgcaaaaacaagacacttacagacatttccagtatatacatccattttcaaatattaccaaagtgtaaacataacttaagataatcatccttctatttctactcttgaatacagtgaaacttccagtgtgatccaggtcacttttttcccaaagataagcaaaaatggcaaaaatttacaatagcaagcactaatattaccagatttttactaatttagtgttttagtatttgaaaagttttgccaaattgtatcactcattaatagtggcttcttatttctcatgatgtgaaaaaataacaaagcaccagacatctcaagacattaatagagtatccaatacggcagtttcattatcatacccctaatgaagacagacagaaaaacataatggtgactttgataactgtaaaacacaatgttacttcatgtcaacgtttctgaggattgaatgaagggtctgtacctaatgacaaaagagctgacgcataaccgacaatactctggcaatgaaaagaaaacaggccttgggggtaaaacagaattaaaaatgtccagtttagataatttctgaattcagattttcagataaaaaaaaatcacactgttattaaaatacaagatggggctacaagggagttcccttaatctgttacactcaaaagccttgccgaggctctaaatatggaatacttctagtggaagatacgagatgctgggaacagagcagagattcccataaagtaaaagaagtaaaatactgtccaagaattcatgtggcctcaagtcttattctgaaacttgtcctttggaaagtggataacctcatttttagagtcaacgcagcaaagagaaccagatacatgagcataaaaaacaaaaaaccctcatcacatgaaatttctcaaaacgagtttattttctccttcttctgccccagtctcctgcacttgacttagtttggtgaaacatggaaatccttaatgctggcttaaaattagtataagttcctccactactaaagtatacctatgcactgccttaaacaaactttttctgtaaaattgagaatctttgaagtatggaaaggaatggttcggaaaaaccattcaaaatctctctaaaatgttaactgacagtttcctctaactggtatttctatttttcttaaaagtacatttgttaaaatactaactgagcccacctgggaaatcttgagtagaaaatatgtgatgagttcctgattgtgacataggcaggctgaagaccagccagaatgttccccaggagaggaaacctgaaaatggtggtttccttaaaaatcaatttcctgttcaatttcttgggttaggtagggggaagaggaactgtgttgtgtttgccagtgttgctgaaatgctgaacacacagcagtagcaaggtcaacagatcccaatatcccatggctgcattaatgtctgatttttttctttcttgttcagccgtatctagaggataaatattaccctcagaaccccaaggtaatacccacatccacattcttaaggcttttgcttttttcagtggttaacaaatagctataatttattttctttctttttgatgcctagcaagcagaatgacttgcttgccttttcccttagtaggtaactacagagcagagcacccatgtttccacagcggggtggtctcactgtccagactgagaattaagagcaaatctttcccacacattggagtaggtgttgcagtcctagaagttaagtactggtctcagatctcatggcagggtgctctctgccatgcagacatgtgcaattgccatttcaggatcccacactgaaaattcacggcgctccattaacaacaccagggtgtgtcatgctcttgggtggggtcacactagttctccaagtgacaaaacacacccaacacaacacaagatgttggtaagttagagaagagcaaaacacagctacttaaatgaaatctctggtttgttaatgaaccaaaggtggcttgggattattttagtagttaaaattaagagtgcattctattgcagaaaatgcagttattcaacacacagttcctcagccggcctagagccgcattacccttatcatttagtttctttttcatcctctggaggagagcagggcaggaagaggtggggacttctcttggagcatctccatcatctgtaagagggtatgtgttactgctcaccagcaccctcggctgtagttgacgtcatcttttctgtctttttggacttcctctgcatttgctcttgctcctttctccttagcttttctctttgtttttccattttctcttgggccttccgagccttctctagagacatcttcatttccttgagtttctttttgaccactgctcggtcctgggatgctgtcattccaagagccttaagtttatttccatccaactgcaggagctgttctccagtgatgttttgggcactgaattcagatacatactgctccagatttaggctcattaaccagtgagaaacctgctgcacactccattcctgaacggcccgattctgacactgactgtgtttgggagactgtccatcatcaaggatctcgtcatctatcatatccaggctctcatctgatgacagtgctaaggactgagagagccctggtgttttaggttctgctcctaagccgctgaggtctgctgaactggtactgctgggactgaagtcatcattgaaggtaaaattctttctctctagactgtcctccccatctgtggaactaacactatcatacagtcttgtcctagagggtctctggcgtctgttcttcacagagagctgggctcgagttttcagtgcttttgaatccaggcgctctgtctctgggactgcttcattcaagtcttgacttaggccatcttggcaagatgtctgcttgccatccaagttctccatggtatcccctttagagacttcaccaagagatgttcttctctcaaagatgttgttattattgttaacttgagtcccattttgcttcagtagcctgaatacctcagcttccaaatctctaatccgcacttggaggccttgcacttccacaagatgagctttttccaaatcttctattttctttctttctgcttcctgtcttttgatgaaatcaagctctttttgttgaaaatccttgatcaacttctttgccttgttgtatttcttttccaaggcctgatactggctttgagtctctttgagatgctcattcactgtgtggcataatgtttgggcctcaatccagtagctttccaacttcaacattctttccttattctcttctatgttttgttggagttgggttttttctagttcccacctcactttctcattttctgctgcctgcagcttggtcttcaatttttgaatctctgcttctgtaactgcatgtttgatttgcaactctttgaacttgtgactgagcttgcttgtgtccagttctgatggggaaaacatgtcctcattctcaggcagctcaaagacttcaatggccatgtcgctgccaggaaggacaggtcctacctcatcttcttcttcatctgtggcatattctcctgtcttaagaaaatagttgttattgttattgcagttgccagacattccttgcaattcagccacagtgttcccccgagtgtcatgaaatagtgctgattgtctgagagatttattgaaatcctccatggcaacctcgtcatcgtcggcatcatactgggcatagtgctgttccagcagctctctctggcgcctctcctgttccagtgtctggcttatcaactgggcaacctcgctcacttgtcctggtttttcccgcccaataacaaatctgacgttgcccttggtgtttctgagaactgttgctgcaaaattctgtgtcacacccaccaagctgattccatccacttccacaatctggtcattgacttgtattctgccatcccgttgagcagcaccaccttctgttactgtcttgacgaatattcccagcttttcaagtccagcatctgctccaacacccattccaataatacttataccaagaccatcctcatctttctctagctccactgggaaaagttccagcttttctacacgtttttcaagttcatactcagctgaagcagccacagggtcaacttcgtcatttctcctgtcatagtcttcattggagtatgtgttgaaaaccttaataggagcactactaaacttaattttcctatttgctgggatttcttcttcttctggcaatccaacaatttccgagtactccatatcaggctgatagtaactgttctcatcactatcttcctcctcatcctgctcagtgcctgtctctccccagtctgaattatacctggatctcaccctatacacattatagtcactgtgcatgtacacatgggaaccatcaaaattatttgaatcttcaggtacttcttttccacaactggatgcagaagcatcaggagaggtgaaatcaccacctgcaagttctttcctctgttgctttgctgcctcccttccaaccaaattagcttcagcatcttctaacagttggctttgtggtgaagggatttcggactttggcattgccttactttcagcacaaggttcttcaggaccatctttgtcaatgctgtcgggagtctgttgattagatgtggagtcctcgggttccttgctctgctggatctcttcaccaggtatcgaagctagagaggtacttttagaagccacttctggtactggagttgcattactcttgtgagcatcctctgtatcaacacctcgcttgtttgaaggaggccaggaattagaatccttcaggtgaccaaatgtgtcaagatttgtaacagtaacagatggtaaattcaagggataatgcccagtcactgagtattcattgttttcagccttctcagaaatgatggcactgggagaatcagtgttctcaaatactgcactcagttgactcacagttggggagacagcctcagttcgggagctaaggctgtccaaggaatcagtactgcctctgttggacttggaacctccccattcatcctgaggttcactccctccagctttctctttctttggggaatagcggttgttctgtcctgattcatgcacacttctctcaaacatctttcgagtctcagtgaacttggaatatgaagggccatcgtacatagtgtcaaatctactaattcgttcagaaacagaagactccaacttaacaactgagccatctgttttttccagaaattctttgggcttcattcttctctgaggagatgaatgtccacctttcccccttgttttggcaatgactgcagcattctcgttgggttccatacccatctgcataaataggtttttaattctgttgacattggagccatatttcctccccctgctctgctgggagccctcaccttcttttgttttttgttccccatctgacttgggtttgtcaaaggtacttttcagtgcctgaaactcagttcgatatgcattcctgtgaggagaggcacttctgagagtggttcgttcacctgaagactcagttttcaacattttcacttcaggggtgaaaagccaatgttcataatgatcaaagaaaaaaaccaaaaaccaagatacctctcttctctaatcaccagtattgggtcaagaaaagtacctctcaaatggtatacggtgtcagtgatcgtcccaacaggtgtattaggaacttagtcacagtcaagagttacacagaatgattttttcaaagcaagactagaggttcatctcggctgatgggattaactctagggccgcagagagagggagcccggcagcaaaatcccgggagag

SEQ ID NO: 17018 - RNA, 338 nt, Homo sapiens
  source 1..338: mol_type = other RNA
taggtagtttcctgttgttgggatccacctttctctcgacagcacgacactgccttcattacttcagttgaaatcgtctccaggtacctctgcgcgcgggggtcgggccgggcggggcatcacggccctggtcgtgccaggcctgcggtggcaacctcggctttccctgctcaggagcctcgtgtctttctccgcagcgctttgccagccggccggctttccccttccaccacacacctccacccttctctctgtaagctcggccgctgctaggagtcgcctctcttttcttccttcttttccctgtcttcccttcctcttttatctcttctttcttt

SEQ ID NO: 17019 - RNA, 495 nt, Homo sapiens
  source 1..495: mol_type = other RNA
tagtactgtgcatatcatctataactagtgaaaatgtctactatgatgagtgtatattagtgaaggtaatgccaagtgttctaataaaagaaacccaataatataccatggcccagcacagtaatgctttgtatgttgctggaataaagtccagttgggtattcctgatcagtcggtggctctccttcaagctgtggttcaggacaagcccatttcctgggcaacagggccccttcctgggtcatctccatccagtcattttatgtgcatttttcccagcatccgtgggtgacaagtttgagaggcacaggcagcagcggccgctgcttctgttggatccaggagggaagggaggttctgagctttggagcgggaagtgaggagcctcagctgtccgcacccttttgcctgttgtgggcagcgtggtcatcacaccaaccttcacatccaacaaatgcttgcagaactgacaggcacatggcacgagcacgccgc

SEQ ID NO: 17020 - RNA, 1365 nt, Homo sapiens
  source 1..1365: mol_type = other RNA
tagtcccttccttgaagcggtccatgtggtagttgacgatgcaggccaaggactgctggtgggcttccctgctgggcaccaggcggtagcggctgatgaccgtcactgtgccattggggttccggatctcctggtactctgcctcaccttttaaccgagtttcccaggataccacactgggaggcttcccattggctgaggtgcaggtggccaccaggaccttgtcatcctgccccttcttggctcgaagcactgcctgggtaccctctatccaattggtgggtttggccatcaccgtgagattgagctggctttctcgattgcccgtagggaaggtagcaaactcgcagatgtagacaccctcatcctccagctccaggcgggagaggcggatagtgccatcggtgaaggagggccgcaggaattccacacgctcgcggtagggagccagcacggacacgcccatggatgggttgtagatggccacgttctgcttggagccattggtggacttctgccatgtgacctgggtgatcttcacgctgggaagcgggttggcaaagctgcagtgcagaaccacgtctgtgccgatgaagccatacatggagtcgttcacctggaccacctgggagtggacgcctgggaggaagaatgcggtcaagccgagagcgagtccccaccagcgtccagcggcgcccgcaagccccatccgagccatcgggggccgggggtccggcgagaggggcggcgagggcagcgctcctcgcgcagcagaaaccagcccggaagatgagggaagatcgctggcggtcggcgggcgctcgaaggatccaggtcagctgcagccgtcggccggggcggggtgggctgggtgggatccgcgcggccgcagtccgggccccgggccgccgccggctcagaggctcggcagatgcccgccgcaagttgcacgagtcatgccccttcgcctcctccgctctcctcccggcgccggtccccgccctcttcttccacgcagagcggggctggggagagggacccacccccggcgcgcccggctgcccggttgcgcggcgcgggctcctggccccggcccgctcacaccctcccgctcggctccaacttgcaggcgtccatggccggccgtcctccgagggtggcgggacgcacccgggcggcgcagaaggctcggggcccaggcggcgggcgcggggctcggcggtcggcggcccgggtggctctggctgcgcggccgggcgcgaggagaacgggtcggaggcgccgcgcgtcccagccgccgccgctctgccgggtgccggcgatccgcaacaatgtggagccgcgctcgctgctctcgctctcttt

SEQ ID NO: 17021 - RNA, 2739 nt, Homo sapiens
  source 1..2739: mol_type = other RNA
tagtggatgatgcactctgtgctcaacagaataatggcctcccaaagatgtccatgtcctaatctccaaaaggtgtcaatgttaccttacacggtaaaaaggaactttgcagatgtggttcagttaaggaccttgagatgcagagagtatcctagattacccaggtgagcccaatgtagtcacaagggggccttacaaaaaggaggctggagggtcaacgttagtggtaggagatgtgacggtgggaacagaagttggaatgatatgagaagaaaccatgagccaaggaacacatgcggcatgtggaagctgaaaatggcaaggaaacgattatcccctgaagcctcccgaaggaaccagccctgtccatatcctgattttagcacttctgacttccagagctcaataaagaagatgctggctgctgatgttgggtggtgatacatatagactgtcacaagaatggctgtggctacaatgaggaccaggatgaggattccaatgatgaggccagcgtggagggttccccctttcttctcagctgcactgtcatctgtagaagctccattatcttttagatgtagtgctatcttggtatcatcttctgtagggaggctggtgggaaactgagaagtcactgctcttctggtggtagttaggaccctgaactgggtggttgtcgctcctacggttgtggtggttcgagaagaagtttccactggttctgtattctcacacatcttctcttttgactcttcagggcatccactgtccacccagtcctgccgatgacgatcaaatccactggaacatctttgaagtttactacaccaactgcagttgaagccaatctgagaagatacacaggggccacatctgttaaactggaggcatgtgggtaatggggtcatctccacagccgaaatgttggtaatttttgacatttgtagctctactcggtggtattcataaattgttcttcttcgaacattgggaatttgttggatcctgtggacaacgacaaatgcatcggacagtccgactttcactggatgattggttgaacttatctgtgtgaccaagacaggaatttctttgtatccaaagatgattcgtccatccatgagcagggttgcctggaatgtgaagcttcccaggttataattatcctggagatgtacatggtcccactggaccacaagtgctgtgccattatcaaaatatctgacagttgaatttctggatacactgggatcgaaatttgccattaaaggtgctatgtactgtgtggctgttagcattcgatgtacgacttctccagtgtatatgaaacccccggttgccacagtgatttcacgtaggaagtggccataaaatggaaaatcgaaggacagattcactcttgcagcttgccgatgagtattggacaatattccatgaatcttcactttatctttttccatttggtctatgttcacccataaatcccggctggcagaatcagatggaccatatattcgagatatatagtaattgtggtctgtatcctcctcgatctgagtgttattgtcctgcccatcatccagcagcaggtctgtgaagcttctgggctcaggagagtcttggccgacgcttgctcggttcgtgtctaccgccttgagaaagtccaagtttcttttccacctgtggctgtacgcgtgtgaatcaacttccacctcctcctctgtgtgagggaaggcctgagtaactccatactgccaatcaaggatttggtctccgggtttcccatcggcgaactgaaactggtccgtgaagaagtggcaaagtaacataactcctgcagcggccaggtcggccttcgggaacctcgccatgccgccgccgccacctccctaccccacccgccagtccttcgccggtgctcgggggctcccgatgcaataggcacgaccgggccaaacgctgcggatcggtctcggtaggacccggaggcctttgtaaatgtcgctgcgatttcacagtagggaaccgagaagaggaagaagcgaacgcgagtaggagcgcagcgctcttcggacctctgaggctctctttgcaacttgccacactcgcagccctcacccgacactgaacaacaaccgcggggaggagaggccacttgcagccgaggctcgcaaactgtcggttccactcgggcagcgccaacccggtgcccgcggacggtgacttccgagccccagcgatgcgctccactgggttcaaaacagatctaattccacagccagcgccgctgcctgccccagatccactagggctggtcggctctgcaggaactttcctctgtctagggatggccccggcaggaggtttaggtttgcgggaaggaggttgatgacgaaaccctcccgacaagttttgcttcttttcttcgcccgacgcagggcgcgcgtcctttctcgcagccggaggaatgggcagctccaaagagctgagccctgggaaggttagggctgcagcagtctgaggtccgaagccaggaaaaaaatgtgtttaaaaaaaaaaaaaaaaaagaggaagaagaaaggaaaagggtggagtgggagggagtcacgctggaacctatcgggagagggttcctccgggctcaggaggaggtggccccaagcccccgcggagccccaggagtttggtggcggaggaggcgctgccgtcgccacgctcccccgcgctccttctcca

SEQ ID NO: 17022 - RNA, 85 nt, Homo sapiens
  source 1..85: mol_type = other RNA
tagtggtcctaaacatttcacaattgcgctacagaactgttgaactgttaagaaccactggacccagcgcgcgagtccccaacac

SEQ ID NO: 17023 - RNA, 5412 nt, Homo sapiens
  source 1..5412: mol_type = other RNA
tagtggtcctaaacatttcacagttctcaaaacttttcacataaaaggggaagattattaaagcttattagattctgtcaattggtcaaaagaaaaaatgtatttcaacacagcttgtcatctttggaaaaaatcaatcataattacgtttccttatactgaatttaaggtagagagacctaaattacaagcactcacaatttggtgggaaagtggcaaatccttgtcatttggtgactgtggcaccaaataaagaggaattcattcacaactgaatgagttattcaaataaaaaaagcagaaagctaatctagacattttaggtcctaaattaaatttttcaggtgtgatatttttagtttgagtaataatgctggtctagtttgctaaaaaattagcaacattctcctttaccttgagctgggtagactcagccacaatgtcctactgtctctttatgtatgtttaaagtaatgcctaaccagactcataatgcatgtagatgcaacatgctagttggcacaaagcaggcagggagaaatgaccctaccttcccaaaaaactcacaggagcatgaccagtaatcattttcctcatatagacaatgtcagtagatatcaagacagatacacataaagttacataaatgtttccaccttttcaccattgagtgaaacatgctgttctttggagaaaaaaatacattcatttttttcaagtatattgcaatatacaaagatgctctggctttgtttcactataaagacaaaaagatttcacatatgtccaagggaaatttcagtttacctttcctttggtgtggatttcatgaagttctgactaaaaaaattaatctaaatatacatctactcattttatctgaaagcatgaactatgttcattttatatatatatttatatgtacatagcaacaacaaaaaccagtctacatatgtccaatggcttaggattggcatgctctgatgagcacgaggtccacctgctgtgactaggcgctcagcaccagtattaggtggttccatcagcttcagggtccagccttgggccagcgacatgcaggctcttcctctctgtagtattctaaggagcactttctgctgaggccgtgcctcttcaattatggcttatttcctatcttggctttgttgttagggttgcagtttaggtctctcagcaacaggtcacaattgactagagcatccgcgggcagcagcttccggagttgctccactgtcttttgataagccattttttcttgttccagggtccggattaaagacttcattttggtctctctcgtcaaaagattttccaggtttgattccaaggcctggattttagtatgagctacctgtaatttttctaggaggtccatgttttgtcttttcagttggctattggccctctccagcttctccaaagtttcactatcctcacaggaatatgaagattcctgaagctcatcctgtagcacatgatattccacctcataggcatgcaactgcttagaaatatccatctcaaaaacctgggtaataattttttccatttcagaggtattcatatcaggtagcgtgtttttaagaaactcaacaatattttcaaagctctcacattccattataagtgtctcttggctgctcagtaggctgagtgcaaccttgaatataacttcagttccctgaagaaaaataatatcaaaaactctggctacaaatcctaatgaaaactgagaggcaaacaatgtgaggaaccagggggcagcataaagactggggctgatttcattttcttcaaggtgattgtagagatctctgtgatagtcatgaaggagcctggacagctggtacatttgaatctgcagcgacatcatgtcaggtctgtactgcttgcggaagccgaggtcatacatgaggaatttcagcatttcaaaggcttgctcttcactcatgtgcagaagcaggactccagccacaaagctgatcccctgacagtatcccacttctttgtccagcaaagaataggctttcaggaggttaaacagtgacagctgtcctggcccaagctgtactgaaaagtaagggtgagtaggaaacgtccttcctaaatccacgagaatcgcatgctgctgagcagtgagctgcttcaaaagttccttataggatatgtcaggaggctgttgtttattaggcaatctgtgtctgagtcggtactgtaaagccagaaactgccaaatttctcctcgtcgacttttgggaactccttctttaagaagagtatgaatatcttccatatcacatctgattttagctctgcagtttaacaacttcttatcccaagttattaagacctctttctgacatgcaccaacttcttcatagtctaatttaacttttctggactggagttcatctctgcttgcttcaagtttctggttttctttttccattcgaagtaacaagatttgttggtgtatagcttttctccacaagctcctcagttcttttgatttctttctttcttcaatcttttctgggtcatcctccccagacaggaatacaaccagcggttcctcctccatggttggagagaggggggacagtggcagcagctcgttcctgtccaatccatcttgctgttgcattgctgagggagatttgttcatgggagaagcaaccctgaggaaaatgcgctgccgccaggagatccggcgaggagtgacagaggttcctcccacacttagggactcattgctgcaggtagatgaggtcctttttctcccttctccatcactgatttcattttcatactgtggggacagtctacctgaattctggtaaaagcttttcaggaaagagggggcagtgaaggaaggggcagagaaggaagtgtgaagacttggaagactggaggaagaattactctccttgtacatgcgtcgaactgacgaaagattgctgcactgttcactggagctctgcctcagcagaggggaacgcacaccctgagccctcccatcctgcaaattcagctttctctttgtgcttgaaggtgggtggctgaacgtgtgtgcccgtcttcgaaactgcggggagtcggaatcctcttcgggaaacgtttgccaagctgaggacggtggggacgctggcggtgtccctggtggagaatcccctggtgagtagtccttctctgaagcaagactgttggaccgttcaaaactgtccacacttccaagccgacctctcattctgttagctccccttgagaagatattttccagggagctagttaaggatctcttagctttatttttcagaatgtcaagtttgaaccttccactgcttgttgcattttctgggattgtactatttgaaatagtagaagggccttccccgatgtgcacgtgtgtcttctgcttggcttcacacagctgcctcaggtgtaaaatcacaagttcattttcttcctggtcactgactggcttcattttctgaactctttcaaagatgtcagcttgctcattatctgtcagtgatgagagatgcctctgtatcaccagcttggctcttggtgggtagagaccttcaatcctttcacagagcttatgcaaagagtgcatcgggcaggcctcacacagtttaatctgcgtcttggcactctgcagggcagccgccgtactgaaggcctgtttcagagtcagcattacctcatcaaccagagattcgctggcacactggaatacataacaaatatactggctaagtccaggctctggagactcccggcagataaagccaaagtgatccacatgctttataccctgagaacaagaggagatatctttaaaattcttttctagcacaactgatttagtgtctggactgataaggttaatctcaaatcgcccaacctggaagagcatggtcctgttcttctccgagtccgagggctggacgtgactgggtgcgctcgcgtgtctccgtcgcggctgggatttctggctgccctcgtgaactctccgttgcacgccggtgacactgctgcaccgagaccgaaactcctgctgctcatcaaagccagaatcttccaaaatccgctcagggaagcagacccgagagctggtcagggcaggctggctggccccggcaggtaagccaaggtgggtgtcggtgccgtcagcctcctccggcaggcagtctccgggggacccgggcaccaccacctccaagtcagccaggtcctctcctgggtccggaccgcgctgctccccttggatcttcaggcgctgctgttcgtgcaggctgaacttctccatgcagtcatcgatgaggcttgagggggccttcttgtgggtcacggtcacctttccacagtacaggacttcgaacttctgagagttgtaaaaggcgtcctcattatctttgctgggtttggcatcctctttcatggccgctttagataattgccttatgctgctaataacatcaggaacctggctggggtctgtggcgcggaaaacgtggcaggccatctgcgactcggggtcgtcgggctgcgccttgatcaggtaggcaaagtaggtgaggtcgtggctgttgtggatgaagcgcgagatatgctgcgccttgtgctcgaagatgaataccgccgggttgggctgcgtggccgacggactagtgccccccgaggccccagcgcccggcgcggggacgcaacgcaggaagggcgcgctgagcaccaggatcacctctcgggccgccggcgccccgcagccgcccgcctcgggcttctggctgcgcctgcggatctcggccatgagccagggcagcataggcagcgtggtcctgtggtccaggcacgaccccccaacgtaccacagccggaaccgcttatcgcttggcttcccggggccgggctgagctgagacgcccggctcgggctccagggggtgcgggaacggctcatcctgaatgcagctgggcggctccataactctcgcctcaccagggcaccgcggaggccggccgggcgcaccgcgccccccactcccgcgcagaaggcgccgccgaaactgtgccaactgccgcaccgggctcccgcgcctgcctgggagcggcgcgaccccgaactccgcgcttcagcagccctgccccatgcagcacttccacgggcgcggctcggaggctccggcggcgggcaccgaggcaagcgcccggcaggcgagggcgggttaaatgggcatcctcctccttgggctggcgcctcgggcaggacctccccttcctccgtcgcgggtttgcagggtcagaggaccacgccgagggtccccgcggccgccggctccagcgctgcagccccgctgcggccgccgcgctcgcctggggcagacac

SEQ ID NO: 17024 - RNA, 5247 nt, Homo sapiens
  source 1..5247: mol_type = other RNA
tagtggtcctaaacatttcacagttctcaaaacttttcacataaaaggggaagattattaaagcttattagattctgtcaattggtcaaaagaaaaaatgtatttcaacacagcttgtcatctttggaaaaaatcaatcataattacgtttccttatactgaatttaaggtagagagacctaaattacaagcactcacaatttggtgggaaagtggcaaatccttgtcatttggtgactgtggcaccaaataaagaggaattcattcacaactgaatgagttattcaaataaaaaaagcagaaagctaatctagacattttaggtcctaaattaaatttttcaggtgtgatatttttagtttgagtaataatgctggtctagtttgctaaaaaattagcaacattctcctttaccttgagctgggtagactcagccacaatgtcctactgtctctttatgtatgtttaaagtaatgcctaaccagactcataatgcatgtagatgcaacatgctagttggcacaaagcaggcagggagaaatgaccctaccttcccaaaaaactcacaggagcatgaccagtaatcattttcctcatatagacaatgtcagtagatatcaagacagatacacataaagttacataaatgtttccaccttttcaccattgagtgaaacatgctgttctttggagaaaaaaatacattcatttttttcaagtatattgcaatatacaaagatgctctggctttgtttcactataaagacaaaaagatttcacatatgtccaagggaaatttcagtttacctttcctttggtgtggatttcatgaagttctgactaaaaaaattaatctaaatatacatctactcattttatctgaaagcatgaactatgttcattttatatatatatttatatgtacatagcaacaacaaaaaccagtctacatatgtccaatggcttaggattggcatgctctgatgagcacgaggtccacctgctgtgactaggcgctcagcaccagtattaggtggttccatcagcttcagggtccagccttgggccagcgacatgcaggctcttcctctctgtagtattctaaggagcactttctgctgaggccgtgcctcttcaattatggcttatttcctatcttggctttgttgttagggttgcagtttaggtctctcagcaacaggtcacaattgactagagcatccgcgggcagcagcttccggagttgctccactgtcttttgataagccattttttcttgttccagggtccggattaaagacttcattttggtctctctcgtcaaaagattttccaggtttgattccaaggcctggattttagtatgagctacctgtaatttttctaggaggtccatgttttgtcttttcagttggctattggccctctccagcttctccaaagtttcactatcctcacaggaatatgaagattcctgaagctcatcctgtagcacatgatattccacctcataggcatgcaactgcttagaaatatccatctcaaaaacctgggtaataattttttccatttcagaggtattcatatcaggtagcgtgtttttaagaaactcaacaatattttcaaagctctcacattccattataagtgtctcttggctgctcagtaggctgagtgcaaccttgaatataacttcagttccctgaagaaaaataatatcaaaaactctggctacaaatcctaatgaaaactgagaggcaaacaatgtgaggaaccagggggcagcataaagactggggctgatttcattttcttcaaggtgattgtagagatctctgtgatagtcatgaaggagcctggacagctggtacatttgaatctgcagcgacatcatgtcaggtctgtactgcttgcggaagccgaggtcatacatgaggaatttcagcatttcaaaggcttgctcttcactcatgtgcagaagcaggactccagccacaaagctgatcccctgacagtatcccacttctttgtccagcaaagaataggctttcaggaggttaaacagtgacagctgtcctggcccaagctgtactgaaaagtaagggtgagtaggaaacgtccttcctaaatccacgagaatcgcatgctgctgagcagtgagctgcttcaaaagttccttataggatatgtcaggaggctgttgtttattaggcaatctgtgtctgagtcggtactgtaaagccagaaactgccaaatttctcctcgtcgacttttgggaactccttctttaagaagagtatgaatatcttccatatcacatctgattttagctctgcagtttaacaacttcttatcccaagttattaagacctctttctgacatgcaccaacttcttcatagtctaatttaacttttctggactggagttcatctctgcttgcttcaagtttctggttttctttttccattcgaagtaacaagatttgttggtgtatagcttttctccacaagctcctcagttcttttgatttctttctttcttcaatcttttctgggtcatcctccccagacaggaatacaaccagcggttcctcctccatggttggagagaggggggacagtggcagcagctcgttcctgtccaatccatcttgctgttgcattgctgagggagatttgttcatgggagaagcaaccctgaggaaaatgcgctgccgccaggagatccggcgaggagtgacagaggttcctcccacacttagggactcattgctgcaggtagatgaggtcctttttctcccttctccatcactgcactgttcactggagctctgcctcagcagaggggaacgcacaccctgagccctcccatcctgcaaattcagctttctctttgtgcttgaaggtgggtggctgaacgtgtgtgcccgtcttcgaaactgcggggagtcggaatcctcttcgggaaacgtttgccaagctgaggacggtggggacgctggcggtgtccctggtggagaatcccctggtgagtagtccttctctgaagcaagactgttggaccgttcaaaactgtccacacttccaagccgacctctcattctgttagctccccttgagaagatattttccagggagctagttaaggatctcttagctttatttttcagaatgtcaagtttgaaccttccactgcttgttgcattttctgggattgtactatttgaaatagtagaagggccttccccgatgtgcacgtgtgtcttctgcttggcttcacacagctgcctcaggtgtaaaatcacaagttcattttcttcctggtcactgactggcttcattttctgaactctttcaaagatgtcagcttgctcattatctgtcagtgatgagagatgcctctgtatcaccagcttggctcttggtgggtagagaccttcaatcctttcacagagcttatgcaaagagtgcatcgggcaggcctcacacagtttaatctgcgtcttggcactctgcagggcagccgccgtactgaaggcctgtttcagagtcagcattacctcatcaaccagagattcgctggcacactggaatacataacaaatatactggctaagtccaggctctggagactcccggcagataaagccaaagtgatccacatgctttataccctgagaacaagaggagatatctttaaaattcttttctagcacaactgatttagtgtctggactgataaggttaatctcaaatcgcccaacctggaagagcatggtcctgttcttctccgagtccgagggctggacgtgactgggtgcgctcgcgtgtctccgtcgcggctgggatttctggctgccctcgtgaactctccgttgcacgccggtgacactgctgcaccgagaccgaaactcctgctgctcatcaaagccagaatcttccaaaatccgctcagggaagcagacccgagagctggtcagggcaggctggctggccccggcaggtaagccaaggtgggtgtcggtgccgtcagcctcctccggcaggcagtctccgggggacccgggcaccaccacctccaagtcagccaggtcctctcctgggtccggaccgcgctgctccccttggatcttcaggcgctgctgttcgtgcaggctgaacttctccatgcagtcatcgatgaggcttgagggggccttcttgtgggtcacggtcacctttccacagtacaggacttcgaacttctgagagttgtaaaaggcgtcctcattatctttgctgggtttggcatcctctttcatggccgctttagataattgccttatgctgctaataacatcaggaacctggctggggtctgtggcgcggaaaacgtggcaggccatctgcgactcggggtcgtcgggctgcgccttgatcaggtaggcaaagtaggtgaggtcgtggctgttgtggatgaagcgcgagatatgctgcgccttgtgctcgaagatgaataccgccgggttgggctgcgtggccgacggactagtgccccccgaggccccagcgcccggcgcggggacgcaacgcaggaagggcgcgctgagcaccaggatcacctctcgggccgccggcgccccgcagccgcccgcctcgggcttctggctgcgcctgcggatctcggccatgagccagggcagcataggcagcgtggtcctgtggtccaggcacgaccccccaacgtaccacagccggaaccgcttatcgcttggcttcccggggccgggctgagctgagacgcccggctcgggctccagggggtgcgggaacggctcatcctgaatgcagctgggcggctccataactctcgcctcaccagggcaccgcggaggccggccgggcgcaccgcgccccccactcccgcgcagaaggcgccgccgaaactgtgccaactgccgcaccgggctcccgcgcctgcctgggagcggcgcgaccccgaactccgcgcttcagcagccctgccccatgcagcacttccacgggcgcggctcggaggctccggcggcgggcaccgaggcaagcgcccggcaggcgagggcgggttaaatgggcatcctcctccttgggctggcgcctcgggcaggacctccccttcctccgtcgcgggtttgcagggtcagaggaccacgccgagggtccccgcggccgccggctccagcgctgcagccccgctgcggccgccgcgctcgcctggggcagacac

SEQ ID NO: 17025 - RNA, 4450 nt, Homo sapiens
  source 1..4450: mol_type = other RNA
tagtggtcctaaacatttcacagttctcaaaacttttcacataaaaggggaagattattaaagcttattagattctgtcaattggtcaaaagaaaaaatgtatttcaacacagcttgtcatctttggaaaaaatcaatcataattacgtttccttatactgaatttaaggtagagagacctaaattacaagcactcacaatttggtgggaaagtggcaaatccttgtcatttggtgactgtggcaccaaataaagaggaattcattcacaactgaatgagttattcaaataaaaaaagcagaaagctaatctagacattttaggtcctaaattaaatttttcaggtgtgatatttttagtttgagtaataatgctggtctagtttgctaaaaaattagcaacattctcctttaccttgagctgggtagactcagccacaatgtcctactgtctctttatgtatgtttaaagtaatgcctaaccagactcataatgcatgtagatgcaacatgctagttggcacaaagcaggcagggagaaatgaccctaccttcccaaaaaactcacaggagcatgaccagtaatcattttcctcatatagacaatgtcagtagatatcaagacagatacacataaagttacataaatgtttccaccttttcaccattgagtgaaacatgctgttctttggagaaaaaaatacattcatttttttcaagtatattgcaatatacaaagatgctctggctttgtttcactataaagacaaaaagatttcacatatgtccaagggaaatttcagtttacctttcctttggtgtggatttcatgaagttctgactaaaaaaattaatctaaatatacatctactcattttatctgaaagcatgaactatgttcattttatatatatatttatatgtacatagcaacaacaaaaaccagtctacatatgtccaatggcttaggattggcatgctctgatgagcacgaggtccacctgctgtgactaggcgctcagcaccagtattaggtggttccatcagcttcagggtccagccttgggccagcgacatgcaggctcttcctctctgtagtattctaaggagcactttctgctgaggccgtgcctcttcaattatggcttatttcctatcttggctttgttgttagggttgcagtttaggtctctcagcaacaggtcacaattgactagagcatccgcgggcagcagcttccggagttgctccactgtcttttgataagccattttttcttgttccagggtccggattaaagacttcattttggtctctctcgtcaaaagattttccaggtttgattccaaggcctggattttagtatgagctacctgtaatttttctaggaggtccatgttttgtcttttcagttggctattggccctctccagcttctccaaagtttcactatcctcacaggaatatgaagattcctgaagctcatcctgtagcacatgatattccacctcataggcatgcaactgcttagaaatatccatctcaaaaacctgggtaataattttttccatttcagaggtattcatatcaggtagcgtgtttttaagaaactcaacaatattttcaaagctctcacattccattataagtgtctcttggctgctcagtaggctgagtgcaaccttgaatataacttcagttccctgaagaaaaataatatcaaaaactctggctacaaatcctaatgaaaactgagaggcaaacaatgtgaggaaccagggggcagcataaagactggggctgatttcattttcttcaaggtgattgtagagatctctgtgatagtcatgaaggagcctggacagctggtacatttgaatctgcagcgacatcatgtcaggtctgtactgcttgcggaagccgaggtcatacatgaggaatttcagcatttcaaaggcttgctcttcactcatgtgcagaagcaggactccagccacaaagctgatcccctgacagtatcccacttctttgtccagcaaagaataggctttcaggaggttaaacagtgacagctgtcctggcccaagctgtactgaaaagtaagggtgagtaggaaacgtccttcctaaatccacgagaatcgcatgctgctgagcagtgagctgcttcaaaagttccttataggatatgtcaggaggctgttgtttattaggcaatctgtgtctgagtcggtactgtaaagccagaaactgccaaatttctcctcgtcgacttttgggaactccttctttaagaagagtatgaatatcttccatatcacatctgattttagctctgcagtttaacaacttcttatcccaagttattaagacctctttctgacatgcaccaacttcttcatagtctaatttaacttttctggactggagttcatctctgcttgcttcaagtttctggttttctttttccattcgaagtaacaagatttgttggtgtatagcttttctccacaagctcctcagttcttttgatttctttctttcttcaatcttttctgggtcatcctccccagacaggaatacaaccagcggttcctcctccatggttggagagaggggggacagtggcagcagctcgttcctgtccaatccatcttgctgttgcattgctgagggagatttgttcatgggagaagcaaccctgaggaaaatgcgctgccgccaggagatccggcgaggagtgacagaggttcctcccacacttagggactcattgctgcaggtagatgaggtcctttttctcccttctccatcactgcactgttcactggagctctgcctcagcagaggggaacgcacaccctgagccctcccatcctgcaaattcagctttctctttgtgcttgaaggtgggtggctgaacgtgtgtgcccgtcttcgaaactgcggggagtcggaatcctcttcgggaaacgtttgccaagctgaggacggtggggacgctggcggtgtccctggtggagaatcccctggtgagtagtccttctctgaagcaagactgttggaccgttcaaaactgtccacacttccaagccgacctctcattctgttagctccccttgagaagatattttccagggagctagttaaggatctcttagctttatttttcagaatgtcaagtttgaaccttccactgcttgttgcattttctgggattgtactatttgaaatagtagaagggccttccccgatgtgcacgtgtgtcttctgcttggcttcacacagctgcctcaggtgtaaaatcacaagttcattttcttcctggtcactgactggcttcattttctgaactctttcaaagatgtcagcttgctcattatctgtcagtgatgagagatgcctctgtatcaccagcttggctcttggtgggtagagaccttcaatcctttcacagagcttatgcaaagagtgcatcgggcaggcctcacacagtttaatctgcgtcttggcactctgcagggcagccgccgtactgaaggcctgtttcagagtcagcattacctcatcaaccagagattcgctggcacactggaatacataacaaatatactggctaagtccaggctctggagactcccggcagataaagccaaagtgatccacatgctttataccctgagaacaagaggagatatctttaaaattcttttctagcacaactgatttagtgtctggactgataaggttaatctcaaatcgcccaacctggaagagcatggtcctgttcttctccgagtccgagggctggacgtgactgggtgcgctcgcgtgtctccgtcgcggctgggatttctggctgccctcgtgaactctccgttgcacgccggtgacactgctgcaccgagaccgaaactcctgctgctcatcaaagccagaatcttccaaaatccgctcagggaagcagacccgagagctggtcagggcaggctggctggccccggcaggtaagccaaggtgggtgtcggtgccgtcagcctcctccggcaggcagtctccgggggacccgggcaccaccacctccaagtcagccaggtcctctcctgggtccggaccgcgctgctccccttggatcttcaggcgctgctgttcgtgcaggctgaacttctccatgcagtcatcgatgaggcttgagggggccttcttgtgggtcacggtcacctttccacagtacaggacttcgaacttctgagagttgtaaaaggcgtcctcattatctttgctgggtttggcatcctctttcatggccgctttagataattgccttatgctgctaataacatcaggaacctttgatcaggaagccagctggaaactggaggtggtcacgaagagcaatgattttgccaaactggtgtagtcctcagtattagctctaagttctctctttct

SEQ ID NO: 17026 - RNA, 4339 nt, Homo sapiens
  source 1..4339: mol_type = other RNA
tagtggtcctaaacatttcacagttctcaaaacttttcacataaaaggggaagattattaaagcttattagattctgtcaattggtcaaaagaaaaaatgtatttcaacacagcttgtcatctttggaaaaaatcaatcataattacgtttccttatactgaatttaaggtagagagacctaaattacaagcactcacaatttggtgggaaagtggcaaatccttgtcatttggtgactgtggcaccaaataaagaggaattcattcacaactgaatgagttattcaaataaaaaaagcagaaagctaatctagacattttaggtcctaaattaaatttttcaggtgtgatatttttagtttgagtaataatgctggtctagtttgctaaaaaattagcaacattctcctttaccttgagctgggtagactcagccacaatgtcctactgtctctttatgtatgtttaaagtaatgcctaaccagactcataatgcatgtagatgcaacatgctagttggcacaaagcaggcagggagaaatgaccctaccttcccaaaaaactcacaggagcatgaccagtaatcattttcctcatatagacaatgtcagtagatatcaagacagatacacataaagttacataaatgtttccaccttttcaccattgagtgaaacatgctgttctttggagaaaaaaatacattcatttttttcaagtatattgcaatatacaaagatgctctggctttgtttcactataaagacaaaaagatttcacatatgtccaagggaaatttcagtttacctttcctttggtgtggatttcatgaagttctgactaaaaaaattaatctaaatatacatctactcattttatctgaaagcatgaactatgttcattttatatatatatttatatgtacatagcaacaacaaaaaccagtctacatatgtccaatggcttaggattggcatgctctgatgagcacgaggtccacctgctgtgactaggcgctcagcaccagtattaggtggttccatcagcttcagggtccagccttgggccagcgacatgcaggctcttcctctctgtagtattctaaggagcactttctgctgaggccgtgcctcttcaattatggcttatttcctatcttggctttgttgttagggttgcagtttaggtctctcagcaacaggtcacaattgactagagcatccgcgggcagcagcttccggagttgctccactgtcttttgataagccattttttcttgttccagggtccggattaaagacttcattttggtctctctcgtcaaaagattttccaggtttgattccaaggcctggattttagtatgagctacctgtaatttttctaggaggtccatgttttgtcttttcagttggctattggccctctccagcttctccaaagtttcactatcctcacaggaatatgaagattcctgaagctcatcctgtagcacatgatattccacctcataggcatgcaactgcttagaaatatccatctcaaaaacctgggtaataattttttccatttcagaggtattcatatcaggtagcgtgtttttaagaaactcaacaatattttcaaagctctcacattccattataagtgtctcttggctgctcagtaggctgagtgcaaccttgaatataacttcagttccctgaagaaaaataatatcaaaaactctggctacaaatcctaatgaaaactgagaggcaaacaatgtgaggaaccagggggcagcataaagactggggctgatttcattttcttcaaggtgattgtagagatctctgtgatagtcatgaaggagcctggacagctggtacatttgaatctgcagcgacatcatgtcaggtctgtactgcttgcggaagccgaggtcatacatgaggaatttcagcatttcaaaggcttgctcttcactcatgtgcagaagcaggactccagccacaaagctgatcccctgacagtatcccacttctttgtccagcaaagaataggctttcaggaggttaaacagtgacagctgtcctggcccaagctgtactgaaaagtaagggtgagtaggaaacgtccttcctaaatccacgagaatcgcatgctgctgagcagtgagctgcttcaaaagttccttataggatatgtcaggaggctgttgtttattaggcaatctgtgtctgagtcggtactgtaaagccagaaactgccaaatttctcctcgtcgacttttgggaactccttctttaagaagagtatgaatatcttccatatcacatctgattttagctctgcagtttaacaacttcttatcccaagttattaagacctctttctgacatgcaccaacttcttcatagtctaatttaacttttctggactggagttcatctctgcttgcttcaagtttctggttttctttttccattcgaagtaacaagatttgttggtgtatagcttttctccacaagctcctcagttcttttgatttctttctttcttcaatcttttctgggtcatcctccccagacaggaatacaaccagcggttcctcctccatggttggagagaggggggacagtggcagcagctcgttcctgtccaatccatcttgctgttgcattgctgagggagatttgttcatgggagaagcaaccctgaggaaaatgcgctgccgccaggagatccggcgaggagtgacagaggttcctcccacacttagggactcattgctgcaggtagatgaggtcctttttctcccttctccatcactgcactgttcactggagctctgcctcagcagaggggaacgcacaccctgagccctcccatcctgcaaattcagctttctctttgtgcttgaaggtgggtggctgaacgtgtgtgcccgtcttcgaaactgcggggagtcggaatcctcttcgggaaacgtttgccaagctgaggacggtggggacgctggcggtgtccctggtggagaatcccctggtgagtagtccttctctgaagcaagactgttggaccgttcaaaactgtccacacttccaagccgacctctcattctgttagctccccttgagaagatattttccagggagctagttaaggatctcttagctttatttttcagaatgtcaagtttgaaccttccactgcttgttgcattttctgggattgtactatttgaaatagtctgaactctttcaaagatgtcagcttgctcattatctgtcagtgatgagagatgcctctgtatcaccagcttggctcttggtgggtagagaccttcaatcctttcacagagcttatgcaaagagtgcatcgggcaggcctcacacagtttaatctgcgtcttggcactctgcagggcagccgccgtactgaaggcctgtttcagagtcagcattacctcatcaaccagagattcgctggcacactggaatacataacaaatatactggctaagtccaggctctggagactcccggcagataaagccaaagtgatccacatgctttataccctgagaacaagaggagatatctttaaaattcttttctagcacaactgatttagtgtctggactgataaggttaatctcaaatcgcccaacctggaagagcatggtcctgttcttctccgagtccgagggctggacgtgactgggtgcgctcgcgtgtctccgtcgcggctgggatttctggctgccctcgtgaactctccgttgcacgccggtgacactgctgcaccgagaccgaaactcctgctgctcatcaaagccagaatcttccaaaatccgctcagggaagcagacccgagagctggtcagggcaggctggctggccccggcaggtaagccaaggtgggtgtcggtgccgtcagcctcctccggcaggcagtctccgggggacccgggcaccaccacctccaagtcagccaggtcctctcctgggtccggaccgcgctgctccccttggatcttcaggcgctgctgttcgtgcaggctgaacttctccatgcagtcatcgatgaggcttgagggggccttcttgtgggtcacggtcacctttccacagtacaggacttcgaacttctgagagttgtaaaaggcgtcctcattatctttgctgggtttggcatcctctttcatggccgctttagataattgccttatgctgctaataacatcaggaacctttgatcaggaagccagctggaaactggaggtggtcacgaagagcaatgattttgccaaactggtgtagtcctcagtattagctctaagttctctctttct

SEQ ID NO: 17027 - RNA, 6337 nt, Homo sapiens
  source 1..6337: mol_type = other RNA
tagtggtcctaaacatttcacagttctcaaaacttttcacataaaaggggaagattattaaagcttattagattctgtcaattggtcaaaagaaaaaatgtatttcaacacagcttgtcatctttggaaaaaatcaatcataattacgtttccttatactgaatttaaggtagagagacctaaattacaagcactcacaatttggtgggaaagtggcaaatccttgtcatttggtgactgtggcaccaaataaagaggaattcattcacaactgaatgagttattcaaataaaaaaagcagaaagctaatctagacattttaggtcctaaattaaatttttcaggtgtgatatttttagtttgagtaataatgctggtctagtttgctaaaaaattagcaacattctcctttaccttgagctgggtagactcagccacaatgtcctactgtctctttatgtatgtttaaagtaatgcctaaccagactcataatgcatgtagatgcaacatgctagttggcacaaagcaggcagggagaaatgaccctaccttcccaaaaaactcacaggagcatgaccagtaatcattttcctcatatagacaatgtcagtagatatcaagacagatacacataaagttacataaatgtttccaccttttcaccattgagtgaaacatgctgttctttggagaaaaaaatacattcatttttttcaagtatattgcaatatacaaagatgctctggctttgtttcactataaagacaaaaagatttcacatatgtccaagggaaatttcagtttacctttcctttggtgtggatttcatgaagttctgactaaaaaaattaatctaaatatacatctactcattttatctgaaagcatgaactatgttcattttatatatatatttatatgtacatagcaacaacaaaaaccagtctacatatgtccaatggcttaggattggcatgctctgatgagcacgaggtccacctgctgtgactaggcgctcagcaccagtattaggtggttccatcagcttcagggtccagccttgggccagcgacatgcaggctcttcctctctgtagtattctaaggagcactttctgctgaggccgtgcctcttcaattatggcttatttcctatcttggctttgttgttagggttgcagtttaggtctctcagcaacaggtcacaattgactagagcatccgcgggcagcagcttccggagttgctccactgtcttttgataagccattttttcttgttccagggtccggattaaagacttcattttggtctctctcgtcaaaagattttccaggtttgattccaaggcctggattttagtatgagctacctgtaatttttctaggaggtccatgttttgtcttttcagttggctattggccctctccagcttctccaaagtttcactatcctcacaggaatatgaagattcctgaagctcatcctgtagcacatgatattccacctcataggcatgcaactgcttagaaatatccatctcaaaaacctgggtaataattttttccatttcagaggtattcatatcaggtagcgtgtttttaagaaactcaacaatattttcaaagctctcacattccattataagtgtctcttggctgctcagtaggctgagtgcaaccttgaatataacttcagttccctgaagaaaaataatatcaaaaactctggctacaaatcctaatgaaaactgagaggcaaacaatgtgaggaaccagggggcagcataaagactggggctgatttcattttcttcaaggtgattgtagagatctctgtgatagtcatgaaggagcctggacagctggtacatttgaatctgcagcgacatcatgtcaggtctgtactgcttgcggaagccgaggtcatacatgaggaatttcagcatttcaaaggcttgctcttcactcatgtgcagaagcaggactccagccacaaagctgatcccctgacagtatcccacttctttgtccagcaaagaataggctttcaggaggttaaacagtgacagctgtcctggcccaagctgtactgaaaagtaagggtgagtaggaaacgtccttcctaaatccacgagaatcgcatgctgctgagcagtgagctgcttcaaaagttccttataggatatgtcaggaggctgttgtttattaggcaatctgtgtctgagtcggtactgtaaagccagaaactgccaaatttctcctcgtcgacttttgggaactccttctttaagaagagtatgaatatcttccatatcacatctgattttagctctgcagtttaacaacttcttatcccaagttattaagacctctttctgacatgcaccaacttcttcatagtctaatttaacttttctggactggagttcatctctgcttgcttcaagtttctggttttctttttccattcgaagtaacaagatttgttggtgtatagcttttctccacaagctcctcagttcttttgatttctttctttcttcaatcttttctgggtcatcctccccagacaggaatacaaccagcggttcctcctccatggttggagagaggggggacagtggcagcagctcgttcctgtccaatccatcttgctgttgcattgctgagggagatttgttcatgggagaagcaaccctgaggaaaatgcgctgccgccaggagatccggcgaggagtgacagaggttcctcccacacttagggactcattgctgcaggtagatgaggtcctttttctcccttctccatcacttgattctgaagcagtgtcttgtctgatttcattttcatactgtggggacagtctacctgaattctggtaaaagcttttcaggaaagagggggcagtgaaggaaggggcagagaaggaagtgtgaagacttggaagactggaggaagaattactctccttgtacatgcgtcgaactgacgaaagattgctgcactgttcactggagctctgcctcagcagaggggaacgcacaccctgagccctcccatcctgcaaattcagctttctctttgtgcttgaaggtgggtggctgaacgtgtgtgcccgtcttcgaaactgcggggagtcggaatcctcttcgggaaacgtttgccaagctgaggacggtggggacgctggcggtgtccctggtggagaatcccctggtgagtagtcccttgagaagatattttccagggagctagttaaggatctcttagctttatttttcagaatgtcaagtttgaaccttccactgcttgttgcattttctgggattgtactatttgaaatagtagaagggccttccccgatgtgcacgtgtgtcttctgcttggcttcacacagctgcctcaggtgtaaaatcacaagttcattttcttcctggtcactgactggcttcattttctgaactctttcaaagatgtcagcttgctcattatctgtcagtgatgagagatgcctctgtatcaccagcttggctcttggtgggtagagaccttcaatcctttcacagagcttatgcaaagagtgcatcgggcaggcctcacacagtttaatctgcgtcttggcactctgcagggcagccgccgtactgaaggcctgtttcagagtcagcattacctcatcaaccagagattcgctggcacactggaatacataacaaatatactggctaagtccaggctctggagactcccggcagataaagccaaagtgatccacatgctttataccctgagaacaagaggagatatctttaaaattcttttctagcacaactgatttagtgtctggactgataaggttaatctcaaatcgcccaacctggaagagcatggtcctgttcttctccgagtccgagggctggacgtgactgggtgcgctcgcgtgtctccgtcgcggctgggatttctggctgccctcgtgaactctccgttgcacgccggtgacactgctgcaccgagaccgaaactcctgctgctcatcaaagccagaatcttccaaaatccgctcagggaagcagacccgagagctggtcagggcaggctggctggccccggcaggtaagccaaggtgggtgtcggtgccgtcagcctcctccggcaggcagtctccgggggacccgggcaccaccacctccaagtcagccaggtcctctcctgggtccggaccgcgctgctccccttggatcttcaggcgctgctgttcgtgcaggctgaacttctccatgcagtcatcgatgaggcttgagggggccttcttgtgggtcacggtcacctttccacagtacaggacttcgaacttctgagagttgtaaaaggcgtcctcattatctttgctgggtttggcatcctctttcatggccgctttagataattgccttatgctgctaataacatcaggaacctggctggggtctgtggcgcggaaaacgtggcaggccatctgcgactcggggtcgtcgggctgcgccttgatcaggtaggcaaagtaggtgaggtcgtggctgttgtggatgaagcgcgagatatgctgcgccttgtgctcgaagatgaataccgccgggttgggctgcgtggccgacggactagtgccccccgaggccccagcgcccggcgcggggacgcaacgcaggaagggcgcgctgagcaccaggatcacctctcgggccgccggcgccccgcagccgcccgcctcgggcttctggctgcgcctgcggatctcggccatgagccagggcagcataggcagcgtggtcctgtggtccaggcacgaccccccaacgtaccacagccggaaccgcttatcgcttggcttcccggggccgggctgagctgagacgcccggctcgggctccagggggtgcgggaacggctcatcctgaatgcagctgggcggctccataactctcgcctcaccagggcaccgcggaggccggccgggcgcaccgcgccccccactcccgcgcagaaggcgccgccgaaactgtgccaactgccgcaccgggctcccgcgcctgcctgggagcggcgcgaccccgaactccgcgcttcagcagccctgccccatgcagcacttccacgggcgcggctcggaggctccggcggcgggcaccgaggcaagcgcccggcaggcgagggcgggttaaatgggcatcctcctccttgggctggcgcctcgggcaggacctccccttcctccgtcgcgggtttgcagggtcagaggaccacgccgagggtccccgcggccgccggctccagcgctgcagccccgctgcggccgccgcgctcgcctggggcagacactgggtggctgggcggggaatggggctgtgggcgggagggggtgacttggggcggagctgactcctaccagggtgaccggctgtcacctggaaggtcggggctgcagggctgcggcgcggtcagtcctcaggaaaggctccggcaactactccagtggaaaataacaaaaacaaaacgtggcctcgcgggggccgctcctcctcccgccgcagctgcagcccagctcgctgctcctcctcctgccgttcccgtccctccctcgctccttccttccttccttccaggctgcttctttaatcgggctgctactccgcctcccgtccggcgggcggagagcgtcgcctgcaaaagcttatccgtgaagccgcctctccgcctcttcgcctcttccttcgacccccgcccttggggctgcagctcagagcctggcgcgggcactgcccggacccacttggcctctcttgagtcgccgcgatctccgtctcctcccgggcgtctctgctgccccctagagagggggccactcgcagtggagaactgggatttttttttaacagtatttgcttggtttcagttccttctaaagcctacacattaatttctgaattatctttcctaataatctcaaaaaacgctcgtgttttcaatcacaatattataaattccagttccaaatttcactttaaaacataatatcgacagcttgaatcttcctagttattaaagcagccaacttcttaaaatatggaaaagttatgttttatttatgttatatccccagttgagagctaatgtagagatttcttgttcttttatatatatgtggtaatacatatttccaaagaactaaaaaaaagtttggaataatttgatcattgtaattttaagacaggtagacaagtattctccctttttactcataccgaatgataattaagaattgggtaagaagtaaagacaaaataaataagaaaga

SEQ ID NO: 17028 - RNA, 5124 nt, Homo sapiens
  source 1..5124: mol_type = other RNA
tagtggtcctaaacatttcacagttctcaaaacttttcacataaaaggggaagattattaaagcttattagattctgtcaattggtcaaaagaaaaaatgtatttcaacacagcttgtcatctttggaaaaaatcaatcataattacgtttccttatactgaatttaaggtagagagacctaaattacaagcactcacaatttggtgggaaagtggcaaatccttgtcatttggtgactgtggcaccaaataaagaggaattcattcacaactgaatgagttattcaaataaaaaaagcagaaagctaatctagacattttaggtcctaaattaaatttttcaggtgtgatatttttagtttgagtaataatgctggtctagtttgctaaaaaattagcaacattctcctttaccttgagctgggtagactcagccacaatgtcctactgtctctttatgtatgtttaaagtaatgcctaaccagactcataatgcatgtagatgcaacatgctagttggcacaaagcaggcagggagaaatgaccctaccttcccaaaaaactcacaggagcatgaccagtaatcattttcctcatatagacaatgtcagtagatatcaagacagatacacataaagttacataaatgtttccaccttttcaccattgagtgaaacatgctgttctttggagaaaaaaatacattcatttttttcaagtatattgcaatatacaaagatgctctggctttgtttcactataaagacaaaaagatttcacatatgtccaagggaaatttcagtttacctttcctttggtgtggatttcatgaagttctgactaaaaaaattaatctaaatatacatctactcattttatctgaaagcatgaactatgttcattttatatatatatttatatgtacatagcaacaacaaaaaccagtctacatatgtccaatggcttaggattggcatgctctgatgagcacgaggtccacctgctgtgactaggcgctcagcaccagtattaggtggttccatcagcttcagggtccagccttgggccagcgacatgcaggctcttcctctctgtagtattctaaggagcactttctgctgaggccgtgcctcttcaattatggcttatttcctatcttggctttgttgttagggttgcagtttaggtctctcagcaacaggtcacaattgactagagcatccgcgggcagcagcttccggagttgctccactgtcttttgataagccattttttcttgttccagggtccggattaaagacttcattttggtctctctcgtcaaaagattttccaggtttgattccaaggcctggattttagtatgagctacctgtaatttttctaggaggtccatgttttgtcttttcagttggctattggccctctccagcttctccaaagtttcactatcctcacaggaatatgaagattcctgaagctcatcctgtagcacatgatattccacctcataggcatgcaactgcttagaaatatccatctcaaaaacctgggtaataattttttccatttcagaggtattcatatcaggtagcgtgtttttaagaaactcaacaatattttcaaagctctcacattccattataagtgtctcttggctgctcagtaggctgagtgcaaccttgaatataacttcagttccctgaagaaaaataatatcaaaaactctggctacaaatcctaatgaaaactgagaggcaaacaatgtgaggaaccagggggcagcataaagactggggctgatttcattttcttcaaggtgattgtagagatctctgtgatagtcatgaaggagcctggacagctggtacatttgaatctgcagcgacatcatgtcaggtctgtactgcttgcggaagccgaggtcatacatgaggaatttcagcatttcaaaggcttgctcttcactcatgtgcagaagcaggactccagccacaaagctgatcccctgacagtatcccacttctttgtccagcaaagaataggctttcaggaggttaaacagtgacagctgtcctggcccaagctgtactgaaaagtaagggtgagtaggaaacgtccttcctaaatccacgagaatcgcatgctgctgagcagtgagctgcttcaaaagttccttataggatatgtcaggaggctgttgtttattaggcaatctgtgtctgagtcggtactgtaaagccagaaactgccaaatttctcctcgtcgacttttgggaactccttctttaagaagagtatgaatatcttccatatcacatctgattttagctctgcagtttaacaacttcttatcccaagttattaagacctctttctgacatgcaccaacttcttcatagtctaatttaacttttctggactggagttcatctctgcttgcttcaagtttctggttttctttttccattcgaagtaacaagatttgttggtgtatagcttttctccacaagctcctcagttcttttgatttctttctttcttcaatcttttctgggtcatcctccccagacaggaatacaaccagcggttcctcctccatggttggagagaggggggacagtggcagcagctcgttcctgtccaatccatcttgctgttgcattgctgagggagatttgttcatgggagaagcaaccctgaggaaaatgcgctgccgccaggagatccggcgaggagtgacagaggttcctcccacacttagggactcattgctgcaggtagatgaggtcctttttctcccttctccatcacttgattctgaagcagtgtcttgtctgatttcattttcatactgtggggacagtctacctgaattctggtaaaagcttttcaggaaagagggggcagtgaaggaaggggcagagaaggaagtgtgaagacttggaagactggaggaagaattactctccttgtacatgcgtcgaactgacgaaagattgctgcactgttcactggagctctgcctcagcagaggggaacgcacaccctgagccctcccatcctgcaaattcagctttctctttgtgcttgaaggtgggtggctgaacgtgtgtgcccgtcttcgaaactgcggggagtcggaatcctcttcgggaaacgtttgccaagctgaggacggtggggacgctggcggtgtccctggtggagaatcccctggtgagtagtccttctctgaagcaagactgttggaccgttcaaaactgtccacacttccaagccgacctctcattctgttagctccccttgagaagatattttccagggagctagttaaggatctcttagctttatttttcagaatgtcaagtttgaaccttccactgcttgttgcattttctgggattgtactatttgaaatagtagaagggccttccccgatgtgcacgtgtgtcttctgcttggcttcacacagctgcctcaggtgtaaaatcacaagttcattttcttcctggtcactgactggcttcattttctgaactctttcaaagatgtcagcttgctcattatctgtcagtgatgagagatgcctctgtatcaccagcttggctcttggtgggtagagaccttcaatcctttcacagagcttatgcaaagagtgcatcgggcaggcctcacacagtttaatctgcgtcttggcactctgcagggcagccgccgtactgaaggcctgtttcagagtcagcattacctcatcaaccagagattcgctggcacactggaatacataacaaatatactggctaagtccaggctctggagactcccggcagataaagccaaagtgatccacatgctttataccctgagaacaagaggagatatctttaaaattcttttctagcacaactgatttagtgtctggactgataaggttaatctcaaatcgcccaacctggaagagcatggtcctgttcttctccgagtccgagggctggacgtgactgggtgcgctcgcgtgtctccgtcgcggctgggatttctggctgccctcgtgaactctccgttgcacgccggtgacactgctgcaccgagaccgaaactcctgctgctcatcaaagccagaatcttccaaaatccgctcagggaagcagacccgagagctggtcagggcaggctggctggccccggcaggtaagccaaggtgggtgtcggtgccgtcagcctcctccggcaggcagtctccgggggacccgggcaccaccacctccaagtcagccaggtcctctcctgggtccggaccgcgctgctccccttggatcttcaggcgctgctgttcgtgcaggctgaacttctccatgcagtcatcgatgaggcttgagggggccttcttgtgggtcacggtcacctttccacagtacaggacttcgaacttctgagagttgtaaaaggcgtcctcattatctttgctgggtttggcatcctctttcatggccgctttagataattgccttatgctgctaataacatcaggaacacaaggtgtctgaacatcttccatcccctgtcaaaatcagaggaagctgtgaagcctgccagccatcaggcccgggttaatgagttccacagtccagtttcacagtatctctggcatttgcagtcatggggaaagaacatgcagcccccgtgctcctgggcccctctctcaagagtctgtttcaggcatgcagggctaaaataaaccaaaccagcagactgaactgcctttcacccatggataaagacctactcctgtccatggccaggtaccaggagatcctgggtcaatgcatttttaattccaccggatcctctacttcacaacatgactttctttatttttaggggaaaagtgtgtggggtttttgcaggggagaaaggattaagataattattagttctagtttcgcagctagcaacaaaatcacttgctaacaactagtttttcattattactaaacaaaatattttaattgtaggctctattcatattgcttaaagaaattacattctaaatgttttgagatattcttgtatgttaacaggtagttacaaaatgtattatttttgatctagcaaatacct

SEQ ID NO: 17029 - RNA, 5437 nt, Homo sapiens
  source 1..5437: mol_type = other RNA
tagtggtcctaaacatttcacagttctcaaaacttttcacataaaaggggaagattattaaagcttattagattctgtcaattggtcaaaagaaaaaatgtatttcaacacagcttgtcatctttggaaaaaatcaatcataattacgtttccttatactgaatttaaggtagagagacctaaattacaagcactcacaatttggtgggaaagtggcaaatccttgtcatttggtgactgtggcaccaaataaagaggaattcattcacaactgaatgagttattcaaataaaaaaagcagaaagctaatctagacattttaggtcctaaattaaatttttcaggtgtgatatttttagtttgagtaataatgctggtctagtttgctaaaaaattagcaacattctcctttaccttgagctgggtagactcagccacaatgtcctactgtctctttatgtatgtttaaagtaatgcctaaccagactcataatgcatgtagatgcaacatgctagttggcacaaagcaggcagggagaaatgaccctaccttcccaaaaaactcacaggagcatgaccagtaatcattttcctcatatagacaatgtcagtagatatcaagacagatacacataaagttacataaatgtttccaccttttcaccattgagtgaaacatgctgttctttggagaaaaaaatacattcatttttttcaagtatattgcaatatacaaagatgctctggctttgtttcactataaagacaaaaagatttcacatatgtccaagggaaatttcagtttacctttcctttggtgtggatttcatgaagttctgactaaaaaaattaatctaaatatacatctactcattttatctgaaagcatgaactatgttcattttatatatatatttatatgtacatagcaacaacaaaaaccagtctacatatgtccaatggcttaggattggcatgctctgatgagcacgaggtccacctgctgtgactaggcgctcagcaccagtattaggtggttccatcagcttcagggtccagccttgggccagcgacatgcaggctcttcctctctgtagtattctaaggagcactttctgctgaggccgtgcctcttcaattatggcttatttcctatcttggctttgttgttagggttgcagtttaggtctctcagcaacaggtcacaattgactagagcatccgcgggcagcagcttccggagttgctccactgtcttttgataagccattttttcttgttccagggtccggattaaagacttcattttggtctctctcgtcaaaagattttccaggtttgattccaaggcctggattttagtatgagctacctgtaatttttctaggaggtccatgttttgtcttttcagttggctattggccctctccagcttctccaaagtttcactatcctcacaggaatatgaagattcctgaagctcatcctgtagcacatgatattccacctcataggcatgcaactgcttagaaatatccatctcaaaaacctgggtaataattttttccatttcagaggtattcatatcaggtagcgtgtttttaagaaactcaacaatattttcaaagctctcacattccattataagtgtctcttggctgctcagtaggctgagtgcaaccttgaatataacttcagttccctgaagaaaaataatatcaaaaactctggctacaaatcctaatgaaaactgagaggcaaacaatgtgaggaaccagggggcagcataaagactggggctgatttcattttcttcaaggtgattgtagagatctctgtgatagtcatgaaggagcctggacagctggtacatttgaatctgcagcgacatcatgtcaggtctgtactgcttgcggaagccgaggtcatacatgaggaatttcagcatttcaaaggcttgctcttcactcatgtgcagaagcaggactccagccacaaagctgatcccctgacagtatcccacttctttgtccagcaaagaataggctttcaggaggttaaacagtgacagctgtcctggcccaagctgtactgaaaagtaagggtgagtaggaaacgtccttcctaaatccacgagaatcgcatgctgctgagcagtgagctgcttcaaaagttccttataggatatgtcaggaggctgttgtttattaggcaatctgtgtctgagtcggtactgtaaagccagaaactgccaaatttctcctcgtcgacttttgggaactccttctttaagaagagtatgaatatcttccatatcacatctgattttagctctgcagtttaacaacttcttatcccaagttattaagacctctttctgacatgcaccaacttcttcatagtctaatttaacttttctggactggagttcatctctgcttgcttcaagtttctggttttctttttccattcgaagtaacaagatttgttggtgtatagcttttctccacaagctcctcagttcttttgatttctttctttcttcaatcttttctgggtcatcctccccagacaggaatacaaccagcggttcctcctccatggttggagagaggggggacagtggcagcagctcgttcctgtccaatccatcttgctgttgcattgctgagggagatttgttcatgggagaagcaaccctgaggaaaatgcgctgccgccaggagatccggcgaggagtgacagaggttcctcccacacttagggactcattgctgcaggtagatgaggtcctttttctcccttctccatcacttgattctgaagcagtgtcttgtctgatttcattttcatactgtggggacagtctacctgaattctggtaaaagcttttcaggaaagagggggcagtgaaggaaggggcagagaaggaagtgtgaagacttggaagactggaggaagaattactctccttgtacatgcgtcgaactgacgaaagattgctgcactgttcactggagctctgcctcagcagaggggaacgcacaccctgagccctcccatcctgcaaattcagctttctctttgtgcttgaaggtgggtggctgaacgtgtgtgcccgtcttcgaaactgcggggagtcggaatcctcttcgggaaacgtttgccaagctgaggacggtggggacgctggcggtgtccctggtggagaatcccctggtgagtagtccttctctgaagcaagactgttggaccgttcaaaactgtccacacttccaagccgacctctcattctgttagctccccttgagaagatattttccagggagctagttaaggatctcttagctttatttttcagaatgtcaagtttgaaccttccactgcttgttgcattttctgggattgtactatttgaaatagtagaagggccttccccgatgtgcacgtgtgtcttctgcttggcttcacacagctgcctcaggtgtaaaatcacaagttcattttcttcctggtcactgactggcttcattttctgaactctttcaaagatgtcagcttgctcattatctgtcagtgatgagagatgcctctgtatcaccagcttggctcttggtgggtagagaccttcaatcctttcacagagcttatgcaaagagtgcatcgggcaggcctcacacagtttaatctgcgtcttggcactctgcagggcagccgccgtactgaaggcctgtttcagagtcagcattacctcatcaaccagagattcgctggcacactggaatacataacaaatatactggctaagtccaggctctggagactcccggcagataaagccaaagtgatccacatgctttataccctgagaacaagaggagatatctttaaaattcttttctagcacaactgatttagtgtctggactgataaggttaatctcaaatcgcccaacctggaagagcatggtcctgttcttctccgagtccgagggctggacgtgactgggtgcgctcgcgtgtctccgtcgcggctgggatttctggctgccctcgtgaactctccgttgcacgccggtgacactgctgcaccgagaccgaaactcctgctgctcatcaaagccagaatcttccaaaatccgctcagggaagcagacccgagagctggtcagggcaggctggctggccccggcaggtaagccaaggtgggtgtcggtgccgtcagcctcctccggcaggcagtctccgggggacccgggcaccaccacctccaagtcagccaggtcctctcctgggtccggaccgcgctgctccccttggatcttcaggcgctgctgttcgtgcaggctgaacttctccatgcagtcatcgatgaggcttgagggggccttcttgtgggtcacggtcacctttccacagtacaggacttcgaacttctgagagttgtaaaaggcgtcctcattatctttgctgggtttggcatcctctttcatggccgctttagataattgccttatgctgctaataacatcaggaacctggctggggtctgtggcgcggaaaacgtggcaggccatctgcgactcggggtcgtcgggctgcgccttgatcaggtaggcaaagtaggtgaggtcgtggctgttgtggatgaagcgcgagatatgctgcgccttgtgctcgaagatgaataccgccgggttgggctgcgtggccgacggactagtgccccccgaggccccagcgcccggcgcggggacgcaacgcaggaagggcgcgctgagcaccaggatcacctctcgggccgccggcgccccgcagccgcccgcctcgggcttctggctgcgcctgcggatctcggccatgagccagggcagcataggcagcgtggtcctgtggtccaggcacgaccccccaacgtaccacagccggaaccgcttatcgcttggcttcccggggccgggctgagctgagacgcccggctcgggctccagggggtgcgggaacggctcatcctgaatgcagctgggcggctccataactctcgcctcaccagggcaccgcggaggccggccgggcgcaccgcgccccccactcccgcgcagaaggcgccgccgaaactgtgccaactgccgcaccgggctcccgcgcctgcctgggagcggcgcgaccccgaactccgcgcttcagcagccctgccccatgcagcacttccacgggcgcggctcggaggctccggcggcgggcaccgaggcaagcgcccggcaggcgagggcgggttaaatgggcatcctcctccttgggctggcgcctcgggcaggacctccccttcctccgtcgcgggtttgcagggtcagaggaccacgccgagggtccccgcggccgccggctccagcgctgcagccccgctgcggccgccgcgctcgcctggggcagacact

SEQ ID NO: 17030 - RNA, 4639 nt, Homo sapiens
  source 1..4639: mol_type = other RNA
tagtggtcctaaacatttcacagttctcaaaacttttcacataaaaggggaagattattaaagcttattagattctgtcaattggtcaaaagaaaaaatgtatttcaacacagcttgtcatctttggaaaaaatcaatcataattacgtttccttatactgaatttaaggtagagagacctaaattacaagcactcacaatttggtgggaaagtggcaaatccttgtcatttggtgactgtggcaccaaataaagaggaattcattcacaactgaatgagttattcaaataaaaaaagcagaaagctaatctagacattttaggtcctaaattaaatttttcaggtgtgatatttttagtttgagtaataatgctggtctagtttgctaaaaaattagcaacattctcctttaccttgagctgggtagactcagccacaatgtcctactgtctctttatgtatgtttaaagtaatgcctaaccagactcataatgcatgtagatgcaacatgctagttggcacaaagcaggcagggagaaatgaccctaccttcccaaaaaactcacaggagcatgaccagtaatcattttcctcatatagacaatgtcagtagatatcaagacagatacacataaagttacataaatgtttccaccttttcaccattgagtgaaacatgctgttctttggagaaaaaaatacattcatttttttcaagtatattgcaatatacaaagatgctctggctttgtttcactataaagacaaaaagatttcacatatgtccaagggaaatttcagtttacctttcctttggtgtggatttcatgaagttctgactaaaaaaattaatctaaatatacatctactcattttatctgaaagcatgaactatgttcattttatatatatatttatatgtacatagcaacaacaaaaaccagtctacatatgtccaatggcttaggattggcatgctctgatgagcacgaggtccacctgctgtgactaggcgctcagcaccagtattaggtggttccatcagcttcagggtccagccttgggccagcgacatgcaggctcttcctctctgtagtattctaaggagcactttctgctgaggccgtgcctcttcaattatggcttatttcctatcttggctttgttgttagggttgcagtttaggtctctcagcaacaggtcacaattgactagagcatccgcgggcagcagcttccggagttgctccactgtcttttgataagccattttttcttgttccagggtccggattaaagacttcattttggtctctctcgtcaaaagattttccaggtttgattccaaggcctggattttagtatgagctacctgtaatttttctaggaggtccatgttttgtcttttcagttggctattggccctctccagcttctccaaagtttcactatcctcacaggaatatgaagattcctgaagctcatcctgtagcacatgatattccacctcataggcatgcaactgcttagaaatatccatctcaaaaacctgggtaataattttttccatttcagaggtattcatatcaggtagcgtgtttttaagaaactcaacaatattttcaaagctctcacattccattataagtgtctcttggctgctcagtaggctgagtgcaaccttgaatataacttcagttccctgaagaaaaataatatcaaaaactctggctacaaatcctaatgaaaactgagaggcaaacaatgtgaggaaccagggggcagcataaagactggggctgatttcattttcttcaaggtgattgtagagatctctgtgatagtcatgaaggagcctggacagctggtacatttgaatctgcagcgacatcatgtcaggtctgtactgcttgcggaagccgaggtcatacatgaggaatttcagcatttcaaaggcttgctcttcactcatgtgcagaagcaggactccagccacaaagctgatcccctgacagtatcccacttctttgtccagcaaagaataggctttcaggaggttaaacagtgacagctgtcctggcccaagctgtactgaaaagtaagggtgagtaggaaacgtccttcctaaatccacgagaatcgcatgctgctgagcagtgagctgcttcaaaagttccttataggatatgtcaggaggctgttgtttattaggcaatctgtgtctgagtcggtactgtaaagccagaaactgccaaatttctcctcgtcgacttttgggaactccttctttaagaagagtatgaatatcttccatatcacatctgattttagctctgcagtttaacaacttcttatcccaagttattaagacctctttctgacatgcaccaacttcttcatagtctaatttaacttttctggactggagttcatctctgcttgcttcaagtttctggttttctttttccattcgaagtaacaagatttgttggtgtatagcttttctccacaagctcctcagttcttttgatttctttctttcttcaatcttttctgggtcatcctccccagacaggaatacaaccagcggttcctcctccatggttggagagaggggggacagtggcagcagctcgttcctgtccaatccatcttgctgttgcattgctgagggagatttgttcatgggagaagcaaccctgaggaaaatgcgctgccgccaggagatccggcgaggagtgacagaggttcctcccacacttagggactcattgctgcaggtagatgaggtcctttttctcccttctccatcacttgattctgaagcagtgtcttgtctgatttcattttcatactgtggggacagtctacctgaattctggtaaaagcttttcaggaaagagggggcagtgaaggaaggggcagagaaggaagtgtgaagacttggaagactggaggaagaattactctccttgtacatgcgtcgaactgacgaaagattgctgcactgttcactggagctctgcctcagcagaggggaacgcacaccctgagccctcccatcctgcaaattcagctttctctttgtgcttgaaggtgggtggctgaacgtgtgtgcccgtcttcgaaactgcggggagtcggaatcctcttcgggaaacgtttgccaagctgaggacggtggggacgctggcggtgtccctggtggagaatcccctggtgagtagtccttctctgaagcaagactgttggaccgttcaaaactgtccacacttccaagccgacctctcattctgttagctccccttgagaagatattttccagggagctagttaaggatctcttagctttatttttcagaatgtcaagtttgaaccttccactgcttgttgcattttctgggattgtactatttgaaatagtagaagggccttccccgatgtgcacgtgtgtcttctgcttggcttcacacagctgcctcaggtgtaaaatcacaagttcattttcttcctggtcactgactggcttcattttctgaactctttcaaagatgtcagcttgctcattatctgtcagtgatgagagatgcctctgtatcaccagcttggctcttggtgggtagagaccttcaatcctttcacagagcttatgcaaagagtgcatcgggcaggcctcacacagtttaatctgcgtcttggcactctgcagggcagccgccgtactgaaggcctgtttcagagtcagcattacctcatcaaccagagattcgctggcacactggaatacataacaaatatactggctaagtccaggctctggagactcccggcagataaagccaaagtgatccacatgctttataccctgagaacaagaggagatatctttaaaattcttttctagcacaactgatttagtgtctggactgataaggttaatctcaaatcgcccaacctggaagagcatggtcctgttcttctccgagtccgagggctggacgtgactgggtgcgctcgcgtgtctccgtcgcggctgggatttctggctgccctcgtgaactctccgttgcacgccggtgacactgctgcaccgagaccgaaactcctgctgctcatcaaagccagaatcttccaaaatccgctcagggaagcagacccgagagctggtcagggcaggctggctggccccggcaggtaagccaaggtgggtgtcggtgccgtcagcctcctccggcaggcagtctccgggggacccgggcaccaccacctccaagtcagccaggtcctctcctgggtccggaccgcgctgctccccttggatcttcaggcgctgctgttcgtgcaggctgaacttctccatgcagtcatcgatgaggcttgagggggccttcttgtgggtcacggtcacctttccacagtacaggacttcgaacttctgagagttgtaaaaggcgtcctcattatctttgctgggtttggcatcctctttcatggccgctttagataattgccttatgctgctaataacatcaggaacctttgatcaggaagccagctggaaactggaggtggtcacgaagagcaatgattttgccaaactggtgtagtcctcagtattagctctaagttctctctttct

SEQ ID NO: 17031 - RNA, 6301 nt, Homo sapiens
  source 1..6301: mol_type = other RNA
tagtggtcctaaacatttcacagttctcaaaacttttcacataaaaggggaagattattaaagcttattagattctgtcaattggtcaaaagaaaaaatgtatttcaacacagcttgtcatctttggaaaaaatcaatcataattacgtttccttatactgaatttaaggtagagagacctaaattacaagcactcacaatttggtgggaaagtggcaaatccttgtcatttggtgactgtggcaccaaataaagaggaattcattcacaactgaatgagttattcaaataaaaaaagcagaaagctaatctagacattttaggtcctaaattaaatttttcaggtgtgatatttttagtttgagtaataatgctggtctagtttgctaaaaaattagcaacattctcctttaccttgagctgggtagactcagccacaatgtcctactgtctctttatgtatgtttaaagtaatgcctaaccagactcataatgcatgtagatgcaacatgctagttggcacaaagcaggcagggagaaatgaccctaccttcccaaaaaactcacaggagcatgaccagtaatcattttcctcatatagacaatgtcagtagatatcaagacagatacacataaagttacataaatgtttccaccttttcaccattgagtgaaacatgctgttctttggagaaaaaaatacattcatttttttcaagtatattgcaatatacaaagatgctctggctttgtttcactataaagacaaaaagatttcacatatgtccaagggaaatttcagtttacctttcctttggtgtggatttcatgaagttctgactaaaaaaattaatctaaatatacatctactcattttatctgaaagcatgaactatgttcattttatatatatatttatatgtacatagcaacaacaaaaaccagtctacatatgtccaatggcttaggattggcatgctctgatgagcacgaggtccacctgctgtgactaggcgctcagcaccagtattaggtggttccatcagcttcagggtccagccttgggccagcgacatgcaggctcttcctctctgtagtattctaaggagcactttctgctgaggccgtgcctcttcaattatggcttatttcctatcttggctttgttgttagggttgcagtttaggtctctcagcaacaggtcacaattgactagagcatccgcgggcagcagcttccggagttgctccactgtcttttgataagccattttttcttgttccagggtccggattaaagacttcattttggtctctctcgtcaaaagattttccaggtttgattccaaggcctggattttagtatgagctacctgtaatttttctaggaggtccatgttttgtcttttcagttggctattggccctctccagcttctccaaagtttcactatcctcacaggaatatgaagattcctgaagctcatcctgtagcacatgatattccacctcataggcatgcaactgcttagaaatatccatctcaaaaacctgggtaataattttttccatttcagaggtattcatatcaggtagcgtgtttttaagaaactcaacaatattttcaaagctctcacattccattataagtgtctcttggctgctcagtaggctgagtgcaaccttgaatataacttcagttccctgaagaaaaataatatcaaaaactctggctacaaatcctaatgaaaactgagaggcaaacaatgtgaggaaccagggggcagcataaagactggggctgatttcattttcttcaaggtgattgtagagatctctgtgatagtcatgaaggagcctggacagctggtacatttgaatctgcagcgacatcatgtcaggtctgtactgcttgcggaagccgaggtcatacatgaggaatttcagcatttcaaaggcttgctcttcactcatgtgcagaagcaggactccagccacaaagctgatcccctgacagtatcccacttctttgtccagcaaagaataggctttcaggaggttaaacagtgacagctgtcctggcccaagctgtactgaaaagtaagggtgagtaggaaacgtccttcctaaatccacgagaatcgcatgctgctgagcagtgagctgcttcaaaagttccttataggatatgtcaggaggctgttgtttattaggcaatctgtgtctgagtcggtactgtaaagccagaaactgccaaatttctcctcgtcgacttttgggaactccttctttaagaagagtatgaatatcttccatatcacatctgattttagctctgcagtttaacaacttcttatcccaagttattaagacctctttctgacatgcaccaacttcttcatagtctaatttaacttttctggactggagttcatctctgcttgcttcaagtttctggttttctttttccattcgaagtaacaagatttgttggtgtatagcttttctccacaagctcctcagttcttttgatttctttctttcttcaatcttttctgggtcatcctccccagacaggaatacaaccagcggttcctcctccatggttggagagaggggggacagtggcagcagctcgttcctgtccaatccatcttgctgttgcattgctgagggagatttgttcatgggagaagcaaccctgaggaaaatgcgctgccgccaggagatccggcgaggagtgacagaggttcctcccacacttagggactcattgctgcaggtagatgaggtcctttttctcccttctccatcacttgattctgaagcagtgtcttgtctgatttcattttcatactgtggggacagtctacctgaattctggtaaaagcttttcaggaaagagggggcagtgaaggaaggggcagagaaggaagtgtgaagacttggaagactggaggaagaattactctccttgtacatgcgtcgaactgacgaaagattgctgcactgttcactggagctctgcctcagcagaggggaacgcacaccctgagccctcccatcctgcaaattcagctttctctttgtgcttgaaggtgggtggctgaacgtgtgtgcccgtcttcgaaactgcggggagtcggaatcctcttcgggaaacgtttgccaagctgaggacggtggggacgctggcggtgtccctggtggagaatcccctggtgagtagtccttctctgaagcaagactgttggaccgttcaaaactgtccacacttccaagccgacctctcattctgttagctccccttgagaagatattttccagggagctagttaaggatctcttagctttatttttcagaatgtcaagtttgaaccttccactgcttgttgcattttctgggattgtactatttgaaatagtctgaactctttcaaagatgtcagcttgctcattatctgtcagtgatgagagatgcctctgtatcaccagcttggctcttggtgggtagagaccttcaatcctttcacagagcttatgcaaagagtgcatcgggcaggcctcacacagtttaatctgcgtcttggcactctgcagggcagccgccgtactgaaggcctgtttcagagtcagcattacctcatcaaccagagattcgctggcacactggaatacataacaaatatactggctaagtccaggctctggagactcccggcagataaagccaaagtgatccacatgctttataccctgagaacaagaggagatatctttaaaattcttttctagcacaactgatttagtgtctggactgataaggttaatctcaaatcgcccaacctggaagagcatggtcctgttcttctccgagtccgagggctggacgtgactgggtgcgctcgcgtgtctccgtcgcggctgggatttctggctgccctcgtgaactctccgttgcacgccggtgacactgctgcaccgagaccgaaactcctgctgctcatcaaagccagaatcttccaaaatccgctcagggaagcagacccgagagctggtcagggcaggctggctggccccggcaggtaagccaaggtgggtgtcggtgccgtcagcctcctccggcaggcagtctccgggggacccgggcaccaccacctccaagtcagccaggtcctctcctgggtccggaccgcgctgctccccttggatcttcaggcgctgctgttcgtgcaggctgaacttctccatgcagtcatcgatgaggcttgagggggccttcttgtgggtcacggtcacctttccacagtacaggacttcgaacttctgagagttgtaaaaggcgtcctcattatctttgctgggtttggcatcctctttcatggccgctttagataattgccttatgctgctaataacatcaggaacctggctggggtctgtggcgcggaaaacgtggcaggccatctgcgactcggggtcgtcgggctgcgccttgatcaggtaggcaaagtaggtgaggtcgtggctgttgtggatgaagcgcgagatatgctgcgccttgtgctcgaagatgaataccgccgggttgggctgcgtggccgacggactagtgccccccgaggccccagcgcccggcgcggggacgcaacgcaggaagggcgcgctgagcaccaggatcacctctcgggccgccggcgccccgcagccgcccgcctcgggcttctggctgcgcctgcggatctcggccatgagccagggcagcataggcagcgtggtcctgtggtccaggcacgaccccccaacgtaccacagccggaaccgcttatcgcttggcttcccggggccgggctgagctgagacgcccggctcgggctccagggggtgcgggaacggctcatcctgaatgcagctgggcggctccataactctcgcctcaccagggcaccgcggaggccggccgggcgcaccgcgccccccactcccgcgcagaaggcgccgccgaaactgtgccaactgccgcaccgggctcccgcgcctgcctgggagcggcgcgaccccgaactccgcgcttcagcagccctgccccatgcagcacttccacgggcgcggctcggaggctccggcggcgggcaccgaggcaagcgcccggcaggcgagggcgggttaaatgggcatcctcctccttgggctggcgcctcgggcaggacctccccttcctccgtcgcgggtttgcagggtcagaggaccacgccgagggtccccgcggccgccggctccagcgctgcagccccgctgcggccgccgcgctcgcctggggcagacactgggtggctgggcggggaatggggctgtgggcgggagggggtgacttggggcggagctgactcctaccagggtgaccggctgtcacctggaaggtcggggctgcagggctgcggcgcggtcagtcctcaggaaaggctccggcaactactccagtggaaaataacaaaaacaaaacgtggcctcgcgggggccgctcctcctcccgccgcagctgcagcccagctcgctgctcctcctcctgccgttcccgtccctccctcgctccttccttccttccttccaggctgcttctttaatcgggctgctactccgcctcccgtccggcgggcggagagcgtcgcctgcaaaagcttatccgtgaagccgcctctccgcctcttcgcctcttccttcgacccccgcccttggggctgcagctcagagcctggcgcgggcactgcccggacccacttggcctctcttgagtcgccgcgatctccgtctcctcccgggcgtctctgctgccccctagagagggggccactcgcagtggagaactgggatttttttttaacagtatttgcttggtttcagttccttctaaagcctacacattaatttctgaattatctttcctaataatctcaaaaaacgctcgtgttttcaatcacaatattataaattccagttccaaatttcactttaaaacataatatcgacagcttgaatcttcctagttattaaagcagccaacttcttaaaatatggaaaagttatgttttatttatgttatatccccagttgagagctaatgtagagatttcttgttcttttatatatatgtggtaatacatatttccaaagaactaaaaaaaagtttggaataatttgatcattgtaattttaagacaggtagacaagtattctccctttttactcataccgaatgataattaagaattgggtaagaagtaaagacaaaataaataagaaaga

SEQ ID NO: 17032 - RNA, 4896 nt, Homo sapiens
  source 1..4896: mol_type = other RNA
tagtggtcctaaacatttcacagttctcaaaacttttcacataaaaggggaagattattaaagcttattagattctgtcaattggtcaaaagaaaaaatgtatttcaacacagcttgtcatctttggaaaaaatcaatcataattacgtttccttatactgaatttaaggtagagagacctaaattacaagcactcacaatttggtgggaaagtggcaaatccttgtcatttggtgactgtggcaccaaataaagaggaattcattcacaactgaatgagttattcaaataaaaaaagcagaaagctaatctagacattttaggtcctaaattaaatttttcaggtgtgatatttttagtttgagtaataatgctggtctagtttgctaaaaaattagcaacattctcctttaccttgagctgggtagactcagccacaatgtcctactgtctctttatgtatgtttaaagtaatgcctaaccagactcataatgcatgtagatgcaacatgctagttggcacaaagcaggcagggagaaatgaccctaccttcccaaaaaactcacaggagcatgaccagtaatcattttcctcatatagacaatgtcagtagatatcaagacagatacacataaagttacataaatgtttccaccttttcaccattgagtgaaacatgctgttctttggagaaaaaaatacattcatttttttcaagtatattgcaatatacaaagatgctctggctttgtttcactataaagacaaaaagatttcacatatgtccaagggaaatttcagtttacctttcctttggtgtggatttcatgaagttctgactaaaaaaattaatctaaatatacatctactcattttatctgaaagcatgaactatgttcattttatatatatatttatatgtacatagcaacaacaaaaaccagtctacatatgtccaatggcttaggattggcatgctctgatgagcacgaggtccacctgctgtgactaggcgctcagcaccagtattaggtggttccatcagcttcagggtccagccttgggccagcgacatgcaggctcttcctctctgtagtattctaaggagcactttctgctgaggccgtgcctcttcaattatggcttatttcctatcttggctttgttgttagggttgcagtttaggtctctcagcaacaggtcacaattgactagagcatccgcgggcagcagcttccggagttgctccactgtcttttgataagccattttttcttgttccagggtccggattaaagacttcattttggtctctctcgtcaaaagattttccaggtttgattccaaggcctggattttagtatgagctacctgtaatttttctaggaggtccatgttttgtcttttcagttggctattggccctctccagcttctccaaagtttcactatcctcacaggaatatgaagattcctgaagctcatcctgtagcacatgatattccacctcataggcatgcaactgcttagaaatatccatctcaaaaacctgggtaataattttttccatttcagaggtattcatatcaggtagcgtgtttttaagaaactcaacaatattttcaaagctctcacattccattataagtgtctcttggctgctcagtaggctgagtgcaaccttgaatataacttcagttccctgaagaaaaataatatcaaaaactctggctacaaatcctaatgaaaactgagaggcaaacaatgtgaggaaccagggggcagcataaagactggggctgatttcattttcttcaaggtgattgtagagatctctgtgatagtcatgaaggagcctggacagctggtacatttgaatctgcagcgacatcatgtcaggtctgtactgcttgcggaagccgaggtcatacatgaggaatttcagcatttcaaaggcttgctcttcactcatgtgcagaagcaggactccagccacaaagctgatcccctgacagtatcccacttctttgtccagcaaagaataggctttcaggaggttaaacagtgacagctgtcctggcccaagctgtactgaaaagtaagggtgagtaggaaacgtccttcctaaatccacgagaatcgcatgctgctgagcagtgagctgcttcaaaagttccttataggatatgtcaggaggctgttgtttattaggcaatctgtgtctgagtcggtactgtaaagccagaaactgccaaatttctcctcgtcgacttttgggaactccttctttaagaagagtatgaatatcttccatatcacatctgattttagctctgcagtttaacaacttcttatcccaagttattaagacctctttctgacatgcaccaacttcttcatagtctaatttaacttttctggactggagttcatctctgcttgcttcaagtttctggttttctttttccattcgaagtaacaagatttgttggtgtatagcttttctccacaagctcctcagttcttttgatttctttctttcttcaatcttttctgggtcatcctccccagacaggaatacaaccagcggttcctcctccatggttggagagaggggggacagtggcagcagctcgttcctgtccaatccatgtatattctctggctgtgaggaacgagattaagtggctaggtatcagtgatctccgaaggtctacatcgatcatcagaatccgtcaggagcatagccactgagcaatgctgggcctctcctggctgagcacagtactccctctgctcattcctcctgcaacacctttttctttttctttttcaatttttattttaggttgaaggggtccatgtgcaggtttgctacatgggtaaattacgtgactctggggtacaatgtacaaatgaaatgacttcgccacccaggtagtgagcacagtacctgagaggtagtttttcaatcctcatcctcctcccaccctccaccctcaagggggtcccggtgtctaatgttcccttctttgtttctatgtgtactcaatgtttagatcccgcttataagtgagaacatgcagtatttggttttctgctcctgtgttaattcttaggataataacctccagctacatccatgtggctccaaaggacatgatttcattatttttcatggctgtgcagtattccatgtgcaacactcccttaacaggtgactcattctctcccttcctactgccaatgattttcctattaacaaccataatcacatctcttaaaacatttcaatggttgcttatatcgcaagaacaaattgggactagcatttaagttccttcagattctggtctccactcagatttccagcctcatatctcaatcttctattctttgcattcatcatgctgaatttctcatgattctctgatctgcaaagttcactcaaatgactccagagcttcgtcattccttccttctaaagcatggttcttccagcaacgagtttaaataaacatctaattgttctgtgaagctttttctgaccacctcgggcagagttaacttcatctttagtaataccagttgttttcttctattttcttctttttttatatatattcattgacctctgcctttacttttattatttacttccatacgttttactgttgttgttttaaaattttaatacctggctctcttactagctttttgagttgaacactcagtgtaactaatttttggccttcttgattttatatcaatatattcatggcttttaactgctccctagatccgtttcaataggtaaggctctaagcattgaattttcttccttctagcttctaagagtagttttctattcccaaacacatgtcattctacttgtcttctaatccttgatttctttctttttttggcattgtggtcagagaatatttgtataaatgattatgattatttggatttcaaaaagatttacttaaaaatctttgtggacaggtacataattacattttatgaatgttccaagtgtgctaaaaatgaatgagttttctccataggaggcgaagttctctataaatattaggtcaagcttatttatttgtgttactcaaatattatttatatttaatttctaaagatgagtatgttaaaatctcccacaggagctattaatttatcgatttcactccagaattcttttaggtgttattttctagctctcaaagctacatcattatgtatgttctcatgattgttctatctgtttgtttactgttacatgtgcttgcctctttggatgcttttgctttagtttaataggtcaattactcaaagagagctgcctgtgctctcttttgctcagtatttgcctagtatattgtatatattcctttattgctcaatatttctatgtcagtttgttttatgtgtggctcttataaaaggctatgttgcttttctaataataaaaagatctttggaagctgaggtaagatgattgcttgagcccaggagttcaaggctacagtgagctatgattacaccactgcaaccccagcctgggcaacagagcaaggcccaatctctgggaaaaaaaaaaagaaagaaagaaagaaagaaagaaaaaggacatacagcttctttcctagcactatcacagttccgtctaccttgtggagtaggcccaagtacaggtttttggaaactgtctcactcattcattcattcaacaagcaggtattgaatgcctaatgttttctaatgatacctgaaagagaaaccactgtatcacatacagaaagatatttctacactgtaatcacttaaatctctttatacacagcacgtgcattccattagctaatttctgacactcagagggat

SEQ ID NO: 17033 - RNA, 1387 nt, Homo sapiens
  source 1..1387: mol_type = other RNA
tagtggtcctaaacatttcacatttcgtacagatcgaggacggtgttcactagtacatacgtgtcataaactggactttcttggctcaatgacaggtgtagaaaatcgtgattcttataagactctctcataaagtccaagaacaaacatattcaacaaaaaaaaaatctaaactatgcacttttgtttcttaaaaaacaaaacagtgtaaatcagattttaagctaggaagaggaaatccgttttttagcctcgcggctgtatccatcctcctgttcagctgaacggatgaagcacaatagcgacaactttgttacagactaaaatccaacaggtaattccaacaccacctgctactctagtaggaaaggctaccaggcggtctagaggggttatccatttactcggcacgacagccacagggacagaataatacttccaaatgagtgagatcatcagggcagcctgcaatacgtagaaagcgacacttatcacccattttatcttggctaattgagctgtccgagctttcacaacaggactaaattttcctccttatttcccagtgtgcacagtacacgaacccctggtgggagtccagcttgtcctgggcctggacaggcccctctgtctgttttcctagccacagagacagctctctgactgtgcacacactgtgaccggggtccctcagcacacgggctgccctgagaaagcgctcttcatcacaggacactggacccgggaggtgacactcagaagaggacactgctgggcatttttctagagagtggaacaaaagcctctgggaatccactgtgagactttttttctgggcttctctcagaaaagtgatgaatttaaaaatgaaaacctacaatttttaagagttagcttaaaattttaaagagttggctctgaggaaaatctgagaggatcttagatatttctgtgcttagaaagcaaaggttcaccagcaaataagaggaaagtaatacttattactgagtttcctccagataacttaagtttccatcaatattcagaacatccaagaagcaaagtatgtattctactaatcttcacatacagacttctctattcatccgctctcatgaagcctccaggctgcaagggacacagtaccatgggttttgagcttatccgtcatcttgttgatctttctttccagcctggcatatctggcaaactcgtccatcatgttgactgtggagagctcctgcttcatgtcctggatctccgctctcatctgtgactcctgctccgcgtccttctgcagcaccctggacataggtctcctccgcctgccgcacagtagggacaactctccatttagagcttggaagccgcgacccgccagtcgcct

SEQ ID NO: 17034 - RNA, 1473 nt, Homo sapiens
  source 1..1473: mol_type = other RNA
tagtggtcctaaacatttcacatttcgtacagatcgaggacggtgttcactagtacatacgtgtcataaactggactttcttggctcaatgacaggtgtagaaaatcgtgattcttataagactctctcataaagtccaagaacaaacatattcaacaaaaaaaaaatctaaactatgcacttttgtttcttaaaaaacaaaacagtgtaaatcagattttaagctaggaagaggaaatccgttttttagcctcgcggctgtatccatcctcctgttcagctgaacggatgaagcacaatagcgacaactttgttacagactaaaatccaacaggtaattccaacaccacctgctactctagtaggaaaggctaccaggcggtctagaggggttatccatttactcggcacgacagccacagggacagaataatacttccaaatgagtgagatcatcagggcagcctgcaatacgtagaaagcgacacttatcacccattttatcttggctaattgagctgtccgagctttcacaacaggactaaattttcctccttatttcccagtgtgcacagtacacgaacccctggtgggagtccagcttgtcctgggcctggacaggcccctctgtctgttttcctagccacagagacagctctctgactgtgcacacactgtgaccggggtccctcagcacacgggctgccctgagaaagcgctcttcatcacaggacactggacccgggaggtgacactcagaagaggacactgctgggcatttttctagagagtggaacaaaagcctctgggaatccactgtgagactttttttctgggcttctctcagaaaagtgatgaatttaaaaatgaaaacctacaatttttaagagttagcttaaaattttaaagagttggctctgaggaaaatctgagaggatcttagatatttctgtgcttagaaagcaaaggttcaccagcaaataagaggaaagtaatacttattactgagtttcctccagataacttaagtttccatcaatattcagaacatccaagaagcaaagtatgtattctactaatcttcacatacagacttctctattcatccgctctcatgaagcctccaggctgcaagggacacagtaccatgggttttgagcttatccgtcatcttgttgatctttctttccagcctggcatatctggcaaactcgtccatcatgttgactgtggagagctcctgcttcatgtcctggatctccgctctcatctgtgactcctgctccgcgtccttctgcagcaccctggacatgaaggatgagaaggacgggaggaggatcctaagaacattgcatccaaacacgaagctgagcaccagcaaccacgcccagtggtcggccgcggctgagctcatcccggacgctcctggctgtgctgggtccgctacggcagctccatggggaccacaacaac

SEQ ID NO: 17035 - RNA, 774 nt, Homo sapiens
  source 1..774: mol_type = other RNA
tagtggtcctaaacatttcacatttcgtacagatcgaggacggtgttcactagtacatacgtgtcataaactggactttcttggctcaatgacaggtgtagaaaatcgtgattcttataagactctctcataaagtccaagaacaaacatattcaacaaaaaaaaaatctaaactatgcacttttgtttcttaaaaaacaaaacagtgtaaatcagattttaagctaggaagaggaaatccgttttttagcctcgcggctgtatccatcctcctgttcagctgaacggatgaagcacaatagcgacaactttgttacagactaaaatccaacaggtaattccaacaccacctgctactctagtaggaaaggctaccaggcggtctagaggggttatccatttactcggcacgacagccacagggacagaataatacttccaaatgagtgagatcatcagggcagcctgcaatacgtagaaagcgacacttatcacccattttatcttggctaattgagctgtccgagctttcacatgggttttgagcttatccgtcatcttgttgatctttctttccagcctggcatatctggcaaactcgtccatcatgttgactgtggagagctcctgcttcatgtcctggatctccgctctcatctgtgactcctgctccgcgtccttctgcagcaccctggacataggtctcctccgcctgccgcacagtagggacaactctccatttagagcttggaagccgcgacccgccagtcgcct

SEQ ID NO: 17036 - RNA, 1295 nt, Homo sapiens
  source 1..1295: mol_type = other RNA
tagtggtcctaaacatttcacatttcgtacagatcgaggacggtgttcactagtacatacgtgtcataaactggactttcttggctcaatgacaggtgtagaaaatcgtgattcttataagactctctcataaagtccaagaacaaacatattcaacaaaaaaaaaatctaaactatgcacttttgtttcttaaaaaacaaaacagtgtaaatcagattttaagctaggaagaggaaatccgttttttagcctcgcggctgtatccatcctcctgttcagctgaacggatgaagcacaatagcgacaactttgttacagactaaaatccaacaggtaattccaacaccacctgctactctagtaggaaaggctaccaggcggtctagaggggttatccatttactcggcacgacagccacagggacagaataatacttccaaatgagtgagatcatcagggcagcctgcaatacgtagaaagcgacacttatcacccattttatcttggctaattgagctgtccgagctttcacatgggttttgagcttatccgtcatcttgttgatctttctttccagcctggcatatctggcaaactcgtccatcatgttgactgtggagagctcctgcttcatgtcctggatctccgctctcatctgtgactcctgctccgcgtccttctgcagcaccctggacatcccaagaatgtgggctcctggacgcgaggatccatctctccgggacctggaacagctgacttcgcccgccaggcctctgggaaaccctggccgagggctgctcgaatgcctctaggaaccaggattaacggaaacgaggctgacagcggggcactaggaactcccagtgtgaggttcgccgccgccacccacagccagaagagtccagggttgcccggtgtttctcccaaccccctagaacccagaaagtctgattttggggtaaagcgtcgtaccttttagacgctaacaactatctcaaaaaagcttacggaccaaccaagacgctactacggccttcagtcgcccagttgagacccctgtacctacgccagacccgccgggggactggggcggcatccccaccggcccttgggaggccaggcagccacttacgaaggatgagaaggacgggaggaggatcctaagaacattgcatccaaacacgaagctgagcaccagcaaccacgcccagtggtcggccgcggctgagctcatcccggacgctcctggctgtgctgggtccgctacggcagctccatggggaccacaacaac

SEQ ID NO: 17037 - RNA, 930 nt, Homo sapiens
  source 1..930: mol_type = other RNA
tagtggtcctaaacatttcacatttcgtacagatcgaggacggtgttcactagtacatacgtgtcataaactggactttcttggctcaatgacaggtgtagaaaatcgtgattcttataagactctctcataaagtccaagaacaaacatattcaacaaaaaaaaaatctaaactatgcacttttgtttcttaaaaaacaaaacagtgtaaatcagattttaagctaggaagaggaaatccgttttttagcctcgcggctgtatccatcctcctgttcagctgaacggatgaagcacaatagcgacaactttgttacagactaaaatccaacaggtaattccaacaccacctgctactctagtaggaaaggctaccaggcggtctagaggggttatccatttactcggcacgacagccacagggacagaataatacttccaaatgagtgagatcatcagggcagcctgcaatacgtagaaagcgacacttatcacccattttatcttggctaattgagctgtccgagctttcacatgggttttgagcttatccgtcatcttgttgatctttctttccagcctggcatatctggcaaactcgtccatcatgttgactgtggagagctcctgcttcatgtcctggatctccgctctcatctgtgactcctgctccgcgtccttctgcagcaccctggacatctacgccagacccgccgggggactggggcggcatccccaccggcccttgggaggccaggcagccacttacgaaggatgagaaggacgggaggaggatcctaagaacattgcatccaaacacgaagctgagcaccagcaaccacgcccagtggtcggccgcggctgagctcatcccggacgctcctggctgtgctgggtccgctacggcagctccatggggaccacaacaac

SEQ ID NO: 17038 - RNA, 1020 nt, Homo sapiens
  source 1..1020: mol_type = other RNA
tagtggtcctaaacatttcacatttcgtacagatcgaggacggtgttcactagtacatacgtgtcataaactggactttcttggctcaatgacaggtgtagaaaatcgtgattcttataagactctctcataaagtccaagaacaaacatattcaacaaaaaaaaaatctaaactatgcacttttgtttcttaaaaaacaaaacagtgtaaatcagattttaagctaggaagaggaaatccgttttttagcctcgcggctgtatccatcctcctgttcagctgaacggatgaagcacaatagcgacaactttgttacagactaaaatccaacaggtaattccaacaccacctgctactctagtaggaaaggctaccaggcggtctagaggggttatccatttactcggcacgacagccacagggacagaataatacttccaaatgagtgagatcatcagggcagcctgcaatacgtagaaagcgacacttatcacccattttatcttggctaattgagctgtccgagctttcacatgggttttgagcttatccgtcatcttgttgatctttctttccagcctggcatatctggcaaactcgtccatcatgttgactgtggagagctcctgcttcatgtcctggatctccgctctcatctgtgactcctgctccgcgtccttctgcagcaccctggacatcttttagacgctaacaactatctcaaaaaagcttacggaccaaccaagacgctactacggccttcagtcgcccagttgagacccctgtacctacgccagacccgccgggggactggggcggcatccccaccggcccttgggaggccaggcagccacttacgaaggatgagaaggacgggaggaggatcctaagaacattgcatccaaacacgaagctgagcaccagcaaccacgcccagtggtcggccgcggctgagctcatcccggacgctcctggctgtgctgggtccgctacggcagctccatggggaccacaacaac

SEQ ID NO: 17039 - RNA, 860 nt, Homo sapiens
  source 1..860: mol_type = other RNA
tagtggtcctaaacatttcacatttcgtacagatcgaggacggtgttcactagtacatacgtgtcataaactggactttcttggctcaatgacaggtgtagaaaatcgtgattcttataagactctctcataaagtccaagaacaaacatattcaacaaaaaaaaaatctaaactatgcacttttgtttcttaaaaaacaaaacagtgtaaatcagattttaagctaggaagaggaaatccgttttttagcctcgcggctgtatccatcctcctgttcagctgaacggatgaagcacaatagcgacaactttgttacagactaaaatccaacaggtaattccaacaccacctgctactctagtaggaaaggctaccaggcggtctagaggggttatccatttactcggcacgacagccacagggacagaataatacttccaaatgagtgagatcatcagggcagcctgcaatacgtagaaagcgacacttatcacccattttatcttggctaattgagctgtccgagctttcacatgggttttgagcttatccgtcatcttgttgatctttctttccagcctggcatatctggcaaactcgtccatcatgttgactgtggagagctcctgcttcatgtcctggatctccgctctcatctgtgactcctgctccgcgtccttctgcagcaccctggacatgaaggatgagaaggacgggaggaggatcctaagaacattgcatccaaacacgaagctgagcaccagcaaccacgcccagtggtcggccgcggctgagctcatcccggacgctcctggctgtgctgggtccgctacggcagctccatggggaccacaacaac

SEQ ID NO: 17040 - RNA, 794 nt, Homo sapiens
  source 1..794: mol_type = other RNA
tagtggtcctaaacatttcacatttcgtacagatcgaggacggtgttcactagtacatacgtgtcataaactggactttcttggctcaatgacaggtgtagaaaatcgtgattcttataagactctctcataaagtccaagaacaaacatattcaacaaaaaaaaaatctaaactatgcacttttgtttcttaaaaaacaaaacagtgtaaatcagattttaagctaggaagaggaaatccgttttttagcctcgcggctgtatccatcctcctgttcagctgaacggatgaagcacaatagcgacaactttgttacagactaaaatccaacaggtaattccaacaccacctgctactctagtaggaaaggctaccaggcggtctagaggggttatccatttactcggcacgacagccacagggacagaataatacttccaaatgagtgagatcatcagggcagcctgcaatacgtagaaagcgacacttatcacccattttatcttggctaattgagctgtccgagctttcacatgggttttgagcttatccgtcatcttgttgatctttctttccagcctggcatatctggcaaactcgtccatcatgttgactgtggagagctcctgcttcatgtcctggatctccgctctcatctgtgactcctgctccgcgtccttctgcagcaccctggacatgccagacccgccgggggactggggcggcatccccaccggcccttgggaggccaggcagccacttacgaaggatgagaaggacgggaggaggatcc

SEQ ID NO: 17041 - RNA, 686 nt, Homo sapiens
  source 1..686: mol_type = other RNA
tagtggtcctaaacatttcacattttttattgtattagacattatgctcttaattcagtttcccattgtccattgcttatatattgtaaaagaaatggtttttatatatcaactggtgtcctgtggctttggaacactcacctattggttttttataggttacaagtattttctatgtacactaacctgtcatctaggaatagaggcagattttcatcttccttcccaatctgtgctttgtatttctttttcttgtcttactgcagtggctgtgaattctagtacaacactgaggggaaaatagtgagaagtgacagtcttaccttatttcttaccttagggaaaataaattcagtttttcaccattcattatgttatctgtagattctccatagattatctttatcagattaaggaagttctcttagatctctagttttgctgaaagtttttctcaataatgggccttgaagtttttcacatttttttctgcatctggaactgaaagatgatgtgttcggcttcaatagatcctgctcgtcacatcagggacagtagtcaatacttttgtatttggacactgggaatcaaggcagaagattctcccttcttttagcttctttaaaagatgttcaattaaagttatgtatgcataatgacattttgatcaataacaggccatgcat

SEQ ID NO: 17042 - RNA, 1294 nt, Homo sapiens
  source 1..1294: mol_type = other RNA
tatacaagggcaagctctctgtggcaccaccctctgagtctcacacccccaggtctcccccacaccccaatgccatcagccaggcccaatggagcagagggctccagatcactcacacccattttccacataagttccccagtgctgggttccaaaaagcatctcacccttccaggcccccaaacccagcaacaatgttcacccaccctgagggtggcaagtccaaagcaggcagaacttggccagcaggtccaaccctccatgttccaagcctcttctgcacctctgtttctggccgaggaataaacactgggggcaccatccttaggctgagcccctggaagtcccactctccaaggatgtactgcaccggcatcctctgcaatcgacggctactcagctcccggatacactgtagttgctgagaggtcaagggctgggtccaaagtgccggcctcaggctctgaaatgttttggctccaaggacatgagccacgatgtactcactggattcccgggcctcagggatacccctcttctcaaagaccccagtccagtggctgaccagttctatggcactggataacccagccagaggtggttggggttgccatgagctgaaggcccagccccgggtacttcccctcctccctgggccagacaggagggcccacagcattcggccccaaagctccatgtctcagggaaaggttctccagagtgcttccaggttcccaagtctgctttatgatgtcagctgctgaggtgagtgctgagagtggcccctggacccagctgggtggagatggagaggtcacaagctctggtgccccaaaatggctctggtcctcagatatagttggttgccaccctgcctgaaaggctgccccacccacccaccagccggagaagctgccccgaactggacgcccggacgtgcgtggcccgtcgcgcgctccctcggacgccccgcttccggggtcggcgcctttaagaaaaggctcgggcggacgccgtagcccagcttcagtgttcctatcgctggtgggttcctcccaggagacccctgcggatgggtggggaggctgtgaattccactccctctacgctcgcaggcctgcatacaggaaagtgcggggatgtgtgtggggttgacccttgggggcccggacctgccggtcttccttaaaatcacagcagggatttggctccagcccaaggggattgctccgagctggcgtttaggaaccaggccgggaggtgtgtgggcggagcccagtagcctgccggaaag

SEQ ID NO: 17043 - RNA, 556 nt, Homo sapiens
  source 1..556: mol_type = other RNA
tatagagagcaggaagattaatgtctgtagcaagaaaaactatatcctctccctgtagggttgtaatggacttatgctgatgcatcagatggggcattacagcatccagagagccttgccatttacaggaagcaccagggcacggacaggaataaggcctaaactcacagagctcttcatggtctgctttttctgtgtgtggcagagttatttcacatccagaagacgcatatttacaggggaaaagtactgaattagccactttctccatagccaagttgcgaatggatcccaaagggccccggcaagttggacaacatgtgagctttgggcgacagttgctacaaacaagatggccactctgacattgaagaatgggcggtaacacatagtcaaagcagactggacactcaaaaagactcgccaagtcattgttggatgcagttgtgccagtcagggcaggcaccctctgggatggtggacacttcgaggtaccggtaggtaatgctgtagcagtctgacggctcatttctccgccatgttggccgcacacccc

SEQ ID NO: 17044 - RNA, 741 nt, Homo sapiens
  source 1..741: mol_type = other RNA
tatagagagcaggaagattaatgtctgtagcaagaaaaactatatcctctccctgtagggttgtaatggacttatgctgatgcatcagatggggcattacagcatccagagagccttgccatttacaggaagcaccagggcacggacaggaataaggcctaaactcacagagctcttcatggtctgctttttctgtgtgtggcagagttatttcacatccagaagacgcatatttacaggggaaaagtactgaattagccactttctccatagccaagttgcgaatggatcccaaagggccccggcaagttggacaacatgtgagctttgggcgacagttgctacaaacaagatggccactctgacattgaagaatgggcggtaacacatagtcaaagcagactggacactcaaaaagactcgccaagtcattgttggatgcagttgtgccagtcagggcaggcaccctctgggatggtggacacttcgaggtaccggtaggtaatgctgtagcagtctgacggctcatttctgtgggcggagagcgcgcctcggaccccggtcctggcaccaacgcgctccgtcgccaacccccgccaccgcgggcagcgccaccgcctcttcccggcgccgagaccgacgggacaccctgggccgccgccgcctctcgagagcgcgccccgcaacggccgccccggctcccccctggccgccgccgccgccgccgtttcgcgcgtcctc

SEQ ID NO: 17045 - RNA, 822 nt, Homo sapiens
  source 1..822: mol_type = other RNA
tatagagagcaggaagattaatgtctgtagcaagaaaaactatatcctctccctgtagggttgtaatggacttatgctgatgcatcagatggggcattacagcatccagagagccttgccatttacaggaagcaccagggcacggacaggaataaggcctaaactcacagagctcttcatggtctgctttttctgtgtgtggcagagttatttcacatccagaagacgcatatttacaggggaaaagtactgaattagccactttctccatagccaagttgcgaatggatcccaaagggccccggcaagttggacaacatgtgagctttgggcgacagttgctacaaacaagatggccactctgacattgaagaatgggcggtaacacatagtcaaagcagactggacactcaaaaagactcgccaagtcattgttggatgcagttgtgccagtcagggcaggcaccctctgggatggtggacacttcgaggtaccggtaggtaatgctgtagcagtctgacggctcatttcttataaactagtggattctcttaaactgcaggggtgcccaggacacagtgtcccctgaggatgccgcacaccagtcttgaagtgctggatcgttgacgtcaggcacccagaagcaacttctgcctctggaattctcaaacgtgcttttcttggcttagtttgtgcctgctctcctctagaagagtccaagttacttcttactttccccacttccctaatgaaacctggtcatcaaagcagtttaaattgccatctcatcagcgctttacacggggcagggggagctgctt

SEQ ID NO: 17046 - RNA, 2157 nt, Homo sapiens
  source 1..2157: mol_type = other RNA
tatagagagcaggaagattaatgtctgtagcaagaaaaactatatcctctccctgtagggttgtaatggacttatgctgatgcatcagatggggcattacagcatccagagagccttgccatttacaggaagcaccagggcacggacaggaataaggcctaaactcacagagctcttcatggtctgctttttctgtgtgtggcagagttatttcacatccagaagacgcatatttacaggggaaaagtactgaattagccactttctccatagccaagttgcgaatggatcccaaagggccccggcaagttggacaacatgtgagctttgggcgacagttgctacaaacaagatggccactctgacattgaagaatgggcggtaacacatagtcaaagcagactggacactcaaaaagactcgccaagtcattgttggatgcagttgtgccagtcagggcaggcaccctctgggatggtggacacttcgaggtaccggtaggtaatgctgtagcagtctgacggctcatttcttataaactagtggattctcttaaactgcaggggtgcccaggacacagtgtcccctgaggatgccgcacaccagtcttgaagtgctggatcgttgacgtcaggcacccagaagcaacttctgcctctggaattctcaaacgtgcttttcttggcttagtttgtgcctgctctcctctagaagagtccaagttacttcttactttccccacttccctgggtaaatcaacaaagtggaggcagaaatctgtctggattgtttggtaagttgtattaagacagaagaggccatggaaactcactgaacttggtatttacatgtatacaatctcagtcttttcatcccttgatcctaatgaaacctggtcatcaaagcagtttaaattgccatctcatcagcgctttacacggggcagggggagctgctttgagccttcagagaccatttcctccatcttccttttgtcctggggagctcccttagaatatgtgtccacttcttgtcactttgagttgatgctttatagactcctaaagatggggggtgcataatgaagaaaaccagcacccttccccaggtgggggaatacagatgttgatgggtcctgagtggggatccttgaccctcgtgccttgtctaagcttcagatgggaggcaaaacatccatccagactgtggagccgatgaccagagagcacccagtaccatttaatgggaaaggccctgggcaggcaccagacacagagaaagaggaatgagctggagccaaggaggcctccccagtgaaacgctgccaggcgcccaacaccagcagagactctagacctggggcacggaggagcaggtgtcccagcagcaagctgtgaggacaggtgggaccccaggccttgatcgcaagccctcgatgacttcctcgatagcaagccctgaggaaaggggcaggcccccaacattgcctgagatgacatttctgccacctagcataacaggggctcagaataaaattgagttataaaaaaaaaagtaagtcccattttactctaatgaggcatcctttaaagaccccaagtgtgcagcctggagcttggcttgctgcatcgtgtggaaacagtatacaccgttctccttatggggcacgggcagcaccactcagcaaacctgttgcttttgtgccttcatgaaagtctttcaggagtagtctacacagcaggtctctcatcactctggggagcccagtggctcagaagccccctgtagtccggggaagtcctgctaaagtacatccagcacaaacaagcttccaagcacaaacaagcttccaactcacccacctccctgtgttcagcttggaatagcaaataccaaaaagtaaacatttgaaactgatggcctcaatgtacagtctggagttcatgggtctaagtttcccactggcgttcccctcaaggtccaccattacctgggctccactgcctgctaggcttcatgacccctctccagggaggcagcatcccaaacacagctgggcgggcatgtccttccttcctctggccccatccttcaccatcccactgcatgccatccacactgcccggtaagcagccctggggacctcaagacttcact

SEQ ID NO: 17047 - RNA, 1387 nt, Homo sapiens
  source 1..1387: mol_type = other RNA
tatagagagcaggaagattaatgtctgtagcaagaaaaactatatcctctccctgtagggttgtaatggacttatgctgatgcatcagatggggcattacagcatccagagagccttgccatttacaggaagcaccagggcacggacaggaataaggcctaaactcacagagctcttcatggtctgctttttctgtgtgtggcagagttatttcacatccagaagacgcatatttacaggggaaaagtactgaattagccactttctccatagccaagttgcgaatggatcccaaagggccccggcaagttggacaacatgtgagctttgggcgacagttgctacaaacaagatggccactctgacattgaagaatgggcggtaacacatagtcaaagcagactggacactcaaaaagactcgccaagtcattgttggatgcagttgtgccagtcagggcaggcaccctctgggatggtggacacttcgaggtaccggtaggtaatgctgtagcagtctgacggctcatttcttataaactagtggattctcttaaactgcaggggtgcccaggacacagtgtcccctgaggatgccgcacaccagtcttgaagtgctggatcgttgacgtcaggcacccagaagcaacttctgcctctggaattctcaaacgtgcttttcttggcttagtttgtgcctgctctcctctagaagagtccaagttacttcttactttccccacttccctgggtaaatcaacaaagtggaggcagaaatctgtctggattgtttggtaagttgtattaagacagaagaggccatggaaactcactgaacttggtatttacatgtatacaatctcagtcttttcatcccttgatcctaatgaaacctggtcatcaaagcagtttaaattgccatctcatcagcgctttacacggggcagggggagctgctttgagccttcagagaccatttcctccatcttccttttgtcctggggagctcccttagaatatgtgtccacttcttgtcactttgagttgatgctttatagactcctaaagatggggggtgcataatgaagaaaaccagcacccttccccaggtgggggaatacagatgttgatgggtcctgagtggggatccttgaccctcgtgccttgtctaagcttcagatgggaggcaaaacatccatccagactgtggagccgatgaccagagagcacccagtaccatttaatgggaaaggccctgggctccactgcctgctaggcttcatgacccctctccagggaggcagcatcccaaacacagctgggcgggcatgtccttccttcctctggccccatccttcaccatcccactgcatgccatccacactgcc

SEQ ID NO: 17048 - RNA, 1032 nt, Homo sapiens
  source 1..1032: mol_type = other RNA
tatagagagcaggaagattaatgtctgtagcaagaaaaactatatcctctccctgtagggttgtaatggacttatgctgatgcatcagatggggcattacagcatccagagagccttgccatttacaggaagcaccagggcacggacaggaataaggcctaaactcacagagctcttcatggtctgctttttctgtgtgtggcagagttatttcacatccagaagacgcatatttacaggggaaaagtactgaattagccactttctccatagccaagttgcgaatggatcccaaagggccccggcaagttggacaacatgtgagctttgggcgacagttgctacaaacaagatggccactctgacattgaagaatgggcggtaacacatagtcaaagcagactggacactcaaaaagactcgccaagtcattgttggatgcagttgtgccagtcagggcaggcaccctctgggatggtggacacttcgaggtaccggtaggtaatgctgtagcagtctgacggctcatttcttttctcttccttgtcctggccgctggtaaacatgtgaacaagactcccctccaggagtacagagaaggtggagtagcctttcccgtcatgagaagtcaggccacgcattgcgtttcccccaagaagtaaaggaacaggcccctcctgggctctttctgctcctaagcacagaagacccaaattcgcgtctgaggtcaggatccaaataccatttacttctcagaagcaccagttacagaggtggagaaaggaagcctttccatccccaggaggcaaccacacctccctgtgagctcaaattcgactgcatctccaaaaatgggagccacagctgcgctgtcctccaatgtgccctaagctttcgtctgtctcccaagtttgttttctccagattcactgggtagggtcctgcccagctccagtggaggccacggatgcagggggcgacgcgctggctgagaaggaagtgcgctccctgagccagctcaagagttactgc

SEQ ID NO: 17049 - RNA, 2611 nt, Homo sapiens
  source 1..2611: mol_type = other RNA
tatagggattggagccgtggcgcacggcggggacagccagcggagggttctgacactgagcaagggggctcaaaaggaggcaggacagtggcacctccctctctcaacccaggctgctggccaggccaacacagccgttcctctattcccacttgcctcttctcccgccagtggtcacaggaagaggtgtgggtcactggacctcatcactggctggacccaccatcccagtgctgggacccccactgaagggctgacttcagggtctggacttggtccccagaggagtggctgaaggaactagggatgttcagcctaggacaagggctgtcacaaggaaacagcactggggggtgggacaaacttcagctcaaccagaagtgcagtatgtggctaagggctgtccaaagacagaaaggacatccatccaacgaggcctacaagctgaggctggagaagccatggtgacagtgccatggtggagtcatggttgggtgggtgggtggctggtcaccccagactgcagtctttaggcctgtcctccctggggtctctgctcacgcacatcaaagctgtcaggagccaagctcaaccctcacacactccagagggatgggcacaggctcccgttatgcgaggcacatcctgcacgtacccagcccagtagaggggtgttaagagtcctgccaggccctggtactgtggctgcagccgtaccacgctcccctcccagcggctcccccgtgaggcctcactctgagggaaggcgcactgagaacccatggcatggtcctatttattttcagacattctcgcttcacagaaagaaacagggtgaggggctcaagagagaggctgcccaagggagaagcacgggaacgctgaactggccgaggggcttgtcctcatcctcaggggtagggggaagcccccatctgccagtctggctggaagggaatagatatagagcagaggccctgagtggaaggtgacagttaaccaaacagccaaggccaaggagaggaggggccctaaggcttagagaggccctgaggaccaaccttgctctgccatctgaccttgcccttgtaggcctcctctgaactcccaaaatgtgacctatgccatcaccgaggccgcaggaacaagaggtgggtgtccatgacattggtacctgtcatccctgtgtgcagcaggtgtgccccaccctggaggcagcagaagaaggtatgtgagtcattgtgggctaggaaggtggctatgtccaggccctcagctgcagcctggctggcaagctcaggtgtgacccaggccccagcagcctctgtgggcccatcctgcccatcggtgccaccgctcaaaaacagcacatctatcggccccagcggccaccttctcaactctgctccaacacgcagggccagttcctggttccggccacccctgcccgagccctgcagctgtactgtgggctcgccaccagccagcaggcagactgggccccttccccatgccatggtctccagagcctcctccagctgcaggtctgggatctgaagctcagctgccagctcatggagctgtgcatcttcctccacagaagccccagccatggatggggtgaggcgggttctagccacatgggccagcagcccgtagaactgggccatactttttacatcaccttgcatggctgcactcagcaccacagcctggtagcccagtgcctcggcctgccgctgggcctcagctagcgccagcacattagagccaatgatcacattcaggacatggccacaggtgtgtggcccatgggggtcagagtcggcccgagacagcacagtcttcacagaacgtggcagggctgcacggaggccgtagcgattgaggatatgcaggcaatcttgcacattgtgggaactggccacggtggggccactggcaatcacctccacagggtcccccaccacatctgacaggatgaggctcaccacctgagatcagcacgagcagcaggtcatcagctgtgagtccctcagccagttgctggatggccagtgcagcccgcagcgcatcgcggtccgggaggttgtcctccgcaccctcgaatacctggacacggctatgtggcttcagcagcatctcctgcttgccggcacgctccatggcagcacggatccccttgggaacgctgatcacgccctgcacaagatgctggcccagtagttcctcagctgcagctgccatacccagcacagccttgccaaagcccaccaggtagaggttttgcctcagctgaaagttccggtcccgcaccttcagctgtctgccaccagggtccaaggatagtgcccggtgcagcatggggcccggcagcactgcacctacagcactctcaaacagctgcctggcctgctctgccaaggccatgctgctggccagacgggccactgagccccgccagaggagtggatgcaagggggctcgggccaagcggggcaggacctgcagggctgcagccatgccccactgctctcagcactgcctggcacccatggctgccagcccacagctccggccgcggtgcccagcgctggagaacggaagtact

SEQ ID NO: 17050 - RNA, 2789 nt, Homo sapiens
  source 1..2789: mol_type = other RNA
tatagggattggagccgtggcgcacggcggggacagccagcggagggttctgacactgagcaagggggctcaaaaggaggcaggacagtggcacctccctctctcaacccaggctgctggccaggccaacacagccgttcctctattcccacttgcctcttctcccgccagtggtcacaggaagaggtgtgggtcactggacctcatcactggctggacccaccatcccagtgctgggacccccactgaagggctgacttcagggtctggacttggtccccagaggagtggctgaaggaactagggatgttcagcctaggacaagggctgtcacaaggaaacagcactggggggtgggacaaacttcagctcaaccagaagtgcagtatgtggctaagggctgtccaaagacagaaaggacatccatccaacgaggcctacaagctgaggctggagaagccatggtgacagtgccatggtggagtcatggttgggtgggtgggtggctggtcaccccagactgcagtctttaggcctgtcctccctggggtctctgctcacgcacatcaaagctgtcaggagccaagctcaaccctcacacactccagagggatgggcacaggctcccgttatgcgaggcacatcctgcacgtacccagcccagtagaggggtgttaagagtcctgccaggccctggtactgtggctgcagccgtaccacgctcccctcccagcggctcccccgtgaggcctcactctgagggaaggcgcactgagaacccatggcatggtcctatttattttcagacattctcgcttcacagaaagaaacagggtgaggggctcaagagagaggctgcccaagggagaagcacgggaacgctgaactggccgaggggcttgtcctcatcctcaggggtagggggaagcccccatctgccagtctggctggaagggaatagatatagagcagaggccctgagtggaaggtgacagttaaccaaacagccaaggccaaggagaggaggggccctaaggcttagagaggccctgaggaccaaccttgctctgccatctgaccttgcccttgtaggcctcctctgaactcccaaaatgtgacctatgccatcaccgaggccgcaggaacaagaggtgggtgtccatgacattggtacctgtcatccctgtgtgcagcaggtgtgccccaccctggaggcagcagaagaaggtatgtgagtcattgtgggctaggaaggtggctatgtccaggccctcagctgcagcctggctggcaagctcaggtgtgacccaggccccagcagcctctgtgggcccatcctgcccatcggtgccaccgctcaaaaacagcacatctatcggccccagcggccaccttctcaactctgctccaacacgcagggccagttcctggttccggccacccctgcccgagccctgcagctgtactgtgggctcgccaccagccagcaggcagactgggccccttccccatgccatggtctccagagcctcctccagctgcaggtctgggatctgaagctcagctgccagctcatggagctgtgcatcttcctccacagaagccccagccatggatggggtgaggcgggttctagccacatgggccagcagcccgtagaactgggccatactttttacatcaccttgcatggctgcactcagcaccacagcctggtagcccagtgcctcggcctgccgctgggcctcagctagcgccagcacattagagccaatgatcacattcaggacatggccacaggtgtgtggcccatgggggtcagagtcggcccgagacagcacagtcttcacagaacgtggcagggctgcacggaggccgtagcgattgaggatatgcaggcaatcttgcacattgtgggaactggccacggtggggccactggcaatcacctccacagggtcccccaccacatctgacaggatgaggctcaccacctgggcagggtaggcggcctgagccagccccccacccttgagctgggacagggccttccgaatggtgttcaactcctggatggtggctccacgggctgccagcagtctagtgagtgtctgcttctcctccagtgtgacaggtgggatgggggcaggcagcagagctgaacccccacctctgagatcagcacgagcagcaggtcatcagctgtgagtccctcagccagttgctggatggccagtgcagcccgcagcgcatcgcggtccgggaggttgtcctccgcaccctcgaatacctggacacggctatgtggcttcagcagcatctcctgcttgccggcacgctccatggcagcacggatccccttgggaacgctgatcacgccctgcacaagatgctggcccagtagttcctcagctgcagctgccatacccagcacagccttgccaaagcccaccaggtagaggttttgcctcagctgaaagttccggtcccgcaccttcagctgtctgccaccagggtccaaggatagtgcccggtgcagcatggggcccggcagcactgcacctacagcactctcaaacagctgcctggcctgctctgccaaggccatgctgctggccagacgggccactgagccccgccagaggagtggatgcaagggggctcgggccaagcggggcaggacctgcagggctgcagccatgccccactgctctcagcactgcctggcacccatggctgccagcccacagctccggccgcggtgcccagcgctggagaacggaagtact

SEQ ID NO: 17051 - RNA, 2787 nt, Homo sapiens
  source 1..2787: mol_type = other RNA
tatagggattggagccgtggcgcacggcggggacagccagcggagggttctgacactgagcaagggggctcaaaaggaggcaggacagtggcacctccctctctcaacccaggctgctggccaggccaacacagccgttcctctattcccacttgcctcttctcccgccagtggtcacaggaagaggtgtgggtcactggacctcatcactggctggacccaccatcccagtgctgggacccccactgaagggctgacttcagggtctggacttggtccccagaggagtggctgaaggaactagggatgttcagcctaggacaagggctgtcacaaggaaacagcactggggggtgggacaaacttcagctcaaccagaagtgcagtatgtggctaagggctgtccaaagacagaaaggacatccatccaacgaggcctacaagctgaggctggagaagccatggtgacagtgccatggtggagtcatggttgggtgggtgggtggctggtcaccccagactgcagtctttaggcctgtcctccctggggtctctgctcacgcacatcaaagctgtcaggagccaagctcaaccctcacacactccagagggatgggcacaggctcccgttatgcgaggcacatcctgcacgtacccagcccagtagaggggtgttaagagtcctgccaggccctggtactgtggctgcagccgtaccacgctcccctcccagcggctcccccgtgaggcctcactctgagggaaggcgcactgagaacccatggcatggtcctatttattttcagacattctcgcttcacagaaagaaacagggtgaggggctcaagagagaggctgcccaagggagaagcacgggaacgctgaactggccgaggggcttgtcctcatcctcaggggtagggggaagcccccatctgccagtctggctggaagggaatagatatagagcagaggccctgagtggaaggtgacagttaaccaaacagccaaggccaaggagaggaggggccctaaggcttagagaggccctgaggaccaaccttgctctgccatctgaccttgcccttgtaggcctcctctgaactcccaaaatgtgacctatgccatcaccgaggccgcaggaacaagaggtgggtgtccatgacattggtacctgtcatccctgtgtgcagcaggtgtgccccaccctggaggcagcagaagaaggtatgtgagtcattgtgggctaggaaggtggctatgtccaggccctcagctgcagcctggctggcaagctcaggtgtgacccaggccccagcagcctctgtgggcccatcctgcccatcggtgccaccgctcaaaaacagcacatctatcggccccagcggccaccttctcaactctgctccaacacgcagggccagttcctggttccggccacccctgcccgagccctgcagctgtactgtgggctcgccaccagccagcaggcagactgggccccttccccatgccatggtctccagagcctcctccagctgcaggtctgggatctgaagctcagctgccagctcatggagctgtgcatcttcctccacagaagccccagccatggatggggtgaggcgggttctagccacatgggccagcagcccgtagaactgggccatactttttacatcaccttgcatggctgcactcagcaccacagcctggtagcccagtgcctcggcctgccgctgggcctcagctagcgccagcacattagagccaatgatcacattcaggacatggccacaggtgtgtggcccatgggggtcagagtcggcccgagacagcacagtcttcacagaacgtggcagggctgcacggaggccgtagcgattgaggatatgcaggcaatcttgcacattgtgggaactggccacggtggggccactggcaatcacctccacagggtcccccaccacatctgacaggatgaggctcaccacctgggcagggtaggcggcctgagccagccccccacccttgagctgggacagggccttccgaatggtgttcaactcctggatggtggctccacgggctgccagcagtctagtgagtgtctgcttctcctccagtgtgacaggtgggatgggggcaggcagcagagctgaacccccacctgagatcagcacgagcagcaggtcatcagctgtgagtccctcagccagttgctggatggccagtgcagcccgcagcgcatcgcggtccgggaggttgtcctccgcaccctcgaatacctggacacggctatgtggcttcagcagcatctcctgcttgccggcacgctccatggcagcacggatccccttgggaacgctgatcacgccctgcacaagatgctggcccagtagttcctcagctgcagctgccatacccagcacagccttgccaaagcccaccaggtagaggttttgcctcagctgaaagttccggtcccgcaccttcagctgtctgccaccagggtccaaggatagtgcccggtgcagcatggggcccggcagcactgcacctacagcactctcaaacagctgcctggcctgctctgccaaggccatgctgctggccagacgggccactgagccccgccagaggagtggatgcaagggggctcgggccaagcggggcaggacctgcagggctgcagccatgccccactgctctcagcactgcctggcacccatggctgccagcccacagctccggccgcggtgcccagcgctggagaacggaagtact

SEQ ID NO: 17052 - RNA, 1711 nt, Homo sapiens
  source 1..1711: mol_type = other RNA
tatagggattggagccgtggcgcacggcggggacagccagcggagggttctgacactgagcaagggggctcaaaaggaggcaggacagtggcacctccctctctcaacccaggctgctggccaggccaacacagccgttcctctattcccacttgcctcttctcccgccagtggtcacaggaagaggtgtgggtcactggacctcatcactggctggacccaccatcccagtgctgggacccccactgaagggctgacttcagggtctggacttggtccccagaggagtggctgaaggaactagggatgttcagcctaggacaagggctgtcacaaggaaacagcactggggggtgggacaaacttcagctcaaccagaagtgcagtatgtggctaagggctgtccaaagacagaaaggacatccatccaacgaggcctacaagctgaggctggagaagccatggtgacagtgccatggtggagtcatggttgggtgggtgggtggctggtcaccccagactgcagtctttaggcctgtcctccctggggtctctgctcacgcacatcaaagctgtcaggagccaagctcaaccctcacacactccagagggatgggcacaggctcccgttatgcgaggcacatcctgcacgtacccagcccagtagaggggtgttaagagtcctgccaggccctggtactgtggctgcagccgtaccacgctcccctcccagcggctcccccgtgaggcctcactctgagggaaggcgcactgagaacccatggcatggtcctatttattttcagacattctcgcttcacagaaagaaacagggtgaggggctcaagagagaggctgcccaagggagaagcacgggaacgctgaactggccgaggggcttgtcctcatcctcaggggtagggggaagcccccatctgccagtctggcttgctctgccatctgaccttgcccttgtaggcctcctctgaactcccaaaatgtgacctatgccatcaccgaggccgcaggaacaagaggtgggtgtccatgacattggtacctgtcatccctgtgtgcagcaggtgtgccccaccctgagatcagcacgagcagcaggtcatcagctgtgagtccctcagccagttgctggatggccagtgcagcccgcagcgcatcgcggtccgggaggttgtcctccgcaccctcgaatacctggacacggctatgtggcttcagcagcatctcctgcttgccggcacgctccatggcagcacggatccccttgggaacgctgatcacgccctgcacaagatgctggcccagtagttcctcagctgcagctgccatacccagcacagccttgccaaagcccaccaggtagaggttttgcctcagctgaaagttccggtcccgcaccttcagctgtctgccaccagggtccaaggatagtgcccggtgcagcatggggcccggcagcactgcacctacagcactctcaaacagctgcctggcctgctctgccaaggccatgctgctggccagacgggccactgagccccgccagaggagtggatgcaagggggctcgggccaagcggggcaggacctgcagggctgcagccatgccccactgctctcagcactgcctggcacccatggctgccagcccacagctccggccgcggtgcccagcgctggagaacggaagtact

SEQ ID NO: 17053 - RNA, 2673 nt, Homo sapiens
  source 1..2673: mol_type = other RNA
tatagggattggagccgtggcgcacggcggggacagccagcggagggttctgacactgagcaagggggctcaaaaggaggcaggacagtggcacctccctctctcaacccaggctgctggccaggccaacacagccgttcctctattcccacttgcctcttctcccgccagtggtcacaggaagaggtgtgggtcactggacctcatcactggctggacccaccatcccagtgctgggacccccactgaagggctgacttcagggtctggacttggtccccagaggagtggctgaaggaactagggatgttcagcctaggacaagggctgtcacaaggaaacagcactggggggtgggacaaacttcagctcaaccagaagtgcagtatgtggctaagggctgtccaaagacagaaaggacatccatccaacgaggcctacaagctgaggctggagaagccatggtgacagtgccatggtggagtcatggttgggtgggtgggtggctggtcaccccagactgcagtctttaggcctgtcctccctggggtctctgctcacgcacatcaaagctgtcaggagccaagctcaaccctcacacactccagagggatgggcacaggctcccgttatgcgaggcacatcctgcacgtacccagcccagtagaggggtgttaagagtcctgccaggccctggtactgtggctgcagccgtaccacgctcccctcccagcggctcccccgtgaggcctcactctgagggaaggcgcactgagaacccatggcatggtcctatttattttcagacattctcgcttcacagaaagaaacagggtgaggggctcaagagagaggctgcccaagggagaagcacgggaacgctgaactggccgaggggcttgtcctcatcctcaggggtagggggaagcccccatctgccagtctggcttgctctgccatctgaccttgcccttgtaggcctcctctgaactcccaaaatgtgacctatgccatcaccgaggccgcaggaacaagaggtgggtgtccatgacattggtacctgtcatccctgtgtgcagcaggtgtgccccaccctggaggcagcagaagaaggtatgtgagtcattgtgggctaggaaggtggctatgtccaggccctcagctgcagcctggctggcaagctcaggtgtgacccaggccccagcagcctctgtgggcccatcctgcccatcggtgccaccgctcaaaaacagcacatctatcggccccagcggccaccttctcaactctgctccaacacgcagggccagttcctggttccggccacccctgcccgagccctgcagctgtactgtgggctcgccaccagccagcaggcagactgggccccttccccatgccatggtctccagagcctcctccagctgcaggtctgggatctgaagctcagctgccagctcatggagctgtgcatcttcctccacagaagccccagccatggatggggtgaggcgggttctagccacatgggccagcagcccgtagaactgggccatactttttacatcaccttgcatggctgcactcagcaccacagcctggtagcccagtgcctcggcctgccgctgggcctcagctagcgccagcacattagagccaatgatcacattcaggacatggccacaggtgtgtggcccatgggggtcagagtcggcccgagacagcacagtcttcacagaacgtggcagggctgcacggaggccgtagcgattgaggatatgcaggcaatcttgcacattgtgggaactggccacggtggggccactggcaatcacctccacagggtcccccaccacatctgacaggatgaggctcaccacctgggcagggtaggcggcctgagccagccccccacccttgagctgggacagggccttccgaatggtgttcaactcctggatggtggctccacgggctgccagcagtctagtgagtgtctgcttctcctccagtgtgacaggtgggatgggggcaggcagcagagctgaacccccacctgagatcagcacgagcagcaggtcatcagctgtgagtccctcagccagttgctggatggccagtgcagcccgcagcgcatcgcggtccgggaggttgtcctccgcaccctcgaatacctggacacggctatgtggcttcagcagcatctcctgcttgccggcacgctccatggcagcacggatccccttgggaacgctgatcacgccctgcacaagatgctggcccagtagttcctcagctgcagctgccatacccagcacagccttgccaaagcccaccaggtagaggttttgcctcagctgaaagttccggtcccgcaccttcagctgtctgccaccagggtccaaggatagtgcccggtgcagcatggggcccggcagcactgcacctacagcactctcaaacagctgcctggcctgctctgccaaggccatgctgctggccagacgggccactgagccccgccagaggagtggatgcaagggggctcgggccaagcggggcaggacctgcagggctgcagccatgccccactgctctcagcactgcctggcacccatggctgccagcccacagctccggccgcggtgcccagcgctggagaacggaagtact

SEQ ID NO: 17054 - RNA, 1781 nt, Homo sapiens
  source 1..1781: mol_type = other RNA
tatagggattggagccgtggcgcacggcggggacagccagcggagggttctgacactgagcaagggggctcaaaaggaggcaggacagtggcacctccctctctcaacccaggctgctggccaggccaacacagccgttcctctattcccacttgcctcttctcccgccagtggtcacaggaagaggtgtgggtcactggacctcatcactggctggacccaccatcccagtgctgggacccccactgaagggctgacttcagggtctggacttggtccccagaggagtggctgaaggaactagggatgttcagcctaggacaagggctgtcacaaggaaacagcactggggggtgggacaaacttcagctcaaccagaagtgcagtatgtggctaagggctgtccaaagacagaaaggacatccatccaacgaggcctacaagctgaggctggagaagccatggtgacagtgccatggtggagtcatggttgggtgggtgggtggctggtcaccccagactgcagtctttaggcctgtcctccctggggtctctgctcacgcacatcaaagctgtcaggagccaagctcaaccctcacacactccagagggatgggcacaggctcccgttatgcgaggcacatcctgcacgtacccagcccagtagaggggtgttaagagtcctgccaggccctggtactgtggctgcagccgtaccacgctcccctcccagcggctcccccgtgaggcctcactctgagggaaggcgcactgagaacccatggcatggtcctatttattttcagacattctcgcttcacagaaagaaacagggtgaggggctcaagagagaggctgcccaagggagaagcacgggaacgctgaactggccgaggggcttgtcctcatcctcaggggtagggggaagcccccatctgccagtctggcttgctctgccatctgaccttgcccttgtaggcctcctctgaactcccaaaatgtgacctatgccatcaccgaggccgcaggaacaagaggtgggtgtccatgacattggtacctgtcatccctgtgtgcagcaggtgtgccccacccttgcatggctgcactcagcaccacagcctggtagcccagtgcctcggcctgccgctgggcctcagctagcgccagcacattagagccaatgatcacattcaggacatggccacaggtgtgtggcccatgggggtcagagtcggcccgagacagcacagtcttcacagaacgtggcagggctgcacggaggccgtagcgattgaggatatgcaggcaatcttgcacattgtgggaactggccacggtggggccactggcaatcacctccacagggtcccccaccacatctgacaggatgaggctcaccacctgggcagggtaggcggcctgagccagccccccacccttgagctgggacagggccttccgaatggtgttcaactcctggatggtggctccacgggctgccagcagtctagtgagtgtctgcttctcctccagtgtgacaggtgggatgggggcaggcagcagagctgaacccccacctgagatcagcacgagcagcaggtcatcagctgtgagtccctcagccagttgctggatggccagtgcagcccgcagcgcatcgcggtccgggaggttgtcctccgcaccctcgaatacctggacacggctatgtggcttcagcagcatctcccagcccacagctccggccgcggtgcccagcgctggagaacggaagtact

SEQ ID NO: 17055 - RNA, 1010 nt, Homo sapiens
  source 1..1010: mol_type = other RNA
tatctgctgggctttctggtgttggcagcccaagatgacaccctgggcccagcaggagccagaagccctagacgctccctgacttctcgaaggcctaccccggctggtcactgtggcagccagagctggcatctctcagggcccactctgctcctgtcagctgtgggactccccgctccccgttctctcttcaacaatagcccctgggacctttcctaaaactgcttcagccatggcatccctgtcccacacccctccgtggctcctcgctgccctctgcaggcaggctgagtgctcagtcaaagcaaagggaagaccccccaacccttcccacttcctggcccagaaggatttggggctccgtgatccccggtttgcagtgtcattcctcacccacctcttatccgggtgaactcctatgcatcccacaaaacccagttccgtcgctgctcactctgcaatgcctgccctttcttgccacgatattaatgcccctcccttgcgctcctctggaacatccctgggggcagggaagcctaccgctcggcccctgctgtctctcagcacccagtgcagaccctgtcctctctcggagatgctatgcccctccacagtgttccccaaaggcctccacctcctgtgggtcctgcccacagtaggtctgggtgcctgctcagaagggcgttggagggatttgcctccaagacctcagcctgaaggctcagcctctggcctcgccctgcggcccgtgagcttctgtcacccagggctgaggcccacccacctgagtccctggtgatggcccttgggtggcccagcctccatgcccagtgtccaggcctggtgaagctctgcatggctcccccgagctcccctcaaggtccccagaaagagtctcatttgcctcccccagggtcggctgctgaggatccctcggtgaggcagctccaggccccccagcaccccgccccagctctgcccagggcggccccagtgctcaggtgcccagg

SEQ ID NO: 17056 - RNA, 125 nt, Homo sapiens
  source 1..125: mol_type = other RNA
tatggaaagactttgccactcttctccacgtccagcgcggtaaaggcgtaccagatggacttgagcagttccttgcgcagggccatggctgaggcgcccgcccggctgggggcggctctgacact

SEQ ID NO: 17057 - RNA, 34 nt, Homo sapiens
  source 1..34: mol_type = other RNA
tatggaaagactttgccactcttgaaagtgaaga

SEQ ID NO: 17058 - RNA, 31 nt, Homo sapiens
  source 1..31: mol_type = other RNA
tatggaaagactttgccactctttaaagtga

SEQ ID NO: 17059 - RNA, 6307 nt, Homo sapiens
  source 1..6307: mol_type = other RNA
tatggaggtctctgtctggccaaagtaaaaatgtataccctcttcaggtgaaggaaaagtggaaattccagaatttgccattttgtgatgatttccagtgtgaaataattaacgccaaaagaaactctccagaacttgctttattcctacagatctttgtgtggagtcaagaacaccccctacctttctgttctgacaatttccttgtatttctagacttgaacttctgggttttcacagaaaaaaaaagttttctccttgctcctttcccttctcaatatgcagccaattcaccttcacaattatctcaaacttggggtacaggctagaagggaaggaccggcttcacatttcgacatggcatcttgcaacttcctgattttttacattgggcccaaattcctcaaggtatatgacctctttttcccccctgcccttagcagcagcagttccttctacattcagacctctcttcaggcacctgaaagaataaagccattgttccgaggtgcacagcctggctcccactgcatgagtctggcccagagcagtggcatgaagagtattttgtggttcttacacacctggggaccaggtggggatgtatcaaaacaaaccaggagagaggagtgtgtgctgggccatttgccacattagttaaaccccttttcagatctgctccccattctctagctctttgagagtatttttccatttctggctgtgctcaggcccgggttactgcaggccaacaacacattgtgcttttttgtgtatctttgtctttggaggtctaacctcaaagaaaaatactaggttggtgcaaaagtaatggctgtttttgccattacttttgcaccaacctaatagaaagcatctctcaaactaacagacgtgtgcttccaaaagctaaatgctctgaaaagcttgtggggtagaaattatctcctttaagtcaacccttgagaggatcattgtctgcagtccagtcttgtgtttagggcttgtgcctcaggcaggctgacccaggaatgactgcattttgccttgaatagattccagcccgatggaaatgggtaaatgtgttactaggtgtaattttctaaagctggtagaggattcagggaaactagaaaaggataccaaatattttccactaaggcagggaccctctctggggccgttttatatgccacacaattgcattacaccttttaaaatcctcccaataatatcttgaggtttatcatattcttttaataaaatagataaccaaagcccaacaagtgtgaggacacaagtttggtcttctagaaagacacagaggcagcatttgaaaacagagcttctgacacctgaaaagagggcatctgacacctgaacttccttaagagctacacagctacctacgtgttctggggagtcatttaaaggcagccataaagttgtgatgaccaacatgtggctatctgaatttactgttctttgcaacatgccctcattgttttccaagttcacccatgtatatgagagcgataacaatccacataagtctcattttctcctcattttcaaatattcaagtgcctcatcttcttcccattttcaaatattcaaatgcagtcagtgtgatggttaagagcactgactccaaggacggatttcctgaatccaaaccatgtttctgccactagtaaaatgtatgactttggacaaattatttaaattgcctgtgtttaactttctccaactttgaaaaataggtacaatagtagtacttgccttcatggtcaacatgaggattaaatgagataatatatgtaaatacttagtaaaatgactggcaatacacgttcaataaatggtagttgttattttatgtaggagttatgttttatatcactgtaataatacacattttatatcactataaaatcattattttatggcagttaaattaaaaatagccttatacattgaacctactttgaggttcaatggaaagaaagtaaagatctggattctcaccatagctctggccaaatttgtgacttacgggccacgtggtcccaggtgaagcatctgacaactctatttcacttacttcatgtgtaaaaaggaagtctgcagttggtcctgatactacttccagatctttccaaatatatgcaatttaacatgtctatgagttatagaatgaatggaataattctagagaattttagaatctactcattacgtagcaagtgttatacttcgtattcatttgctcacttacatgtcacaaaaacattcccattttatagatgacactagtgaggtttagagaaattaagcaacttgtccaaaatccaaaattcatcctaaacacctaacttaaaacaaagcagtgcttgaaatgaaaagcagcagtagtggaagtgatggaagatgtgtgcaaatgtggctgattctgtgtgctggccctaacccgtgactctccctccatctgttcagctagggacccattaataaattcagtaacaatggtctttgttttaaccatccaagttaactaaaagttcattataaacagaaaatactaaatcaatttcctattagcaacaatggctattttcactgctaaaaagattagtaagtgtgagaagctaaatttaaatctacaattggcgagagattaaactaattcgggtctattttggaaggaagcttttaaaagaccagaactcaacttttcaagttaacaggattcaagctttcaatgctttcctttcttcttccctttaaccaaattcaactttgtagttttcatcttgtttttggaatctttccaggtcacctctgttaagaaacacaaggcccttggcactgaacttttgggaatgtgcccacatctgcctctgaatgtctgcctgcctacctttgatgccgcattcaacacctaacttaaaacaaagcagtgcttgaaacaaaaatctccttagagcacaatggtggacccattgctcaccagtcagtagcctcagtgataaatggcatgagcaaaaaggcctgaaaaccccaaatagttcaatattctaggacatgcccaactgattttcatttgggagaggaaaaggagcagtgcttcattatagggaaagaaaggaataaatgatgatgacagctgtgctgattcattgtttttttaaataattctgaaacattctaactatgttggtgtcacatagatccctcccagagctgaagaggttttgctcctatgtgtatatgtacttttatttataataaggttttcattttgacatgatactccaatttaaaaatgcagaattcttcttcacttcagttccttagaattgaatatgtcattcatcatcttggtggtcccagtaaaatgccctggaattctcatcccagttttcaatagttacgtattaatccatatggtaacaatattaccacaaccaaattcctgctaccagagacatcagattgttcagcttcagccccaggaatatttttttgtctctaagaagtaaatttcaatctgtaaattattggaagaggataaatataagctaaagcaatatcatttattgccctacaagtggggtgaccattcacataaggaggaaaagaagagattaaggcacatttctctttcaaacaagatgagcctctgcaaagcttggaggaattgagtcaaaaaaccactgtgactgaaaagcaggcagctgtagcagagctctgtgtatttgtctcttaacaatagctttattaatctcggaatctgaagatgtctgaggcaaagagttgcttctactggaaaatgaatggaaggaggagaatgtgctggggccttccattgtctgacagatcatctcctgttttgggatctgcccatgtgagattgagcctttcgagttcagaagaggcagggtgtggtggtagttaaaaacactgtaaggaatcaggtggcctcagttcttcctctgttttcttgttaattagcgggtgacttcaaaaacgtctaaagatttctggacttcagtttcctcattcaaaaaggaaagaatccaactagccaaaatcgaaggccacttttacttctaaagtttcaactgtgtgcaatgtagtcaagcaggactttctatactcctgggggagtaacagtagctatcatttcctaaacgcttttctgttccaggcacagtgctagggttttcttcatatggatgttcaacctcctggatgactctccaaggtagatttgattcctactttacagatgagaaaacccttacttgcttagagtcactcagctagtatgtgggaaacctgaagtgcaaacccagactgcccagctccaaaagctcgagctcttttgctaccatacagtgggtaccatccaaccctgctctgagaaaggcactgataagactgataatagtgacgctgaactagctggatgcccaagaggctggctatatgcagtgtctaggaacattaataggcaaaagtgatgacaaattcctacaaagtgggggtaacactaggattacctcatcgtctcatcattgtagggattcatgtttgtaaagtactaagatcaatgtgtttgttaaatttaaacaaataaataaaaacctgaggaaacagaaggctaatggatgtgtagcatacagggtcagggataaggtacagattggagatgattagaagtgggttgatccaggaacagagcaggaccagagagtcacaaaaggagcaacatgagagggccaggaccactgctacagagtgggctgcagtccctgacttgtttgtttacagggcctgcagtccttgagtggatctccatgttcaattcctcatcattgatttggggtatcacctgtcacatggtcttctggatgctaaggggccaattctgcagctcagggttctgtgttgtgccaatggcatgtgagctatggaaccccatggtggctgctacagaagcagctcctctcacctctgagatgcatgttcattccctttcccatctgccctgaggatattctccagtggtgcttgccgctgcagtgtttaccctaagataactttgccacaaaatatcttaattttattattatttttgcatcactctagtgtatcgactttggaacaaaagacatcatactctttatagcattctgtttttagtagtggtatctccgtttataaaatatagtaattctcgatcactgaaaatgtcaaatcctagaaaacatagcattcctacacgtgatgttaacatcattctcgaagagttattggccaaagattcatttgataaattcaattttttctgaaatagaggattctgatgattcggatgtttctgatgttagttcttcttagaaacaactctaagaacagtttttagattttattttcacattgaaaatgagttagatttgcttcagcctcaaatactgtgtttatgtacaattaaatgagcattggcagtgagctgcacttttttttttctaaacaggaaaagggttaacttgtatattcctttatttaggccgtggccaatatgttgtctgacttatggatatgcttgacagacacttagatcctgtagggaactggaagtcagagtgaaagtgaatgtgaggaaagtataacactgtctctggatgatcagaccaaatctccagggacaggagaaggaggtcagagtcacctggccactctcatgtttgtcggaagccaggaccatgcctttgagcttagtggagggatatccacagggctgtcaaaagagggcctcccgaggggagctctgcttaaatagctccactgggatgaggaaagagcttccaaggtcccctgctgggcttccttcagaaccccatgggttctgaactcaaatcaagtcttgaatgttagttttcaagcatgtggtgtgtttagacttggcgcctgttgctactgatgtttccacctccaccccacagttgttcattttcccagccctgtagctccacttctgtctgccccaggattttgctttgctgctcctgtatcaatgttaatggccaaagggaacactaggattcaacaaccgccaattcattgtcactgtacacacttgggattggacttctccatacggaatgctaaaatttattctatcattaccatcaacaagagcctatttgtgaatctcacatgtgtattgtgcacttaaaggtttccaaatttaaaagatacatatagatatggtgcagaatatgtcattaaaaataattaa

SEQ ID NO: 17060 - RNA, 828 nt, Homo sapiens
  source 1..828: mol_type = other RNA
tatggaggtctctgtctggctgggccgggtggggggcccaagagggcggggtggggagcggaaaggggcgtggccgaggggcggggtctcccgggccgaggggcgggatctcctggtatctgccagagcccgccgctgcctccccgacttcagtccccgcagatgcctcgcagacggtgaacggccacaggcgccaggccagccatagcgggtgaggaactggagctgggaacaggggagggaccagcggatgaaggggaggcccctgactcaggcccattggcgcctcgcggaggagggacgcgcagtggtgggcaaacttcgcatctccctctcgggcctcaacgagtgtttggagagcaagaaaagtgggcgccagggggcttgagggcgcgaatccaggcagacgtgaacgagggagtgcttttcagaatccaaaacgcgggagcctcccagtcctccggtgaggggcgtgttggattttcgtgctgtctgctccgttggatccaggatggcaccgtggtgctactgtttcctctgcctcctggtaccttcacttctgggagggcagtgcctgggaggaagtcaaggggactcacagcttcaagggttccaagtggccatccttacctcataaggtcactgcaaatgttatccaagataagtcctggcacagacggaataaaagcactcactaagggtgacccctcttactcatcagcctgtttactcctcacacagggaaaaggctcagggcagcaaagggccctcccgagatcacactctgagtggtgggatttgaatccaggtctgactgcagagtctgca

SEQ ID NO: 17061 - RNA, 1580 nt, Homo sapiens
  source 1..1580: mol_type = other RNA
tatggaggtctctgtctggctgggccgggtggggggcccaagagggcggggtggggagcggaaaggggcgtggccgaggggcggggtctcccgggccgaggggcgggatctcctggtatctgccagagcccgccgctgcctccccgacttcagtccccgcagatgcctcgcagacggtgaacggccacaggcgccaggccagccatagcgggtgaggaactggagctgggaacaggggagggaccagcggatgaaggggaggcccctgactcaggcccattggcgcctcgcggaggagggacgcgcagtggtgggcaaacttcgcatctccctctcgggcctcaacgagtgtttggagagcaagaaaagtgggcgccagggggcttgagggcgcgaatccaggcagacgtgaacgagggagtgcttttcagaatccaaaacgcgggagcctcccagtcctccggtgaggggcgtgttggattttcgtgctgtctggaaaagggaaaaggggtgaatgatcactggtgatggctcagatgccgtcaccaggtggcatgaggccaggtgtcaggacaccgtgttttctcaggcacatttgtgtaaagccagggctggagcagagacccaggaggctcttccctgcctgcagagccccccaggttgacgggagtgaccccagatcacccagggttagggtatccccgctgagcacagcgtctggctgtggcacacccaccagccggaaccacaagctgaacctggaggtggtactactgagagactgggaggcagtccaggcaggagggatggcatggtcacaggtccagaggagggaaactcagaaatggacgcaccttggggagcaggggaaaggtggctgcacggagcagcggtggacaggtgaggccagagaactcggcagaggcctgatgaagcagaaccttggcggagaacctcaaggaacacaaagcccacctggacctgagcttcccccacccgctgcagggaccctgagctctgtttcgcccctctctggccagcgactgctgctgcctccccctctcccagctctccagggcgacagtgtttccctgcttcggtcctgaaggggctcctggagaccatcttttgtgcaagtaaatgtcgtccctactaggtgggccaccccatcctgggcttccagcccactggttggttcccagctcagtggggtctgggagtcaaacaaagggcaaacggaccctgcagaagtccaagggcgaagcaaggcaggatgcccagctgctttcctgcgacttttttttcctcagtccaagttggcctgcctgtgacccctgctgtctgtcacctgctccgttggatccaggatggcaccgtggtgctactgtttcctctgcctcctggtaccttcacttctgggagggcagtgcctgggaggaagtcaaggggactcacagcttcaagggttccaagtggccatccttacctcataaggtcacaggccctgcgaggaacgcttcactggtttccgtctcattcctgccattgcgcagatgacgaaaagagctctgcaagaggac

SEQ ID NO: 17062 - RNA, 1602 nt, Homo sapiens
  source 1..1602: mol_type = other RNA
tatggaggtctctgtctggctgggccgggtggggggcccaagagggcggggtggggagcggaaaggggcgtggccgaggggcggggtctcccgggccgaggggcgggatctcctggtatctgccagagcccgccgctgcctccccgacttcagtccccgcagatgcctcgcagacggtgaacggccacaggcgccaggccagccatagcgggtgaggaactggagctgggaacaggggagggaccagcggatgaaggggaggcccctgactcaggcccattggcgcctcgcggaggagggacgcgcagtggtgggcaaacttcgcatctccctctcgggcctcaacgagtgtttggagagcaagaaaagtgggcgccagggggcttgagggcgcgaatccaggcagacgtgaacgagggagtgcttttcagaatccaaaacgcgggagcctcccagtcctccggtgaggggcgtgttggattttcgtgctgtctggaaaagggaaaaggggtgaatgatcactggtgatggctcagatgccgtcaccaggtggcatgaggccaggtgtcaggacaccgtgttttctcaggcacatttgtgtaaagccagggctggagcagagacccaggaggctcttccctgcctgcagagccccccaggttgacgggagtgaccccagatcacccagggttagggtatccccgctgagcacagcgtctggctgtggcacacccaccagccggaaccacaagctgaacctggaggtggtactactgagagactgggaggcagtccaggcaggagggatggcatggtcacaggtccagaggagggaaactcagaaatggacgcaccttggggagcaggggaaaggtggctgcacggagcagcggtggacaggtgaggccagagaactcggcagaggcctgatgaagcagaaccttggcggagaacctcaaggaacacaaagcccacctggacctgagcttcccccacccgctgcagggaccctgagctctgtttcgcccctctctggccagcgactgctgctgcctccccctctcccagctctccagggcgacagtgtttccctgcttcggtcctgaaggggctcctggagaccatcttttgtgcaagtaaatgtcgtccctactaggtgggccaccccatcctgggcttccagcccactggttggttcccagctcagtggggtctgggagtcaaacaaagggcaaacggaccctgcagaagtccaagggcgaagcaaggcaggatgcccagctgctttcctgcgacttttttttcctcagtccaagttggcctgcctgtgacccctgctgtctgtcacctgctccgttggatccaggatggcaccgtggtgctactgtttcctctgcctcctggtaccttcacttctgggagggcagtgcctgggaggaagtcaaggggactcacagcttcaagggttccaagtggccatccttacctcataaggtcactgcaaatgttatccaagataagtccaggccctgcgaggaacgcttcactggtttccgtctcattcctgccattgcgcagatgacgaaaagagctctgcaagag

SEQ ID NO: 17063 - RNA, 720 nt, Homo sapiens
  source 1..720: mol_type = other RNA
tatggcactggtagaattcactaccgcctgagggtgggtggaagctgtgacctgcctttaactaacagaatatggcaaaggtgatggaatgcacatgattatattaccttgtgtttttacaatttttacacagtgagtctgcagtgtcttaagaagactatcccttggtggatttgaagaagcaagctgccttgttgtttgagctctcatttggagagggctgcaggttgaggagctgacagccagcagaaatgggggccatccctcagacagccatcagggagctgcatgctgccaacaccatgagagcttggcagtgaatcctcccccagtcaagcctcagatgagaccacagtcccagctgacctcttggtttcagcctccaaactcccaactcagaaaaacccaaagaggcaacaccaggttctttgcttttcttcccccgatctctcatgagcacccattgttccaccatgtagtgaatgcaggatgaggagatgctgtctttttctagtaggaagatgactttgctggatttggtaacctccataaagggtattcatgcaacacagtggcaggaagaagagtgaatcaagaggtatccaagaggtatcttatctgaaacacgcaggttcccagccctgttgtcctgaagcttccactccaggtgattgtgtatcttgggagatacctgtgaccaaactggcaggtaggttgtgg

SEQ ID NO: 17064 - RNA, 756 nt, Homo sapiens
  source 1..756: mol_type = other RNA
tatggcactggtagaattcactaccgcctgagggtgggtggaagctgtgacctgcctttaactaacagaatatggcaaaggtgatggaatgcacatgattatattaccttgtgtttttacaatttttacacagtgagtctgcagtgtcttaagaagactatcccttggtggatttgaagaagcaagctgccttgttgtttgagctctcatttggagagggctgcaggttgaggagctgacagccagcagaaatgggggccatccctcagacagccatcagggagctgcatgctgccaacaccatgagagcttggcagtgaatcctcccccagtcaagcctcagatgagaccacagtcccagctgacctcttggtttcagcctccaaactcccaactcagaaaaacccaaagaggcaacaccaggttctttgcttttcttcccccgatctctcatgagcacccattgttccaccatgtagtgaatgcaggatgaggagatgctgtctttttctagtaggaagatgactttgctggatttggtaacctccataaagggtattcatgcaactgcataaagctggtcaaagactcaatgatcctcaccacagtggcaggaagaagagtgaatcaagaggtatccaagaggtatcttatctgaaacacgcaggttcccagccctgttgtcctgaagcttccactccaggtgattgtgtatcttgggagatacctgtgaccaaactggcaggtaggttgtgg

SEQ ID NO: 17065 - RNA, 710 nt, Homo sapiens
  source 1..710: mol_type = other RNA
tatggcactggtagaattcactaccgcctgagggtgggtggaagctgtgacctgcctttaactaacagaatatggcaaaggtgatggaatgcacatgattatattaccttgtgtttttacaatttttacacagtgagtctgcagtgtcttaagaagactatcccttggtggatttgaagaagcaagctgccttgttgtttgagctctcatttggagagggctgcaggttgaggagctgacagccagcagaaatgggggccatccctcagacagccatcagggagctgcatgctgccaacaccatgagagcttggcagtgaatcctcccccagtcaagcctcagatgagaccacagtcccagctgacctcttggtttcagcctccaaactcccaactcagaaaaacccaaagaggcaacaccaggttctttgcttttcttcccccgatctctcatgagcacccattgttccaccatgtagtgaatgcaggatgaggagatgctgtctttttctagtaggaagatgactttgctggatttggtaacctccataaagggtattcatgcaactgcataaagctggtcaaagactcaatgatcctcaccacagtggcaggaagaagagtgaatcaagaggtatccaagaggtatcttatctgaaacacgcaggttcctgtaatttcagctactctggaggctgaggcaggagaat

SEQ ID NO: 17066 - RNA, 98 nt, Homo sapiens
  source 1..98: mol_type = other RNA
tatggcactggtagaattcactgtggactggaggtggtgggggccacaggaagaggcttttctgccacctcggtatttagatgaatcagaacaaatac

SEQ ID NO: 17067 - RNA, 2650 nt, Homo sapiens
  source 1..2650: mol_type = other RNA
tatggctttttattcctatgtgattctactgctcactcatatagggattggagccgtggcgcacggcggggacagccagcggagggttctgacactgagcaagggggctcaaaaggaggcaggacagtggcacctccctctctcaacccaggctgctggccaggccaacacagccgttcctctattcccacttgcctcttctcccgccagtggtcacaggaagaggtgtgggtcactggacctcatcactggctggacccaccatcccagtgctgggacccccactgaagggctgacttcagggtctggacttggtccccagaggagtggctgaaggaactagggatgttcagcctaggacaagggctgtcacaaggaaacagcactggggggtgggacaaacttcagctcaaccagaagtgcagtatgtggctaagggctgtccaaagacagaaaggacatccatccaacgaggcctacaagctgaggctggagaagccatggtgacagtgccatggtggagtcatggttgggtgggtgggtggctggtcaccccagactgcagtctttaggcctgtcctccctggggtctctgctcacgcacatcaaagctgtcaggagccaagctcaaccctcacacactccagagggatgggcacaggctcccgttatgcgaggcacatcctgcacgtacccagcccagtagaggggtgttaagagtcctgccaggccctggtactgtggctgcagccgtaccacgctcccctcccagcggctcccccgtgaggcctcactctgagggaaggcgcactgagaacccatggcatggtcctatttattttcagacattctcgcttcacagaaagaaacagggtgaggggctcaagagagaggctgcccaagggagaagcacgggaacgctgaactggccgaggggcttgtcctcatcctcaggggtagggggaagcccccatctgccagtctggctggaagggaatagatatagagcagaggccctgagtggaaggtgacagttaaccaaacagccaaggccaaggagaggaggggccctaaggcttagagaggccctgaggaccaaccttgctctgccatctgaccttgcccttgtaggcctcctctgaactcccaaaatgtgacctatgccatcaccgaggccgcaggaacaagaggtgggtgtccatgacattggtacctgtcatccctgtgtgcagcaggtgtgccccaccctggaggcagcagaagaaggtatgtgagtcattgtgggctaggaaggtggctatgtccaggccctcagctgcagcctggctggcaagctcaggtgtgacccaggccccagcagcctctgtgggcccatcctgcccatcggtgccaccgctcaaaaacagcacatctatcggccccagcggccaccttctcaactctgctccaacacgcagggccagttcctggttccggccacccctgcccgagccctgcagctgtactgtgggctcgccaccagccagcaggcagactgggccccttccccatgccatggtctccagagcctcctccagctgcaggtctgggatctgaagctcagctgccagctcatggagctgtgcatcttcctccacagaagccccagccatggatggggtgaggcgggttctagccacatgggccagcagcccgtagaactgggccatactttttacatcaccttgcatggctgcactcagcaccacagcctggtagcccagtgcctcggcctgccgctgggcctcagctagcgccagcacattagagccaatgatcacattcaggacatggccacaggtgtgtggcccatgggggtcagagtcggcccgagacagcacagtcttcacagaacgtggcagggctgcacggaggccgtagcgattgaggatatgcaggcaatcttgcacattgtgggaactggccacggtggggccactggcaatcacctccacagggtcccccaccacatctgacaggatgaggctcaccacctgagatcagcacgagcagcaggtcatcagctgtgagtccctcagccagttgctggatggccagtgcagcccgcagcgcatcgcggtccgggaggttgtcctccgcaccctcgaatacctggacacggctatgtggcttcagcagcatctcctgcttgccggcacgctccatggcagcacggatccccttgggaacgctgatcacgccctgcacaagatgctggcccagtagttcctcagctgcagctgccatacccagcacagccttgccaaagcccaccaggtagaggttttgcctcagctgaaagttccggtcccgcaccttcagctgtctgccaccagggtccaaggatagtgcccggtgcagcatggggcccggcagcactgcacctacagcactctcaaacagctgcctggcctgctctgccaaggccatgctgctggccagacgggccactgagccccgccagaggagtggatgcaagggggctcgggccaagcggggcaggacctgcagggctgcagccatgccccactgctctcagcactgcctggcacccatggctgccagcccacagctccggccgcggtgcccagcgctggagaacggaagtact

SEQ ID NO: 17068 - RNA, 2828 nt, Homo sapiens
  source 1..2828: mol_type = other RNA
tatggctttttattcctatgtgattctactgctcactcatatagggattggagccgtggcgcacggcggggacagccagcggagggttctgacactgagcaagggggctcaaaaggaggcaggacagtggcacctccctctctcaacccaggctgctggccaggccaacacagccgttcctctattcccacttgcctcttctcccgccagtggtcacaggaagaggtgtgggtcactggacctcatcactggctggacccaccatcccagtgctgggacccccactgaagggctgacttcagggtctggacttggtccccagaggagtggctgaaggaactagggatgttcagcctaggacaagggctgtcacaaggaaacagcactggggggtgggacaaacttcagctcaaccagaagtgcagtatgtggctaagggctgtccaaagacagaaaggacatccatccaacgaggcctacaagctgaggctggagaagccatggtgacagtgccatggtggagtcatggttgggtgggtgggtggctggtcaccccagactgcagtctttaggcctgtcctccctggggtctctgctcacgcacatcaaagctgtcaggagccaagctcaaccctcacacactccagagggatgggcacaggctcccgttatgcgaggcacatcctgcacgtacccagcccagtagaggggtgttaagagtcctgccaggccctggtactgtggctgcagccgtaccacgctcccctcccagcggctcccccgtgaggcctcactctgagggaaggcgcactgagaacccatggcatggtcctatttattttcagacattctcgcttcacagaaagaaacagggtgaggggctcaagagagaggctgcccaagggagaagcacgggaacgctgaactggccgaggggcttgtcctcatcctcaggggtagggggaagcccccatctgccagtctggctggaagggaatagatatagagcagaggccctgagtggaaggtgacagttaaccaaacagccaaggccaaggagaggaggggccctaaggcttagagaggccctgaggaccaaccttgctctgccatctgaccttgcccttgtaggcctcctctgaactcccaaaatgtgacctatgccatcaccgaggccgcaggaacaagaggtgggtgtccatgacattggtacctgtcatccctgtgtgcagcaggtgtgccccaccctggaggcagcagaagaaggtatgtgagtcattgtgggctaggaaggtggctatgtccaggccctcagctgcagcctggctggcaagctcaggtgtgacccaggccccagcagcctctgtgggcccatcctgcccatcggtgccaccgctcaaaaacagcacatctatcggccccagcggccaccttctcaactctgctccaacacgcagggccagttcctggttccggccacccctgcccgagccctgcagctgtactgtgggctcgccaccagccagcaggcagactgggccccttccccatgccatggtctccagagcctcctccagctgcaggtctgggatctgaagctcagctgccagctcatggagctgtgcatcttcctccacagaagccccagccatggatggggtgaggcgggttctagccacatgggccagcagcccgtagaactgggccatactttttacatcaccttgcatggctgcactcagcaccacagcctggtagcccagtgcctcggcctgccgctgggcctcagctagcgccagcacattagagccaatgatcacattcaggacatggccacaggtgtgtggcccatgggggtcagagtcggcccgagacagcacagtcttcacagaacgtggcagggctgcacggaggccgtagcgattgaggatatgcaggcaatcttgcacattgtgggaactggccacggtggggccactggcaatcacctccacagggtcccccaccacatctgacaggatgaggctcaccacctgggcagggtaggcggcctgagccagccccccacccttgagctgggacagggccttccgaatggtgttcaactcctggatggtggctccacgggctgccagcagtctagtgagtgtctgcttctcctccagtgtgacaggtgggatgggggcaggcagcagagctgaacccccacctctgagatcagcacgagcagcaggtcatcagctgtgagtccctcagccagttgctggatggccagtgcagcccgcagcgcatcgcggtccgggaggttgtcctccgcaccctcgaatacctggacacggctatgtggcttcagcagcatctcctgcttgccggcacgctccatggcagcacggatccccttgggaacgctgatcacgccctgcacaagatgctggcccagtagttcctcagctgcagctgccatacccagcacagccttgccaaagcccaccaggtagaggttttgcctcagctgaaagttccggtcccgcaccttcagctgtctgccaccagggtccaaggatagtgcccggtgcagcatggggcccggcagcactgcacctacagcactctcaaacagctgcctggcctgctctgccaaggccatgctgctggccagacgggccactgagccccgccagaggagtggatgcaagggggctcgggccaagcggggcaggacctgcagggctgcagccatgccccactgctctcagcactgcctggcacccatggctgccagcccacagctccggccgcggtgcccagcgctggagaacggaagtact

SEQ ID NO: 17069 - RNA, 2826 nt, Homo sapiens
  source 1..2826: mol_type = other RNA
tatggctttttattcctatgtgattctactgctcactcatatagggattggagccgtggcgcacggcggggacagccagcggagggttctgacactgagcaagggggctcaaaaggaggcaggacagtggcacctccctctctcaacccaggctgctggccaggccaacacagccgttcctctattcccacttgcctcttctcccgccagtggtcacaggaagaggtgtgggtcactggacctcatcactggctggacccaccatcccagtgctgggacccccactgaagggctgacttcagggtctggacttggtccccagaggagtggctgaaggaactagggatgttcagcctaggacaagggctgtcacaaggaaacagcactggggggtgggacaaacttcagctcaaccagaagtgcagtatgtggctaagggctgtccaaagacagaaaggacatccatccaacgaggcctacaagctgaggctggagaagccatggtgacagtgccatggtggagtcatggttgggtgggtgggtggctggtcaccccagactgcagtctttaggcctgtcctccctggggtctctgctcacgcacatcaaagctgtcaggagccaagctcaaccctcacacactccagagggatgggcacaggctcccgttatgcgaggcacatcctgcacgtacccagcccagtagaggggtgttaagagtcctgccaggccctggtactgtggctgcagccgtaccacgctcccctcccagcggctcccccgtgaggcctcactctgagggaaggcgcactgagaacccatggcatggtcctatttattttcagacattctcgcttcacagaaagaaacagggtgaggggctcaagagagaggctgcccaagggagaagcacgggaacgctgaactggccgaggggcttgtcctcatcctcaggggtagggggaagcccccatctgccagtctggctggaagggaatagatatagagcagaggccctgagtggaaggtgacagttaaccaaacagccaaggccaaggagaggaggggccctaaggcttagagaggccctgaggaccaaccttgctctgccatctgaccttgcccttgtaggcctcctctgaactcccaaaatgtgacctatgccatcaccgaggccgcaggaacaagaggtgggtgtccatgacattggtacctgtcatccctgtgtgcagcaggtgtgccccaccctggaggcagcagaagaaggtatgtgagtcattgtgggctaggaaggtggctatgtccaggccctcagctgcagcctggctggcaagctcaggtgtgacccaggccccagcagcctctgtgggcccatcctgcccatcggtgccaccgctcaaaaacagcacatctatcggccccagcggccaccttctcaactctgctccaacacgcagggccagttcctggttccggccacccctgcccgagccctgcagctgtactgtgggctcgccaccagccagcaggcagactgggccccttccccatgccatggtctccagagcctcctccagctgcaggtctgggatctgaagctcagctgccagctcatggagctgtgcatcttcctccacagaagccccagccatggatggggtgaggcgggttctagccacatgggccagcagcccgtagaactgggccatactttttacatcaccttgcatggctgcactcagcaccacagcctggtagcccagtgcctcggcctgccgctgggcctcagctagcgccagcacattagagccaatgatcacattcaggacatggccacaggtgtgtggcccatgggggtcagagtcggcccgagacagcacagtcttcacagaacgtggcagggctgcacggaggccgtagcgattgaggatatgcaggcaatcttgcacattgtgggaactggccacggtggggccactggcaatcacctccacagggtcccccaccacatctgacaggatgaggctcaccacctgggcagggtaggcggcctgagccagccccccacccttgagctgggacagggccttccgaatggtgttcaactcctggatggtggctccacgggctgccagcagtctagtgagtgtctgcttctcctccagtgtgacaggtgggatgggggcaggcagcagagctgaacccccacctgagatcagcacgagcagcaggtcatcagctgtgagtccctcagccagttgctggatggccagtgcagcccgcagcgcatcgcggtccgggaggttgtcctccgcaccctcgaatacctggacacggctatgtggcttcagcagcatctcctgcttgccggcacgctccatggcagcacggatccccttgggaacgctgatcacgccctgcacaagatgctggcccagtagttcctcagctgcagctgccatacccagcacagccttgccaaagcccaccaggtagaggttttgcctcagctgaaagttccggtcccgcaccttcagctgtctgccaccagggtccaaggatagtgcccggtgcagcatggggcccggcagcactgcacctacagcactctcaaacagctgcctggcctgctctgccaaggccatgctgctggccagacgggccactgagccccgccagaggagtggatgcaagggggctcgggccaagcggggcaggacctgcagggctgcagccatgccccactgctctcagcactgcctggcacccatggctgccagcccacagctccggccgcggtgcccagcgctggagaacggaagtact

SEQ ID NO: 17070 - RNA, 1750 nt, Homo sapiens
  source 1..1750: mol_type = other RNA
tatggctttttattcctatgtgattctactgctcactcatatagggattggagccgtggcgcacggcggggacagccagcggagggttctgacactgagcaagggggctcaaaaggaggcaggacagtggcacctccctctctcaacccaggctgctggccaggccaacacagccgttcctctattcccacttgcctcttctcccgccagtggtcacaggaagaggtgtgggtcactggacctcatcactggctggacccaccatcccagtgctgggacccccactgaagggctgacttcagggtctggacttggtccccagaggagtggctgaaggaactagggatgttcagcctaggacaagggctgtcacaaggaaacagcactggggggtgggacaaacttcagctcaaccagaagtgcagtatgtggctaagggctgtccaaagacagaaaggacatccatccaacgaggcctacaagctgaggctggagaagccatggtgacagtgccatggtggagtcatggttgggtgggtgggtggctggtcaccccagactgcagtctttaggcctgtcctccctggggtctctgctcacgcacatcaaagctgtcaggagccaagctcaaccctcacacactccagagggatgggcacaggctcccgttatgcgaggcacatcctgcacgtacccagcccagtagaggggtgttaagagtcctgccaggccctggtactgtggctgcagccgtaccacgctcccctcccagcggctcccccgtgaggcctcactctgagggaaggcgcactgagaacccatggcatggtcctatttattttcagacattctcgcttcacagaaagaaacagggtgaggggctcaagagagaggctgcccaagggagaagcacgggaacgctgaactggccgaggggcttgtcctcatcctcaggggtagggggaagcccccatctgccagtctggcttgctctgccatctgaccttgcccttgtaggcctcctctgaactcccaaaatgtgacctatgccatcaccgaggccgcaggaacaagaggtgggtgtccatgacattggtacctgtcatccctgtgtgcagcaggtgtgccccaccctgagatcagcacgagcagcaggtcatcagctgtgagtccctcagccagttgctggatggccagtgcagcccgcagcgcatcgcggtccgggaggttgtcctccgcaccctcgaatacctggacacggctatgtggcttcagcagcatctcctgcttgccggcacgctccatggcagcacggatccccttgggaacgctgatcacgccctgcacaagatgctggcccagtagttcctcagctgcagctgccatacccagcacagccttgccaaagcccaccaggtagaggttttgcctcagctgaaagttccggtcccgcaccttcagctgtctgccaccagggtccaaggatagtgcccggtgcagcatggggcccggcagcactgcacctacagcactctcaaacagctgcctggcctgctctgccaaggccatgctgctggccagacgggccactgagccccgccagaggagtggatgcaagggggctcgggccaagcggggcaggacctgcagggctgcagccatgccccactgctctcagcactgcctggcacccatggctgccagcccacagctccggccgcggtgcccagcgctggagaacggaagtact

SEQ ID NO: 17071 - RNA, 2712 nt, Homo sapiens
  source 1..2712: mol_type = other RNA
tatggctttttattcctatgtgattctactgctcactcatatagggattggagccgtggcgcacggcggggacagccagcggagggttctgacactgagcaagggggctcaaaaggaggcaggacagtggcacctccctctctcaacccaggctgctggccaggccaacacagccgttcctctattcccacttgcctcttctcccgccagtggtcacaggaagaggtgtgggtcactggacctcatcactggctggacccaccatcccagtgctgggacccccactgaagggctgacttcagggtctggacttggtccccagaggagtggctgaaggaactagggatgttcagcctaggacaagggctgtcacaaggaaacagcactggggggtgggacaaacttcagctcaaccagaagtgcagtatgtggctaagggctgtccaaagacagaaaggacatccatccaacgaggcctacaagctgaggctggagaagccatggtgacagtgccatggtggagtcatggttgggtgggtgggtggctggtcaccccagactgcagtctttaggcctgtcctccctggggtctctgctcacgcacatcaaagctgtcaggagccaagctcaaccctcacacactccagagggatgggcacaggctcccgttatgcgaggcacatcctgcacgtacccagcccagtagaggggtgttaagagtcctgccaggccctggtactgtggctgcagccgtaccacgctcccctcccagcggctcccccgtgaggcctcactctgagggaaggcgcactgagaacccatggcatggtcctatttattttcagacattctcgcttcacagaaagaaacagggtgaggggctcaagagagaggctgcccaagggagaagcacgggaacgctgaactggccgaggggcttgtcctcatcctcaggggtagggggaagcccccatctgccagtctggcttgctctgccatctgaccttgcccttgtaggcctcctctgaactcccaaaatgtgacctatgccatcaccgaggccgcaggaacaagaggtgggtgtccatgacattggtacctgtcatccctgtgtgcagcaggtgtgccccaccctggaggcagcagaagaaggtatgtgagtcattgtgggctaggaaggtggctatgtccaggccctcagctgcagcctggctggcaagctcaggtgtgacccaggccccagcagcctctgtgggcccatcctgcccatcggtgccaccgctcaaaaacagcacatctatcggccccagcggccaccttctcaactctgctccaacacgcagggccagttcctggttccggccacccctgcccgagccctgcagctgtactgtgggctcgccaccagccagcaggcagactgggccccttccccatgccatggtctccagagcctcctccagctgcaggtctgggatctgaagctcagctgccagctcatggagctgtgcatcttcctccacagaagccccagccatggatggggtgaggcgggttctagccacatgggccagcagcccgtagaactgggccatactttttacatcaccttgcatggctgcactcagcaccacagcctggtagcccagtgcctcggcctgccgctgggcctcagctagcgccagcacattagagccaatgatcacattcaggacatggccacaggtgtgtggcccatgggggtcagagtcggcccgagacagcacagtcttcacagaacgtggcagggctgcacggaggccgtagcgattgaggatatgcaggcaatcttgcacattgtgggaactggccacggtggggccactggcaatcacctccacagggtcccccaccacatctgacaggatgaggctcaccacctgggcagggtaggcggcctgagccagccccccacccttgagctgggacagggccttccgaatggtgttcaactcctggatggtggctccacgggctgccagcagtctagtgagtgtctgcttctcctccagtgtgacaggtgggatgggggcaggcagcagagctgaacccccacctgagatcagcacgagcagcaggtcatcagctgtgagtccctcagccagttgctggatggccagtgcagcccgcagcgcatcgcggtccgggaggttgtcctccgcaccctcgaatacctggacacggctatgtggcttcagcagcatctcctgcttgccggcacgctccatggcagcacggatccccttgggaacgctgatcacgccctgcacaagatgctggcccagtagttcctcagctgcagctgccatacccagcacagccttgccaaagcccaccaggtagaggttttgcctcagctgaaagttccggtcccgcaccttcagctgtctgccaccagggtccaaggatagtgcccggtgcagcatggggcccggcagcactgcacctacagcactctcaaacagctgcctggcctgctctgccaaggccatgctgctggccagacgggccactgagccccgccagaggagtggatgcaagggggctcgggccaagcggggcaggacctgcagggctgcagccatgccccactgctctcagcactgcctggcacccatggctgccagcccacagctccggccgcggtgcccagcgctggagaacggaagtact

SEQ ID NO: 17072 - RNA, 1820 nt, Homo sapiens
  source 1..1820: mol_type = other RNA
tatggctttttattcctatgtgattctactgctcactcatatagggattggagccgtggcgcacggcggggacagccagcggagggttctgacactgagcaagggggctcaaaaggaggcaggacagtggcacctccctctctcaacccaggctgctggccaggccaacacagccgttcctctattcccacttgcctcttctcccgccagtggtcacaggaagaggtgtgggtcactggacctcatcactggctggacccaccatcccagtgctgggacccccactgaagggctgacttcagggtctggacttggtccccagaggagtggctgaaggaactagggatgttcagcctaggacaagggctgtcacaaggaaacagcactggggggtgggacaaacttcagctcaaccagaagtgcagtatgtggctaagggctgtccaaagacagaaaggacatccatccaacgaggcctacaagctgaggctggagaagccatggtgacagtgccatggtggagtcatggttgggtgggtgggtggctggtcaccccagactgcagtctttaggcctgtcctccctggggtctctgctcacgcacatcaaagctgtcaggagccaagctcaaccctcacacactccagagggatgggcacaggctcccgttatgcgaggcacatcctgcacgtacccagcccagtagaggggtgttaagagtcctgccaggccctggtactgtggctgcagccgtaccacgctcccctcccagcggctcccccgtgaggcctcactctgagggaaggcgcactgagaacccatggcatggtcctatttattttcagacattctcgcttcacagaaagaaacagggtgaggggctcaagagagaggctgcccaagggagaagcacgggaacgctgaactggccgaggggcttgtcctcatcctcaggggtagggggaagcccccatctgccagtctggcttgctctgccatctgaccttgcccttgtaggcctcctctgaactcccaaaatgtgacctatgccatcaccgaggccgcaggaacaagaggtgggtgtccatgacattggtacctgtcatccctgtgtgcagcaggtgtgccccacccttgcatggctgcactcagcaccacagcctggtagcccagtgcctcggcctgccgctgggcctcagctagcgccagcacattagagccaatgatcacattcaggacatggccacaggtgtgtggcccatgggggtcagagtcggcccgagacagcacagtcttcacagaacgtggcagggctgcacggaggccgtagcgattgaggatatgcaggcaatcttgcacattgtgggaactggccacggtggggccactggcaatcacctccacagggtcccccaccacatctgacaggatgaggctcaccacctgggcagggtaggcggcctgagccagccccccacccttgagctgggacagggccttccgaatggtgttcaactcctggatggtggctccacgggctgccagcagtctagtgagtgtctgcttctcctccagtgtgacaggtgggatgggggcaggcagcagagctgaacccccacctgagatcagcacgagcagcaggtcatcagctgtgagtccctcagccagttgctggatggccagtgcagcccgcagcgcatcgcggtccgggaggttgtcctccgcaccctcgaatacctggacacggctatgtggcttcagcagcatctcccagcccacagctccggccgcggtgcccagcgctggagaacggaagtact

SEQ ID NO: 17073 - RNA, 503 nt, Homo sapiens
  source 1..503: mol_type = other RNA
tatggggcttctgtagagatttcattggatagaaatgattgaagcatggacaatccttctgtgttgatctcactgggaactgcagaccggagctgttcctattcaaccatcttgccagccacctatccttccatttttgatttctggtttgatttcatcttttggtaaaacaggctgcatggctccactgctccgcgtcacccgcctggcctcccaccgcttagcggaaggggaggtgcggttcctaattccgacaggcacgtagtcttccacaagtggcactactcggggctctcctggctaggggcgttcgagccactaggggcgggtctcctgggatgggaagactggggctagggaggttcaacgccgcccccggaaacctaagggacgctccctgaaactcaccgggacgcgcttccgacccattccggtcacttgccttgaaatcgccgcagggctgcgcaaacctgccacccagggcccaagcgaccggggcgggg

SEQ ID NO: 17074 - RNA, 401 nt, Homo sapiens
  source 1..401: mol_type = other RNA
tatggggcttctgtagagatttcattggatagaaatgattgaagcatggacaatctcttttggtaaaacaggctgcatggctccactgctccgcgtcacccgcctggcctcccaccgcttagcggaaggggaggtgcggttcctaattccgacaggcacgtagtcttccacaagtggcactactcggggctctcctggctaggggcgttcgagccactaggggcgggtctcctgggatgggaagactggggctagggaggttcaacgccgcccccggaaacctaagggacgctccctgaaactcaccgggacgcgcttccgacccattccggtcacttgccttgaaatcgccgcagggctgcgcaaacctgccacccagggcccaagcgaccggggcgggg

SEQ ID NO: 17075 - RNA, 23 nt, Homo sapiens
  source 1..23: mol_type = other RNA
tatgtagtagtcaaaggcattta

SEQ ID NO: 17076 - RNA, 880 nt, Homo sapiens
  source 1..880: mol_type = other RNA
tatgtctgctgaccatcaccttgacagacttttaaaatggagcacaatgaaccatcccttgtgactcctttcagtatcttatgatggaaggaaactgtccccaaaatacatgactgggagttgtgaaggttactcttcctgtcttgtctcccatctgcctgatattcatctggatagatccaatttgatatgtctccctttatgatccatggctcttctccttgttccaacttggagatgacatctggtttggaaactggataccccattgagaccaggtggctgtagttctccagcatcacatccctgtacagggtcctctgagaagggtcaagttgctgccactcctcctgggtgaaatccacagccacatccttgaatgatactaacccctgggacttcatcattttttgctcttccaaaaggccagatgaagaagtctcagcaggcaccatgtggaggagggatcattctttactcctcttgtacctggtaaattttcctcagtcccaggacaagtcatgcagacagagctgaactatttcagaggacgtgggggctcccatgacagacagattattttatatgggggtatcaaaacatccttcaccgcacacatcccgcctctgactcccagctcgattatcaggtcccaaaaccaccatcaccgcttaatgggaaccgctgtcacatccctattggcaaactctcctgcttcctgtccgcgagcaccacaccgggctcccgaggctgcgccgttccgtactgggcggttttgcccgttccgcatcttcagaggctttgttcaggaagcaacatggctgctccctggagctgtttccgcatggggccgccatcttgagagcccggtcgtcttcgt

SEQ ID NO: 17077 - RNA, 825 nt, Homo sapiens
  source 1..825: mol_type = other RNA
tatgtctgctgaccatcaccttgacagacttttaaaatggagcacaatgaaccatcccttgtgactcctttcagtatcttatgatggaaggaaactgtccccaaaatacatgactgggagttgtgaaggttactcttcctgtcttgtctcccatctgcctgatattcatctggatagatccaatttgatatgtctccctttatgatccatggctcttctccttgttccaacttggagatgacatctggtttggaaactggataccccattgagaccaggtggctgtagttctccagcatcacatccctgtacagggtcctctgagaagggtcaagttgctgccactcctcctgggtgaaatccacagccacatccttgaatgatactaacccctgggacttcatcattttttgctcttccaaaaggccagatgactggtaaattttcctcagtcccaggacaagtcatgcagacagagctgaactatttcagaggacgtgggggctcccatgacagacagattattttatatgggggtatcaaaacatccttcaccgcacacatcccgcctctgactcccagctcgattatcaggtcccaaaaccaccatcaccgcttaatgggaaccgctgtcacatccctattggcaaactctcctgcttcctgtccgcgagcaccacaccgggctcccgaggctgcgccgttccgtactgggcggttttgcccgttccgcatcttcagaggctttgttcaggaagcaacatggctgctccctggagctgtttccgcatggggccgccatcttgagagcccggtcgtcttcgt

SEQ ID NO: 17078 - RNA, 783 nt, Homo sapiens
  source 1..783: mol_type = other RNA
tatgtctgctgaccatcaccttgacagacttttaaaatggagcacaatgaaccatcccttgtgactcctttcagtatcttatgatggaaggaaactgtccccaaaatacatgactgggagttgtgaaggttactcttcctgtcttgtctcccatctgcctgatattcatctggatagatccaatttgatatgtctccctttatgatccatggctcttctccttgttccaacttggagatgacatctggtttggaaactggataccccattgagaccaggtggctgtagttctccagcatcacatccctgtacagggtcctctgagaagggtcaagttgctgccactcctcctgggtgaaatccacagccacatccttgaatgatactaacccctggtaaattttcctcagtcccaggacaagtcatgcagacagagctgaactatttcagaggacgtgggggctcccatgacagacagattattttatatgggggtatcaaaacatccttcaccgcacacatcccgcctctgactcccagctcgattatcaggtcccaaaaccaccatcaccgcttaatgggaaccgctgtcacatccctattggcaaactctcctgcttcctgtccgcgagcaccacaccgggctcccgaggctgcgccgttccgtactgggcggttttgcccgttccgcatcttcagaggctttgttcaggaagcaacatggctgctccctggagctgtttccgcatggggccgccatcttgagagcccggtcgtcttcgt

SEQ ID NO: 17079 - RNA, 983 nt, Homo sapiens
  source 1..983: mol_type = other RNA
tatgtctgctgaccatcaccttgacagacttttaaaatggagcacaatgaaccatcccttgtgactcctttcagtatcttatgatggaaggaaactgtccccaaaatacatgactgggagttgtgaaggttactcttcctgtcttgtctcccatctgcctgatattcatctggatagatccaatttgatatgtctccctttatgatccatggctcttctccttgttccaacttggagatgacatctggtttggaaactggataccccattgagaccaggtggctgtagttctccagcatcacatccctgtacagggtcctctgagaagggtcaagttgctgccactcctcctgggtgaaatccacagccacatccttgaatgatactaacccctgtggataaagctggacaataggaagcatctgtaatcaatttgttccttgaaagcaggggtcaacaaactttttcagtaaagtttacatttttggcattgcaggccatacggtttctgttgtaactactcaactctgccattgtagctagaaaaaagctgggacttcatcattttttgctcttccaaaaggccagatgactggtaaattttcctcagtcccaggacaagtcatgcagacagagctgaactatttcagaggacgtgggggctcccatgacagacagattattttatatgggggtatcaaaacatccttcaccgcacacatcccgcctctgactcccagctcgattatcaggtcccaaaaccaccatcaccgcttaatgggaaccgctgtcacatccctattggcaaactctcctgcttcctgtccgcgagcaccacaccgggctcccgaggctgcgccgttccgtactgggcggttttgcccgttccgcatcttcagaggctttgttcaggaagcaacatggctgctccctggagctgtttccgcatggggccgccatcttgagagcccggtcgtcttcgt

SEQ ID NO: 17080 - RNA, 103 nt, Homo sapiens
  source 1..103: mol_type = other RNA
tattcaggaaggtgttacttaattcatgcttgaaggacataacaattaatagacacgcaagcctgtaccgacgctcacgcccgtaccgacgctcacgcccgta

SEQ ID NO: 17081 - RNA, 1566 nt, Homo sapiens
  source 1..1566: mol_type = other RNA
tattgcacttgtcccggcctgtgggagcctcctccccagactctgaattcagtggcggccctggcatctcctcttggggcactgtctctggcatccggctttcctgactctgcttcttcctcttcttggtggatcccggagttgccctggcttcaggctgtccctcccctggcagttcaggctctagtggctgaattggctcagtcactgtgtgacctctctctttcttcttcttcttcttcttggtggatgtgggagctgcctgaggctcaaggtcatccggcagctcaggccccaccacctctgtctctggctccactgtggcatcttgctgtttttctttcttcgtcttctttttgggagctgccagagctgcctgggcctgaggcttcgctccttctggctgttgaggcgccatggtcccccctggggactccagaggcttcatctccggctccactggctccatcgcctccgtccctggctccatcattgccatctgtcccttttcttttttcctcttcttcgtagggggcagagggatggcttcctccagtggctccaccttcacctgtggctgagactcaactgtcaccccctcctctggctccatcccttccgtccccttttgcctctttctctttttggtcggggacaggactgtgtcttctagaggctcagtgttaatctgttcctgcttcactgtcttgtcttctggctcgaaggtttctttccctttgggcttcttcctcttcttggtggtggacgggaacagcactcccagaggctccagtgtctccactgtgggctctgtccccacaggccctgctgcctctggttctttcagctgctgattttttttcttcttcttcttccgcacatccatttctggcgaccccaaagccatgtccacctccagggccccgtgcccattcactgcctcctgagtgactggggcctctgtcacctgcatctcctttttcttcttccctgaggtgagcaggttgggggccaaggctgacctaggccctgtgactggtgggttgcccccaaaggcacagaaccgaggcctcaggccaggagggatctgtggtgggggacttgctgggatgggctgcagagggctccctgacagggattgctggggaccctcaaggatccttagggtgccctggggggctgaggcacaggtgagtccacctcctgcctccgttgagggggccagcagggtcgcttctccagcttggggacagctgctgaggactcgatagcggtgccgcttgcctgccaatttgcccttgacgatctgggagccagagagaggcacatgccgcccattgaagcattctggggcaaagtctgcaggggcctgaataagccacagctccgtatctggacccgtcagcgcctccaaggagaaacgaggggactctgaggctgggggcttcgcggtaaagttggggggacaagagaaccgagcagcatcctcaccgccggcctggggctcctccatcctgggacccacacctcaggcaaccctgtagcccgggctgctcgcaccaggtt

SEQ ID NO: 17082 - RNA, 1560 nt, Homo sapiens
  source 1..1560: mol_type = other RNA
tattgcacttgtcccggcctgtgggagcctcctccccagactctgaattcagtggcggccctggcatctcctcttggggcactgtctctggcatccggctttcctgactctgcttcttcctcttcttggtggatcccggagttgccctggcttcaggctgtccctcccctggcagttcaggctctagtggctgaattggctcagtcactgtgtgacctctctctttcttcttcttcttcttcttggtggatgtgggagctgcctgaggctcaaggtcatccggcagctcaggccccaccacctctgtctctggctccactgtggcatcttgctgtttttctttcttcgtcttctttttgggagctgccagagctgcctgggcctgaggcttcgctccttctggctgttgaggcgccatggtcccccctggggactccagaggcttcatctccggctccactggctccatcgcctccgtccctggctccatcattgccatctgtcccttttcttttttcctcttcttcgtagggggcagagggatggcttcctccagtggctccaccttcacctgtggctgagactcaactgtcaccccctcctctggctccatcccttccgtccccttttgcctctttctctttttggtcggggacaggactgtgtcttctagaggctcagtgttaatctgttcctgcttcactgtcttgtcttctggctcgaaggtttctttccctttgggcttcttcctcttcttggtggtggacgggaacagcactcccagaggctccagtgtctccactgtgggctctgtccccacaggccctgctgcctctggttctttcagctgctgattttttttcttcttcttcttccgcacatccatttctggcgaccccaaagccatgtccacctccagggccccgtgcccattcactgcctcctgagtgactggggcctctgtcacctgcatctcctttttcttcttccctgaggtgagcaggttgggggccaaggctgacctaggccctgtgactggtgggttgcccccaaaggcacagaaccgaggcctcaggccaggagggatctgtggtgggggacttgctgggatgggctgcagagggctccctgacagggattgctggggaccctcaaggatccttagggtgccctggggggctgaggcacaggtgagtccacctcctgcctccgttgagggggccagcagggtcgcttctccagcttggggacagctgctgaggactcgatagcggtgccgcttgcctgccaatttgcccttgacgatctgggagccagagagaggcacatgccgcccattgaagcattctggggcaaagtctgcaggggcctgaataagccacagctccgtatctggacccgtcagcgcctccaaggagaaacgaggggactctgaggctgggggcttcgcggtaaagttggggggacaagagaaccgagcagcatcgccggcctggggctcctccatcctgggacccacacctcaggcaaccctgtagcccgggctgctcgcaccaggtt

SEQ ID NO: 17083 - RNA, 9172 nt, Homo sapiens
  source 1..9172: mol_type = other RNA
tcaaaactgaggggcattttcttcttgcggagggtatctggatcaagtgtgtaagagtctgatttagaacgttcccgaggaggatcaagctttgtcttaacaggagcagtacttttttgaggtagatttttatcatgtggtgaggaggagcgtggagaactagcacccgatgggctagacctattggctgggagagtctttggcttaggagatgacaaccgagaacctggtcctggggattcagctctggagctagaaggcatcctcccatcagatttcaatgtctgcaaggtgttatggttgggggataatgacctactgtgggaatctgacctcaactttgcagcatcagattttaagatgagggattcactagcagataaactttctgtgccccttggcttcttctgatcagcagtagtccggctcatacgtccatcaggtttaagcgatctgctgtgtttagaggacagctctgattttcctgatgtagaggctggtttagaagatgttgagatgtttcctcgatcacccttcagtttgtgagacagagatgagagagcagaggcaggcccagctacaccataatttttgtaaatgcgctcacgagaagcaaggttgcgagatggagattctttgctatttccgagtccataatcaaatccttgggcactgcaacttgcccctttattaaaagcttgcactgagaaagggcttggaggaggagtttgagaattctgatccagaagagcttgttcatcttcatgtcggaggtactggtttccgcctctgtctctagctaaggaccatgcctctccttcatcactctcacagaactctaccatgctgttctgatccagttgcacccatgtcccttcagaattggttacctctcccactgctttgactttgtttcccagaactaacattccaattgggatacctctaaggttagggcagcttctgatgttgtgacctgaaggtcccgtcttcactaccttgtacatgcctggccctcctcgcaagaatggcatatcttgttcttgcattgttgcttcctgtgggcagcaggagtttatgtctttgaaaaagtcatcagtattagttttagattcctgggggaaaaaagctttggaagtccatgaaaatacgtccaaatccctgactccttggctagcattaaagatattgtcaacagggaccagaagactcttgccaagatgttgattaaaagagaggcaccaggcttcagtgtaaccattcatgttagggacatacttctttattgtctcatcattcagcctcagccacacaccatcatcattatggatctcatcaataaaagtgatagttccattgactttcactatgcctatctgctcactctgaagggaagggtggctacggatgcgaagccccgcactgtccttggccacaaattttcgaaccttattaggctgaggttcagactttggtttgaccaactgagttcctggtggtatcatcccttttggtgggtcttttacttttacttccagaccagcatcgatttcaatgccatcaatggtaacatgaagagtgtagagtccaatagcccctggagtccaatttgcacaataagtcccatcattattgacacggatcagcatattctcactgggtctcttaggagttggtgatgcaaaacgtagttcttcaaatgaataattttcataaaccttcatcattgttatggcaatatatcgagcttccttcactatcattggttcatatgaaacatctagctttggtgatgccagccctccataagtcatgtcagtattagaagatgcagctgttactgcaggactgccaggaatcctttgaggtttctttgcttgatcttgttgtaaagacatttttttctgagaaacagggacagctttcacttccaccttcatattgggaacatgtaccacatccccatactggtcttttgtttgaacagttatggtggtaggccaaccacaacgaatatcatccttattcaggatcaaagatgttttctgaggatccgcatatgaatctggctgaagccaccttgcaagccttccaccacttgatcctgggacacaggcaataaaatcatccagaaaagactgttcattgctttggatttggagtggtaaatttccctcaagtgcttctaatatagttggtgaatgagaaagagctagaccctttccaagaattccagaatgggttttgcacacctgcaatgcagcctcctcaagaatttcaaggtcttcttctaattcattaccaataggaagtgctaggtccttcttcatcagagctgctgcacaaaccccaccaagattggctaattctttttccaattggatgactccctcatcaggtccagggctaaattcatatccaattgcaaaacacttaaaaccatagaaagaagctttgtcatctttcacataatctgatgcagtctccaatgaaaaaagggcctcatttcctggcaacaccaaaaccatagtaggccacccagaggatcctgaaaatttctttaattctatccatgaattaagattttcatgaacagatgtcaattttggtccatatcctgaattctgaacagttctgacaggaatcaacaaacgaaggacatcttctgactgtgcagtaccacactgagggtcaaattcgattgtcatccacctcacacattctgggaatgtcaccttgtaatgcatcacacaggcaggtttatacgggtgctcactctctatgacagcatagtgactggaggttgtacaagcagagaggccctgttcaggctggtttcctgtggtgctatctgtcgactgattagggttgaaggcaggcggtgcatacttctgattcaaaatggcaactgacggaagcaattgttggacaaggccaaagacttctacagccaccttgggaatagcagcagctactggtcctatgtaggctataataagggggagcagcatggaaaacagactggaagaactcagcagttctggaatgtcatcagcatccacagcaagagctctgtgcaggaggtccttagaggctcgaacgacagtgcttacaacagacaatgctctgctacagtttttatcttcttcattggctttactcagaagttgggattgtaaatctccatcaaattcactcctatagtagagtatctgtgggatctgtcctctggtttggtttgtgccgttactgctcaagctgcacgtgctgaatgtgaatgtcacaccatcagggcactgaactgtggtcattcctccatctccattggctgtacggcttccatagttcctcaagcgcacagcatatttaacattttcctttaaaggaaccactttgtcaagtctgatctcagctatatcactgggtgagtcatccgttgtgtacgttcctttcactaattccagagatgtccatctgtgggaatgagttgaatctcctgcatgttcactatcatcaaccaacacctctaattcatattcatgaattccacctcctccatagacagagaaaccaaccacaactattccaggtttgtctactgaaaaacagattgcatcaggggacccgttcccagtgttccaacttctgccctgacttgtttttgtaaatcggttagcactagcttttacagagtgaagagaattaagtccatcaacctcagatcccagggctgacgctgtcagttcactgacaatgctggccagtaatccacaggtgttagagacgaggtgggaggagaagagttcattttctctcctcaggctgttcctgactggtagcacaacaatgaccagcattttctccagaacttcacggaagcttgtcatccctgagatattctcttcactctggctgagtttttccatatgtgccaccaaaaggggaaaacgatgaactagtgttgagtcgttctctgtactaacttgtttaacaattgatcgtagtaatacttctccatcatacgcaatcgggaagatggaagtcagcttaacagacgtgtgacacagagctgacataacagctgcaaggagtcggctacttgatgtcttgaagtttgcttcttggatatcctgatccaaacaattcagcagatcacaaaggcaagcccactgtaaggcaggagttgggtagaaagaatgaaagcaggcagtgaaagtattatgacattcctgaaggacagcttctagaagactcaagggttgactgagatatccttgaggatcattatccaatttcaccatgcagtgatcaactccttctgataaaatttttcttaacaaagttctggtttttccaatacactctgctaatttgctagtttcttctacaactgcttttcctgtagctgacactgggtaaatttcacaggtatagacacgcaataacctcagacaacaggtacccacaaagcgcagtctctctaaatctaggagtgtagctgtgaactggaatccttttaatcctctaagttcttcaactcctaagactaaggtggtccagctccagtgaagaatactcaacaatgactcaaaacattccactgagacagttcttgcaaaagacctctttaaaatgtgtacaggttcactggtttgctgtttgccttttgaagcactgccatcactggttggaagtctgtataataactgaggtatctgacccgcattaacatctgtaccattatttgatttctttgaactcttgaactggaaaacaaccccatcatctgtggtaatagatgcctgtccatgagatccacagtcactgctgggtcctgacactcgggcccatgccacataccaccacccagcttgcaggagaacaggctcatcaaacatcattgcatatttttctctagcagcacagtcataagccaatacatcagtctctgcaagaaggtcaccatcagtttcatgatctcctccatcaggacccaattcaaacagcttaattttagcagtatattctcctctacctccaaacagaccaagaccaccaagtaaaatatcagtgtcggcactgaaacgtatagcttctactgaatgggcagaataaccccagcctcctccatgactttcaaacctgtttaccacactataatcttctttagaataaaccttcattactgcttgagtctcttcctctgtacttgcaacacccatttttaagtcctgcatagctgccaaggtatcaagacaacctaaaatgtgcaaagctgcatgagatcgggtagtgagggcccttgatcctgttggtaaggcaagttcaggacttaggatactacatctggactgcatgtctgctgcagagggaagcctggcatcagcaaccaccgcattgtaacaccacagctctctagtatttggtcgaaacctccaaattacatcatatacaggatcaagacacacaccaaatccttgcagatcctcttgttctgagtcattaaaagttttacaactcccatccactttatttatcagaaggcatttaaatggaggaggttctgatatagaagcaggtaccaagcctattatgtgtttactggcaaaaatttctgatgtagcaagtacatgagaattaataagtgcttcatcaattcgtaaaaaagtttggtccccacttgcacctatccaagtagcttttcttccatattttgatccaatgttaggcatgggagctggctttgcattccaatatggcacatccaaaattggtctgcccagttgtcctttagaaaaacttccaaatgtgaagacctgtccatccattaaaagtactgccgtatggttgctgcctgcagtgacttgtgtgctagggcctggcaatgcttgaacaagagtgggacatcccctggagttgacatctccatgtcctagctgcccatgctgcccataaccaaatgtatagacatctccattttccattaaaaccactgaatggtgaaatccacagctgacttggactgcccggagctcacagtcaaatcgcacagagcctggagggtatgttgtgattttgcttgcatccttttcgcctctttctccacttccatctttgtgcttgtcccgtttatgctttagctgtgctggatgggatctgagtctggctagagcctgttctcgatggttcataaaaataggaccagcaaatacaagggggcctcttccttcctctaatctgtgccttctgattacacgttgccgtttttcttcttgtcgtaactgaaggtgttcttcaatgttaaccccgggcactgggacagctaaaagaagatctaaaggtatcatttctttcactgcatcaagaattcctctttgtcttgcctcttgaccatctaactctcttgcacaggccttgcaacatccacacacagcacaaccagattctccggaaccacaaccacagatccctccggggactctgtctggccgtccactactgacacagctggctccataacctgtacagtctccacagacagtgcaaaccatgcactgctccagcttccatttgtgcatgcctggagggcacatcatagacttctcatctttttcatctagttcttcttccaggtcttcatccattgctgttgccatattttcaactccaaaccctttcccaccttggttcatggcaccagtatctcgtccacactgtcctttattatttacaccaaatgtccacacctctccattcttcattaaaacacaagtgtgagctttgcccatagctacctgagttacaaaatggcccttcaaatcagttaccaaacttgaactatcagagtaaatggcatcttttccaaacatgtagagttctccatctttagaaataacagaactacttccattattgcaggctgtatataccacaatctttccttccatcttaattatctttttaggtttataaggtttggattgccgtctgctcttagttgattctccatcttctcctttactagcagatcctgtaaagaatatgctcccatcttctgcaactaaaagggcgtgagagccatcgtgtccaactgagaagtgtactatctttggagattttgtaattggtagctcaacccattttcctgctgaaggaccaccttgtttgattccaagactctggtatttgccagtgtaatatatctttccatttgctgttttcattagcgcaaactctcgtcctgcaccaagaattgctgactcctcatcaaatcctgtacttataatatgcaagtccttttccagatcgaatagtgagataccacaggcatgtaagcattttctagccagtttaagttgcaattcttgctgtagaacaggttcagtgcttgtggcaaatattctgacaacaaagccatcatctcttgaagcagctatctgattaatatattctccatcagtgaataaaatattttgaccttcagtgtggcaatctggtaacatcacagtaccatcttgctccagtgtttcagggcttatccttatggctgtcatgctgtggttattcacatctctatataataaataaccctgagcataccctaaccaagactttttttcttttctgtttctaatacgggatgtagaattgtatatatggcccctaactgttccactgtatccagagcctattttatataatccatccttgcataatagataaagaaaaaatccatcattctgaagtagacattggtcatcttcatcaacagatatttcttttaatggccacttgtgcattaaagctgctttcttaatgccattactaaaccagtcctgaatttgaatttttcccaccaaaactgcttgtacacttctctgtagcgaatttagaattgttggcacctgaatagtttggcaagcatggcttccattgttggtgaggatagcagagatggcctgaagtgtccttcctgtttctccccaagaagccaccagactaaagaggcaagcacaggaaagtgctgttaaggactgtcctgtgctgtcattcatcccagtacttcgaacggtgatttccaaaagaagctggaagagagactctaggacctcaggtggctcagactggaggccttctggctgctggccctgcagcacgttgagcagggcttggagactcctgagacacagggatggatgagaaaatcgtgtctctttgatcaattcaaaaacttcacaaaggccaacctcaataatctttggaagcttgatagggggctctttggattcctcttcttcatcactatctgattctccactctgcacagagttcttagatgcggctgccaatgatatttcctttttctgccattccagaacgcaatggcgtacattacagtaaatattgaaagcagaaggattgctatgtagtttgatatctggtatgattactgtattctctaagttttcagacttgcttcttgtcttcacttttgatttgctcttctgttttcttttcaatttcttcttatttaaaattttcttattcctggaggctgggtgtccagcgctgccgcccccctggtccctgtcattgagcgcagcggtataaatcctccggtagcggtcggccagggcccggcctgacagcagcagctggtagtgaccccgggagtccgcggcgggtagccccagccccagccccgcagcagccacggagccgtcgggaaccggcatgaacagcgcccccggcgccggggaggaagagaaggtggcggctgggtagaatccgtccccgccgagccccgaggaggcggcggcgggggaggcagtcgctgcgcacatcatcatcctcgccgccgccgccgccgccgccgcctcgtccccgcgggccgggcgggcagacacgcgcgcgcacacacagcccttttccaacgacgacggctccggcggcggcctctggctcccgcagcagggagactacaaagacagcgacctccttctcctcctccttcttctcctcctcccccccgcgccgccctcgccgctactggggccgctcatctaaccccgccaccccgggaatgtgaggaggaggcggtgccgccactgccgccgccaccaccgctaccaccgccaccaccgccggggctacccgcaatgggaagctgccg

SEQ ID NO: 17084 - RNA, 8872 nt, Homo sapiens
  source 1..8872: mol_type = other RNA
tcaaaactgaggggcattttcttcttgcggagggtatctggatcaagtgtgtaagagtctgatttagaacgttcccgaggaggatcaagctttgtcttaacaggagcagtacttttttgaggtagatttttatcatgtggtgaggaggagcgtggagaactagcacccgatgggctagacctattggctgggagagtctttggcttaggagatgacaaccgagaacctggtcctggggattcagctctggagctagaaggcatcctcccatcagatttcaatgtctgcaaggtgttatggttgggggataatgacctactgtgggaatctgacctcaactttgcagcatcagattttaagatgagggattcactagcagataaactttctgtgccccttggcttcttctgatcagcagtagtccggctcatacgtccatcaggtttaagcgatctgctgtgtttagaggacagctctgattttcctgatgtagaggctggtttagaagatgttgagatgtttcctcgatcacccttcagtttgtgagacagagatgagagagcagaggcaggcccagctacaccataatttttgtaaatgcgctcacgagaagcaaggttgcgagatggagattctttgctatttccgagtccataatcaaatccttgggcactgcaacttgcccctttattaaaagcttgcactgagaaagggcttggaggaggagtttgagaattctgatccagaagagcttgttcatcttcatgtcggaggtactggtttccgcctctgtctctagctaaggaccatgcctctccttcatcactctcacagaactctaccatgctgttctgatccagttgcacccatgtcccttcagaattggttacgtcaacagggaccagaagactcttgccaagatgttgattaaaagagaggcaccaggcttcagtgtaaccattcatgttagggacatacttctttattgtctcatcattcagcctcagccacacaccatcatcattatggatctcatcaataaaagtgatagttccattgactttcactatgcctatctgctcactctgaagggaagggtggctacggatgcgaagccccgcactgtccttggccacaaattttcgaaccttattaggctgaggttcagactttggtttgaccaactgagttcctggtggtatcatcccttttggtgggtcttttacttttacttccagaccagcatcgatttcaatgccatcaatggtaacatgaagagtgtagagtccaatagcccctggagtccaatttgcacaataagtcccatcattattgacacggatcagcatattctcactgggtctcttaggagttggtgatgcaaaacgtagttcttcaaatgaataattttcataaaccttcatcattgttatggcaatatatcgagcttccttcactatcattggttcatatgaaacatctagctttggtgatgccagccctccataagtcatgtcagtattagaagatgcagctgttactgcaggactgccaggaatcctttgaggtttctttgcttgatcttgttgtaaagacatttttttctgagaaacagggacagctttcacttccaccttcatattgggaacatgtaccacatccccatactggtcttttgtttgaacagttatggtggtaggccaaccacaacgaatatcatccttattcaggatcaaagatgttttctgaggatccgcatatgaatctggctgaagccaccttgcaagccttccaccacttgatcctgggacacaggcaataaaatcatccagaaaagactgttcattgctttggatttggagtggtaaatttccctcaagtgcttctaatatagttggtgaatgagaaagagctagaccctttccaagaattccagaatgggttttgcacacctgcaatgcagcctcctcaagaatttcaaggtcttcttctaattcattaccaataggaagtgctaggtccttcttcatcagagctgctgcacaaaccccaccaagattggctaattctttttccaattggatgactccctcatcaggtccagggctaaattcatatccaattgcaaaacacttaaaaccatagaaagaagctttgtcatctttcacataatctgatgcagtctccaatgaaaaaagggcctcatttcctggcaacaccaaaaccatagtaggccacccagaggatcctgaaaatttctttaattctatccatgaattaagattttcatgaacagatgtcaattttggtccatatcctgaattctgaacagttctgacaggaatcaacaaacgaaggacatcttctgactgtgcagtaccacactgagggtcaaattcgattgtcatccacctcacacattctgggaatgtcaccttgtaatgcatcacacaggcaggtttatacgggtgctcactctctatgacagcatagtgactggaggttgtacaagcagagaggccctgttcaggctggtttcctgtggtgctatctgtcgactgattagggttgaaggcaggcggtgcatacttctgattcaaaatggcaactgacggaagcaattgttggacaaggccaaagacttctacagccaccttgggaatagcagcagctactggtcctatgtaggctataataagggggagcagcatggaaaacagactggaagaactcagcagttctggaatgtcatcagcatccacagcaagagctctgtgcaggaggtccttagaggctcgaacgacagtgcttacaacagacaatgctctgctacagtttttatcttcttcattggctttactcagaagttgggattgtaaatctccatcaaattcactcctatagtagagtatctgtgggatctgtcctctggtttggtttgtgccgttactgctcaagctgcacgtgctgaatgtgaatgtcacaccatcagggcactgaactgtggtcattcctccatctccattggctgtacggcttccatagttcctcaagcgcacagcatatttaacattttcctttaaaggaaccactttgtcaagtctgatctcagctatatcactgggtgagtcatccgttgtgtacgttcctttcactaattccagagatgtccatctgtgggaatgagttgaatctcctgcatgttcactatcatcaaccaacacctctaattcatattcatgaattccacctcctccatagacagagaaaccaaccacaactattccaggtttgtctactgaaaaacagattgcatcaggggacccgttcccagtgttccaacttctgccctgacttgtttttgtaaatcggttagcactagcttttacagagtgaagagaattaagtccatcaacctcagatcccagggctgacgctgtcagttcactgacaatgctggccagtaatccacaggtgttagagacgaggtgggaggagaagagttcattttctctcctcaggctgttcctgactggtagcacaacaatgaccagcattttctccagaacttcacggaagcttgtcatccctgagatattctcttcactctggctgagtttttccatatgtgccaccaaaaggggaaaacgatgaactagtgttgagtcgttctctgtactaacttgtttaacaattgatcgtagtaatacttctccatcatacgcaatcgggaagatggaagtcagcttaacagacgtgtgacacagagctgacataacagctgcaaggagtcggctacttgatgtcttgaagtttgcttcttggatatcctgatccaaacaattcagcagatcacaaaggcaagcccactgtaaggcaggagttgggtagaaagaatgaaagcaggcagtgaaagtattatgacattcctgaaggacagcttctagaagactcaagggttgactgagatatccttgaggatcattatccaatttcaccatgcagtgatcaactccttctgataaaatttttcttaacaaagttctggtttttccaatacactctgctaatttgctagtttcttctacaactgcttttcctgtagctgacactgggtaaatttcacaggtatagacacgcaataacctcagacaacaggtacccacaaagcgcagtctctctaaatctaggagtgtagctgtgaactggaatccttttaatcctctaagttcttcaactcctaagactaaggtggtccagctccagtgaagaatactcaacaatgactcaaaacattccactgagacagttcttgcaaaagacctctttaaaatgtgtacaggttcactggtttgctgtttgccttttgaagcactgccatcactggttggaagtctgtataataactgaggtatctgacccgcattaacatctgtaccattatttgatttctttgaactcttgaactggaaaacaaccccatcatctgtggtaatagatgcctgtccatgagatccacagtcactgctgggtcctgacactcgggcccatgccacataccaccacccagcttgcaggagaacaggctcatcaaacatcattgcatatttttctctagcagcacagtcataagccaatacatcagtctctgcaagaaggtcaccatcagtttcatgatctcctccatcaggacccaattcaaacagcttaattttagcagtatattctcctctacctccaaacagaccaagaccaccaagtaaaatatcagtgtcggcactgaaacgtatagcttctactgaatgggcagaataaccccagcctcctccatgactttcaaacctgtttaccacactataatcttctttagaataaaccttcattactgcttgagtctcttcctctgtacttgcaacacccatttttaagtcctgcatagctgccaaggtatcaagacaacctaaaatgtgcaaagctgcatgagatcgggtagtgagggcccttgatcctgttggtaaggcaagttcaggacttaggatactacatctggactgcatgtctgctgcagagggaagcctggcatcagcaaccaccgcattgtaacaccacagctctctagtatttggtcgaaacctccaaattacatcatatacaggatcaagacacacaccaaatccttgcagatcctcttgttctgagtcattaaaagttttacaactcccatccactttatttatcagaaggcatttaaatggaggaggttctgatatagaagcaggtaccaagcctattatgtgtttactggcaaaaatttctgatgtagcaagtacatgagaattaataagtgcttcatcaattcgtaaaaaagtttggtccccacttgcacctatccaagtagcttttcttccatattttgatccaatgttaggcatgggagctggctttgcattccaatatggcacatccaaaattggtctgcccagttgtcctttagaaaaacttccaaatgtgaagacctgtccatccattaaaagtactgccgtatggttgctgcctgcagtgacttgtgtgctagggcctggcaatgcttgaacaagagtgggacatcccctggagttgacatctccatgtcctagctgcccatgctgcccataaccaaatgtatagacatctccattttccattaaaaccactgaatggtgaaatccacagctgacttggactgcccggagctcacagtcaaatcgcacagagcctggagggtatgttgtgattttgcttgcatccttttcgcctctttctccacttccatctttgtgcttgtcccgtttatgctttagctgtgctggatgggatctgagtctggctagagcctgttctcgatggttcataaaaataggaccagcaaatacaagggggcctcttccttcctctaatctgtgccttctgattacacgttgccgtttttcttcttgtcgtaactgaaggtgttcttcaatgttaaccccgggcactgggacagctaaaagaagatctaaaggtatcatttctttcactgcatcaagaattcctctttgtcttgcctcttgaccatctaactctcttgcacaggccttgcaacatccacacacagcacaaccagattctccggaaccacaaccacagatccctccggggactctgtctggccgtccactactgacacagctggctccataacctgtacagtctccacagacagtgcaaaccatgcactgctccagcttccatttgtgcatgcctggagggcacatcatagacttctcatctttttcatctagttcttcttccaggtcttcatccattgctgttgccatattttcaactccaaaccctttcccaccttggttcatggcaccagtatctcgtccacactgtcctttattatttacaccaaatgtccacacctctccattcttcattaaaacacaagtgtgagctttgcccatagctacctgagttacaaaatggcccttcaaatcagttaccaaacttgaactatcagagtaaatggcatcttttccaaacatgtagagttctccatctttagaaataacagaactacttccattattgcaggctgtatataccacaatctttccttccatcttaattatctttttaggtttataaggtttggattgccgtctgctcttagttgattctccatcttctcctttactagcagatcctgtaaagaatatgctcccatcttctgcaactaaaagggcgtgagagccatcgtgtccaactgagaagtgtactatctttggagattttgtaattggtagctcaacccattttcctgctgaaggaccaccttgtttgattccaagactctggtatttgccagtgtaatatatctttccatttgctgttttcattagcgcaaactctcgtcctgcaccaagaattgctgactcctcatcaaatcctgtacttataatatgcaagtccttttccagatcgaatagtgagataccacaggcatgtaagcattttctagccagtttaagttgcaattcttgctgtagaacaggttcagtgcttgtggcaaatattctgacaacaaagccatcatctcttgaagcagctatctgattaatatattctccatcagtgaataaaatattttgaccttcagtgtggcaatctggtaacatcacagtaccatcttgctccagtgtttcagggcttatccttatggctgtcatgctgtggttattcacatctctatataataaataaccctgagcataccctaaccaagactttttttcttttctgtttctaatacgggatgtagaattgtatatatggcccctaactgttccactgtatccagagcctattttatataatccatccttgcataatagataaagaaaaaatccatcattctgaagtagacattggtcatcttcatcaacagatatttcttttaatggccacttgtgcattaaagctgctttcttaatgccattactaaaccagtcctgaatttgaatttttcccaccaaaactgcttgtacacttctctgtagcgaatttagaattgttggcacctgaatagtttggcaagcatggcttccattgttggtgaggatagcagagatggcctgaagtgtccttcctgtttctccccaagaagccaccagactaaagaggcaagcacaggaaagtgctgttaaggactgtcctgtgctgtcattcatcccagtacttcgaacggtgatttccaaaagaagctggaagagagactctaggacctcaggtggctcagactggaggccttctggctgctggccctgcagcacgttgagcagggcttggagactcctgagacacagggatggatgagaaaatcgtgtctctttgatcaattcaaaaacttcacaaaggccaacctcaataatctttggaagcttgatagggggctctttggattcctcttcttcatcactatctgattctccactctgcacagagttcttagatgcggctgccaatgatatttcctttttctgccattccagaacgcaatggcgtacattacagtaaatattgaaagcagaaggattgctatgtagtttgatatctggtatgattactgtattctctaagttttcagacttgcttcttgtcttcacttttgatttgctcttctgttttcttttcaatttcttcttatttaaaattttcttattcctggaggctgggtgtccagcgctgccgcccccctggtccctgtcattgagcgcagcggtataaatcctccggtagcggtcggccagggcccggcctgacagcagcagctggtagtgaccccgggagtccgcggcgggtagccccagccccagccccgcagcagccacggagccgtcgggaaccggcatgaacagcgcccccggcgccggggaggaagagaaggtggcggctgggtagaatccgtccccgccgagccccgaggaggcggcggcgggggaggcagtcgctgcgcacatcatcatcctcgccgccgccgccgccgccgccgcctcgtccccgcgggccgggcgggcagacacgcgcgcgcacacacagcccttttccaacgacgacggctccggcggcggcctctggctcccgcagcagggagactacaaagacagcgacctccttctcctcctccttcttctcctcctcccccccgcgccgccctcgccgctactggggccgctcatctaaccccgccaccccgggaatgtgaggaggaggcggtgccgccactgccgccgccaccaccgctaccaccgccaccaccgccggggctacccgcaatgggaagctgccg

SEQ ID NO: 17085 - RNA, 9295 nt, Homo sapiens
  source 1..9295: mol_type = other RNA
tcaaaactgaggggcattttcttcttgcggagggtatctggatcaagtgtgtaagagtctgatttagaacgttcccgaggaggatcaagctttgtcttaacaggagcagtacttttttgaggtagatttttatcatgtggtgaggaggagcgtggagaactagcacccgatgggctagacctattggctgggagagtctttggcttaggagatgacaaccgagaacctggtcctggggattcagctctggagctagaaggcatcctcccatcagatttcaatgtctgcaaggtgttatggttgggggataatgacctactgtgggaatctgacctcaactttgcagcatcagattttaagatgagggattcactagcagataaactttctgtgccccttggcttcttctgatcagcagtagtccggctcatacgtccatcaggtttaagcgatctgctgtgtttagaggacagctctgattttcctgatgtagaggctggtttagaagatgttgagatgtttcctcgatcacccttcagtttgtgagacagagatgagagagcagaggcaggcccagctacaccataatttttgtaaatgcgctcacgagaagcaaggttgcgagatggagatttctgaagctgaggctgctggaaggaaaggggctgtccgaacacaaatgggctgtgtactagggaagagggaggttttgcagcttgatcaaagatggaaggagctgggagattgggtcgtgactgaatggaattcaatatggcactcagttggtcacctgcagtgggtaaaacagtcaaaactttgctatttccgagtccataatcaaatccttgggcactgcaacttgcccctttattaaaagcttgcactgagaaagggcttggaggaggagtttgagaattctgatccagaagagcttgttcatcttcatgtcggaggtactggtttccgcctctgtctctagctaaggaccatgcctctccttcatcactctcacagaactctaccatgctgttctgatccagttgcacccatgtcccttcagaattggttacctctcccactgctttgactttgtttcccagaactaacattccaattgggatacctctaaggttagggcagcttctgatgttgtgacctgaaggtcccgtcttcactaccttgtacatgcctggccctcctcgcaagaatggcatatcttgttcttgcattgttgcttcctgggggaaaaaagctttggaagtccatgaaaatacgtccaaatccctgactccttggctagcattaaagatattgtcaacagggaccagaagactcttgccaagatgttgattaaaagagaggcaccaggcttcagtgtaaccattcatgttagggacatacttctttattgtctcatcattcagcctcagccacacaccatcatcattatggatctcatcaataaaagtgatagttccattgactttcactatgcctatctgctcactctgaagggaagggtggctacggatgcgaagccccgcactgtccttggccacaaattttcgaaccttattaggctgaggttcagactttggtttgaccaactgagttcctggtggtatcatcccttttggtgggtcttttacttttacttccagaccagcatcgatttcaatgccatcaatggtaacatgaagagtgtagagtccaatagcccctggagtccaatttgcacaataagtcccatcattattgacacggatcagcatattctcactgggtctcttaggagttggtgatgcaaaacgtagttcttcaaatgaataattttcataaaccttcatcattgttatggcaatatatcgagcttccttcactatcattggttcatatgaaacatctagctttggtgatgccagccctccataagtcatgtcagtattagaagatgcagctgttactgcaggactgccaggaatcctttgaggtttctttgcttgatcttgttgtaaagacatttttttctgagaaacagggacagctttcacttccaccttcatattgggaacatgtaccacatccccatactggtcttttgtttgaacagttatggtggtaggccaaccacaacgaatatcatccttattcaggatcaaagatgttttctgaggatccgcatatgaatctggctgaagccaccttgcaagccttccaccacttgatcctgggacacaggcaataaaatcatccagaaaagactgttcattgctttggatttggagtggtaaatttccctcaagtgcttctaatatagttggtgaatgagaaagagctagaccctttccaagaattccagaatgggttttgcacacctgcaatgcagcctcctcaagaatttcaaggtcttcttctaattcattaccaataggaagtgctaggtccttcttcatcagagctgctgcacaaaccccaccaagattggctaattctttttccaattggatgactccctcatcaggtccagggctaaattcatatccaattgcaaaacacttaaaaccatagaaagaagctttgtcatctttcacataatctgatgcagtctccaatgaaaaaagggcctcatttcctggcaacaccaaaaccatagtaggccacccagaggatcctgaaaatttctttaattctatccatgaattaagattttcatgaacagatgtcaattttggtccatatcctgaattctgaacagttctgacaggaatcaacaaacgaaggacatcttctgactgtgcagtaccacactgagggtcaaattcgattgtcatccacctcacacattctgggaatgtcaccttgtaatgcatcacacaggcaggtttatacgggtgctcactctctatgacagcatagtgactggaggttgtacaagcagagaggccctgttcaggctggtttcctgtggtgctatctgtcgactgattagggttgaaggcaggcggtgcatacttctgattcaaaatggcaactgacggaagcaattgttggacaaggccaaagacttctacagccaccttgggaatagcagcagctactggtcctatgtaggctataataagggggagcagcatggaaaacagactggaagaactcagcagttctggaatgtcatcagcatccacagcaagagctctgtgcaggaggtccttagaggctcgaacgacagtgcttacaacagacaatgctctgctacagtttttatcttcttcattggctttactcagaagttgggattgtaaatctccatcaaattcactcctatagtagagtatctgtgggatctgtcctctggtttggtttgtgccgttactgctcaagctgcacgtgctgaatgtgaatgtcacaccatcagggcactgaactgtggtcattcctccatctccattggctgtacggcttccatagttcctcaagcgcacagcatatttaacattttcctttaaaggaaccactttgtcaagtctgatctcagctatatcactgggtgagtcatccgttgtgtacgttcctttcactaattccagagatgtccatctgtgggaatgagttgaatctcctgcatgttcactatcatcaaccaacacctctaattcatattcatgaattccacctcctccatagacagagaaaccaaccacaactattccaggtttgtctactgaaaaacagattgcatcaggggacccgttcccagtgttccaacttctgccctgacttgtttttgtaaatcggttagcactagcttttacagagtgaagagaattaagtccatcaacctcagatcccagggctgacgctgtcagttcactgacaatgctggccagtaatccacaggtgttagagacgaggtgggaggagaagagttcattttctctcctcaggctgttcctgactggtagcacaacaatgaccagcattttctccagaacttcacggaagcttgtcatccctgagatattctcttcactctggctgagtttttccatatgtgccaccaaaaggggaaaacgatgaactagtgttgagtcgttctctgtactaacttgtttaacaattgatcgtagtaatacttctccatcatacgcaatcgggaagatggaagtcagcttaacagacgtgtgacacagagctgacataacagctgcaaggagtcggctacttgatgtcttgaagtttgcttcttggatatcctgatccaaacaattcagcagatcacaaaggcaagcccactgtaaggcaggagttgggtagaaagaatgaaagcaggcagtgaaagtattatgacattcctgaaggacagcttctagaagactcaagggttgactgagatatccttgaggatcattatccaatttcaccatgcagtgatcaactccttctgataaaatttttcttaacaaagttctggtttttccaatacactctgctaatttgctagtttcttctacaactgcttttcctgtagctgacactgggtaaatttcacaggtatagacacgcaataacctcagacaacaggtacccacaaagcgcagtctctctaaatctaggagtgtagctgtgaactggaatccttttaatcctctaagttcttcaactcctaagactaaggtggtccagctccagtgaagaatactcaacaatgactcaaaacattccactgagacagttcttgcaaaagacctctttaaaatgtgtacaggttcactggtttgctgtttgccttttgaagcactgccatcactggttggaagtctgtataataactgaggtatctgacccgcattaacatctgtaccattatttgatttctttgaactcttgaactggaaaacaaccccatcatctgtggtaatagatgcctgtccatgagatccacagtcactgctgggtcctgacactcgggcccatgccacataccaccacccagcttgcaggagaacaggctcatcaaacatcattgcatatttttctctagcagcacagtcataagccaatacatcagtctctgcaagaaggtcaccatcagtttcatgatctcctccatcaggacccaattcaaacagcttaattttagcagtatattctcctctacctccaaacagaccaagaccaccaagtaaaatatcagtgtcggcactgaaacgtatagcttctactgaatgggcagaataaccccagcctcctccatgactttcaaacctgtttaccacactataatcttctttagaataaaccttcattactgcttgagtctcttcctctgtacttgcaacacccatttttaagtcctgcatagctgccaaggtatcaagacaacctaaaatgtgcaaagctgcatgagatcgggtagtgagggcccttgatcctgttggtaaggcaagttcaggacttaggatactacatctggactgcatgtctgctgcagagggaagcctggcatcagcaaccaccgcattgtaacaccacagctctctagtatttggtcgaaacctccaaattacatcatatacaggatcaagacacacaccaaatccttgcagatcctcttgttctgagtcattaaaagttttacaactcccatccactttatttatcagaaggcatttaaatggaggaggttctgatatagaagcaggtaccaagcctattatgtgtttactggcaaaaatttctgatgtagcaagtacatgagaattaataagtgcttcatcaattcgtaaaaaagtttggtccccacttgcacctatccaagtagcttttcttccatattttgatccaatgttaggcatgggagctggctttgcattccaatatggcacatccaaaattggtctgcccagttgtcctttagaaaaacttccaaatgtgaagacctgtccatccattaaaagtactgccgtatggttgctgcctgcagtgacttgtgtgctagggcctggcaatgcttgaacaagagtgggacatcccctggagttgacatctccatgtcctagctgcccatgctgcccataaccaaatgtatagacatctccattttccattaaaaccactgaatggtgaaatccacagctgacttggactgcccggagctcacagtcaaatcgcacagagcctggagggtatgttgtgattttgcttgcatccttttcgcctctttctccacttccatctttgtgcttgtcccgtttatgctttagctgtgctggatgggatctgagtctggctagagcctgttctcgatggttcataaaaataggaccagcaaatacaagggggcctcttccttcctctaatctgtgccttctgattacacgttgccgtttttcttcttgtcgtaactgaaggtgttcttcaatgttaaccccgggcactgggacagctaaaagaagatctaaaggtatcatttctttcactgcatcaagaattcctctttgtcttgcctcttgaccatctaactctcttgcacaggccttgcaacatccacacacagcacaaccagattctccggaaccacaaccacagatccctccggggactctgtctggccgtccactactgacacagctggctccataacctgtacagtctccacagacagtgcaaaccatgcactgctccagcttccatttgtgcatgcctggagggcacatcatagacttctcatctttttcatctagttcttcttccaggtcttcatccattgctgttgccatattttcaactccaaaccctttcccaccttggttcatggcaccagtatctcgtccacactgtcctttattatttacaccaaatgtccacacctctccattcttcattaaaacacaagtgtgagctttgcccatagctacctgagttacaaaatggcccttcaaatcagttaccaaacttgaactatcagagtaaatggcatcttttccaaacatgtagagttctccatctttagaaataacagaactacttccattattgcaggctgtatataccacaatctttccttccatcttaattatctttttaggtttataaggtttggattgccgtctgctcttagttgattctccatcttctcctttactagcagatcctgtaaagaatatgctcccatcttctgcaactaaaagggcgtgagagccatcgtgtccaactgagaagtgtactatctttggagattttgtaattggtagctcaacccattttcctgctgaaggaccaccttgtttgattccaagactctggtatttgccagtgtaatatatctttccatttgctgttttcattagcgcaaactctcgtcctgcaccaagaattgctgactcctcatcaaatcctgtacttataatatgcaagtccttttccagatcgaatagtgagataccacaggcatgtaagcattttctagccagtttaagttgcaattcttgctgtagaacaggttcagtgcttgtggcaaatattctgacaacaaagccatcatctcttgaagcagctatctgattaatatattctccatcagtgaataaaatattttgaccttcagtgtggcaatctggtaacatcacagtaccatcttgctccagtgtttcagggcttatccttatggctgtcatgctgtggttattcacatctctatataataaataaccctgagcataccctaaccaagactttttttcttttctgtttctaatacgggatgtagaattgtatatatggcccctaactgttccactgtatccagagcctattttatataatccatccttgcataatagataaagaaaaaatccatcattctgaagtagacattggtcatcttcatcaacagatatttcttttaatggccacttgtgcattaaagctgctttcttaatgccattactaaaccagtcctgaatttgaatttttcccaccaaaactgcttgtacacttctctgtagcgaatttagaattgttggcacctgaatagtttggcaagcatggcttccattgttggtgaggatagcagagatggcctgaagtgtccttcctgtttctccccaagaagccaccagactaaagaggcaagcacaggaaagtgctgttaaggactgtcctgtgctgtcattcatcccagtacttcgaacggtgatttccaaaagaagctggaagagagactctaggacctcaggtggctcagactggaggccttctggctgctggccctgcagcacgttgagcagggcttggagactcctgagacacagggatggatgagaaaatcgtgtctctttgatcaattcaaaaacttcacaaaggccaacctcaataatctttggaagcttgatagggggctctttggattcctcttcttcatcactatctgattctccactctgcacagagttcttagatgcggctgccaatgatatttcctttttctgccattccagaacgcaatggcgtacattacagtaaatattgaaagcagaaggattgctatgtagtttgatatctggtatgattactgtattctctaagttttcagacttgcttcttgtcttcacttttgatttgctcttctgttttcttttcaatttcttcttatttaaaattttcttattcctggaggctgggtgtccagcgctgccgcccccctggtccctgtcattgagcgcagcggtataaatcctccggtagcggtcggccagggcccggcctgacagcagcagctggtagtgaccccgggagtccgcggcgggtagccccagccccagccccgcagcagccacggagccgtcgggaaccggcatgaacagcgcccccggcgccggggaggaagagaaggtggcggctgggtagaatccgtccccgccgagccccgaggaggcggcggcgggggaggcagtcgctgcgcacatcatcatcctcgccgccgccgccgccgccgccgcctcgtccccgcgggccgggcgggcagacacgcgcgcgcacacacagcccttttccaacgacgacggctccggcggcggcctctggctcccgcagcagggagactacaaagacagcgacctccttctcctcctccttcttctcctcctcccccccgcgccgccctcgccgctactggggccgctcatctaaccccgccaccccgggaatgtgaggaggaggcggtgccgccactgccgccgccaccaccgctaccaccgccaccaccgccggggctacccgcaatgggaagctgccg

SEQ ID NO: 17086 - RNA, 6400 nt, Homo sapiens
  source 1..6400: mol_type = other RNA
tcaaaactgaggggcattttcttcttgcggagggtatctggatcaagtgtgtaagagtctgatttagaacgttcccgaggaggatcaagctttgtcttaacaggagcagtacttttttgaggtagatttttatcatgtggtgaggaggagcgtggagaactagcacccgatgggctagacctattggctgggagagtctttggcttaggagatgacaaccgagaacctggtcctggggattcagctctggagctagaaggcatcctcccatcagatttcaatgtctgcaaggtgttatggttgggggataatgacctactgtgggaatctgacctcaactttgcagcatcagattttaagatgagggattcactagcagataaactttctgtgccccttggcttcttctgatcagcagtagtccggctcatacgtccatcaggtttaagcgatctgctgtgtttagaggacagctctgattttcctgatgtagaggctggtttagaagatgttgagatgtttcctcgatcacccttcagtttgtgagacagagatgagagagcagaggcaggcccagctacaccataatttttgtaaatgcgctcacgagaagcaaggttgcgagatggagatttctgaagctgaggctgctggaaggaaaggggctgtccgaacacaaatgggctgtgtactagggaagagggaggttttgcagcttgatcaaagatggaaggagctgggagattgggtcgtgactgaatggaattcaatatggcactcagttggtcacctgcagtgggtaaaacagtcaaaactttgctatttccgagtccataatcaaatccttgggcactgcaacttgcccctttattaaaagcttgcactgagaaagggcttggaggaggagtttgagaattctgatccagaagagcttgttcatcttcatgtcggaggtactggtttccgcctctgtctctagctaaggaccatgcctctccttcatcactctcacagaactctaccatgctgttctgatccagttgcacccatgtcccttcagaattggttacctctcccactgctttgactttgtttcccagaactaacattccaattgggatacctctaaggttagggcagcttctgatgttgtgacctgaaggtcccgtcttcactaccttgtacatgcctggccctcctcgcaagaatggcatatcttgttcttgcattgttgcttcctgtgggcagcaggagtttatgtctttgaaaaagtcatcagtattagttttagattcctgggggaaaaaagctttggaagtccatgaaaatacgtccaaatccctgactccttggctagcattaaagatattgtcaacagggaccagaagactcttgccaagatgttgattaaaagagaggcaccaggcttcagtgtaaccattcatgttagggacatacttctttattgtctcatcattcagcctcagccacacaccatcatcattatggatctcatcaataaaagtgatagttccattgactttcactatgcctatctgctcactctgaagggaagggtggctacggatgcgaagccccgcactgtccttggccacaaattttcgaaccttattaggctgaggttcagactttggtttgaccaactgagttcctggtggtatcatcccttttggtgggtcttttacttttacttccagaccagcatcgatttcaatgccatcaatggtaacatgaagagtgtagagtccaatagcccctggagtccaatttgcacaataagtcccatcattattgacacggatcagcatattctcactgggtctcttaggagttggtgatgcaaaacgtagttcttcaaatgaataattttcataaaccttcatcattgttatggcaatatatcgagcttccttcactatcattggttcatatgaaacatctagctttggtgatgccagccctccataagtcatgtcagtattagaagatgcagctgttactgcaggactgccaggaatcctttgaggtttctttgcttgatcttgttgtaaagacatttttttctgagaaacagggacagctttcacttccaccttcatattgggaacatgtaccacatccccatactggtcttttgtttgaacagttatggtggtaggccaaccacaacgaatatcatccttattcaggatcaaagatgttttctgaggatccgcatatgaatctggctgaagccaccttgcaagccttccaccacttgatcctgggacacaggcaataaaatcatccagaaaagactgttcattgctttggatttggagtggtaaatttccctcaagtgcttctaatatagttggtgaatgagaaagagctagaccctttccaagaattccagaatgggttttgcacacctgcaatgcagcctcctcaagaatttcaaggtcttcttctaattcattaccaataggaagtgctaggtccttcttcatcagagctgctgcacaaaccccaccaagattggctaattctttttccaattggatgactccctcatcaggtccagggctaaattcatatccaattgcaaaacacttaaaaccatagaaagaagctttgtcatctttcacataatctgatgcagtctccaatgaaaaaagggcctcatttcctggcaacaccaaaaccatagtaggccacccagaggatcctgaaaatttctttaattctatccatgaattaagattttcatgaacagatgtcaattttggtccatatcctgaattctgaacagttctgacaggaatcaacaaacgaaggacatcttctgactgtgcagtaccacactgagggtcaaattcgattgtcatccacctcacacattctgggaatgtcaccttgtaatgcatcacacaggcaggtttatacgggtgctcactctctatgacagcatagtgactggaggttgtacaagcagagaggccctgttcaggctggtttcctgtggtgctatctgtcgactgattagggttgaaggcaggcggtgcatacttctgattcaaaatggcaactgacggaagcaattgttggacaaggccaaagacttctacagccaccttgggaatagcagcagctactggtcctatgtaggctataataagggggagcagcatggaaaacagactggaagaactcagcagttctggaatgtcatcagcatccacagcaagagctctgtgcaggaggtccttagaggctcgaacgacagtgcttacaacagacaatgctctgctacagtttttatcttcttcattggctttactcagaagttgggattgtaaatctccatcaaattcactcctatagtagagtatctgtgggatctgtcctctggtttggtttgtgccgttactgctcaagctgcacgtgctgaatgtgaatgtcacaccatcagggcactgaactgtggtcattcctccatctccattggctgtacggcttccatagttcctcaagcgcacagcatatttaacattttcctttaaaggaaccactttgtcaagtctgatctcagctatatcactgggtgagtcatccgttgtgtacgttcctttcactaattccagagatgtccatctgtgggaatgagttgaatctcctgcatgttcactatcatcaaccaacacctctaattcatattcatgaattccacctcctccatagacagagaaaccaaccacaactattccaggtttgtctactgaaaaacagattgcatcaggggacccgttcccagtgttccaacttctgccctgacttgtttttgtaaatcggttagcactagcttttacagagtgaagagaattaagtccatcaacctcagatcccagggctgacgctgtcagttcactgacaatgctggccagtaatccacaggtgttagagacgaggtgggaggagaagagttcattttctctcctcaggctgttcctgactggtagcacaacaatgaccagcattttctccagaacttcacggaagcttgtcatccctgagatattctcttcactctggctgagtttttccatatgtgccaccaaaaggggaaaacgatgaactagtgttgagtcgttctctgtactaacttgtttaacaattgatcgtagtaatacttctccatcatacgcaatcgggaagatggaagtcagcttaacagacgtgtgacacagagctgacataacagctgcaaggagtcggctacttgatgtcttgaagtttgcttcttggatatcctgatccaaacaattcagcagatcacaaaggcaagcccactgtaaggcaggagttgggtagaaagaatgaaagcaggcagtgaaagtattatgacattcctgaaggacagcttctagaagactcaagggttgactgagatatccttgaggatcattatccaatttcaccatgcagtgatcaactccttctgataaaatttttcttaacaaagttctggtttttccaatacactctgctaatttgctagtttcttctacaactgcttttcctgtagctgacactgggtaaatttcacaggtatagacacgcaataacctcagacaacaggtacccacaaagcgcagtctctctaaatctaggagtgtagctgtgaactggaatccttttaatcctctaagttcttcaactcctaagactaaggtggtccagctccagtgaagaatactcaacaatgactcaaaacattccactgagacagttcttgcaaaagacctctttaaaatgtgtacaggttcactggtttgctgtttgccttttgaagcactgccatcactggttggaagtctgtataataactgaggtatctgacccgcattaacatctgtaccattatttgatttctttgaactcttgaactggaaaacaaccccatcatctgtggtaatagatgcctgtccatgagatccacagtcactgctgggtcctgacactcgggcccatgccacataccaccacccagcttgcaggagaacaggctcatcaaacatcattgcatatttttctctagcagcacagtcataagccaatacatcagtctctgcaagaaggtcaccatcagtttcatgatctcctccatcaggacccaattcaaacagcttaattttagcagtatattctcctctacctccaaacagaccaagaccaccaagtaaaatatcagtgtcggcactgaaacgtatagcttctactgaatgggcagaataaccccagcctcctccatgactttcaaacctgtttaccacactataatcttctttagaataaaccttcattactgcttgagtctcttcctctgtacttgcaacacccatttttaagtcctgcatagctgccaaggtatcaagacaacctaaaatgtgcaaagctgcatgagatcgggtagtgagggcccttgatcctgttggtaaggcaagttcaggacttaggatactacatctggactgcatgtctgctgcagagggaagcctggcatcagcaaccaccgcattgtaacaccacagctctctagtatttggtcgaaacctccaaattacatcatatacaggatcaagacacacaccaaatccttgcagatcctcttgttctgagtcattaaaagttttacaactcccatccactttatttatcagaaggcatttaaatggaggaggttctgatatagaagcaggtaccaagcctattatgtgtttactggcaaaaatttctgatgtagcaagtacatgagaattaataagtgcttcatcaattcgtaaaaaagtttggtccccacttgcacctatccaagtagcttttcttccatattttgatccaatgttaggcatgggagctggctttgcattccaatatggcacatccaaaattggtctgcccagttgtcctttagaaaaacttccaaatgtgaagacctgtccatccattaaaagtactgccgtatggttgctgcctgcagtgacttgtgtgctagggcctggcaatgcttgaacaagagtgggacatcccctggagttgacatctccatgtcctagctgcccatgctgcccataaccaaatgtatagacatctccattttccattaaaaccactgaatggtgaaatccacagctgacttggactgcccggagctcacagtcaaatcgcacagagcctggagggtatgttgtgattttgcttgcatccttttcgcctctttctccacttccataagaattaactgctggacccagaggctgaaggcacgttgaaggaatccttcatttcttgagcccttggtttgaaaagctagtgattttagacaggtttccccttataa

SEQ ID NO: 17087 - RNA, 9244 nt, Homo sapiens
  source 1..9244: mol_type = other RNA
tcaaaactgaggggcattttcttcttgcggagggtatctggatcaagtgtgtaagagtctgatttagaacgttcccgaggaggatcaagctttgtcttaacaggagcagtacttttttgaggtagatttttatcatgtggtgaggaggagcgtggagaactagcacccgatgggctagacctattggctgggagagtctttggcttaggagatgacaaccgagaacctggtcctggggattcagctctggagctagaaggcatcctcccatcagatttcaatgtctgcaaggtgttatggttgggggataatgacctactgtgggaatctgacctcaactttgcagcatcagattttaagatgagggattcactagcagataaactttctgtgccccttggcttcttctgatcagcagtagtccggctcatacgtccatcaggtttaagcgatctgctgtgtttagaggacagctctgattttcctgatgtagaggctggtttagaagatgttgagatgtttcctcgatcacccttcagtttgtgagacagagatgagagagcagaggcaggcccagctacaccataatttttgtaaatgcgctcacgagaagcaaggttgcgagatggagatttctgaagctgaggctgctggaaggaaaggggctgtccgaacacaaatgggctgtgtactagggaagagggaggttttgcagcttgatcaaagatggaaggagctgggagattgggtcgtgactgaatggaattcaatatggcactcagttggtcacctgcagtgggtaaaacagtcaaaactttgctatttccgagtccataatcaaatccttgggcactgcaacttgcccctttattaaaagcttgcactgagaaagggcttggaggaggagtttgagaattctgatccagaagagcttgttcatcttcatgtcggaggtactggtttccgcctctgtctctagctaaggaccatgcctctccttcatcactctcacagaactctaccatgctgttctgatccagttgcacccatgtcccttcagaattggttacctctcccactgctttgactttgtttcccagaactaacattccaattgggatacctctaaggttagggcagcttctgatgttgtgacctgaaggtcccgtcttcactaccttgtacatgcctggccctcctcgcaagaatggcatatcttgttcttgcattgttgcttcctgtgggcagcaggagtttatgtctttgaaaaagtcatcagtattagttttagattcctgggggaaaaaagctttggaagtccatgaaaatacgtccaaatccctgactccttggctagcattaaagatattgtcaacagggaccagaagactcttgccaagatgttgattaaaagagaggcaccaggcttcagtgtaaccattcatgttagggacatacttctttattgtctcatcattcagcctcagccacacaccatcatcattatggatctcatcaataaaagtgatagttccattgactttcactatgcctatctgctcactctgaagggaagggtggctacggatgcgaagccccgcactgtccttggccacaaattttcgaaccttattaggctgaggttcagactttggtttgaccaactgagttcctggtggtatcatcccttttggtgggtcttttacttttacttccagaccagcatcgatttcaatgccatcaatggtaacatgaagagtgtagagtccaatagcccctggagtccaatttgcacaataagtcccatcattattgacacggatcagcatattctcactgggtctcttaggagttggtgatgcaaaacgtagttcttcaaatgaataattttcataaaccttcatcattgttatggcaatatatcgagcttccttcactatcattggttcatatgaaacatctagctttggtgatgccagccctccataagtcatgtcagtattagaagatgcagctgttactgcaggactgccaggaatcctttgaggtttctttgcttgatcttgttgtaaagacatttttttctgagaaacagggacagctttcacttccaccttcatattgggaacatgtaccacatccccatactggtcttttgtttgaacagttatggtggtaggccaaccacaacgaatatcatccttattcaggatcaaagatgttttctgaggatccgcatatgaatctggctgaagccaccttgcaagccttccaccacttgatcctgggacacaggcaataaaatcatccagaaaagactgttcattgctttggatttggagtggtaaatttccctcaagtgcttctaatatagttggtgaatgagaaagagctagaccctttccaagaattccagaatgggttttgcacacctgcaatgcagcctcctcaagaatttcaaggtcttcttctaattcattaccaataggaagtgctaggtccttcttcatcagagctgctgcacaaaccccaccaagattggctaattctttttccaattggatgactccctcatcaggtccagggctaaattcatatccaattgcaaaacacttaaaaccatagaaagaagctttgtcatctttcacataatctgatgcagtctccaatgaaaaaagggcctcatttcctggcaacaccaaaaccatagtaggccacccagaggatcctgaaaatttctttaattctatccatgaattaagattttcatgaacagatgtcaattttggtccatatcctgaattctgaacagttctgacaggaatcaacaaacgaaggacatcttctgactgtgcagtaccacactgagggtcaaattcgattgtcatccacctcacacattctgggaatgtcaccttgtaatgcatcacacaggcaggtttatacgggtgctcactctctatgacagcatagtgactggaggttgtacaagcagagaggccctgttcaggctggtttcctgtggtgctatctgtcgactgattagggttgaaggcaggcggtgcatacttctgattcaaaatggcaactgacggaagcaattgttggacaaggccaaagacttctacagccaccttgggaatagcagcagctactggtcctatgtaggctataataagggggagcagcatggaaaacagactggaagaactcagcagttctggaatgtcatcagcatccacagcaagagctctgtgcaggaggtccttagaggctcgaacgacagtgcttacaacagacaatgctctgctacagtttttatcttcttcattggctttactcagaagttgggattgtaaatctccatcaaattcactcctatagtagagtatctgtgggatctgtcctctggtttggtttgtgccgttactgctcaagctgcacgtgctgaatgtgaatgtcacaccatcagggcactgaactgtggtcattcctccatctccattggctgtacggcttccatagttcctcaagcgcacagcatatttaacattttcctttaaaggaaccactttgtcaagtctgatctcagctatatcactgggtgagtcatccgttgtgtacgttcctttcactaattccagagatgtccatctgtgggaatgagttgaatctcctgcatgttcactatcatcaaccaacacctctaattcatattcatgaattccacctcctccatagacagagaaaccaaccacaactattccaggtttgtctactgaaaaacagattgcatcaggggacccgttcccagtgttccaacttctgccctgacttgtttttgtaaatcggttagcactagcttttacagagtgaagagaattaagtccatcaacctcagatcccagggctgacgctgtcagttcactgacaatgctggccagtaatccacaggtgttagagacgaggtgggaggagaagagttcattttctctcctcaggctgttcctgactggtagcacaacaatgaccagcattttctccagaacttcacggaagcttgtcatccctgagatattctcttcactctggctgagtttttccatatgtgccaccaaaaggggaaaacgatgaactagtgttgagtcgttctctgtactaacttgtttaacaattgatcgtagtaatacttctccatcatacgcaatcgggaagatggaagtcagcttaacagacgtgtgacacagagctgacataacagctgcaaggagtcggctacttgatgtcttgaagtttgcttcttggatatcctgatccaaacaattcagcagatcacaaaggcaagcccactgtaaggcaggagttgggtagaaagaatgaaagcaggcagtgaaagtattatgacattcctgaaggacagcttctagaagactcaagggttgactgagatatccttgaggatcattatccaatttcaccatgcagtgatcaactccttctgataaaatttttcttaacaaagttctggtttttccaatacactctgctaatttgctagtttcttctacaactgcttttcctgtagctgacactgggtaaatttcacaggtatagacacgcaataacctcagacaacaggtacccacaaagcgcagtctctctaaatctaggagtgtagctgtgaactggaatccttttaatcctctaagttcttcaactcctaagactaaggtggtccagctccagtgaagaatactcaacaatgactcaaaacattccactgagacagttcttgcaaaagacctctttaaaatgtgtacaggttcactggtttgctgtttgccttttgaagcactgccatcactggttggaagtctgtataataactgaggtatctgacccgcattaacatctgtaccattatttgatttctttgaactcttgaactggaaaacaaccccatcatctgtggtaatagatgcctgtccatgagatccacagtcactgctgggtcctgacactcgggcccatgccacataccaccacccagcttgcaggagaacaggctcatcaaacatcattgcatatttttctctagcagcacagtcataagccaatacatcagtctctgcaagaaggtcaccatcagtttcatgatctcctccatcaggacccaattcaaacagcttaattttagcagtatattctcctctacctccaaacagaccaagaccaccaagtaaaatatcagtgtcggcactgaaacgtatagcttctactgaatgggcagaataaccccagcctcctccatgactttcaaacctgtttaccacactataatcttctttagaataaaccttcattactgcttgagtctcttcctctgtacttgcaacacccatttttaagtcctgcatagctgccaaggtatcaagacaacctaaaatgtgcaaagctgcatgagatcgggtagtgagggcccttgatcctgttggtaaggcaagttcaggacttaggatactacatctggactgcatgtctgctgcagagggaagcctggcatcagcaaccaccgcattgtaacaccacagctctctagtatttggtcgaaacctccaaattacatcatatacaggatcaagacacacaccaaatccttgcagatcctcttgttctgagtcattaaaagttttacaactcccatccactttatttatcagaaggcatttaaatggaggaggttctgatatagaagcaggtaccaagcctattatgtgtttactggcaaaaatttctgatgtagcaagtacatgagaattaataagtgcttcatcaattcgtaaaaaagtttggtccccacttgcacctatccaagtagcttttcttccatattttgatccaatgttaggcatgggagctggctttgcattccaatatggcacatccaaaattggtctgcccagttgtcctttagaaaaacttccaaatgtgaagacctgtccatccattaaaagtactgccgtatggttgctgcctgcagtgacttgtgtgctagggcctggcaatgcttgaacaagagtgggacatcccctggagttgacatctccatgtcctagctgcccatgctgcccataaccaaatgtatagacatctccattttccattaaaaccactgaatggtgaaatccacagctgacttggactgcccggagctcacagtcaaatcgcacagagcctggagggtatgttgtgattttgcttgcatccttttcgcctctttctccacttccatctcttccttcctctaatctgtgccttctgattacacgttgccgtttttcttcttgtcgtaactgaaggtgttcttcaatgttaaccccgggcactgggacagctaaaagaagatctaaaggtatcatttctttcactgcatcaagaattcctctttgtcttgcctcttgaccatctaactctcttgcacaggccttgcaacatccacacacagcacaaccagattctccggaaccacaaccacagatccctccggggactctgtctggccgtccactactgacacagctggctccataacctgtacagtctccacagacagtgcaaaccatgcactgctccagcttccatttgtgcatgcctggagggcacatcatagacttctcatctttttcatctagttcttcttccaggtcttcatccattgctgttgccatattttcaactccaaaccctttcccaccttggttcatggcaccagtatctcgtccacactgtcctttattatttacaccaaatgtccacacctctccattcttcattaaaacacaagtgtgagctttgcccatagctacctgagttacaaaatggcccttcaaatcagttaccaaacttgaactatcagagtaaatggcatcttttccaaacatgtagagttctccatctttagaaataacagaactacttccattattgcaggctgtatataccacaatctttccttccatcttaattatctttttaggtttataaggtttggattgccgtctgctcttagttgattctccatcttctcctttactagcagatcctgtaaagaatatgctcccatcttctgcaactaaaagggcgtgagagccatcgtgtccaactgagaagtgtactatctttggagattttgtaattggtagctcaacccattttcctgctgaaggaccaccttgtttgattccaagactctggtatttgccagtgtaatatatctttccatttgctgttttcattagcgcaaactctcgtcctgcaccaagaattgctgactcctcatcaaatcctgtacttataatatgcaagtccttttccagatcgaatagtgagataccacaggcatgtaagcattttctagccagtttaagttgcaattcttgctgtagaacaggttcagtgcttgtggcaaatattctgacaacaaagccatcatctcttgaagcagctatctgattaatatattctccatcagtgaataaaatattttgaccttcagtgtggcaatctggtaacatcacagtaccatcttgctccagtgtttcagggcttatccttatggctgtcatgctgtggttattcacatctctatataataaataaccctgagcataccctaaccaagactttttttcttttctgtttctaatacgggatgtagaattgtatatatggcccctaactgttccactgtatccagagcctattttatataatccatccttgcataatagataaagaaaaaatccatcattctgaagtagacattggtcatcttcatcaacagatatttcttttaatggccacttgtgcattaaagctgctttcttaatgccattactaaaccagtcctgaatttgaatttttcccaccaaaactgcttgtacacttctctgtagcgaatttagaattgttggcacctgaatagtttggcaagcatggcttccattgttggtgaggatagcagagatggcctgaagtgtccttcctgtttctccccaagaagccaccagactaaagaggcaagcacaggaaagtgctgttaaggactgtcctgtgctgtcattcatcccagtacttcgaacggtgatttccaaaagaagctggaagagagactctaggacctcaggtggctcagactggaggccttctggctgctggccctgcagcacgttgagcagggcttggagactcctgagacacagggatggatgagaaaatcgtgtctctttgatcaattcaaaaacttcacaaaggccaacctcaataatctttggaagcttgatagggggctctttggattcctcttcttcatcactatctgattctccactctgcacagagttcttagatgcggctgccaatgatatttcctttttctgccattccagaacgcaatggcgtacattacagtaaatattgaaagcagaaggattgctatgtagtttgatatctggtatgattactgtattctctaagttttcagacttgcttcttgtcttcacttttgatttgctcttctgttttcttttcaatttcttcttatttaaaattttcttattcctggaggctgggtgtccagcgctgccgcccccctggtccctgtcattgagcgcagcggtataaatcctccggtagcggtcggccagggcccggcctgacagcagcagctggtagtgaccccgggagtccgcggcgggtagccccagccccagccccgcagcagccacggagccgtcgggaaccggcatgaacagcgcccccggcgccggggaggaagagaaggtggcggctgggtagaatccgtccccgccgagccccgaggaggcggcggcgggggaggcagtcgctgcgcacatcatcatcctcgccgccgccgccgccgccgccgcctcgtccccgcgggccgggcgggcagacacgcgcgcgcacacacagcccttttccaacgacgacggctccggcggcggcctctggctcccgcagcagggagactacaaagacagcgacctccttctcctcctccttcttctcctcctcccccccgcgccgccctcgccgctactggggccgctcatctaaccccgccaccccgggaatgtgaggaggaggcggtgccgccactgccgccgccaccaccgctaccaccgccaccaccgccggggctacccgcaatgggaagctgccg

SEQ ID NO: 17088 - RNA, 8807 nt, Homo sapiens
  source 1..8807: mol_type = other RNA
tcaaaactgaggggcattttcttcttgcggagggtatctggatcaagtgtgtaagagtctgatttagaacgttcccgaggaggatcaagctttgtcttaacaggagcagtacttttttgaggtagatttttatcatgtggtgaggaggagcgtggagaactagcacccgatgggctagacctattggctgggagagtctttggcttaggagatgacaaccgagaacctggtcctggggattcagctctggagctagaaggcatcctcccatcagatttcaatgtctgcaaggtgttatggttgggggataatgacctactgtgggaatctgacctcaactttgcagcatcagattttaagatgagggattcactagcagataaactttctgtgccccttggcttcttctgatcagcagtagtccggctcatacgtccatcaggtttaagcgatctgctgtgtttagaggacagctctgattttcctgatgtagaggctggtttagaagatgttgagatgtttcctcgatcacccttcagtttgtgagacagagatgagagagcagaggcaggcccagctacaccataatttttgtaaatgcgctcacgagaagcaaggttgcgagatggagatttctgaagctgaggctgctggaaggaaaggggctgtccgaacacaaatgggctgtgtactagggaagagggaggttttgcagcttgatcaaagatggaaggagctgggagattgggtcgtgactgaatggaattcaatatggcactcagttggtcacctgcagtgggtaaaacagtcaaaactttgctatttccgagtccataatcaaatccttgggcactgcaacttgcccctttattaaaagcttgcactgagaaagggcttggaggaggagtttgagaattctgatccagaagagcttgttcatcttcatgtcggaggtactggtttccgcctctgtctctagctaaggaccatgcctctccttcatcactctcacagaactctaccatgctgttctgatccagttgcacccatgtcccttcagaattggttacctctcccactgctttgactttgtttcccagaactaacattccaattgggatacctctaaggttagggcagcttctgatgttgtgacctgaaggtcccgtcttcactaccttgtacatgcctggccctcctcgcaagaatggcatatcttgttcttgcattgttgcttcctgtgggcagcaggagtttatgtctttgaaaaagtcatcagtattagttttagattcctgggggaaaaaagctttggaagtccatgaaaatacgtccaaatccctgactccttggctagcattaaagatattgtcaacagggaccagaagactcttgccaagatgttgattaaaagagaggcaccaggcttcagtgtaaccattcatgttagggacatacttctttattgtctcatcattcagcctcagccacacaccatcatcattatggatctcatcaataaaagtgatagttccattgactttcactatgcctatctgctcactctgaagggaagggtggctacggatgcgaagccccgcactgtccttggccacaaattttcgaaccttattaggctgaggttcagactttggtttgaccaactgagttcctggtggtatcatcccttttggtgggtcttttacttttacttccagaccagcatcgatttcaatgccatcaatggtaacatgaagagtgtagagtccaatagcccctggagtccaatttgcacaataagtcccatcattattgacacggatcagcatattctcactgggtctcttaggagttggtgatgcaaaacgtagttcttcaaatgaataattttcataaaccttcatcattgttatggcaatatatcgagcttccttcactatcattggttcatatgaaacatctagctttggtgatgccagccctccataagtcatgtcagtattagaagatgcagctgttactgcaggactgccaggaatcctttgaggtttctttgcttgatcttgttgtaaagacatttttttctgagaaacagggacagctttcacttccaccttcatattgggaacatgtaccacatccccatactggtcttttgtttgaacagttatggtggtaggccaaccacaacgaatatcatccttattcaggatcaaagatgttttctgaggatccgcatatgaatctggctgaagccaccttgcaagccttccaccacttgatcctgggacacaggcaataaaatcatccagaaaagactgttcattgctttggatttggagtggtaaatttccctcaagtgcttctaatatagttggtgaatgagaaagagctagaccctttccaagaattccagaatgggttttgcacacctgcaatgcagcctcctcaagaatttcaaggtcttcttctaattcattaccaataggaagtgctaggtccttcttcatcagagctgctgcacaaaccccaccaagattggctaattctttttccaattggatgactccctcatcaggtccagggctaaattcatatccaattgcaaaacacttaaaaccatagaaagaagctttgtcatctttcacataatctgatgcagtctccaatgaaaaaagggcctcatttcctggcaacaccaaaaccatagtaggccacccagaggatcctgaaaatttctttaattctatccatgaattaagattttcatgaacagatgtcaattttggtccatatcctgaattctgaacagttctgacaggaatcaacaaacgaaggacatcttctgactgtgcagtaccacactgagggtcaaattcgattgtcatccacctcacacattctgggaatgtcaccttgtaatgcatcacacaggcaggtttatacgggtgctcactctctatgacagcatagtgactggaggttgtacaagcagagaggccctgttcaggctggtttcctgtggtgctatctgtcgactgattagggttgaaggcaggcggtgcatacttctgattcaaaatggcaactgacggaagcaattgttggacaaggccaaagacttctacagccaccttgggaatagcagcagctactggtcctatgtaggctataataagggggagcagcatggaaaacagactggaagaactcagcagttctggaatgtcatcagcatccacagcaagagctctgtgcaggaggtccttagaggctcgaacgacagtgcttacaacagacaatgctctgctacagtttttatcttcttcattggctttactcagaagttgggattgtaaatctccatcaaattcactcctatagtagagtatctgtgggatctgtcctctggtttggtttgtgccgttactgctcaagctgcacgtgctgaatgtgaatgtcacaccatcagggcactgaactgtggtcattcctccatctccattggctgtacggcttccatagttcctcaagcgcacagcatatttaacattttcctttaaaggaaccactttgtcaagtctgatctcagctatatcactgggtgagtcatccgttgtgtacgttcctttcactaattccagagatgtccatctgtgggaatgagttgaatctcctgcatgttcactatcatcaaccaacacctctaattcatattcatgaattccacctcctccatagacagagaaaccaaccacaactattccaggtttgtctactgaaaaacagattgcatcaggggacccgttcccagtgttccaacttctgccctgacttgtttttgtaaatcggttagcactagcttttacagagtgaagagaattaagtccatcaacctcagatcccagggctgacgctgtcagttcactgacaatgctggccagtaatccacaggtgttagagacgaggtgggaggagaagagttcattttctctcctcaggctgttcctgactggtagcacaacaatgaccagcattttctccagaacttcacggaagcttgtcatccctgagatattctcttcactctggctgagtttttccatatgtgccaccaaaaggggaaaacgatgaactagtgttgagtcgttctctgtactaacttgtttaacaattgatcgtagtaatacttctccatcatacgcaatcgggaagatggaagtcagcttaacagacgtgtgacacagagctgacataacagctgcaaggagtcggctacttgatgtcttgaagtttgcttcttggatatcctgatccaaacaattcagcagatcacaaaggcaagcccactgtaaggcaggagttgggtagaaagaatgaaagcaggcagtgaaagtattatgacattcctgaaggacagcttctagaagactcaagggttgactgagatatccttgaggatcattatccaatttcaccatgcagtgatcaactccttctgataaaatttttcttaacaaagttctggtttttccaatacactctgctaatttgctagtttcttctacaactgcttttcctgtagctgacactgggtaaatttcacaggtatagacacgcaataacctcagacaacaggtacccacaaagcgcagtctctctaaatctaggagtgtagctgtgaactggaatccttttaatcctctaagttcttcaactcctaagactaaggtggtccagctccagtgaagaatactcaacaatgactcaaaacattccactgagacagttcttgcaaaagacctctttaaaatgtgtacaggttcactggtttgctgtttgccttttgaagcactgccatcactggttggaagtctgtataataactgaggtatctgacccgcattaacatctgtaccattatttgatttctttgaactcttgaactggaaaacaaccccatcatctgtggtaatagatgcctgtccatgagatccacagtcactgctgggtcctgacactcgggcccatgccacataccaccacccagcttgcaggagaacaggctcatcaaacatcattgcatatttttctctagcagcacagtcataagccaatacatcagtctctgcaagaaggtcaccatcagtttcatgatctcctccatcaggacccaattcaaacagcttaattttagcagtatattctcctctacctccaaacagaccaagaccaccaagtaaaatatcagtgtcggcactgaaacgtatagcttctactgaatgggcagaataaccccagcctcctccatgactttcaaacctgtttaccacactataatcttctttagaataaaccttcattactgcttgagtctcttcctctgtacttgcaacacccatttttaagtcctgcatagctgccaaggtatcaagacaacctaaaatgtgcaaagctgcatgagatcgggtagtgagggcccttgatcctgttggtaaggcaagttcaggacttaggatactacatctggactgcatgtctgctgcagagggaagcctggcatcagcaaccaccgcattgtaacaccacagctctctagtatttggtcgaaacctccaaattacatcatatacaggatcaagacacacaccaaatccttgcagatcctcttgttctgagtcattaaaagttttacaactcccatccactttatttatcagaaggcatttaaatggaggaggttctgatatagaagcaggtaccaagcctattatgtgtttactggcaaaaatttctgatgtagcaagtacatgagaattaataagtgcttcatcaattcgtaaaaaagtttggtccccacttgcacctatccaagtagcttttcttccatattttgatccaatgttaggcatgggagctggctttgcattccaatatggcacatccaaaattggtctgcccagttgtcctttagaaaaacttccaaatgtgaagacctgtccatccattaaaagtactgccgtatggttgctgcctgcagtgacttgtgtgctagggcctggcaatgcttgaacaagagtgggacatcccctggagttgacatctccatgtcctagctgcccatgctgcccataaccaaatgtatagacatctccattttccattaaaaccactgaatggtgaaatccacagctgacttggactgcccggagctcacagtcaaatcgcacagagcctggagggtatgttgtgattttgcttgcatccttttcgcctctttctccacttccatctttgtgcttgtcccgtttatgctttagctgtgctggatgggatctgagtctggctagagcctgttctcgatggttcataaaaataggaccagcaaatacaagggggcctcttccttcctctaatctgtgccttctgattacacgttgccgtttttcttcttgtcgtaactgaaggtgttcttcaatgttaaccccgggcactgggacagctaaaagaagatctaaaggtatcatttctttcactgcatcaagaattcctctttgtcttgcctcttgaccatctaactctcttgcacaggccttgcaacatccacacacagcacaaccagattctccggaaccacaaccacagatccctccggggactctgtctggccgtccactactgacacagctggctccataacctgtacagtctccacagacagtgcaaaccatgcactgctccagcttccatttgtgcatgcctggagggcacatcatagacttctcatctttttcatctagttcttcttccaggtcttcatccattgctgttgccatattttcaactccaaaccctttcccaccttggttcatggcaccagtatctcgtccacactgtcctttattatttacaccaaatgtccacacctctccattcttcattaaaacacaagtgtgagctttgcccatagctacctgagttacaaaatggcccttcaaatcagttaccaaacttgaactatcagagtaaatggcatcttttccaaacatgtagagttctccatctttagaaataacagaactacttccattattgcaggctgtatataccacaatctttccttccatcttaattatctttttaggtttataaggtttggattgccgtctgctcttagttgattctccatcttctcctttactagcagatcctgtaaagaatatgctcccatcttctgcaactaaaagggcgtgagagccatcgtgtccaactgagaagtgtactatctttggagattttgtaattggtagctcaacccattttcctgctgaaggaccaccttgtttgattccaagactctggtatttgccagtgtaatatatctttccatttgctgttttcattagcgcaaactctcgtcctgcaccaagaattgctgactcctcatcaaatcctgtacttataatatgcaagtccttttccagatcgaatagtgagataccacaggcatgtaagcattttctagccagtttaagttgcaattcttgctgtagaacaggttcagtgcttgtggcaaatattctgacaacaaagccatcatctcttgaagcagctatctgattaatatattctccatcagtgaataaaatattttgaccttcagtgtggcaatctggtaacatcacagtaccatcttgctccagtgtttcagggcttatccttatggctgtcatgctgtggttattcacatctctatataataaataaccctgagcataccctaaccaagactttttttcttttctgtttctaatacgggatgtagaattgtatatatggcccctaactgttccactgtatccagagcctattttatataatccatccttgcataatagataaagaaaaaatccatcattctgaagtagacattggtcatcttcatcaacagatatttcttttaatggccacttgtgcattaaagctgctttcttaatgccattactaaaccagtcctgaatttgaatttttcccaccaaaactgcttgtacacttctctgtagcgaatttagaattgttggcacctgaatagtttggcaagcatggcttccattgttggtgaggatagcagagatggcctgaagtgtccttcctgtttctccccaagaagccaccagactaaagaggcaagcacaggaaagtgctgttaaggactgtcctgtgctgtcattcatcccagtacttcgaacggtgatttccaaaagaagctggaagagagactctaggacctcaggtggctcagactggaggccttctggctgctggccctgcagcacgttgagcagggcttggagactcctgagacacagggatggatgagaaaatcgtgtctctttgatcaattcaaaaacttcacaaaggccaacctcaataatctttggaagcttgatagggggctctttggattcctcttcttcatcactatctgattctccactctgcacagagttcttagatgcggctgccaatgatatttcctttttctgccattccagaacgcaatggcgtacattacagtaaatattgaaagcagaaggattgctatgtagtttgatatctggtatgattactgtattctctaagttttcagactgtggctataaaggatatcacagagaatccttgtgatggaactgctgtatatccagactgtggtaagagtcacatggacctacacatgtgataaaattacacagacttaggtgcacacaaacacatacacactgcattcatactgaaatcatctc

SEQ ID NO: 17089 - RNA, 9352 nt, Homo sapiens
  source 1..9352: mol_type = other RNA
tcaaaactgaggggcattttcttcttgcggagggtatctggatcaagtgtgtaagagtctgatttagaacgttcccgaggaggatcaagctttgtcttaacaggagcagtacttttttgaggtagatttttatcatgtggtgaggaggagcgtggagaactagcacccgatgggctagacctattggctgggagagtctttggcttaggagatgacaaccgagaacctggtcctggggattcagctctggagctagaaggcatcctcccatcagatttcaatgtctgcaaggtgttatggttgggggataatgacctactgtgggaatctgacctcaactttgcagcatcagattttaagatgagggattcactagcagataaactttctgtgccccttggcttcttctgatcagcagtagtccggctcatacgtccatcaggtttaagcgatctgctgtgtttagaggacagctctgattttcctgatgtagaggctggtttagaagatgttgagatgtttcctcgatcacccttcagtttgtgagacagagatgagagagcagaggcaggcccagctacaccataatttttgtaaatgcgctcacgagaagcaaggttgcgagatggagatttctgaagctgaggctgctggaaggaaaggggctgtccgaacacaaatgggctgtgtactagggaagagggaggttttgcagcttgatcaaagatggaaggagctgggagattgggtcgtgactgaatggaattcaatatggcactcagttggtcacctgcagtgggtaaaacagtcaaaactttgctatttccgagtccataatcaaatccttgggcactgcaacttgcccctttattaaaagcttgcactgagaaagggcttggaggaggagtttgagaattctgatccagaagagcttgttcatcttcatgtcggaggtactggtttccgcctctgtctctagctaaggaccatgcctctccttcatcactctcacagaactctaccatgctgttctgatccagttgcacccatgtcccttcagaattggttacctctcccactgctttgactttgtttcccagaactaacattccaattgggatacctctaaggttagggcagcttctgatgttgtgacctgaaggtcccgtcttcactaccttgtacatgcctggccctcctcgcaagaatggcatatcttgttcttgcattgttgcttcctgtgggcagcaggagtttatgtctttgaaaaagtcatcagtattagttttagattcctgggggaaaaaagctttggaagtccatgaaaatacgtccaaatccctgactccttggctagcattaaagatattgtcaacagggaccagaagactcttgccaagatgttgattaaaagagaggcaccaggcttcagtgtaaccattcatgttagggacatacttctttattgtctcatcattcagcctcagccacacaccatcatcattatggatctcatcaataaaagtgatagttccattgactttcactatgcctatctgctcactctgaagggaagggtggctacggatgcgaagccccgcactgtccttggccacaaattttcgaaccttattaggctgaggttcagactttggtttgaccaactgagttcctggtggtatcatcccttttggtgggtcttttacttttacttccagaccagcatcgatttcaatgccatcaatggtaacatgaagagtgtagagtccaatagcccctggagtccaatttgcacaataagtcccatcattattgacacggatcagcatattctcactgggtctcttaggagttggtgatgcaaaacgtagttcttcaaatgaataattttcataaaccttcatcattgttatggcaatatatcgagcttccttcactatcattggttcatatgaaacatctagctttggtgatgccagccctccataagtcatgtcagtattagaagatgcagctgttactgcaggactgccaggaatcctttgaggtttctttgcttgatcttgttgtaaagacatttttttctgagaaacagggacagctttcacttccaccttcatattgggaacatgtaccacatccccatactggtcttttgtttgaacagttatggtggtaggccaaccacaacgaatatcatccttattcaggatcaaagatgttttctgaggatccgcatatgaatctggctgaagccaccttgcaagccttccaccacttgatcctgggacacaggcaataaaatcatccagaaaagactgttcattgctttggatttggagtggtaaatttccctcaagtgcttctaatatagttggtgaatgagaaagagctagaccctttccaagaattccagaatgggttttgcacacctgcaatgcagcctcctcaagaatttcaaggtcttcttctaattcattaccaataggaagtgctaggtccttcttcatcagagctgctgcacaaaccccaccaagattggctaattctttttccaattggatgactccctcatcaggtccagggctaaattcatatccaattgcaaaacacttaaaaccatagaaagaagctttgtcatctttcacataatctgatgcagtctccaatgaaaaaagggcctcatttcctggcaacaccaaaaccatagtaggccacccagaggatcctgaaaatttctttaattctatccatgaattaagattttcatgaacagatgtcaattttggtccatatcctgaattctgaacagttctgacaggaatcaacaaacgaaggacatcttctgactgtgcagtaccacactgagggtcaaattcgattgtcatccacctcacacattctgggaatgtcaccttgtaatgcatcacacaggcaggtttatacgggtgctcactctctatgacagcatagtgactggaggttgtacaagcagagaggccctgttcaggctggtttcctgtggtgctatctgtcgactgattagggttgaaggcaggcggtgcatacttctgattcaaaatggcaactgacggaagcaattgttggacaaggccaaagacttctacagccaccttgggaatagcagcagctactggtcctatgtaggctataataagggggagcagcatggaaaacagactggaagaactcagcagttctggaatgtcatcagcatccacagcaagagctctgtgcaggaggtccttagaggctcgaacgacagtgcttacaacagacaatgctctgctacagtttttatcttcttcattggctttactcagaagttgggattgtaaatctccatcaaattcactcctatagtagagtatctgtgggatctgtcctctggtttggtttgtgccgttactgctcaagctgcacgtgctgaatgtgaatgtcacaccatcagggcactgaactgtggtcattcctccatctccattggctgtacggcttccatagttcctcaagcgcacagcatatttaacattttcctttaaaggaaccactttgtcaagtctgatctcagctatatcactgggtgagtcatccgttgtgtacgttcctttcactaattccagagatgtccatctgtgggaatgagttgaatctcctgcatgttcactatcatcaaccaacacctctaattcatattcatgaattccacctcctccatagacagagaaaccaaccacaactattccaggtttgtctactgaaaaacagattgcatcaggggacccgttcccagtgttccaacttctgccctgacttgtttttgtaaatcggttagcactagcttttacagagtgaagagaattaagtccatcaacctcagatcccagggctgacgctgtcagttcactgacaatgctggccagtaatccacaggtgttagagacgaggtgggaggagaagagttcattttctctcctcaggctgttcctgactggtagcacaacaatgaccagcattttctccagaacttcacggaagcttgtcatccctgagatattctcttcactctggctgagtttttccatatgtgccaccaaaaggggaaaacgatgaactagtgttgagtcgttctctgtactaacttgtttaacaattgatcgtagtaatacttctccatcatacgcaatcgggaagatggaagtcagcttaacagacgtgtgacacagagctgacataacagctgcaaggagtcggctacttgatgtcttgaagtttgcttcttggatatcctgatccaaacaattcagcagatcacaaaggcaagcccactgtaaggcaggagttgggtagaaagaatgaaagcaggcagtgaaagtattatgacattcctgaaggacagcttctagaagactcaagggttgactgagatatccttgaggatcattatccaatttcaccatgcagtgatcaactccttctgataaaatttttcttaacaaagttctggtttttccaatacactctgctaatttgctagtttcttctacaactgcttttcctgtagctgacactgggtaaatttcacaggtatagacacgcaataacctcagacaacaggtacccacaaagcgcagtctctctaaatctaggagtgtagctgtgaactggaatccttttaatcctctaagttcttcaactcctaagactaaggtggtccagctccagtgaagaatactcaacaatgactcaaaacattccactgagacagttcttgcaaaagacctctttaaaatgtgtacaggttcactggtttgctgtttgccttttgaagcactgccatcactggttggaagtctgtataataactgaggtatctgacccgcattaacatctgtaccattatttgatttctttgaactcttgaactggaaaacaaccccatcatctgtggtaatagatgcctgtccatgagatccacagtcactgctgggtcctgacactcgggcccatgccacataccaccacccagcttgcaggagaacaggctcatcaaacatcattgcatatttttctctagcagcacagtcataagccaatacatcagtctctgcaagaaggtcaccatcagtttcatgatctcctccatcaggacccaattcaaacagcttaattttagcagtatattctcctctacctccaaacagaccaagaccaccaagtaaaatatcagtgtcggcactgaaacgtatagcttctactgaatgggcagaataaccccagcctcctccatgactttcaaacctgtttaccacactataatcttctttagaataaaccttcattactgcttgagtctcttcctctgtacttgcaacacccatttttaagtcctgcatagctgccaaggtatcaagacaacctaaaatgtgcaaagctgcatgagatcgggtagtgagggcccttgatcctgttggtaaggcaagttcaggacttaggatactacatctggactgcatgtctgctgcagagggaagcctggcatcagcaaccaccgcattgtaacaccacagctctctagtatttggtcgaaacctccaaattacatcatatacaggatcaagacacacaccaaatccttgcagatcctcttgttctgagtcattaaaagttttacaactcccatccactttatttatcagaaggcatttaaatggaggaggttctgatatagaagcaggtaccaagcctattatgtgtttactggcaaaaatttctgatgtagcaagtacatgagaattaataagtgcttcatcaattcgtaaaaaagtttggtccccacttgcacctatccaagtagcttttcttccatattttgatccaatgttaggcatgggagctggctttgcattccaatatggcacatccaaaattggtctgcccagttgtcctttagaaaaacttccaaatgtgaagacctgtccatccattaaaagtactgccgtatggttgctgcctgcagtgacttgtgtgctagggcctggcaatgcttgaacaagagtgggacatcccctggagttgacatctccatgtcctagctgcccatgctgcccataaccaaatgtatagacatctccattttccattaaaaccactgaatggtgaaatccacagctgacttggactgcccggagctcacagtcaaatcgcacagagcctggagggtatgttgtgattttgcttgcatccttttcgcctctttctccacttccatctttgtgcttgtcccgtttatgctttagctgtgctggatgggatctgagtctggctagagcctgttctcgatggttcataaaaataggaccagcaaatacaagggggcctcttccttcctctaatctgtgccttctgattacacgttgccgtttttcttcttgtcgtaactgaaggtgttcttcaatgttaaccccgggcactgggacagctaaaagaagatctaaaggtatcatttctttcactgcatcaagaattcctctttgtcttgcctcttgaccatctaactctcttgcacaggccttgcaacatccacacacagcacaaccagattctccggaaccacaaccacagatccctccggggactctgtctggccgtccactactgacacagctggctccataacctgtacagtctccacagacagtgcaaaccatgcactgctccagcttccatttgtgcatgcctggagggcacatcatagacttctcatctttttcatctagttcttcttccaggtcttcatccattgctgttgccatattttcaactccaaaccctttcccaccttggttcatggcaccagtatctcgtccacactgtcctttattatttacaccaaatgtccacacctctccattcttcattaaaacacaagtgtgagctttgcccatagctacctgagttacaaaatggcccttcaaatcagttaccaaacttgaactatcagagtaaatggcatcttttccaaacatgtagagttctccatctttagaaataacagaactacttccattattgcaggctgtatataccacaatctttccttccatcttaattatctttttaggtttataaggtttggattgccgtctgctcttagttgattctccatcttctcctttactagcagatcctgtaaagaatatgctcccatcttctgcaactaaaagggcgtgagagccatcgtgtccaactgagaagtgtactatctttggagattttgtaattggtagctcaacccattttcctgctgaaggaccaccttgtttgattccaagactctggtatttgccagtgtaatatatctttccatttgctgttttcattagcgcaaactctcgtcctgcaccaagaattgctgactcctcatcaaatcctgtacttataatatgcaagtccttttccagatcgaatagtgagataccacaggcatgtaagcattttctagccagtttaagttgcaattcttgctgtagaacaggttcagtgcttgtggcaaatattctgacaacaaagccatcatctcttgaagcagctatctgattaatatattctccatcagtgaataaaatattttgaccttcagtgtggcaatctggtaacatcacagtaccatcttgctccagtgtttcagggcttatccttatggctgtcatgctgtggttattcacatctctatataataaataaccctgagcataccctaaccaagactttttttcttttctgtttctaatacgggatgtagaattgtatatatggcccctaactgttccactgtatccagagcctattttatataatccatccttgcataatagataaagaaaaaatccatcattctgaagtagacattggtcatcttcatcaacagatatttcttttaatggccacttgtgcattaaagctgctttcttaatgccattactaaaccagtcctgaatttgaatttttcccaccaaaactgcttgtacacttctctgtagcgaatttagaattgttggcacctgaatagtttggcaagcatggcttccattgttggtgaggatagcagagatggcctgaagtgtccttcctgtttctccccaagaagccaccagactaaagaggcaagcacaggaaagtgctgttaaggactgtcctgtgctgtcattcatcccagtacttcgaacggtgatttccaaaagaagctggaagagagactctaggacctcaggtggctcagactggaggccttctggctgctggccctgcagcacgttgagcagggcttggagactcctgagacacagggatggatgagaaaatcgtgtctctttgatcaattcaaaaacttcacaaaggccaacctcaataatctttggaagcttgatagggggctctttggattcctcttcttcatcactatctgattctccactctgcacagagttcttagatgcggctgccaatgatatttcctttttctgccattccagaacgcaatggcgtacattacagtaaatattgaaagcagaaggattgctatgtagtttgatatctggtatgattactgtattctctaagttttcagacttgcttcttgtcttcacttttgatttgctcttctgttttcttttcaatttcttcttatttaaaattttcttattcctggaggctgggtgtccagcgctgccgcccccctggtccctgtcattgagcgcagcggtataaatcctccggtagcggtcggccagggcccggcctgacagcagcagctggtagtgaccccgggagtccgcggcgggtagccccagccccagccccgcagcagccacggagccgtcgggaaccggcatgaacagcgcccccggcgccggggaggaagagaaggtggcggctgggtagaatccgtccccgccgagccccgaggaggcggcggcgggggaggcagtcgctgcgcacatcatcatcctcgccgccgccgccgccgccgccgcctcgtccccgcgggccgggcgggcagacacgcgcgcgcacacacagcccttttccaacgacgacggctccggcggcggcctctggctcccgcagcagggagactacaaagacagcgacctccttctcctcctccttcttctcctcctcccccccgcgccgccctcgccgctactggggccgctcatctaaccccgccaccccgggaatgtgaggaggaggcggtgccgccactgccgccgccaccaccgctaccaccgccaccaccgccggggctacccgcaatgggaagctgccg

SEQ ID NO: 17090 - RNA, 8859 nt, Homo sapiens
  source 1..8859: mol_type = other RNA
tcaaaactgaggggcattttcttcttgcggagggtatctggatcaagtgtgtaagagtctgatttagaacgttcccgaggaggatcaagctttgtcttaacaggagcagtacttttttgaggtagatttttatcatgtggtgaggaggagcgtggagaactagcacccgatgggctagacctattggctgggagagtctttggcttaggagatgacaaccgagaacctggtcctggggattcagctctggagctagaaggcatcctcccatcagatttcaatgtctgcaaggtgttatggttgggggataatgacctactgtgggaatctgacctcaactttgcagcatcagattttaagatgagggattcactagcagataaactttctgtgccccttggcttcttctgatcagcagtagtccggctcatacgtccatcaggtttaagcgatctgctgtgtttagaggacagctctgattttcctgatgtagaggctggtttagaagatgttgagatgtttcctcgatcacccttcagtttgtgagacagagatgagagagcagaggcaggcccagctacaccataatttttgtaaatgcgctcacgagaagcaaggttgcgagatggagatttctgaagctgaggctgctggaaggaaaggggctgtccgaacacaaatgggctgtgtactagggaagagggaggttttgcagcttgatcaaagatggaaggagctgggagattgggtcgtgactgaatggaattcaatatggcactcagttggtcacctgcagtgggtaaaacagtcaaaactttgctatttccgagtccataatcaaatccttgggcactgcaacttgcccctttattaaaagcttgcactgagaaagggcttggaggaggagtttgagaattctgatccagaagagcttgttcatcttcatgtcggaggtactggtttccgcctctgtctctagctaaggaccatgcctctccttcatcactctcacagaactctaccatgctgttctgatccagttgcacccatgtcccttcagaattggttacctctcccactgctttgactttgtttcccagaactaacattccaattgggatacctctaaggttagggcagcttctgatgttgtgacctgaaggtcccgtcttcactaccttgtacatgcctggccctcctcgcaagaatggcatatcttgttcttgcattgttgcttcctgtgggcagcaggagtttatgtctttgaaaaagtcatcagtattagttttagattcctgggggaaaaaagctttggaagtccatgaaaatacgtccaaatccctgactccttggctagcattaaagatattgtcaacagggaccagaagactcttgccaagatgttgattaaaagagaggcaccaggcttcagtgtaaccattcatgttagggacatacttctttattgtctcatcattcagcctcagccacacaccatcatcattatggatctcatcaataaaagtgatagttccattgactttcactatgcctatctgctcactctgaagggaagggtggctacggatgcgaagccccgcactgtccttggccacaaattttcgaaccttattaggctgaggttcagactttggtttgaccaactgagttcctggtggtatcatcccttttggtgggtcttttacttttacttccagaccagcatcgatttcaatgccatcaatggtaacatgaagagtgtagagtccaatagcccctggagtccaatttgcacaataagtcccatcattattgacacggatcagcatattctcactgggtctcttaggagttggtgatgcaaaacgtagttcttcaaatgaataattttcataaaccttcatcattgttatggcaatatatcgagcttccttcactatcattggttcatatgaaacatctagctttggtgatgccagccctccataagtcatgtcagtattagaagatgcagctgttactgcaggactgccaggaatcctttgaggtttctttgcttgatcttgttgtaaagacatttttttctgagaaacagggacagctttcacttccaccttcatattgggaacatgtaccacatccccatactggtcttttgtttgaacagttatggtggtaggccaaccacaacgaatatcatccttattcaggatcaaagatgttttctgaggatccgcatatgaatctggctgaagccaccttgcaagccttccaccacttgatcctgggacacaggcaataaaatcatccagaaaagactgttcattgctttggatttggagtggtaaatttccctcaagtgcttctaatatagttggtgaatgagaaagagctagaccctttccaagaattccagaatgggttttgcacacctgcaatgcagcctcctcaagaatttcaaggtcttcttctaattcattaccaataggaagtgctaggtccttcttcatcagagctgctgcacaaaccccaccaagattggctaattctttttccaattggatgactccctcatcaggtccagggctaaattcatatccaattgcaaaacacttaaaaccatagaaagaagctttgtcatctttcacataatctgatgcagtctccaatgaaaaaagggcctcatttcctggcaacaccaaaaccatagtaggccacccagaggatcctgaaaatttctttaattctatccatgaattaagattttcatgaacagatgtcaattttggtccatatcctgaattctgaacagttctgacaggaatcaacaaacgaaggacatcttctgactgtgcagtaccacactgagggtcaaattcgattgtcatccacctcacacattctgggaatgtcaccttgtaatgcatcacacaggcaggtttatacgggtgctcactctctatgacagcatagtgactggaggttgtacaagcagagaggccctgttcaggctggtttcctgtggtgctatctgtcgactgattagggttgaaggcaggcggtgcatacttctgattcaaaatggcaactgacggaagcaattgttggacaaggccaaagacttctacagccaccttgggaatagcagcagctactggtcctatgtaggctataataagggggagcagcatggaaaacagactggaagaactcagcagttctggaatgtcatcagcatccacagcaagagctctgtgcaggaggtccttagaggctcgaacgacagtgcttacaacagacaatgctctgctacagtttttatcttcttcattggctttactcagaagttgggattgtaaatctccatcaaattcactcctatagtagagtatctgtgggatctgtcctctggtttggtttgtgccgttactgctcaagctgcacgtgctgaatgtgaatgtcacaccatcagggcactgaactgtggtcattcctccatctccattggctgtacggcttccatagttcctcaagcgcacagcatatttaacattttcctttaaaggaaccactttgtcaagtctgatctcagctatatcactgggtgagtcatccgttgtgtacgttcctttcactaattccagagatgtccatctgtgggaatgagttgaatctcctgcatgttcactatcatcaaccaacacctctaattcatattcatgaattccacctcctccatagacagagaaaccaaccacaactattccaggtttgtctactgaaaaacagattgcatcaggggacccgttcccagtgttccaacttctgccctgacttgtttttgtaaatcggttagcactagcttttacagagtgaagagaattaagtccatcaacctcagatcccagggctgacgctgtcagttcactgacaatgctggccagtaatccacaggtgttagagacgaggtgggaggagaagagttcattttctctcctcaggctgttcctgactggtagcacaacaatgaccagcattttctccagaacttcacggaagcttgtcatccctgagatattctcttcactctggctgagtttttccatatgtgccaccaaaaggggaaaacgatgaactagtgttgagtcgttctctgtactaacttgtttaacaattgatcgtagtaatacttctccatcatacgcaatcgggaagatggaagtcagcttaacagacgtgtgacacagagctgacataacagctgcaaggagtcggctacttgatgtcttgaagtttgcttcttggatatcctgatccaaacaattcagcagatcacaaaggcaagcccactgtaaggcaggagttgggtagaaagaatgaaagcaggcagtgaaagtattatgacattcctgaaggacagcttctagaagactcaagggttgactgagatatccttgaggatcattatccaatttcaccatgcagtgatcaactccttctgataaaatttttcttaacaaagttctggtttttccaatacactctgctaatttgctagtttcttctacaactgcttttcctgtagctgacactgggtaaatttcacaggtatagacacgcaataacctcagacaacaggtacccacaaagcgcagtctctctaaatctaggagtgtagctgtgaactggaatccttttaatcctctaagttcttcaactcctaagactaaggtggtccagctccagtgaagaatactcaacaatgactcaaaacattccactgagacagttcttgcaaaagacctctttaaaatgtgtacaggttcactggtttgctgtttgccttttgaagcactgccatcactggttggaagtctgtataataactgaggtatctgacccgcattaacatctgtaccattatttgatttctttgaactcttgaactggaaaacaaccccatcatctgtggtaatagatgcctgtccatgagatccacagtcactgctgggtcctgacactcgggcccatgccacataccaccacccagcttgcaggagaacaggctcatcaaacatcattgcatatttttctctagcagcacagtcataagccaatacatcagtctctgcaagaaggtcaccatcagtttcatgatctcctccatcaggacccaattcaaacagcttaattttagcagtatattctcctctacctccaaacagaccaagaccaccaagtaaaatatcagtgtcggcactgaaacgtatagcttctactgaatgggcagaataaccccagcctcctccatgactttcaaacctgtttaccacactataatcttctttagaataaaccttcattactgcttgagtctcttcctctgtacttgcaacacccatttttaagtcctgcatagctgccaaggtatcaagacaacctaaaatgtgcaaagctgcatgagatcgggtagtgagggcccttgatcctgttggtaaggcaagttcaggacttaggatactacatctggactgcatgtctgctgcagagggaagcctggcatcagcaaccaccgcattgtaacaccacagctctctagtatttggtcgaaacctccaaattacatcatatacaggatcaagacacacaccaaatccttgcagatcctcttgttctgagtcattaaaagttttacaactcccatccactttatttatcagaaggcatttaaatggaggaggttctgatatagaagcaggtaccaagcctattatgtgtttactggcaaaaatttctgatgtagcaagtacatgagaattaataagtgcttcatcaattcgtaaaaaagtttggtccccacttgcacctatccaagtagcttttcttccatattttgatccaatgttaggcatgggagctggctttgcattccaatatggcacatccaaaattggtctgcccagttgtcctttagaaaaacttccaaatgtgaagacctgtccatccattaaaagtactgccgtatggttgctgcctgcagtgacttgtgtgctagggcctggcaatgcttgaacaagagtgggacatcccctggagttgacatctccatgtcctagctgcccatgctgcccataaccaaatgtatagacatctccattttccattaaaaccactgaatggtgaaatccacagctgacttggactgcccggagctcacagtcaaatcgcacagagcctggagggtatgttgtgattttgcttgcatccttttcgcctctttctccacttccatctttgtgcttgtcccgtttatgctttagctgtgctggatgggatctgagtctggctagagcctgttctcgatggttcataaaaataggaccagcaaatacaagggggcctcttccttcctctaatctgtgccttctgattacacgttgccgtttttcttcttgtcgtaactgaaggtgttcttcaatgttaaccccgggcactgggacagctaaaagaagatctaaaggtatcatttctttcactgcatcaagaattcctctttgtcttgcctcttgaccatctaactctcttgcacaggccttgcaacatccacacacagcacaaccagattctccggaaccacaaccacagatccctccggggactctgtctggccgtccactactgacacagctggctccataacctgtacagtctccacagacagtgcaaaccatgcactgctccagcttccatttgtgcatgcctggagggcacatcatagacttctcatctttttcatctagttcttcttccaggtcttcatccattgctgttgccatattttcaactccaaaccctttcccaccttggttcatggcaccagtatctcgtccacactgtcctttattatttacaccaaatgtccacacctctccattcttcattaaaacacaagtgtgagctttgcccatagctacctgagttacaaaatggcccttcaaatcagttaccaaacttgaactatcagagtaaatggcatcttttccaaacatgtagagttctccatctttagaaataacagaactacttccattattgcaggctgtatataccacaatctttccttccatcttaattatctttttaggtttataaggtttggattgccgtctgctcttagttgattctccatcttctcctttactagcagatcctgtaaagaatatgctcccatcttctgcaactaaaagggcgtgagagccatcgtgtccaactgagaagtgtactatctttggagattttgtaattggtagctcaacccattttcctgctgaaggaccaccttgtttgattccaagactctggtatttgccagtgtaatatatctttccatttgctgttttcattagcgcaaactctcgtcctgcaccaagaattgctgactcctcatcaaatcctgtacttataatatgcaagtccttttccagatcgaatagtgagataccacaggcatgtaagcattttctagccagtttaagttgcaattcttgctgtagaacaggttcagtgcttgtggcaaatattctgacaacaaagccatcatctcttgaagcagctatctgattaatatattctccatcagtgaataaaatattttgaccttcagtgtggcaatctggtaacatcacagtaccatcttgctccagtgtttcagggcttatccttatggctgtcatgctgtggttattcacatctctatataataaataaccctgagcataccctaaccaagactttttttcttttctgtttctaatacgggatgtagaattgtatatatggcccctaactgttccactgtatccagagcctattttatataatccatccttgcataatagataaagaaaaaatccatcattctgaagtagacattggtcatcttcatcaacagatatttcttttaatggccacttgtgcattaaagctgctttcttaatgccattactaaaccagtcctgaatttgaatttttcccaccaaaactgcttgtacacttctctgtagcgaatttagaattgttggcacctgaatagtttggcaagcatggcttccattgttggtgaggatagcagagatggcctgaagtgtccttcctgtttctccccaagaagccaccagactaaagaggcaagcacaggaaagtgctgttaaggactgtcctgtgctgtcattcatcccagtacttcgaacggtgatttccaaaagaagctggaagagagactctaggacctcaggtggctcagactggaggccttctggctgctggccctgcagcacgttgagcagggcttggagactcctgagacacagggatggatgagaaaatcgtgtctctttgatcaattcaaaaacttcacaaaggccaacctcaataatctttggaagcttgatagggggctctttggattcctcttcttcatcactatctgattctccactctgcacagagttcttagatgcggctgccaatgatatttcctttttctgccattccagaacgcaatggcgtacattacagtaaatattgaaagcagaaggattgctatgtagtttgatatctggtatgattactgtattctctaagttttcagactttttcctgctgcttgctctgtatcctttgttgtaataaatcttagccatgagtataaattgcttgtgagatttatgagtccttctggcaaatcaaaggaaaaaccacctaaacattccactcctcagtatgcacccaagaaaactgaacacacacacatacacacacaagtgcatatatatgtatataaaatcagcaaaaaaatgg

SEQ ID NO: 17091 - RNA, 9277 nt, Homo sapiens
  source 1..9277: mol_type = other RNA
tcaaaactgaggggcattttcttcttgcggagggtatctggatcaagtgtgtaagagtctgatttagaacgttcccgaggaggatcaagctttgtcttaacaggagcagtacttttttgaggtagatttttatcatgtggtgaggaggagcgtggagaactagcacccgatgggctagacctattggctgggagagtctttggcttaggagatgacaaccgagaacctggtcctggggattcagctctggagctagaaggcatcctcccatcagatttcaatgtctgcaaggtgttatggttgggggataatgacctactgtgggaatctgacctcaactttgcagcatcagattttaagatgagggattcactagcagataaactttctgtgccccttggcttcttctgatcagcagtagtccggctcatacgtccatcaggtttaagcgatctgctgtgtttagaggacagctctgattttcctgatgtagaggctggtttagaagatgttgagatgtttcctcgatcacccttcagtttgtgagacagagatgagagagcagaggcaggcccagctacaccataatttttgtaaatgcgctcacgagaagcaaggttgcgagatggagatttctgaagctgaggctgctggaaggaaaggggctgtccgaacacaaatgggctgtgtactagggaagagggaggttttgcagcttgatcaaagatggaaggagctgggagattgggtcgtgactgaatggaattcaatatggcactcagttggtcacctgcagtgggtaaaacagtcaaaactttgctatttccgagtccataatcaaatccttgggcactgcaacttgcccctttattaaaagcttgcactgagaaagggcttggaggaggagtttgagaattctgatccagaagagcttgttcatcttcatgtcggaggtactggtttccgcctctgtctctagctaaggaccatgcctctccttcatcactctcacagaactctaccatgctgttctgatccagttgcacccatgtcccttcagaattggttacctctcccactgctttgactttgtttcccagaactaacattccaattgggatacctctaaggttagggcagcttctgatgttgtgacctgaaggtcccgtcttcactaccttgtacatgcctggccctcctcgcaagaatggcatatcttgttcttgcattgttgcttcctgtgggcagcaggagtttatgtctttgaaaaagtcatcagtattagttttagattcgtcaacagggaccagaagactcttgccaagatgttgattaaaagagaggcaccaggcttcagtgtaaccattcatgttagggacatacttctttattgtctcatcattcagcctcagccacacaccatcatcattatggatctcatcaataaaagtgatagttccattgactttcactatgcctatctgctcactctgaagggaagggtggctacggatgcgaagccccgcactgtccttggccacaaattttcgaaccttattaggctgaggttcagactttggtttgaccaactgagttcctggtggtatcatcccttttggtgggtcttttacttttacttccagaccagcatcgatttcaatgccatcaatggtaacatgaagagtgtagagtccaatagcccctggagtccaatttgcacaataagtcccatcattattgacacggatcagcatattctcactgggtctcttaggagttggtgatgcaaaacgtagttcttcaaatgaataattttcataaaccttcatcattgttatggcaatatatcgagcttccttcactatcattggttcatatgaaacatctagctttggtgatgccagccctccataagtcatgtcagtattagaagatgcagctgttactgcaggactgccaggaatcctttgaggtttctttgcttgatcttgttgtaaagacatttttttctgagaaacagggacagctttcacttccaccttcatattgggaacatgtaccacatccccatactggtcttttgtttgaacagttatggtggtaggccaaccacaacgaatatcatccttattcaggatcaaagatgttttctgaggatccgcatatgaatctggctgaagccaccttgcaagccttccaccacttgatcctgggacacaggcaataaaatcatccagaaaagactgttcattgctttggatttggagtggtaaatttccctcaagtgcttctaatatagttggtgaatgagaaagagctagaccctttccaagaattccagaatgggttttgcacacctgcaatgcagcctcctcaagaatttcaaggtcttcttctaattcattaccaataggaagtgctaggtccttcttcatcagagctgctgcacaaaccccaccaagattggctaattctttttccaattggatgactccctcatcaggtccagggctaaattcatatccaattgcaaaacacttaaaaccatagaaagaagctttgtcatctttcacataatctgatgcagtctccaatgaaaaaagggcctcatttcctggcaacaccaaaaccatagtaggccacccagaggatcctgaaaatttctttaattctatccatgaattaagattttcatgaacagatgtcaattttggtccatatcctgaattctgaacagttctgacaggaatcaacaaacgaaggacatcttctgactgtgcagtaccacactgagggtcaaattcgattgtcatccacctcacacattctgggaatgtcaccttgtaatgcatcacacaggcaggtttatacgggtgctcactctctatgacagcatagtgactggaggttgtacaagcagagaggccctgttcaggctggtttcctgtggtgctatctgtcgactgattagggttgaaggcaggcggtgcatacttctgattcaaaatggcaactgacggaagcaattgttggacaaggccaaagacttctacagccaccttgggaatagcagcagctactggtcctatgtaggctataataagggggagcagcatggaaaacagactggaagaactcagcagttctggaatgtcatcagcatccacagcaagagctctgtgcaggaggtccttagaggctcgaacgacagtgcttacaacagacaatgctctgctacagtttttatcttcttcattggctttactcagaagttgggattgtaaatctccatcaaattcactcctatagtagagtatctgtgggatctgtcctctggtttggtttgtgccgttactgctcaagctgcacgtgctgaatgtgaatgtcacaccatcagggcactgaactgtggtcattcctccatctccattggctgtacggcttccatagttcctcaagcgcacagcatatttaacattttcctttaaaggaaccactttgtcaagtctgatctcagctatatcactgggtgagtcatccgttgtgtacgttcctttcactaattccagagatgtccatctgtgggaatgagttgaatctcctgcatgttcactatcatcaaccaacacctctaattcatattcatgaattccacctcctccatagacagagaaaccaaccacaactattccaggtttgtctactgaaaaacagattgcatcaggggacccgttcccagtgttccaacttctgccctgacttgtttttgtaaatcggttagcactagcttttacagagtgaagagaattaagtccatcaacctcagatcccagggctgacgctgtcagttcactgacaatgctggccagtaatccacaggtgttagagacgaggtgggaggagaagagttcattttctctcctcaggctgttcctgactggtagcacaacaatgaccagcattttctccagaacttcacggaagcttgtcatccctgagatattctcttcactctggctgagtttttccatatgtgccaccaaaaggggaaaacgatgaactagtgttgagtcgttctctgtactaacttgtttaacaattgatcgtagtaatacttctccatcatacgcaatcgggaagatggaagtcagcttaacagacgtgtgacacagagctgacataacagctgcaaggagtcggctacttgatgtcttgaagtttgcttcttggatatcctgatccaaacaattcagcagatcacaaaggcaagcccactgtaaggcaggagttgggtagaaagaatgaaagcaggcagtgaaagtattatgacattcctgaaggacagcttctagaagactcaagggttgactgagatatccttgaggatcattatccaatttcaccatgcagtgatcaactccttctgataaaatttttcttaacaaagttctggtttttccaatacactctgctaatttgctagtttcttctacaactgcttttcctgtagctgacactgggtaaatttcacaggtatagacacgcaataacctcagacaacaggtacccacaaagcgcagtctctctaaatctaggagtgtagctgtgaactggaatccttttaatcctctaagttcttcaactcctaagactaaggtggtccagctccagtgaagaatactcaacaatgactcaaaacattccactgagacagttcttgcaaaagacctctttaaaatgtgtacaggttcactggtttgctgtttgccttttgaagcactgccatcactggttggaagtctgtataataactgaggtatctgacccgcattaacatctgtaccattatttgatttctttgaactcttgaactggaaaacaaccccatcatctgtggtaatagatgcctgtccatgagatccacagtcactgctgggtcctgacactcgggcccatgccacataccaccacccagcttgcaggagaacaggctcatcaaacatcattgcatatttttctctagcagcacagtcataagccaatacatcagtctctgcaagaaggtcaccatcagtttcatgatctcctccatcaggacccaattcaaacagcttaattttagcagtatattctcctctacctccaaacagaccaagaccaccaagtaaaatatcagtgtcggcactgaaacgtatagcttctactgaatgggcagaataaccccagcctcctccatgactttcaaacctgtttaccacactataatcttctttagaataaaccttcattactgcttgagtctcttcctctgtacttgcaacacccatttttaagtcctgcatagctgccaaggtatcaagacaacctaaaatgtgcaaagctgcatgagatcgggtagtgagggcccttgatcctgttggtaaggcaagttcaggacttaggatactacatctggactgcatgtctgctgcagagggaagcctggcatcagcaaccaccgcattgtaacaccacagctctctagtatttggtcgaaacctccaaattacatcatatacaggatcaagacacacaccaaatccttgcagatcctcttgttctgagtcattaaaagttttacaactcccatccactttatttatcagaaggcatttaaatggaggaggttctgatatagaagcaggtaccaagcctattatgtgtttactggcaaaaatttctgatgtagcaagtacatgagaattaataagtgcttcatcaattcgtaaaaaagtttggtccccacttgcacctatccaagtagcttttcttccatattttgatccaatgttaggcatgggagctggctttgcattccaatatggcacatccaaaattggtctgcccagttgtcctttagaaaaacttccaaatgtgaagacctgtccatccattaaaagtactgccgtatggttgctgcctgcagtgacttgtgtgctagggcctggcaatgcttgaacaagagtgggacatcccctggagttgacatctccatgtcctagctgcccatgctgcccataaccaaatgtatagacatctccattttccattaaaaccactgaatggtgaaatccacagctgacttggactgcccggagctcacagtcaaatcgcacagagcctggagggtatgttgtgattttgcttgcatccttttcgcctctttctccacttccatctttgtgcttgtcccgtttatgctttagctgtgctggatgggatctgagtctggctagagcctgttctcgatggttcataaaaataggaccagcaaatacaagggggcctcttccttcctctaatctgtgccttctgattacacgttgccgtttttcttcttgtcgtaactgaaggtgttcttcaatgttaaccccgggcactgggacagctaaaagaagatctaaaggtatcatttctttcactgcatcaagaattcctctttgtcttgcctcttgaccatctaactctcttgcacaggccttgcaacatccacacacagcacaaccagattctccggaaccacaaccacagatccctccggggactctgtctggccgtccactactgacacagctggctccataacctgtacagtctccacagacagtgcaaaccatgcactgctccagcttccatttgtgcatgcctggagggcacatcatagacttctcatctttttcatctagttcttcttccaggtcttcatccattgctgttgccatattttcaactccaaaccctttcccaccttggttcatggcaccagtatctcgtccacactgtcctttattatttacaccaaatgtccacacctctccattcttcattaaaacacaagtgtgagctttgcccatagctacctgagttacaaaatggcccttcaaatcagttaccaaacttgaactatcagagtaaatggcatcttttccaaacatgtagagttctccatctttagaaataacagaactacttccattattgcaggctgtatataccacaatctttccttccatcttaattatctttttaggtttataaggtttggattgccgtctgctcttagttgattctccatcttctcctttactagcagatcctgtaaagaatatgctcccatcttctgcaactaaaagggcgtgagagccatcgtgtccaactgagaagtgtactatctttggagattttgtaattggtagctcaacccattttcctgctgaaggaccaccttgtttgattccaagactctggtatttgccagtgtaatatatctttccatttgctgttttcattagcgcaaactctcgtcctgcaccaagaattgctgactcctcatcaaatcctgtacttataatatgcaagtccttttccagatcgaatagtgagataccacaggcatgtaagcattttctagccagtttaagttgcaattcttgctgtagaacaggttcagtgcttgtggcaaatattctgacaacaaagccatcatctcttgaagcagctatctgattaatatattctccatcagtgaataaaatattttgaccttcagtgtggcaatctggtaacatcacagtaccatcttgctccagtgtttcagggcttatccttatggctgtcatgctgtggttattcacatctctatataataaataaccctgagcataccctaaccaagactttttttcttttctgtttctaatacgggatgtagaattgtatatatggcccctaactgttccactgtatccagagcctattttatataatccatccttgcataatagataaagaaaaaatccatcattctgaagtagacattggtcatcttcatcaacagatatttcttttaatggccacttgtgcattaaagctgctttcttaatgccattactaaaccagtcctgaatttgaatttttcccaccaaaactgcttgtacacttctctgtagcgaatttagaattgttggcacctgaatagtttggcaagcatggcttccattgttggtgaggatagcagagatggcctgaagtgtccttcctgtttctccccaagaagccaccagactaaagaggcaagcacaggaaagtgctgttaaggactgtcctgtgctgtcattcatcccagtacttcgaacggtgatttccaaaagaagctggaagagagactctaggacctcaggtggctcagactggaggccttctggctgctggccctgcagcacgttgagcagggcttggagactcctgagacacagggatggatgagaaaatcgtgtctctttgatcaattcaaaaacttcacaaaggccaacctcaataatctttggaagcttgatagggggctctttggattcctcttcttcatcactatctgattctccactctgcacagagttcttagatgcggctgccaatgatatttcctttttctgccattccagaacgcaatggcgtacattacagtaaatattgaaagcagaaggattgctatgtagtttgatatctggtatgattactgtattctctaagttttcagacttgcttcttgtcttcacttttgatttgctcttctgttttcttttcaatttcttcttatttaaaattttcttattcctggaggctgggtgtccagcgctgccgcccccctggtccctgtcattgagcgcagcggtataaatcctccggtagcggtcggccagggcccggcctgacagcagcagctggtagtgaccccgggagtccgcggcgggtagccccagccccagccccgcagcagccacggagccgtcgggaaccggcatgaacagcgcccccggcgccggggaggaagagaaggtggcggctgggtagaatccgtccccgccgagccccgaggaggcggcggcgggggaggcagtcgctgcgcacatcatcatcctcgccgccgccgccgccgccgccgcctcgtccccgcgggccgggcgggcagacacgcgcgcgcacacacagcccttttccaacgacgacggctccggcggcggcctctggctcccgcagcagggagactacaaagacagcgacctccttctcctcctccttcttctcctcctcccccccgcgccgccctcgccgctactggggccgctcatctaaccccgccaccccgggaatgtgaggaggaggcggtgccgccactgccgccgccaccaccgctaccaccgccaccaccgccggggctacccgcaatgggaagctgccg

SEQ ID NO: 17092 - RNA, 9220 nt, Homo sapiens
  source 1..9220: mol_type = other RNA
tcaaaactgaggggcattttcttcttgcggagggtatctggatcaagtgtgtaagagtctgatttagaacgttcccgaggaggatcaagctttgtcttaacaggagcagtacttttttgaggtagatttttatcatgtggtgaggaggagcgtggagaactagcacccgatgggctagacctattggctgggagagtctttggcttaggagatgacaaccgagaacctggtcctggggattcagctctggagctagaaggcatcctcccatcagatttcaatgtctgcaaggtgttatggttgggggataatgacctactgtgggaatctgacctcaactttgcagcatcagattttaagatgagggattcactagcagataaactttctgtgccccttggcttcttctgatcagcagtagtccggctcatacgtccatcaggtttaagcgatctgctgtgtttagaggacagctctgattttcctgatgtagaggctggtttagaagatgttgagatgtttcctcgatcacccttcagtttgtgagacagagatgagagagcagaggcaggcccagctacaccataatttttgtaaatgcgctcacgagaagcaaggttgcgagatggagatttctgaagctgaggctgctggaaggaaaggggctgtccgaacacaaatgggctgtgtactagggaagagggaggttttgcagcttgatcaaagatggaaggagctgggagattgggtcgtgactgaatggaattcaatatggcactcagttggtcacctgcagtgggtaaaacagtcaaaactttgctatttccgagtccataatcaaatccttgggcactgcaacttgcccctttattaaaagcttgcactgagaaagggcttggaggaggagtttgagaattctgatccagaagagcttgttcatcttcatgtcggaggtactggtttccgcctctgtctctagctaaggaccatgcctctccttcatcactctcacagaactctaccatgctgttctgatccagttgcacccatgtcccttcagaattggttacctctcccactgctttgactttgtttcccagaactaacattccaattgggatacctctaaggttagggcagcttctgatgttgtgacctgaaggtcccgtcttcactaccttgtacatgcctggccctcctcgcaagaatggcatatcttgttcttgcattgttgcttcgtcaacagggaccagaagactcttgccaagatgttgattaaaagagaggcaccaggcttcagtgtaaccattcatgttagggacatacttctttattgtctcatcattcagcctcagccacacaccatcatcattatggatctcatcaataaaagtgatagttccattgactttcactatgcctatctgctcactctgaagggaagggtggctacggatgcgaagccccgcactgtccttggccacaaattttcgaaccttattaggctgaggttcagactttggtttgaccaactgagttcctggtggtatcatcccttttggtgggtcttttacttttacttccagaccagcatcgatttcaatgccatcaatggtaacatgaagagtgtagagtccaatagcccctggagtccaatttgcacaataagtcccatcattattgacacggatcagcatattctcactgggtctcttaggagttggtgatgcaaaacgtagttcttcaaatgaataattttcataaaccttcatcattgttatggcaatatatcgagcttccttcactatcattggttcatatgaaacatctagctttggtgatgccagccctccataagtcatgtcagtattagaagatgcagctgttactgcaggactgccaggaatcctttgaggtttctttgcttgatcttgttgtaaagacatttttttctgagaaacagggacagctttcacttccaccttcatattgggaacatgtaccacatccccatactggtcttttgtttgaacagttatggtggtaggccaaccacaacgaatatcatccttattcaggatcaaagatgttttctgaggatccgcatatgaatctggctgaagccaccttgcaagccttccaccacttgatcctgggacacaggcaataaaatcatccagaaaagactgttcattgctttggatttggagtggtaaatttccctcaagtgcttctaatatagttggtgaatgagaaagagctagaccctttccaagaattccagaatgggttttgcacacctgcaatgcagcctcctcaagaatttcaaggtcttcttctaattcattaccaataggaagtgctaggtccttcttcatcagagctgctgcacaaaccccaccaagattggctaattctttttccaattggatgactccctcatcaggtccagggctaaattcatatccaattgcaaaacacttaaaaccatagaaagaagctttgtcatctttcacataatctgatgcagtctccaatgaaaaaagggcctcatttcctggcaacaccaaaaccatagtaggccacccagaggatcctgaaaatttctttaattctatccatgaattaagattttcatgaacagatgtcaattttggtccatatcctgaattctgaacagttctgacaggaatcaacaaacgaaggacatcttctgactgtgcagtaccacactgagggtcaaattcgattgtcatccacctcacacattctgggaatgtcaccttgtaatgcatcacacaggcaggtttatacgggtgctcactctctatgacagcatagtgactggaggttgtacaagcagagaggccctgttcaggctggtttcctgtggtgctatctgtcgactgattagggttgaaggcaggcggtgcatacttctgattcaaaatggcaactgacggaagcaattgttggacaaggccaaagacttctacagccaccttgggaatagcagcagctactggtcctatgtaggctataataagggggagcagcatggaaaacagactggaagaactcagcagttctggaatgtcatcagcatccacagcaagagctctgtgcaggaggtccttagaggctcgaacgacagtgcttacaacagacaatgctctgctacagtttttatcttcttcattggctttactcagaagttgggattgtaaatctccatcaaattcactcctatagtagagtatctgtgggatctgtcctctggtttggtttgtgccgttactgctcaagctgcacgtgctgaatgtgaatgtcacaccatcagggcactgaactgtggtcattcctccatctccattggctgtacggcttccatagttcctcaagcgcacagcatatttaacattttcctttaaaggaaccactttgtcaagtctgatctcagctatatcactgggtgagtcatccgttgtgtacgttcctttcactaattccagagatgtccatctgtgggaatgagttgaatctcctgcatgttcactatcatcaaccaacacctctaattcatattcatgaattccacctcctccatagacagagaaaccaaccacaactattccaggtttgtctactgaaaaacagattgcatcaggggacccgttcccagtgttccaacttctgccctgacttgtttttgtaaatcggttagcactagcttttacagagtgaagagaattaagtccatcaacctcagatcccagggctgacgctgtcagttcactgacaatgctggccagtaatccacaggtgttagagacgaggtgggaggagaagagttcattttctctcctcaggctgttcctgactggtagcacaacaatgaccagcattttctccagaacttcacggaagcttgtcatccctgagatattctcttcactctggctgagtttttccatatgtgccaccaaaaggggaaaacgatgaactagtgttgagtcgttctctgtactaacttgtttaacaattgatcgtagtaatacttctccatcatacgcaatcgggaagatggaagtcagcttaacagacgtgtgacacagagctgacataacagctgcaaggagtcggctacttgatgtcttgaagtttgcttcttggatatcctgatccaaacaattcagcagatcacaaaggcaagcccactgtaaggcaggagttgggtagaaagaatgaaagcaggcagtgaaagtattatgacattcctgaaggacagcttctagaagactcaagggttgactgagatatccttgaggatcattatccaatttcaccatgcagtgatcaactccttctgataaaatttttcttaacaaagttctggtttttccaatacactctgctaatttgctagtttcttctacaactgcttttcctgtagctgacactgggtaaatttcacaggtatagacacgcaataacctcagacaacaggtacccacaaagcgcagtctctctaaatctaggagtgtagctgtgaactggaatccttttaatcctctaagttcttcaactcctaagactaaggtggtccagctccagtgaagaatactcaacaatgactcaaaacattccactgagacagttcttgcaaaagacctctttaaaatgtgtacaggttcactggtttgctgtttgccttttgaagcactgccatcactggttggaagtctgtataataactgaggtatctgacccgcattaacatctgtaccattatttgatttctttgaactcttgaactggaaaacaaccccatcatctgtggtaatagatgcctgtccatgagatccacagtcactgctgggtcctgacactcgggcccatgccacataccaccacccagcttgcaggagaacaggctcatcaaacatcattgcatatttttctctagcagcacagtcataagccaatacatcagtctctgcaagaaggtcaccatcagtttcatgatctcctccatcaggacccaattcaaacagcttaattttagcagtatattctcctctacctccaaacagaccaagaccaccaagtaaaatatcagtgtcggcactgaaacgtatagcttctactgaatgggcagaataaccccagcctcctccatgactttcaaacctgtttaccacactataatcttctttagaataaaccttcattactgcttgagtctcttcctctgtacttgcaacacccatttttaagtcctgcatagctgccaaggtatcaagacaacctaaaatgtgcaaagctgcatgagatcgggtagtgagggcccttgatcctgttggtaaggcaagttcaggacttaggatactacatctggactgcatgtctgctgcagagggaagcctggcatcagcaaccaccgcattgtaacaccacagctctctagtatttggtcgaaacctccaaattacatcatatacaggatcaagacacacaccaaatccttgcagatcctcttgttctgagtcattaaaagttttacaactcccatccactttatttatcagaaggcatttaaatggaggaggttctgatatagaagcaggtaccaagcctattatgtgtttactggcaaaaatttctgatgtagcaagtacatgagaattaataagtgcttcatcaattcgtaaaaaagtttggtccccacttgcacctatccaagtagcttttcttccatattttgatccaatgttaggcatgggagctggctttgcattccaatatggcacatccaaaattggtctgcccagttgtcctttagaaaaacttccaaatgtgaagacctgtccatccattaaaagtactgccgtatggttgctgcctgcagtgacttgtgtgctagggcctggcaatgcttgaacaagagtgggacatcccctggagttgacatctccatgtcctagctgcccatgctgcccataaccaaatgtatagacatctccattttccattaaaaccactgaatggtgaaatccacagctgacttggactgcccggagctcacagtcaaatcgcacagagcctggagggtatgttgtgattttgcttgcatccttttcgcctctttctccacttccatctttgtgcttgtcccgtttatgctttagctgtgctggatgggatctgagtctggctagagcctgttctcgatggttcataaaaataggaccagcaaatacaagggggcctcttccttcctctaatctgtgccttctgattacacgttgccgtttttcttcttgtcgtaactgaaggtgttcttcaatgttaaccccgggcactgggacagctaaaagaagatctaaaggtatcatttctttcactgcatcaagaattcctctttgtcttgcctcttgaccatctaactctcttgcacaggccttgcaacatccacacacagcacaaccagattctccggaaccacaaccacagatccctccggggactctgtctggccgtccactactgacacagctggctccataacctgtacagtctccacagacagtgcaaaccatgcactgctccagcttccatttgtgcatgcctggagggcacatcatagacttctcatctttttcatctagttcttcttccaggtcttcatccattgctgttgccatattttcaactccaaaccctttcccaccttggttcatggcaccagtatctcgtccacactgtcctttattatttacaccaaatgtccacacctctccattcttcattaaaacacaagtgtgagctttgcccatagctacctgagttacaaaatggcccttcaaatcagttaccaaacttgaactatcagagtaaatggcatcttttccaaacatgtagagttctccatctttagaaataacagaactacttccattattgcaggctgtatataccacaatctttccttccatcttaattatctttttaggtttataaggtttggattgccgtctgctcttagttgattctccatcttctcctttactagcagatcctgtaaagaatatgctcccatcttctgcaactaaaagggcgtgagagccatcgtgtccaactgagaagtgtactatctttggagattttgtaattggtagctcaacccattttcctgctgaaggaccaccttgtttgattccaagactctggtatttgccagtgtaatatatctttccatttgctgttttcattagcgcaaactctcgtcctgcaccaagaattgctgactcctcatcaaatcctgtacttataatatgcaagtccttttccagatcgaatagtgagataccacaggcatgtaagcattttctagccagtttaagttgcaattcttgctgtagaacaggttcagtgcttgtggcaaatattctgacaacaaagccatcatctcttgaagcagctatctgattaatatattctccatcagtgaataaaatattttgaccttcagtgtggcaatctggtaacatcacagtaccatcttgctccagtgtttcagggcttatccttatggctgtcatgctgtggttattcacatctctatataataaataaccctgagcataccctaaccaagactttttttcttttctgtttctaatacgggatgtagaattgtatatatggcccctaactgttccactgtatccagagcctattttatataatccatccttgcataatagataaagaaaaaatccatcattctgaagtagacattggtcatcttcatcaacagatatttcttttaatggccacttgtgcattaaagctgctttcttaatgccattactaaaccagtcctgaatttgaatttttcccaccaaaactgcttgtacacttctctgtagcgaatttagaattgttggcacctgaatagtttggcaagcatggcttccattgttggtgaggatagcagagatggcctgaagtgtccttcctgtttctccccaagaagccaccagactaaagaggcaagcacaggaaagtgctgttaaggactgtcctgtgctgtcattcatcccagtacttcgaacggtgatttccaaaagaagctggaagagagactctaggacctcaggtggctcagactggaggccttctggctgctggccctgcagcacgttgagcagggcttggagactcctgagacacagggatggatgagaaaatcgtgtctctttgatcaattcaaaaacttcacaaaggccaacctcaataatctttggaagcttgatagggggctctttggattcctcttcttcatcactatctgattctccactctgcacagagttcttagatgcggctgccaatgatatttcctttttctgccattccagaacgcaatggcgtacattacagtaaatattgaaagcagaaggattgctatgtagtttgatatctggtatgattactgtattctctaagttttcagacttgcttcttgtcttcacttttgatttgctcttctgttttcttttcaatttcttcttatttaaaattttcttattcctggaggctgggtgtccagcgctgccgcccccctggtccctgtcattgagcgcagcggtataaatcctccggtagcggtcggccagggcccggcctgacagcagcagctggtagtgaccccgggagtccgcggcgggtagccccagccccagccccgcagcagccacggagccgtcgggaaccggcatgaacagcgcccccggcgccggggaggaagagaaggtggcggctgggtagaatccgtccccgccgagccccgaggaggcggcggcgggggaggcagtcgctgcgcacatcatcatcctcgccgccgccgccgccgccgccgcctcgtccccgcgggccgggcgggcagacacgcgcgcgcacacacagcccttttccaacgacgacggctccggcggcggcctctggctcccgcagcagggagactacaaagacagcgacctccttctcctcctccttcttctcctcctcccccccgcgccgccctcgccgctactggggccgctcatctaaccccgccaccccgggaatgtgaggaggaggcggtgccgccactgccgccgccaccaccgctaccaccgccaccaccgccggggctacccgcaatgggaagctgccg

SEQ ID NO: 17093 - RNA, 9052 nt, Homo sapiens
  source 1..9052: mol_type = other RNA
tcaaaactgaggggcattttcttcttgcggagggtatctggatcaagtgtgtaagagtctgatttagaacgttcccgaggaggatcaagctttgtcttaacaggagcagtacttttttgaggtagatttttatcatgtggtgaggaggagcgtggagaactagcacccgatgggctagacctattggctgggagagtctttggcttaggagatgacaaccgagaacctggtcctggggattcagctctggagctagaaggcatcctcccatcagatttcaatgtctgcaaggtgttatggttgggggataatgacctactgtgggaatctgacctcaactttgcagcatcagattttaagatgagggattcactagcagataaactttctgtgccccttggcttcttctgatcagcagtagtccggctcatacgtccatcaggtttaagcgatctgctgtgtttagaggacagctctgattttcctgatgtagaggctggtttagaagatgttgagatgtttcctcgatcacccttcagtttgtgagacagagatgagagagcagaggcaggcccagctacaccataatttttgtaaatgcgctcacgagaagcaaggttgcgagatggagatttctgaagctgaggctgctggaaggaaaggggctgtccgaacacaaatgggctgtgtactagggaagagggaggttttgcagcttgatcaaagatggaaggagctgggagattgggtcgtgactgaatggaattcaatatggcactcagttggtcacctgcagtgggtaaaacagtcaaaactttgctatttccgagtccataatcaaatccttgggcactgcaacttgcccctttattaaaagcttgcactgagaaagggcttggaggaggagtttgagaattctgatccagaagagcttgttcatcttcatgtcggaggtactggtttccgcctctgtctctagctaaggaccatgcctctccttcatcactctcacagaactctaccatgctgttctgatccagttgcacccatgtcccttcagaattggttacgtcaacagggaccagaagactcttgccaagatgttgattaaaagagaggcaccaggcttcagtgtaaccattcatgttagggacatacttctttattgtctcatcattcagcctcagccacacaccatcatcattatggatctcatcaataaaagtgatagttccattgactttcactatgcctatctgctcactctgaagggaagggtggctacggatgcgaagccccgcactgtccttggccacaaattttcgaaccttattaggctgaggttcagactttggtttgaccaactgagttcctggtggtatcatcccttttggtgggtcttttacttttacttccagaccagcatcgatttcaatgccatcaatggtaacatgaagagtgtagagtccaatagcccctggagtccaatttgcacaataagtcccatcattattgacacggatcagcatattctcactgggtctcttaggagttggtgatgcaaaacgtagttcttcaaatgaataattttcataaaccttcatcattgttatggcaatatatcgagcttccttcactatcattggttcatatgaaacatctagctttggtgatgccagccctccataagtcatgtcagtattagaagatgcagctgttactgcaggactgccaggaatcctttgaggtttctttgcttgatcttgttgtaaagacatttttttctgagaaacagggacagctttcacttccaccttcatattgggaacatgtaccacatccccatactggtcttttgtttgaacagttatggtggtaggccaaccacaacgaatatcatccttattcaggatcaaagatgttttctgaggatccgcatatgaatctggctgaagccaccttgcaagccttccaccacttgatcctgggacacaggcaataaaatcatccagaaaagactgttcattgctttggatttggagtggtaaatttccctcaagtgcttctaatatagttggtgaatgagaaagagctagaccctttccaagaattccagaatgggttttgcacacctgcaatgcagcctcctcaagaatttcaaggtcttcttctaattcattaccaataggaagtgctaggtccttcttcatcagagctgctgcacaaaccccaccaagattggctaattctttttccaattggatgactccctcatcaggtccagggctaaattcatatccaattgcaaaacacttaaaaccatagaaagaagctttgtcatctttcacataatctgatgcagtctccaatgaaaaaagggcctcatttcctggcaacaccaaaaccatagtaggccacccagaggatcctgaaaatttctttaattctatccatgaattaagattttcatgaacagatgtcaattttggtccatatcctgaattctgaacagttctgacaggaatcaacaaacgaaggacatcttctgactgtgcagtaccacactgagggtcaaattcgattgtcatccacctcacacattctgggaatgtcaccttgtaatgcatcacacaggcaggtttatacgggtgctcactctctatgacagcatagtgactggaggttgtacaagcagagaggccctgttcaggctggtttcctgtggtgctatctgtcgactgattagggttgaaggcaggcggtgcatacttctgattcaaaatggcaactgacggaagcaattgttggacaaggccaaagacttctacagccaccttgggaatagcagcagctactggtcctatgtaggctataataagggggagcagcatggaaaacagactggaagaactcagcagttctggaatgtcatcagcatccacagcaagagctctgtgcaggaggtccttagaggctcgaacgacagtgcttacaacagacaatgctctgctacagtttttatcttcttcattggctttactcagaagttgggattgtaaatctccatcaaattcactcctatagtagagtatctgtgggatctgtcctctggtttggtttgtgccgttactgctcaagctgcacgtgctgaatgtgaatgtcacaccatcagggcactgaactgtggtcattcctccatctccattggctgtacggcttccatagttcctcaagcgcacagcatatttaacattttcctttaaaggaaccactttgtcaagtctgatctcagctatatcactgggtgagtcatccgttgtgtacgttcctttcactaattccagagatgtccatctgtgggaatgagttgaatctcctgcatgttcactatcatcaaccaacacctctaattcatattcatgaattccacctcctccatagacagagaaaccaaccacaactattccaggtttgtctactgaaaaacagattgcatcaggggacccgttcccagtgttccaacttctgccctgacttgtttttgtaaatcggttagcactagcttttacagagtgaagagaattaagtccatcaacctcagatcccagggctgacgctgtcagttcactgacaatgctggccagtaatccacaggtgttagagacgaggtgggaggagaagagttcattttctctcctcaggctgttcctgactggtagcacaacaatgaccagcattttctccagaacttcacggaagcttgtcatccctgagatattctcttcactctggctgagtttttccatatgtgccaccaaaaggggaaaacgatgaactagtgttgagtcgttctctgtactaacttgtttaacaattgatcgtagtaatacttctccatcatacgcaatcgggaagatggaagtcagcttaacagacgtgtgacacagagctgacataacagctgcaaggagtcggctacttgatgtcttgaagtttgcttcttggatatcctgatccaaacaattcagcagatcacaaaggcaagcccactgtaaggcaggagttgggtagaaagaatgaaagcaggcagtgaaagtattatgacattcctgaaggacagcttctagaagactcaagggttgactgagatatccttgaggatcattatccaatttcaccatgcagtgatcaactccttctgataaaatttttcttaacaaagttctggtttttccaatacactctgctaatttgctagtttcttctacaactgcttttcctgtagctgacactgggtaaatttcacaggtatagacacgcaataacctcagacaacaggtacccacaaagcgcagtctctctaaatctaggagtgtagctgtgaactggaatccttttaatcctctaagttcttcaactcctaagactaaggtggtccagctccagtgaagaatactcaacaatgactcaaaacattccactgagacagttcttgcaaaagacctctttaaaatgtgtacaggttcactggtttgctgtttgccttttgaagcactgccatcactggttggaagtctgtataataactgaggtatctgacccgcattaacatctgtaccattatttgatttctttgaactcttgaactggaaaacaaccccatcatctgtggtaatagatgcctgtccatgagatccacagtcactgctgggtcctgacactcgggcccatgccacataccaccacccagcttgcaggagaacaggctcatcaaacatcattgcatatttttctctagcagcacagtcataagccaatacatcagtctctgcaagaaggtcaccatcagtttcatgatctcctccatcaggacccaattcaaacagcttaattttagcagtatattctcctctacctccaaacagaccaagaccaccaagtaaaatatcagtgtcggcactgaaacgtatagcttctactgaatgggcagaataaccccagcctcctccatgactttcaaacctgtttaccacactataatcttctttagaataaaccttcattactgcttgagtctcttcctctgtacttgcaacacccatttttaagtcctgcatagctgccaaggtatcaagacaacctaaaatgtgcaaagctgcatgagatcgggtagtgagggcccttgatcctgttggtaaggcaagttcaggacttaggatactacatctggactgcatgtctgctgcagagggaagcctggcatcagcaaccaccgcattgtaacaccacagctctctagtatttggtcgaaacctccaaattacatcatatacaggatcaagacacacaccaaatccttgcagatcctcttgttctgagtcattaaaagttttacaactcccatccactttatttatcagaaggcatttaaatggaggaggttctgatatagaagcaggtaccaagcctattatgtgtttactggcaaaaatttctgatgtagcaagtacatgagaattaataagtgcttcatcaattcgtaaaaaagtttggtccccacttgcacctatccaagtagcttttcttccatattttgatccaatgttaggcatgggagctggctttgcattccaatatggcacatccaaaattggtctgcccagttgtcctttagaaaaacttccaaatgtgaagacctgtccatccattaaaagtactgccgtatggttgctgcctgcagtgacttgtgtgctagggcctggcaatgcttgaacaagagtgggacatcccctggagttgacatctccatgtcctagctgcccatgctgcccataaccaaatgtatagacatctccattttccattaaaaccactgaatggtgaaatccacagctgacttggactgcccggagctcacagtcaaatcgcacagagcctggagggtatgttgtgattttgcttgcatccttttcgcctctttctccacttccatctttgtgcttgtcccgtttatgctttagctgtgctggatgggatctgagtctggctagagcctgttctcgatggttcataaaaataggaccagcaaatacaagggggcctcttccttcctctaatctgtgccttctgattacacgttgccgtttttcttcttgtcgtaactgaaggtgttcttcaatgttaaccccgggcactgggacagctaaaagaagatctaaaggtatcatttctttcactgcatcaagaattcctctttgtcttgcctcttgaccatctaactctcttgcacaggccttgcaacatccacacacagcacaaccagattctccggaaccacaaccacagatccctccggggactctgtctggccgtccactactgacacagctggctccataacctgtacagtctccacagacagtgcaaaccatgcactgctccagcttccatttgtgcatgcctggagggcacatcatagacttctcatctttttcatctagttcttcttccaggtcttcatccattgctgttgccatattttcaactccaaaccctttcccaccttggttcatggcaccagtatctcgtccacactgtcctttattatttacaccaaatgtccacacctctccattcttcattaaaacacaagtgtgagctttgcccatagctacctgagttacaaaatggcccttcaaatcagttaccaaacttgaactatcagagtaaatggcatcttttccaaacatgtagagttctccatctttagaaataacagaactacttccattattgcaggctgtatataccacaatctttccttccatcttaattatctttttaggtttataaggtttggattgccgtctgctcttagttgattctccatcttctcctttactagcagatcctgtaaagaatatgctcccatcttctgcaactaaaagggcgtgagagccatcgtgtccaactgagaagtgtactatctttggagattttgtaattggtagctcaacccattttcctgctgaaggaccaccttgtttgattccaagactctggtatttgccagtgtaatatatctttccatttgctgttttcattagcgcaaactctcgtcctgcaccaagaattgctgactcctcatcaaatcctgtacttataatatgcaagtccttttccagatcgaatagtgagataccacaggcatgtaagcattttctagccagtttaagttgcaattcttgctgtagaacaggttcagtgcttgtggcaaatattctgacaacaaagccatcatctcttgaagcagctatctgattaatatattctccatcagtgaataaaatattttgaccttcagtgtggcaatctggtaacatcacagtaccatcttgctccagtgtttcagggcttatccttatggctgtcatgctgtggttattcacatctctatataataaataaccctgagcataccctaaccaagactttttttcttttctgtttctaatacgggatgtagaattgtatatatggcccctaactgttccactgtatccagagcctattttatataatccatccttgcataatagataaagaaaaaatccatcattctgaagtagacattggtcatcttcatcaacagatatttcttttaatggccacttgtgcattaaagctgctttcttaatgccattactaaaccagtcctgaatttgaatttttcccaccaaaactgcttgtacacttctctgtagcgaatttagaattgttggcacctgaatagtttggcaagcatggcttccattgttggtgaggatagcagagatggcctgaagtgtccttcctgtttctccccaagaagccaccagactaaagaggcaagcacaggaaagtgctgttaaggactgtcctgtgctgtcattcatcccagtacttcgaacggtgatttccaaaagaagctggaagagagactctaggacctcaggtggctcagactggaggccttctggctgctggccctgcagcacgttgagcagggcttggagactcctgagacacagggatggatgagaaaatcgtgtctctttgatcaattcaaaaacttcacaaaggccaacctcaataatctttggaagcttgatagggggctctttggattcctcttcttcatcactatctgattctccactctgcacagagttcttagatgcggctgccaatgatatttcctttttctgccattccagaacgcaatggcgtacattacagtaaatattgaaagcagaaggattgctatgtagtttgatatctggtatgattactgtattctctaagttttcagacttgcttcttgtcttcacttttgatttgctcttctgttttcttttcaatttcttcttatttaaaattttcttattcctggaggctgggtgtccagcgctgccgcccccctggtccctgtcattgagcgcagcggtataaatcctccggtagcggtcggccagggcccggcctgacagcagcagctggtagtgaccccgggagtccgcggcgggtagccccagccccagccccgcagcagccacggagccgtcgggaaccggcatgaacagcgcccccggcgccggggaggaagagaaggtggcggctgggtagaatccgtccccgccgagccccgaggaggcggcggcgggggaggcagtcgctgcgcacatcatcatcctcgccgccgccgccgccgccgccgcctcgtccccgcgggccgggcgggcagacacgcgcgcgcacacacagcccttttccaacgacgacggctccggcggcggcctctggctcccgcagcagggagactacaaagacagcgacctccttctcctcctccttcttctcctcctcccccccgcgccgccctcgccgctactggggccgctcatctaaccccgccaccccgggaatgtgaggaggaggcggtgccgccactgccgccgccaccaccgctaccaccgccaccaccgccggggctacccgcaatgggaagctgccg

SEQ ID NO: 17094 - RNA, 9328 nt, Homo sapiens
  source 1..9328: mol_type = other RNA
tcaaaactgaggggcattttcttcttgcggagggtatctggatcaagtgtgtaagagtctgatttagaacgttcccgaggaggatcaagctttgtcttaacaggagcagtacttttttgaggtagatttttatcatgtggtgaggaggagcgtggagaactagcacccgatgggctagacctattggctgggagagtctttggcttaggagatgacaaccgagaacctggtcctggggattcagctctggagctagaaggcatcctcccatcagatttcaatgtctgcaaggtgttatggttgggggataatgacctactgtgggaatctgacctcaactttgcagcatcagattttaagatgagggattcactagcagataaactttctgtgccccttggcttcttctgatcagcagtagtccggctcatacgtccatcaggtttaagcgatctgctgtgtttagaggacagctctgattttcctgatgtagaggctggtttagaagatgttgagatgtttcctcgatcacccttcagtttgtgagacagagatgagagagcagaggcaggcccagctacaccataatttttgtaaatgcgctcacgagaagcaaggttgcgagatggagatttctgaagctgaggctgctggaaggaaaggggctgtccgaacacaaatgggctgtgtactagggaagagggaggttttgcagcttgatcaaagatggaaggagctgggagattgggtcgtgactgaatggaattcaatatggcactcagttggtcacctttgctatttccgagtccataatcaaatccttgggcactgcaacttgcccctttattaaaagcttgcactgagaaagggcttggaggaggagtttgagaattctgatccagaagagcttgttcatcttcatgtcggaggtactggtttccgcctctgtctctagctaaggaccatgcctctccttcatcactctcacagaactctaccatgctgttctgatccagttgcacccatgtcccttcagaattggttacctctcccactgctttgactttgtttcccagaactaacattccaattgggatacctctaaggttagggcagcttctgatgttgtgacctgaaggtcccgtcttcactaccttgtacatgcctggccctcctcgcaagaatggcatatcttgttcttgcattgttgcttcctgtgggcagcaggagtttatgtctttgaaaaagtcatcagtattagttttagattcctgggggaaaaaagctttggaagtccatgaaaatacgtccaaatccctgactccttggctagcattaaagatattgtcaacagggaccagaagactcttgccaagatgttgattaaaagagaggcaccaggcttcagtgtaaccattcatgttagggacatacttctttattgtctcatcattcagcctcagccacacaccatcatcattatggatctcatcaataaaagtgatagttccattgactttcactatgcctatctgctcactctgaagggaagggtggctacggatgcgaagccccgcactgtccttggccacaaattttcgaaccttattaggctgaggttcagactttggtttgaccaactgagttcctggtggtatcatcccttttggtgggtcttttacttttacttccagaccagcatcgatttcaatgccatcaatggtaacatgaagagtgtagagtccaatagcccctggagtccaatttgcacaataagtcccatcattattgacacggatcagcatattctcactgggtctcttaggagttggtgatgcaaaacgtagttcttcaaatgaataattttcataaaccttcatcattgttatggcaatatatcgagcttccttcactatcattggttcatatgaaacatctagctttggtgatgccagccctccataagtcatgtcagtattagaagatgcagctgttactgcaggactgccaggaatcctttgaggtttctttgcttgatcttgttgtaaagacatttttttctgagaaacagggacagctttcacttccaccttcatattgggaacatgtaccacatccccatactggtcttttgtttgaacagttatggtggtaggccaaccacaacgaatatcatccttattcaggatcaaagatgttttctgaggatccgcatatgaatctggctgaagccaccttgcaagccttccaccacttgatcctgggacacaggcaataaaatcatccagaaaagactgttcattgctttggatttggagtggtaaatttccctcaagtgcttctaatatagttggtgaatgagaaagagctagaccctttccaagaattccagaatgggttttgcacacctgcaatgcagcctcctcaagaatttcaaggtcttcttctaattcattaccaataggaagtgctaggtccttcttcatcagagctgctgcacaaaccccaccaagattggctaattctttttccaattggatgactccctcatcaggtccagggctaaattcatatccaattgcaaaacacttaaaaccatagaaagaagctttgtcatctttcacataatctgatgcagtctccaatgaaaaaagggcctcatttcctggcaacaccaaaaccatagtaggccacccagaggatcctgaaaatttctttaattctatccatgaattaagattttcatgaacagatgtcaattttggtccatatcctgaattctgaacagttctgacaggaatcaacaaacgaaggacatcttctgactgtgcagtaccacactgagggtcaaattcgattgtcatccacctcacacattctgggaatgtcaccttgtaatgcatcacacaggcaggtttatacgggtgctcactctctatgacagcatagtgactggaggttgtacaagcagagaggccctgttcaggctggtttcctgtggtgctatctgtcgactgattagggttgaaggcaggcggtgcatacttctgattcaaaatggcaactgacggaagcaattgttggacaaggccaaagacttctacagccaccttgggaatagcagcagctactggtcctatgtaggctataataagggggagcagcatggaaaacagactggaagaactcagcagttctggaatgtcatcagcatccacagcaagagctctgtgcaggaggtccttagaggctcgaacgacagtgcttacaacagacaatgctctgctacagtttttatcttcttcattggctttactcagaagttgggattgtaaatctccatcaaattcactcctatagtagagtatctgtgggatctgtcctctggtttggtttgtgccgttactgctcaagctgcacgtgctgaatgtgaatgtcacaccatcagggcactgaactgtggtcattcctccatctccattggctgtacggcttccatagttcctcaagcgcacagcatatttaacattttcctttaaaggaaccactttgtcaagtctgatctcagctatatcactgggtgagtcatccgttgtgtacgttcctttcactaattccagagatgtccatctgtgggaatgagttgaatctcctgcatgttcactatcatcaaccaacacctctaattcatattcatgaattccacctcctccatagacagagaaaccaaccacaactattccaggtttgtctactgaaaaacagattgcatcaggggacccgttcccagtgttccaacttctgccctgacttgtttttgtaaatcggttagcactagcttttacagagtgaagagaattaagtccatcaacctcagatcccagggctgacgctgtcagttcactgacaatgctggccagtaatccacaggtgttagagacgaggtgggaggagaagagttcattttctctcctcaggctgttcctgactggtagcacaacaatgaccagcattttctccagaacttcacggaagcttgtcatccctgagatattctcttcactctggctgagtttttccatatgtgccaccaaaaggggaaaacgatgaactagtgttgagtcgttctctgtactaacttgtttaacaattgatcgtagtaatacttctccatcatacgcaatcgggaagatggaagtcagcttaacagacgtgtgacacagagctgacataacagctgcaaggagtcggctacttgatgtcttgaagtttgcttcttggatatcctgatccaaacaattcagcagatcacaaaggcaagcccactgtaaggcaggagttgggtagaaagaatgaaagcaggcagtgaaagtattatgacattcctgaaggacagcttctagaagactcaagggttgactgagatatccttgaggatcattatccaatttcaccatgcagtgatcaactccttctgataaaatttttcttaacaaagttctggtttttccaatacactctgctaatttgctagtttcttctacaactgcttttcctgtagctgacactgggtaaatttcacaggtatagacacgcaataacctcagacaacaggtacccacaaagcgcagtctctctaaatctaggagtgtagctgtgaactggaatccttttaatcctctaagttcttcaactcctaagactaaggtggtccagctccagtgaagaatactcaacaatgactcaaaacattccactgagacagttcttgcaaaagacctctttaaaatgtgtacaggttcactggtttgctgtttgccttttgaagcactgccatcactggttggaagtctgtataataactgaggtatctgacccgcattaacatctgtaccattatttgatttctttgaactcttgaactggaaaacaaccccatcatctgtggtaatagatgcctgtccatgagatccacagtcactgctgggtcctgacactcgggcccatgccacataccaccacccagcttgcaggagaacaggctcatcaaacatcattgcatatttttctctagcagcacagtcataagccaatacatcagtctctgcaagaaggtcaccatcagtttcatgatctcctccatcaggacccaattcaaacagcttaattttagcagtatattctcctctacctccaaacagaccaagaccaccaagtaaaatatcagtgtcggcactgaaacgtatagcttctactgaatgggcagaataaccccagcctcctccatgactttcaaacctgtttaccacactataatcttctttagaataaaccttcattactgcttgagtctcttcctctgtacttgcaacacccatttttaagtcctgcatagctgccaaggtatcaagacaacctaaaatgtgcaaagctgcatgagatcgggtagtgagggcccttgatcctgttggtaaggcaagttcaggacttaggatactacatctggactgcatgtctgctgcagagggaagcctggcatcagcaaccaccgcattgtaacaccacagctctctagtatttggtcgaaacctccaaattacatcatatacaggatcaagacacacaccaaatccttgcagatcctcttgttctgagtcattaaaagttttacaactcccatccactttatttatcagaaggcatttaaatggaggaggttctgatatagaagcaggtaccaagcctattatgtgtttactggcaaaaatttctgatgtagcaagtacatgagaattaataagtgcttcatcaattcgtaaaaaagtttggtccccacttgcacctatccaagtagcttttcttccatattttgatccaatgttaggcatgggagctggctttgcattccaatatggcacatccaaaattggtctgcccagttgtcctttagaaaaacttccaaatgtgaagacctgtccatccattaaaagtactgccgtatggttgctgcctgcagtgacttgtgtgctagggcctggcaatgcttgaacaagagtgggacatcccctggagttgacatctccatgtcctagctgcccatgctgcccataaccaaatgtatagacatctccattttccattaaaaccactgaatggtgaaatccacagctgacttggactgcccggagctcacagtcaaatcgcacagagcctggagggtatgttgtgattttgcttgcatccttttcgcctctttctccacttccatctttgtgcttgtcccgtttatgctttagctgtgctggatgggatctgagtctggctagagcctgttctcgatggttcataaaaataggaccagcaaatacaagggggcctcttccttcctctaatctgtgccttctgattacacgttgccgtttttcttcttgtcgtaactgaaggtgttcttcaatgttaaccccgggcactgggacagctaaaagaagatctaaaggtatcatttctttcactgcatcaagaattcctctttgtcttgcctcttgaccatctaactctcttgcacaggccttgcaacatccacacacagcacaaccagattctccggaaccacaaccacagatccctccggggactctgtctggccgtccactactgacacagctggctccataacctgtacagtctccacagacagtgcaaaccatgcactgctccagcttccatttgtgcatgcctggagggcacatcatagacttctcatctttttcatctagttcttcttccaggtcttcatccattgctgttgccatattttcaactccaaaccctttcccaccttggttcatggcaccagtatctcgtccacactgtcctttattatttacaccaaatgtccacacctctccattcttcattaaaacacaagtgtgagctttgcccatagctacctgagttacaaaatggcccttcaaatcagttaccaaacttgaactatcagagtaaatggcatcttttccaaacatgtagagttctccatctttagaaataacagaactacttccattattgcaggctgtatataccacaatctttccttccatcttaattatctttttaggtttataaggtttggattgccgtctgctcttagttgattctccatcttctcctttactagcagatcctgtaaagaatatgctcccatcttctgcaactaaaagggcgtgagagccatcgtgtccaactgagaagtgtactatctttggagattttgtaattggtagctcaacccattttcctgctgaaggaccaccttgtttgattccaagactctggtatttgccagtgtaatatatctttccatttgctgttttcattagcgcaaactctcgtcctgcaccaagaattgctgactcctcatcaaatcctgtacttataatatgcaagtccttttccagatcgaatagtgagataccacaggcatgtaagcattttctagccagtttaagttgcaattcttgctgtagaacaggttcagtgcttgtggcaaatattctgacaacaaagccatcatctcttgaagcagctatctgattaatatattctccatcagtgaataaaatattttgaccttcagtgtggcaatctggtaacatcacagtaccatcttgctccagtgtttcagggcttatccttatggctgtcatgctgtggttattcacatctctatataataaataaccctgagcataccctaaccaagactttttttcttttctgtttctaatacgggatgtagaattgtatatatggcccctaactgttccactgtatccagagcctattttatataatccatccttgcataatagataaagaaaaaatccatcattctgaagtagacattggtcatcttcatcaacagatatttcttttaatggccacttgtgcattaaagctgctttcttaatgccattactaaaccagtcctgaatttgaatttttcccaccaaaactgcttgtacacttctctgtagcgaatttagaattgttggcacctgaatagtttggcaagcatggcttccattgttggtgaggatagcagagatggcctgaagtgtccttcctgtttctccccaagaagccaccagactaaagaggcaagcacaggaaagtgctgttaaggactgtcctgtgctgtcattcatcccagtacttcgaacggtgatttccaaaagaagctggaagagagactctaggacctcaggtggctcagactggaggccttctggctgctggccctgcagcacgttgagcagggcttggagactcctgagacacagggatggatgagaaaatcgtgtctctttgatcaattcaaaaacttcacaaaggccaacctcaataatctttggaagcttgatagggggctctttggattcctcttcttcatcactatctgattctccactctgcacagagttcttagatgcggctgccaatgatatttcctttttctgccattccagaacgcaatggcgtacattacagtaaatattgaaagcagaaggattgctatgtagtttgatatctggtatgattactgtattctctaagttttcagacttgcttcttgtcttcacttttgatttgctcttctgttttcttttcaatttcttcttatttaaaattttcttattcctggaggctgggtgtccagcgctgccgcccccctggtccctgtcattgagcgcagcggtataaatcctccggtagcggtcggccagggcccggcctgacagcagcagctggtagtgaccccgggagtccgcggcgggtagccccagccccagccccgcagcagccacggagccgtcgggaaccggcatgaacagcgcccccggcgccggggaggaagagaaggtggcggctgggtagaatccgtccccgccgagccccgaggaggcggcggcgggggaggcagtcgctgcgcacatcatcatcctcgccgccgccgccgccgccgccgcctcgtccccgcgggccgggcgggcagacacgcgcgcgcacacacagcccttttccaacgacgacggctccggcggcggcctctggctcccgcagcagggagactacaaagacagcgacctccttctcctcctccttcttctcctcctcccccccgcgccgccctcgccgctactggggccgctcatctaaccccgccaccccgggaatgtgaggaggaggcggtgccgccactgccgccgccaccaccgctaccaccgccaccaccgccggggctacccgcaatgggaagctgccg

SEQ ID NO: 17095 - RNA, 9028 nt, Homo sapiens
  source 1..9028: mol_type = other RNA
tcaaaactgaggggcattttcttcttgcggagggtatctggatcaagtgtgtaagagtctgatttagaacgttcccgaggaggatcaagctttgtcttaacaggagcagtacttttttgaggtagatttttatcatgtggtgaggaggagcgtggagaactagcacccgatgggctagacctattggctgggagagtctttggcttaggagatgacaaccgagaacctggtcctggggattcagctctggagctagaaggcatcctcccatcagatttcaatgtctgcaaggtgttatggttgggggataatgacctactgtgggaatctgacctcaactttgcagcatcagattttaagatgagggattcactagcagataaactttctgtgccccttggcttcttctgatcagcagtagtccggctcatacgtccatcaggtttaagcgatctgctgtgtttagaggacagctctgattttcctgatgtagaggctggtttagaagatgttgagatgtttcctcgatcacccttcagtttgtgagacagagatgagagagcagaggcaggcccagctacaccataatttttgtaaatgcgctcacgagaagcaaggttgcgagatggagatttctgaagctgaggctgctggaaggaaaggggctgtccgaacacaaatgggctgtgtactagggaagagggaggttttgcagcttgatcaaagatggaaggagctgggagattgggtcgtgactgaatggaattcaatatggcactcagttggtcacctttgctatttccgagtccataatcaaatccttgggcactgcaacttgcccctttattaaaagcttgcactgagaaagggcttggaggaggagtttgagaattctgatccagaagagcttgttcatcttcatgtcggaggtactggtttccgcctctgtctctagctaaggaccatgcctctccttcatcactctcacagaactctaccatgctgttctgatccagttgcacccatgtcccttcagaattggttacgtcaacagggaccagaagactcttgccaagatgttgattaaaagagaggcaccaggcttcagtgtaaccattcatgttagggacatacttctttattgtctcatcattcagcctcagccacacaccatcatcattatggatctcatcaataaaagtgatagttccattgactttcactatgcctatctgctcactctgaagggaagggtggctacggatgcgaagccccgcactgtccttggccacaaattttcgaaccttattaggctgaggttcagactttggtttgaccaactgagttcctggtggtatcatcccttttggtgggtcttttacttttacttccagaccagcatcgatttcaatgccatcaatggtaacatgaagagtgtagagtccaatagcccctggagtccaatttgcacaataagtcccatcattattgacacggatcagcatattctcactgggtctcttaggagttggtgatgcaaaacgtagttcttcaaatgaataattttcataaaccttcatcattgttatggcaatatatcgagcttccttcactatcattggttcatatgaaacatctagctttggtgatgccagccctccataagtcatgtcagtattagaagatgcagctgttactgcaggactgccaggaatcctttgaggtttctttgcttgatcttgttgtaaagacatttttttctgagaaacagggacagctttcacttccaccttcatattgggaacatgtaccacatccccatactggtcttttgtttgaacagttatggtggtaggccaaccacaacgaatatcatccttattcaggatcaaagatgttttctgaggatccgcatatgaatctggctgaagccaccttgcaagccttccaccacttgatcctgggacacaggcaataaaatcatccagaaaagactgttcattgctttggatttggagtggtaaatttccctcaagtgcttctaatatagttggtgaatgagaaagagctagaccctttccaagaattccagaatgggttttgcacacctgcaatgcagcctcctcaagaatttcaaggtcttcttctaattcattaccaataggaagtgctaggtccttcttcatcagagctgctgcacaaaccccaccaagattggctaattctttttccaattggatgactccctcatcaggtccagggctaaattcatatccaattgcaaaacacttaaaaccatagaaagaagctttgtcatctttcacataatctgatgcagtctccaatgaaaaaagggcctcatttcctggcaacaccaaaaccatagtaggccacccagaggatcctgaaaatttctttaattctatccatgaattaagattttcatgaacagatgtcaattttggtccatatcctgaattctgaacagttctgacaggaatcaacaaacgaaggacatcttctgactgtgcagtaccacactgagggtcaaattcgattgtcatccacctcacacattctgggaatgtcaccttgtaatgcatcacacaggcaggtttatacgggtgctcactctctatgacagcatagtgactggaggttgtacaagcagagaggccctgttcaggctggtttcctgtggtgctatctgtcgactgattagggttgaaggcaggcggtgcatacttctgattcaaaatggcaactgacggaagcaattgttggacaaggccaaagacttctacagccaccttgggaatagcagcagctactggtcctatgtaggctataataagggggagcagcatggaaaacagactggaagaactcagcagttctggaatgtcatcagcatccacagcaagagctctgtgcaggaggtccttagaggctcgaacgacagtgcttacaacagacaatgctctgctacagtttttatcttcttcattggctttactcagaagttgggattgtaaatctccatcaaattcactcctatagtagagtatctgtgggatctgtcctctggtttggtttgtgccgttactgctcaagctgcacgtgctgaatgtgaatgtcacaccatcagggcactgaactgtggtcattcctccatctccattggctgtacggcttccatagttcctcaagcgcacagcatatttaacattttcctttaaaggaaccactttgtcaagtctgatctcagctatatcactgggtgagtcatccgttgtgtacgttcctttcactaattccagagatgtccatctgtgggaatgagttgaatctcctgcatgttcactatcatcaaccaacacctctaattcatattcatgaattccacctcctccatagacagagaaaccaaccacaactattccaggtttgtctactgaaaaacagattgcatcaggggacccgttcccagtgttccaacttctgccctgacttgtttttgtaaatcggttagcactagcttttacagagtgaagagaattaagtccatcaacctcagatcccagggctgacgctgtcagttcactgacaatgctggccagtaatccacaggtgttagagacgaggtgggaggagaagagttcattttctctcctcaggctgttcctgactggtagcacaacaatgaccagcattttctccagaacttcacggaagcttgtcatccctgagatattctcttcactctggctgagtttttccatatgtgccaccaaaaggggaaaacgatgaactagtgttgagtcgttctctgtactaacttgtttaacaattgatcgtagtaatacttctccatcatacgcaatcgggaagatggaagtcagcttaacagacgtgtgacacagagctgacataacagctgcaaggagtcggctacttgatgtcttgaagtttgcttcttggatatcctgatccaaacaattcagcagatcacaaaggcaagcccactgtaaggcaggagttgggtagaaagaatgaaagcaggcagtgaaagtattatgacattcctgaaggacagcttctagaagactcaagggttgactgagatatccttgaggatcattatccaatttcaccatgcagtgatcaactccttctgataaaatttttcttaacaaagttctggtttttccaatacactctgctaatttgctagtttcttctacaactgcttttcctgtagctgacactgggtaaatttcacaggtatagacacgcaataacctcagacaacaggtacccacaaagcgcagtctctctaaatctaggagtgtagctgtgaactggaatccttttaatcctctaagttcttcaactcctaagactaaggtggtccagctccagtgaagaatactcaacaatgactcaaaacattccactgagacagttcttgcaaaagacctctttaaaatgtgtacaggttcactggtttgctgtttgccttttgaagcactgccatcactggttggaagtctgtataataactgaggtatctgacccgcattaacatctgtaccattatttgatttctttgaactcttgaactggaaaacaaccccatcatctgtggtaatagatgcctgtccatgagatccacagtcactgctgggtcctgacactcgggcccatgccacataccaccacccagcttgcaggagaacaggctcatcaaacatcattgcatatttttctctagcagcacagtcataagccaatacatcagtctctgcaagaaggtcaccatcagtttcatgatctcctccatcaggacccaattcaaacagcttaattttagcagtatattctcctctacctccaaacagaccaagaccaccaagtaaaatatcagtgtcggcactgaaacgtatagcttctactgaatgggcagaataaccccagcctcctccatgactttcaaacctgtttaccacactataatcttctttagaataaaccttcattactgcttgagtctcttcctctgtacttgcaacacccatttttaagtcctgcatagctgccaaggtatcaagacaacctaaaatgtgcaaagctgcatgagatcgggtagtgagggcccttgatcctgttggtaaggcaagttcaggacttaggatactacatctggactgcatgtctgctgcagagggaagcctggcatcagcaaccaccgcattgtaacaccacagctctctagtatttggtcgaaacctccaaattacatcatatacaggatcaagacacacaccaaatccttgcagatcctcttgttctgagtcattaaaagttttacaactcccatccactttatttatcagaaggcatttaaatggaggaggttctgatatagaagcaggtaccaagcctattatgtgtttactggcaaaaatttctgatgtagcaagtacatgagaattaataagtgcttcatcaattcgtaaaaaagtttggtccccacttgcacctatccaagtagcttttcttccatattttgatccaatgttaggcatgggagctggctttgcattccaatatggcacatccaaaattggtctgcccagttgtcctttagaaaaacttccaaatgtgaagacctgtccatccattaaaagtactgccgtatggttgctgcctgcagtgacttgtgtgctagggcctggcaatgcttgaacaagagtgggacatcccctggagttgacatctccatgtcctagctgcccatgctgcccataaccaaatgtatagacatctccattttccattaaaaccactgaatggtgaaatccacagctgacttggactgcccggagctcacagtcaaatcgcacagagcctggagggtatgttgtgattttgcttgcatccttttcgcctctttctccacttccatctttgtgcttgtcccgtttatgctttagctgtgctggatgggatctgagtctggctagagcctgttctcgatggttcataaaaataggaccagcaaatacaagggggcctcttccttcctctaatctgtgccttctgattacacgttgccgtttttcttcttgtcgtaactgaaggtgttcttcaatgttaaccccgggcactgggacagctaaaagaagatctaaaggtatcatttctttcactgcatcaagaattcctctttgtcttgcctcttgaccatctaactctcttgcacaggccttgcaacatccacacacagcacaaccagattctccggaaccacaaccacagatccctccggggactctgtctggccgtccactactgacacagctggctccataacctgtacagtctccacagacagtgcaaaccatgcactgctccagcttccatttgtgcatgcctggagggcacatcatagacttctcatctttttcatctagttcttcttccaggtcttcatccattgctgttgccatattttcaactccaaaccctttcccaccttggttcatggcaccagtatctcgtccacactgtcctttattatttacaccaaatgtccacacctctccattcttcattaaaacacaagtgtgagctttgcccatagctacctgagttacaaaatggcccttcaaatcagttaccaaacttgaactatcagagtaaatggcatcttttccaaacatgtagagttctccatctttagaaataacagaactacttccattattgcaggctgtatataccacaatctttccttccatcttaattatctttttaggtttataaggtttggattgccgtctgctcttagttgattctccatcttctcctttactagcagatcctgtaaagaatatgctcccatcttctgcaactaaaagggcgtgagagccatcgtgtccaactgagaagtgtactatctttggagattttgtaattggtagctcaacccattttcctgctgaaggaccaccttgtttgattccaagactctggtatttgccagtgtaatatatctttccatttgctgttttcattagcgcaaactctcgtcctgcaccaagaattgctgactcctcatcaaatcctgtacttataatatgcaagtccttttccagatcgaatagtgagataccacaggcatgtaagcattttctagccagtttaagttgcaattcttgctgtagaacaggttcagtgcttgtggcaaatattctgacaacaaagccatcatctcttgaagcagctatctgattaatatattctccatcagtgaataaaatattttgaccttcagtgtggcaatctggtaacatcacagtaccatcttgctccagtgtttcagggcttatccttatggctgtcatgctgtggttattcacatctctatataataaataaccctgagcataccctaaccaagactttttttcttttctgtttctaatacgggatgtagaattgtatatatggcccctaactgttccactgtatccagagcctattttatataatccatccttgcataatagataaagaaaaaatccatcattctgaagtagacattggtcatcttcatcaacagatatttcttttaatggccacttgtgcattaaagctgctttcttaatgccattactaaaccagtcctgaatttgaatttttcccaccaaaactgcttgtacacttctctgtagcgaatttagaattgttggcacctgaatagtttggcaagcatggcttccattgttggtgaggatagcagagatggcctgaagtgtccttcctgtttctccccaagaagccaccagactaaagaggcaagcacaggaaagtgctgttaaggactgtcctgtgctgtcattcatcccagtacttcgaacggtgatttccaaaagaagctggaagagagactctaggacctcaggtggctcagactggaggccttctggctgctggccctgcagcacgttgagcagggcttggagactcctgagacacagggatggatgagaaaatcgtgtctctttgatcaattcaaaaacttcacaaaggccaacctcaataatctttggaagcttgatagggggctctttggattcctcttcttcatcactatctgattctccactctgcacagagttcttagatgcggctgccaatgatatttcctttttctgccattccagaacgcaatggcgtacattacagtaaatattgaaagcagaaggattgctatgtagtttgatatctggtatgattactgtattctctaagttttcagacttgcttcttgtcttcacttttgatttgctcttctgttttcttttcaatttcttcttatttaaaattttcttattcctggaggctgggtgtccagcgctgccgcccccctggtccctgtcattgagcgcagcggtataaatcctccggtagcggtcggccagggcccggcctgacagcagcagctggtagtgaccccgggagtccgcggcgggtagccccagccccagccccgcagcagccacggagccgtcgggaaccggcatgaacagcgcccccggcgccggggaggaagagaaggtggcggctgggtagaatccgtccccgccgagccccgaggaggcggcggcgggggaggcagtcgctgcgcacatcatcatcctcgccgccgccgccgccgccgccgcctcgtccccgcgggccgggcgggcagacacgcgcgcgcacacacagcccttttccaacgacgacggctccggcggcggcctctggctcccgcagcagggagactacaaagacagcgacctccttctcctcctccttcttctcctcctcccccccgcgccgccctcgccgctactggggccgctcatctaaccccgccaccccgggaatgtgaggaggaggcggtgccgccactgccgccgccaccaccgctaccaccgccaccaccgccggggctacccgcaatgggaagctgccg

SEQ ID NO: 17096 - RNA, 8962 nt, Homo sapiens
  source 1..8962: mol_type = other RNA
tcaaaactgaggggcattttcttcttgcggagggtatctggatcaagtgtgtaagagtctgatttagaacgttcccgaggaggatcaagctttgtcttaacaggagcagtacttttttgaggtagatttttatcatgtggtgaggaggagcgtggagaactagcacccgatgggctagacctattggctgggagagtctttggcttaggagatgacaaccgagaacctggtcctggggattcagctctggagctagaaggcatcctcccatcagatttcaatgtctgcaaggtgttatggttgggggataatgacctactgtgggaatctgacctcaactttgcagcatcagattttaagatgagggattcactagcagataaactttctgtgccccttggcttcttctgatcagcagtagtccggctcatacgtccatcaggtttaagcgatctgctgtgtttagaggacagctctgattttcctgatgtagaggctggtttagaagatgttgagatgtttcctcgatcacctttgctatttccgagtccataatcaaatccttgggcactgcaacttgcccctttattaaaagcttgcactgagaaagggcttggaggaggagtttgagaattctgatccagaagagcttgttcatcttcatgtcggaggtactggtttccgcctctgtctctagctaaggaccatgcctctccttcatcactctcacagaactctaccatgctgttctgatccagttgcacccatgtcccttcagaattggttacctctcccactgctttgactttgtttcccagaactaacattccaattgggatacctctaaggttagggcagcttctgatgttgtgacctgaaggtcccgtcttcactaccttgtacatgcctggccctcctcgcaagaatggcatatcttgttcttgcattgttgcttcctgtgggcagcaggagtttatgtctttgaaaaagtcatcagtattagttttagattcctgggggaaaaaagctttggaagtccatgaaaatacgtccaaatccctgactccttggctagcattaaagatattgtcaacagggaccagaagactcttgccaagatgttgattaaaagagaggcaccaggcttcagtgtaaccattcatgttagggacatacttctttattgtctcatcattcagcctcagccacacaccatcatcattatggatctcatcaataaaagtgatagttccattgactttcactatgcctatctgctcactctgaagggaagggtggctacggatgcgaagccccgcactgtccttggccacaaattttcgaaccttattaggctgaggttcagactttggtttgaccaactgagttcctggtggtatcatcccttttggtgggtcttttacttttacttccagaccagcatcgatttcaatgccatcaatggtaacatgaagagtgtagagtccaatagcccctggagtccaatttgcacaataagtcccatcattattgacacggatcagcatattctcactgggtctcttaggagttggtgatgcaaaacgtagttcttcaaatgaataattttcataaaccttcatcattgttatggcaatatatcgagcttccttcactatcattggttcatatgaaacatctagctttggtgatgccagccctccataagtcatgtcagtattagaagatgcagctgttactgcaggactgccaggaatcctttgaggtttctttgcttgatcttgttgtaaagacatttttttctgagaaacagggacagctttcacttccaccttcatattgggaacatgtaccacatccccatactggtcttttgtttgaacagttatggtggtaggccaaccacaacgaatatcatccttattcaggatcaaagatgttttctgaggatccgcatatgaatctggctgaagccaccttgcaagccttccaccacttgatcctgggacacaggcaataaaatcatccagaaaagactgttcattgctttggatttggagtggtaaatttccctcaagtgcttctaatatagttggtgaatgagaaagagctagaccctttccaagaattccagaatgggttttgcacacctgcaatgcagcctcctcaagaatttcaaggtcttcttctaattcattaccaataggaagtgctaggtccttcttcatcagagctgctgcacaaaccccaccaagattggctaattctttttccaattggatgactccctcatcaggtccagggctaaattcatatccaattgcaaaacacttaaaaccatagaaagaagctttgtcatctttcacataatctgatgcagtctccaatgaaaaaagggcctcatttcctggcaacaccaaaaccatagtaggccacccagaggatcctgaaaatttctttaattctatccatgaattaagattttcatgaacagatgtcaattttggtccatatcctgaattctgaacagttctgacaggaatcaacaaacgaaggacatcttctgactgtgcagtaccacactgagggtcaaattcgattgtcatccacctcacacattctgggaatgtcaccttgtaatgcatcacacaggcaggtttatacgggtgctcactctctatgacagcatagtgactggaggttgtacaagcagagaggccctgttcaggctggtttcctgtggtgctatctgtcgactgattagggttgaaggcaggcggtgcatacttctgattcaaaatggcaactgacggaagcaattgttggacaaggccaaagacttctacagccaccttgggaatagcagcagctactggtcctatgtaggctataataagggggagcagcatggaaaacagactggaagaactcagcagttctggaatgtcatcagcatccacagcaagagctctgtgcaggaggtccttagaggctcgaacgacagtgcttacaacagacaatgctctgctacagtttttatcttcttcattggctttactcagaagttgggattgtaaatctccatcaaattcactcctatagtagagtatctgtgggatctgtcctctggtttggtttgtgccgttactgctcaagctgcacgtgctgaatgtgaatgtcacaccatcagggcactgaactgtggtcattcctccatctccattggctgtacggcttccatagttcctcaagcgcacagcatatttaacattttcctttaaaggaaccactttgtcaagtctgatctcagctatatcactgggtgagtcatccgttgtgtacgttcctttcactaattccagagatgtccatctgtgggaatgagttgaatctcctgcatgttcactatcatcaaccaacacctctaattcatattcatgaattccacctcctccatagacagagaaaccaaccacaactattccaggtttgtctactgaaaaacagattgcatcaggggacccgttcccagtgttccaacttctgccctgacttgtttttgtaaatcggttagcactagcttttacagagtgaagagaattaagtccatcaacctcagatcccagggctgacgctgtcagttcactgacaatgctggccagtaatccacaggtgttagagacgaggtgggaggagaagagttcattttctctcctcaggctgttcctgactggtagcacaacaatgaccagcattttctccagaacttcacggaagcttgtcatccctgagatattctcttcactctggctgagtttttccatatgtgccaccaaaaggggaaaacgatgaactagtgttgagtcgttctctgtactaacttgtttaacaattgatcgtagtaatacttctccatcatacgcaatcgggaagatggaagtcagcttaacagacgtgtgacacagagctgacataacagctgcaaggagtcggctacttgatgtcttgaagtttgcttcttggatatcctgatccaaacaattcagcagatcacaaaggcaagcccactgtaaggcaggagttgggtagaaagaatgaaagcaggcagtgaaagtattatgacattcctgaaggacagcttctagaagactcaagggttgactgagatatccttgaggatcattatccaatttcaccatgcagtgatcaactccttctgataaaatttttcttaacaaagttctggtttttccaatacactctgctaatttgctagtttcttctacaactgcttttcctgtagctgacactgggtaaatttcacaggtatagacacgcaataacctcagacaacaggtacccacaaagcgcagtctctctaaatctaggagtgtagctgtgaactggaatccttttaatcctctaagttcttcaactcctaagactaaggtggtccagctccagtgaagaatactcaacaatgactcaaaacattccactgagacagttcttgcaaaagacctctttaaaatgtgtacaggttcactggtttgctgtttgccttttgaagcactgccatcactggttggaagtctgtataataactgaggtatctgacccgcattaacatctgtaccattatttgatttctttgaactcttgaactggaaaacaaccccatcatctgtggtaatagatgcctgtccatgagatccacagtcactgctgggtcctgacactcgggcccatgccacataccaccacccagcttgcaggagaacaggctcatcaaacatcattgcatatttttctctagcagcacagtcataagccaatacatcagtctctgcaagaaggtcaccatcagtttcatgatctcctccatcaggacccaattcaaacagcttaattttagcagtatattctcctctacctccaaacagaccaagaccaccaagtaaaatatcagtgtcggcactgaaacgtatagcttctactgaatgggcagaataaccccagcctcctccatgactttcaaacctgtttaccacactataatcttctttagaataaaccttcattactgcttgagtctcttcctctgtacttgcaacacccatttttaagtcctgcatagctgccaaggtatcaagacaacctaaaatgtgcaaagctgcatgagatcgggtagtgagggcccttgatcctgttggtaaggcaagttcaggacttaggatactacatctggactgcatgtctgctgcagagggaagcctggcatcagcaaccaccgcattgtaacaccacagctctctagtatttggtcgaaacctccaaattacatcatatacaggatcaagacacacaccaaatccttgcagatcctcttgttctgagtcattaaaagttttacaactcccatccactttatttatcagaaggcatttaaatggaggaggttctgatatagaagcaggtaccaagcctattatgtgtttactggcaaaaatttctgatgtagcaagtacatgagaattaataagtgcttcatcaattcgtaaaaaagtttggtccccacttgcacctatccaagtagcttttcttccatattttgatccaatgttaggcatgggagctggctttgcattccaatatggcacatccaaaattggtctgcccagttgtcctttagaaaaacttccaaatgtgaagacctgtccatccattaaaagtactgccgtatggttgctgcctgcagtgacttgtgtgctagggcctggcaatgcttgaacaagagtgggacatcccctggagttgacatctccatgtcctagctgcccatgctgcccataaccaaatgtatagacatctccattttccattaaaaccactgaatggtgaaatccacagctgacttggactgcccggagctcacagtcaaatcgcacagagcctggagggtatgttgtgattttgcttgcatccttttcgcctctttctccacttccatctcttccttcctctaatctgtgccttctgattacacgttgccgtttttcttcttgtcgtaactgaaggtgttcttcaatgttaaccccgggcactgggacagctaaaagaagatctaaaggtatcatttctttcactgcatcaagaattcctctttgtcttgcctcttgaccatctaactctcttgcacaggccttgcaacatccacacacagcacaaccagattctccggaaccacaaccacagatccctccggggactctgtctggccgtccactactgacacagctggctccataacctgtacagtctccacagacagtgcaaaccatgcactgctccagcttccatttgtgcatgcctggagggcacatcatagacttctcatctttttcatctagttcttcttccaggtcttcatccattgctgttgccatattttcaactccaaaccctttcccaccttggttcatggcaccagtatctcgtccacactgtcctttattatttacaccaaatgtccacacctctccattcttcattaaaacacaagtgtgagctttgcccatagctacctgagttacaaaatggcccttcaaatcagttaccaaacttgaactatcagagtaaatggcatcttttccaaacatgtagagttctccatctttagaaataacagaactacttccattattgcaggctgtatataccacaatctttccttccatcttaattatctttttaggtttataaggtttggattgccgtctgctcttagttgattctccatcttctcctttactagcagatcctgtaaagaatatgctcccatcttctgcaactaaaagggcgtgagagccatcgtgtccaactgagaagtgtactatctttggagattttgtaattggtagctcaacccattttcctgctgaaggaccaccttgtttgattccaagactctggtatttgccagtgtaatatatctttccatttgctgttttcattagcgcaaactctcgtcctgcaccaagaattgctgactcctcatcaaatcctgtacttataatatgcaagtccttttccagatcgaatagtgagataccacaggcatgtaagcattttctagccagtttaagttgcaattcttgctgtagaacaggttcagtgcttgtggcaaatattctgacaacaaagccatcatctcttgaagcagctatctgattaatatattctccatcagtgaataaaatattttgaccttcagtgtggcaatctggtaacatcacagtaccatcttgctccagtgtttcagggcttatccttatggctgtcatgctgtggttattcacatctctatataataaataaccctgagcataccctaaccaagactttttttcttttctgtttctaatacgggatgtagaattgtatatatggcccctaactgttccactgtatccagagcctattttatataatccatccttgcataatagataaagaaaaaatccatcattctgaagtagacattggtcatcttcatcaacagatatttcttttaatggccacttgtgcattaaagctgctttcttaatgccattactaaaccagtcctgaatttgaatttttcccaccaaaactgcttgtacacttctctgtagcgaatttagaattgttggcacctgaatagtttggcaagcatggcttccattgttggtgaggatagcagagatggcctgaagtgtccttcctgtttctccccaagaagccaccagactaaagaggcaagcacaggaaagtgctgttaaggactgtcctgtgctgtcattcatcccagtacttcgaacggtgatttccaaaagaagctggaagagagactctaggacctcaggtggctcagactggaggccttctggctgctggccctgcagcacgttgagcagggcttggagactcctgagacacagggatggatgagaaaatcgtgtctctttgatcaattcaaaaacttcacaaaggccaacctcaataatctttggaagcttgatagggggctctttggattcctcttcttcatcactatctgattctccactctgcacagagttcttagatgcggctgccaatgatatttcctttttctgccattccagaacgcaatggcgtacattacagtaaatattgaaagcagaaggattgctatgtagtttgatatctggtatgattactgtattctctaagttttcagacttgcttcttgtcttcacttttgatttgctcttctgttttcttttcaatttcttcttatttaaaattttcttattcctggaggctgggtgtccagcgctgccgcccccctggtccctgtcattgagcgcagcggtataaatcctccggtagcggtcggccagggcccggcctgacagcagcagctggtagtgaccccgggagtccgcggcgggtagccccagccccagccccgcagcagccacggagccgtcgggaaccggcatgaacagcgcccccggcgccggggaggaagagaaggtggcggctgggtagaatccgtccccgccgagccccgaggaggcggcggcgggggaggcagtcgctgcgcacatcatcatcctcgccgccgccgccgccgccgccgcctcgtccccgcgggccgggcgggcagacacgcgcgcgcacacacagcccttttccaacgacgacggctccggcggcggcctctggctcccgcagcagggagactacaaagacagcgacctccttctcctcctccttcttctcctcctcccccccgcgccgccctcgccgctactggggccgctcatctaaccccgccaccccgggaatgtgaggaggaggcggtgccgccactgccgccgccaccaccgctaccaccgccaccaccgccggggctacccgcaatgggaagctgccg

SEQ ID NO: 17097 - RNA, 9070 nt, Homo sapiens
  source 1..9070: mol_type = other RNA
tcaaaactgaggggcattttcttcttgcggagggtatctggatcaagtgtgtaagagtctgatttagaacgttcccgaggaggatcaagctttgtcttaacaggagcagtacttttttgaggtagatttttatcatgtggtgaggaggagcgtggagaactagcacccgatgggctagacctattggctgggagagtctttggcttaggagatgacaaccgagaacctggtcctggggattcagctctggagctagaaggcatcctcccatcagatttcaatgtctgcaaggtgttatggttgggggataatgacctactgtgggaatctgacctcaactttgcagcatcagattttaagatgagggattcactagcagataaactttctgtgccccttggcttcttctgatcagcagtagtccggctcatacgtccatcaggtttaagcgatctgctgtgtttagaggacagctctgattttcctgatgtagaggctggtttagaagatgttgagatgtttcctcgatcacctttgctatttccgagtccataatcaaatccttgggcactgcaacttgcccctttattaaaagcttgcactgagaaagggcttggaggaggagtttgagaattctgatccagaagagcttgttcatcttcatgtcggaggtactggtttccgcctctgtctctagctaaggaccatgcctctccttcatcactctcacagaactctaccatgctgttctgatccagttgcacccatgtcccttcagaattggttacctctcccactgctttgactttgtttcccagaactaacattccaattgggatacctctaaggttagggcagcttctgatgttgtgacctgaaggtcccgtcttcactaccttgtacatgcctggccctcctcgcaagaatggcatatcttgttcttgcattgttgcttcctgtgggcagcaggagtttatgtctttgaaaaagtcatcagtattagttttagattcctgggggaaaaaagctttggaagtccatgaaaatacgtccaaatccctgactccttggctagcattaaagatattgtcaacagggaccagaagactcttgccaagatgttgattaaaagagaggcaccaggcttcagtgtaaccattcatgttagggacatacttctttattgtctcatcattcagcctcagccacacaccatcatcattatggatctcatcaataaaagtgatagttccattgactttcactatgcctatctgctcactctgaagggaagggtggctacggatgcgaagccccgcactgtccttggccacaaattttcgaaccttattaggctgaggttcagactttggtttgaccaactgagttcctggtggtatcatcccttttggtgggtcttttacttttacttccagaccagcatcgatttcaatgccatcaatggtaacatgaagagtgtagagtccaatagcccctggagtccaatttgcacaataagtcccatcattattgacacggatcagcatattctcactgggtctcttaggagttggtgatgcaaaacgtagttcttcaaatgaataattttcataaaccttcatcattgttatggcaatatatcgagcttccttcactatcattggttcatatgaaacatctagctttggtgatgccagccctccataagtcatgtcagtattagaagatgcagctgttactgcaggactgccaggaatcctttgaggtttctttgcttgatcttgttgtaaagacatttttttctgagaaacagggacagctttcacttccaccttcatattgggaacatgtaccacatccccatactggtcttttgtttgaacagttatggtggtaggccaaccacaacgaatatcatccttattcaggatcaaagatgttttctgaggatccgcatatgaatctggctgaagccaccttgcaagccttccaccacttgatcctgggacacaggcaataaaatcatccagaaaagactgttcattgctttggatttggagtggtaaatttccctcaagtgcttctaatatagttggtgaatgagaaagagctagaccctttccaagaattccagaatgggttttgcacacctgcaatgcagcctcctcaagaatttcaaggtcttcttctaattcattaccaataggaagtgctaggtccttcttcatcagagctgctgcacaaaccccaccaagattggctaattctttttccaattggatgactccctcatcaggtccagggctaaattcatatccaattgcaaaacacttaaaaccatagaaagaagctttgtcatctttcacataatctgatgcagtctccaatgaaaaaagggcctcatttcctggcaacaccaaaaccatagtaggccacccagaggatcctgaaaatttctttaattctatccatgaattaagattttcatgaacagatgtcaattttggtccatatcctgaattctgaacagttctgacaggaatcaacaaacgaaggacatcttctgactgtgcagtaccacactgagggtcaaattcgattgtcatccacctcacacattctgggaatgtcaccttgtaatgcatcacacaggcaggtttatacgggtgctcactctctatgacagcatagtgactggaggttgtacaagcagagaggccctgttcaggctggtttcctgtggtgctatctgtcgactgattagggttgaaggcaggcggtgcatacttctgattcaaaatggcaactgacggaagcaattgttggacaaggccaaagacttctacagccaccttgggaatagcagcagctactggtcctatgtaggctataataagggggagcagcatggaaaacagactggaagaactcagcagttctggaatgtcatcagcatccacagcaagagctctgtgcaggaggtccttagaggctcgaacgacagtgcttacaacagacaatgctctgctacagtttttatcttcttcattggctttactcagaagttgggattgtaaatctccatcaaattcactcctatagtagagtatctgtgggatctgtcctctggtttggtttgtgccgttactgctcaagctgcacgtgctgaatgtgaatgtcacaccatcagggcactgaactgtggtcattcctccatctccattggctgtacggcttccatagttcctcaagcgcacagcatatttaacattttcctttaaaggaaccactttgtcaagtctgatctcagctatatcactgggtgagtcatccgttgtgtacgttcctttcactaattccagagatgtccatctgtgggaatgagttgaatctcctgcatgttcactatcatcaaccaacacctctaattcatattcatgaattccacctcctccatagacagagaaaccaaccacaactattccaggtttgtctactgaaaaacagattgcatcaggggacccgttcccagtgttccaacttctgccctgacttgtttttgtaaatcggttagcactagcttttacagagtgaagagaattaagtccatcaacctcagatcccagggctgacgctgtcagttcactgacaatgctggccagtaatccacaggtgttagagacgaggtgggaggagaagagttcattttctctcctcaggctgttcctgactggtagcacaacaatgaccagcattttctccagaacttcacggaagcttgtcatccctgagatattctcttcactctggctgagtttttccatatgtgccaccaaaaggggaaaacgatgaactagtgttgagtcgttctctgtactaacttgtttaacaattgatcgtagtaatacttctccatcatacgcaatcgggaagatggaagtcagcttaacagacgtgtgacacagagctgacataacagctgcaaggagtcggctacttgatgtcttgaagtttgcttcttggatatcctgatccaaacaattcagcagatcacaaaggcaagcccactgtaaggcaggagttgggtagaaagaatgaaagcaggcagtgaaagtattatgacattcctgaaggacagcttctagaagactcaagggttgactgagatatccttgaggatcattatccaatttcaccatgcagtgatcaactccttctgataaaatttttcttaacaaagttctggtttttccaatacactctgctaatttgctagtttcttctacaactgcttttcctgtagctgacactgggtaaatttcacaggtatagacacgcaataacctcagacaacaggtacccacaaagcgcagtctctctaaatctaggagtgtagctgtgaactggaatccttttaatcctctaagttcttcaactcctaagactaaggtggtccagctccagtgaagaatactcaacaatgactcaaaacattccactgagacagttcttgcaaaagacctctttaaaatgtgtacaggttcactggtttgctgtttgccttttgaagcactgccatcactggttggaagtctgtataataactgaggtatctgacccgcattaacatctgtaccattatttgatttctttgaactcttgaactggaaaacaaccccatcatctgtggtaatagatgcctgtccatgagatccacagtcactgctgggtcctgacactcgggcccatgccacataccaccacccagcttgcaggagaacaggctcatcaaacatcattgcatatttttctctagcagcacagtcataagccaatacatcagtctctgcaagaaggtcaccatcagtttcatgatctcctccatcaggacccaattcaaacagcttaattttagcagtatattctcctctacctccaaacagaccaagaccaccaagtaaaatatcagtgtcggcactgaaacgtatagcttctactgaatgggcagaataaccccagcctcctccatgactttcaaacctgtttaccacactataatcttctttagaataaaccttcattactgcttgagtctcttcctctgtacttgcaacacccatttttaagtcctgcatagctgccaaggtatcaagacaacctaaaatgtgcaaagctgcatgagatcgggtagtgagggcccttgatcctgttggtaaggcaagttcaggacttaggatactacatctggactgcatgtctgctgcagagggaagcctggcatcagcaaccaccgcattgtaacaccacagctctctagtatttggtcgaaacctccaaattacatcatatacaggatcaagacacacaccaaatccttgcagatcctcttgttctgagtcattaaaagttttacaactcccatccactttatttatcagaaggcatttaaatggaggaggttctgatatagaagcaggtaccaagcctattatgtgtttactggcaaaaatttctgatgtagcaagtacatgagaattaataagtgcttcatcaattcgtaaaaaagtttggtccccacttgcacctatccaagtagcttttcttccatattttgatccaatgttaggcatgggagctggctttgcattccaatatggcacatccaaaattggtctgcccagttgtcctttagaaaaacttccaaatgtgaagacctgtccatccattaaaagtactgccgtatggttgctgcctgcagtgacttgtgtgctagggcctggcaatgcttgaacaagagtgggacatcccctggagttgacatctccatgtcctagctgcccatgctgcccataaccaaatgtatagacatctccattttccattaaaaccactgaatggtgaaatccacagctgacttggactgcccggagctcacagtcaaatcgcacagagcctggagggtatgttgtgattttgcttgcatccttttcgcctctttctccacttccatctttgtgcttgtcccgtttatgctttagctgtgctggatgggatctgagtctggctagagcctgttctcgatggttcataaaaataggaccagcaaatacaagggggcctcttccttcctctaatctgtgccttctgattacacgttgccgtttttcttcttgtcgtaactgaaggtgttcttcaatgttaaccccgggcactgggacagctaaaagaagatctaaaggtatcatttctttcactgcatcaagaattcctctttgtcttgcctcttgaccatctaactctcttgcacaggccttgcaacatccacacacagcacaaccagattctccggaaccacaaccacagatccctccggggactctgtctggccgtccactactgacacagctggctccataacctgtacagtctccacagacagtgcaaaccatgcactgctccagcttccatttgtgcatgcctggagggcacatcatagacttctcatctttttcatctagttcttcttccaggtcttcatccattgctgttgccatattttcaactccaaaccctttcccaccttggttcatggcaccagtatctcgtccacactgtcctttattatttacaccaaatgtccacacctctccattcttcattaaaacacaagtgtgagctttgcccatagctacctgagttacaaaatggcccttcaaatcagttaccaaacttgaactatcagagtaaatggcatcttttccaaacatgtagagttctccatctttagaaataacagaactacttccattattgcaggctgtatataccacaatctttccttccatcttaattatctttttaggtttataaggtttggattgccgtctgctcttagttgattctccatcttctcctttactagcagatcctgtaaagaatatgctcccatcttctgcaactaaaagggcgtgagagccatcgtgtccaactgagaagtgtactatctttggagattttgtaattggtagctcaacccattttcctgctgaaggaccaccttgtttgattccaagactctggtatttgccagtgtaatatatctttccatttgctgttttcattagcgcaaactctcgtcctgcaccaagaattgctgactcctcatcaaatcctgtacttataatatgcaagtccttttccagatcgaatagtgagataccacaggcatgtaagcattttctagccagtttaagttgcaattcttgctgtagaacaggttcagtgcttgtggcaaatattctgacaacaaagccatcatctcttgaagcagctatctgattaatatattctccatcagtgaataaaatattttgaccttcagtgtggcaatctggtaacatcacagtaccatcttgctccagtgtttcagggcttatccttatggctgtcatgctgtggttattcacatctctatataataaataaccctgagcataccctaaccaagactttttttcttttctgtttctaatacgggatgtagaattgtatatatggcccctaactgttccactgtatccagagcctattttatataatccatccttgcataatagataaagaaaaaatccatcattctgaagtagacattggtcatcttcatcaacagatatttcttttaatggccacttgtgcattaaagctgctttcttaatgccattactaaaccagtcctgaatttgaatttttcccaccaaaactgcttgtacacttctctgtagcgaatttagaattgttggcacctgaatagtttggcaagcatggcttccattgttggtgaggatagcagagatggcctgaagtgtccttcctgtttctccccaagaagccaccagactaaagaggcaagcacaggaaagtgctgttaaggactgtcctgtgctgtcattcatcccagtacttcgaacggtgatttccaaaagaagctggaagagagactctaggacctcaggtggctcagactggaggccttctggctgctggccctgcagcacgttgagcagggcttggagactcctgagacacagggatggatgagaaaatcgtgtctctttgatcaattcaaaaacttcacaaaggccaacctcaataatctttggaagcttgatagggggctctttggattcctcttcttcatcactatctgattctccactctgcacagagttcttagatgcggctgccaatgatatttcctttttctgccattccagaacgcaatggcgtacattacagtaaatattgaaagcagaaggattgctatgtagtttgatatctggtatgattactgtattctctaagttttcagacttgcttcttgtcttcacttttgatttgctcttctgttttcttttcaatttcttcttatttaaaattttcttattcctggaggctgggtgtccagcgctgccgcccccctggtccctgtcattgagcgcagcggtataaatcctccggtagcggtcggccagggcccggcctgacagcagcagctggtagtgaccccgggagtccgcggcgggtagccccagccccagccccgcagcagccacggagccgtcgggaaccggcatgaacagcgcccccggcgccggggaggaagagaaggtggcggctgggtagaatccgtccccgccgagccccgaggaggcggcggcgggggaggcagtcgctgcgcacatcatcatcctcgccgccgccgccgccgccgccgcctcgtccccgcgggccgggcgggcagacacgcgcgcgcacacacagcccttttccaacgacgacggctccggcggcggcctctggctcccgcagcagggagactacaaagacagcgacctccttctcctcctccttcttctcctcctcccccccgcgccgccctcgccgctactggggccgctcatctaaccccgccaccccgggaatgtgaggaggaggcggtgccgccactgccgccgccaccaccgctaccaccgccaccaccgccggggctacccgcaatgggaagctgccg

SEQ ID NO: 17098 - RNA, 8887 nt, Homo sapiens
  source 1..8887: mol_type = other RNA
tcaaaactgaggggcattttcttcttgcggagggtatctggatcaagtgtgtaagagtctgatttagaacgttcccgaggaggatcaagctttgtcttaacaggagcagtacttttttgaggtagatttttatcatgtggtgaggaggagcgtggagaactagcacccgatgggctagacctattggctgggagagtctttggcttaggagatgacaaccgagaacctggtcctggggattcagctctggagctagaaggcatcctcccatcagatttcaatgtctgcaaggtgttatggttgggggataatgacctactgtgggaatctgacctcaactttgcagcatcagattttaagatgagggattcactagcagataaactttctgtgccccttggcttcttctgatcagcagtagtccggctcatacgtccatcaggtttaagcgatctgctgtgtttagaggacagctctgattttcctgatgtagaggctggtttagaagatgttgagatgtttcctcgatcacctttgctatttccgagtccataatcaaatccttgggcactgcaacttgcccctttattaaaagcttgcactgagaaagggcttggaggaggagtttgagaattctgatccagaagagcttgttcatcttcatgtcggaggtactggtttccgcctctgtctctagctaaggaccatgcctctccttcatcactctcacagaactctaccatgctgttctgatccagttgcacccatgtcccttcagaattggttacctctcccactgctttgactttgtttcccagaactaacattccaattgggatacctctaaggttagggcagcttctgatgttgtgacctgaaggtcccgtcttcactaccttgtacatgcctggccctcctcgcaagaatggcatatcttgttcttgcattgttgcttcctgtgggcagcaggagtttatgtctttgaaaaagtcatcagtattagttttagattcgtcaacagggaccagaagactcttgccaagatgttgattaaaagagaggcaccaggcttcagtgtaaccattcatgttagggacatacttctttattgtctcatcattcagcctcagccacacaccatcatcattatggatctcatcaataaaagtgatagttccattgactttcactatgcctatctgctcactctgaagggaagggtggctacggatgcgaagccccgcactgtccttggccacaaattttcgaaccttattaggctgaggttcagactttggtttgaccaactgagttcctggtggtatcatcccttttggtgggtcttttacttttacttccagaccagcatcgatttcaatgccatcaatggtaacatgaagagtgtagagtccaatagcccctggagtccaatttgcacaataagtcccatcattattgacacggatcagcatattctcactgggtctcttaggagttggtgatgcaaaacgtagttcttcaaatgaataattttcataaaccttcatcattgttatggcaatatatcgagcttccttcactatcattggttcatatgaaacatctagctttggtgatgccagccctccataagtcatgtcagtattagaagatgcagctgttactgcaggactgccaggaatcctttgaggtttctttgcttgatcttgttgtaaagacatttttttctgagaaacagggacagctttcacttccaccttcatattgggaacatgtaccacatccccatactggtcttttgtttgaacagttatggtggtaggccaaccacaacgaatatcatccttattcaggatcaaagatgttttctgaggatccgcatatgaatctggctgaagccaccttgcaagccttccaccacttgatcctgggacacaggcaataaaatcatccagaaaagactgttcattgctttggatttggagtggtaaatttccctcaagtgcttctaatatagttggtgaatgagaaagagctagaccctttccaagaattccagaatgggttttgcacacctgcaatgcagcctcctcaagaatttcaaggtcttcttctaattcattaccaataggaagtgctaggtccttcttcatcagagctgctgcacaaaccccaccaagattggctaattctttttccaattggatgactccctcatcaggtccagggctaaattcatatccaattgcaaaacacttaaaaccatagaaagaagctttgtcatctttcacataatctgatgcagtctccaatgaaaaaagggcctcatttcctggcaacaccaaaaccatagtaggccacccagaggatcctgaaaatttctttaattctatccatgaattaagattttcatgaacagatgtcaattttggtccatatcctgaattctgaacagttctgacaggaatcaacaaacgaaggacatcttctgactgtgcagtaccacactgagggtcaaattcgattgtcatccacctcacacattctgggaatgtcaccttgtaatgcatcacacaggcaggtttatacgggtgctcactctctatgacagcatagtgactggaggttgtacaagcagagaggccctgttcaggctggtttcctgtggtgctatctgtcgactgattagggttgaaggcaggcggtgcatacttctgattcaaaatggcaactgacggaagcaattgttggacaaggccaaagacttctacagccaccttgggaatagcagcagctactggtcctatgtaggctataataagggggagcagcatggaaaacagactggaagaactcagcagttctggaatgtcatcagcatccacagcaagagctctgtgcaggaggtccttagaggctcgaacgacagtgcttacaacagacaatgctctgctacagtttttatcttcttcattggctttactcagaagttgggattgtaaatctccatcaaattcactcctatagtagagtatctgtgggatctgtcctctggtttggtttgtgccgttactgctcaagctgcacgtgctgaatgtgaatgtcacaccatcagggcactgaactgtggtcattcctccatctccattggctgtacggcttccatagttcctcaagcgcacagcatatttaacattttcctttaaaggaaccactttgtcaagtctgatctcagctatatcactgggtgagtcatccgttgtgtacgttcctttcactaattccagagatgtccatctgtgggaatgagttgaatctcctgcatgttcactatcatcaaccaacacctctaattcatattcatgaattccacctcctccatagacagagaaaccaaccacaactattccaggtttgtctactgaaaaacagattgcatcaggggacccgttcccagtgttccaacttctgccctgacttgtttttgtaaatcggttagcactagcttttacagagtgaagagaattaagtccatcaacctcagatcccagggctgacgctgtcagttcactgacaatgctggccagtaatccacaggtgttagagacgaggtgggaggagaagagttcattttctctcctcaggctgttcctgactggtagcacaacaatgaccagcattttctccagaacttcacggaagcttgtcatccctgagatattctcttcactctggctgagtttttccatatgtgccaccaaaaggggaaaacgatgaactagtgttgagtcgttctctgtactaacttgtttaacaattgatcgtagtaatacttctccatcatacgcaatcgggaagatggaagtcagcttaacagacgtgtgacacagagctgacataacagctgcaaggagtcggctacttgatgtcttgaagtttgcttcttggatatcctgatccaaacaattcagcagatcacaaaggcaagcccactgtaaggcaggagttgggtagaaagaatgaaagcaggcagtgaaagtattatgacattcctgaaggacagcttctagaagactcaagggttgactgagatatccttgaggatcattatccaatttcaccatgcagtgatcaactccttctgataaaatttttcttaacaaagttctggtttttccaatacactctgctaatttgctagtttcttctacaactgcttttcctgtagctgacactgggtaaatttcacaggtatagacacgcaataacctcagacaacaggtacccacaaagcgcagtctctctaaatctaggagtgtagctgtgaactggaatccttttaatcctctaagttcttcaactcctaagactaaggtggtccagctccagtgaagaatactcaacaatgactcaaaacattccactgagacagttcttgcaaaagacctctttaaaatgtgtacaggttcactggtttgctgtttgccttttgaagcactgccatcactggttggaagtctgtataataactgaggtatctgacccgcattaacatctgtaccattatttgatttctttgaactcttgaactggaaaacaaccccatcatctgtggtaatagatgcctgtccatgagatccacagtcactgctgggtcctgacactcgggcccatgccacataccaccacccagcttgcaggagaacaggctcatcaaacatcattgcatatttttctctagcagcacagtcataagccaatacatcagtctctgcaagaaggtcaccatcagtttcatgatctcctccatcaggacccaattcaaacagcttaattttagcagtatattctcctctacctccaaacagaccaagaccaccaagtaaaatatcagtgtcggcactgaaacgtatagcttctactgaatgggcagaataaccccagcctcctccatgactttcaaacctgtttaccacactataatcttctttagaataaaccttcattactgcttgagtctcttcctctgtacttgcaacacccatttttaagtcctgcatagctgccaaggtatcaagacaacctaaaatgtgcaaagctgcatgagatcgggtagtgagggcccttgatcctgttggtaaggcaagttcaggacttaggatactacatctggactgcatgtctgctgcagagggaagcctggcatcagcaaccaccgcattgtaacaccacagctctctagtatttggtcgaaacctccaaattacatcatatacaggatcaagacacacaccaaatccttgcagatcctcttgttctgagtcattaaaagttttacaactcccatccactttatttatcagaaggcatttaaatggaggaggttctgatatagaagcaggtaccaagcctattatgtgtttactggcaaaaatttctgatgtagcaagtacatgagaattaataagtgcttcatcaattcgtaaaaaagtttggtccccacttgcacctatccaagtagcttttcttccatattttgatccaatgttaggcatgggagctggctttgcattccaatatggcacatccaaaattggtctgcccagttgtcctttagaaaaacttccaaatgtgaagacctgtccatccattaaaagtactgccgtatggttgctgcctgcagtgacttgtgtgctagggcctggcaatgcttgaacaagagtgggacatcccctggagttgacatctccatgtcctagctgcccatgctgcccataaccaaatgtatagacatctccattttccattaaaaccactgaatggtgaaatccacagctgacttggactgcccggagctcacagtcaaatcgcacagagcctggagggtatgttgtgattttgcttgcatccttttcgcctctttctccacttccatctcttccttcctctaatctgtgccttctgattacacgttgccgtttttcttcttgtcgtaactgaaggtgttcttcaatgttaaccccgggcactgggacagctaaaagaagatctaaaggtatcatttctttcactgcatcaagaattcctctttgtcttgcctcttgaccatctaactctcttgcacaggccttgcaacatccacacacagcacaaccagattctccggaaccacaaccacagatccctccggggactctgtctggccgtccactactgacacagctggctccataacctgtacagtctccacagacagtgcaaaccatgcactgctccagcttccatttgtgcatgcctggagggcacatcatagacttctcatctttttcatctagttcttcttccaggtcttcatccattgctgttgccatattttcaactccaaaccctttcccaccttggttcatggcaccagtatctcgtccacactgtcctttattatttacaccaaatgtccacacctctccattcttcattaaaacacaagtgtgagctttgcccatagctacctgagttacaaaatggcccttcaaatcagttaccaaacttgaactatcagagtaaatggcatcttttccaaacatgtagagttctccatctttagaaataacagaactacttccattattgcaggctgtatataccacaatctttccttccatcttaattatctttttaggtttataaggtttggattgccgtctgctcttagttgattctccatcttctcctttactagcagatcctgtaaagaatatgctcccatcttctgcaactaaaagggcgtgagagccatcgtgtccaactgagaagtgtactatctttggagattttgtaattggtagctcaacccattttcctgctgaaggaccaccttgtttgattccaagactctggtatttgccagtgtaatatatctttccatttgctgttttcattagcgcaaactctcgtcctgcaccaagaattgctgactcctcatcaaatcctgtacttataatatgcaagtccttttccagatcgaatagtgagataccacaggcatgtaagcattttctagccagtttaagttgcaattcttgctgtagaacaggttcagtgcttgtggcaaatattctgacaacaaagccatcatctcttgaagcagctatctgattaatatattctccatcagtgaataaaatattttgaccttcagtgtggcaatctggtaacatcacagtaccatcttgctccagtgtttcagggcttatccttatggctgtcatgctgtggttattcacatctctatataataaataaccctgagcataccctaaccaagactttttttcttttctgtttctaatacgggatgtagaattgtatatatggcccctaactgttccactgtatccagagcctattttatataatccatccttgcataatagataaagaaaaaatccatcattctgaagtagacattggtcatcttcatcaacagatatttcttttaatggccacttgtgcattaaagctgctttcttaatgccattactaaaccagtcctgaatttgaatttttcccaccaaaactgcttgtacacttctctgtagcgaatttagaattgttggcacctgaatagtttggcaagcatggcttccattgttggtgaggatagcagagatggcctgaagtgtccttcctgtttctccccaagaagccaccagactaaagaggcaagcacaggaaagtgctgttaaggactgtcctgtgctgtcattcatcccagtacttcgaacggtgatttccaaaagaagctggaagagagactctaggacctcaggtggctcagactggaggccttctggctgctggccctgcagcacgttgagcagggcttggagactcctgagacacagggatggatgagaaaatcgtgtctctttgatcaattcaaaaacttcacaaaggccaacctcaataatctttggaagcttgatagggggctctttggattcctcttcttcatcactatctgattctccactctgcacagagttcttagatgcggctgccaatgatatttcctttttctgccattccagaacgcaatggcgtacattacagtaaatattgaaagcagaaggattgctatgtagtttgatatctggtatgattactgtattctctaagttttcagacttgcttcttgtcttcacttttgatttgctcttctgttttcttttcaatttcttcttatttaaaattttcttattcctggaggctgggtgtccagcgctgccgcccccctggtccctgtcattgagcgcagcggtataaatcctccggtagcggtcggccagggcccggcctgacagcagcagctggtagtgaccccgggagtccgcggcgggtagccccagccccagccccgcagcagccacggagccgtcgggaaccggcatgaacagcgcccccggcgccggggaggaagagaaggtggcggctgggtagaatccgtccccgccgagccccgaggaggcggcggcgggggaggcagtcgctgcgcacatcatcatcctcgccgccgccgccgccgccgccgcctcgtccccgcgggccgggcgggcagacacgcgcgcgcacacacagcccttttccaacgacgacggctccggcggcggcctctggctcccgcagcagggagactacaaagacagcgacctccttctcctcctccttcttctcctcctcccccccgcgccgccctcgccgctactggggccgctcatctaaccccgccaccccgggaatgtgaggaggaggcggtgccgccactgccgccgccaccaccgctaccaccgccaccaccgccggggctacccgcaatgggaagctgccg

SEQ ID NO: 17099 - RNA, 8991 nt, Homo sapiens
  source 1..8991: mol_type = other RNA
tcaaaactgaggggcattttcttcttgcggagggtatctggatcaagtgtgtaagagtctgatttagaacgttcccgaggaggatcaagctttgtcttaacaggagcagtacttttttgaggtagatttttatcatgtggtgaggaggagcgtggagaactagcacccgatgggctagacctattggctgggagagtctttggcttaggagatgacaaccgagaacctggtcctggggattcagctctggagctagaaggcatcctcccatcagatttcaatgtctgcaaggtgttatggttgggggataatgacctactgtgggaatctgacctcaactttgcagcatcagattttaagatgagggattcactagcagataaactttctgtgccccttggcttcttctgatcagcagtagtccggctcatacgtccatcaggtttaagcgatctgctgtgtttagaggacagctctgattttcctgatgtagaggctggtttagaagatgttgagatgtttcctcgatcacctttgctatttccgagtccataatcaaatccttgggcactgcaacttgcccctttattaaaagcttgcactgagaaagggcttggaggaggagtttgagaattctgatccagaagagcttgttcatcttcatgtcggaggtactggtttccgcctctgtctctagctaaggaccatgcctctccttcatcactctcacagaactctaccatgctgttctgatccagttgcacccatgtcccttcagaattggttacctctcccactgctttgactttgtttcccagaactaacattccaattgggatacctctaaggttagggcagcttctgatgttgtgacctgaaggtcccgtcttcactaccttgtacatgcctggccctcctcgcaagaatggcatatcttgttcttgcattgttgcttcctgtgggcagcaggagtttatgtctttgaaaaagtcatcagtattagttttagattcgtcaacagggaccagaagactcttgccaagatgttgattaaaagagaggcaccaggcttcagtgtaaccattcatgttagggacatacttctttattgtctcatcattcagcctcagccacacaccatcatcattatggatctcatcaataaaagtgatagttccattgactttcactatgcctatctgctcactctgaagggaagggtggctacggatgcgaagccccgcactgtccttggccacaaattttcgaaccttattaggctgaggttcagactttggtttgaccaactgagttcctggtggtatcatcccttttggtgggtcttttacttttacttccagaccagcatcgatttcaatgccatcaatggtaacatgaagagtgtagagtccaatagcccctggagtccaatttgcacaataagtcccatcattattgacacggatcagcatattctcactgggtctcttaggagttggtgatgcaaaacgtagttcttcaaatgaataattttcataaaccttcatcattgttatggcaatatatcgagcttccttcactatcattggttcatatgaaacatctagctttggtgatgccagccctccataagtcatgtcagtattagaagatgcagctgttactgcaggactgccaggaatcctttgaggtttctttgcttgatcttgttgtaaagacatttttttctgagaaacagggacagctttcacttccaccttcatattgggaacatgtaccacatccccatactggtcttttgtttgaacagttatggtggtaggccaaccacaacgaatatcatccttattcaggatcaaagatgttttctgaggatccgcatatgaatctggctgaagccaccttgcaagccttccaccacttgatcctgggacacaggcaataaaatcatccagaaaagactgttcattgctttggatttggagtggtaaatttccctcaagtgcttctaatatagttggtgaatgagaaagagctagaccctttccaagaattccagaatgggttttgcacacctgcaatgcagcctcctcaagaatttcaaggtcttcttctaattcattaccaataggaagtgctaggtccttcttcatcagagctgctgcacaaaccccaccaagattggctaattctttttccaattggatgactccctcatcaggtccagggctaaattcatatccaattgcaaaacacttaaaaccatagaaagaagctttgtcatctttcacataatctgatgcagtctccaatgaaaaaagggcctcatttcctggcaacaccaaaaccatagtaggccacccagaggatcctgaaaatttctttaattctatccatgaattaagattttcatgaacagatgtcaattttggtccatatcctgaattctgaacagttctgacaggaatcaacaaacgaaggacatcttctgactgtgcagtaccacactgagggtcaaattcgattgtcatccacctcacacattctgggaatgtcaccttgtaatgcatcacacaggcaggtttatacgggtgctcactctctatgacagcatagtgactggaggttgtacaagcagagaggccctgttcaggctggtttcctgtggtgctatctgtcgactgattagggttgaaggcaggcggtgcatacttctgattcaaaatggcaactgacggaagcaattgttggacaaggccaaagacttctacagccaccttgggaatagcagcagctactggtcctatgtaggctataataagggggagcagcatggaaaacagactggaagaactcagcagttctggaatgtcatcagcatccacagcaagagctctgtgcaggaggtccttagaggctcgaacgacagtgcttacaacagacaatgctctgctacagtttttatcttcttcattggctttactcagaagttgggattgtaaatctccatcaaattcactcctatagtagagtatctgtgggatctgtcctctggtttggtttgtgccgttactgctcaagctgcacgtgctgaatgtgaatgtcacaccatcagggcactgaactgtggtcattcctccatctccattggctgtacggcttccatagttcctcaagcgcacagcatatttaacattttcctttaaaggaaccactttgtcaagtctgatctcagctatatcactgggtgagtcatccgttgtgtacgttcctttcactaattccagagatgtccatctgtgggaatgagttgaatctcctgcatgttcactatcatcaaccaacacctctaattcatattcatgaattccacctcctccatagacagagaaaccaaccacaactattccaggtttgtctactgaaaaacagattgcatcaggggacccgttcccagtgttccaacttctgccctgacttgtttttgtaaatcggttagcactagcttttacagagtgaagagaattaagtccatcaacctcagatcccagggctgacgctgtcagttcactgacaatgctggccagtaatccacaggtgttagagacgaggtgggaggagaagagttcattttctctcctcaggctgttcctgactggtagcacaacaatgaccagcattttctccagaacttcacggaagcttgtcatccctgagatattctcttcactctggctgagtttttccatatgtgccaccaaaaggggaaaacgatgaactagtgttgagtcgttctctgtactaacttgtttaacaattgatcgtagtaatacttctccatcatacgcaatcgggaagatggaagtcagcttaacagacgtgtgacacagagctgacataacagctgcaaggagtcggctacttgatgtcttgaagtttgcttcttggatatcctgatccaaacaattcagcagatcacaaaggcaagcccactgtaaggcaggagttgggtagaaagaatgaaagcaggcagtgaaagtattatgacattcctgaaggacagcttctagaagactcaagggttgactgagatatccttgaggatcattatccaatttcaccatgcagtgatcaactccttctgataaaatttttcttaacaaagttctggtttttccaatacactctgctaatttgctagtttcttctacaactgcttttcctgtagctgacactgggtaaatttcacaggtatagacacgcaataacctcagacaacaggtacccacaaagcgcagtctctctaaatctaggagtgtagctgtgaactggaatccttttaatcctctaagttcttcaactcctaagactaaggtggtccagctccagtgaagaatactcaacaatgactcaaaacattccactgagacagttcttgcaaaagacctctttaaaatgtgtacaggttcactggtttgctgtttgccttttgaagcactgccatcactggttggaagtctgtataataactgaggtatctgacccgcattaacatctgtaccattatttgatttctttgaactcttgaactggaaaacaaccccatcatctgtggtaatagatgcctgtccatgagatccacagtcactgctgggtcctgacactcgggcccatgccacataccaccacccagcttgcaggagaacaggctcatcaaacatcattgcatatttttctctagcagcacagtcataagccaatacatcagtctctgcaagaaggtcaccatcagtttcatgatctcctccatcaggacccaattcaaacagcttaattttagcagtatattctcctctacctccaaacagaccaagaccaccaagtaaaatatcagtgtcggcactgaaacgtatagcttctactgaatgggcagaataaccccagcctcctccatgactttcaaacctgtttaccacactataatcttctttagaataaaccttcattactgcttgagtctcttcctctgtacttgcaacacccatttttaagtcctgcatagctgccaaggtatcaagacaacctaaaatgtgcaaagctgcatgagatcgggtagtgagggcccttgatcctgttggtaaggcaagttcaggacttaggatactacatctggactgcatgtctgctgcagagggaagcctggcatcagcaaccaccgcattgtaacaccacagctctctagtatttggtcgaaacctccaaattacatcatatacaggatcaagacacacaccaaatccttgcagatcctcttgttctgagtcattaaaagttttacaactcccatccactttatttatcagaaggcatttaaatggaggaggttctgatatagaagcaggtaccaagcctattatgtgtttactggcaaaaatttctgatgtagcaagtacatgagaattaataagtgcttcatcaattcgtaaaaaagtttggtccccacttgcacctatccaagtagcttttcttccatattttgatccaatgttaggcatgggagctggctttgcattccaatatggcacatccaaaattggtctgcccagttgtcctttagaaaaacttccaaatgtgaagacctgtccatccattaaaagtactgccgtatggttgctgcctgcagtgacttgtgtgctagggcctggcaatgcttgaacaagagtgggacatcccctggagttgacatctccatgtcctagctgcccatgctgcccataaccaaatgtatagacatctccattttccattaaaaccactgaatggtgaaatccacagctgacttggactgcccggagctcacagtcaaatcgcacagagcctggagggtatgttgtgattttgcttgcatccttttcgcctctttctccacttccatctttgtgcttgtcccgtttatgctttagctgtgctggatgggatctgagtctggctagagcctgttctcgatggttcataaaaataggaccagcaaatacaagggggcctcttccttcctctaatctgtgccttctgattacacgttgccgtttttcttcttgtcgtaactgaaggtgttcttcaatgttaaccccgggcactgggacagctaaaagaagatctaaaggtatcatttctttcactgcatcaagaattcctctttgtcttgcctcttgaccatctaactctcttgcacaggccttgcaacatccacacacagcacaaccagattctccggaaccacaaccacagatccctccggggactctgtctggccgtccactactgacacagctggctccataacctgtacagtctccacagacagtgcaaaccatgcactgctccagcttccatttgtgcatgcctggagggcacatcatagacttctcatctttttcatctagttcttcttccaggtcttcatccattgctgttgccatattttcaactccaaaccctttcccaccttggttcatggcaccagtatctcgtccacactgtcctttattatttacaccaaatgtccacacctctccattcttcattaaaacacaagtgtgagctttgcccatagctacctgagttacaaaatggcccttcaaatcagttaccaaacttgaactatcagagtaaatggcatcttttccaaacatgtagagttctccatctttagaaataacagaactacttccattattgcaggctgtatataccacaatctttccttccatcttaattatctttttaggtttataaggtttggattgccgtctgctcttagttgattctccatcttctcctttactagcagatcctgtaaagaatatgctcccatcttctgcaactaaaagggcgtgagagccatcgtgtccaactgagaagtgtactatctttggagattttgtaattggtagctcaacccattttcctgctgaaggaccaccttgtttgattccaagactctggtatttgccagtgtaatatatctttccatttgctgttttcattagcgcaaactctcgtcctgcaccaagaattgctgactcctcatcaaatcctgtacttataatatgcaagtccttttccagatcgaatagtgagataccacaggcatgtaagcattttctagccagtttaagttgcaattcttgctgtagaacaggttcagtgcttgtggcaaatattctgacaacaaagccatcatctcttgaagcagctatctgattaatatattctccatcagtgaataaaatattttgaccttcagtgtggcaatctggtaacatcacagtaccatcttgctccagtgtttcagggcttatccttatggctgtcatgctgtggttattcacatctctatataataaataaccctgagcataccctaaccaagactttttttcttttctgtttctaatacgggatgtagaattgtatatatggcccctaactgttccactgtatccagagcctattttatataatccatccttgcataatagataaagaaaaaatccatcattctgaagtagacattggtcatcttcatcaacagatatttcttttaatggccacttgtgcattaaagctgctttcttaatgccattactaaaccagtcctgaatttgaatttttcccaccaaaactgcttgtacacttctctgtagcgaatttagaattgttggcacctgaatagtttggcaagcatggcttccattgttggtgaggatagcagagatggcctgaagtgtccttcctgtttctccccaagaagccaccagactaaagaggcaagcacaggaaagtgctgttaaggactgtcctgtgctgtcattcatcccagtacttcgaacggtgatttccaaaagaagctggaagagagactctaggacctcaggtggctcagactggaggccttctggctgctggccctgcagcacgttgagcagggcttggagactcctgagacacagggatggatgagaaaatcgtgtctctttgatcaattcaaaaacttcacaaaggccaacctcaataatctttggaagcttgatagggggctctttggattcctcttcttcatcactatctgattctccactctgcacagagttcttagatgcggctgccaatgatatttcctttttctgccattccagaacgcaatggcgtacattacagtaaatattgaaagcagaaggattgctatgtagtttgatatctggtatgattactgtattctctaagttttcagacttgcttcttgtcttcacttttgatttgctcttctgttttcttttcaatttcttcttatttaaaattttcttattcctggaggctgggtgtccagcgctgccgcccccctggtccctgtcattgagcgcagcggtataaatcctccggtagcggtcggccagggcccggcctgacagcagcagctggtagtgaccccgggagtccgcggcgggtagccccagccccagccccgcagcagccacggagccgtcgggaaccggcatgaacagcgcccccggcgccggggaggaagagaaggtggcggctgggtagaatccgtccccgccgagccccgaggaggcggcggcgggggaggcagtcgctgcgcacatcatcatcctcgccgccgccgccgccgccgccgcctcgtccccgcgggccgggcgggcagacacgcgcgcgcacacacagcccttttccaacgacgacggctccggcggcggcctctggctcccgcagcagggagactacaaagacagcgacctccttctcctcctccttcttctcctcctcccccccgcgccgccctcgccgctactggggccgctcatctaaccccgccaccccgggaatgtgaggaggaggcggtgccgccactgccgccgccaccaccgctaccaccgccaccaccgccggggctacccgcaatgggaagct

SEQ ID NO: 17100 - RNA, 8938 nt, Homo sapiens
  source 1..8938: mol_type = other RNA
tcaaaactgaggggcattttcttcttgcggagggtatctggatcaagtgtgtaagagtctgatttagaacgttcccgaggaggatcaagctttgtcttaacaggagcagtacttttttgaggtagatttttatcatgtggtgaggaggagcgtggagaactagcacccgatgggctagacctattggctgggagagtctttggcttaggagatgacaaccgagaacctggtcctggggattcagctctggagctagaaggcatcctcccatcagatttcaatgtctgcaaggtgttatggttgggggataatgacctactgtgggaatctgacctcaactttgcagcatcagattttaagatgagggattcactagcagataaactttctgtgccccttggcttcttctgatcagcagtagtccggctcatacgtccatcaggtttaagcgatctgctgtgtttagaggacagctctgattttcctgatgtagaggctggtttagaagatgttgagatgtttcctcgatcacctttgctatttccgagtccataatcaaatccttgggcactgcaacttgcccctttattaaaagcttgcactgagaaagggcttggaggaggagtttgagaattctgatccagaagagcttgttcatcttcatgtcggaggtactggtttccgcctctgtctctagctaaggaccatgcctctccttcatcactctcacagaactctaccatgctgttctgatccagttgcacccatgtcccttcagaattggttacctctcccactgctttgactttgtttcccagaactaacattccaattgggatacctctaaggttagggcagcttctgatgttgtgacctgaaggtcccgtcttcactaccttgtacatgcctggccctcctcgcaagaatggcatatcttgttcttgcattgttgcttcgtcaacagggaccagaagactcttgccaagatgttgattaaaagagaggcaccaggcttcagtgtaaccattcatgttagggacatacttctttattgtctcatcattcagcctcagccacacaccatcatcattatggatctcatcaataaaagtgatagttccattgactttcactatgcctatctgctcactctgaagggaagggtggctacggatgcgaagccccgcactgtccttggccacaaattttcgaaccttattaggctgaggttcagactttggtttgaccaactgagttcctggtggtatcatcccttttggtgggtcttttacttttacttccagaccagcatcgatttcaatgccatcaatggtaacatgaagagtgtagagtccaatagcccctggagtccaatttgcacaataagtcccatcattattgacacggatcagcatattctcactgggtctcttaggagttggtgatgcaaaacgtagttcttcaaatgaataattttcataaaccttcatcattgttatggcaatatatcgagcttccttcactatcattggttcatatgaaacatctagctttggtgatgccagccctccataagtcatgtcagtattagaagatgcagctgttactgcaggactgccaggaatcctttgaggtttctttgcttgatcttgttgtaaagacatttttttctgagaaacagggacagctttcacttccaccttcatattgggaacatgtaccacatccccatactggtcttttgtttgaacagttatggtggtaggccaaccacaacgaatatcatccttattcaggatcaaagatgttttctgaggatccgcatatgaatctggctgaagccaccttgcaagccttccaccacttgatcctgggacacaggcaataaaatcatccagaaaagactgttcattgctttggatttggagtggtaaatttccctcaagtgcttctaatatagttggtgaatgagaaagagctagaccctttccaagaattccagaatgggttttgcacacctgcaatgcagcctcctcaagaatttcaaggtcttcttctaattcattaccaataggaagtgctaggtccttcttcatcagagctgctgcacaaaccccaccaagattggctaattctttttccaattggatgactccctcatcaggtccagggctaaattcatatccaattgcaaaacacttaaaaccatagaaagaagctttgtcatctttcacataatctgatgcagtctccaatgaaaaaagggcctcatttcctggcaacaccaaaaccatagtaggccacccagaggatcctgaaaatttctttaattctatccatgaattaagattttcatgaacagatgtcaattttggtccatatcctgaattctgaacagttctgacaggaatcaacaaacgaaggacatcttctgactgtgcagtaccacactgagggtcaaattcgattgtcatccacctcacacattctgggaatgtcaccttgtaatgcatcacacaggcaggtttatacgggtgctcactctctatgacagcatagtgactggaggttgtacaagcagagaggccctgttcaggctggtttcctgtggtgctatctgtcgactgattagggttgaaggcaggcggtgcatacttctgattcaaaatggcaactgacggaagcaattgttggacaaggccaaagacttctacagccaccttgggaatagcagcagctactggtcctatgtaggctataataagggggagcagcatggaaaacagactggaagaactcagcagttctggaatgtcatcagcatccacagcaagagctctgtgcaggaggtccttagaggctcgaacgacagtgcttacaacagacaatgctctgctacagtttttatcttcttcattggctttactcagaagttgggattgtaaatctccatcaaattcactcctatagtagagtatctgtgggatctgtcctctggtttggtttgtgccgttactgctcaagctgcacgtgctgaatgtgaatgtcacaccatcagggcactgaactgtggtcattcctccatctccattggctgtacggcttccatagttcctcaagcgcacagcatatttaacattttcctttaaaggaaccactttgtcaagtctgatctcagctatatcactgggtgagtcatccgttgtgtacgttcctttcactaattccagagatgtccatctgtgggaatgagttgaatctcctgcatgttcactatcatcaaccaacacctctaattcatattcatgaattccacctcctccatagacagagaaaccaaccacaactattccaggtttgtctactgaaaaacagattgcatcaggggacccgttcccagtgttccaacttctgccctgacttgtttttgtaaatcggttagcactagcttttacagagtgaagagaattaagtccatcaacctcagatcccagggctgacgctgtcagttcactgacaatgctggccagtaatccacaggtgttagagacgaggtgggaggagaagagttcattttctctcctcaggctgttcctgactggtagcacaacaatgaccagcattttctccagaacttcacggaagcttgtcatccctgagatattctcttcactctggctgagtttttccatatgtgccaccaaaaggggaaaacgatgaactagtgttgagtcgttctctgtactaacttgtttaacaattgatcgtagtaatacttctccatcatacgcaatcgggaagatggaagtcagcttaacagacgtgtgacacagagctgacataacagctgcaaggagtcggctacttgatgtcttgaagtttgcttcttggatatcctgatccaaacaattcagcagatcacaaaggcaagcccactgtaaggcaggagttgggtagaaagaatgaaagcaggcagtgaaagtattatgacattcctgaaggacagcttctagaagactcaagggttgactgagatatccttgaggatcattatccaatttcaccatgcagtgatcaactccttctgataaaatttttcttaacaaagttctggtttttccaatacactctgctaatttgctagtttcttctacaactgcttttcctgtagctgacactgggtaaatttcacaggtatagacacgcaataacctcagacaacaggtacccacaaagcgcagtctctctaaatctaggagtgtagctgtgaactggaatccttttaatcctctaagttcttcaactcctaagactaaggtggtccagctccagtgaagaatactcaacaatgactcaaaacattccactgagacagttcttgcaaaagacctctttaaaatgtgtacaggttcactggtttgctgtttgccttttgaagcactgccatcactggttggaagtctgtataataactgaggtatctgacccgcattaacatctgtaccattatttgatttctttgaactcttgaactggaaaacaaccccatcatctgtggtaatagatgcctgtccatgagatccacagtcactgctgggtcctgacactcgggcccatgccacataccaccacccagcttgcaggagaacaggctcatcaaacatcattgcatatttttctctagcagcacagtcataagccaatacatcagtctctgcaagaaggtcaccatcagtttcatgatctcctccatcaggacccaattcaaacagcttaattttagcagtatattctcctctacctccaaacagaccaagaccaccaagtaaaatatcagtgtcggcactgaaacgtatagcttctactgaatgggcagaataaccccagcctcctccatgactttcaaacctgtttaccacactataatcttctttagaataaaccttcattactgcttgagtctcttcctctgtacttgcaacacccatttttaagtcctgcatagctgccaaggtatcaagacaacctaaaatgtgcaaagctgcatgagatcgggtagtgagggcccttgatcctgttggtaaggcaagttcaggacttaggatactacatctggactgcatgtctgctgcagagggaagcctggcatcagcaaccaccgcattgtaacaccacagctctctagtatttggtcgaaacctccaaattacatcatatacaggatcaagacacacaccaaatccttgcagatcctcttgttctgagtcattaaaagttttacaactcccatccactttatttatcagaaggcatttaaatggaggaggttctgatatagaagcaggtaccaagcctattatgtgtttactggcaaaaatttctgatgtagcaagtacatgagaattaataagtgcttcatcaattcgtaaaaaagtttggtccccacttgcacctatccaagtagcttttcttccatattttgatccaatgttaggcatgggagctggctttgcattccaatatggcacatccaaaattggtctgcccagttgtcctttagaaaaacttccaaatgtgaagacctgtccatccattaaaagtactgccgtatggttgctgcctgcagtgacttgtgtgctagggcctggcaatgcttgaacaagagtgggacatcccctggagttgacatctccatgtcctagctgcccatgctgcccataaccaaatgtatagacatctccattttccattaaaaccactgaatggtgaaatccacagctgacttggactgcccggagctcacagtcaaatcgcacagagcctggagggtatgttgtgattttgcttgcatccttttcgcctctttctccacttccatctttgtgcttgtcccgtttatgctttagctgtgctggatgggatctgagtctggctagagcctgttctcgatggttcataaaaataggaccagcaaatacaagggggcctcttccttcctctaatctgtgccttctgattacacgttgccgtttttcttcttgtcgtaactgaaggtgttcttcaatgttaaccccgggcactgggacagctaaaagaagatctaaaggtatcatttctttcactgcatcaagaattcctctttgtcttgcctcttgaccatctaactctcttgcacaggccttgcaacatccacacacagcacaaccagattctccggaaccacaaccacagatccctccggggactctgtctggccgtccactactgacacagctggctccataacctgtacagtctccacagacagtgcaaaccatgcactgctccagcttccatttgtgcatgcctggagggcacatcatagacttctcatctttttcatctagttcttcttccaggtcttcatccattgctgttgccatattttcaactccaaaccctttcccaccttggttcatggcaccagtatctcgtccacactgtcctttattatttacaccaaatgtccacacctctccattcttcattaaaacacaagtgtgagctttgcccatagctacctgagttacaaaatggcccttcaaatcagttaccaaacttgaactatcagagtaaatggcatcttttccaaacatgtagagttctccatctttagaaataacagaactacttccattattgcaggctgtatataccacaatctttccttccatcttaattatctttttaggtttataaggtttggattgccgtctgctcttagttgattctccatcttctcctttactagcagatcctgtaaagaatatgctcccatcttctgcaactaaaagggcgtgagagccatcgtgtccaactgagaagtgtactatctttggagattttgtaattggtagctcaacccattttcctgctgaaggaccaccttgtttgattccaagactctggtatttgccagtgtaatatatctttccatttgctgttttcattagcgcaaactctcgtcctgcaccaagaattgctgactcctcatcaaatcctgtacttataatatgcaagtccttttccagatcgaatagtgagataccacaggcatgtaagcattttctagccagtttaagttgcaattcttgctgtagaacaggttcagtgcttgtggcaaatattctgacaacaaagccatcatctcttgaagcagctatctgattaatatattctccatcagtgaataaaatattttgaccttcagtgtggcaatctggtaacatcacagtaccatcttgctccagtgtttcagggcttatccttatggctgtcatgctgtggttattcacatctctatataataaataaccctgagcataccctaaccaagactttttttcttttctgtttctaatacgggatgtagaattgtatatatggcccctaactgttccactgtatccagagcctattttatataatccatccttgcataatagataaagaaaaaatccatcattctgaagtagacattggtcatcttcatcaacagatatttcttttaatggccacttgtgcattaaagctgctttcttaatgccattactaaaccagtcctgaatttgaatttttcccaccaaaactgcttgtacacttctctgtagcgaatttagaattgttggcacctgaatagtttggcaagcatggcttccattgttggtgaggatagcagagatggcctgaagtgtccttcctgtttctccccaagaagccaccagactaaagaggcaagcacaggaaagtgctgttaaggactgtcctgtgctgtcattcatcccagtacttcgaacggtgatttccaaaagaagctggaagagagactctaggacctcaggtggctcagactggaggccttctggctgctggccctgcagcacgttgagcagggcttggagactcctgagacacagggatggatgagaaaatcgtgtctctttgatcaattcaaaaacttcacaaaggccaacctcaataatctttggaagcttgatagggggctctttggattcctcttcttcatcactatctgattctccactctgcacagagttcttagatgcggctgccaatgatatttcctttttctgccattccagaacgcaatggcgtacattacagtaaatattgaaagcagaaggattgctatgtagtttgatatctggtatgattactgtattctctaagttttcagacttgcttcttgtcttcacttttgatttgctcttctgttttcttttcaatttcttcttatttaaaattttcttattcctggaggctgggtgtccagcgctgccgcccccctggtccctgtcattgagcgcagcggtataaatcctccggtagcggtcggccagggcccggcctgacagcagcagctggtagtgaccccgggagtccgcggcgggtagccccagccccagccccgcagcagccacggagccgtcgggaaccggcatgaacagcgcccccggcgccggggaggaagagaaggtggcggctgggtagaatccgtccccgccgagccccgaggaggcggcggcgggggaggcagtcgctgcgcacatcatcatcctcgccgccgccgccgccgccgccgcctcgtccccgcgggccgggcgggcagacacgcgcgcgcacacacagcccttttccaacgacgacggctccggcggcggcctctggctcccgcagcagggagactacaaagacagcgacctccttctcctcctccttcttctcctcctcccccccgcgccgccctcgccgctactggggccgctcatctaaccccgccaccccgggaatgtgaggaggaggcggtgccgccactgccgccgccaccaccgctaccaccgccaccaccgccggggctacccgcaatgggaagctgccg

SEQ ID NO: 17101 - RNA, 8770 nt, Homo sapiens
  source 1..8770: mol_type = other RNA
tcaaaactgaggggcattttcttcttgcggagggtatctggatcaagtgtgtaagagtctgatttagaacgttcccgaggaggatcaagctttgtcttaacaggagcagtacttttttgaggtagatttttatcatgtggtgaggaggagcgtggagaactagcacccgatgggctagacctattggctgggagagtctttggcttaggagatgacaaccgagaacctggtcctggggattcagctctggagctagaaggcatcctcccatcagatttcaatgtctgcaaggtgttatggttgggggataatgacctactgtgggaatctgacctcaactttgcagcatcagattttaagatgagggattcactagcagataaactttctgtgccccttggcttcttctgatcagcagtagtccggctcatacgtccatcaggtttaagcgatctgctgtgtttagaggacagctctgattttcctgatgtagaggctggtttagaagatgttgagatgtttcctcgatcacctttgctatttccgagtccataatcaaatccttgggcactgcaacttgcccctttattaaaagcttgcactgagaaagggcttggaggaggagtttgagaattctgatccagaagagcttgttcatcttcatgtcggaggtactggtttccgcctctgtctctagctaaggaccatgcctctccttcatcactctcacagaactctaccatgctgttctgatccagttgcacccatgtcccttcagaattggttacgtcaacagggaccagaagactcttgccaagatgttgattaaaagagaggcaccaggcttcagtgtaaccattcatgttagggacatacttctttattgtctcatcattcagcctcagccacacaccatcatcattatggatctcatcaataaaagtgatagttccattgactttcactatgcctatctgctcactctgaagggaagggtggctacggatgcgaagccccgcactgtccttggccacaaattttcgaaccttattaggctgaggttcagactttggtttgaccaactgagttcctggtggtatcatcccttttggtgggtcttttacttttacttccagaccagcatcgatttcaatgccatcaatggtaacatgaagagtgtagagtccaatagcccctggagtccaatttgcacaataagtcccatcattattgacacggatcagcatattctcactgggtctcttaggagttggtgatgcaaaacgtagttcttcaaatgaataattttcataaaccttcatcattgttatggcaatatatcgagcttccttcactatcattggttcatatgaaacatctagctttggtgatgccagccctccataagtcatgtcagtattagaagatgcagctgttactgcaggactgccaggaatcctttgaggtttctttgcttgatcttgttgtaaagacatttttttctgagaaacagggacagctttcacttccaccttcatattgggaacatgtaccacatccccatactggtcttttgtttgaacagttatggtggtaggccaaccacaacgaatatcatccttattcaggatcaaagatgttttctgaggatccgcatatgaatctggctgaagccaccttgcaagccttccaccacttgatcctgggacacaggcaataaaatcatccagaaaagactgttcattgctttggatttggagtggtaaatttccctcaagtgcttctaatatagttggtgaatgagaaagagctagaccctttccaagaattccagaatgggttttgcacacctgcaatgcagcctcctcaagaatttcaaggtcttcttctaattcattaccaataggaagtgctaggtccttcttcatcagagctgctgcacaaaccccaccaagattggctaattctttttccaattggatgactccctcatcaggtccagggctaaattcatatccaattgcaaaacacttaaaaccatagaaagaagctttgtcatctttcacataatctgatgcagtctccaatgaaaaaagggcctcatttcctggcaacaccaaaaccatagtaggccacccagaggatcctgaaaatttctttaattctatccatgaattaagattttcatgaacagatgtcaattttggtccatatcctgaattctgaacagttctgacaggaatcaacaaacgaaggacatcttctgactgtgcagtaccacactgagggtcaaattcgattgtcatccacctcacacattctgggaatgtcaccttgtaatgcatcacacaggcaggtttatacgggtgctcactctctatgacagcatagtgactggaggttgtacaagcagagaggccctgttcaggctggtttcctgtggtgctatctgtcgactgattagggttgaaggcaggcggtgcatacttctgattcaaaatggcaactgacggaagcaattgttggacaaggccaaagacttctacagccaccttgggaatagcagcagctactggtcctatgtaggctataataagggggagcagcatggaaaacagactggaagaactcagcagttctggaatgtcatcagcatccacagcaagagctctgtgcaggaggtccttagaggctcgaacgacagtgcttacaacagacaatgctctgctacagtttttatcttcttcattggctttactcagaagttgggattgtaaatctccatcaaattcactcctatagtagagtatctgtgggatctgtcctctggtttggtttgtgccgttactgctcaagctgcacgtgctgaatgtgaatgtcacaccatcagggcactgaactgtggtcattcctccatctccattggctgtacggcttccatagttcctcaagcgcacagcatatttaacattttcctttaaaggaaccactttgtcaagtctgatctcagctatatcactgggtgagtcatccgttgtgtacgttcctttcactaattccagagatgtccatctgtgggaatgagttgaatctcctgcatgttcactatcatcaaccaacacctctaattcatattcatgaattccacctcctccatagacagagaaaccaaccacaactattccaggtttgtctactgaaaaacagattgcatcaggggacccgttcccagtgttccaacttctgccctgacttgtttttgtaaatcggttagcactagcttttacagagtgaagagaattaagtccatcaacctcagatcccagggctgacgctgtcagttcactgacaatgctggccagtaatccacaggtgttagagacgaggtgggaggagaagagttcattttctctcctcaggctgttcctgactggtagcacaacaatgaccagcattttctccagaacttcacggaagcttgtcatccctgagatattctcttcactctggctgagtttttccatatgtgccaccaaaaggggaaaacgatgaactagtgttgagtcgttctctgtactaacttgtttaacaattgatcgtagtaatacttctccatcatacgcaatcgggaagatggaagtcagcttaacagacgtgtgacacagagctgacataacagctgcaaggagtcggctacttgatgtcttgaagtttgcttcttggatatcctgatccaaacaattcagcagatcacaaaggcaagcccactgtaaggcaggagttgggtagaaagaatgaaagcaggcagtgaaagtattatgacattcctgaaggacagcttctagaagactcaagggttgactgagatatccttgaggatcattatccaatttcaccatgcagtgatcaactccttctgataaaatttttcttaacaaagttctggtttttccaatacactctgctaatttgctagtttcttctacaactgcttttcctgtagctgacactgggtaaatttcacaggtatagacacgcaataacctcagacaacaggtacccacaaagcgcagtctctctaaatctaggagtgtagctgtgaactggaatccttttaatcctctaagttcttcaactcctaagactaaggtggtccagctccagtgaagaatactcaacaatgactcaaaacattccactgagacagttcttgcaaaagacctctttaaaatgtgtacaggttcactggtttgctgtttgccttttgaagcactgccatcactggttggaagtctgtataataactgaggtatctgacccgcattaacatctgtaccattatttgatttctttgaactcttgaactggaaaacaaccccatcatctgtggtaatagatgcctgtccatgagatccacagtcactgctgggtcctgacactcgggcccatgccacataccaccacccagcttgcaggagaacaggctcatcaaacatcattgcatatttttctctagcagcacagtcataagccaatacatcagtctctgcaagaaggtcaccatcagtttcatgatctcctccatcaggacccaattcaaacagcttaattttagcagtatattctcctctacctccaaacagaccaagaccaccaagtaaaatatcagtgtcggcactgaaacgtatagcttctactgaatgggcagaataaccccagcctcctccatgactttcaaacctgtttaccacactataatcttctttagaataaaccttcattactgcttgagtctcttcctctgtacttgcaacacccatttttaagtcctgcatagctgccaaggtatcaagacaacctaaaatgtgcaaagctgcatgagatcgggtagtgagggcccttgatcctgttggtaaggcaagttcaggacttaggatactacatctggactgcatgtctgctgcagagggaagcctggcatcagcaaccaccgcattgtaacaccacagctctctagtatttggtcgaaacctccaaattacatcatatacaggatcaagacacacaccaaatccttgcagatcctcttgttctgagtcattaaaagttttacaactcccatccactttatttatcagaaggcatttaaatggaggaggttctgatatagaagcaggtaccaagcctattatgtgtttactggcaaaaatttctgatgtagcaagtacatgagaattaataagtgcttcatcaattcgtaaaaaagtttggtccccacttgcacctatccaagtagcttttcttccatattttgatccaatgttaggcatgggagctggctttgcattccaatatggcacatccaaaattggtctgcccagttgtcctttagaaaaacttccaaatgtgaagacctgtccatccattaaaagtactgccgtatggttgctgcctgcagtgacttgtgtgctagggcctggcaatgcttgaacaagagtgggacatcccctggagttgacatctccatgtcctagctgcccatgctgcccataaccaaatgtatagacatctccattttccattaaaaccactgaatggtgaaatccacagctgacttggactgcccggagctcacagtcaaatcgcacagagcctggagggtatgttgtgattttgcttgcatccttttcgcctctttctccacttccatctttgtgcttgtcccgtttatgctttagctgtgctggatgggatctgagtctggctagagcctgttctcgatggttcataaaaataggaccagcaaatacaagggggcctcttccttcctctaatctgtgccttctgattacacgttgccgtttttcttcttgtcgtaactgaaggtgttcttcaatgttaaccccgggcactgggacagctaaaagaagatctaaaggtatcatttctttcactgcatcaagaattcctctttgtcttgcctcttgaccatctaactctcttgcacaggccttgcaacatccacacacagcacaaccagattctccggaaccacaaccacagatccctccggggactctgtctggccgtccactactgacacagctggctccataacctgtacagtctccacagacagtgcaaaccatgcactgctccagcttccatttgtgcatgcctggagggcacatcatagacttctcatctttttcatctagttcttcttccaggtcttcatccattgctgttgccatattttcaactccaaaccctttcccaccttggttcatggcaccagtatctcgtccacactgtcctttattatttacaccaaatgtccacacctctccattcttcattaaaacacaagtgtgagctttgcccatagctacctgagttacaaaatggcccttcaaatcagttaccaaacttgaactatcagagtaaatggcatcttttccaaacatgtagagttctccatctttagaaataacagaactacttccattattgcaggctgtatataccacaatctttccttccatcttaattatctttttaggtttataaggtttggattgccgtctgctcttagttgattctccatcttctcctttactagcagatcctgtaaagaatatgctcccatcttctgcaactaaaagggcgtgagagccatcgtgtccaactgagaagtgtactatctttggagattttgtaattggtagctcaacccattttcctgctgaaggaccaccttgtttgattccaagactctggtatttgccagtgtaatatatctttccatttgctgttttcattagcgcaaactctcgtcctgcaccaagaattgctgactcctcatcaaatcctgtacttataatatgcaagtccttttccagatcgaatagtgagataccacaggcatgtaagcattttctagccagtttaagttgcaattcttgctgtagaacaggttcagtgcttgtggcaaatattctgacaacaaagccatcatctcttgaagcagctatctgattaatatattctccatcagtgaataaaatattttgaccttcagtgtggcaatctggtaacatcacagtaccatcttgctccagtgtttcagggcttatccttatggctgtcatgctgtggttattcacatctctatataataaataaccctgagcataccctaaccaagactttttttcttttctgtttctaatacgggatgtagaattgtatatatggcccctaactgttccactgtatccagagcctattttatataatccatccttgcataatagataaagaaaaaatccatcattctgaagtagacattggtcatcttcatcaacagatatttcttttaatggccacttgtgcattaaagctgctttcttaatgccattactaaaccagtcctgaatttgaatttttcccaccaaaactgcttgtacacttctctgtagcgaatttagaattgttggcacctgaatagtttggcaagcatggcttccattgttggtgaggatagcagagatggcctgaagtgtccttcctgtttctccccaagaagccaccagactaaagaggcaagcacaggaaagtgctgttaaggactgtcctgtgctgtcattcatcccagtacttcgaacggtgatttccaaaagaagctggaagagagactctaggacctcaggtggctcagactggaggccttctggctgctggccctgcagcacgttgagcagggcttggagactcctgagacacagggatggatgagaaaatcgtgtctctttgatcaattcaaaaacttcacaaaggccaacctcaataatctttggaagcttgatagggggctctttggattcctcttcttcatcactatctgattctccactctgcacagagttcttagatgcggctgccaatgatatttcctttttctgccattccagaacgcaatggcgtacattacagtaaatattgaaagcagaaggattgctatgtagtttgatatctggtatgattactgtattctctaagttttcagacttgcttcttgtcttcacttttgatttgctcttctgttttcttttcaatttcttcttatttaaaattttcttattcctggaggctgggtgtccagcgctgccgcccccctggtccctgtcattgagcgcagcggtataaatcctccggtagcggtcggccagggcccggcctgacagcagcagctggtagtgaccccgggagtccgcggcgggtagccccagccccagccccgcagcagccacggagccgtcgggaaccggcatgaacagcgcccccggcgccggggaggaagagaaggtggcggctgggtagaatccgtccccgccgagccccgaggaggcggcggcgggggaggcagtcgctgcgcacatcatcatcctcgccgccgccgccgccgccgccgcctcgtccccgcgggccgggcgggcagacacgcgcgcgcacacacagcccttttccaacgacgacggctccggcggcggcctctggctcccgcagcagggagactacaaagacagcgacctccttctcctcctccttcttctcctcctcccccccgcgccgccctcgccgctactggggccgctcatctaaccccgccaccccgggaatgtgaggaggaggcggtgccgccactgccgccgccaccaccgctaccaccgccaccaccgccggggctacccgcaatgggaagctgccg

SEQ ID NO: 17102 - RNA, 9250 nt, Homo sapiens
  source 1..9250: mol_type = other RNA
tcaaaactgaggggcattttcttcttgcggagggtatctggatcaagtgtgtaagagtctgatttagaacgttcccgaggaggatcaagctttgtcttaacaggagcagtacttttttgaggtagatttttatcatgtggtgaggaggagcgtggagaactagcacccgatgggctagacctattggctgggagagtctttggcttaggagatgacaaccgagaacctggtcctggggattcagctctggagctagaaggcatcctcccatcagatttcaatgtctgcaaggtgttatggttgggggataatgacctactgtgggaatctgacctcaactttgcagcatcagattttaagatgagggattcactagcagataaactttctgtgccccttggcttcttctgatcagcagtagtccggctcatacgtccatcaggtttaagcgatctgctgtgtttagaggacagctctgattttcctgatgtagaggctggtttagaagatgttgagatgtttcctcgatcactctgaagctgaggctgctggaaggaaaggggctgtccgaacacaaatgggctgtgtactagggaagagggaggttttgcagcttgatcaaagatggaaggagctgggagattgggtcgtgactgaatggaattcaatatggcactcagttggtcacctgcagtgggtaaaacagtcaaaactttgctatttccgagtccataatcaaatccttgggcactgcaacttgcccctttattaaaagcttgcactgagaaagggcttggaggaggagtttgagaattctgatccagaagagcttgttcatcttcatgtcggaggtactggtttccgcctctgtctctagctaaggaccatgcctctccttcatcactctcacagaactctaccatgctgttctgatccagttgcacccatgtcccttcagaattggttacctctcccactgctttgactttgtttcccagaactaacattccaattgggatacctctaaggttagggcagcttctgatgttgtgacctgaaggtcccgtcttcactaccttgtacatgcctggccctcctcgcaagaatggcatatcttgttcttgcattgttgcttcctgtgggcagcaggagtttatgtctttgaaaaagtcatcagtattagttttagattcctgggggaaaaaagctttggaagtccatgaaaatacgtccaaatccctgactccttggctagcattaaagatattgtcaacagggaccagaagactcttgccaagatgttgattaaaagagaggcaccaggcttcagtgtaaccattcatgttagggacatacttctttattgtctcatcattcagcctcagccacacaccatcatcattatggatctcatcaataaaagtgatagttccattgactttcactatgcctatctgctcactctgaagggaagggtggctacggatgcgaagccccgcactgtccttggccacaaattttcgaaccttattaggctgaggttcagactttggtttgaccaactgagttcctggtggtatcatcccttttggtgggtcttttacttttacttccagaccagcatcgatttcaatgccatcaatggtaacatgaagagtgtagagtccaatagcccctggagtccaatttgcacaataagtcccatcattattgacacggatcagcatattctcactgggtctcttaggagttggtgatgcaaaacgtagttcttcaaatgaataattttcataaaccttcatcattgttatggcaatatatcgagcttccttcactatcattggttcatatgaaacatctagctttggtgatgccagccctccataagtcatgtcagtattagaagatgcagctgttactgcaggactgccaggaatcctttgaggtttctttgcttgatcttgttgtaaagacatttttttctgagaaacagggacagctttcacttccaccttcatattgggaacatgtaccacatccccatactggtcttttgtttgaacagttatggtggtaggccaaccacaacgaatatcatccttattcaggatcaaagatgttttctgaggatccgcatatgaatctggctgaagccaccttgcaagccttccaccacttgatcctgggacacaggcaataaaatcatccagaaaagactgttcattgctttggatttggagtggtaaatttccctcaagtgcttctaatatagttggtgaatgagaaagagctagaccctttccaagaattccagaatgggttttgcacacctgcaatgcagcctcctcaagaatttcaaggtcttcttctaattcattaccaataggaagtgctaggtccttcttcatcagagctgctgcacaaaccccaccaagattggctaattctttttccaattggatgactccctcatcaggtccagggctaaattcatatccaattgcaaaacacttaaaaccatagaaagaagctttgtcatctttcacataatctgatgcagtctccaatgaaaaaagggcctcatttcctggcaacaccaaaaccatagtaggccacccagaggatcctgaaaatttctttaattctatccatgaattaagattttcatgaacagatgtcaattttggtccatatcctgaattctgaacagttctgacaggaatcaacaaacgaaggacatcttctgactgtgcagtaccacactgagggtcaaattcgattgtcatccacctcacacattctgggaatgtcaccttgtaatgcatcacacaggcaggtttatacgggtgctcactctctatgacagcatagtgactggaggttgtacaagcagagaggccctgttcaggctggtttcctgtggtgctatctgtcgactgattagggttgaaggcaggcggtgcatacttctgattcaaaatggcaactgacggaagcaattgttggacaaggccaaagacttctacagccaccttgggaatagcagcagctactggtcctatgtaggctataataagggggagcagcatggaaaacagactggaagaactcagcagttctggaatgtcatcagcatccacagcaagagctctgtgcaggaggtccttagaggctcgaacgacagtgcttacaacagacaatgctctgctacagtttttatcttcttcattggctttactcagaagttgggattgtaaatctccatcaaattcactcctatagtagagtatctgtgggatctgtcctctggtttggtttgtgccgttactgctcaagctgcacgtgctgaatgtgaatgtcacaccatcagggcactgaactgtggtcattcctccatctccattggctgtacggcttccatagttcctcaagcgcacagcatatttaacattttcctttaaaggaaccactttgtcaagtctgatctcagctatatcactgggtgagtcatccgttgtgtacgttcctttcactaattccagagatgtccatctgtgggaatgagttgaatctcctgcatgttcactatcatcaaccaacacctctaattcatattcatgaattccacctcctccatagacagagaaaccaaccacaactattccaggtttgtctactgaaaaacagattgcatcaggggacccgttcccagtgttccaacttctgccctgacttgtttttgtaaatcggttagcactagcttttacagagtgaagagaattaagtccatcaacctcagatcccagggctgacgctgtcagttcactgacaatgctggccagtaatccacaggtgttagagacgaggtgggaggagaagagttcattttctctcctcaggctgttcctgactggtagcacaacaatgaccagcattttctccagaacttcacggaagcttgtcatccctgagatattctcttcactctggctgagtttttccatatgtgccaccaaaaggggaaaacgatgaactagtgttgagtcgttctctgtactaacttgtttaacaattgatcgtagtaatacttctccatcatacgcaatcgggaagatggaagtcagcttaacagacgtgtgacacagagctgacataacagctgcaaggagtcggctacttgatgtcttgaagtttgcttcttggatatcctgatccaaacaattcagcagatcacaaaggcaagcccactgtaaggcaggagttgggtagaaagaatgaaagcaggcagtgaaagtattatgacattcctgaaggacagcttctagaagactcaagggttgactgagatatccttgaggatcattatccaatttcaccatgcagtgatcaactccttctgataaaatttttcttaacaaagttctggtttttccaatacactctgctaatttgctagtttcttctacaactgcttttcctgtagctgacactgggtaaatttcacaggtatagacacgcaataacctcagacaacaggtacccacaaagcgcagtctctctaaatctaggagtgtagctgtgaactggaatccttttaatcctctaagttcttcaactcctaagactaaggtggtccagctccagtgaagaatactcaacaatgactcaaaacattccactgagacagttcttgcaaaagacctctttaaaatgtgtacaggttcactggtttgctgtttgccttttgaagcactgccatcactggttggaagtctgtataataactgaggtatctgacccgcattaacatctgtaccattatttgatttctttgaactcttgaactggaaaacaaccccatcatctgtggtaatagatgcctgtccatgagatccacagtcactgctgggtcctgacactcgggcccatgccacataccaccacccagcttgcaggagaacaggctcatcaaacatcattgcatatttttctctagcagcacagtcataagccaatacatcagtctctgcaagaaggtcaccatcagtttcatgatctcctccatcaggacccaattcaaacagcttaattttagcagtatattctcctctacctccaaacagaccaagaccaccaagtaaaatatcagtgtcggcactgaaacgtatagcttctactgaatgggcagaataaccccagcctcctccatgactttcaaacctgtttaccacactataatcttctttagaataaaccttcattactgcttgagtctcttcctctgtacttgcaacacccatttttaagtcctgcatagctgccaaggtatcaagacaacctaaaatgtgcaaagctgcatgagatcgggtagtgagggcccttgatcctgttggtaaggcaagttcaggacttaggatactacatctggactgcatgtctgctgcagagggaagcctggcatcagcaaccaccgcattgtaacaccacagctctctagtatttggtcgaaacctccaaattacatcatatacaggatcaagacacacaccaaatccttgcagatcctcttgttctgagtcattaaaagttttacaactcccatccactttatttatcagaaggcatttaaatggaggaggttctgatatagaagcaggtaccaagcctattatgtgtttactggcaaaaatttctgatgtagcaagtacatgagaattaataagtgcttcatcaattcgtaaaaaagtttggtccccacttgcacctatccaagtagcttttcttccatattttgatccaatgttaggcatgggagctggctttgcattccaatatggcacatccaaaattggtctgcccagttgtcctttagaaaaacttccaaatgtgaagacctgtccatccattaaaagtactgccgtatggttgctgcctgcagtgacttgtgtgctagggcctggcaatgcttgaacaagagtgggacatcccctggagttgacatctccatgtcctagctgcccatgctgcccataaccaaatgtatagacatctccattttccattaaaaccactgaatggtgaaatccacagctgacttggactgcccggagctcacagtcaaatcgcacagagcctggagggtatgttgtgattttgcttgcatccttttcgcctctttctccacttccatctttgtgcttgtcccgtttatgctttagctgtgctggatgggatctgagtctggctagagcctgttctcgatggttcataaaaataggaccagcaaatacaagggggcctcttccttcctctaatctgtgccttctgattacacgttgccgtttttcttcttgtcgtaactgaaggtgttcttcaatgttaaccccgggcactgggacagctaaaagaagatctaaaggtatcatttctttcactgcatcaagaattcctctttgtcttgcctcttgaccatctaactctcttgcacaggccttgcaacatccacacacagcacaaccagattctccggaaccacaaccacagatccctccggggactctgtctggccgtccactactgacacagctggctccataacctgtacagtctccacagacagtgcaaaccatgcactgctccagcttccatttgtgcatgcctggagggcacatcatagacttctcatctttttcatctagttcttcttccaggtcttcatccattgctgttgccatattttcaactccaaaccctttcccaccttggttcatggcaccagtatctcgtccacactgtcctttattatttacaccaaatgtccacacctctccattcttcattaaaacacaagtgtgagctttgcccatagctacctgagttacaaaatggcccttcaaatcagttaccaaacttgaactatcagagtaaatggcatcttttccaaacatgtagagttctccatctttagaaataacagaactacttccattattgcaggctgtatataccacaatctttccttccatcttaattatctttttaggtttataaggtttggattgccgtctgctcttagttgattctccatcttctcctttactagcagatcctgtaaagaatatgctcccatcttctgcaactaaaagggcgtgagagccatcgtgtccaactgagaagtgtactatctttggagattttgtaattggtagctcaacccattttcctgctgaaggaccaccttgtttgattccaagactctggtatttgccagtgtaatatatctttccatttgctgttttcattagcgcaaactctcgtcctgcaccaagaattgctgactcctcatcaaatcctgtacttataatatgcaagtccttttccagatcgaatagtgagataccacaggcatgtaagcattttctagccagtttaagttgcaattcttgctgtagaacaggttcagtgcttgtggcaaatattctgacaacaaagccatcatctcttgaagcagctatctgattaatatattctccatcagtgaataaaatattttgaccttcagtgtggcaatctggtaacatcacagtaccatcttgctccagtgtttcagggcttatccttatggctgtcatgctgtggttattcacatctctatataataaataaccctgagcataccctaaccaagactttttttcttttctgtttctaatacgggatgtagaattgtatatatggcccctaactgttccactgtatccagagcctattttatataatccatccttgcataatagataaagaaaaaatccatcattctgaagtagacattggtcatcttcatcaacagatatttcttttaatggccacttgtgcattaaagctgctttcttaatgccattactaaaccagtcctgaatttgaatttttcccaccaaaactgcttgtacacttctctgtagcgaatttagaattgttggcacctgaatagtttggcaagcatggcttccattgttggtgaggatagcagagatggcctgaagtgtccttcctgtttctccccaagaagccaccagactaaagaggcaagcacaggaaagtgctgttaaggactgtcctgtgctgtcattcatcccagtacttcgaacggtgatttccaaaagaagctggaagagagactctaggacctcaggtggctcagactggaggccttctggctgctggccctgcagcacgttgagcagggcttggagactcctgagacacagggatggatgagaaaatcgtgtctctttgatcaattcaaaaacttcacaaaggccaacctcaataatctttggaagcttgatagggggctctttggattcctcttcttcatcactatctgattctccactctgcacagagttcttagatgcggctgccaatgatatttcctttttctgccattccagaacgcaatggcgtacattacagtaaatattgaaagcagaaggattgctatgtagtttgatatctggtatgattactgtattctctaagttttcagacttgcttcttgtcttcacttttgatttgctcttctgttttcttttcaatttcttcttatttaaaattttcttattcctggaggctgggtgtccagcgctgccgcccccctggtccctgtcattgagcgcagcggtataaatcctccggtagcggtcggccagggcccggcctgacagcagcagctggtagtgaccccgggagtccgcggcgggtagccccagccccagccccgcagcagccacggagccgtcgggaaccggcatgaacagcgcccccggcgccggggaggaagagaaggtggcggctgggtagaatccgtccccgccgagccccgaggaggcggcggcgggggaggcagtcgctgcgcacatcatcatcctcgccgccgccgccgccgccgccgcctcgtccccgcgggccgggcgggcagacacgcgcgcgcacacacagcccttttccaacgacgacggctccggcggcggcctctggctcccgcagcagggagactacaaagacagcgacctccttctcctcctccttcttctcctcctcccccccgcgccgccctcgccgctactggggccgctcatctaaccccgccaccccgggaatgtgaggaggaggcggtgccgccactgccgccgccaccaccgctaccaccgccaccaccgccggggctacccgcaatgggaagctgccg

SEQ ID NO: 17103 - RNA, 8950 nt, Homo sapiens
  source 1..8950: mol_type = other RNA
tcaaaactgaggggcattttcttcttgcggagggtatctggatcaagtgtgtaagagtctgatttagaacgttcccgaggaggatcaagctttgtcttaacaggagcagtacttttttgaggtagatttttatcatgtggtgaggaggagcgtggagaactagcacccgatgggctagacctattggctgggagagtctttggcttaggagatgacaaccgagaacctggtcctggggattcagctctggagctagaaggcatcctcccatcagatttcaatgtctgcaaggtgttatggttgggggataatgacctactgtgggaatctgacctcaactttgcagcatcagattttaagatgagggattcactagcagataaactttctgtgccccttggcttcttctgatcagcagtagtccggctcatacgtccatcaggtttaagcgatctgctgtgtttagaggacagctctgattttcctgatgtagaggctggtttagaagatgttgagatgtttcctcgatcactctgaagctgaggctgctggaaggaaaggggctgtccgaacacaaatgggctgtgtactagggaagagggaggttttgcagcttgatcaaagatggaaggagctgggagattgggtcgtgactgaatggaattcaatatggcactcagttggtcacctgcagtgggtaaaacagtcaaaactttgctatttccgagtccataatcaaatccttgggcactgcaacttgcccctttattaaaagcttgcactgagaaagggcttggaggaggagtttgagaattctgatccagaagagcttgttcatcttcatgtcggaggtactggtttccgcctctgtctctagctaaggaccatgcctctccttcatcactctcacagaactctaccatgctgttctgatccagttgcacccatgtcccttcagaattggttacgtcaacagggaccagaagactcttgccaagatgttgattaaaagagaggcaccaggcttcagtgtaaccattcatgttagggacatacttctttattgtctcatcattcagcctcagccacacaccatcatcattatggatctcatcaataaaagtgatagttccattgactttcactatgcctatctgctcactctgaagggaagggtggctacggatgcgaagccccgcactgtccttggccacaaattttcgaaccttattaggctgaggttcagactttggtttgaccaactgagttcctggtggtatcatcccttttggtgggtcttttacttttacttccagaccagcatcgatttcaatgccatcaatggtaacatgaagagtgtagagtccaatagcccctggagtccaatttgcacaataagtcccatcattattgacacggatcagcatattctcactgggtctcttaggagttggtgatgcaaaacgtagttcttcaaatgaataattttcataaaccttcatcattgttatggcaatatatcgagcttccttcactatcattggttcatatgaaacatctagctttggtgatgccagccctccataagtcatgtcagtattagaagatgcagctgttactgcaggactgccaggaatcctttgaggtttctttgcttgatcttgttgtaaagacatttttttctgagaaacagggacagctttcacttccaccttcatattgggaacatgtaccacatccccatactggtcttttgtttgaacagttatggtggtaggccaaccacaacgaatatcatccttattcaggatcaaagatgttttctgaggatccgcatatgaatctggctgaagccaccttgcaagccttccaccacttgatcctgggacacaggcaataaaatcatccagaaaagactgttcattgctttggatttggagtggtaaatttccctcaagtgcttctaatatagttggtgaatgagaaagagctagaccctttccaagaattccagaatgggttttgcacacctgcaatgcagcctcctcaagaatttcaaggtcttcttctaattcattaccaataggaagtgctaggtccttcttcatcagagctgctgcacaaaccccaccaagattggctaattctttttccaattggatgactccctcatcaggtccagggctaaattcatatccaattgcaaaacacttaaaaccatagaaagaagctttgtcatctttcacataatctgatgcagtctccaatgaaaaaagggcctcatttcctggcaacaccaaaaccatagtaggccacccagaggatcctgaaaatttctttaattctatccatgaattaagattttcatgaacagatgtcaattttggtccatatcctgaattctgaacagttctgacaggaatcaacaaacgaaggacatcttctgactgtgcagtaccacactgagggtcaaattcgattgtcatccacctcacacattctgggaatgtcaccttgtaatgcatcacacaggcaggtttatacgggtgctcactctctatgacagcatagtgactggaggttgtacaagcagagaggccctgttcaggctggtttcctgtggtgctatctgtcgactgattagggttgaaggcaggcggtgcatacttctgattcaaaatggcaactgacggaagcaattgttggacaaggccaaagacttctacagccaccttgggaatagcagcagctactggtcctatgtaggctataataagggggagcagcatggaaaacagactggaagaactcagcagttctggaatgtcatcagcatccacagcaagagctctgtgcaggaggtccttagaggctcgaacgacagtgcttacaacagacaatgctctgctacagtttttatcttcttcattggctttactcagaagttgggattgtaaatctccatcaaattcactcctatagtagagtatctgtgggatctgtcctctggtttggtttgtgccgttactgctcaagctgcacgtgctgaatgtgaatgtcacaccatcagggcactgaactgtggtcattcctccatctccattggctgtacggcttccatagttcctcaagcgcacagcatatttaacattttcctttaaaggaaccactttgtcaagtctgatctcagctatatcactgggtgagtcatccgttgtgtacgttcctttcactaattccagagatgtccatctgtgggaatgagttgaatctcctgcatgttcactatcatcaaccaacacctctaattcatattcatgaattccacctcctccatagacagagaaaccaaccacaactattccaggtttgtctactgaaaaacagattgcatcaggggacccgttcccagtgttccaacttctgccctgacttgtttttgtaaatcggttagcactagcttttacagagtgaagagaattaagtccatcaacctcagatcccagggctgacgctgtcagttcactgacaatgctggccagtaatccacaggtgttagagacgaggtgggaggagaagagttcattttctctcctcaggctgttcctgactggtagcacaacaatgaccagcattttctccagaacttcacggaagcttgtcatccctgagatattctcttcactctggctgagtttttccatatgtgccaccaaaaggggaaaacgatgaactagtgttgagtcgttctctgtactaacttgtttaacaattgatcgtagtaatacttctccatcatacgcaatcgggaagatggaagtcagcttaacagacgtgtgacacagagctgacataacagctgcaaggagtcggctacttgatgtcttgaagtttgcttcttggatatcctgatccaaacaattcagcagatcacaaaggcaagcccactgtaaggcaggagttgggtagaaagaatgaaagcaggcagtgaaagtattatgacattcctgaaggacagcttctagaagactcaagggttgactgagatatccttgaggatcattatccaatttcaccatgcagtgatcaactccttctgataaaatttttcttaacaaagttctggtttttccaatacactctgctaatttgctagtttcttctacaactgcttttcctgtagctgacactgggtaaatttcacaggtatagacacgcaataacctcagacaacaggtacccacaaagcgcagtctctctaaatctaggagtgtagctgtgaactggaatccttttaatcctctaagttcttcaactcctaagactaaggtggtccagctccagtgaagaatactcaacaatgactcaaaacattccactgagacagttcttgcaaaagacctctttaaaatgtgtacaggttcactggtttgctgtttgccttttgaagcactgccatcactggttggaagtctgtataataactgaggtatctgacccgcattaacatctgtaccattatttgatttctttgaactcttgaactggaaaacaaccccatcatctgtggtaatagatgcctgtccatgagatccacagtcactgctgggtcctgacactcgggcccatgccacataccaccacccagcttgcaggagaacaggctcatcaaacatcattgcatatttttctctagcagcacagtcataagccaatacatcagtctctgcaagaaggtcaccatcagtttcatgatctcctccatcaggacccaattcaaacagcttaattttagcagtatattctcctctacctccaaacagaccaagaccaccaagtaaaatatcagtgtcggcactgaaacgtatagcttctactgaatgggcagaataaccccagcctcctccatgactttcaaacctgtttaccacactataatcttctttagaataaaccttcattactgcttgagtctcttcctctgtacttgcaacacccatttttaagtcctgcatagctgccaaggtatcaagacaacctaaaatgtgcaaagctgcatgagatcgggtagtgagggcccttgatcctgttggtaaggcaagttcaggacttaggatactacatctggactgcatgtctgctgcagagggaagcctggcatcagcaaccaccgcattgtaacaccacagctctctagtatttggtcgaaacctccaaattacatcatatacaggatcaagacacacaccaaatccttgcagatcctcttgttctgagtcattaaaagttttacaactcccatccactttatttatcagaaggcatttaaatggaggaggttctgatatagaagcaggtaccaagcctattatgtgtttactggcaaaaatttctgatgtagcaagtacatgagaattaataagtgcttcatcaattcgtaaaaaagtttggtccccacttgcacctatccaagtagcttttcttccatattttgatccaatgttaggcatgggagctggctttgcattccaatatggcacatccaaaattggtctgcccagttgtcctttagaaaaacttccaaatgtgaagacctgtccatccattaaaagtactgccgtatggttgctgcctgcagtgacttgtgtgctagggcctggcaatgcttgaacaagagtgggacatcccctggagttgacatctccatgtcctagctgcccatgctgcccataaccaaatgtatagacatctccattttccattaaaaccactgaatggtgaaatccacagctgacttggactgcccggagctcacagtcaaatcgcacagagcctggagggtatgttgtgattttgcttgcatccttttcgcctctttctccacttccatctttgtgcttgtcccgtttatgctttagctgtgctggatgggatctgagtctggctagagcctgttctcgatggttcataaaaataggaccagcaaatacaagggggcctcttccttcctctaatctgtgccttctgattacacgttgccgtttttcttcttgtcgtaactgaaggtgttcttcaatgttaaccccgggcactgggacagctaaaagaagatctaaaggtatcatttctttcactgcatcaagaattcctctttgtcttgcctcttgaccatctaactctcttgcacaggccttgcaacatccacacacagcacaaccagattctccggaaccacaaccacagatccctccggggactctgtctggccgtccactactgacacagctggctccataacctgtacagtctccacagacagtgcaaaccatgcactgctccagcttccatttgtgcatgcctggagggcacatcatagacttctcatctttttcatctagttcttcttccaggtcttcatccattgctgttgccatattttcaactccaaaccctttcccaccttggttcatggcaccagtatctcgtccacactgtcctttattatttacaccaaatgtccacacctctccattcttcattaaaacacaagtgtgagctttgcccatagctacctgagttacaaaatggcccttcaaatcagttaccaaacttgaactatcagagtaaatggcatcttttccaaacatgtagagttctccatctttagaaataacagaactacttccattattgcaggctgtatataccacaatctttccttccatcttaattatctttttaggtttataaggtttggattgccgtctgctcttagttgattctccatcttctcctttactagcagatcctgtaaagaatatgctcccatcttctgcaactaaaagggcgtgagagccatcgtgtccaactgagaagtgtactatctttggagattttgtaattggtagctcaacccattttcctgctgaaggaccaccttgtttgattccaagactctggtatttgccagtgtaatatatctttccatttgctgttttcattagcgcaaactctcgtcctgcaccaagaattgctgactcctcatcaaatcctgtacttataatatgcaagtccttttccagatcgaatagtgagataccacaggcatgtaagcattttctagccagtttaagttgcaattcttgctgtagaacaggttcagtgcttgtggcaaatattctgacaacaaagccatcatctcttgaagcagctatctgattaatatattctccatcagtgaataaaatattttgaccttcagtgtggcaatctggtaacatcacagtaccatcttgctccagtgtttcagggcttatccttatggctgtcatgctgtggttattcacatctctatataataaataaccctgagcataccctaaccaagactttttttcttttctgtttctaatacgggatgtagaattgtatatatggcccctaactgttccactgtatccagagcctattttatataatccatccttgcataatagataaagaaaaaatccatcattctgaagtagacattggtcatcttcatcaacagatatttcttttaatggccacttgtgcattaaagctgctttcttaatgccattactaaaccagtcctgaatttgaatttttcccaccaaaactgcttgtacacttctctgtagcgaatttagaattgttggcacctgaatagtttggcaagcatggcttccattgttggtgaggatagcagagatggcctgaagtgtccttcctgtttctccccaagaagccaccagactaaagaggcaagcacaggaaagtgctgttaaggactgtcctgtgctgtcattcatcccagtacttcgaacggtgatttccaaaagaagctggaagagagactctaggacctcaggtggctcagactggaggccttctggctgctggccctgcagcacgttgagcagggcttggagactcctgagacacagggatggatgagaaaatcgtgtctctttgatcaattcaaaaacttcacaaaggccaacctcaataatctttggaagcttgatagggggctctttggattcctcttcttcatcactatctgattctccactctgcacagagttcttagatgcggctgccaatgatatttcctttttctgccattccagaacgcaatggcgtacattacagtaaatattgaaagcagaaggattgctatgtagtttgatatctggtatgattactgtattctctaagttttcagacttgcttcttgtcttcacttttgatttgctcttctgttttcttttcaatttcttcttatttaaaattttcttattcctggaggctgggtgtccagcgctgccgcccccctggtccctgtcattgagcgcagcggtataaatcctccggtagcggtcggccagggcccggcctgacagcagcagctggtagtgaccccgggagtccgcggcgggtagccccagccccagccccgcagcagccacggagccgtcgggaaccggcatgaacagcgcccccggcgccggggaggaagagaaggtggcggctgggtagaatccgtccccgccgagccccgaggaggcggcggcgggggaggcagtcgctgcgcacatcatcatcctcgccgccgccgccgccgccgccgcctcgtccccgcgggccgggcgggcagacacgcgcgcgcacacacagcccttttccaacgacgacggctccggcggcggcctctggctcccgcagcagggagactacaaagacagcgacctccttctcctcctccttcttctcctcctcccccccgcgccgccctcgccgctactggggccgctcatctaaccccgccaccccgggaatgtgaggaggaggcggtgccgccactgccgccgccaccaccgctaccaccgccaccaccgccggggctacccgcaatgggaagctgccg

SEQ ID NO: 17104 - RNA, 9169 nt, Homo sapiens
  source 1..9169: mol_type = other RNA
tcaaaactgaggggcattttcttcttgcggagggtatctggatcaagtgtgtaagagtctgatttagaacgttcccgaggaggatcaagctttgtcttaacaggagcagtacttttttgaggtagatttttatcatgtggtgaggaggagcgtggagaactagcacccgatgggctagacctattggctgggagagtctttggcttaggagatgacaaccgagaacctggtcctggggattcagctctggagctagaaggcatcctcccatcagatttcaatgtctgcaaggtgttatggttgggggataatgacctactgtgggaatctgacctcaactttgcagcatcagattttaagatgagggattcactagcagataaactttctgtgccccttggcttcttctgatcagcagtagtccggctcatacgtccatcaggtttaagcgatctgctgtgtttagaggacagctctgattttcctgatgtagaggctggtttagaagatgttgagatgtttcctcgatcactctgaagctgaggctgctggaaggaaaggggctgtccgaacacaaatgggctgtgtactagggaagagggaggttttgcagcttgatcaaagatggaaggagctgggagattgggtcgtgactgaatggaattcaatatggcactcagttggtcacctttgctatttccgagtccataatcaaatccttgggcactgcaacttgcccctttattaaaagcttgcactgagaaagggcttggaggaggagtttgagaattctgatccagaagagcttgttcatcttcatgtcggaggtactggtttccgcctctgtctctagctaaggaccatgcctctccttcatcactctcacagaactctaccatgctgttctgatccagttgcacccatgtcccttcagaattggttacctctcccactgctttgactttgtttcccagaactaacattccaattgggatacctctaaggttagggcagcttctgatgttgtgacctgaaggtcccgtcttcactaccttgtacatgcctggccctcctcgcaagaatggcatatcttgttcttgcattgttgcttcctgggggaaaaaagctttggaagtccatgaaaatacgtccaaatccctgactccttggctagcattaaagatattgtcaacagggaccagaagactcttgccaagatgttgattaaaagagaggcaccaggcttcagtgtaaccattcatgttagggacatacttctttattgtctcatcattcagcctcagccacacaccatcatcattatggatctcatcaataaaagtgatagttccattgactttcactatgcctatctgctcactctgaagggaagggtggctacggatgcgaagccccgcactgtccttggccacaaattttcgaaccttattaggctgaggttcagactttggtttgaccaactgagttcctggtggtatcatcccttttggtgggtcttttacttttacttccagaccagcatcgatttcaatgccatcaatggtaacatgaagagtgtagagtccaatagcccctggagtccaatttgcacaataagtcccatcattattgacacggatcagcatattctcactgggtctcttaggagttggtgatgcaaaacgtagttcttcaaatgaataattttcataaaccttcatcattgttatggcaatatatcgagcttccttcactatcattggttcatatgaaacatctagctttggtgatgccagccctccataagtcatgtcagtattagaagatgcagctgttactgcaggactgccaggaatcctttgaggtttctttgcttgatcttgttgtaaagacatttttttctgagaaacagggacagctttcacttccaccttcatattgggaacatgtaccacatccccatactggtcttttgtttgaacagttatggtggtaggccaaccacaacgaatatcatccttattcaggatcaaagatgttttctgaggatccgcatatgaatctggctgaagccaccttgcaagccttccaccacttgatcctgggacacaggcaataaaatcatccagaaaagactgttcattgctttggatttggagtggtaaatttccctcaagtgcttctaatatagttggtgaatgagaaagagctagaccctttccaagaattccagaatgggttttgcacacctgcaatgcagcctcctcaagaatttcaaggtcttcttctaattcattaccaataggaagtgctaggtccttcttcatcagagctgctgcacaaaccccaccaagattggctaattctttttccaattggatgactccctcatcaggtccagggctaaattcatatccaattgcaaaacacttaaaaccatagaaagaagctttgtcatctttcacataatctgatgcagtctccaatgaaaaaagggcctcatttcctggcaacaccaaaaccatagtaggccacccagaggatcctgaaaatttctttaattctatccatgaattaagattttcatgaacagatgtcaattttggtccatatcctgaattctgaacagttctgacaggaatcaacaaacgaaggacatcttctgactgtgcagtaccacactgagggtcaaattcgattgtcatccacctcacacattctgggaatgtcaccttgtaatgcatcacacaggcaggtttatacgggtgctcactctctatgacagcatagtgactggaggttgtacaagcagagaggccctgttcaggctggtttcctgtggtgctatctgtcgactgattagggttgaaggcaggcggtgcatacttctgattcaaaatggcaactgacggaagcaattgttggacaaggccaaagacttctacagccaccttgggaatagcagcagctactggtcctatgtaggctataataagggggagcagcatggaaaacagactggaagaactcagcagttctggaatgtcatcagcatccacagcaagagctctgtgcaggaggtccttagaggctcgaacgacagtgcttacaacagacaatgctctgctacagtttttatcttcttcattggctttactcagaagttgggattgtaaatctccatcaaattcactcctatagtagagtatctgtgggatctgtcctctggtttggtttgtgccgttactgctcaagctgcacgtgctgaatgtgaatgtcacaccatcagggcactgaactgtggtcattcctccatctccattggctgtacggcttccatagttcctcaagcgcacagcatatttaacattttcctttaaaggaaccactttgtcaagtctgatctcagctatatcactgggtgagtcatccgttgtgtacgttcctttcactaattccagagatgtccatctgtgggaatgagttgaatctcctgcatgttcactatcatcaaccaacacctctaattcatattcatgaattccacctcctccatagacagagaaaccaaccacaactattccaggtttgtctactgaaaaacagattgcatcaggggacccgttcccagtgttccaacttctgccctgacttgtttttgtaaatcggttagcactagcttttacagagtgaagagaattaagtccatcaacctcagatcccagggctgacgctgtcagttcactgacaatgctggccagtaatccacaggtgttagagacgaggtgggaggagaagagttcattttctctcctcaggctgttcctgactggtagcacaacaatgaccagcattttctccagaacttcacggaagcttgtcatccctgagatattctcttcactctggctgagtttttccatatgtgccaccaaaaggggaaaacgatgaactagtgttgagtcgttctctgtactaacttgtttaacaattgatcgtagtaatacttctccatcatacgcaatcgggaagatggaagtcagcttaacagacgtgtgacacagagctgacataacagctgcaaggagtcggctacttgatgtcttgaagtttgcttcttggatatcctgatccaaacaattcagcagatcacaaaggcaagcccactgtaaggcaggagttgggtagaaagaatgaaagcaggcagtgaaagtattatgacattcctgaaggacagcttctagaagactcaagggttgactgagatatccttgaggatcattatccaatttcaccatgcagtgatcaactccttctgataaaatttttcttaacaaagttctggtttttccaatacactctgctaatttgctagtttcttctacaactgcttttcctgtagctgacactgggtaaatttcacaggtatagacacgcaataacctcagacaacaggtacccacaaagcgcagtctctctaaatctaggagtgtagctgtgaactggaatccttttaatcctctaagttcttcaactcctaagactaaggtggtccagctccagtgaagaatactcaacaatgactcaaaacattccactgagacagttcttgcaaaagacctctttaaaatgtgtacaggttcactggtttgctgtttgccttttgaagcactgccatcactggttggaagtctgtataataactgaggtatctgacccgcattaacatctgtaccattatttgatttctttgaactcttgaactggaaaacaaccccatcatctgtggtaatagatgcctgtccatgagatccacagtcactgctgggtcctgacactcgggcccatgccacataccaccacccagcttgcaggagaacaggctcatcaaacatcattgcatatttttctctagcagcacagtcataagccaatacatcagtctctgcaagaaggtcaccatcagtttcatgatctcctccatcaggacccaattcaaacagcttaattttagcagtatattctcctctacctccaaacagaccaagaccaccaagtaaaatatcagtgtcggcactgaaacgtatagcttctactgaatgggcagaataaccccagcctcctccatgactttcaaacctgtttaccacactataatcttctttagaataaaccttcattactgcttgagtctcttcctctgtacttgcaacacccatttttaagtcctgcatagctgccaaggtatcaagacaacctaaaatgtgcaaagctgcatgagatcgggtagtgagggcccttgatcctgttggtaaggcaagttcaggacttaggatactacatctggactgcatgtctgctgcagagggaagcctggcatcagcaaccaccgcattgtaacaccacagctctctagtatttggtcgaaacctccaaattacatcatatacaggatcaagacacacaccaaatccttgcagatcctcttgttctgagtcattaaaagttttacaactcccatccactttatttatcagaaggcatttaaatggaggaggttctgatatagaagcaggtaccaagcctattatgtgtttactggcaaaaatttctgatgtagcaagtacatgagaattaataagtgcttcatcaattcgtaaaaaagtttggtccccacttgcacctatccaagtagcttttcttccatattttgatccaatgttaggcatgggagctggctttgcattccaatatggcacatccaaaattggtctgcccagttgtcctttagaaaaacttccaaatgtgaagacctgtccatccattaaaagtactgccgtatggttgctgcctgcagtgacttgtgtgctagggcctggcaatgcttgaacaagagtgggacatcccctggagttgacatctccatgtcctagctgcccatgctgcccataaccaaatgtatagacatctccattttccattaaaaccactgaatggtgaaatccacagctgacttggactgcccggagctcacagtcaaatcgcacagagcctggagggtatgttgtgattttgcttgcatccttttcgcctctttctccacttccatctttgtgcttgtcccgtttatgctttagctgtgctggatgggatctgagtctggctagagcctgttctcgatggttcataaaaataggaccagcaaatacaagggggcctcttccttcctctaatctgtgccttctgattacacgttgccgtttttcttcttgtcgtaactgaaggtgttcttcaatgttaaccccgggcactgggacagctaaaagaagatctaaaggtatcatttctttcactgcatcaagaattcctctttgtcttgcctcttgaccatctaactctcttgcacaggccttgcaacatccacacacagcacaaccagattctccggaaccacaaccacagatccctccggggactctgtctggccgtccactactgacacagctggctccataacctgtacagtctccacagacagtgcaaaccatgcactgctccagcttccatttgtgcatgcctggagggcacatcatagacttctcatctttttcatctagttcttcttccaggtcttcatccattgctgttgccatattttcaactccaaaccctttcccaccttggttcatggcaccagtatctcgtccacactgtcctttattatttacaccaaatgtccacacctctccattcttcattaaaacacaagtgtgagctttgcccatagctacctgagttacaaaatggcccttcaaatcagttaccaaacttgaactatcagagtaaatggcatcttttccaaacatgtagagttctccatctttagaaataacagaactacttccattattgcaggctgtatataccacaatctttccttccatcttaattatctttttaggtttataaggtttggattgccgtctgctcttagttgattctccatcttctcctttactagcagatcctgtaaagaatatgctcccatcttctgcaactaaaagggcgtgagagccatcgtgtccaactgagaagtgtactatctttggagattttgtaattggtagctcaacccattttcctgctgaaggaccaccttgtttgattccaagactctggtatttgccagtgtaatatatctttccatttgctgttttcattagcgcaaactctcgtcctgcaccaagaattgctgactcctcatcaaatcctgtacttataatatgcaagtccttttccagatcgaatagtgagataccacaggcatgtaagcattttctagccagtttaagttgcaattcttgctgtagaacaggttcagtgcttgtggcaaatattctgacaacaaagccatcatctcttgaagcagctatctgattaatatattctccatcagtgaataaaatattttgaccttcagtgtggcaatctggtaacatcacagtaccatcttgctccagtgtttcagggcttatccttatggctgtcatgctgtggttattcacatctctatataataaataaccctgagcataccctaaccaagactttttttcttttctgtttctaatacgggatgtagaattgtatatatggcccctaactgttccactgtatccagagcctattttatataatccatccttgcataatagataaagaaaaaatccatcattctgaagtagacattggtcatcttcatcaacagatatttcttttaatggccacttgtgcattaaagctgctttcttaatgccattactaaaccagtcctgaatttgaatttttcccaccaaaactgcttgtacacttctctgtagcgaatttagaattgttggcacctgaatagtttggcaagcatggcttccattgttggtgaggatagcagagatggcctgaagtgtccttcctgtttctccccaagaagccaccagactaaagaggcaagcacaggaaagtgctgttaaggactgtcctgtgctgtcattcatcccagtacttcgaacggtgatttccaaaagaagctggaagagagactctaggacctcaggtggctcagactggaggccttctggctgctggccctgcagcacgttgagcagggcttggagactcctgagacacagggatggatgagaaaatcgtgtctctttgatcaattcaaaaacttcacaaaggccaacctcaataatctttggaagcttgatagggggctctttggattcctcttcttcatcactatctgattctccactctgcacagagttcttagatgcggctgccaatgatatttcctttttctgccattccagaacgcaatggcgtacattacagtaaatattgaaagcagaaggattgctatgtagtttgatatctggtatgattactgtattctctaagttttcagacttgcttcttgtcttcacttttgatttgctcttctgttttcttttcaatttcttcttatttaaaattttcttattcctggaggctgggtgtccagcgctgccgcccccctggtccctgtcattgagcgcagcggtataaatcctccggtagcggtcggccagggcccggcctgacagcagcagctggtagtgaccccgggagtccgcggcgggtagccccagccccagccccgcagcagccacggagccgtcgggaaccggcatgaacagcgcccccggcgccggggaggaagagaaggtggcggctgggtagaatccgtccccgccgagccccgaggaggcggcggcgggggaggcagtcgctgcgcacatcatcatcctcgccgccgccgccgccgccgccgcctcgtccccgcgggccgggcgggcagacacgcgcgcgcacacacagcccttttccaacgacgacggctccggcggcggcctctggctcccgcagcagggagactacaaagacagcgacctccttctcctcctccttcttctcctcctcccccccgcgccgccctcgccgctactggggccgctcatctaaccccgccaccccgggaatgtgaggaggaggcggtgccgccactgccgccgccaccaccgctaccaccgccaccaccgccggggctacccgcaatgggaagctgccg

SEQ ID NO: 17105 - RNA, 9118 nt, Homo sapiens
  source 1..9118: mol_type = other RNA
tcaaaactgaggggcattttcttcttgcggagggtatctggatcaagtgtgtaagagtctgatttagaacgttcccgaggaggatcaagctttgtcttaacaggagcagtacttttttgaggtagatttttatcatgtggtgaggaggagcgtggagaactagcacccgatgggctagacctattggctgggagagtctttggcttaggagatgacaaccgagaacctggtcctggggattcagctctggagctagaaggcatcctcccatcagatttcaatgtctgcaaggtgttatggttgggggataatgacctactgtgggaatctgacctcaactttgcagcatcagattttaagatgagggattcactagcagataaactttctgtgccccttggcttcttctgatcagcagtagtccggctcatacgtccatcaggtttaagcgatctgctgtgtttagaggacagctctgattttcctgatgtagaggctggtttagaagatgttgagatgtttcctcgatcactctgaagctgaggctgctggaaggaaaggggctgtccgaacacaaatgggctgtgtactagggaagagggaggttttgcagcttgatcaaagatggaaggagctgggagattgggtcgtgactgaatggaattcaatatggcactcagttggtcacctttgctatttccgagtccataatcaaatccttgggcactgcaacttgcccctttattaaaagcttgcactgagaaagggcttggaggaggagtttgagaattctgatccagaagagcttgttcatcttcatgtcggaggtactggtttccgcctctgtctctagctaaggaccatgcctctccttcatcactctcacagaactctaccatgctgttctgatccagttgcacccatgtcccttcagaattggttacctctcccactgctttgactttgtttcccagaactaacattccaattgggatacctctaaggttagggcagcttctgatgttgtgacctgaaggtcccgtcttcactaccttgtacatgcctggccctcctcgcaagaatggcatatcttgttcttgcattgttgcttcctgtgggcagcaggagtttatgtctttgaaaaagtcatcagtattagttttagattcctgggggaaaaaagctttggaagtccatgaaaatacgtccaaatccctgactccttggctagcattaaagatattgtcaacagggaccagaagactcttgccaagatgttgattaaaagagaggcaccaggcttcagtgtaaccattcatgttagggacatacttctttattgtctcatcattcagcctcagccacacaccatcatcattatggatctcatcaataaaagtgatagttccattgactttcactatgcctatctgctcactctgaagggaagggtggctacggatgcgaagccccgcactgtccttggccacaaattttcgaaccttattaggctgaggttcagactttggtttgaccaactgagttcctggtggtatcatcccttttggtgggtcttttacttttacttccagaccagcatcgatttcaatgccatcaatggtaacatgaagagtgtagagtccaatagcccctggagtccaatttgcacaataagtcccatcattattgacacggatcagcatattctcactgggtctcttaggagttggtgatgcaaaacgtagttcttcaaatgaataattttcataaaccttcatcattgttatggcaatatatcgagcttccttcactatcattggttcatatgaaacatctagctttggtgatgccagccctccataagtcatgtcagtattagaagatgcagctgttactgcaggactgccaggaatcctttgaggtttctttgcttgatcttgttgtaaagacatttttttctgagaaacagggacagctttcacttccaccttcatattgggaacatgtaccacatccccatactggtcttttgtttgaacagttatggtggtaggccaaccacaacgaatatcatccttattcaggatcaaagatgttttctgaggatccgcatatgaatctggctgaagccaccttgcaagccttccaccacttgatcctgggacacaggcaataaaatcatccagaaaagactgttcattgctttggatttggagtggtaaatttccctcaagtgcttctaatatagttggtgaatgagaaagagctagaccctttccaagaattccagaatgggttttgcacacctgcaatgcagcctcctcaagaatttcaaggtcttcttctaattcattaccaataggaagtgctaggtccttcttcatcagagctgctgcacaaaccccaccaagattggctaattctttttccaattggatgactccctcatcaggtccagggctaaattcatatccaattgcaaaacacttaaaaccatagaaagaagctttgtcatctttcacataatctgatgcagtctccaatgaaaaaagggcctcatttcctggcaacaccaaaaccatagtaggccacccagaggatcctgaaaatttctttaattctatccatgaattaagattttcatgaacagatgtcaattttggtccatatcctgaattctgaacagttctgacaggaatcaacaaacgaaggacatcttctgactgtgcagtaccacactgagggtcaaattcgattgtcatccacctcacacattctgggaatgtcaccttgtaatgcatcacacaggcaggtttatacgggtgctcactctctatgacagcatagtgactggaggttgtacaagcagagaggccctgttcaggctggtttcctgtggtgctatctgtcgactgattagggttgaaggcaggcggtgcatacttctgattcaaaatggcaactgacggaagcaattgttggacaaggccaaagacttctacagccaccttgggaatagcagcagctactggtcctatgtaggctataataagggggagcagcatggaaaacagactggaagaactcagcagttctggaatgtcatcagcatccacagcaagagctctgtgcaggaggtccttagaggctcgaacgacagtgcttacaacagacaatgctctgctacagtttttatcttcttcattggctttactcagaagttgggattgtaaatctccatcaaattcactcctatagtagagtatctgtgggatctgtcctctggtttggtttgtgccgttactgctcaagctgcacgtgctgaatgtgaatgtcacaccatcagggcactgaactgtggtcattcctccatctccattggctgtacggcttccatagttcctcaagcgcacagcatatttaacattttcctttaaaggaaccactttgtcaagtctgatctcagctatatcactgggtgagtcatccgttgtgtacgttcctttcactaattccagagatgtccatctgtgggaatgagttgaatctcctgcatgttcactatcatcaaccaacacctctaattcatattcatgaattccacctcctccatagacagagaaaccaaccacaactattccaggtttgtctactgaaaaacagattgcatcaggggacccgttcccagtgttccaacttctgccctgacttgtttttgtaaatcggttagcactagcttttacagagtgaagagaattaagtccatcaacctcagatcccagggctgacgctgtcagttcactgacaatgctggccagtaatccacaggtgttagagacgaggtgggaggagaagagttcattttctctcctcaggctgttcctgactggtagcacaacaatgaccagcattttctccagaacttcacggaagcttgtcatccctgagatattctcttcactctggctgagtttttccatatgtgccaccaaaaggggaaaacgatgaactagtgttgagtcgttctctgtactaacttgtttaacaattgatcgtagtaatacttctccatcatacgcaatcgggaagatggaagtcagcttaacagacgtgtgacacagagctgacataacagctgcaaggagtcggctacttgatgtcttgaagtttgcttcttggatatcctgatccaaacaattcagcagatcacaaaggcaagcccactgtaaggcaggagttgggtagaaagaatgaaagcaggcagtgaaagtattatgacattcctgaaggacagcttctagaagactcaagggttgactgagatatccttgaggatcattatccaatttcaccatgcagtgatcaactccttctgataaaatttttcttaacaaagttctggtttttccaatacactctgctaatttgctagtttcttctacaactgcttttcctgtagctgacactgggtaaatttcacaggtatagacacgcaataacctcagacaacaggtacccacaaagcgcagtctctctaaatctaggagtgtagctgtgaactggaatccttttaatcctctaagttcttcaactcctaagactaaggtggtccagctccagtgaagaatactcaacaatgactcaaaacattccactgagacagttcttgcaaaagacctctttaaaatgtgtacaggttcactggtttgctgtttgccttttgaagcactgccatcactggttggaagtctgtataataactgaggtatctgacccgcattaacatctgtaccattatttgatttctttgaactcttgaactggaaaacaaccccatcatctgtggtaatagatgcctgtccatgagatccacagtcactgctgggtcctgacactcgggcccatgccacataccaccacccagcttgcaggagaacaggctcatcaaacatcattgcatatttttctctagcagcacagtcataagccaatacatcagtctctgcaagaaggtcaccatcagtttcatgatctcctccatcaggacccaattcaaacagcttaattttagcagtatattctcctctacctccaaacagaccaagaccaccaagtaaaatatcagtgtcggcactgaaacgtatagcttctactgaatgggcagaataaccccagcctcctccatgactttcaaacctgtttaccacactataatcttctttagaataaaccttcattactgcttgagtctcttcctctgtacttgcaacacccatttttaagtcctgcatagctgccaaggtatcaagacaacctaaaatgtgcaaagctgcatgagatcgggtagtgagggcccttgatcctgttggtaaggcaagttcaggacttaggatactacatctggactgcatgtctgctgcagagggaagcctggcatcagcaaccaccgcattgtaacaccacagctctctagtatttggtcgaaacctccaaattacatcatatacaggatcaagacacacaccaaatccttgcagatcctcttgttctgagtcattaaaagttttacaactcccatccactttatttatcagaaggcatttaaatggaggaggttctgatatagaagcaggtaccaagcctattatgtgtttactggcaaaaatttctgatgtagcaagtacatgagaattaataagtgcttcatcaattcgtaaaaaagtttggtccccacttgcacctatccaagtagcttttcttccatattttgatccaatgttaggcatgggagctggctttgcattccaatatggcacatccaaaattggtctgcccagttgtcctttagaaaaacttccaaatgtgaagacctgtccatccattaaaagtactgccgtatggttgctgcctgcagtgacttgtgtgctagggcctggcaatgcttgaacaagagtgggacatcccctggagttgacatctccatgtcctagctgcccatgctgcccataaccaaatgtatagacatctccattttccattaaaaccactgaatggtgaaatccacagctgacttggactgcccggagctcacagtcaaatcgcacagagcctggagggtatgttgtgattttgcttgcatccttttcgcctctttctccacttccatctcttccttcctctaatctgtgccttctgattacacgttgccgtttttcttcttgtcgtaactgaaggtgttcttcaatgttaaccccgggcactgggacagctaaaagaagatctaaaggtatcatttctttcactgcatcaagaattcctctttgtcttgcctcttgaccatctaactctcttgcacaggccttgcaacatccacacacagcacaaccagattctccggaaccacaaccacagatccctccggggactctgtctggccgtccactactgacacagctggctccataacctgtacagtctccacagacagtgcaaaccatgcactgctccagcttccatttgtgcatgcctggagggcacatcatagacttctcatctttttcatctagttcttcttccaggtcttcatccattgctgttgccatattttcaactccaaaccctttcccaccttggttcatggcaccagtatctcgtccacactgtcctttattatttacaccaaatgtccacacctctccattcttcattaaaacacaagtgtgagctttgcccatagctacctgagttacaaaatggcccttcaaatcagttaccaaacttgaactatcagagtaaatggcatcttttccaaacatgtagagttctccatctttagaaataacagaactacttccattattgcaggctgtatataccacaatctttccttccatcttaattatctttttaggtttataaggtttggattgccgtctgctcttagttgattctccatcttctcctttactagcagatcctgtaaagaatatgctcccatcttctgcaactaaaagggcgtgagagccatcgtgtccaactgagaagtgtactatctttggagattttgtaattggtagctcaacccattttcctgctgaaggaccaccttgtttgattccaagactctggtatttgccagtgtaatatatctttccatttgctgttttcattagcgcaaactctcgtcctgcaccaagaattgctgactcctcatcaaatcctgtacttataatatgcaagtccttttccagatcgaatagtgagataccacaggcatgtaagcattttctagccagtttaagttgcaattcttgctgtagaacaggttcagtgcttgtggcaaatattctgacaacaaagccatcatctcttgaagcagctatctgattaatatattctccatcagtgaataaaatattttgaccttcagtgtggcaatctggtaacatcacagtaccatcttgctccagtgtttcagggcttatccttatggctgtcatgctgtggttattcacatctctatataataaataaccctgagcataccctaaccaagactttttttcttttctgtttctaatacgggatgtagaattgtatatatggcccctaactgttccactgtatccagagcctattttatataatccatccttgcataatagataaagaaaaaatccatcattctgaagtagacattggtcatcttcatcaacagatatttcttttaatggccacttgtgcattaaagctgctttcttaatgccattactaaaccagtcctgaatttgaatttttcccaccaaaactgcttgtacacttctctgtagcgaatttagaattgttggcacctgaatagtttggcaagcatggcttccattgttggtgaggatagcagagatggcctgaagtgtccttcctgtttctccccaagaagccaccagactaaagaggcaagcacaggaaagtgctgttaaggactgtcctgtgctgtcattcatcccagtacttcgaacggtgatttccaaaagaagctggaagagagactctaggacctcaggtggctcagactggaggccttctggctgctggccctgcagcacgttgagcagggcttggagactcctgagacacagggatggatgagaaaatcgtgtctctttgatcaattcaaaaacttcacaaaggccaacctcaataatctttggaagcttgatagggggctctttggattcctcttcttcatcactatctgattctccactctgcacagagttcttagatgcggctgccaatgatatttcctttttctgccattccagaacgcaatggcgtacattacagtaaatattgaaagcagaaggattgctatgtagtttgatatctggtatgattactgtattctctaagttttcagacttgcttcttgtcttcacttttgatttgctcttctgttttcttttcaatttcttcttatttaaaattttcttattcctggaggctgggtgtccagcgctgccgcccccctggtccctgtcattgagcgcagcggtataaatcctccggtagcggtcggccagggcccggcctgacagcagcagctggtagtgaccccgggagtccgcggcgggtagccccagccccagccccgcagcagccacggagccgtcgggaaccggcatgaacagcgcccccggcgccggggaggaagagaaggtggcggctgggtagaatccgtccccgccgagccccgaggaggcggcggcgggggaggcagtcgctgcgcacatcatcatcctcgccgccgccgccgccgccgccgcctcgtccccgcgggccgggcgggcagacacgcgcgcgcacacacagcccttttccaacgacgacggctccggcggcggcctctggctcccgcagcagggagactacaaagacagcgacctccttctcctcctccttcttctcctcctcccccccgcgccgccctcgccgctactggggccgctcatctaaccccgccaccccgggaatgtgaggaggaggcggtgccgccactgccgccgccaccaccgctaccaccgccaccaccgccggggctacccgcaatgggaagctgccg

SEQ ID NO: 17106 - RNA, 9226 nt, Homo sapiens
  source 1..9226: mol_type = other RNA
tcaaaactgaggggcattttcttcttgcggagggtatctggatcaagtgtgtaagagtctgatttagaacgttcccgaggaggatcaagctttgtcttaacaggagcagtacttttttgaggtagatttttatcatgtggtgaggaggagcgtggagaactagcacccgatgggctagacctattggctgggagagtctttggcttaggagatgacaaccgagaacctggtcctggggattcagctctggagctagaaggcatcctcccatcagatttcaatgtctgcaaggtgttatggttgggggataatgacctactgtgggaatctgacctcaactttgcagcatcagattttaagatgagggattcactagcagataaactttctgtgccccttggcttcttctgatcagcagtagtccggctcatacgtccatcaggtttaagcgatctgctgtgtttagaggacagctctgattttcctgatgtagaggctggtttagaagatgttgagatgtttcctcgatcactctgaagctgaggctgctggaaggaaaggggctgtccgaacacaaatgggctgtgtactagggaagagggaggttttgcagcttgatcaaagatggaaggagctgggagattgggtcgtgactgaatggaattcaatatggcactcagttggtcacctttgctatttccgagtccataatcaaatccttgggcactgcaacttgcccctttattaaaagcttgcactgagaaagggcttggaggaggagtttgagaattctgatccagaagagcttgttcatcttcatgtcggaggtactggtttccgcctctgtctctagctaaggaccatgcctctccttcatcactctcacagaactctaccatgctgttctgatccagttgcacccatgtcccttcagaattggttacctctcccactgctttgactttgtttcccagaactaacattccaattgggatacctctaaggttagggcagcttctgatgttgtgacctgaaggtcccgtcttcactaccttgtacatgcctggccctcctcgcaagaatggcatatcttgttcttgcattgttgcttcctgtgggcagcaggagtttatgtctttgaaaaagtcatcagtattagttttagattcctgggggaaaaaagctttggaagtccatgaaaatacgtccaaatccctgactccttggctagcattaaagatattgtcaacagggaccagaagactcttgccaagatgttgattaaaagagaggcaccaggcttcagtgtaaccattcatgttagggacatacttctttattgtctcatcattcagcctcagccacacaccatcatcattatggatctcatcaataaaagtgatagttccattgactttcactatgcctatctgctcactctgaagggaagggtggctacggatgcgaagccccgcactgtccttggccacaaattttcgaaccttattaggctgaggttcagactttggtttgaccaactgagttcctggtggtatcatcccttttggtgggtcttttacttttacttccagaccagcatcgatttcaatgccatcaatggtaacatgaagagtgtagagtccaatagcccctggagtccaatttgcacaataagtcccatcattattgacacggatcagcatattctcactgggtctcttaggagttggtgatgcaaaacgtagttcttcaaatgaataattttcataaaccttcatcattgttatggcaatatatcgagcttccttcactatcattggttcatatgaaacatctagctttggtgatgccagccctccataagtcatgtcagtattagaagatgcagctgttactgcaggactgccaggaatcctttgaggtttctttgcttgatcttgttgtaaagacatttttttctgagaaacagggacagctttcacttccaccttcatattgggaacatgtaccacatccccatactggtcttttgtttgaacagttatggtggtaggccaaccacaacgaatatcatccttattcaggatcaaagatgttttctgaggatccgcatatgaatctggctgaagccaccttgcaagccttccaccacttgatcctgggacacaggcaataaaatcatccagaaaagactgttcattgctttggatttggagtggtaaatttccctcaagtgcttctaatatagttggtgaatgagaaagagctagaccctttccaagaattccagaatgggttttgcacacctgcaatgcagcctcctcaagaatttcaaggtcttcttctaattcattaccaataggaagtgctaggtccttcttcatcagagctgctgcacaaaccccaccaagattggctaattctttttccaattggatgactccctcatcaggtccagggctaaattcatatccaattgcaaaacacttaaaaccatagaaagaagctttgtcatctttcacataatctgatgcagtctccaatgaaaaaagggcctcatttcctggcaacaccaaaaccatagtaggccacccagaggatcctgaaaatttctttaattctatccatgaattaagattttcatgaacagatgtcaattttggtccatatcctgaattctgaacagttctgacaggaatcaacaaacgaaggacatcttctgactgtgcagtaccacactgagggtcaaattcgattgtcatccacctcacacattctgggaatgtcaccttgtaatgcatcacacaggcaggtttatacgggtgctcactctctatgacagcatagtgactggaggttgtacaagcagagaggccctgttcaggctggtttcctgtggtgctatctgtcgactgattagggttgaaggcaggcggtgcatacttctgattcaaaatggcaactgacggaagcaattgttggacaaggccaaagacttctacagccaccttgggaatagcagcagctactggtcctatgtaggctataataagggggagcagcatggaaaacagactggaagaactcagcagttctggaatgtcatcagcatccacagcaagagctctgtgcaggaggtccttagaggctcgaacgacagtgcttacaacagacaatgctctgctacagtttttatcttcttcattggctttactcagaagttgggattgtaaatctccatcaaattcactcctatagtagagtatctgtgggatctgtcctctggtttggtttgtgccgttactgctcaagctgcacgtgctgaatgtgaatgtcacaccatcagggcactgaactgtggtcattcctccatctccattggctgtacggcttccatagttcctcaagcgcacagcatatttaacattttcctttaaaggaaccactttgtcaagtctgatctcagctatatcactgggtgagtcatccgttgtgtacgttcctttcactaattccagagatgtccatctgtgggaatgagttgaatctcctgcatgttcactatcatcaaccaacacctctaattcatattcatgaattccacctcctccatagacagagaaaccaaccacaactattccaggtttgtctactgaaaaacagattgcatcaggggacccgttcccagtgttccaacttctgccctgacttgtttttgtaaatcggttagcactagcttttacagagtgaagagaattaagtccatcaacctcagatcccagggctgacgctgtcagttcactgacaatgctggccagtaatccacaggtgttagagacgaggtgggaggagaagagttcattttctctcctcaggctgttcctgactggtagcacaacaatgaccagcattttctccagaacttcacggaagcttgtcatccctgagatattctcttcactctggctgagtttttccatatgtgccaccaaaaggggaaaacgatgaactagtgttgagtcgttctctgtactaacttgtttaacaattgatcgtagtaatacttctccatcatacgcaatcgggaagatggaagtcagcttaacagacgtgtgacacagagctgacataacagctgcaaggagtcggctacttgatgtcttgaagtttgcttcttggatatcctgatccaaacaattcagcagatcacaaaggcaagcccactgtaaggcaggagttgggtagaaagaatgaaagcaggcagtgaaagtattatgacattcctgaaggacagcttctagaagactcaagggttgactgagatatccttgaggatcattatccaatttcaccatgcagtgatcaactccttctgataaaatttttcttaacaaagttctggtttttccaatacactctgctaatttgctagtttcttctacaactgcttttcctgtagctgacactgggtaaatttcacaggtatagacacgcaataacctcagacaacaggtacccacaaagcgcagtctctctaaatctaggagtgtagctgtgaactggaatccttttaatcctctaagttcttcaactcctaagactaaggtggtccagctccagtgaagaatactcaacaatgactcaaaacattccactgagacagttcttgcaaaagacctctttaaaatgtgtacaggttcactggtttgctgtttgccttttgaagcactgccatcactggttggaagtctgtataataactgaggtatctgacccgcattaacatctgtaccattatttgatttctttgaactcttgaactggaaaacaaccccatcatctgtggtaatagatgcctgtccatgagatccacagtcactgctgggtcctgacactcgggcccatgccacataccaccacccagcttgcaggagaacaggctcatcaaacatcattgcatatttttctctagcagcacagtcataagccaatacatcagtctctgcaagaaggtcaccatcagtttcatgatctcctccatcaggacccaattcaaacagcttaattttagcagtatattctcctctacctccaaacagaccaagaccaccaagtaaaatatcagtgtcggcactgaaacgtatagcttctactgaatgggcagaataaccccagcctcctccatgactttcaaacctgtttaccacactataatcttctttagaataaaccttcattactgcttgagtctcttcctctgtacttgcaacacccatttttaagtcctgcatagctgccaaggtatcaagacaacctaaaatgtgcaaagctgcatgagatcgggtagtgagggcccttgatcctgttggtaaggcaagttcaggacttaggatactacatctggactgcatgtctgctgcagagggaagcctggcatcagcaaccaccgcattgtaacaccacagctctctagtatttggtcgaaacctccaaattacatcatatacaggatcaagacacacaccaaatccttgcagatcctcttgttctgagtcattaaaagttttacaactcccatccactttatttatcagaaggcatttaaatggaggaggttctgatatagaagcaggtaccaagcctattatgtgtttactggcaaaaatttctgatgtagcaagtacatgagaattaataagtgcttcatcaattcgtaaaaaagtttggtccccacttgcacctatccaagtagcttttcttccatattttgatccaatgttaggcatgggagctggctttgcattccaatatggcacatccaaaattggtctgcccagttgtcctttagaaaaacttccaaatgtgaagacctgtccatccattaaaagtactgccgtatggttgctgcctgcagtgacttgtgtgctagggcctggcaatgcttgaacaagagtgggacatcccctggagttgacatctccatgtcctagctgcccatgctgcccataaccaaatgtatagacatctccattttccattaaaaccactgaatggtgaaatccacagctgacttggactgcccggagctcacagtcaaatcgcacagagcctggagggtatgttgtgattttgcttgcatccttttcgcctctttctccacttccatctttgtgcttgtcccgtttatgctttagctgtgctggatgggatctgagtctggctagagcctgttctcgatggttcataaaaataggaccagcaaatacaagggggcctcttccttcctctaatctgtgccttctgattacacgttgccgtttttcttcttgtcgtaactgaaggtgttcttcaatgttaaccccgggcactgggacagctaaaagaagatctaaaggtatcatttctttcactgcatcaagaattcctctttgtcttgcctcttgaccatctaactctcttgcacaggccttgcaacatccacacacagcacaaccagattctccggaaccacaaccacagatccctccggggactctgtctggccgtccactactgacacagctggctccataacctgtacagtctccacagacagtgcaaaccatgcactgctccagcttccatttgtgcatgcctggagggcacatcatagacttctcatctttttcatctagttcttcttccaggtcttcatccattgctgttgccatattttcaactccaaaccctttcccaccttggttcatggcaccagtatctcgtccacactgtcctttattatttacaccaaatgtccacacctctccattcttcattaaaacacaagtgtgagctttgcccatagctacctgagttacaaaatggcccttcaaatcagttaccaaacttgaactatcagagtaaatggcatcttttccaaacatgtagagttctccatctttagaaataacagaactacttccattattgcaggctgtatataccacaatctttccttccatcttaattatctttttaggtttataaggtttggattgccgtctgctcttagttgattctccatcttctcctttactagcagatcctgtaaagaatatgctcccatcttctgcaactaaaagggcgtgagagccatcgtgtccaactgagaagtgtactatctttggagattttgtaattggtagctcaacccattttcctgctgaaggaccaccttgtttgattccaagactctggtatttgccagtgtaatatatctttccatttgctgttttcattagcgcaaactctcgtcctgcaccaagaattgctgactcctcatcaaatcctgtacttataatatgcaagtccttttccagatcgaatagtgagataccacaggcatgtaagcattttctagccagtttaagttgcaattcttgctgtagaacaggttcagtgcttgtggcaaatattctgacaacaaagccatcatctcttgaagcagctatctgattaatatattctccatcagtgaataaaatattttgaccttcagtgtggcaatctggtaacatcacagtaccatcttgctccagtgtttcagggcttatccttatggctgtcatgctgtggttattcacatctctatataataaataaccctgagcataccctaaccaagactttttttcttttctgtttctaatacgggatgtagaattgtatatatggcccctaactgttccactgtatccagagcctattttatataatccatccttgcataatagataaagaaaaaatccatcattctgaagtagacattggtcatcttcatcaacagatatttcttttaatggccacttgtgcattaaagctgctttcttaatgccattactaaaccagtcctgaatttgaatttttcccaccaaaactgcttgtacacttctctgtagcgaatttagaattgttggcacctgaatagtttggcaagcatggcttccattgttggtgaggatagcagagatggcctgaagtgtccttcctgtttctccccaagaagccaccagactaaagaggcaagcacaggaaagtgctgttaaggactgtcctgtgctgtcattcatcccagtacttcgaacggtgatttccaaaagaagctggaagagagactctaggacctcaggtggctcagactggaggccttctggctgctggccctgcagcacgttgagcagggcttggagactcctgagacacagggatggatgagaaaatcgtgtctctttgatcaattcaaaaacttcacaaaggccaacctcaataatctttggaagcttgatagggggctctttggattcctcttcttcatcactatctgattctccactctgcacagagttcttagatgcggctgccaatgatatttcctttttctgccattccagaacgcaatggcgtacattacagtaaatattgaaagcagaaggattgctatgtagtttgatatctggtatgattactgtattctctaagttttcagacttgcttcttgtcttcacttttgatttgctcttctgttttcttttcaatttcttcttatttaaaattttcttattcctggaggctgggtgtccagcgctgccgcccccctggtccctgtcattgagcgcagcggtataaatcctccggtagcggtcggccagggcccggcctgacagcagcagctggtagtgaccccgggagtccgcggcgggtagccccagccccagccccgcagcagccacggagccgtcgggaaccggcatgaacagcgcccccggcgccggggaggaagagaaggtggcggctgggtagaatccgtccccgccgagccccgaggaggcggcggcgggggaggcagtcgctgcgcacatcatcatcctcgccgccgccgccgccgccgccgcctcgtccccgcgggccgggcgggcagacacgcgcgcgcacacacagcccttttccaacgacgacggctccggcggcggcctctggctcccgcagcagggagactacaaagacagcgacctccttctcctcctccttcttctcctcctcccccccgcgccgccctcgccgctactggggccgctcatctaaccccgccaccccgggaatgtgaggaggaggcggtgccgccactgccgccgccaccaccgctaccaccgccaccaccgccggggctacccgcaatgggaagctgccg

SEQ ID NO: 17107 - RNA, 9151 nt, Homo sapiens
  source 1..9151: mol_type = other RNA
tcaaaactgaggggcattttcttcttgcggagggtatctggatcaagtgtgtaagagtctgatttagaacgttcccgaggaggatcaagctttgtcttaacaggagcagtacttttttgaggtagatttttatcatgtggtgaggaggagcgtggagaactagcacccgatgggctagacctattggctgggagagtctttggcttaggagatgacaaccgagaacctggtcctggggattcagctctggagctagaaggcatcctcccatcagatttcaatgtctgcaaggtgttatggttgggggataatgacctactgtgggaatctgacctcaactttgcagcatcagattttaagatgagggattcactagcagataaactttctgtgccccttggcttcttctgatcagcagtagtccggctcatacgtccatcaggtttaagcgatctgctgtgtttagaggacagctctgattttcctgatgtagaggctggtttagaagatgttgagatgtttcctcgatcactctgaagctgaggctgctggaaggaaaggggctgtccgaacacaaatgggctgtgtactagggaagagggaggttttgcagcttgatcaaagatggaaggagctgggagattgggtcgtgactgaatggaattcaatatggcactcagttggtcacctttgctatttccgagtccataatcaaatccttgggcactgcaacttgcccctttattaaaagcttgcactgagaaagggcttggaggaggagtttgagaattctgatccagaagagcttgttcatcttcatgtcggaggtactggtttccgcctctgtctctagctaaggaccatgcctctccttcatcactctcacagaactctaccatgctgttctgatccagttgcacccatgtcccttcagaattggttacctctcccactgctttgactttgtttcccagaactaacattccaattgggatacctctaaggttagggcagcttctgatgttgtgacctgaaggtcccgtcttcactaccttgtacatgcctggccctcctcgcaagaatggcatatcttgttcttgcattgttgcttcctgtgggcagcaggagtttatgtctttgaaaaagtcatcagtattagttttagattcgtcaacagggaccagaagactcttgccaagatgttgattaaaagagaggcaccaggcttcagtgtaaccattcatgttagggacatacttctttattgtctcatcattcagcctcagccacacaccatcatcattatggatctcatcaataaaagtgatagttccattgactttcactatgcctatctgctcactctgaagggaagggtggctacggatgcgaagccccgcactgtccttggccacaaattttcgaaccttattaggctgaggttcagactttggtttgaccaactgagttcctggtggtatcatcccttttggtgggtcttttacttttacttccagaccagcatcgatttcaatgccatcaatggtaacatgaagagtgtagagtccaatagcccctggagtccaatttgcacaataagtcccatcattattgacacggatcagcatattctcactgggtctcttaggagttggtgatgcaaaacgtagttcttcaaatgaataattttcataaaccttcatcattgttatggcaatatatcgagcttccttcactatcattggttcatatgaaacatctagctttggtgatgccagccctccataagtcatgtcagtattagaagatgcagctgttactgcaggactgccaggaatcctttgaggtttctttgcttgatcttgttgtaaagacatttttttctgagaaacagggacagctttcacttccaccttcatattgggaacatgtaccacatccccatactggtcttttgtttgaacagttatggtggtaggccaaccacaacgaatatcatccttattcaggatcaaagatgttttctgaggatccgcatatgaatctggctgaagccaccttgcaagccttccaccacttgatcctgggacacaggcaataaaatcatccagaaaagactgttcattgctttggatttggagtggtaaatttccctcaagtgcttctaatatagttggtgaatgagaaagagctagaccctttccaagaattccagaatgggttttgcacacctgcaatgcagcctcctcaagaatttcaaggtcttcttctaattcattaccaataggaagtgctaggtccttcttcatcagagctgctgcacaaaccccaccaagattggctaattctttttccaattggatgactccctcatcaggtccagggctaaattcatatccaattgcaaaacacttaaaaccatagaaagaagctttgtcatctttcacataatctgatgcagtctccaatgaaaaaagggcctcatttcctggcaacaccaaaaccatagtaggccacccagaggatcctgaaaatttctttaattctatccatgaattaagattttcatgaacagatgtcaattttggtccatatcctgaattctgaacagttctgacaggaatcaacaaacgaaggacatcttctgactgtgcagtaccacactgagggtcaaattcgattgtcatccacctcacacattctgggaatgtcaccttgtaatgcatcacacaggcaggtttatacgggtgctcactctctatgacagcatagtgactggaggttgtacaagcagagaggccctgttcaggctggtttcctgtggtgctatctgtcgactgattagggttgaaggcaggcggtgcatacttctgattcaaaatggcaactgacggaagcaattgttggacaaggccaaagacttctacagccaccttgggaatagcagcagctactggtcctatgtaggctataataagggggagcagcatggaaaacagactggaagaactcagcagttctggaatgtcatcagcatccacagcaagagctctgtgcaggaggtccttagaggctcgaacgacagtgcttacaacagacaatgctctgctacagtttttatcttcttcattggctttactcagaagttgggattgtaaatctccatcaaattcactcctatagtagagtatctgtgggatctgtcctctggtttggtttgtgccgttactgctcaagctgcacgtgctgaatgtgaatgtcacaccatcagggcactgaactgtggtcattcctccatctccattggctgtacggcttccatagttcctcaagcgcacagcatatttaacattttcctttaaaggaaccactttgtcaagtctgatctcagctatatcactgggtgagtcatccgttgtgtacgttcctttcactaattccagagatgtccatctgtgggaatgagttgaatctcctgcatgttcactatcatcaaccaacacctctaattcatattcatgaattccacctcctccatagacagagaaaccaaccacaactattccaggtttgtctactgaaaaacagattgcatcaggggacccgttcccagtgttccaacttctgccctgacttgtttttgtaaatcggttagcactagcttttacagagtgaagagaattaagtccatcaacctcagatcccagggctgacgctgtcagttcactgacaatgctggccagtaatccacaggtgttagagacgaggtgggaggagaagagttcattttctctcctcaggctgttcctgactggtagcacaacaatgaccagcattttctccagaacttcacggaagcttgtcatccctgagatattctcttcactctggctgagtttttccatatgtgccaccaaaaggggaaaacgatgaactagtgttgagtcgttctctgtactaacttgtttaacaattgatcgtagtaatacttctccatcatacgcaatcgggaagatggaagtcagcttaacagacgtgtgacacagagctgacataacagctgcaaggagtcggctacttgatgtcttgaagtttgcttcttggatatcctgatccaaacaattcagcagatcacaaaggcaagcccactgtaaggcaggagttgggtagaaagaatgaaagcaggcagtgaaagtattatgacattcctgaaggacagcttctagaagactcaagggttgactgagatatccttgaggatcattatccaatttcaccatgcagtgatcaactccttctgataaaatttttcttaacaaagttctggtttttccaatacactctgctaatttgctagtttcttctacaactgcttttcctgtagctgacactgggtaaatttcacaggtatagacacgcaataacctcagacaacaggtacccacaaagcgcagtctctctaaatctaggagtgtagctgtgaactggaatccttttaatcctctaagttcttcaactcctaagactaaggtggtccagctccagtgaagaatactcaacaatgactcaaaacattccactgagacagttcttgcaaaagacctctttaaaatgtgtacaggttcactggtttgctgtttgccttttgaagcactgccatcactggttggaagtctgtataataactgaggtatctgacccgcattaacatctgtaccattatttgatttctttgaactcttgaactggaaaacaaccccatcatctgtggtaatagatgcctgtccatgagatccacagtcactgctgggtcctgacactcgggcccatgccacataccaccacccagcttgcaggagaacaggctcatcaaacatcattgcatatttttctctagcagcacagtcataagccaatacatcagtctctgcaagaaggtcaccatcagtttcatgatctcctccatcaggacccaattcaaacagcttaattttagcagtatattctcctctacctccaaacagaccaagaccaccaagtaaaatatcagtgtcggcactgaaacgtatagcttctactgaatgggcagaataaccccagcctcctccatgactttcaaacctgtttaccacactataatcttctttagaataaaccttcattactgcttgagtctcttcctctgtacttgcaacacccatttttaagtcctgcatagctgccaaggtatcaagacaacctaaaatgtgcaaagctgcatgagatcgggtagtgagggcccttgatcctgttggtaaggcaagttcaggacttaggatactacatctggactgcatgtctgctgcagagggaagcctggcatcagcaaccaccgcattgtaacaccacagctctctagtatttggtcgaaacctccaaattacatcatatacaggatcaagacacacaccaaatccttgcagatcctcttgttctgagtcattaaaagttttacaactcccatccactttatttatcagaaggcatttaaatggaggaggttctgatatagaagcaggtaccaagcctattatgtgtttactggcaaaaatttctgatgtagcaagtacatgagaattaataagtgcttcatcaattcgtaaaaaagtttggtccccacttgcacctatccaagtagcttttcttccatattttgatccaatgttaggcatgggagctggctttgcattccaatatggcacatccaaaattggtctgcccagttgtcctttagaaaaacttccaaatgtgaagacctgtccatccattaaaagtactgccgtatggttgctgcctgcagtgacttgtgtgctagggcctggcaatgcttgaacaagagtgggacatcccctggagttgacatctccatgtcctagctgcccatgctgcccataaccaaatgtatagacatctccattttccattaaaaccactgaatggtgaaatccacagctgacttggactgcccggagctcacagtcaaatcgcacagagcctggagggtatgttgtgattttgcttgcatccttttcgcctctttctccacttccatctttgtgcttgtcccgtttatgctttagctgtgctggatgggatctgagtctggctagagcctgttctcgatggttcataaaaataggaccagcaaatacaagggggcctcttccttcctctaatctgtgccttctgattacacgttgccgtttttcttcttgtcgtaactgaaggtgttcttcaatgttaaccccgggcactgggacagctaaaagaagatctaaaggtatcatttctttcactgcatcaagaattcctctttgtcttgcctcttgaccatctaactctcttgcacaggccttgcaacatccacacacagcacaaccagattctccggaaccacaaccacagatccctccggggactctgtctggccgtccactactgacacagctggctccataacctgtacagtctccacagacagtgcaaaccatgcactgctccagcttccatttgtgcatgcctggagggcacatcatagacttctcatctttttcatctagttcttcttccaggtcttcatccattgctgttgccatattttcaactccaaaccctttcccaccttggttcatggcaccagtatctcgtccacactgtcctttattatttacaccaaatgtccacacctctccattcttcattaaaacacaagtgtgagctttgcccatagctacctgagttacaaaatggcccttcaaatcagttaccaaacttgaactatcagagtaaatggcatcttttccaaacatgtagagttctccatctttagaaataacagaactacttccattattgcaggctgtatataccacaatctttccttccatcttaattatctttttaggtttataaggtttggattgccgtctgctcttagttgattctccatcttctcctttactagcagatcctgtaaagaatatgctcccatcttctgcaactaaaagggcgtgagagccatcgtgtccaactgagaagtgtactatctttggagattttgtaattggtagctcaacccattttcctgctgaaggaccaccttgtttgattccaagactctggtatttgccagtgtaatatatctttccatttgctgttttcattagcgcaaactctcgtcctgcaccaagaattgctgactcctcatcaaatcctgtacttataatatgcaagtccttttccagatcgaatagtgagataccacaggcatgtaagcattttctagccagtttaagttgcaattcttgctgtagaacaggttcagtgcttgtggcaaatattctgacaacaaagccatcatctcttgaagcagctatctgattaatatattctccatcagtgaataaaatattttgaccttcagtgtggcaatctggtaacatcacagtaccatcttgctccagtgtttcagggcttatccttatggctgtcatgctgtggttattcacatctctatataataaataaccctgagcataccctaaccaagactttttttcttttctgtttctaatacgggatgtagaattgtatatatggcccctaactgttccactgtatccagagcctattttatataatccatccttgcataatagataaagaaaaaatccatcattctgaagtagacattggtcatcttcatcaacagatatttcttttaatggccacttgtgcattaaagctgctttcttaatgccattactaaaccagtcctgaatttgaatttttcccaccaaaactgcttgtacacttctctgtagcgaatttagaattgttggcacctgaatagtttggcaagcatggcttccattgttggtgaggatagcagagatggcctgaagtgtccttcctgtttctccccaagaagccaccagactaaagaggcaagcacaggaaagtgctgttaaggactgtcctgtgctgtcattcatcccagtacttcgaacggtgatttccaaaagaagctggaagagagactctaggacctcaggtggctcagactggaggccttctggctgctggccctgcagcacgttgagcagggcttggagactcctgagacacagggatggatgagaaaatcgtgtctctttgatcaattcaaaaacttcacaaaggccaacctcaataatctttggaagcttgatagggggctctttggattcctcttcttcatcactatctgattctccactctgcacagagttcttagatgcggctgccaatgatatttcctttttctgccattccagaacgcaatggcgtacattacagtaaatattgaaagcagaaggattgctatgtagtttgatatctggtatgattactgtattctctaagttttcagacttgcttcttgtcttcacttttgatttgctcttctgttttcttttcaatttcttcttatttaaaattttcttattcctggaggctgggtgtccagcgctgccgcccccctggtccctgtcattgagcgcagcggtataaatcctccggtagcggtcggccagggcccggcctgacagcagcagctggtagtgaccccgggagtccgcggcgggtagccccagccccagccccgcagcagccacggagccgtcgggaaccggcatgaacagcgcccccggcgccggggaggaagagaaggtggcggctgggtagaatccgtccccgccgagccccgaggaggcggcggcgggggaggcagtcgctgcgcacatcatcatcctcgccgccgccgccgccgccgccgcctcgtccccgcgggccgggcgggcagacacgcgcgcgcacacacagcccttttccaacgacgacggctccggcggcggcctctggctcccgcagcagggagactacaaagacagcgacctccttctcctcctccttcttctcctcctcccccccgcgccgccctcgccgctactggggccgctcatctaaccccgccaccccgggaatgtgaggaggaggcggtgccgccactgccgccgccaccaccgctaccaccgccaccaccgccggggctacccgcaatgggaagctgccg

SEQ ID NO: 17108 - RNA, 8818 nt, Homo sapiens
  source 1..8818: mol_type = other RNA
tcaaaactgaggggcattttcttcttgcggagggtatctggatcaagtgtgtaagagtctgatttagaacgttcccgaggaggatcaagctttgtcttaacaggagcagtacttttttgaggtagatttttatcatgtggtgaggaggagcgtggagaactagcacccgatgggctagacctattggctgggagagtctttggcttaggagatgacaaccgagaacctggtcctggggattcagctctggagctagaaggcatcctcccatcagatttcaatgtctgcaaggtgttatggttgggggataatgacctactgtgggaatctgacctcaactttgcagcatcagattttaagatgagggattcactagcagataaactttctgtgccccttggcttcttctgatcagcagtagtccggctcatacgtccatcaggtttaagcgatctgctgtgtttagaggacagctctgattttcctgatgtagaggctggtttagaagatgttgagatgtttcctcgatcactctgaagctgaggctgctggaaggaaaggggctgtccgaacacaaatgggctgtgtactagggaagagggaggttttgcagcttgatcaaagatggaaggagctgggagattgggtcgtgactgaatggaattcaatatggcactcagttggtcacctttgctatttccgagtccataatcaaatccttgggcactgcaacttgcccctttattaaaagcttgcactgagaaagggcttggaggaggagtttgagaattctgatccagaagagcttgttcatcttcatgtcggaggtactggtttccgcctctgtctctagctaaggaccatgcctctccttcatcactctcacagaactctaccatgctgttctgatccagttgcacccatgtcccttcagaattggttacgtcaacagggaccagaagactcttgccaagatgttgattaaaagagaggcaccaggcttcagtgtaaccattcatgttagggacatacttctttattgtctcatcattcagcctcagccacacaccatcatcattatggatctcatcaataaaagtgatagttccattgactttcactatgcctatctgctcactctgaagggaagggtggctacggatgcgaagccccgcactgtccttggccacaaattttcgaaccttattaggctgaggttcagactttggtttgaccaactgagttcctggtggtatcatcccttttggtgggtcttttacttttacttccagaccagcatcgatttcaatgccatcaatggtaacatgaagagtgtagagtccaatagcccctggagtccaatttgcacaataagtcccatcattattgacacggatcagcatattctcactgggtctcttaggagttggtgatgcaaaacgtagttcttcaaatgaataattttcataaaccttcatcattgttatggcaatatatcgagcttccttcactatcattggttcatatgaaacatctagctttggtgatgccagccctccataagtcatgtcagtattagaagatgcagctgttactgcaggactgccaggaatcctttgaggtttctttgcttgatcttgttgtaaagacatttttttctgagaaacagggacagctttcacttccaccttcatattgggaacatgtaccacatccccatactggtcttttgtttgaacagttatggtggtaggccaaccacaacgaatatcatccttattcaggatcaaagatgttttctgaggatccgcatatgaatctggctgaagccaccttgcaagccttccaccacttgatcctgggacacaggcaataaaatcatccagaaaagactgttcattgctttggatttggagtggtaaatttccctcaagtgcttctaatatagttggtgaatgagaaagagctagaccctttccaagaattccagaatgggttttgcacacctgcaatgcagcctcctcaagaatttcaaggtcttcttctaattcattaccaataggaagtgctaggtccttcttcatcagagctgctgcacaaaccccaccaagattggctaattctttttccaattggatgactccctcatcaggtccagggctaaattcatatccaattgcaaaacacttaaaaccatagaaagaagctttgtcatctttcacataatctgatgcagtctccaatgaaaaaagggcctcatttcctggcaacaccaaaaccatagtaggccacccagaggatcctgaaaatttctttaattctatccatgaattaagattttcatgaacagatgtcaattttggtccatatcctgaattctgaacagttctgacaggaatcaacaaacgaaggacatcttctgactgtgcagtaccacactgagggtcaaattcgattgtcatccacctcacacattctgggaatgtcaccttgtaatgcatcacacaggcaggtttatacgggtgctcactctctatgacagcatagtgactggaggttgtacaagcagagaggccctgttcaggctggtttcctgtggtgctatctgtcgactgattagggttgaaggcaggcggtgcatacttctgattcaaaatggcaactgacggaagcaattgttggacaaggccaaagacttctacagccaccttgggaatagcagcagctactggtcctatgtaggctataataagggggagcagcatggaaaacagactggaagaactcagcagttctggaatgtcatcagcatccacagcaagagctctgtgcaggaggtccttagaggctcgaacgacagtgcttacaacagacaatgctctgctacagtttttatcttcttcattggctttactcagaagttgggattgtaaatctccatcaaattcactcctatagtagagtatctgtgggatctgtcctctggtttggtttgtgccgttactgctcaagctgcacgtgctgaatgtgaatgtcacaccatcagggcactgaactgtggtcattcctccatctccattggctgtacggcttccatagttcctcaagcgcacagcatatttaacattttcctttaaaggaaccactttgtcaagtctgatctcagctatatcactgggtgagtcatccgttgtgtacgttcctttcactaattccagagatgtccatctgtgggaatgagttgaatctcctgcatgttcactatcatcaaccaacacctctaattcatattcatgaattccacctcctccatagacagagaaaccaaccacaactattccaggtttgtctactgaaaaacagattgcatcaggggacccgttcccagtgttccaacttctgccctgacttgtttttgtaaatcggttagcactagcttttacagagtgaagagaattaagtccatcaacctcagatcccagggctgacgctgtcagttcactgacaatgctggccagtaatccacaggtgttagagacgaggtgggaggagaagagttcattttctctcctcaggctgttcctgactggtagcacaacaatgaccagcattttctccagaacttcacggaagcttgtcatccctgagatattctcttcactctggctgagtttttccatatgtgccaccaaaaggggaaaacgatgaactagtgttgagtcgttctctgtactaacttgtttaacaattgatcgtagtaatacttctccatcatacgcaatcgggaagatggaagtcagcttaacagacgtgtgacacagagctgacataacagctgcaaggagtcggctacttgatgtcttgaagtttgcttcttggatatcctgatccaaacaattcagcagatcacaaaggcaagcccactgtaaggcaggagttgggtagaaagaatgaaagcaggcagtgaaagtattatgacattcctgaaggacagcttctagaagactcaagggttgactgagatatccttgaggatcattatccaatttcaccatgcagtgatcaactccttctgataaaatttttcttaacaaagttctggtttttccaatacactctgctaatttgctagtttcttctacaactgcttttcctgtagctgacactgggtaaatttcacaggtatagacacgcaataacctcagacaacaggtacccacaaagcgcagtctctctaaatctaggagtgtagctgtgaactggaatccttttaatcctctaagttcttcaactcctaagactaaggtggtccagctccagtgaagaatactcaacaatgactcaaaacattccactgagacagttcttgcaaaagacctctttaaaatgtgtacaggttcactggtttgctgtttgccttttgaagcactgccatcactggttggaagtctgtataataactgaggtatctgacccgcattaacatctgtaccattatttgatttctttgaactcttgaactggaaaacaaccccatcatctgtggtaatagatgcctgtccatgagatccacagtcactgctgggtcctgacactcgggcccatgccacataccaccacccagcttgcaggagaacaggctcatcaaacatcattgcatatttttctctagcagcacagtcataagccaatacatcagtctctgcaagaaggtcaccatcagtttcatgatctcctccatcaggacccaattcaaacagcttaattttagcagtatattctcctctacctccaaacagaccaagaccaccaagtaaaatatcagtgtcggcactgaaacgtatagcttctactgaatgggcagaataaccccagcctcctccatgactttcaaacctgtttaccacactataatcttctttagaataaaccttcattactgcttgagtctcttcctctgtacttgcaacacccatttttaagtcctgcatagctgccaaggtatcaagacaacctaaaatgtgcaaagctgcatgagatcgggtagtgagggcccttgatcctgttggtaaggcaagttcaggacttaggatactacatctggactgcatgtctgctgcagagggaagcctggcatcagcaaccaccgcattgtaacaccacagctctctagtatttggtcgaaacctccaaattacatcatatacaggatcaagacacacaccaaatccttgcagatcctcttgttctgagtcattaaaagttttacaactcccatccactttatttatcagaaggcatttaaatggaggaggttctgatatagaagcaggtaccaagcctattatgtgtttactggcaaaaatttctgatgtagcaagtacatgagaattaataagtgcttcatcaattcgtaaaaaagtttggtccccacttgcacctatccaagtagcttttcttccatattttgatccaatgttaggcatgggagctggctttgcattccaatatggcacatccaaaattggtctgcccagttgtcctttagaaaaacttccaaatgtgaagacctgtccatccattaaaagtactgccgtatggttgctgcctgcagtgacttgtgtgctagggcctggcaatgcttgaacaagagtgggacatcccctggagttgacatctccatgtcctagctgcccatgctgcccataaccaaatgtatagacatctccattttccattaaaaccactgaatggtgaaatccacagctgacttggactgcccggagctcacagtcaaatcgcacagagcctggagggtatgttgtgattttgcttgcatccttttcgcctctttctccacttccatctcttccttcctctaatctgtgccttctgattacacgttgccgtttttcttcttgtcgtaactgaaggtgttcttcaatgttaaccccgggcactgggacagctaaaagaagatctaaaggtatcatttctttcactgcatcaagaattcctctttgtcttgcctcttgaccatctaactctcttgcacaggccttgcaacatccacacacagcacaaccagattctccggaaccacaaccacagatccctccggggactctgtctggccgtccactactgacacagctggctccataacctgtacagtctccacagacagtgcaaaccatgcactgctccagcttccatttgtgcatgcctggagggcacatcatagacttctcatctttttcatctagttcttcttccaggtcttcatccattgctgttgccatattttcaactccaaaccctttcccaccttggttcatggcaccagtatctcgtccacactgtcctttattatttacaccaaatgtccacacctctccattcttcattaaaacacaagtgtgagctttgcccatagctacctgagttacaaaatggcccttcaaatcagttaccaaacttgaactatcagagtaaatggcatcttttccaaacatgtagagttctccatctttagaaataacagaactacttccattattgcaggctgtatataccacaatctttccttccatcttaattatctttttaggtttataaggtttggattgccgtctgctcttagttgattctccatcttctcctttactagcagatcctgtaaagaatatgctcccatcttctgcaactaaaagggcgtgagagccatcgtgtccaactgagaagtgtactatctttggagattttgtaattggtagctcaacccattttcctgctgaaggaccaccttgtttgattccaagactctggtatttgccagtgtaatatatctttccatttgctgttttcattagcgcaaactctcgtcctgcaccaagaattgctgactcctcatcaaatcctgtacttataatatgcaagtccttttccagatcgaatagtgagataccacaggcatgtaagcattttctagccagtttaagttgcaattcttgctgtagaacaggttcagtgcttgtggcaaatattctgacaacaaagccatcatctcttgaagcagctatctgattaatatattctccatcagtgaataaaatattttgaccttcagtgtggcaatctggtaacatcacagtaccatcttgctccagtgtttcagggcttatccttatggctgtcatgctgtggttattcacatctctatataataaataaccctgagcataccctaaccaagactttttttcttttctgtttctaatacgggatgtagaattgtatatatggcccctaactgttccactgtatccagagcctattttatataatccatccttgcataatagataaagaaaaaatccatcattctgaagtagacattggtcatcttcatcaacagatatttcttttaatggccacttgtgcattaaagctgctttcttaatgccattactaaaccagtcctgaatttgaatttttcccaccaaaactgcttgtacacttctctgtagcgaatttagaattgttggcacctgaatagtttggcaagcatggcttccattgttggtgaggatagcagagatggcctgaagtgtccttcctgtttctccccaagaagccaccagactaaagaggcaagcacaggaaagtgctgttaaggactgtcctgtgctgtcattcatcccagtacttcgaacggtgatttccaaaagaagctggaagagagactctaggacctcaggtggctcagactggaggccttctggctgctggccctgcagcacgttgagcagggcttggagactcctgagacacagggatggatgagaaaatcgtgtctctttgatcaattcaaaaacttcacaaaggccaacctcaataatctttggaagcttgatagggggctctttggattcctcttcttcatcactatctgattctccactctgcacagagttcttagatgcggctgccaatgatatttcctttttctgccattccagaacgcaatggcgtacattacagtaaatattgaaagcagaaggattgctatgtagtttgatatctggtatgattactgtattctctaagttttcagacttgcttcttgtcttcacttttgatttgctcttctgttttcttttcaatttcttcttatttaaaattttcttattcctggaggctgggtgtccagcgctgccgcccccctggtccctgtcattgagcgcagcggtataaatcctccggtagcggtcggccagggcccggcctgacagcagcagctggtagtgaccccgggagtccgcggcgggtagccccagccccagccccgcagcagccacggagccgtcgggaaccggcatgaacagcgcccccggcgccggggaggaagagaaggtggcggctgggtagaatccgtccccgccgagccccgaggaggcggcggcgggggaggcagtcgctgcgcacatcatcatcctcgccgccgccgccgccgccgccgcctcgtccccgcgggccgggcgggcagacacgcgcgcgcacacacagcccttttccaacgacgacggctccggcggcggcctctggctcccgcagcagggagactacaaagacagcgacctccttctcctcctccttcttctcctcctcccccccgcgccgccctcgccgctactggggccgctcatctaaccccgccaccccgggaatgtgaggaggaggcggtgccgccactgccgccgccaccaccgctaccaccgccaccaccgccggggctacccgcaatgggaagctgccg

SEQ ID NO: 17109 - RNA, 8926 nt, Homo sapiens
  source 1..8926: mol_type = other RNA
tcaaaactgaggggcattttcttcttgcggagggtatctggatcaagtgtgtaagagtctgatttagaacgttcccgaggaggatcaagctttgtcttaacaggagcagtacttttttgaggtagatttttatcatgtggtgaggaggagcgtggagaactagcacccgatgggctagacctattggctgggagagtctttggcttaggagatgacaaccgagaacctggtcctggggattcagctctggagctagaaggcatcctcccatcagatttcaatgtctgcaaggtgttatggttgggggataatgacctactgtgggaatctgacctcaactttgcagcatcagattttaagatgagggattcactagcagataaactttctgtgccccttggcttcttctgatcagcagtagtccggctcatacgtccatcaggtttaagcgatctgctgtgtttagaggacagctctgattttcctgatgtagaggctggtttagaagatgttgagatgtttcctcgatcactctgaagctgaggctgctggaaggaaaggggctgtccgaacacaaatgggctgtgtactagggaagagggaggttttgcagcttgatcaaagatggaaggagctgggagattgggtcgtgactgaatggaattcaatatggcactcagttggtcacctttgctatttccgagtccataatcaaatccttgggcactgcaacttgcccctttattaaaagcttgcactgagaaagggcttggaggaggagtttgagaattctgatccagaagagcttgttcatcttcatgtcggaggtactggtttccgcctctgtctctagctaaggaccatgcctctccttcatcactctcacagaactctaccatgctgttctgatccagttgcacccatgtcccttcagaattggttacgtcaacagggaccagaagactcttgccaagatgttgattaaaagagaggcaccaggcttcagtgtaaccattcatgttagggacatacttctttattgtctcatcattcagcctcagccacacaccatcatcattatggatctcatcaataaaagtgatagttccattgactttcactatgcctatctgctcactctgaagggaagggtggctacggatgcgaagccccgcactgtccttggccacaaattttcgaaccttattaggctgaggttcagactttggtttgaccaactgagttcctggtggtatcatcccttttggtgggtcttttacttttacttccagaccagcatcgatttcaatgccatcaatggtaacatgaagagtgtagagtccaatagcccctggagtccaatttgcacaataagtcccatcattattgacacggatcagcatattctcactgggtctcttaggagttggtgatgcaaaacgtagttcttcaaatgaataattttcataaaccttcatcattgttatggcaatatatcgagcttccttcactatcattggttcatatgaaacatctagctttggtgatgccagccctccataagtcatgtcagtattagaagatgcagctgttactgcaggactgccaggaatcctttgaggtttctttgcttgatcttgttgtaaagacatttttttctgagaaacagggacagctttcacttccaccttcatattgggaacatgtaccacatccccatactggtcttttgtttgaacagttatggtggtaggccaaccacaacgaatatcatccttattcaggatcaaagatgttttctgaggatccgcatatgaatctggctgaagccaccttgcaagccttccaccacttgatcctgggacacaggcaataaaatcatccagaaaagactgttcattgctttggatttggagtggtaaatttccctcaagtgcttctaatatagttggtgaatgagaaagagctagaccctttccaagaattccagaatgggttttgcacacctgcaatgcagcctcctcaagaatttcaaggtcttcttctaattcattaccaataggaagtgctaggtccttcttcatcagagctgctgcacaaaccccaccaagattggctaattctttttccaattggatgactccctcatcaggtccagggctaaattcatatccaattgcaaaacacttaaaaccatagaaagaagctttgtcatctttcacataatctgatgcagtctccaatgaaaaaagggcctcatttcctggcaacaccaaaaccatagtaggccacccagaggatcctgaaaatttctttaattctatccatgaattaagattttcatgaacagatgtcaattttggtccatatcctgaattctgaacagttctgacaggaatcaacaaacgaaggacatcttctgactgtgcagtaccacactgagggtcaaattcgattgtcatccacctcacacattctgggaatgtcaccttgtaatgcatcacacaggcaggtttatacgggtgctcactctctatgacagcatagtgactggaggttgtacaagcagagaggccctgttcaggctggtttcctgtggtgctatctgtcgactgattagggttgaaggcaggcggtgcatacttctgattcaaaatggcaactgacggaagcaattgttggacaaggccaaagacttctacagccaccttgggaatagcagcagctactggtcctatgtaggctataataagggggagcagcatggaaaacagactggaagaactcagcagttctggaatgtcatcagcatccacagcaagagctctgtgcaggaggtccttagaggctcgaacgacagtgcttacaacagacaatgctctgctacagtttttatcttcttcattggctttactcagaagttgggattgtaaatctccatcaaattcactcctatagtagagtatctgtgggatctgtcctctggtttggtttgtgccgttactgctcaagctgcacgtgctgaatgtgaatgtcacaccatcagggcactgaactgtggtcattcctccatctccattggctgtacggcttccatagttcctcaagcgcacagcatatttaacattttcctttaaaggaaccactttgtcaagtctgatctcagctatatcactgggtgagtcatccgttgtgtacgttcctttcactaattccagagatgtccatctgtgggaatgagttgaatctcctgcatgttcactatcatcaaccaacacctctaattcatattcatgaattccacctcctccatagacagagaaaccaaccacaactattccaggtttgtctactgaaaaacagattgcatcaggggacccgttcccagtgttccaacttctgccctgacttgtttttgtaaatcggttagcactagcttttacagagtgaagagaattaagtccatcaacctcagatcccagggctgacgctgtcagttcactgacaatgctggccagtaatccacaggtgttagagacgaggtgggaggagaagagttcattttctctcctcaggctgttcctgactggtagcacaacaatgaccagcattttctccagaacttcacggaagcttgtcatccctgagatattctcttcactctggctgagtttttccatatgtgccaccaaaaggggaaaacgatgaactagtgttgagtcgttctctgtactaacttgtttaacaattgatcgtagtaatacttctccatcatacgcaatcgggaagatggaagtcagcttaacagacgtgtgacacagagctgacataacagctgcaaggagtcggctacttgatgtcttgaagtttgcttcttggatatcctgatccaaacaattcagcagatcacaaaggcaagcccactgtaaggcaggagttgggtagaaagaatgaaagcaggcagtgaaagtattatgacattcctgaaggacagcttctagaagactcaagggttgactgagatatccttgaggatcattatccaatttcaccatgcagtgatcaactccttctgataaaatttttcttaacaaagttctggtttttccaatacactctgctaatttgctagtttcttctacaactgcttttcctgtagctgacactgggtaaatttcacaggtatagacacgcaataacctcagacaacaggtacccacaaagcgcagtctctctaaatctaggagtgtagctgtgaactggaatccttttaatcctctaagttcttcaactcctaagactaaggtggtccagctccagtgaagaatactcaacaatgactcaaaacattccactgagacagttcttgcaaaagacctctttaaaatgtgtacaggttcactggtttgctgtttgccttttgaagcactgccatcactggttggaagtctgtataataactgaggtatctgacccgcattaacatctgtaccattatttgatttctttgaactcttgaactggaaaacaaccccatcatctgtggtaatagatgcctgtccatgagatccacagtcactgctgggtcctgacactcgggcccatgccacataccaccacccagcttgcaggagaacaggctcatcaaacatcattgcatatttttctctagcagcacagtcataagccaatacatcagtctctgcaagaaggtcaccatcagtttcatgatctcctccatcaggacccaattcaaacagcttaattttagcagtatattctcctctacctccaaacagaccaagaccaccaagtaaaatatcagtgtcggcactgaaacgtatagcttctactgaatgggcagaataaccccagcctcctccatgactttcaaacctgtttaccacactataatcttctttagaataaaccttcattactgcttgagtctcttcctctgtacttgcaacacccatttttaagtcctgcatagctgccaaggtatcaagacaacctaaaatgtgcaaagctgcatgagatcgggtagtgagggcccttgatcctgttggtaaggcaagttcaggacttaggatactacatctggactgcatgtctgctgcagagggaagcctggcatcagcaaccaccgcattgtaacaccacagctctctagtatttggtcgaaacctccaaattacatcatatacaggatcaagacacacaccaaatccttgcagatcctcttgttctgagtcattaaaagttttacaactcccatccactttatttatcagaaggcatttaaatggaggaggttctgatatagaagcaggtaccaagcctattatgtgtttactggcaaaaatttctgatgtagcaagtacatgagaattaataagtgcttcatcaattcgtaaaaaagtttggtccccacttgcacctatccaagtagcttttcttccatattttgatccaatgttaggcatgggagctggctttgcattccaatatggcacatccaaaattggtctgcccagttgtcctttagaaaaacttccaaatgtgaagacctgtccatccattaaaagtactgccgtatggttgctgcctgcagtgacttgtgtgctagggcctggcaatgcttgaacaagagtgggacatcccctggagttgacatctccatgtcctagctgcccatgctgcccataaccaaatgtatagacatctccattttccattaaaaccactgaatggtgaaatccacagctgacttggactgcccggagctcacagtcaaatcgcacagagcctggagggtatgttgtgattttgcttgcatccttttcgcctctttctccacttccatctttgtgcttgtcccgtttatgctttagctgtgctggatgggatctgagtctggctagagcctgttctcgatggttcataaaaataggaccagcaaatacaagggggcctcttccttcctctaatctgtgccttctgattacacgttgccgtttttcttcttgtcgtaactgaaggtgttcttcaatgttaaccccgggcactgggacagctaaaagaagatctaaaggtatcatttctttcactgcatcaagaattcctctttgtcttgcctcttgaccatctaactctcttgcacaggccttgcaacatccacacacagcacaaccagattctccggaaccacaaccacagatccctccggggactctgtctggccgtccactactgacacagctggctccataacctgtacagtctccacagacagtgcaaaccatgcactgctccagcttccatttgtgcatgcctggagggcacatcatagacttctcatctttttcatctagttcttcttccaggtcttcatccattgctgttgccatattttcaactccaaaccctttcccaccttggttcatggcaccagtatctcgtccacactgtcctttattatttacaccaaatgtccacacctctccattcttcattaaaacacaagtgtgagctttgcccatagctacctgagttacaaaatggcccttcaaatcagttaccaaacttgaactatcagagtaaatggcatcttttccaaacatgtagagttctccatctttagaaataacagaactacttccattattgcaggctgtatataccacaatctttccttccatcttaattatctttttaggtttataaggtttggattgccgtctgctcttagttgattctccatcttctcctttactagcagatcctgtaaagaatatgctcccatcttctgcaactaaaagggcgtgagagccatcgtgtccaactgagaagtgtactatctttggagattttgtaattggtagctcaacccattttcctgctgaaggaccaccttgtttgattccaagactctggtatttgccagtgtaatatatctttccatttgctgttttcattagcgcaaactctcgtcctgcaccaagaattgctgactcctcatcaaatcctgtacttataatatgcaagtccttttccagatcgaatagtgagataccacaggcatgtaagcattttctagccagtttaagttgcaattcttgctgtagaacaggttcagtgcttgtggcaaatattctgacaacaaagccatcatctcttgaagcagctatctgattaatatattctccatcagtgaataaaatattttgaccttcagtgtggcaatctggtaacatcacagtaccatcttgctccagtgtttcagggcttatccttatggctgtcatgctgtggttattcacatctctatataataaataaccctgagcataccctaaccaagactttttttcttttctgtttctaatacgggatgtagaattgtatatatggcccctaactgttccactgtatccagagcctattttatataatccatccttgcataatagataaagaaaaaatccatcattctgaagtagacattggtcatcttcatcaacagatatttcttttaatggccacttgtgcattaaagctgctttcttaatgccattactaaaccagtcctgaatttgaatttttcccaccaaaactgcttgtacacttctctgtagcgaatttagaattgttggcacctgaatagtttggcaagcatggcttccattgttggtgaggatagcagagatggcctgaagtgtccttcctgtttctccccaagaagccaccagactaaagaggcaagcacaggaaagtgctgttaaggactgtcctgtgctgtcattcatcccagtacttcgaacggtgatttccaaaagaagctggaagagagactctaggacctcaggtggctcagactggaggccttctggctgctggccctgcagcacgttgagcagggcttggagactcctgagacacagggatggatgagaaaatcgtgtctctttgatcaattcaaaaacttcacaaaggccaacctcaataatctttggaagcttgatagggggctctttggattcctcttcttcatcactatctgattctccactctgcacagagttcttagatgcggctgccaatgatatttcctttttctgccattccagaacgcaatggcgtacattacagtaaatattgaaagcagaaggattgctatgtagtttgatatctggtatgattactgtattctctaagttttcagacttgcttcttgtcttcacttttgatttgctcttctgttttcttttcaatttcttcttatttaaaattttcttattcctggaggctgggtgtccagcgctgccgcccccctggtccctgtcattgagcgcagcggtataaatcctccggtagcggtcggccagggcccggcctgacagcagcagctggtagtgaccccgggagtccgcggcgggtagccccagccccagccccgcagcagccacggagccgtcgggaaccggcatgaacagcgcccccggcgccggggaggaagagaaggtggcggctgggtagaatccgtccccgccgagccccgaggaggcggcggcgggggaggcagtcgctgcgcacatcatcatcctcgccgccgccgccgccgccgccgcctcgtccccgcgggccgggcgggcagacacgcgcgcgcacacacagcccttttccaacgacgacggctccggcggcggcctctggctcccgcagcagggagactacaaagacagcgacctccttctcctcctccttcttctcctcctcccccccgcgccgccctcgccgctactggggccgctcatctaaccccgccaccccgggaatgtgaggaggaggcggtgccgccactgccgccgccaccaccgctaccaccgccaccaccgccggggctacccgcaatgggaagctgccg

SEQ ID NO: 17110 - RNA, 1865 nt, Homo sapiens
  source 1..1865: mol_type = other RNA
tcaaaatgtagaggaagaccccagcagtgaccccaaacacccagggagtgagggggacagggcccaggctgagccccacccccaggactgcaccccccaatcccagggctccagacacgaggctcagcagcagcagccgccgaaaggacagccctgactggagcagcatggcaaagtcacccagttcgtggggcagctcatggcagaagaccgctaaggtggtactgaggccgctggagaagccatcagagaaggcagcacctatggccagcccatcagtgaggttgtgtagaccatctcccaggaggaccatccacgtgatatcagtgccaccctggtgcccatgactgtggccttggtgcccaggaggggccagagctggtgggtgctggctgttcttctccctctggccctgagcccctggctctggagctgcctgtaggggctgaagggccatcccactgccattctccggatccaagttgcgtgtttcgagattccttcgttttcgcctgcagcatctctgaaataggagggcatccctctggcctgagccctcggtgccgcaaaagccccagcatgttctccagcacaaagagcaggaagaggcctccgagcactgacagccccgggcccaggtccttctctggtagtccgccaggtcctgcgtgccgcccttcttgtgcatgcggtagcagatgtagcagtgcatccccacaaagagtgcccaccgccagggcccccaggaagcccagcaagggccgtagtagacgaggtcccaggagccgcagcagcagcagggataggggagaagggaggctgagcaacaggactgccagggcactctgaagcagggcagatagtagatcccctgggggtgcaggggccggagcgccgatgcagacgcggctgtcgatctgataaagcagggctgggcacagcagagcaaactgacgaggggtcagaggagcagcggggctcaagccaaaattgaccagcagctgggagccgttcagacaatcctcattcaggtggtcagccaatgagtggtccagcaacagaagcctgtgaaggaggtccaggcccgagggggctggcccacggggtaggtgaggggcctttgactcttccaggtcaccccaccctgagggacccagaggcatccctgcccagacatccacactcagctcagggttctgtggcctgtgtgtggaattgtctgcagctggggatgcagcccgtccagtcagaggcccatgctgtcccaggcgaagcccctgaactcggcctagccccaggctgtggagaagccgcgccaagccccctgcagtcagcgtcccattctcgccgtacaggccaaacagctgggccaggtaatggttctgctcctgctcagcagggcccaggttggggactgagccccctacccagcccaagacgacccacacacagaagccggccagcagatgactcactggggaccccatcattggtgaggggaatagcttaggggctcaggttctggctcctattctccccgaaacatcctgaggactgtgccccctactggcaacataagagctgtcacctcaggtcccctattaggccttgctgtagacgttaagcagttcctgagtcagggaagggggaatccaggcttagcctccaggtgtccaggtggatcggaggccacgtcacatagaaggctgagatggacatgcaccccctcctagcccacctgccccaagaagagaaagagccagagctctagggatcgatgaccaagaaaggggaagccctgatagcaggagacaaggacacccagaggaagggggacacaaccttcttggttccagctggggggg

SEQ ID NO: 17111 - RNA, 1678 nt, Homo sapiens
  source 1..1678: mol_type = other RNA
tcaaaatgtagaggaagaccccagcagtgaccccaaacacccagggagtgagggggacagggcccaggctgagccccacccccaggactgcaccccccaatcccagggctccagacacgaggctcagcagcagcagccgccgaaaggacagccctgactggagcagcatggcaaagtcacccagttcgtggggcagctcatggcagaagaccgctaaggtggtactgaggccgctggagaagccatcagagaaggcagcacctatggccagcccatcagtgaggttgtgtagaccatctcccaggaggaccatccacgtgatatcagtgccaccctggtgcccatgactgtggccttggtgcccaggaggggccagagctggtgggtgctggctgttcttctccctctggccctgagcccctggctctggagctgcctgtaggggctgaagggccatcccactgccattctccggatccaagttgcgtgtttcgagattccttcgttttcgcctgcagcatctctgaaataggagggcatccctctggcctgagccctcggtgccgcaaaagccccagcatgttctccagcacaaagagcaggaagaggcctccgagcactgacagccccgggcccaggtccttctctggtagtccgccaggtcctgcgtgccgcccttcttgtgcatgcggtagcagatgtagcagtgcatccccacaaagagtgcccaccgccagggcccccaggaagcccagcaagggccgtagtagacgaggtcccaggagccgcagcagcagcagggataggggagaagggaggctgagcaacaggactgccagggcactctgaagcagggcagatagtagatcccctgggggtgcaggggccggagcgccgatgcagacgcggctgtcgatctgataaagcagggctgggcacagcagagcaaactgacgaggggtcagaggagcagcggggctcaagccaaaattgaccagcagctgggagccgttcagacaatcctcattcaggtggtcagccaatgagtggtccagcaacagaagcctgtgaaggaggtccaggcccgagggggctggcccacggggtaggtgaggggcctttgactcttccaggtcaccccaccctgagggacccagaggcatccctgcccagacatccacactcagctcagggttctgtggcctgtgtgtggaattgtctgcagctggggatgcagcccgtccagtcagaggcccatgctgtcccaggcgaagcccctgaactcggcctagccccaggctgtggagaagccgcgccaagccccctgcagtcagcgtcccattctcgccgtacaggccaaacagctgggccaggtaatggttctgctcctgctcagcagggcccaggttggggactgagccccctacccagcccaagacgacccacacacagaagccggccagcagatgactcactggggaccccatcattggtgaggggaatagcttaggggctcaggttctggctcctattctccccgaaacatcctgaggactgtgccctcaggtcccctattaggccttgctgtagacgttaagcagttcctgagtcagggaagggggaatccaggcttagcctccaggtgtccaggtggatcggaggccacgtcacatagaag

SEQ ID NO: 17112 - RNA, 1612 nt, Homo sapiens
  source 1..1612: mol_type = other RNA
tcaaaatgtagaggaagaccccagcagtgaccccaaacacccagggagtgagggggacagggcccaggctgagccccacccccaggactgcaccccccaatcccagggctccagacacgaggctcagcagcagcagccgccgaaaggacagccctgactggagcagcatggcaaagtcacccagttcgtggggcagctcatggcagaagaccgctaaggtggtactgaggccgctggagaagccatcagagaaggcagcacctatggccagcccatcagtgaggttgtgtagaccatctcccaggaggaccatccacgtgatatcagtgccaccctggtgcccatgactgtggccttggtgcccaggaggggccagagctggtgggtgctggctgttcttctccctctggccctgagcccctggctctggagctgcctgtaggggctgaagggccatcccactgccattctccggatccaagttgcgtgtttcgagattccttcgttttcgcctgcagcatctctgaaataggagggcatccctctggcctgagccctcggtgccgcaaaagccccagcatgttctccagcacaaagagcaggaagaggcctccgagcactgacagccccgggcccaggtccttctctggtagtccgccaggtcctgcgtgccgcccttcttgtgcatgcggtagcagatgtagcagtgcatccccacaaagagtgcccaccgccagggcccccaggaagcccagcaagggccgtagtagacgaggtcccaggagccgcagcagcagcagggataggggagaagggaggctgagcaacaggactgccagggcactctgaagcagggcagatagtagatcccctgggggtgcaggggccggagcgccgatgcagacgcggctgtcgatctgataaagcagggctgggcacagcagagcaaactgacgaggggtcagaggagcagcggggctcaagccaaaattgaccagcagctgggagccgttcagacaatcctcattcaggtggtcagccaatgagtggtccagcaacagaagcctgtgaaggaggtccaggcccgagggggctggcccacggggtaggtgaggggcctttgactcttccaggtcaccccaccctgagggacccagaggcatccctgcccagacatccacactcagctcagggttctgtggcctgtgtgtggaattgtctgcagctggggatgcagcccgtccagtcagaggcccatgctgtcccaggcgaagcccctgaactcggcctagccccaggctgtggagaagccgcgccaagccccctgcagtcagcgtcccattctcgccgtacaggccaaacagctgggccaggtaatggttctgctcctgctcagcagggcccaggttggggactgagccccctacccagcccaagacgacccacacacagaagccggccagcagatgactcactggggaccccatcattggtgaggggaatagcttaggggctcaggttctggctcctattctccccgaaacatcctgaggactgtgccctgatagcaggagacaaggacacccagaggaagggggacacaaccttcttg

SEQ ID NO: 17113 - RNA, 1682 nt, Homo sapiens
  source 1..1682: mol_type = other RNA
tcaaaatgtagaggaagaccccagcagtgaccccaaacacccagggagtgagggggacagggcccaggctgagccccacccccaggactgcaccccccaatcccagggctccagacacgaggctcagcagcagcagccgccgaaaggacagccctgactggagcagcatggcaaagtcacccagttcgtggggcagctcatggcagaagaccgctaaggtggtactgaggccgctggagaagccatcagagaaggcagcacctatggccagcccatcagtgaggttgtgtagaccatctcccaggaggaccatccacgtgatatcagtgccaccctggtgcccatgactgtggccttggtgcccaggaggggccagagctggtgggtgctggctgttcttctccctctggccctgagcccctggctctggagctgcctgtaggggctgaagggccatcccactgccattctccggatccaagttgcgtgtttcgagattccttcgttttcgcctgcagcatcttggcctgagccctcggtgccgcaaaagccccagcatgttctccagcacaaagagcaggaagaggcctccgagcactgacagccccgggcccaggtccttctctggtagtccgccaggtcctgcgtgccgcccttcttgtgcatgcggtagcagatgtagcagtgcatccccacaaagagtgcccaccgccagggcccccaggaagcccagcaagggccgtagtagacgaggtcccaggagccgcagcagcagcagggataggggagaagggaggctgagcaacaggactgccagggcactctgaagcagggcagatagtagatcccctgggggtgcaggggccggagcgccgatgcagacgcggctgtcgatctgataaagcagggctgggcacagcagagcaaactgacgaggggtcagaggagcagcggggctcaagccaaaattgaccagcagctgggagccgttcagacaatcctcattcaggtggtcagccaatgagtggtccagcaacagaagcctgtgaaggaggtccaggcccgagggggctggcccacggggtaggtgaggggcctttgactcttccaggtcaccccaccctgagggacccagaggcatccctgcccagacatccacactcagctcagggttctgtggcctgtgtgtggaattgtctgcagctggggatgcagcccgtccagtcagaggcccatgctgtcccaggcgaagcccctgaactcggcctagccccaggctgtggagaagccgcgccaagccccctgcagtcagcgtcccattctcgccgtacaggccaaacagctgggccaggtaatggttctgctcctgctcagcagggcccaggttggggactgagccccctacccagcccaagacgacccacacacagaagccggccagcagatgactcactggggaccccatcattggtgaggggaatagcttaggggctcaggttctggctcctattctccccgaaacatcctgaggactgtgcccccaagaagagaaagagccagagctctagggatcgatgaccaagaaaggggaagccctgatagcaggagacaaggacacccagaggaagggggacacaaccttcttggttccagctgggggggcaggcaggcaggcgggcaag

SEQ ID NO: 17114 - RNA, 1732 nt, Homo sapiens
  source 1..1732: mol_type = other RNA
tcaaaatgtagaggaagaccccagcagtgaccccaaacacccagggagtgagggggacagggcccaggctgagccccacccccaggactgcaccccccaatcccagggctccagacacgaggctcagcagcagcagccgccgaaaggacagccctgactggagcagcatggcaaagtcacccagttcgtggggcagctcatggcagaagaccgctaaggtggtactgaggccgctggagaagccatcagagaaggcagcacctatggccagcccatcagtgaggttgtgtagaccatctcccaggaggaccatccacgtgatatcagtgccaccctggtgcccatgactgtggccttggtgcccaggaggggccagagctggtgggtgctggctgttcttctccctctggccctgagcccctggctctggagctgcctgtaggggctgaagggccatcccactgccattctccggatccaagttgcgtgtttcgagattccttcgttttcgcctgcagcatcttggcctgagccctcggtgccgcaaaagccccagcatgttctccagcacaaagagcaggaagaggcctccgagcactgacagccccgggcccaggtccttctctggtagtccgccaggtcctgcgtgccgcccttcttgtgcatgcggtagcagatgtagcagtgcatccccacaaagagtgcccaccgccagggcccccaggaagcccagcaagggccgtagtagacgaggtcccaggagccgcagcagcagcagggataggggagaagggaggctgagcaacaggactgccagggcactctgaagcagggcagatagtagatcccctgggggtgcaggggccggagcgccgatgcagacgcggctgtcgatctgataaagcagggctgggcacagcagagcaaactgacgaggggtcagaggagcagcggggctcaagccaaaattgaccagcagctgggagccgttcagacaatcctcattcaggtggtcagccaatgagtggtccagcaacagaagcctgtgaaggaggtccaggcccgagggggctggcccacggggtaggtgaggggcctttgactcttccaggtcaccccaccctgagggacccagaggcatccctgcccagacatccacactcagctcagggttctgtggcctgtgtgtggaattgtctgcagctggggatgcagcccgtccagtcagaggcccatgctgtcccaggcgaagcccctgaactcggcctagccccaggctgtggagaagccgcgccaagccccctgcagtcagcgtcccattctcgccgtacaggccaaacagctgggccaggtaatggttctgctcctgctcagcagggcccaggttggggactgagccccctacccagcccaagacgacccacacacagaagccggccagcagatgactcactggggaccccatcattggtgaggggaatagcttaggggctcaggttctggctcctattctccccgaaacatcctgaggactgtgccccctactggcaacataagagctgtcacctcaggtcccctattaggccttgctgtagacgttaagcagttccccaagaagagaaagagccagagctctagggatcgatgaccaagaaaggggaagccctgatagcaggagacaaggacacccagaggaagggggacacaaccttcttggttccagctggggggg

SEQ ID NO: 17115 - RNA, 1678 nt, Homo sapiens
  source 1..1678: mol_type = other RNA
tcaaaatgtagaggaagaccccagcagtgaccccaaacacccagggagtgagggggacagggcccaggctgagccccacccccaggactgcaccccccaatcccagggctccagacacgaggctcagcagcagcagccgccgaaaggacagccctgactggagcagcatggcaaagtcacccagttcgtggggcagctcatggcagaagaccgctaaggtggtactgaggccgctggagaagccatcagagaaggcagcacctatggccagcccatcagtgaggttgtgtagaccatctcccaggaggaccatccacgtgatatcagtgccaccctggtgcccatgactgtggccttggtgcccaggaggggccagagctggtgggtgctggctgttcttctccctctggccctgagcccctggctctggagctgcctgtaggggctgaagggccatcccactgccattctccggatccaagttgcgtgtttcgagattccttcgttttcgcctgcagcatcttggcctgagccctcggtgccgcaaaagccccagcatgttctccagcacaaagagcaggaagaggcctccgagcactgacagccccgggcccaggtccttctctggtagtccgccaggtcctgcgtgccgcccttcttgtgcatgcggtagcagatgtagcagtgcatccccacaaagagtgcccaccgccagggcccccaggaagcccagcaagggccgtagtagacgaggtcccaggagccgcagcagcagcagggataggggagaagggaggctgagcaacaggactgccagggcactctgaagcagggcagatagtagatcccctgggggtgcaggggccggagcgccgatgcagacgcggctgtcgatctgataaagcagggctgggcacagcagagcaaactgacgaggggtcagaggagcagcggggctcaagccaaaattgaccagcagctgggagccgttcagacaatcctcattcaggtggtcagccaatgagtggtccagcaacagaagcctgtgaaggaggtccaggcccgagggggctggcccacggggtaggtgaggggcctttgactcttccaggtcaccccaccctgagggacccagaggcatccctgcccagacatccacactcagctcagggttctgtggcctgtgtgtggaattgtctgcagctggggatgcagcccgtccagtcagaggcccatgctgtcccaggcgaagcccctgaactcggcctagccccaggctgtggagaagccgcgccaagccccctgcagtcagcgtcccattctcgccgtacaggccaaacagctgggccaggtaatggttctgctcctgctcagcagggcccaggttggggactgagccccctacccagcccaagacgacccacacacagaagccggccagcagatgactcactggggaccccatcattggtgaggggaatagcttaggggctcaggttctggctcctattctccccgaaacatcctgaggactgtgccccctactggcaacataagagctgtcacctcaggtcccctattaggccttgctgtagacgttaagcagttcctgagtcagggaagggggaatccaggcttagcctccaggtgtccaggtggatcggaggccacgtcacat

SEQ ID NO: 17116 - RNA, 1710 nt, Homo sapiens
  source 1..1710: mol_type = other RNA
tcaaaatgtagaggaagaccccagcagtgaccccaaacacccagggagtgagggggacagggcccaggctgagccccacccccaggactgcaccccccaatcccagggctccagacacgaggctcagcagcagcagccgccgaaaggacagccctgactggagcagcatggcaaagtcacccagttcgtggggcagctcatggcagaagaccgctaaggtggtactgaggccgctggagaagccatcagagaaggcagcacctatggccagcccatcagtgaggttgtgtagaccatctcccaggaggaccatccacgtgatatcagtgccaccctggtgcccatgactgtggccttggtgcccaggaggggccagagctggtgggtgctggctgttcttctccctctggccctgagcccctggctctggagctgcctgtaggggctgaagggccatcccactgccattctccggatccaagttgcgtgtttcgagattccttcgttttcgcctgcagcatcttggcctgagccctcggtgccgcaaaagccccagcatgttctccagcacaaagagcaggaagaggcctccgagcactgacagccccgggcccaggtccttctctggtagtccgccaggtcctgcgtgccgcccttcttgtgcatgcggtagcagatgtagcagtgcatccccacaaagagtgcccaccgccagggcccccaggaagcccagcaagggccgtagtagacgaggtcccaggagccgcagcagcagcagggataggggagaagggaggctgagcaacaggactgccagggcactctgaagcagggcagatagtagatcccctgggggtgcaggggccggagcgccgatgcagacgcggctgtcgatctgataaagcagggctgggcacagcagagcaaactgacgaggggtcagaggagcagcggggctcaagccaaaattgaccagcagctgggagccgttcagacaatcctcattcaggtggtcagccaatgagtggtccagcaacagaagcctgtgaaggaggtccaggcccgagggggctggcccacggggtaggtgaggggcctttgactcttccaggtcaccccaccctgagggacccagaggcatccctgcccagacatccacactcagctcagggttctgtggcctgtgtgtggaattgtctgcagctggggatgcagcccgtccagtcagaggcccatgctgtcccaggcgaagcccctgaactcggcctagccccaggctgtggagaagccgcgccaagccccctgcagtcagcgtcccattctcgccgtacaggccaaacagctgggccaggtaatggttctgctcctgctcagcagggcccaggttggggactgagccccctacccagcccaagacgacccacacacagaagccggccagcagatgactcactggggaccccatcattggtgaggggaatagcttaggggctcaggttctggctcctattctccccgaaacatcctgaggactgtgccctcaggtcccctattaggccttgctgtagacgttaagcagttccccaagaagagaaagagccagagctctagggatcgatgaccaagaaaggggaagccctgatagcaggagacaaggacacccagaggaagggggacacaaccttcttggttccagctgggggggcaggc

SEQ ID NO: 17117 - RNA, 1656 nt, Homo sapiens
  source 1..1656: mol_type = other RNA
tcaaaatgtagaggaagaccccagcagtgaccccaaacacccagggagtgagggggacagggcccaggctgagccccacccccaggactgcaccccccaatcccagggctccagacacgaggctcagcagcagcagccgccgaaaggacagccctgactggagcagcatggcaaagtcacccagttcgtggggcagctcatggcagaagaccgctaaggtggtactgaggccgctggagaagccatcagagaaggcagcacctatggccagcccatcagtgaggttgtgtagaccatctcccaggaggaccatccacgtgatatcagtgccaccctggtgcccatgactgtggccttggtgcccaggaggggccagagctggtgggtgctggctgttcttctccctctggccctgagcccctggctctggagctgcctgtaggggctgaagggccatcccactgccattctccggatccaagttgcgtgtttcgagattccttcgttttcgcctgcagcatcttggcctgagccctcggtgccgcaaaagccccagcatgttctccagcacaaagagcaggaagaggcctccgagcactgacagccccgggcccaggtccttctctggtagtccgccaggtcctgcgtgccgcccttcttgtgcatgcggtagcagatgtagcagtgcatccccacaaagagtgcccaccgccagggcccccaggaagcccagcaagggccgtagtagacgaggtcccaggagccgcagcagcagcagggataggggagaagggaggctgagcaacaggactgccagggcactctgaagcagggcagatagtagatcccctgggggtgcaggggccggagcgccgatgcagacgcggctgtcgatctgataaagcagggctgggcacagcagagcaaactgacgaggggtcagaggagcagcggggctcaagccaaaattgaccagcagctgggagccgttcagacaatcctcattcaggtggtcagccaatgagtggtccagcaacagaagcctgtgaaggaggtccaggcccgagggggctggcccacggggtaggtgaggggcctttgactcttccaggtcaccccaccctgagggacccagaggcatccctgcccagacatccacactcagctcagggttctgtggcctgtgtgtggaattgtctgcagctggggatgcagcccgtccagtcagaggcccatgctgtcccaggcgaagcccctgaactcggcctagccccaggctgtggagaagccgcgccaagccccctgcagtcagcgtcccattctcgccgtacaggccaaacagctgggccaggtaatggttctgctcctgctcagcagggcccaggttggggactgagccccctacccagcccaagacgacccacacacagaagccggccagcagatgactcactggggaccccatcattggtgaggggaatagcttaggggctcaggttctggctcctattctccccgaaacatcctgaggactgtgccctcaggtcccctattaggccttgctgtagacgttaagcagttcctgatagcaggagacaaggacacccagaggaagggggacacaaccttcttggttccagctgggggggcaggcag

SEQ ID NO: 17118 - RNA, 1606 nt, Homo sapiens
  source 1..1606: mol_type = other RNA
tcaaaatgtagaggaagaccccagcagtgaccccaaacacccagggagtgagggggacagggcccaggctgagccccacccccaggactgcaccccccaatcccagggctccagacacgaggctcagcagcagcagccgccgaaaggacagccctgactggagcagcatggcaaagtcacccagttcgtggggcagctcatggcagaagaccgctaaggtggtactgaggccgctggagaagccatcagagaaggcagcacctatggccagcccatcagtgaggttgtgtagaccatctcccaggaggaccatccacgtgatatcagtgccaccctggtgcccatgactgtggccttggtgcccaggaggggccagagctggtgggtgctggctgttcttctccctctggccctgagcccctggctctggagctgcctgtaggggctgaagggccatcccactgccattctccggatccaagttgcgtgtttcgagattccttcgttttcgcctgcagcatcttggcctgagccctcggtgccgcaaaagccccagcatgttctccagcacaaagagcaggaagaggcctccgagcactgacagccccgggcccaggtccttctctggtagtccgccaggtcctgcgtgccgcccttcttgtgcatgcggtagcagatgtagcagtgcatccccacaaagagtgcccaccgccagggcccccaggaagcccagcaagggccgtagtagacgaggtcccaggagccgcagcagcagcagggataggggagaagggaggctgagcaacaggactgccagggcactctgaagcagggcagatagtagatcccctgggggtgcaggggccggagcgccgatgcagacgcggctgtcgatctgataaagcagggctgggcacagcagagcaaactgacgaggggtcagaggagcagcggggctcaagccaaaattgaccagcagctgggagccgttcagacaatcctcattcaggtggtcagccaatgagtggtccagcaacagaagcctgtgaaggaggtccaggcccgagggggctggcccacggggtaggtgaggggcctttgactcttccaggtcaccccaccctgagggacccagaggcatccctgcccagacatccacactcagctcagggttctgtggcctgtgtgtggaattgtctgcagctggggatgcagcccgtccagtcagaggcccatgctgtcccaggcgaagcccctgaactcggcctagccccaggctgtggagaagccgcgccaagccccctgcagtcagcgtcccattctcgccgtacaggccaaacagctgggccaggtaatggttctgctcctgctcagcagggcccaggttggggactgagccccctacccagcccaagacgacccacacacagaagccggccagcagatgactcactggggaccccatcattggtgaggggaatagcttaggggctcaggttctggctcctattctccccgaaacatcctgaggactgtgccctgatagcaggagacaaggacacccagaggaagggggacacaaccttcttggttccagctggggggg

SEQ ID NO: 17119 - RNA, 1696 nt, Homo sapiens
  source 1..1696: mol_type = other RNA
tcaaaatgtagaggaagaccccagcagtgaccccaaacacccagggagtgagggggacagggcccaggctgagccccacccccaggactgcaccccccaatcccagggctccagacacgaggctcagcagcagcagccgccgaaaggacagccctgactggagcagcatggcaaagtcacccagttcgtggggcagctcatggcagaagaccgctaaggtggtactgaggccgctggagaagccatcagagaaggcagcacctatggccagcccatcagtgaggttgtgtagaccatctcccaggaggaccatccacgtgatatcagtgccaccctggtgcccatgactgtggccttggtgcccaggaggggccagagctggtgggtgctggctgttcttctccctctggccctgagcccctggctctggagctgcctgtaggggctgaagggccatcccactgccattctccggatccaagttgcgtgtttcgagattccttcgttttcgcctgcagcatcttggcctgagccctcggtgccgcaaaagccccagcatgttctccagcacaaagagcaggaagaggcctccgagcactgacagccccgggcccaggtccttctctggtagtccgccaggtcctgcgtgccgcccttcttgtgcatgcggtagcagatgtagcagtgcatccccacaaagagtgcccaccgccagggcccccaggaagcccagcaagggccgtagtagacgaggtcccaggagccgcagcagcagcagggataggggagaagggaggctgagcaacaggactgccagggcactctgaagcagggcagatagtagatcccctgggggtgcaggggccggagcgccgatgcagacgcggctgtcgatctgataaagcagggctgggcacagcagagcaaactgacgaggggtcagaggagcagcggggctcaagccaaaattgaccagcagctgggagccgttcagacaatcctcattcaggtggtcagccaatgagtggtccagcaacagaagcctgtgaaggaggtccaggcccgagggggctggcccacggggtaggtgaggggcctttgactcttccaggtcaccccaccctgagggacccagaggcatccctgcccagacatccacactcagctcagggttctgtggcctgtgtgtggaattgtctgcagctggggatgcagcccgtccagtcagaggcccatgctgtcccaggcgaagcccctgaactcggcctagccccaggctgtggagaagccgcgccaagccccctgcagtcagcgtcccattctcgccgtacaggccaaacagctgggccaggtaatggttctgctcctgctcagcagggcccaggttggggactgagccccctacccagcccaagacgacccacacacagaagccggccagcagatgactcactggggaccccatcattggtgaggggaatggcttaggggctcaggttctggctcctattctccccgaaacatcctgaggactgtgccctcaggtcccctattaggccttgctgtagacgttaagcagttcctgagtcagggaagggggaatccaggcttagcctccaggtgtccaggtggatcggaggccacgtcacatagaaggctgagatggacatgcaccccctcctagcccacctgcctt

SEQ ID NO: 17120 - RNA, 32 nt, Homo sapiens
  source 1..32: mol_type = other RNA
tcaaaatgtagaggaagaccccaggagaagca

SEQ ID NO: 17121 - RNA, 67 nt, Homo sapiens
  source 1..67: mol_type = other RNA
tcaaatgcagatcctgacttcactggtgcagtaagaagtcagagaatctgcatctgtaacaagctcc

SEQ ID NO: 17122 - RNA, 64 nt, Homo sapiens
  source 1..64: mol_type = other RNA
tcaacaaaatcactgatgctggagtcgcctgagtcatcactcagcaccaggatattgttggaga

SEQ ID NO: 17123 - RNA, 70 nt, Homo sapiens
  source 1..70: mol_type = other RNA
tcaagtagtttcatgataaagggttgatctctcatacaccctttatcatgaaactacttgagaatatgct

SEQ ID NO: 17124 - RNA, 1207 nt, Homo sapiens
  source 1..1207: mol_type = other RNA
tcacaagtcaggctcttgggacatcgtggaggtactgggcaccgctgaggtcttcaagctgcccacagtaacctcttccttttcctcctgccgcaggtgccggagaacctcctgggacagcgagaagctgctgtcatctgcaggttccgctgcccgttctccagaagctcatagatgctgttgctgtaaacccgatccttgatgccagcatggtcaccggtctgctggggcagtttatccaggaagcgaatgttggggtcagccatactcaggttatcaggcaccccacagtccaatgggaggagaatatacagccgctggctcactgcaccccgtagcaggttgttgtaatgctgattgtaagttcgaatccgggcctggagctctggcaggatcagccgcagatatccgatgtaatatgaccatgccagcccatgggccacgttgaaattccctttttcacacactgcagagatctcagctggggccaggcccttgaggcccaggaggatgttcagtgcctgcgagaggcccaggagggcaagcatccaagtgaagggcgggccgaccgcatttgggagggagtagtagaaatagatggacagcagcaacagggccccacggcggagggggcagcccaggcaggcccgcacagtcctccagtagctgccccggtacctggagtggatgtggcgcagctcctcagccaggctgcagaccccgtttaacagcagtcccagctgcagggaggctaggtggagcaccaggtaccggagagtgtgctctggtggctctcctagcccccaaagggtcaccaggcaggcactcagcagaaccaaggctgccttctgggccccgtgacccctgggacacgggatggatggatgcaggctggagtggggcatcttctgcctcccggacactggctgctctggatgatgacgaggagagaaggcccggcgctacgagcagccaagggcagcttctctgagtgcagccgcagtcacagctctgaacagcgggttcccctcaagccaccacgatcaaacacactgtacctaacacctgagcaggactccacacactcagccaaaggcagcacacacatcacacgatgattccccgtctcatatttttcttctggtttccaggatgcagattctttttctgaaaagtgtgacctaggagggaggagtgaaaaatgaac

SEQ ID NO: 17125 - RNA, 1394 nt, Homo sapiens
  source 1..1394: mol_type = other RNA
tcacaagtcaggctcttgggacatcgtggaggtactgggcaccgctgaggtcttcaagctgcccacagtaacctcttccttttcctcctgccgcaggtgccggagaacctcctgggacagcgagaagctgctgtcatctgcaggttcctggtaggcaatgaggcggcagttgttctgagactcaggggcatctgccaggatgtcctcaagtgtccggcagaagagtttggcctgctcaagcctatcctcccggctaaagccagcttgactgtattgtgacatggcaaacaaagtctgcaagggggtggcgtactccaggacacaggtgcccgcccgctgcccgttctccagaagctcatagatgctgttgctgtaaacccgatccttgatgccagcatggtcaccggtctgctggggcagtttatccaggaagcgaatgttggggtcagccatactcaggttatcaggcaccccacagtccaatgggaggagaatatacagccgctggctcactgcaccccgtagcaggttgttgtaatgctgattgtaagttcgaatccgggcctggagctctggcaggatcagccgcagatatccgatgtaatatgaccatgccagcccatgggccacgttgaaattccctttttcacacactgcagagatctcagctggggccaggcccttgaggcccaggaggatgttcagtgcctgcgagaggcccaggagggcaagcatccaagtgaagggcgggccgaccgcatttgggagggagtagtagaaatagatggacagcagcaacagggccccacggcggagggggcagcccaggcaggcccgcacagtcctccagtagctgccccggtacctggagtggatgtggcgcagctcctcagccaggctgcagaccccgtttaacagcagtcccagctgcagggaggctaggtggagcaccaggtaccggagagtgtgctctggtggctctcctagcccccaaagggtcaccaggcaggcactcagcagaaccaaggctgccttctgggccccgtgacccctgggacacgggatggatggatgcaggctggagtggggcatcttctgcctcccggacactggctgctctggatgatgacgaggagagaaggcccggcgctacgagcagccaagggcagcttctctgagtgcagccgcagtcacagctctgaacagcgggttcccctcaagccaccacgatcaaacacactgtacctaacacctgagcaggactccacacactcagccaaaggcagcacacacatcacacgatgattccccgtctcatatttttcttctggtttccaggatgcagattctttttctgaaaagtgtgacctaggagggaggagtgaaaaatgaac

SEQ ID NO: 17126 - RNA, 1167 nt, Homo sapiens
  source 1..1167: mol_type = other RNA
tcacaagtcaggctcttgggacatcgtggaggtactgggcaccgctgaggtcttcaagctgcccacagtaacctcttccttttcctcctgccgcaggtgccggagaacctcctgggacagcgagaagctgctgtcatctgcaggttcctggtaggcaatgaggcggcagttgttctgagactcaggggcatctgccaggatgtcctcaagtgtccggcagaagagtttggcctgctcaagcctatcctcccggctaaagccagcttgactgtattgtgacatggcaaacaaagtctgcaagggggtggcgtactccaggacacaggtgcccgcccgctgcccgttctccagaagctcatagatgctgttgctgtaaacccgatccttgatgccagcatggtcaccggtctgctggggcagtttatccaggaagcgaatgttggggtcagccatactcaggttatcaggcaccccacagtccaatgggaggagaatatacagccgctggctcactgcaccccgtagcaggttgttgtaatgctgattgtaagttcgaatccgggcctggagctctggcaggatcagccgcagatatccgatgtaatatgaccatgccagcccatgggccacgttgaaattccctttttcacacactgcagagatctcagctggggccaggcccttgaggcccaggaggatgttcagtgcctgcgagaggcccaggagggcaagcatccaagtgaagggcgggccgaccgcatttgggagggagtagtagaaatagatggacagcagcaacagggccccacggcggagggggcagcccaggcaggcccgcacagtcctccagtagctgccccggtaccttctgcctcccggacactggctgctctggatgatgacgaggagagaaggcccggcgctacgagcagccaagggcagcttctctgagtgcagccgcagtcacagctctgaacagcgggttcccctcaagccaccacgatcaaacacactgtacctaacacctgagcaggactccacacactcagccaaaggcagcacacacatcacacgatgattccccgtctcatatttttcttctggtttccaggatgcagattctttttctgaaaagtgtgacctaggagggaggagtgaaaaatgaac

SEQ ID NO: 17127 - RNA, 42 nt, Homo sapiens
  source 1..42: mol_type = other RNA
tcacctgacctcccatgcctgtgcaccctctattatatcact

SEQ ID NO: 17128 - RNA, 1579 nt, Homo sapiens
  source 1..1579: mol_type = other RNA
tcacctgacctcccatgcctgtggccaaacatgtgcacccctgcacacacaagggcttcctcacatacacctaatacaagcctgcacactcaaactcactcatagacacacacatcttctgcctatacatcctcactcatgcgcatatacacacactgctgggtacctgtctacacatgcacataccgagttcctcattcttacatactacacacacacacatatgttcactcttacatgctcacatataggtctgcagataaattagctgtgtgtacacatgtgcacacagcacacttaagctcatttatacatgcttattcacacatgcctacacacaccagcctacatgttagcacatacacactcatgcctacctgcaatcatgccagcaaattatgtacttactagtgcgcctcacacatgcctgcaaatatatacatatacccttgcacacttgtggaggcacacccttaggcctggtcctggggcctggatggtgctgccctctgctggagacagcgaataagctccttccggttgtctaggatggtgtcgaagctctcctgcagtcgggcctgctggtcaatcaactgatgctgcaggccccggatccactggagcagtgccaggcgacggtacatcaccaagtgcacgtggtgcttttccttctcctgctctttgtagcgctcctggacttgtaagtgctgcacagcctgggccactgagggcagaaggggatcgggagggccagggcctcgcggggtcccacaggcaggctcaggactgctgctacggctgtcaatgctcagggaactgctggcatagccgttgtcctccagaggggagcagactgtgccagcaccacccatcttctcaggctcagccccgggaatctctgccccctctggggggctgcgcaccccttcctcaggggatccaggggcctggaaggcttggttgtcagagggtgactcagaggagctcctcctcaggataggttccactctgcctggcatcccatgccaattctcgttagcatccttggcacttgccatgaagttggagttgctgtctggttggagctcgggctgacataatccaggaggtgggtcccccaggaattggcccccctcagctagccctggctggatggcgaacatctagcctgttcattctcagtctcctgcaaagggtttttcctccgtcctcagagccaggctgtcttctgattttgtgcatttctctccagaggacctcattctctgctgtagcttcaaagaccatcatatgctggtgactctcagatctgtcttcagcccagatccaactgctatccaaccctgcaaccaaccatagtctcctcaaattctacataaccagtccaggcatggtggctcatacctgtaatcccagcactttgggaggccgaggcaggcagatcacctgaggtcaggagttcgagactagactggccaacatggtgaaaccccatctctactaaaaatacaaaaattagccaggcatggtgacaggcacctgtaatcccagctatttgggaggctgaggcaggggaatc

SEQ ID NO: 17129 - RNA, 1346 nt, Homo sapiens
  source 1..1346: mol_type = other RNA
tcacctgacctcccatgcctgtggccaaacatgtgcacccctgcacacacaagggcttcctcacatacacctaatacaagcctgcacactcaaactcactcatagacacacacatcttctgcctatacatcctcactcatgcgcatatacacacactgctgggtacctgtctacacatgcacataccgagttcctcattcttacatactacacacacacacatatgttcactcttacatgctcacatataggtctgcagataaattagctgtgtgtacacatgtgcacacagcacacttaagctcatttatacatgcttattcacacatgcctacacacaccagcctacatgttagcacatacacactcatgcctacctgcaatcatgccagcaaattatgtacttactagtgcgcctcacacatgcctgcaaatatatacatatacccttgcacacttgtggaggcacacccttaggcctggtcctggggcctggatggtgctgccctctgctggagacagcgaataagctccttccggttgtctaggatggtgtcgaagctctcctgcagtcgggcctgctggtcaatcaactgatgctgcaggccccggatccactggagcagtgccaggcgacggtacatcaccaagtgcacgtggtgcttttccttctcctgctctttgtagcgctcctggacttgtaagtgctgcacagcctgggccactgagggcagaaggggatcgggagggccagggcctcgcggggtcccacaggcaggctcaggactgctgctacggctgtcaatgctcagggaactgctggcatagccgttgtcctccagaggggagcagactgtgccagcaccacccatcttctcaggctcagccccgggaatctctgccccctctggggggctgcgcaccccttcctcaggggatccaggggcctggaaggcttggttgtcagagggtgactcagaggagctcctcctcaggataggttccactctgcctggcatcccatgccaattctcgttagcatccttggcacttgccatgaagttggagttgctgtctggttggagctcgggctgacataatccaggaggtgggtcccccaggaattggcccccctcagctagccctggctggatggcgaacatctagcggcgtagaggcgcccgctccggcgcgtctggctctggctccgcccggccctggtggtgtctagtccctgggctgggggttcctcggcctgggcgtctccgcggtccaggcgtgggtgcggggctcccgggcagcgcgcccagccccagtcccggactgcggagtcaggcggcgtctgc

SEQ ID NO: 17130 - RNA, 34 nt, Homo sapiens
  source 1..34: mol_type = other RNA
tcacctgagctcccgtgcctgtgcaccctctatt

SEQ ID NO: 17131 - RNA, 118 nt, Homo sapiens
  source 1..118: mol_type = other RNA
tcacgcggagagatggctttgtttttgctttcgtgcggttctgcgaggcgctccacgatcccgccccctggcatggcagcacctaccggcggcgcgaactcggctgctgtgggctgct

SEQ ID NO: 17132 - RNA, 75 nt, Homo sapiens
  source 1..75: mol_type = other RNA
tcacgtctgcggctgtcacgttggctgggcccgacctggggaaacacgcctgtccaaaggaagagacgtggactc

SEQ ID NO: 17133 - RNA, 1062 nt, Homo sapiens
  source 1..1062: mol_type = other RNA
tcactacctgacaatacagtataagtggctcaggtaggaaagatagcacggcatctcatattattgattttaattagcaggtagagtggactgaaaagaaacaaaaggaacttccttcataaacaaaaggttttgctacaatgattggttaagatttgctcccgttttgtaaggccaacatctagggcacataatctaagttgtctgtcttctttctctctctcttccccctccaactgttctttccctcttactttttcaaatatagctaattgggggatgaagtggtggacacaggcacagggggcctagaagaagaagatttcgctatgtatctgggtgttgtgggttggttgtattctgtctccctgcccctcacaaaattcatatattgacgcattaatctttaatagttcagaatgtgatggtatttggagataaggtctttaaagaggtaatcaagttaaaattaggttattagggtgttcctttttccaatatgactactgtccttataagaagaggaaatttggaaacaaatacagagggaagacgtgagaagacacagagagaatatggccaatggcaagccaaagggaaagtcctggaacagattcttcctcaaggccctcaggaaccaatcctgctgacatcttggtcttggatggttagcctccagagcacattaaaaacatttcatcttttgcagcactgactttaccactctttatgctgttgacttgcaggcatcagtgtctattggtggatatcaattttagtccatatggtcaaagataggtgatagattgttttaaaatcctttctggctctttgtgtccatctgtcatatggagtcaggactagaaaatcgcccaggatccttgcagtccacagtttaagcacattatgaaaactccagttgggctgaatcatttcctttcatttatttcaaagctatagttagattcatgtaggtgccatttgaaagtgcagtctattcaacccacacatacgaaatcagcagagtgcctctagcaaccacactgcagtagccatactgtc

SEQ ID NO: 17134 - RNA, 653 nt, Homo sapiens
  source 1..653: mol_type = other RNA
tcactctcaccttgctttgcaaagcgtttcttacgcctcattttggtccggtgtctagcaaacaagtcactgatcctctcagcccaggccgcataactgttggtatctgtaaccccgcagcggggacgagtcatctggcgcagggtggcgcggtccaacacgccgctgacaggtagctgggacacccactgaaacgctctgatggcatcgctgaatcgagtggaggtgggagctttggggacctgttcattgaggtatccgtacttctctaggaatgcctccgcctccttgcgcagctcctggcctccgcgctccgcgggctgggcgtccaggtggccccacagtagcagctgcagggcgcgcagcaggaggccgacgcgcgcgaccatctcgccgcctccggtgcagcccggctcggggagctactgcgcgcagggaaccagccggcagtcagccgcgcccgggaccccggggatgggactgctctgcgccgcccccgcacggagagggactgtcccggggtttcgccagtgccctagctgcgcgctctgggccgctcctccgctgcccttcgccgggagccggccagacgtcgtccagcccgggcagtgcctgcccgcgggtccgccggccccggggaccgagggagggag

SEQ ID NO: 17135 - RNA, 29 nt, Homo sapiens
  source 1..29: mol_type = other RNA
tcagatgatctaaaggcctatacataaat

SEQ ID NO: 17136 - RNA, 24 nt, Homo sapiens
  source 1..24: mol_type = other RNA
tcagcaccaggatattgttggaga

SEQ ID NO: 17137 - RNA, 2429 nt, Homo sapiens
  source 1..2429: mol_type = other RNA
tcagcaggcaggctggtgcagcttcttcactcacagaccggcaatgacatcccctgtcacctgtaaatcaccgaggtgccattaatcaacaatatgcatccagtgagggccaactctgggcccagcatgggcaggtgctatgaggtggaaaaaaaggaaacaaaagataaagtcagccttcagagaaggactaacacacaagaaacaaggaagaaaacaattgcactcccttaacggcacagtgcttactatatgtgtaatgagagttctaagaaaaatgaggtaagtgtgggcaagaaggctgcgaggaagagggtgggctcatgctcaggctgagccagcagcagaccagggtgctgaggttggagacaggaggtggacctcagcacctgtcacctcaggactgtgggcagagccaccccagccactaccgattcccctgcccctgccttccaggcagggggtgctgctttgaccagttaatcggttgcccacttactgagcaccacgtgtgcacaaacagcctcctgcacagggggccgactccccctgaaggcagatgaattctaactctctgtgacagaagctttcacatctcagttgatttcaggagccaaccagagccagagaggaagagaagcatgtgcatctatgtccagctccaagaactctggtcaatccacagcgatccagagcaatgctctagaaaggcctctattagaaatgcaagcaaggctcaggtagaagcagtggagaaggcagaaagaggaggaaagaggccaagtcaaggacattgcaaagggaaaaggaatttcaaaagatggctttgcagggggcagaaaagagagcaagtggcatctaaagagaccaaccatcctagaactcaggactttcatactaaaaccaggacagtcccaagcaaaccaggacgagttggtcaacccagccataccatcctcagggatgctatgaagttgcctgataactgggtactctttctcccatcctttgtggaactgtcattgctcgttagcacccctggggccaatggaaaggaagaagtggtcaacccagggaggtgactactgtgtccttcctgctgtcctcctggcttgtatcctctcatctcaaccatggaggtttccaaaggggctcaggtagaataaaatgctttattgctgttcttaaaataaaacctagaatcacagccactatcctttattccactgtttcacagacacgagcttatcagccatccagttgggagaggaccccatgtatccctcttggagaaataagcaccttatctgtaacaaacttggaaatcagaagaagctggaggggttggcacactcagctcttgaagccatctccattcattctccatctccctcttccttcttagagcttcagttcccacccacctctcccaaaggcaggctctaagagagtactccacccacataatctgttcattcaacgaggatttactgagcatttactatgtggcagaaagtttgttaggcaagattcagaacacaaagcacaataagacacaatctatgccttccaagaatttatggttcagttgatggggagagggagtggaggtgtgggcaaggatggtgtagaggtgagaatcattcaattattcaacacatatttactttcctcttaatatgtgccaagaactgtactgagagaatgtagataagtaatggaacaactgcaaaaccatgtataaatgctggtcatgtcggagacctcaggacagcaaccgccccagccaccgaggcaaataccaactgatcaccgcttctccttcgcatggcagtatgtgctgtggaggactaaaaacaaaagaaaagcggtaagaccaagccctgacctcaaagagtgaaccaaatgatcaaggagataaaacccccacaaataaagcaattcgcaaaccaccaggtatggtgaagagctaactgtgggacacagaacttcagcacaaggagcaacagagctggacaaagtctgcagagcttcccagagggagcggaggtaaaacctgagaagtaataccgaacggggagcattttccaggcaggaagaacataacaggtatctgtgatttttctcaaaaatcaaaggtgaatgtatagttattactgaaagtgtttctaaatggcacacctatccacgcatctttggcttgagtaaataggaaccttgccaatagtgaccttcacaaatgtgagttacactggaatagaaagatgggcatcaaatctaacttcagctgtccacactatgaaggtggggaattgaaacatacttaaccctgtaatgcaagtcagtgtgcacgtctgtataaacatacacacacacacatacacacacacacccatacttccctggctctttttttcttttttcttttt

SEQ ID NO: 17138 - RNA, 897 nt, Homo sapiens
  source 1..897: mol_type = other RNA
tcagcaggcaggctggtgcagcttcttcactcacagaccggcaatgacatcccctgtcacctgtaaatcaccgaggtgccattaatcaacaatatgcatccagtgagggccaactctgggcccagcatgggcaggtggactgctttgctgtaaaatattccaacaccaagaactcccgagaagcgacctgtttgaggatgaagaggctgaatctttcagggtcgtcctgcttctgcgtcttcttccttcagcattctccacagccagggccttggctgtttctgcaacaagtgcatgggcaatccgacgagaagaccagtatccgcttggggggtgagatggggggcgagcagagtagtgagcaagcgtgcaggctctcctgatgctggaaacttactcccagatatagcgcccgccagccccctttcccagccctgctccccttcctgccctccgccgcaagcaactccaaactctccgcatccagccgttctccctccccagtggaaatttgcagcgccgggctgcgcgcgtgcatccaccctccccttcaggaaacttactccccatctgcatgcaccgcctctcagccatcgcttagagggaagggggtgtgctggggagacagaaatacatatgtatctctcgcccctcccccggtcgcagcccactcggggccgagccgcggtaacctggccttacctttgcattgctccccatcctcgccccctcccttaaccctccttatccgctccccggtaccccccttttttcacccattacccacccctagcaaccgttcccaagctcctctcggccttttttttttttttaaatccaggatgcaaattcctcccttgtcagcaaatcgactgtcaaattattttcttgcaaaag

SEQ ID NO: 17139 - RNA, 790 nt, Homo sapiens
  source 1..790: mol_type = other RNA
tcagcaggcaggctggtgcagcttcttcactcacagaccggcaatgctgtaaatcaccgaggtgccattaatcaacaatatgcatccagtgagggccaactctgggcccagcatgggcaggtggactgctttgctgtaaaatattccaacaccaagaactcccgagaagcgacctgtttgaggatgaagaggctgaatctttcagggtcgtcctgcttctgcgtcttcttccttcagcattctccacagccagggccttggctgtttctgcaacaagtgcatgggcaatccgacgagaagaccagtatccgcttggggggtgagatggggggcgagcagagtagtgagcaagcgtgcaggctctcctgatgctggaaacttactcccagatatagcgcccgccagccccctttcccagccctgctccccttcctgccctccgccgcaagcaactccaaactctccgcatccagccgttctccctccccagtggaaatttgcagcgccgggctgcgcgcgtgcatccaccctccccttcaggaaacttactccccatctgcatgcaccgcctctcagccatcgcttagagggaagggggtgtgctggggagacagaaatacatatgtatctctcgcccctcccccggtcgcagcccactcggggccgagccgcggtaacctggccttacctttgcattgctccccatcctcgccccctcccttaaccctccttatccgctccccggtaccccccttttttcacccattacccacccctagcaaccgttccc

SEQ ID NO: 17140 - RNA, 883 nt, Homo sapiens
  source 1..883: mol_type = other RNA
tcagcaggcaggctggtgcagcttcttcactcacagaccggcaatgctgtaaatcaccgaggtgccattaatcaacaatatgcatccagtgagggccaactctgggcccagcatgggcaggtggactgctttgctgtaaaatattccaacaccaagaactcccgagaagcgacctgtttgaggatgaagaggctgaatctttcagggtcgtcctgcttctgcgtcttcttccttcagcattctccacagccagggccttggctgtttctgcaacaagtgcatgggcaatccgacgagaagaccagtatccgcttggggggtgagatggggggcgagcagagtagtgagcaagcgtgcaggctctcctgatgctggaaacttactcccagatatagcgcccgccagccccctttcccagccctgctccccttcctgccctccgccgcaagcaactccaaactctccgcatccagccgttctccctccccagtggaaatttgcagcgccgggctgcgcgcgtgcatccaccctccccttcaggaaacttactccccatctgcatgcaccgcctctcagccatcgcttagagggaagggggtgtgctggggagacagaaatacatatgtatctctcgcccctcccccggtcgcagcccactcggggccgagccgcggtaacctggccttacctttgcattgctccccatcctcgccccctcccttaaccctccttatccgctccccggtaccccccttttttcacccattacccacccctagcaaccgttcccaagctcctctcggccttttttttttttttaaatccaggatgcaaattcctcccttgtcagcaaatcgactgtcaaattattttcttgcaaaag

SEQ ID NO: 17141 - RNA, 806 nt, Homo sapiens
  source 1..806: mol_type = other RNA
tcagcaggcaggctggtgcagcttcttcactcacagaccggcaatggactgctttgctgtaaaatattccaacaccaagaactcccgagaagcgacctgtttgaggatgaagaggctgaatctttcagggtcgtcctgcttctgcgtcttcttccttcagcattctccacagccagggccttggctgtttctgcaacaagtgcatgggcaatccgacgagaagaccagtatccgcttggggggtgagatggggggcgagcagagtagtgagcaagcgtgcaggctctcctgatgctggaaacttactcccagatatagcgcccgccagccccctttcccagccctgctccccttcctgccctccgccgcaagcaactccaaactctccgcatccagccgttctccctccccagtggaaatttgcagcgccgggctgcgcgcgtgcatccaccctccccttcaggaaacttactccccatctgcatgcaccgcctctcagccatcgcttagagggaagggggtgtgctggggagacagaaatacatatgtatctctcgcccctcccccggtcgcagcccactcggggccgagccgcggtaacctggccttacctttgcattgctccccatcctcgccccctcccttaaccctccttatccgctccccggtaccccccttttttcacccattacccacccctagcaaccgttcccaagctcctctcggccttttttttttttttaaatccaggatgcaaattcctcccttgtcagcaaatcgactgtcaaattattttcttgcaaaag

SEQ ID NO: 17142 - RNA, 3000 nt, Homo sapiens
  source 1..3000: mol_type = other RNA
tcaggccaggcacagtggctcaaacgtgtaatcccagcactttgggaggccgaggcaggtagatcacctgaggtcaggagttcgagaccagcctagccaacatggtgaaaccctgtctctacaaaaaatacaaaaattagccgggcttggtggcaggcatctaatcccagctactcgggaggctgaggcaggagaatcacttgaacacaggaggtggagtttgcagtgagccaaaattgtgcgattgtactccagcctaggcaacaagagcaagactccattaaaaaaaaaaaaaagtaacaaaagagcaaagtaagccagctgataggctgtttttatatagttcccaattcacttcgatgacagtcactaccacacagcacactctagggtcctgtggtctgggggtaaagaaaagttatcagcagtgactgggaatgagccttggtggagatctcagactctgctagcaggaaaaagcatgagggtaagtcctggagtcctcaagagctccttccttgaagagcccctggggagcagacatcctattgaaaagaggcaaggtcatgggataaggaggtttacagtgggagactggaaagaagaacctaatgtcctttctggaaaataaatgttttcattagtgtatataataatgctgttaagaactcagctgtctgggcttaaattctggctgtcacttattagctgtatgacctttgataagtcacttactcacttcaggatccaatttcttaatgggttaacagcatcttcctcatatgatgctatgaggatcaatgtcaagtgctcattagagtagctggtatacattaactgctcaataaatgttagctatttattattgttgttcttattataattattttattattgtttgatcatcttctctcgagacttgacatcaggacagaaacgccagtatatatacaggatatttgaataaggaggcatttaaccatcgaaagtaaataaaccagaaattggataggcgtggtagctcatgcctgtaatcccagcactttgggaggttgaggtgggcagatcactagagtccaggagttcaagaccagcctgggcaacatggcaaagccttgtctccacacacaaaaaaatacaaaaattagctaggtgtggtggtgtgtgcctttagtcccagttatgcagaaggatgaggcgggaggattgataaactaccccacgtggtagtttaacctgttgcctatactttggaaacaaagagaaaaatgcatccaagtttggcaaaggaaagcagcaatcacctatctgtcttgtgcccaccatcaagagagttcttgagatcaaagtttccaaatggagacttagctctggcaactgcagaaaagtttacgaagaatctgaaggaccagactgatggctagacttcatccagagacaacaatggggtgggacccagtgaaggaagtgaattgggttatgagttccacagcataagtaatcccaaaagcagggactgtgagtgctttttattccatgcaaaagagagaagtgggtctctgaggagtatctggggctggctggctagagacgctagggaaaggtagacaaggcttcctgagtgtgtggtgctttcttgctgacttgccctatatacctaaagtccatggtagaaacctgaacctacagaacctccaccaaaagagaggagagcacgggattctcagagactggcttccacttgaacagggaaggccaattccctgtgggcctgtcaacatcaacttcagttctctcgcccttacaggaggcctctgactgtatcactattttagaaatattgctgccatgtaagcttctttcaaggtgaagcttggaagctgttctccaagtccatcctcagcagctgaggccacaacagattaactgaagagaccccttggcttcttcctcttgacctttgacagctgaggtctctgcagagggcctgaagtacccgtggactctttctcaggtgctgagagggttggggctgaggagaccagttgttctggctggtttacacattggctatcgattccttgcagggaagcactgtttgaggtatgaggatctccagcgccttgatgcttctgtcccacttggacctcttgtgtggtgactgccatatacagatcctgcagattcatgacaaagggctttccatcaccaatgctgcatgcctctggcagtttcatgataaaaagagaccgatgcagcatgtagagttctaggccaatatgccgggtctccagttttgatgggtatatcttttaactctatcataaattgttccaagaaggaattttcttcaaatggttctgtcttcaatcgatctcgaatcagcgtagccccactctcctggtagtcttggatctctaggtctttcatatgaagtaacgttgctagctccctcacttggcactgtaatgccagactcatgcccatcagaggacgaatcaaatgttgggagaccagggaaggactagctagcatgcagtggaaattccaatagaaggggaggccagagagctcacttcgcacccgtagaatcagtgcatctgccacacaatcacaggagaaggtagcttcgctagggtgagcagcgtccttcaacaatgggcgaaggagattatccaaatgacagaggaaagctgcaggaggagcagtgagccgcttgttcagctccttggctcgctggctgaccacactagtgtccacctgttcatgccacacctgttgaagatctgaaaccaacaaggcatagccctgcttggtgataaaaaccttggccaagagggagttctctgcaagctgtagccacgcccatggctgcatcaacaggccttgctccagttcttccatcgtcagcggccgcgagagcgcccactctcttagccgcacgcacgctttcctgcccgctcgcgcaaaccgaaaggcctagagtaagaggccgctttc

SEQ ID NO: 17143 - RNA, 2918 nt, Homo sapiens
  source 1..2918: mol_type = other RNA
tcaggccaggcacagtggctcaaacgtgtaatcccagcactttgggaggccgaggcaggtagatcacctgaggtcaggagttcgagaccagcctagccaacatggtgaaaccctgtctctacaaaaaatacaaaaattagccgggcttggtggcaggcatctaatcccagctactcgggaggctgaggcaggagaatcacttgaacacaggaggtggagtttgcagtgagccaaaattgtgcgattgtactccagcctaggcaacaagagcaagactccattaaaaaaaaaaaaaagtaacaaaagagcaaagtaagccagctgataggctgtttttatatagttcccaattcacttcgatgacagtcactaccacacagcacactctagggtcctgtggtctgggggtaaagaaaagttatcagcagtgactgggaatgagccttggtggagatctcagactctgctagcaggaaaaagcatgagggtaagtcctggagtcctcaagagctccttccttgaagagcccctggggagcagacatcctattgaaaagaggcaaggtcatgggataaggaggtttacagtgggagactggaaagaagaacctaatgtcctttctggaaaataaatgttttcattagtgtatataataatgctgttaagaactcagctgtctgggcttaaattctggctgtcacttattagctgtatgacctttgataagtcacttactcacttcaggatccaatttcttaatgggttaacagcatcttcctcatatgatgctatgaggatcaatgtcaagtgctcattagagtagctggtatacattaactgctcaataaatgttagctatttattattgttgttcttattataattattttattattgtttgatcatcttctctcgagacttgacatcaggacagaaacgccagtatatatacaggatatttgaataaggaggcatttaaccatcgaaagtaaataaaccagaaattggataggcgtggtagctcatgcctgtaatcccagcactttgggaggttgaggtgggcagatcactagagtccaggagttcaagaccagcctgggcaacatggcaaagccttgtctccacacacaaaaaaatacaaaaattagctaggtgtggtggtgtgtgcctttagtcccagttatgcagaaggatgaggcgggaggattgataaactaccccacgtggtagtttaacctgttgcctatactttggaaacaaagagaaaaatgcatccaagtttggcaaaggaaagcagcaatcacctatctgtcttgtgcccaccatcaagagagttcttgagatcaaagtttccaaatggagacttagctctggcaactgcagaaaagtttacgaagaatctgaaggaccagactgatggctagacttcatccagagacaacaatggggtgggacccagtgaaggaagtgaattgggttatgagttccacagcataagtaatcccaaaagcagggactgtgagtgctttttattccatgcaaaagagagaagtgggtctctgaggagtatctggggctggctggctagagacgctagggaaaggtagacaaggcttcctgagtgtgtggtgctttcttgctgacttgccctatatacctaaagtccatggtagaaacctgaacctacagaacctccaccaaaagagaggagagcacgggattctcagagactggcttccacttgaacagggaaggccaattccctgtgggcctgtcaacatcaacttcagttctctcgcccttacaggaggcctctgactgtatcactattttagaaatattgctgccatgtaagcttctttcaaggtgaagcttggaagctgttctccaagtccatcctcagcagctgaggccacaacagattaactgaagagaccccttggcttcttcctcttgacctttgacagctgaggtctctgcagagggcctgaagtacccgtggactctttctcaggtgctgagagggttggggctgaggagaccagttgttctggctggtttacacattggctatcgattccttgcagggaagcactgtttgaggtatgaggatctccagcgccttgatgcttctgtcccacttggacctcttgtgtggtgactgccatatacagatcctgcagattcatgacaaagggctttccatcaccaatgctgcatgcctctggcagtttctctatcataaattgttccaagaaggaattttcttcaaatggttctgtcttcaatcgatctcgaatcagcgtagccccactctcctggtagtcttggatctctaggtctttcatatgaagtaacgttgctagctccctcacttggcactgtaatgccagactcatgcccatcagaggacgaatcaaatgttgggagaccagggaaggactagctagcatgcagtggaaattccaatagaaggggaggccagagagctcacttcgcacccgtagaatcagtgcatctgccacacaatcacaggagaaggtagcttcgctagggtgagcagcgtccttcaacaatgggcgaaggagattatccaaatgacagaggaaagctgcaggaggagcagtgagccgcttgttcagctccttggctcgctggctgaccacactagtgtccacctgttcatgccacacctgttgaagatctgaaaccaacaaggcatagccctgcttggtgataaaaaccttggccaagagggagttctctgcaagctgtagccacgcccatggctgcatcaacaggccttgctccagttcttccatcgtcagcggccgcgagagcgcccactctcttagccgcacgcacgctttcctgcccgctcgcgcaaaccgaaaggcctagagtaagaggccgctttc

SEQ ID NO: 17144 - RNA, 2868 nt, Homo sapiens
  source 1..2868: mol_type = other RNA
tcaggccaggcacagtggctcaaacgtgtaatcccagcactttgggaggccgaggcaggtagatcacctgaggtcaggagttcgagaccagcctagccaacatggtgaaaccctgtctctacaaaaaatacaaaaattagccgggcttggtggcaggcatctaatcccagctactcgggaggctgaggcaggagaatcacttgaacacaggaggtggagtttgcagtgagccaaaattgtgcgattgtactccagcctaggcaacaagagcaagactccattaaaaaaaaaaaaaagtaacaaaagagcaaagtaagccagctgataggctgtttttatatagttcccaattcacttcgatgacagtcactaccacacagcacactctagggtcctgtggtctgggggtaaagaaaagttatcagcagtgactgggaatgagccttggtggagatctcagactctgctagcaggaaaaagcatgagggtaagtcctggagtcctcaagagctccttccttgaagagcccctggggagcagacatcctattgaaaagaggcaaggtcatgggataaggaggtttacagtgggagactggaaagaagaacctaatgtcctttctggaaaataaatgttttcattagtgtatataataatgctgttaagaactcagctgtctgggcttaaattctggctgtcacttattagctgtatgacctttgataagtcacttactcacttcaggatccaatttcttaatgggttaacagcatcttcctcatatgatgctatgaggatcaatgtcaagtgctcattagagtagctggtatacattaactgctcaataaatgttagctatttattattgttgttcttattataattattttattattgtttgatcatcttctctcgagacttgacatcaggacagaaacgccagtatatatacaggatatttgaataaggaggcatttaaccatcgaaagtaaataaaccagaaattggataggcgtggtagctcatgcctgtaatcccagcactttgggaggttgaggtgggcagatcactagagtccaggagttcaagaccagcctgggcaacatggcaaagccttgtctccacacacaaaaaaatacaaaaattagctaggtgtggtggtgtgtgcctttagtcccagttatgcagaaggatgaggcgggaggattgataaactaccccacgtggtagtttaacctgttgcctatactttggaaacaaagagaaaaatgcatccaagtttggcaaaggaaagcagcaatcacctatctgtcttgtgcccaccatcaagagagttcttgagatcaaagtttccaaatggagacttagctctggcaactgcagaaaagtttacgaagaatctgaaggaccagactgatggctagacttcatccagagacaacaatggggtgggacccagtgaaggaagtgaattgggttatgagttccacagcataagtaatcccaaaagcagggactgtgagtgctttttattccatgcaaaagagagaagtgggtctctgaggagtatctggggctggctggctagagacgctagggaaaggtagacaaggcttcctgagtgtgtggtgctttcttgctgacttgccctatatacctaaagtccatggtagaaacctgaacctacagaacctccaccaaaagagaggagagcacgggattctcagagactggcttccacttgaacagggaaggccaattccctgtgggcctgtcaacatcaacttcagttctctcgcccttacaggaggcctctgactgtatcactattttagaaatattgctgccatgtaagcttctttcaaggtgaagcttggaagctgttctccaagtccatcctcagcagctgaggccacaacagattaactgaagagaccccttggcttcttcctcttgacctttgacagctgaggtctctgcagagggcctgaagtacccgtggactctttctcaggtgctgagagggttggggctgaggagaccagttgttctggctggtttacacattggctatcgattccttgcagggaagcactgtttgaggtatgaggatctccagcgccttgatgcttctgtcccacttggacctcttgtgtggtgactgccatatacagatcctgcagattcatgacaaagggctttccatcaccaatgctgcatgcctctggcagtttctctatcataaattgttccaagaaggaattttcttcaaatggttctgtcttcaatcgatctcgaatcagcgtagccccactctcctggtagtcttggatctctaggtctttcatatgaagtaacgttgctagctccctcacttggcactgtaatgccagactcatgcccatcagaggacgaatcaaatgttgggagaccagggaaggactagctagcatgcagtggaaattccaatagaaggggaggccagagagctcacttcgcacccgtagaatcagtgcatctgccacacaatcacaggagaaggtagcttcgctagggtgagcagcgtccttcaacaatgggcgaaggagattatccaaatgacagaggaaagctgcaggaggagcagtgagccgcttgttcagctccttggctcgctggctgaccacactagtgtccacctgttcatgccacacctgttgaagatctgaaaccaacaaggcatagccctgcttggtgataaaaaccttggccaagagggagttctctgcaagctgtagccacgcccatggctgcatcaacaggccttgctccagttcttccatcttcactcgagccctaccatccacgccgggcagcagccagcggact

SEQ ID NO: 17145 - RNA, 2933 nt, Homo sapiens
  source 1..2933: mol_type = other RNA
tcaggccaggcacagtggctcaaacgtgtaatcccagcactttgggaggccgaggcaggtagatcacctgaggtcaggagttcgagaccagcctagccaacatggtgaaaccctgtctctacaaaaaatacaaaaattagccgggcttggtggcaggcatctaatcccagctactcgggaggctgaggcaggagaatcacttgaacacaggaggtggagtttgcagtgagccaaaattgtgcgattgtactccagcctaggcaacaagagcaagactccattaaaaaaaaaaaaaagtaacaaaagagcaaagtaagccagctgataggctgtttttatatagttcccaattcacttcgatgacagtcactaccacacagcacactctagggtcctgtggtctgggggtaaagaaaagttatcagcagtgactgggaatgagccttggtggagatctcagactctgctagcaggaaaaagcatgagggtaagtcctggagtcctcaagagctccttccttgaagagcccctggggagcagacatcctattgaaaagaggcaaggtcatgggataaggaggtttacagtgggagactggaaagaagaacctaatgtcctttctggaaaataaatgttttcattagtgtatataataatgctgttaagaactcagctgtctgggcttaaattctggctgtcacttattagctgtatgacctttgataagtcacttactcacttcaggatccaatttcttaatgggttaacagcatcttcctcatatgatgctatgaggatcaatgtcaagtgctcattagagtagctggtatacattaactgctcaataaatgttagctatttattattgttgttcttattataattattttattattgtttgatcatcttctctcgagacttgacatcaggacagaaacgccagtatatatacaggatatttgaataaggaggcatttaaccatcgaaagtaaataaaccagaaattggataggcgtggtagctcatgcctgtaatcccagcactttgggaggttgaggtgggcagatcactagagtccaggagttcaagaccagcctgggcaacatggcaaagccttgtctccacacacaaaaaaatacaaaaattagctaggtgtggtggtgtgtgcctttagtcccagttatgcagaaggatgaggcgggaggattgataaactaccccacgtggtagtttaacctgttgcctatactttggaaacaaagagaaaaatgcatccaagtttggcaaaggaaagcagcaatcacctatctgtcttgtgcccaccatcaagagagttcttgagatcaaagtttccaaatggagacttagctctggcaactgcagaaaagtttacgaagaatctgaaggaccagactgatggctagacttcatccagagacaacaatggggtgggacccagtgaaggaagtgaattgggttatgagttccacagcataagtaatcccaaaagcagggactgtgagtgctttttattccatgcaaaagagagaagtgggtctctgaggagtatctggggctggctggctagagacgctagggaaaggtagacaaggcttcctgagtgtgtggtgctttcttgctgacttgccctatatacctaaagtccatggtagaaacctgaacctacagaacctccaccaaaagagaggagagcacgggattctcagagactggcttccacttgaacagggaaggccaattccctgtgggcctgtcaacatcaacttcagttctctcgcccttacaggaggcctctgactgtatcactattttagaaatattgctgccatgtaagcttctttcaaggtgaagcttggaagctgttctccaagtccatcctcagcagctgaggccacaacagattaactgaagagaccccttggcttcttcctcttgacctttgacagctgaggtctctgcagagggcctgaagtacccgtggactctttctcaggtgctgagagggttggggctgaggagaccagttgttctggctggtttacacattggctatcgattccttgcagggaagcactgtttgaggtatgaggatctcctctggagggctcaccagcgccttgatgcttctgtcccacttggacctcttgtgtggtgactgccatatacagatcctgcagattcatgacaaagggctttccatcaccaatgctgcatgcctctggcagtttctctatcataaattgttccaagaaggaattttcttcaaatggttctgtcttcaatcgatctcgaatcagcgtagccccactctcctggtagtcttggatctctaggtctttcatatgaagtaacgttgctagctccctcacttggcactgtaatgccagactcatgcccatcagaggacgaatcaaatgttgggagaccagggaaggactagctagcatgcagtggaaattccaatagaaggggaggccagagagctcacttcgcacccgtagaatcagtgcatctgccacacaatcacaggagaaggtagcttcgctagggtgagcagcgtccttcaacaatgggcgaaggagattatccaaatgacagaggaaagctgcaggaggagcagtgagccgcttgttcagctccttggctcgctggctgaccacactagtgtccacctgttcatgccacacctgttgaagatctgaaaccaacaaggcatagccctgcttggtgataaaaaccttggccaagagggagttctctgcaagctgtagccacgcccatggctgcatcaacaggccttgctccagttcttccatcgtcagcggccgcgagagcgcccactctcttagccgcacgcacgctttcctgcccgctcgcgcaaaccgaaaggcctagagtaagaggccgctttc

SEQ ID NO: 17146 - RNA, 11487 nt, Homo sapiens
  source 1..11487: mol_type = other RNA
tcaggccaggcacagtggctcaaccctgtcatcctagcattttgggaggctgatgcagaaggataacttgaacaggatttcaagaccagcctgggcaatatagtgagacacagtctcgaccaaaaaaaaaaaaatttaaaaataaaaaaattagccgggcctggtggtacatgcctgcattcccagctactcagaaggctgaggtgagaggattgcttgagcccaggaggtcgaggctgcagtgagctatgattgcaccactgcactccagcctaggtgacatggcaagacactgtctctggaaaaaaaaaaaaaaaaaaagaacaccaccggccactgtggctcattcctgtaatcccagcactttgggaggttgaatcaggctgaatcaggggggtctcaggagttcaagaccatcctggccaacatggcaaaaccccgcctctactgaaaatacaaaaattagctgggtgtggtggtgcacacctgtaatcccaggtacttgggaggctgaggcaggagaatcacttgaacccaggaattggaggttgcagtgagctgagatcacgccactgcactccagcctgggtgacagagcgagactctgtcattcataaataaataagtttagaaaaaaaaaatgtgtctgaaagggtcttgagcatccctctgggcaaattccaggcatcatccataatgatgaatgcacaaatacaaagatacgaatgagccagagccaaccttatattcctgcagtaaatgccactgggtttactattttcttatcaagcagttggaatttatttgctaatccgttccttcctagcttccttttttccttcttttttttttttttttaaatggagtcttgctctgttgcccaggctggaatgcagtggcatgatcttggctcactgcattttttaatttttaagttttttgtagatggggggcttgctatgctgtccaggcaggtctcgaactcctgagctcaagtaatccttttgcctcctttcaaagtgttgagactccaggcataagccactttgcccagttgctactattatacttagcgcatttttttgtttgtttgttttttgagacagtcttactctgtatcccaggctggagtgcagtggtgtgatctcggttcactgtaacctcctgcctcagcctcccgagtagctaggaatacatgcacatgccaccacgcccagctatatttttttagttttagtagatacaaggtttcaccgttttagccaggatcatctcaatctgaccttgtgatccacctgcctcagcctcccaaagtgctgggattacaggcatgtgagccaccgtacctggcttacttagtgaatttgtaccaatattcattaccaatataattctgtagtttttaatgactgtactgtttttatcagtgataaaaacgatacatatatacatcttgtactgcatcataaaaagatttagcaagatttgcttcattgttaatactctgaaaggatttatggagaattaggaccaattggaccttgaaaatgtcatgtaaagatgtctggctgggcatggtggctcatgcttgtaatcccagcactttgggaggcccagaagagaggattactctagctcaggagtttgaggacagcctgggcaatggagtgagataccttctctaccaaaataaaaaagtgtgagtttaggtgctgtgttccttgttgttgttacagtgtgagccaccgtgcctggccgagactgggtaagttatgaagaaaaagaggtttaatggactcacagttccacatggctggggaggcctcaaaatcatgacagaaggtgaaggaggagcaaaggcacatcttatatggcagaaggcaagagagcctgtccaggggaacagctgcttataaaactgacagacctcatgagatttactcactgtgacaaaaacagcacacgcctattatcccagctacttggctgactgaggcatgagaattacttgaacagcatggggaaacccccccccatgattctattacctcccacctggtctctccctcgacaccatggggattatgggagctacaattcaagatgacatttgggtggggacacagccaaaccatatcagctggcaacttgcttgcagctcataacatcaactgtttctttgggccttcagtcctgctgacttccggcctcctgagtccctaagcagaggaatacgaattcaaatcttgattttctcattgcagctcatagtgggagatgcccagtctctctgtgaacattgacagaattttttttttttttttgagacagagtctcacactgtcaccaggctggagtgccgtggcgcaatatcagctcactgtaacctccacctcccaggttgaagtgattctcccatctcagcccccaagtagctgggactacaggtgagtgccaccacacccagctaatttttgtatttttagtagagatgggggttcaccatgttgcccaaaatggtctcaatctcttggcctcgtgatccaaccatctcagcctcccaaagtgctgggtttaaaggcatgagccactgtgcctggcccagaattctttactgctaacacgagtgggcctggttctggaggatttcccagtgggtcctgaagaaccacagtttattggcttgtgggcaaaggggtatgtgtatcagttggcctttactgtgtaataaacagccacaaaaattactagctgaaaacagcagctacttaattagcagaagcctcttgaggatggacttgcaaaccaaagttgtgctggtttctactggtcaaagcaaggactggctcacataaaaaggagagagattgcaccttcagagagtaatctcaagacatctgtaatctaccacagggtgtcactgggcctctgtcaaggagcctattctttctgccaccagatctgtctaatagcttgtgtgacaatgcacttccttctgggtctctctccaagtgtagtaagtgtatatgggaatcactttattcaaacagtgtagtgcacttagttagaaagaaaaggtattaaggaagacttatatttaaaattgttatttatggtaacaacgaaaagtaacatacaaatttcaaacatcaagaataaaataaattaaaggtatgatcaatacacatcagtacaaagaggggaacacaatgaaacaaacaaaaaaaattagatgctagaaattaatccaaattattactaattaaatgtcaggcactaaatgtgcaacataaaaggattgttaattggtattattcaagtattttttctttttttttttttttttgtgacagagtttcactcttgttgcccaggctgcagtgcaatggcgtgatctcggctcactgcaacctctgcctcccgggttcaaatgattctcctgcctcagcctcccaagtagctggcattacaggcatgcaccactaggcacagctaattttgtatttttagtagagatggggtttctcagtgttggtcaggctggtctcgaactcccgacctcaggtgatcacctgccttggcctcccaaagtgctgtgattacagacatcagccactatgcccagcggtatacagattttttaaaactccagctaaagtatgtataaaaagacacatttttttaaaaagcatacagaaagactaagaagtagaggaaaatcaagctgatgtaactatataaatatctaacagaattagtggaacagaaaacatgcaagaaatagtgtagatttttcaagcgaaatatctgaaagaattcataaacctgggtactctctaccaagattaacacaagcaaagggaaagaatgcacaattaataagttattccagaatgcaaaaggagactgaagttatacaaccagcaaaaatgaaaaatataaaaagtataaatttttgctacacatttggaaataaaaacatgcctagaagaatattctcaaaatacttatgcaagccttagttgtctttttttttttttttttatgagatggagttttgctcttgtcacccaggctggagtgcagtggcaagaactcaactcactgcaaccttcgcctcccagattcaagcaattctcctgcctcagcctcccaagcggctgggattacaggcgcccgccaactcacctggctaattttattttttgaatttttagtagagacaaaagtttcaccgcattggccaggctggtctcgaactcctgacctcaggtgaccccctgccttgacctcccaaagtgctgtgattaaagccgtgaagcaccgtgcccaacctagttgtctttttttttttttttgagacggattctcgctctgtcgtcaggctggagtgcagtggtgtgatctaggctcattgaaacctccacttcaggggttcaagagattctcctgcctcagcctcctgagtagctgggattacaggggcacaataccgtgcccagctaatttttgtatttttagtaaagacggggtttcaacatgttggccaggatggtcttgatctcttgacctcatgatctgcctgcctcagcctcccaaagtggtgggattacaggcatgagccaccactcccagcctgataactgttttatttatttatttttatttttttggagatatggggtctgtgttgcccagactgatcttgaactcctggcctcaaggaatccttctgactgagcttcccagtgtgctgggattaaaagtgtgagccactatgaccagccagaagagataattttaactttttaaaatattttgcagtattggccgggcacagtggcttgtgcctgtaatcccagtactttgggagtatgaggcatgcagatcacctgaggtcaggagtttgagaccagcctggccaacttgatgaaaccgtctctactaaaaatacaaaaatcagccaggcaaggtggaggctgtctgtaatctcagctactcgggaggctgaggcaggagaaccactggaacccaggaggtggaatttgcagtaagttgagatcacaccattgcactccagcctgggcaacgagtgaaacactaactcaaaaacaaagaaacaaacaccaactcaaaaacaaagaaacaaaccaaaaaaatgaaaatatcttgtagtatttttaaatagagatgtggtttcgctatgttgcccaggctggtttgaactccttggctcaagggatctttttgcctcagcctccaaaagtgctgggattacaggcctgagccactattcccaacctagatgactcttatagattaagaatttagaaatagtaggaacatgccccactacagtatatgacagtcattatatacaaatatcattaagggacaattttttaaaaatcacaatgttattcaaacatagctccataacatattagtaaaggtcatgaagtatttttaagtgatccattatgtcacagtcgagcttatccaggaatacaaggttgatgtaacattggaaaagcaataaatacaaataccacatttatttaatttaatttatttatttttgacagagtcgcaccctgtcacccagcatggagtgcagtggtgcaatcttggctcaatgcaacctccacctcccaggttcaagtgattctcctgcttcagcctcccaagtagctgggattacaggtgcacatcaccacacccagctaatttttgtattgttagtagagatggggtttcaccatgttggctgggctggtctcgaactcttgacctcaaatgatctgcccacccccacctcccaaattgctgggattacaggcataagcccccacacccagcctgaccacatttgttttagaaaagcgcctttccatgcattcacttcttcaagttttttttttgttttgtttttgtttttttttttgagatggggtcttgctatgttgcctaagctggtctagaacccctgggctcaggccaccctcccaagtagctaaaactataggcatgcatcaccacatcatttcattgaagtatttattaggtaccatcatgagctaggtgcagttctaggtattgagttttatcagtaaataaacatgatcatcacagaggatgtgaaggaagcatttaataaattcaagaggaattcagcctcataaactatgaaatattgggaaataattcatcatgtaaaaactggatataaagaaaaaacttttcctgcaggacattgttgcaggaagtcagggaccccaaacggggggactggctgaagccatggcagaaaaacatggattgtgaaggtttcatggacatttattagttccccaaattaatacttttataatttcttatgcctgtctttactgcaatctctaaacataaattgtaaagatttcatggacacttatcacttccccagtcaatacccttgtgatttcctatgcctgtctttactttaatctctcaatcctgtcagctgaggaggatgtatattacctcaggaccctgtaataattgcattaactgcacaaattatacagcatgtgtgtttgagcaatatgaaatctgggcaccttgaaaaaagaacaggataacagcaatgtttaggaaacaagagagataaccttaaattctgaccgccggtgagccaggtggaacaaagccacatttctcttctttcacaagcaaatgggagaaatatcactgaattctttttctcagcaaggaacatccttgagaaagagaatgcacacctgggagtgggtctctgaactggcccccctgggtgtagccatctcttatggtcgagactgcaggggtgaaatagaccccagtctcccatagcactcccaggcttattaggaagaggaaattcccacctaataaattttagtcagaccagttgatctcaaaaccgtctcctgataagatgttatcaatgacaatggtgcccaaaacttcattagcaattttaatttcaccttggtcctgtgatctcgccctgcctccacttgccttgtgatattctattaccttgtaaagtacttgatgtctgtgacccacacctatttgcacactccctccccttttgaaaatccctaataaaaacttgctggtttttgcggcttgtggggcatcacggaacctaccgacatgtgatgtctgccccggacacccagctttaaaatttctctcttttgtactctgtccctttatttctcaagttggctgacacttagggaaaatagaaaagaacctatgtgaatatcggggctggttccctgacaggacataacctcttcaaaaaataaaaaagaaataaaagcctacagccaaaccaacaaaatagagtgcatatctcaccagaactgcaaagacaagtatgctggtattactacttttagttggtgttgtgcagcgggttaaaatcagtccagtaaagcaagaaaatatttagagagagcttcatcatcatacgaattttgggggtcattgttcagtccaaagtacttaatatgattcttttctctttccacatagagaatcagataatctataaataatgactcttactgttccactttaggagttaggtatacatacatatgtgtatatatatgtatatatatatacacatacacacacacacacacacacacacagtgaccccccaaatttcatatgaagttccaaacctcaatgtgactgtatgtgaaaagagaagggggcggggaggggggagaccgaccgacctatttgttggtctccatcgtgtgaaaacatgaggaagtgggcacttacatgccaggaagagagctctcactagaggttgaccatgctggcactctgatctcagacttccagcctccagatatgtgagaatataaatttgtgttttgggccagatacggtggctcaggcctgtaatcccagcactttgggaggccaaggcaggtggatcaccaaaggtcagatctgaccaacatggagatcagcctaaccaacatggagaaaccctgtctctactaaaaatacaaacttagctaaggtttgtggtgcatgccaataatcccagctactgagggtgaggcaggagaatcactggaactcaggaggtggaggttgcggtgagccaagatcataccattgcactccagcctgggcaacaagagcaaaactccatctcaaaaaaaaaaaaaaaaaaaaaaaaaaaatcctgtgtttttaacctcattgatttaaaattaaattaatttctaagccatttggtctgcggtattctcttatggttgtctgagctgactaaggcagatattggtactgagaagtgaggtactgcaattaaaaacaaacaaaaaaactaaaaatgtgaagcagctttgaaactgacaaatgagtagaggctggaaaaattctgatgtgcaagctggaaataaggttggtaagggttattctggtgaggtgtcattggggaatgaggaacatgctattgggaaatgaagaaaagacaacccttgatataaagtggtgaagaacttggcagaactgtattctagcattttacggaaggtagagcttgagacagataaaatggtatgtatcactaagatctgtaattaaagtgttaaaggacacaggaagcttcattattcctgagtgcttacaggaaaatgtgctgggaacaggccccccaaatctggccataaacaggcaatgagaaactggccataaacaaaatctctgcagcactgtgacatgctcgtgatggctatgacgcccatgctggaggctgctggtttaccagaatgagggcaagcaacacctggcccacccagggcagaaaactggaaaactgctcaaggcattcctaaaccacaaacaatagcatgagtgatttgtgccttaaggacatattcctgttgcagataacaagccagagcctgtccctttctttctcataaggaatacttatagctgatctacaatctataggaataatgtttatcacaggcttactgtcaataaatatgtgggtcaaactctgttcaagctcagctctgaaggctgtgagccccgattcccactctgcactatatttctgtgtctttgtcttaattcctctagagccactgggttagggtctccacgacccagctggtctcggcaaaaatgcaaaaggagacctgaattgcagaagaaattgttaaggaaaaaggaaccagaacttggagatttggaaaattctcagcctatccatactgcaaaaattagaaaacttgtactgaagagaatcctcaaagtgtggctgaacaatcatttgataaagagatcatgagtgggattcatggactatatcagccatcttaacagaagtgagaagagagactggattatactataagagacactgccacttacattgtgccacctaaaatggacagagaagacagaacagaacagtcaaggttgtcacacttcttattttacaagaaggggacatagaaataatcagctgtgaaagggcactggcagttatggatggtttcactcctgacatgctctgcaggatccatgggaacagaagagaaccttggaggagcatctttttaacaatccacctctggggcctacatcatcttggcttctggtaaattttgacatgaatgtgccacactggcagccactaaccaacaggggctgggatcaatctgcatgatttatctcgtacagaacttgttaatgctatgatcttaggaatctaatcaccaaggtgaggcagcctgcagtactgacctcaccatccatgacccttcttcacagatgcccagactcaggtaaccatgatgttgtattcagaacctgtaggtttaatttcagaccctcgggatgcatctaaggccaatctgtgagccattacaacctccaaaaggcatttaggactaatctgatgatctttgcactgccaataattaaagatggcaaccaatgggctaaatggtaacaacactcatatccttacattcatagtatttctccccagtgtgaattctttcatgcatacttaggcatgaggaaagagcaaatgctttcccaaattctttacatacaaaaggtttctctctggtaggagttcacaggtggggtgaggaatacagaaattctttcccacatatcttgcatttacctttctccactgtgagttttcaaatgtttactacgatgggaagaagtaatgaaggtcttcccacattcaacacattcataaggcttctctcctgtgtgaattcttctatgttgagtaagcgttgaagatctattgaaggctttcccacattccttacactgatagggtttctctccagtgtgatttcgtatgtgtatagcaaggcccgtgtactgagtgaaggcttggccacattccttacattcatagggttttattccagtgtgagttcttacatgttgagtaaggtgagttgatctagtgaaggctttcccacattccgtacatttgtgtggttttattccagtgtgaatttgaatgtgaacattaaaggatgaggaatttctaaaggatcttccacattctttacattcaaaggacttctctcctttatgagtttttgcatgtgcagaaagttgagaaaaattagtgaaggatttcccacagttcttagtcttttcggatttctttccagtatgaactgctacacactgctttaagtgtgaggaagttgtgatggctctctcacattcctgaaattcacagagtttctctccaatgtggattcccatgtgattatcaaggcttgcaaaatacttaaagccttttccacattccttacatttgtagggttgtcttccattgagaatttcaagatgcacagcaaggcctggagttaaggtgaagacttttccacatggattaaatttggaaagttcttgtccaatagaggcttccttgtgcacactgatgctgtcttttccataacaattaccctcaaaagtgttccctccattctgagctctcatgtgtgtcttaaggcaaaactgttcactgaagacctctccacaattctcacagagtttccatccactgtagcttcttgtctgcatttgtatcccagtgaatatttgattcttcaaaaaaccctgctgaagtgatgaccgtttggttctaggttgtatttcccattctgaagttaagcagaaaaagaaatcatgggacatatcaaaggctgacatcctctgaagctgatggtgagatgtgcctcaatgctgtctttcttgatgccaagatcgcctcagggcagcttatgaatctaggtggatacaggcaatctccattcccctttgtacagggttatctgaggcccacagcggggtggactccaccacaataaaggttaaacggcactgaccatgctgagccacagccggtaaagatggcggtggcacact

SEQ ID NO: 17147 - RNA, 11650 nt, Homo sapiens
  source 1..11650: mol_type = other RNA
tcaggccaggcacagtggctcaaccctgtcatcctagcattttgggaggctgatgcagaaggataacttgaacaggatttcaagaccagcctgggcaatatagtgagacacagtctcgaccaaaaaaaaaaaaatttaaaaataaaaaaattagccgggcctggtggtacatgcctgcattcccagctactcagaaggctgaggtgagaggattgcttgagcccaggaggtcgaggctgcagtgagctatgattgcaccactgcactccagcctaggtgacatggcaagacactgtctctggaaaaaaaaaaaaaaaaaaagaacaccaccggccactgtggctcattcctgtaatcccagcactttgggaggttgaatcaggctgaatcaggggggtctcaggagttcaagaccatcctggccaacatggcaaaaccccgcctctactgaaaatacaaaaattagctgggtgtggtggtgcacacctgtaatcccaggtacttgggaggctgaggcaggagaatcacttgaacccaggaattggaggttgcagtgagctgagatcacgccactgcactccagcctgggtgacagagcgagactctgtcattcataaataaataagtttagaaaaaaaaaatgtgtctgaaagggtcttgagcatccctctgggcaaattccaggcatcatccataatgatgaatgcacaaatacaaagatacgaatgagccagagccaaccttatattcctgcagtaaatgccactgggtttactattttcttatcaagcagttggaatttatttgctaatccgttccttcctagcttccttttttccttcttttttttttttttttaaatggagtcttgctctgttgcccaggctggaatgcagtggcatgatcttggctcactgcattttttaatttttaagttttttgtagatggggggcttgctatgctgtccaggcaggtctcgaactcctgagctcaagtaatccttttgcctcctttcaaagtgttgagactccaggcataagccactttgcccagttgctactattatacttagcgcatttttttgtttgtttgttttttgagacagtcttactctgtatcccaggctggagtgcagtggtgtgatctcggttcactgtaacctcctgcctcagcctcccgagtagctaggaatacatgcacatgccaccacgcccagctatatttttttagttttagtagatacaaggtttcaccgttttagccaggatcatctcaatctgaccttgtgatccacctgcctcagcctcccaaagtgctgggattacaggcatgtgagccaccgtacctggcttacttagtgaatttgtaccaatattcattaccaatataattctgtagtttttaatgactgtactgtttttatcagtgataaaaacgatacatatatacatcttgtactgcatcataaaaagatttagcaagatttgcttcattgttaatactctgaaaggatttatggagaattaggaccaattggaccttgaaaatgtcatgtaaagatgtctggctgggcatggtggctcatgcttgtaatcccagcactttgggaggcccagaagagaggattactctagctcaggagtttgaggacagcctgggcaatggagtgagataccttctctaccaaaataaaaaagtgtgagtttaggtgctgtgttccttgttgttgttacagtgtgagccaccgtgcctggccgagactgggtaagttatgaagaaaaagaggtttaatggactcacagttccacatggctggggaggcctcaaaatcatgacagaaggtgaaggaggagcaaaggcacatcttatatggcagaaggcaagagagcctgtccaggggaacagctgcttataaaactgacagacctcatgagatttactcactgtgacaaaaacagcacacgcctattatcccagctacttggctgactgaggcatgagaattacttgaacagcatggggaaacccccccccatgattctattacctcccacctggtctctccctcgacaccatggggattatgggagctacaattcaagatgacatttgggtggggacacagccaaaccatatcagctggcaacttgcttgcagctcataacatcaactgtttctttgggccttcagtcctgctgacttccggcctcctgagtccctaagcagaggaatacgaattcaaatcttgattttctcattgcagctcatagtgggagatgcccagtctctctgtgaacattgacagaattttttttttttttttgagacagagtctcacactgtcaccaggctggagtgccgtggcgcaatatcagctcactgtaacctccacctcccaggttgaagtgattctcccatctcagcccccaagtagctgggactacaggtgagtgccaccacacccagctaatttttgtatttttagtagagatgggggttcaccatgttgcccaaaatggtctcaatctcttggcctcgtgatccaaccatctcagcctcccaaagtgctgggtttaaaggcatgagccactgtgcctggcccagaattctttactgctaacacgagtgggcctggttctggaggatttcccagtgggtcctgaagaaccacagtttattggcttgtgggcaaaggggtatgtgtatcagttggcctttactgtgtaataaacagccacaaaaattactagctgaaaacagcagctacttaattagcagaagcctcttgaggatggacttgcaaaccaaagttgtgctggtttctactggtcaaagcaaggactggctcacataaaaaggagagagattgcaccttcagagagtaatctcaagacatctgtaatctaccacagggtgtcactgggcctctgtcaaggagcctattctttctgccaccagatctgtctaatagcttgtgtgacaatgcacttccttctgggtctctctccaagtgtagtaagtgtatatgggaatcactttattcaaacagtgtagtgcacttagttagaaagaaaaggtattaaggaagacttatatttaaaattgttatttatggtaacaacgaaaagtaacatacaaatttcaaacatcaagaataaaataaattaaaggtatgatcaatacacatcagtacaaagaggggaacacaatgaaacaaacaaaaaaaattagatgctagaaattaatccaaattattactaattaaatgtcaggcactaaatgtgcaacataaaaggattgttaattggtattattcaagtattttttctttttttttttttttttgtgacagagtttcactcttgttgcccaggctgcagtgcaatggcgtgatctcggctcactgcaacctctgcctcccgggttcaaatgattctcctgcctcagcctcccaagtagctggcattacaggcatgcaccactaggcacagctaattttgtatttttagtagagatggggtttctcagtgttggtcaggctggtctcgaactcccgacctcaggtgatcacctgccttggcctcccaaagtgctgtgattacagacatcagccactatgcccagcggtatacagattttttaaaactccagctaaagtatgtataaaaagacacatttttttaaaaagcatacagaaagactaagaagtagaggaaaatcaagctgatgtaactatataaatatctaacagaattagtggaacagaaaacatgcaagaaatagtgtagatttttcaagcgaaatatctgaaagaattcataaacctgggtactctctaccaagattaacacaagcaaagggaaagaatgcacaattaataagttattccagaatgcaaaaggagactgaagttatacaaccagcaaaaatgaaaaatataaaaagtataaatttttgctacacatttggaaataaaaacatgcctagaagaatattctcaaaatacttatgcaagccttagttgtctttttttttttttttttatgagatggagttttgctcttgtcacccaggctggagtgcagtggcaagaactcaactcactgcaaccttcgcctcccagattcaagcaattctcctgcctcagcctcccaagcggctgggattacaggcgcccgccaactcacctggctaattttattttttgaatttttagtagagacaaaagtttcaccgcattggccaggctggtctcgaactcctgacctcaggtgaccccctgccttgacctcccaaagtgctgtgattaaagccgtgaagcaccgtgcccaacctagttgtctttttttttttttttgagacggattctcgctctgtcgtcaggctggagtgcagtggtgtgatctaggctcattgaaacctccacttcaggggttcaagagattctcctgcctcagcctcctgagtagctgggattacaggggcacaataccgtgcccagctaatttttgtatttttagtaaagacggggtttcaacatgttggccaggatggtcttgatctcttgacctcatgatctgcctgcctcagcctcccaaagtggtgggattacaggcatgagccaccactcccagcctgataactgttttatttatttatttttatttttttggagatatggggtctgtgttgcccagactgatcttgaactcctggcctcaaggaatccttctgactgagcttcccagtgtgctgggattaaaagtgtgagccactatgaccagccagaagagataattttaactttttaaaatattttgcagtattggccgggcacagtggcttgtgcctgtaatcccagtactttgggagtatgaggcatgcagatcacctgaggtcaggagtttgagaccagcctggccaacttgatgaaaccgtctctactaaaaatacaaaaatcagccaggcaaggtggaggctgtctgtaatctcagctactcgggaggctgaggcaggagaaccactggaacccaggaggtggaatttgcagtaagttgagatcacaccattgcactccagcctgggcaacgagtgaaacactaactcaaaaacaaagaaacaaacaccaactcaaaaacaaagaaacaaaccaaaaaaatgaaaatatcttgtagtatttttaaatagagatgtggtttcgctatgttgcccaggctggtttgaactccttggctcaagggatctttttgcctcagcctccaaaagtgctgggattacaggcctgagccactattcccaacctagatgactcttatagattaagaatttagaaatagtaggaacatgccccactacagtatatgacagtcattatatacaaatatcattaagggacaattttttaaaaatcacaatgttattcaaacatagctccataacatattagtaaaggtcatgaagtatttttaagtgatccattatgtcacagtcgagcttatccaggaatacaaggttgatgtaacattggaaaagcaataaatacaaataccacatttatttaatttaatttatttatttttgacagagtcgcaccctgtcacccagcatggagtgcagtggtgcaatcttggctcaatgcaacctccacctcccaggttcaagtgattctcctgcttcagcctcccaagtagctgggattacaggtgcacatcaccacacccagctaatttttgtattgttagtagagatggggtttcaccatgttggctgggctggtctcgaactcttgacctcaaatgatctgcccacccccacctcccaaattgctgggattacaggcataagcccccacacccagcctgaccacatttgttttagaaaagcgcctttccatgcattcacttcttcaagttttttttttgttttgtttttgtttttttttttgagatggggtcttgctatgttgcctaagctggtctagaacccctgggctcaggccaccctcccaagtagctaaaactataggcatgcatcaccacatcatttcattgaagtatttattaggtaccatcatgagctaggtgcagttctaggtattgagttttatcagtaaataaacatgatcatcacagaggatgtgaaggaagcatttaataaattcaagaggaattcagcctcataaactatgaaatattgggaaataattcatcatgtaaaaactggatataaagaaaaaacttttcctgcaggacattgttgcaggaagtcagggaccccaaacggggggactggctgaagccatggcagaaaaacatggattgtgaaggtttcatggacatttattagttccccaaattaatacttttataatttcttatgcctgtctttactgcaatctctaaacataaattgtaaagatttcatggacacttatcacttccccagtcaatacccttgtgatttcctatgcctgtctttactttaatctctcaatcctgtcagctgaggaggatgtatattacctcaggaccctgtaataattgcattaactgcacaaattatacagcatgtgtgtttgagcaatatgaaatctgggcaccttgaaaaaagaacaggataacagcaatgtttaggaaacaagagagataaccttaaattctgaccgccggtgagccaggtggaacaaagccacatttctcttctttcacaagcaaatgggagaaatatcactgaattctttttctcagcaaggaacatccttgagaaagagaatgcacacctgggagtgggtctctgaactggcccccctgggtgtagccatctcttatggtcgagactgcaggggtgaaatagaccccagtctcccatagcactcccaggcttattaggaagaggaaattcccacctaataaattttagtcagaccagttgatctcaaaaccgtctcctgataagatgttatcaatgacaatggtgcccaaaacttcattagcaattttaatttcaccttggtcctgtgatctcgccctgcctccacttgccttgtgatattctattaccttgtaaagtacttgatgtctgtgacccacacctatttgcacactccctccccttttgaaaatccctaataaaaacttgctggtttttgcggcttgtggggcatcacggaacctaccgacatgtgatgtctgccccggacacccagctttaaaatttctctcttttgtactctgtccctttatttctcaagttggctgacacttagggaaaatagaaaagaacctatgtgaatatcggggctggttccctgacaggacataacctcttcaaaaaataaaaaagaaataaaagcctacagccaaaccaacaaaatagagtgcatatctcaccagaactgcaaagacaagtatgctggtattactacttttagttggtgttgtgcagcgggttaaaatcagtccagtaaagcaagaaaatatttagagagagcttcatcatcatacgaattttgggggtcattgttcagtccaaagtacttaatatgattcttttctctttccacatagagaatcagataatctataaataatgactcttactgttccactttaggagttaggtatacatacatatgtgtatatatatgtatatatatatacacatacacacacacacacacacacacacagtgaccccccaaatttcatatgaagttccaaacctcaatgtgactgtatgtgaaaagagaagggggcggggaggggggagaccgaccgacctatttgttggtctccatcgtgtgaaaacatgaggaagtgggcacttacatgccaggaagagagctctcactagaggttgaccatgctggcactctgatctcagacttccagcctccagatatgtgagaatataaatttgtgttttgggccagatacggtggctcaggcctgtaatcccagcactttgggaggccaaggcaggtggatcaccaaaggtcagatctgaccaacatggagatcagcctaaccaacatggagaaaccctgtctctactaaaaatacaaacttagctaaggtttgtggtgcatgccaataatcccagctactgagggtgaggcaggagaatcactggaactcaggaggtggaggttgcggtgagccaagatcataccattgcactccagcctgggcaacaagagcaaaactccatctcaaaaaaaaaaaaaaaaaaaaaaaaaaaatcctgtgtttttaacctcattgatttaaaattaaattaatttctaagccatttggtctgcggtattctcttatggttgtctgagctgactaaggcagatattggtactgagaagtgaggtactgcaattaaaaacaaacaaaaaaactaaaaatgtgaagcagctttgaaactgacaaatgagtagaggctggaaaaattctgatgtgcaagctggaaataaggttggtaagggttattctggtgaggtgtcattggggaatgaggaacatgctattgggaaatgaagaaaagacaacccttgatataaagtggtgaagaacttggcagaactgtattctagcattttacggaaggtagagcttgagacagataaaatggtatgtatcactaagatctgtaattaaagtgttaaaggacacaggaagcttcattattcctgagtgcttacaggaaaatgtgctgggaacaggccccccaaatctggccataaacaggcaatgagaaactggccataaacaaaatctctgcagcactgtgacatgctcgtgatggctatgacgcccatgctggaggctgctggtttaccagaatgagggcaagcaacacctggcccacccagggcagaaaactggaaaactgctcaaggcattcctaaaccacaaacaatagcatgagtgatttgtgccttaaggacatattcctgttgcagataacaagccagagcctgtccctttctttctcataaggaatacttatagctgatctacaatctataggaataatgtttatcacaggcttactgtcaataaatatgtgggtcaaactctgttcaagctcagctctgaaggctgtgagccccgattcccactctgcactatatttctgtgtctttgtcttaattcctctagagccactgggttagggtctccacgacccagctggtctcggcaaaaatgcaaaaggagacctgaattgcagaagaaattgttaaggaaaaaggaaccagaacttggagatttggaaaattctcagcctatccatactgcaaaaattagaaaacttgtactgaagagaatcctcaaagtgtggctgaacaatcatttgataaagagatcatgagtgggattcatggactatatcagccatcttaacagaagtgagaagagagactggattatactataagagacactgccacttacattgtgccacctaaaatggacagagaagacagaacagaacagtcaaggttgtcacacttcttattttacaagaaggggacatagaaataatcagctgtgaaagggcactggcagttatggatggtttcactcctgacatgctctgcaggatccatgggaacagaagagaaccttggaggagcatctttttaacaatccacctctggggcctacatcatcttggcttctggtaaattttgacatgaatgtgccacactggcagccactaaccaacaggggctgggatcaatctgcatgatttatctcgtacagaacttgttaatgctatgatcttaggaatctaatcaccaaggtgaggcagcctgcagtactgacctcaccatccatgacccttcttcacagatgcccagactcaggtaaccatgatgttgtattcagaacctgtaggtttaatttcagaccctcgggatgcatctaaggccaatctgtgagccattacaacctccaaaaggcatttaggactaatctgatgatctttgcactgccaataattaaagatggcaaccaatgggctaaatggtaacaacactcatatccttacattcatagtatttctccccagtgtgaattctttcatgcatacttaggcatgaggaaagagcaaatgctttcccaaattctttacatacaaaaggtttctctctggtaggagttcacaggtggggtgaggaatacagaaattctttcccacatatcttgcatttacctttctccactgtgagttttcaaatgtttactacgatgggaagaagtaatgaaggtcttcccacattcaacacattcataaggcttctctcctgtgtgaattcttctatgttgagtaagcgttgaagatctattgaaggctttcccacattccttacactgatagggtttctctccagtgtgatttcgtatgtgtatagcaaggcccgtgtactgagtgaaggcttggccacattccttacattcatagggttttattccagtgtgagttcttacatgttgagtaaggtgagttgatctagtgaaggctttcccacattccgtacatttgtgtggttttattccagtgtgaatttgaatgtgaacattaaaggatgaggaatttctaaaggatcttccacattctttacattcaaaggacttctctcctttatgagtttttgcatgtgcagaaagttgagaaaaattagtgaaggatttcccacagttcttagtcttttcggatttctttccagtatgaactgctacacactgctttaagtgtgaggaagttgtgatggctctctcacattcctgaaattcacagagtttctctccaatgtggattcccatgtgattatcaaggcttgcaaaatacttaaagccttttccacattccttacatttgtagggttgtcttccattgagaatttcaagatgcacagcaaggcctggagttaaggtgaagacttttccacatggattaaatttggaaagttcttgtccaatagaggcttccttgtgcacactgatgctgtcttttccataacaattaccctcaaaagtgttccctccattctgagctctcatgtgtgtcttaaggcaaaactgttcactgaagacctctccacaattctcacagagtttccatccactgtagcttcttgtctgcatttgtatcccagtgaatatttgattcttcaaaaaaccctgctgaagtgatgaccgtttggttctaggttgtatttcccattctgaagttaagcagaaaaagaaatccacagaggccaggttcatgtagttctccagcatcacatctctgtagaggtatttctgagttgtgtccagtaaagcccactcctctggggtgaactccacagccacatcatcaaacgtcactgaatcctggtaagaatttgaccggtggtcctctaccatcgttcctatctttgtcttttcttcaaaaggacagattggttccctgggaaaaaacccatgggacatatcaaaggctgacatcctctgaagctgatggtgagatgtgcctcaatgctgtctttcttgatgccaagatcgcctcagggcagcttatgaatcacagcggggtggactccaccacaataaaggttaaacggcactgaccatgctgagccacagccggtaaagatggcggtggcacact

SEQ ID NO: 17148 - RNA, 11703 nt, Homo sapiens
  source 1..11703: mol_type = other RNA
tcaggccaggcacagtggctcaaccctgtcatcctagcattttgggaggctgatgcagaaggataacttgaacaggatttcaagaccagcctgggcaatatagtgagacacagtctcgaccaaaaaaaaaaaaatttaaaaataaaaaaattagccgggcctggtggtacatgcctgcattcccagctactcagaaggctgaggtgagaggattgcttgagcccaggaggtcgaggctgcagtgagctatgattgcaccactgcactccagcctaggtgacatggcaagacactgtctctggaaaaaaaaaaaaaaaaaaagaacaccaccggccactgtggctcattcctgtaatcccagcactttgggaggttgaatcaggctgaatcaggggggtctcaggagttcaagaccatcctggccaacatggcaaaaccccgcctctactgaaaatacaaaaattagctgggtgtggtggtgcacacctgtaatcccaggtacttgggaggctgaggcaggagaatcacttgaacccaggaattggaggttgcagtgagctgagatcacgccactgcactccagcctgggtgacagagcgagactctgtcattcataaataaataagtttagaaaaaaaaaatgtgtctgaaagggtcttgagcatccctctgggcaaattccaggcatcatccataatgatgaatgcacaaatacaaagatacgaatgagccagagccaaccttatattcctgcagtaaatgccactgggtttactattttcttatcaagcagttggaatttatttgctaatccgttccttcctagcttccttttttccttcttttttttttttttttaaatggagtcttgctctgttgcccaggctggaatgcagtggcatgatcttggctcactgcattttttaatttttaagttttttgtagatggggggcttgctatgctgtccaggcaggtctcgaactcctgagctcaagtaatccttttgcctcctttcaaagtgttgagactccaggcataagccactttgcccagttgctactattatacttagcgcatttttttgtttgtttgttttttgagacagtcttactctgtatcccaggctggagtgcagtggtgtgatctcggttcactgtaacctcctgcctcagcctcccgagtagctaggaatacatgcacatgccaccacgcccagctatatttttttagttttagtagatacaaggtttcaccgttttagccaggatcatctcaatctgaccttgtgatccacctgcctcagcctcccaaagtgctgggattacaggcatgtgagccaccgtacctggcttacttagtgaatttgtaccaatattcattaccaatataattctgtagtttttaatgactgtactgtttttatcagtgataaaaacgatacatatatacatcttgtactgcatcataaaaagatttagcaagatttgcttcattgttaatactctgaaaggatttatggagaattaggaccaattggaccttgaaaatgtcatgtaaagatgtctggctgggcatggtggctcatgcttgtaatcccagcactttgggaggcccagaagagaggattactctagctcaggagtttgaggacagcctgggcaatggagtgagataccttctctaccaaaataaaaaagtgtgagtttaggtgctgtgttccttgttgttgttacagtgtgagccaccgtgcctggccgagactgggtaagttatgaagaaaaagaggtttaatggactcacagttccacatggctggggaggcctcaaaatcatgacagaaggtgaaggaggagcaaaggcacatcttatatggcagaaggcaagagagcctgtccaggggaacagctgcttataaaactgacagacctcatgagatttactcactgtgacaaaaacagcacacgcctattatcccagctacttggctgactgaggcatgagaattacttgaacagcatggggaaacccccccccatgattctattacctcccacctggtctctccctcgacaccatggggattatgggagctacaattcaagatgacatttgggtggggacacagccaaaccatatcagctggcaacttgcttgcagctcataacatcaactgtttctttgggccttcagtcctgctgacttccggcctcctgagtccctaagcagaggaatacgaattcaaatcttgattttctcattgcagctcatagtgggagatgcccagtctctctgtgaacattgacagaattttttttttttttttgagacagagtctcacactgtcaccaggctggagtgccgtggcgcaatatcagctcactgtaacctccacctcccaggttgaagtgattctcccatctcagcccccaagtagctgggactacaggtgagtgccaccacacccagctaatttttgtatttttagtagagatgggggttcaccatgttgcccaaaatggtctcaatctcttggcctcgtgatccaaccatctcagcctcccaaagtgctgggtttaaaggcatgagccactgtgcctggcccagaattctttactgctaacacgagtgggcctggttctggaggatttcccagtgggtcctgaagaaccacagtttattggcttgtgggcaaaggggtatgtgtatcagttggcctttactgtgtaataaacagccacaaaaattactagctgaaaacagcagctacttaattagcagaagcctcttgaggatggacttgcaaaccaaagttgtgctggtttctactggtcaaagcaaggactggctcacataaaaaggagagagattgcaccttcagagagtaatctcaagacatctgtaatctaccacagggtgtcactgggcctctgtcaaggagcctattctttctgccaccagatctgtctaatagcttgtgtgacaatgcacttccttctgggtctctctccaagtgtagtaagtgtatatgggaatcactttattcaaacagtgtagtgcacttagttagaaagaaaaggtattaaggaagacttatatttaaaattgttatttatggtaacaacgaaaagtaacatacaaatttcaaacatcaagaataaaataaattaaaggtatgatcaatacacatcagtacaaagaggggaacacaatgaaacaaacaaaaaaaattagatgctagaaattaatccaaattattactaattaaatgtcaggcactaaatgtgcaacataaaaggattgttaattggtattattcaagtattttttctttttttttttttttttgtgacagagtttcactcttgttgcccaggctgcagtgcaatggcgtgatctcggctcactgcaacctctgcctcccgggttcaaatgattctcctgcctcagcctcccaagtagctggcattacaggcatgcaccactaggcacagctaattttgtatttttagtagagatggggtttctcagtgttggtcaggctggtctcgaactcccgacctcaggtgatcacctgccttggcctcccaaagtgctgtgattacagacatcagccactatgcccagcggtatacagattttttaaaactccagctaaagtatgtataaaaagacacatttttttaaaaagcatacagaaagactaagaagtagaggaaaatcaagctgatgtaactatataaatatctaacagaattagtggaacagaaaacatgcaagaaatagtgtagatttttcaagcgaaatatctgaaagaattcataaacctgggtactctctaccaagattaacacaagcaaagggaaagaatgcacaattaataagttattccagaatgcaaaaggagactgaagttatacaaccagcaaaaatgaaaaatataaaaagtataaatttttgctacacatttggaaataaaaacatgcctagaagaatattctcaaaatacttatgcaagccttagttgtctttttttttttttttttatgagatggagttttgctcttgtcacccaggctggagtgcagtggcaagaactcaactcactgcaaccttcgcctcccagattcaagcaattctcctgcctcagcctcccaagcggctgggattacaggcgcccgccaactcacctggctaattttattttttgaatttttagtagagacaaaagtttcaccgcattggccaggctggtctcgaactcctgacctcaggtgaccccctgccttgacctcccaaagtgctgtgattaaagccgtgaagcaccgtgcccaacctagttgtctttttttttttttttgagacggattctcgctctgtcgtcaggctggagtgcagtggtgtgatctaggctcattgaaacctccacttcaggggttcaagagattctcctgcctcagcctcctgagtagctgggattacaggggcacaataccgtgcccagctaatttttgtatttttagtaaagacggggtttcaacatgttggccaggatggtcttgatctcttgacctcatgatctgcctgcctcagcctcccaaagtggtgggattacaggcatgagccaccactcccagcctgataactgttttatttatttatttttatttttttggagatatggggtctgtgttgcccagactgatcttgaactcctggcctcaaggaatccttctgactgagcttcccagtgtgctgggattaaaagtgtgagccactatgaccagccagaagagataattttaactttttaaaatattttgcagtattggccgggcacagtggcttgtgcctgtaatcccagtactttgggagtatgaggcatgcagatcacctgaggtcaggagtttgagaccagcctggccaacttgatgaaaccgtctctactaaaaatacaaaaatcagccaggcaaggtggaggctgtctgtaatctcagctactcgggaggctgaggcaggagaaccactggaacccaggaggtggaatttgcagtaagttgagatcacaccattgcactccagcctgggcaacgagtgaaacactaactcaaaaacaaagaaacaaacaccaactcaaaaacaaagaaacaaaccaaaaaaatgaaaatatcttgtagtatttttaaatagagatgtggtttcgctatgttgcccaggctggtttgaactccttggctcaagggatctttttgcctcagcctccaaaagtgctgggattacaggcctgagccactattcccaacctagatgactcttatagattaagaatttagaaatagtaggaacatgccccactacagtatatgacagtcattatatacaaatatcattaagggacaattttttaaaaatcacaatgttattcaaacatagctccataacatattagtaaaggtcatgaagtatttttaagtgatccattatgtcacagtcgagcttatccaggaatacaaggttgatgtaacattggaaaagcaataaatacaaataccacatttatttaatttaatttatttatttttgacagagtcgcaccctgtcacccagcatggagtgcagtggtgcaatcttggctcaatgcaacctccacctcccaggttcaagtgattctcctgcttcagcctcccaagtagctgggattacaggtgcacatcaccacacccagctaatttttgtattgttagtagagatggggtttcaccatgttggctgggctggtctcgaactcttgacctcaaatgatctgcccacccccacctcccaaattgctgggattacaggcataagcccccacacccagcctgaccacatttgttttagaaaagcgcctttccatgcattcacttcttcaagttttttttttgttttgtttttgtttttttttttgagatggggtcttgctatgttgcctaagctggtctagaacccctgggctcaggccaccctcccaagtagctaaaactataggcatgcatcaccacatcatttcattgaagtatttattaggtaccatcatgagctaggtgcagttctaggtattgagttttatcagtaaataaacatgatcatcacagaggatgtgaaggaagcatttaataaattcaagaggaattcagcctcataaactatgaaatattgggaaataattcatcatgtaaaaactggatataaagaaaaaacttttcctgcaggacattgttgcaggaagtcagggaccccaaacggggggactggctgaagccatggcagaaaaacatggattgtgaaggtttcatggacatttattagttccccaaattaatacttttataatttcttatgcctgtctttactgcaatctctaaacataaattgtaaagatttcatggacacttatcacttccccagtcaatacccttgtgatttcctatgcctgtctttactttaatctctcaatcctgtcagctgaggaggatgtatattacctcaggaccctgtaataattgcattaactgcacaaattatacagcatgtgtgtttgagcaatatgaaatctgggcaccttgaaaaaagaacaggataacagcaatgtttaggaaacaagagagataaccttaaattctgaccgccggtgagccaggtggaacaaagccacatttctcttctttcacaagcaaatgggagaaatatcactgaattctttttctcagcaaggaacatccttgagaaagagaatgcacacctgggagtgggtctctgaactggcccccctgggtgtagccatctcttatggtcgagactgcaggggtgaaatagaccccagtctcccatagcactcccaggcttattaggaagaggaaattcccacctaataaattttagtcagaccagttgatctcaaaaccgtctcctgataagatgttatcaatgacaatggtgcccaaaacttcattagcaattttaatttcaccttggtcctgtgatctcgccctgcctccacttgccttgtgatattctattaccttgtaaagtacttgatgtctgtgacccacacctatttgcacactccctccccttttgaaaatccctaataaaaacttgctggtttttgcggcttgtggggcatcacggaacctaccgacatgtgatgtctgccccggacacccagctttaaaatttctctcttttgtactctgtccctttatttctcaagttggctgacacttagggaaaatagaaaagaacctatgtgaatatcggggctggttccctgacaggacataacctcttcaaaaaataaaaaagaaataaaagcctacagccaaaccaacaaaatagagtgcatatctcaccagaactgcaaagacaagtatgctggtattactacttttagttggtgttgtgcagcgggttaaaatcagtccagtaaagcaagaaaatatttagagagagcttcatcatcatacgaattttgggggtcattgttcagtccaaagtacttaatatgattcttttctctttccacatagagaatcagataatctataaataatgactcttactgttccactttaggagttaggtatacatacatatgtgtatatatatgtatatatatatacacatacacacacacacacacacacacacagtgaccccccaaatttcatatgaagttccaaacctcaatgtgactgtatgtgaaaagagaagggggcggggaggggggagaccgaccgacctatttgttggtctccatcgtgtgaaaacatgaggaagtgggcacttacatgccaggaagagagctctcactagaggttgaccatgctggcactctgatctcagacttccagcctccagatatgtgagaatataaatttgtgttttgggccagatacggtggctcaggcctgtaatcccagcactttgggaggccaaggcaggtggatcaccaaaggtcagatctgaccaacatggagatcagcctaaccaacatggagaaaccctgtctctactaaaaatacaaacttagctaaggtttgtggtgcatgccaataatcccagctactgagggtgaggcaggagaatcactggaactcaggaggtggaggttgcggtgagccaagatcataccattgcactccagcctgggcaacaagagcaaaactccatctcaaaaaaaaaaaaaaaaaaaaaaaaaaaatcctgtgtttttaacctcattgatttaaaattaaattaatttctaagccatttggtctgcggtattctcttatggttgtctgagctgactaaggcagatattggtactgagaagtgaggtactgcaattaaaaacaaacaaaaaaactaaaaatgtgaagcagctttgaaactgacaaatgagtagaggctggaaaaattctgatgtgcaagctggaaataaggttggtaagggttattctggtgaggtgtcattggggaatgaggaacatgctattgggaaatgaagaaaagacaacccttgatataaagtggtgaagaacttggcagaactgtattctagcattttacggaaggtagagcttgagacagataaaatggtatgtatcactaagatctgtaattaaagtgttaaaggacacaggaagcttcattattcctgagtgcttacaggaaaatgtgctgggaacaggccccccaaatctggccataaacaggcaatgagaaactggccataaacaaaatctctgcagcactgtgacatgctcgtgatggctatgacgcccatgctggaggctgctggtttaccagaatgagggcaagcaacacctggcccacccagggcagaaaactggaaaactgctcaaggcattcctaaaccacaaacaatagcatgagtgatttgtgccttaaggacatattcctgttgcagataacaagccagagcctgtccctttctttctcataaggaatacttatagctgatctacaatctataggaataatgtttatcacaggcttactgtcaataaatatgtgggtcaaactctgttcaagctcagctctgaaggctgtgagccccgattcccactctgcactatatttctgtgtctttgtcttaattcctctagagccactgggttagggtctccacgacccagctggtctcggcaaaaatgcaaaaggagacctgaattgcagaagaaattgttaaggaaaaaggaaccagaacttggagatttggaaaattctcagcctatccatactgcaaaaattagaaaacttgtactgaagagaatcctcaaagtgtggctgaacaatcatttgataaagagatcatgagtgggattcatggactatatcagccatcttaacagaagtgagaagagagactggattatactataagagacactgccacttacattgtgccacctaaaatggacagagaagacagaacagaacagtcaaggttgtcacacttcttattttacaagaaggggacatagaaataatcagctgtgaaagggcactggcagttatggatggtttcactcctgacatgctctgcaggatccatgggaacagaagagaaccttggaggagcatctttttaacaatccacctctggggcctacatcatcttggcttctggtaaattttgacatgaatgtgccacactggcagccactaaccaacaggggctgggatcaatctgcatgatttatctcgtacagaacttgttaatgctatgatcttaggaatctaatcaccaaggtgaggcagcctgcagtactgacctcaccatccatgacccttcttcacagatgcccagactcaggtaaccatgatgttgtattcagaacctgtaggtttaatttcagaccctcgggatgcatctaaggccaatctgtgagccattacaacctccaaaaggcatttaggactaatctgatgatctttgcactgccaataattaaagatggcaaccaatgggctaaatggtaacaacactcatatccttacattcatagtatttctccccagtgtgaattctttcatgcatacttaggcatgaggaaagagcaaatgctttcccaaattctttacatacaaaaggtttctctctggtaggagttcacaggtggggtgaggaatacagaaattctttcccacatatcttgcatttacctttctccactgtgagttttcaaatgtttactacgatgggaagaagtaatgaaggtcttcccacattcaacacattcataaggcttctctcctgtgtgaattcttctatgttgagtaagcgttgaagatctattgaaggctttcccacattccttacactgatagggtttctctccagtgtgatttcgtatgtgtatagcaaggcccgtgtactgagtgaaggcttggccacattccttacattcatagggttttattccagtgtgagttcttacatgttgagtaaggtgagttgatctagtgaaggctttcccacattccgtacatttgtgtggttttattccagtgtgaatttgaatgtgaacattaaaggatgaggaatttctaaaggatcttccacattctttacattcaaaggacttctctcctttatgagtttttgcatgtgcagaaagttgagaaaaattagtgaaggatttcccacagttcttagtcttttcggatttctttccagtatgaactgctacacactgctttaagtgtgaggaagttgtgatggctctctcacattcctgaaattcacagagtttctctccaatgtggattcccatgtgattatcaaggcttgcaaaatacttaaagccttttccacattccttacatttgtagggttgtcttccattgagaatttcaagatgcacagcaaggcctggagttaaggtgaagacttttccacatggattaaatttggaaagttcttgtccaatagaggcttccttgtgcacactgatgctgtcttttccataacaattaccctcaaaagtgttccctccattctgagctctcatgtgtgtcttaaggcaaaactgttcactgaagacctctccacaattctcacagagtttccatccactgtagcttcttgtctgcatttgtatcccagtgaatatttgattcttcaaaaaaccctgctgaagtgatgaccgtttggttctaggttgtatttcccattctgaagttaagcagaaaaagaaatccacagaggccaggttcatgtagttctccagcatcacatctctgtagaggtatttctgagttgtgtccagtaaagcccactcctctggggtgaactccacagccacatcatcaaacgtcactgaatcctggtaagaatttgaccggtggtcctctaccatcgttcctatctttgtcttttcttcaaaaggacagattggttccctgggaaaaaacccatgggacatatcaaaggctgacatcctctgaagctgatggtgagatgtgcctcaatgctgtctttcttgatgccaagatcgcctcagggcagcttatgaatctaggtggatacaggcaatctccattcccctttgtacagggttatctgaggcccacagcggggtggactccaccacaataaaggttaaacggcactgaccatgctgagccacagccggtaaagatggcggtggcacact

SEQ ID NO: 17149 - RNA, 33 nt, Homo sapiens
  source 1..33: mol_type = other RNA
tcaggccaggcacagtggctcaagcctgtaatc

SEQ ID NO: 17150 - RNA, 66 nt, Homo sapiens
  source 1..66: mol_type = other RNA
tcaggccaggcacagtggctcaagcctgtaatcccaagctctttgggaggacgaggtaggaagact

SEQ ID NO: 17151 - RNA, 984 nt, Homo sapiens
  source 1..984: mol_type = other RNA
tcaggccaggcacagtggctcaagcctgtaatcccagcactttaggaggccaaggtgggcagatcacttgaagccaggagttggagatcagcctgggcaacatagtgaaaccccatctctacaaaaatacaaaaattatctgggattggtggcacatgcctgtaatcccagctacttgggaggctaaggcacgagaatcacttgaacccaggaggcagaggttacagtgagctgagatcacaccactgcactccagtatgagcaacagagcaagactgtcaaaaaaaaaaaaaaagaagaaagaaaaaagaaggaaagaagaaagaaagaaagaaagaaagaaagaaagaaagaaagaaagaaagaaagaaagaaagaaagagaaagaaagaaaaagaaattcacagccaaactggtatgcattgagtctctggaggctgaagacaaaaaagtttttaatcttatttgtgccatttaaatatttataagatttaagaaaaggattttccttttcttttttaatccgtgactgtaagggaccaatttggaagtcagaaaatttagagaaaattgtgctattgacgtgctgactttggcaaatgagccttagattcctctttgtatacctgccttcttgcttcagttaattggaagtacatgcaatgacagaaataaaatctctggctctttgaaaagtaggatgccatgggagaaagactttttaataattttctctattatgaagggcttaggtctggaggatagaggcaaaaactgcaaatcccccttgttgtgcattcactcacattcactaccaaggctcccattttgatcattccccttgaccagaaaatggagagtgcaaatgtgtgttcttagatgcaggaaaaataaacatccaccagcttcagcttcagaaacacgcatgaggagccttcagtttgcaaagcaacagcctcacgtaatagacgacgatgtgtacat

SEQ ID NO: 17152 - RNA, 481 nt, Homo sapiens
  source 1..481: mol_type = other RNA
tcaggccaggcacagtggctcaagcctgtaatcccagcactttgggaggctgaggcgggcagatcacgaagtcaggagatcgagaccatcctggctaacacagtcgaatctcttgtctctgctctttgcagcattaatttctggttcgtgtttagtgagccaggaagcagtcatgggtttggaaaggtgatgtctcaactcgggttttaaatagcattctttttcaacactgttaggtgctgtgaacacagagctgtctctttgtgttaaagtggggacaagcaaagtagcagaggagagagtcgaccgaggcgggagggaggtggcaggtggaatgaaatatcgggcagtttcatgtgcggagctgatgtcgccggcataacaagaaagggttgcacagaacaaatctctattgttccctgtcatctttaaatgagtgtcaaagtaggcaggggggctttgaccgttaaccgcacaattt

SEQ ID NO: 17153 - RNA, 10021 nt, Homo sapiens
  source 1..10021: mol_type = other RNA
tcaggccaggcacagtggctcaatgcctgtaatcccagcactttgggaggccgaggcaggtggaccacatgaggtcaggaattcgagaccagcctggccaacatggcaaaaccccatctccactaaaaatgaaaaaattagctgaaataacacagctacttgggaggctaaagcaggagaatcacttgaacccaggaggtggaggctgcagtgagccaagatcacgccattgcactccaccctgggcaacagagcaagacgccatctcaaaaaaacaaacaaaaaatcacaatcagtgagattaatgtttaatgaacatactgttattttttatttttttaagagacaagtctccatctgtctcctaagcagagtgtagtggcgcaatcatagctcattgtaacattggactcctgggctcaagtgatcctcccacctcagtctcccatgcatgccaccacaattttttggatacagggtgtcattatgttgcccaggctgatctcaaactcctggcctcaagtgatcctccttccttggcctcccaaagtgttgagattacaggcgtgagtcacagagcctggcccaggatgttattttaaaattgtctttttgtcttctaaatcaacaagaacttgatagttgctttcaatgccaatcaacatcctttactactgtatacacaatgtatttatttgacatttgaaaggagatacggctgggcgcggtggctcacgcctgtaatcccagcactttgggaggccgaggcgggcggatcacaaggtcaggagatcgagaccatcttggctaacacggtgaaaccccgtctctactaaaaatacaaaaaattagccaggcgcggtggcgggcgcctgtagtcccagctactcgggaggctgaggcaggagaatggcgtgaacctgggaggcggagcttgcagtgagccgagattgcgccactgcaatccggcctgggctaaacagcgggactccgtctcaaaaaaaaaaaaaaaaaaagaaaggagatacaaaaggatgttacaacctgctatggcaagaagatacaaaggaacatattggtatgaacagaatacctcagagttgagtgtataaaaaaggcttaattcaccagatgcagtggctcgcacctgtaatcccagcattttgagaggtcaaggtcaagacacgaggattgcttgagcccaggagttcaaggccagcctgggcaacatagcaggactctgcctctaaaaaaagtatatatatatatataatgtacacacacatacatacataaacacatatgtattatatatatatatgtaatatatgtatattatatataatatatatattagccaggcatggtggcaacaggcctgtgttcccagctactcaggaggctgcagtgagtcatgtttgcgccactatactccagcctgggtgacagaatgagaccctgtctcagcaaaaaacaaataaaaaacttcaaggtggagtaggggttaattcaaggctacctaagctggatttggggtgattatggtcgagtggatgcaaacagaatattaaacttccattcattaaaagtgcttactacctgccagaccccatactaggctctatagatttattgtctctaaggtcactaggcgagtaagtaccagatctgtgactttgaacttcccactacaataagcttatgaactttgtttaagcaaaaaaggtttgaaaagtgaaaagcaagcacccatttcatagtgttctaaaagtctaaaataatccagtagaacatcagagataaaatccaaaaagcaagtttttcccccaatatttaaatcagggaagcaacatgatggtatctgtaaactataactgaaccaaaaataggaccaaacgtagtgaaatccatttagggagatattactgtgatcttgaaggaaggcctacttaatacaggacagtgggctggggaggtgtgaaccaaaaatagacacaggcaaaagcgctaaaatttaaccctgagaaataaatgaaattcacctacaaaataaatggaataaatttaaaaggtgaaattttgggcttggcgtggtggcttacacctgtaatctcagcactttgggaagccaagacgggcagatcacttgaccccaggagtttgagaccagcctgggcaacatggtgaaactgtctctacaaaaaatacaaaaattaggccgggcacggtggctcacgcctgtaatcccagtactttgggaggccgaggtgggcggatcatgaggtcaggagttcgagaccagcctggacaacatgctgaaaccccatctctactaaaaatacaaaaaaaattagccaggtgtggttggcgagcacctataattccagctactcaggaggctgaggcagaattgcttgaacctgggaggtggaggttgcaatgagccgagattgcaccactgcactccagtctgggtgaaagagcaagactctgtctcagggcgggtggcagcggggtcgggggaggtggggggaaggttagctggacctggtggcttgcacctgtggtccccagctacttgggaggctgaggtgggaggattgcttgagcccaggaggttgaggctgtagtgagtcatgtttgcagcactgcattccagcctgggcgacagagcaagaccgcatctcaaaacaaaacaaacaaaaggtgaaattttggaattaggaaagatgctatttttataaattggctttaagctgttggctggacatctaagttgtagcattctgaaggcagcagagatgtgggattgtaggactgaaacatgaaaatgcctatcgaattttttttaaagtctttaaaggagagctttaaaggaaagcaatacgaattcaagtatgtttcagtaccactcctctctctaaagacaatcaactatggttttcattcaaaatactattactctaacgttaaatatttgagtacagcaatcatttcagatgcattatgaataagttactgaacacgcctcccatctgcttgctttacggttttattttgcctttcgtttgttagctcattttataatttgttacttctgaacaccttccaagtgctggtgctttcagatatctacctcaaagtattatttgtaaatgtcaaaaagtccctcttacatataattgaaagctggctacatggtagacaatatgatcacaaacttttaaacaattttttaagctgaagaaatactttttctttttataagtatcaaatcaaaatgtaattcagcatccacccataaagcgcaactaaaaacttttcacaatgccattaacaacttgtggttaccatcataagcctacagacctacacactaattatctttaaaacccttattaggctgggcgtggcggctcacgcctgtaatcacagcactttggggggccaaggcgggcagatcacttgaggtcaggagtttgagcccagcctggccaacatagtgaaacttcatctctgctagaaatacaaaaattagcggggcgtggtgacagggtgctctaaccccagctacttgggaggctgaagcagaaccacttgaacacagccaggaggcagaggttgcagtgagccaagattgcaccactgtactccagcctgagccacagagcaagactccgtctcaaaaaataaataaaaataaaataaaacccttattaaggatttaaaaaatcttaattatataatgccaaaagctagtccccgtctggcttaggggcccacaagctcctgctttaaagccagtttttttgtttttttctgatgtacttacatttgtgcctcacaatcaagaggttcccagcttggtggaactttcaaagatgaggcagaaaactaaacaggcaattacaatcttacttttcacgctgacaagtggtacggtggctagcccaaactcccctccctgtcccagctacctcccttatagaccattcacgatcacttaggccaggctgccatgtgacctaagagaagacagggagaacacagcatttcttactcctactaacttgcaacatcattctctcaagttgctctcattggaggctcccaactgcttcaagctgcccagtgatatttgtatttctaaagtgggcaggcatggccattccagaaaaagaaacacattcagacttgtgccttttgttacccaaatatatgatattcaaataatttctattttaacaactcataaaaatttaagatcaaataattgcattcttgaaacaattcttaatcatttattttcaacacgtgtactataaagaacctaagaaatcagacaattttaataacccataaacatgttgaatccatttgcagatttaaattttgtaaaaatagctgtcactgcctccatatatcaagtgtactatgtttataatcacatttatgctaccgatactcctcagaaaaaaacagattctgcttggttctagcttcagtattatgaactccaataatgctttgaggacctccaaaggaaaaaaacagattctactaggttctagctgaaatattatcaactccaaattgaagctgaagtattatcaactccaaataatgcttcgaggacctccaaaaaaaagagattctgcttggttgtagctgaagtattatcaactccaaataatgcttggaggacctccacaggtaaactactaatccctttggccatttattgagacagacagagagagagagagagagttttgaagcaacaatgtaccattagtaaagttgctgtgcagaattacctcagtcctattctaagcttacagttcagttgattttattgtcttcacctaagtatatacaattcacatatgggagaaaaacactaaatcaagatggttattttcactgttttgcttaagattcatatttaaatataaatcaagaagttaatccacagtttgagagatacttatattagaaattttaaatgttaaatacataattgtaaatatggtgtatgtactgtttcacatacaatgggtattgatcaaatcagtgtaattagcacacccatcagctcaaatatcatttatttgtagcaagaacattcaatacattaactatagtcaccctactctctctctctctctctctcaataaatggccaaagggattagtacttttacctttggaggtcctcaaagcattatttggagttcataatacttcagctagaacttattccttcaaatttaactctgtacccattaaaagtggttttgtgtgcaattaacagacacatgttctacccatacattgttttccaaaattattgtgtggctttaaaaaaaaaaaaacccacacaacaaattgcaaaaggcactgagataacatctgcttctagatcattgctaggctcgaaaaataaagcttgttctaccaggaatgacaagttagaacttagtatttgccaaagcagaaattatatagtgtcagttatttcaggcaaaccttattcggctctcatccccaactatctgtcagaacaattaaaagagatcaaaacagtccagcataactaggcttcattatataaggccattttgttctaagacactaataaaccaaaataagaaatattaaaatcaaaataaaagatattatttgagctattttcatacaaactgttggttccttatatcctcccttctataataaagggcatattttactgcaaagaaaattttactttatatatatcactagccataaatttttgaatgtcattaattacatgttgtctagtaccattaaccaaatagcgtaactattttatgtccacatttcacttctgtatttacaaacatatcagtaaagagttaacaatgagatgcgatcaaacatccatattatctgttttgtagacagcaatgtagatgattttgtaatcacctttcatcggagtgaccttatataaaaaataagtcaataatttagaggttctaagtctccaaaggagattttcaaatgtaaatatagaaatggttatagataatgagatttttaggaaacctctgccatgtctgcatcctgttaactgttatatcatcttttcttccagctgcgttcctttgcctgcaacaggggtcaagatgagttttgcctgacttctttgatgtcctgaactttccgtagtcctttttcttgaatttgttcattataaatatagcttggcatttgtttgatcttttcaactgtcttcactgcatcagtagttttattccatagttcttgcagatatttgacaggcttgttactatatttttcaaattcaaatccactgtaagctcattattagcagttgctttacagaatgctttagtccacctaaccttttgagaattgcacttcttttaaagtttttgtgacatttatgtttatacaatctgaacaccttgcaacagctgcagatgaacatcatgatgtggtcagggtagatgggtcccaaagaaactaacacttctcagtgctgagctcggatgggcctccactgaccaaacacggagcttgagaggaagtcaagaggtatcttggaattccacatgctgaccctgtcattcttgaaggaaaatgatgcataatttctgaataattcagaaagaacttaacaatctttccagttagtttttaaataacaattctgtttatcaaatttctgaattaacttttctgaattcacgggtttctaaaactggccttaagcaaaagtctgaaacctaggctgggaaccatgtaacccaggccaagaaggtactttaaagtgtcttagagttgtttttcaacttagggggaaacaacagattccattaaatcccataaaggatttttttgtgtgtgaaaaagggcctgatgtaatctaggttagactcaggaggctttaacaagttttgtcttacgggtaaatggtggctattttcacagataacatcattactcccatcccttactatggtttatacaaaagaggctggagaataagtacatttttacagccgggtgtggtggctaacgcctgtaatcctacttagcactttgcgaggccaagacaggaggatctcttgagcccaggagttcgagaccagcctgggcaacacagggagaccctgtctctattgttaaatcaagaaaacctaaaaaacattttcatttacatagcaccaaatataagagcctttttttttttaacctagaaagagtattttggagagagaaactaaggatcagaaggtttaagagtatcaaaaatctgaggccaggtgcctcacatctgtaatcccagcattttgggaggctgaggtgagtagatcacttgagtttaggagttcaagatcagcctggctaacatggtgaaaccctgtctttactaaaaatacaaaaaaatcagctggtatggtggtacatgcctgtaatcccagttacttggaaggctgaggcaggagaatagcttgaacccagaaggcggaagttgcagtgagccgagatcactccactgcactctagcatgggtgatggagcaagactctgtctcaaaaaaaaaaaaaaaaaaaaaaaaaaagagtatctaaaatttaaatactaattcttggctggacatggtggctcacatctgcaatcccagcacttcgggaggccgaggcgggtgacctcacttgaggtcaggagttcgtgaccagcctggccaacatggtgaaaccctatctctactaaaaatacaaaaattagctgggcatggtggtgcatgcctgtaatcccagctgctccagaggctgagccaggagaatggcttgaacccgggaagcggagactgctagatcatgacactgcactccagcctgggcgacagagagactcatctcaaaacaaacaaacaaacaaacaaacaaaaaaacaaaaaactaaatctttcacacattttctctttatatcaaaggtactaagtgacatttaggccggacgcggtggctcatgcctgtaatcccagcactttgggaggccgaggtgggcggatcacgaggtcaggagatcgagaccatcctggctaacacggtgaaaccctgtctctactaaaagtacaaaaaattagccaggtgtggtggcagatgactgtaggccaagctaattgggaggctgaggcaggagaatggtgcgaacccgggaggcagagcttgcagtgagccaagatcacgccactgcactccagcctgggtaacagagcaagactcggtctcaaaaaaaataataagttacatttaaatgtcatatacatatttaagaaaaaaaaaaaccaagtacttctcatttaagacagagtagaaattatttaaaattaggagttggtgtaaaggatgagctacatattcaagtcaaattatagtaagtattcactattccactaccaaagtaggtcaattatactaaagagaagaaatctatgtgaattgaggcattttctcactttgatatatgtgaataaatttcaggttgtctaaattcctagggttatatagttagaaatatataattctcttatagacaggtcaactaggggaaataagttagcacaatcatttgaattggttgtctacatactgggcagggcttattccttttctttagcttctttgcacatgtaaagcaggccataagatgtcctgttttgccatggacaatgcaaccatttttaggtcgaccttgacaaatcacacaaggttcaatggcattaaggggcaaactagattccacactctcttctttgtcttgggtttcttccctttcaaactctttcacatcttcttggctgctataaataatgctactagaagttgatggctgagaatagtcttcactttcttgtgattgtgaagcttgtgtaattttatcatcattttcctcaacacatgactctctggaatcattcactatagtttttttacaatcaggaacatcaaagccctcttcagcttgtgttgagttttccagtttggctttctcagagatttcccctttatctttccctttatcttcaggaagccaattctcacgaagggcccaacatctgttgcaatgtgatggaagggggggattcatttcattgcatgaagtgcatttccaatagtcagctaaggaaatttcaggatcttcttcaaatgaatctgtatcactctcccctgcctgatacacagtaacttgatatacaccagcatcaagatccggattcgatggcgtccctgtagattcactgctactgcttctttcacaacatatctcccttattacacacagagccaggctttcatcaaaggaaagggaaatactatcagatttgtggcgttttctttgtcgttcaccagataattcatctgaattttcttctgtctcactaattgctctccttctagatgaggtagatggtctagaaaccaaatgtgaagatgaaggtttctcttcctgaagctcttgtacaaggtccttttgatcactcccaccttcaaggtgacacctgttctcactcacagatgtacctgagtccgatgattcctgctgattgactactaccaagttcctgtagatcatggtatatattttcctgtgctctttcacagagaagcttggcacgccaaacaaatctcctagaagatcatttgaacaatatacaatatgttgttgcttctcatcatataatcgtttagtcataatatactggccaagataaaaaagaacctctttcatagtataagtgtctttttgtgcaccaacagactttaataacttcaaaagcaatggctttggtctaaccagggtctcttgttccgaagctggaatctgtgaggtggttacagcaccatcagtaggtacagacatgttggtattgcacatttgcctggatcagcagagaaaaagtggcgtgcgtccgtgcccacaggtctaccctccaatcgccact

SEQ ID NO: 17154 - RNA, 9652 nt, Homo sapiens
  source 1..9652: mol_type = other RNA
tcaggccaggcacagtggctcaatgcctgtaatcccagcactttgggaggccgaggcaggtggaccacatgaggtcaggaattcgagaccagcctggccaacatggcaaaaccccatctccactaaaaatgaaaaaattagctgaaataacacagctacttgggaggctaaagcaggagaatcacttgaacccaggaggtggaggctgcagtgagccaagatcacgccattgcactccaccctgggcaacagagcaagacgccatctcaaaaaaacaaacaaaaaatcacaatcagtgagattaatgtttaatgaacatactgttattttttatttttttaagagacaagtctccatctgtctcctaagcagagtgtagtggcgcaatcatagctcattgtaacattggactcctgggctcaagtgatcctcccacctcagtctcccatgcatgccaccacaattttttggatacagggtgtcattatgttgcccaggctgatctcaaactcctggcctcaagtgatcctccttccttggcctcccaaagtgttgagattacaggcgtgagtcacagagcctggcccaggatgttattttaaaattgtctttttgtcttctaaatcaacaagaacttgatagttgctttcaatgccaatcaacatcctttactactgtatacacaatgtatttatttgacatttgaaaggagatacggctgggcgcggtggctcacgcctgtaatcccagcactttgggaggccgaggcgggcggatcacaaggtcaggagatcgagaccatcttggctaacacggtgaaaccccgtctctactaaaaatacaaaaaattagccaggcgcggtggcgggcgcctgtagtcccagctactcgggaggctgaggcaggagaatggcgtgaacctgggaggcggagcttgcagtgagccgagattgcgccactgcaatccggcctgggctaaacagcgggactccgtctcaaaaaaaaaaaaaaaaaaagaaaggagatacaaaaggatgttacaacctgctatggcaagaagatacaaaggaacatattggtatgaacagaatacctcagagttgagtgtataaaaaaggcttaattcaccagatgcagtggctcgcacctgtaatcccagcattttgagaggtcaaggtcaagacacgaggattgcttgagcccaggagttcaaggccagcctgggcaacatagcaggactctgcctctaaaaaaagtatatatatatatataatgtacacacacatacatacataaacacatatgtattatatatatatatgtaatatatgtatattatatataatatatatattagccaggcatggtggcaacaggcctgtgttcccagctactcaggaggctgcagtgagtcatgtttgcgccactatactccagcctgggtgacagaatgagaccctgtctcagcaaaaaacaaataaaaaacttcaaggtggagtaggggttaattcaaggctacctaagctggatttggggtgattatggtcgagtggatgcaaacagaatattaaacttccattcattaaaagtgcttactacctgccagaccccatactaggctctatagatttattgtctctaaggtcactaggcgagtaagtaccagatctgtgactttgaacttcccactacaataagcttatgaactttgtttaagcaaaaaaggtttgaaaagtgaaaagcaagcacccatttcatagtgttctaaaagtctaaaataatccagtagaacatcagagataaaatccaaaaagcaagtttttcccccaatatttaaatcagggaagcaacatgatggtatctgtaaactataactgaaccaaaaataggaccaaacgtagtgaaatccatttagggagatattactgtgatcttgaaggaaggcctacttaatacaggacagtgggctggggaggtgtgaaccaaaaatagacacaggcaaaagcgctaaaatttaaccctgagaaataaatgaaattcacctacaaaataaatggaataaatttaaaaggtgaaattttgggcttggcgtggtggcttacacctgtaatctcagcactttgggaagccaagacgggcagatcacttgaccccaggagtttgagaccagcctgggcaacatggtgaaactgtctctacaaaaaatacaaaaattaggccgggcacggtggctcacgcctgtaatcccagtactttgggaggccgaggtgggcggatcatgaggtcaggagttcgagaccagcctggacaacatgctgaaaccccatctctactaaaaatacaaaaaaaattagccaggtgtggttggcgagcacctataattccagctactcaggaggctgaggcagaattgcttgaacctgggaggtggaggttgcaatgagccgagattgcaccactgcactccagtctgggtgaaagagcaagactctgtctcagggcgggtggcagcggggtcgggggaggtggggggaaggttagctggacctggtggcttgcacctgtggtccccagctacttgggaggctgaggtgggaggattgcttgagcccaggaggttgaggctgtagtgagtcatgtttgcagcactgcattccagcctgggcgacagagcaagaccgcatctcaaaacaaaacaaacaaaaggtgaaattttggaattaggaaagatgctatttttataaattggctttaagctgttggctggacatctaagttgtagcattctgaaggcagcagagatgtgggattgtaggactgaaacatgaaaatgcctatcgaattttttttaaagtctttaaaggagagctttaaaggaaagcaatacgaattcaagtatgtttcagtaccactcctctctctaaagacaatcaactatggttttcattcaaaatactattactctaacgttaaatatttgagtacagcaatcatttcagatgcattatgaataagttactgaacacgcctcccatctgcttgctttacggttttattttgcctttcgtttgttagctcattttataatttgttacttctgaacaccttccaagtgctggtgctttcagatatctacctcaaagtattatttgtaaatgtcaaaaagtccctcttacatataattgaaagctggctacatggtagacaatatgatcacaaacttttaaacaattttttaagctgaagaaatactttttctttttataagtatcaaatcaaaatgtaattcagcatccacccataaagcgcaactaaaaacttttcacaatgccattaacaacttgtggttaccatcataagcctacagacctacacactaattatctttaaaacccttattaggctgggcgtggcggctcacgcctgtaatcacagcactttggggggccaaggcgggcagatcacttgaggtcaggagtttgagcccagcctggccaacatagtgaaacttcatctctgctagaaatacaaaaattagcggggcgtggtgacagggtgctctaaccccagctacttgggaggctgaagcagaaccacttgaacacagccaggaggcagaggttgcagtgagccaagattgcaccactgtactccagcctgagccacagagcaagactccgtctcaaaaaataaataaaaataaaataaaacccttattaaggatttaaaaaatcttaattatataatgccaaaagctagtccccgtctggcttaggggcccacaagctcctgctttaaagccagtttttttgtttttttctgatgtacttacatttgtgcctcacaatcaagaggttcccagcttggtggaactttcaaagatgaggcagaaaactaaacaggcaattacaatcttacttttcacgctgacaagtggtacggtggctagcccaaactcccctccctgtcccagctacctcccttatagaccattcacgatcacttaggccaggctgccatgtgacctaagagaagacagggagaacacagcatttcttactcctactaacttgcaacatcattctctcaagttgctctcattggaggctcccaactgcttcaagctgcccagtgatatttgtatttctaaagtgggcaggcatggccattccagaaaaagaaacacattcagacttgtgccttttgttacccaaatatatgatattcaaataatttctattttaacaactcataaaaatttaagatcaaataattgcattcttgaaacaattcttaatcatttattttcaacacgtgtactataaagaacctaagaaatcagacaattttaataacccataaacatgttgaatccatttgcagatttaaattttgtaaaaatagctgtcactgcctccatatatcaagtgtactatgtttataatcacatttatgctaccgatactcctcagaaaaaaacagattctgcttggttctagcttcagtattatgaactccaataatgctttgaggacctccaaaggaaaaaaacagattctactaggttctagctgaaatattatcaactccaaattgaagctgaagtattatcaactccaaataatgcttcgaggacctccaaaaaaaagagattctgcttggttgtagctgaagtattatcaactccaaataatgcttggaggacctccacaggtaaactactaatccctttggccatttattgagacagacagagagagagagagagagttttgaagcaacaatgtaccattagtaaagttgctgtgcagaattacctcagtcctattctaagcttacagttcagttgattttattgtcttcacctaagtatatacaattcacatatgggagaaaaacactaaatcaagatggttattttcactgttttgcttaagattcatatttaaatataaatcaagaagttaatccacagtttgagagatacttatattagaaattttaaatgttaaatacataattgtaaatatggtgtatgtactgtttcacatacaatgggtattgatcaaatcagtgtaattagcacacccatcagctcaaatatcatttatttgtagcaagaacattcaatacattaactatagtcaccctactctctctctctctctctctcaataaatggccaaagggattagtacttttacctttggaggtcctcaaagcattatttggagttcataatacttcagctagaacttattccttcaaatttaactctgtacccattaaaagtggttttgtgtgcaattaacagacacatgttctacccatacattgttttccaaaattattgtgtggctttaaaaaaaaaaaaacccacacaacaaattgcaaaaggcactgagataacatctgcttctagatcattgctaggctcgaaaaataaagcttgttctaccaggaatgacaagttagaacttagtatttgccaaagcagaaattatatagtgtcagttatttcaggcaaaccttattcggctctcatccccaactatctgtcagaacaattaaaagagatcaaaacagtccagcataactaggcttcattatataaggccattttgttctaagacactaataaaccaaaataagaaatattaaaatcaaaataaaagatattatttgagctattttcatacaaactgttggttccttatatcctcccttctataataaagggcatattttactgcaaagaaaattttactttatatatatcactagccataaatttttgaatgtcattaattacatgttgtctagtaccattaaccaaatagcgtaactattttatgtccacatttcacttctgtatttacaaacatatcagtaaagagttaacaatgagatgcgatcaaacatccatattatctgttttgtagacagcaatgtagatgattttgtaatcacctttcatcggagtgaccttatataaaaaataagtcaataatttagaggttctaagtctccaaaggagattttcaaatgtaaatatagaaatggttatagataatgagatttttaggaaacctctgccatgtctgcatcctgttaactgttatatcatcttttcttccagctgcgttcctttgcctgcaacaggggtcaagatgagttttgcctgacttctttgatgtcctgaactttccgtagtcctttttcttgaatttgttcattataaatatagcttggcatttgtttgatcttttcaactgtcttcactgcatcagtagttttattccatagttcttgcagatatttgacaggcttgttactatatttttcaaattcaaatccactgtaagctcattattagcagttgctttacagaatgctttagtccacctaaccttttgagaattgcacttcttttaaagtttttgtgacatttatgtttatacaatctgaacaccttgcaacagctgcagatgaacatcatgatgtggtcagggtagatgggtcccaaagaaactaacacttctcagtgctgagctcggatgggcctccactgaccaaacacggagcttgagaggaagtcaagaggtatcttggaattccacatgctgaccctgtcattcttgaaggaaaatgatgcataatttctgaataattcagaaagaacttaacaatctttccagttagtttttaaataacaattctgtttatcaaatttctgaattaacttttctgaattcacgggtttctaaaactggccttaagcaaaagtctgaaacctaggctgggaaccatgtaacccaggccaagaaggtactttaaagtgtcttagagttgtttttcaacttagggggaaacaacagattccattaaatcccataaaggatttttttgtgtgtgaaaaagggcctgatgtaatctaggttagactcaggaggctttaacaagttttgtcttacgggtaaatggtggctattttcacagataacatcattactcccatcccttactatggtttatacaaaagaggctggagaataagtacatttttacagccgggtgtggtggctaacgcctgtaatcctacttagcactttgcgaggccaagacaggaggatctcttgagcccaggagttcgagaccagcctgggcaacacagggagaccctgtctctattgttaaatcaagaaaacctaaaaaacattttcatttacatagcaccaaatataagagcctttttttttttaacctagaaagagtattttggagagagaaactaaggatcagaaggtttaagagtatcaaaaatctgaggccaggtgcctcacatctgtaatcccagcattttgggaggctgaggtgagtagatcacttgagtttaggagttcaagatcagcctggctaacatggtgaaaccctgtctttactaaaaatacaaaaaaatcagctggtatggtggtacatgcctgtaatcccagttacttggaaggctgaggcaggagaatagcttgaacccagaaggcggaagttgcagtgagccgagatcactccactgcactctagcatgggtgatggagcaagactctgtctcaaaaaaaaaaaaaaaaaaaaaaaaaaagagtatctaaaatttaaatactaattcttggctggacatggtggctcacatctgcaatcccagcacttcgggaggccgaggcgggtgacctcacttgaggtcaggagttcgtgaccagcctggccaacatggtgaaaccctatctctactaaaaatacaaaaattagctgggcatggtggtgcatgcctgtaatcccagctgctccagaggctgagccaggagaatggcttgaacccgggaagcggagactgctagatcatgacactgcactccagcctgggcgacagagagactcatctcaaaacaaacaaacaaacaaacaaacaaaaaaacaaaaaactaaatctttcacacattttctctttatatcaaaggtactaagtgacatttaggccggacgcggtggctcatgcctgtaatcccagcactttgggaggccgaggtgggcggatcacgaggtcaggagatcgagaccatcctggctaacacggtgaaaccctgtctctactaaaagtacaaaaaattagccaggtgtggtggcagatgactgtaggccaagctaattgggaggctgaggcaggagaatggtgcgaacccgggaggcagagcttgcagtgagccaagatcacgccactgcactccagcctgggtaacagagcaagactcggtctcaaaaaaaataataagttacatttaaatgtcatatacatatttaagaaaaaaaaaaaccaagtacttctcatttaagacagagtagaaattatttaaaattaggagttggtgtaaaggatgagctacatattcaagtcaaattatagtaagtattcactattccactaccaaagtaggtcaattatactaaagagaagaaatctatgtgaattgaggcattttctcactttgatatatgtgaataaatttcaggttgtctaaattcctagggttatatagttagaaatatataattctcttatagacaggtcaactaggggaaataagttagcacaatcatttgaattggttgtctacatactgggcagggcttattccttttctttagcttctttgcacatgtaaagcaggccataagatgtcctgttttgccatggacaatgcaaccatttttaggtcgaccttgacaaatcacacaaggttcaatggcattaaggggcaaactagattccacactctcttctttgtcttgggtttcttccctttcaaactctttcacatcttcttggctgctataaataatgctactagaagttgatggctgagaatagtcttcactttcttgtgattgtgaagcttgtgtaattttatcatcattttcctcaacacatgactctctggaatcattcactatagtttttttacaatcaggaacatcaaagccctcttcagcttgtgttgagttttccagtttggctttctcagagatttcccctttatctttccctttatcttcaggaagccaattctcacgaagggcccaacatctgttgcaatgtgatggaagggggggattcatttcattgcatgaagtgcatttccaatagtcagctaaggaaatttcaggatcttcttcaaatgaatctgtatcactctcccctgcctgatacacagtaacttgatatacctcatcatcttcatctgagagttcttgtccttcttcactaaggctataatcttctgagtcgagagattcaacttcaaattctacactaaactgatctgaaactgaatcctgatccaaccaatcacctgaatgttcacttacaccagcatcaagatcctctttcatagtataagtgtctttttgtgcaccaacagactttaataacttcaaaagcaatggctttggtctaaccagggtctcttgttccgaagctggaatctgtgaggtggttacagcaccatcagtaggtacagacatgttggtattgcacatttgcctggatcagcagagaaaaagtggcgtgcgtccgtgcccacaggtctaccctccaatcgccact

SEQ ID NO: 17155 - RNA, 9574 nt, Homo sapiens
  source 1..9574: mol_type = other RNA
tcaggccaggcacagtggctcaatgcctgtaatcccagcactttgggaggccgaggcaggtggaccacatgaggtcaggaattcgagaccagcctggccaacatggcaaaaccccatctccactaaaaatgaaaaaattagctgaaataacacagctacttgggaggctaaagcaggagaatcacttgaacccaggaggtggaggctgcagtgagccaagatcacgccattgcactccaccctgggcaacagagcaagacgccatctcaaaaaaacaaacaaaaaatcacaatcagtgagattaatgtttaatgaacatactgttattttttatttttttaagagacaagtctccatctgtctcctaagcagagtgtagtggcgcaatcatagctcattgtaacattggactcctgggctcaagtgatcctcccacctcagtctcccatgcatgccaccacaattttttggatacagggtgtcattatgttgcccaggctgatctcaaactcctggcctcaagtgatcctccttccttggcctcccaaagtgttgagattacaggcgtgagtcacagagcctggcccaggatgttattttaaaattgtctttttgtcttctaaatcaacaagaacttgatagttgctttcaatgccaatcaacatcctttactactgtatacacaatgtatttatttgacatttgaaaggagatacggctgggcgcggtggctcacgcctgtaatcccagcactttgggaggccgaggcgggcggatcacaaggtcaggagatcgagaccatcttggctaacacggtgaaaccccgtctctactaaaaatacaaaaaattagccaggcgcggtggcgggcgcctgtagtcccagctactcgggaggctgaggcaggagaatggcgtgaacctgggaggcggagcttgcagtgagccgagattgcgccactgcaatccggcctgggctaaacagcgggactccgtctcaaaaaaaaaaaaaaaaaaagaaaggagatacaaaaggatgttacaacctgctatggcaagaagatacaaaggaacatattggtatgaacagaatacctcagagttgagtgtataaaaaaggcttaattcaccagatgcagtggctcgcacctgtaatcccagcattttgagaggtcaaggtcaagacacgaggattgcttgagcccaggagttcaaggccagcctgggcaacatagcaggactctgcctctaaaaaaagtatatatatatatataatgtacacacacatacatacataaacacatatgtattatatatatatatgtaatatatgtatattatatataatatatatattagccaggcatggtggcaacaggcctgtgttcccagctactcaggaggctgcagtgagtcatgtttgcgccactatactccagcctgggtgacagaatgagaccctgtctcagcaaaaaacaaataaaaaacttcaaggtggagtaggggttaattcaaggctacctaagctggatttggggtgattatggtcgagtggatgcaaacagaatattaaacttccattcattaaaagtgcttactacctgccagaccccatactaggctctatagatttattgtctctaaggtcactaggcgagtaagtaccagatctgtgactttgaacttcccactacaataagcttatgaactttgtttaagcaaaaaaggtttgaaaagtgaaaagcaagcacccatttcatagtgttctaaaagtctaaaataatccagtagaacatcagagataaaatccaaaaagcaagtttttcccccaatatttaaatcagggaagcaacatgatggtatctgtaaactataactgaaccaaaaataggaccaaacgtagtgaaatccatttagggagatattactgtgatcttgaaggaaggcctacttaatacaggacagtgggctggggaggtgtgaaccaaaaatagacacaggcaaaagcgctaaaatttaaccctgagaaataaatgaaattcacctacaaaataaatggaataaatttaaaaggtgaaattttgggcttggcgtggtggcttacacctgtaatctcagcactttgggaagccaagacgggcagatcacttgaccccaggagtttgagaccagcctgggcaacatggtgaaactgtctctacaaaaaatacaaaaattaggccgggcacggtggctcacgcctgtaatcccagtactttgggaggccgaggtgggcggatcatgaggtcaggagttcgagaccagcctggacaacatgctgaaaccccatctctactaaaaatacaaaaaaaattagccaggtgtggttggcgagcacctataattccagctactcaggaggctgaggcagaattgcttgaacctgggaggtggaggttgcaatgagccgagattgcaccactgcactccagtctgggtgaaagagcaagactctgtctcagggcgggtggcagcggggtcgggggaggtggggggaaggttagctggacctggtggcttgcacctgtggtccccagctacttgggaggctgaggtgggaggattgcttgagcccaggaggttgaggctgtagtgagtcatgtttgcagcactgcattccagcctgggcgacagagcaagaccgcatctcaaaacaaaacaaacaaaaggtgaaattttggaattaggaaagatgctatttttataaattggctttaagctgttggctggacatctaagttgtagcattctgaaggcagcagagatgtgggattgtaggactgaaacatgaaaatgcctatcgaattttttttaaagtctttaaaggagagctttaaaggaaagcaatacgaattcaagtatgtttcagtaccactcctctctctaaagacaatcaactatggttttcattcaaaatactattactctaacgttaaatatttgagtacagcaatcatttcagatgcattatgaataagttactgaacacgcctcccatctgcttgctttacggttttattttgcctttcgtttgttagctcattttataatttgttacttctgaacaccttccaagtgctggtgctttcagatatctacctcaaagtattatttgtaaatgtcaaaaagtccctcttacatataattgaaagctggctacatggtagacaatatgatcacaaacttttaaacaattttttaagctgaagaaatactttttctttttataagtatcaaatcaaaatgtaattcagcatccacccataaagcgcaactaaaaacttttcacaatgccattaacaacttgtggttaccatcataagcctacagacctacacactaattatctttaaaacccttattaggctgggcgtggcggctcacgcctgtaatcacagcactttggggggccaaggcgggcagatcacttgaggtcaggagtttgagcccagcctggccaacatagtgaaacttcatctctgctagaaatacaaaaattagcggggcgtggtgacagggtgctctaaccccagctacttgggaggctgaagcagaaccacttgaacacagccaggaggcagaggttgcagtgagccaagattgcaccactgtactccagcctgagccacagagcaagactccgtctcaaaaaataaataaaaataaaataaaacccttattaaggatttaaaaaatcttaattatataatgccaaaagctagtccccgtctggcttaggggcccacaagctcctgctttaaagccagtttttttgtttttttctgatgtacttacatttgtgcctcacaatcaagaggttcccagcttggtggaactttcaaagatgaggcagaaaactaaacaggcaattacaatcttacttttcacgctgacaagtggtacggtggctagcccaaactcccctccctgtcccagctacctcccttatagaccattcacgatcacttaggccaggctgccatgtgacctaagagaagacagggagaacacagcatttcttactcctactaacttgcaacatcattctctcaagttgctctcattggaggctcccaactgcttcaagctgcccagtgatatttgtatttctaaagtgggcaggcatggccattccagaaaaagaaacacattcagacttgtgccttttgttacccaaatatatgatattcaaataatttctattttaacaactcataaaaatttaagatcaaataattgcattcttgaaacaattcttaatcatttattttcaacacgtgtactataaagaacctaagaaatcagacaattttaataacccataaacatgttgaatccatttgcagatttaaattttgtaaaaatagctgtcactgcctccatatatcaagtgtactatgtttataatcacatttatgctaccgatactcctcagaaaaaaacagattctgcttggttctagcttcagtattatgaactccaataatgctttgaggacctccaaaggaaaaaaacagattctactaggttctagctgaaatattatcaactccaaattgaagctgaagtattatcaactccaaataatgcttcgaggacctccaaaaaaaagagattctgcttggttgtagctgaagtattatcaactccaaataatgcttggaggacctccacaggtaaactactaatccctttggccatttattgagacagacagagagagagagagagagttttgaagcaacaatgtaccattagtaaagttgctgtgcagaattacctcagtcctattctaagcttacagttcagttgattttattgtcttcacctaagtatatacaattcacatatgggagaaaaacactaaatcaagatggttattttcactgttttgcttaagattcatatttaaatataaatcaagaagttaatccacagtttgagagatacttatattagaaattttaaatgttaaatacataattgtaaatatggtgtatgtactgtttcacatacaatgggtattgatcaaatcagtgtaattagcacacccatcagctcaaatatcatttatttgtagcaagaacattcaatacattaactatagtcaccctactctctctctctctctctctcaataaatggccaaagggattagtacttttacctttggaggtcctcaaagcattatttggagttcataatacttcagctagaacttattccttcaaatttaactctgtacccattaaaagtggttttgtgtgcaattaacagacacatgttctacccatacattgttttccaaaattattgtgtggctttaaaaaaaaaaaaacccacacaacaaattgcaaaaggcactgagataacatctgcttctagatcattgctaggctcgaaaaataaagcttgttctaccaggaatgacaagttagaacttagtatttgccaaagcagaaattatatagtgtcagttatttcaggcaaaccttattcggctctcatccccaactatctgtcagaacaattaaaagagatcaaaacagtccagcataactaggcttcattatataaggccattttgttctaagacactaataaaccaaaataagaaatattaaaatcaaaataaaagatattatttgagctattttcatacaaactgttggttccttatatcctcccttctataataaagggcatattttactgcaaagaaaattttactttatatatatcactagccataaatttttgaatgtcattaattacatgttgtctagtaccattaaccaaatagcgtaactattttatgtccacatttcacttctgtatttacaaacatatcagtaaagagttaacaatgagatgcgatcaaacatccatattatctgttttgtagacagcaatgtagatgattttgtaatcacctttcatcggagtgaccttatataaaaaataagtcaataatttagaggttctaagtctccaaaggagattttcaaatgtaaatatagaaatggttatagataatgagatttttaggaaacctctgccatgtctgcatcctgttaactgttatatcatcttttcttccagctgcgttcctttgcctgcaacaggggtcaagatgagttttgcctgacttctttgatgtcctgaactttccgtagtcctttttcttgaatttgttcattataaatatagcttggcatttgtttgatcttttcaactgtcttcactgcatcagtagttttattccatagttcttgcagatatttgacaggcttgttactatatttttcaaattcaaatccactgtaagctcattattagcagttgctttacagaatgctttagtccacctaaccttttgagaattgcacttcttttaaagtttttgtgacatttatgtttatacaatctgaacaccttgcaacagctgcagatgaacatcatgatgtggtcagggtagatgggtcccaaagaaactaacacttctcagtgctgagctcggatgggcctccactgaccaaacacggagcttgagaggaagtcaagaggtatcttggaattccacatgctgaccctgtcattcttgaaggaaaatgatgcataatttctgaataattcagaaagaacttaacaatctttccagttagtttttaaataacaattctgtttatcaaatttctgaattaacttttctgaattcacgggtttctaaaactggccttaagcaaaagtctgaaacctaggctgggaaccatgtaacccaggccaagaaggtactttaaagtgtcttagagttgtttttcaacttagggggaaacaacagattccattaaatcccataaaggatttttttgtgtgtgaaaaagggcctgatgtaatctaggttagactcaggaggctttaacaagttttgtcttacgggtaaatggtggctattttcacagataacatcattactcccatcccttactatggtttatacaaaagaggctggagaataagtacatttttacagccgggtgtggtggctaacgcctgtaatcctacttagcactttgcgaggccaagacaggaggatctcttgagcccaggagttcgagaccagcctgggcaacacagggagaccctgtctctattgttaaatcaagaaaacctaaaaaacattttcatttacatagcaccaaatataagagcctttttttttttaacctagaaagagtattttggagagagaaactaaggatcagaaggtttaagagtatcaaaaatctgaggccaggtgcctcacatctgtaatcccagcattttgggaggctgaggtgagtagatcacttgagtttaggagttcaagatcagcctggctaacatggtgaaaccctgtctttactaaaaatacaaaaaaatcagctggtatggtggtacatgcctgtaatcccagttacttggaaggctgaggcaggagaatagcttgaacccagaaggcggaagttgcagtgagccgagatcactccactgcactctagcatgggtgatggagcaagactctgtctcaaaaaaaaaaaaaaaaaaaaaaaaaaagagtatctaaaatttaaatactaattcttggctggacatggtggctcacatctgcaatcccagcacttcgggaggccgaggcgggtgacctcacttgaggtcaggagttcgtgaccagcctggccaacatggtgaaaccctatctctactaaaaatacaaaaattagctgggcatggtggtgcatgcctgtaatcccagctgctccagaggctgagccaggagaatggcttgaacccgggaagcggagactgctagatcatgacactgcactccagcctgggcgacagagagactcatctcaaaacaaacaaacaaacaaacaaacaaaaaaacaaaaaactaaatctttcacacattttctctttatatcaaaggtactaagtgacatttaggccggacgcggtggctcatgcctgtaatcccagcactttgggaggccgaggtgggcggatcacgaggtcaggagatcgagaccatcctggctaacacggtgaaaccctgtctctactaaaagtacaaaaaattagccaggtgtggtggcagatgactgtaggccaagctaattgggaggctgaggcaggagaatggtgcgaacccgggaggcagagcttgcagtgagccaagatcacgccactgcactccagcctgggtaacagagcaagactcggtctcaaaaaaaataataagttacatttaaatgtcatatacatatttaagaaaaaaaaaaaccaagtacttctcatttaagacagagtagaaattatttaaaattaggagttggtgtaaaggatgagctacatattcaagtcaaattatagtaagtattcactattccactaccaaagtaggtcaattatactaaagagaagaaatctatgtgaattgaggcattttctcactttgatatatgtgaataaatttcaggttgtctaaattcctagggttatatagttagaaatatataattctcttatagacaggtcaactaggggaaataagttagcacaatcatttgaattggttgtctacatactgggcagggcttattccttttctttagcttctttgcacatgtaaagcaggccataagatgtcctgttttgccatggacaatgcaaccatttttaggtcgaccttgacaaatcacacaaggttcaatggcattaaggggcaaactagattccacactctcttctttgtcttgggtttcttccctttcaaactctttcacatcttcttggctgctataaataatgctactagaagttgatggctgagaatagtcttcactttcttgtgattgtgaagcttgtgtaattttatcatcattttcctcaacacatgactctctggaatcattcactatagtttttttacaatcaggaacatcaaagccctcttcagcttgtgttgagttttccagtttggctttctcagagatttcccctttatctttccctttatcttcaggaagccaattctcacgaagggcccaacatctgttgcaatgtgatggaagggggggattcatttcattgcatgaagtgcatttccaatagtcctcatcatcttcatctgagagttcttgtccttcttcactaaggctataatcttctgagtcgagagattcaacttcaaattctacactaaactgatctgaaactgaatcctgatccaaccaatcacctgaatgttcacttacaccagcatcaagatcctctttcatagtataagtgtctttttgtgcaccaacagactttaataacttcaaaagcaatggctttggtctaaccagggtctcttgttccgaagctggaatctgtgaggtggttacagcaccatcagtaggtacagacatgttggtattgcacatttgcctggatcagcagagaaaaagtggcgtgcgtccgtgcccacaggtctaccctccaatcgccact

SEQ ID NO: 17156 - RNA, 3746 nt, Homo sapiens
  source 1..3746: mol_type = other RNA
tcaggccaggcacagtggctcacaaccgtaatcccagcactctgggacgctgaggtgtgaggatcgcttgagcccaggagtctgagatctgcctgggcaacatagggagaccccccacctctacaaaaaaaaattgaaaaaaattatctggatatgaggtgcacacctgtggtcctaactacttgggaggctgaggtaggaggatcacttgagctgggaaggtcaaggctgcaatcagctgtaattgtgtcactgcactaagccttggtgacagagtgaaaccctttttcaacaacaaaggcaaaatcttaaaaacaggaaacaggctattgaggaaaaagggttataaaactgcctaagaatcttcactaaagtaatcttctagtccttccatatccatttccagagaggaatttaaagaggccagagcagatgatgcatccttggttttctggacacttggtttgggttgaggagtttctggttggataggttccttctttatgtctttaccaccatttagaatacgttggctctcacaaaagaactgattaggatgattcaaagaaaagccacaatcatccacattgtgtatcatctcaaagtatttttgacaggctacctggtaatgtgtcccctttactaaatccaaaatctggcttatccctccaggagagatcttgtatgactgcaacttttgcttcagcagctctggatcactgtgacggaatgggcacccatgataatccccttggcttggtggattggacagaataatcttcaggcaactgaaaggtgtatagtctgtcctcttgccttcctttccaaagctgtgacggatgttgtaagagtaacctttatcaaacttgtctggatccatctttcctttgataaattcttgcttccagaactgcaatgcctgttccaaagttaaaccaatgcccttcagaaataggccatactgcattcggcctccatgacgaagatggtgattttcccgcaaggctttatgtaactgacgcatgcaaggtgggaaggatttggtagaaagcaaatcaatctgatctaaagaaatcttcccaacatttccctgggtactgtaatcttggccagtgtaggaatgactgaggtgattgagcagaggctgaagtctttcatcagactgcacagcaggcaaggacctggctgttaacaagggttcatggaataggttttgctggctgcccagacgactgcccatttcttccccacgagttatcttcaaaacagtatctctgcatgagctttctctttccttatccctcctctcatctccacattgcttaactaaaccctgacttttccttctctttcatggatcgtatcatccttaaatatagacttttatctgtcttgagatgagatgagagacttctagtttccttgattctaatcctcctgtgacaaggtacatcttttttatctgtgtcattaatcaataaagagctgacaagagagtcactcaatattatgaaccgttcagttaagctggaacattgctcaggtaaaatttagaataagaagtcatcaggcttcataaaattgatcttaccccaataaaacttggttagcagtccttctccatttgtcatagggaaaatccaaaagcaaggaaaacacagcttagaagtagtcttataaaattaatgatattacttttgcagtaaatcaaatccatagagattttagaagttataactagtggtcaacctgaaagttcaattgaaaagcttttttttttttttttaaatcaggatgacagccataagacaggcctatcaaaagacttaaatcagtaaactcttaaaagacattctttaaaatggcagtcatttaaaatccagtagatatcatatttaactggctaaagacagaacttacgagcattacagaataatatccttttgatggttttcggaagtactgccttctgtggaattgcagagactcttcaattctctaaggagaagcttactgagactcaggcatattcctaaaatcctagtaaagctttccaaaagctcaccaaaaactatcactaaattaagcactccatcaagttaaacatgttcctaacttttctgttggtggcaaattagaacattttttctaattcagtacactctctgatatctaacaagccacttttagctctaagtataagtaaaatgttctacttttctttcaagtttgaaaaaaaaaaaaaatagacccctggtctgtatggagaccgcaacaaaaaccatttgcactggcttatatgctcctgcccccaccatacaacatcaaatgtactgaaaaagcatggagaacaaggctgccacaacctttaatgcttcatgactaggtgaagcatgacttcaatgtttcatgaccaggagggggctctgtgcccctcacaccctcttctgctgcaggcagtaccttttcacctaggggtgcttaatttttatgtgtcagcttggctacataatgatgcctagttagttggtcaaatactaatcgaggtggcactgtgaaggttttgtagagatgattaacaattgacaatcagctgactttaagtaaagggaaagtaccctggataacatggctggctctcatcccaccagctcaaggccttaaaagcaaaaacatgtttttgaagaaggaattctgcctcaatattgtaatatagaaatcctgcccaagtttcctgcatggaggccttccctatgaatttcagactcaagattacaacttcaactcttacctgagtttccgggcagccctacagacttcagccctcccatttcataagccaggtatgttgtagtgtggtctagttagctcagtttaaaaatctagtttatcactgtacaggaacctgccatttgtgaaaaagatcagttataagagcatcttagattctcttcaagaagaaattcttaaatttgggctaaaaatgtccacctaataagatcattttattcaattcctaatctcacagctgattcctttctatgaggtttttaacaagtaatcatgcacttgaataactctaccaacagggacagcaaggtggaaagtaaaggaaagggaaatgacatttattgaattcttctcatgtgttgagtgctaccctgagcattttacaaaagtcatccactttaatcctcacatcataactgtgagataggcattattaacatcattttacagataaagaaacccagcctcagagaacttaaactgatgcaaaaatcacaaaacaagcatacttaacactcagcccaggtggtcttactccaaaactcattgtgttaagtcagctcttgctgataataacaatcccaaaatctcagtgacttaccacaccaaatagttatttttttgttcatactaaacaaaagttaagggctgagtaaagctctgctcaacgctgcaggtcctcttcacaggtcttctcattctgggatgcaagctaaaggaggaagttaccagatgtcacctggttaagactacaaatacataattcctcccatacaatttttttatgaagacaaagtgtgtattctgggtaggaaacaaaaatgaagtgaatgcctagtagctaggggggctaactgtaagagtcactagtgttttcatcaaataatcgtagatttgtttctgtttgtttgtttgtttgtcttttttgagacagagtttcactcttgttgcccagg

SEQ ID NO: 17157 - RNA, 2162 nt, Homo sapiens
  source 1..2162: mol_type = other RNA
tcaggccaggcacagtggctcacaaccgtaatcccagcactctgggacgctgaggtgtgaggatcgcttgagcccaggagtctgagatctgcctgggcaacatagggagaccccccacctctacaaaaaaaaattgaaaaaaattatctggatatgaggtgcacacctgtggtcctaactacttgggaggctgaggtaggaggatcacttgagctgggaaggtcaaggctgcaatcagctgtaattgtgtcactgcactaagccttggtgacagagtgaaaccctttttcaacaacaaaggcaaaatcttaaaaacaggaaacaggctattgaggaaaaagggttataaaactgcctaagaatcttcactaaagtaatcttctagtccttccatatccatttccagagaggaatttaaagaggccagagcagatgatgcatccttggttttctggacacttggtttgggttgaggagtttctggttggataggttccttctttatgtctttaccaccatttagaatacgttggctctcacaaaagaactgattaggatgattcaaagaaaagccacaatcatccacattgtgtatcatctcaaagtatttttgacaggctacctggtaatgtgtcccctttactaaatccaaaatctggcttatccctccaggagagatcttgtatgactgcaacttttgcttcagcagctctggatcactgtgacggaatgggcacccatgataatccccttggcttggtggattggacagaataatcttcaggcaactgaaaggtgtatagtctgtcctcttgccttcctttccaaagctgtgacggatgttgtaagagtaacctttatcaaacttgtctggatccatctttcctttgataaattcttgcttccagaactgcaatgcctgttccaaagttaaaccaatgcccttcagaaataggccatactgcattcggcctccatgacgaagatggtgattttcccgcaaggctttatgtaactgacgcatgcaaggtgggaaggatttggtagaaagcaaatcaatctgatctaaagaaatcttcccaacatttccctgggtactgtaatcttggccagtgtaggaatgactgaggtgattgagcagaggctgaagtctttcatcagactgcacagcaggcaaggacctggctgttaatactgaagctgactttgccacctcttctctatgtgagtaaagactgttccatccacagcctgtgtgagtcgtgtatctcttcaggaatccaacaattgcaaccatgtggtgggctgacatcctgggactgctgctcctgacagtaggtgttgttatgctccttgctgtcctccacacagtgggactcctccctgccaaagccttggacagtttggctctaaattcattcaggatgattgccacaatgtccttaagtggtacgtaagcaaagccatcttccaaatagactttccttcctcgaaacaaatccagagcatcagcaaaagggatcttataaatggactcgaaccccaacttaagtccacttaaacttggtgatgaggcaacaatctcctgttctcgaagagtcttctcttcatcacttatagcctcaaactgcaattggctatcctttaagaaatcctgaattttatccttgggtaaaatactaaatctaaatcgaaggagatccatttcttgttgaatgaaccagcgtctaagttcttcagactggcaataagcaagccgcaaaataaaatgagaaatatgatctcttcttcgtggttcatattcatcttctaagttttctctgtaggaaaacttgagcttccgaagctcactctccaacttactctggtattgttcagttcctttcacatagctcactccaagattttcaactgattttaacaatttaactctatcaatagccaagttttcaaattctattaaagatatgttttcagaaggtggctgcaagtaaaactgaaggcaatgagggtaggaagcattcctctggtcacctgccaacctcagcttcctccactttcttccagaaaactccatcttggtcacctgcaagaattcaaactcgggaaaacacaaacggtggcagccactgttcccgggtggcgggagagttcatatgaaa

SEQ ID NO: 17158 - RNA, 1966 nt, Homo sapiens
  source 1..1966: mol_type = other RNA
tcaggccaggcacagtggctcacaaccgtaatcccagcactctgggacgctgaggtgtgaggatcgcttgagcccaggagtctgagatctgcctgggcaacatagggagaccccccacctctacaaaaaaaaattgaaaaaaattatctggatatgaggtgcacacctgtggtcctaactacttgggaggctgaggtaggaggatcacttgagctgggaaggtcaaggctgcaatcagctgtaattgtgtcactgcactaagccttggtgacagagtgaaaccctttttcaacaacaaaggcaaaatcttaaaaacaggaaacaggctattgaggaaaaagggttataaaactgcctaagaatcttcactaaagtaatcttctagtccttccatatccatttccagagaggaatttaaagaggccagagcagatgatgcatccttggttttctggacacttggtttgggttgaggagtttctggttggataggttccttctttatgtctttaccaccatttagaatacgttggctctcacaaaagaactgattaggatgattcaaagaaaagccacaatcatccacattgtgtatcatctcaaagtatttttgacaggctacctggtaatgtgtcccctttactaaatccaaaatctggcttatccctccaggagagatcttgtatgactgcaacttttgcttcagcagctctggatcactgtgacggaatgggcacccatgataatccccttggcttggtggattggacagaataatcttcaggcaactgaaaggtgtatagtctgtcctcttgccttcctttccaaagctgtgacggatgttgtaagagtaacctttatcaaacttgtctggatccatctttcctttgataaattcttgcttccagaactgcaatgcctgttccaaagttaaaccaatgcccttcagaaataggccatactgcattcggcctccatgacgaagatggtgattttcccgcaaggctttatgtaactgacgcatgcaaggtgggaaggatttggtagaaagcaaatcaatctgatctaaagaaatcttcccaacatttccctgggtactgtaatcttggccagtgtaggaatgactgaggtgattgagcagaggctgaagtctttcatcagactgcacagcaggcaaggacctggctgttaatgccaaagccttggacagtttggctctaaattcattcaggatgattgccacaatgtccttaagtggtacgtaagcaaagccatcttccaaatagactttccttcctcgaaacaaatccagagcatcagcaaaagggatcttataaatggactcgaaccccaacttaagtccacttaaacttggtgatgaggcaacaatctcctgttctcgaagagtcttctcttcatcacttatagcctcaaactgcaattggctatcctttaagaaatcctgaattttatccttgggtaaaatactaaatctaaatcgaaggagatccatttcttgttgaatgaaccagcgtctaagttcttcagactggcaataagcaagccgcaaaataaaatgagaaatatgatctcttcttcgtggttcatattcatcttctaagttttctctgtaggaaaacttgagcttccgaagctcactctccaacttactctggtattgttcagttcctttcacatagctcactccaagattttcaactgattttaacaatttaactctatcaatagccaagttttcaaattctattaaagatatgttttcagaaggtggctgcaagtaaaactgaaggcaatgagggtaggaagcattcctctggtcacctgccaacctcagcttcctccactttcttccagaaaactccatcttggtcacctgcaagaattcaaactcgggaaaacacaaacggtggcagccactgttcccgggtggcgggagagttcatat

SEQ ID NO: 17159 - RNA, 1893 nt, Homo sapiens
  source 1..1893: mol_type = other RNA
tcaggccaggcacagtggctcacaaccgtaatcccagcactctgggacgctgaggtgtgaggatcgcttgagcccaggagtctgagatctgcctgggcaacatagggagaccccccacctctacaaaaaaaaattgaaaaaaattatctggatatgaggtgcacacctgtggtcctaactacttgggaggctgaggtaggaggatcacttgagctgggaaggtcaaggctgcaatcagctgtaattgtgtcactgcactaagccttggtgacagagtgaaaccctttttcaacaacaaaggcaaaatcttaaaaacaggaaacaggctattgaggaaaaagggttataaaactgcctaagaatcttcactaaagtaatcttctagtccttccatatccatttccagagaggaatttaaagaggccagagcagatgatgcatccttggttttctggacacttggtttgggttgaggagtttctggttggataggttccttctttatgtctttaccaccatttagaatacgttggctctcacaaaagaactgattaggatgattcaaagaaaagccacaatcatccacattgtgtatcatctcaaagtatttttgacaggctacctggtaatgtgtcccctttactaaatccaaaatctggcttatccctccaggagagatcttgtatgactgcaacttttgcttcagcagctctggatcactgtgacggaatgggcacccatgataatccccttggcttggtggattggacagaataatcttcaggcaactgaaaggtgtatagtctgtcctcttgccttcctttccaaagctgtgacggatgttgtaagagtaacctttatcaaacttgtctggatccatctttcctttgataaattcttgcttccagaactgcaatgcctgttccaaagttaaaccaatgcccttcagaaataggccatactgcattcggcctccatgacgaagatggtgattttcccgcaaggctttatgtaactgacgcatgcaaggtgggaaggatttggtagaaagcaaatcaatctgatctaaagaaatcttcccaacatttccctgggtactgtaatcttggccagtgtaggaatgatgccaaagccttggacagtttggctctaaattcattcaggatgattgccacaatgtccttaagtggtacgtaagcaaagccatcttccaaatagactttccttcctcgaaacaaatccagagcatcagcaaaagggatcttataaatggactcgaaccccaacttaagtccacttaaacttggtgatgaggcaacaatctcctgttctcgaagagtcttctcttcatcacttatagcctcaaactgcaattggctatcctttaagaaatcctgaattttatccttgggtaaaatactaaatctaaatcgaaggagatccatttcttgttgaatgaaccagcgtctaagttcttcagactggcaataagcaagccgcaaaataaaatgagaaatatgatctcttcttcgtggttcatattcatcttctaagttttctctgtaggaaaacttgagcttccgaagctcactctccaacttactctggtattgttcagttcctttcacatagctcactccaagattttcaactgattttaacaatttaactctatcaatagccaagttttcaaattctattaaagatatgttttcagaaggtggctgcaagtaaaactgaaggcaatgagggtaggaagcattcctctggtcacctgccaacctcagcttcctccactttcttccagaaaactccatcttggtcacctgcaagaattcaaactcgggaaaacacaaacggtggcagccactgttcccgggtggcgggagagtt

SEQ ID NO: 17160 - RNA, 1170 nt, Homo sapiens
  source 1..1170: mol_type = other RNA
tcaggccaggcacagtggctcacaactgtaatcccagcactctgggaggctgaggtgtgaggatcgcttgagtccaggagtctgagatctgcctgggcaacatagggagaccctcacctctacaaaaaaaaattgaaaaaaattagttggatatggggtacacacctgtggtcccaactacttgggaggctgaggtagcaggatcacctgagctgggaaggtcaaggctgcaatcagctgtaattgtgtcactgcactaagccttggtgacagagtgaaaccctttttcaacaacaaaggcaaaatcttaaaaacaggaaacaggctattgaggaaaatgggttagaaaactgcctaagaatcttcactaaagtaatcttctagtccttccatatccatttccagagaggaatttaaagaggccagagcagatgatgcatccttggttttctggacacttggtttgggttgaggagtttctggttggataggttccttctttatgtctttaccaccatttagaatactttggctctcacaaaagaactgattaggatgattcaaagaaaagccacaatcatccacattgtgtatcatctcaaagtatttttgacaggctacctggtaatgtgtcccctttactaaatccaaaatctggcttatccctccaggagagatcttgtatgactgcaacttttgcttcagcagctctggatcactgtgacggaatgggcacccatgataatccccttggcttggtggattggatagaataatcttcaggcaactgaaaggtgtatagtctgtcctcttgccttcctttccaaagctgtgacagatgttgtaagagcaacctttaccaaactccctgtaaccaaaaggttcactggcctccatctccttcagatgaagcccaggatcagccagtacctgttcccaagtgaggcttccctctcctttcttacaccattttaaaccagacaaatacccattgtgagaaaaacctctgaatatgctccagtctatccttgcaagggtcatgtccactcgcatcataattttaccatcaattcttttctgggaacaagcatttgtcattacacttctccagccatcattaaatgtaacataatgcctccaagccactacaggttcctggacatctctcat

SEQ ID NO: 17161 - RNA, 1061 nt, Homo sapiens
  source 1..1061: mol_type = other RNA
tcaggccaggcacagtggctcacaactgtaatcttagcactttgggaggccaagggttgggggatcacttgagcccaggagtttgagaccagtctgggcaacacagcaagaccccatccctacaaaaaatttaaaaattagccagacgtcttggcacatgcctgtagttgcagctactcaggagacaggtgggaggatcacttgagcccgggaggttgaagcttcaagtgagctgtgttcgagccactacgctccagcctgggcgaccctgtcatgtttcactgatgaaattagaaagatccaaaagtttgataatgttttattccaaggctttggggaaacaggatctctcacacgttgcaccatgcctgacacttctcatgtgctccacaaatcttcatttagaaaagtatctatggaatttattgaagaatttttttgacacctaaaagaggagaagagtctttgaagagctgcttaagcaaaaacccatctcttagaacaagtacagttgtcaaaagacattcactcatgccacctctagggtatgctttccttcattttacagttttctcatgttaaaaaaagaagacaaatactgcctttcaaatttgatgcgtaacatgtgagctagtcacgttgtttcccttgggtaatttttccaacattaactgctaacaacagggctgcaaattgctgtctcttcccccagggactagagaagatgagtaagtacctgaaagagactggccaaatacttacctagacagagtttaccatctgcagctgtagagaggttatttcccttacttccaactatatgcatcctgaatgacattttatttgcaccactgtttatttcagtttctaagacaagattaaggcatttacctccccactaaacaaacttaatgaacagcgtgaacactgtttcccaaatcattgtgtgactgaattactaatccctgacatttggcagttcttaagtcagaaggcaatttactgtagctagatgagaacatgaatatacattgcattagaaaactcagtggtacatgggg

SEQ ID NO: 17162 - RNA, 950 nt, Homo sapiens
  source 1..950: mol_type = other RNA
tcaggccaggcacagtggctcacacactttggaggctgagacaggtggatcacttgagcccggaagtttgagaccagcttaggcaacatggtgaaaccctatctctacaaaatacaaaaaattagccaggcgtggtggcacatgactgtagtcccagttattcaggaggcagaggtgggagaatcacctgagcccaggagctcgaggctgcagggagccatgatcgtgccactgcactccagcttggataacagaatgagacccttgctgcatccacaagagggagcctcgtgccagcttctccagccaggatggtagcccccaagactcttcctcttccatccacctttaggtgcagcatccaacaaggtcaaaatcacaatgtcttgcatgttttggagtcctctccagaggcagtgttcctcttcaatgttccatcccagattattgtctccttctctggcctcacccacatttctactttctttgatctcttcctgatcctcacagctgactacccagacgagctgaagtgcctggatgctccggtgctgacccaggctgagtgtaaagcctcctaccatagcgggagcccgactgcgacttgggaatcaagcccagcactgcacgctgcattttcatcttctttgcctttgtggtaggacgctgcagtgaatcccacagctaacaccagctccccactctgacctcagtcactggttctttcaaaatgccctttgtcctcaccatgccaccaagtttgccaacctttttttctacaggtagaagtatccacaaagggtggaacgagtcatgtagggagactgatagcttcctactttcagagacaaaattgaaacctgctcaagtggttaactctagctaaaggggtggtctcacagatgacaagtatcatctgaggcgagatcgtttctctgggtgggatgtat

SEQ ID NO: 17163 - RNA, 1939 nt, Homo sapiens
  source 1..1939: mol_type = other RNA
tcaggccaggcacagtggctcacaccaataatcccagcattttgggaggctgaagtggatggatcacttgaggtcaggatttcaagaccagcctggccaacatggcaaaaccccatctctactaaaaatacaaaaattagctgggcgtggtggcatgcacctggagtcccagctacttgggaggctaagacacgagaatagcttgaacccaggaggcagaggttgcagtgagccaagattgcaccactgcactccagcctggatggcagagccagaccctgtctccgaaaaaaaaaaaaaaaatcacacactaaccctcttctcttcctccctctcctggcttagccagtgcagtcaagtccttgaatggcgtgctccctggccctcaggagaggacattgcctatcgagtggagacttggtaaggaaattgttcccatttctaagatggagagttctggactctggaccttctattaggagtttacaggcctgtactgccacctccctgggccagagcttttgcagatattcctagagaacaggtaaaagcaatgagcttggggtaagagcttagaccaactgaaggctctctgcctccctcctcctctaagaggcctgccctggctgtgacaccaaaaagcgcactcgggcctctgtgcccaactctgccctttcaccatctgcccctgtcacaccaacgtcagcatgagttacacagttgtgttgccctttgtggctactctccccacacttactagaatgtgagccccatgcggcagcgatcttcatcctttttcttttcctctattccaagtacctagaatagtgcctggcaaaggcacttagtgcacaattagtgttttttaaaaaaaaaatgataggaagcaagcaggagatacatagcaagtacaagacattttcagtggcttgcagtcaaaagtgtcactgaggtccccccagctgcccctgccccggctggcccaaggatgagataggtggctgctctggggtcatgtcttgctttatagcctggcctgttgggtctccaggagccttttgagtcttgcctgtttgacagagaagactgaggcccagaggacggaagggatgggactggcacccagtgagcttttcccttcatcaagatgcttacacaggtgatgtccatcattcagcttgggtcaggtgcagaccatgcacgtggtggtggtgcgtgcgatggacatgaagtagctgaccctgtgtagagatgacatttcccatcgggtgtggaactgggagttcaaccctttggcttaccaccctaatctgcatccacactagagagtcacacagcccaggtagtatttggatttcaaccccgggaaagaatagcaacctgccgcttggtggcagcatgggagctggggtttagtgaggaggggaagcagttgtgtaggcatcagcagtcatagcaccaggccgaggcgagaccctccgagcggagtccggctggttaaagggcctgcacgggtctctcacagaagaaggaaagctggtcctgagggtggagccaggggaatctgggggccacttcagcattctttgttgccattggctttggttcagtaagctttgttgatttattttgttgttgttattgttgttagagtgatggggctgattgcttataagttctgaggttcttatttgcgtttccagctccctgggtattcattcatacctggtttctggctgtggtgaaatgtcttctgaccaagtgggttgataaacagggggcttcgctggagcgggggcagggggcgcggtcacaccctggcagtctcctcctcttggaagttttaactattcaagactcaatggccaggcgcggcggctcatgcctgtaatcccagcactttgggaagctgaggcaggaagatcacttgaggtcagga

SEQ ID NO: 17164 - RNA, 818 nt, Homo sapiens
  source 1..818: mol_type = other RNA
tcaggccaggcacagtggctcacacctataatcccaacactttggaaggacaagctgggaggatcacttgaggccaggagttggagaccagcctgggcaacataacaagacccaattttcttcttttttgtcaagcttgtcctgggcagggtctcagcactgtgcggatgtgcggctccttgcactattttgttctgcctttgaggcctctgctgaaatgtctgcgtgtccctctgcgctccgactggtgcgacttctccctgcgctagcgaggcagggttttggcctcgcctctcgcgagatcgcctcctgttgctgccgccgccgctcctggccactgactggcggcgcctgcgcagccgccatgttcggttgctatgctgcggcctaggagagggggtgtgcttgagggaggaggaagagatagaggaggaggagggggaggaagaggaggtggagaaggaggggggtgactgagctcctcttgcactctcacacacaaacgctgcccaggattacccgccagctcacgccgcgcagtgcgcttttccgctcctcgcgccccaccaccaacattgttctctcaggactcctgggtcccaggggccggaattgggcctgagcgggagaggaaagagacttggctttggccgcggggtcggaggattggggccaggccccctcccccacgcacttttgggggtgtggattatctcatccctgcagggaggtaggagaggtcgccggctgcccgcctccctgccacctccccagcggcgccggcccgcggctgcccagcagcatgaggtggtgctggc

SEQ ID NO: 17165 - RNA, 1208 nt, Homo sapiens
  source 1..1208: mol_type = other RNA
tcaggccaggcacagtggctcacacctatactcccagcattttgggaggctgaggcgggtggatcacctgaggtcaggagtttgagaccagcctggccaacatggtgaaaccctgtctctactaaaattacaaaaattagctgggtttggtggtgggcatctgtaatcccagctacttgggaggctgaggcaggagaatcacctgaacccaggaggcggaggttgcagtgagctgaggtcttgccattgcactccagcctgggcgacaagaatgaaactccatctcaaacaaacaaacaaaaaactaaccacatgctcgatgtttctgtgtcttccctgctggttagtgacatccaaggcaggccacatgagtaagaaccctctgagatcttccacccttcacttccctaacctggaatccagtcattctccaggttttggggctcccaactccaaatgttcattcctctttgtcccccacttccatgtgacactgcctgggtgtgtagcctcagcaccccttttgtcgaattggtctctggctctggggtttcctcgcttggtcctccacactgggtcagttctctcaatggccacctccttccttgcacaagatcaagtgcagactcctgacctgggtgctggagggcagtcctttccatcgcccccgttctcctcacccagattctcaggccacatgggcgggcttgccatggttatggttgactcgtgcgctgcccccatcttggtccatttgcattgctcatggtaccggcctgcaagccatttcctggggcctccccgtcgcctcttccagaaacaactcctggaactccccttggaggtcaggccaatgacctgtgccccgcattgccctccatcctctaagcttcccgtgggtagggacaattcccagttctgaagggctccccctgccccgggcctggctcttggcagaagcttaacaacagaccggccacgttcgtgtgacctgattctctccggctttcaggacgtcctgaggctgcacccacgtggcaatggtgtctgtcgcgctgtcgcctggatccggcaccactagcggagccgagcagagcccagggctccaacgcgtagggaaaaggctgcgccgctcccggggtggccccacgccccttctctgagcttgagcggcggcgcgggacggggacggctctggccgggaccag

SEQ ID NO: 17166 - RNA, 3051 nt, Homo sapiens
  source 1..3051: mol_type = other RNA
tcaggccaggcacagtggctcacacctctaatcccagcactttgaggggccaagatgggcagatcacttgaggtcaggagttcgagaccagcctggccgatacggtggaactctctccattaaaaacaaaaattagcggccaggcacggtggctcacgcctgtaatcccagcatttgggaggccaaggcaggcggatcacgaggtcaagagattgagacaatcctggcaaacatggtgaaaccccgtctctactaaaaatacaaaaattagctgggcatggtgacacgtgcctgtaatcccagctactcaggaggctgaggcaggagaatcacttgaacccgggaggcagaggttgcagtgagccgcgattgcgccactgcactccagcctggcgacagagagagactccatctcaagaaaaaaaaaaaaaaaattagctgggcgtggtggtgggcgcccgtaatcccagctacttgggagcttaaggctcgagaatcacttgaatccaggaggtggaggttgcagtgagctgacattgcaacaccactctagcctggcaaaagagtaagactccatctcaaaaaaaccccacaaaatttatattacttcctttttcagttttccctcgtaaaacttgtgaagtcattacatgtcagcaccaatttcattattaataaacaaaaaatatactctagttggaattaaactctcatcatcaatgtagttagacccatgcaattaatacctaatgccccttttctccactaactaatatggcatctaatttataataaaatattttaagtctcctgttatatttaaattgcatcaaatttaaattatgttaattataagactggcatgccaagccaaattatcacagaagattacatgaacaagcaatgttagtgatagatgctttttgttatccatcaaataattactaagttttctttttaaaaaaaatcagtgtttatgggcacacaattaaataccatttagaaaatccttaacttaggaccaggtcactggcttagttaaagtatatttatatttgatagtttccaaggtaaggttaccattggggaaattgtgataattaagtcaaacagttgtaccactgacctaaccagtacattaaggatttctaaatgtatcttattgtgtatttagcataagtggccatgctaatattatcaataccaaactgcagacaagattagttaagaactatgcagaaaacctgagcatcctacctttactttctatacattcgcattaccaattttttcttttcaaaacatcccttgcatcaagtgctactttctaacagctcttaagattctctgttcaccagaacaagcaacattaaagataacattggttcccatgttatatattcattactaatagcacttatcaaagctaaacctagataatattccttctttcctgacatactgctcagtggcaagtacacttcttctcaaccagcataggaaacctttcctttgggtcatttcccttctcaaaaaactttgcttaagggaaattggagctaaagagcttaccaacaaatagccctactagagttcaataaatatgctttgctattaagtctaatatacaaatatgatagaagtttgaaaatggaaccttatcccagtgctatattggcacgtaacatggctagtgatcatttcaaaaggagtcatgttatgttttgagtttgtttgtgataaacctattgtctaaacagatttattctttaagaatatacacaagaggttttcctccattattttcacacatcagatatggtgtttggttttttgaaggagggagggggtactatctacaacaaatacttcattcatagccataaaccatttgtatcttgggcttgagcccctggttaaatcaggaatgctcttcagcgctgctgctgaatgatctgctccggatgtgatttctcagttgctctataagttcaggattttgttgctgtatctgctgagcaaactgctgtcccgcttggatgaggcttgacaggtcagttaggcccccaactccagcagcaggtcccccaatggcatttgtcatcattcctgacattagctgttgaacttgagggttctgcattaaacttgccgccatactaatgaaggctggattatttatcaagctagccatgtcaaagctcagtccagttcctgtaggactggatacctctcttaacttctgttctgctattttcagatttgacttataggaatcattttcagggtcaagatctaatgccttttgataacttgtaactgcttcttcaaatttattcaaggcagtgagggccagccccattctcccataggccttgctgtactttgaatcaattgctattgctttttcacaatcctttatcgcatctgtgtagtgacctaatttgctctgagcagcagccctgttgcaatagtaaactgcattattgggatccaattctattgcctgtgtgtaacaatccactgcagcagcataattttcttctttcatgtggttattgccttcatcttttaattggtcagcttttcccacatcttcaggcactgagtttgaaaggggcagaacgtcattcttacagaaggaactggtaaacatttctgtcaaaggctgtgaaactgctaggtgtgtatcttctgggctgatcttaaaaactgtctccaagcactgaattgcaacttccaaactttcttgttcatccgaggtgtaagtgtccatctgactttgttcccgtaagaaacgaataactgcataaaccaggtgcttgatagatgacattttagaagcttaaacacttttccaagcaggaggacgcgagacgactgctgctggcccgcggggttccgtaggcaggcccgcccgacccctggtcctcggggctggagcccggctcgggatcgcagcactggtcgcggcggcgcaaacttccccggcccctaggccgtagaccccagaacccaccaggctgtgctctctctcaggcggcagggtct

SEQ ID NO: 17167 - RNA, 2923 nt, Homo sapiens
  source 1..2923: mol_type = other RNA
tcaggccaggcacagtggctcacacctctaatcccagcactttgaggggccaagatgggcagatcacttgaggtcaggagttcgagaccagcctggccgatacggtggaactctctccattaaaaacaaaaattagcggccaggcacggtggctcacgcctgtaatcccagcatttgggaggccaaggcaggcggatcacgaggtcaagagattgagacaatcctggcaaacatggtgaaaccccgtctctactaaaaatacaaaaattagctgggcatggtgacacgtgcctgtaatcccagctactcaggaggctgaggcaggagaatcacttgaacccgggaggcagaggttgcagtgagccgcgattgcgccactgcactccagcctggcgacagagagagactccatctcaagaaaaaaaaaaaaaaaattagctgggcgtggtggtgggcgcccgtaatcccagctacttgggagcttaaggctcgagaatcacttgaatccaggaggtggaggttgcagtgagctgacattgcaacaccactctagcctggcaaaagagtaagactccatctcaaaaaaaccccacaaaatttatattacttcctttttcagttttccctcgtaaaacttgtgaagtcattacatgtcagcaccaatttcattattaataaacaaaaaatatactctagttggaattaaactctcatcatcaatgtagttagacccatgcaattaatacctaatgccccttttctccactaactaatatggcatctaatttataataaaatattttaagtctcctgttatatttaaattgcatcaaatttaaattatgttaattataagactggcatgccaagccaaattatcacagaagattacatgaacaagcaatgttagtgatagatgctttttgttatccatcaaataattactaagttttctttttaaaaaaaatcagtgtttatgggcacacaattaaataccatttagaaaatccttaacttaggaccaggtcactggcttagttaaagtatatttatatttgatagtttccaaggtaaggttaccattggggaaattgtgataattaagtcaaacagttgtaccactgacctaaccagtacattaaggatttctaaatgtatcttattgtgtatttagcataagtggccatgctaatattatcaataccaaactgcagacaagattagttaagaactatgcagaaaacctgagcatcctacctttactttctatacattcgcattaccaattttttcttttcaaaacatcccttgcatcaagtgctactttctaacagctcttaagattctctgttcaccagaacaagcaacattaaagataacattggttcccatgttatatattcattactaatagcacttatcaaagctaaacctagataatattccttctttcctgacatactgctcagtggcaagtacacttcttctcaaccagcataggaaacctttcctttgggtcatttcccttctcaaaaaactttgcttaagggaaattggagctaaagagcttaccaacaaatagccctactagagttcaataaatatgctttgctattaagtctaatatacaaatatgatagaagtttgaaaatggaaccttatcccagtgctatattggcacgtaacatggctagtgatcatttcaaaaggagtcatgttatgttttgagtttgtttgtgataaacctattgtctaaacagatttattctttaagaatatacacaagaggttttcctccattattttcacacatcagatatggtgtttggttttttgaaggagggagggggtactatctacaacaaatacttcattcatagccataaaccatttgtatcttgggcttgagcccctggttaaatcaggaatgctcttcagcgctgctgctgaatgatctgctccggatgtgatttctcagttgctctataagttcaggattttgttgctgtatctgctgagcaaactgctgtcccgcttggatgaggcttgacaggtcagttaggcccccaactccagcagcaggtcccccaatggcatttgtcatcattcctgacattagctgttgaacttgagggttctgcattaaacttgccgccatactaatgaaggctggattatttatcaagctagccatgtcaaagctcagtccagttcctgtaggactggatacctctcttaacttctgttctgctattttcagatttgacttataggaatcattttcagggtcaagatctaatgccttttgataacttgtaactgcttcttcaaatttattcaaggcagtgagggccagccccattctcccataggccttgctgtactttgaatcaattgctattgctttttcacaatcctttatcgcatctgtgtagtgacctaatttgctctgagcagcagccctgttgcaatagtaaactgcattattgggatccaattctattgcctgtgtgtaacaatccactgcagcagcataattttcttctttcatgtggttattgccttcatcttttaattggtcagcttttcccacatcttcaggcactgagtttgaaaggggcagaacgtcattcttacagaaggaactggtaaacatttctgtcaaaggctgtgaaactgctaggtgtgtatcttctgggctgatcttaaaaactgtctccaagcactgaattgcaacttccaaactttcttgttcatccgaggtgtaagtgtccatctgactttgttcccgtaagaaacgaataactgcataaaccaggtgcttgatagatgacattttagaagcttaaacacttttcctgtcattaaaagtgccgcagctgtggactcagaacaattgtgtttgctcctcgcgcccattatt

SEQ ID NO: 17168 - RNA, 3192 nt, Homo sapiens
  source 1..3192: mol_type = other RNA
tcaggccaggcacagtggctcacacctctaatcccagcactttgaggggccaagatgggcagatcacttgaggtcaggagttcgagaccagcctggccgatacggtggaactctctccattaaaaacaaaaattagcggccaggcacggtggctcacgcctgtaatcccagcatttgggaggccaaggcaggcggatcacgaggtcaagagattgagacaatcctggcaaacatggtgaaaccccgtctctactaaaaatacaaaaattagctgggcatggtgacacgtgcctgtaatcccagctactcaggaggctgaggcaggagaatcacttgaacccgggaggcagaggttgcagtgagccgcgattgcgccactgcactccagcctggcgacagagagagactccatctcaagaaaaaaaaaaaaaaaattagctgggcgtggtggtgggcgcccgtaatcccagctacttgggagcttaaggctcgagaatcacttgaatccaggaggtggaggttgcagtgagctgacattgcaacaccactctagcctggcaaaagagtaagactccatctcaaaaaaaccccacaaaatttatattacttcctttttcagttttccctcgtaaaacttgtgaagtcattacatgtcagcaccaatttcattattaataaacaaaaaatatactctagttggaattaaactctcatcatcaatgtagttagacccatgcaattaatacctaatgccccttttctccactaactaatatggcatctaatttataataaaatattttaagtctcctgttatatttaaattgcatcaaatttaaattatgttaattataagactggcatgccaagccaaattatcacagaagattacatgaacaagcaatgttagtgatagatgctttttgttatccatcaaataattactaagttttctttttaaaaaaaatcagtgtttatgggcacacaattaaataccatttagaaaatccttaacttaggaccaggtcactggcttagttaaagtatatttatatttgatagtttccaaggtaaggttaccattggggaaattgtgataattaagtcaaacagttgtaccactgacctaaccagtacattaaggatttctaaatgtatcttattgtgtatttagcataagtggccatgctaatattatcaataccaaactgcagacaagattagttaagaactatgcagaaaacctgagcatcctacctttactttctatacattcgcattaccaattttttcttttcaaaacatcccttgcatcaagtgctactttctaacagctcttaagattctctgttcaccagaacaagcaacattaaagataacattggttcccatgttatatattcattactaatagcacttatcaaagctaaacctagataatattccttctttcctgacatactgctcagtggcaagtacacttcttctcaaccagcataggaaacctttcctttgggtcatttcccttctcaaaaaactttgcttaagggaaattggagctaaagagcttaccaacaaatagccctactagagttcaataaatatgctttgctattaagtctaatatacaaatatgatagaagtttgaaaatggaaccttatcccagtgctatattggcacgtaacatggctagtgatcatttcaaaaggagtcatgttatgttttgagtttgtttgtgataaacctattgtctaaacagatttattctttaagaatatacacaagaggttttcctccattattttcacacatcagatatggtgtttggttttttgaaggagggagggggtactatctacaacaaatacttcattcatagccataaaccatttgtatcttgggcttgagcccctggttaaatcaggaatgctcttcagcgctgctgctgaatgatctgctccggatgtgatttctcagttgctctataagttcaggattttgttgctgtatctgctgagcaaactgctgtcccgcttggatgaggcttgacaggtcagttaggcccccaactccagcagcaggtcccccaatggcatttgtcatcattcctgacattagctgttgaacttgagggttctgcattaaacttgccgccatactaatgaaggctggattatttatcaagctagccatgtcaaagctcagtccagttcctgtaggactggatacctctcttaacttctgttctgctattttcagatttgacttataggaatcattttcagggtcaagatctaatgccttttgataacttgtaactgcttcttcaaatttattcaaggcagtgagggccagccccattctcccataggccttgctgtactttgaatcaattgctattgctttttcacaatcctttatcgcatctgtgtagtgacctaatttgctctgagcagcagccctgttgcaatagtaaactgcattattgggatccaattctattgcctgtgtgtaacaatccactgcagcagcataattttcttctttcatgtggttattgccttccttatcttcatctctctcctcccttttagagctgccccagcccgttccagatgcaacaccctccctaatcaccatctcaatctggacctggtcttccactctttcccttcatcttttaattggtcagcttttcccacatcttcaggcactgagtttgaaaggggcagaacgtcattcttacagaaggaactggtaaacatttctgtcaaaggctgtgaaactgctaggtgtgtatcttctgggctgatcttaaaaactgtctccaagcactgaattgcaacttccaaactttcttgttcatccgaggtgtaagtgtccatctgactttgttcccgtaagaaacgaataactgcataaaccaggtgcttgatagatgacattttagaagcttaaacacttttccaagcaggaggacgcgagacgactgctgctggcccgcggggttccgtaggcaggcccgcccgacccctggtcctcggggctggagcccggctcgggatcgcagcactggtcgcggcggcgcaaacttccccggcccctaggccgtagaccccagaacccaccaggctgtgctctctctcaggcggcagggtctggccagcaccgcccctggggcggggccggac

SEQ ID NO: 17169 - RNA, 1529 nt, Homo sapiens
  source 1..1529: mol_type = other RNA
tcaggccaggcacagtggctcacacctgcaatcctagcactttggcaggcccaggcaggaggatcacttgagcccaggattttgagatgagcctgagccacatagcaagaccctggctcaattttttataataataaaattaaaggctgagcgtggtggctcacgcctgtaatcccagcactttgggagaccaaggcgggtggatcacgaggtcaggagtttgagaccagcctggccaatatggtgaaaccccgtctctactaaaaaaaaatacaaaaattagctgggtgtggtggcgcgctcctgtagtcccagctactcaggaagctgaggcaggggaattgcttgaacctgggaggcagaagttgcagtgagctgagatcatgccactgcactctagcctgggcgagagtaaaactccatctcaaaaataaaaaataaaataataataataataataaaaaaattaaaaaagaaaagctctggccttgactttcacagggctgctgtactgagccacccctatcttttccctatttctccagagtggcacagagcactggccctaagctggggctaggatcacctgtccccaaagcagcagaacgaaggttctgtatcacttggcagaaaatgaagcagaagggtcacagcaggctacactgggtaacctgaggtcttaggaacagagtatcaaccagtgagaagaggtggctcctctgtcctccagcacataagggttagggaaagacagaaccaccaatgactgctgcagggtctgctggccagcatcctcagcacttttctgtggtccagttctggaatggcaggtgacagggcacatacaaggcctctgctccactgtcattgtcaactcatctcagctctgattcatttgttcacctcgaatcaacaacaggggcactggctttacccaatacttatcagctggtgcccactgcgctgtcaggcagtgagatttctggctgacttggaggcgctctgggcccgctgaacaatggcagaacacttctcacgtcgcagcagcttgttgttctcaaagagaccttcattgcgggggattccatgagaaccatcagggaaagtcagcaggccaaaaccatctactctgccatttttaaattccccctcaaaggtcatgttgtcatatcgaatgaagactccgacgccattaaacttgccctgggcaaactccccctcataccttgaaccatctgagaaggtcaataccccaaagccattaaagagcccattctcaaaatgacccaggtaggtgccaccatctgcaaacatcagttgaccaaaaccatgcctgcggccctccttccactcgccacgatattcctccccactggagtaggtgaaggaaccttttgtcagggtcatggtgacagattacaggataaaaggatgaaactgcgcccgaagcaacagtgaccatcaacgcgagcggctctgatcttgctccagtccccactgctgtcaagggccccgccgcggagtttaag

SEQ ID NO: 17170 - RNA, 1589 nt, Homo sapiens
  source 1..1589: mol_type = other RNA
tcaggccaggcacagtggctcacacctgcaatcctagcactttggcaggcccaggcaggaggatcacttgagcccaggattttgagatgagcctgagccacatagcaagaccctggctcaattttttataataataaaattaaaggctgagcgtggtggctcacgcctgtaatcccagcactttgggagaccaaggcgggtggatcacgaggtcaggagtttgagaccagcctggccaatatggtgaaaccccgtctctactaaaaaaaaatacaaaaattagctgggtgtggtggcgcgctcctgtagtcccagctactcaggaagctgaggcaggggaattgcttgaacctgggaggcagaagttgcagtgagctgagatcatgccactgcactctagcctgggcgagagtaaaactccatctcaaaaataaaaaataaaataataataataataataaaaaaattaaaaaagaaaagctctggccttgactttcacagggctgctgtactgagccacccctatcttttccctatttctccagagtggcacagagcactggccctaagctggggctaggatcacctgtccccaaagcagcagaacgaaggttctgtatcacttggcagaaaatgaagcagaagggtcacagcaggctacactgggtaacctgaggtcttaggaacagagtatcaaccagtgagaagaggtggctcctctgtcctccagcacataagggttagggaaagacagaaccaccaatgactgctgcagggtctgctggccagcatcctcagcacttttctgtggtccagttctggaatggcaggtgacagggcacatacaaggcctctgctccactgtcattgtcaactcatctcagctctgattcatttgttcacctcgaatcaacaacaggggcactggctttacccaatacttatcagctggtgcccactgcgctgtcaggcagtgagatttctggctgacttggaggcgctctgggcccgctgaacaatggcagaacacttctcacgtcgcagcagcttgttgttctcaaagagaccttcattgcgggggattccatgagaaccatcagggaaagtcagcaggccaaaaccatctactctgccatttttaaattccccctcaaaggtcatgttgtcatatcgaatgaagactccgacgccattaaacttgccctgggcaaactccccctcataccttgaaccatctgagaaggtcaataccccaaagccattaaagagcccattctcaaaatgacccaggtaggtgccaccatctgcaaacatcagttgaccaaaaccatgcctgcggccctccttccactcgccacgatattcctccccactggagtaggtgaaggaaccttttgtcagggtcatggtgacagattacaggataaaaggatgaaactggccaggcgcagtggctcacatctgtaatcccagcacttcgggaggccgcggcttgagctcaggagtgcgggaggcttgagcccaagagttctagatcagcctgggcaacgcagggagactccgtatctacagaagaaaaaaattaccca

SEQ ID NO: 17171 - RNA, 1591 nt, Homo sapiens
  source 1..1591: mol_type = other RNA
tcaggccaggcacagtggctcacacctgcaatcctagcactttggcaggcccaggcaggaggatcacttgagcccaggattttgagatgagcctgagccacatagcaagaccctggctcaattttttataataataaaattaaaggctgagcgtggtggctcacgcctgtaatcccagcactttgggagaccaaggcgggtggatcacgaggtcaggagtttgagaccagcctggccaatatggtgaaaccccgtctctactaaaaaaaaatacaaaaattagctgggtgtggtggcgcgctcctgtagtcccagctactcaggaagctgaggcaggggaattgcttgaacctgggaggcagaagttgcagtgagctgagatcatgccactgcactctagcctgggcgagagtaaaactccatctcaaaaataaaaaataaaataataataataataataaaaaaattaaaaaagaaaagctctggccttgactttcacagggctgctgtactgagccacccctatcttttccctatttctccagagtggcacagagcactggccctaagctggggctaggatcacctgtccccaaagcagcagaacgaaggttctgtatcacttggcagaaaatgaagcagaagggtcacagcaggctacactgggtaacctgaggtcttaggaacagagtatcaaccagtgagaagaggtggctcctctgtcctccagcacataagggttagggaaagacagaaccaccaatgactgctgcagggtctgctggccagcatcctcagcacttttctgtggtccagttctggaatggcaggtgacagggcacatacaaggcctctgctccactgtcattgtcaactcatctcagctctgattcatttgttcacctcgaatcaacaacaggggcactggctttacccaatacttatcagctggtgcccactgcgctgtcaggcagtgagatttctggctgacttggaggcgctctgggcccgctgaacaatggcagaacacttctcacgtcgcagcagcttgttgttctcaaagagaccttcattgcgggggattccatgagaaccatcagggaaagtcagcaggccaaaaccatctactctgccatttttaaattccccctcaaaggtcatgttgtcatatcgaatgaagactccgacgccattaaacttgccctgggcaaactccccctcataccttgaaccatctgagaaggtcaataccccaaagccattaaagagcccattctcaaaatgacccaggtaggtgccaccatctgcaaacatcagttgaccaaaaccatgcctgcggccctccttccactcgccacgatattcctccccactggagtaggtgaaggaaccttttgtcagggtcatggtgacagattacaggataaaaggatgaaactggggccggcctttcgggatgaccgtcacgcctggacgcagggttccagcgcctcggacttttcctctgatgggctcccggctgccaccttgctctccgccacctccaccagcgattgccccacttgacgccgccatcctgggcgaccgcact

SEQ ID NO: 17172 - RNA, 1712 nt, Homo sapiens
  source 1..1712: mol_type = other RNA
tcaggccaggcacagtggctcacacctgcaatcctagcactttggcaggcccaggcaggaggatcacttgagcccaggattttgagatgagcctgagccacatagcaagaccctggctcaattttttataataataaaattaaaggctgagcgtggtggctcacgcctgtaatcccagcactttgggagaccaaggcgggtggatcacgaggtcaggagtttgagaccagcctggccaatatggtgaaaccccgtctctactaaaaaaaaatacaaaaattagctgggtgtggtggcgcgctcctgtagtcccagctactcaggaagctgaggcaggggaattgcttgaacctgggaggcagaagttgcagtgagctgagatcatgccactgcactctagcctgggcgagagtaaaactccatctcaaaaataaaaaataaaataataataataataataaaaaaattaaaaaagaaaagctctggccttgactttcacagggctgctgtactgagccacccctatcttttccctatttctccagagtggcacagagcactggccctaagctggggctaggatcacctgtccccaaagcagcagaacgaaggttctgtatcacttggcagaaaatgaagcagaagggtcacagcaggctacactgggtaacctgaggtcttaggaacagagtatcaaccagtgagaagaggtggctcctctgtcctccagcacataagggttagggaaagacagaaccaccaatgactgctgcagggtctgctggccagcatcctcagcacttttctgtggtccagttctggaatggcaggtgacagggcacatacaaggcctctgctccactgtcattgtcaactcatctcagctctgattcatttgttcacctcgaatcaacaacaggggcactggctttacccaatacttatcagctggtgcccactgcgctgtcaggcagtgagatttctggctgacttggaggcgctctgggcccgctgaacaatggcagaacacttctcacgtcgcagcagcttgttgttctcaaagagaccttcattgcgggggattccatgagaaccatcagggaaagtcagcaggccaaaaccatctactctgccatttttaaattccccctcaaaggtcatgttgtcatatcgaatgaagactccgacgccattaaacttgccctgggcaaactccccctcataccttgaaccatctgagaaggtcaataccccaaagccattaaagagcccattctcaaaatgacccaggtaggtgccaccatctgcaaacatcagttgaccaaaaccatgcctgcggcctggggccggcctttcgggatgaccgtcacgcctggacgcagggttccagcgcctcggacttttcctctgatgggctcccggctgccaccttgctctccgccacctccaccagcgattgccccacttgacgccgccatcctgggcgaccgcactgggtacaattcccgctgcccattggctgttacctaggcaaccgggagcaacgccactccgcattggcccagcccggctccacgccatctttgtgcggggccgagtgtttgcgaacccgggctgactatgtgaaagaggggtggtcccacctctgcaacgcagataaagacagaggatccagatctggcctacccagaggccgtctagttgaaatggca

SEQ ID NO: 17173 - RNA, 36 nt, Homo sapiens
  source 1..36: mol_type = other RNA
tcaggccaggcacagtggctcacacctgtaaaccca

SEQ ID NO: 17174 - RNA, 32 nt, Homo sapiens
  source 1..32: mol_type = other RNA
tcaggccaggcacagtggctcacacctgtaat

SEQ ID NO: 17175 - RNA, 2365 nt, Homo sapiens
  source 1..2365: mol_type = other RNA
tcaggccaggcacagtggctcacacctgtaatcccaacactttcggaggccgaggcaggcagatcatttgaagtcaggagttcaagaccagcctgggcaacatggtgaaaccccatctcgactaaaaatacaaaaattagctgggtgtggtggtgcatgcctgtaatcccagctacttgggaggcagaggcaggagaatcacttgaacctgggaggcagaggttgcagtgagccaaaatcatgccactgcattctagcctaaacaacagagcgagactcaaaaaaaaaaaaaaaaaaatcatagacacagtgacaatggaaatgtttattgctggtggttgggtctgtcatttcctagaggacatagctggccagcagattttcatttcttttttacaaaataaacaaatgcctactttattatttatacacagaaaattatatagaaacaccacacaaactgcttgaaatacaaatattctttggtttacttatcaaagtaaaaaataacaaaaatcttatcagttaaataaaaaagtgacattctttatcaagccttcttaaacactgaaacgcacgcatttttatgctcatgttctttagcagtatttctccccttttgcccctcattcccctaaattgtttcaatgagttcatctgtagaatgaagattgttacctttcttaatgctacttactttttattatctcaatatcaagaccaatctagacttttttgtctcttacatgtgaaatggatgtaaaaaatggaaaattcaccagcactttttaagataacataaaagaagccctaagcaagcatttcaaggcaatgacacaccattacatttctgagaaatttaagtatcattggtacttaaaaggagaactcaattccagaagcatattcttatactggacattattcataatagctaatatagttcatttccacagtactgatttcagataagccattttttttttcctgagggttgactacctcagacttaaatcctgaatgtcgatgactcaatcttaacaaaacagtcagctgtagacatgaaaattgaattgtttcaaaaggagcaatgatagcaagagaaagttcttggcattttaagaaaagtacatatacatagcaagaaatgaaagtaaatcaaaatacatagctttgtacatgttagaaatatccaatgtgccaccaacacaacaactgccctattaaaaagtcctcaggtctggagacatctgtatttttctttgtataactacatttgcattacccaaccacatatctctcccatggtctgttacccgttaggaagcttttaaccagaatttttggcaatatgcttttcttcaaataaaacaagccttcaaataaatcattatgtctgacaactgaattgggtaaagtctttctgaaatatgtgtaatctttagaaaattcttcttttttccttcataaatcagcagtgctccatcttcaaataaatcatgatcagtcacaatcttaactcatgtgctcatatgttctcttcatccaacattttgttgataccatcacatagtttttgtaagtggggtttaaaattcccaaaaggattatacaaggcagccaaaaattcacaatctgaaaaatgatcaaacacattattaacccgtccatgtgacttggcagtgaggtggcgctgaatgatttggtgcagcatctctctgcattcatttaacagcctggataacacattccggtcaaaggtataatccacctgatggaaactgaccacggtcatagcaagctgatgaactttcttcttaaatttctccatcaatgctagctcatcttgattaaactgattattcctataaagaatggccagcttgatgactgtcttgatgaggttcttgatgatcttctctgcctccttcttgttttgggtgtactccctggtcactctgtagagctcatccagcacctcactacttgtgtcgtctattaaggtggtggcgatggatttggacaccattttacccaagatcttcttttgtgcctgaacggccaggtttttggaattaaagacatctgtggccactgtggttccagctactcaggagactgaggtgggaggatcgcttgagcccaggagttagaggctgcagtgagctatgatctcaccactgcacttcagcctgggtgacacaggaagatcctgttcggaggagtggcgcgacggcgccgggacgctgaagcgcgagctgggctgtttggcggcgccgagttctctgctctctcggtggctcacgggttcccgcggaccttagccaagcgcgggttagagccggcgggagaaaaggaggcagag

SEQ ID NO: 17176 - RNA, 2361 nt, Homo sapiens
  source 1..2361: mol_type = other RNA
tcaggccaggcacagtggctcacacctgtaatcccaacactttcggaggccgaggcaggcagatcatttgaagtcaggagttcaagaccagcctgggcaacatggtgaaaccccatctcgactaaaaatacaaaaattagctgggtgtggtggtgcatgcctgtaatcccagctacttgggaggcagaggcaggagaatcacttgaacctgggaggcagaggttgcagtgagccaaaatcatgccactgcattctagcctaaacaacagagcgagactcaaaaaaaaaaaaaaaaaaatcatagacacagtgacaatggaaatgtttattgctggtggttgggtctgtcatttcctagaggacatagctggccagcagattttcatttcttttttacaaaataaacaaatgcctactttattatttatacacagaaaattatatagaaacaccacacaaactgcttgaaatacaaatattctttggtttacttatcaaagtaaaaaataacaaaaatcttatcagttaaataaaaaagtgacattctttatcaagccttcttaaacactgaaacgcacgcatttttatgctcatgttctttagcagtatttctccccttttgcccctcattcccctaaattgtttcaatgagttcatctgtagaatgaagattgttacctttcttaatgctacttactttttattatctcaatatcaagaccaatctagacttttttgtctcttacatgtgaaatggatgtaaaaaatggaaaattcaccagcactttttaagataacataaaagaagccctaagcaagcatttcaaggcaatgacacaccattacatttctgagaaatttaagtatcattggtacttaaaaggagaactcaattccagaagcatattcttatactggacattattcataatagctaatatagttcatttccacagtactgatttcagataagccattttttttttcctgagggttgactacctcagacttaaatcctgaatgtcgatgactcaatcttaacaaaacagtcagctgtagacatgaaaattgaattgtttcaaaaggagcaatgatagcaagagaaagttcttggcattttaagaaaagtacatatacatagcaagaaatgaaagtaaatcaaaatacatagctttgtacatgttagaaatatccaatgtgccaccaacacaacaactgccctattaaaaagtcctcaggtctggagacatctgtatttttctttgtataactacatttgcattacccaaccacatatctctcccatggtctgttacccgttaggaagcttttaaccagaatttttggcaatatgcttttcttcaaataaaacaagccttcaaataaatcattatgtctgacaactgaattgggtaaagtctttctgaaatatgtgtaatctttagaaaattcttcttttttccttcataaatcagcagtgctccatcttcaaataaatcatgatcagtcacaatcttaactcatgtgctcatatgttctcttcatccaacattttgttgataccatcacatagtttttgtaagtggggtttaaaattcccaaaaggattatacaaggcagccaaaaattcacaatctgaaaaatgatcaaacacattattaacccgtccatgtgacttggcagtgaggtggcgctgaatgatttggtgcagcatctctctgcattcatttaacagcctggataacacattccggtcaaaggtataatccacctgatggaaactgaccacggtcatagcaagctgatgaactttcttcttaaatttctccatcaatgctagctcatcttgattaaactgattattcctataaagaatggccagcttgatgactgtcttgatgaggttcttgatgatcttctctgcctccttcttgttttgggtgtactccctggtcactctgtagagctcatccagcacctcactacttgtgtcgtctattaaggtggtggcgatggatttggacaccattttacccaagatcttcttttgtgcctgaacggccaggtttttggaattaaagacatctgtggccactgtggttccagctactcaggagactgaggtgggaggatcgcttgagcccaggagttagaggctgcagtgagctatgatctcaccactgcacttcagcctgggtgacacaggaagatctcggaggagtggcgcgacggcgccgggacgctgaagcgcgagctgggctgtttggcggcgccgagttctctgctctctcggtggctcacgggttcccgcggaccttagccaagcgcgggttagagccggcgggagaaaaggaggcagag

SEQ ID NO: 17177 - RNA, 2197 nt, Homo sapiens
  source 1..2197: mol_type = other RNA
tcaggccaggcacagtggctcacacctgtaatcccaacactttcggaggccgaggcaggcagatcatttgaagtcaggagttcaagaccagcctgggcaacatggtgaaaccccatctcgactaaaaatacaaaaattagctgggtgtggtggtgcatgcctgtaatcccagctacttgggaggcagaggcaggagaatcacttgaacctgggaggcagaggttgcagtgagccaaaatcatgccactgcattctagcctaaacaacagagcgagactcaaaaaaaaaaaaaaaaaaatcatagacacagtgacaatggaaatgtttattgctggtggttgggtctgtcatttcctagaggacatagctggccagcagattttcatttcttttttacaaaataaacaaatgcctactttattatttatacacagaaaattatatagaaacaccacacaaactgcttgaaatacaaatattctttggtttacttatcaaagtaaaaaataacaaaaatcttatcagttaaataaaaaagtgacattctttatcaagccttcttaaacactgaaacgcacgcatttttatgctcatgttctttagcagtatttctccccttttgcccctcattcccctaaattgtttcaatgagttcatctgtagaatgaagattgttacctttcttaatgctacttactttttattatctcaatatcaagaccaatctagacttttttgtctcttacatgtgaaatggatgtaaaaaatggaaaattcaccagcactttttaagataacataaaagaagccctaagcaagcatttcaaggcaatgacacaccattacatttctgagaaatttaagtatcattggtacttaaaaggagaactcaattccagaagcatattcttatactggacattattcataatagctaatatagttcatttccacagtactgatttcagataagccattttttttttcctgagggttgactacctcagacttaaatcctgaatgtcgatgactcaatcttaacaaaacagtcagctgtagacatgaaaattgaattgtttcaaaaggagcaatgatagcaagagaaagttcttggcattttaagaaaagtacatatacatagcaagaaatgaaagtaaatcaaaatacatagctttgtacatgttagaaatatccaatgtgccaccaacacaacaactgccctattaaaaagtcctcaggtctggagacatctgtatttttctttgtataactacatttgcattacccaaccacatatctctcccatggtctgttacccgttaggaagcttttaaccagaatttttggcaatatgcttttcttcaaataaaacaagccttcaaataaatcattatgtctgacaactgaattgggtaaagtctttctgaaatatgtgtaatctttagaaaattcttcttttttccttcataaatcagcagtgctccatcttcaaataaatcatgatcagtcacaatcttaactcatgtgctcatatgttctcttcatccaacattttgttgataccatcacatagtttttgtaagtggggtttaaaattcccaaaaggattatacaaggcagccaaaaattcacaatctgaaaaatgatcaaacacattattaacccgtccatgtgacttggcagtgaggtggcgctgaatgatttggtgcagcatctctctgcattcatttaacagcctggataacacattccggtcaaaggtataatccacctgatggaaactgaccacggtcatagcaagctgatgaactttcttcttaaatttctccatcaatgctagctcatcttgattaaactgattattcctataaagaatggccagcttgatgactgtcttgatgaggttcttgatgatcttctctgcctccttcttgttttgggtgtactccctggtcactctgtagagctcatccagcacctcactacttgtgtcgtctattaaggtggtggcgatggatttggacaccattttacccaagatcttcttttgtgcctgaacggccaggtttttggaattaaagacatctgtggccacttccttggattcttctgcttcggagtgcataatgtcaggataaccagctgcaggggcgattaccgctcacatgtactcggacgagccgcaagttcgctctgc

SEQ ID NO: 17178 - RNA, 2813 nt, Homo sapiens
  source 1..2813: mol_type = other RNA
tcaggccaggcacagtggctcacacctgtaatcccaacactttcggaggccgaggcaggcagatcatttgaagtcaggagttcaagaccagcctgggcaacatggtgaaaccccatctcgactaaaaatacaaaaattagctgggtgtggtggtgcatgcctgtaatcccagctacttgggaggcagaggcaggagaatcacttgaacctgggaggcagaggttgcagtgagccaaaatcatgccactgcattctagcctaaacaacagagcgagactcaaaaaaaaaaaaaaaaaaatcatagacacagtgacaatggaaatgtttattgctggtggttgggtctgtcatttcctagaggacatagctggccagcagattttcatttcttttttacaaaataaacaaatgcctactttattatttatacacagaaaattatatagaaacaccacacaaactgcttgaaatacaaatattctttggtttacttatcaaagtaaaaaataacaaaaatcttatcagttaaataaaaaagtgacattctttatcaagccttcttaaacactgaaacgcacgcatttttatgctcatgttctttagcagtatttctccccttttgcccctcattcccctaaattgtttcaatgagttcatctgtagaatgaagattgttacctttcttaatgctacttactttttattatctcaatatcaagaccaatctagacttttttgtctcttacatgtgaaatggatgtaaaaaatggaaaattcaccagcactttttaagataacataaaagaagccctaagcaagcatttcaaggcaatgacacaccattacatttctgagaaatttaagtatcattggtacttaaaaggagaactcaattccagaagcatattcttatactggacattattcataatagctaatatagttcatttccacagtactgatttcagataagccattttttttttcctgagggttgactacctcagacttaaatcctgaatgtcgatgactcaatcttaacaaaacagtcagctgtagacatgaaaattgaattgtttcaaaaggagcaatgatagcaagagaaagttcttggcattttaagaaaagtacatatacatagcaagaaatgaaagtaaatcaaaatacatagctttgtacatgttagaaatatccaatgtgccaccaacacaacaactgccctattaaaaagtcctcaggtctggagacatctgtatttttctttgtataactacatttgcattacccaaccacatatctctcccatggtctgttacccgttaggaagcttttaaccagaatttttggcaatatgcttttcttcaaataaaacaagccttcaaataaatcattatgtctgacaactgaattgggtaaagtctttctgaaatatgtgtaatctttagaaaattcttcttttttccttcataaatcagcagtgctccatcttcaaataaatcatgatcagtcacaatcttaactcatgtgctcatatgttctcttcatccaacattttgttgataccatcacatagtttttgtaagtggggtttaaaattcccaaaaggattatacaaggcagccaaaaattcacaatctgaaaaatgatcaaacacattattaacccgtccatgtgacttggcagtgaggtggcgctgaatgatttggtgcagcatctctctgcattcatttaacagcctggataacacattccggtcaaaggtataatccacctgatggaaactgaccacggtcatagcaagctgatgaactttcttcttaaatttctccatcaatgctagctcatcttgattaaactgattattcctataaagaatggccagcttgatgactgtcttgatgaggttcttgatgatcttctctgcctccttcttgttttgggtgtactccctggtcactctgtagagctcatccagcacctcactacttgtgtcgtctattaaggtggtggcgatggatttggacaccattttacccaagatcttcttttgtgcctgaacggccaggtttttggaattaaagacatctgtggccacttccttggattcttctgcttcggagtgcataatgtcaggataaccagctgcaggggcgattaccgctcacatgtactcggacgagccgcaagttcgctctttgcacagcaaaagcagacggggctgcttactcattcagtatagccccgggcgagcactggtactccaagcacagcccgggcactcattgctgcagttactccaaagggccttcctcagggggagagcacggttccctcccggctaccagcaaaaactggggatgaattccttcaaaatgccaaaggggaggttttcaggatttgaaatgctgatagaataaagaagccggacagccttcacaacagatctcaattctgcccccgggtctggcccacaggcccctacaaattggctgagaggaagtccccttagctctgtggagccttggttttcccttctgcaaagcggggacaagagctgccactgataggcctgtcttacggaggtattttgtagaacacttgttttatcgccagtctgaggcaaaaagtcctcaaataacatatctgaaagatccgcttggaaattatgagaaaaaaatatactcttttgacaaatttattttccagttcgtttctttttcttcgtttccgattttatataggcaaaaaccaatagaaacactatggcaaatttagtgaaaagaacgtacaaaagacatggatttaaggagtct

SEQ ID NO: 17179 - RNA, 2243 nt, Homo sapiens
  source 1..2243: mol_type = other RNA
tcaggccaggcacagtggctcacacctgtaatcccaacactttcggaggccgaggcaggcagatcatttgaagtcaggagttcaagaccagcctgggcaacatggtgaaaccccatctcgactaaaaatacaaaaattagctgggtgtggtggtgcatgcctgtaatcccagctacttgggaggcagaggcaggagaatcacttgaacctgggaggcagaggttgcagtgagccaaaatcatgccactgcattctagcctaaacaacagagcgagactcaaaaaaaaaaaaaaaaaaatcatagacacagtgacaatggaaatgtttattgctggtggttgggtctgtcatttcctagaggacatagctggccagcagattttcatttcttttttacaaaataaacaaatgcctactttattatttatacacagaaaattatatagaaacaccacacaaactgcttgaaatacaaatattctttggtttacttatcaaagtaaaaaataacaaaaatcttatcagttaaataaaaaagtgacattctttatcaagccttcttaaacactgaaacgcacgcatttttatgctcatgttctttagcagtatttctccccttttgcccctcattcccctaaattgtttcaatgagttcatctgtagaatgaagattgttacctttcttaatgctacttactttttattatctcaatatcaagaccaatctagacttttttgtctcttacatgtgaaatggatgtaaaaaatggaaaattcaccagcactttttaagataacataaaagaagccctaagcaagcatttcaaggcaatgacacaccattacatttctgagaaatttaagtatcattggtacttaaaaggagaactcaattccagaagcatattcttatactggacattattcataatagctaatatagttcatttccacagtactgatttcagataagccattttttttttcctgagggttgactacctcagacttaaatcctgaatgtcgatgactcaatcttaacaaaacagtcagctgtagacatgaaaattgaattgtttcaaaaggagcaatgatagcaagagaaagttcttggcattttaagaaaagtacatatacatagcaagaaatgaaagtaaatcaaaatacatagctttgtacatgttagaaatatccaatgtgccaccaacacaacaactgccctattaaaaagtcctcaggtctggagacatctgtatttttctttgtataactacatttgcattacccaaccacatatctctcccatggtctgttacccgttaggaagcttttaaccagaatttttggcaatatgcttttcttcaaataaaacaagccttcaaataaatcattatgtctgacaactgaattgggtaaagtctttctgaaatatgtgtaatctttagaaaattcttcttttttccttcataaatcagcagtgctccatcttcaaataaatcatgatcagtcacaatcttaactcatgtgctcatatgttctcttcatccaacattttgttgataccatcacatagtttttgtaagtggggtttaaaattcccaaaaggattatacaaggcagccaaaaattcacaatctgaaaaatgatcaaacacattattaacccgtccatgtgacttggcagtgaggtggcgctgaatgatttggtgcagcatctctctgcattcatttaacagcctggataacacattccggtcaaaggtataatccacctgatggaaactgaccacggtcatagcaagctgatgaactttcttcttaaatttctccatcaatgctagctcatcttgattaaactgattattcctataaagaatggccagcttgatgactgtcttgatgaggttcttgatgatcttctctgcctccttcttgttttgggtgtactccctggtcactctgtagagctcatccagcacctcactacttgtgtcgtctattaaggtggtggcgatggatttggacaccattttacccaagatcttcttttgtgcctgaacggccaggtttttggaattaaagacatctgtggccatcggaggagtggcgcgacggcgccgggacgctgaagcgcgagctgggctgtttggcggcgccgagttctctgctctctcggtggctcacgggttcccgcggaccttagccaagcgcgggttagagccggcgggagaaaaggaggcagag

SEQ ID NO: 17180 - RNA, 2936 nt, Homo sapiens
  source 1..2936: mol_type = other RNA
tcaggccaggcacagtggctcacacctgtaatcccaacactttgggaggctgaggcgagaggatcacctgaggtcaggagttcgagaccagccgggccaccatgctgaaaccccatctctactaaaaaaaaaaaaaaaaaaagccatacgtggtggtgcacgcctgtagtcccagctactaaagaggttgaggcaggagaatcgcttgaatctgggaggcagaggctgcagtgagccaagatcgtgccactgcactccagcttgggtgacagagtgagaatctgtctcaaaaaaaaaaaaacgggcaaataaaacacaaaacttttagaatccagggctttaccttctaattggtcaacatataattgcataaccaaattcttacgggcaaatcaggtcttttagagaagaaaaaaaataaagtttaattcagtggaattaacatggttggaaaaatgatttgtttgggcagagtcccagagctaacagtaataaacataatacttaactttaaaaatgcttgaacttttctccaaagaacatatttccaccatcaggggaagtgttgattttcatattattcaagctatcttttatccctctaaatatgaacattttgcaagtagtgtggctactcatttcctgataatagacatattctaatagctagacacggaagtattttctaaaatgccacatttgctatctagagacacaaccactgaaaggaagtctgctaattaagaccccaagatgactatcattttataaactaacagacctactttcatcataaattaggccaggcgcggtggctcatgcctgtaatcccagcattttgggaggccaaggcgggcggatcaccttaggtcaggagtttgagaccagcttggctaacatggcaaaaccctgtctctactaaaaatacaaaaaatagccaggcgtggtggtgggcgcctgtaatcccagctactcgggtcggggaggcaaaggaattgcttgaacccaggaggtggaggttgcagtgagccgagatcgcgccaccgtactccagcctgggcaacagggtgagactgtctcaaaaattaattaattaattagtttttcattttactaagaggctcagcagagttttcaatcccctacttcatttaaaatacaaacccaaaatatcaaaatttgaaacttgttgagattttccatgtagtgtaaaatgaccagtgactgtgcttcactctggatatgctggactcactgcaccaggagatccctccatgttttcaatccgaggaaactgcaggcatctaggtctgagacagaatacaacagcagaaacagccttcagtgacggacattcctgtggctaaatgactgctgaatggccctgctgctctctcaaggctaagacatcgaagctgaagacaacgcttcgtggccaggacgcttgtgagacctacgcttcgccatctgtgtggtgttgccatttcattttcatcaggcctgtggtactgcacaggcagcgaatatgactctgatcactccacagctcaaaaaaggcagacagacaggtcacccatagctggaactggagctgtcatcagcttcatctgccctcttcaaaacttgacggggtttgaagctggcccattaagaatgatcaaaatatagtccttcaggtagtgaggttgtagggatcaaatggcagaatgtccggaagcgcaggtcatagcagtggcttttggattaggagcctgactaactgtgagacatgaggctcatcactgcacttttagtgttggtctcctcctgttgtaaatggaaccaatagtggctgccttgaaagagcaaaggccaccacgcagatgaaccccgaaactcagctgtggtcagtgtacctctcccggccattagcaggggctgccctggtggcgtctcacgacaagaatgtatcatagtggtttacaactgcttcctagcatttccagttgcctaaactgtgaatttttctaattcaattttgtatgtccctctcaccacttatccctcttctcccaagtctagcactgtacacagcacatagaagagccttaataaatgtttggtgaatgaaatatatgagtgaatgactaacacagagaatttgtaaaatggaagtactactgtagctacgaaaaactgctctggaaacgatcattcaaaccccttgccatttttttccccatggtgtatggctgaaacaagtaatctgtgagataataagacaaaattatctggcatatctagaaaatacctatcgaaatagcatgaagttgattctctctcgtcctttatgaaagtcacacacttctaatatattttaagatccgacagtaaaactgtctgaatttttaatactgtgcctgctacctgatgcctgtgtttttcttttgcaaatttttttggccagtgtttgaaaggctgaagaccaattcgttttcatggatccaaacctggttctgtattttcttaaatgataacaattaagaaattcccatcagtagatgctacttgtaaacgaagaaactttttttttccctttggaatctagtagtattctaactttttcatgtcttctatcagaccacaattcaaatattttccaaagcagaggacgacggtactaagcagatgatagctcagaagcctgattccctacccaagggacagaggctgtgagatgacattgagaaagagacccgggtccagtgaagcatcagacacgctggcgcatggggacgaggagccctggagactcagggcccgtctggtgcggcccgggctttgctccgcgctcgccccctgcagctgccggggccgccgcaacttttcaaacctcaccgcaccgacagctctgtcccttcttttatctggagacgctgagcctcatcaactctcac

SEQ ID NO: 17181 - RNA, 1640 nt, Homo sapiens
  source 1..1640: mol_type = other RNA
tcaggccaggcacagtggctcacacctgtaatcccagaactttgggagggccaggcaggcggcagatcgcttgagctcaggagtttgagagcagcctgggcaacatggggaaactctgtctctacaaaaaatacaaaaactagccagacatggtggcgcgcgccgctcctcccagctacttgggaggttgcggtgggagggtcacttgagaccgggaggcggaagttgcagtgagcagagatcacaccactgcactccatcctggacgacagagcgagaccctgtctcgaaaaacaaaagacaaaaacaaaaacaaaggtcatcctgcaggacaaccaggagggcacaaatgtgtgtctgtgggaagctgaaatgttggcgggggaaaaaagcagggaaaggcattccagaaaaaggaaactgtaaacagcacacgaaaaagcatagtgaatgaataggaagcctgagaccaaacttagggtttcctacacttatttcaaagcccttcattatctatatggaaagggggagtctttaaacacaaatatttagatcatattgactgagatttagatataaatgaatgctaataattacttttcgttattttggggtgttaaacatttactgtacaagattgtattcgttttaagtatcttctaacatgagccattttgtaatgattcagttgtttatattcaatttcaagtagaatgctgatcacagcgccaaatgggtatcttctacagaaaaagttattttaataaagaaaaatatagtcagttttaggatttcctgagagattatagaaacaataaaagcattaaaactgttaagtcattaaatacgagtaccttgtattttgaaggctcttaaaatttagtttataaattgcttttacataacatatgcactgaaataccacttaagattagttttgaaaataggtgttcgtttcaaccacatcattaggtattttattcaaagctctttataaaaagagctttactatgttccagtatagtaaacttatccagaaaataagacaaaaatttaacttcatgctatagctgcaaagttttcggaaagcgggatttaaaacttccattgtaactttaactagcggtcatgtcaaatttcacaactaagaacattttaacgcatgtaatactgagcacaacatgggcacgtttttgttgctatgagaaccttctattttgtattagacattgcagccttgacgacgcaatgtttgtgctattttgcgcatgttttcctgcagctattcctctcctctagcaatagtcgaatggctctggtttcctcttgcgcccggcccagtttttccgttttagcttcggttgtcataggctgtgctgtcgctttctctgggaaaggacggtgaagactggacgggagaaaccgggagggcaggcgcggccgttctgcagcagccgggccgcttcccggcgggaggcgggctgcgaatgggaagcgggaggaggaggccgggccgcgggctggttctatcacccccttgggagcccagctcttcacctagctctccggcgcttttcaaaatatcctgcgcgggctgcgccggaggcgccggcagggggtgctgataatggcgtcgttgt

SEQ ID NO: 17182 - RNA, 40 nt, Homo sapiens
  source 1..40: mol_type = other RNA
tcaggccaggcacagtggctcacacctgtaatcccagcac

SEQ ID NO: 17183 - RNA, 188 nt, Homo sapiens
  source 1..188: mol_type = other RNA
tcaggccaggcacagtggctcacacctgtaatcccagcacagtagctataaaacaacaacaacaaaaaacaaaaaacagtagctattagtaatgaagttttgataattggccaatctgtcaatcagcagggtttgtttgtttttggttctgttttttaagacagcatcttgctgtgtgtgcccaggct

SEQ ID NO: 17184 - RNA, 1305 nt, Homo sapiens
  source 1..1305: mol_type = other RNA
tcaggccaggcacagtggctcacacctgtaatcccagcacttagggaagacaagtcaggaggattgattgaagttaggagttagagaccagcctgggcaacgtattgagaccatgtctattaaaaaataaaatggaaaagcaagaatagccttattttcaaaatatggaaagaaatttatatgaaaatttatctgagtcattaaaattctccttaagtgatacttttttagaagtacattatggctagagttgccagataaaatgctggatatcatgcaataaatttgcaaaacatcatctaaaatttaaatttgtcctacatttgtacttgctaaatctggcagccttaattattacacaactataacacaacacaaacagtaatctctcccctagtttagagtcctttgcatgaaatttagcaaatctatcattttgaatacagtacaagcctggtaatccagtgtatttgggataggccagtggaactcagaactgatacatatatacatgtatgtctatcatattcaatgtctattaggtgtaaatcatctcttcatgtaaaagacactactggtttgagggtagactcgtctaggaatattttgtccttctgtgacagcaccactatccatcccaatgtaacatttctacaaagggaagatatcttaaccaggcatacttatatttgctagttggaaaatcattctgaacagttttaattccattctattgaatggattattgtatgagctatttggggatcagatataaatgacaatcacacagaaccacttttattcaacatagataaaatgtgatgagtgttaacattttaaataagcaatctgcttaatggacattggtatgaaggggaagtgtcattctttacctcactcctcaaacacttttctatccaaaggttggtttgagtcagtattggcatcatacaaccacttactgtaaaataagtttattagtggtaacgtgatagaatttattcccgatatctgatgttacaaactttagggtccttgagatatgcaggatccttgtatgtaactggcataaaccccattatttgagctctcttaattgcttttgtgatttctttctgtttcttcccacaaagaccaggtcctcattgctggatacctgttgtgaacaacctcttctccaaagcaccgtgtgagtcccgggatgtgtaaggctgacagcagccgttaccaagtgtgtcaacttcttcctccctagaccaccgcaaacagcaaccacagcggccatggttccgcgtttcttccact

SEQ ID NO: 17185 - RNA, 1363 nt, Homo sapiens
  source 1..1363: mol_type = other RNA
tcaggccaggcacagtggctcacacctgtaatcccagcacttagggaagacaagtcaggaggattgattgaagttaggagttagagaccagcctgggcaacgtattgagaccatgtctattaaaaaataaaatggaaaagcaagaatagccttattttcaaaatatggaaagaaatttatatgaaaatttatctgagtcattaaaattctccttaagtgatacttttttagaagtacattatggctagagttgccagataaaatgctggatatcatgcaataaatttgcaaaacatcatctaaaatttaaatttgtcctacatttgtacttgctaaatctggcagccttaattattacacaactataacacaacacaaacagtaatctctcccctagtttagagtcctttgcatgaaatttagcaaatctatcattttgaatacagtacaagcctggtaatccagtgtatttgggataggccagtggaactcagaactgatacatatatacatgtatgtctatcatattcaatgtctattaggtgtaaatcatctcttcatgtaaaagacactactggtttgagggtagactcgtctaggaatattttgtccttctgtgacagcaccactatccatcccaatgtaacatttctacaaagggaagatatcttaaccaggcatacttatatttgctagttggaaaatcattctgaacagttttaattccattctattgaatggattattgtatgagctatttggggatcagatataaatgacaatcacacagaaccacttttattcaacatagataaaatgtgatgagtgttaacattttaaataagcaatctgcttaatggacattggtatgaaggggaagtgtcattctttacctcactcctcaaacacttttctatccaaaggttggtttgagtcagtattggcatcatacaaccacttactgtaaaataagtttattagtggtaacgtgatagaatttattcccgatatctgatgttacaaactttagggtccttgagatatgcaggatccttgtatgtaactggcataaaccccattatttgagctctcttaattgcttttgtgatttctttctgtttcttcccacaaagacctgtaatgtgccttccataaatgcatccagtaaatggagaaacaaactgggacaaaagcaggtcctcattgctggatacctgttgtgaacaacctcttctccaaagcaccgtgtgagtcccgggatgtgtaaggctgacagcagccgttaccaagtgtgtcaacttcttcctccctagaccaccgcaaacagcaaccacagcggccatggttccgcgtttcttccact

SEQ ID NO: 17186 - RNA, 1447 nt, Homo sapiens
  source 1..1447: mol_type = other RNA
tcaggccaggcacagtggctcacacctgtaatcccagcacttagggaagacaagtcaggaggattgattgaagttaggagttagagaccagcctgggcaacgtattgagaccatgtctattaaaaaataaaatggaaaagcaagaatagccttattttcaaaatatggaaagaaatttatatgaaaatttatctgagtcattaaaattctccttaagtgatacttttttagaagtacattatggctagagttgccagataaaatgctggatatcatgcaataaatttgcaaaacatcatctaaaatttaaatttgtcctacatttgtacttgctaaatctggcagccttaattattacacaactataacacaacacaaacagtaatctctcccctagtttagagtcctttgcatgaaatttagcaaatctatcattttgaatacagtacaagcctggtaatccagtgtatttgggataggccagtggaactcagaactgatacatatatacatgtatgtctatcatattcaatgtctattaggtgtaaatcatctcttcatgtaaaagacactactggtttgagggtagactcgtctaggaatattttgtccttctgtgacagcaccactatccatcccaatgtaacatttctacaaagggaagatatcttaaccaggcatacttatatttgctagttggaaaatcattctgaacagttttaattccattctattgaatggattattgtatgagctatttggggatcagatataaatgacaatcacacagaaccacttttattcaacatagataaaatgtgatgagtgttaacattttaaataagcaatctgcttaatggacattggtatgaaggggaagtgtcattctttacctcactcctcaaacacttttctatccaaaggttggtttgagtcagtattggcatcatacaaccacttactgtaaaataagtttattagtggtaacgtgatagaatttattcccgatatctgatgttacaaactttagggtccttgagatatgcaggatccttgtatgtaactggcataaaccccattatttgagctctcttaattgcttttgtgatttctttctgtttcttcccacaaagacctgtaatgtgccttccataaatgcatccagtaaatggagaaacaaactgggacaaaagctgtacattcttataatctacatgctttccacacaagatacatttcttaagaggttctttataaggattttccattgaaatgggcaggtcctcattgctggatacctgttgtgaacaacctcttctccaaagcaccgtgtgagtcccgggatgtgtaaggctgacagcagccgttaccaagtgtgtcaacttcttcctccctagaccaccgcaaacagcaaccacagcggccatggttccgcgtttcttccact

SEQ ID NO: 17187 - RNA, 1389 nt, Homo sapiens
  source 1..1389: mol_type = other RNA
tcaggccaggcacagtggctcacacctgtaatcccagcacttagggaagacaagtcaggaggattgattgaagttaggagttagagaccagcctgggcaacgtattgagaccatgtctattaaaaaataaaatggaaaagcaagaatagccttattttcaaaatatggaaagaaatttatatgaaaatttatctgagtcattaaaattctccttaagtgatacttttttagaagtacattatggctagagttgccagataaaatgctggatatcatgcaataaatttgcaaaacatcatctaaaatttaaatttgtcctacatttgtacttgctaaatctggcagccttaattattacacaactataacacaacacaaacagtaatctctcccctagtttagagtcctttgcatgaaatttagcaaatctatcattttgaatacagtacaagcctggtaatccagtgtatttgggataggccagtggaactcagaactgatacatatatacatgtatgtctatcatattcaatgtctattaggtgtaaatcatctcttcatgtaaaagacactactggtttgagggtagactcgtctaggaatattttgtccttctgtgacagcaccactatccatcccaatgtaacatttctacaaagggaagatatcttaaccaggcatacttatatttgctagttggaaaatcattctgaacagttttaattccattctattgaatggattattgtatgagctatttggggatcagatataaatgacaatcacacagaaccacttttattcaacatagataaaatgtgatgagtgttaacattttaaataagcaatctgcttaatggacattggtatgaaggggaagtgtcattctttacctcactcctcaaacacttttctatccaaaggttggtttgagtcagtattggcatcatacaaccacttactgtaaaataagtttattagtggtaacgtgatagaatttattcccgatatctgatgttacaaactttagggtccttgagatatgcaggatccttgtatgtaactggcataaaccccattatttgagctctcttaattgcttttgtgatttctttctgtttcttcccacaaagacctgtacattcttataatctacatgctttccacacaagatacatttcttaagaggttctttataaggattttccattgaaatgggcaggtcctcattgctggatacctgttgtgaacaacctcttctccaaagcaccgtgtgagtcccgggatgtgtaaggctgacagcagccgttaccaagtgtgtcaacttcttcctccctagaccaccgcaaacagcaaccacagcggccatggttccgcgtttcttccact

SEQ ID NO: 17188 - RNA, 7249 nt, Homo sapiens
  source 1..7249: mol_type = other RNA
tcaggccaggcacagtggctcacacctgtaatcccagcacttcgggaggccgaggcaggtggatcaccagatcaggaaatcgagaccatcctggctaacacagtgaaaccccgtctctactaaaaatacaaaaaattagccgggcatggtggcgggcacctgtagtcccagctactcgggaggctgaggcaggagaatggcatgaacccgggaggcagagcttgcagtgagcagagatcgcgccactgcactccagcctgggcaacagagcaaagagtctgtctcaaaaaaacaaaacaaaacaaaacaaaacaaatggaaattaaacaactgaaaaatacaaaaaccaaaacgaaaactcattggacaagctcaacagtagactgcatatggcagaaaaaaagaatcagtgagctgaaaaaaagtcaacagaaattaaccaatatgaaaaaaagggaaaaatagaccagaaaaagggggtaaacatgaaagcacaagagacctctgagacagtaacaaaagctctaccattcatatcacagagaggagaaagagtagggatgaaaaaatatttcaagaaataatggttaaaaattcccaaatttggcaaagggcataaaccgacaaatcaaaaagctaaacaaaaaccaaacatgatacactcaaaaaaattccatgtcacacacctcataaccaaacttctgaacactacaaaaaaaacaaaacactttgaacgcaggttgataaaaatggcacattatgaactagggaacaatggttcaaatggcaacagatttctcatctgaaaccatagcggacagaaggaacaaacatgtttctcaagtactaaaagaactgcagaccctaaatcctattatcccacaaaaatatccctcaggaatgaagggaacataaagacacttttagagacaccagcagactgaccctagaaaaaaggttacacaagttcgccaaacagaaagaaaatgttaatagaaggtggcttagaatttcaagaaagaatagtggaatgggtaaagagatcaacaagcaatacttcctgtgacttttgtaaaatatatttgacagtggaagcaaaaattacattttccaacatggtgctcaattttgaagaggaattactttagacaattatattaacaggcaaggtgaagggaccaagtaaggtttctatacatcaaagtgctaaatttttcataccattaactgtaattatgttacatatgtacattatactacttaaagcaaccactaaaaaattaatacaaaaatacaaagaaatatatttaaaaaacactacaaatatatcaaatggaattctaaaaaatgttaaagacaaaaaaaaaaaaacccaaacaaaccaagaaagaagcaacaggaaacacaaaaaactaatcataaaatagcagacatagcactaacataattattgtaaactttaaatggtctaaatacaccaataaaagacagaaatatgcaaactggggccagacacagtgacacatacctgtaatcccagcactttgggaggctgaggtgggcagatcacctgaggtcaggagtttgagaccagcctgaccaacatgatgaaaccccgtctctactaaaaatataaaaattagctaggtgtggtggcaggcacctgtaatcccagctacttgggaggctgaggcaagagaatggcttgaacccgggaggcagaggttgcagactgcgccactgcactccagccagggcgacagagcaagactccgtctcaaaaaaaaaaaaaaaaaaaaaatgctgtgcgtggttgctcataccagtaatcctagcactttgggaggctgaggcaggtggatcacctgaggtcaggagttcgagaccagcctggccaacatggtgaaactccatctctactaaaaatacaaaaaatcagtcaggcatggtggcggatgcctgtaatcccagctactcaagagcctgaggcaggagaatcacttgaacccaggaggcggaggttgcagtgagcggagatcgcaccactccactccagcctgggcaacaagaacaaaactccgtctcaaaaaaaaaaaaaaaaaaaaaaaaagatacgcaaactggatataaaaccacagcccaaatatacgccattcacaagaaacttactcccaatatagtgatatagataaggtttaaaaaaatgatgaagtgtaaatcatgcaagcattaaccaaaacgtaagactgaccacacaaatatcagataaaaattgataagagtattaacaggaacaaaaagggacattacttaattataaaagggtcaatacaccaagaatactaagcaaacctacatgtgtatataccaaacaacagagctttaaattatgtggagcaaaaactgatagaacttaaaggaggaataggtaattccacaattatagctcaggacttcaacatccttctcttggcaattgatagaaatactagacagaaaatcagcaaggatacaggagacctaaataacaccaccaactaacaggatcatacaaacttttacagaaactccaccaaatgaccgagaacacacattcttttcaagcagctatgtaaaacaagacagcctatatcctgggtcataaggaaaaaaagtcaacaaatttcaacagtaacatcaaatgcaaaacaaattagaaatcaataacaaatagcagggaatactccaaacactattaaacaatatacttctaaataattcctgggttagagaagatgtctcaaaaggaatcaggcaatcttagaactgagtaagataatcaaaagcatattaagacttgtgggatgaaactaacagcagtgtaagaaaaatgtatagaacttaaagcttatattaaaaaagaaaaaaagcctcaaatcaataacctaaacatccacgtcaggaaaccactgagtcaaatacaaccagagcaagtaggagaaaggatacaatacacatcagagcagatatcagtgaaattaagaacagagactggagaaaaatcagtgatataaagtgctatttctttgaaatgatcaatgaaattgacatatgtctacaaagactgacaataataagtgatacatttccaatatcaagaatacaacaaggaacataagtacagatcctgctgccatcaagaggataaaaggaaatatttcaaagaatgctacaaattagaacatttacataaaatgaacacttccttaagaaaatctataaaaattcatccaatatgaaatactctgaatagttctatacctattaaataaaataaatacataattaaaaagcattcaaaaggaaaatctccaggtcccacttcttcactggagaaagctaccaaacattaaaggaacaaataacaccaattctacacatgatcttccaaaaaaacagaagagaattccttccaattcatgttaggaggttagttatcatctagacatcaaaaccaaacagtaacagttgaagaaagaaaactacagattatcactcatgaaatcagaggaaagcttcctcaacaaaatactagcaaatgaaatactgtagcatagtacacaaacaaaattatactccatgatcaagtagggcttatcacaaagatgtgaggctggttcaatacttgaaactcaatcaaggtaacacatcatatcaactgactatagaagtaacatcacataattaaatcaattggtggagaaaaagcatatgacaaaattcaacacttattaataataaccaaaaaaatcccagcaaattaggaatagagggaaactttctaaactcgatagagaaactctttggaagcaactttcaacatcataataatgagaaactgaacatttccccctaatatcaggaacaaggcatggataacttgtcactattcgtattcaacatcacactggaaatcctacctagtacaataacatgagaaaagcaaataaaaggtatacagatgggaagcaagaaataaaactgtcccaaattgcaaatgacatttctatatttaaaatcctaaggattctcccaaaagaaatggcaagaaataatgagtttaggaaggttgcaagacagcaaaataagattgaaaaaataatgtttctgtatactagccaacatcatgtgaatattgaaactttaaatatcaatgccatttacaatcactcaaaaaactatgcagctataattcttattttaaatgtgcaggagttatactgtgtaaactataaaacagtaatgaaatatatcaaagaaaatttaaataatgaaaagataggctatgttcatgaattggaagactaagatgccaatttccaacacattgatctatagatttaactcaatttctatcaaaatccaagcaagaatatttgaaaaacagaaaaaccaatcctaaagtgtatatggaaagtcaaactaggaatgctaaatgaattttaaataaaaatagtaagaaaaaagaaatcacattacctaattttgagatttaccatacagctatagcaatcaagtaaaccaacagatgggaatcaagaaaaattctcagtgttagtgtttaaaacccattaaaaaagaatttttttaaaaaatcaaagacctaaacagtattaagtggtacaataaaatgtgcgcattcatgtttcttttaatccttaaatataaaagtatttcataactcaaggcttcattatttctcataaaaacaatgcttcttaagaagagacaatgttgtagaacaaagacattgagtaagtttccagaccttcccttactaactttcctgacacaggacagaaatgtacatacaagacaacagtataaaagcagtgtctgcatttcattttcttttctatgtcacctctttctgtttataaaaattcctgagataacattgcactgtaaactaatgagaaagatggagctaaaggttttcccaagtgcgtaataaccactgggtgtttttccaggatgaattcggatggagaataaggctctaagctgcgtgattttctaatatgactccttaggtgacaaatgacatttggcaacagaaggttttctcacagtgaagacacttgtggggtttctctttggtatgtacgatcagatgccatgtaagatgcttcctcttgcaaaagattttcctcagtggtgacattcaaaaagtttttccccaataaaagttcttggatgttgactgaggtctgcccacttgtaaaaggtcttcccacatctgttacactgataggatttctcccagtatgcatcctttgatgctgagtgagggacgagctgcgactgaaggcctttccacattcactgcactcatacggcttctctccagtgtggatgatagagtgtcgaatgaggtttgtgctccagcaaaatgttttcccacactcgatgcattcatagggcttctctccactatgaatccgctggtgccttgtgaggcctgacctgcggttgaaggcctttccacactccatgcactcatagggcttctctccagtgtggatgctgaagtggcgaatgaggtctgccctattgctaaaggctttcccacactctttgcactcgaaaggtttttctccagtgtgggcccttttatgcaagatgaaagtagagcagtgggtgaaggcctttccgcattcactacacacatatggcttctccccagtgtgaatccgctggtgccttttgaggtaggatcggtggttgaaagccttcccacactcgaggcactcaaagggcttctctccagtgtggatgacatagtggtgaatcagcgctgcgctctcacagaaggccttcccacattcactgcactcatagggcttctccccggtatgagtctgctggtgccacatgaggtatgatctgtgtttgaagaccttgccacattcgaagcactcgtagggattctcaccactgtggatgatgtagtgtcgaatgaaacctggcctatctcgaaaggctttgccacactctttgcacacaaagggtttttctccagtgtggctcctgttatgcaagacaaaagtggagcggtgggtgaaggcctttccacattcactgcacttataaggcttctctccactgtgaatccgctggtgctgggtaaggtgtgacttccgattaaaagccttcccacactccatgcacttatagggcttctccccagtgtggaccatgtggtgctgcaggaggtatgtactcttgctaaaggtttttccacactctgtgcattcatagggcttcactccagagtgaatcctctcatgccgagcaagcaggcgtttcttgttaaacactttttcacattcattgcatttaaagatattttcctcttcctgaataactggatttttacctgatccatgtgagtcacagtcatggacatcatctcctaaggagactcgatcctgtataatccttgaacacacactatcagctgtccctaaaccatcatgtttggggctcatttttccaggaagcttctccttttgggaatctaaccctggtctcaagcgttctccctgcatttctgaaaacccatcctgatccttgggttgccccaactgggagtcccctgaagctccttgtgttagttgtccccaaaaagagattccttcagacaaggctagctcacaggtggtaggttctgtgctcttgggttttcctttgtcacctggacaggtgccttgggagaggtcttccttcctggtccatggctcctgcccatgctctaggtggtagatcagctcaggtctgggaacaggacaccccagagataccaggagcccacagttttccagcatcacctcctggtacagggtccgctgagctaggtccagctggccccactcctcctgggtgaaagtcacagccacatcatcaaaggtcacagacacctgcgccgggtccgtcaaagccatcgccataccgggaccctgtggccctagcggggcgggggctgcggcgagcagggcgggtctcgcgggctcagccgagccccaccccttccctgcgccgggcccggtgaccttggctgacagtcaaactctctcgttacggggaggctcacggttcgctccgagacgcggaggtcgctgtcggcctcctacctgctcatttccccagcgccgccagggaggcggccacggaacaccgccccctccctagagccggcgtggacggaacc

SEQ ID NO: 17189 - RNA, 7122 nt, Homo sapiens
  source 1..7122: mol_type = other RNA
tcaggccaggcacagtggctcacacctgtaatcccagcacttcgggaggccgaggcaggtggatcaccagatcaggaaatcgagaccatcctggctaacacagtgaaaccccgtctctactaaaaatacaaaaaattagccgggcatggtggcgggcacctgtagtcccagctactcgggaggctgaggcaggagaatggcatgaacccgggaggcagagcttgcagtgagcagagatcgcgccactgcactccagcctgggcaacagagcaaagagtctgtctcaaaaaaacaaaacaaaacaaaacaaaacaaatggaaattaaacaactgaaaaatacaaaaaccaaaacgaaaactcattggacaagctcaacagtagactgcatatggcagaaaaaaagaatcagtgagctgaaaaaaagtcaacagaaattaaccaatatgaaaaaaagggaaaaatagaccagaaaaagggggtaaacatgaaagcacaagagacctctgagacagtaacaaaagctctaccattcatatcacagagaggagaaagagtagggatgaaaaaatatttcaagaaataatggttaaaaattcccaaatttggcaaagggcataaaccgacaaatcaaaaagctaaacaaaaaccaaacatgatacactcaaaaaaattccatgtcacacacctcataaccaaacttctgaacactacaaaaaaaacaaaacactttgaacgcaggttgataaaaatggcacattatgaactagggaacaatggttcaaatggcaacagatttctcatctgaaaccatagcggacagaaggaacaaacatgtttctcaagtactaaaagaactgcagaccctaaatcctattatcccacaaaaatatccctcaggaatgaagggaacataaagacacttttagagacaccagcagactgaccctagaaaaaaggttacacaagttcgccaaacagaaagaaaatgttaatagaaggtggcttagaatttcaagaaagaatagtggaatgggtaaagagatcaacaagcaatacttcctgtgacttttgtaaaatatatttgacagtggaagcaaaaattacattttccaacatggtgctcaattttgaagaggaattactttagacaattatattaacaggcaaggtgaagggaccaagtaaggtttctatacatcaaagtgctaaatttttcataccattaactgtaattatgttacatatgtacattatactacttaaagcaaccactaaaaaattaatacaaaaatacaaagaaatatatttaaaaaacactacaaatatatcaaatggaattctaaaaaatgttaaagacaaaaaaaaaaaaacccaaacaaaccaagaaagaagcaacaggaaacacaaaaaactaatcataaaatagcagacatagcactaacataattattgtaaactttaaatggtctaaatacaccaataaaagacagaaatatgcaaactggggccagacacagtgacacatacctgtaatcccagcactttgggaggctgaggtgggcagatcacctgaggtcaggagtttgagaccagcctgaccaacatgatgaaaccccgtctctactaaaaatataaaaattagctaggtgtggtggcaggcacctgtaatcccagctacttgggaggctgaggcaagagaatggcttgaacccgggaggcagaggttgcagactgcgccactgcactccagccagggcgacagagcaagactccgtctcaaaaaaaaaaaaaaaaaaaaaatgctgtgcgtggttgctcataccagtaatcctagcactttgggaggctgaggcaggtggatcacctgaggtcaggagttcgagaccagcctggccaacatggtgaaactccatctctactaaaaatacaaaaaatcagtcaggcatggtggcggatgcctgtaatcccagctactcaagagcctgaggcaggagaatcacttgaacccaggaggcggaggttgcagtgagcggagatcgcaccactccactccagcctgggcaacaagaacaaaactccgtctcaaaaaaaaaaaaaaaaaaaaaaaaagatacgcaaactggatataaaaccacagcccaaatatacgccattcacaagaaacttactcccaatatagtgatatagataaggtttaaaaaaatgatgaagtgtaaatcatgcaagcattaaccaaaacgtaagactgaccacacaaatatcagataaaaattgataagagtattaacaggaacaaaaagggacattacttaattataaaagggtcaatacaccaagaatactaagcaaacctacatgtgtatataccaaacaacagagctttaaattatgtggagcaaaaactgatagaacttaaaggaggaataggtaattccacaattatagctcaggacttcaacatccttctcttggcaattgatagaaatactagacagaaaatcagcaaggatacaggagacctaaataacaccaccaactaacaggatcatacaaacttttacagaaactccaccaaatgaccgagaacacacattcttttcaagcagctatgtaaaacaagacagcctatatcctgggtcataaggaaaaaaagtcaacaaatttcaacagtaacatcaaatgcaaaacaaattagaaatcaataacaaatagcagggaatactccaaacactattaaacaatatacttctaaataattcctgggttagagaagatgtctcaaaaggaatcaggcaatcttagaactgagtaagataatcaaaagcatattaagacttgtgggatgaaactaacagcagtgtaagaaaaatgtatagaacttaaagcttatattaaaaaagaaaaaaagcctcaaatcaataacctaaacatccacgtcaggaaaccactgagtcaaatacaaccagagcaagtaggagaaaggatacaatacacatcagagcagatatcagtgaaattaagaacagagactggagaaaaatcagtgatataaagtgctatttctttgaaatgatcaatgaaattgacatatgtctacaaagactgacaataataagtgatacatttccaatatcaagaatacaacaaggaacataagtacagatcctgctgccatcaagaggataaaaggaaatatttcaaagaatgctacaaattagaacatttacataaaatgaacacttccttaagaaaatctataaaaattcatccaatatgaaatactctgaatagttctatacctattaaataaaataaatacataattaaaaagcattcaaaaggaaaatctccaggtcccacttcttcactggagaaagctaccaaacattaaaggaacaaataacaccaattctacacatgatcttccaaaaaaacagaagagaattccttccaattcatgttaggaggttagttatcatctagacatcaaaaccaaacagtaacagttgaagaaagaaaactacagattatcactcatgaaatcagaggaaagcttcctcaacaaaatactagcaaatgaaatactgtagcatagtacacaaacaaaattatactccatgatcaagtagggcttatcacaaagatgtgaggctggttcaatacttgaaactcaatcaaggtaacacatcatatcaactgactatagaagtaacatcacataattaaatcaattggtggagaaaaagcatatgacaaaattcaacacttattaataataaccaaaaaaatcccagcaaattaggaatagagggaaactttctaaactcgatagagaaactctttggaagcaactttcaacatcataataatgagaaactgaacatttccccctaatatcaggaacaaggcatggataacttgtcactattcgtattcaacatcacactggaaatcctacctagtacaataacatgagaaaagcaaataaaaggtatacagatgggaagcaagaaataaaactgtcccaaattgcaaatgacatttctatatttaaaatcctaaggattctcccaaaagaaatggcaagaaataatgagtttaggaaggttgcaagacagcaaaataagattgaaaaaataatgtttctgtatactagccaacatcatgtgaatattgaaactttaaatatcaatgccatttacaatcactcaaaaaactatgcagctataattcttattttaaatgtgcaggagttatactgtgtaaactataaaacagtaatgaaatatatcaaagaaaatttaaataatgaaaagataggctatgttcatgaattggaagactaagatgccaatttccaacacattgatctatagatttaactcaatttctatcaaaatccaagcaagaatatttgaaaaacagaaaaaccaatcctaaagtgtatatggaaagtcaaactaggaatgctaaatgaattttaaataaaaatagtaagaaaaaagaaatcacattacctaattttgagatttaccatacagctatagcaatcaagtaaaccaacagatgggaatcaagaaaaattctcagtgttagtgtttaaaacccattaaaaaagaatttttttaaaaaatcaaagacctaaacagtattaagtggtacaataaaatgtgcgcattcatgtttcttttaatccttaaatataaaagtatttcataactcaaggcttcattatttctcataaaaacaatgcttcttaagaagagacaatgttgtagaacaaagacattgagtaagtttccagaccttcccttactaactttcctgacacaggacagaaatgtacatacaagacaacagtataaaagcagtgtctgcatttcattttcttttctatgtcacctctttctgtttataaaaattcctgagataacattgcactgtaaactaatgagaaagatggagctaaaggttttcccaagtgcgtaataaccactgggtgtttttccaggatgaattcggatggagaataaggctctaagctgcgtgattttctaatatgactccttaggtgacaaatgacatttggcaacagaaggttttctcacagtgaagacacttgtggggtttctctttggtatgtacgatcagatgccatgtaagatgcttcctcttgcaaaagattttcctcagtggtgacattcaaaaagtttttccccaataaaagttcttggatgttgactgaggtctgcccacttgtaaaaggtcttcccacatctgttacactgataggatttctcccagtatgcatcctttgatgctgagtgagggacgagctgcgactgaaggcctttccacattcactgcactcatacggcttctctccagtgtggatgatagagtgtcgaatgaggtttgtgctccagcaaaatgttttcccacactcgatgcattcatagggcttctctccactatgaatccgctggtgccttgtgaggcctgacctgcggttgaaggcctttccacactccatgcactcatagggcttctctccagtgtggatgctgaagtggcgaatgaggtctgccctattgctaaaggctttcccacactctttgcactcgaaaggtttttctccagtgtgggcccttttatgcaagatgaaagtagagcagtgggtgaaggcctttccgcattcactacacacatatggcttctccccagtgtgaatccgctggtgccttttgaggtaggatcggtggttgaaagccttcccacactcgaggcactcaaagggcttctctccagtgtggatgacatagtggtgaatcagcgctgcgctctcacagaaggccttcccacattcactgcactcatagggcttctccccggtatgagtctgctggtgccacatgaggtatgatctgtgtttgaagaccttgccacattcgaagcactcgtagggattctcaccactgtggatgatgtagtgtcgaatgaaacctggcctatctcgaaaggctttgccacactctttgcacacaaagggtttttctccagtgtggctcctgttatgcaagacaaaagtggagcggtgggtgaaggcctttccacattcactgcacttataaggcttctctccactgtgaatccgctggtgctgggtaaggtgtgacttccgattaaaagccttcccacactccatgcacttatagggcttctccccagtgtggaccatgtggtgctgcaggaggtatgtactcttgctaaaggtttttccacactctgtgcattcatagggcttcactccagagtgaatcctctcatgccgagcaagcaggcgtttcttgttaaacactttttcacattcattgcatttaaagatattttcctcttcctgaataactggatttttacctgatccatgtgagtcacagtcatggacatcatctcctaaggagactcgatcctgtataatccttgaacacacactatcagctgtccctaaaccatcatgtttggggctcatttttccaggaagcttctccttttgggaatctaaccctggtctcaagcgttctccctgcatttctgaaaacccatcctgatccttgggttgccccaactgggagtcccctgaagctccttgtgttagttgtccccaaaaagagattccttcagacaaggctagctcacaggtggtaggttctgtgctcttgggttttcctttgtcacctggacaggtgccttgggagaggtcttccttcctggtccatggctcctgcccatgctctaggtggtagatcagctcaggtctgggaacaggacaccctgcgccgggtccgtcaaagccatcgccataccgggaccctgtggccctagcggggcgggggctgcggcgagcagggcgggtctcgcgggctcagccgagccccaccccttccctgcgccgggcccggtgaccttggctgacagtcaaactctctcgttacggggaggctcacggttcgctccgagacgcggaggtcgctgtcggcctcctacctgctcatttccccagcgccgccagggaggcggccacggaacaccgccccctccctagagccggcgtggacggaacc

SEQ ID NO: 17190 - RNA, 1794 nt, Homo sapiens
  source 1..1794: mol_type = other RNA
tcaggccaggcacagtggctcacacctgtaatcccagcactttggaaggttgaggcaggcagatcacctgaagtcagaagttcgagatcagcctggccaacatggagaaaccccgtctctactaaaaatacaaaaattagctgggtgtggtggtgtgtgcctgtagtcccagctactcgggaggctgaggcaggagaatcgcttgaacccaggaggtggaggctgcagtgagccaagattgcaccactgcactccagcctgggcaacagagtgagactccaatttaaaaaagaaaaatgaaaaaagaagaaaagtaagaaaagaaaaagaaataacatataacaaataagaaaagtaaaataaatagaaggaaaagaaataagaaaaaaatgaaaagaaagaaaaaaataagaaaagtaaaagaaagaaaacaagttaaaatcaattacattgaagaacaagttggtggactttggaaacagaaggaaaatccaggtacaatttgtgtttttcagggatatgagagaatccaaggaagacggccgcagaggctccgtgctcaaatgtgtgaatagggacctgaccacccaccaattcccaacacgccttacagtgtgaagatcaggagatgtttaggtgattcctcaacgtatgaattttgtttttctaggaaccaaggtgtgtacctgtttggaacactgatcacagaaagagttaagaactgcttcataggaagtgcagtgagaaatgcaagtcaacggccaaaaacgttgaagatttaaaaatccatgcatgacctggaaggtcaaatccttaggacgtgagtgagcttaacctaggacactgcagggaagagggtggccaccctgggccccagtttgttcccttggcagggatggacttagggacaaaactcattaaaacatggaagtcactgccctgtttctgttagattcatgtttaaaagaaaatatctgcatttctcttcattttctgaagctcttatgcagaaatatgatttgctataatgagcttctgtgcatccagaaaggcaaaagcatatggaactgaaggcagagaatccgccatgtgattgagaatcccatcgtggtgggaatttgccagcagggcgaggggagcggcagatggaagggtttgctttaaggctatgtcttagcagataaaacgattacggtcaggacgctccgcaggcctgggctgggttctctgctcacccctaggtcttcagccatcattttctttgaagcatagcttctttttctggtaagcaatgaagctagagatggctccagccacggcgaccacgacagcccccacaatcccggggatcacgcctggggcgtcggcctcttccccttctttcctgtggctgcctccaccatcactgcctccttttccttctccacctgaaacgccatccgcaaggtcagcatctgaaaagctaccggaggaactagggtggttggggtttggatttggcatcggtttgggtgggttcggtggtcgtgggtcgtcattttctccatcaacaacagcatctcctaagtcaaagtcatccccagcactgggtttcttggggattgcagtgggtttcttgttttcattgtcaggaagggcatcggataaatcgaaaccaccatccggggcggcgaccagaacacccagcaggccgaagagcagcagcgccagcgcagccccgcgggccatggtgcgcccagagcgcgcagggacggtcccggagtgcagggcgtgggcgaaggcggcaggacagat

SEQ ID NO: 17191 - RNA, 473 nt, Homo sapiens
  source 1..473: mol_type = other RNA
tcaggccaggcacagtggctcacacctgtaatcccagcactttgggaggcagaggccagcattatcatttgaggtcaggagtttgagaccagcctggccaacatgacgaaaccccgtctctactaaaaatacaaaaattagctgggcgtggtggcacacatctgtagtcccagccactcgggaggctgaggcacgagaatcacgtgaacctaggagatggagtttgcagtgagccaagattgcaccactgcactccagcctgggcaacggagcaagactatgtcttaaaaaaaaaaaacactcatcaccgtcctcccaaagcctgctctccctaaccatgtcctcaatctcaggaagtgctgcccctgtctttgatcagaaatctcacccctctctgacactctacagatcccagcaactaatcagaataaatagtgatgacgtctctacatggcggtactcacccccaagcc

SEQ ID NO: 17192 - RNA, 4594 nt, Homo sapiens
  source 1..4594: mol_type = other RNA
tcaggccaggcacagtggctcacacctgtaatcccagcactttgggaggccaagacgggtggatcacgaggtcagatcgagaccatcctggttaacacggtgaaaccctgtctctacttaaaatacaaaaaatagccgggtgtggtggcgggcgcctgtagtcccagctactcaggaggctgaggcaggagaatggcgtgaacccgggaggcggagcttgcagtgagccgagatcgcgccactgcactccagcccgggtgacagcgcgactctgtctcaaaaaaataaaaaaaataaaaaaaaataaaaaacaagacagctaggaggaaagcctgtatgctttggaaaatgcatatcttgtgtgtttacccttttaaaggtaactatactttgaaacaggtgaactgcagaaagttaacaaagacttctttttttaccatgtttacctttctaagaattctatgcatttcctagggcatacatgcaaaagccttcacatttccccctttttaaaagagatatttctcaaacttatacgtatacagttcagtagtgttaagtacaatcacacttgttttgcaacagatctctagaattcttgcaacacaagctctgtacccactaaatacaaattcaccctctccccttcccccaaccgttgcttggcaaccacctttctactttctattgtatgattttgactactttgcatacttcacatggaggaatcatatagcatttgttcttttgttggctggcttatttcacttggcataatgccttcaaggttcatccacattgtacatttgacaggatttccttctttttaaaggctgaataatattccattgactgtatataccacatttcctttatctattcatctgttgatggacatttgggatgcttccagaacctcttggctattgtgaataatgctgctatgaacatgggtgtacaaatatctctttgagatcccgctttggtggtaattcttatggtaattctgttttcagttatttgggaaacctgtgtactgttttccgtaatgactgcaccgttttacattaccaccaacagtgcacaagggtttcaacttctctgcatcctccccaatacttgttatttttttgttcttctgatagtggccatcatgatgggcgtgagacgatatctcattgtggttttgatttgcatttccctaataattggcaatgttgagcatattttcatgttcttattggccaattgtataacttctttggagaaatgtctgtgcaagtcctttgcccatttttaaaaattgagttatttggttttttgttgttgagttgtagaagttcctcatatattctggatttgggctccttataagatagacgatttgcaattattttctctcattctagagcttgcgttttcactttgttgattgcttcctttgacacacagacatttttaagtttgatgtagtcccgtttccttcctaacgatctttaagtgtacagttcagtagtgttaagtatattcatccaaccctatcttgcagaccagatgacaaacatattaatgaaagaaatactaccagtcattgacgcaacagagtctgaacataggcttagaggcattcagaaacattccaagatatttataagcaagagccacaggagcatgaattcctcagaatatgtagaattatctagattttagcctatctgacaagtttctctccctattaccataacaaaagtcttttaaaccactgtataaactgagatatttaagttaatcacctgccttgcaaagaaccttgactaatgagtaaataaagttcagacagttgtaaagggaagacgggatagctctttcactgtagaaaacattatcattatatactatgtaacagcgtgcaaataatacaaaataataatataaactataggctattagattactagtcctttgaaaaatatttctggaaggccgggcacggtggctcacgcctgtaatcccagcactttgggaggccaaggcgggtggatcacctgaggtcaggagttcaagaccagcctggccaacatagtgaaaccccatctctactaaaaatacaaaaattagctgggcgtggtggcatgtgcctgtagtcccagttactcaggaggctgaggcaggagaatcgcttaaacccgggaggtggaggttgcagtgagccaagatagtgccactgcactccagcctgggggacagagcgagactccatctcaaaaaaaaaaaaaaaaaagaaaagaaaaatatttctggaaatgtgcaatgaaagaattctaagttctaggcactttaagcattttttcttttcttttctttttttttttttattagacacagagtctcactctgttgcccaggctggagtgcagtggtgtgatcttggttcactacaaccaccacctcctgggttcaagcgattctccagcctcagcttcccgagtagctggcattacaggtgctcaccaccatgcctggctaattttttatttgtagtagtgacagggtttcatcatgttggccaggctggtctcaaactcctgacctcaagtgagctacccgcctcagcctcccaaagtgctgggattacaggtgtgagccactgtgcccagccaggcattttctttaaaatgttctgcatatatttcctatatgatcagacctttaagcaaaatatctgatcttcggaaatgcaaagggatttctgggtataggaaaagtcttgttttcttataattacaaaatatattttctacatcataaactgatagtaagtaagcatatcatgtccttgtaacaactaaacactggggcaaatatactgactgataagcccttatgaaagaatacacattcatgttataaaataaaatacatctaaaaccatggccaatattcagccaggaagtaccagtctgggcccataggctgtttctgcaaggcctgagttctggtcagtgtctgtgccttaccacatgttaaaaattttgattataatccctatgtatagtgctatagaaccactaatggataaacataaaaagatagctcaaaaatgtcagacataaaaagatattacaagctgggccaggcggccagcacctgtagccccagctactctagaggctaaggcaggaggactgcttgagcctaggagttcaaggctgcagtgagctatcatttggccactgcactctagcctgggcagcagagcaagacctagtctcttaaagaaaaaaaaaaggcattacaattaccaacaggtatctgtaagagaaacttgtgtctcttgctggtaccgaatagccttcctcaaagactgatgaagcactctcatgctaagaaatgcacatctgtaaatattatcaaatgcaggcacttagaatagtctagttaacaatttatagtaagctagtatatattaaagcaaaagcaaaatactgcctagatatgaatgttttagggggttgcttggctggtggccggcttgggtttcgcttgtacattcagcacataatcatgccggaaggatgaacgaacagtgcgattcatcagtggctgaagggggcggaagttgtccaccattcttttctctttctccccttcggaagtgaaaagcagggtccgaaattgctcaagctgatcatgatcaacctctactggttgcttcttaatgatccaggtgacagactcggagaggggtggggtagtcagagaccctgagtaggtccagtaatctgggcaggtaggcatcaggcaggaagggtcaaatgacccaaattccacaagggcgtccttatgcttaattgacggcaaagtatccactaatttctgtagctccttatgatgtttgcctagctttaaaaatactcctatcacagccaaaccattttcttccagtgctgcatcctcaaagttttcaaatctgactgcgttccaatgcactaagtgcagctctgctgggaagcatttgctgtccacggtgtgctcagaaccccaggcatcgatggccccccagtgaaaatggaactgcttcaatcggtagttgtgttccaggggtcctcccttgatcactgatttatctgtagaatcttcaaattccacgaggaaagagtacccattattccagacgtggaggcaggtggctgggtcataagagatggtcagtggttttaagccgggatcataaacactgtccctccaccgaatgttgatgggtgactggcgatcgcccccaggaaccaggtccacgctctcccagagtggatgcaaggctcggttccgggttttgtaagtacaagtatagaggctgcagggcctcgctggcatgaatctcggaatctggaactttctccacagcaatttgcctggagaggcttgaagaatgaccctcaggctgttcatcaccaccatctttagcttgaaatcttgatcagttcccagttaagttgcaggaacttaataatctgagcgtctctccagatcacgaacctagccgctcgctcgcctacggggatccgcagcctgcacgtccggccatcgaagctac

SEQ ID NO: 17193 - RNA, 5873 nt, Homo sapiens
  source 1..5873: mol_type = other RNA
tcaggccaggcacagtggctcacacctgtaatcccagcactttgggaggccaagacgggtggatcacgaggtcagatcgagaccatcctggttaacacggtgaaaccctgtctctacttaaaatacaaaaaatagccgggtgtggtggcgggcgcctgtagtcccagctactcaggaggctgaggcaggagaatggcgtgaacccgggaggcggagcttgcagtgagccgagatcgcgccactgcactccagcccgggtgacagcgcgactctgtctcaaaaaaataaaaaaaataaaaaaaaataaaaaacaagacagctaggaggaaagcctgtatgctttggaaaatgcatatcttgtgtgtttacccttttaaaggtaactatactttgaaacaggtgaactgcagaaagttaacaaagacttctttttttaccatgtttacctttctaagaattctatgcatttcctagggcatacatgcaaaagccttcacatttccccctttttaaaagagatatttctcaaacttatacgtatacagttcagtagtgttaagtacaatcacacttgttttgcaacagatctctagaattcttgcaacacaagctctgtacccactaaatacaaattcaccctctccccttcccccaaccgttgcttggcaaccacctttctactttctattgtatgattttgactactttgcatacttcacatggaggaatcatatagcatttgttcttttgttggctggcttatttcacttggcataatgccttcaaggttcatccacattgtacatttgacaggatttccttctttttaaaggctgaataatattccattgactgtatataccacatttcctttatctattcatctgttgatggacatttgggatgcttccagaacctcttggctattgtgaataatgctgctatgaacatgggtgtacaaatatctctttgagatcccgctttggtggtaattcttatggtaattctgttttcagttatttgggaaacctgtgtactgttttccgtaatgactgcaccgttttacattaccaccaacagtgcacaagggtttcaacttctctgcatcctccccaatacttgttatttttttgttcttctgatagtggccatcatgatgggcgtgagacgatatctcattgtggttttgatttgcatttccctaataattggcaatgttgagcatattttcatgttcttattggccaattgtataacttctttggagaaatgtctgtgcaagtcctttgcccatttttaaaaattgagttatttggttttttgttgttgagttgtagaagttcctcatatattctggatttgggctccttataagatagacgatttgcaattattttctctcattctagagcttgcgttttcactttgttgattgcttcctttgacacacagacatttttaagtttgatgtagtcccgtttccttcctaacgatctttaagtgtacagttcagtagtgttaagtatattcatccaaccctatcttgcagaccagatgacaaacatattaatgaaagaaatactaccagtcattgacgcaacagagtctgaacataggcttagaggcattcagaaacattccaagatatttataagcaagagccacaggagcatgaattcctcagaatatgtagaattatctagattttagcctatctgacaagtttctctccctattaccataacaaaagtcttttaaaccactgtataaactgagatatttaagttaatcacctgccttgcaaagaaccttgactaatgagtaaataaagttcagacagttgtaaagggaagacgggatagctctttcactgtagaaaacattatcattatatactatgtaacagcgtgcaaataatacaaaataataatataaactataggctattagattactagtcctttgaaaaatatttctggaaggccgggcacggtggctcacgcctgtaatcccagcactttgggaggccaaggcgggtggatcacctgaggtcaggagttcaagaccagcctggccaacatagtgaaaccccatctctactaaaaatacaaaaattagctgggcgtggtggcatgtgcctgtagtcccagttactcaggaggctgaggcaggagaatcgcttaaacccgggaggtggaggttgcagtgagccaagatagtgccactgcactccagcctgggggacagagcgagactccatctcaaaaaaaaaaaaaaaaaagaaaagaaaaatatttctggaaatgtgcaatgaaagaattctaagttctaggcactttaagcattttttcttttcttttctttttttttttttattagacacagagtctcactctgttgcccaggctggagtgcagtggtgtgatcttggttcactacaaccaccacctcctgggttcaagcgattctccagcctcagcttcccgagtagctggcattacaggtgctcaccaccatgcctggctaattttttatttgtagtagtgacagggtttcatcatgttggccaggctggtctcaaactcctgacctcaagtgagctacccgcctcagcctcccaaagtgctgggattacaggtgtgagccactgtgcccagccaggcattttctttaaaatgttctgcatatatttcctatatgatcagacctttaagcaaaatatctgatcttcggaaatgcaaagggatttctgggtataggaaaagtcttgttttcttataattacaaaatatattttctacatcataaactgatagtaagtaagcatatcatgtccttgtaacaactaaacactggggcaaatatactgactgataagcccttatgaaagaatacacattcatgttataaaataaaatacatctaaaaccatggccaatattcagccaggaagtaccagtctgggcccataggctgtttctgcaaggcctgagttctggtcagtgtctgtgccttaccacatgttaaaaattttgattataatccctatgtatagtgctatagaaccactaatggataaacataaaaagatagctcaaaaatgtcagacataaaaagatattacaagctgggccaggcggccagcacctgtagccccagctactctagaggctaaggcaggaggactgcttgagcctaggagttcaaggctgcagtgagctatcatttggccactgcactctagcctgggcagcagagcaagacctagtctcttaaagaaaaaaaaaaggcattacaattaccaacaggtatctgtaagagaaacttgtgtctcttgctggtaccgaatagccttcctcaaagactgatgaagcactctcatgctaagaaatgcacatctgtaaatattatcaaatgcaggcacttagaatagtctagttaacaatttatagtaagctagtatatattaaagcaaaagcaaaatactgcctagatatgaatgttttagggggttgcttggctggtggccggcttgggtttcgcttgtacattcagcacataatcatgccggaaggatgaacgaacagtgcgattcatcagtggctgaagggggcggaagttgtccaccattcttttctctttctccccttcggaagtgaaaagcagggtccgaaattgctcaagctgatcatgatcaacctctactggttgcttcttaatgatccaggtgacagactcggagaggggtggggtagtcagagaccctgagtaggtccagtaatctgggcaggtaggcatcaggcaggaagggtcaaatgacccaaattccacaagggcgtccttatgcttaattgacggcaaagtatccactaatttctgtagctccttatgatgtttgcctagctttaaaaatactcctatcacagccaaaccattttcttccagtgctgcatcctcaaagttttcaaatctgactgcgttccaatgcactaagtgcagctctgctgggaagcatttgctgtccacggtgtgctcagaaccccaggcatcgatggccccccagtgaaaatggaactgcttcaatcggtagttgtgttccaggggtcctcccttgatcacttctcttataatcctatcaaggtaggtaggtcatgttgtcctctctttcattccagagtttagtaatttgagtcttcttttatttttttcttggtctcccccaattaaaagtttgtgaactttgttgatcttcccaaagaaccaacttttgatttcattgatttctgctcgttctttattatgcccttctctctacttgcttttgggtttagtttgttcttctttttctagtttcttaaggcggaaagctgagatactgacttgagaaagttcttctctattgtaggcattttcatctatacatttccctctaagcactgctttagctgcatcccaaaaggactggtatgatgtttttgtcacataccttccccagctccttttccttgcactttattccaatcctcacaaagcacactgtggcagcatttcttagggttttgtctttgaaatttatagacatcgatatttattaggtttttacttttctagaattgtttcttgcctttgtttctaaaatgtcttgctttctttcactttttattttttatgttcattcactctttttttcctctttgcatgctattgattgttttgcaacaacatggagaaatagcagcaaagaataaacaggaaataagaggcagtcactgatttatctgtagaatcttcaaattccacgaggaaagagtacccattattccagacgtggaggcaggtggctgggtcataagagatggtcagtggttttaagccgggatcataaacactgtccctccaccgaatgttgatgggtgactggcgatcgcccccaggaaccaggtccacgctctcccagagtggatgcaaggctcggttccgggttttgtaagtacaagtatagaggctgcagggcctcgctggcatgaatctcggaatctggaactttctccacagcaatttgcctggagaggcttgaagaatgaccctcaggctgttcatcaccaccatctttagcttgaaatcttgatcagttcccagttaagttgcaggaacttaataatcagattatgtggagtagaaatagtcccattacagtaaggaagaagacaagtgtccatgttatcccaccattatgtcactctgttgtgatagtgccactttaaaaatactcctatcacagccaaaccattttcttccagtgctgcatcctcaaagttttcaaatttgactgcgttccaatgcactaagtgcagctgatttatctgtagaatcttcaaattccacgaggaaagagtacccattattccagacgtggaggcaggtggctgggtcataagagatggtcagtggttttaagccgggatcataaacactgtccctccaccgaatgttgatgggtgactggcgatcgcccccaggaaccaggtccacgctctcccagagtggatgcactgagccagaacctcctcgttcgctcccggtacccgaggatcccgcacgcggccatcttggccacgccccctcacgtttagccacgtccctacgcagcaaacgtcatttcgtcattccaggttacgcccctatcagtccccattctgtccccgacccaggctgaaatctcgccctggccacgcttccccagcgccggagtccacacctgctctgcgctctggctacacatctcctgtcgctgccacgcgcctgcacgctaacttgccgacgcctctgccctccgcctgctccaccatctttgttacgcccctcagagcaac

SEQ ID NO: 17194 - RNA, 811 nt, Homo sapiens
  source 1..811: mol_type = other RNA
tcaggccaggcacagtggctcacacctgtaatcccagcactttgggaggccaaggcagcaggatctcatgaggtcaggggtttgagacagaccatctgggcaacatagtgagacctcacctcttaaaaaaaaaaaaaaaattggccgggcacggtggctcacgcctgtaatcctagcacgttgggaggccgaggcggacagattgcctgagctcaggagttcgcaaccagcctgggcaacacggtgaaaccccgtcagcagtgttgtcttgagcatgtcacttaacctctccaagtctgtttcctcatctgtgatacttgttaagccattgaagatgcccagatcccaccctcagaaaggtccagaaacaatgctgagaaaaattggctgaattttttaaattatacttgactgctgtattttctctctgttgtaaaactctttcctttgcaagcacagcaagtccctgtaataagataggcacaactgtctgatccaggtaggcacgagttggcaaagactggagatctaccttctgctttgatgacttttctgcattaatcttctcattttctactattctctcaacgttgtctgtgagaccgtactcagagtgaggattttctgcaacctgcgtttgtccctccagcatctgctctggctccatggcggaccctgcaagtcacagtccccggataccagtccgcgcccaagccgttcgttcttaagagccctgcaccgcgccaccagctcccagcacaaacagctccggccgtaagtgacggctgtcgcacgactgccgcgcctgcgc

SEQ ID NO: 17195 - RNA, 64 nt, Homo sapiens
  source 1..64: mol_type = other RNA
tcaggccaggcacagtggctcacacctgtaatcccagcactttgggaggccaaggtgggtggat

SEQ ID NO: 17196 - RNA, 2057 nt, Homo sapiens
  source 1..2057: mol_type = other RNA
tcaggccaggcacagtggctcacacctgtaatcccagcactttgggaggccgaggtgggcagatcactggaggtcaggagtttgagactagcctggccaacatggtgaaaccccatctctactaaaaatacaaaaattagccgggcgtggtgacacacacctgtagtcccagctacttgggaggctgaggccagagaatcacttgaacccgggaggtggaggttgcagtgagccaagatcacgacactagactccagcctgggtgacagagcgagacgcctaccaacaaaaacaaaaataaaaatatataaatacaaataaaaacaaatttttttgtagagacaggatctcactatgttgcccaggctggtctggaactcctggcctcaagctatcctcctgctttggcctcccaacaaagtgttgggattacaggcatcagtcactatgcctggctgaagtataaatttaaaaggcaaaagctaagaaatggaaactacacaattaaaaatcaaagttattttcatatttatagtacatgaaaataagtcttatatccaataatccaacagataatatattgaaggttatgcttttgaaaatttatcactgaccttcctgttggaagcacactttaagaacacacaaagttctaaataaaacaaataaaaaaagttctaaataaaacaaataaaagaaaaaaaaatgcaccatgtccttaaaacggtatcacaaagtgtaggagcatcttagtaacaccaaattataaccgcttttggggttgcaatattgatttagaaattccttcctagaaacaataatcaatgaggcatgtttgtcactgatcactcttctgttaatctgcttcatcctgttggaggactactttccctcttgttcattcttgttcgtatttgcatgcgttaggatgtgggctttcaggttatttgactgaataaacctcctgttgcagccttgaaagggacacacgaaacgtttctcccccgtgtggatgcgcacgtgcgtacgcaaattaaagtccagagagaagcgctttccgcacccttcaaaagtgcaccgaaacggcttctctccagtatgaaccaggaaatgtctctttagttttgagctctcaacgaacgctttcccacattccgcacagacgtggtctcggggaccatgaatgaggagatgctttctcagggcagctctattcctcaacttcctagtgcatccactctgaggacaagcgattgcgctcagactgtcatattctttatttatggggggcttctttctagcaaattctgcgagctgtttaggatctgataggtcaatgccaggtattcctccaggcggaagcttcttgcctgtcatgtactcagaatactcaagcgaattctctccaactatcttttgtggaagctctttctttaccccttttttcatgtattccaaagaacattcaagggagcttgcttcgaaaaccttttgagaaagctgttgttctgatcctttctttaggtattccaaggactcaaaaagtgagtcctcttccaggatgggttgagaaaactcaccccttatgacgcattctatgtaacagtctgagaaatcatcccctccgagagcctgagggccaggctcatagcacacatagccatcacataaggcccacaccgcgctgacaggttctatttccgcctgcaggtcttggcttgacttgccttgcctgggcttagccccactgggggctcttccacccaggcctttctggtgtcttgtctttgcccgtttcttcagttgctggctcatgttttcctgcctgtgcccttcttgaaggtttacaccaggatatatcaaccacctccaggcagtagtgatctgagtaagctgtcttcagcaaacacctgctggactgtgagcactactagagtgaaggcctcttctgttctgttcacacaggctccagcctcagtacatttgtccctgttaccgcgaagcactctgctatttccaatgccacctcctcccaaacgtaaaacaaaggagaaact

SEQ ID NO: 17197 - RNA, 2223 nt, Homo sapiens
  source 1..2223: mol_type = other RNA
tcaggccaggcacagtggctcacacctgtaatcccagcactttgggaggccgaggtgggcagatcactggaggtcaggagtttgagactagcctggccaacatggtgaaaccccatctctactaaaaatacaaaaattagccgggcgtggtgacacacacctgtagtcccagctacttgggaggctgaggccagagaatcacttgaacccgggaggtggaggttgcagtgagccaagatcacgacactagactccagcctgggtgacagagcgagacgcctaccaacaaaaacaaaaataaaaatatataaatacaaataaaaacaaatttttttgtagagacaggatctcactatgttgcccaggctggtctggaactcctggcctcaagctatcctcctgctttggcctcccaacaaagtgttgggattacaggcatcagtcactatgcctggctgaagtataaatttaaaaggcaaaagctaagaaatggaaactacacaattaaaaatcaaagttattttcatatttatagtacatgaaaataagtcttatatccaataatccaacagataatatattgaaggttatgcttttgaaaatttatcactgaccttcctgttggaagcacactttaagaacacacaaagttctaaataaaacaaataaaaaaagttctaaataaaacaaataaaagaaaaaaaaatgcaccatgtccttaaaacggtatcacaaagtgtaggagcatcttagtaacaccaaattataaccgcttttggggttgcaatattgatttagaaattccttcctagaaacaataatcaatgaggcatgtttgtcactgatcactcttctgttaatctgcttcatcctgttggaggactactttccctcttgttcattcttgttcgtatttgcatgcgttaggatgtgggctttcaggttatttgactgaataaacctcctgttgcagccttgaaagggacacacgaaacgtttctcccccgtgtggatgcgcacgtgcgtacgcaaattaaagtccagagagaagcgctttccgcacccttcaaaagtgcaccgaaacggcttctctccagtatgaaccaggaaatgtctctttagttttgagctctcaacgaacgctttcccacattccgcacagacgtggtctcggggaccatgaatgaggagatgctttctcagggcagctctattcctcaacttcctagtgcatccactctgaggacaagcgattgcgctcagactgtcatattctttatttatggggggcttctttctagcaaattctgcgagctgtttaggatctgataggtcaatgccaggtattcctccaggcggaagcttcttgcctgtcatgtactcagaatactcaagcgaattctctccaactatcttttgtggaagctctttctttaccccttttttcatgtattccaaagaacattcaagggagcttgcttcgaaaaccttttgagaaagctgttgttctgatcctttctttaggtattccaaggactcaaaaagtgagtcctcttccaggatgggttgagaaaactcaccccttatgacgcattctatgtaacagtctgagaaatcatcccctccgagagcctgagggccaggctcatagcacacatagccatcacataaggcccacaccgcgctgacaggttctatttccgcctgcaggtcttggcttgacttgccttgcctgggcttagccccactgggggctcttccacccaggcctttctggtgtcttgtctttgcccgtttcttcagttgctggctcatgttttcctgcctgtgcccttcttgaaggtttacaccaggatatatcaaccacctccaggcagtagtgatctgagtaagctgtcttcagcaaacacctgctggactgtgagcactactagagtgaaggcctcttctgttctgttcacacaggctccagcctcagtacatttgtttcagctcagcgatggttaggtctgaattcccaagggaggccgtgagtggggtgggtttgcctagtgtgctggtggtcagctattcaggaggctgaggtgggaggatcgctggagcctgggaggcaggggttgcagtgagctgagatcacaccattgcactccaacccctgttaccgcgaagcactctgctatttccaatgccacctcctcccaaacgtaaaacaaaggagaaact

SEQ ID NO: 17198 - RNA, 2771 nt, Homo sapiens
  source 1..2771: mol_type = other RNA
tcaggccaggcacagtggctcacacctgtaatcccagcactttgggaggccgaggtgggcgtatcacctgaggtcaggagttcaagaccagcctggccaacatggtgaaaccctgtctctactaaaaatagaagaattagctgggtggggtggcaggtgcctgtagtcccagctactcaggaggttgaggcaggagaatcgcttgaacctgggaggtggaggttgcagtgagatgagatcgcgccactgcactccagcctgggcaacagagtgagactctgtcttaaaaaaaaaacaaaaaaaagaactaaaagtagaactacctttcagtccagcagttccactactgggtatctacccaaaggaaacaaagtcattatgtgaaaaagacacatacacctgcatgtttatagcaacataattagcaattacaaaggcatggaaccaacctaagtgcccatcaaccaatgagtgataaagattgtggtatatgtacagcatggaatactacttatccataaaaaggaaccaaataatgtcttttgtagcaacttggatggaactggaggtcattactctaggtgaagtaactcaggaatgaaaaacctggacttgtttgtatgttcaaccaacatacataagatccatatgaacatatcgtatgttctcagttataagtgggagctaagctatgaggacacaaagggatatgaacaatataatgaactttggtgacttgaagggagaaaggttgggaggggggtgaggaataagagactactaccacttgggtgacgggtacactaaaaactcagaagtcaccactaaagaactcatccgtgtaatgaaaaaccacatgtaccccaaaaactactgacataaaaataaatttttttaaaaaaagaaaacatggtatgtatctacatatgtctatatctatatagatatcgaggatatatacaatggagtactactcagccataaaaaaggatgaaatcatgtcttttgcagcaacatcgatgggactggaagccattctcttaagtaaggtagtaaagaaacaaagtcaaatgctgcatgatctcacttataattgggagctaaacaatgtatacgcatgggcattataacagaataatggacactggagactgcaaaaggtgagaggggagtgagagtttaaaaactgccttggccgggcgtggtggctcacacctgtaatcccagcactttgagaggccaaggcaggtggatcacaaggtcaggagttcgagaccagcctggccaagatggtgaaaccccgtctctactaaaaggcatgggtggcacacacctgtaatctcagctactcaggaggctgagacagaagaatcacttgaacccgggaggcggaggttgcagtgagccgagatcactccactgcactccagcctgggagacagagtgagactccgtctcaaaaaagaaaaaaaagtgccttatgttcactattcaggtaattggtacgccaaaagctcagacttcacccttatgcaaatgcatgttaagaaatctgcatttgtactctcaaagtataaaaaaatgtttttaattttaaagagtaagaatttcaaaataaaacatttttgccattggtgctcacaaaacttcttagtcctggggccaagggatccatcacaaacaagaggctgccctgctgaggagactccccagggctcccttcacatccttgttcctcaggctgtagatgaaggggttcaacatgggggtgaccacagtgtacatcaccgaggccacggagattttctgggaagagtgagtcaccgcagaagtgaagtggaccccaatgcctgtcccataaaataaagaaacgacggagaggtgagacccacaggtggaaagtgctttttgttttcccccagatgaggacatcttccttatggatgaagcaattcgtgaataagagaaaatgatcccaaggaggggaaaaacgcccagcacacccgtcataaagtatatcaacgtgctgttcaggaaggtatcagagcaggccagctggaggatgtacgtcagttcgcagaaaaaatgtggaatttcaaaatctttacagaagattagatgcatcatcagagaaatatggaggagggatgtcatgacaccaatgagccaggtgacaaaaaccaggaggccacagaggtgggggttcatgatgatcatatagtgcagagggtggcagacagccacaaaccggtcataggccatcacggtcaggagtagcgtgtccagaataggaaaaaacatggagaaatagacctgtgtgaggcagtccatgtaggagatggctttgttctcggtctggatgttcaccagcatcttggggacgatgcaagtgctgaaacagatgtcaacccaggacaggttggagaggaagaagtacatgggggtgtggaggtgggagtcagagctgatggccaggatgatgagcaggtttcccagcaccgtcaccaggtacatggacaggaacagcccaaatatgaacggctgtagttctggatcctcagagagtccgagaaggataaactctaaaaatcctgtttggtttcctgcttccatgtagctgatgtatattgcttgaaaaaaaaaaatgctggtatgacgtcttcctcccctgactgttgaatgctgaagacagaatctagcagggaaaggcggggagatggaacttgtcatgaagtcatcctaactctcctctctaagatgcatgagtgtgg

SEQ ID NO: 17199 - RNA, 2862 nt, Homo sapiens
  source 1..2862: mol_type = other RNA
tcaggccaggcacagtggctcacacctgtaatcccagcactttgggaggccgaggtgggcgtatcacctgaggtcaggagttcaagaccagcctggccaacatggtgaaaccctgtctctactaaaaatagaagaattagctgggtggggtggcaggtgcctgtagtcccagctactcaggaggttgaggcaggagaatcgcttgaacctgggaggtggaggttgcagtgagatgagatcgcgccactgcactccagcctgggcaacagagtgagactctgtcttaaaaaaaaaacaaaaaaaagaactaaaagtagaactacctttcagtccagcagttccactactgggtatctacccaaaggaaacaaagtcattatgtgaaaaagacacatacacctgcatgtttatagcaacataattagcaattacaaaggcatggaaccaacctaagtgcccatcaaccaatgagtgataaagattgtggtatatgtacagcatggaatactacttatccataaaaaggaaccaaataatgtcttttgtagcaacttggatggaactggaggtcattactctaggtgaagtaactcaggaatgaaaaacctggacttgtttgtatgttcaaccaacatacataagatccatatgaacatatcgtatgttctcagttataagtgggagctaagctatgaggacacaaagggatatgaacaatataatgaactttggtgacttgaagggagaaaggttgggaggggggtgaggaataagagactactaccacttgggtgacgggtacactaaaaactcagaagtcaccactaaagaactcatccgtgtaatgaaaaaccacatgtaccccaaaaactactgacataaaaataaatttttttaaaaaaagaaaacatggtatgtatctacatatgtctatatctatatagatatcgaggatatatacaatggagtactactcagccataaaaaaggatgaaatcatgtcttttgcagcaacatcgatgggactggaagccattctcttaagtaaggtagtaaagaaacaaagtcaaatgctgcatgatctcacttataattgggagctaaacaatgtatacgcatgggcattataacagaataatggacactggagactgcaaaaggtgagaggggagtgagagtttaaaaactgccttggccgggcgtggtggctcacacctgtaatcccagcactttgagaggccaaggcaggtggatcacaaggtcaggagttcgagaccagcctggccaagatggtgaaaccccgtctctactaaaaggcatgggtggcacacacctgtaatctcagctactcaggaggctgagacagaagaatcacttgaacccgggaggcggaggttgcagtgagccgagatcactccactgcactccagcctgggagacagagtgagactccgtctcaaaaaagaaaaaaaagtgccttatgttcactattcaggtaattggtacgccaaaagctcagacttcacccttatgcaaatgcatgttaagaaatctgcatttgtactctcaaagtataaaaaaatgtttttaattttaaagagtaagaatttcaaaataaaacatttttgccattggtgctcacaaaacttcttagtcctggggccaagggatccatcacaaacaagaggctgccctgctgaggagactccccagggctcccttcacatccttgttcctcaggctgtagatgaaggggttcaacatgggggtgaccacagtgtacatcaccgaggccacggagattttctgggaagagtgagtcaccgcagaagtgaagtggaccccaatgcctgtcccataaaataaagaaacgacggagaggtgagacccacaggtggaaagtgctttttgttttcccccagatgaggacatcttccttatggatgaagcaattcgtgaataagagaaaatgatcccaaggaggggaaaaacgcccagcacacccgtcataaagtatatcaacgtgctgttcaggaaggtatcagagcaggccagctggaggatgtacgtcagttcgcagaaaaaatgtggaatttcaaaatctttacagaagattagatgcatcatcagagaaatatggaggagggatgtcatgacaccaatgagccaggtgacaaaaaccaggaggccacagaggtgggggttcatgatgatcatatagtgcagagggtggcagacagccacaaaccggtcataggccatcacggtcaggagtagcgtgtccagaataggaaaaaacatggagaaatagacctgtgtgaggcagtccatgtaggagatggctttgttctcggtctggatgttcaccagcatcttggggacgatgcaagtgctgaaacagatgtcaacccaggacaggttggagaggaagaagtacatgggggtgtggaggtgggagtcagagctgatggccaggatgatgagcaggtttcccagcaccgtcaccaggtacatggacaggaacagcccaaatatgaacggctgtagttctggatcctcagagagtccgagaaggataaactctaaaaatcctgtttggtttcctgcttccatgtagctgatgtatctgaagtttctttgtggcaagtccagatcacattctagaaaattttactttatccagatattccccaaggctttgtactcatcatggaaagattgcttgaaaaaaaaaaatgctggtatgacgtcttcctcccctgactgttgaatgctgaagacagaatctagcagggaaaggcggggagatggaacttgtcatgaagtcatcctaactctcctctctaagatgcatgagtgtgg

SEQ ID NO: 17200 - RNA, 506 nt, Homo sapiens
  source 1..506: mol_type = other RNA
tcaggccaggcacagtggctcacacctgtaatcccagcactttgggaggctgaggcgagcagatggcttgagttcatgagttcgagaccttggatgataattaaattggtaaattttttaagggaagaaaatacttatttcttcaagttgaatgtaacgcattgtcaattgctttcaggaagatcatgagaaaacactgttcacaatcttaggaagcagctaaaatttaggtttctgagtgtttaatacatttgttttagtgctttatttgatttagaattctgagaccaatatgagacaccatagccttctagaatttttactatggtgacacaaatcttcatctctcttgtcttctatccatccacaacatcatattttcctgacactcaagtaaagaacaaaagtgaaagtttgcatatccatgccttctggattagtccattttcatgctgctgataaagacatacccaagactgggcaatttacaaaagaaagaggtttca

SEQ ID NO: 17201 - RNA, 76 nt, Homo sapiens
  source 1..76: mol_type = other RNA
tcaggccaggcacagtggctcacacctgtaatcccagcattttgggagtccaaggcaggtggatcacttgagctcg

SEQ ID NO: 17202 - RNA, 2859 nt, Homo sapiens
  source 1..2859: mol_type = other RNA
tcaggccaggcacagtggctcacacctgtaatcccagcgctttgggaggccaagataggaggatgagttgagcccatgagttggagaccagcctgggcaacatagtgagaccccatctctactaaaaagtattaaaaagtagcagggtgaccaggcatggtggctcacacctgtaatcccagcactttgggaggctgaggcaggcagatcacaaggtcaagagatcgagactatcctggcaaacatggtgaaaccctgtctctactaaaaatacaaaacaaaacaaaacaaaacaaaagccaggcatggtggcacgcgcctgtagtcccagttactcgggaggctgaggcaggagaatcacttgaacctgggaggcagaggttgcagtgagctgagattgtgtcactgcactccagcctgggtaacagatcgagactcccatctcaaaaaaaaaaaaaaaaaaggagcagggcatggtggtgtgtgattgtggtcccagctactccagaggctgaggtgggaggatcccttgagccctggaggcggaggctacagtgacctatgatgccactgcactcccgcctaggcaacagaccctgtctcaaaaaaaaaaaaagtaattaaaaattttaaaattccttgaggagggctaaacaaggcatgcctgtgggcactgctgtgaggtctggcctagggatttgtagggccacagttagggggagctgaggcccatatatgaatggtggggcagagcactcagccaaacctggtggcctctctgcctcccgtcgaatgcagaatctcacccaagcgatgcccagtggctctgaccccgcctcagggtgcggcccctgggggtgagcctgccaggcacccccacctccctcccacaacatccagaagctctgggaaggaggggggaggtggttcccctccacaggggccaagggtcttggtcccactctccaagtacctgccacgacactgcaggaaggtgggctgcaggatgggggggtcagggaaccccgaagcacagacgggaacgtccttgtccccttggacgacccagggcccggggcgccctctggtggcgaatcttctcacagcctgactcaggatgcccccagcgctccaggggcaagaagagcacgaggcagacgcggtgggtctctgagaacttaaaataaccctcaccacgtggcggggtgggcgaggagggggctcacagcagaagcagagtggccccggggtgggggcgccacaggacactgagggttcacaccaccccagcctgggcctggtaagtagcaggtcagcataaatccaaccccgcgaggcacatccaaaccccacccagaggggttcaaatgacaggagtgggaacagaggggctccctgaggcttcaggccccatccccaggaagactggcccggcctcagccaccttcaagcacaggagtgaggcctcgggttccagggacgatgggggacccagcattaaatatgtcataaataggtgggcggacactgtgcggacaggcggggctcacattcctctagaccactggggtccactgggggaccagggcctgggccctctcccagcgatgccacgggcctgagagggctgctgggaaggagcccgggagccccctgcagtctgaagtccgggccgagggcacaggagcccgaggctcacggctgctttgtcttgcctctgttcttctggagcttggcatgcacgactttgagcgtggtcaggaagttgccgaggaagaggatgaggaaggtgaacgccagtacgaacacctgccattctctgcattcctcgtggctggagagctcaaacagcgtgacggcattgtagagctgccagaaatggccacagaagaggaagggcaggagaaaggtgaggccccgccacatccaggactggaacccttccactgtgagatccaggtggttcctctcccccagggcccgcagccggtagaggcagcccctctggtaataatattgcaggaactggacgcagctctgaaaaatggaaaatgctaagaactggttgcgaaacttctgataaatgggtccattaggccaggtcagcatcactccggacaggaatgtggagacgtagtggtgagacacccaccagcctttaattcttgagccgttgctgatgagaatgctctcccgaatggtcagggtgcagtaataccacaccagcaggaagttgaagacttcgtcagtcaccctgtagtgaaggacaaatcgacatgccacggcacccaggagcaggatgatggtcaggtagagcttgaacttctcatattcgtccttgtaggcgaacttggcctggttgctgaggagggtcacgttcacattgccgaggaccaggttcaagtagagcccgttcttcttgggcaggtaggcctccatgtcgaagaagacgtcctgccgctccttgatgttcgctgccatctgctgaacgagctccgcctcctcccgactggcatggcgtttgcacctctggagtgtaagcttcaagtccttgaggtgcttcttctgcttactgatggaactgctacacagcgtctgcagcgcagccagctcctccagcttctgcttgtagatcctgtgcgtctcctgcagttcttgaaattctccctccagctcgtgccattcgcgctcgcaacgctccagctgcccggacatgatgcgatggtgcaaggcggcggtgccggcggctgctcccgcagcgctgcccgaccggccccccagcgccccacgcccgcgcgctcgccgaccgccctcggaggcaccagctgttcctgcgcagccagagccacgcgcgcaact

SEQ ID NO: 17203 - RNA, 3303 nt, Homo sapiens
  source 1..3303: mol_type = other RNA
tcaggccaggcacagtggctcacacctgtaatcccagtgctttgggaggctgaggcaggaggatcatgaggtcaggagttcgagaccagcctggccaacatagtgaaaccccatgtctactaaaaatacaaaaaattagctgggcgtggtgtcaggcgcccgtaattccagtgactcaggaggctgaggcaggagaatcgcttgaactggggaggcggaggttgcagtgagctgagatcgcgccgttgcactccagcctgggcaacgagtgaaactcctgtgaatgttgtaactaccaggctgaaattcatgtctgttggtcagcacatgctcttcctggtaggaaaaatctgtgtagatgacttgcttttattgtaacaaaggcaactggccctgtaatcggagtcaccaggctgctgtttactgtgttccgaaatgccttctctaaggactatccatagagacagctctctggtctcaattcagagatggttgggttcctctgagcactggtttgcctttatctgataggcacagacattatctattagtaaaaataaaataataattttattaagacccctaaatcatgatgcccaaaccccttgcaatcaggaagtctagataaataacaggagtttcccttcatagagatttctggaattacccaaggatattaacatgcatgacccagatgcctccctaagccttatggtgtgctggcaaatgtttaacaaccattattcagaaataagacaggaaaactgccatctatgactggtaagattataggtgatttttgtattttttttcttcattttcccaacttccttcaggaaacacattttactctgaagggggtgagggtggtggctaatacttgggattatggtgagctgccctagaaactatcgggttattaagtaacacttaatatatgtaccagtttcacttcaaaatctgaagcattctgaactcttaattattttggagggatatcccacagaaaagttggctgaggccctagtgataaagctctttcttacagtggcccattcctgcccaagactccaggcactggaaaacctggtgggggtggagaaggtaacatcagcaggcaagtactcggaaccactctcctatctcctacctcttcttctcacgacctccaaaactctgctgagaccggcctccctctgcctcacttgtggtgattttctctcggatgctcactttctctctgtgcaatctttcctttgggtgtcccttgtctttaaacatgtctgcgtatacctgaactctaattgtggacagggttcaaagttctttttcatgggattcatgggccccatgaaaattagaggctaagtaggcatctaagtaggagcatttacgtgctcccaggcattctgttacacttaaagaggctcatggaagagatttgggcaagtggtataactctacaagctgctatattcaagtcctagttccagcttagccaaaacacctactccgattgcaactgatctttttcttggttgctagaaaactgagagtcatatgtgtggcctacctccagcaaaccaataggaccttacaccatgcattttgcatacaaaactgctggcttaatcttatctttcacactcacggttttcttttgtcctatttttctctgtacttatttttaatttaccctgatgtacacatttatgtaaactacgttaaatcctttcctctggaataaagtagggtgtaaataaatttaacaaaacaacaaagagtgatgatgagccaggtcttcactcctgaaggcctcaaaacgaactggcagtgatctgtgaaaactacagagaactgcccgttcatctccacagattactgaagtctgtgaaaactactccagccaggaccaccattatagcctgctgcctgttgtgttcacaatcgatgcacaaactcaaccctgaaatggagagaaaaataggggaaaaaagacattaggaaatcctagctctatgtcatctggacattagaaagcacttggttggacaaagctttttctcccccacagcacatgcctgtttcagcatctcagcccacattcacggagagggagaatatagcaattgttaagaatgcagactctagcactgcatgctctgctgtttatttgtgttatttgggctaggttttttaaccgtctgtgcctcggtgaatcccatctacaaagtagagataataatagtacctacctcacagggcagttgtaaggattaaatgaggtaacccgggtgtaacatttaaaacagtggcagagtacatacagggatctgaacaaatgttagctactattagtgatatgtgagtgggggaagcacactgccttggacttgaggcaatatcaagtctgagtttctggaaaaacacttgtggaataagtaagggctggccacctcctaaaaccggacaaaagatctggcttgcctagatccttagcgtgactgcttctcctcctgcctttctagaggcagtattacgtgatggaaatacttggtgggtgctgtgggcacaaagataagttaatgtgtttttattccctaggagctgagtcgagagtaggagaaaaatgcataaataattaccaggtaggatgattaagcaatatactggaggcagcaacagaaacacaccgtggaaaaaaaatacccacggcgtggatgaagatatgagatgtgtgaaagcgctagacacaggcagccacctgcacccatgtaaaattggattattgctgactcctacaaggcccactttaacgcttctttcaaccagaatccctgcagaactaattttgtagaaccgccggggataaagacctttatttgcaatgtcgaactccagcagagtaaccccttttgctttccacacgcgcaaacccgggtcccaaacgctgcagttcgcgtttcccggctaacggaagaaacacgaggaactgtttgcagatctaggggatgaagccaaaaaacggaaagcgaggccgaaagggcgcaaccaccacgtctggaggaggccagtgaagtagagaaaggggaaggtcagccctgccccagcgcgctctgcgtaaccgggacttcctccgcgcggcaaagccggggaacctccctggcgcctgcgccaccgtggcgagactcggcgccgtggacgtggagagagggcgacgcacctgcgcgaagacggcagcgggagaagccgctccagtgcggttgcgcggcggcccaggcgtcgaggggagcctcggcgggg

SEQ ID NO: 17204 - RNA, 3321 nt, Homo sapiens
  source 1..3321: mol_type = other RNA
tcaggccaggcacagtggctcacacctgtaatcccagtgctttgggaggctgaggcaggaggatcatgaggtcaggagttcgagaccagcctggccaacatagtgaaaccccatgtctactaaaaatacaaaaaattagctgggcgtggtgtcaggcgcccgtaattccagtgactcaggaggctgaggcaggagaatcgcttgaactggggaggcggaggttgcagtgagctgagatcgcgccgttgcactccagcctgggcaacgagtgaaactcctgtgtagatgacttgcttttattgtaacaaaggcaactggccctgtaatcggagtcaccaggctgctgtttactgtgttccgaaatgccttctctaaggactatccatagagacagctctctggtctcaattcagagatggttgggttcctctgagcactggtttgcctttatctgataggcacagacattatctattagtaaaaataaaataataattttattaagacccctaaatcatgatgcccaaaccccttgcaatcaggaagtctagataaataacaggagtttcccttcatagagatttctggaattacccaaggatattaacatgcatgacccagatgcctccctaagccttatggtgtgctggcaaatgtttaacaaccattattcagaaataagacaggaaaactgccatctatgactggtaagattataggtgatttttgtattttttttcttcattttcccaacttccttcaggaaacacattttactctgaagggggtgagggtggtggctaatacttgggattatggtgagctgccctagaaactatcgggttattaagtaacacttaatatatgtaccagtttcacttcaaaatctgaagcattctgaactcttaattattttggagggatatcccacagaaaagttggctgaggccctagtgataaagctctttcttacagtggcccattcctgcccaagactccaggcactggaaaacctggtgggggtggagaaggtaacatcagcaggcaagtactcggaaccactctcctatctcctacctcttcttctcacgacctccaaaactctgctgagaccggcctccctctgcctcacttgtggtgattttctctcggatgctcactttctctctgtgcaatctttcctttgggtgtcccttgtctttaaacatgtctgcgtatacctgaactctaattgtggacagggttcaaagttctttttcatgggattcatgggccccatgaaaattagaggctaagtaggcatctaagtaggagcatttacgtgctcccaggcattctgttacacttaaagaggctcatggaagagatttgggcaagtggtataactctacaagctgctatattcaagtcctagttccagcttagccaaaacacctactccgattgcaactgatctttttcttggttgctagaaaactgagagtcatatgtgtggcctacctccagcaaaccaataggaccttacaccatgcattttgcatacaaaactgctggcttaatcttatctttcacactcacggttttcttttgtcctatttttctctgtacttatttttaatttaccctgatgtacacatttatgtaaactacgttaaatcctttcctctggaataaagtagggtgtaaataaatttaacaaaacaacaaagagtgatgatgagccaggtcttcactcctgaaggcctcaaaacgaactggcagtgatctgtgaaaactacagagaactgcccgttcatctccacagattactgaagtctgtgaaaactactccagccaggaccaccattatagcctgctgcctgttgtgttcacaatcgatgcacaaactcaaccctgaaatggagagaaaaataggggaaaaaagacattaggaaatcctagctctatgtcatctggacattagaaagcacttggttggacaaagctttttctcccccacagcacatgcctgtttcagcatctcagcccacattcacggagagggagaatatagcaattgttaagaatgcagactctagcactgcatgctctgctgtttatttgtgttatttgggctaggttttttaaccgtctgtgcctcggtgaatcccatctacaaagtagagataataatagtacctacctcacagggcagttgtaaggattaaatgaggtaacccgggtgtaacatttaaaacagtggcagagtacatacagggatctgaacaaatgttagctactattagtgatatgtgagtgggggaagcacactgccttggacttgaggcaatatcaagtctgagtttctggaaaaacacttgtggaataagtaagggctggccacctcctaaaaccggacaaaagatctggcttgcctagatccttagcgtgactgcttctcctcctgcctttctagaggcagtattacgtgatggaaatacttggtgggtgctgtgggcacaaagataagttaatgtgtttttattccctaggagctgagtcgagagtaggagaaaaatgcataaataattaccaggtaggatgattaagcaatatactggaggcagcaacagaaacacaccgtggaaaaaaaatacccacggcgtggatgaagatatgagatgtgtgaaagcgctagacacaggcagccacctgcacccatgtaaaattggattattgctgactcctacaaggcccactttaacgcttctttcaaccagaatccctgcagaactaattttgtagaaccgccggggataaagacctttatttgcaatgtcgaactccagcagagtaaccccttttgctttccacacgcgcaaacccgggtcccaaacgctgcagttcgcgtttcccggctaacggaagaaacacgaggaactgtttgcagatctaggggatgaagccaaaaaacggaaagcgaggccgaaagggcgcaaccaccacgtctggaggaggccagtgaagtagagaaaggggaaggtcagccctgccccagcgcgctctgcgtaaccgggacttcctccgcgcggcaaagccggggaacctccctggcgcctgcgccaccgtggcgagactcggcgccgtggacgtggagagagggcgacgcacctgcgcgaagacggcagcgggagaagccgctccagtgcggttgcgcggcggcccaggcgtcgaggggagcctcggcggggagcgcaccgcgcgcctgcgcggagagctgcgtgacgcggcggcgcgcaagggacgtgcggagtgagtggcgctgcgggtggggccgtcggc

SEQ ID NO: 17205 - RNA, 3260 nt, Homo sapiens
  source 1..3260: mol_type = other RNA
tcaggccaggcacagtggctcacacctgtaatccgagcactttgggaagccgaggtaggagggtaactgtagcccaggagttcaagactagactgggcaacatagtgagaccccatctctactgctaccctccaaaaccattaaaaaaacaggaatgcaggctgggtgcggtggctcatgcctgtaatcccagcactttgggaggtcaaggcgggcggatcatgaggtcaggagttcgagaccagcctggccaacatggtgaaaccctgtctctactaaaaataccacaaattagctgggcgtagtggcgggcgcctgtaatcctagctactcgggaggctgatgcaggagaatcgcttgaacccgggaggcagaggtttcagtgagctgaggtcgcaccactgcactccagcctgggtgacagagcgagactctgtctcaaaaaaaaaaaaaaaaaaaaaaaacaaaaaacacacagaaaacaggaatgcataggataaaactatgtacgtagctggttgaggaggaggttctctaggacagcattcctgtctacaaacagtaaaaatttgagttttatttaaagttatcaccacttggactatcatgctgtaaacttctgcttattctgttacaaccaggtggcttctctagtctgtttttctttagattatgtctaagaaataatgatagacctatggtcttttaaagatagttcatcaaacacaagtgaatacaactttagactttggtggaacctcttactaatgatgtagagttccgcctcttagattcatgaactgtgataactcagataaggatggtaactgcagaaataatatatataaagagaaatcactcctgggtgatgtcattttccatgtagcccagtatgcccatgttgaaaagttttgttttcaaagcagtgtactgatgtgataatggggaataacatttttttatgagggaaccctttaaaatggatgcacacagtggcattttctcctaggctcaaagctgagtacactcccgtaattttaataatattttaggcaagtcctatgacaattataccaacaagtttcttcaaccccaccaccaccccaccatctctatgctttgcttgcccagactcccttcaccctttcctctgctattaccgcttatggttgaaagtaaaaagcatctccagattacagcaaattcagtggccctgctccatagcctggcctctgctgaaggaagaaaaggggtgaaacatgaacagccatcatgggttgtgatgaggcactaccagaagcccagcttgtgtttcaaaaacaggctcttggacactttcccagcagataactcttcactggcttggagaacaggaaggactatttcacaaacaccactgtgtttgaatttctagaggctacccaggccaagaatacatccctgcagtgcttcaccacacactcattgctgcagtattcattgtcccagtccttactcacaatgggagggttctcacaaccagacctcacacatcgaggctggggtgagagtgccacaggagacccactcaccaattcaacatccatctgagaaggagactcaacctcaggaactacatctgtgatcatctcacagatagtctcaggagaaggtgcctccactgtatgggcctcagggctgttgttcataggccgctcaggactactttccacagttggtgggactaaggtagtctgcattttcaaagtgggtagaggcacactcttgatctgcagaggaggaggctgttgctgtaaattgattcgaactttctgaggtggaggctgttgcatggcctggagtggaggaggctgctgcagaatggtaacttgctgctgagtcgggggctgtggcatctgttgtaatggagggggctgtagtcggggtggaggcagttgcatagaagcagcagcagcagcagctgctgctgcctgcaacactgaccgagtgacaatctgggcttgttgactgggctggatagtagctgtactggtttggcctagttggagcccccgggaggtcaccactgtggctgggataacagtaaccatccctccttgagacatagtaatagaagagggcaacatttgtttggtaataatcaacttggtgatattgggctgacccccagctccagaagatgcctggtttgccacataggatgaaagggtggagttaacaacaatggatggggacagggcagggggctctattgaagctggtgctggagatgctgggtcaacagtagccataggaggtggagaaggagtttgtgatggtggtgctggatccaattccactgtttccacagtggcctgacactcctggttgtctttgtaagcagccagtgccttcagatactctttcttggcagcctcagttttcctcttatatacctgtttttgctcctctccaagactatcccacatggaggccacaatttttgaaacctcaccaaaagtggcattaggattctgtcccttgatggcagcctgtgtatcacgaaagaataaagcatatgctgaaactggtttctgaggttcattaggatctttcttttttctcttctttggggccttctgctttttccctgcttccaccacgactgtcttctggctgggaagttgcctccggaaatcctcaacaccatcctcgtgaagtgaactagtaggtgaaggggtggttgaaagacgatcttcaggtgactgggcaggtggcaggatggtgccaccccctaggctcaaacccagctgggaactcagttctgactgatcaatggtggtcaactggctatgccccatcaagccagatgtcatgtctgtcattggtacatcaattgtaacaggtgggttggcactatactgagttcctatagagtggtccaagtccatggtcaagcccccactcaggagccccccgccctgctccatcaagccatgggtcatgcccacaggcatgtccaatgtctggaccccatactgggctgaaaaactgccatcctgtgaagaggaagggtctgccaggtcatcaaagtggccaaccacatctgagacagccaatgagggatcagaatccaaggagataggtgggatttcaaattcctcatcacccaagcttggtgtatggaatgtctccatcttcacacaaccgctcccaccgtctcagaccctcatcgctcccaccgcccccactggactcggaactgccgtcacttccgcaag

SEQ ID NO: 17206 - RNA, 3329 nt, Homo sapiens
  source 1..3329: mol_type = other RNA
tcaggccaggcacagtggctcacacctgtaatccgagcactttgggaagccgaggtaggagggtaactgtagcccaggagttcaagactagactgggcaacatagtgagaccccatctctactgctaccctccaaaaccattaaaaaaacaggaatgcaggctgggtgcggtggctcatgcctgtaatcccagcactttgggaggtcaaggcgggcggatcatgaggtcaggagttcgagaccagcctggccaacatggtgaaaccctgtctctactaaaaataccacaaattagctgggcgtagtggcgggcgcctgtaatcctagctactcgggaggctgatgcaggagaatcgcttgaacccgggaggcagaggtttcagtgagctgaggtcgcaccactgcactccagcctgggtgacagagcgagactctgtctcaaaaaaaaaaaaaaaaaaaaaaaacaaaaaacacacagaaaacaggaatgcataggataaaactatgtacgtagctggttgaggaggaggttctctaggacagcattcctgtctacaaacagtaaaaatttgagttttatttaaagttatcaccacttggactatcatgctgtaaacttctgcttattctgttacaaccaggtggcttctctagtctgtttttctttagattatgtctaagaaataatgatagacctatggtcttttaaagatagttcatcaaacacaagtgaatacaactttagactttggtggaacctcttactaatgatgtagagttccgcctcttagattcatgaactgtgataactcagataaggatggtaactgcagaaataatatatataaagagaaatcactcctgggtgatgtcattttccatgtagcccagtatgcccatgttgaaaagttttgttttcaaagcagtgtactgatgtgataatggggaataacatttttttatgagggaaccctttaaaatggatgcacacagtggcattttctcctaggctcaaagctgagtacactcccgtaattttaataatattttaggcaagtcctatgacaattataccaacaagtttcttcaaccccaccaccaccccaccatctctatgctttgcttgcccagactcccttcaccctttcctctgctattaccgcttatggttgaaagtaaaaagcatctccagattacagcaaattcagtggccctgctccatagcctggcctctgctgaaggaagaaaaggggtgaaacatgaacagccatcatgggttgtgatgaggcactaccagaagcccagcttgtgtttcaaaaacaggctcttggacactttcccagcagataactcttcactggcttggagaacaggaaggactatttcacaaacaccactgtgtttgaatttctagaggctacccaggccaagaatacatccctgcagtgcttcaccacacactcattgctgcagtattcattgtcccagtccttactcacaatgggagggttctcacaaccagacctcacacatcgaggctggggtgagagtgccacaggagacccactcaccaattcaacatccatctgagaaggagactcaacctcaggaactacatctgtgatcatctcacagatagtctcaggagaaggtgcctccactgtatgggcctcagggctgttgttcataggccgctcaggactactttccacagttggtgggactaaggtagtctgcattttcaaagtgggtagaggcacactcttgatctgcagaggaggaggctgttgctgtaaattgattcgaactttctgaggtggaggctgttgcatggcctggagtggaggaggctgctgcagaatggtaacttgctgctgagtcgggggctgtggcatctgttgtaatggagggggctgtagtcggggtggaggcagttgcatagaagcagcagcagcagcagctgctgctgcctgcaacactgaccgagtgacaatctgggcttgttgactgggctggatagtagctgtactggtttggcctagttggagcccccgggaggtcaccactgtggctgggataacagtaaccatccctccttgagacatagtaatagaagagggcaacatttgtttggtaataatcaacttggtgatattgggctgacccccagctccagaagatgcctggtttgccacataggatgaaagggtggagttaacaacaatggatggggacagggcagggggctctattgaagctggtgctggagatgctgggtcaacagtagccataggaggtggagaaggagtttgtgatggtggtgctggatccaattccactgtttccacagtggcctgacactcctggttgtctttgtaagcagccagtgccttcagatactctttcttggcagcctcagttttcctcttatatacctgtttttgctcctctccaagactatcccacatggaggccacaatttttgaaacctcaccaaaagtggcattaggattctgtcccttgatggcagcctgtgtatcacgaaagaataaagcatatgctgaaactggtttctgaggttcattaggatctttcttttttctcttctttggggccttctgctttttccctgcttccaccacgactgtcttctggctgggaagttgcctccggaaatcctcaacaccatcctcgtgaagtgaactagtaggtgaaggggtggttgaaagacgatcttcaggtgactgggcaggtggcaggatggtgccaccccctaggctcaaacccagctgggaactcagttctgactgatcaatggtggtcaactggctatgccccatcaagccagatgtcatgtctgtcattggtacatcaattgtaacaggtgggttggcactatactgagttcctatagagtggtccaagtccatggtcaagcccccactcaggagccccccgccctgctccatcaagccatgggtcatgcccacaggcatgtccaatgtctggaccccatactgggctgaaaaactgccatcctgtgaagaggaagggtctgccaggtcatcaaagtggccaaccacatctgagacagccaatgagggatcagaatccaaggagataggtgggatttcaaattcctcatcacccaagcttggtgtatggaatgtctcggcccctgacaggaaggggtgcgaaggccctgtgatcgtcaggtaattgtcatttcctccgggaaactccatcttcacacaaccgctcccaccgtctcagaccctcatcgctcccaccgcccccactggactcggaactgccgtcacttccgcaag

SEQ ID NO: 17207 - RNA, 4710 nt, Homo sapiens
  source 1..4710: mol_type = other RNA
tcaggccaggcacagtggctcacacctgtaatcctagcactttcggaggccgaggtgggtggatcacttgaggtcagggtcttcaagacagggtcttcctatattacccaggctgtccttgaactcctgcactcaaatgatcctcccacctcagcctctcaaatagcagggactatagatgcacagcaccatgcctggcttccaaaatggatgaatcttatttcactatgctaagtgaaataagccagtcacaggacaaatattgcatgatcccactatatgagatatctgtaatagtcaaactcatagaaacagggtagaagggtggttgctaggggccagggaaatggagagttgttcaacaggtataaagcttcagttatgcaagacaagtaaggtctaaagatctgttgtacaacatggtgcctggaattaacaatactatatcgtgcacttaaagatttgttaagagggtaggtcttgagttaagtgttcttaccacagaagacaaaacaaaaactcaacagcaaccaaaaagcaaaaaacaaaggggcaggaggaaacttgtggagatgacaggtatgtttattaccctgattgtggtgatggtatcaaaggtgtgtgcatatagtcagacccatcaaattgtattcattaaatatgtaacaactgtacttctataaagctggtaaaaaacactgtacctgtttgtttttacttcaacgtggctataagaaaatataaaattacattacagcttgcattctatttgtatagtactgtcctgctcaagatggattaacaggtgtgtgacactcactgcctgctgagagcagggtgtagggaacctggggttggaaaggagacttgtcaccgtatgctcttccatttatcaatatttcatattttgagaagacatgaactttttgaacaaagataacagaaaatcattgtcaatagttaatctaccagagagattcagaaaccttgcatacttggttttcaggtcttggttgagagttctaacaccgttgaaaaatctcaagagtaacctggtaatgatatcttcattgaattaaaattacattttgctttaatctgatagtcctcttaatccaaaaggtcaacatcaagttaaacaacatccagtttcactttgatgttcatagctgccagttcagctacaaaataccgaaaaacataaggcacagaaacagtatcgatagtgtcactgcgactacacagagtacagttgtattttctgttgcgcatggcagaccaagaagggggtggcttctccaacagtggagagagtaaactgccacacttcacacacacatgggctaccgaccgatctgagcagttgaagaggcggtcatgaaggagaaaagatgtaccatgagctaaaagcgcatcccgttccatctccccaaaacggattccaccctggacatttcttcccccaataggctggttggtgactctgtctcgggctccagttgtccttacttgaaatttgtctgagaccatatggcgtaagcgctgataataaaccactcctatgaagatgtctgcttccagttctagcccactgatgccactatataacctctcggtgccatagaaattgtagccagcagcctttaacatctcaccaaagtattctaaggccgagttctcctctgagaagatgaagggtgtagcatcatggcagagaccatgcaaagctgcagacttcccggccatactctcaattaacatcccaatggtcatgcgggatggaaaaccatggggattgaacagaatgtctgggaccatcccactctcagtaaaaggcatgtcctcagccggccacaatctgcttaaaatgcccttctgcccatggcgactggcaaatttatctccgatagttgggttccgaggcactctcatagtgatgcaaacacacttgaattttccactcccagtgtcattactgcacactttgatgttatccacaacacaattttctttactcttatagtacatcacaaaactttccccggtgttgaggttgaggtagctgtaatacggatctccgtactgcagttttgctcctataaacggcaatccatcgtcatctaacttctgcagaacgcgtgggtcaccaggtttgatgccaaacaccaggctactatctccttgtttaattttttcagagaggtctatgaactcagacttgtagacacttccatgggcaaagcctcgttcccaagaggccttattcacaatcatggcatcttccatatcatagccagtgtaagaaatcacagcaacgatggcattggtcccaattggatagttatccatgtcataataatcatacatggagggtctcaccaagggactctgaggagtctgaagacgatacagtttgttatccgatcggtcttgataagtgagaagtggaaagcccatagtttgcttacccatctggcattggtacatgttccgtggactctggttgtgatcagagaaagggatgaagttggcaatcacactcagcaggctgtgtggaaagagttcctggtgtgtggtaactccagcaaaaacttcatcctcaaagatagcgacattcatgaagatctgttccatagttccaattagctcttctttgcccaatgctaagttctgcacaggccgtaccagtctacaaggagtggtaaaaaggaacaatcctgggtacagacttggttttcctgtcatgggtataaggaccacttccatccagggaggaattcttttctctctcaacacccaggcatggtggtgtgcacctgtaatcccagctacttgggagaccgaggcaggagaattgcttgaacatgggaggcggaggctgcagtgagccaagatcacaccactgcactgcagcctgggcgacagagcgagactcttaaaatgacgaagagaatctgcgatgcctggagcaagatccttatccacccagccaaccatgacaccgtccagcaggacagggtagcactcactgtatgatcggtggggagctccatcaatgggagtgacccccaagttgcacagtaaagctggaatagatgccgtatacacaaactgtgtgacaacctcacatacggcagttaggtggttcatcaggccacagggctccccgtctggggtatgcacgggacaaaggaagccccaggactctggcagcagcctgcgtactgtggtggtcctcatcttggcaaaatcagcccctctgtgcacgcagcggaaatgggagaggtagcgtatgaagttcagcttgtcagccacaacacaaagtccagaatcttgtaggaggccaagacctgttttagaacgcagattcccagtagcaaaaaggtattcaaatggttttgtaaggtctatgcccattgtaaaaatcctcatcaaattgtcagtgttcatggaaacactggtcttctgagccttcttatcaaaagctattttaatagacactaaccaaccttccagtttttccttcaggaacataaggaagagctgacccggtgtgaggacttcctggttcaccaaactatcaggattgtcctccatgcactctcctttggctaaagcaaagagctttcgcgtcatgagacaaagcatataaaacttttcagtattggatttcaagtggatacagatgcactggttaaacaggaactccgcagcttgctcatttgggtaccagtcaggaacattgagttttactctgaagcattcacctaggtagttaaggacctgtttttgtgtcgaacaaccctcttccattacaatccttaacatctgagaaacagagttcctaaggaaagaatcatcctcttttcctttgatgagctcctgaaagatctgataatcagaaaagctgacaagtgccttaagtgcaaatcccaaaggaagaaagaacagttcttttcggtaaataaagttcaacataacagtgccattttccaagtagtggaggttcatattgacagcggaatgttcttccctcacacagtgcattgaaactccatactgagtataaccaggccctctggttttccattttggtcttatcattgcaatgggaaaatttctccgaggcataatcaacattcggatgactttttcaatgccattgattataaaatagccccccatttcctctgcctcctcatggtgctcaatgagggcttgtgggggaaggttacgtaagttgcaaagcttggatttcaccatgatgggaacatagccaagaaactgcttaatgattccttttgagattccattcactgcccagttgatatcagctgtcaacttcccacggtaggtactccttcggccccggcattctgctggataaacattggcctctttgcagatggtcccttttggaactgtaggtggactgataacagcatccagaatagtaaaagagatacgctcatctttgaaagcaaattcaaagggaggtatagcctgcaccgcgaggccgagaccctcgtgcacagcgtagttgaaggactccacgtgcgcccgcgtcagctcctgcaacgctgccttttgctgttcccgcgggattccataagaggggtcagtcaagtgctttaggctaggcccgctgggcaggttccgccaccggctgccaggatccatgtggccacctgcacaccggacgccagtctc

SEQ ID NO: 17208 - RNA, 4404 nt, Homo sapiens
  source 1..4404: mol_type = other RNA
tcaggccaggcacagtggctcacacctgtaatcctagcactttcggaggccgaggtgggtggatcacttgaggtcagggtcttcaagacagggtcttcctatattacccaggctgtccttgaactcctgcactcaaatgatcctcccacctcagcctctcaaatagcagggactatagatgcacagcaccatgcctggcttccaaaatggatgaatcttatttcactatgctaagtgaaataagccagtcacaggacaaatattgcatgatcccactatatgagatatctgtaatagtcaaactcatagaaacagggtagaagggtggttgctaggggccagggaaatggagagttgttcaacaggtataaagcttcagttatgcaagacaagtaaggtctaaagatctgttgtacaacatggtgcctggaattaacaatactatatcgtgcacttaaagatttgttaagagggtaggtcttgagttaagtgttcttaccacagaagacaaaacaaaaactcaacagcaaccaaaaagcaaaaaacaaaggggcaggaggaaacttgtggagatgacaggtatgtttattaccctgattgtggtgatggtatcaaaggtgtgtgcatatagtcagacccatcaaattgtattcattaaatatgtaacaactgtacttctataaagctggtaaaaaacactgtacctgtttgtttttacttcaacgtggctataagaaaatataaaattacattacagcttgcattctatttgtatagtactgtcctgctcaagatggattaacaggtgtgtgacactcactgcctgctgagagcagggtgtagggaacctggggttggaaaggagacttgtcaccgtatgctcttccatttatcaatatttcatattttgagaagacatgaactttttgaacaaagataacagaaaatcattgtcaatagttaatctaccagagagattcagaaaccttgcatacttggttttcaggtcttggttgagagttctaacaccgttgaaaaatctcaagagtaacctggtaatgatatcttcattgaattaaaattacattttgctttaatctgatagtcctcttaatccaaaaggtcaacatcaagttaaacaacatccagtttcactttgatgttcatagctgccagttcagctacaaaataccgaaaaacataaggcacagaaacagtatcgatagtgtcactgcgactacacagagtacagttgtattttctgttgcgcatggcagaccaagaagggggtggcttctccaacagtggagagagtaaactgccacacttcacacacacatgggctaccgaccgatctgagcagttgaagaggcggtcatgaaggagaaaagatgtaccatgagctaaaagcgcatcccgttccatctccccaaaacggattccaccctggacatttcttcccccaataggctggttggtgactctgtctcgggctccagttgtccttacttgaaatttgtctgagaccatatggcgtaagcgctgataataaaccactcctatgaagatgtctgcttccagttctagcccactgatgccactatataacctctcggtgccatagaaattgtagccagcagcctttaacatctcaccaaagtattctaaggccgagttctcctctgagaagatgaagggtgtagcatcatggcagagaccatgcaaagctgcagacttcccggccatactctcaattaacatcccaatggtcatgcgggatggaaaaccatggggattgaacagaatgtctgggaccatcccactctcagtaaaaggcatgtcctcagccggccacaatctgcttaaaatgcccttctgcccatggcgactggcaaatttatctccgatagttgggttccgaggcactctcatagtgatgcaaacacacttgaattttccactcccagtgtcattactgcacactttgatgttatccacaacacaattttctttactcttatagtacatcacaaaactttccccggtgttgaggttgaggtagctgtaatacggatctccgtactgcagttttgctcctataaacggcaatccatcgtcatctaacttctgcagaacgcgtgggtcaccaggtttgatgccaaacaccaggctactatctccttgtttaattttttcagagaggtctatgaactcagacttgtagacacttccatgggcaaagcctcgttcccaagaggccttattcacaatcatggcatcttccatatcatagccagtgtaagaaatcacagcaacgatggcattggtcccaattggatagttatccatgtcataataatcatacatggagggtctcaccaagggactctgaggagtctgaagacgatacagtttgttatccgatcggtcttgataagtgagaagtggaaagcccatagtttgcttacccatctggcattggtacatgttccgtggactctggttgtgatcagagaaagggatgaagttggcaatcacactcagcaggctgtgtggaaagagttcctggtgtgtggtaactccagcaaaaacttcatcctcaaagatagcgacattcatgaagatctgttccatagttccaattagctcttctttgcccaatgctaagttctgcacaggccgtaccagtctacaaggagtggtaaaaaggaacaatcctgggtacagacttggttttcctgtcatgggtataaggaccacttccatccagggaggaattcttttctctctcaacaccttaaaatgacgaagagaatctgcgatgcctggagcaagatccttatccacccagccaaccatgacaccgtccagcaggacagggtagcactcactgtatgatcggtggggagctccatcaatgggagtgacccccaagttgcacagtaaagctggaatagatgccgtatacacaaactgtgtgacaacctcacatacggcagttaggtggttcatcaggccacagggctccccgtctggggtatgcacgggacaaaggaagccccaggactctggcagcagcctgcgtactgtggtggtcctcatcttggcaaaatcagcccctctgtgcacgcagcggaaatgggagaggtagcgtatgaagttcagcttgtcagccacaacacaaagtccagaatcttgtaggaggccaagacctgttttagaacgcagattcccagtagcaaaaaggtattcaaatggttttgtaaggtctatgcccattgtaaaaatcctcatcaaattgtcagtgttcatggaaacactggtcttctgagccttcttatcaaaagctattttaatagacactaaccaaccttccagtttttccttcaggaacataaggaagagctgacccggtgtgaggacttcctggttcaccaaactatcaggattgtcctccatgcactctcctttggctaaagcaaagagctttcgcgtcatgagacaaagcatataaaacttttcagtattggatttcaagtggatacagatgcactggttaaacaggaactccgcagcttgctcatttgggtaccagtcaggaacattgagttttactctgaagcattcacctaggtagttaaggacctgtttttgtgtcgaacaaccctcttccattacaatccttaacatctgagaaacagagttcctaaggaaagaatcatcctcttttcctttgatgagctcctgaaagatctgataatcagaaaagctgacaagtgccttaagtgcaaatcccaaaggaagaaagaacagttcttttcggtaaataaagttcaacataacagtgccattttccaagtagtggaggttcatattgacagcggaatgttcttccctcacacagtgcattgaaactccatactgagtataaccaggccctctggttttccattttggtcttatcattgcaatgggaaaatttctccgaggcataatcaacattcggatgactttttcaatgccattgattataaaatagccccccatttcctctgcctcctcatggtgctcaatgagggcttgtgggggaaggttacgtaagttgcaaagcttggatttcaccatgatgggaacatagccaagaaactgcttaatgattccttttgagattccattcactgcccagttgatatcagcctgcaccgcgaggccgagaccctcgtgcacagcgtagttgaaggactccacgtgcgcccgcgtcagctcctgcaacgctgccttttgctgttcccgcgggattccataagaggggtcagtcaagtgctttaggctaggcccgctgggcaggttccgccaccggctgccaggatccatgtggccacctgcacaccggacgccagtctc

SEQ ID NO: 17209 - RNA, 4572 nt, Homo sapiens
  source 1..4572: mol_type = other RNA
tcaggccaggcacagtggctcacacctgtaatcctagcactttcggaggccgaggtgggtggatcacttgaggtcagggtcttcaagacagggtcttcctatattacccaggctgtccttgaactcctgcactcaaatgatcctcccacctcagcctctcaaatagcagggactatagatgcacagcaccatgcctggcttccaaaatggatgaatcttatttcactatgctaagtgaaataagccagtcacaggacaaatattgcatgatcccactatatgagatatctgtaatagtcaaactcatagaaacagggtagaagggtggttgctaggggccagggaaatggagagttgttcaacaggtataaagcttcagttatgcaagacaagtaaggtctaaagatctgttgtacaacatggtgcctggaattaacaatactatatcgtgcacttaaagatttgttaagagggtaggtcttgagttaagtgttcttaccacagaagacaaaacaaaaactcaacagcaaccaaaaagcaaaaaacaaaggggcaggaggaaacttgtggagatgacaggtatgtttattaccctgattgtggtgatggtatcaaaggtgtgtgcatatagtcagacccatcaaattgtattcattaaatatgtaacaactgtacttctataaagctggtaaaaaacactgtacctgtttgtttttacttcaacgtggctataagaaaatataaaattacattacagcttgcattctatttgtatagtactgtcctgctcaagatggattaacaggtgtgtgacactcactgcctgctgagagcagggtgtagggaacctggggttggaaaggagacttgtcaccgtatgctcttccatttatcaatatttcatattttgagaagacatgaactttttgaacaaagataacagaaaatcattgtcaatagttaatctaccagagagattcagaaaccttgcatacttggttttcaggtcttggttgagagttctaacaccgttgaaaaatctcaagagtaacctggtaatgatatcttcattgaattaaaattacattttgctttaatctgatagtcctcttaatccaaaaggtcaacatcaagttaaacaacatccagtttcactttgatgttcatagctgccagttcagctacaaaataccgaaaaacataaggcacagaaacagtatcgatagtgtcactgcgactacacagagtacagttgtattttctgttgcgcatggcagaccaagaagggggtggcttctccaacagtggagagagtaaactgccacacttcacacacacatgggctaccgaccgatctgagcagttgaagaggcggtcatgaaggagaaaagatgtaccatgagctaaaagcgcatcccgttccatctccccaaaacggattccaccctggacatttcttcccccaataggctggttggtgactctgtctcgggctccagttgtccttacttgaaatttgtctgagaccatatggcgtaagcgctgataataaaccactcctatgaagatgtctgcttccagttctagcccactgatgccactatataacctctcggtgccatagaaattgtagccagcagcctttaacatctcaccaaagtattctaaggccgagttctcctctgagaagatgaagggtgtagcatcatggcagagaccatgcaaagctgcagacttcccggccatactctcaattaacatcccaatggtcatgcgggatggaaaaccatggggattgaacagaatgtctgggaccatcccactctcagtaaaaggcatgtcctcagccggccacaatctgcttaaaatgcccttctgcccatggcgactggcaaatttatctccgatagttgggttccgaggcactctcatagtgatgcaaacacacttgaattttccactcccagtgtcattactgcacactttgatgttatccacaacacaattttctttactcttatagtacatcacaaaactttccccggtgttgaggttgaggtagctgtaatacggatctccgtactgcagttttgctcctataaacggcaatccatcgtcatctaacttctgcagaacgcgtgggtcaccaggtttgatgccaaacaccaggctactatctccttgtttaattttttcagagaggtctatgaactcagacttgtagacacttccatgggcaaagcctcgttcccaagaggccttattcacaatcatggcatcttccatatcatagccagtgtaagaaatcacagcaacgatggcattggtcccaattggatagttatccatgtcataataatcatacatggagggtctcaccaagggactctgaggagtctgaagacgatacagtttgttatccgatcggtcttgataagtgagaagtggaaagcccatagtttgcttacccatctggcattggtacatgttccgtggactctggttgtgatcagagaaagggatgaagttggcaatcacactcagcaggctgtgtggaaagagttcctggtgtgtggtaactccagcaaaaacttcatcctcaaagatagcgacattcatgaagatctgttccatagttccaattagctcttctttgcccaatgctaagttctgcacaggccgtaccagtctacaaggagtggtaaaaaggaacaatcctgggtacagacttggttttcctgtcatgggtataaggaccacttccatccagggaggaattcttttctctctcaacaccttaaaatgacgaagagaatctgcgatgcctggagcaagatccttatccacccagccaaccatgacaccgtccagcaggacagggtagcactcactgtatgatcggtggggagctccatcaatgggagtgacccccaagttgcacagtaaagctggaatagatgccgtatacacaaactgtgtgacaacctcacatacggcagttaggtggttcatcaggccacagggctccccgtctggggtatgcacgggacaaaggaagccccaggactctggcagcagcctgcgtactgtggtggtcctcatcttggcaaaatcagcccctctgtgcacgcagcggaaatgggagaggtagcgtatgaagttcagcttgtcagccacaacacaaagtccagaatcttgtaggaggccaagacctgttttagaacgcagattcccagtagcaaaaaggtattcaaatggttttgtaaggtctatgcccattgtaaaaatcctcatcaaattgtcagtgttcatggaaacactggtcttctgagccttcttatcaaaagctattttaatagacactaaccaaccttccagtttttccttcaggaacataaggaagagctgacccggtgtgaggacttcctggttcaccaaactatcaggattgtcctccatgcactctcctttggctaaagcaaagagctttcgcgtcatgagacaaagcatataaaacttttcagtattggatttcaagtggatacagatgcactggttaaacaggaactccgcagcttgctcatttgggtaccagtcaggaacattgagttttactctgaagcattcacctaggtagttaaggacctgtttttgtgtcgaacaaccctcttccattacaatccttaacatctgagaaacagagttcctaaggaaagaatcatcctcttttcctttgatgagctcctgaaagatctgataatcagaaaagctgacaagtgccttaagtgcaaatcccaaaggaagaaagaacagttcttttcggtaaataaagttcaacataacagtgccattttccaagtagtggaggttcatattgacagcggaatgttcttccctcacacagtgcattgaaactccatactgagtataaccaggccctctggttttccattttggtcttatcattgcaatgggaaaatttctccgaggcataatcaacattcggatgactttttcaatgccattgattataaaatagccccccatttcctctgcctcctcatggtgctcaatgagggcttgtgggggaaggttacgtaagttgcaaagcttggatttcaccatgatgggaacatagccaagaaactgcttaatgattccttttgagattccattcactgcccagttgatatcagctgtcaacttcccacggtaggtactccttcggccccggcattctgctggataaacattggcctctttgcagatggtcccttttggaactgtaggtggactgataacagcatccagaatagtaaaagagatacgctcatctttgaaagcaaattcaaagggaggtatagcctgcaccgcgaggccgagaccctcgtgcacagcgtagttgaaggactccacgtgcgcccgcgtcagctcctgcaacgctgccttttgctgttcccgcgggattccataagaggggtcagtcaagtgctttaggctaggcccgctgggcaggttccgccaccggctgccaggatccatgtggccacctgcacaccggacgccagtctc

SEQ ID NO: 17210 - RNA, 4772 nt, Homo sapiens
  source 1..4772: mol_type = other RNA
tcaggccaggcacagtggctcacacctgtaatcctagcactttcggaggccgaggtgggtggatcacttgaggtcagggtcttcaagacagggtcttcctatattacccaggctgtccttgaactcctgcactcaaatgatcctcccacctcagcctctcaaatagcagggactatagatgcacagcaccatgcctggcttccaaaatggatgaatcttatttcactatgctaagtgaaataagccagtcacaggacaaatattgcatgatcccactatatgagatatctgtaatagtcaaactcatagaaacagggtagaagggtggttgctaggggccagggaaatggagagttgttcaacaggtataaagcttcagttatgcaagacaagtaaggtctaaagatctgttgtacaacatggtgcctggaattaacaatactatatcgtgcacttaaagatttgttaagagggtaggtcttgagttaagtgttcttaccacagaagacaaaacaaaaactcaacagcaaccaaaaagcaaaaaacaaaggggcaggaggaaacttgtggagatgacaggtatgtttattaccctgattgtggtgatggtatcaaaggtgtgtgcatatagtcagacccatcaaattgtattcattaaatatgtaacaactgtacttctataaagctggtaaaaaacactgtacctgtttgtttttacttcaacgtggctataagaaaatataaaattacattacagcttgcattctatttgtatagtactgtcctgctcaagatggattaacaggtgtgtgacactcactgcctgctgagagcagggtgtagggaacctggggttggaaaggagacttgtcaccgtatgctcttccatttatcaatatttcatattttgagaagacatgaactttttgaacaaagataacagaaaatcattgtcaatagttaatctaccagagagattcagaaaccttgcatacttggttttcaggtcttggttgagagttctaacaccgttgaaaaatctcaagagtaacctggtaatgatatcttcattgaattaaaattacattttgctttaatctgatagtcctcttaatccaaaaggtcaacatcaagttaaacaacatccagtttcactttgatgttcatagctgccagttcagctacaaaataccgaaaaacataaggcacagaaacagtatcgatagtgtcactgcgactacacagagtacagttgtattttctgttgcgcatggcagaccaagaagggggtggcttctccaacagtggagagagtaaactgccacacttcacacacacatgggctaccgaccgatctgagcagttgaagaggcggtcatgaaggagaaaagatgtaccatgagctaaaagcgcatcccgttccatctccccaaaacggattccaccctggacatttcttcccccaataggctggttggtgactctgtctcgggctccagttgtccttacttgaaatttgtctgagaccatatggcgtaagcgctgataataaaccactcctatgaagatgtctgcttccagttctagcccactgatgccactatataacctctcggtgccatagaaattgtagccagcagcctttaacatctcaccaaagtattctaaggccgagttctcctctgagaagatgaagggtgtagcatcatggcagagaccatgcaaagctgcagacttcccggccatactctcaattaacatcccaatggtcatgcgggatggaaaaccatggggattgaacagaatgtctgggaccatcccactctcagtaaaaggcatgtcctcagccggccacaatctgcttaaaatgcccttctgcccatggcgactggcaaatttatctccgatagttgggttccgaggcactctcatagtgatgcaaacacacttgaattttccactcccagtgtcattactgcacactttgatgttatccacaacacaattttctttactcttatagtacatcacaaaactttccccggtgttgaggttgaggtagctgtaatacggatctccgtactgcagttttgctcctataaacggcaatccatcgtcatctaacttctgcagaacgcgtgggtcaccaggtttgatgccaaacaccaggctactatctccttgtttaattttttcagagaggtctatgaactcagacttgtagacacttccatgggcaaagcctcgttcccaagaggccttattcacaatcatggcatcttccatatcatagccagtgtaagaaatcacagcaacgatggcattggtcccaattggatagttatccatgtcataataatcatacatggagggtctcaccaagggactctgaggagtctgaagacgatacagtttgttatccgatcggtcttgataagtgagaagtggaaagcccatagtttgcttacccatctggcattggtacatgttccgtggactctggttgtgatcagagaaagggatgaagttggcaatcacactcagcaggctgtgtggaaagagttcctggtgtgtggtaactccagcaaaaacttcatcctcaaagatagcgacattcatgaagatctgttccatagttccaattagctcttctttgcccaatgctaagttctgcacaggccgtaccagtctacaaggagtggtaaaaaggaacaatcctgggtacagacttggttttcctgtcatgggtataaggaccacttccatccagggaggaattcttttctctctcaacaccttaaaatgacgaagagaatctgcgatgcctggagcaagatccttatccacccagccaaccatgacaccgtccagcaggacagggtagcactcactgtatgatcggtggggagctccatcaatgggagtgacccccaagttgcacagtaaagctggaatagatgccgtatacacaaactgtgtgacaacctcacatacggcagttaggtggttcatcaggccacagggctccccgtctggggtatgcacgggacaaaggaagccccaggactctggcagcagcctgcgtactgtggtggtcctcatcttggcaaaatcagcccctctgtgcacgcagcggaaatgggagaggtagcgtatgaagttcagcttgtcagccacaacacaaagtccagaatcttgtaggaggccaagacctgttttagaacgcagattcccagtagcaaaaaggtattcaaatggttttgtaaggtctatgcccattgtaaaaatcctcatcaaattgtcagtgttcatggaaacactggtcttctgagccttcttatcaaaagctattttaatagacactaaccaaccttccagtttttccttcaggaacataaggaagagctgacccggtgtgaggacttcctggttcaccaaactatcaggattgtcctccatgcactctcctttggctaaagcaaagagctttcgcgtcatgagacaaagcatataaaacttttcagtattggatttcaagtggatacagatgcactggttaaacaggaactccgcagcttgctcatttgggtaccagtcaggaacattgagttttactctgaagcattcacctaggtagttaaggacctgtttttgtgtcgaacaaccctcttccattacaatccttaacatctgagaaacagagttcctaaggaaagaatcatcctcttttcctttgatgagctcctgaaagatctgataatcagaaaagctgacaagtgccttaagtgcaaatcccaaaggaagaaagaacagttcttttcggtaaataaagttcaacataacagtgccattttccaagtagtggaggttcatattgacagcggaatgttcttccctcacacagtgcattgaaactccatactgagtataaccaggccctctggttttccattttggtcttatcattgcaatgggaaaatttctccgaggcataatcaacattcggatgactttttcaatgccattgattataaaatagccccccatttcctctgcctcctcatggtgctcaatgagggcttgtgggggaaggttacgtaagttgcaaagcttggatttcaccatgatgggaacatagccaagaaactgcttaatgattccttttgagattccattcactgcccagttgatatcagctgtcaacttcccacggtaggtactccttcggccccggcattctgctggataaacattggcctctttgcagatggtcccttttggaactgtaggtggactgataacagcatccagaatagtaaaagagatacgctcatctttgaaagcaaattcaaagggaggtatagcctgcaccgcgaggccgagaccctcgtgcacagcgtagttgaaggactccacgtgcgcccgcgtcagctcctgcaacgctgccttttgctgttcccgcgggattccataagaggggtcagtcaagtgctttaggctaggcccgctgggcaggttccgccaccggctgccaggatccatgtggccacctgcacaccggacgccagtctctcggtacacgccggacgccagtctctcggtacacgccggaagtagtggccgcagtcccgtttccgcagcctctttggctctcattggctcagtcaattaggatcggaggagagcggtcttctcaggctctcttctgtttcccttcacctgttcccagtcccacgctgatgccgaccctggggagtcatccggccaaagtc

SEQ ID NO: 17211 - RNA, 4830 nt, Homo sapiens
  source 1..4830: mol_type = other RNA
tcaggccaggcacagtggctcacacctgtaatcctagcactttcggaggccgaggtgggtggatcacttgaggtcagggtcttcaagacagggtcttcctatattacccaggctgtccttgaactcctgcactcaaatgatcctcccacctcagcctctcaaatagcagggactatagatgcacagcaccatgcctggcttccaaaatggatgaatcttatttcactatgctaagtgaaataagccagtcacaggacaaatattgcatgatcccactatatgagatatctgtaatagtcaaactcatagaaacagggtagaagggtggttgctaggggccagggaaatggagagttgttcaacaggtataaagcttcagttatgcaagacaagtaaggtctaaagatctgttgtacaacatggtgcctggaattaacaatactatatcgtgcacttaaagatttgttaagagggtaggtcttgagttaagtgttcttaccacagaagacaaaacaaaaactcaacagcaaccaaaaagcaaaaaacaaaggggcaggaggaaacttgtggagatgacaggtatgtttattaccctgattgtggtgatggtatcaaaggtgtgtgcatatagtcagacccatcaaattgtattcattaaatatgtaacaactgtacttctataaagctggtaaaaaacactgtacctgtttgtttttacttcaacgtggctataagaaaatataaaattacattacagcttgcattctatttgtatagtactgtcctgctcaagatggattaacaggtgtgtgacactcactgcctgctgagagcagggtgtagggaacctggggttggaaaggagacttgtcaccgtatgctcttccatttatcaatatttcatattttgagaagacatgaactttttgaacaaagataacagaaaatcattgtcaatagttaatctaccagagagattcagaaaccttgcatacttggttttcaggtcttggttgagagttctaacaccgttgaaaaatctcaagagtaacctggtaatgatatcttcattgaattaaaattacattttgctttaatctgatagtcctcttaatccaaaaggtcaacatcaagttaaacaacatccagtttcactttgatgttcatagctgccagttcagctacaaaataccgaaaaacataaggcacagaaacagtatcgatagtgtcactgcgactacacagagtacagttgtattttctgttgcgcatggcagaccaagaagggggtggcttctccaacagtggagagagtaaactgccacacttcacacacacatgggctaccgaccgatctgagcagttgaagaggcggtcatgaaggagaaaagatgtaccatgagctaaaagcgcatcccgttccatctccccaaaacggattccaccctggacatttcttcccccaataggctggttggtgactctgtctcgggctccagttgtccttacttgaaatttgtctgagaccatatggcgtaagcgctgataataaaccactcctatgaagatgtctgcttccagttctagcccactgatgccactatataacctctcggtgccatagaaattgtagccagcagcctttaacatctcaccaaagtattctaaggccgagttctcctctgagaagatgaagggtgtagcatcatggcagagaccatgcaaagctgcagacttcccggccatactctcaattaacatcccaatggtcatgcgggatggaaaaccatggggattgaacagaatgtctgggaccatcccactctcagtaaaaggcatgtcctcagccggccacaatctgcttaaaatgcccttctgcccatggcgactggcaaatttatctccgatagttgggttccgaggcactctcatagtgatgcaaacacacttgaattttccactcccagtgtcattactgcacactttgatgttatccacaacacaattttctttactcttatagtacatcacaaaactttccccggtgttgaggttgaggtagctgtaatacggatctccgtactgcagttttgctcctataaacggcaatccatcgtcatctaacttctgcagaacgcgtgggtcaccaggtttgatgccaaacaccaggctactatctccttgtttaattttttcagagaggtctatgaactcagacttgtagacacttccatgggcaaagcctcgttcccaagaggccttattcacaatcatggcatcttccatatcatagccagtgtaagaaatcacagcaacgatggcattggtcccaattggatagttatccatgtcataataatcatacatggagggtctcaccaagggactctgaggagtctgaagacgatacagtttgttatccgatcggtcttgataagtgagaagtggaaagcccatagtttgcttacccatctggcattggtacatgttccgtggactctggttgtgatcagagaaagggatgaagttggcaatcacactcagcaggctgtgtggaaagagttcctggtgtgtggtaactccagcaaaaacttcatcctcaaagatagcgacattcatgaagatctgttccatagttccaattagctcttctttgcccaatgctaagttctgcacaggccgtaccagtctacaaggagtggtaaaaaggaacaatcctgggtacagacttggttttcctgtcatgggtataaggaccacttccatccagggaggaattcttttctctctcaacaccttaaaatgacgaagagaatctgcgatgcctggagcaagatccttatccacccagccaaccatgacaccgtccagcaggacagggtagcactcactgtatgatcggtggggagctccatcaatgggagtgacccccaagttgcacagtaaagctggaatagatgccgtatacacaaactgtgtgacaacctcacatacggcagttaggtggttcatcaggccacagggctccccgtctggggtatgcacgggacaaaggaagccccaggactctggcagcagcctgcgtactgtggtggtcctcatcttggcaaaatcagcccctctgtgcacgcagcggaaatgggagaggtagcgtatgaagttcagcttgtcagccacaacacaaagtccagaatcttgtaggaggccaagacctgttttagaacgcagattcccagtagcaaaaaggtattcaaatggttttgtaaggtctatgcccattgtaaaaatcctcatcaaattgtcagtgttcatggaaacactggtcttctgagccttcttatcaaaagctattttaatagacactaaccaaccttccagtttttccttcaggaacataaggaagagctgacccggtgtgaggacttcctggttcaccaaactatcaggattgtcctccatgcactctcctttggctaaagcaaagagctttcgcgtcatgagacaaagcatataaaacttttcagtattggatttcaagtggatacagatgcactggttaaacaggaactccgcagcttgctcatttgggtaccagtcaggaacattgagttttactctgaagcattcacctaggtagttaaggacctgtttttgtgtcgaacaaccctcttccattacaatccttaacatctgagaaacagagttcctaaggaaagaatcatcctcttttcctttgatgagctcctgaaagatctgataatcagaaaagctgacaagtgccttaagtgcaaatcccaaaggaagaaagaacagttcttttcggtaaataaagttcaacataacagtgccattttccaagtagtggaggttcatattgacagcggaatgttcttccctcacacagtgcattgaaactccatactgagtataaccaggccctctggttttccattttggtcttatcattgcaatgggaaaatttctccgaggcataatcaacattcggatgactttttcaatgccattgattataaaatagccccccatttcctctgcctcctcatggtgctcaatgagggcttgtgggggaaggttacgtaagttgcaaagcttggatttcaccatgatgggaacatagccaagaaactgcttaatgattccttttgagattccattcactgcccagttgatatcagctgtcaacttcccacggtaggtactccttcggccccggcattctgctggataaacattggcctctttgcagatggtcccttttggaactgtaggtggactgataacagcatccagaatagtaaaagagatacgctcatctttgaaagcaaattcaaagggaggtatagcctgtaatcccaatatttgggagaccgagagaggaggactacttgagctcaggagtttgagaccaggctgggccacatagggagaccccgtctctacaaaaaataaaaataaaaaaattagccgggcatagtggtgcacgcctgtggtcccagctactcaagaggttgacgtgggaggatcacttgatcctggaaggtcgaggctgcagtgagctataaccatgccactgcattccagcctaggtgacaaagtgagatcctgcaccgcgaggccgagaccctcgtgcacagcgtagttgaaggactccacgtgcgcccgcgtcagctcctgcaacgctgccttttgctgttcccgcgggattccataagaggggtcagtcaagtgctttaggctaggcccgctgggcaggttccgccaccggctgccaggatccatgtggccacctgcacaccggacgccagtctc

SEQ ID NO: 17212 - RNA, 4664 nt, Homo sapiens
  source 1..4664: mol_type = other RNA
tcaggccaggcacagtggctcacacctgtaatcctagcactttcggaggccgaggtgggtggatcacttgaggtcagggtcttcaagacagggtcttcctatattacccaggctgtccttgaactcctgcactcaaatgatcctcccacctcagcctctcaaatagcagggactatagatgcacagcaccatgcctggcttccaaaatggatgaatcttatttcactatgctaagtgaaataagccagtcacaggacaaatattgcatgatcccactatatgagatatctgtaatagtcaaactcatagaaacagggtagaagggtggttgctaggggccagggaaatggagagttgttcaacaggtataaagcttcagttatgcaagacaagtaaggtctaaagatctgttgtacaacatggtgcctggaattaacaatactatatcgtgcacttaaagatttgttaagagggtaggtcttgagttaagtgttcttaccacagaagacaaaacaaaaactcaacagcaaccaaaaagcaaaaaacaaaggggcaggaggaaacttgtggagatgacaggtatgtttattaccctgattgtggtgatggtatcaaaggtgtgtgcatatagtcagacccatcaaattgtattcattaaatatgtaacaactgtacttctataaagctggtaaaaaacactgtacctgtttgtttttacttcaacgtggctataagaaaatataaaattacattacagcttgcattctatttgtatagtactgtcctgctcaagatggattaacaggtgtgtgacactcactgcctgctgagagcagggtgtagggaacctggggttggaaaggagacttgtcaccgtatgctcttccatttatcaatatttcatattttgagaagacatgaactttttgaacaaagataacagaaaatcattgtcaatagttaatctaccagagagattcagaaaccttgcatacttggttttcaggtcttggttgagagttctaacaccgttgaaaaatctcaagagtaacctggtaatgatatcttcattgaattaaaattacattttgctttaatctgatagtcctcttaatccaaaaggtcaacatcaagttaaacaacatccagtttcactttgatgttcatagctgccagttcagctacaaaataccgaaaaacataaggcacagaaacagtatcgatagtgtcactgcgactacacagagtacagttgtattttctgttgcgcatggcagaccaagaagggggtggcttctccaacagtggagagagtaaactgccacacttcacacacacatgggctaccgaccgatctgagcagttgaagaggcggtcatgaaggagaaaagatgtaccatgagctaaaagcgcatcccgttccatctccccaaaacggattccaccctggacatttcttcccccaataggctggttggtgactctgtctcgggctccagttgtccttacttgaaatttgtctgagaccatatggcgtaagcgctgataataaaccactcctatgaagatgtctgcttccagttctagcccactgatgccactatataacctctcggtgccatagaaattgtagccagcagcctttaacatctcaccaaagtattctaaggccgagttctcctctgagaagatgaagggtgtagcatcatggcagagaccatgcaaagctgcagacttcccggccatactctcaattaacatcccaatggtcatgcgggatggaaaaccatggggattgaacagaatgtctgggaccatcccactctcagtaaaaggcatgtcctcagccggccacaatctgcttaaaatgcccttctgcccatggcgactggcaaatttatctccgatagttgggttccgaggcactctcatagtgatgcaaacacacttgaattttccactcccagtgtcattactgcacactttgatgttatccacaacacaattttctttactcttatagtacatcacaaaactttccccggtgttgaggttgaggtagctgtaatacggatctccgtactgcagttttgctcctataaacggcaatccatcgtcatctaacttctgcagaacgcgtgggtcaccaggtttgatgccaaacaccaggctactatctccttgtttaattttttcagagaggtctatgaactcagacttgtagacacttccatgggcaaagcctcgttcccaagaggccttattcacaatcatggcatcttccatatcatagccagtgtaagaaatcacagcaacgatggcattggtcccaattggatagttatccatgtcataataatcatacatggagggtctcaccaagggactctgaggagtctgaagacgatacagtttgttatccgatcggtcttgataagtgagaagtggaaagcccatagtttgcttacccatctggcattggtacatgttccgtggactctggttgtgatcagagaaagggatgaagttggcaatcacactcagcaggctgtgtggaaagagttcctggtgtgtggtaactccagcaaaaacttcatcctcaaagatagcgacattcatgaagatctgttccatagttccaattagctcttctttgcccaatgctaagttctgcacaggccgtaccagtctacaaggagtggtaaaaaggaacaatcctgggtacagacttggttttcctgtcatgggtataaggaccacttccatccagggaggaattcttttctctctcaacaccttaaaatgacgaagagaatctgcgatgcctggagcaagatccttatccacccagccaaccatgacaccgtccagcaggacagggtagcactcactgtatgatcggtggggagctccatcaatgggagtgacccccaagttgcacagtaaagctggaatagatgccgtatacacaaactgtgtgacaacctcacatacggcagttaggtggttcatcaggccacagggctccccgtctggggtatgcacgggacaaaggaagccccaggactctggcagcagcctgcgtactgtggtggtcctcatcttggcaaaatcagcccctctgtgcacgcagcggaaatgggagaggtagcgtatgaagttcagcttgtcagccacaacacaaagtccagaatcttgtaggaggccaagacctgttttagaacgcagattcccagtagcaaaaaggtattcaaatggttttgtaaggtctatgcccattgtaaaaatcctcatcaaattgtcagtgttcatggaaacactggtcttctgagccttcttatcaaaagctattttaatagacactaaccaaccttccagtttttccttcaggaacataaggaagagctgacccggtgtgaggacttcctggttcaccaaactatcaggattgtcctccatgcactctcctttggctaaagcaaagagctttcgcgtcatgagacaaagcatataaaacttttcagtattggatttcaagtggatacagatgcactggttaaacaggaactccgcagcttgctcatttgggtaccagtcaggaacattgagttttactctgaagcattcacctaggtagttaaggacctgtttttgtgtcgaacaaccctcttccattacaatccttaacatctgagaaacagagttcctaaggaaagaatcatcctcttttcctttgatgagctcctgaaagatctgataatcagaaaagctgacaagtgccttaagtgcaaatcccaaaggaagaaagaacagttcttttcggtaaataaagttcaacataacagtgccattttccaagtagtggaggttcatattgacagcggaatgttcttccctcacacagtgcattgaaactccatactgagtataaccaggccctctggttttccattttggtcttatcattgcaatgggaaaatttctccgaggcataatcaacattcggatgactttttcaatgccattgattataaaatagccccccatttcctctgcctcctcatggtgctcaatgagggcttgtgggggaaggttacgtaagttgcaaagcttggatttcaccatgatgggaacatagccaagaaactgcttaatgattccttttgagattccattcactgcccagttgatatcagctgtcaacttcccacggtaggtactccttcggccccggcattctgctggataaacattggcctctttgcagatggtcccttttggaactgtaggtggactgataacagcatccagaatagtaaaagagatacgctcatctttgaaagcaaattcaaagggaggtatagcctgtaatcccaatatttgggagaccgagagaggaggactacttgagctcaggagtttgagaccaggctgggccacatagggagaccccgtctctgcaccgcgaggccgagaccctcgtgcacagcgtagttgaaggactccacgtgcgcccgcgtcagctcctgcaacgctgccttttgctgttcccgcgggattccataagaggggtcagtcaagtgctttaggctaggcccgctgggcaggttccgccaccggctgccaggatccatgtggccacctgcacaccggacgccagtctc

SEQ ID NO: 17213 - RNA, 4501 nt, Homo sapiens
  source 1..4501: mol_type = other RNA
tcaggccaggcacagtggctcacacctgtaatcctagcactttcggaggccgaggtgggtggatcacttgaggtcagggtcttcaagacagggtcttcctatattacccaggctgtccttgaactcctgcactcaaatgatcctcccacctcagcctctcaaatagcagggactatagatgcacagcaccatgcctggcttccaaaatggatgaatcttatttcactatgctaagtgaaataagccagtcacaggacaaatattgcatgatcccactatatgagatatctgtaatagtcaaactcatagaaacagggtagaagggtggttgctaggggccagggaaatggagagttgttcaacaggtataaagcttcagttatgcaagacaagtaaggtctaaagatctgttgtacaacatggtgcctggaattaacaatactatatcgtgcacttaaagatttgttaagagggtaggtcttgagttaagtgttcttaccacagaagacaaaacaaaaactcaacagcaaccaaaaagcaaaaaacaaaggggcaggaggaaacttgtggagatgacaggtatgtttattaccctgattgtggtgatggtatcaaaggtgtgtgcatatagtcagacccatcaaattgtattcattaaatatgtaacaactgtacttctataaagctggtaaaaaacactgtacctgtttgtttttacttcaacgtggctataagaaaatataaaattacattacagcttgcattctatttgtatagtactgtcctgctcaagatggattaacaggtgtgtgacactcactgcctgctgagagcagggtgtagggaacctggggttggaaaggagacttgtcaccgtatgctcttccatttatcaatatttcatattttgagaagacatgaactttttgaacaaagataacagaaaatcattgtcaatagttaatctaccagagagattcagaaaccttgcatacttggttttcaggtcttggttgagagttctaacaccgttgaaaaatctcaagagtaacctggtaatgatatcttcattgaattaaaattacattttgctttaatctgatagtcctcttaatccaaaaggtcaacatcaagttaaacaacatccagtttcactttgatgttcatagctgccagttcagctacaaaataccgaaaaacataaggcacagaaacagtatcgatagtgtcactgcgactacacagagtacagttgtattttctgttgcgcatggcagaccaagaagggggtggcttctccaacagtggagagagtaaactgccacacttcacacacacatgggctaccgaccgatctgagcagttgaagaggcggtcatgaaggagaaaagatgtaccatgagctaaaagcgcatcccgttccatctccccaaaacggattccaccctggacatttcttcccccaataggctggttggtgactctgtctcgggctccagttgtccttacttgaaatttgtctgagaccatatggcgtaagcgctgataataaaccactcctatgaagatgtctgcttccagttctagcccactgatgccactatataacctctcggtgccatagaaattgtagccagcagcctttaacatctcaccaaagtattctaaggccgagttctcctctgagaagatgaagggtgtagcatcatggcagagaccatgcaaagctgcagacttcccggccatactctcaattaacatcccaatggtcatgcgggatggaaaaccatggggattgaacagaatgtctgggaccatcccactctcagtaaaaggcatgtcctcagccggccacaatctgcttaaaatgcccttctgcccatggcgactggcaaatttatctccgatagttgggttccgaggcactctcatagtgatgcaaacacacttgaattttccactcccagtgtcattactgcacactttgatgttatccacaacacaattttctttactcttatagtacatcacaaaactttccccggtgttgaggttgaggtagctgtaatacggatctccgtactgcagttttgctcctataaacggcaatccatcgtcatctaacttctgcagaacgcgtgggtcaccaggtttgatgccaaacaccaggctactatctccttgtttaattttttcagagaggtctatgaactcagacttgtagacacttccatgggcaaagcctcgttcccaagaggccttattcacaatcatggcatcttccatatcatagccagtgtaagaaatcacagcaacgatggcattggtcccaattggatagttatccatgtcataataatcatacatggagggtctcaccaagggactctgaggagtctgaagacgatacagtttgttatccgatcggtcttgataagtgagaagtggaaagcccatagtttgcttacccatctggcattggtacatgttccgtggactctggttgtgatcagagaaagggatgaagttggcaatcacactcagcaggctgtgtggaaagagttcctggtgtgtggtaactccagcaaaaacttcatcctcaaagatagcgacattcatgaagatctgttccatagttccaattagctcttctttgcccaatgctaagttctgcacaggccgtaccagtctacaaggagtggtaaaaaggaacaatcctgggtacagacttggttttcctgtcatgggtataaggaccacttccatccagggaggaattcttttctctctcaacaccttaaaatgacgaagagaatctgcgatgcctggagcaagatccttatccacccagccaaccatgacaccgtccagcaggacagggtagcactcactgtatgatcggtggggagctccatcaatgggagtgacccccaagttgcacagtaaagctggaatagatgccgtatacacaaactgtgtgacaacctcacatacggcagttaggtggttcatcaggccacagggctccccgtctggggtatgcacgggacaaaggaagccccaggactctggcagcagcctgcgtactgtggtggtcctcatcttggcaaaatcagcccctctgtgcacgcagcggaaatgggagaggtagcgtatgaagttcagcttgtcagccacaacacaaagtccagaatcttgtaggaggccaagacctgttttagaacgcagattcccagtagcaaaaaggtattcaaatggttttgtaaggtctatgcccattgtaaaaatcctcatcaaattgtcagtgttcatggaaacactggtcttctgagccttcttatcaaaagctattttaatagacactaaccaaccttccagtttttccttcaggaacataaggaagagctgacccggtgtgaggacttcctggttcaccaaactatcaggattgtcctccatgcactctcctttggctaaagcaaagagctttcgcgtcatgagacaaagcatataaaacttttcagtattggatttcaagtggatacagatgcactggttaaacaggaactccgcagcttgctcatttgggtaccagtcaggaacattgagttttactctgaagcattcacctaggtagttaaggacctgtttttgtgtcgaacaaccctcttccattacaatccttaacatctgagaaacagagttcctaaggaaagaatcatcctcttttcctttgatgagctcctgaaagatctgataatcagaaaagctgacaagtgccttaagtgcaaatcccaaaggaagaaagaacagttcttttcggtaaataaagttcaacataacagtgccattttccaagtagtggaggttcatattgacagcggaatgttcttccctcacacagtgcattgaaactccatactgagtataaccaggccctctggttttccattttggtcttatcattgcaatgggaaaatttctccgaggcataatcaacattcggatgactttttcaatgccattgattataaaatagccccccatttcctctgcctcctcatggtgctcaatgagggcttgtgggggaaggttacgtaagttgcaaagcttggatttcaccatgatgggaacatagccaagaaactgcttaatgattccttttgagattccattcactgcccagttgatatcagctgtcaacttcccacggtaggtactccttcggccccggcattctgctggataaacattggcctctttgcagatggtcccttttggaactgtaggtggactgcaccgcgaggccgagaccctcgtgcacagcgtagttgaaggactccacgtgcgcccgcgtcagctcctgcaacgctgccttttgctgttcccgcgggattccataagaggggtcagtcaagtgctttaggctaggcccgctgggcaggttccgccaccggctgccaggatccatgtggccacctgcacaccggacgccagtctc

SEQ ID NO: 17214 - RNA, 4439 nt, Homo sapiens
  source 1..4439: mol_type = other RNA
tcaggccaggcacagtggctcacacctgtaatcctagcactttcggaggccgaggtgggtggatcacttgaggtcagggtcttcaagacagggtcttcctatattacccaggctgtccttgaactcctgcactcaaatgatcctcccacctcagcctctcaaatagcagggactatagatgcacagcaccatgcctggcttccaaaatggatgaatcttatttcactatgctaagtgaaataagccagtcacaggacaaatattgcatgatcccactatatgagatatctgtaatagtcaaactcatagaaacagggtagaagggtggttgctaggggccagggaaatggagagttgttcaacaggtataaagcttcagttatgcaagacaagtaaggtctaaagatctgttgtacaacatggtgcctggaattaacaatactatatcgtgcacttaaagatttgttaagagggtaggtcttgagttaagtgttcttaccacagaagacaaaacaaaaactcaacagcaaccaaaaagcaaaaaacaaaggggcaggaggaaacttgtggagatgacaggtatgtttattaccctgattgtggtgatggtatcaaaggtgtgtgcatatagtcagacccatcaaattgtattcattaaatatgtaacaactgtacttctataaagctggtaaaaaacactgtacctgtttgtttttacttcaacgtggctataagaaaatataaaattacattacagcttgcattctatttgtatagtactgtcctgctcaagatggattaacaggtgtgtgacactcactgcctgctgagagcagggtgtagggaacctggggttggaaaggagacttgtcaccgtatgctcttccatttatcaatatttcatattttgagaagacatgaactttttgaacaaagataacagaaaatcattgtcaatagttaatctaccagagagattcagaaaccttgcatacttggttttcaggtcttggttgagagttctaacaccgttgaaaaatctcaagagtaacctggtaatgatatcttcattgaattaaaattacattttgctttaatctgatagtcctcttaatccaaaaggtcaacatcaagttaaacaacatccagtttcactttgatgttcatagctgccagttcagctacaaaataccgaaaaacataaggcacagaaacagtatcgatagtgtcactgcgactacacagagtacagttgtattttctgttgcgcatggcagaccaagaagggggtggcttctccaacagtggagagagtaaactgccacacttcacacacacatgggctaccgaccgatctgagcagttgaagaggcggtcatgaaggagaaaagatgtaccatgagctaaaagcgcatcccgttccatctccccaaaacggattccaccctggacatttcttcccccaataggctggttggtgactctgtctcgggctccagttgtccttacttgaaatttgtctgagaccatatggcgtaagcgctgataataaaccactcctatgaagatgtctgcttccagttctagcccactgatgccactatataacctctcggtgccatagaaattgtagccagcagcctttaacatctcaccaaagtattctaaggccgagttctcctctgagaagatgaagggtgtagcatcatggcagagaccatgcaaagctgcagacttcccggccatactctcaattaacatcccaatggtcatgcgggatggaaaaccatggggattgaacagaatgtctgggaccatcccactctcagtaaaaggcatgtcctcagccggccacaatctgcttaaaatgcccttctgcccatggcgactggcaaatttatctccgatagttgggttccgaggcactctcatagtgatgcaaacacacttgaattttccactcccagtgtcattactgcacactttgatgttatccacaacacaattttctttactcttatagtacatcacaaaactttccccggtgttgaggttgaggtagctgtaatacggatctccgtactgcagttttgctcctataaacggcaatccatcgtcatctaacttctgcagaacgcgtgggtcaccaggtttgatgccaaacaccaggctactatctccttgtttaattttttcagagaggtctatgaactcagacttgtagacacttccatgggcaaagcctcgttcccaagaggccttattcacaatcatggcatcttccatatcatagccagtgtaagaaatcacagcaacgatggcattggtcccaattggatagttatccatgtcataataatcatacatggagggtctcaccaagggactctgaggagtctgaagacgatacagtttgttatccgatcggtcttgataagtgagaagtggaaagcccatagtttgcttacccatctggcattggtacatgttccgtggactctggttgtgatcagagaaagggatgaagttggcaatcacactcagcaggctgtgtggaaagagttcctggtgtgtggtaactccagcaaaaacttcatcctcaaagatagcgacattcatgaagatctgttccatagttccaattagctcttctttgcccaatgctaagttctgcacaggccgtaccagtctacaaggagtggtaaaaaggaacaatcctgggtacagacttggttttcctgtcatgggtataaggaccacttccatccagggaggaattcttttctctctcaacaccttaaaatgacgaagagaatctgcgatgcctggagcaagatccttatccacccagccaaccatgacaccgtccagcaggacagggtagcactcactgtatgatcggtggggagctccatcaatgggagtgacccccaagttgcacagtaaagctggaatagatgccgtatacacaaactgtgtgacaacctcacatacggcagttaggtggttcatcaggccacagggctccccgtctggggtatgcacgggacaaaggaagccccaggactctggcagcagcctgcgtactgtggtggtcctcatcttggcaaaatcagcccctctgtgcacgcagcggaaatgggagaggtagcgtatgaagttcagcttgtcagccacaacacaaagtccagaatcttgtaggaggccaagacctgttttagaacgcagattcccagtagcaaaaaggtattcaaatggttttgtaaggtctatgcccattgtaaaaatcctcatcaaattgtcagtgttcatggaaacactggtcttctgagccttcttatcaaaagctattttaatagacactaaccaaccttccagtttttccttcaggaacataaggaagagctgacccggtgtgaggacttcctggttcaccaaactatcaggattgtcctccatgcactctcctttggctaaagcaaagagctttcgcgtcatgagacaaagcatataaaacttttcagtattggatttcaagtggatacagatgcactggttaaacaggaactccgcagcttgctcatttgggtaccagtcaggaacattgagttttactctgaagcattcacctaggtagttaaggacctgtttttgtgtcgaacaaccctcttccattacaatccttaacatctgagaaacagagttcctaaggaaagaatcatcctcttttcctttgatgagctcctgaaagatctgataatcagaaaagctgacaagtgccttaagtgcaaatcccaaaggaagaaagaacagttcttttcggtaaataaagttcaacataacagtgccattttccaagtagtggaggttcatattgacagcggaatgttcttccctcacacagtgcattgaaactcctctgcctcctcatggtgctcaatgagggcttgtgggggaaggttacgtaagttgcaaagcttggatttcaccatgatgggaacatagccaagaaactgcttaatgattccttttgagattccattcactgcccagttgatatcagctgtcaacttcccacggtaggtactccttcggccccggcattctgctggataaacattggcctctttgcagatggtcccttttggaactgtaggtggactgataacagcatccagaatagtaaaagagatacgctcatctttgaaagcaaattcaaagggaggtatagcctgcaccgcgaggccgagaccctcgtgcacagcgtagttgaaggactccacgtgcgcccgcgtcagctcctgcaacgctgccttttgctgttcccgcgggattccataagaggggtcagtcaagtgctttaggctaggcccgctgggcaggttccgccaccggctgccaggatccatgtggccacctgcacaccggacgccagtctc

SEQ ID NO: 17215 - RNA, 4124 nt, Homo sapiens
  source 1..4124: mol_type = other RNA
tcaggccaggcacagtggctcacacctgtaatcctagcactttcggaggccgaggtgggtggatcacttgaggtcagggtcttcaagacagggtcttcctatattacccaggctgtccttgaactcctgcactcaaatgatcctcccacctcagcctctcaaatagcagggactatagatgcacagcaccatgcctggcttccaaaatggatgaatcttatttcactatgctaagtgaaataagccagtcacaggacaaatattgcatgatcccactatatgagatatctgtaatagtcaaactcatagaaacagggtagaagggtggttgctaggggccagggaaatggagagttgttcaacaggtataaagcttcagttatgcaagacaagtaaggtctaaagatctgttgtacaacatggtgcctggaattaacaatactatatcgtgcacttaaagatttgttaagagggtaggtcttgagttaagtgttcttaccacagaagacaaaacaaaaactcaacagcaaccaaaaagcaaaaaacaaaggggcaggaggaaacttgtggagatgacaggtatgtttattaccctgattgtggtgatggtatcaaaggtgtgtgcatatagtcagacccatcaaattgtattcattaaatatgtaacaactgtacttctataaagctggtaaaaaacactgtacctgtttgtttttacttcaacgtggctataagaaaatataaaattacattacagcttgcattctatttgtatagtactgtcctgctcaagatggattaacaggtgtgtgacactcactgcctgctgagagcagggtgtagggaacctggggttggaaaggagacttgtcaccgtatgctcttccatttatcaatatttcatattttgagaagacatgaactttttgaacaaagataacagaaaatcattgtcaatagttaatctaccagagagattcagaaaccttgcatacttggttttcaggtcttggttgagagttctaacaccgttgaaaaatctcaagagtaacctggtaatgatatcttcattgaattaaaattacattttgctttaatctgatagtcctcttaatccaaaaggtcaacatcaagttaaacaacatccagtttcactttgatgttcatagctgccagttcagctacaaaataccgaaaaacataaggcacagaaacagtatcgatagtgtcactgcgactacacagagtacagttgtattttctgttgcgcatggcagaccaagaagggggtggcttctccaacagtggagagagtaaactgccacacttcacacacacatgggctaccgaccgatctgagcagttgaagaggcggtcatgaaggagaaaagatgtaccatgagctaaaagcgcatcccgttccatctccccaaaacggattccaccctggacatttcttcccccaataggctggttggtgactctgtctcgggctccagttgtccttacttgaaatttgtctgagaccatatggcgtaagcgctgataataaaccactcctatgaagatgtctgcttccagttctagcccactgatgccactatataacctctcggtgccatagaaattgtagccagcagcctttaacatctcaccaaagtattctaaggccgagttctcctctgagaagatgaagggtgtagcatcatggcagagaccatgcaaagctgcagacttcccggccatactctcaattaacatcccaatggtcatgcgggatggaaaaccatggggattgaacagaatgtctgggaccatcccactctcagtaaaaggcatgtcctcagccggccacaatctgcttaaaatgcccttctgcccatggcgactggcaaatttatctccgatagttgggttccgaggcactctcatagtgatgcaaacacacttgaattttccactcccagtgtcattactgcacactttgatgttatccacaacacaattttctttactcttatagtacatcacaaaactttccccggtgttgaggttgaggtagctgtaatacggatctccgtactgcagttttgctcctataaacggcaatccatcgtcatctaacttctgcagaacgcgtgggtcaccaggtttgatgccaaacaccaggctactatctccttgtttaattttttcagagaggtctatgaactcagacttgtagacacttccatgggcaaagcctcgttcccaagaggccttattcacaatcatggcatcttccatatcatagccagtgtaagaaatcacagcaacgatggcattggtcccaattggatagttatccatgtcataataatcatacatggagggtctcaccaagggactctgaggagtctgaagacgatacagtttgttatccgatcggtcttgataagtgagaagtggaaagcccatagtttgcttacccatctggcattggtacatgttccgtggactctggttgtgatcagagaaagggatgaagttggcaatcacactcagcaggctgtgtggaaagagttcctggtgtgtggtaactccagcaaaaacttcatcctcaaagatagcgacattcatgaagatctgttccatagttccaattagctcttctttgcccaatgctaagttctgcacaggccgtaccagtctacaaggagtggtaaaaaggaacaatcctgggtacagacttggttttcctgtcatgggtataaggaccacttccatccagggaggaattcttttctctctcaacaccttaaaatgacgaagagaatctgcgatgcctggagcaagatccttatccacccagccaaccatgacaccgtccagcaggacagggtagcactcactgtatgatcggtggggagctccatcaatgggagtgacccccaagttgcacagtaaagctggaatagatgccgtatacacaaactgtgtgacaacctcacatacggcagttaggtggttcatcaggccacagggctccccgtctggggtatgcacgggacaaaggaagccccaggactctggcagcagcctgcgtactgtggtggtcctcatcttggcaaaatcagcccctctgtgcacgcagcggaaatgggagaggtagcgtatgaagttcagcttgtcagccacaacacaaagtccagaatcttgtaggaggccaagacctgttttagaacgcagattcccagtagcaaaaaggtattcaaatggttttgtaaggtctatgcccattgtaaaaatcctcatcaaattgtcagtgttcatggaaacactggtcttctgagccttcttatcaaaagctattttaatagacactaaccaaccttccagtttttccttcaggaacataaggaagagctgacccggtgtgaggacttcctggttcaccaaactatcaggattgtcctccatgcactctcctttggctaaagcaaagagctttcgcgtcatgagacaaagcatataaaacttttcagtattggatttcaagtggatacagatgcactggttaaacaggaactccgcagcttgctcatttgggtaccagtcaggaacattgagttttactctgaagcattcacctaggtagttaaggacctgtttttgtgtcgaacaaccctcttccattacaatccttaacatctgagaaacagagttcctaaggaaagaatcatcctcttttcctttgatgagctcctgaaagatctgataatcagaaaagctgacaagtgccttaagtgcaaatcccaaaggaagaaagaacagttcttttcggtaaataaagttcaacataacagtgccattttccaagtagtggaggttcatattgacagcggaatgttcttccctcacacagtgcattgaaactcctgcaccgcgaggccgagaccctcgtgcacagcgtagttgaaggactccacgtgcgcccgcgtcagctcctgcaacgctgccttttgctgttcccgcgggattccataagaggggtcagtcaagtgctttaggctaggcccgctgggcaggttccgccaccggctgccaggatccatgtggccacctgcacaccggacgccagtctc

SEQ ID NO: 17216 - RNA, 4023 nt, Homo sapiens
  source 1..4023: mol_type = other RNA
tcaggccaggcacagtggctcacacctgtaatcctagcactttcggaggccgaggtgggtggatcacttgaggtcagggtcttcaagacagggtcttcctatattacccaggctgtccttgaactcctgcactcaaatgatcctcccacctcagcctctcaaatagcagggactatagatgcacagcaccatgcctggcttccaaaatggatgaatcttatttcactatgctaagtgaaataagccagtcacaggacaaatattgcatgatcccactatatgagatatctgtaatagtcaaactcatagaaacagggtagaagggtggttgctaggggccagggaaatggagagttgttcaacaggtataaagcttcagttatgcaagacaagtaaggtctaaagatctgttgtacaacatggtgcctggaattaacaatactatatcgtgcacttaaagatttgttaagagggtaggtcttgagttaagtgttcttaccacagaagacaaaacaaaaactcaacagcaaccaaaaagcaaaaaacaaaggggcaggaggaaacttgtggagatgacaggtatgtttattaccctgattgtggtgatggtatcaaaggtgtgtgcatatagtcagacccatcaaattgtattcattaaatatgtaacaactgtacttctataaagctggtaaaaaacactgtacctgtttgtttttacttcaacgtggctataagaaaatataaaattacattacagcttgcattctatttgtatagtactgtcctgctcaagatggattaacaggtgtgtgacactcactgcctgctgagagcagggtgtagggaacctggggttggaaaggagacttgtcaccgtatgctcttccatttatcaatatttcatattttgagaagacatgaactttttgaacaaagataacagaaaatcattgtcaatagttaatctaccagagagattcagaaaccttgcatacttggttttcaggtcttggttgagagttctaacaccgttgaaaaatctcaagagtaacctggtaatgatatcttcattgaattaaaattacattttgctttaatctgatagtcctcttaatccaaaaggtcaacatcaagttaaacaacatccagtttcactttgatgttcatagctgccagttcagctacaaaataccgaaaaacataaggcacagaaacagtatcgatagtgtcactgcgactacacagagtacagttgtattttctgttgcgcatggcagaccaagaagggggtggcttctccaacagtggagagagtaaactgccacacttcacacacacatgggctaccgaccgatctgagcagttgaagaggcggtcatgaaggagaaaagatgtaccatgagctaaaagcgcatcccgttccatctccccaaaacggattccaccctggacatttcttcccccaataggctggttggtgactctgtctcgggctccagttgtccttacttgaaatttgtctgagaccatatggcgtaagcgctgataataaaccactcctatgaagatgtctgcttccagttctagcccactgatgccactatataacctctcggtgccatagaaattgtagccagcagcctttaacatctcaccaaagtattctaaggccgagttctcctctgagaagatgaagggtgtagcatcatggcagagaccatgcaaagctgcagacttcccggccatactctcaattaacatcccaatggtcatgcgggatggaaaaccatggggattgaacagaatgtctgggaccatcccactctcagtaaaaggcatgtcctcagccggccacaatctgcttaaaatgcccttctgcccatggcgactggcaaatttatctccgatagttgggttccgaggcactctcatagtgatgcaaacacacttgaattttccactcccagtgtcattactgcacactttgatgttatccacaacacaattttctttactcttatagtacatcacaaaactttccccggtgttgaggttgaggtagctgtaatacggatctccgtactgcagttttgctcctataaacggcaatccatcgtcatctaacttctgcagaacgcgtgggtcaccaggtttgatgccaaacaccaggctactatctccttgtttaattttttcagagaggtctatgaactcagacttgtagacacttccatgggcaaagcctcgttcccaagaggccttattcacaatcatggcatcttccatatcatagccagtgtaagaaatcacagcaacgatggcattggtcccaattggatagttatccatgtcataataatcatacatggagggtctcaccaagggactctgaggagtctgaagacgatacagtttgttatccgatcggtcttgataagtgagaagtggaaagcccatagtttgcttacccatctggcattggtacatgttccgtggactctggttgtgatcagagaaagggatgaagttggcaatcacactcagcaggctgtgtggaaagagttcctggtgtgtggtaactccagcaaaaacttcatcctcaaagatagcgacattcatgaagatctgttccatagttccaattagctcttctttgcccaatgctaagttctgcacaggccgtaccagtctacaaggagtggtaaaaaggaacaatcctgggtacagacttggttttcctgtcatgggtataaggaccacttccatccagggaggaattcttttctctctcaacactgtatgatcggtggggagctccatcaatgggagtgaccccttcaggaacataaggaagagctgacccggtgtgaggacttcctggttcaccaaactatcaggattgtcctccatgcactctcctttggctaaagcaaagagctttcgcgtcatgagacaaagcatataaaacttttcagtattggatttcaagtggatacagatgcactggttaaacaggaactccgcagcttgctcatttgggtaccagtcaggaacattgagttttactctgaagcattcacctaggtagttaaggacctgtttttgtgtcgaacaaccctcttccattacaatccttaacatctgagaaacagagttcctaaggaaagaatcatcctcttttcctttgatgagctcctgaaagatctgataatcagaaaagctgacaagtgccttaagtgcaaatcccaaaggaagaaagaacagttcttttcggtaaataaagttcaacataacagtgccattttccaagtagtggaggttcatattgacagcggaatgttcttccctcacacagtgcattgaaactccatactgagtataaccaggccctctggttttccattttggtcttatcattgcaatgggaaaatttctccgaggcataatcaacattcggatgactttttcaatgccattgattataaaatagccccccatttcctctgcctcctcatggtgctcaatgagggcttgtgggggaaggttacgtaagttgcaaagcttggatttcaccatgatgggaacatagccaagaaactgcttaatgattccttttgagattccattcactgcccagttgatatcagctgtcaacttcccacggtaggtactccttcggccccggcattctgctggataaacattggcctctttgcagatggtcccttttggaactgtaggtggactgataacagcatccagaatagtaaaagagatacgctcatctttgaaagcaaattcaaagggaggtatagcctgcaccgcgaggccgagaccctcgtgcacagcgtagttgaaggactccacgtgcgcccgcgtcagctcctgcaacgctgccttttgctgttcccgcgggattccataagaggggtcagtcaagtgctttaggctaggcccgctgggcaggttccgccaccggctgccaggatccatgtggccacctgcacaccggacgccagtctc

SEQ ID NO: 17217 - RNA, 1689 nt, Homo sapiens
  source 1..1689: mol_type = other RNA
tcaggccaggcacagtggctcacacctgtaatcctcacaatttgggaagcccaagtaggaggatccattgaggcaaggagtttgagactggcctgggcaacatagtgagactccctctctttaaatgctacaaaaaattggccaggcatggtggtgcgcatgtgtagtcccagctactcaggaggctgagatgggaggatcacctgagcccagaagtttgaggctgcaggaaaaggagcccagtcccagctctttgtggttcacaggcgccaggatatttcatcccaggttcaacaccagccccagggtcctcagggctagtatcacttcccaagagtcatgatcaggaacttagtgaagatcctttcaaccccagaagtgggagacctcccaccaccaagctctgagcatcctcccagctcaccatctactagggcaagcccaagtcctcactctagaaacagcctgacttgcacccctgggaacttgctgcatccagggtgccaatcctgtttgaggcacatctgtgtgtccactcacgaagaggcaaggccgtccacgaaagggcaggagattctcatctcaaagagacactcagatatggacccccagcctcggccctgggcttcaacaggaacatttccgctcacaaatccaatacgtagttttgtagcaagagagatcattccaggtgccacctttgttcatggtagcacagtcctcatcgtggatgttattgggttcctctggctcccagaagcttaatgtcacaggagacccatccagccacctccagtccccttcctgggccctgtcattcagccccagccagtacacccgtggagagccatgggccttggccacaaaattctaataagccccaaagttccaccagggactggttggtgtcagctcttacacgggcaatgtcatgcttcaggccagctagccctgccatgccagtcatatttgttcgccacgtcatctgctgaaagcttaacattctcagttcttccatcaactcctggtacttaatcagggtcacagtgagaccaaggcagcccaggaacagggaagtcaccaccagcagacacaggtacaccatccacctcttctggcagcagccaggacctccagacctctgattgagccaggggactggagttgcggccagggatggctgcaatggagaaggctcaagattcacagccagttgaggaggtggacaggtgacagcggcgaggtccaggcctgtcatgttccggggcttgcaaggaagtgggggtttctctgtttcctttgctgcccttggaggtcttggtggagcacttgaacctggcttgggaggaaggtccttgtagggaggtgttgagttctcatagtcatcatcctcctcctcctcctccatggtccctggcttgggaggaaggtccttgtagggaggtgttgagttctcatagtcatcatcctcctcctcctcctccatggtccctggcttgggaggaaggtccttgtagggaggtgttgagttctcatagtcatcatcctcctcctcctcctccatggtccctggtgggtccgggtacccagtgatggaatacagattatgcatgtctagcacagggaacctgacaagtggcagccagggcttggcaacctctgccccctgtctctccgactcaggcgtct

SEQ ID NO: 17218 - RNA, 2186 nt, Homo sapiens
  source 1..2186: mol_type = other RNA
tcaggccaggcacagtggctcacacctgtaatcctcacaatttgggaagcccaagtaggaggatccattgaggcaaggagtttgagactggcctgggcaacatagtgagactccctctctttaaatgctacaaaaaattggccaggcatggtggtgcgcatgtgtagtcccagctactcaggaggctgagatgggaggatcacctgagcccagaagtttgaggctgcaggaaaaggagcccagtcccagctctttgtggttcacaggcgccaggatatttcatcccaggttcaacaccagccccagggtcctcagggctagtatcacttcccaagagtcatgatcaggaacttagtgaagatcctttcaaccccagaagtgggagacctcccaccaccaagctctgagcatcctcccagctcaccatctactagggcaagcccaagtcctcactctagaaacagcctgacttgcacccctgggaacttgctgcatccagggtgccaatcctgtttgaggcacatctgtgtgtccactcacgaagaggcaaggccgtccacgaaagggcaggagattctcatctcaaagagacactcagatatggacccccagcctcggccctgggcttcaacaggaacatttccgctcacaaatccaatacgtagttttgtagcaagagagatcattccaggtgccacctttgttcatggtagcacagtcctcatcgtggatgttattgggttcctctggctcccagaagcttaatgtcacaggagacccatccagccacctccagtccccttcctgggccctgtcattcagccccagccagtacacccgtggagagccatgggccttggccacaaaattgtgctcagcaaagctattgatgatgaccaagtgagagtaattctcctggcagaacatccgggcctcatcccatgacttggtgcttggggagaagtagtaacacttgccctcaaagggcagccagccttcaggacaggtaattcggcggcagtctaataagccccaaagttccaccagggactggttggtgtcagctcttacacgggcaatgtcatgcttcaggccagctagccctgccatgccagtcacggccagggatggctgcaatggagaaggctcaagattcacagccagttgaggaggtggacaggtgacagcggcgaggtccaggcctgtcatgttccggggcttgcaaggaagtgggggtttctctgtttcctttgctgcccttggaggtcttggtggagcacttgaacctggcttgggaggaaggtccttgtagggaggtgttgagttctcatagtcatcatcctcctcctcctcctccatggtccagtttctgtggttcaggaatctgagagcagcttagctgggtagttctagcttgagatctcttgcgtgattgtagtcaagatgttgcctgggactgcaagtcatctgcaggcttgactggggctagaggatctgcttccaagatgatgcactcacatggctgttggtgggaggcctcagttccttgccatgtgagcctctccaaagggatgactgggcatcttcacaacatggcagaggcaaagatagaagccaccatgctcctatgatctagcctcacaagtcacaaaggatggtctccactatacagtattctatttatcacatggaccagctctgagtcgttgtgggaagagactggcttgggaggaaggtccttgtagggaggtgttgagttctcatagtcatcatcctcctcctcctcctccatggtccctggcttgggaggaaggtccttgtagggaggtgttgagttctcatagtcatcatcctcctcctcctcctccatggtccctggtgggtccgggtacccagtgatggaatacagattatgcatgtctagcacagggaacctgacaagtggcagccagggcttggcaacctctgccccctgtctctccgactcaggcgtctgggggctctctcagttcccttttcctttcaaagtcaaatacatgcaaattcattttgacaggaagccctcagacctcacacgtgctcacacaaacacacacacacacacacacacacatacacacagagcctttctccccagtttggattcacgcacagaaggaataatgacaactggcctggtgtggtgg

SEQ ID NO: 17219 - RNA, 1904 nt, Homo sapiens
  source 1..1904: mol_type = other RNA
tcaggccaggcacagtggctcacacctgtaatcctcacaatttgggaagcccaagtaggaggatccattgaggcaaggagtttgagactggcctgggcaacatagtgagactccctctctttaaatgctacaaaaaattggccaggcatggtggtgcgcatgtgtagtcccagctactcaggaggctgagatgggaggatcacctgagcccagaagtttgaggctgcaggaaaaggagcccagtcccagctctttgtggttcacaggcgccaggatatttcatcccaggttcaacaccagccccagggtcctcagggctagtatcacttcccaagagtcatgatcaggaacttagtgaagatcctttcaaccccagaagtgggagacctcccaccaccaagctctgagcatcctcccagctcaccatctactagggcaagcccaagtcctcactctagaaacagcctgacttgcacccctgggaacttgctgcatccagggtgccaatcctgtttgaggcacatctgtgtgtccactcacgaagaggcaaggccgtccacgaaagggcaggagattctcatctcaaagagacactcagatatggacccccagcctcggccctgggcttcaacaggaacatttccgctcacaaatccaatacgtagttttgtagcaagagagatcattccaggtgccacctttgttcatggtagcacagtcctcatcgtggatgttattgggttcctctggctcccagaagcttaatgtcacaggagacccatccagccacctccagtccccttcctgggccctgtcattcagccccagccagtacacccgtggagagccatgggccttggccacaaaattgtgctcagcaaagctattgatgatgaccaagtgagagtaattctcctggcagaacatccgggcctcatcccatgacttggtgcttggggagaagtagtaacacttgccctcaaagggcagccagccttcaggacaggtaattcggcggcagtctaataagccccaaagttccaccagggactggttggtgtcagctcttacacgggcaatgtcatgcttcaggccagctagccctgccatgccagtcactgtcagaagggatgggcttgagggctacagactgagaacccatcctacccatccaccacggatatttgttcgccacgtcatctgctgaaagcttaacattctcagttcttccatcaactcctggtacttaatcagggtcacagtgagaccaaggcagcccaggaacagggaagtcaccaccagcagacacaggtacaccatccacctcttctggcagcagccaggacctccagacctctgattgagccaggggactggagttgcggccagggatggctgcaatggagaaggctcaagattcacagccagttgaggaggtggacaggtgacagcggcgaggtccaggcctgtcatgttccggggcttgcaaggaagtgggggtttctctgtttcctttgctgcccttggaggtcttggtggagcacttgaacctggcttgggaggaaggtccttgtagggaggtgttgagttctcatagtcatcatcctcctcctcctcctccatggtccctggcttgggaggaaggtccttgtagggaggtgttgagttctcatagtcatcatcctcctcctcctcctccatggtccctggcttgggaggaaggtccttgtagggaggtgttgagttctcatagtcatcatcctcctcctcctcctccatggtccctggtgggtccgggtacccagtgatggaatacagattatgcatgtctagcacagggaacctgacaagtggcagccagggcttggcaacctctgccccctgtctctccgactcaggcgtct

SEQ ID NO: 17220 - RNA, 2337 nt, Homo sapiens
  source 1..2337: mol_type = other RNA
tcaggccaggcacagtggctcacacctgtaatcctcacaatttgggaagcccaagtaggaggatccattgaggcaaggagtttgagactggcctgggcaacatagtgagactccctctctttaaatgctacaaaaaattggccaggcatggtggtgcgcatgtgtagtcccagctactcaggaggctgagatgggaggatcacctgagcccagaagtttgaggctgcaggaaaaggagcccagtcccagctctttgtggttcacaggcgccaggatatttcatcccaggttcaacaccagccccagggtcctcagggctagtatcacttcccaagagtcatgatcaggaacttagtgaagatcctttcaaccccagaagtgggagacctcccaccaccaagctctgagcatcctcccagctcaccatctactagggcaagcccaagtcctcactctagaaacagcctgacttgcacccctgggaacttgctgcatccagggtgccaatcctgtttgaggcacatctgtgtgtccactcacgaagaggcaaggccgtccacgaaagggcaggagattctcatctcaaagagacactcagatatggacccccagcctcggccctgggcttcaacaggaacatttccgctcacaaatccaatacgtagttttgtagcaagagagatcattccaggtgccacctttgttcatggtagcacagtcctcatcgtggatgttattgggttcctctggctcccagaagcttaatgtcacaggagacccatccagccacctccagtccccttcctgggccctgtcattcagccccagccagtacacccgtggagagccatgggccttggccacaaaattgtgctcagcaaagctattgatgatgaccaagtgagagtaattctcctggcagaacatccgggcctcatcccatgacttggtgcttggggagaagtagtaacacttgccctcaaagggcagccagccttcaggacaggtaattcggcggcagtctaataagccccaaagttccaccagggactggttggtgtcagctcttacacgggcaatgtcatgcttcaggccagctagccctgccatgccagtcatatttgttcgccacgtcatctgctgaaagcttaacattctcagttcttccatcaactcctggtacttaatcagggtcacagtgagaccaaggcagcccaggaacagggaagtcaccaccagcagacacaggtacaccatccacctcttctggcagcagccaggacctccagacctctgattgagccaggggactggagttgcggccagggatggctgcaatggagaaggctcaagattcacagccagttgaggaggtggacaggtgacagcggcgaggtccaggcctgcccttggaggtcttggtggagcacttgaacctggcttgggaggaaggtccttgtagggaggtgttgagttctcatagtcatcatcctcctcctcctcctccatggtccagtttctgtggttcaggaatctgagagcagcttagctgggtagttctagcttgagatctcttgcgtgattgtagtcaagatgttgcctgggactgcaagtcatctgcaggcttgactggggctagaggatctgcttccaagatgatgcactcacatggctgttggtgggaggcctcagttccttgccatgtgagcctctccaaagggatgactgggcatcttcacaacatggcagaggcaaagatagaagccaccatgctcctatgatctagcctcacaagtcacaaaggatggtctccactatacagtattctatttatcacatggaccagctctgagtcgttgtgggaagagactggcttgggaggaaggtccttgtagggaggtgttgagttctcatagtcatcatcctcctcctcctcctccatggtccctggcttgggaggaaggtccttgtagggaggtgttgagttctcatagtcatcatcctcctcctcctcctccatggtccctggtgggtccgggtacccagtgatggaatacagattatgcatgtctagcacagggaacctgacaagtggcagccagggcttggcaacctctgccccctgtctctccgactcaggcgtctgggggctctctcagttcccttttcctttcaaagtcaaatacatgcaaattcattttgacaggaagccctcagacctcacacgtgctcacacaaacacacacacacacacacacacacatacacacagagcctttctccccagtttggattcacgcacagaaggaataatgacaactggcctggtgtggtggc

SEQ ID NO: 17221 - RNA, 2249 nt, Homo sapiens
  source 1..2249: mol_type = other RNA
tcaggccaggcacagtggctcacacctgtaatcctcacaatttgggaagcccaagtaggaggatccattgaggcaaggagtttgagactggcctgggcaacatagtgagactccctctctttaaatgctacaaaaaattggccaggcatggtggtgcgcatgtgtagtcccagctactcaggaggctgagatgggaggatcacctgagcccagaagtttgaggctgcaggaaaaggagcccagtcccagctctttgtggttcacaggcgccaggatatttcatcccaggttcaacaccagccccagggtcctcagggctagtatcacttcccaagagtcatgatcaggaacttagtgaagatcctttcaaccccagaagtgggagacctcccaccaccaagctctgagcatcctcccagctcaccatctactagggcaagcccaagtcctcactctagaaacagcctgacttgcacccctgggaacttgctgcatccagggtgccaatcctgtttgaggcacatctgtgtgtccactcacgaagaggcaaggccgtccacgaaagggcaggagattctcatctcaaagagacactcagatatggacccccagcctcggccctgggcttcaacaggaacatttccgctcacaaatccaatacgtagttttgtagcaagagagatcattccaggtgccacctttgttcatggtagcacagtcctcatcgtggatgttattgggttcctctggctcccagaagcttaatgtcacaggagacccatccagccacctccagtccccttcctgggccctgtcattcagccccagccagtacacccgtggagagccatgggccttggccacaaaattgtgctcagcaaagctattgatgatgaccaagtgagagtaattctcctggcagaacatccgggcctcatcccatgacttggtgcttggggagaagtagtaacacttgccctcaaagggcagccagccttcaggacaggtaattcggcggcagtctaataagccccaaagttccaccagggactggttggtgtcagctcttacacgggcaatgtcatgcttcaggccagctagccctgccatgccagtcatatttgttcgccacgtcatctgctgaaagcttaacattctcagttcttccatcaactcctggtacttaatcagggtcacagtgagaccaaggcagcccaggaacagggaagtcaccaccagcagacacaggtacaccatccacctcttctggcagcagccaggacctccagacctctgattgagccaggggactggagttgcggccagggatggctgcaatggagaaggctcaagattcacagccagttgaggaggtggacaggtgacagcggcgaggtccaggcctgtcatgttccggggcttgcaaggaagtgggggtttctctgtttcctttgctgcccttggaggtcttggtggagcacttgaacctggcttgggaggaaggtccttgtagggaggtgttgagttctcatagtcatcatcctcctcctcctcctccatggtccagtttctgtggttcaggaatctgagagcagcttagctgggtagttctagcttgagatctcttgcgtgattgtagtcaagatgttgcctgggactgcaagtcatctgcaggcttgactggggctagaggatctgcttccaagatgatgcactcacatggctgttggtgggaggcctcagttccttgccatgtgagcctctccaaagggatgactgggcatctggcttgggaggaaggtccttgtagggaggtgttgagttctcatagtcatcatcctcctcctcctcctccatggtccctggcttgggaggaaggtccttgtagggaggtgttgagttctcatagtcatcatcctcctcctcctcctccatggtccctggtgggtccgggtacccagtgatggaatacagattatgcatgtctagcacagggaacctgacaagtggcagccagggcttggcaacctctgccccctgtctctccgactcaggcgtctgggggctctctcagttcccttttcctttcaaagtcaaatacatgcaaattcattttgacaggaagccctcagacctcacacgtgctcacacaaacacacacacacacacacacacacatacacacagagcctttctccccagtttggattcacgcacagaaggaataatgacaactggcctggtgtggt

SEQ ID NO: 17222 - RNA, 2604 nt, Homo sapiens
  source 1..2604: mol_type = other RNA
tcaggccaggcacagtggctcacacctgtaatcctcacaatttgggaagcccaagtaggaggatccattgaggcaaggagtttgagactggcctgggcaacatagtgagactccctctctttaaatgctacaaaaaattggccaggcatggtggtgcgcatgtgtagtcccagctactcaggaggctgagatgggaggatcacctgagcccagaagtttgaggctgcaggaaaaggagcccagtcccagctctttgtggttcacaggcgccaggatatttcatcccaggttcaacaccagccccagggtcctcagggctagtatcacttcccaagagtcatgatcaggaacttagtgaagatcctttcaaccccagaagtgggagacctcccaccaccaagctctgagcatcctcccagctcaccatctactagggcaagcccaagtcctcactctagaaacagcctgacttgcacccctgggaacttgctgcatccagggtgccaatcctgtttgaggcacatctgtgtgtccactcacgaagaggcaaggccgtccacgaaagggcaggagattctcatctcaaagagacactcagatatggacccccagcctcggccctgggcttcaacaggaacatttccgctcacaaatccaatacgtagttttgtagcaagagagatcattccaggtgccacctttgttcatggtagcacagtcctcatcgtggatgttattgggttcctctggctcccagaagcttaatgtcacaggagacccatccagccacctccagtccccttcctgggccctgtcattcagccccagccagtacacccgtggagagccatgggccttggccacaaaattgtgctcagcaaagctattgatgatgaccaagtgagagtaattctcctggcagaacatccgggcctcatcccatgacttggtgcttggggagaagtagtaacacttgccctcaaagggcagccagccttcaggacaggtaattcggcggcagtctaataagccccaaagttccaccagggactggttggtgtcagctcttacacgggcaatgtcatgcttcaggccagctagccctgccatgccagtcatatttgttcgccacgtcatctgctgaaagcttaacattctcagttcttccatcaactcctggtacttaatcagggtcacagtgagaccaaggcagcccaggaacagggaagtcaccaccagcagacacaggtacaccatccacctcttctggcagcagccaggacctccagacctctgattgagccaggggactggagttgcggccagggatggctgcaatggagaaggctcaagattcacagccagttgaggaggtggacaggtgacagcggcgaggtccaggcctgtcatgttccggggcttgcaaggaagtgggggtttctctgtttcctttgctgcccttggaggtcttggtggagcacttgaacctggcttgggaggaaggtccttgtagggaggtgttgagttctcatagtcatcatcctcctcctcctcctccatggtccagtttctgtggttcaggaatctgagagcagcttagctgggtagttctagcttgagatctcttgcgtgattgtagtcaagatgttgcctgggactgcaagtcatctgcaggcttgactggggctagaggatctgcttccaagatgatgcactcacatggctgttggtgggaggcctcagttccttgccatgtgagcctctccaaagggatgactgggcatcttcacaacatggcagaggcaaagatagaagccaccatgctcctatgatctagcctcacaagtcacaaaggatggtctccactatacagtattctatttatcacatggaccagctctgagtcgttgtgggaagagactggcttgggaggaaggtccttgtagggaggtgttgagttctcatagtcatcatcctcctcctcctcctccatggtccagtttctgtggttcaggaatctgagagcagcttagctgggtagttctagcttgagatctcttgcgtgattgtagtcaagatgttgcctgggactgcaagtcatctgcaggcttgactggggctagaggatctgcttccaagatgatgcactcacatggctgttggtgggaggcctcagttccttgccatgtgagcctctccaaagggatgactgggcatctggcttgggaggaaggtccttgtagggaggtgttgagttctcatagtcatcatcctcctcctcctcctccatggtccctggtgggtccgggtacccagtgatggaatacagattatgcatgtctagcacagggaacctgacaagtggcagccagggcttggcaacctctgccccctgtctctccgactcaggcgtctgggggctctctcagttcccttttcctttcaaagtcaaatacatgcaaattcattttgacaggaagccctcagacctcacacgtgctcacacaaacacacacacacacacacacacacatacacacagagcctttctccccagtttggattcacgcacagaaggaataatgacaactggcctggtgtggt

SEQ ID NO: 17223 - RNA, 2361 nt, Homo sapiens
  source 1..2361: mol_type = other RNA
tcaggccaggcacagtggctcacacctgtaatcctcacaatttgggaagcccaagtaggaggatccattgaggcaaggagtttgagactggcctgggcaacatagtgagactccctctctttaaatgctacaaaaaattggccaggcatggtggtgcgcatgtgtagtcccagctactcaggaggctgagatgggaggatcacctgagcccagaagtttgaggctgcaggaaaaggagcccagtcccagctctttgtggttcacaggcgccaggatatttcatcccaggttcaacaccagccccagggtcctcagggctagtatcacttcccaagagtcatgatcaggaacttagtgaagatcctttcaaccccagaagtgggagacctcccaccaccaagctctgagcatcctcccagctcaccatctactagggcaagcccaagtcctcactctagaaacagcctgacttgcacccctgggaacttgctgcatccagggtgccaatcctgtttgaggcacatctgtgtgtccactcacgaagaggcaaggccgtccacgaaagggcaggagattctcatctcaaagagacactcagatatggacccccagcctcggccctgggcttcaacaggaacatttccgctcacaaatccaatacgtagttttgtagcaagagagatcattccaggtgccacctttgttcatggtagcacagtcctcatcgtggatgttattgggttcctctggctcccagaagcttaatgtcacaggagacccatccagccacctccagtccccttcctgggccctgtcattcagccccagccagtacacccgtggagagccatgggccttggccacaaaattgtgctcagcaaagctattgatgatgaccaagtgagagtaattctcctggcagaacatccgggcctcatcccatgacttggtgcttggggagaagtagtaacacttgccctcaaagggcagccagccttcaggacaggtaattcggcggcagtctaataagccccaaagttccaccagggactggttggtgtcagctcttacacgggcaatgtcatgcttcaggccagctagccctgccatgccagtcatatttgttcgccacgtcatctgctgaaagcttaacattctcagttcttccatcaactcctggtacttaatcagggtcacagtgagaccaaggcagcccaggaacagggaagtcaccaccagcagacacaggtacaccatccacctcttctggcagcagccaggacctccagacctctgattgagccaggggactggagttgcggccagggatggctgcaatggagaaggctcaagattcacagccagttgaggaggtggacaggtgacagcggcgaggtccaggcctgtcatgttccggggcttgcaaggaagtgggggtttctctgtttcctttgctgcccttggaggtcttggtggagcacttgaacctggcttgggaggaaggtccttgtagggaggtgttgagttctcatagtcatcatcctcctcctcctcctccatggtccagtttctgtggttcaggaatctgagagcagcttagctgggtagttctagcttgagatctcttgcgtgattgtagtcaagatgttgcctgggactgcaagtcatctgcaggcttgactggggctagaggatctgcttccaagatgatgcactcacatggctgttggtgggaggcctcagttccttgccatgtgagcctctccaaagggatgactgggcatcttcacaacatggcagaggcaaagatagaagccaccatgctcctatgatctagcctcacaagtcacaaaggatggtctccactatacagtattctatttatcacatggaccagctctgagtcgttgtgggaagagactggcttgggaggaaggtccttgtagggaggtgttgagttctcatagtcatcatcctcctcctcctcctccatggtccctggcttgggaggaaggtccttgtagggaggtgttgagttctcatagtcatcatcctcctcctcctcctccatggtccctgacaggctcagtataagcaagtgagagcctctaacaaatggaaaaaccttcccccgcaccgcacgtgggcaatggggtagccccggtcttaattgaggtaggagggcagcagcagattaacctccctttccattcaaagctgactctaggggctgggctttcccctcttacatggcctgatgtcatagagccttcccagcctgtaggagggcaaacgtgactgtacccattccaacctgtaggagggcaaatgtgactgtacccattctagagatgggaaaat

SEQ ID NO: 17224 - RNA, 2385 nt, Homo sapiens
  source 1..2385: mol_type = other RNA
tcaggccaggcacagtggctcacacctgtaatcctcacaatttgggaagcccaagtaggaggatccattgaggcaaggagtttgagactggcctgggcaacatagtgagactccctctctttaaatgctacaaaaaattggccaggcatggtggtgcgcatgtgtagtcccagctactcaggaggctgagatgggaggatcacctgagcccagaagtttgaggctgcaggaaaaggagcccagtcccagctctttgtggttcacaggcgccaggatatttcatcccaggttcaacaccagccccagggtcctcagggctagtatcacttcccaagagtcatgatcaggaacttagtgaagatcctttcaaccccagaagtgggagacctcccaccaccaagctctgagcatcctcccagctcaccatctactagggcaagcccaagtcctcactctagaaacagcctgacttgcacccctgggaacttgctgcatccagggtgccaatcctgtttgaggcacatctgtgtgtccactcacgaagaggcaaggccgtccacgaaagggcaggagattctcatctcaaagagacactcagatatggacccccagcctcggccctgggcttcaacaggaacatttccgctcacaaatccaatacgtagttttgtagcaagagagatcattccaggtgccacctttgttcatggtagcacagtcctcatcgtggatgttattgggttcctctggctcccagaagcttaatgtcacaggagacccatccagccacctccagtccccttcctgggccctgtcattcagccccagccagtacacccgtggagagccatgggccttggccacaaaattgtgctcagcaaagctattgatgatgaccaagtgagagtaattctcctggcagaacatccgggcctcatcccatgacttggtgcttggggagaagtagtaacacttgccctcaaagggcagccagccttcaggacaggtaattcggcggcagtctaataagccccaaagttccaccagggactggttggtgtcagctcttacacgggcaatgtcatgcttcaggccagctagccctgccatgccagtcatatttgttcgccacgtcatctgctgaaagcttaacattctcagttcttccatcaactcctggtacttaatcagggtcacagtgagaccaaggcagcccaggaacagggaagtcaccaccagcagacacaggtacaccatccacctcttctggcagcagccaggacctccagacctctgattgagccaggggactggagttgcggccagggatggctgcaatggagaaggctcaagattcacagccagttgaggaggtggacaggtgacagcggcgaggtccaggcctgtcatgttccggggcttgcaaggaagtgggggtttctctgtttcctttgctgcccttggaggtcttggtggagcacttgaacctggcttgggaggaaggtccttgtagggaggtgttgagttctcatagtcatcatcctcctcctcctcctccatggtccagtttctgtggttcaggaatctgagagcagcttagctgggtagttctagcttgagatctcttgcgtgattgtagtcaagatgttgcctgggactgcaagtcatctgcaggcttgactggggctagaggatctgcttccaagatgatgcactcacatggctgttggtgggaggcctcagttccttgccatgtgagcctctccaaagggatgactgggcatcttcacaacatggcagaggcaaagatagaagccaccatgctcctatgatctagcctcacaagtcacaaaggatggtctccactatacagtattctatttatcacatggaccagctctgagtcgttgtgggaagagactggcttgggaggaaggtccttgtagggaggtgttgagttctcatagtcatcatcctcctcctcctcctccatggtccctggcttgggaggaaggtccttgtagggaggtgttgagttctcatagtcatcatcctcctcctcctcctccatggtccctggtgggtccgggtacccagtgatggaatacagattatgcatgtctagcacagggaacctgacaagtggcagccagggcttggcaacctctgccccctgtctctccgactcaggcgtctgggggctctctcagttcccttttcctttcaaagtcaaatacatgcaaattcattttgacaggaagccctcagacctcacacgtgctcacacaaacacacacacacacacacacacacatacacacagagcctttctccccagtttggattcacgcacagaaggaataatgacaactggcctggtgtggt

SEQ ID NO: 17225 - RNA, 1841 nt, Homo sapiens
  source 1..1841: mol_type = other RNA
tcaggccaggcacagtggctcacacctgtaatcctcacaatttgggaagcccaagtaggaggatccattgaggcaaggagtttgagactggcctgggcaacatagtgagactccctctctttaaatgctacaaaaaattggccaggcatggtggtgcgcatgtgtagtcccagctactcaggaggctgagatgggaggatcacctgagcccagaagtttgaggctgcaggaaaaggagcccagtcccagctctttgtggttcacaggcgccaggatatttcatcccaggttcaacaccagccccagggtcctcagggctagtatcacttcccaagagtcatgatcaggaacttagtgaagatcctttcaaccccagaagtgggagacctcccaccaccaagctctgagcatcctcccagctcaccatctactagggcaagcccaagtcctcactctagaaacagcctgacttgcacccctgggaacttgctgcatccagggtgccaatcctgtttgaggcacatctgtgtgtccactcacgaagaggcaaggccgtccacgaaagggcaggagattctcatctcaaagagacactcagatatggacccccagcctcggccctgggcttcaacaggaacatttccgctcacaaatccaatacgtagttttgtagcaagagagatcattccaggtgccacctttgttcatggtagcacagtcctcatcgtggatgttattgggttcctctggctcccagaagcttaatgtcacaggagacccatccagccacctccagtccccttcctgggccctgtcattcagccccagccagtacacccgtggagagccatgggccttggccacaaaattgtgctcagcaaagctattgatgatgaccaagtgagagtaattctcctggcagaacatccgggcctcatcccatgacttggtgcttggggagaagtagtaacacttgccctcaaagggcagccagccttcaggacaggtaattcggcggcagtctaataagccccaaagttccaccagggactggttggtgtcagctcttacacgggcaatgtcatgcttcaggccagctagccctgccatgccagtcatatttgttcgccacgtcatctgctgaaagcttaacattctcagttcttccatcaactcctggtacttaatcagggtcacagtgagaccaaggcagcccaggaacagggaagtcaccaccagcagacacaggtacaccatccacctcttctggcagcagccaggacctccagacctctgattgagccaggggactggagttgcggccagggatggctgcaatggagaaggctcaagattcacagccagttgaggaggtggacaggtgacagcggcgaggtccaggcctgtcatgttccggggcttgcaaggaagtgggggtttctctgtttcctttgctgcccttggaggtcttggtggagcacttgaacctggcttgggaggaaggtccttgtagggaggtgttgagttctcatagtcatcatcctcctcctcctcctccatggtccctggcttgggaggaaggtccttgtagggaggtgttgagttctcatagtcatcatcctcctcctcctcctccatggtccctggcttgggaggaaggtccttgtagggaggtgttgagttctcatagtcatcatcctcctcctcctcctccatggtccctggtgggtccgggtacccagtgatggaatacagattatgcatgtctagcacagggaacctgacaagtggcagccagggcttggcaacctctgccccctgtctctccgactcaggcgtct

SEQ ID NO: 17226 - RNA, 2063 nt, Homo sapiens
  source 1..2063: mol_type = other RNA
tcaggccaggcacagtggctcacacctgtaatcctcacaatttgggaagcccaagtaggaggatccattgaggcaaggagtttgagactggcctgggcaacatagtgagactccctctctttaaatgctacaaaaaattggccaggcatggtggtgcgcatgtgtagtcccagctactcaggaggctgagatgggaggatcacctgagcccagaagtttgaggctgcaggaaaaggagcccagtcccagctctttgtggttcacaggcgccaggatatttcatcccaggttcaacaccagccccagggtcctcagggctagtatcacttcccaagagtcatgatcaggaacttagtgaagatcctttcaaccccagaagtgggagacctcccaccaccaagctctgagcatcctcccagctcaccatctactagggcaagcccaagtcctcactctagaaacagcctgacttgcacccctgggaacttgctgcatccagggtgccaatcctgtttgaggcacatctgtgtgtccactcacgaagaggcaaggccgtccacgaaagggcaggagattctcatctcaaagagacactcagatatggacccccagcctcggccctgggcttcaacaggaacatttccgctcacaaatccaatacgtagttttgtagcaagagagatcattccaggtgccacctttgttcatggtagcacagtcctcatcgtggatgttattgggttcctctggctcccagaagcttaatgtcacaggagacccatccagccacctccagtccccttcctgggccctgtcattcagccccagccagtacacccgtggagagccatgggccttggccacaaaattgtgctcagcaaagctattgatgatgaccaagtgagagtaattctcctggcagaacatccgggcctcatcccatgacttggtgcttggggagaagtagtaacacttgccctcaaagggcagccagccttcaggacaggtaattcggcggcagtctaataagccccaaagttccaccagggactggttggtgtcagctcttacacgggcaatgtcatgcttcaggccagctagccctgccatgccagtcatatttgttcgccacgtcatctgctgaaagcttaacattctcagttcttccatcaactcctggtacttaatcagggtcacagtgagaccaaggcagcccaggaacagggaagtcaccaccagcagacacaggtacaccatccacctcttctggcagcagccaggacctccagacctctgattgagccaggggactggagttgcggccagggatggctgcaatggagaaggctcaagattcacagccagttgaggaggtggacaggtgacagcggcgaggtccaggcctgtcatgttccggggcttgcaaggaagtgggggtttctctgtttcctttgctgcccttggaggtcttggtggagcacttgaacctggcttgggaggaaggtccttgtagggaggtgttgagttctcatagtcatcatcctcctcctcctcctccatggtcccttccaggggaaaggcaagtcagagcccagccattccctcctccctccatccctcaagccctggtctctgcctcagctgccccatgatggggattctgtaccctggatcttgaccacacctgggccccagccccagcctggccagggccttacctggtgggtctggacacccagcgatagtatacatgttgtgcatggctacagctaacaccaggaacatgacaagtggtagccaggtcttgtccctcctactcagatgtctaaggcatctgtctgtttccctttcctttcaaagtcaagtacaggcaaatccatcttggggggaagcccctggacctcacacaaacacacacacacacacacacacacacacacacacacatttttctccggagtttggattcacacacggaagaaacaatgggccgggagtggtggctcacatctgtaatcccagcactttgggaggctgaggctggcaggttgcctgagtttggg

SEQ ID NO: 17227 - RNA, 1731 nt, Homo sapiens
  source 1..1731: mol_type = other RNA
tcaggccaggcacagtggctcacacctgtaatcctcacaatttgggaagcccaagtaggaggatccattgaggcaaggagtttgagactggcctgggcaacatagtgagactccctctctttaaatgctacaaaaaattggccaggcatggtggtgcgcatgtgtagtcccagctactcaggaggctgagatgggaggatcacctgagcccagaagtttgaggctgcaggaaaaggagcccagtcccagctctttgtggttcacaggcgccaggatatttcatcccaggttcaacaccagccccagggtcctcagggctagtatcacttcccaagagtcatgatcaggaacttagtgaagatcctttcaaccccagaagtgggagacctcccaccaccaagctctgagcatcctcccagctcaccatctactagggcaagcccaagtcctcactctagaaacagcctgacttgcacccctgggaacttgctgcatccagggtgccaatcctgtttgaggcacatctgtgtgtccactcacgaagaggcaaggccgtccacgaaagggcaggagattctcatctcaaagagacactcagatatggacccccagcctcggccctgggcttcaacaggaacatttccgctcacaaatccaatacgtagttttgtagcaagagagatcattccaggtgccacctttgttcatggtagcacagtcctcatcgtggatgttattgggttcctctggctcccagaaggtgctcagcaaagctattgatgatgaccaagtgagagtaattctcctggcagaacatccgggcctcatcccatgacttggtgcttggggagaagtagtaacacttgccctcaaagggcagccagccttcaggacaggtaattcggcggcagtctaataagccccaaagttccaccagggactggttggtgtcagctcttacacgggcaatgtcatgcttcaggccagctagccctgccatgccagtcatatttgttcgccacgtcatctgctgaaagcttaacattctcagttcttccatcaactcctggtacttaatcagggtcacagtgagaccaaggcagcccaggaacagggaagtcaccaccagcagacacaggtacaccatccacctcttctggcagcagccaggacctccagacctctgattgagccaggggactggagttgcggccagggatggctgcaatggagaaggctcaagattcacagccagttgaggaggtggacaggtgacagcggcgaggtccaggcctgtcatgttccggggcttgcaaggaagtgggggtttctctgtttcctttgctgcccttggaggtcttggtggagcacttgaacctggcttgggaggaaggtccttgtagggaggtgttgagttctcatagtcatcatcctcctcctcctcctccatggtccctggcttgggaggaaggtccttgtagggaggtgttgagttctcatagtcatcatcctcctcctcctcctccatggtccctggcttgggaggaaggtccttgtagggaggtgttgagttctcatagtcatcatcctcctcctcctcctccatggtccctggtgggtccgggtacccagtgatggaatacagattatgcatgtctagcacagggaacctgacaagtggcagccagggcttggcaacctctgccccctgtctctccgactcaggcgtct

SEQ ID NO: 17228 - RNA, 1830 nt, Homo sapiens
  source 1..1830: mol_type = other RNA
tcaggccaggcacagtggctcacacctgtaatccttgctctttgggaagctgaggcagatggatcacttgaggtcaggagtttgagaccagcctggctaacatggcaataccatctccactaaaaatacaaaaattagctgggtgtggtggtgtaagcctgtagttccagttacttgggaggccgaggcaggagaatcacttgaacccaggagatggaggctgcaaggagccaagatcacgtcactgcactccagcctgggtgacagagcgagatagtcaagttttctctctcaatcctttgttgttccttctgtctgttgagagcactgtgatataactttgggggatgatcagccgatctaggaattgtacttttgcttcccggcttttccgcctgtcttgacagttctttcaaaagcctctgattttcccgatcgatctgtctcacctcttctcttgtgaaagagtagtttttcccgggtgctactgaaggctgatcaaagtgatgtttttgtggtccttttttatctaattgcagaaaagctttcaagagatgattcagatccattgtgtcatgtaagactttctgtttatgtctgtggtctaaactggagtctaacactgaagacgactttgaggagacatcaggctcatgtttttctttcccttttttggctgctttcaaatattttgaattatttttcaaatcctcaacatcttcatatatttcttggctcacattttcttgctttttaattttcactttttgatcatttgctatgcccagttcaaaagactgaagagggctaatgtctggagttgataagggacttacgtcagtcacagtatcttcagactcctcagggtagtggccacattttggtgtagtacttgaaggctgtgtttctgtcgattttattcctgatttatacttgtgttttggtgacaggagggttataccagatacatgtttcttagatgacttagatgacggagacgaatcagatagatggctatcagaccctgcatctaaacaatctgtacctgaacctgaagatgaggaagataaagaggaggaggaagaggagctaactttgcaatactttttccttatgctttttttaacgttagtagatggtttagcggacttggacttcacatggtatttcttcccatcatcactgctttcctctccatctgtgtagtaatcatcttcaccttcttttacaattttgggaattctatttggaatggacacgtgtattttaagtcctgttgtaacatcacacaatttttttgatcttgaagaggctggcaatgagaaagaacttacagtttgtgtaacatcattctctacggggtgttctgggggaaatttcacgtttctttcatttcccttctcagtaagataattttctgttgtttgcattccagtgttcgaatttacattttttgtatctttatctattctttcctttgggtcatcattttgcttgtcaaaaactgagttagtttcacatttctttccttcttcaaagtcactgtcaaagaaagaatggtccacttcaccttctaatatatctccaaactgatccatgatggcaaaaatatatcccgagtactcgccgccgcctgggctccggagcggggagacggatgcgaacggaaaggagcgtggcgggcgccccgcgagcagggagccaggagccgctcgcgcgcccctcacctgagagccgcggccaccacagccccacgcgcggcgctggcgcactcccgcggccctgaacgggctcccggcgccgcgcgcccgcgcttccggaggcggagag

SEQ ID NO: 17229 - RNA, 2778 nt, Homo sapiens
  source 1..2778: mol_type = other RNA
tcaggccaggcacagtggctcacacctgtaatctcagcactttgagatgccaaagcgggaggactgcttgagcccataagatgagaccagcctggacaacatagcaaggcctcatctctacaaaaataagaaagaaaataactctacgattaacactacactttcttgcccaccctacactactttgtagaaaactatgagaaaatggaaaatggttaataggaaaaataatgaaaactactttacctttaccagttacaattttctcacgttctaatctaacgctttatattatgcaattggaaatcttgtcagatgatacaggaataacaacattcagctgatggccttccttgataatctattcgctctcctcgccagtactccaaaggtttcaaacgtgttctcttggtcctgcgaacatttggtgtgttggagggcaatactagtttgtgatggattctgttctttggtatcactttagattgttttgagtcatctgaacttccatgaacttcctcatcatccacatcattctttccagacattaaataattattattgagcctggaaggtccactttcctctaaaactgaagtcttatgctctccagaatccaagtttgactctgttggtatattacatgtatatccactggtctgaggctttaggggaacattctgtgcagtcataatgttatcttcattctttgagcttcttgtagatctagaacaatcaagatttttcttcttagccaagtctgcctcatcactttccaatggctcactcagcgaacatctggaaatttcatcatgaccaacgatacctccagaaccttcagcatttaaaaacttctgtactctttggttgcctttagttgctgtcttctgccttttaagtggaatagtttttttcctaatattcttagatgactgatttgttttcttagtagattttcggctactattgtgatgcattggtaattcatttcttactgaagaattgctataaacaggactctcctctgattttaccacccaccaatcagatggacgcctggaaattcttcgacttttcgtgacagttgaagtcacttcttcaggtacaagtttgttcttggactcactggaaaagcgcttctttttagattcttccttatcttttctagtgctacttttcttgcttcccacaggtggcatctgttttttggaaacacaatcatttcccatctcttcatgctcttccatatttctgtctgaatttctttgaaattcgtcttgggtaatatgtgatgtatgtatgttttcatctttagactgtcccacatcaagctgttcttcagctggtttagccatgaattttcttctctgtttttgttttatagtccttttgcttctagatggtttttctgcattcttggaatacatttcatattttgtagatctataattatttactgtttcacctatcaaagcataacttgtatccagtactgttttatcagagggctgagatgtctctactgggtgaggtttatgggaatgtttgtcatttgccaaagtcttaggtaatatattatgatgcttttctcttgactttctaccttgaaggagtgcagtgctctcagccggggatattgtgcgttgtttcagagaccctgcctttcttggtattgtaatccaagatctactggcaaaactttgatccgactcatcaattataaattcatcctctatcaacttcgtatcatcgggaggacacgaatgaggtggagcagttgccgcatgcctaacaatgggactggattcactttttcgttttactgtttctaaaaacaatgttgaaaaactttttttagcttgtcgttgaatttcatattctgaatctcgtattctattctgagatgatcctgatggttttctttcttgtccttccgatgttttatcctcttcatctgatactttattatctatttctattttctttaacataactttatcatcaaagtttaacctttttttggttttaactgaaacctctgtacttgaaggcagcatatttactgaattttcaaaagtgtaagtctctctcttttgggcactagatggaataacattttgtgatacagatgtttttgcatccaaaagaacagaaggtgagccaacggataagtaaaattcttcatcagcttcactgtgatgatcatttatgtttctacttgatatttttttcgagtcaggtgtatttttggaactaacatcagttgccagaattttctgatgaacttcatgggcctgaactgatctgtttgtggcttcacttggttctacaacaaactgtagagaggcttctttcttctttgaagaaactggaactgactttggatgtgatttctggcactctttgcttggtgactgaatacaagtgtcttttattttgcgtgttgaattaggcactgattttgtagaatttgtactaaaatcattggcaagacttttttcttcaaaacagtcttgtaagatttccagaacattctggccttgctctgtgttaatgtcacgtgccctggaaggtcgacaaaatcttcttctgtagccatttttgagatgatccagaccggacgcagccatgttccggccccgctgagccagcgcaactgtctgaggtggaagcccacacggaccacagctccaggaagccgagcaagaaacgaatcgccggaataccaggccgcggccaagcaataaccttaagtctcaggcgactgccgcgagagct

SEQ ID NO: 17230 - RNA, 14919 nt, Homo sapiens
  source 1..14919: mol_type = other RNA
tcaggccaggcacagtggctcacacctgtaatcttatcactttgggaggctgaggcaggtggatcgcttgagcccaggagttcaagaccagcctgggcaacatggtgaaaccccatcgctataaaaaacaacaattagccgggtgtggtggcacatgcctgtagtccctgctactcaggaggctgaggtgggaggatcacttgagcctggggaggtcaaggctttagtgagctgtgatggtgccactgcactccagcctgggtgacagagtgagaccccatttaaaaaacaaaaacaaaaacaaaaaaaaatgtgacatatagttgactaagaagtacatttcaatacaggattgaaagaacccacatatgttaattaaacacaagcgcagaatttgtgccttttacataaaggaagaatgcacataggcatgctttcagacaagcaattcatctagcagaaaaggaaggaatacatttttcagcccttccaggaataaaatccataaatgggctctatttcgtcctccaacacttgtatttcccacgtcatttactcctgcacacccccactcactagaagcctgctaaactgttccagtgagatattttaacacctgatagggaataaatatgcttctgttttggccttcaaaaataagctctgggccagttgcagtggctcacgcctgtaatcccaacactttgggaggccgaggtgggcggatcacgaggtcaggagtttgggatcagcctggccaatatggtgaaactccatctctactaaaaatacaaaaattagccaggcatggtgcctgtaatcccagctacttgggaggctgaaggagaagaatcgcttgaacctgggaggcacaggttgcagtgagccgagatcacaccactgcactccaggccaggtgacagagcgacactctgtctcaaaaaaataaataaatcaactctgtagcatagcatttgtaattctattattttgccttacatttccattatccttttaataaaattgtttttttacatcttcctaatcaagaagtattatgaggccaggcacagtggctcatacctggaatcccagcactttgggaggccgaggcaggcagatcacctgaggtcaaggtatttgagaccagcctggccaacatggtgaaaccccatctctactaaaaatacagaaattagctgggtgtggtggtgcacacctgtaatgctagctactcgggaggctgaggtaggagaatcgcttgaacctgggaggcagaggttgcaataagcctagatcatgccactgcactcaagcctgggagacagagcgagactacatcttaaaaaaaaaaaaaaaagtattatgagagaggataatgtattgtaatgtattgtagaggctaaataaaattatgctcatgtcagaaaaaaagagtatttctcaaaataaaattcactgaaactggatgtttattttgactgagatatagtatatcctcaaattgccatagaaagtttacaagaatattagaggtaaattataaatatcagggcctttttaaaaaaaaaagattctgcttataacttggtatttgtttataataaaaattatagtagccaataatgaacacttactctggcttggttatttacttaggtcaaaagaaggaggagcggttaaactgtgggatcaggaactgaggcggtgccgtgccttcaggcttgagacaggacaagccacagattgtgttcgttctgtgtgcagaggcaaagtaagatgttccatgagctgatacagtgcagcagaaaacagaaagtggttattactgtgattccctcaccctttgcagcctaatgaacaatacttaataatgcataacgatggatttgcttgccaacattactctgtctttgctgctttctttgccaaagttagcaccagtgtggtgcataagctaggaagctattctgtctaaatactgtatgtaaacctccaatattttctagaatctgccaatttaacaactctagtagacataattgaaagcccttggcagttgactcatattaggacagctgtctccattttttaaaaaaacacacattccctagataaaacgtgcagtaaacaaacaatgaaatactactcagccataaaaaataatgaaattctgtcattcttggtggcaacatggatgagactggaggacatgatgtgaagtgaaataagccaggcacagaaagataaatacatgttctcactcctgtgcagaaactaaaaaagttgatcccacagaggtggagagtagaatagtggttactggaggcggacaagggggagggggagggggatagggaaggactggttaaaggatacaagtttacacagccagataggaatagtatgttttagtattctgtagtactgtaggatgactatagttaagaatcacgtatttatgtattttcaggtatttacaagagaggattttgaaagtttccatcacaaagaaatgataaatgtctgaggtgatggttatgcgtattaccctatgccctatagatatgtataattatgtgtcaatttcaaaataaaaattcaaaactacaactcctatgaaaatttttgagcgtgtttgtacttattaagtgtatttataaatcatacggatattatcttcagcctgcatattaaattgtagttaagcttttactttttaactaaaaaataaattctattattttttcctatatcccactgcactgaccccagtttggaaatcctaagattatcaaataaaaactttgattattgaagaatccaggtgtactgccacagaaaagttctattctgtagcatggactctaatatgtaatctagcccattgtgcttacagatagatgtgtgcctgtagtcatagaaaaatttgcatgagctaatgactgccttgctactagattagctcaaagcaaaaagttctctgaaagcaggtcaatagggtcatttttatattatgaagaagaaaagcagctgttgtattacattcactgtattggtcctgcttgtgtttcagggcaagatccttgttgggacaaggaatgctgaaataatcgaagttggagagaaaaatgcagcttgtaatattttagttaacggtcatgtggatgggccaatctggggactagcaacacatccttccagggattttttcctttctgctgcagaagatgggacagtgagactttgggatattgctgataaagtaagtacagataatttttttaaaagaggttacaacttctaaaaagaaaagttggaagttctaaattgctagtacttaaagaactgccagaattctgttgagcattttgaggggaaactggtataatttagaagtacttcacttaatgtttcctatgactctttttttttttttttttaaatgcagaagatgttaaacaaagtgaatttgggacatgctgctcgtactgtgtgttacagccctgaaggggacatggtggctattggaatgaaaaatggagaatttatcattttactagtgagttctctaaaaatatggggaaagaagagagacaggagatgtgcaatccatgatatcaggttagtgaacaaatggaatagagtttctagtatatacttgatttaacttccatttgtaaaattttccatagccttgccttcaaaaagaggtccccagggcctgtagcatttcccgtattataaattgtatgctaaaatatggctgtttgtatactacttaattcttcttgctaaattataaacccactgggcaccaactataatagcaagtactagtaggtaatgtttgatgaattcatgttaacacttagccatgtccattaagttcatcccaccaagaggtatctcccactgtaatacaagagagctatctgcccttcaaaagttgtcaccctggaaaactaaagttgtgatttcaaacatatcttctcttagtaacctcagtttgggaatatgtagttcattaatttaatcaatacctattgattaaatgttccagaatccaaattaatttaaatgtttcttaaacctttgtttttcagtgcttaagcatttttcaacagtggctaccatttacggagtacttccgtgtgatcagtagataagattattgaatctaggtctgtcaaaagcttgtacacttttcatcagtaaaatccttttacaaatgaaaccttcctcagaacttcaatatataaaatagtaacagtggcttcccttagcttttacatgtctctatcgtacctcagtaagactcatgggccatttcaagagactgaattgtcccatatgactccaaagattgctaggcaaatagcatttcactttgtcttttaaataagttcttcaggccgggcgcggtggctcatgcctgtaatcccagcactttgggaggccgaggcaggcagatcacctgaagtcaggagtactcgaccagcctggccaacatagtgaaaccccatctcaactaaaaatacaaaaatcagccgggcgtggtggcaggcgcctgtaatcccagctactcagggggctgaaacaggagaatcgcttgaacccgggaggcggaggttgcgccatcgcactccagcctgggagacaagagcgagacttcgtctcaaaaaaaaaaaattcttcttccaagattcaagttgtgtcatttcaccttaataactggaggttagttaagctgggctgtgttctttgcttaatattaagacaacgttttttccagatggaagaaaactatcttaatgaattgttagcttattaattatgtaatgctaatggcttttaaaagctgagatgttctgactgggtgttgtggctcacacctgtaatcccagtaccttgggaggccaagggggaaggattgcttgaggccaggagtttgggaccatagtgagaccccgcctctatttaaaaaattaaattttgttttgttttgttttgagttggagttttgctcttgttgcccatgctgaagtgcaatggtgcaatctcagctcaccacaacctgtgcctcctgggttcaagcgattctcctgcttcagcctcccgagtagatgggattacaggcgtgcaccaccatgcctggctaattttgtatttttagtagagacagggtttctctatgttggtcaggctggtctcaaactctcgacctcaggtgatctgcccgcctccgcttcccaaagttctgggattataggtgtgagccactgggcctggcctaagaaagtttttttaagccattagacgtttttaaaggaattgggagatgacaattggggaaatatttaaaatttaagtaaaatataaagcttccttatttcatgtaacccagacaatctcagtatacatgatcagttgtgtctgacaggtaaatctatttgaggccttatcacacgttacttttaagaactagaaaggaaaagtcactgatcttaagtatttataatacttcatgtggtctaatactttttacgttttgttttgattcagatttagtccggattcccggtatctggcagtaggttctagtgagaactcagtggatttttatgacctaacgctgggccccactcttaacagaatcagctactgcaaagacattccaagctttgtcattcaaatggacttctctgcagatagcagttatctccaggtacagtaccaatactgtatacccaggtggcaagttcttctgcttttacatttcgtgttagtgaatgcatttaaagttcctgagctccagagctccagcttctcaactcctccctttgtaccttctgacctacagctcccctttcctcccccacttatcagagcttttctcctattaagtttttgtagtgatcttttgcatacttaataatgttagacatgtaaatcaagtagcaatatgctagtattctgtaaaccccctgtggattttgtctctcacctaatggaattcttgtcccattttaatctgatgaaaaaggtctctagtggctgctataaacggcatgtctatgaagtgccttcaggaaaacatcttatggatcatgccgctattgacagaattacttgggctacatggactaggtaaatacttatatattcacaaggcaagaactgactttgaaggccagttagaaaatcctatttctgaactgttagagccattccaataaggaatagtaattgagtttcaagtttttgttaccatattttgaaatggtatgttcatgttgggacccctttttattgaatatatttccatgttttatcagtttccatgatttatcaagttttttttttaaggaaatcaaagttttaactttaaagataccctgatatttttcttaatgctaaatttaatgactggcaaaaaggtattgggtgctgttaagcaactgttattaattctctatctaaaggaatgctatcttgaatctattagaagtcaaagcttccaaatttgttcaaatttcctggctgtatgacaggtaaccatgactatccatttttttggccaatgaaaaatgccatcaaattcctgtatcagccaggcatatagtggctcatgcctgtaatctctgatgtagcaggccgaggtgggaggatcacttgagcctagaagttttgataccagcctgggcaacatagcaagaccccatctctgaaatttttttaattcctatgtcataagtcatttttatttttgtagagatagggatctcacaatattgcccaggctggtctcaaactcttggcctcaagcagtcctcctgcctcagcctcccaaaatgttgggattactggtatgtgctgctggacccagccaagtagcacttttaatttgaaaaatagttctatcagttttcagtcaggcgcggtggctcagcctgtaatcccagcactttgggaggccgagcgggggtgatcacctgaggtcgggagttcgagactagcctgaccaacatggagaaaccctgtctctactaaaaatacaaaataagccgggcatgttagcgcatgcctgtgatcccagctactcgggaggctgaggcaggagaattgcttgaacccaggaggcagaggttgcggtgagccgagatcatgccattgcactccagcctgggtaacaagagcgaaaactccgtctcaaaaaaaaaaaaagaaaaaatagttctatcagttttcataaagtactactttaatcttaaaaagattaatctagaaacccttcaaattataaaatgtcatttttaaaaggcaggagttgatatcctgatgaaattcaggtctccaaacaacttaccataatttacttcctgtattttaagtaacatgatagggtacttagagattaattgccaagaaactttttgaatatagtcaacctgcccgcacttgccatgatgagttttcttttgttccttccctctagtattctaggagatgaggttttgggaatctggtccagacatgctgagaaagctgatgtcaactgtgcctgtgtatctcattcaggaatcagtcttgttacaggagatgactttggcatggttaagttatttgacttcccatgtccagaaaaatttgtaagtttgtgttttgtttactattatcagtttactcctaattttgatgtcttatcatcagcacttttccccatatatttaaaatgttttgtcctaatttctaaatttttccccaaactttctaaatctatttactttgaaataaaagctattagaaacaaatcctctccctcgagtaataccatctttggaaccatcctacaaaagctgtaattagcttttcaccaaacctataatcagttatcaaatttcaaatgcttttccttagagaaaaatggtcagagtacctggagacatctgactgcccacacagcctggttttgcagatccactactcatgctgaaaagcattctaatcactggctgcggtgctaactccctactctctccacagctcttgtcatagagattatagttcctaataagagcctttgacttctgtgtgcaccaaatgccctgagcttgtctgtcattgttttttaggcaaaacacaaaaggttcttgggtcattcgccccatgtgacaaatattcgatttaccagtggtgatcgacatgttgttagtgctggaggtgatgactgcaggttagtaactttctcagcccatgaagagcagactatgttactagttaagagacttaatacaacaactcctacagctttggtttatgaaatcagctagtcaacattagtagaaggtagtataaccagatggctcttcagaatctcatatttatgcaaatacagaataaaaggagttaaagaggaaaaatattacacatgtaacctgaaagcacaactgaaaaatattaaactgttatgaaaatctaaaaacataattaactccctgcaattttcttctctgattgcagcttatttgtctggaaatgtgtacatacacctcactgagagatgctgagatgactacagaaattaactttgagaccagaattacagagaagaaaaaccaaaacccaaccctgcatggtcaagtggtgctaacccaagactgtaacagggagaaatgcccagaatcatcaaaatagtgaaagactgatctgttcaaaatatttgctatatgcactgggtataatccgtaatccatacactgccagataatgccatttcaaggaaggatcgaatacttgatggtaaaggccaagtccccctgtattgggaagtgtgtgatttcggcagacctgctgggaaaatttagggtagagcactctttacagaagaactcaaaaacccaatttggataattttcattatctttttagcaaaatggtttcttaatgtttatattttattttcaaggttcattgtttaatgaaatattttattcttgcatttccataaggaaagggaaagtcatgatcatcctaaaggatcacagtttttaaaaggcaaacattttccctaaggaaacagacacaagctttcctagagaatatgatgttttttaggcattaataaggtccttttttataaaggacacttttctcctagtagttttgaattcaggaacagatccaaagttagcagtatatggctgctacatttccattttcattttcgagccatcagtttatgttcagatgccatctctgtaatcgcacatttaaaacataactgtagcctcactaatggaaaagtagtatgatgaacaatcattcccaatggtgtacaatgtaagggttttagggagcaacagtatttaactggaagaaagaattgcatatttaatgtagtctaatatatacacatttgtttaacatgtaaacaaaagtgttaaattcacatatacaacattatacaatttaatcactcttggaataaaatttttatagccttttttctattgggaaaatttgtttagatgtgtgccactccataggtttatttccaaaatgaatgagcccaactccatttgtaaaaacttgtcagttagaattcctttttttagtggattagggctgaattcttagatccttatttcttttcactttaaatgctgccaaagatcactactcatcattcaggaattcgctgtctagcctatctgtagtttcctgaagattgaaaattatgtagactgctatttaaaaatatatttttctaagtgtgaggtttaagatgctgtattgaccctatgagtttttaatgtgttaattatctttatagcataatagatcgctttaggttcctggaatcccatttggtctgacaggatatatgaagattcttaatacctattttctgtgtctaatacttggttaatactaaaaatagaaatgactaaattacatcacagaaagcataaccagtgattgaacctggtagttttaaagctctaaatagctgtggctgaaggactgattatggggctaagaagcttgaaacgtaagttggtacttgttcatcagtggattctcctaaattaagccaaattttgaaatacatgactattaagtttctactcatgtatttacagtcagtcaataaattaaaggaggaaaaaaatccctgaacaacctgcccataaaaagaaaaatactctacatttgagcctgctgcagttttaaattttccctctgggtcaagtttgccagcttttggctacagagaaattatatttccattacagtgcaggtagaaactctgtaaccttaagcatgtaaactacatagaataaaactgtttccactgcatttctgtccttcaaagtggccaacctgattaagtcagccttaatcactgctgctgtcagtttcacgactaaaggtcatattgactaagtagtcatcagctgaccacctcgctgtatcagccagcaacgaggggaaggtgaagaaacatgataggccatatagaatctgccctatgtttacttttttaacccagataattatttttgtgtgcagtatctaagctcctgattgtgtaacctgggacttctggcaccttttgttccattcattttatgtataaaatgcatgccaaagcacactgtgccctctggtacccttgcttccaatcgccaaccatgctcatttccttcctttttttgtggtccctttttgtggtgatcattttaaaccacgtcatccaacaaatgttttatggtcaaccttagcttgttcataagccatagcaactgaaagattaaactcttaaatatgtgtctgggcagtggctattaaatagcaaaaaacaatcagattttagtattttattatttccttgtaaaatggctgaactaaattaaacccttgtttcccatttgttctataatttatagtgaaactgagaacaaaactatctttataaatgatagctaaaagtatttccagatatttaaacaatttaaaataaatttcttctgcagagatgcaaagcatctcaacactggaatgaacaaatgccttaaattcaatggagtaaacctttagaatgaagaggaactgtcatttcacccaagccgaagacaacagccttatgcacttgtgtgctctgtctttgctgcttctcgtgtttcaagcctttcctgtgggatcagcacagcaaagtgcaacttaccaaatggtttaatgactggttaattctttcttctcccaatggaaaagcaatggcaacacaacagtagactgctggcttgacaatcttaaacgtgagcctttgcacatgtaggtttatcatcatttgagtatacgactaagcaagtcaatgaactttttttttttttttagcagtttaatttggtcctgagaatgttgcagtctttattaccccttttgcattaatccacttttctaaccaccttttaagctttaatttttaacactatacaccaagtctttgaaatcagtgatctgttatttaactctaaagcatttgacacttcttgccttaacagttttaaaaaccacacacaaaaaaactctgtaagtaatacagtaggccaaaagtttcatcctatctatcttgcagtttacctatctgatctgatctctgtaattatagttctgtcatttaaaatatactatttaaatctaatttttacatttcaaaaattatcttcagtagtaactaagtatattttctgtggattctgagaatgttatttttcagaatgtgagaatatatatgtacatttataatcttgtgactttaaagtctgttttcagatacagtatgtaaatacttgtaaaaaaatttgtataattttgtgataatgtagtttcccaaaaaaattatttagaaggcattatgttattagtaaatgagagcactgtatagaactgttcctattttctgcacttgccattccagctgcctccactgtccatacccacctcattcatcctgtcacagaaggcaggaaaactgggaactttaccaaagtagcactcagcctgagaggcctgtataatcatgcttttcaaactaaattcacttaaaaattaaaaagcagaattgaatattttaagcagcctcagtacctttggccaatgctgttttcatggtggattatgaacattatataatctttgggaaaagtgaaagtagtacaatttttagaataatgacaactgcctcactgcatctctccactcacacagcaaccgtgtagccccctaagctgcagtaccatgactaaccatgatgtcaatttcatatgctgatcctcacaacagcagtgcacaaacatgccccaaatattttaacagaatttagctcttccttaagctgtcttttcatagtaaaaacaaaacaaaaacacccaatgttaaaaccacataataaacttacaaacttgaaaaattagacacttcagatagataggcaataaaacttcatattatgaaagcaatatattccaagtttcaaagatttgacaagttctgtagagtatctttcatcagtacatgaaaacttccaaactgcatgatcttctgccaggcaggactgggtgctattcgctggtttgaggtcgaatccatttcaaggcatgtcgtggtgggacattaatggtgggatggtagaatgtgcagtccggtcttgtacattgagtgttaaacctacaatgttttggatgatagaagggacattccatcttcttacaagcagggaagtaacggcagagctgactactggaaggtggtgctggtggtgcaactgctggttttggagacagtactggaattcttctactcacatgagtgaagggacaatctggtttagtacactttgcatcatatttacaatttgggtgaacaaacaaacatttttcagcaaatttacaattggggaaggctttgcagggtgagatggggtgatggtaggcacactcatccccatttttacaagcaggccagtacttgcagcgctccaaaagtttttctggtttctgtgccacactcagttcactcatctcagcatttgggtcctcaagctgcctgctcagcaagtgcaactgctgtgggtggaggagacctctgagtcccttgtttgaggctgcagtttggtttacgggtttcattccttcaaagcacatgtcctcctcttgatctgacatgtatcctggggggctggggacaccatccagcgtcactataaacttgggacttgcaggtttatctggttgtacaagatctcgtgtctgcataaggtgtcctgaaagtacccgaagggaatctgcagtcttcatccccgactcttggtttggtgccactactacttcctcagacagctttggcttcttcagaataaatgatcttgtgtctgcatggaccatggattccatgtcatagtaatcttgactcatctgcagagtttctgccattactgggtcgatttgcagtcgggataataattgcctctgttgagttccttgatttttttctacagaatctccttttgtttcctcttctttaatggggggacttattctgggggtcctactttgtccctggaccacttctgctagcaattcttcttgagaagttcgagttctgggagcaactggaagtgtctgtttctgtggaactgtagagtagttagttgtttttgttacggattcttgagcttcagatatagccttcaaaatcagattcttgttagcttgtttagaaggtggaagagaaggtctcctttcaggctttgcaggcacagacacactgctggagatgcttcctgttcgagacccgtaatcatcatcttcttcctcctcttctccatcatgattgaatttttttactttaacaactgaacttaccacaggcaactttctcttccgaaagttttcatcctccatactcattttctccgagttgtttctaaagaacggactatacgtttcttctaagctgttaagcacctctggttcacacaaacgtcctgtttcatatacccaactactctgcatatcaagctgcttggcagcatgaatactattctgctgctgttgaaattgcaacctgtttaaatgaacaccactatctgcatttctacttgcaggtggtcgataaatttcaatagaagggcgagaagaaccatatgtaagtgtcactgtaggttttttctgagataagggattctcctgcacaaagttgaggtcttcgtcaatgagatcatctggttctggcttaatatcaatcacatcttcagagggtgctggctccctcaaaggtttcactgttgacattagtcgggttgcagctccatcatcgtaagtctgtctgacatttgtggtttttgactcctgcgaacttgtagaaactctggaatctcttttttcaggtctcgcgctaggaatggcaagtggtggcactgcagcttcatgcctcctctcatctccccgactgaaattgctcttgtttgaaggcacgttactatcaaagatgttggtatcagaagacttcagactagagggttcagttgtaacagagcgaagtttatctaatacaccatgaagccatacggtgaatcgaattgtgttgttccctagaaacagggacagatcctctgtcatttggtcctgacttttcttgttggccaccatcaccataatgtaatcaggaagttcttcatcaacataagctcctaattcttgtaatttccccttaatggcactccggatcttgcggctgatctcggtgccgatctccatggctctgcggcgtgcgggaactcagcactgcgcggcgcttggcttacccggaggctgccgcggactcctaccccgcagccgggacaccaccgcctcc

SEQ ID NO: 17231 - RNA, 14844 nt, Homo sapiens
  source 1..14844: mol_type = other RNA
tcaggccaggcacagtggctcacacctgtaatcttatcactttgggaggctgaggcaggtggatcgcttgagcccaggagttcaagaccagcctgggcaacatggtgaaaccccatcgctataaaaaacaacaattagccgggtgtggtggcacatgcctgtagtccctgctactcaggaggctgaggtgggaggatcacttgagcctggggaggtcaaggctttagtgagctgtgatggtgccactgcactccagcctgggtgacagagtgagaccccatttaaaaaacaaaaacaaaaacaaaaaaaaatgtgacatatagttgactaagaagtacatttcaatacaggattgaaagaacccacatatgttaattaaacacaagcgcagaatttgtgccttttacataaaggaagaatgcacataggcatgctttcagacaagcaattcatctagcagaaaaggaaggaatacatttttcagcccttccaggaataaaatccataaatgggctctatttcgtcctccaacacttgtatttcccacgtcatttactcctgcacacccccactcactagaagcctgctaaactgttccagtgagatattttaacacctgatagggaataaatatgcttctgttttggccttcaaaaataagctctgggccagttgcagtggctcacgcctgtaatcccaacactttgggaggccgaggtgggcggatcacgaggtcaggagtttgggatcagcctggccaatatggtgaaactccatctctactaaaaatacaaaaattagccaggcatggtgcctgtaatcccagctacttgggaggctgaaggagaagaatcgcttgaacctgggaggcacaggttgcagtgagccgagatcacaccactgcactccaggccaggtgacagagcgacactctgtctcaaaaaaataaataaatcaactctgtagcatagcatttgtaattctattattttgccttacatttccattatccttttaataaaattgtttttttacatcttcctaatcaagaagtattatgaggccaggcacagtggctcatacctggaatcccagcactttgggaggccgaggcaggcagatcacctgaggtcaaggtatttgagaccagcctggccaacatggtgaaaccccatctctactaaaaatacagaaattagctgggtgtggtggtgcacacctgtaatgctagctactcgggaggctgaggtaggagaatcgcttgaacctgggaggcagaggttgcaataagcctagatcatgccactgcactcaagcctgggagacagagcgagactacatcttaaaaaaaaaaaaaaaagtattatgagagaggataatgtattgtaatgtattgtagaggctaaataaaattatgctcatgtcagaaaaaaagagtatttctcaaaataaaattcactgaaactggatgtttattttgactgagatatagtatatcctcaaattgccatagaaagtttacaagaatattagaggtaaattataaatatcagggcctttttaaaaaaaaaagattctgcttataacttggtatttgtttataataaaaattatagtagccaataatgaacacttactctggcttggttatttacttaggtcaaaagaaggaggagcggttaaactgtgggatcaggaactgaggcggtgccgtgccttcaggcttgagacaggacaagccacagattgtgttcgttctgtgtgcagaggcaaagtaagatgttccatgagctgatacagtgcagcagaaaacagaaagtggttattactgtgattccctcaccctttgcagcctaatgaacaatacttaataatgcataacgatggatttgcttgccaacattactctgtctttgctgctttctttgccaaagttagcaccagtgtggtgcataagctaggaagctattctgtctaaatactgtatgtaaacctccaatattttctagaatctgccaatttaacaactctagtagacataattgaaagcccttggcagttgactcatattaggacagctgtctccattttttaaaaaaacacacattccctagataaaacgtgcagtaaacaaacaatgaaatactactcagccataaaaaataatgaaattctgtcattcttggtggcaacatggatgagactggaggacatgatgtgaagtgaaataagccaggcacagaaagataaatacatgttctcactcctgtgcagaaactaaaaaagttgatcccacagaggtggagagtagaatagtggttactggaggcggacaagggggagggggagggggatagggaaggactggttaaaggatacaagtttacacagccagataggaatagtatgttttagtattctgtagtactgtaggatgactatagttaagaatcacgtatttatgtattttcaggtatttacaagagaggattttgaaagtttccatcacaaagaaatgataaatgtctgaggtgatggttatgcgtattaccctatgccctatagatatgtataattatgtgtcaatttcaaaataaaaattcaaaactacaactcctatgaaaatttttgagcgtgtttgtacttattaagtgtatttataaatcatacggatattatcttcagcctgcatattaaattgtagttaagcttttactttttaactaaaaaataaattctattattttttcctatatcccactgcactgaccccagtttggaaatcctaagattatcaaataaaaactttgattattgaagaatccaggtgtactgccacagaaaagttctattctgtagcatggactctaatatgtaatctagcccattgtgcttacagatagatgtgtgcctgtagtcatagaaaaatttgcatgagctaatgactgccttgctactagattagctcaaagcaaaaagttctctgaaagcaggtcaatagggtcatttttatattatgaagaagaaaagcagctgttgtattacattcactgtattggtcctgcttgtgtttcagggcaagatccttgttgggacaaggaatgctgaaataatcgaagttggagagaaaaatgcagcttgtaatattttagttaacggtcatgtggatgggccaatctggggactagcaacacatccttccagggattttttcctttctgctgcagaagatgggacagtgagactttgggatattgctgataaagtaagtacagataatttttttaaaagaggttacaacttctaaaaagaaaagttggaagttctaaattgctagtacttaaagaactgccagaattctgttgagcattttgaggggaaactggtataatttagaagtacttcacttaatgtttcctatgactctttttttttttttttttaaatgcagaagatgttaaacaaagtgaatttgggacatgctgctcgtactgtgtgttacagccctgaaggggacatggtggctattggaatgaaaaatggagaatttatcattttactagtgagttctctaaaaatatggggaaagaagagagacaggagatgtgcaatccatgatatcaggttagtgaacaaatggaatagagtttctagtatatacttgatttaacttccatttgtaaaattttccatagccttgccttcaaaaagaggtccccagggcctgtagcatttcccgtattataaattgtatgctaaaatatggctgtttgtatactacttaattcttcttgctaaattataaacccactgggcaccaactataatagcaagtactagtaggtaatgtttgatgaattcatgttaacacttagccatgtccattaagttcatcccaccaagaggtatctcccactgtaatacaagagagctatctgcccttcaaaagttgtcaccctggaaaactaaagttgtgatttcaaacatatcttctcttagtaacctcagtttgggaatatgtagttcattaatttaatcaatacctattgattaaatgttccagaatccaaattaatttaaatgtttcttaaacctttgtttttcagtgcttaagcatttttcaacagtggctaccatttacggagtacttccgtgtgatcagtagataagattattgaatctaggtctgtcaaaagcttgtacacttttcatcagtaaaatccttttacaaatgaaaccttcctcagaacttcaatatataaaatagtaacagtggcttcccttagcttttacatgtctctatcgtacctcagtaagactcatgggccatttcaagagactgaattgtcccatatgactccaaagattgctaggcaaatagcatttcactttgtcttttaaataagttcttcaggccgggcgcggtggctcatgcctgtaatcccagcactttgggaggccgaggcaggcagatcacctgaagtcaggagtactcgaccagcctggccaacatagtgaaaccccatctcaactaaaaatacaaaaatcagccgggcgtggtggcaggcgcctgtaatcccagctactcagggggctgaaacaggagaatcgcttgaacccgggaggcggaggttgcgccatcgcactccagcctgggagacaagagcgagacttcgtctcaaaaaaaaaaaattcttcttccaagattcaagttgtgtcatttcaccttaataactggaggttagttaagctgggctgtgttctttgcttaatattaagacaacgttttttccagatggaagaaaactatcttaatgaattgttagcttattaattatgtaatgctaatggcttttaaaagctgagatgttctgactgggtgttgtggctcacacctgtaatcccagtaccttgggaggccaagggggaaggattgcttgaggccaggagtttgggaccatagtgagaccccgcctctatttaaaaaattaaattttgttttgttttgttttgagttggagttttgctcttgttgcccatgctgaagtgcaatggtgcaatctcagctcaccacaacctgtgcctcctgggttcaagcgattctcctgcttcagcctcccgagtagatgggattacaggcgtgcaccaccatgcctggctaattttgtatttttagtagagacagggtttctctatgttggtcaggctggtctcaaactctcgacctcaggtgatctgcccgcctccgcttcccaaagttctgggattataggtgtgagccactgggcctggcctaagaaagtttttttaagccattagacgtttttaaaggaattgggagatgacaattggggaaatatttaaaatttaagtaaaatataaagcttccttatttcatgtaacccagacaatctcagtatacatgatcagttgtgtctgacaggtaaatctatttgaggccttatcacacgttacttttaagaactagaaaggaaaagtcactgatcttaagtatttataatacttcatgtggtctaatactttttacgttttgttttgattcagatttagtccggattcccggtatctggcagtaggttctagtgagaactcagtggatttttatgacctaacgctgggccccactcttaacagaatcagctactgcaaagacattccaagctttgtcattcaaatggacttctctgcagatagcagttatctccaggtacagtaccaatactgtatacccaggtggcaagttcttctgcttttacatttcgtgttagtgaatgcatttaaagttcctgagctccagagctccagcttctcaactcctccctttgtaccttctgacctacagctcccctttcctcccccacttatcagagcttttctcctattaagtttttgtagtgatcttttgcatacttaataatgttagacatgtaaatcaagtagcaatatgctagtattctgtaaaccccctgtggattttgtctctcacctaatggaattcttgtcccattttaatctgatgaaaaaggtctctagtggctgctataaacggcatgtctatgaagtgccttcaggaaaacatcttatggatcatgccgctattgacagaattacttgggctacatggactaggtaaatacttatatattcacaaggcaagaactgactttgaaggccagttagaaaatcctatttctgaactgttagagccattccaataaggaatagtaattgagtttcaagtttttgttaccatattttgaaatggtatgttcatgttgggacccctttttattgaatatatttccatgttttatcagtttccatgatttatcaagttttttttttaaggaaatcaaagttttaactttaaagataccctgatatttttcttaatgctaaatttaatgactggcaaaaaggtattgggtgctgttaagcaactgttattaattctctatctaaaggaatgctatcttgaatctattagaagtcaaagcttccaaatttgttcaaatttcctggctgtatgacaggtaaccatgactatccatttttttggccaatgaaaaatgccatcaaattcctgtatcagccaggcatatagtggctcatgcctgtaatctctgatgtagcaggccgaggtgggaggatcacttgagcctagaagttttgataccagcctgggcaacatagcaagaccccatctctgaaatttttttaattcctatgtcataagtcatttttatttttgtagagatagggatctcacaatattgcccaggctggtctcaaactcttggcctcaagcagtcctcctgcctcagcctcccaaaatgttgggattactggtatgtgctgctggacccagccaagtagcacttttaatttgaaaaatagttctatcagttttcagtcaggcgcggtggctcagcctgtaatcccagcactttgggaggccgagcgggggtgatcacctgaggtcgggagttcgagactagcctgaccaacatggagaaaccctgtctctactaaaaatacaaaataagccgggcatgttagcgcatgcctgtgatcccagctactcgggaggctgaggcaggagaattgcttgaacccaggaggcagaggttgcggtgagccgagatcatgccattgcactccagcctgggtaacaagagcgaaaactccgtctcaaaaaaaaaaaaagaaaaaatagttctatcagttttcataaagtactactttaatcttaaaaagattaatctagaaacccttcaaattataaaatgtcatttttaaaaggcaggagttgatatcctgatgaaattcaggtctccaaacaacttaccataatttacttcctgtattttaagtaacatgatagggtacttagagattaattgccaagaaactttttgaatatagtcaacctgcccgcacttgccatgatgagttttcttttgttccttccctctagtattctaggagatgaggttttgggaatctggtccagacatgctgagaaagctgatgtcaactgtgcctgtgtatctcattcaggaatcagtcttgttacaggagatgactttggcatggttaagttatttgacttcccatgtccagaaaaatttgtaagtttgtgttttgtttactattatcagtttactcctaattttgatgtcttatcatcagcacttttccccatatatttaaaatgttttgtcctaatttctaaatttttccccaaactttctaaatctatttactttgaaataaaagctattagaaacaaatcctctccctcgagtaataccatctttggaaccatcctacaaaagctgtaattagcttttcaccaaacctataatcagttatcaaatttcaaatgcttttccttagagaaaaatggtcagagtacctggagacatctgactgcccacacagcctggttttgcagatccactactcatgctgaaaagcattctaatcactggctgcggtgctaactccctactctctccacagctcttgtcatagagattatagttcctaataagagcctttgacttctgtgtgcaccaaatgccctgagcttgtctgtcattgttttttaggcaaaacacaaaaggttcttgggtcattcgccccatgtgacaaatattcgatttaccagtggtgatcgacatgttgttagtgctggaggtgatgactgcaggttagtaactttctcagcccatgaagagcagactatgttactagttaagagacttaatacaacaactcctacagctttggtttatgaaatcagctagtcaacattagtagaaggtagtataaccagatggctcttcagaatctcatatttatgcaaatacagaataaaaggagttaaagaggaaaaatattacacatgtaacctgaaagcacaactgaaaaatattaaactgttatgaaaatctaaaaacataattaactccctgcaattttcttctctgattgcagcttatttgtctggaaatgtgtacatacacctcactgagagatgctgagatgactacagaaattaactttgagaccagaattacagagaagaaaaaccaaaacccaaccctgcatggtcaagtggtgctaacccaagactgtaacagggagaaatgcccagaatcatcaaaatagtgaaagactgatctgttcaaaatatttgctatatgcactgggtataatccgtaatccatacactgccagataatgccatttcaaggaaggatcgaatacttgatggtaaaggccaagtccccctgtattgggaagtgtgtgatttcggcagacctgctgggaaaatttagggtagagcactctttacagaagaactcaaaaacccaatttggataattttcattatctttttagcaaaatggtttcttaatgtttatattttattttcaaggttcattgtttaatgaaatattttattcttgcatttccataaggaaagggaaagtcatgatcatcctaaaggatcacagtttttaaaaggcaaacattttccctaaggaaacagacacaagctttcctagagaatatgatgttttttaggcattaataaggtccttttttataaaggacacttttctcctagtagttttgaattcaggaacagatccaaagttagcagtatatggctgctacatttccattttcattttcgagccatcagtttatgttcagatgccatctctgtaatcgcacatttaaaacataactgtagcctcactaatggaaaagtagtatgatgaacaatcattcccaatggtgtacaatgtaagggttttagggagcaacagtatttaactggaagaaagaattgcatatttaatgtagtctaatatatacacatttgtttaacatgtaaacaaaagtgttaaattcacatatacaacattatacaatttaatcactcttggaataaaatttttatagccttttttctattgggaaaatttgtttagatgtgtgccactccataggtttatttccaaaatgaatgagcccaactccatttgtaaaaacttgtcagttagaattcctttttttagtggattagggctgaattcttagatccttatttcttttcactttaaatgctgccaaagatcactactcatcattcaggaattcgctgtctagcctatctgtagtttcctgaagattgaaaattatgtagactgctatttaaaaatatatttttctaagtgtgaggtttaagatgctgtattgaccctatgagtttttaatgtgttaattatctttatagcataatagatcgctttaggttcctggaatcccatttggtctgacaggatatatgaagattcttaatacctattttctgtgtctaatacttggttaatactaaaaatagaaatgactaaattacatcacagaaagcataaccagtgattgaacctggtagttttaaagctctaaatagctgtggctgaaggactgattatggggctaagaagcttgaaacgtaagttggtacttgttcatcagtggattctcctaaattaagccaaattttgaaatacatgactattaagtttctactcatgtatttacagtcagtcaataaattaaaggaggaaaaaaatccctgaacaacctgcccataaaaagaaaaatactctacatttgagcctgctgcagttttaaattttccctctgggtcaagtttgccagcttttggctacagagaaattatatttccattacagtgcaggtagaaactctgtaaccttaagcatgtaaactacatagaataaaactgtttccactgcatttctgtccttcaaagtggccaacctgattaagtcagccttaatcactgctgctgtcagtttcacgactaaaggtcatattgactaagtagtcatcagctgaccacctcgctgtatcagccagcaacgaggggaaggtgaagaaacatgataggccatatagaatctgccctatgtttacttttttaacccagataattatttttgtgtgcagtatctaagctcctgattgtgtaacctgggacttctggcaccttttgttccattcattttatgtataaaatgcatgccaaagcacactgtgccctctggtacccttgcttccaatcgccaaccatgctcatttccttcctttttttgtggtccctttttgtggtgatcattttaaaccacgtcatccaacaaatgttttatggtcaaccttagcttgttcataagccatagcaactgaaagattaaactcttaaatatgtgtctgggcagtggctattaaatagcaaaaaacaatcagattttagtattttattatttccttgtaaaatggctgaactaaattaaacccttgtttcccatttgttctataatttatagtgaaactgagaacaaaactatctttataaatgatagctaaaagtatttccagatatttaaacaatttaaaataaatttcttctgcagagatgcaaagcatctcaacactggaatgaacaaatgccttaaattcaatggagtaaacctttagaatgaagaggaactgtcatttcacccaagccgaagacaacagccttatgcacttgtgtgctctgtctttgctgcttctcgtgtttcaagcctttcctgtgggatcagcacagcaaagtgcaacttaccaaatggtttaatgactggttaattctttcttctcccaatggaaaagcaatggcaacacaacagtagactgctggcttgacaatcttaaacgtgagcctttgcacatgtaggtttatcatcatttgagtatacgactaagcaagtcaatgaactttttttttttttttagcagtttaatttggtcctgagaatgttgcagtctttattaccccttttgcattaatccacttttctaaccaccttttaagctttaatttttaacactatacaccaagtctttgaaatcagtgatctgttatttaactctaaagcatttgacacttcttgccttaacagttttaaaaaccacacacaaaaaaactctgtaagtaatacagtaggccaaaagtttcatcctatctatcttgcagtttacctatctgatctgatctctgtaattatagttctgtcatttaaaatatactatttaaatctaatttttacatttcaaaaattatcttcagtagtaactaagtatattttctgtggattctgagaatgttatttttcagaatgtgagaatatatatgtacatttataatcttgtgactttaaagtctgttttcagatacagtatgtaaatacttgtaaaaaaatttgtataattttgtgataatgtagtttcccaaaaaaattatttagaaggcattatgttattagtaaatgagagcactgtatagaactgttcctattttctgcacttgccattccagctgcctccactgtccatacccacctcattcatcctgtcacagaaggcaggaaaactgggaactttaccaaagtagcactcagcctgagaggcctgtataatcatgcttttcaaactaaattcacttaaaaattaaaaagcagaattgaatattttaagcagcctcagtacctttggccaatgctgttttcatggtggattatgaacattatataatctttgggaaaagtgaaagtagtacaatttttagaataatgacaactgcctcactgcatctctccactcacacagcaaccgtgtagccccctaagctgcagtaccatgactaaccatgatgtcaatttcatatgctgatcctcacaacagcagtgcacaaacatgccccaaatattttaacagaatttagctcttccttaagctgtcttttcatagtaaaaacaaaacaaaaacacccaatgttaaaaccacataataaacttacaaacttgaaaaattagacacttcagatagataggcaataaaacttcatattatgaaagcaatatattccaagtttcaaagatttgacaagttctgtagagtatctttcatcagtacatgaaaacttccaaactgcatgatcttctgccaggcaggactgggtgctattcgctggtttgaggtcgaatccatttcaaggcatgtcgtggtgggacattaatggtgggatggtagaatgtgcagtccggtcttgtacattgagtgttaaacctacaatgttttggatgatagaagggacattccatcttcttacaagcagggaagtaacggcagagctgactactggaaggtggtgctggtggtgcaactgctggttttggagacagtactggaattcttctactcacatgagtgaagggacaatctggtttagtacactttgcatcatatttacaatttgggtgaacaaacaaacatttttcagcaaatttacaattggggaaggctttgcagggtgagatggggtgatggtaggcacactcatccccatttttacaagcaggccagtacttgcagcgctccaaaagtttttctggtttctgtgccacactcagttcactcatctcagcatttgggtcctcaagctgcctgctcagcaagtgcaactgctgtgggtggaggagacctctgagtcccttgtttgaggctgcagtttggtttacgggtttcattccttcaaagcacatgtcctcctcttgatctgacatgtatcctggggggctggggacaccatccagcgtcactataaacttgggacttgcaggtttatctggttgtacaagatctcgtgtctgcataaggtgtcctgaaagtacccgaagggaatctgcagtcttcatccccgactcttggtttggtgccactactacttcctcagacagctttggcttcttcagaataaatgatcttgtgtctgcatggaccatggattccatgtcatagtaatcttgatttttttctacagaatctccttttgtttcctcttctttaatggggggacttattctgggggtcctactttgtccctggaccacttctgctagcaattcttcttgagaagttcgagttctgggagcaactggaagtgtctgtttctgtggaactgtagagtagttagttgtttttgttacggattcttgagcttcagatatagccttcaaaatcagattcttgttagcttgtttagaaggtggaagagaaggtctcctttcaggctttgcaggcacagacacactgctggagatgcttcctgttcgagacccgtaatcatcatcttcttcctcctcttctccatcatgattgaatttttttactttaacaactgaacttaccacaggcaactttctcttccgaaagttttcatcctccatactcattttctccgagttgtttctaaagaacggactatacgtttcttctaagctgttaagcacctctggttcacacaaacgtcctgtttcatatacccaactactctgcatatcaagctgcttggcagcatgaatactattctgctgctgttgaaattgcaacctgtttaaatgaacaccactatctgcatttctacttgcaggtggtcgataaatttcaatagaagggcgagaagaaccatatgtaagtgtcactgtaggttttttctgagataagggattctcctgcacaaagttgaggtcttcgtcaatgagatcatctggttctggcttaatatcaatcacatcttcagagggtgctggctccctcaaaggtttcactgttgacattagtcgggttgcagctccatcatcgtaagtctgtctgacatttgtggtttttgactcctgcgaacttgtagaaactctggaatctcttttttcaggtctcgcgctaggaatggcaagtggtggcactgcagcttcatgcctcctctcatctccccgactgaaattgctcttgtttgaaggcacgttactatcaaagatgttggtatcagaagacttcagactagagggttcagttgtaacagagcgaagtttatctaatacaccatgaagccatacggtgaatcgaattgtgttgttccctagaaacagggacagatcctctgtcatttggtcctgacttttcttgttggccaccatcaccataatgtaatcaggaagttcttcatcaacataagctcctaattcttgtaatttccccttaatggcactccggatcttgcggctgatctcggtgccgatctccatggctctgcggcgtgcgggaactcagcactgcgcggcgcttggcttacccggaggctgccgcggactcctaccccgcagccgggacaccaccgcctcc

SEQ ID NO: 17232 - RNA, 14819 nt, Homo sapiens
  source 1..14819: mol_type = other RNA
tcaggccaggcacagtggctcacacctgtaatcttatcactttgggaggctgaggcaggtggatcgcttgagcccaggagttcaagaccagcctgggcaacatggtgaaaccccatcgctataaaaaacaacaattagccgggtgtggtggcacatgcctgtagtccctgctactcaggaggctgaggtgggaggatcacttgagcctggggaggtcaaggctttagtgagctgtgatggtgccactgcactccagcctgggtgacagagtgagaccccatttaaaaaacaaaaacaaaaacaaaaaaaaatgtgacatatagttgactaagaagtacatttcaatacaggattgaaagaacccacatatgttaattaaacacaagcgcagaatttgtgccttttacataaaggaagaatgcacataggcatgctttcagacaagcaattcatctagcagaaaaggaaggaatacatttttcagcccttccaggaataaaatccataaatgggctctatttcgtcctccaacacttgtatttcccacgtcatttactcctgcacacccccactcactagaagcctgctaaactgttccagtgagatattttaacacctgatagggaataaatatgcttctgttttggccttcaaaaataagctctgggccagttgcagtggctcacgcctgtaatcccaacactttgggaggccgaggtgggcggatcacgaggtcaggagtttgggatcagcctggccaatatggtgaaactccatctctactaaaaatacaaaaattagccaggcatggtgcctgtaatcccagctacttgggaggctgaaggagaagaatcgcttgaacctgggaggcacaggttgcagtgagccgagatcacaccactgcactccaggccaggtgacagagcgacactctgtctcaaaaaaataaataaatcaactctgtagcatagcatttgtaattctattattttgccttacatttccattatccttttaataaaattgtttttttacatcttcctaatcaagaagtattatgaggccaggcacagtggctcatacctggaatcccagcactttgggaggccgaggcaggcagatcacctgaggtcaaggtatttgagaccagcctggccaacatggtgaaaccccatctctactaaaaatacagaaattagctgggtgtggtggtgcacacctgtaatgctagctactcgggaggctgaggtaggagaatcgcttgaacctgggaggcagaggttgcaataagcctagatcatgccactgcactcaagcctgggagacagagcgagactacatcttaaaaaaaaaaaaaaaagtattatgagagaggataatgtattgtaatgtattgtagaggctaaataaaattatgctcatgtcagaaaaaaagagtatttctcaaaataaaattcactgaaactggatgtttattttgactgagatatagtatatcctcaaattgccatagaaagtttacaagaatattagaggtaaattataaatatcagggcctttttaaaaaaaaaagattctgcttataacttggtatttgtttataataaaaattatagtagccaataatgaacacttactctggcttggttatttacttaggtcaaaagaaggaggagcggttaaactgtgggatcaggaactgaggcggtgccgtgccttcaggcttgagacaggacaagccacagattgtgttcgttctgtgtgcagaggcaaagtaagatgttccatgagctgatacagtgcagcagaaaacagaaagtggttattactgtgattccctcaccctttgcagcctaatgaacaatacttaataatgcataacgatggatttgcttgccaacattactctgtctttgctgctttctttgccaaagttagcaccagtgtggtgcataagctaggaagctattctgtctaaatactgtatgtaaacctccaatattttctagaatctgccaatttaacaactctagtagacataattgaaagcccttggcagttgactcatattaggacagctgtctccattttttaaaaaaacacacattccctagataaaacgtgcagtaaacaaacaatgaaatactactcagccataaaaaataatgaaattctgtcattcttggtggcaacatggatgagactggaggacatgatgtgaagtgaaataagccaggcacagaaagataaatacatgttctcactcctgtgcagaaactaaaaaagttgatcccacagaggtggagagtagaatagtggttactggaggcggacaagggggagggggagggggatagggaaggactggttaaaggatacaagtttacacagccagataggaatagtatgttttagtattctgtagtactgtaggatgactatagttaagaatcacgtatttatgtattttcaggtatttacaagagaggattttgaaagtttccatcacaaagaaatgataaatgtctgaggtgatggttatgcgtattaccctatgccctatagatatgtataattatgtgtcaatttcaaaataaaaattcaaaactacaactcctatgaaaatttttgagcgtgtttgtacttattaagtgtatttataaatcatacggatattatcttcagcctgcatattaaattgtagttaagcttttactttttaactaaaaaataaattctattattttttcctatatcccactgcactgaccccagtttggaaatcctaagattatcaaataaaaactttgattattgaagaatccaggtgtactgccacagaaaagttctattctgtagcatggactctaatatgtaatctagcccattgtgcttacagatagatgtgtgcctgtagtcatagaaaaatttgcatgagctaatgactgccttgctactagattagctcaaagcaaaaagttctctgaaagcaggtcaatagggtcatttttatattatgaagaagaaaagcagctgttgtattacattcactgtattggtcctgcttgtgtttcagggcaagatccttgttgggacaaggaatgctgaaataatcgaagttggagagaaaaatgcagcttgtaatattttagttaacggtcatgtggatgggccaatctggggactagcaacacatccttccagggattttttcctttctgctgcagaagatgggacagtgagactttgggatattgctgataaagtaagtacagataatttttttaaaagaggttacaacttctaaaaagaaaagttggaagttctaaattgctagtacttaaagaactgccagaattctgttgagcattttgaggggaaactggtataatttagaagtacttcacttaatgtttcctatgactctttttttttttttttttaaatgcagaagatgttaaacaaagtgaatttgggacatgctgctcgtactgtgtgttacagccctgaaggggacatggtggctattggaatgaaaaatggagaatttatcattttactagtgagttctctaaaaatatggggaaagaagagagacaggagatgtgcaatccatgatatcaggttagtgaacaaatggaatagagtttctagtatatacttgatttaacttccatttgtaaaattttccatagccttgccttcaaaaagaggtccccagggcctgtagcatttcccgtattataaattgtatgctaaaatatggctgtttgtatactacttaattcttcttgctaaattataaacccactgggcaccaactataatagcaagtactagtaggtaatgtttgatgaattcatgttaacacttagccatgtccattaagttcatcccaccaagaggtatctcccactgtaatacaagagagctatctgcccttcaaaagttgtcaccctggaaaactaaagttgtgatttcaaacatatcttctcttagtaacctcagtttgggaatatgtagttcattaatttaatcaatacctattgattaaatgttccagaatccaaattaatttaaatgtttcttaaacctttgtttttcagtgcttaagcatttttcaacagtggctaccatttacggagtacttccgtgtgatcagtagataagattattgaatctaggtctgtcaaaagcttgtacacttttcatcagtaaaatccttttacaaatgaaaccttcctcagaacttcaatatataaaatagtaacagtggcttcccttagcttttacatgtctctatcgtacctcagtaagactcatgggccatttcaagagactgaattgtcccatatgactccaaagattgctaggcaaatagcatttcactttgtcttttaaataagttcttcaggccgggcgcggtggctcatgcctgtaatcccagcactttgggaggccgaggcaggcagatcacctgaagtcaggagtactcgaccagcctggccaacatagtgaaaccccatctcaactaaaaatacaaaaatcagccgggcgtggtggcaggcgcctgtaatcccagctactcagggggctgaaacaggagaatcgcttgaacccgggaggcggaggttgcgccatcgcactccagcctgggagacaagagcgagacttcgtctcaaaaaaaaaaaattcttcttccaagattcaagttgtgtcatttcaccttaataactggaggttagttaagctgggctgtgttctttgcttaatattaagacaacgttttttccagatggaagaaaactatcttaatgaattgttagcttattaattatgtaatgctaatggcttttaaaagctgagatgttctgactgggtgttgtggctcacacctgtaatcccagtaccttgggaggccaagggggaaggattgcttgaggccaggagtttgggaccatagtgagaccccgcctctatttaaaaaattaaattttgttttgttttgttttgagttggagttttgctcttgttgcccatgctgaagtgcaatggtgcaatctcagctcaccacaacctgtgcctcctgggttcaagcgattctcctgcttcagcctcccgagtagatgggattacaggcgtgcaccaccatgcctggctaattttgtatttttagtagagacagggtttctctatgttggtcaggctggtctcaaactctcgacctcaggtgatctgcccgcctccgcttcccaaagttctgggattataggtgtgagccactgggcctggcctaagaaagtttttttaagccattagacgtttttaaaggaattgggagatgacaattggggaaatatttaaaatttaagtaaaatataaagcttccttatttcatgtaacccagacaatctcagtatacatgatcagttgtgtctgacaggtaaatctatttgaggccttatcacacgttacttttaagaactagaaaggaaaagtcactgatcttaagtatttataatacttcatgtggtctaatactttttacgttttgttttgattcagatttagtccggattcccggtatctggcagtaggttctagtgagaactcagtggatttttatgacctaacgctgggccccactcttaacagaatcagctactgcaaagacattccaagctttgtcattcaaatggacttctctgcagatagcagttatctccaggtacagtaccaatactgtatacccaggtggcaagttcttctgcttttacatttcgtgttagtgaatgcatttaaagttcctgagctccagagctccagcttctcaactcctccctttgtaccttctgacctacagctcccctttcctcccccacttatcagagcttttctcctattaagtttttgtagtgatcttttgcatacttaataatgttagacatgtaaatcaagtagcaatatgctagtattctgtaaaccccctgtggattttgtctctcacctaatggaattcttgtcccattttaatctgatgaaaaaggtctctagtggctgctataaacggcatgtctatgaagtgccttcaggaaaacatcttatggatcatgccgctattgacagaattacttgggctacatggactaggtaaatacttatatattcacaaggcaagaactgactttgaaggccagttagaaaatcctatttctgaactgttagagccattccaataaggaatagtaattgagtttcaagtttttgttaccatattttgaaatggtatgttcatgttgggacccctttttattgaatatatttccatgttttatcagtttccatgatttatcaagttttttttttaaggaaatcaaagttttaactttaaagataccctgatatttttcttaatgctaaatttaatgactggcaaaaaggtattgggtgctgttaagcaactgttattaattctctatctaaaggaatgctatcttgaatctattagaagtcaaagcttccaaatttgttcaaatttcctggctgtatgacaggtaaccatgactatccatttttttggccaatgaaaaatgccatcaaattcctgtatcagccaggcatatagtggctcatgcctgtaatctctgatgtagcaggccgaggtgggaggatcacttgagcctagaagttttgataccagcctgggcaacatagcaagaccccatctctgaaatttttttaattcctatgtcataagtcatttttatttttgtagagatagggatctcacaatattgcccaggctggtctcaaactcttggcctcaagcagtcctcctgcctcagcctcccaaaatgttgggattactggtatgtgctgctggacccagccaagtagcacttttaatttgaaaaatagttctatcagttttcagtcaggcgcggtggctcagcctgtaatcccagcactttgggaggccgagcgggggtgatcacctgaggtcgggagttcgagactagcctgaccaacatggagaaaccctgtctctactaaaaatacaaaataagccgggcatgttagcgcatgcctgtgatcccagctactcgggaggctgaggcaggagaattgcttgaacccaggaggcagaggttgcggtgagccgagatcatgccattgcactccagcctgggtaacaagagcgaaaactccgtctcaaaaaaaaaaaaagaaaaaatagttctatcagttttcataaagtactactttaatcttaaaaagattaatctagaaacccttcaaattataaaatgtcatttttaaaaggcaggagttgatatcctgatgaaattcaggtctccaaacaacttaccataatttacttcctgtattttaagtaacatgatagggtacttagagattaattgccaagaaactttttgaatatagtcaacctgcccgcacttgccatgatgagttttcttttgttccttccctctagtattctaggagatgaggttttgggaatctggtccagacatgctgagaaagctgatgtcaactgtgcctgtgtatctcattcaggaatcagtcttgttacaggagatgactttggcatggttaagttatttgacttcccatgtccagaaaaatttgtaagtttgtgttttgtttactattatcagtttactcctaattttgatgtcttatcatcagcacttttccccatatatttaaaatgttttgtcctaatttctaaatttttccccaaactttctaaatctatttactttgaaataaaagctattagaaacaaatcctctccctcgagtaataccatctttggaaccatcctacaaaagctgtaattagcttttcaccaaacctataatcagttatcaaatttcaaatgcttttccttagagaaaaatggtcagagtacctggagacatctgactgcccacacagcctggttttgcagatccactactcatgctgaaaagcattctaatcactggctgcggtgctaactccctactctctccacagctcttgtcatagagattatagttcctaataagagcctttgacttctgtgtgcaccaaatgccctgagcttgtctgtcattgttttttaggcaaaacacaaaaggttcttgggtcattcgccccatgtgacaaatattcgatttaccagtggtgatcgacatgttgttagtgctggaggtgatgactgcaggttagtaactttctcagcccatgaagagcagactatgttactagttaagagacttaatacaacaactcctacagctttggtttatgaaatcagctagtcaacattagtagaaggtagtataaccagatggctcttcagaatctcatatttatgcaaatacagaataaaaggagttaaagaggaaaaatattacacatgtaacctgaaagcacaactgaaaaatattaaactgttatgaaaatctaaaaacataattaactccctgcaattttcttctctgattgcagcttatttgtctggaaatgtgtacatacacctcactgagagatgctgagatgactacagaaattaactttgagaccagaattacagagaagaaaaaccaaaacccaaccctgcatggtcaagtggtgctaacccaagactgtaacagggagaaatgcccagaatcatcaaaatagtgaaagactgatctgttcaaaatatttgctatatgcactgggtataatccgtaatccatacactgccagataatgccatttcaaggaaggatcgaatacttgatggtaaaggccaagtccccctgtattgggaagtgtgtgatttcggcagacctgctgggaaaatttagggtagagcactctttacagaagaactcaaaaacccaatttggataattttcattatctttttagcaaaatggtttcttaatgtttatattttattttcaaggttcattgtttaatgaaatattttattcttgcatttccataaggaaagggaaagtcatgatcatcctaaaggatcacagtttttaaaaggcaaacattttccctaaggaaacagacacaagctttcctagagaatatgatgttttttaggcattaataaggtccttttttataaaggacacttttctcctagtagttttgaattcaggaacagatccaaagttagcagtatatggctgctacatttccattttcattttcgagccatcagtttatgttcagatgccatctctgtaatcgcacatttaaaacataactgtagcctcactaatggaaaagtagtatgatgaacaatcattcccaatggtgtacaatgtaagggttttagggagcaacagtatttaactggaagaaagaattgcatatttaatgtagtctaatatatacacatttgtttaacatgtaaacaaaagtgttaaattcacatatacaacattatacaatttaatcactcttggaataaaatttttatagccttttttctattgggaaaatttgtttagatgtgtgccactccataggtttatttccaaaatgaatgagcccaactccatttgtaaaaacttgtcagttagaattcctttttttagtggattagggctgaattcttagatccttatttcttttcactttaaatgctgccaaagatcactactcatcattcaggaattcgctgtctagcctatctgtagtttcctgaagattgaaaattatgtagactgctatttaaaaatatatttttctaagtgtgaggtttaagatgctgtattgaccctatgagtttttaatgtgttaattatctttatagcataatagatcgctttaggttcctggaatcccatttggtctgacaggatatatgaagattcttaatacctattttctgtgtctaatacttggttaatactaaaaatagaaatgactaaattacatcacagaaagcataaccagtgattgaacctggtagttttaaagctctaaatagctgtggctgaaggactgattatggggctaagaagcttgaaacgtaagttggtacttgttcatcagtggattctcctaaattaagccaaattttgaaatacatgactattaagtttctactcatgtatttacagtcagtcaataaattaaaggaggaaaaaaatccctgaacaacctgcccataaaaagaaaaatactctacatttgagcctgctgcagttttaaattttccctctgggtcaagtttgccagcttttggctacagagaaattatatttccattacagtgcaggtagaaactctgtaaccttaagcatgtaaactacatagaataaaactgtttccactgcatttctgtccttcaaagtggccaacctgattaagtcagccttaatcactgctgctgtcagtttcacgactaaaggtcatattgactaagtagtcatcagctgaccacctcgctgtatcagccagcaacgaggggaaggtgaagaaacatgataggccatatagaatctgccctatgtttacttttttaacccagataattatttttgtgtgcagtatctaagctcctgattgtgtaacctgggacttctggcaccttttgttccattcattttatgtataaaatgcatgccaaagcacactgtgccctctggtacccttgcttccaatcgccaaccatgctcatttccttcctttttttgtggtccctttttgtggtgatcattttaaaccacgtcatccaacaaatgttttatggtcaaccttagcttgttcataagccatagcaactgaaagattaaactcttaaatatgtgtctgggcagtggctattaaatagcaaaaaacaatcagattttagtattttattatttccttgtaaaatggctgaactaaattaaacccttgtttcccatttgttctataatttatagtgaaactgagaacaaaactatctttataaatgatagctaaaagtatttccagatatttaaacaatttaaaataaatttcttctgcagagatgcaaagcatctcaacactggaatgaacaaatgccttaaattcaatggagtaaacctttagaatgaagaggaactgtcatttcacccaagccgaagacaacagccttatgcacttgtgtgctctgtctttgctgcttctcgtgtttcaagcctttcctgtgggatcagcacagcaaagtgcaacttaccaaatggtttaatgactggttaattctttcttctcccaatggaaaagcaatggcaacacaacagtagactgctggcttgacaatcttaaacgtgagcctttgcacatgtaggtttatcatcatttgagtatacgactaagcaagtcaatgaactttttttttttttttagcagtttaatttggtcctgagaatgttgcagtctttattaccccttttgcattaatccacttttctaaccaccttttaagctttaatttttaacactatacaccaagtctttgaaatcagtgatctgttatttaactctaaagcatttgacacttcttgccttaacagttttaaaaaccacacacaaaaaaactctgtaagtaatacagtaggccaaaagtttcatcctatctatcttgcagtttacctatctgatctgatctctgtaattatagttctgtcatttaaaatatactatttaaatctaatttttacatttcaaaaattatcttcagtagtaactaagtatattttctgtggattctgagaatgttatttttcagaatgtgagaatatatatgtacatttataatcttgtgactttaaagtctgttttcagatacagtatgtaaatacttgtaaaaaaatttgtataattttgtgataatgtagtttcccaaaaaaattatttagaaggcattatgttattagtaaatgagagcactgtatagaactgttcctattttctgcacttgccattccagctgcctccactgtccatacccacctcattcatcctgtcacagaaggcaggaaaactgggaactttaccaaagtagcactcagcctgagaggcctgtataatcatgcttttcaaactaaattcacttaaaaattaaaaagcagaattgaatattttaagcagcctcagtacctttggccaatgctgttttcatggtggattatgaacattatataatctttgggaaaagtgaaagtagtacaatttttagaataatgacaactgcctcactgcatctctccactcacacagcaaccgtgtagccccctaagctgcagtaccatgactaaccatgatgtcaatttcatatgctgatcctcacaacagcagtgcacaaacatgccccaaatattttaacagaatttagctcttccttaagctgtcttttcatagtaaaaacaaaacaaaaacacccaatgttaaaaccacataataaacttacaaacttgaaaaattagacacttcagatagataggcaataaaacttcatattatgaaagcaatatattccaagtttcaaagatttgacaagttctgtagagtatctttcatcagtacatgaaaacttccaaactgcatgatcttctgccaggcaggactgggtgctattcgctggtttgaggtcgaatccatttcaaggcatgtcgtggtgggacattaatggtgggatggtagaatgtgcagtccggtcttgtacattgagtgttaaacctacaatgttttggatgatagaagggacattccatcttcttacaagcagggaagtaacggcagagctgactactggaaggtggtgctggtggtgcaactgctggttttggagacagtactggaattcttctactcacatgagtgaagggacaatctggtttagtacactttgcatcatatttacaatttgggtgaacaaacaaacatttttcagcaaatttacaattggggaaggctttgcagggtgagatggggtgatggtaggcacactcatccccatttttacaagcaggccagtacttgcagcgctccaaaagtttttctggtttctgtgccacactcagttcactcatctcagcgttagaaaagctaccatttgggtcctcaagctgcctgctcagcaagtgcaactgctgtgggtggaggagacctctgagtcccttgtttgaggctgcagtttggtttacgggtttcattccttcaaagcacatgtcctcctcttgatctgacatgtatcctggggggctggggacaccatccagcgtcactataaacttgggacttgcaggtttatctggttgtacaagatctcgtgtctgcataaggtgtcctgaaagtacccgaagggaatctgcagtcttcatccccgactcttggtttggtgccactactacttcctcagacagctttggcttcttcagaataaatgatcttgtgtctgcatggaccatggattccatgtcatagtaatcttgactcatctgcagagtttctgccattactgggtcgatttgcagtcgggataataattgcctctgttgagttccttgatttttttctacagaatctccttttgtttcctcttctttaatggggggacttattctgggggtcctactttgtccctggaccacttctgctagcaattcttcttgagaagttcgagttctgggagcaactggaagtgtctgtttctgtggaactgtagagtagttagttgtttttgttacggattcttgagcttcagatatagccttcaaaatcagattcttgttagcttgtttagaaggtggaagagaaggtctcctttcaggctttgcaggcacagacacactgctggagatgcttcctgttcgagacccgtaatcatcatcttcttcctcctcttctccatcatgattgaatttttttactttaacaactgaacttaccacaggcaactttctcttccgaaagttttcatcctccatactcattttctccgagttgtttctaaagaacggactatacgtttcttctaagctgttaagcacctctggttcacacaaacgtcctgtttcatatacccaactactctgcatatcaagctgcttggcagcatgaatactattctgctgctgttgaaattgcaacctgtttaaatgaacaccactatctgcatttctacttgcaggtggtcgataaatttcaatagaagggcgagaagaaccatatgtaagtgtcactgtaggttttttctgagataagggattctcctgcacaaagttgaggtcttcgtcaatgagatcatctggttctggcttaatatcaatcacatcttcagagggtgctggctccctcaaaggtttcactgttgacattagtcgggttgcagctccatcatcgtaagtctgtctgacatttgtggtttttgactcctgcgaacttgtagaaactctggaatctcttttttcaggtctcgcgctaggaatggcaagtggtggcactgcagcttcatgcctcctctcatctccccgactgaaattgctcttgtttgaaggcacgttactatcaaagatgttggtatcagaagacttcagactagagggttcagttgtaacagagcgaagtttatctaatacaccatgaagccaacataagctcctaattcttgtaatttccccttaatggcactccggatcttgcggctgatctcggtgccgatctccatggctctgcggcgtgcgggaactcagcactgcgcggcgcttggcttacccggaggctgccgcggactcctaccccgcagccgggacaccaccgcctcc

SEQ ID NO: 17233 - RNA, 14934 nt, Homo sapiens
  source 1..14934: mol_type = other RNA
tcaggccaggcacagtggctcacacctgtaatcttatcactttgggaggctgaggcaggtggatcgcttgagcccaggagttcaagaccagcctgggcaacatggtgaaaccccatcgctataaaaaacaacaattagccgggtgtggtggcacatgcctgtagtccctgctactcaggaggctgaggtgggaggatcacttgagcctggggaggtcaaggctttagtgagctgtgatggtgccactgcactccagcctgggtgacagagtgagaccccatttaaaaaacaaaaacaaaaacaaaaaaaaatgtgacatatagttgactaagaagtacatttcaatacaggattgaaagaacccacatatgttaattaaacacaagcgcagaatttgtgccttttacataaaggaagaatgcacataggcatgctttcagacaagcaattcatctagcagaaaaggaaggaatacatttttcagcccttccaggaataaaatccataaatgggctctatttcgtcctccaacacttgtatttcccacgtcatttactcctgcacacccccactcactagaagcctgctaaactgttccagtgagatattttaacacctgatagggaataaatatgcttctgttttggccttcaaaaataagctctgggccagttgcagtggctcacgcctgtaatcccaacactttgggaggccgaggtgggcggatcacgaggtcaggagtttgggatcagcctggccaatatggtgaaactccatctctactaaaaatacaaaaattagccaggcatggtgcctgtaatcccagctacttgggaggctgaaggagaagaatcgcttgaacctgggaggcacaggttgcagtgagccgagatcacaccactgcactccaggccaggtgacagagcgacactctgtctcaaaaaaataaataaatcaactctgtagcatagcatttgtaattctattattttgccttacatttccattatccttttaataaaattgtttttttacatcttcctaatcaagaagtattatgaggccaggcacagtggctcatacctggaatcccagcactttgggaggccgaggcaggcagatcacctgaggtcaaggtatttgagaccagcctggccaacatggtgaaaccccatctctactaaaaatacagaaattagctgggtgtggtggtgcacacctgtaatgctagctactcgggaggctgaggtaggagaatcgcttgaacctgggaggcagaggttgcaataagcctagatcatgccactgcactcaagcctgggagacagagcgagactacatcttaaaaaaaaaaaaaaaagtattatgagagaggataatgtattgtaatgtattgtagaggctaaataaaattatgctcatgtcagaaaaaaagagtatttctcaaaataaaattcactgaaactggatgtttattttgactgagatatagtatatcctcaaattgccatagaaagtttacaagaatattagaggtaaattataaatatcagggcctttttaaaaaaaaaagattctgcttataacttggtatttgtttataataaaaattatagtagccaataatgaacacttactctggcttggttatttacttaggtcaaaagaaggaggagcggttaaactgtgggatcaggaactgaggcggtgccgtgccttcaggcttgagacaggacaagccacagattgtgttcgttctgtgtgcagaggcaaagtaagatgttccatgagctgatacagtgcagcagaaaacagaaagtggttattactgtgattccctcaccctttgcagcctaatgaacaatacttaataatgcataacgatggatttgcttgccaacattactctgtctttgctgctttctttgccaaagttagcaccagtgtggtgcataagctaggaagctattctgtctaaatactgtatgtaaacctccaatattttctagaatctgccaatttaacaactctagtagacataattgaaagcccttggcagttgactcatattaggacagctgtctccattttttaaaaaaacacacattccctagataaaacgtgcagtaaacaaacaatgaaatactactcagccataaaaaataatgaaattctgtcattcttggtggcaacatggatgagactggaggacatgatgtgaagtgaaataagccaggcacagaaagataaatacatgttctcactcctgtgcagaaactaaaaaagttgatcccacagaggtggagagtagaatagtggttactggaggcggacaagggggagggggagggggatagggaaggactggttaaaggatacaagtttacacagccagataggaatagtatgttttagtattctgtagtactgtaggatgactatagttaagaatcacgtatttatgtattttcaggtatttacaagagaggattttgaaagtttccatcacaaagaaatgataaatgtctgaggtgatggttatgcgtattaccctatgccctatagatatgtataattatgtgtcaatttcaaaataaaaattcaaaactacaactcctatgaaaatttttgagcgtgtttgtacttattaagtgtatttataaatcatacggatattatcttcagcctgcatattaaattgtagttaagcttttactttttaactaaaaaataaattctattattttttcctatatcccactgcactgaccccagtttggaaatcctaagattatcaaataaaaactttgattattgaagaatccaggtgtactgccacagaaaagttctattctgtagcatggactctaatatgtaatctagcccattgtgcttacagatagatgtgtgcctgtagtcatagaaaaatttgcatgagctaatgactgccttgctactagattagctcaaagcaaaaagttctctgaaagcaggtcaatagggtcatttttatattatgaagaagaaaagcagctgttgtattacattcactgtattggtcctgcttgtgtttcagggcaagatccttgttgggacaaggaatgctgaaataatcgaagttggagagaaaaatgcagcttgtaatattttagttaacggtcatgtggatgggccaatctggggactagcaacacatccttccagggattttttcctttctgctgcagaagatgggacagtgagactttgggatattgctgataaagtaagtacagataatttttttaaaagaggttacaacttctaaaaagaaaagttggaagttctaaattgctagtacttaaagaactgccagaattctgttgagcattttgaggggaaactggtataatttagaagtacttcacttaatgtttcctatgactctttttttttttttttttaaatgcagaagatgttaaacaaagtgaatttgggacatgctgctcgtactgtgtgttacagccctgaaggggacatggtggctattggaatgaaaaatggagaatttatcattttactagtgagttctctaaaaatatggggaaagaagagagacaggagatgtgcaatccatgatatcaggttagtgaacaaatggaatagagtttctagtatatacttgatttaacttccatttgtaaaattttccatagccttgccttcaaaaagaggtccccagggcctgtagcatttcccgtattataaattgtatgctaaaatatggctgtttgtatactacttaattcttcttgctaaattataaacccactgggcaccaactataatagcaagtactagtaggtaatgtttgatgaattcatgttaacacttagccatgtccattaagttcatcccaccaagaggtatctcccactgtaatacaagagagctatctgcccttcaaaagttgtcaccctggaaaactaaagttgtgatttcaaacatatcttctcttagtaacctcagtttgggaatatgtagttcattaatttaatcaatacctattgattaaatgttccagaatccaaattaatttaaatgtttcttaaacctttgtttttcagtgcttaagcatttttcaacagtggctaccatttacggagtacttccgtgtgatcagtagataagattattgaatctaggtctgtcaaaagcttgtacacttttcatcagtaaaatccttttacaaatgaaaccttcctcagaacttcaatatataaaatagtaacagtggcttcccttagcttttacatgtctctatcgtacctcagtaagactcatgggccatttcaagagactgaattgtcccatatgactccaaagattgctaggcaaatagcatttcactttgtcttttaaataagttcttcaggccgggcgcggtggctcatgcctgtaatcccagcactttgggaggccgaggcaggcagatcacctgaagtcaggagtactcgaccagcctggccaacatagtgaaaccccatctcaactaaaaatacaaaaatcagccgggcgtggtggcaggcgcctgtaatcccagctactcagggggctgaaacaggagaatcgcttgaacccgggaggcggaggttgcgccatcgcactccagcctgggagacaagagcgagacttcgtctcaaaaaaaaaaaattcttcttccaagattcaagttgtgtcatttcaccttaataactggaggttagttaagctgggctgtgttctttgcttaatattaagacaacgttttttccagatggaagaaaactatcttaatgaattgttagcttattaattatgtaatgctaatggcttttaaaagctgagatgttctgactgggtgttgtggctcacacctgtaatcccagtaccttgggaggccaagggggaaggattgcttgaggccaggagtttgggaccatagtgagaccccgcctctatttaaaaaattaaattttgttttgttttgttttgagttggagttttgctcttgttgcccatgctgaagtgcaatggtgcaatctcagctcaccacaacctgtgcctcctgggttcaagcgattctcctgcttcagcctcccgagtagatgggattacaggcgtgcaccaccatgcctggctaattttgtatttttagtagagacagggtttctctatgttggtcaggctggtctcaaactctcgacctcaggtgatctgcccgcctccgcttcccaaagttctgggattataggtgtgagccactgggcctggcctaagaaagtttttttaagccattagacgtttttaaaggaattgggagatgacaattggggaaatatttaaaatttaagtaaaatataaagcttccttatttcatgtaacccagacaatctcagtatacatgatcagttgtgtctgacaggtaaatctatttgaggccttatcacacgttacttttaagaactagaaaggaaaagtcactgatcttaagtatttataatacttcatgtggtctaatactttttacgttttgttttgattcagatttagtccggattcccggtatctggcagtaggttctagtgagaactcagtggatttttatgacctaacgctgggccccactcttaacagaatcagctactgcaaagacattccaagctttgtcattcaaatggacttctctgcagatagcagttatctccaggtacagtaccaatactgtatacccaggtggcaagttcttctgcttttacatttcgtgttagtgaatgcatttaaagttcctgagctccagagctccagcttctcaactcctccctttgtaccttctgacctacagctcccctttcctcccccacttatcagagcttttctcctattaagtttttgtagtgatcttttgcatacttaataatgttagacatgtaaatcaagtagcaatatgctagtattctgtaaaccccctgtggattttgtctctcacctaatggaattcttgtcccattttaatctgatgaaaaaggtctctagtggctgctataaacggcatgtctatgaagtgccttcaggaaaacatcttatggatcatgccgctattgacagaattacttgggctacatggactaggtaaatacttatatattcacaaggcaagaactgactttgaaggccagttagaaaatcctatttctgaactgttagagccattccaataaggaatagtaattgagtttcaagtttttgttaccatattttgaaatggtatgttcatgttgggacccctttttattgaatatatttccatgttttatcagtttccatgatttatcaagttttttttttaaggaaatcaaagttttaactttaaagataccctgatatttttcttaatgctaaatttaatgactggcaaaaaggtattgggtgctgttaagcaactgttattaattctctatctaaaggaatgctatcttgaatctattagaagtcaaagcttccaaatttgttcaaatttcctggctgtatgacaggtaaccatgactatccatttttttggccaatgaaaaatgccatcaaattcctgtatcagccaggcatatagtggctcatgcctgtaatctctgatgtagcaggccgaggtgggaggatcacttgagcctagaagttttgataccagcctgggcaacatagcaagaccccatctctgaaatttttttaattcctatgtcataagtcatttttatttttgtagagatagggatctcacaatattgcccaggctggtctcaaactcttggcctcaagcagtcctcctgcctcagcctcccaaaatgttgggattactggtatgtgctgctggacccagccaagtagcacttttaatttgaaaaatagttctatcagttttcagtcaggcgcggtggctcagcctgtaatcccagcactttgggaggccgagcgggggtgatcacctgaggtcgggagttcgagactagcctgaccaacatggagaaaccctgtctctactaaaaatacaaaataagccgggcatgttagcgcatgcctgtgatcccagctactcgggaggctgaggcaggagaattgcttgaacccaggaggcagaggttgcggtgagccgagatcatgccattgcactccagcctgggtaacaagagcgaaaactccgtctcaaaaaaaaaaaaagaaaaaatagttctatcagttttcataaagtactactttaatcttaaaaagattaatctagaaacccttcaaattataaaatgtcatttttaaaaggcaggagttgatatcctgatgaaattcaggtctccaaacaacttaccataatttacttcctgtattttaagtaacatgatagggtacttagagattaattgccaagaaactttttgaatatagtcaacctgcccgcacttgccatgatgagttttcttttgttccttccctctagtattctaggagatgaggttttgggaatctggtccagacatgctgagaaagctgatgtcaactgtgcctgtgtatctcattcaggaatcagtcttgttacaggagatgactttggcatggttaagttatttgacttcccatgtccagaaaaatttgtaagtttgtgttttgtttactattatcagtttactcctaattttgatgtcttatcatcagcacttttccccatatatttaaaatgttttgtcctaatttctaaatttttccccaaactttctaaatctatttactttgaaataaaagctattagaaacaaatcctctccctcgagtaataccatctttggaaccatcctacaaaagctgtaattagcttttcaccaaacctataatcagttatcaaatttcaaatgcttttccttagagaaaaatggtcagagtacctggagacatctgactgcccacacagcctggttttgcagatccactactcatgctgaaaagcattctaatcactggctgcggtgctaactccctactctctccacagctcttgtcatagagattatagttcctaataagagcctttgacttctgtgtgcaccaaatgccctgagcttgtctgtcattgttttttaggcaaaacacaaaaggttcttgggtcattcgccccatgtgacaaatattcgatttaccagtggtgatcgacatgttgttagtgctggaggtgatgactgcaggttagtaactttctcagcccatgaagagcagactatgttactagttaagagacttaatacaacaactcctacagctttggtttatgaaatcagctagtcaacattagtagaaggtagtataaccagatggctcttcagaatctcatatttatgcaaatacagaataaaaggagttaaagaggaaaaatattacacatgtaacctgaaagcacaactgaaaaatattaaactgttatgaaaatctaaaaacataattaactccctgcaattttcttctctgattgcagcttatttgtctggaaatgtgtacatacacctcactgagagatgctgagatgactacagaaattaactttgagaccagaattacagagaagaaaaaccaaaacccaaccctgcatggtcaagtggtgctaacccaagactgtaacagggagaaatgcccagaatcatcaaaatagtgaaagactgatctgttcaaaatatttgctatatgcactgggtataatccgtaatccatacactgccagataatgccatttcaaggaaggatcgaatacttgatggtaaaggccaagtccccctgtattgggaagtgtgtgatttcggcagacctgctgggaaaatttagggtagagcactctttacagaagaactcaaaaacccaatttggataattttcattatctttttagcaaaatggtttcttaatgtttatattttattttcaaggttcattgtttaatgaaatattttattcttgcatttccataaggaaagggaaagtcatgatcatcctaaaggatcacagtttttaaaaggcaaacattttccctaaggaaacagacacaagctttcctagagaatatgatgttttttaggcattaataaggtccttttttataaaggacacttttctcctagtagttttgaattcaggaacagatccaaagttagcagtatatggctgctacatttccattttcattttcgagccatcagtttatgttcagatgccatctctgtaatcgcacatttaaaacataactgtagcctcactaatggaaaagtagtatgatgaacaatcattcccaatggtgtacaatgtaagggttttagggagcaacagtatttaactggaagaaagaattgcatatttaatgtagtctaatatatacacatttgtttaacatgtaaacaaaagtgttaaattcacatatacaacattatacaatttaatcactcttggaataaaatttttatagccttttttctattgggaaaatttgtttagatgtgtgccactccataggtttatttccaaaatgaatgagcccaactccatttgtaaaaacttgtcagttagaattcctttttttagtggattagggctgaattcttagatccttatttcttttcactttaaatgctgccaaagatcactactcatcattcaggaattcgctgtctagcctatctgtagtttcctgaagattgaaaattatgtagactgctatttaaaaatatatttttctaagtgtgaggtttaagatgctgtattgaccctatgagtttttaatgtgttaattatctttatagcataatagatcgctttaggttcctggaatcccatttggtctgacaggatatatgaagattcttaatacctattttctgtgtctaatacttggttaatactaaaaatagaaatgactaaattacatcacagaaagcataaccagtgattgaacctggtagttttaaagctctaaatagctgtggctgaaggactgattatggggctaagaagcttgaaacgtaagttggtacttgttcatcagtggattctcctaaattaagccaaattttgaaatacatgactattaagtttctactcatgtatttacagtcagtcaataaattaaaggaggaaaaaaatccctgaacaacctgcccataaaaagaaaaatactctacatttgagcctgctgcagttttaaattttccctctgggtcaagtttgccagcttttggctacagagaaattatatttccattacagtgcaggtagaaactctgtaaccttaagcatgtaaactacatagaataaaactgtttccactgcatttctgtccttcaaagtggccaacctgattaagtcagccttaatcactgctgctgtcagtttcacgactaaaggtcatattgactaagtagtcatcagctgaccacctcgctgtatcagccagcaacgaggggaaggtgaagaaacatgataggccatatagaatctgccctatgtttacttttttaacccagataattatttttgtgtgcagtatctaagctcctgattgtgtaacctgggacttctggcaccttttgttccattcattttatgtataaaatgcatgccaaagcacactgtgccctctggtacccttgcttccaatcgccaaccatgctcatttccttcctttttttgtggtccctttttgtggtgatcattttaaaccacgtcatccaacaaatgttttatggtcaaccttagcttgttcataagccatagcaactgaaagattaaactcttaaatatgtgtctgggcagtggctattaaatagcaaaaaacaatcagattttagtattttattatttccttgtaaaatggctgaactaaattaaacccttgtttcccatttgttctataatttatagtgaaactgagaacaaaactatctttataaatgatagctaaaagtatttccagatatttaaacaatttaaaataaatttcttctgcagagatgcaaagcatctcaacactggaatgaacaaatgccttaaattcaatggagtaaacctttagaatgaagaggaactgtcatttcacccaagccgaagacaacagccttatgcacttgtgtgctctgtctttgctgcttctcgtgtttcaagcctttcctgtgggatcagcacagcaaagtgcaacttaccaaatggtttaatgactggttaattctttcttctcccaatggaaaagcaatggcaacacaacagtagactgctggcttgacaatcttaaacgtgagcctttgcacatgtaggtttatcatcatttgagtatacgactaagcaagtcaatgaactttttttttttttttagcagtttaatttggtcctgagaatgttgcagtctttattaccccttttgcattaatccacttttctaaccaccttttaagctttaatttttaacactatacaccaagtctttgaaatcagtgatctgttatttaactctaaagcatttgacacttcttgccttaacagttttaaaaaccacacacaaaaaaactctgtaagtaatacagtaggccaaaagtttcatcctatctatcttgcagtttacctatctgatctgatctctgtaattatagttctgtcatttaaaatatactatttaaatctaatttttacatttcaaaaattatcttcagtagtaactaagtatattttctgtggattctgagaatgttatttttcagaatgtgagaatatatatgtacatttataatcttgtgactttaaagtctgttttcagatacagtatgtaaatacttgtaaaaaaatttgtataattttgtgataatgtagtttcccaaaaaaattatttagaaggcattatgttattagtaaatgagagcactgtatagaactgttcctattttctgcacttgccattccagctgcctccactgtccatacccacctcattcatcctgtcacagaaggcaggaaaactgggaactttaccaaagtagcactcagcctgagaggcctgtataatcatgcttttcaaactaaattcacttaaaaattaaaaagcagaattgaatattttaagcagcctcagtacctttggccaatgctgttttcatggtggattatgaacattatataatctttgggaaaagtgaaagtagtacaatttttagaataatgacaactgcctcactgcatctctccactcacacagcaaccgtgtagccccctaagctgcagtaccatgactaaccatgatgtcaatttcatatgctgatcctcacaacagcagtgcacaaacatgccccaaatattttaacagaatttagctcttccttaagctgtcttttcatagtaaaaacaaaacaaaaacacccaatgttaaaaccacataataaacttacaaacttgaaaaattagacacttcagatagataggcaataaaacttcatattatgaaagcaatatattccaagtttcaaagatttgacaagttctgtagagtatctttcatcagtacatgaaaacttccaaactgcatgatcttctgccaggcaggactgggtgctattcgctggtttgaggtcgaatccatttcaaggcatgtcgtggtgggacattaatggtgggatggtagaatgtgcagtccggtcttgtacattgagtgttaaacctacaatgttttggatgatagaagggacattccatcttcttacaagcagggaagtaacggcagagctgactactggaaggtggtgctggtggtgcaactgctggttttggagacagtactggaattcttctactcacatgagtgaagggacaatctggtttagtacactttgcatcatatttacaatttgggtgaacaaacaaacatttttcagcaaatttacaattggggaaggctttgcagggtgagatggggtgatggtaggcacactcatccccatttttacaagcaggccagtacttgcagcgctccaaaagtttttctggtttctgtgccacactcagttcactcatctcagcgttagaaaagctaccatttgggtcctcaagctgcctgctcagcaagtgcaactgctgtgggtggaggagacctctgagtcccttgtttgaggctgcagtttggtttacgggtttcattccttcaaagcacatgtcctcctcttgatctgacatgtatcctggggggctggggacaccatccagcgtcactataaacttgggacttgcaggtttatctggttgtacaagatctcgtgtctgcataaggtgtcctgaaagtacccgaagggaatctgcagtcttcatccccgactcttggtttggtgccactactacttcctcagacagctttggcttcttcagaataaatgatcttgtgtctgcatggaccatggattccatgtcatagtaatcttgactcatctgcagagtttctgccattactgggtcgatttgcagtcgggataataattgcctctgttgagttccttgatttttttctacagaatctccttttgtttcctcttctttaatggggggacttattctgggggtcctactttgtccctggaccacttctgctagcaattcttcttgagaagttcgagttctgggagcaactggaagtgtctgtttctgtggaactgtagagtagttagttgtttttgttacggattcttgagcttcagatatagccttcaaaatcagattcttgttagcttgtttagaaggtggaagagaaggtctcctttcaggctttgcaggcacagacacactgctggagatgcttcctgttcgagacccgtaatcatcatcttcttcctcctcttctccatcatgattgaatttttttactttaacaactgaacttaccacaggcaactttctcttccgaaagttttcatcctccatactcattttctccgagttgtttctaaagaacggactatacgtttcttctaagctgttaagcacctctggttcacacaaacgtcctgtttcatatacccaactactctgcatatcaagctgcttggcagcatgaatactattctgctgctgttgaaattgcaacctgtttaaatgaacaccactatctgcatttctacttgcaggtggtcgataaatttcaatagaagggcgagaagaaccatatgtaagtgtcactgtaggttttttctgagataagggattctcctgcacaaagttgaggtcttcgtcaatgagatcatctggttctggcttaatatcaatcacatcttcagagggtgctggctccctcaaaggtttcactgttgacattagtcgggttgcagctccatcatcgtaagtctgtctgacatttgtggtttttgactcctgcgaacttgtagaaactctggaatctcttttttcaggtctcgcgctaggaatggcaagtggtggcactgcagcttcatgcctcctctcatctccccgactgaaattgctcttgtttgaaggcacgttactatcaaagatgttggtatcagaagacttcagactagagggttcagttgtaacagagcgaagtttatctaatacaccatgaagccatacggtgaatcgaattgtgttgttccctagaaacagggacagatcctctgtcatttggtcctgacttttcttgttggccaccatcaccataatgtaatcaggaagttcttcatcaacataagctcctaattcttgtaatttccccttaatggcactccggatcttgcggctgatctcggtgccgatctccatggctctgcggcgtgcgggaactcagcactgcgcggcgcttggcttacccggaggctgccgcggactcctaccccgcagccgggacaccaccgcctcc

SEQ ID NO: 17234 - RNA, 15115 nt, Homo sapiens
  source 1..15115: mol_type = other RNA
tcaggccaggcacagtggctcacacctgtaatcttatcactttgggaggctgaggcaggtggatcgcttgagcccaggagttcaagaccagcctgggcaacatggtgaaaccccatcgctataaaaaacaacaattagccgggtgtggtggcacatgcctgtagtccctgctactcaggaggctgaggtgggaggatcacttgagcctggggaggtcaaggctttagtgagctgtgatggtgccactgcactccagcctgggtgacagagtgagaccccatttaaaaaacaaaaacaaaaacaaaaaaaaatgtgacatatagttgactaagaagtacatttcaatacaggattgaaagaacccacatatgttaattaaacacaagcgcagaatttgtgccttttacataaaggaagaatgcacataggcatgctttcagacaagcaattcatctagcagaaaaggaaggaatacatttttcagcccttccaggaataaaatccataaatgggctctatttcgtcctccaacacttgtatttcccacgtcatttactcctgcacacccccactcactagaagcctgctaaactgttccagtgagatattttaacacctgatagggaataaatatgcttctgttttggccttcaaaaataagctctgggccagttgcagtggctcacgcctgtaatcccaacactttgggaggccgaggtgggcggatcacgaggtcaggagtttgggatcagcctggccaatatggtgaaactccatctctactaaaaatacaaaaattagccaggcatggtgcctgtaatcccagctacttgggaggctgaaggagaagaatcgcttgaacctgggaggcacaggttgcagtgagccgagatcacaccactgcactccaggccaggtgacagagcgacactctgtctcaaaaaaataaataaatcaactctgtagcatagcatttgtaattctattattttgccttacatttccattatccttttaataaaattgtttttttacatcttcctaatcaagaagtattatgaggccaggcacagtggctcatacctggaatcccagcactttgggaggccgaggcaggcagatcacctgaggtcaaggtatttgagaccagcctggccaacatggtgaaaccccatctctactaaaaatacagaaattagctgggtgtggtggtgcacacctgtaatgctagctactcgggaggctgaggtaggagaatcgcttgaacctgggaggcagaggttgcaataagcctagatcatgccactgcactcaagcctgggagacagagcgagactacatcttaaaaaaaaaaaaaaaagtattatgagagaggataatgtattgtaatgtattgtagaggctaaataaaattatgctcatgtcagaaaaaaagagtatttctcaaaataaaattcactgaaactggatgtttattttgactgagatatagtatatcctcaaattgccatagaaagtttacaagaatattagaggtaaattataaatatcagggcctttttaaaaaaaaaagattctgcttataacttggtatttgtttataataaaaattatagtagccaataatgaacacttactctggcttggttatttacttaggtcaaaagaaggaggagcggttaaactgtgggatcaggaactgaggcggtgccgtgccttcaggcttgagacaggacaagccacagattgtgttcgttctgtgtgcagaggcaaagtaagatgttccatgagctgatacagtgcagcagaaaacagaaagtggttattactgtgattccctcaccctttgcagcctaatgaacaatacttaataatgcataacgatggatttgcttgccaacattactctgtctttgctgctttctttgccaaagttagcaccagtgtggtgcataagctaggaagctattctgtctaaatactgtatgtaaacctccaatattttctagaatctgccaatttaacaactctagtagacataattgaaagcccttggcagttgactcatattaggacagctgtctccattttttaaaaaaacacacattccctagataaaacgtgcagtaaacaaacaatgaaatactactcagccataaaaaataatgaaattctgtcattcttggtggcaacatggatgagactggaggacatgatgtgaagtgaaataagccaggcacagaaagataaatacatgttctcactcctgtgcagaaactaaaaaagttgatcccacagaggtggagagtagaatagtggttactggaggcggacaagggggagggggagggggatagggaaggactggttaaaggatacaagtttacacagccagataggaatagtatgttttagtattctgtagtactgtaggatgactatagttaagaatcacgtatttatgtattttcaggtatttacaagagaggattttgaaagtttccatcacaaagaaatgataaatgtctgaggtgatggttatgcgtattaccctatgccctatagatatgtataattatgtgtcaatttcaaaataaaaattcaaaactacaactcctatgaaaatttttgagcgtgtttgtacttattaagtgtatttataaatcatacggatattatcttcagcctgcatattaaattgtagttaagcttttactttttaactaaaaaataaattctattattttttcctatatcccactgcactgaccccagtttggaaatcctaagattatcaaataaaaactttgattattgaagaatccaggtgtactgccacagaaaagttctattctgtagcatggactctaatatgtaatctagcccattgtgcttacagatagatgtgtgcctgtagtcatagaaaaatttgcatgagctaatgactgccttgctactagattagctcaaagcaaaaagttctctgaaagcaggtcaatagggtcatttttatattatgaagaagaaaagcagctgttgtattacattcactgtattggtcctgcttgtgtttcagggcaagatccttgttgggacaaggaatgctgaaataatcgaagttggagagaaaaatgcagcttgtaatattttagttaacggtcatgtggatgggccaatctggggactagcaacacatccttccagggattttttcctttctgctgcagaagatgggacagtgagactttgggatattgctgataaagtaagtacagataatttttttaaaagaggttacaacttctaaaaagaaaagttggaagttctaaattgctagtacttaaagaactgccagaattctgttgagcattttgaggggaaactggtataatttagaagtacttcacttaatgtttcctatgactctttttttttttttttttaaatgcagaagatgttaaacaaagtgaatttgggacatgctgctcgtactgtgtgttacagccctgaaggggacatggtggctattggaatgaaaaatggagaatttatcattttactagtgagttctctaaaaatatggggaaagaagagagacaggagatgtgcaatccatgatatcaggttagtgaacaaatggaatagagtttctagtatatacttgatttaacttccatttgtaaaattttccatagccttgccttcaaaaagaggtccccagggcctgtagcatttcccgtattataaattgtatgctaaaatatggctgtttgtatactacttaattcttcttgctaaattataaacccactgggcaccaactataatagcaagtactagtaggtaatgtttgatgaattcatgttaacacttagccatgtccattaagttcatcccaccaagaggtatctcccactgtaatacaagagagctatctgcccttcaaaagttgtcaccctggaaaactaaagttgtgatttcaaacatatcttctcttagtaacctcagtttgggaatatgtagttcattaatttaatcaatacctattgattaaatgttccagaatccaaattaatttaaatgtttcttaaacctttgtttttcagtgcttaagcatttttcaacagtggctaccatttacggagtacttccgtgtgatcagtagataagattattgaatctaggtctgtcaaaagcttgtacacttttcatcagtaaaatccttttacaaatgaaaccttcctcagaacttcaatatataaaatagtaacagtggcttcccttagcttttacatgtctctatcgtacctcagtaagactcatgggccatttcaagagactgaattgtcccatatgactccaaagattgctaggcaaatagcatttcactttgtcttttaaataagttcttcaggccgggcgcggtggctcatgcctgtaatcccagcactttgggaggccgaggcaggcagatcacctgaagtcaggagtactcgaccagcctggccaacatagtgaaaccccatctcaactaaaaatacaaaaatcagccgggcgtggtggcaggcgcctgtaatcccagctactcagggggctgaaacaggagaatcgcttgaacccgggaggcggaggttgcgccatcgcactccagcctgggagacaagagcgagacttcgtctcaaaaaaaaaaaattcttcttccaagattcaagttgtgtcatttcaccttaataactggaggttagttaagctgggctgtgttctttgcttaatattaagacaacgttttttccagatggaagaaaactatcttaatgaattgttagcttattaattatgtaatgctaatggcttttaaaagctgagatgttctgactgggtgttgtggctcacacctgtaatcccagtaccttgggaggccaagggggaaggattgcttgaggccaggagtttgggaccatagtgagaccccgcctctatttaaaaaattaaattttgttttgttttgttttgagttggagttttgctcttgttgcccatgctgaagtgcaatggtgcaatctcagctcaccacaacctgtgcctcctgggttcaagcgattctcctgcttcagcctcccgagtagatgggattacaggcgtgcaccaccatgcctggctaattttgtatttttagtagagacagggtttctctatgttggtcaggctggtctcaaactctcgacctcaggtgatctgcccgcctccgcttcccaaagttctgggattataggtgtgagccactgggcctggcctaagaaagtttttttaagccattagacgtttttaaaggaattgggagatgacaattggggaaatatttaaaatttaagtaaaatataaagcttccttatttcatgtaacccagacaatctcagtatacatgatcagttgtgtctgacaggtaaatctatttgaggccttatcacacgttacttttaagaactagaaaggaaaagtcactgatcttaagtatttataatacttcatgtggtctaatactttttacgttttgttttgattcagatttagtccggattcccggtatctggcagtaggttctagtgagaactcagtggatttttatgacctaacgctgggccccactcttaacagaatcagctactgcaaagacattccaagctttgtcattcaaatggacttctctgcagatagcagttatctccaggtacagtaccaatactgtatacccaggtggcaagttcttctgcttttacatttcgtgttagtgaatgcatttaaagttcctgagctccagagctccagcttctcaactcctccctttgtaccttctgacctacagctcccctttcctcccccacttatcagagcttttctcctattaagtttttgtagtgatcttttgcatacttaataatgttagacatgtaaatcaagtagcaatatgctagtattctgtaaaccccctgtggattttgtctctcacctaatggaattcttgtcccattttaatctgatgaaaaaggtctctagtggctgctataaacggcatgtctatgaagtgccttcaggaaaacatcttatggatcatgccgctattgacagaattacttgggctacatggactaggtaaatacttatatattcacaaggcaagaactgactttgaaggccagttagaaaatcctatttctgaactgttagagccattccaataaggaatagtaattgagtttcaagtttttgttaccatattttgaaatggtatgttcatgttgggacccctttttattgaatatatttccatgttttatcagtttccatgatttatcaagttttttttttaaggaaatcaaagttttaactttaaagataccctgatatttttcttaatgctaaatttaatgactggcaaaaaggtattgggtgctgttaagcaactgttattaattctctatctaaaggaatgctatcttgaatctattagaagtcaaagcttccaaatttgttcaaatttcctggctgtatgacaggtaaccatgactatccatttttttggccaatgaaaaatgccatcaaattcctgtatcagccaggcatatagtggctcatgcctgtaatctctgatgtagcaggccgaggtgggaggatcacttgagcctagaagttttgataccagcctgggcaacatagcaagaccccatctctgaaatttttttaattcctatgtcataagtcatttttatttttgtagagatagggatctcacaatattgcccaggctggtctcaaactcttggcctcaagcagtcctcctgcctcagcctcccaaaatgttgggattactggtatgtgctgctggacccagccaagtagcacttttaatttgaaaaatagttctatcagttttcagtcaggcgcggtggctcagcctgtaatcccagcactttgggaggccgagcgggggtgatcacctgaggtcgggagttcgagactagcctgaccaacatggagaaaccctgtctctactaaaaatacaaaataagccgggcatgttagcgcatgcctgtgatcccagctactcgggaggctgaggcaggagaattgcttgaacccaggaggcagaggttgcggtgagccgagatcatgccattgcactccagcctgggtaacaagagcgaaaactccgtctcaaaaaaaaaaaaagaaaaaatagttctatcagttttcataaagtactactttaatcttaaaaagattaatctagaaacccttcaaattataaaatgtcatttttaaaaggcaggagttgatatcctgatgaaattcaggtctccaaacaacttaccataatttacttcctgtattttaagtaacatgatagggtacttagagattaattgccaagaaactttttgaatatagtcaacctgcccgcacttgccatgatgagttttcttttgttccttccctctagtattctaggagatgaggttttgggaatctggtccagacatgctgagaaagctgatgtcaactgtgcctgtgtatctcattcaggaatcagtcttgttacaggagatgactttggcatggttaagttatttgacttcccatgtccagaaaaatttgtaagtttgtgttttgtttactattatcagtttactcctaattttgatgtcttatcatcagcacttttccccatatatttaaaatgttttgtcctaatttctaaatttttccccaaactttctaaatctatttactttgaaataaaagctattagaaacaaatcctctccctcgagtaataccatctttggaaccatcctacaaaagctgtaattagcttttcaccaaacctataatcagttatcaaatttcaaatgcttttccttagagaaaaatggtcagagtacctggagacatctgactgcccacacagcctggttttgcagatccactactcatgctgaaaagcattctaatcactggctgcggtgctaactccctactctctccacagctcttgtcatagagattatagttcctaataagagcctttgacttctgtgtgcaccaaatgccctgagcttgtctgtcattgttttttaggcaaaacacaaaaggttcttgggtcattcgccccatgtgacaaatattcgatttaccagtggtgatcgacatgttgttagtgctggaggtgatgactgcaggttagtaactttctcagcccatgaagagcagactatgttactagttaagagacttaatacaacaactcctacagctttggtttatgaaatcagctagtcaacattagtagaaggtagtataaccagatggctcttcagaatctcatatttatgcaaatacagaataaaaggagttaaagaggaaaaatattacacatgtaacctgaaagcacaactgaaaaatattaaactgttatgaaaatctaaaaacataattaactccctgcaattttcttctctgattgcagcttatttgtctggaaatgtgtacatacacctcactgagagatgctgagatgactacagaaattaactttgagaccagaattacagagaagaaaaaccaaaacccaaccctgcatggtcaagtggtgctaacccaagactgtaacagggagaaatgcccagaatcatcaaaatagtgaaagactgatctgttcaaaatatttgctatatgcactgggtataatccgtaatccatacactgccagataatgccatttcaaggaaggatcgaatacttgatggtaaaggccaagtccccctgtattgggaagtgtgtgatttcggcagacctgctgggaaaatttagggtagagcactctttacagaagaactcaaaaacccaatttggataattttcattatctttttagcaaaatggtttcttaatgtttatattttattttcaaggttcattgtttaatgaaatattttattcttgcatttccataaggaaagggaaagtcatgatcatcctaaaggatcacagtttttaaaaggcaaacattttccctaaggaaacagacacaagctttcctagagaatatgatgttttttaggcattaataaggtccttttttataaaggacacttttctcctagtagttttgaattcaggaacagatccaaagttagcagtatatggctgctacatttccattttcattttcgagccatcagtttatgttcagatgccatctctgtaatcgcacatttaaaacataactgtagcctcactaatggaaaagtagtatgatgaacaatcattcccaatggtgtacaatgtaagggttttagggagcaacagtatttaactggaagaaagaattgcatatttaatgtagtctaatatatacacatttgtttaacatgtaaacaaaagtgttaaattcacatatacaacattatacaatttaatcactcttggaataaaatttttatagccttttttctattgggaaaatttgtttagatgtgtgccactccataggtttatttccaaaatgaatgagcccaactccatttgtaaaaacttgtcagttagaattcctttttttagtggattagggctgaattcttagatccttatttcttttcactttaaatgctgccaaagatcactactcatcattcaggaattcgctgtctagcctatctgtagtttcctgaagattgaaaattatgtagactgctatttaaaaatatatttttctaagtgtgaggtttaagatgctgtattgaccctatgagtttttaatgtgttaattatctttatagcataatagatcgctttaggttcctggaatcccatttggtctgacaggatatatgaagattcttaatacctattttctgtgtctaatacttggttaatactaaaaatagaaatgactaaattacatcacagaaagcataaccagtgattgaacctggtagttttaaagctctaaatagctgtggctgaaggactgattatggggctaagaagcttgaaacgtaagttggtacttgttcatcagtggattctcctaaattaagccaaattttgaaatacatgactattaagtttctactcatgtatttacagtcagtcaataaattaaaggaggaaaaaaatccctgaacaacctgcccataaaaagaaaaatactctacatttgagcctgctgcagttttaaattttccctctgggtcaagtttgccagcttttggctacagagaaattatatttccattacagtgcaggtagaaactctgtaaccttaagcatgtaaactacatagaataaaactgtttccactgcatttctgtccttcaaagtggccaacctgattaagtcagccttaatcactgctgctgtcagtttcacgactaaaggtcatattgactaagtagtcatcagctgaccacctcgctgtatcagccagcaacgaggggaaggtgaagaaacatgataggccatatagaatctgccctatgtttacttttttaacccagataattatttttgtgtgcagtatctaagctcctgattgtgtaacctgggacttctggcaccttttgttccattcattttatgtataaaatgcatgccaaagcacactgtgccctctggtacccttgcttccaatcgccaaccatgctcatttccttcctttttttgtggtccctttttgtggtgatcattttaaaccacgtcatccaacaaatgttttatggtcaaccttagcttgttcataagccatagcaactgaaagattaaactcttaaatatgtgtctgggcagtggctattaaatagcaaaaaacaatcagattttagtattttattatttccttgtaaaatggctgaactaaattaaacccttgtttcccatttgttctataatttatagtgaaactgagaacaaaactatctttataaatgatagctaaaagtatttccagatatttaaacaatttaaaataaatttcttctgcagagatgcaaagcatctcaacactggaatgaacaaatgccttaaattcaatggagtaaacctttagaatgaagaggaactgtcatttcacccaagccgaagacaacagccttatgcacttgtgtgctctgtctttgctgcttctcgtgtttcaagcctttcctgtgggatcagcacagcaaagtgcaacttaccaaatggtttaatgactggttaattctttcttctcccaatggaaaagcaatggcaacacaacagtagactgctggcttgacaatcttaaacgtgagcctttgcacatgtaggtttatcatcatttgagtatacgactaagcaagtcaatgaactttttttttttttttagcagtttaatttggtcctgagaatgttgcagtctttattaccccttttgcattaatccacttttctaaccaccttttaagctttaatttttaacactatacaccaagtctttgaaatcagtgatctgttatttaactctaaagcatttgacacttcttgccttaacagttttaaaaaccacacacaaaaaaactctgtaagtaatacagtaggccaaaagtttcatcctatctatcttgcagtttacctatctgatctgatctctgtaattatagttctgtcatttaaaatatactatttaaatctaatttttacatttcaaaaattatcttcagtagtaactaagtatattttctgtggattctgagaatgttatttttcagaatgtgagaatatatatgtacatttataatcttgtgactttaaagtctgttttcagatacagtatgtaaatacttgtaaaaaaatttgtataattttgtgataatgtagtttcccaaaaaaattatttagaaggcattatgttattagtaaatgagagcactgtatagaactgttcctattttctgcacttgccattccagctgcctccactgtccatacccacctcattcatcctgtcacagaaggcaggaaaactgggaactttaccaaagtagcactcagcctgagaggcctgtataatcatgcttttcaaactaaattcacttaaaaattaaaaagcagaattgaatattttaagcagcctcagtacctttggccaatgctgttttcatggtggattatgaacattatataatctttgggaaaagtgaaagtagtacaatttttagaataatgacaactgcctcactgcatctctccactcacacagcaaccgtgtagccccctaagctgcagtaccatgactaaccatgatgtcaatttcatatgctgatcctcacaacagcagtgcacaaacatgccccaaatattttaacagaatttagctcttccttaagctgtcttttcatagtaaaaacaaaacaaaaacacccaatgttaaaaccacataataaacttacaaacttgaaaaattagacacttcagatagataggcaataaaacttcatattatgaaagcaatatattccaagtttcaaagatttgacaagttctgtagagtatctttcatcagtacatgaaaacttccaaactgcatgatcttctgccaggcaggactgggtgctattcgctggtttgaggtcgaatccatttcaaggcatgtcgtggtgggacattaatggtgggatggtagaatgtgcagtccggtcttgtacattgagtgttaaacctacaatgttttggatgatagaagggacattccatcttcttacaagcagggaagtaacggcagagctgactactggaaggtggtgctggtggtgcaactgctggttttggagacagtactggaattcttctactcacatgagtgaagggacaatctggtttagtacactttgcatcatatttacaatttgggtgaacaaacaaacatttttcagcaaatttacaattggggaaggctttgcagggtgagatggggtgatggtaggcacactcatccccatttttacaagcaggccagtacttgcagcgctccaaaagtttttctggtttctgtgccacactcagttcactcatctcagcgttagaaaagctaccatttgggtcctcaagctgcctgctcagcaagtgcaactgctgtgggtggaggagacctctgagtcccttgtttgaggctgcagtttggtttacgggtttcattccttcaaagcacatgtcctcctcttgatctgacatgtatcctggggggctggggacaccatccagcgtcactataaacttgggacttgcaggtttatctggttgtacaagatctcgtgtctgcataaggtgtcctgaaagtacccgaagggaatctgcagtcttcatccccgactcttggtttggtgccactactacttcctcagacagctttggcttcttcagaataaatgatcttgtgtctgcatggaccatggattccatgtcatagtaatcttgactcatctgcagagtttctgccattactgggtcgatttgcagtcgggataataattgcctctgttgagttccttgatttttttctacagaatctccttttgtttcctcttctttaatggggggacttattctgggggtcctactttgtccctggaccacttctgctagcaattcttcttgagaagttcgagttctgggagcaactggaagtgtctgtttctgtggaactgtagagtagttagttgtttttgttacggattcttgagcttcagatatagccttcaaaatcagattcttgttagcttgtttagaaggtggaagagaaggtctcctttcaggctttgcaggcacagacacactgctggagatgcttcctgttcgagacccgtaatcatcatcttcttcctcctcttctccatcatgattgaatttttttactttaacaactgaacttaccacaggcaactttctcttccgaaagttttcatcctccatactcattttctccgagttgtttctaaagaacggactatacgtttcttctaagctgttaagcacctctggttcacacaaacgtcctgtttcatatacccaactactctgcatatcaagctgcttggcagcatgaatactattctgctgctgttgaaattgcaacctgtttaaatgaacaccactatctgcatttctacttgcaggtggtcgataaatttcaatagaagggcgagaagaaccatatgtaagtgtcactgtaggttttttctgagataagggattctcctgcacaaagttgaggtcttcgtcaatgagatcatctggttctggcttaatatcaatcacatcttcagagggtgctggctccctcaaaggtttcactgttgacattagtcgggttgcagctccatcatcgtaagtctgtctgacatttgtggtttttgactcctgcgaacttgtagaaactctggaatctcttttttcaggtctcgcgctaggaatggcaagtggtggcactgcagcttcatgcctcctctcatctccccgactgaaattgctcttgtttgaaggcacgttactatcaaagatgttggtatcagaagacttcagactagagggttcagttgtaacagagcgaagtttatctaatacaccatgaagccatacggtgaatcgaattgtgttgttccctagaaacagggacagatcctctgtcatttggtcctgacttttcttgttggccaccatcaccataatgtaatcaggaagttcttcatctatttaaaaggaaaggtagatcaaaactttgtttcctcaaaactttcttcttaaagttgatgtgcttgaaaatatagatgtagctctaagctttagagtcgcagagctctactggaattacattggacaagatggcttagctttaatttttttctcttcattccacaggtatttcaaatacaacataagctcctaattcttgtaatttccccttaatggcactccggatcttgcggctgatctcggtgccgatctccatggctctgcggcgtgcgggaactcagcactgcgcggcgcttggcttacccggaggctgccgcggactcctaccccgcagccgggacaccaccgcctcc

SEQ ID NO: 17235 - RNA, 14744 nt, Homo sapiens
  source 1..14744: mol_type = other RNA
tcaggccaggcacagtggctcacacctgtaatcttatcactttgggaggctgaggcaggtggatcgcttgagcccaggagttcaagaccagcctgggcaacatggtgaaaccccatcgctataaaaaacaacaattagccgggtgtggtggcacatgcctgtagtccctgctactcaggaggctgaggtgggaggatcacttgagcctggggaggtcaaggctttagtgagctgtgatggtgccactgcactccagcctgggtgacagagtgagaccccatttaaaaaacaaaaacaaaaacaaaaaaaaatgtgacatatagttgactaagaagtacatttcaatacaggattgaaagaacccacatatgttaattaaacacaagcgcagaatttgtgccttttacataaaggaagaatgcacataggcatgctttcagacaagcaattcatctagcagaaaaggaaggaatacatttttcagcccttccaggaataaaatccataaatgggctctatttcgtcctccaacacttgtatttcccacgtcatttactcctgcacacccccactcactagaagcctgctaaactgttccagtgagatattttaacacctgatagggaataaatatgcttctgttttggccttcaaaaataagctctgggccagttgcagtggctcacgcctgtaatcccaacactttgggaggccgaggtgggcggatcacgaggtcaggagtttgggatcagcctggccaatatggtgaaactccatctctactaaaaatacaaaaattagccaggcatggtgcctgtaatcccagctacttgggaggctgaaggagaagaatcgcttgaacctgggaggcacaggttgcagtgagccgagatcacaccactgcactccaggccaggtgacagagcgacactctgtctcaaaaaaataaataaatcaactctgtagcatagcatttgtaattctattattttgccttacatttccattatccttttaataaaattgtttttttacatcttcctaatcaagaagtattatgaggccaggcacagtggctcatacctggaatcccagcactttgggaggccgaggcaggcagatcacctgaggtcaaggtatttgagaccagcctggccaacatggtgaaaccccatctctactaaaaatacagaaattagctgggtgtggtggtgcacacctgtaatgctagctactcgggaggctgaggtaggagaatcgcttgaacctgggaggcagaggttgcaataagcctagatcatgccactgcactcaagcctgggagacagagcgagactacatcttaaaaaaaaaaaaaaaagtattatgagagaggataatgtattgtaatgtattgtagaggctaaataaaattatgctcatgtcagaaaaaaagagtatttctcaaaataaaattcactgaaactggatgtttattttgactgagatatagtatatcctcaaattgccatagaaagtttacaagaatattagaggtaaattataaatatcagggcctttttaaaaaaaaaagattctgcttataacttggtatttgtttataataaaaattatagtagccaataatgaacacttactctggcttggttatttacttaggtcaaaagaaggaggagcggttaaactgtgggatcaggaactgaggcggtgccgtgccttcaggcttgagacaggacaagccacagattgtgttcgttctgtgtgcagaggcaaagtaagatgttccatgagctgatacagtgcagcagaaaacagaaagtggttattactgtgattccctcaccctttgcagcctaatgaacaatacttaataatgcataacgatggatttgcttgccaacattactctgtctttgctgctttctttgccaaagttagcaccagtgtggtgcataagctaggaagctattctgtctaaatactgtatgtaaacctccaatattttctagaatctgccaatttaacaactctagtagacataattgaaagcccttggcagttgactcatattaggacagctgtctccattttttaaaaaaacacacattccctagataaaacgtgcagtaaacaaacaatgaaatactactcagccataaaaaataatgaaattctgtcattcttggtggcaacatggatgagactggaggacatgatgtgaagtgaaataagccaggcacagaaagataaatacatgttctcactcctgtgcagaaactaaaaaagttgatcccacagaggtggagagtagaatagtggttactggaggcggacaagggggagggggagggggatagggaaggactggttaaaggatacaagtttacacagccagataggaatagtatgttttagtattctgtagtactgtaggatgactatagttaagaatcacgtatttatgtattttcaggtatttacaagagaggattttgaaagtttccatcacaaagaaatgataaatgtctgaggtgatggttatgcgtattaccctatgccctatagatatgtataattatgtgtcaatttcaaaataaaaattcaaaactacaactcctatgaaaatttttgagcgtgtttgtacttattaagtgtatttataaatcatacggatattatcttcagcctgcatattaaattgtagttaagcttttactttttaactaaaaaataaattctattattttttcctatatcccactgcactgaccccagtttggaaatcctaagattatcaaataaaaactttgattattgaagaatccaggtgtactgccacagaaaagttctattctgtagcatggactctaatatgtaatctagcccattgtgcttacagatagatgtgtgcctgtagtcatagaaaaatttgcatgagctaatgactgccttgctactagattagctcaaagcaaaaagttctctgaaagcaggtcaatagggtcatttttatattatgaagaagaaaagcagctgttgtattacattcactgtattggtcctgcttgtgtttcagggcaagatccttgttgggacaaggaatgctgaaataatcgaagttggagagaaaaatgcagcttgtaatattttagttaacggtcatgtggatgggccaatctggggactagcaacacatccttccagggattttttcctttctgctgcagaagatgggacagtgagactttgggatattgctgataaagtaagtacagataatttttttaaaagaggttacaacttctaaaaagaaaagttggaagttctaaattgctagtacttaaagaactgccagaattctgttgagcattttgaggggaaactggtataatttagaagtacttcacttaatgtttcctatgactctttttttttttttttttaaatgcagaagatgttaaacaaagtgaatttgggacatgctgctcgtactgtgtgttacagccctgaaggggacatggtggctattggaatgaaaaatggagaatttatcattttactagtgagttctctaaaaatatggggaaagaagagagacaggagatgtgcaatccatgatatcaggttagtgaacaaatggaatagagtttctagtatatacttgatttaacttccatttgtaaaattttccatagccttgccttcaaaaagaggtccccagggcctgtagcatttcccgtattataaattgtatgctaaaatatggctgtttgtatactacttaattcttcttgctaaattataaacccactgggcaccaactataatagcaagtactagtaggtaatgtttgatgaattcatgttaacacttagccatgtccattaagttcatcccaccaagaggtatctcccactgtaatacaagagagctatctgcccttcaaaagttgtcaccctggaaaactaaagttgtgatttcaaacatatcttctcttagtaacctcagtttgggaatatgtagttcattaatttaatcaatacctattgattaaatgttccagaatccaaattaatttaaatgtttcttaaacctttgtttttcagtgcttaagcatttttcaacagtggctaccatttacggagtacttccgtgtgatcagtagataagattattgaatctaggtctgtcaaaagcttgtacacttttcatcagtaaaatccttttacaaatgaaaccttcctcagaacttcaatatataaaatagtaacagtggcttcccttagcttttacatgtctctatcgtacctcagtaagactcatgggccatttcaagagactgaattgtcccatatgactccaaagattgctaggcaaatagcatttcactttgtcttttaaataagttcttcaggccgggcgcggtggctcatgcctgtaatcccagcactttgggaggccgaggcaggcagatcacctgaagtcaggagtactcgaccagcctggccaacatagtgaaaccccatctcaactaaaaatacaaaaatcagccgggcgtggtggcaggcgcctgtaatcccagctactcagggggctgaaacaggagaatcgcttgaacccgggaggcggaggttgcgccatcgcactccagcctgggagacaagagcgagacttcgtctcaaaaaaaaaaaattcttcttccaagattcaagttgtgtcatttcaccttaataactggaggttagttaagctgggctgtgttctttgcttaatattaagacaacgttttttccagatggaagaaaactatcttaatgaattgttagcttattaattatgtaatgctaatggcttttaaaagctgagatgttctgactgggtgttgtggctcacacctgtaatcccagtaccttgggaggccaagggggaaggattgcttgaggccaggagtttgggaccatagtgagaccccgcctctatttaaaaaattaaattttgttttgttttgttttgagttggagttttgctcttgttgcccatgctgaagtgcaatggtgcaatctcagctcaccacaacctgtgcctcctgggttcaagcgattctcctgcttcagcctcccgagtagatgggattacaggcgtgcaccaccatgcctggctaattttgtatttttagtagagacagggtttctctatgttggtcaggctggtctcaaactctcgacctcaggtgatctgcccgcctccgcttcccaaagttctgggattataggtgtgagccactgggcctggcctaagaaagtttttttaagccattagacgtttttaaaggaattgggagatgacaattggggaaatatttaaaatttaagtaaaatataaagcttccttatttcatgtaacccagacaatctcagtatacatgatcagttgtgtctgacaggtaaatctatttgaggccttatcacacgttacttttaagaactagaaaggaaaagtcactgatcttaagtatttataatacttcatgtggtctaatactttttacgttttgttttgattcagatttagtccggattcccggtatctggcagtaggttctagtgagaactcagtggatttttatgacctaacgctgggccccactcttaacagaatcagctactgcaaagacattccaagctttgtcattcaaatggacttctctgcagatagcagttatctccaggtacagtaccaatactgtatacccaggtggcaagttcttctgcttttacatttcgtgttagtgaatgcatttaaagttcctgagctccagagctccagcttctcaactcctccctttgtaccttctgacctacagctcccctttcctcccccacttatcagagcttttctcctattaagtttttgtagtgatcttttgcatacttaataatgttagacatgtaaatcaagtagcaatatgctagtattctgtaaaccccctgtggattttgtctctcacctaatggaattcttgtcccattttaatctgatgaaaaaggtctctagtggctgctataaacggcatgtctatgaagtgccttcaggaaaacatcttatggatcatgccgctattgacagaattacttgggctacatggactaggtaaatacttatatattcacaaggcaagaactgactttgaaggccagttagaaaatcctatttctgaactgttagagccattccaataaggaatagtaattgagtttcaagtttttgttaccatattttgaaatggtatgttcatgttgggacccctttttattgaatatatttccatgttttatcagtttccatgatttatcaagttttttttttaaggaaatcaaagttttaactttaaagataccctgatatttttcttaatgctaaatttaatgactggcaaaaaggtattgggtgctgttaagcaactgttattaattctctatctaaaggaatgctatcttgaatctattagaagtcaaagcttccaaatttgttcaaatttcctggctgtatgacaggtaaccatgactatccatttttttggccaatgaaaaatgccatcaaattcctgtatcagccaggcatatagtggctcatgcctgtaatctctgatgtagcaggccgaggtgggaggatcacttgagcctagaagttttgataccagcctgggcaacatagcaagaccccatctctgaaatttttttaattcctatgtcataagtcatttttatttttgtagagatagggatctcacaatattgcccaggctggtctcaaactcttggcctcaagcagtcctcctgcctcagcctcccaaaatgttgggattactggtatgtgctgctggacccagccaagtagcacttttaatttgaaaaatagttctatcagttttcagtcaggcgcggtggctcagcctgtaatcccagcactttgggaggccgagcgggggtgatcacctgaggtcgggagttcgagactagcctgaccaacatggagaaaccctgtctctactaaaaatacaaaataagccgggcatgttagcgcatgcctgtgatcccagctactcgggaggctgaggcaggagaattgcttgaacccaggaggcagaggttgcggtgagccgagatcatgccattgcactccagcctgggtaacaagagcgaaaactccgtctcaaaaaaaaaaaaagaaaaaatagttctatcagttttcataaagtactactttaatcttaaaaagattaatctagaaacccttcaaattataaaatgtcatttttaaaaggcaggagttgatatcctgatgaaattcaggtctccaaacaacttaccataatttacttcctgtattttaagtaacatgatagggtacttagagattaattgccaagaaactttttgaatatagtcaacctgcccgcacttgccatgatgagttttcttttgttccttccctctagtattctaggagatgaggttttgggaatctggtccagacatgctgagaaagctgatgtcaactgtgcctgtgtatctcattcaggaatcagtcttgttacaggagatgactttggcatggttaagttatttgacttcccatgtccagaaaaatttgtaagtttgtgttttgtttactattatcagtttactcctaattttgatgtcttatcatcagcacttttccccatatatttaaaatgttttgtcctaatttctaaatttttccccaaactttctaaatctatttactttgaaataaaagctattagaaacaaatcctctccctcgagtaataccatctttggaaccatcctacaaaagctgtaattagcttttcaccaaacctataatcagttatcaaatttcaaatgcttttccttagagaaaaatggtcagagtacctggagacatctgactgcccacacagcctggttttgcagatccactactcatgctgaaaagcattctaatcactggctgcggtgctaactccctactctctccacagctcttgtcatagagattatagttcctaataagagcctttgacttctgtgtgcaccaaatgccctgagcttgtctgtcattgttttttaggcaaaacacaaaaggttcttgggtcattcgccccatgtgacaaatattcgatttaccagtggtgatcgacatgttgttagtgctggaggtgatgactgcaggttagtaactttctcagcccatgaagagcagactatgttactagttaagagacttaatacaacaactcctacagctttggtttatgaaatcagctagtcaacattagtagaaggtagtataaccagatggctcttcagaatctcatatttatgcaaatacagaataaaaggagttaaagaggaaaaatattacacatgtaacctgaaagcacaactgaaaaatattaaactgttatgaaaatctaaaaacataattaactccctgcaattttcttctctgattgcagcttatttgtctggaaatgtgtacatacacctcactgagagatgctgagatgactacagaaattaactttgagaccagaattacagagaagaaaaaccaaaacccaaccctgcatggtcaagtggtgctaacccaagactgtaacagggagaaatgcccagaatcatcaaaatagtgaaagactgatctgttcaaaatatttgctatatgcactgggtataatccgtaatccatacactgccagataatgccatttcaaggaaggatcgaatacttgatggtaaaggccaagtccccctgtattgggaagtgtgtgatttcggcagacctgctgggaaaatttagggtagagcactctttacagaagaactcaaaaacccaatttggataattttcattatctttttagcaaaatggtttcttaatgtttatattttattttcaaggttcattgtttaatgaaatattttattcttgcatttccataaggaaagggaaagtcatgatcatcctaaaggatcacagtttttaaaaggcaaacattttccctaaggaaacagacacaagctttcctagagaatatgatgttttttaggcattaataaggtccttttttataaaggacacttttctcctagtagttttgaattcaggaacagatccaaagttagcagtatatggctgctacatttccattttcattttcgagccatcagtttatgttcagatgccatctctgtaatcgcacatttaaaacataactgtagcctcactaatggaaaagtagtatgatgaacaatcattcccaatggtgtacaatgtaagggttttagggagcaacagtatttaactggaagaaagaattgcatatttaatgtagtctaatatatacacatttgtttaacatgtaaacaaaagtgttaaattcacatatacaacattatacaatttaatcactcttggaataaaatttttatagccttttttctattgggaaaatttgtttagatgtgtgccactccataggtttatttccaaaatgaatgagcccaactccatttgtaaaaacttgtcagttagaattcctttttttagtggattagggctgaattcttagatccttatttcttttcactttaaatgctgccaaagatcactactcatcattcaggaattcgctgtctagcctatctgtagtttcctgaagattgaaaattatgtagactgctatttaaaaatatatttttctaagtgtgaggtttaagatgctgtattgaccctatgagtttttaatgtgttaattatctttatagcataatagatcgctttaggttcctggaatcccatttggtctgacaggatatatgaagattcttaatacctattttctgtgtctaatacttggttaatactaaaaatagaaatgactaaattacatcacagaaagcataaccagtgattgaacctggtagttttaaagctctaaatagctgtggctgaaggactgattatggggctaagaagcttgaaacgtaagttggtacttgttcatcagtggattctcctaaattaagccaaattttgaaatacatgactattaagtttctactcatgtatttacagtcagtcaataaattaaaggaggaaaaaaatccctgaacaacctgcccataaaaagaaaaatactctacatttgagcctgctgcagttttaaattttccctctgggtcaagtttgccagcttttggctacagagaaattatatttccattacagtgcaggtagaaactctgtaaccttaagcatgtaaactacatagaataaaactgtttccactgcatttctgtccttcaaagtggccaacctgattaagtcagccttaatcactgctgctgtcagtttcacgactaaaggtcatattgactaagtagtcatcagctgaccacctcgctgtatcagccagcaacgaggggaaggtgaagaaacatgataggccatatagaatctgccctatgtttacttttttaacccagataattatttttgtgtgcagtatctaagctcctgattgtgtaacctgggacttctggcaccttttgttccattcattttatgtataaaatgcatgccaaagcacactgtgccctctggtacccttgcttccaatcgccaaccatgctcatttccttcctttttttgtggtccctttttgtggtgatcattttaaaccacgtcatccaacaaatgttttatggtcaaccttagcttgttcataagccatagcaactgaaagattaaactcttaaatatgtgtctgggcagtggctattaaatagcaaaaaacaatcagattttagtattttattatttccttgtaaaatggctgaactaaattaaacccttgtttcccatttgttctataatttatagtgaaactgagaacaaaactatctttataaatgatagctaaaagtatttccagatatttaaacaatttaaaataaatttcttctgcagagatgcaaagcatctcaacactggaatgaacaaatgccttaaattcaatggagtaaacctttagaatgaagaggaactgtcatttcacccaagccgaagacaacagccttatgcacttgtgtgctctgtctttgctgcttctcgtgtttcaagcctttcctgtgggatcagcacagcaaagtgcaacttaccaaatggtttaatgactggttaattctttcttctcccaatggaaaagcaatggcaacacaacagtagactgctggcttgacaatcttaaacgtgagcctttgcacatgtaggtttatcatcatttgagtatacgactaagcaagtcaatgaactttttttttttttttagcagtttaatttggtcctgagaatgttgcagtctttattaccccttttgcattaatccacttttctaaccaccttttaagctttaatttttaacactatacaccaagtctttgaaatcagtgatctgttatttaactctaaagcatttgacacttcttgccttaacagttttaaaaaccacacacaaaaaaactctgtaagtaatacagtaggccaaaagtttcatcctatctatcttgcagtttacctatctgatctgatctctgtaattatagttctgtcatttaaaatatactatttaaatctaatttttacatttcaaaaattatcttcagtagtaactaagtatattttctgtggattctgagaatgttatttttcagaatgtgagaatatatatgtacatttataatcttgtgactttaaagtctgttttcagatacagtatgtaaatacttgtaaaaaaatttgtataattttgtgataatgtagtttcccaaaaaaattatttagaaggcattatgttattagtaaatgagagcactgtatagaactgttcctattttctgcacttgccattccagctgcctccactgtccatacccacctcattcatcctgtcacagaaggcaggaaaactgggaactttaccaaagtagcactcagcctgagaggcctgtataatcatgcttttcaaactaaattcacttaaaaattaaaaagcagaattgaatattttaagcagcctcagtacctttggccaatgctgttttcatggtggattatgaacattatataatctttgggaaaagtgaaagtagtacaatttttagaataatgacaactgcctcactgcatctctccactcacacagcaaccgtgtagccccctaagctgcagtaccatgactaaccatgatgtcaatttcatatgctgatcctcacaacagcagtgcacaaacatgccccaaatattttaacagaatttagctcttccttaagctgtcttttcatagtaaaaacaaaacaaaaacacccaatgttaaaaccacataataaacttacaaacttgaaaaattagacacttcagatagataggcaataaaacttcatattatgaaagcaatatattccaagtttcaaagatttgacaagttctgtagagtatctttcatcagtacatgaaaacttccaaactgcatgatcttctgccaggcaggactgggtgctattcgctggtttgaggtcgaatccatttcaaggcatgtcgtggtgggacattaatggtgggatggtagaatgtgcagtccggtcttgtacattgagtgttaaacctacaatgttttggatgatagaagggacattccatcttcttacaagcagggaagtaacggcagagctgactactggaaggtggtgctggtggtgcaactgctggttttggagacagtactggaattcttctactcacatgagtgaagggacaatctggtttagtacactttgcatcatatttacaatttgggtgaacaaacaaacatttttcagcaaatttacaattggggaaggctttgcagggtgagatggggtgatggtaggcacactcatccccatttttacaagcaggccagtacttgcagcgctccaaaagtttttctggtttctgtgccacactcagttcactcatctcagcgttagaaaagctaccatttgggtcctcaagctgcctgctcagcaagtgcaactgctgtgggtggaggagacctctgagtcccttgtttgaggctgcagtttggtttacgggtttcattccttcaaagcacatgtcctcctcttgatctgacatgtatcctggggggctggggacaccatccagcgtcactataaacttgggacttgcaggtttatctggttgtacaagatctcgtgtctgcataaggtgtcctgaaagtacccgaagggaatctgcagtcttcatccccgactcttggtttggtgccactactacttcctcagacagctttggcttcttcagaataaatgatcttgtgtctgcatggaccatggattccatgtcatagtaatcttgatttttttctacagaatctccttttgtttcctcttctttaatggggggacttattctgggggtcctactttgtccctggaccacttctgctagcaattcttcttgagaagttcgagttctgggagcaactggaagtgtctgtttctgtggaactgtagagtagttagttgtttttgttacggattcttgagcttcagatatagccttcaaaatcagattcttgttagcttgtttagaaggtggaagagaaggtctcctttcaggctttgcaggcacagacacactgctggagatgcttcctgttcgagacccgtaatcatcatcttcttcctcctcttctccatcatgattgaatttttttactttaacaactgaacttaccacaggcaactttctcttccgaaagttttcatcctccatactcattttctccgagttgtttctaaagaacggactatacgtttcttctaagctgttaagcacctctggttcacacaaacgtcctgtttcatatacccaactactctgcatatcaagctgcttggcagcatgaatactattctgctgctgttgaaattgcaacctgtttaaatgaacaccactatctgcatttctacttgcaggtggtcgataaatttcaatagaagggcgagaagaaccatatgtaagtgtcactgtaggttttttctgagataagggattctcctgcacaaagttgaggtcttcgtcaatgagatcatctggttctggcttaatatcaatcacatcttcagagggtgctggctccctcaaaggtttcactgttgacattagtcgggttgcagctccatcatcgtaagtctgtctgacatttgtggtttttgactcctgcgaacttgtagaaactctggaatctcttttttcaggtctcgcgctaggaatggcaagtggtggcactgcagcttcatgcctcctctcatctccccgactgaaattgctcttgtttgaaggcacgttactatcaaagatgttggtatcagaagacttcagactagagggttcagttgtaacagagcgaagtttatctaatacaccatgaagccaacataagctcctaattcttgtaatttccccttaatggcactccggatcttgcggctgatctcggtgccgatctccatggctctgcggcgtgcgggaactcagcactgcgcggcgcttggcttacccggaggctgccgcggactcctaccccgcagccgggacaccaccgcctcc

SEQ ID NO: 17236 - RNA, 14859 nt, Homo sapiens
  source 1..14859: mol_type = other RNA
tcaggccaggcacagtggctcacacctgtaatcttatcactttgggaggctgaggcaggtggatcgcttgagcccaggagttcaagaccagcctgggcaacatggtgaaaccccatcgctataaaaaacaacaattagccgggtgtggtggcacatgcctgtagtccctgctactcaggaggctgaggtgggaggatcacttgagcctggggaggtcaaggctttagtgagctgtgatggtgccactgcactccagcctgggtgacagagtgagaccccatttaaaaaacaaaaacaaaaacaaaaaaaaatgtgacatatagttgactaagaagtacatttcaatacaggattgaaagaacccacatatgttaattaaacacaagcgcagaatttgtgccttttacataaaggaagaatgcacataggcatgctttcagacaagcaattcatctagcagaaaaggaaggaatacatttttcagcccttccaggaataaaatccataaatgggctctatttcgtcctccaacacttgtatttcccacgtcatttactcctgcacacccccactcactagaagcctgctaaactgttccagtgagatattttaacacctgatagggaataaatatgcttctgttttggccttcaaaaataagctctgggccagttgcagtggctcacgcctgtaatcccaacactttgggaggccgaggtgggcggatcacgaggtcaggagtttgggatcagcctggccaatatggtgaaactccatctctactaaaaatacaaaaattagccaggcatggtgcctgtaatcccagctacttgggaggctgaaggagaagaatcgcttgaacctgggaggcacaggttgcagtgagccgagatcacaccactgcactccaggccaggtgacagagcgacactctgtctcaaaaaaataaataaatcaactctgtagcatagcatttgtaattctattattttgccttacatttccattatccttttaataaaattgtttttttacatcttcctaatcaagaagtattatgaggccaggcacagtggctcatacctggaatcccagcactttgggaggccgaggcaggcagatcacctgaggtcaaggtatttgagaccagcctggccaacatggtgaaaccccatctctactaaaaatacagaaattagctgggtgtggtggtgcacacctgtaatgctagctactcgggaggctgaggtaggagaatcgcttgaacctgggaggcagaggttgcaataagcctagatcatgccactgcactcaagcctgggagacagagcgagactacatcttaaaaaaaaaaaaaaaagtattatgagagaggataatgtattgtaatgtattgtagaggctaaataaaattatgctcatgtcagaaaaaaagagtatttctcaaaataaaattcactgaaactggatgtttattttgactgagatatagtatatcctcaaattgccatagaaagtttacaagaatattagaggtaaattataaatatcagggcctttttaaaaaaaaaagattctgcttataacttggtatttgtttataataaaaattatagtagccaataatgaacacttactctggcttggttatttacttaggtcaaaagaaggaggagcggttaaactgtgggatcaggaactgaggcggtgccgtgccttcaggcttgagacaggacaagccacagattgtgttcgttctgtgtgcagaggcaaagtaagatgttccatgagctgatacagtgcagcagaaaacagaaagtggttattactgtgattccctcaccctttgcagcctaatgaacaatacttaataatgcataacgatggatttgcttgccaacattactctgtctttgctgctttctttgccaaagttagcaccagtgtggtgcataagctaggaagctattctgtctaaatactgtatgtaaacctccaatattttctagaatctgccaatttaacaactctagtagacataattgaaagcccttggcagttgactcatattaggacagctgtctccattttttaaaaaaacacacattccctagataaaacgtgcagtaaacaaacaatgaaatactactcagccataaaaaataatgaaattctgtcattcttggtggcaacatggatgagactggaggacatgatgtgaagtgaaataagccaggcacagaaagataaatacatgttctcactcctgtgcagaaactaaaaaagttgatcccacagaggtggagagtagaatagtggttactggaggcggacaagggggagggggagggggatagggaaggactggttaaaggatacaagtttacacagccagataggaatagtatgttttagtattctgtagtactgtaggatgactatagttaagaatcacgtatttatgtattttcaggtatttacaagagaggattttgaaagtttccatcacaaagaaatgataaatgtctgaggtgatggttatgcgtattaccctatgccctatagatatgtataattatgtgtcaatttcaaaataaaaattcaaaactacaactcctatgaaaatttttgagcgtgtttgtacttattaagtgtatttataaatcatacggatattatcttcagcctgcatattaaattgtagttaagcttttactttttaactaaaaaataaattctattattttttcctatatcccactgcactgaccccagtttggaaatcctaagattatcaaataaaaactttgattattgaagaatccaggtgtactgccacagaaaagttctattctgtagcatggactctaatatgtaatctagcccattgtgcttacagatagatgtgtgcctgtagtcatagaaaaatttgcatgagctaatgactgccttgctactagattagctcaaagcaaaaagttctctgaaagcaggtcaatagggtcatttttatattatgaagaagaaaagcagctgttgtattacattcactgtattggtcctgcttgtgtttcagggcaagatccttgttgggacaaggaatgctgaaataatcgaagttggagagaaaaatgcagcttgtaatattttagttaacggtcatgtggatgggccaatctggggactagcaacacatccttccagggattttttcctttctgctgcagaagatgggacagtgagactttgggatattgctgataaagtaagtacagataatttttttaaaagaggttacaacttctaaaaagaaaagttggaagttctaaattgctagtacttaaagaactgccagaattctgttgagcattttgaggggaaactggtataatttagaagtacttcacttaatgtttcctatgactctttttttttttttttttaaatgcagaagatgttaaacaaagtgaatttgggacatgctgctcgtactgtgtgttacagccctgaaggggacatggtggctattggaatgaaaaatggagaatttatcattttactagtgagttctctaaaaatatggggaaagaagagagacaggagatgtgcaatccatgatatcaggttagtgaacaaatggaatagagtttctagtatatacttgatttaacttccatttgtaaaattttccatagccttgccttcaaaaagaggtccccagggcctgtagcatttcccgtattataaattgtatgctaaaatatggctgtttgtatactacttaattcttcttgctaaattataaacccactgggcaccaactataatagcaagtactagtaggtaatgtttgatgaattcatgttaacacttagccatgtccattaagttcatcccaccaagaggtatctcccactgtaatacaagagagctatctgcccttcaaaagttgtcaccctggaaaactaaagttgtgatttcaaacatatcttctcttagtaacctcagtttgggaatatgtagttcattaatttaatcaatacctattgattaaatgttccagaatccaaattaatttaaatgtttcttaaacctttgtttttcagtgcttaagcatttttcaacagtggctaccatttacggagtacttccgtgtgatcagtagataagattattgaatctaggtctgtcaaaagcttgtacacttttcatcagtaaaatccttttacaaatgaaaccttcctcagaacttcaatatataaaatagtaacagtggcttcccttagcttttacatgtctctatcgtacctcagtaagactcatgggccatttcaagagactgaattgtcccatatgactccaaagattgctaggcaaatagcatttcactttgtcttttaaataagttcttcaggccgggcgcggtggctcatgcctgtaatcccagcactttgggaggccgaggcaggcagatcacctgaagtcaggagtactcgaccagcctggccaacatagtgaaaccccatctcaactaaaaatacaaaaatcagccgggcgtggtggcaggcgcctgtaatcccagctactcagggggctgaaacaggagaatcgcttgaacccgggaggcggaggttgcgccatcgcactccagcctgggagacaagagcgagacttcgtctcaaaaaaaaaaaattcttcttccaagattcaagttgtgtcatttcaccttaataactggaggttagttaagctgggctgtgttctttgcttaatattaagacaacgttttttccagatggaagaaaactatcttaatgaattgttagcttattaattatgtaatgctaatggcttttaaaagctgagatgttctgactgggtgttgtggctcacacctgtaatcccagtaccttgggaggccaagggggaaggattgcttgaggccaggagtttgggaccatagtgagaccccgcctctatttaaaaaattaaattttgttttgttttgttttgagttggagttttgctcttgttgcccatgctgaagtgcaatggtgcaatctcagctcaccacaacctgtgcctcctgggttcaagcgattctcctgcttcagcctcccgagtagatgggattacaggcgtgcaccaccatgcctggctaattttgtatttttagtagagacagggtttctctatgttggtcaggctggtctcaaactctcgacctcaggtgatctgcccgcctccgcttcccaaagttctgggattataggtgtgagccactgggcctggcctaagaaagtttttttaagccattagacgtttttaaaggaattgggagatgacaattggggaaatatttaaaatttaagtaaaatataaagcttccttatttcatgtaacccagacaatctcagtatacatgatcagttgtgtctgacaggtaaatctatttgaggccttatcacacgttacttttaagaactagaaaggaaaagtcactgatcttaagtatttataatacttcatgtggtctaatactttttacgttttgttttgattcagatttagtccggattcccggtatctggcagtaggttctagtgagaactcagtggatttttatgacctaacgctgggccccactcttaacagaatcagctactgcaaagacattccaagctttgtcattcaaatggacttctctgcagatagcagttatctccaggtacagtaccaatactgtatacccaggtggcaagttcttctgcttttacatttcgtgttagtgaatgcatttaaagttcctgagctccagagctccagcttctcaactcctccctttgtaccttctgacctacagctcccctttcctcccccacttatcagagcttttctcctattaagtttttgtagtgatcttttgcatacttaataatgttagacatgtaaatcaagtagcaatatgctagtattctgtaaaccccctgtggattttgtctctcacctaatggaattcttgtcccattttaatctgatgaaaaaggtctctagtggctgctataaacggcatgtctatgaagtgccttcaggaaaacatcttatggatcatgccgctattgacagaattacttgggctacatggactaggtaaatacttatatattcacaaggcaagaactgactttgaaggccagttagaaaatcctatttctgaactgttagagccattccaataaggaatagtaattgagtttcaagtttttgttaccatattttgaaatggtatgttcatgttgggacccctttttattgaatatatttccatgttttatcagtttccatgatttatcaagttttttttttaaggaaatcaaagttttaactttaaagataccctgatatttttcttaatgctaaatttaatgactggcaaaaaggtattgggtgctgttaagcaactgttattaattctctatctaaaggaatgctatcttgaatctattagaagtcaaagcttccaaatttgttcaaatttcctggctgtatgacaggtaaccatgactatccatttttttggccaatgaaaaatgccatcaaattcctgtatcagccaggcatatagtggctcatgcctgtaatctctgatgtagcaggccgaggtgggaggatcacttgagcctagaagttttgataccagcctgggcaacatagcaagaccccatctctgaaatttttttaattcctatgtcataagtcatttttatttttgtagagatagggatctcacaatattgcccaggctggtctcaaactcttggcctcaagcagtcctcctgcctcagcctcccaaaatgttgggattactggtatgtgctgctggacccagccaagtagcacttttaatttgaaaaatagttctatcagttttcagtcaggcgcggtggctcagcctgtaatcccagcactttgggaggccgagcgggggtgatcacctgaggtcgggagttcgagactagcctgaccaacatggagaaaccctgtctctactaaaaatacaaaataagccgggcatgttagcgcatgcctgtgatcccagctactcgggaggctgaggcaggagaattgcttgaacccaggaggcagaggttgcggtgagccgagatcatgccattgcactccagcctgggtaacaagagcgaaaactccgtctcaaaaaaaaaaaaagaaaaaatagttctatcagttttcataaagtactactttaatcttaaaaagattaatctagaaacccttcaaattataaaatgtcatttttaaaaggcaggagttgatatcctgatgaaattcaggtctccaaacaacttaccataatttacttcctgtattttaagtaacatgatagggtacttagagattaattgccaagaaactttttgaatatagtcaacctgcccgcacttgccatgatgagttttcttttgttccttccctctagtattctaggagatgaggttttgggaatctggtccagacatgctgagaaagctgatgtcaactgtgcctgtgtatctcattcaggaatcagtcttgttacaggagatgactttggcatggttaagttatttgacttcccatgtccagaaaaatttgtaagtttgtgttttgtttactattatcagtttactcctaattttgatgtcttatcatcagcacttttccccatatatttaaaatgttttgtcctaatttctaaatttttccccaaactttctaaatctatttactttgaaataaaagctattagaaacaaatcctctccctcgagtaataccatctttggaaccatcctacaaaagctgtaattagcttttcaccaaacctataatcagttatcaaatttcaaatgcttttccttagagaaaaatggtcagagtacctggagacatctgactgcccacacagcctggttttgcagatccactactcatgctgaaaagcattctaatcactggctgcggtgctaactccctactctctccacagctcttgtcatagagattatagttcctaataagagcctttgacttctgtgtgcaccaaatgccctgagcttgtctgtcattgttttttaggcaaaacacaaaaggttcttgggtcattcgccccatgtgacaaatattcgatttaccagtggtgatcgacatgttgttagtgctggaggtgatgactgcaggttagtaactttctcagcccatgaagagcagactatgttactagttaagagacttaatacaacaactcctacagctttggtttatgaaatcagctagtcaacattagtagaaggtagtataaccagatggctcttcagaatctcatatttatgcaaatacagaataaaaggagttaaagaggaaaaatattacacatgtaacctgaaagcacaactgaaaaatattaaactgttatgaaaatctaaaaacataattaactccctgcaattttcttctctgattgcagcttatttgtctggaaatgtgtacatacacctcactgagagatgctgagatgactacagaaattaactttgagaccagaattacagagaagaaaaaccaaaacccaaccctgcatggtcaagtggtgctaacccaagactgtaacagggagaaatgcccagaatcatcaaaatagtgaaagactgatctgttcaaaatatttgctatatgcactgggtataatccgtaatccatacactgccagataatgccatttcaaggaaggatcgaatacttgatggtaaaggccaagtccccctgtattgggaagtgtgtgatttcggcagacctgctgggaaaatttagggtagagcactctttacagaagaactcaaaaacccaatttggataattttcattatctttttagcaaaatggtttcttaatgtttatattttattttcaaggttcattgtttaatgaaatattttattcttgcatttccataaggaaagggaaagtcatgatcatcctaaaggatcacagtttttaaaaggcaaacattttccctaaggaaacagacacaagctttcctagagaatatgatgttttttaggcattaataaggtccttttttataaaggacacttttctcctagtagttttgaattcaggaacagatccaaagttagcagtatatggctgctacatttccattttcattttcgagccatcagtttatgttcagatgccatctctgtaatcgcacatttaaaacataactgtagcctcactaatggaaaagtagtatgatgaacaatcattcccaatggtgtacaatgtaagggttttagggagcaacagtatttaactggaagaaagaattgcatatttaatgtagtctaatatatacacatttgtttaacatgtaaacaaaagtgttaaattcacatatacaacattatacaatttaatcactcttggaataaaatttttatagccttttttctattgggaaaatttgtttagatgtgtgccactccataggtttatttccaaaatgaatgagcccaactccatttgtaaaaacttgtcagttagaattcctttttttagtggattagggctgaattcttagatccttatttcttttcactttaaatgctgccaaagatcactactcatcattcaggaattcgctgtctagcctatctgtagtttcctgaagattgaaaattatgtagactgctatttaaaaatatatttttctaagtgtgaggtttaagatgctgtattgaccctatgagtttttaatgtgttaattatctttatagcataatagatcgctttaggttcctggaatcccatttggtctgacaggatatatgaagattcttaatacctattttctgtgtctaatacttggttaatactaaaaatagaaatgactaaattacatcacagaaagcataaccagtgattgaacctggtagttttaaagctctaaatagctgtggctgaaggactgattatggggctaagaagcttgaaacgtaagttggtacttgttcatcagtggattctcctaaattaagccaaattttgaaatacatgactattaagtttctactcatgtatttacagtcagtcaataaattaaaggaggaaaaaaatccctgaacaacctgcccataaaaagaaaaatactctacatttgagcctgctgcagttttaaattttccctctgggtcaagtttgccagcttttggctacagagaaattatatttccattacagtgcaggtagaaactctgtaaccttaagcatgtaaactacatagaataaaactgtttccactgcatttctgtccttcaaagtggccaacctgattaagtcagccttaatcactgctgctgtcagtttcacgactaaaggtcatattgactaagtagtcatcagctgaccacctcgctgtatcagccagcaacgaggggaaggtgaagaaacatgataggccatatagaatctgccctatgtttacttttttaacccagataattatttttgtgtgcagtatctaagctcctgattgtgtaacctgggacttctggcaccttttgttccattcattttatgtataaaatgcatgccaaagcacactgtgccctctggtacccttgcttccaatcgccaaccatgctcatttccttcctttttttgtggtccctttttgtggtgatcattttaaaccacgtcatccaacaaatgttttatggtcaaccttagcttgttcataagccatagcaactgaaagattaaactcttaaatatgtgtctgggcagtggctattaaatagcaaaaaacaatcagattttagtattttattatttccttgtaaaatggctgaactaaattaaacccttgtttcccatttgttctataatttatagtgaaactgagaacaaaactatctttataaatgatagctaaaagtatttccagatatttaaacaatttaaaataaatttcttctgcagagatgcaaagcatctcaacactggaatgaacaaatgccttaaattcaatggagtaaacctttagaatgaagaggaactgtcatttcacccaagccgaagacaacagccttatgcacttgtgtgctctgtctttgctgcttctcgtgtttcaagcctttcctgtgggatcagcacagcaaagtgcaacttaccaaatggtttaatgactggttaattctttcttctcccaatggaaaagcaatggcaacacaacagtagactgctggcttgacaatcttaaacgtgagcctttgcacatgtaggtttatcatcatttgagtatacgactaagcaagtcaatgaactttttttttttttttagcagtttaatttggtcctgagaatgttgcagtctttattaccccttttgcattaatccacttttctaaccaccttttaagctttaatttttaacactatacaccaagtctttgaaatcagtgatctgttatttaactctaaagcatttgacacttcttgccttaacagttttaaaaaccacacacaaaaaaactctgtaagtaatacagtaggccaaaagtttcatcctatctatcttgcagtttacctatctgatctgatctctgtaattatagttctgtcatttaaaatatactatttaaatctaatttttacatttcaaaaattatcttcagtagtaactaagtatattttctgtggattctgagaatgttatttttcagaatgtgagaatatatatgtacatttataatcttgtgactttaaagtctgttttcagatacagtatgtaaatacttgtaaaaaaatttgtataattttgtgataatgtagtttcccaaaaaaattatttagaaggcattatgttattagtaaatgagagcactgtatagaactgttcctattttctgcacttgccattccagctgcctccactgtccatacccacctcattcatcctgtcacagaaggcaggaaaactgggaactttaccaaagtagcactcagcctgagaggcctgtataatcatgcttttcaaactaaattcacttaaaaattaaaaagcagaattgaatattttaagcagcctcagtacctttggccaatgctgttttcatggtggattatgaacattatataatctttgggaaaagtgaaagtagtacaatttttagaataatgacaactgcctcactgcatctctccactcacacagcaaccgtgtagccccctaagctgcagtaccatgactaaccatgatgtcaatttcatatgctgatcctcacaacagcagtgcacaaacatgccccaaatattttaacagaatttagctcttccttaagctgtcttttcatagtaaaaacaaaacaaaaacacccaatgttaaaaccacataataaacttacaaacttgaaaaattagacacttcagatagataggcaataaaacttcatattatgaaagcaatatattccaagtttcaaagatttgacaagttctgtagagtatctttcatcagtacatgaaaacttccaaactgcatgatcttctgccaggcaggactgggtgctattcgctggtttgaggtcgaatccatttcaaggcatgtcgtggtgggacattaatggtgggatggtagaatgtgcagtccggtcttgtacattgagtgttaaacctacaatgttttggatgatagaagggacattccatcttcttacaagcagggaagtaacggcagagctgactactggaaggtggtgctggtggtgcaactgctggttttggagacagtactggaattcttctactcacatgagtgaagggacaatctggtttagtacactttgcatcatatttacaatttgggtgaacaaacaaacatttttcagcaaatttacaattggggaaggctttgcagggtgagatggggtgatggtaggcacactcatccccatttttacaagcaggccagtacttgcagcgctccaaaagtttttctggtttctgtgccacactcagttcactcatctcagcgttagaaaagctaccatttgggtcctcaagctgcctgctcagcaagtgcaactgctgtgggtggaggagacctctgagtcccttgtttgaggctgcagtttggtttacgggtttcattccttcaaagcacatgtcctcctcttgatctgacatgtatcctggggggctggggacaccatccagcgtcactataaacttgggacttgcaggtttatctggttgtacaagatctcgtgtctgcataaggtgtcctgaaagtacccgaagggaatctgcagtcttcatccccgactcttggtttggtgccactactacttcctcagacagctttggcttcttcagaataaatgatcttgtgtctgcatggaccatggattccatgtcatagtaatcttgatttttttctacagaatctccttttgtttcctcttctttaatggggggacttattctgggggtcctactttgtccctggaccacttctgctagcaattcttcttgagaagttcgagttctgggagcaactggaagtgtctgtttctgtggaactgtagagtagttagttgtttttgttacggattcttgagcttcagatatagccttcaaaatcagattcttgttagcttgtttagaaggtggaagagaaggtctcctttcaggctttgcaggcacagacacactgctggagatgcttcctgttcgagacccgtaatcatcatcttcttcctcctcttctccatcatgattgaatttttttactttaacaactgaacttaccacaggcaactttctcttccgaaagttttcatcctccatactcattttctccgagttgtttctaaagaacggactatacgtttcttctaagctgttaagcacctctggttcacacaaacgtcctgtttcatatacccaactactctgcatatcaagctgcttggcagcatgaatactattctgctgctgttgaaattgcaacctgtttaaatgaacaccactatctgcatttctacttgcaggtggtcgataaatttcaatagaagggcgagaagaaccatatgtaagtgtcactgtaggttttttctgagataagggattctcctgcacaaagttgaggtcttcgtcaatgagatcatctggttctggcttaatatcaatcacatcttcagagggtgctggctccctcaaaggtttcactgttgacattagtcgggttgcagctccatcatcgtaagtctgtctgacatttgtggtttttgactcctgcgaacttgtagaaactctggaatctcttttttcaggtctcgcgctaggaatggcaagtggtggcactgcagcttcatgcctcctctcatctccccgactgaaattgctcttgtttgaaggcacgttactatcaaagatgttggtatcagaagacttcagactagagggttcagttgtaacagagcgaagtttatctaatacaccatgaagccatacggtgaatcgaattgtgttgttccctagaaacagggacagatcctctgtcatttggtcctgacttttcttgttggccaccatcaccataatgtaatcaggaagttcttcatcaacataagctcctaattcttgtaatttccccttaatggcactccggatcttgcggctgatctcggtgccgatctccatggctctgcggcgtgcgggaactcagcactgcgcggcgcttggcttacccggaggctgccgcggactcctaccccgcagccgggacaccaccgcctcc

SEQ ID NO: 17237 - RNA, 15040 nt, Homo sapiens
  source 1..15040: mol_type = other RNA
tcaggccaggcacagtggctcacacctgtaatcttatcactttgggaggctgaggcaggtggatcgcttgagcccaggagttcaagaccagcctgggcaacatggtgaaaccccatcgctataaaaaacaacaattagccgggtgtggtggcacatgcctgtagtccctgctactcaggaggctgaggtgggaggatcacttgagcctggggaggtcaaggctttagtgagctgtgatggtgccactgcactccagcctgggtgacagagtgagaccccatttaaaaaacaaaaacaaaaacaaaaaaaaatgtgacatatagttgactaagaagtacatttcaatacaggattgaaagaacccacatatgttaattaaacacaagcgcagaatttgtgccttttacataaaggaagaatgcacataggcatgctttcagacaagcaattcatctagcagaaaaggaaggaatacatttttcagcccttccaggaataaaatccataaatgggctctatttcgtcctccaacacttgtatttcccacgtcatttactcctgcacacccccactcactagaagcctgctaaactgttccagtgagatattttaacacctgatagggaataaatatgcttctgttttggccttcaaaaataagctctgggccagttgcagtggctcacgcctgtaatcccaacactttgggaggccgaggtgggcggatcacgaggtcaggagtttgggatcagcctggccaatatggtgaaactccatctctactaaaaatacaaaaattagccaggcatggtgcctgtaatcccagctacttgggaggctgaaggagaagaatcgcttgaacctgggaggcacaggttgcagtgagccgagatcacaccactgcactccaggccaggtgacagagcgacactctgtctcaaaaaaataaataaatcaactctgtagcatagcatttgtaattctattattttgccttacatttccattatccttttaataaaattgtttttttacatcttcctaatcaagaagtattatgaggccaggcacagtggctcatacctggaatcccagcactttgggaggccgaggcaggcagatcacctgaggtcaaggtatttgagaccagcctggccaacatggtgaaaccccatctctactaaaaatacagaaattagctgggtgtggtggtgcacacctgtaatgctagctactcgggaggctgaggtaggagaatcgcttgaacctgggaggcagaggttgcaataagcctagatcatgccactgcactcaagcctgggagacagagcgagactacatcttaaaaaaaaaaaaaaaagtattatgagagaggataatgtattgtaatgtattgtagaggctaaataaaattatgctcatgtcagaaaaaaagagtatttctcaaaataaaattcactgaaactggatgtttattttgactgagatatagtatatcctcaaattgccatagaaagtttacaagaatattagaggtaaattataaatatcagggcctttttaaaaaaaaaagattctgcttataacttggtatttgtttataataaaaattatagtagccaataatgaacacttactctggcttggttatttacttaggtcaaaagaaggaggagcggttaaactgtgggatcaggaactgaggcggtgccgtgccttcaggcttgagacaggacaagccacagattgtgttcgttctgtgtgcagaggcaaagtaagatgttccatgagctgatacagtgcagcagaaaacagaaagtggttattactgtgattccctcaccctttgcagcctaatgaacaatacttaataatgcataacgatggatttgcttgccaacattactctgtctttgctgctttctttgccaaagttagcaccagtgtggtgcataagctaggaagctattctgtctaaatactgtatgtaaacctccaatattttctagaatctgccaatttaacaactctagtagacataattgaaagcccttggcagttgactcatattaggacagctgtctccattttttaaaaaaacacacattccctagataaaacgtgcagtaaacaaacaatgaaatactactcagccataaaaaataatgaaattctgtcattcttggtggcaacatggatgagactggaggacatgatgtgaagtgaaataagccaggcacagaaagataaatacatgttctcactcctgtgcagaaactaaaaaagttgatcccacagaggtggagagtagaatagtggttactggaggcggacaagggggagggggagggggatagggaaggactggttaaaggatacaagtttacacagccagataggaatagtatgttttagtattctgtagtactgtaggatgactatagttaagaatcacgtatttatgtattttcaggtatttacaagagaggattttgaaagtttccatcacaaagaaatgataaatgtctgaggtgatggttatgcgtattaccctatgccctatagatatgtataattatgtgtcaatttcaaaataaaaattcaaaactacaactcctatgaaaatttttgagcgtgtttgtacttattaagtgtatttataaatcatacggatattatcttcagcctgcatattaaattgtagttaagcttttactttttaactaaaaaataaattctattattttttcctatatcccactgcactgaccccagtttggaaatcctaagattatcaaataaaaactttgattattgaagaatccaggtgtactgccacagaaaagttctattctgtagcatggactctaatatgtaatctagcccattgtgcttacagatagatgtgtgcctgtagtcatagaaaaatttgcatgagctaatgactgccttgctactagattagctcaaagcaaaaagttctctgaaagcaggtcaatagggtcatttttatattatgaagaagaaaagcagctgttgtattacattcactgtattggtcctgcttgtgtttcagggcaagatccttgttgggacaaggaatgctgaaataatcgaagttggagagaaaaatgcagcttgtaatattttagttaacggtcatgtggatgggccaatctggggactagcaacacatccttccagggattttttcctttctgctgcagaagatgggacagtgagactttgggatattgctgataaagtaagtacagataatttttttaaaagaggttacaacttctaaaaagaaaagttggaagttctaaattgctagtacttaaagaactgccagaattctgttgagcattttgaggggaaactggtataatttagaagtacttcacttaatgtttcctatgactctttttttttttttttttaaatgcagaagatgttaaacaaagtgaatttgggacatgctgctcgtactgtgtgttacagccctgaaggggacatggtggctattggaatgaaaaatggagaatttatcattttactagtgagttctctaaaaatatggggaaagaagagagacaggagatgtgcaatccatgatatcaggttagtgaacaaatggaatagagtttctagtatatacttgatttaacttccatttgtaaaattttccatagccttgccttcaaaaagaggtccccagggcctgtagcatttcccgtattataaattgtatgctaaaatatggctgtttgtatactacttaattcttcttgctaaattataaacccactgggcaccaactataatagcaagtactagtaggtaatgtttgatgaattcatgttaacacttagccatgtccattaagttcatcccaccaagaggtatctcccactgtaatacaagagagctatctgcccttcaaaagttgtcaccctggaaaactaaagttgtgatttcaaacatatcttctcttagtaacctcagtttgggaatatgtagttcattaatttaatcaatacctattgattaaatgttccagaatccaaattaatttaaatgtttcttaaacctttgtttttcagtgcttaagcatttttcaacagtggctaccatttacggagtacttccgtgtgatcagtagataagattattgaatctaggtctgtcaaaagcttgtacacttttcatcagtaaaatccttttacaaatgaaaccttcctcagaacttcaatatataaaatagtaacagtggcttcccttagcttttacatgtctctatcgtacctcagtaagactcatgggccatttcaagagactgaattgtcccatatgactccaaagattgctaggcaaatagcatttcactttgtcttttaaataagttcttcaggccgggcgcggtggctcatgcctgtaatcccagcactttgggaggccgaggcaggcagatcacctgaagtcaggagtactcgaccagcctggccaacatagtgaaaccccatctcaactaaaaatacaaaaatcagccgggcgtggtggcaggcgcctgtaatcccagctactcagggggctgaaacaggagaatcgcttgaacccgggaggcggaggttgcgccatcgcactccagcctgggagacaagagcgagacttcgtctcaaaaaaaaaaaattcttcttccaagattcaagttgtgtcatttcaccttaataactggaggttagttaagctgggctgtgttctttgcttaatattaagacaacgttttttccagatggaagaaaactatcttaatgaattgttagcttattaattatgtaatgctaatggcttttaaaagctgagatgttctgactgggtgttgtggctcacacctgtaatcccagtaccttgggaggccaagggggaaggattgcttgaggccaggagtttgggaccatagtgagaccccgcctctatttaaaaaattaaattttgttttgttttgttttgagttggagttttgctcttgttgcccatgctgaagtgcaatggtgcaatctcagctcaccacaacctgtgcctcctgggttcaagcgattctcctgcttcagcctcccgagtagatgggattacaggcgtgcaccaccatgcctggctaattttgtatttttagtagagacagggtttctctatgttggtcaggctggtctcaaactctcgacctcaggtgatctgcccgcctccgcttcccaaagttctgggattataggtgtgagccactgggcctggcctaagaaagtttttttaagccattagacgtttttaaaggaattgggagatgacaattggggaaatatttaaaatttaagtaaaatataaagcttccttatttcatgtaacccagacaatctcagtatacatgatcagttgtgtctgacaggtaaatctatttgaggccttatcacacgttacttttaagaactagaaaggaaaagtcactgatcttaagtatttataatacttcatgtggtctaatactttttacgttttgttttgattcagatttagtccggattcccggtatctggcagtaggttctagtgagaactcagtggatttttatgacctaacgctgggccccactcttaacagaatcagctactgcaaagacattccaagctttgtcattcaaatggacttctctgcagatagcagttatctccaggtacagtaccaatactgtatacccaggtggcaagttcttctgcttttacatttcgtgttagtgaatgcatttaaagttcctgagctccagagctccagcttctcaactcctccctttgtaccttctgacctacagctcccctttcctcccccacttatcagagcttttctcctattaagtttttgtagtgatcttttgcatacttaataatgttagacatgtaaatcaagtagcaatatgctagtattctgtaaaccccctgtggattttgtctctcacctaatggaattcttgtcccattttaatctgatgaaaaaggtctctagtggctgctataaacggcatgtctatgaagtgccttcaggaaaacatcttatggatcatgccgctattgacagaattacttgggctacatggactaggtaaatacttatatattcacaaggcaagaactgactttgaaggccagttagaaaatcctatttctgaactgttagagccattccaataaggaatagtaattgagtttcaagtttttgttaccatattttgaaatggtatgttcatgttgggacccctttttattgaatatatttccatgttttatcagtttccatgatttatcaagttttttttttaaggaaatcaaagttttaactttaaagataccctgatatttttcttaatgctaaatttaatgactggcaaaaaggtattgggtgctgttaagcaactgttattaattctctatctaaaggaatgctatcttgaatctattagaagtcaaagcttccaaatttgttcaaatttcctggctgtatgacaggtaaccatgactatccatttttttggccaatgaaaaatgccatcaaattcctgtatcagccaggcatatagtggctcatgcctgtaatctctgatgtagcaggccgaggtgggaggatcacttgagcctagaagttttgataccagcctgggcaacatagcaagaccccatctctgaaatttttttaattcctatgtcataagtcatttttatttttgtagagatagggatctcacaatattgcccaggctggtctcaaactcttggcctcaagcagtcctcctgcctcagcctcccaaaatgttgggattactggtatgtgctgctggacccagccaagtagcacttttaatttgaaaaatagttctatcagttttcagtcaggcgcggtggctcagcctgtaatcccagcactttgggaggccgagcgggggtgatcacctgaggtcgggagttcgagactagcctgaccaacatggagaaaccctgtctctactaaaaatacaaaataagccgggcatgttagcgcatgcctgtgatcccagctactcgggaggctgaggcaggagaattgcttgaacccaggaggcagaggttgcggtgagccgagatcatgccattgcactccagcctgggtaacaagagcgaaaactccgtctcaaaaaaaaaaaaagaaaaaatagttctatcagttttcataaagtactactttaatcttaaaaagattaatctagaaacccttcaaattataaaatgtcatttttaaaaggcaggagttgatatcctgatgaaattcaggtctccaaacaacttaccataatttacttcctgtattttaagtaacatgatagggtacttagagattaattgccaagaaactttttgaatatagtcaacctgcccgcacttgccatgatgagttttcttttgttccttccctctagtattctaggagatgaggttttgggaatctggtccagacatgctgagaaagctgatgtcaactgtgcctgtgtatctcattcaggaatcagtcttgttacaggagatgactttggcatggttaagttatttgacttcccatgtccagaaaaatttgtaagtttgtgttttgtttactattatcagtttactcctaattttgatgtcttatcatcagcacttttccccatatatttaaaatgttttgtcctaatttctaaatttttccccaaactttctaaatctatttactttgaaataaaagctattagaaacaaatcctctccctcgagtaataccatctttggaaccatcctacaaaagctgtaattagcttttcaccaaacctataatcagttatcaaatttcaaatgcttttccttagagaaaaatggtcagagtacctggagacatctgactgcccacacagcctggttttgcagatccactactcatgctgaaaagcattctaatcactggctgcggtgctaactccctactctctccacagctcttgtcatagagattatagttcctaataagagcctttgacttctgtgtgcaccaaatgccctgagcttgtctgtcattgttttttaggcaaaacacaaaaggttcttgggtcattcgccccatgtgacaaatattcgatttaccagtggtgatcgacatgttgttagtgctggaggtgatgactgcaggttagtaactttctcagcccatgaagagcagactatgttactagttaagagacttaatacaacaactcctacagctttggtttatgaaatcagctagtcaacattagtagaaggtagtataaccagatggctcttcagaatctcatatttatgcaaatacagaataaaaggagttaaagaggaaaaatattacacatgtaacctgaaagcacaactgaaaaatattaaactgttatgaaaatctaaaaacataattaactccctgcaattttcttctctgattgcagcttatttgtctggaaatgtgtacatacacctcactgagagatgctgagatgactacagaaattaactttgagaccagaattacagagaagaaaaaccaaaacccaaccctgcatggtcaagtggtgctaacccaagactgtaacagggagaaatgcccagaatcatcaaaatagtgaaagactgatctgttcaaaatatttgctatatgcactgggtataatccgtaatccatacactgccagataatgccatttcaaggaaggatcgaatacttgatggtaaaggccaagtccccctgtattgggaagtgtgtgatttcggcagacctgctgggaaaatttagggtagagcactctttacagaagaactcaaaaacccaatttggataattttcattatctttttagcaaaatggtttcttaatgtttatattttattttcaaggttcattgtttaatgaaatattttattcttgcatttccataaggaaagggaaagtcatgatcatcctaaaggatcacagtttttaaaaggcaaacattttccctaaggaaacagacacaagctttcctagagaatatgatgttttttaggcattaataaggtccttttttataaaggacacttttctcctagtagttttgaattcaggaacagatccaaagttagcagtatatggctgctacatttccattttcattttcgagccatcagtttatgttcagatgccatctctgtaatcgcacatttaaaacataactgtagcctcactaatggaaaagtagtatgatgaacaatcattcccaatggtgtacaatgtaagggttttagggagcaacagtatttaactggaagaaagaattgcatatttaatgtagtctaatatatacacatttgtttaacatgtaaacaaaagtgttaaattcacatatacaacattatacaatttaatcactcttggaataaaatttttatagccttttttctattgggaaaatttgtttagatgtgtgccactccataggtttatttccaaaatgaatgagcccaactccatttgtaaaaacttgtcagttagaattcctttttttagtggattagggctgaattcttagatccttatttcttttcactttaaatgctgccaaagatcactactcatcattcaggaattcgctgtctagcctatctgtagtttcctgaagattgaaaattatgtagactgctatttaaaaatatatttttctaagtgtgaggtttaagatgctgtattgaccctatgagtttttaatgtgttaattatctttatagcataatagatcgctttaggttcctggaatcccatttggtctgacaggatatatgaagattcttaatacctattttctgtgtctaatacttggttaatactaaaaatagaaatgactaaattacatcacagaaagcataaccagtgattgaacctggtagttttaaagctctaaatagctgtggctgaaggactgattatggggctaagaagcttgaaacgtaagttggtacttgttcatcagtggattctcctaaattaagccaaattttgaaatacatgactattaagtttctactcatgtatttacagtcagtcaataaattaaaggaggaaaaaaatccctgaacaacctgcccataaaaagaaaaatactctacatttgagcctgctgcagttttaaattttccctctgggtcaagtttgccagcttttggctacagagaaattatatttccattacagtgcaggtagaaactctgtaaccttaagcatgtaaactacatagaataaaactgtttccactgcatttctgtccttcaaagtggccaacctgattaagtcagccttaatcactgctgctgtcagtttcacgactaaaggtcatattgactaagtagtcatcagctgaccacctcgctgtatcagccagcaacgaggggaaggtgaagaaacatgataggccatatagaatctgccctatgtttacttttttaacccagataattatttttgtgtgcagtatctaagctcctgattgtgtaacctgggacttctggcaccttttgttccattcattttatgtataaaatgcatgccaaagcacactgtgccctctggtacccttgcttccaatcgccaaccatgctcatttccttcctttttttgtggtccctttttgtggtgatcattttaaaccacgtcatccaacaaatgttttatggtcaaccttagcttgttcataagccatagcaactgaaagattaaactcttaaatatgtgtctgggcagtggctattaaatagcaaaaaacaatcagattttagtattttattatttccttgtaaaatggctgaactaaattaaacccttgtttcccatttgttctataatttatagtgaaactgagaacaaaactatctttataaatgatagctaaaagtatttccagatatttaaacaatttaaaataaatttcttctgcagagatgcaaagcatctcaacactggaatgaacaaatgccttaaattcaatggagtaaacctttagaatgaagaggaactgtcatttcacccaagccgaagacaacagccttatgcacttgtgtgctctgtctttgctgcttctcgtgtttcaagcctttcctgtgggatcagcacagcaaagtgcaacttaccaaatggtttaatgactggttaattctttcttctcccaatggaaaagcaatggcaacacaacagtagactgctggcttgacaatcttaaacgtgagcctttgcacatgtaggtttatcatcatttgagtatacgactaagcaagtcaatgaactttttttttttttttagcagtttaatttggtcctgagaatgttgcagtctttattaccccttttgcattaatccacttttctaaccaccttttaagctttaatttttaacactatacaccaagtctttgaaatcagtgatctgttatttaactctaaagcatttgacacttcttgccttaacagttttaaaaaccacacacaaaaaaactctgtaagtaatacagtaggccaaaagtttcatcctatctatcttgcagtttacctatctgatctgatctctgtaattatagttctgtcatttaaaatatactatttaaatctaatttttacatttcaaaaattatcttcagtagtaactaagtatattttctgtggattctgagaatgttatttttcagaatgtgagaatatatatgtacatttataatcttgtgactttaaagtctgttttcagatacagtatgtaaatacttgtaaaaaaatttgtataattttgtgataatgtagtttcccaaaaaaattatttagaaggcattatgttattagtaaatgagagcactgtatagaactgttcctattttctgcacttgccattccagctgcctccactgtccatacccacctcattcatcctgtcacagaaggcaggaaaactgggaactttaccaaagtagcactcagcctgagaggcctgtataatcatgcttttcaaactaaattcacttaaaaattaaaaagcagaattgaatattttaagcagcctcagtacctttggccaatgctgttttcatggtggattatgaacattatataatctttgggaaaagtgaaagtagtacaatttttagaataatgacaactgcctcactgcatctctccactcacacagcaaccgtgtagccccctaagctgcagtaccatgactaaccatgatgtcaatttcatatgctgatcctcacaacagcagtgcacaaacatgccccaaatattttaacagaatttagctcttccttaagctgtcttttcatagtaaaaacaaaacaaaaacacccaatgttaaaaccacataataaacttacaaacttgaaaaattagacacttcagatagataggcaataaaacttcatattatgaaagcaatatattccaagtttcaaagatttgacaagttctgtagagtatctttcatcagtacatgaaaacttccaaactgcatgatcttctgccaggcaggactgggtgctattcgctggtttgaggtcgaatccatttcaaggcatgtcgtggtgggacattaatggtgggatggtagaatgtgcagtccggtcttgtacattgagtgttaaacctacaatgttttggatgatagaagggacattccatcttcttacaagcagggaagtaacggcagagctgactactggaaggtggtgctggtggtgcaactgctggttttggagacagtactggaattcttctactcacatgagtgaagggacaatctggtttagtacactttgcatcatatttacaatttgggtgaacaaacaaacatttttcagcaaatttacaattggggaaggctttgcagggtgagatggggtgatggtaggcacactcatccccatttttacaagcaggccagtacttgcagcgctccaaaagtttttctggtttctgtgccacactcagttcactcatctcagcgttagaaaagctaccatttgggtcctcaagctgcctgctcagcaagtgcaactgctgtgggtggaggagacctctgagtcccttgtttgaggctgcagtttggtttacgggtttcattccttcaaagcacatgtcctcctcttgatctgacatgtatcctggggggctggggacaccatccagcgtcactataaacttgggacttgcaggtttatctggttgtacaagatctcgtgtctgcataaggtgtcctgaaagtacccgaagggaatctgcagtcttcatccccgactcttggtttggtgccactactacttcctcagacagctttggcttcttcagaataaatgatcttgtgtctgcatggaccatggattccatgtcatagtaatcttgatttttttctacagaatctccttttgtttcctcttctttaatggggggacttattctgggggtcctactttgtccctggaccacttctgctagcaattcttcttgagaagttcgagttctgggagcaactggaagtgtctgtttctgtggaactgtagagtagttagttgtttttgttacggattcttgagcttcagatatagccttcaaaatcagattcttgttagcttgtttagaaggtggaagagaaggtctcctttcaggctttgcaggcacagacacactgctggagatgcttcctgttcgagacccgtaatcatcatcttcttcctcctcttctccatcatgattgaatttttttactttaacaactgaacttaccacaggcaactttctcttccgaaagttttcatcctccatactcattttctccgagttgtttctaaagaacggactatacgtttcttctaagctgttaagcacctctggttcacacaaacgtcctgtttcatatacccaactactctgcatatcaagctgcttggcagcatgaatactattctgctgctgttgaaattgcaacctgtttaaatgaacaccactatctgcatttctacttgcaggtggtcgataaatttcaatagaagggcgagaagaaccatatgtaagtgtcactgtaggttttttctgagataagggattctcctgcacaaagttgaggtcttcgtcaatgagatcatctggttctggcttaatatcaatcacatcttcagagggtgctggctccctcaaaggtttcactgttgacattagtcgggttgcagctccatcatcgtaagtctgtctgacatttgtggtttttgactcctgcgaacttgtagaaactctggaatctcttttttcaggtctcgcgctaggaatggcaagtggtggcactgcagcttcatgcctcctctcatctccccgactgaaattgctcttgtttgaaggcacgttactatcaaagatgttggtatcagaagacttcagactagagggttcagttgtaacagagcgaagtttatctaatacaccatgaagccatacggtgaatcgaattgtgttgttccctagaaacagggacagatcctctgtcatttggtcctgacttttcttgttggccaccatcaccataatgtaatcaggaagttcttcatctatttaaaaggaaaggtagatcaaaactttgtttcctcaaaactttcttcttaaagttgatgtgcttgaaaatatagatgtagctctaagctttagagtcgcagagctctactggaattacattggacaagatggcttagctttaatttttttctcttcattccacaggtatttcaaatacaacataagctcctaattcttgtaatttccccttaatggcactccggatcttgcggctgatctcggtgccgatctccatggctctgcggcgtgcgggaactcagcactgcgcggcgcttggcttacccggaggctgccgcggactcctaccccgcagccgggacaccaccgcctcc

SEQ ID NO: 17238 - RNA, 14774 nt, Homo sapiens
  source 1..14774: mol_type = other RNA
tcaggccaggcacagtggctcacacctgtaatcttatcactttgggaggctgaggcaggtggatcgcttgagcccaggagttcaagaccagcctgggcaacatggtgaaaccccatcgctataaaaaacaacaattagccgggtgtggtggcacatgcctgtagtccctgctactcaggaggctgaggtgggaggatcacttgagcctggggaggtcaaggctttagtgagctgtgatggtgccactgcactccagcctgggtgacagagtgagaccccatttaaaaaacaaaaacaaaaacaaaaaaaaatgtgacatatagttgactaagaagtacatttcaatacaggattgaaagaacccacatatgttaattaaacacaagcgcagaatttgtgccttttacataaaggaagaatgcacataggcatgctttcagacaagcaattcatctagcagaaaaggaaggaatacatttttcagcccttccaggaataaaatccataaatgggctctatttcgtcctccaacacttgtatttcccacgtcatttactcctgcacacccccactcactagaagcctgctaaactgttccagtgagatattttaacacctgatagggaataaatatgcttctgttttggccttcaaaaataagctctgggccagttgcagtggctcacgcctgtaatcccaacactttgggaggccgaggtgggcggatcacgaggtcaggagtttgggatcagcctggccaatatggtgaaactccatctctactaaaaatacaaaaattagccaggcatggtgcctgtaatcccagctacttgggaggctgaaggagaagaatcgcttgaacctgggaggcacaggttgcagtgagccgagatcacaccactgcactccaggccaggtgacagagcgacactctgtctcaaaaaaataaataaatcaactctgtagcatagcatttgtaattctattattttgccttacatttccattatccttttaataaaattgtttttttacatcttcctaatcaagaagtattatgaggccaggcacagtggctcatacctggaatcccagcactttgggaggccgaggcaggcagatcacctgaggtcaaggtatttgagaccagcctggccaacatggtgaaaccccatctctactaaaaatacagaaattagctgggtgtggtggtgcacacctgtaatgctagctactcgggaggctgaggtaggagaatcgcttgaacctgggaggcagaggttgcaataagcctagatcatgccactgcactcaagcctgggagacagagcgagactacatcttaaaaaaaaaaaaaaaagtattatgagagaggataatgtattgtaatgtattgtagaggctaaataaaattatgctcatgtcagaaaaaaagagtatttctcaaaataaaattcactgaaactggatgtttattttgactgagatatagtatatcctcaaattgccatagaaagtttacaagaatattagaggtaaattataaatatcagggcctttttaaaaaaaaaagattctgcttataacttggtatttgtttataataaaaattatagtagccaataatgaacacttactctggcttggttatttacttaggtcaaaagaaggaggagcggttaaactgtgggatcaggaactgaggcggtgccgtgccttcaggcttgagacaggacaagccacagattgtgttcgttctgtgtgcagaggcaaagtaagatgttccatgagctgatacagtgcagcagaaaacagaaagtggttattactgtgattccctcaccctttgcagcctaatgaacaatacttaataatgcataacgatggatttgcttgccaacattactctgtctttgctgctttctttgccaaagttagcaccagtgtggtgcataagctaggaagctattctgtctaaatactgtatgtaaacctccaatattttctagaatctgccaatttaacaactctagtagacataattgaaagcccttggcagttgactcatattaggacagctgtctccattttttaaaaaaacacacattccctagataaaacgtgcagtaaacaaacaatgaaatactactcagccataaaaaataatgaaattctgtcattcttggtggcaacatggatgagactggaggacatgatgtgaagtgaaataagccaggcacagaaagataaatacatgttctcactcctgtgcagaaactaaaaaagttgatcccacagaggtggagagtagaatagtggttactggaggcggacaagggggagggggagggggatagggaaggactggttaaaggatacaagtttacacagccagataggaatagtatgttttagtattctgtagtactgtaggatgactatagttaagaatcacgtatttatgtattttcaggtatttacaagagaggattttgaaagtttccatcacaaagaaatgataaatgtctgaggtgatggttatgcgtattaccctatgccctatagatatgtataattatgtgtcaatttcaaaataaaaattcaaaactacaactcctatgaaaatttttgagcgtgtttgtacttattaagtgtatttataaatcatacggatattatcttcagcctgcatattaaattgtagttaagcttttactttttaactaaaaaataaattctattattttttcctatatcccactgcactgaccccagtttggaaatcctaagattatcaaataaaaactttgattattgaagaatccaggtgtactgccacagaaaagttctattctgtagcatggactctaatatgtaatctagcccattgtgcttacagatagatgtgtgcctgtagtcatagaaaaatttgcatgagctaatgactgccttgctactagattagctcaaagcaaaaagttctctgaaagcaggtcaatagggtcatttttatattatgaagaagaaaagcagctgttgtattacattcactgtattggtcctgcttgtgtttcagggcaagatccttgttgggacaaggaatgctgaaataatcgaagttggagagaaaaatgcagcttgtaatattttagttaacggtcatgtggatgggccaatctggggactagcaacacatccttccagggattttttcctttctgctgcagaagatgggacagtgagactttgggatattgctgataaagtaagtacagataatttttttaaaagaggttacaacttctaaaaagaaaagttggaagttctaaattgctagtacttaaagaactgccagaattctgttgagcattttgaggggaaactggtataatttagaagtacttcacttaatgtttcctatgactctttttttttttttttttaaatgcagaagatgttaaacaaagtgaatttgggacatgctgctcgtactgtgtgttacagccctgaaggggacatggtggctattggaatgaaaaatggagaatttatcattttactagtgagttctctaaaaatatggggaaagaagagagacaggagatgtgcaatccatgatatcaggttagtgaacaaatggaatagagtttctagtatatacttgatttaacttccatttgtaaaattttccatagccttgccttcaaaaagaggtccccagggcctgtagcatttcccgtattataaattgtatgctaaaatatggctgtttgtatactacttaattcttcttgctaaattataaacccactgggcaccaactataatagcaagtactagtaggtaatgtttgatgaattcatgttaacacttagccatgtccattaagttcatcccaccaagaggtatctcccactgtaatacaagagagctatctgcccttcaaaagttgtcaccctggaaaactaaagttgtgatttcaaacatatcttctcttagtaacctcagtttgggaatatgtagttcattaatttaatcaatacctattgattaaatgttccagaatccaaattaatttaaatgtttcttaaacctttgtttttcagtgcttaagcatttttcaacagtggctaccatttacggagtacttccgtgtgatcagtagataagattattgaatctaggtctgtcaaaagcttgtacacttttcatcagtaaaatccttttacaaatgaaaccttcctcagaacttcaatatataaaatagtaacagtggcttcccttagcttttacatgtctctatcgtacctcagtaagactcatgggccatttcaagagactgaattgtcccatatgactccaaagattgctaggcaaatagcatttcactttgtcttttaaataagttcttcaggccgggcgcggtggctcatgcctgtaatcccagcactttgggaggccgaggcaggcagatcacctgaagtcaggagtactcgaccagcctggccaacatagtgaaaccccatctcaactaaaaatacaaaaatcagccgggcgtggtggcaggcgcctgtaatcccagctactcagggggctgaaacaggagaatcgcttgaacccgggaggcggaggttgcgccatcgcactccagcctgggagacaagagcgagacttcgtctcaaaaaaaaaaaattcttcttccaagattcaagttgtgtcatttcaccttaataactggaggttagttaagctgggctgtgttctttgcttaatattaagacaacgttttttccagatggaagaaaactatcttaatgaattgttagcttattaattatgtaatgctaatggcttttaaaagctgagatgttctgactgggtgttgtggctcacacctgtaatcccagtaccttgggaggccaagggggaaggattgcttgaggccaggagtttgggaccatagtgagaccccgcctctatttaaaaaattaaattttgttttgttttgttttgagttggagttttgctcttgttgcccatgctgaagtgcaatggtgcaatctcagctcaccacaacctgtgcctcctgggttcaagcgattctcctgcttcagcctcccgagtagatgggattacaggcgtgcaccaccatgcctggctaattttgtatttttagtagagacagggtttctctatgttggtcaggctggtctcaaactctcgacctcaggtgatctgcccgcctccgcttcccaaagttctgggattataggtgtgagccactgggcctggcctaagaaagtttttttaagccattagacgtttttaaaggaattgggagatgacaattggggaaatatttaaaatttaagtaaaatataaagcttccttatttcatgtaacccagacaatctcagtatacatgatcagttgtgtctgacaggtaaatctatttgaggccttatcacacgttacttttaagaactagaaaggaaaagtcactgatcttaagtatttataatacttcatgtggtctaatactttttacgttttgttttgattcagatttagtccggattcccggtatctggcagtaggttctagtgagaactcagtggatttttatgacctaacgctgggccccactcttaacagaatcagctactgcaaagacattccaagctttgtcattcaaatggacttctctgcagatagcagttatctccaggtacagtaccaatactgtatacccaggtggcaagttcttctgcttttacatttcgtgttagtgaatgcatttaaagttcctgagctccagagctccagcttctcaactcctccctttgtaccttctgacctacagctcccctttcctcccccacttatcagagcttttctcctattaagtttttgtagtgatcttttgcatacttaataatgttagacatgtaaatcaagtagcaatatgctagtattctgtaaaccccctgtggattttgtctctcacctaatggaattcttgtcccattttaatctgatgaaaaaggtctctagtggctgctataaacggcatgtctatgaagtgccttcaggaaaacatcttatggatcatgccgctattgacagaattacttgggctacatggactaggtaaatacttatatattcacaaggcaagaactgactttgaaggccagttagaaaatcctatttctgaactgttagagccattccaataaggaatagtaattgagtttcaagtttttgttaccatattttgaaatggtatgttcatgttgggacccctttttattgaatatatttccatgttttatcagtttccatgatttatcaagttttttttttaaggaaatcaaagttttaactttaaagataccctgatatttttcttaatgctaaatttaatgactggcaaaaaggtattgggtgctgttaagcaactgttattaattctctatctaaaggaatgctatcttgaatctattagaagtcaaagcttccaaatttgttcaaatttcctggctgtatgacaggtaaccatgactatccatttttttggccaatgaaaaatgccatcaaattcctgtatcagccaggcatatagtggctcatgcctgtaatctctgatgtagcaggccgaggtgggaggatcacttgagcctagaagttttgataccagcctgggcaacatagcaagaccccatctctgaaatttttttaattcctatgtcataagtcatttttatttttgtagagatagggatctcacaatattgcccaggctggtctcaaactcttggcctcaagcagtcctcctgcctcagcctcccaaaatgttgggattactggtatgtgctgctggacccagccaagtagcacttttaatttgaaaaatagttctatcagttttcagtcaggcgcggtggctcagcctgtaatcccagcactttgggaggccgagcgggggtgatcacctgaggtcgggagttcgagactagcctgaccaacatggagaaaccctgtctctactaaaaatacaaaataagccgggcatgttagcgcatgcctgtgatcccagctactcgggaggctgaggcaggagaattgcttgaacccaggaggcagaggttgcggtgagccgagatcatgccattgcactccagcctgggtaacaagagcgaaaactccgtctcaaaaaaaaaaaaagaaaaaatagttctatcagttttcataaagtactactttaatcttaaaaagattaatctagaaacccttcaaattataaaatgtcatttttaaaaggcaggagttgatatcctgatgaaattcaggtctccaaacaacttaccataatttacttcctgtattttaagtaacatgatagggtacttagagattaattgccaagaaactttttgaatatagtcaacctgcccgcacttgccatgatgagttttcttttgttccttccctctagtattctaggagatgaggttttgggaatctggtccagacatgctgagaaagctgatgtcaactgtgcctgtgtatctcattcaggaatcagtcttgttacaggagatgactttggcatggttaagttatttgacttcccatgtccagaaaaatttgtaagtttgtgttttgtttactattatcagtttactcctaattttgatgtcttatcatcagcacttttccccatatatttaaaatgttttgtcctaatttctaaatttttccccaaactttctaaatctatttactttgaaataaaagctattagaaacaaatcctctccctcgagtaataccatctttggaaccatcctacaaaagctgtaattagcttttcaccaaacctataatcagttatcaaatttcaaatgcttttccttagagaaaaatggtcagagtacctggagacatctgactgcccacacagcctggttttgcagatccactactcatgctgaaaagcattctaatcactggctgcggtgctaactccctactctctccacagctcttgtcatagagattatagttcctaataagagcctttgacttctgtgtgcaccaaatgccctgagcttgtctgtcattgttttttaggcaaaacacaaaaggttcttgggtcattcgccccatgtgacaaatattcgatttaccagtggtgatcgacatgttgttagtgctggaggtgatgactgcaggttagtaactttctcagcccatgaagagcagactatgttactagttaagagacttaatacaacaactcctacagctttggtttatgaaatcagctagtcaacattagtagaaggtagtataaccagatggctcttcagaatctcatatttatgcaaatacagaataaaaggagttaaagaggaaaaatattacacatgtaacctgaaagcacaactgaaaaatattaaactgttatgaaaatctaaaaacataattaactccctgcaattttcttctctgattgcagcttatttgtctggaaatgtgtacatacacctcactgagagatgctgagatgactacagaaattaactttgagaccagaattacagagaagaaaaaccaaaacccaaccctgcatggtcaagtggtgctaacccaagactgtaacagggagaaatgcccagaatcatcaaaatagtgaaagactgatctgttcaaaatatttgctatatgcactgggtataatccgtaatccatacactgccagataatgccatttcaaggaaggatcgaatacttgatggtaaaggccaagtccccctgtattgggaagtgtgtgatttcggcagacctgctgggaaaatttagggtagagcactctttacagaagaactcaaaaacccaatttggataattttcattatctttttagcaaaatggtttcttaatgtttatattttattttcaaggttcattgtttaatgaaatattttattcttgcatttccataaggaaagggaaagtcatgatcatcctaaaggatcacagtttttaaaaggcaaacattttccctaaggaaacagacacaagctttcctagagaatatgatgttttttaggcattaataaggtccttttttataaaggacacttttctcctagtagttttgaattcaggaacagatccaaagttagcagtatatggctgctacatttccattttcattttcgagccatcagtttatgttcagatgccatctctgtaatcgcacatttaaaacataactgtagcctcactaatggaaaagtagtatgatgaacaatcattcccaatggtgtacaatgtaagggttttagggagcaacagtatttaactggaagaaagaattgcatatttaatgtagtctaatatatacacatttgtttaacatgtaaacaaaagtgttaaattcacatatacaacattatacaatttaatcactcttggaataaaatttttatagccttttttctattgggaaaatttgtttagatgtgtgccactccataggtttatttccaaaatgaatgagcccaactccatttgtaaaaacttgtcagttagaattcctttttttagtggattagggctgaattcttagatccttatttcttttcactttaaatgctgccaaagatcactactcatcattcaggaattcgctgtctagcctatctgtagtttcctgaagattgaaaattatgtagactgctatttaaaaatatatttttctaagtgtgaggtttaagatgctgtattgaccctatgagtttttaatgtgttaattatctttatagcataatagatcgctttaggttcctggaatcccatttggtctgacaggatatatgaagattcttaatacctattttctgtgtctaatacttggttaatactaaaaatagaaatgactaaattacatcacagaaagcataaccagtgattgaacctggtagttttaaagctctaaatagctgtggctgaaggactgattatggggctaagaagcttgaaacgtaagttggtacttgttcatcagtggattctcctaaattaagccaaattttgaaatacatgactattaagtttctactcatgtatttacagtcagtcaataaattaaaggaggaaaaaaatccctgaacaacctgcccataaaaagaaaaatactctacatttgagcctgctgcagttttaaattttccctctgggtcaagtttgccagcttttggctacagagaaattatatttccattacagtgcaggtagaaactctgtaaccttaagcatgtaaactacatagaataaaactgtttccactgcatttctgtccttcaaagtggccaacctgattaagtcagccttaatcactgctgctgtcagtttcacgactaaaggtcatattgactaagtagtcatcagctgaccacctcgctgtatcagccagcaacgaggggaaggtgaagaaacatgataggccatatagaatctgccctatgtttacttttttaacccagataattatttttgtgtgcagtatctaagctcctgattgtgtaacctgggacttctggcaccttttgttccattcattttatgtataaaatgcatgccaaagcacactgtgccctctggtacccttgcttccaatcgccaaccatgctcatttccttcctttttttgtggtccctttttgtggtgatcattttaaaccacgtcatccaacaaatgttttatggtcaaccttagcttgttcataagccatagcaactgaaagattaaactcttaaatatgtgtctgggcagtggctattaaatagcaaaaaacaatcagattttagtattttattatttccttgtaaaatggctgaactaaattaaacccttgtttcccatttgttctataatttatagtgaaactgagaacaaaactatctttataaatgatagctaaaagtatttccagatatttaaacaatttaaaataaatttcttctgcagagatgcaaagcatctcaacactggaatgaacaaatgccttaaattcaatggagtaaacctttagaatgaagaggaactgtcatttcacccaagccgaagacaacagccttatgcacttgtgtgctctgtctttgctgcttctcgtgtttcaagcctttcctgtgggatcagcacagcaaagtgcaacttaccaaatggtttaatgactggttaattctttcttctcccaatggaaaagcaatggcaacacaacagtagactgctggcttgacaatcttaaacgtgagcctttgcacatgtaggtttatcatcatttgagtatacgactaagcaagtcaatgaactttttttttttttttagcagtttaatttggtcctgagaatgttgcagtctttattaccccttttgcattaatccacttttctaaccaccttttaagctttaatttttaacactatacaccaagtctttgaaatcagtgatctgttatttaactctaaagcatttgacacttcttgccttaacagttttaaaaaccacacacaaaaaaactctgtaagtaatacagtaggccaaaagtttcatcctatctatcttgcagtttacctatctgatctgatctctgtaattatagttctgtcatttaaaatatactatttaaatctaatttttacatttcaaaaattatcttcagtagtaactaagtatattttctgtggattctgagaatgttatttttcagaatgtgagaatatatatgtacatttataatcttgtgactttaaagtctgttttcagatacagtatgtaaatacttgtaaaaaaatttgtataattttgtgataatgtagtttcccaaaaaaattatttagaaggcattatgttattagtaaatgagagcactgtatagaactgttcctattttctgcacttgccattccagctgcctccactgtccatacccacctcattcatcctgtcacagaaggcaggaaaactgggaactttaccaaagtagcactcagcctgagaggcctgtataatcatgcttttcaaactaaattcacttaaaaattaaaaagcagaattgaatattttaagcagcctcagtacctttggccaatgctgttttcatggtggattatgaacattatataatctttgggaaaagtgaaagtagtacaatttttagaataatgacaactgcctcactgcatctctccactcacacagcaaccgtgtagccccctaagctgcagtaccatgactaaccatgatgtcaatttcatatgctgatcctcacaacagcagtgcacaaacatgccccaaatattttaacagaatttagctcttccttaagctgtcttttcatagtaaaaacaaaacaaaaacacccaatgttaaaaccacataataaacttacaaacttgaaaaattagacacttcagatagataggcaataaaacttcatattatgaaagcaatatattccaagtttcaaagatttgacaagttctgtagagtatctttcatcagtacatgaaaacttccaaactgcatgatcttctgccaggcaggactgggtgctattcgctggtttgaggtcgaatccatttcaaggcatgtcgtggtgggacattaatggtgggatggtagaatgtgcagtccggtcttgtacattgagtgttaaacctacaatgttttggatgatagaagggacattccatcttcttacaagcagggaagtaacggcagagctgactactggaaggtggtgctggtggtgcaactgctggttttggagacagtactggaattcttctactcacatgagtgaagggacaatctggtttagtacactttgcatcatatttacaatttgggtgaacaaacaaacatttttcagcaaatttacaattggggaaggctttgcagggtgagatggggtgatggtaggcacactcatccccatttttacaagcaggccagtacttgcagcgctccaaaagtttttctggtttctgtgccacactcagttcactcatctcagcgttagaaaagctaccatttgggtcctcaagctgcctgctcagcaagtgcaactgctgtgggtggaggagacctctgagtcccttgtttgaggctgcagtttggtttacgggtttcattccttcaaagcacatgtcctcctcttgatctgacatgtatcctggggggctggggacaccatccagcgtcactataaacttgggacttgcaggtttatctggttgtacaagatctcttgactcatctgcagagtttctgccattactgggtcgatttgcagtcgggataataattgcctctgttgagttccttgatttttttctacagaatctccttttgtttcctcttctttaatggggggacttattctgggggtcctactttgtccctggaccacttctgctagcaattcttcttgagaagttcgagttctgggagcaactggaagtgtctgtttctgtggaactgtagagtagttagttgtttttgttacggattcttgagcttcagatatagccttcaaaatcagattcttgttagcttgtttagaaggtggaagagaaggtctcctttcaggctttgcaggcacagacacactgctggagatgcttcctgttcgagacccgtaatcatcatcttcttcctcctcttctccatcatgattgaatttttttactttaacaactgaacttaccacaggcaactttctcttccgaaagttttcatcctccatactcattttctccgagttgtttctaaagaacggactatacgtttcttctaagctgttaagcacctctggttcacacaaacgtcctgtttcatatacccaactactctgcatatcaagctgcttggcagcatgaatactattctgctgctgttgaaattgcaacctgtttaaatgaacaccactatctgcatttctacttgcaggtggtcgataaatttcaatagaagggcgagaagaaccatatgtaagtgtcactgtaggttttttctgagataagggattctcctgcacaaagttgaggtcttcgtcaatgagatcatctggttctggcttaatatcaatcacatcttcagagggtgctggctccctcaaaggtttcactgttgacattagtcgggttgcagctccatcatcgtaagtctgtctgacatttgtggtttttgactcctgcgaacttgtagaaactctggaatctcttttttcaggtctcgcgctaggaatggcaagtggtggcactgcagcttcatgcctcctctcatctccccgactgaaattgctcttgtttgaaggcacgttactatcaaagatgttggtatcagaagacttcagactagagggttcagttgtaacagagcgaagtttatctaatacaccatgaagccatacggtgaatcgaattgtgttgttccctagaaacagggacagatcctctgtcatttggtcctgacttttcttgttggccaccatcaccataatgtaatcaggaagttcttcatcaacataagctcctaattcttgtaatttccccttaatggcactccggatcttgcggctgatctcggtgccgatctccatggctctgcggcgtgcgggaactcagcactgcgcggcgcttggcttacccggaggctgccgcggactcctaccccgcagccgggacaccaccgcctcc

SEQ ID NO: 17239 - RNA, 14310 nt, Homo sapiens
  source 1..14310: mol_type = other RNA
tcaggccaggcacagtggctcacacctgtaatcttatcactttgggaggctgaggcaggtggatcgcttgagcccaggagttcaagaccagcctgggcaacatggtgaaaccccatcgctataaaaaacaacaattagccgggtgtggtggcacatgcctgtagtccctgctactcaggaggctgaggtgggaggatcacttgagcctggggaggtcaaggctttagtgagctgtgatggtgccactgcactccagcctgggtgacagagtgagaccccatttaaaaaacaaaaacaaaaacaaaaaaaaatgtgacatatagttgactaagaagtacatttcaatacaggattgaaagaacccacatatgttaattaaacacaagcgcagaatttgtgccttttacataaaggaagaatgcacataggcatgctttcagacaagcaattcatctagcagaaaaggaaggaatacatttttcagcccttccaggaataaaatccataaatgggctctatttcgtcctccaacacttgtatttcccacgtcatttactcctgcacacccccactcactagaagcctgctaaactgttccagtgagatattttaacacctgatagggaataaatatgcttctgttttggccttcaaaaataagctctgggccagttgcagtggctcacgcctgtaatcccaacactttgggaggccgaggtgggcggatcacgaggtcaggagtttgggatcagcctggccaatatggtgaaactccatctctactaaaaatacaaaaattagccaggcatggtgcctgtaatcccagctacttgggaggctgaaggagaagaatcgcttgaacctgggaggcacaggttgcagtgagccgagatcacaccactgcactccaggccaggtgacagagcgacactctgtctcaaaaaaataaataaatcaactctgtagcatagcatttgtaattctattattttgccttacatttccattatccttttaataaaattgtttttttacatcttcctaatcaagaagtattatgaggccaggcacagtggctcatacctggaatcccagcactttgggaggccgaggcaggcagatcacctgaggtcaaggtatttgagaccagcctggccaacatggtgaaaccccatctctactaaaaatacagaaattagctgggtgtggtggtgcacacctgtaatgctagctactcgggaggctgaggtaggagaatcgcttgaacctgggaggcagaggttgcaataagcctagatcatgccactgcactcaagcctgggagacagagcgagactacatcttaaaaaaaaaaaaaaaagtattatgagagaggataatgtattgtaatgtattgtagaggctaaataaaattatgctcatgtcagaaaaaaagagtatttctcaaaataaaattcactgaaactggatgtttattttgactgagatatagtatatcctcaaattgccatagaaagtttacaagaatattagaggtaaattataaatatcagggcctttttaaaaaaaaaagattctgcttataacttggtatttgtttataataaaaattatagtagccaataatgaacacttactctggcttggttatttacttaggtcaaaagaaggaggagcggttaaactgtgggatcaggaactgaggcggtgccgtgccttcaggcttgagacaggacaagccacagattgtgttcgttctgtgtgcagaggcaaagtaagatgttccatgagctgatacagtgcagcagaaaacagaaagtggttattactgtgattccctcaccctttgcagcctaatgaacaatacttaataatgcataacgatggatttgcttgccaacattactctgtctttgctgctttctttgccaaagttagcaccagtgtggtgcataagctaggaagctattctgtctaaatactgtatgtaaacctccaatattttctagaatctgccaatttaacaactctagtagacataattgaaagcccttggcagttgactcatattaggacagctgtctccattttttaaaaaaacacacattccctagataaaacgtgcagtaaacaaacaatgaaatactactcagccataaaaaataatgaaattctgtcattcttggtggcaacatggatgagactggaggacatgatgtgaagtgaaataagccaggcacagaaagataaatacatgttctcactcctgtgcagaaactaaaaaagttgatcccacagaggtggagagtagaatagtggttactggaggcggacaagggggagggggagggggatagggaaggactggttaaaggatacaagtttacacagccagataggaatagtatgttttagtattctgtagtactgtaggatgactatagttaagaatcacgtatttatgtattttcaggtatttacaagagaggattttgaaagtttccatcacaaagaaatgataaatgtctgaggtgatggttatgcgtattaccctatgccctatagatatgtataattatgtgtcaatttcaaaataaaaattcaaaactacaactcctatgaaaatttttgagcgtgtttgtacttattaagtgtatttataaatcatacggatattatcttcagcctgcatattaaattgtagttaagcttttactttttaactaaaaaataaattctattattttttcctatatcccactgcactgaccccagtttggaaatcctaagattatcaaataaaaactttgattattgaagaatccaggtgtactgccacagaaaagttctattctgtagcatggactctaatatgtaatctagcccattgtgcttacagatagatgtgtgcctgtagtcatagaaaaatttgcatgagctaatgactgccttgctactagattagctcaaagcaaaaagttctctgaaagcaggtcaatagggtcatttttatattatgaagaagaaaagcagctgttgtattacattcactgtattggtcctgcttgtgtttcagggcaagatccttgttgggacaaggaatgctgaaataatcgaagttggagagaaaaatgcagcttgtaatattttagttaacggtcatgtggatgggccaatctggggactagcaacacatccttccagggattttttcctttctgctgcagaagatgggacagtgagactttgggatattgctgataaagtaagtacagataatttttttaaaagaggttacaacttctaaaaagaaaagttggaagttctaaattgctagtacttaaagaactgccagaattctgttgagcattttgaggggaaactggtataatttagaagtacttcacttaatgtttcctatgactctttttttttttttttttaaatgcagaagatgttaaacaaagtgaatttgggacatgctgctcgtactgtgtgttacagccctgaaggggacatggtggctattggaatgaaaaatggagaatttatcattttactagtgagttctctaaaaatatggggaaagaagagagacaggagatgtgcaatccatgatatcaggttagtgaacaaatggaatagagtttctagtatatacttgatttaacttccatttgtaaaattttccatagccttgccttcaaaaagaggtccccagggcctgtagcatttcccgtattataaattgtatgctaaaatatggctgtttgtatactacttaattcttcttgctaaattataaacccactgggcaccaactataatagcaagtactagtaggtaatgtttgatgaattcatgttaacacttagccatgtccattaagttcatcccaccaagaggtatctcccactgtaatacaagagagctatctgcccttcaaaagttgtcaccctggaaaactaaagttgtgatttcaaacatatcttctcttagtaacctcagtttgggaatatgtagttcattaatttaatcaatacctattgattaaatgttccagaatccaaattaatttaaatgtttcttaaacctttgtttttcagtgcttaagcatttttcaacagtggctaccatttacggagtacttccgtgtgatcagtagataagattattgaatctaggtctgtcaaaagcttgtacacttttcatcagtaaaatccttttacaaatgaaaccttcctcagaacttcaatatataaaatagtaacagtggcttcccttagcttttacatgtctctatcgtacctcagtaagactcatgggccatttcaagagactgaattgtcccatatgactccaaagattgctaggcaaatagcatttcactttgtcttttaaataagttcttcaggccgggcgcggtggctcatgcctgtaatcccagcactttgggaggccgaggcaggcagatcacctgaagtcaggagtactcgaccagcctggccaacatagtgaaaccccatctcaactaaaaatacaaaaatcagccgggcgtggtggcaggcgcctgtaatcccagctactcagggggctgaaacaggagaatcgcttgaacccgggaggcggaggttgcgccatcgcactccagcctgggagacaagagcgagacttcgtctcaaaaaaaaaaaattcttcttccaagattcaagttgtgtcatttcaccttaataactggaggttagttaagctgggctgtgttctttgcttaatattaagacaacgttttttccagatggaagaaaactatcttaatgaattgttagcttattaattatgtaatgctaatggcttttaaaagctgagatgttctgactgggtgttgtggctcacacctgtaatcccagtaccttgggaggccaagggggaaggattgcttgaggccaggagtttgggaccatagtgagaccccgcctctatttaaaaaattaaattttgttttgttttgttttgagttggagttttgctcttgttgcccatgctgaagtgcaatggtgcaatctcagctcaccacaacctgtgcctcctgggttcaagcgattctcctgcttcagcctcccgagtagatgggattacaggcgtgcaccaccatgcctggctaattttgtatttttagtagagacagggtttctctatgttggtcaggctggtctcaaactctcgacctcaggtgatctgcccgcctccgcttcccaaagttctgggattataggtgtgagccactgggcctggcctaagaaagtttttttaagccattagacgtttttaaaggaattgggagatgacaattggggaaatatttaaaatttaagtaaaatataaagcttccttatttcatgtaacccagacaatctcagtatacatgatcagttgtgtctgacaggtaaatctatttgaggccttatcacacgttacttttaagaactagaaaggaaaagtcactgatcttaagtatttataatacttcatgtggtctaatactttttacgttttgttttgattcagatttagtccggattcccggtatctggcagtaggttctagtgagaactcagtggatttttatgacctaacgctgggccccactcttaacagaatcagctactgcaaagacattccaagctttgtcattcaaatggacttctctgcagatagcagttatctccaggtacagtaccaatactgtatacccaggtggcaagttcttctgcttttacatttcgtgttagtgaatgcatttaaagttcctgagctccagagctccagcttctcaactcctccctttgtaccttctgacctacagctcccctttcctcccccacttatcagagcttttctcctattaagtttttgtagtgatcttttgcatacttaataatgttagacatgtaaatcaagtagcaatatgctagtattctgtaaaccccctgtggattttgtctctcacctaatggaattcttgtcccattttaatctgatgaaaaaggtctctagtggctgctataaacggcatgtctatgaagtgccttcaggaaaacatcttatggatcatgccgctattgacagaattacttgggctacatggactaggtaaatacttatatattcacaaggcaagaactgactttgaaggccagttagaaaatcctatttctgaactgttagagccattccaataaggaatagtaattgagtttcaagtttttgttaccatattttgaaatggtatgttcatgttgggacccctttttattgaatatatttccatgttttatcagtttccatgatttatcaagttttttttttaaggaaatcaaagttttaactttaaagataccctgatatttttcttaatgctaaatttaatgactggcaaaaaggtattgggtgctgttaagcaactgttattaattctctatctaaaggaatgctatcttgaatctattagaagtcaaagcttccaaatttgttcaaatttcctggctgtatgacaggtaaccatgactatccatttttttggccaatgaaaaatgccatcaaattcctgtatcagccaggcatatagtggctcatgcctgtaatctctgatgtagcaggccgaggtgggaggatcacttgagcctagaagttttgataccagcctgggcaacatagcaagaccccatctctgaaatttttttaattcctatgtcataagtcatttttatttttgtagagatagggatctcacaatattgcccaggctggtctcaaactcttggcctcaagcagtcctcctgcctcagcctcccaaaatgttgggattactggtatgtgctgctggacccagccaagtagcacttttaatttgaaaaatagttctatcagttttcagtcaggcgcggtggctcagcctgtaatcccagcactttgggaggccgagcgggggtgatcacctgaggtcgggagttcgagactagcctgaccaacatggagaaaccctgtctctactaaaaatacaaaataagccgggcatgttagcgcatgcctgtgatcccagctactcgggaggctgaggcaggagaattgcttgaacccaggaggcagaggttgcggtgagccgagatcatgccattgcactccagcctgggtaacaagagcgaaaactccgtctcaaaaaaaaaaaaagaaaaaatagttctatcagttttcataaagtactactttaatcttaaaaagattaatctagaaacccttcaaattataaaatgtcatttttaaaaggcaggagttgatatcctgatgaaattcaggtctccaaacaacttaccataatttacttcctgtattttaagtaacatgatagggtacttagagattaattgccaagaaactttttgaatatagtcaacctgcccgcacttgccatgatgagttttcttttgttccttccctctagtattctaggagatgaggttttgggaatctggtccagacatgctgagaaagctgatgtcaactgtgcctgtgtatctcattcaggaatcagtcttgttacaggagatgactttggcatggttaagttatttgacttcccatgtccagaaaaatttgtaagtttgtgttttgtttactattatcagtttactcctaattttgatgtcttatcatcagcacttttccccatatatttaaaatgttttgtcctaatttctaaatttttccccaaactttctaaatctatttactttgaaataaaagctattagaaacaaatcctctccctcgagtaataccatctttggaaccatcctacaaaagctgtaattagcttttcaccaaacctataatcagttatcaaatttcaaatgcttttccttagagaaaaatggtcagagtacctggagacatctgactgcccacacagcctggttttgcagatccactactcatgctgaaaagcattctaatcactggctgcggtgctaactccctactctctccacagctcttgtcatagagattatagttcctaataagagcctttgacttctgtgtgcaccaaatgccctgagcttgtctgtcattgttttttaggcaaaacacaaaaggttcttgggtcattcgccccatgtgacaaatattcgatttaccagtggtgatcgacatgttgttagtgctggaggtgatgactgcaggttagtaactttctcagcccatgaagagcagactatgttactagttaagagacttaatacaacaactcctacagctttggtttatgaaatcagctagtcaacattagtagaaggtagtataaccagatggctcttcagaatctcatatttatgcaaatacagaataaaaggagttaaagaggaaaaatattacacatgtaacctgaaagcacaactgaaaaatattaaactgttatgaaaatctaaaaacataattaactccctgcaattttcttctctgattgcagcttatttgtctggaaatgtgtacatacacctcactgagagatgctgagatgactacagaaattaactttgagaccagaattacagagaagaaaaaccaaaacccaaccctgcatggtcaagtggtgctaacccaagactgtaacagggagaaatgcccagaatcatcaaaatagtgaaagactgatctgttcaaaatatttgctatatgcactgggtataatccgtaatccatacactgccagataatgccatttcaaggaaggatcgaatacttgatggtaaaggccaagtccccctgtattgggaagtgtgtgatttcggcagacctgctgggaaaatttagggtagagcactctttacagaagaactcaaaaacccaatttggataattttcattatctttttagcaaaatggtttcttaatgtttatattttattttcaaggttcattgtttaatgaaatattttattcttgcatttccataaggaaagggaaagtcatgatcatcctaaaggatcacagtttttaaaaggcaaacattttccctaaggaaacagacacaagctttcctagagaatatgatgttttttaggcattaataaggtccttttttataaaggacacttttctcctagtagttttgaattcaggaacagatccaaagttagcagtatatggctgctacatttccattttcattttcgagccatcagtttatgttcagatgccatctctgtaatcgcacatttaaaacataactgtagcctcactaatggaaaagtagtatgatgaacaatcattcccaatggtgtacaatgtaagggttttagggagcaacagtatttaactggaagaaagaattgcatatttaatgtagtctaatatatacacatttgtttaacatgtaaacaaaagtgttaaattcacatatacaacattatacaatttaatcactcttggaataaaatttttatagccttttttctattgggaaaatttgtttagatgtgtgccactccataggtttatttccaaaatgaatgagcccaactccatttgtaaaaacttgtcagttagaattcctttttttagtggattagggctgaattcttagatccttatttcttttcactttaaatgctgccaaagatcactactcatcattcaggaattcgctgtctagcctatctgtagtttcctgaagattgaaaattatgtagactgctatttaaaaatatatttttctaagtgtgaggtttaagatgctgtattgaccctatgagtttttaatgtgttaattatctttatagcataatagatcgctttaggttcctggaatcccatttggtctgacaggatatatgaagattcttaatacctattttctgtgtctaatacttggttaatactaaaaatagaaatgactaaattacatcacagaaagcataaccagtgattgaacctggtagttttaaagctctaaatagctgtggctgaaggactgattatggggctaagaagcttgaaacgtaagttggtacttgttcatcagtggattctcctaaattaagccaaattttgaaatacatgactattaagtttctactcatgtatttacagtcagtcaataaattaaaggaggaaaaaaatccctgaacaacctgcccataaaaagaaaaatactctacatttgagcctgctgcagttttaaattttccctctgggtcaagtttgccagcttttggctacagagaaattatatttccattacagtgcaggtagaaactctgtaaccttaagcatgtaaactacatagaataaaactgtttccactgcatttctgtccttcaaagtggccaacctgattaagtcagccttaatcactgctgctgtcagtttcacgactaaaggtcatattgactaagtagtcatcagctgaccacctcgctgtatcagccagcaacgaggggaaggtgaagaaacatgataggccatatagaatctgccctatgtttacttttttaacccagataattatttttgtgtgcagtatctaagctcctgattgtgtaacctgggacttctggcaccttttgttccattcattttatgtataaaatgcatgccaaagcacactgtgccctctggtacccttgcttccaatcgccaaccatgctcatttccttcctttttttgtggtccctttttgtggtgatcattttaaaccacgtcatccaacaaatgttttatggtcaaccttagcttgttcataagccatagcaactgaaagattaaactcttaaatatgtgtctgggcagtggctattaaatagcaaaaaacaatcagattttagtattttattatttccttgtaaaatggctgaactaaattaaacccttgtttcccatttgttctataatttatagtgaaactgagaacaaaactatctttataaatgatagctaaaagtatttccagatatttaaacaatttaaaataaatttcttctgcagagatgcaaagcatctcaacactggaatgaacaaatgccttaaattcaatggagtaaacctttagaatgaagaggaactgtcatttcacccaagccgaagacaacagccttatgcacttgtgtgctctgtctttgctgcttctcgtgtttcaagcctttcctgtgggatcagcacagcaaagtgcaacttaccaaatggtttaatgactggttaattctttcttctcccaatggaaaagcaatggcaacacaacagtagactgctggcttgacaatcttaaacgtgagcctttgcacatgtaggtttatcatcatttgagtatacgactaagcaagtcaatgaactttttttttttttttagcagtttaatttggtcctgagaatgttgcagtctttattaccccttttgcattaatccacttttctaaccaccttttaagctttaatttttaacactatacaccaagtctttgaaatcagtgatctgttatttaactctaaagcatttgacacttcttgccttaacagttttaaaaaccacacacaaaaaaactctgtaagtaatacagtaggccaaaagtttcatcctatctatcttgcagtttacctatctgatctgatctctgtaattatagttctgtcatttaaaatatactatttaaatctaatttttacatttcaaaaattatcttcagtagtaactaagtatattttctgtggattctgagaatgttatttttcagaatgtgagaatatatatgtacatttataatcttgtgactttaaagtctgttttcagatacagtatgtaaatacttgtaaaaaaatttgtataattttgtgataatgtagtttcccaaaaaaattatttagaaggcattatgttattagtaaatgagagcactgtatagaactgttcctattttctgcacttgccattccagctgcctccactgtccatacccacctcattcatcctgtcacagaaggcaggaaaactgggaactttaccaaagtagcactcagcctgagaggcctgtataatcatgcttttcaaactaaattcacttaaaaattaaaaagcagaattgaatattttaagcagcctcagtacctttggccaatgctgttttcatggtggattatgaacattatataatctttgggaaaagtgaaagtagtacaatttttagaataatgacaactgcctcactgcatctctccactcacacagcaaccgtgtagccccctaagctgcagtaccatgactaaccatgatgtcaatttcatatgctgatcctcacaacagcagtgcacaaacatgccccaaatattttaacagaatttagctcttccttaagctgtcttttcatagtaaaaacaaaacaaaaacacccaatgttaaaaccacataataaacttacaaacttgaaaaattagacacttcagatagataggcaataaaacttcatattatgaaagcaatatattccaagtttcaaagatttgacaagttctgtagagtatctttcatcagtacatgaaaacttccaaactgcatgatcttctgccaggcaggactgggtgctattcgctggtttgaggtcgaatccatttcaaggcatgtcgtggtgggacattaatggtgggatggtagaatgtgcagtccggtcttgtacattgagtgttaaacctacaatgttttggatgatagaagggacattccatcttcttacaagcagggaagtaacggcagagctgactactggaaggtggtgctggtggtgcaactgctggttttggagacagtactggaattcttctactcacatgagtgaagggacaatctggtttagtacactttgcatcatatttacaatttgggtgaacaaacaaacatttttcagcaaatttacaattggggaaggctttgcagggtgagatggggtgatggtaggcacactcatccccatttttacaagcaggccagtacttgcagcgctccaaaagtttttctggtttctgtgccacactcagttcactcatctcagctgtagagtagttagttgtttttgttacggattcttgagcttcagatatagccttcaaaatcagattcttgttagcttgtttagaaggtggaagagaaggtctcctttcaggctttgcaggcacagacacactgctggagatgcttcctgttcgagacccgtaatcatcatcttcttcctcctcttctccatcatgattgaatttttttactttaacaactgaacttaccacaggcaactttctcttccgaaagttttcatcctccatactcattttctccgagttgtttctaaagaacggactatacgtttcttctaagctgttaagcacctctggttcacacaaacgtcctgtttcatatacccaactactctgcatatcaagctgcttggcagcatgaatactattctgctgctgttgaaattgcaacctgtttaaatgaacaccactatctgcatttctacttgcaggtggtcgataaatttcaatagaagggcgagaagaaccatatgtaagtgtcactgtaggttttttctgagataagggattctcctgcacaaagttgaggtcttcgtcaatgagatcatctggttctggcttaatatcaatcacatcttcagagggtgctggctccctcaaaggtttcactgttgacattagtcgggttgcagctccatcatcgtaagtctgtctgacatttgtggtttttgactcctgcgaacttgtagaaactctggaatctcttttttcaggtctcgcgctaggaatggcaagtggtggcactgcagcttcatgcctcctctcatctccccgactgaaattgctcttgtttgaaggcacgttactatcaaagatgttggtatcagaagacttcagactagagggttcagttgtaacagagcgaagtttatctaatacaccatgaagccatacggtgaatcgaattgtgttgttccctagaaacagggacagatcctctgtcatttggtcctgacttttcttgttggccaccatcaccataatgtaatcaggaagttcttcatcaacataagctcctaattcttgtaatttccccttaatggcactccggatcttgcggctgatctcggtgccgatctccatggctctgcggcgtgcgggaactcagcactgcgcggcgcttggcttacccggaggctgccgcggactcctaccccgcagccgggacaccaccgcctcc

SEQ ID NO: 17240 - RNA, 14426 nt, Homo sapiens
  source 1..14426: mol_type = other RNA
tcaggccaggcacagtggctcacacctgtaatcttatcactttgggaggctgaggcaggtggatcgcttgagcccaggagttcaagaccagcctgggcaacatggtgaaaccccatcgctataaaaaacaacaattagccgggtgtggtggcacatgcctgtagtccctgctactcaggaggctgaggtgggaggatcacttgagcctggggaggtcaaggctttagtgagctgtgatggtgccactgcactccagcctgggtgacagagtgagaccccatttaaaaaacaaaaacaaaaacaaaaaaaaatgtgacatatagttgactaagaagtacatttcaatacaggattgaaagaacccacatatgttaattaaacacaagcgcagaatttgtgccttttacataaaggaagaatgcacataggcatgctttcagacaagcaattcatctagcagaaaaggaaggaatacatttttcagcccttccaggaataaaatccataaatgggctctatttcgtcctccaacacttgtatttcccacgtcatttactcctgcacacccccactcactagaagcctgctaaactgttccagtgagatattttaacacctgatagggaataaatatgcttctgttttggccttcaaaaataagctctgggccagttgcagtggctcacgcctgtaatcccaacactttgggaggccgaggtgggcggatcacgaggtcaggagtttgggatcagcctggccaatatggtgaaactccatctctactaaaaatacaaaaattagccaggcatggtgcctgtaatcccagctacttgggaggctgaaggagaagaatcgcttgaacctgggaggcacaggttgcagtgagccgagatcacaccactgcactccaggccaggtgacagagcgacactctgtctcaaaaaaataaataaatcaactctgtagcatagcatttgtaattctattattttgccttacatttccattatccttttaataaaattgtttttttacatcttcctaatcaagaagtattatgaggccaggcacagtggctcatacctggaatcccagcactttgggaggccgaggcaggcagatcacctgaggtcaaggtatttgagaccagcctggccaacatggtgaaaccccatctctactaaaaatacagaaattagctgggtgtggtggtgcacacctgtaatgctagctactcgggaggctgaggtaggagaatcgcttgaacctgggaggcagaggttgcaataagcctagatcatgccactgcactcaagcctgggagacagagcgagactacatcttaaaaaaaaaaaaaaaagtattatgagagaggataatgtattgtaatgtattgtagaggctaaataaaattatgctcatgtcagaaaaaaagagtatttctcaaaataaaattcactgaaactggatgtttattttgactgagatatagtatatcctcaaattgccatagaaagtttacaagaatattagaggtaaattataaatatcagggcctttttaaaaaaaaaagattctgcttataacttggtatttgtttataataaaaattatagtagccaataatgaacacttactctggcttggttatttacttaggtcaaaagaaggaggagcggttaaactgtgggatcaggaactgaggcggtgccgtgccttcaggcttgagacaggacaagccacagattgtgttcgttctgtgtgcagaggcaaagtaagatgttccatgagctgatacagtgcagcagaaaacagaaagtggttattactgtgattccctcaccctttgcagcctaatgaacaatacttaataatgcataacgatggatttgcttgccaacattactctgtctttgctgctttctttgccaaagttagcaccagtgtggtgcataagctaggaagctattctgtctaaatactgtatgtaaacctccaatattttctagaatctgccaatttaacaactctagtagacataattgaaagcccttggcagttgactcatattaggacagctgtctccattttttaaaaaaacacacattccctagataaaacgtgcagtaaacaaacaatgaaatactactcagccataaaaaataatgaaattctgtcattcttggtggcaacatggatgagactggaggacatgatgtgaagtgaaataagccaggcacagaaagataaatacatgttctcactcctgtgcagaaactaaaaaagttgatcccacagaggtggagagtagaatagtggttactggaggcggacaagggggagggggagggggatagggaaggactggttaaaggatacaagtttacacagccagataggaatagtatgttttagtattctgtagtactgtaggatgactatagttaagaatcacgtatttatgtattttcaggtatttacaagagaggattttgaaagtttccatcacaaagaaatgataaatgtctgaggtgatggttatgcgtattaccctatgccctatagatatgtataattatgtgtcaatttcaaaataaaaattcaaaactacaactcctatgaaaatttttgagcgtgtttgtacttattaagtgtatttataaatcatacggatattatcttcagcctgcatattaaattgtagttaagcttttactttttaactaaaaaataaattctattattttttcctatatcccactgcactgaccccagtttggaaatcctaagattatcaaataaaaactttgattattgaagaatccaggtgtactgccacagaaaagttctattctgtagcatggactctaatatgtaatctagcccattgtgcttacagatagatgtgtgcctgtagtcatagaaaaatttgcatgagctaatgactgccttgctactagattagctcaaagcaaaaagttctctgaaagcaggtcaatagggtcatttttatattatgaagaagaaaagcagctgttgtattacattcactgtattggtcctgcttgtgtttcagggcaagatccttgttgggacaaggaatgctgaaataatcgaagttggagagaaaaatgcagcttgtaatattttagttaacggtcatgtggatgggccaatctggggactagcaacacatccttccagggattttttcctttctgctgcagaagatgggacagtgagactttgggatattgctgataaagtaagtacagataatttttttaaaagaggttacaacttctaaaaagaaaagttggaagttctaaattgctagtacttaaagaactgccagaattctgttgagcattttgaggggaaactggtataatttagaagtacttcacttaatgtttcctatgactctttttttttttttttttaaatgcagaagatgttaaacaaagtgaatttgggacatgctgctcgtactgtgtgttacagccctgaaggggacatggtggctattggaatgaaaaatggagaatttatcattttactagtgagttctctaaaaatatggggaaagaagagagacaggagatgtgcaatccatgatatcaggttagtgaacaaatggaatagagtttctagtatatacttgatttaacttccatttgtaaaattttccatagccttgccttcaaaaagaggtccccagggcctgtagcatttcccgtattataaattgtatgctaaaatatggctgtttgtatactacttaattcttcttgctaaattataaacccactgggcaccaactataatagcaagtactagtaggtaatgtttgatgaattcatgttaacacttagccatgtccattaagttcatcccaccaagaggtatctcccactgtaatacaagagagctatctgcccttcaaaagttgtcaccctggaaaactaaagttgtgatttcaaacatatcttctcttagtaacctcagtttgggaatatgtagttcattaatttaatcaatacctattgattaaatgttccagaatccaaattaatttaaatgtttcttaaacctttgtttttcagtgcttaagcatttttcaacagtggctaccatttacggagtacttccgtgtgatcagtagataagattattgaatctaggtctgtcaaaagcttgtacacttttcatcagtaaaatccttttacaaatgaaaccttcctcagaacttcaatatataaaatagtaacagtggcttcccttagcttttacatgtctctatcgtacctcagtaagactcatgggccatttcaagagactgaattgtcccatatgactccaaagattgctaggcaaatagcatttcactttgtcttttaaataagttcttcaggccgggcgcggtggctcatgcctgtaatcccagcactttgggaggccgaggcaggcagatcacctgaagtcaggagtactcgaccagcctggccaacatagtgaaaccccatctcaactaaaaatacaaaaatcagccgggcgtggtggcaggcgcctgtaatcccagctactcagggggctgaaacaggagaatcgcttgaacccgggaggcggaggttgcgccatcgcactccagcctgggagacaagagcgagacttcgtctcaaaaaaaaaaaattcttcttccaagattcaagttgtgtcatttcaccttaataactggaggttagttaagctgggctgtgttctttgcttaatattaagacaacgttttttccagatggaagaaaactatcttaatgaattgttagcttattaattatgtaatgctaatggcttttaaaagctgagatgttctgactgggtgttgtggctcacacctgtaatcccagtaccttgggaggccaagggggaaggattgcttgaggccaggagtttgggaccatagtgagaccccgcctctatttaaaaaattaaattttgttttgttttgttttgagttggagttttgctcttgttgcccatgctgaagtgcaatggtgcaatctcagctcaccacaacctgtgcctcctgggttcaagcgattctcctgcttcagcctcccgagtagatgggattacaggcgtgcaccaccatgcctggctaattttgtatttttagtagagacagggtttctctatgttggtcaggctggtctcaaactctcgacctcaggtgatctgcccgcctccgcttcccaaagttctgggattataggtgtgagccactgggcctggcctaagaaagtttttttaagccattagacgtttttaaaggaattgggagatgacaattggggaaatatttaaaatttaagtaaaatataaagcttccttatttcatgtaacccagacaatctcagtatacatgatcagttgtgtctgacaggtaaatctatttgaggccttatcacacgttacttttaagaactagaaaggaaaagtcactgatcttaagtatttataatacttcatgtggtctaatactttttacgttttgttttgattcagatttagtccggattcccggtatctggcagtaggttctagtgagaactcagtggatttttatgacctaacgctgggccccactcttaacagaatcagctactgcaaagacattccaagctttgtcattcaaatggacttctctgcagatagcagttatctccaggtacagtaccaatactgtatacccaggtggcaagttcttctgcttttacatttcgtgttagtgaatgcatttaaagttcctgagctccagagctccagcttctcaactcctccctttgtaccttctgacctacagctcccctttcctcccccacttatcagagcttttctcctattaagtttttgtagtgatcttttgcatacttaataatgttagacatgtaaatcaagtagcaatatgctagtattctgtaaaccccctgtggattttgtctctcacctaatggaattcttgtcccattttaatctgatgaaaaaggtctctagtggctgctataaacggcatgtctatgaagtgccttcaggaaaacatcttatggatcatgccgctattgacagaattacttgggctacatggactaggtaaatacttatatattcacaaggcaagaactgactttgaaggccagttagaaaatcctatttctgaactgttagagccattccaataaggaatagtaattgagtttcaagtttttgttaccatattttgaaatggtatgttcatgttgggacccctttttattgaatatatttccatgttttatcagtttccatgatttatcaagttttttttttaaggaaatcaaagttttaactttaaagataccctgatatttttcttaatgctaaatttaatgactggcaaaaaggtattgggtgctgttaagcaactgttattaattctctatctaaaggaatgctatcttgaatctattagaagtcaaagcttccaaatttgttcaaatttcctggctgtatgacaggtaaccatgactatccatttttttggccaatgaaaaatgccatcaaattcctgtatcagccaggcatatagtggctcatgcctgtaatctctgatgtagcaggccgaggtgggaggatcacttgagcctagaagttttgataccagcctgggcaacatagcaagaccccatctctgaaatttttttaattcctatgtcataagtcatttttatttttgtagagatagggatctcacaatattgcccaggctggtctcaaactcttggcctcaagcagtcctcctgcctcagcctcccaaaatgttgggattactggtatgtgctgctggacccagccaagtagcacttttaatttgaaaaatagttctatcagttttcagtcaggcgcggtggctcagcctgtaatcccagcactttgggaggccgagcgggggtgatcacctgaggtcgggagttcgagactagcctgaccaacatggagaaaccctgtctctactaaaaatacaaaataagccgggcatgttagcgcatgcctgtgatcccagctactcgggaggctgaggcaggagaattgcttgaacccaggaggcagaggttgcggtgagccgagatcatgccattgcactccagcctgggtaacaagagcgaaaactccgtctcaaaaaaaaaaaaagaaaaaatagttctatcagttttcataaagtactactttaatcttaaaaagattaatctagaaacccttcaaattataaaatgtcatttttaaaaggcaggagttgatatcctgatgaaattcaggtctccaaacaacttaccataatttacttcctgtattttaagtaacatgatagggtacttagagattaattgccaagaaactttttgaatatagtcaacctgcccgcacttgccatgatgagttttcttttgttccttccctctagtattctaggagatgaggttttgggaatctggtccagacatgctgagaaagctgatgtcaactgtgcctgtgtatctcattcaggaatcagtcttgttacaggagatgactttggcatggttaagttatttgacttcccatgtccagaaaaatttgtaagtttgtgttttgtttactattatcagtttactcctaattttgatgtcttatcatcagcacttttccccatatatttaaaatgttttgtcctaatttctaaatttttccccaaactttctaaatctatttactttgaaataaaagctattagaaacaaatcctctccctcgagtaataccatctttggaaccatcctacaaaagctgtaattagcttttcaccaaacctataatcagttatcaaatttcaaatgcttttccttagagaaaaatggtcagagtacctggagacatctgactgcccacacagcctggttttgcagatccactactcatgctgaaaagcattctaatcactggctgcggtgctaactccctactctctccacagctcttgtcatagagattatagttcctaataagagcctttgacttctgtgtgcaccaaatgccctgagcttgtctgtcattgttttttaggcaaaacacaaaaggttcttgggtcattcgccccatgtgacaaatattcgatttaccagtggtgatcgacatgttgttagtgctggaggtgatgactgcaggttagtaactttctcagcccatgaagagcagactatgttactagttaagagacttaatacaacaactcctacagctttggtttatgaaatcagctagtcaacattagtagaaggtagtataaccagatggctcttcagaatctcatatttatgcaaatacagaataaaaggagttaaagaggaaaaatattacacatgtaacctgaaagcacaactgaaaaatattaaactgttatgaaaatctaaaaacataattaactccctgcaattttcttctctgattgcagcttatttgtctggaaatgtgtacatacacctcactgagagatgctgagatgactacagaaattaactttgagaccagaattacagagaagaaaaaccaaaacccaaccctgcatggtcaagtggtgctaacccaagactgtaacagggagaaatgcccagaatcatcaaaatagtgaaagactgatctgttcaaaatatttgctatatgcactgggtataatccgtaatccatacactgccagataatgccatttcaaggaaggatcgaatacttgatggtaaaggccaagtccccctgtattgggaagtgtgtgatttcggcagacctgctgggaaaatttagggtagagcactctttacagaagaactcaaaaacccaatttggataattttcattatctttttagcaaaatggtttcttaatgtttatattttattttcaaggttcattgtttaatgaaatattttattcttgcatttccataaggaaagggaaagtcatgatcatcctaaaggatcacagtttttaaaaggcaaacattttccctaaggaaacagacacaagctttcctagagaatatgatgttttttaggcattaataaggtccttttttataaaggacacttttctcctagtagttttgaattcaggaacagatccaaagttagcagtatatggctgctacatttccattttcattttcgagccatcagtttatgttcagatgccatctctgtaatcgcacatttaaaacataactgtagcctcactaatggaaaagtagtatgatgaacaatcattcccaatggtgtacaatgtaagggttttagggagcaacagtatttaactggaagaaagaattgcatatttaatgtagtctaatatatacacatttgtttaacatgtaaacaaaagtgttaaattcacatatacaacattatacaatttaatcactcttggaataaaatttttatagccttttttctattgggaaaatttgtttagatgtgtgccactccataggtttatttccaaaatgaatgagcccaactccatttgtaaaaacttgtcagttagaattcctttttttagtggattagggctgaattcttagatccttatttcttttcactttaaatgctgccaaagatcactactcatcattcaggaattcgctgtctagcctatctgtagtttcctgaagattgaaaattatgtagactgctatttaaaaatatatttttctaagtgtgaggtttaagatgctgtattgaccctatgagtttttaatgtgttaattatctttatagcataatagatcgctttaggttcctggaatcccatttggtctgacaggatatatgaagattcttaatacctattttctgtgtctaatacttggttaatactaaaaatagaaatgactaaattacatcacagaaagcataaccagtgattgaacctggtagttttaaagctctaaatagctgtggctgaaggactgattatggggctaagaagcttgaaacgtaagttggtacttgttcatcagtggattctcctaaattaagccaaattttgaaatacatgactattaagtttctactcatgtatttacagtcagtcaataaattaaaggaggaaaaaaatccctgaacaacctgcccataaaaagaaaaatactctacatttgagcctgctgcagttttaaattttccctctgggtcaagtttgccagcttttggctacagagaaattatatttccattacagtgcaggtagaaactctgtaaccttaagcatgtaaactacatagaataaaactgtttccactgcatttctgtccttcaaagtggccaacctgattaagtcagccttaatcactgctgctgtcagtttcacgactaaaggtcatattgactaagtagtcatcagctgaccacctcgctgtatcagccagcaacgaggggaaggtgaagaaacatgataggccatatagaatctgccctatgtttacttttttaacccagataattatttttgtgtgcagtatctaagctcctgattgtgtaacctgggacttctggcaccttttgttccattcattttatgtataaaatgcatgccaaagcacactgtgccctctggtacccttgcttccaatcgccaaccatgctcatttccttcctttttttgtggtccctttttgtggtgatcattttaaaccacgtcatccaacaaatgttttatggtcaaccttagcttgttcataagccatagcaactgaaagattaaactcttaaatatgtgtctgggcagtggctattaaatagcaaaaaacaatcagattttagtattttattatttccttgtaaaatggctgaactaaattaaacccttgtttcccatttgttctataatttatagtgaaactgagaacaaaactatctttataaatgatagctaaaagtatttccagatatttaaacaatttaaaataaatttcttctgcagagatgcaaagcatctcaacactggaatgaacaaatgccttaaattcaatggagtaaacctttagaatgaagaggaactgtcatttcacccaagccgaagacaacagccttatgcacttgtgtgctctgtctttgctgcttctcgtgtttcaagcctttcctgtgggatcagcacagcaaagtgcaacttaccaaatggtttaatgactggttaattctttcttctcccaatggaaaagcaatggcaacacaacagtagactgctggcttgacaatcttaaacgtgagcctttgcacatgtaggtttatcatcatttgagtatacgactaagcaagtcaatgaactttttttttttttttagcagtttaatttggtcctgagaatgttgcagtctttattaccccttttgcattaatccacttttctaaccaccttttaagctttaatttttaacactatacaccaagtctttgaaatcagtgatctgttatttaactctaaagcatttgacacttcttgccttaacagttttaaaaaccacacacaaaaaaactctgtaagtaatacagtaggccaaaagtttcatcctatctatcttgcagtttacctatctgatctgatctctgtaattatagttctgtcatttaaaatatactatttaaatctaatttttacatttcaaaaattatcttcagtagtaactaagtatattttctgtggattctgagaatgttatttttcagaatgtgagaatatatatgtacatttataatcttgtgactttaaagtctgttttcagatacagtatgtaaatacttgtaaaaaaatttgtataattttgtgataatgtagtttcccaaaaaaattatttagaaggcattatgttattagtaaatgagagcactgtatagaactgttcctattttctgcacttgccattccagctgcctccactgtccatacccacctcattcatcctgtcacagaaggcaggaaaactgggaactttaccaaagtagcactcagcctgagaggcctgtataatcatgcttttcaaactaaattcacttaaaaattaaaaagcagaattgaatattttaagcagcctcagtacctttggccaatgctgttttcatggtggattatgaacattatataatctttgggaaaagtgaaagtagtacaatttttagaataatgacaactgcctcactgcatctctccactcacacagcaaccgtgtagccccctaagctgcagtaccatgactaaccatgatgtcaatttcatatgctgatcctcacaacagcagtgcacaaacatgccccaaatattttaacagaatttagctcttccttaagctgtcttttcatagtaaaaacaaaacaaaaacacccaatgttaaaaccacataataaacttacaaacttgaaaaattagacacttcagatagataggcaataaaacttcatattatgaaagcaatatattccaagtttcaaagatttgacaagttctgtagagtatctttcatcagtacatgaaaacttccaaactgcatgatcttctgccaggcaggactgggtgctattcgctggtttgaggtcgaatccatttcaaggcatgtcgtggtgggacattaatggtgggatggtagaatgtgcagtccggtcttgtacattgagtgttaaacctacaatgttttggatgatagaagggacattccatcttcttacaagcagggaagtaacggcagagctgactactggaaggtggtgctggtggtgcaactgctggttttggagacagtactggaattcttctactcacatgagtgaagggacaatctggtttagtacactttgcatcatatttacaatttgggtgaacaaacaaacatttttcagcaaatttacaattggggaaggctttgcagggtgagatggggtgatggtaggcacactcatccccatttttacaagcaggccagtacttgcagcgctccaaaagtttttctggtttctgtgccacactcagttcactcatctcagcttgactcatctgcagagtttctgccattactgggtcgatttgcagtcgggataataattgcctctgttgagttccttgatttttttctacagaatctccttttgtttcctcttctttaatggggggacttattctgggggtcctactttgtccctggaccacttctgctagcaattcttcttgagaagttcgagttctgggagcaactggaagtgtctgtttctgtggaactgtagagtagttagttgtttttgttacggattcttgagcttcagatatagccttcaaaatcagattcttgttagcttgtttagaaggtggaagagaaggtctcctttcaggctttgcaggcacagacacactgctggagatgcttcctgttcgagacccgtaatcatcatcttcttcctcctcttctccatcatgattgaatttttttactttaacaactgaacttaccacaggcaactttctcttccgaaagttttcatcctccatactcattttctccgagttgtttctaaagaacggactatacgtttcttctaagctgttaagcacctctggttcacacaaacgtcctgtttcatatacccaactactctgcatatcaagctgcttggcagcatgaatactattctgctgctgttgaaattgcaacctgtttaaatgaacaccactatctgcatttctacttgcaggtggtcgataaatttcaatagaagggcgagaagaaccatatgtaagtgtcactgtaggttttttctgagataagggattctcctgcacaaagttgaggtcttcgtcaatgagatcatctggttctggcttaatatcaatcacatcttcagagggtgctggctccctcaaaggtttcactgttgacattagtcgggttgcagctccatcatcgtaagtctgtctgacatttgtggtttttgactcctgcgaacttgtagaaactctggaatctcttttttcaggtctcgcgctaggaatggcaagtggtggcactgcagcttcatgcctcctctcatctccccgactgaaattgctcttgtttgaaggcacgttactatcaaagatgttggtatcagaagacttcagactagagggttcagttgtaacagagcgaagtttatctaatacaccatgaagccaacataagctcctaattcttgtaatttccccttaatggcactccggatcttgcggctgatctcggtgccgatctccatggctctgcggcgtgcgggaactcagcactgcgcggcgcttggcttacccggaggctgccgcggactcctaccccgcagccgggacaccaccgcctcc

SEQ ID NO: 17241 - RNA, 14541 nt, Homo sapiens
  source 1..14541: mol_type = other RNA
tcaggccaggcacagtggctcacacctgtaatcttatcactttgggaggctgaggcaggtggatcgcttgagcccaggagttcaagaccagcctgggcaacatggtgaaaccccatcgctataaaaaacaacaattagccgggtgtggtggcacatgcctgtagtccctgctactcaggaggctgaggtgggaggatcacttgagcctggggaggtcaaggctttagtgagctgtgatggtgccactgcactccagcctgggtgacagagtgagaccccatttaaaaaacaaaaacaaaaacaaaaaaaaatgtgacatatagttgactaagaagtacatttcaatacaggattgaaagaacccacatatgttaattaaacacaagcgcagaatttgtgccttttacataaaggaagaatgcacataggcatgctttcagacaagcaattcatctagcagaaaaggaaggaatacatttttcagcccttccaggaataaaatccataaatgggctctatttcgtcctccaacacttgtatttcccacgtcatttactcctgcacacccccactcactagaagcctgctaaactgttccagtgagatattttaacacctgatagggaataaatatgcttctgttttggccttcaaaaataagctctgggccagttgcagtggctcacgcctgtaatcccaacactttgggaggccgaggtgggcggatcacgaggtcaggagtttgggatcagcctggccaatatggtgaaactccatctctactaaaaatacaaaaattagccaggcatggtgcctgtaatcccagctacttgggaggctgaaggagaagaatcgcttgaacctgggaggcacaggttgcagtgagccgagatcacaccactgcactccaggccaggtgacagagcgacactctgtctcaaaaaaataaataaatcaactctgtagcatagcatttgtaattctattattttgccttacatttccattatccttttaataaaattgtttttttacatcttcctaatcaagaagtattatgaggccaggcacagtggctcatacctggaatcccagcactttgggaggccgaggcaggcagatcacctgaggtcaaggtatttgagaccagcctggccaacatggtgaaaccccatctctactaaaaatacagaaattagctgggtgtggtggtgcacacctgtaatgctagctactcgggaggctgaggtaggagaatcgcttgaacctgggaggcagaggttgcaataagcctagatcatgccactgcactcaagcctgggagacagagcgagactacatcttaaaaaaaaaaaaaaaagtattatgagagaggataatgtattgtaatgtattgtagaggctaaataaaattatgctcatgtcagaaaaaaagagtatttctcaaaataaaattcactgaaactggatgtttattttgactgagatatagtatatcctcaaattgccatagaaagtttacaagaatattagaggtaaattataaatatcagggcctttttaaaaaaaaaagattctgcttataacttggtatttgtttataataaaaattatagtagccaataatgaacacttactctggcttggttatttacttaggtcaaaagaaggaggagcggttaaactgtgggatcaggaactgaggcggtgccgtgccttcaggcttgagacaggacaagccacagattgtgttcgttctgtgtgcagaggcaaagtaagatgttccatgagctgatacagtgcagcagaaaacagaaagtggttattactgtgattccctcaccctttgcagcctaatgaacaatacttaataatgcataacgatggatttgcttgccaacattactctgtctttgctgctttctttgccaaagttagcaccagtgtggtgcataagctaggaagctattctgtctaaatactgtatgtaaacctccaatattttctagaatctgccaatttaacaactctagtagacataattgaaagcccttggcagttgactcatattaggacagctgtctccattttttaaaaaaacacacattccctagataaaacgtgcagtaaacaaacaatgaaatactactcagccataaaaaataatgaaattctgtcattcttggtggcaacatggatgagactggaggacatgatgtgaagtgaaataagccaggcacagaaagataaatacatgttctcactcctgtgcagaaactaaaaaagttgatcccacagaggtggagagtagaatagtggttactggaggcggacaagggggagggggagggggatagggaaggactggttaaaggatacaagtttacacagccagataggaatagtatgttttagtattctgtagtactgtaggatgactatagttaagaatcacgtatttatgtattttcaggtatttacaagagaggattttgaaagtttccatcacaaagaaatgataaatgtctgaggtgatggttatgcgtattaccctatgccctatagatatgtataattatgtgtcaatttcaaaataaaaattcaaaactacaactcctatgaaaatttttgagcgtgtttgtacttattaagtgtatttataaatcatacggatattatcttcagcctgcatattaaattgtagttaagcttttactttttaactaaaaaataaattctattattttttcctatatcccactgcactgaccccagtttggaaatcctaagattatcaaataaaaactttgattattgaagaatccaggtgtactgccacagaaaagttctattctgtagcatggactctaatatgtaatctagcccattgtgcttacagatagatgtgtgcctgtagtcatagaaaaatttgcatgagctaatgactgccttgctactagattagctcaaagcaaaaagttctctgaaagcaggtcaatagggtcatttttatattatgaagaagaaaagcagctgttgtattacattcactgtattggtcctgcttgtgtttcagggcaagatccttgttgggacaaggaatgctgaaataatcgaagttggagagaaaaatgcagcttgtaatattttagttaacggtcatgtggatgggccaatctggggactagcaacacatccttccagggattttttcctttctgctgcagaagatgggacagtgagactttgggatattgctgataaagtaagtacagataatttttttaaaagaggttacaacttctaaaaagaaaagttggaagttctaaattgctagtacttaaagaactgccagaattctgttgagcattttgaggggaaactggtataatttagaagtacttcacttaatgtttcctatgactctttttttttttttttttaaatgcagaagatgttaaacaaagtgaatttgggacatgctgctcgtactgtgtgttacagccctgaaggggacatggtggctattggaatgaaaaatggagaatttatcattttactagtgagttctctaaaaatatggggaaagaagagagacaggagatgtgcaatccatgatatcaggttagtgaacaaatggaatagagtttctagtatatacttgatttaacttccatttgtaaaattttccatagccttgccttcaaaaagaggtccccagggcctgtagcatttcccgtattataaattgtatgctaaaatatggctgtttgtatactacttaattcttcttgctaaattataaacccactgggcaccaactataatagcaagtactagtaggtaatgtttgatgaattcatgttaacacttagccatgtccattaagttcatcccaccaagaggtatctcccactgtaatacaagagagctatctgcccttcaaaagttgtcaccctggaaaactaaagttgtgatttcaaacatatcttctcttagtaacctcagtttgggaatatgtagttcattaatttaatcaatacctattgattaaatgttccagaatccaaattaatttaaatgtttcttaaacctttgtttttcagtgcttaagcatttttcaacagtggctaccatttacggagtacttccgtgtgatcagtagataagattattgaatctaggtctgtcaaaagcttgtacacttttcatcagtaaaatccttttacaaatgaaaccttcctcagaacttcaatatataaaatagtaacagtggcttcccttagcttttacatgtctctatcgtacctcagtaagactcatgggccatttcaagagactgaattgtcccatatgactccaaagattgctaggcaaatagcatttcactttgtcttttaaataagttcttcaggccgggcgcggtggctcatgcctgtaatcccagcactttgggaggccgaggcaggcagatcacctgaagtcaggagtactcgaccagcctggccaacatagtgaaaccccatctcaactaaaaatacaaaaatcagccgggcgtggtggcaggcgcctgtaatcccagctactcagggggctgaaacaggagaatcgcttgaacccgggaggcggaggttgcgccatcgcactccagcctgggagacaagagcgagacttcgtctcaaaaaaaaaaaattcttcttccaagattcaagttgtgtcatttcaccttaataactggaggttagttaagctgggctgtgttctttgcttaatattaagacaacgttttttccagatggaagaaaactatcttaatgaattgttagcttattaattatgtaatgctaatggcttttaaaagctgagatgttctgactgggtgttgtggctcacacctgtaatcccagtaccttgggaggccaagggggaaggattgcttgaggccaggagtttgggaccatagtgagaccccgcctctatttaaaaaattaaattttgttttgttttgttttgagttggagttttgctcttgttgcccatgctgaagtgcaatggtgcaatctcagctcaccacaacctgtgcctcctgggttcaagcgattctcctgcttcagcctcccgagtagatgggattacaggcgtgcaccaccatgcctggctaattttgtatttttagtagagacagggtttctctatgttggtcaggctggtctcaaactctcgacctcaggtgatctgcccgcctccgcttcccaaagttctgggattataggtgtgagccactgggcctggcctaagaaagtttttttaagccattagacgtttttaaaggaattgggagatgacaattggggaaatatttaaaatttaagtaaaatataaagcttccttatttcatgtaacccagacaatctcagtatacatgatcagttgtgtctgacaggtaaatctatttgaggccttatcacacgttacttttaagaactagaaaggaaaagtcactgatcttaagtatttataatacttcatgtggtctaatactttttacgttttgttttgattcagatttagtccggattcccggtatctggcagtaggttctagtgagaactcagtggatttttatgacctaacgctgggccccactcttaacagaatcagctactgcaaagacattccaagctttgtcattcaaatggacttctctgcagatagcagttatctccaggtacagtaccaatactgtatacccaggtggcaagttcttctgcttttacatttcgtgttagtgaatgcatttaaagttcctgagctccagagctccagcttctcaactcctccctttgtaccttctgacctacagctcccctttcctcccccacttatcagagcttttctcctattaagtttttgtagtgatcttttgcatacttaataatgttagacatgtaaatcaagtagcaatatgctagtattctgtaaaccccctgtggattttgtctctcacctaatggaattcttgtcccattttaatctgatgaaaaaggtctctagtggctgctataaacggcatgtctatgaagtgccttcaggaaaacatcttatggatcatgccgctattgacagaattacttgggctacatggactaggtaaatacttatatattcacaaggcaagaactgactttgaaggccagttagaaaatcctatttctgaactgttagagccattccaataaggaatagtaattgagtttcaagtttttgttaccatattttgaaatggtatgttcatgttgggacccctttttattgaatatatttccatgttttatcagtttccatgatttatcaagttttttttttaaggaaatcaaagttttaactttaaagataccctgatatttttcttaatgctaaatttaatgactggcaaaaaggtattgggtgctgttaagcaactgttattaattctctatctaaaggaatgctatcttgaatctattagaagtcaaagcttccaaatttgttcaaatttcctggctgtatgacaggtaaccatgactatccatttttttggccaatgaaaaatgccatcaaattcctgtatcagccaggcatatagtggctcatgcctgtaatctctgatgtagcaggccgaggtgggaggatcacttgagcctagaagttttgataccagcctgggcaacatagcaagaccccatctctgaaatttttttaattcctatgtcataagtcatttttatttttgtagagatagggatctcacaatattgcccaggctggtctcaaactcttggcctcaagcagtcctcctgcctcagcctcccaaaatgttgggattactggtatgtgctgctggacccagccaagtagcacttttaatttgaaaaatagttctatcagttttcagtcaggcgcggtggctcagcctgtaatcccagcactttgggaggccgagcgggggtgatcacctgaggtcgggagttcgagactagcctgaccaacatggagaaaccctgtctctactaaaaatacaaaataagccgggcatgttagcgcatgcctgtgatcccagctactcgggaggctgaggcaggagaattgcttgaacccaggaggcagaggttgcggtgagccgagatcatgccattgcactccagcctgggtaacaagagcgaaaactccgtctcaaaaaaaaaaaaagaaaaaatagttctatcagttttcataaagtactactttaatcttaaaaagattaatctagaaacccttcaaattataaaatgtcatttttaaaaggcaggagttgatatcctgatgaaattcaggtctccaaacaacttaccataatttacttcctgtattttaagtaacatgatagggtacttagagattaattgccaagaaactttttgaatatagtcaacctgcccgcacttgccatgatgagttttcttttgttccttccctctagtattctaggagatgaggttttgggaatctggtccagacatgctgagaaagctgatgtcaactgtgcctgtgtatctcattcaggaatcagtcttgttacaggagatgactttggcatggttaagttatttgacttcccatgtccagaaaaatttgtaagtttgtgttttgtttactattatcagtttactcctaattttgatgtcttatcatcagcacttttccccatatatttaaaatgttttgtcctaatttctaaatttttccccaaactttctaaatctatttactttgaaataaaagctattagaaacaaatcctctccctcgagtaataccatctttggaaccatcctacaaaagctgtaattagcttttcaccaaacctataatcagttatcaaatttcaaatgcttttccttagagaaaaatggtcagagtacctggagacatctgactgcccacacagcctggttttgcagatccactactcatgctgaaaagcattctaatcactggctgcggtgctaactccctactctctccacagctcttgtcatagagattatagttcctaataagagcctttgacttctgtgtgcaccaaatgccctgagcttgtctgtcattgttttttaggcaaaacacaaaaggttcttgggtcattcgccccatgtgacaaatattcgatttaccagtggtgatcgacatgttgttagtgctggaggtgatgactgcaggttagtaactttctcagcccatgaagagcagactatgttactagttaagagacttaatacaacaactcctacagctttggtttatgaaatcagctagtcaacattagtagaaggtagtataaccagatggctcttcagaatctcatatttatgcaaatacagaataaaaggagttaaagaggaaaaatattacacatgtaacctgaaagcacaactgaaaaatattaaactgttatgaaaatctaaaaacataattaactccctgcaattttcttctctgattgcagcttatttgtctggaaatgtgtacatacacctcactgagagatgctgagatgactacagaaattaactttgagaccagaattacagagaagaaaaaccaaaacccaaccctgcatggtcaagtggtgctaacccaagactgtaacagggagaaatgcccagaatcatcaaaatagtgaaagactgatctgttcaaaatatttgctatatgcactgggtataatccgtaatccatacactgccagataatgccatttcaaggaaggatcgaatacttgatggtaaaggccaagtccccctgtattgggaagtgtgtgatttcggcagacctgctgggaaaatttagggtagagcactctttacagaagaactcaaaaacccaatttggataattttcattatctttttagcaaaatggtttcttaatgtttatattttattttcaaggttcattgtttaatgaaatattttattcttgcatttccataaggaaagggaaagtcatgatcatcctaaaggatcacagtttttaaaaggcaaacattttccctaaggaaacagacacaagctttcctagagaatatgatgttttttaggcattaataaggtccttttttataaaggacacttttctcctagtagttttgaattcaggaacagatccaaagttagcagtatatggctgctacatttccattttcattttcgagccatcagtttatgttcagatgccatctctgtaatcgcacatttaaaacataactgtagcctcactaatggaaaagtagtatgatgaacaatcattcccaatggtgtacaatgtaagggttttagggagcaacagtatttaactggaagaaagaattgcatatttaatgtagtctaatatatacacatttgtttaacatgtaaacaaaagtgttaaattcacatatacaacattatacaatttaatcactcttggaataaaatttttatagccttttttctattgggaaaatttgtttagatgtgtgccactccataggtttatttccaaaatgaatgagcccaactccatttgtaaaaacttgtcagttagaattcctttttttagtggattagggctgaattcttagatccttatttcttttcactttaaatgctgccaaagatcactactcatcattcaggaattcgctgtctagcctatctgtagtttcctgaagattgaaaattatgtagactgctatttaaaaatatatttttctaagtgtgaggtttaagatgctgtattgaccctatgagtttttaatgtgttaattatctttatagcataatagatcgctttaggttcctggaatcccatttggtctgacaggatatatgaagattcttaatacctattttctgtgtctaatacttggttaatactaaaaatagaaatgactaaattacatcacagaaagcataaccagtgattgaacctggtagttttaaagctctaaatagctgtggctgaaggactgattatggggctaagaagcttgaaacgtaagttggtacttgttcatcagtggattctcctaaattaagccaaattttgaaatacatgactattaagtttctactcatgtatttacagtcagtcaataaattaaaggaggaaaaaaatccctgaacaacctgcccataaaaagaaaaatactctacatttgagcctgctgcagttttaaattttccctctgggtcaagtttgccagcttttggctacagagaaattatatttccattacagtgcaggtagaaactctgtaaccttaagcatgtaaactacatagaataaaactgtttccactgcatttctgtccttcaaagtggccaacctgattaagtcagccttaatcactgctgctgtcagtttcacgactaaaggtcatattgactaagtagtcatcagctgaccacctcgctgtatcagccagcaacgaggggaaggtgaagaaacatgataggccatatagaatctgccctatgtttacttttttaacccagataattatttttgtgtgcagtatctaagctcctgattgtgtaacctgggacttctggcaccttttgttccattcattttatgtataaaatgcatgccaaagcacactgtgccctctggtacccttgcttccaatcgccaaccatgctcatttccttcctttttttgtggtccctttttgtggtgatcattttaaaccacgtcatccaacaaatgttttatggtcaaccttagcttgttcataagccatagcaactgaaagattaaactcttaaatatgtgtctgggcagtggctattaaatagcaaaaaacaatcagattttagtattttattatttccttgtaaaatggctgaactaaattaaacccttgtttcccatttgttctataatttatagtgaaactgagaacaaaactatctttataaatgatagctaaaagtatttccagatatttaaacaatttaaaataaatttcttctgcagagatgcaaagcatctcaacactggaatgaacaaatgccttaaattcaatggagtaaacctttagaatgaagaggaactgtcatttcacccaagccgaagacaacagccttatgcacttgtgtgctctgtctttgctgcttctcgtgtttcaagcctttcctgtgggatcagcacagcaaagtgcaacttaccaaatggtttaatgactggttaattctttcttctcccaatggaaaagcaatggcaacacaacagtagactgctggcttgacaatcttaaacgtgagcctttgcacatgtaggtttatcatcatttgagtatacgactaagcaagtcaatgaactttttttttttttttagcagtttaatttggtcctgagaatgttgcagtctttattaccccttttgcattaatccacttttctaaccaccttttaagctttaatttttaacactatacaccaagtctttgaaatcagtgatctgttatttaactctaaagcatttgacacttcttgccttaacagttttaaaaaccacacacaaaaaaactctgtaagtaatacagtaggccaaaagtttcatcctatctatcttgcagtttacctatctgatctgatctctgtaattatagttctgtcatttaaaatatactatttaaatctaatttttacatttcaaaaattatcttcagtagtaactaagtatattttctgtggattctgagaatgttatttttcagaatgtgagaatatatatgtacatttataatcttgtgactttaaagtctgttttcagatacagtatgtaaatacttgtaaaaaaatttgtataattttgtgataatgtagtttcccaaaaaaattatttagaaggcattatgttattagtaaatgagagcactgtatagaactgttcctattttctgcacttgccattccagctgcctccactgtccatacccacctcattcatcctgtcacagaaggcaggaaaactgggaactttaccaaagtagcactcagcctgagaggcctgtataatcatgcttttcaaactaaattcacttaaaaattaaaaagcagaattgaatattttaagcagcctcagtacctttggccaatgctgttttcatggtggattatgaacattatataatctttgggaaaagtgaaagtagtacaatttttagaataatgacaactgcctcactgcatctctccactcacacagcaaccgtgtagccccctaagctgcagtaccatgactaaccatgatgtcaatttcatatgctgatcctcacaacagcagtgcacaaacatgccccaaatattttaacagaatttagctcttccttaagctgtcttttcatagtaaaaacaaaacaaaaacacccaatgttaaaaccacataataaacttacaaacttgaaaaattagacacttcagatagataggcaataaaacttcatattatgaaagcaatatattccaagtttcaaagatttgacaagttctgtagagtatctttcatcagtacatgaaaacttccaaactgcatgatcttctgccaggcaggactgggtgctattcgctggtttgaggtcgaatccatttcaaggcatgtcgtggtgggacattaatggtgggatggtagaatgtgcagtccggtcttgtacattgagtgttaaacctacaatgttttggatgatagaagggacattccatcttcttacaagcagggaagtaacggcagagctgactactggaaggtggtgctggtggtgcaactgctggttttggagacagtactggaattcttctactcacatgagtgaagggacaatctggtttagtacactttgcatcatatttacaatttgggtgaacaaacaaacatttttcagcaaatttacaattggggaaggctttgcagggtgagatggggtgatggtaggcacactcatccccatttttacaagcaggccagtacttgcagcgctccaaaagtttttctggtttctgtgccacactcagttcactcatctcagcttgactcatctgcagagtttctgccattactgggtcgatttgcagtcgggataataattgcctctgttgagttccttgatttttttctacagaatctccttttgtttcctcttctttaatggggggacttattctgggggtcctactttgtccctggaccacttctgctagcaattcttcttgagaagttcgagttctgggagcaactggaagtgtctgtttctgtggaactgtagagtagttagttgtttttgttacggattcttgagcttcagatatagccttcaaaatcagattcttgttagcttgtttagaaggtggaagagaaggtctcctttcaggctttgcaggcacagacacactgctggagatgcttcctgttcgagacccgtaatcatcatcttcttcctcctcttctccatcatgattgaatttttttactttaacaactgaacttaccacaggcaactttctcttccgaaagttttcatcctccatactcattttctccgagttgtttctaaagaacggactatacgtttcttctaagctgttaagcacctctggttcacacaaacgtcctgtttcatatacccaactactctgcatatcaagctgcttggcagcatgaatactattctgctgctgttgaaattgcaacctgtttaaatgaacaccactatctgcatttctacttgcaggtggtcgataaatttcaatagaagggcgagaagaaccatatgtaagtgtcactgtaggttttttctgagataagggattctcctgcacaaagttgaggtcttcgtcaatgagatcatctggttctggcttaatatcaatcacatcttcagagggtgctggctccctcaaaggtttcactgttgacattagtcgggttgcagctccatcatcgtaagtctgtctgacatttgtggtttttgactcctgcgaacttgtagaaactctggaatctcttttttcaggtctcgcgctaggaatggcaagtggtggcactgcagcttcatgcctcctctcatctccccgactgaaattgctcttgtttgaaggcacgttactatcaaagatgttggtatcagaagacttcagactagagggttcagttgtaacagagcgaagtttatctaatacaccatgaagccatacggtgaatcgaattgtgttgttccctagaaacagggacagatcctctgtcatttggtcctgacttttcttgttggccaccatcaccataatgtaatcaggaagttcttcatcaacataagctcctaattcttgtaatttccccttaatggcactccggatcttgcggctgatctcggtgccgatctccatggctctgcggcgtgcgggaactcagcactgcgcggcgcttggcttacccggaggctgccgcggactcctaccccgcagccgggacaccaccgcctcc

SEQ ID NO: 17242 - RNA, 14517 nt, Homo sapiens
  source 1..14517: mol_type = other RNA
tcaggccaggcacagtggctcacacctgtaatcttatcactttgggaggctgaggcaggtggatcgcttgagcccaggagttcaagaccagcctgggcaacatggtgaaaccccatcgctataaaaaacaacaattagccgggtgtggtggcacatgcctgtagtccctgctactcaggaggctgaggtgggaggatcacttgagcctggggaggtcaaggctttagtgagctgtgatggtgccactgcactccagcctgggtgacagagtgagaccccatttaaaaaacaaaaacaaaaacaaaaaaaaatgtgacatatagttgactaagaagtacatttcaatacaggattgaaagaacccacatatgttaattaaacacaagcgcagaatttgtgccttttacataaaggaagaatgcacataggcatgctttcagacaagcaattcatctagcagaaaaggaaggaatacatttttcagcccttccaggaataaaatccataaatgggctctatttcgtcctccaacacttgtatttcccacgtcatttactcctgcacacccccactcactagaagcctgctaaactgttccagtgagatattttaacacctgatagggaataaatatgcttctgttttggccttcaaaaataagctctgggccagttgcagtggctcacgcctgtaatcccaacactttgggaggccgaggtgggcggatcacgaggtcaggagtttgggatcagcctggccaatatggtgaaactccatctctactaaaaatacaaaaattagccaggcatggtgcctgtaatcccagctacttgggaggctgaaggagaagaatcgcttgaacctgggaggcacaggttgcagtgagccgagatcacaccactgcactccaggccaggtgacagagcgacactctgtctcaaaaaaataaataaatcaactctgtagcatagcatttgtaattctattattttgccttacatttccattatccttttaataaaattgtttttttacatcttcctaatcaagaagtattatgaggccaggcacagtggctcatacctggaatcccagcactttgggaggccgaggcaggcagatcacctgaggtcaaggtatttgagaccagcctggccaacatggtgaaaccccatctctactaaaaatacagaaattagctgggtgtggtggtgcacacctgtaatgctagctactcgggaggctgaggtaggagaatcgcttgaacctgggaggcagaggttgcaataagcctagatcatgccactgcactcaagcctgggagacagagcgagactacatcttaaaaaaaaaaaaaaaagtattatgagagaggataatgtattgtaatgtattgtagaggctaaataaaattatgctcatgtcagaaaaaaagagtatttctcaaaataaaattcactgaaactggatgtttattttgactgagatatagtatatcctcaaattgccatagaaagtttacaagaatattagaggtaaattataaatatcagggcctttttaaaaaaaaaagattctgcttataacttggtatttgtttataataaaaattatagtagccaataatgaacacttactctggcttggttatttacttaggtcaaaagaaggaggagcggttaaactgtgggatcaggaactgaggcggtgccgtgccttcaggcttgagacaggacaagccacagattgtgttcgttctgtgtgcagaggcaaagtaagatgttccatgagctgatacagtgcagcagaaaacagaaagtggttattactgtgattccctcaccctttgcagcctaatgaacaatacttaataatgcataacgatggatttgcttgccaacattactctgtctttgctgctttctttgccaaagttagcaccagtgtggtgcataagctaggaagctattctgtctaaatactgtatgtaaacctccaatattttctagaatctgccaatttaacaactctagtagacataattgaaagcccttggcagttgactcatattaggacagctgtctccattttttaaaaaaacacacattccctagataaaacgtgcagtaaacaaacaatgaaatactactcagccataaaaaataatgaaattctgtcattcttggtggcaacatggatgagactggaggacatgatgtgaagtgaaataagccaggcacagaaagataaatacatgttctcactcctgtgcagaaactaaaaaagttgatcccacagaggtggagagtagaatagtggttactggaggcggacaagggggagggggagggggatagggaaggactggttaaaggatacaagtttacacagccagataggaatagtatgttttagtattctgtagtactgtaggatgactatagttaagaatcacgtatttatgtattttcaggtatttacaagagaggattttgaaagtttccatcacaaagaaatgataaatgtctgaggtgatggttatgcgtattaccctatgccctatagatatgtataattatgtgtcaatttcaaaataaaaattcaaaactacaactcctatgaaaatttttgagcgtgtttgtacttattaagtgtatttataaatcatacggatattatcttcagcctgcatattaaattgtagttaagcttttactttttaactaaaaaataaattctattattttttcctatatcccactgcactgaccccagtttggaaatcctaagattatcaaataaaaactttgattattgaagaatccaggtgtactgccacagaaaagttctattctgtagcatggactctaatatgtaatctagcccattgtgcttacagatagatgtgtgcctgtagtcatagaaaaatttgcatgagctaatgactgccttgctactagattagctcaaagcaaaaagttctctgaaagcaggtcaatagggtcatttttatattatgaagaagaaaagcagctgttgtattacattcactgtattggtcctgcttgtgtttcagggcaagatccttgttgggacaaggaatgctgaaataatcgaagttggagagaaaaatgcagcttgtaatattttagttaacggtcatgtggatgggccaatctggggactagcaacacatccttccagggattttttcctttctgctgcagaagatgggacagtgagactttgggatattgctgataaagtaagtacagataatttttttaaaagaggttacaacttctaaaaagaaaagttggaagttctaaattgctagtacttaaagaactgccagaattctgttgagcattttgaggggaaactggtataatttagaagtacttcacttaatgtttcctatgactctttttttttttttttttaaatgcagaagatgttaaacaaagtgaatttgggacatgctgctcgtactgtgtgttacagccctgaaggggacatggtggctattggaatgaaaaatggagaatttatcattttactagtgagttctctaaaaatatggggaaagaagagagacaggagatgtgcaatccatgatatcaggttagtgaacaaatggaatagagtttctagtatatacttgatttaacttccatttgtaaaattttccatagccttgccttcaaaaagaggtccccagggcctgtagcatttcccgtattataaattgtatgctaaaatatggctgtttgtatactacttaattcttcttgctaaattataaacccactgggcaccaactataatagcaagtactagtaggtaatgtttgatgaattcatgttaacacttagccatgtccattaagttcatcccaccaagaggtatctcccactgtaatacaagagagctatctgcccttcaaaagttgtcaccctggaaaactaaagttgtgatttcaaacatatcttctcttagtaacctcagtttgggaatatgtagttcattaatttaatcaatacctattgattaaatgttccagaatccaaattaatttaaatgtttcttaaacctttgtttttcagtgcttaagcatttttcaacagtggctaccatttacggagtacttccgtgtgatcagtagataagattattgaatctaggtctgtcaaaagcttgtacacttttcatcagtaaaatccttttacaaatgaaaccttcctcagaacttcaatatataaaatagtaacagtggcttcccttagcttttacatgtctctatcgtacctcagtaagactcatgggccatttcaagagactgaattgtcccatatgactccaaagattgctaggcaaatagcatttcactttgtcttttaaataagttcttcaggccgggcgcggtggctcatgcctgtaatcccagcactttgggaggccgaggcaggcagatcacctgaagtcaggagtactcgaccagcctggccaacatagtgaaaccccatctcaactaaaaatacaaaaatcagccgggcgtggtggcaggcgcctgtaatcccagctactcagggggctgaaacaggagaatcgcttgaacccgggaggcggaggttgcgccatcgcactccagcctgggagacaagagcgagacttcgtctcaaaaaaaaaaaattcttcttccaagattcaagttgtgtcatttcaccttaataactggaggttagttaagctgggctgtgttctttgcttaatattaagacaacgttttttccagatggaagaaaactatcttaatgaattgttagcttattaattatgtaatgctaatggcttttaaaagctgagatgttctgactgggtgttgtggctcacacctgtaatcccagtaccttgggaggccaagggggaaggattgcttgaggccaggagtttgggaccatagtgagaccccgcctctatttaaaaaattaaattttgttttgttttgttttgagttggagttttgctcttgttgcccatgctgaagtgcaatggtgcaatctcagctcaccacaacctgtgcctcctgggttcaagcgattctcctgcttcagcctcccgagtagatgggattacaggcgtgcaccaccatgcctggctaattttgtatttttagtagagacagggtttctctatgttggtcaggctggtctcaaactctcgacctcaggtgatctgcccgcctccgcttcccaaagttctgggattataggtgtgagccactgggcctggcctaagaaagtttttttaagccattagacgtttttaaaggaattgggagatgacaattggggaaatatttaaaatttaagtaaaatataaagcttccttatttcatgtaacccagacaatctcagtatacatgatcagttgtgtctgacaggtaaatctatttgaggccttatcacacgttacttttaagaactagaaaggaaaagtcactgatcttaagtatttataatacttcatgtggtctaatactttttacgttttgttttgattcagatttagtccggattcccggtatctggcagtaggttctagtgagaactcagtggatttttatgacctaacgctgggccccactcttaacagaatcagctactgcaaagacattccaagctttgtcattcaaatggacttctctgcagatagcagttatctccaggtacagtaccaatactgtatacccaggtggcaagttcttctgcttttacatttcgtgttagtgaatgcatttaaagttcctgagctccagagctccagcttctcaactcctccctttgtaccttctgacctacagctcccctttcctcccccacttatcagagcttttctcctattaagtttttgtagtgatcttttgcatacttaataatgttagacatgtaaatcaagtagcaatatgctagtattctgtaaaccccctgtggattttgtctctcacctaatggaattcttgtcccattttaatctgatgaaaaaggtctctagtggctgctataaacggcatgtctatgaagtgccttcaggaaaacatcttatggatcatgccgctattgacagaattacttgggctacatggactaggtaaatacttatatattcacaaggcaagaactgactttgaaggccagttagaaaatcctatttctgaactgttagagccattccaataaggaatagtaattgagtttcaagtttttgttaccatattttgaaatggtatgttcatgttgggacccctttttattgaatatatttccatgttttatcagtttccatgatttatcaagttttttttttaaggaaatcaaagttttaactttaaagataccctgatatttttcttaatgctaaatttaatgactggcaaaaaggtattgggtgctgttaagcaactgttattaattctctatctaaaggaatgctatcttgaatctattagaagtcaaagcttccaaatttgttcaaatttcctggctgtatgacaggtaaccatgactatccatttttttggccaatgaaaaatgccatcaaattcctgtatcagccaggcatatagtggctcatgcctgtaatctctgatgtagcaggccgaggtgggaggatcacttgagcctagaagttttgataccagcctgggcaacatagcaagaccccatctctgaaatttttttaattcctatgtcataagtcatttttatttttgtagagatagggatctcacaatattgcccaggctggtctcaaactcttggcctcaagcagtcctcctgcctcagcctcccaaaatgttgggattactggtatgtgctgctggacccagccaagtagcacttttaatttgaaaaatagttctatcagttttcagtcaggcgcggtggctcagcctgtaatcccagcactttgggaggccgagcgggggtgatcacctgaggtcgggagttcgagactagcctgaccaacatggagaaaccctgtctctactaaaaatacaaaataagccgggcatgttagcgcatgcctgtgatcccagctactcgggaggctgaggcaggagaattgcttgaacccaggaggcagaggttgcggtgagccgagatcatgccattgcactccagcctgggtaacaagagcgaaaactccgtctcaaaaaaaaaaaaagaaaaaatagttctatcagttttcataaagtactactttaatcttaaaaagattaatctagaaacccttcaaattataaaatgtcatttttaaaaggcaggagttgatatcctgatgaaattcaggtctccaaacaacttaccataatttacttcctgtattttaagtaacatgatagggtacttagagattaattgccaagaaactttttgaatatagtcaacctgcccgcacttgccatgatgagttttcttttgttccttccctctagtattctaggagatgaggttttgggaatctggtccagacatgctgagaaagctgatgtcaactgtgcctgtgtatctcattcaggaatcagtcttgttacaggagatgactttggcatggttaagttatttgacttcccatgtccagaaaaatttgtaagtttgtgttttgtttactattatcagtttactcctaattttgatgtcttatcatcagcacttttccccatatatttaaaatgttttgtcctaatttctaaatttttccccaaactttctaaatctatttactttgaaataaaagctattagaaacaaatcctctccctcgagtaataccatctttggaaccatcctacaaaagctgtaattagcttttcaccaaacctataatcagttatcaaatttcaaatgcttttccttagagaaaaatggtcagagtacctggagacatctgactgcccacacagcctggttttgcagatccactactcatgctgaaaagcattctaatcactggctgcggtgctaactccctactctctccacagctcttgtcatagagattatagttcctaataagagcctttgacttctgtgtgcaccaaatgccctgagcttgtctgtcattgttttttaggcaaaacacaaaaggttcttgggtcattcgccccatgtgacaaatattcgatttaccagtggtgatcgacatgttgttagtgctggaggtgatgactgcaggttagtaactttctcagcccatgaagagcagactatgttactagttaagagacttaatacaacaactcctacagctttggtttatgaaatcagctagtcaacattagtagaaggtagtataaccagatggctcttcagaatctcatatttatgcaaatacagaataaaaggagttaaagaggaaaaatattacacatgtaacctgaaagcacaactgaaaaatattaaactgttatgaaaatctaaaaacataattaactccctgcaattttcttctctgattgcagcttatttgtctggaaatgtgtacatacacctcactgagagatgctgagatgactacagaaattaactttgagaccagaattacagagaagaaaaaccaaaacccaaccctgcatggtcaagtggtgctaacccaagactgtaacagggagaaatgcccagaatcatcaaaatagtgaaagactgatctgttcaaaatatttgctatatgcactgggtataatccgtaatccatacactgccagataatgccatttcaaggaaggatcgaatacttgatggtaaaggccaagtccccctgtattgggaagtgtgtgatttcggcagacctgctgggaaaatttagggtagagcactctttacagaagaactcaaaaacccaatttggataattttcattatctttttagcaaaatggtttcttaatgtttatattttattttcaaggttcattgtttaatgaaatattttattcttgcatttccataaggaaagggaaagtcatgatcatcctaaaggatcacagtttttaaaaggcaaacattttccctaaggaaacagacacaagctttcctagagaatatgatgttttttaggcattaataaggtccttttttataaaggacacttttctcctagtagttttgaattcaggaacagatccaaagttagcagtatatggctgctacatttccattttcattttcgagccatcagtttatgttcagatgccatctctgtaatcgcacatttaaaacataactgtagcctcactaatggaaaagtagtatgatgaacaatcattcccaatggtgtacaatgtaagggttttagggagcaacagtatttaactggaagaaagaattgcatatttaatgtagtctaatatatacacatttgtttaacatgtaaacaaaagtgttaaattcacatatacaacattatacaatttaatcactcttggaataaaatttttatagccttttttctattgggaaaatttgtttagatgtgtgccactccataggtttatttccaaaatgaatgagcccaactccatttgtaaaaacttgtcagttagaattcctttttttagtggattagggctgaattcttagatccttatttcttttcactttaaatgctgccaaagatcactactcatcattcaggaattcgctgtctagcctatctgtagtttcctgaagattgaaaattatgtagactgctatttaaaaatatatttttctaagtgtgaggtttaagatgctgtattgaccctatgagtttttaatgtgttaattatctttatagcataatagatcgctttaggttcctggaatcccatttggtctgacaggatatatgaagattcttaatacctattttctgtgtctaatacttggttaatactaaaaatagaaatgactaaattacatcacagaaagcataaccagtgattgaacctggtagttttaaagctctaaatagctgtggctgaaggactgattatggggctaagaagcttgaaacgtaagttggtacttgttcatcagtggattctcctaaattaagccaaattttgaaatacatgactattaagtttctactcatgtatttacagtcagtcaataaattaaaggaggaaaaaaatccctgaacaacctgcccataaaaagaaaaatactctacatttgagcctgctgcagttttaaattttccctctgggtcaagtttgccagcttttggctacagagaaattatatttccattacagtgcaggtagaaactctgtaaccttaagcatgtaaactacatagaataaaactgtttccactgcatttctgtccttcaaagtggccaacctgattaagtcagccttaatcactgctgctgtcagtttcacgactaaaggtcatattgactaagtagtcatcagctgaccacctcgctgtatcagccagcaacgaggggaaggtgaagaaacatgataggccatatagaatctgccctatgtttacttttttaacccagataattatttttgtgtgcagtatctaagctcctgattgtgtaacctgggacttctggcaccttttgttccattcattttatgtataaaatgcatgccaaagcacactgtgccctctggtacccttgcttccaatcgccaaccatgctcatttccttcctttttttgtggtccctttttgtggtgatcattttaaaccacgtcatccaacaaatgttttatggtcaaccttagcttgttcataagccatagcaactgaaagattaaactcttaaatatgtgtctgggcagtggctattaaatagcaaaaaacaatcagattttagtattttattatttccttgtaaaatggctgaactaaattaaacccttgtttcccatttgttctataatttatagtgaaactgagaacaaaactatctttataaatgatagctaaaagtatttccagatatttaaacaatttaaaataaatttcttctgcagagatgcaaagcatctcaacactggaatgaacaaatgccttaaattcaatggagtaaacctttagaatgaagaggaactgtcatttcacccaagccgaagacaacagccttatgcacttgtgtgctctgtctttgctgcttctcgtgtttcaagcctttcctgtgggatcagcacagcaaagtgcaacttaccaaatggtttaatgactggttaattctttcttctcccaatggaaaagcaatggcaacacaacagtagactgctggcttgacaatcttaaacgtgagcctttgcacatgtaggtttatcatcatttgagtatacgactaagcaagtcaatgaactttttttttttttttagcagtttaatttggtcctgagaatgttgcagtctttattaccccttttgcattaatccacttttctaaccaccttttaagctttaatttttaacactatacaccaagtctttgaaatcagtgatctgttatttaactctaaagcatttgacacttcttgccttaacagttttaaaaaccacacacaaaaaaactctgtaagtaatacagtaggccaaaagtttcatcctatctatcttgcagtttacctatctgatctgatctctgtaattatagttctgtcatttaaaatatactatttaaatctaatttttacatttcaaaaattatcttcagtagtaactaagtatattttctgtggattctgagaatgttatttttcagaatgtgagaatatatatgtacatttataatcttgtgactttaaagtctgttttcagatacagtatgtaaatacttgtaaaaaaatttgtataattttgtgataatgtagtttcccaaaaaaattatttagaaggcattatgttattagtaaatgagagcactgtatagaactgttcctattttctgcacttgccattccagctgcctccactgtccatacccacctcattcatcctgtcacagaaggcaggaaaactgggaactttaccaaagtagcactcagcctgagaggcctgtataatcatgcttttcaaactaaattcacttaaaaattaaaaagcagaattgaatattttaagcagcctcagtacctttggccaatgctgttttcatggtggattatgaacattatataatctttgggaaaagtgaaagtagtacaatttttagaataatgacaactgcctcactgcatctctccactcacacagcaaccgtgtagccccctaagctgcagtaccatgactaaccatgatgtcaatttcatatgctgatcctcacaacagcagtgcacaaacatgccccaaatattttaacagaatttagctcttccttaagctgtcttttcatagtaaaaacaaaacaaaaacacccaatgttaaaaccacataataaacttacaaacttgaaaaattagacacttcagatagataggcaataaaacttcatattatgaaagcaatatattccaagtttcaaagatttgacaagttctgtagagtatctttcatcagtacatgaaaacttccaaactgcatgatcttctgccaggcaggactgggtgctattcgctggtttgaggtcgaatccatttcaaggcatgtcgtggtgggacattaatggtgggatggtagaatgtgcagtccggtcttgtacattgagtgttaaacctacaatgttttggatgatagaagggacattccatcttcttacaagcagggaagtaacggcagagctgactactggaaggtggtgctggtggtgcaactgctggttttggagacagtactggaattcttctactcacatgagtgaagggacaatctggtttagtacactttgcatcatatttacaatttgggtgaacaaacaaacatttttcagcaaatttacaattggggaaggctttgcagggtgagatggggtgatggtaggcacactcatccccatttttacaagcaggccagtacttgcagcgctccaaaagtttttctggtttctgtgccacactcagttcactcatctcagcttgactcatctgcagagtttctgccattactgggtcgatttgcagtcgggataataattgcctctgttgagttccttgatttttttctacagaatctccttttgtttcctcttctttaatggggggacttattctgggggtcctactttgtccctggaccacttctgctagcaattcttcttgagaagttcgagttctgggagcaactggaagtgtctgtttctgtggaactgtagagtagttagttgtttttgttacggattcttgagcttcagatatagccttcaaaatcagattcttgttagcttgtttagaaggtggaagagaaggtctcctttcaggctttgcaggcacagacacactgctggagatgcttcctgttcgagacccgtaatcatcatcttcttcctcctcttctccatcatgattgaatttttttactttaacaactgaacttaccacaggcaactttctcttccgaaagttttcatcctccatactcattttctccgagttgtttctaaagaacggactatacgtttcttctaagctgttaagcacctctggttcacacaaacgtcctgtttcatatacccaactactctgcatatcaagctgcttggcagcatgaatactattctgctgctgttgaaattgcaacctgtttaaatgaacaccactatctgcatttctacttgcaggtggtcgataaatttcaatagaagggcgagaagaaccatatgtaagtgtcactgtaggttttttctgagataagggattctcctgcacaaagttgaggtcttcgtcaatgagatcatctggttctggcttaatatcaatcacatcttcagagggtgctggctccctcaaaggtttcactgttgacattagtcgggttgcagctccatcatcgtaagtctgtctgacatttgtggtttttgactcctgcgaacttgtagaaactctggaatctcttttttcaggtctcgcgctaggaatggcaagtggtggcactgcagcttcatgcctcctctcatctccccgactgaaattgctcttgtttgaaggcacgttactatcaaagatgttggtatcagaagacttcagactagagggttcagttgtaacagagcgaagtttatctaatacaccatgaagccatacggtgaatcgaattgtgttgttccctagaaacagggacagatcctctgtcatttggtcctgacttttcttgttggccaccatcaccataatgtaatcaggaagttcttcatcaacataagctcctaattcttgtaatttccccttaatggcactctcccgcagcggatccaaagcggcgccgtgcgccgcggtggtggctccagccgggcctgcgcctgtccttccatttcccggcggctacttcagccgcagccacgctccg

SEQ ID NO: 17243 - RNA, 14351 nt, Homo sapiens
  source 1..14351: mol_type = other RNA
tcaggccaggcacagtggctcacacctgtaatcttatcactttgggaggctgaggcaggtggatcgcttgagcccaggagttcaagaccagcctgggcaacatggtgaaaccccatcgctataaaaaacaacaattagccgggtgtggtggcacatgcctgtagtccctgctactcaggaggctgaggtgggaggatcacttgagcctggggaggtcaaggctttagtgagctgtgatggtgccactgcactccagcctgggtgacagagtgagaccccatttaaaaaacaaaaacaaaaacaaaaaaaaatgtgacatatagttgactaagaagtacatttcaatacaggattgaaagaacccacatatgttaattaaacacaagcgcagaatttgtgccttttacataaaggaagaatgcacataggcatgctttcagacaagcaattcatctagcagaaaaggaaggaatacatttttcagcccttccaggaataaaatccataaatgggctctatttcgtcctccaacacttgtatttcccacgtcatttactcctgcacacccccactcactagaagcctgctaaactgttccagtgagatattttaacacctgatagggaataaatatgcttctgttttggccttcaaaaataagctctgggccagttgcagtggctcacgcctgtaatcccaacactttgggaggccgaggtgggcggatcacgaggtcaggagtttgggatcagcctggccaatatggtgaaactccatctctactaaaaatacaaaaattagccaggcatggtgcctgtaatcccagctacttgggaggctgaaggagaagaatcgcttgaacctgggaggcacaggttgcagtgagccgagatcacaccactgcactccaggccaggtgacagagcgacactctgtctcaaaaaaataaataaatcaactctgtagcatagcatttgtaattctattattttgccttacatttccattatccttttaataaaattgtttttttacatcttcctaatcaagaagtattatgaggccaggcacagtggctcatacctggaatcccagcactttgggaggccgaggcaggcagatcacctgaggtcaaggtatttgagaccagcctggccaacatggtgaaaccccatctctactaaaaatacagaaattagctgggtgtggtggtgcacacctgtaatgctagctactcgggaggctgaggtaggagaatcgcttgaacctgggaggcagaggttgcaataagcctagatcatgccactgcactcaagcctgggagacagagcgagactacatcttaaaaaaaaaaaaaaaagtattatgagagaggataatgtattgtaatgtattgtagaggctaaataaaattatgctcatgtcagaaaaaaagagtatttctcaaaataaaattcactgaaactggatgtttattttgactgagatatagtatatcctcaaattgccatagaaagtttacaagaatattagaggtaaattataaatatcagggcctttttaaaaaaaaaagattctgcttataacttggtatttgtttataataaaaattatagtagccaataatgaacacttactctggcttggttatttacttaggtcaaaagaaggaggagcggttaaactgtgggatcaggaactgaggcggtgccgtgccttcaggcttgagacaggacaagccacagattgtgttcgttctgtgtgcagaggcaaagtaagatgttccatgagctgatacagtgcagcagaaaacagaaagtggttattactgtgattccctcaccctttgcagcctaatgaacaatacttaataatgcataacgatggatttgcttgccaacattactctgtctttgctgctttctttgccaaagttagcaccagtgtggtgcataagctaggaagctattctgtctaaatactgtatgtaaacctccaatattttctagaatctgccaatttaacaactctagtagacataattgaaagcccttggcagttgactcatattaggacagctgtctccattttttaaaaaaacacacattccctagataaaacgtgcagtaaacaaacaatgaaatactactcagccataaaaaataatgaaattctgtcattcttggtggcaacatggatgagactggaggacatgatgtgaagtgaaataagccaggcacagaaagataaatacatgttctcactcctgtgcagaaactaaaaaagttgatcccacagaggtggagagtagaatagtggttactggaggcggacaagggggagggggagggggatagggaaggactggttaaaggatacaagtttacacagccagataggaatagtatgttttagtattctgtagtactgtaggatgactatagttaagaatcacgtatttatgtattttcaggtatttacaagagaggattttgaaagtttccatcacaaagaaatgataaatgtctgaggtgatggttatgcgtattaccctatgccctatagatatgtataattatgtgtcaatttcaaaataaaaattcaaaactacaactcctatgaaaatttttgagcgtgtttgtacttattaagtgtatttataaatcatacggatattatcttcagcctgcatattaaattgtagttaagcttttactttttaactaaaaaataaattctattattttttcctatatcccactgcactgaccccagtttggaaatcctaagattatcaaataaaaactttgattattgaagaatccaggtgtactgccacagaaaagttctattctgtagcatggactctaatatgtaatctagcccattgtgcttacagatagatgtgtgcctgtagtcatagaaaaatttgcatgagctaatgactgccttgctactagattagctcaaagcaaaaagttctctgaaagcaggtcaatagggtcatttttatattatgaagaagaaaagcagctgttgtattacattcactgtattggtcctgcttgtgtttcagggcaagatccttgttgggacaaggaatgctgaaataatcgaagttggagagaaaaatgcagcttgtaatattttagttaacggtcatgtggatgggccaatctggggactagcaacacatccttccagggattttttcctttctgctgcagaagatgggacagtgagactttgggatattgctgataaagtaagtacagataatttttttaaaagaggttacaacttctaaaaagaaaagttggaagttctaaattgctagtacttaaagaactgccagaattctgttgagcattttgaggggaaactggtataatttagaagtacttcacttaatgtttcctatgactctttttttttttttttttaaatgcagaagatgttaaacaaagtgaatttgggacatgctgctcgtactgtgtgttacagccctgaaggggacatggtggctattggaatgaaaaatggagaatttatcattttactagtgagttctctaaaaatatggggaaagaagagagacaggagatgtgcaatccatgatatcaggttagtgaacaaatggaatagagtttctagtatatacttgatttaacttccatttgtaaaattttccatagccttgccttcaaaaagaggtccccagggcctgtagcatttcccgtattataaattgtatgctaaaatatggctgtttgtatactacttaattcttcttgctaaattataaacccactgggcaccaactataatagcaagtactagtaggtaatgtttgatgaattcatgttaacacttagccatgtccattaagttcatcccaccaagaggtatctcccactgtaatacaagagagctatctgcccttcaaaagttgtcaccctggaaaactaaagttgtgatttcaaacatatcttctcttagtaacctcagtttgggaatatgtagttcattaatttaatcaatacctattgattaaatgttccagaatccaaattaatttaaatgtttcttaaacctttgtttttcagtgcttaagcatttttcaacagtggctaccatttacggagtacttccgtgtgatcagtagataagattattgaatctaggtctgtcaaaagcttgtacacttttcatcagtaaaatccttttacaaatgaaaccttcctcagaacttcaatatataaaatagtaacagtggcttcccttagcttttacatgtctctatcgtacctcagtaagactcatgggccatttcaagagactgaattgtcccatatgactccaaagattgctaggcaaatagcatttcactttgtcttttaaataagttcttcaggccgggcgcggtggctcatgcctgtaatcccagcactttgggaggccgaggcaggcagatcacctgaagtcaggagtactcgaccagcctggccaacatagtgaaaccccatctcaactaaaaatacaaaaatcagccgggcgtggtggcaggcgcctgtaatcccagctactcagggggctgaaacaggagaatcgcttgaacccgggaggcggaggttgcgccatcgcactccagcctgggagacaagagcgagacttcgtctcaaaaaaaaaaaattcttcttccaagattcaagttgtgtcatttcaccttaataactggaggttagttaagctgggctgtgttctttgcttaatattaagacaacgttttttccagatggaagaaaactatcttaatgaattgttagcttattaattatgtaatgctaatggcttttaaaagctgagatgttctgactgggtgttgtggctcacacctgtaatcccagtaccttgggaggccaagggggaaggattgcttgaggccaggagtttgggaccatagtgagaccccgcctctatttaaaaaattaaattttgttttgttttgttttgagttggagttttgctcttgttgcccatgctgaagtgcaatggtgcaatctcagctcaccacaacctgtgcctcctgggttcaagcgattctcctgcttcagcctcccgagtagatgggattacaggcgtgcaccaccatgcctggctaattttgtatttttagtagagacagggtttctctatgttggtcaggctggtctcaaactctcgacctcaggtgatctgcccgcctccgcttcccaaagttctgggattataggtgtgagccactgggcctggcctaagaaagtttttttaagccattagacgtttttaaaggaattgggagatgacaattggggaaatatttaaaatttaagtaaaatataaagcttccttatttcatgtaacccagacaatctcagtatacatgatcagttgtgtctgacaggtaaatctatttgaggccttatcacacgttacttttaagaactagaaaggaaaagtcactgatcttaagtatttataatacttcatgtggtctaatactttttacgttttgttttgattcagatttagtccggattcccggtatctggcagtaggttctagtgagaactcagtggatttttatgacctaacgctgggccccactcttaacagaatcagctactgcaaagacattccaagctttgtcattcaaatggacttctctgcagatagcagttatctccaggtacagtaccaatactgtatacccaggtggcaagttcttctgcttttacatttcgtgttagtgaatgcatttaaagttcctgagctccagagctccagcttctcaactcctccctttgtaccttctgacctacagctcccctttcctcccccacttatcagagcttttctcctattaagtttttgtagtgatcttttgcatacttaataatgttagacatgtaaatcaagtagcaatatgctagtattctgtaaaccccctgtggattttgtctctcacctaatggaattcttgtcccattttaatctgatgaaaaaggtctctagtggctgctataaacggcatgtctatgaagtgccttcaggaaaacatcttatggatcatgccgctattgacagaattacttgggctacatggactaggtaaatacttatatattcacaaggcaagaactgactttgaaggccagttagaaaatcctatttctgaactgttagagccattccaataaggaatagtaattgagtttcaagtttttgttaccatattttgaaatggtatgttcatgttgggacccctttttattgaatatatttccatgttttatcagtttccatgatttatcaagttttttttttaaggaaatcaaagttttaactttaaagataccctgatatttttcttaatgctaaatttaatgactggcaaaaaggtattgggtgctgttaagcaactgttattaattctctatctaaaggaatgctatcttgaatctattagaagtcaaagcttccaaatttgttcaaatttcctggctgtatgacaggtaaccatgactatccatttttttggccaatgaaaaatgccatcaaattcctgtatcagccaggcatatagtggctcatgcctgtaatctctgatgtagcaggccgaggtgggaggatcacttgagcctagaagttttgataccagcctgggcaacatagcaagaccccatctctgaaatttttttaattcctatgtcataagtcatttttatttttgtagagatagggatctcacaatattgcccaggctggtctcaaactcttggcctcaagcagtcctcctgcctcagcctcccaaaatgttgggattactggtatgtgctgctggacccagccaagtagcacttttaatttgaaaaatagttctatcagttttcagtcaggcgcggtggctcagcctgtaatcccagcactttgggaggccgagcgggggtgatcacctgaggtcgggagttcgagactagcctgaccaacatggagaaaccctgtctctactaaaaatacaaaataagccgggcatgttagcgcatgcctgtgatcccagctactcgggaggctgaggcaggagaattgcttgaacccaggaggcagaggttgcggtgagccgagatcatgccattgcactccagcctgggtaacaagagcgaaaactccgtctcaaaaaaaaaaaaagaaaaaatagttctatcagttttcataaagtactactttaatcttaaaaagattaatctagaaacccttcaaattataaaatgtcatttttaaaaggcaggagttgatatcctgatgaaattcaggtctccaaacaacttaccataatttacttcctgtattttaagtaacatgatagggtacttagagattaattgccaagaaactttttgaatatagtcaacctgcccgcacttgccatgatgagttttcttttgttccttccctctagtattctaggagatgaggttttgggaatctggtccagacatgctgagaaagctgatgtcaactgtgcctgtgtatctcattcaggaatcagtcttgttacaggagatgactttggcatggttaagttatttgacttcccatgtccagaaaaatttgtaagtttgtgttttgtttactattatcagtttactcctaattttgatgtcttatcatcagcacttttccccatatatttaaaatgttttgtcctaatttctaaatttttccccaaactttctaaatctatttactttgaaataaaagctattagaaacaaatcctctccctcgagtaataccatctttggaaccatcctacaaaagctgtaattagcttttcaccaaacctataatcagttatcaaatttcaaatgcttttccttagagaaaaatggtcagagtacctggagacatctgactgcccacacagcctggttttgcagatccactactcatgctgaaaagcattctaatcactggctgcggtgctaactccctactctctccacagctcttgtcatagagattatagttcctaataagagcctttgacttctgtgtgcaccaaatgccctgagcttgtctgtcattgttttttaggcaaaacacaaaaggttcttgggtcattcgccccatgtgacaaatattcgatttaccagtggtgatcgacatgttgttagtgctggaggtgatgactgcaggttagtaactttctcagcccatgaagagcagactatgttactagttaagagacttaatacaacaactcctacagctttggtttatgaaatcagctagtcaacattagtagaaggtagtataaccagatggctcttcagaatctcatatttatgcaaatacagaataaaaggagttaaagaggaaaaatattacacatgtaacctgaaagcacaactgaaaaatattaaactgttatgaaaatctaaaaacataattaactccctgcaattttcttctctgattgcagcttatttgtctggaaatgtgtacatacacctcactgagagatgctgagatgactacagaaattaactttgagaccagaattacagagaagaaaaaccaaaacccaaccctgcatggtcaagtggtgctaacccaagactgtaacagggagaaatgcccagaatcatcaaaatagtgaaagactgatctgttcaaaatatttgctatatgcactgggtataatccgtaatccatacactgccagataatgccatttcaaggaaggatcgaatacttgatggtaaaggccaagtccccctgtattgggaagtgtgtgatttcggcagacctgctgggaaaatttagggtagagcactctttacagaagaactcaaaaacccaatttggataattttcattatctttttagcaaaatggtttcttaatgtttatattttattttcaaggttcattgtttaatgaaatattttattcttgcatttccataaggaaagggaaagtcatgatcatcctaaaggatcacagtttttaaaaggcaaacattttccctaaggaaacagacacaagctttcctagagaatatgatgttttttaggcattaataaggtccttttttataaaggacacttttctcctagtagttttgaattcaggaacagatccaaagttagcagtatatggctgctacatttccattttcattttcgagccatcagtttatgttcagatgccatctctgtaatcgcacatttaaaacataactgtagcctcactaatggaaaagtagtatgatgaacaatcattcccaatggtgtacaatgtaagggttttagggagcaacagtatttaactggaagaaagaattgcatatttaatgtagtctaatatatacacatttgtttaacatgtaaacaaaagtgttaaattcacatatacaacattatacaatttaatcactcttggaataaaatttttatagccttttttctattgggaaaatttgtttagatgtgtgccactccataggtttatttccaaaatgaatgagcccaactccatttgtaaaaacttgtcagttagaattcctttttttagtggattagggctgaattcttagatccttatttcttttcactttaaatgctgccaaagatcactactcatcattcaggaattcgctgtctagcctatctgtagtttcctgaagattgaaaattatgtagactgctatttaaaaatatatttttctaagtgtgaggtttaagatgctgtattgaccctatgagtttttaatgtgttaattatctttatagcataatagatcgctttaggttcctggaatcccatttggtctgacaggatatatgaagattcttaatacctattttctgtgtctaatacttggttaatactaaaaatagaaatgactaaattacatcacagaaagcataaccagtgattgaacctggtagttttaaagctctaaatagctgtggctgaaggactgattatggggctaagaagcttgaaacgtaagttggtacttgttcatcagtggattctcctaaattaagccaaattttgaaatacatgactattaagtttctactcatgtatttacagtcagtcaataaattaaaggaggaaaaaaatccctgaacaacctgcccataaaaagaaaaatactctacatttgagcctgctgcagttttaaattttccctctgggtcaagtttgccagcttttggctacagagaaattatatttccattacagtgcaggtagaaactctgtaaccttaagcatgtaaactacatagaataaaactgtttccactgcatttctgtccttcaaagtggccaacctgattaagtcagccttaatcactgctgctgtcagtttcacgactaaaggtcatattgactaagtagtcatcagctgaccacctcgctgtatcagccagcaacgaggggaaggtgaagaaacatgataggccatatagaatctgccctatgtttacttttttaacccagataattatttttgtgtgcagtatctaagctcctgattgtgtaacctgggacttctggcaccttttgttccattcattttatgtataaaatgcatgccaaagcacactgtgccctctggtacccttgcttccaatcgccaaccatgctcatttccttcctttttttgtggtccctttttgtggtgatcattttaaaccacgtcatccaacaaatgttttatggtcaaccttagcttgttcataagccatagcaactgaaagattaaactcttaaatatgtgtctgggcagtggctattaaatagcaaaaaacaatcagattttagtattttattatttccttgtaaaatggctgaactaaattaaacccttgtttcccatttgttctataatttatagtgaaactgagaacaaaactatctttataaatgatagctaaaagtatttccagatatttaaacaatttaaaataaatttcttctgcagagatgcaaagcatctcaacactggaatgaacaaatgccttaaattcaatggagtaaacctttagaatgaagaggaactgtcatttcacccaagccgaagacaacagccttatgcacttgtgtgctctgtctttgctgcttctcgtgtttcaagcctttcctgtgggatcagcacagcaaagtgcaacttaccaaatggtttaatgactggttaattctttcttctcccaatggaaaagcaatggcaacacaacagtagactgctggcttgacaatcttaaacgtgagcctttgcacatgtaggtttatcatcatttgagtatacgactaagcaagtcaatgaactttttttttttttttagcagtttaatttggtcctgagaatgttgcagtctttattaccccttttgcattaatccacttttctaaccaccttttaagctttaatttttaacactatacaccaagtctttgaaatcagtgatctgttatttaactctaaagcatttgacacttcttgccttaacagttttaaaaaccacacacaaaaaaactctgtaagtaatacagtaggccaaaagtttcatcctatctatcttgcagtttacctatctgatctgatctctgtaattatagttctgtcatttaaaatatactatttaaatctaatttttacatttcaaaaattatcttcagtagtaactaagtatattttctgtggattctgagaatgttatttttcagaatgtgagaatatatatgtacatttataatcttgtgactttaaagtctgttttcagatacagtatgtaaatacttgtaaaaaaatttgtataattttgtgataatgtagtttcccaaaaaaattatttagaaggcattatgttattagtaaatgagagcactgtatagaactgttcctattttctgcacttgccattccagctgcctccactgtccatacccacctcattcatcctgtcacagaaggcaggaaaactgggaactttaccaaagtagcactcagcctgagaggcctgtataatcatgcttttcaaactaaattcacttaaaaattaaaaagcagaattgaatattttaagcagcctcagtacctttggccaatgctgttttcatggtggattatgaacattatataatctttgggaaaagtgaaagtagtacaatttttagaataatgacaactgcctcactgcatctctccactcacacagcaaccgtgtagccccctaagctgcagtaccatgactaaccatgatgtcaatttcatatgctgatcctcacaacagcagtgcacaaacatgccccaaatattttaacagaatttagctcttccttaagctgtcttttcatagtaaaaacaaaacaaaaacacccaatgttaaaaccacataataaacttacaaacttgaaaaattagacacttcagatagataggcaataaaacttcatattatgaaagcaatatattccaagtttcaaagatttgacaagttctgtagagtatctttcatcagtacatgaaaacttccaaactgcatgatcttctgccaggcaggactgggtgctattcgctggtttgaggtcgaatccatttcaaggcatgtcgtggtgggacattaatggtgggatggtagaatgtgcagtccggtcttgtacattgagtgttaaacctacaatgttttggatgatagaagggacattccatcttcttacaagcagggaagtaacggcagagctgactactggaaggtggtgctggtggtgcaactgctggttttggagacagtactggaattcttctactcacatgagtgaagggacaatctggtttagtacactttgcatcatatttacaatttgggtgaacaaacaaacatttttcagcaaatttacaattggggaaggctttgcagggtgagatggggtgatggtaggcacactcatccccatttttacaagcaggccagtacttgcagcgctccaaaagtttttctggtttctgtgccacactcagttcactcatctcagcttgatttttttctacagaatctccttttgtttcctcttctttaatggggggacttattctgggggtcctactttgtccctggaccacttctgctagcaattcttcttgagaagttcgagttctgggagcaactggaagtgtctgtttctgtggaactgtagagtagttagttgtttttgttacggattcttgagcttcagatatagccttcaaaatcagattcttgttagcttgtttagaaggtggaagagaaggtctcctttcaggctttgcaggcacagacacactgctggagatgcttcctgttcgagacccgtaatcatcatcttcttcctcctcttctccatcatgattgaatttttttactttaacaactgaacttaccacaggcaactttctcttccgaaagttttcatcctccatactcattttctccgagttgtttctaaagaacggactatacgtttcttctaagctgttaagcacctctggttcacacaaacgtcctgtttcatatacccaactactctgcatatcaagctgcttggcagcatgaatactattctgctgctgttgaaattgcaacctgtttaaatgaacaccactatctgcatttctacttgcaggtggtcgataaatttcaatagaagggcgagaagaaccatatgtaagtgtcactgtaggttttttctgagataagggattctcctgcacaaagttgaggtcttcgtcaatgagatcatctggttctggcttaatatcaatcacatcttcagagggtgctggctccctcaaaggtttcactgttgacattagtcgggttgcagctccatcatcgtaagtctgtctgacatttgtggtttttgactcctgcgaacttgtagaaactctggaatctcttttttcaggtctcgcgctaggaatggcaagtggtggcactgcagcttcatgcctcctctcatctccccgactgaaattgctcttgtttgaaggcacgttactatcaaagatgttggtatcagaagacttcagactagagggttcagttgtaacagagcgaagtttatctaatacaccatgaagccaacataagctcctaattcttgtaatttccccttaatggcactccggatcttgcggctgatctcggtgccgatctccatggctctgcggcgtgcgggaactcagcactgcgcggcgcttggcttacccggaggctgccgcggactcctaccccgcagccgggacaccaccgcctcc

SEQ ID NO: 17244 - RNA, 14466 nt, Homo sapiens
  source 1..14466: mol_type = other RNA
tcaggccaggcacagtggctcacacctgtaatcttatcactttgggaggctgaggcaggtggatcgcttgagcccaggagttcaagaccagcctgggcaacatggtgaaaccccatcgctataaaaaacaacaattagccgggtgtggtggcacatgcctgtagtccctgctactcaggaggctgaggtgggaggatcacttgagcctggggaggtcaaggctttagtgagctgtgatggtgccactgcactccagcctgggtgacagagtgagaccccatttaaaaaacaaaaacaaaaacaaaaaaaaatgtgacatatagttgactaagaagtacatttcaatacaggattgaaagaacccacatatgttaattaaacacaagcgcagaatttgtgccttttacataaaggaagaatgcacataggcatgctttcagacaagcaattcatctagcagaaaaggaaggaatacatttttcagcccttccaggaataaaatccataaatgggctctatttcgtcctccaacacttgtatttcccacgtcatttactcctgcacacccccactcactagaagcctgctaaactgttccagtgagatattttaacacctgatagggaataaatatgcttctgttttggccttcaaaaataagctctgggccagttgcagtggctcacgcctgtaatcccaacactttgggaggccgaggtgggcggatcacgaggtcaggagtttgggatcagcctggccaatatggtgaaactccatctctactaaaaatacaaaaattagccaggcatggtgcctgtaatcccagctacttgggaggctgaaggagaagaatcgcttgaacctgggaggcacaggttgcagtgagccgagatcacaccactgcactccaggccaggtgacagagcgacactctgtctcaaaaaaataaataaatcaactctgtagcatagcatttgtaattctattattttgccttacatttccattatccttttaataaaattgtttttttacatcttcctaatcaagaagtattatgaggccaggcacagtggctcatacctggaatcccagcactttgggaggccgaggcaggcagatcacctgaggtcaaggtatttgagaccagcctggccaacatggtgaaaccccatctctactaaaaatacagaaattagctgggtgtggtggtgcacacctgtaatgctagctactcgggaggctgaggtaggagaatcgcttgaacctgggaggcagaggttgcaataagcctagatcatgccactgcactcaagcctgggagacagagcgagactacatcttaaaaaaaaaaaaaaaagtattatgagagaggataatgtattgtaatgtattgtagaggctaaataaaattatgctcatgtcagaaaaaaagagtatttctcaaaataaaattcactgaaactggatgtttattttgactgagatatagtatatcctcaaattgccatagaaagtttacaagaatattagaggtaaattataaatatcagggcctttttaaaaaaaaaagattctgcttataacttggtatttgtttataataaaaattatagtagccaataatgaacacttactctggcttggttatttacttaggtcaaaagaaggaggagcggttaaactgtgggatcaggaactgaggcggtgccgtgccttcaggcttgagacaggacaagccacagattgtgttcgttctgtgtgcagaggcaaagtaagatgttccatgagctgatacagtgcagcagaaaacagaaagtggttattactgtgattccctcaccctttgcagcctaatgaacaatacttaataatgcataacgatggatttgcttgccaacattactctgtctttgctgctttctttgccaaagttagcaccagtgtggtgcataagctaggaagctattctgtctaaatactgtatgtaaacctccaatattttctagaatctgccaatttaacaactctagtagacataattgaaagcccttggcagttgactcatattaggacagctgtctccattttttaaaaaaacacacattccctagataaaacgtgcagtaaacaaacaatgaaatactactcagccataaaaaataatgaaattctgtcattcttggtggcaacatggatgagactggaggacatgatgtgaagtgaaataagccaggcacagaaagataaatacatgttctcactcctgtgcagaaactaaaaaagttgatcccacagaggtggagagtagaatagtggttactggaggcggacaagggggagggggagggggatagggaaggactggttaaaggatacaagtttacacagccagataggaatagtatgttttagtattctgtagtactgtaggatgactatagttaagaatcacgtatttatgtattttcaggtatttacaagagaggattttgaaagtttccatcacaaagaaatgataaatgtctgaggtgatggttatgcgtattaccctatgccctatagatatgtataattatgtgtcaatttcaaaataaaaattcaaaactacaactcctatgaaaatttttgagcgtgtttgtacttattaagtgtatttataaatcatacggatattatcttcagcctgcatattaaattgtagttaagcttttactttttaactaaaaaataaattctattattttttcctatatcccactgcactgaccccagtttggaaatcctaagattatcaaataaaaactttgattattgaagaatccaggtgtactgccacagaaaagttctattctgtagcatggactctaatatgtaatctagcccattgtgcttacagatagatgtgtgcctgtagtcatagaaaaatttgcatgagctaatgactgccttgctactagattagctcaaagcaaaaagttctctgaaagcaggtcaatagggtcatttttatattatgaagaagaaaagcagctgttgtattacattcactgtattggtcctgcttgtgtttcagggcaagatccttgttgggacaaggaatgctgaaataatcgaagttggagagaaaaatgcagcttgtaatattttagttaacggtcatgtggatgggccaatctggggactagcaacacatccttccagggattttttcctttctgctgcagaagatgggacagtgagactttgggatattgctgataaagtaagtacagataatttttttaaaagaggttacaacttctaaaaagaaaagttggaagttctaaattgctagtacttaaagaactgccagaattctgttgagcattttgaggggaaactggtataatttagaagtacttcacttaatgtttcctatgactctttttttttttttttttaaatgcagaagatgttaaacaaagtgaatttgggacatgctgctcgtactgtgtgttacagccctgaaggggacatggtggctattggaatgaaaaatggagaatttatcattttactagtgagttctctaaaaatatggggaaagaagagagacaggagatgtgcaatccatgatatcaggttagtgaacaaatggaatagagtttctagtatatacttgatttaacttccatttgtaaaattttccatagccttgccttcaaaaagaggtccccagggcctgtagcatttcccgtattataaattgtatgctaaaatatggctgtttgtatactacttaattcttcttgctaaattataaacccactgggcaccaactataatagcaagtactagtaggtaatgtttgatgaattcatgttaacacttagccatgtccattaagttcatcccaccaagaggtatctcccactgtaatacaagagagctatctgcccttcaaaagttgtcaccctggaaaactaaagttgtgatttcaaacatatcttctcttagtaacctcagtttgggaatatgtagttcattaatttaatcaatacctattgattaaatgttccagaatccaaattaatttaaatgtttcttaaacctttgtttttcagtgcttaagcatttttcaacagtggctaccatttacggagtacttccgtgtgatcagtagataagattattgaatctaggtctgtcaaaagcttgtacacttttcatcagtaaaatccttttacaaatgaaaccttcctcagaacttcaatatataaaatagtaacagtggcttcccttagcttttacatgtctctatcgtacctcagtaagactcatgggccatttcaagagactgaattgtcccatatgactccaaagattgctaggcaaatagcatttcactttgtcttttaaataagttcttcaggccgggcgcggtggctcatgcctgtaatcccagcactttgggaggccgaggcaggcagatcacctgaagtcaggagtactcgaccagcctggccaacatagtgaaaccccatctcaactaaaaatacaaaaatcagccgggcgtggtggcaggcgcctgtaatcccagctactcagggggctgaaacaggagaatcgcttgaacccgggaggcggaggttgcgccatcgcactccagcctgggagacaagagcgagacttcgtctcaaaaaaaaaaaattcttcttccaagattcaagttgtgtcatttcaccttaataactggaggttagttaagctgggctgtgttctttgcttaatattaagacaacgttttttccagatggaagaaaactatcttaatgaattgttagcttattaattatgtaatgctaatggcttttaaaagctgagatgttctgactgggtgttgtggctcacacctgtaatcccagtaccttgggaggccaagggggaaggattgcttgaggccaggagtttgggaccatagtgagaccccgcctctatttaaaaaattaaattttgttttgttttgttttgagttggagttttgctcttgttgcccatgctgaagtgcaatggtgcaatctcagctcaccacaacctgtgcctcctgggttcaagcgattctcctgcttcagcctcccgagtagatgggattacaggcgtgcaccaccatgcctggctaattttgtatttttagtagagacagggtttctctatgttggtcaggctggtctcaaactctcgacctcaggtgatctgcccgcctccgcttcccaaagttctgggattataggtgtgagccactgggcctggcctaagaaagtttttttaagccattagacgtttttaaaggaattgggagatgacaattggggaaatatttaaaatttaagtaaaatataaagcttccttatttcatgtaacccagacaatctcagtatacatgatcagttgtgtctgacaggtaaatctatttgaggccttatcacacgttacttttaagaactagaaaggaaaagtcactgatcttaagtatttataatacttcatgtggtctaatactttttacgttttgttttgattcagatttagtccggattcccggtatctggcagtaggttctagtgagaactcagtggatttttatgacctaacgctgggccccactcttaacagaatcagctactgcaaagacattccaagctttgtcattcaaatggacttctctgcagatagcagttatctccaggtacagtaccaatactgtatacccaggtggcaagttcttctgcttttacatttcgtgttagtgaatgcatttaaagttcctgagctccagagctccagcttctcaactcctccctttgtaccttctgacctacagctcccctttcctcccccacttatcagagcttttctcctattaagtttttgtagtgatcttttgcatacttaataatgttagacatgtaaatcaagtagcaatatgctagtattctgtaaaccccctgtggattttgtctctcacctaatggaattcttgtcccattttaatctgatgaaaaaggtctctagtggctgctataaacggcatgtctatgaagtgccttcaggaaaacatcttatggatcatgccgctattgacagaattacttgggctacatggactaggtaaatacttatatattcacaaggcaagaactgactttgaaggccagttagaaaatcctatttctgaactgttagagccattccaataaggaatagtaattgagtttcaagtttttgttaccatattttgaaatggtatgttcatgttgggacccctttttattgaatatatttccatgttttatcagtttccatgatttatcaagttttttttttaaggaaatcaaagttttaactttaaagataccctgatatttttcttaatgctaaatttaatgactggcaaaaaggtattgggtgctgttaagcaactgttattaattctctatctaaaggaatgctatcttgaatctattagaagtcaaagcttccaaatttgttcaaatttcctggctgtatgacaggtaaccatgactatccatttttttggccaatgaaaaatgccatcaaattcctgtatcagccaggcatatagtggctcatgcctgtaatctctgatgtagcaggccgaggtgggaggatcacttgagcctagaagttttgataccagcctgggcaacatagcaagaccccatctctgaaatttttttaattcctatgtcataagtcatttttatttttgtagagatagggatctcacaatattgcccaggctggtctcaaactcttggcctcaagcagtcctcctgcctcagcctcccaaaatgttgggattactggtatgtgctgctggacccagccaagtagcacttttaatttgaaaaatagttctatcagttttcagtcaggcgcggtggctcagcctgtaatcccagcactttgggaggccgagcgggggtgatcacctgaggtcgggagttcgagactagcctgaccaacatggagaaaccctgtctctactaaaaatacaaaataagccgggcatgttagcgcatgcctgtgatcccagctactcgggaggctgaggcaggagaattgcttgaacccaggaggcagaggttgcggtgagccgagatcatgccattgcactccagcctgggtaacaagagcgaaaactccgtctcaaaaaaaaaaaaagaaaaaatagttctatcagttttcataaagtactactttaatcttaaaaagattaatctagaaacccttcaaattataaaatgtcatttttaaaaggcaggagttgatatcctgatgaaattcaggtctccaaacaacttaccataatttacttcctgtattttaagtaacatgatagggtacttagagattaattgccaagaaactttttgaatatagtcaacctgcccgcacttgccatgatgagttttcttttgttccttccctctagtattctaggagatgaggttttgggaatctggtccagacatgctgagaaagctgatgtcaactgtgcctgtgtatctcattcaggaatcagtcttgttacaggagatgactttggcatggttaagttatttgacttcccatgtccagaaaaatttgtaagtttgtgttttgtttactattatcagtttactcctaattttgatgtcttatcatcagcacttttccccatatatttaaaatgttttgtcctaatttctaaatttttccccaaactttctaaatctatttactttgaaataaaagctattagaaacaaatcctctccctcgagtaataccatctttggaaccatcctacaaaagctgtaattagcttttcaccaaacctataatcagttatcaaatttcaaatgcttttccttagagaaaaatggtcagagtacctggagacatctgactgcccacacagcctggttttgcagatccactactcatgctgaaaagcattctaatcactggctgcggtgctaactccctactctctccacagctcttgtcatagagattatagttcctaataagagcctttgacttctgtgtgcaccaaatgccctgagcttgtctgtcattgttttttaggcaaaacacaaaaggttcttgggtcattcgccccatgtgacaaatattcgatttaccagtggtgatcgacatgttgttagtgctggaggtgatgactgcaggttagtaactttctcagcccatgaagagcagactatgttactagttaagagacttaatacaacaactcctacagctttggtttatgaaatcagctagtcaacattagtagaaggtagtataaccagatggctcttcagaatctcatatttatgcaaatacagaataaaaggagttaaagaggaaaaatattacacatgtaacctgaaagcacaactgaaaaatattaaactgttatgaaaatctaaaaacataattaactccctgcaattttcttctctgattgcagcttatttgtctggaaatgtgtacatacacctcactgagagatgctgagatgactacagaaattaactttgagaccagaattacagagaagaaaaaccaaaacccaaccctgcatggtcaagtggtgctaacccaagactgtaacagggagaaatgcccagaatcatcaaaatagtgaaagactgatctgttcaaaatatttgctatatgcactgggtataatccgtaatccatacactgccagataatgccatttcaaggaaggatcgaatacttgatggtaaaggccaagtccccctgtattgggaagtgtgtgatttcggcagacctgctgggaaaatttagggtagagcactctttacagaagaactcaaaaacccaatttggataattttcattatctttttagcaaaatggtttcttaatgtttatattttattttcaaggttcattgtttaatgaaatattttattcttgcatttccataaggaaagggaaagtcatgatcatcctaaaggatcacagtttttaaaaggcaaacattttccctaaggaaacagacacaagctttcctagagaatatgatgttttttaggcattaataaggtccttttttataaaggacacttttctcctagtagttttgaattcaggaacagatccaaagttagcagtatatggctgctacatttccattttcattttcgagccatcagtttatgttcagatgccatctctgtaatcgcacatttaaaacataactgtagcctcactaatggaaaagtagtatgatgaacaatcattcccaatggtgtacaatgtaagggttttagggagcaacagtatttaactggaagaaagaattgcatatttaatgtagtctaatatatacacatttgtttaacatgtaaacaaaagtgttaaattcacatatacaacattatacaatttaatcactcttggaataaaatttttatagccttttttctattgggaaaatttgtttagatgtgtgccactccataggtttatttccaaaatgaatgagcccaactccatttgtaaaaacttgtcagttagaattcctttttttagtggattagggctgaattcttagatccttatttcttttcactttaaatgctgccaaagatcactactcatcattcaggaattcgctgtctagcctatctgtagtttcctgaagattgaaaattatgtagactgctatttaaaaatatatttttctaagtgtgaggtttaagatgctgtattgaccctatgagtttttaatgtgttaattatctttatagcataatagatcgctttaggttcctggaatcccatttggtctgacaggatatatgaagattcttaatacctattttctgtgtctaatacttggttaatactaaaaatagaaatgactaaattacatcacagaaagcataaccagtgattgaacctggtagttttaaagctctaaatagctgtggctgaaggactgattatggggctaagaagcttgaaacgtaagttggtacttgttcatcagtggattctcctaaattaagccaaattttgaaatacatgactattaagtttctactcatgtatttacagtcagtcaataaattaaaggaggaaaaaaatccctgaacaacctgcccataaaaagaaaaatactctacatttgagcctgctgcagttttaaattttccctctgggtcaagtttgccagcttttggctacagagaaattatatttccattacagtgcaggtagaaactctgtaaccttaagcatgtaaactacatagaataaaactgtttccactgcatttctgtccttcaaagtggccaacctgattaagtcagccttaatcactgctgctgtcagtttcacgactaaaggtcatattgactaagtagtcatcagctgaccacctcgctgtatcagccagcaacgaggggaaggtgaagaaacatgataggccatatagaatctgccctatgtttacttttttaacccagataattatttttgtgtgcagtatctaagctcctgattgtgtaacctgggacttctggcaccttttgttccattcattttatgtataaaatgcatgccaaagcacactgtgccctctggtacccttgcttccaatcgccaaccatgctcatttccttcctttttttgtggtccctttttgtggtgatcattttaaaccacgtcatccaacaaatgttttatggtcaaccttagcttgttcataagccatagcaactgaaagattaaactcttaaatatgtgtctgggcagtggctattaaatagcaaaaaacaatcagattttagtattttattatttccttgtaaaatggctgaactaaattaaacccttgtttcccatttgttctataatttatagtgaaactgagaacaaaactatctttataaatgatagctaaaagtatttccagatatttaaacaatttaaaataaatttcttctgcagagatgcaaagcatctcaacactggaatgaacaaatgccttaaattcaatggagtaaacctttagaatgaagaggaactgtcatttcacccaagccgaagacaacagccttatgcacttgtgtgctctgtctttgctgcttctcgtgtttcaagcctttcctgtgggatcagcacagcaaagtgcaacttaccaaatggtttaatgactggttaattctttcttctcccaatggaaaagcaatggcaacacaacagtagactgctggcttgacaatcttaaacgtgagcctttgcacatgtaggtttatcatcatttgagtatacgactaagcaagtcaatgaactttttttttttttttagcagtttaatttggtcctgagaatgttgcagtctttattaccccttttgcattaatccacttttctaaccaccttttaagctttaatttttaacactatacaccaagtctttgaaatcagtgatctgttatttaactctaaagcatttgacacttcttgccttaacagttttaaaaaccacacacaaaaaaactctgtaagtaatacagtaggccaaaagtttcatcctatctatcttgcagtttacctatctgatctgatctctgtaattatagttctgtcatttaaaatatactatttaaatctaatttttacatttcaaaaattatcttcagtagtaactaagtatattttctgtggattctgagaatgttatttttcagaatgtgagaatatatatgtacatttataatcttgtgactttaaagtctgttttcagatacagtatgtaaatacttgtaaaaaaatttgtataattttgtgataatgtagtttcccaaaaaaattatttagaaggcattatgttattagtaaatgagagcactgtatagaactgttcctattttctgcacttgccattccagctgcctccactgtccatacccacctcattcatcctgtcacagaaggcaggaaaactgggaactttaccaaagtagcactcagcctgagaggcctgtataatcatgcttttcaaactaaattcacttaaaaattaaaaagcagaattgaatattttaagcagcctcagtacctttggccaatgctgttttcatggtggattatgaacattatataatctttgggaaaagtgaaagtagtacaatttttagaataatgacaactgcctcactgcatctctccactcacacagcaaccgtgtagccccctaagctgcagtaccatgactaaccatgatgtcaatttcatatgctgatcctcacaacagcagtgcacaaacatgccccaaatattttaacagaatttagctcttccttaagctgtcttttcatagtaaaaacaaaacaaaaacacccaatgttaaaaccacataataaacttacaaacttgaaaaattagacacttcagatagataggcaataaaacttcatattatgaaagcaatatattccaagtttcaaagatttgacaagttctgtagagtatctttcatcagtacatgaaaacttccaaactgcatgatcttctgccaggcaggactgggtgctattcgctggtttgaggtcgaatccatttcaaggcatgtcgtggtgggacattaatggtgggatggtagaatgtgcagtccggtcttgtacattgagtgttaaacctacaatgttttggatgatagaagggacattccatcttcttacaagcagggaagtaacggcagagctgactactggaaggtggtgctggtggtgcaactgctggttttggagacagtactggaattcttctactcacatgagtgaagggacaatctggtttagtacactttgcatcatatttacaatttgggtgaacaaacaaacatttttcagcaaatttacaattggggaaggctttgcagggtgagatggggtgatggtaggcacactcatccccatttttacaagcaggccagtacttgcagcgctccaaaagtttttctggtttctgtgccacactcagttcactcatctcagcttgatttttttctacagaatctccttttgtttcctcttctttaatggggggacttattctgggggtcctactttgtccctggaccacttctgctagcaattcttcttgagaagttcgagttctgggagcaactggaagtgtctgtttctgtggaactgtagagtagttagttgtttttgttacggattcttgagcttcagatatagccttcaaaatcagattcttgttagcttgtttagaaggtggaagagaaggtctcctttcaggctttgcaggcacagacacactgctggagatgcttcctgttcgagacccgtaatcatcatcttcttcctcctcttctccatcatgattgaatttttttactttaacaactgaacttaccacaggcaactttctcttccgaaagttttcatcctccatactcattttctccgagttgtttctaaagaacggactatacgtttcttctaagctgttaagcacctctggttcacacaaacgtcctgtttcatatacccaactactctgcatatcaagctgcttggcagcatgaatactattctgctgctgttgaaattgcaacctgtttaaatgaacaccactatctgcatttctacttgcaggtggtcgataaatttcaatagaagggcgagaagaaccatatgtaagtgtcactgtaggttttttctgagataagggattctcctgcacaaagttgaggtcttcgtcaatgagatcatctggttctggcttaatatcaatcacatcttcagagggtgctggctccctcaaaggtttcactgttgacattagtcgggttgcagctccatcatcgtaagtctgtctgacatttgtggtttttgactcctgcgaacttgtagaaactctggaatctcttttttcaggtctcgcgctaggaatggcaagtggtggcactgcagcttcatgcctcctctcatctccccgactgaaattgctcttgtttgaaggcacgttactatcaaagatgttggtatcagaagacttcagactagagggttcagttgtaacagagcgaagtttatctaatacaccatgaagccatacggtgaatcgaattgtgttgttccctagaaacagggacagatcctctgtcatttggtcctgacttttcttgttggccaccatcaccataatgtaatcaggaagttcttcatcaacataagctcctaattcttgtaatttccccttaatggcactccggatcttgcggctgatctcggtgccgatctccatggctctgcggcgtgcgggaactcagcactgcgcggcgcttggcttacccggaggctgccgcggactcctaccccgcagccgggacaccaccgcctcc

SEQ ID NO: 17245 - RNA, 14916 nt, Homo sapiens
  source 1..14916: mol_type = other RNA
tcaggccaggcacagtggctcacacctgtaatcttatcactttgggaggctgaggcaggtggatcgcttgagcccaggagttcaagaccagcctgggcaacatggtgaaaccccatcgctataaaaaacaacaattagccgggtgtggtggcacatgcctgtagtccctgctactcaggaggctgaggtgggaggatcacttgagcctggggaggtcaaggctttagtgagctgtgatggtgccactgcactccagcctgggtgacagagtgagaccccatttaaaaaacaaaaacaaaaacaaaaaaaaatgtgacatatagttgactaagaagtacatttcaatacaggattgaaagaacccacatatgttaattaaacacaagcgcagaatttgtgccttttacataaaggaagaatgcacataggcatgctttcagacaagcaattcatctagcagaaaaggaaggaatacatttttcagcccttccaggaataaaatccataaatgggctctatttcgtcctccaacacttgtatttcccacgtcatttactcctgcacacccccactcactagaagcctgctaaactgttccagtgagatattttaacacctgatagggaataaatatgcttctgttttggccttcaaaaataagctctgggccagttgcagtggctcacgcctgtaatcccaacactttgggaggccgaggtgggcggatcacgaggtcaggagtttgggatcagcctggccaatatggtgaaactccatctctactaaaaatacaaaaattagccaggcatggtgcctgtaatcccagctacttgggaggctgaaggagaagaatcgcttgaacctgggaggcacaggttgcagtgagccgagatcacaccactgcactccaggccaggtgacagagcgacactctgtctcaaaaaaataaataaatcaactctgtagcatagcatttgtaattctattattttgccttacatttccattatccttttaataaaattgtttttttacatcttcctaatcaagaagtattatgaggccaggcacagtggctcatacctggaatcccagcactttgggaggccgaggcaggcagatcacctgaggtcaaggtatttgagaccagcctggccaacatggtgaaaccccatctctactaaaaatacagaaattagctgggtgtggtggtgcacacctgtaatgctagctactcgggaggctgaggtaggagaatcgcttgaacctgggaggcagaggttgcaataagcctagatcatgccactgcactcaagcctgggagacagagcgagactacatcttaaaaaaaaaaaaaaaagtattatgagagaggataatgtattgtaatgtattgtagaggctaaataaaattatgctcatgtcagaaaaaaagagtatttctcaaaataaaattcactgaaactggatgtttattttgactgagatatagtatatcctcaaattgccatagaaagtttacaagaatattagaggtaaattataaatatcagggcctttttaaaaaaaaaagattctgcttataacttggtatttgtttataataaaaattatagtagccaataatgaacacttactctggcttggttatttacttaggtcaaaagaaggaggagcggttaaactgtgggatcaggaactgaggcggtgccgtgccttcaggcttgagacaggacaagccacagattgtgttcgttctgtgtgcagaggcaaagtaagatgttccatgagctgatacagtgcagcagaaaacagaaagtggttattactgtgattccctcaccctttgcagcctaatgaacaatacttaataatgcataacgatggatttgcttgccaacattactctgtctttgctgctttctttgccaaagttagcaccagtgtggtgcataagctaggaagctattctgtctaaatactgtatgtaaacctccaatattttctagaatctgccaatttaacaactctagtagacataattgaaagcccttggcagttgactcatattaggacagctgtctccattttttaaaaaaacacacattccctagataaaacgtgcagtaaacaaacaatgaaatactactcagccataaaaaataatgaaattctgtcattcttggtggcaacatggatgagactggaggacatgatgtgaagtgaaataagccaggcacagaaagataaatacatgttctcactcctgtgcagaaactaaaaaagttgatcccacagaggtggagagtagaatagtggttactggaggcggacaagggggagggggagggggatagggaaggactggttaaaggatacaagtttacacagccagataggaatagtatgttttagtattctgtagtactgtaggatgactatagttaagaatcacgtatttatgtattttcaggtatttacaagagaggattttgaaagtttccatcacaaagaaatgataaatgtctgaggtgatggttatgcgtattaccctatgccctatagatatgtataattatgtgtcaatttcaaaataaaaattcaaaactacaactcctatgaaaatttttgagcgtgtttgtacttattaagtgtatttataaatcatacggatattatcttcagcctgcatattaaattgtagttaagcttttactttttaactaaaaaataaattctattattttttcctatatcccactgcactgaccccagtttggaaatcctaagattatcaaataaaaactttgattattgaagaatccaggtgtactgccacagaaaagttctattctgtagcatggactctaatatgtaatctagcccattgtgcttacagatagatgtgtgcctgtagtcatagaaaaatttgcatgagctaatgactgccttgctactagattagctcaaagcaaaaagttctctgaaagcaggtcaatagggtcatttttatattatgaagaagaaaagcagctgttgtattacattcactgtattggtcctgcttgtgtttcagggcaagatccttgttgggacaaggaatgctgaaataatcgaagttggagagaaaaatgcagcttgtaatattttagttaacggtcatgtggatgggccaatctggggactagcaacacatccttccagggattttttcctttctgctgcagaagatgggacagtgagactttgggatattgctgataaagtaagtacagataatttttttaaaagaggttacaacttctaaaaagaaaagttggaagttctaaattgctagtacttaaagaactgccagaattctgttgagcattttgaggggaaactggtataatttagaagtacttcacttaatgtttcctatgactctttttttttttttttttaaatgcagaagatgttaaacaaagtgaatttgggacatgctgctcgtactgtgtgttacagccctgaaggggacatggtggctattggaatgaaaaatggagaatttatcattttactagtgagttctctaaaaatatggggaaagaagagagacaggagatgtgcaatccatgatatcaggttagtgaacaaatggaatagagtttctagtatatacttgatttaacttccatttgtaaaattttccatagccttgccttcaaaaagaggtccccagggcctgtagcatttcccgtattataaattgtatgctaaaatatggctgtttgtatactacttaattcttcttgctaaattataaacccactgggcaccaactataatagcaagtactagtaggtaatgtttgatgaattcatgttaacacttagccatgtccattaagttcatcccaccaagaggtatctcccactgtaatacaagagagctatctgcccttcaaaagttgtcaccctggaaaactaaagttgtgatttcaaacatatcttctcttagtaacctcagtttgggaatatgtagttcattaatttaatcaatacctattgattaaatgttccagaatccaaattaatttaaatgtttcttaaacctttgtttttcagtgcttaagcatttttcaacagtggctaccatttacggagtacttccgtgtgatcagtagataagattattgaatctaggtctgtcaaaagcttgtacacttttcatcagtaaaatccttttacaaatgaaaccttcctcagaacttcaatatataaaatagtaacagtggcttcccttagcttttacatgtctctatcgtacctcagtaagactcatgggccatttcaagagactgaattgtcccatatgactccaaagattgctaggcaaatagcatttcactttgtcttttaaataagttcttcaggccgggcgcggtggctcatgcctgtaatcccagcactttgggaggccgaggcaggcagatcacctgaagtcaggagtactcgaccagcctggccaacatagtgaaaccccatctcaactaaaaatacaaaaatcagccgggcgtggtggcaggcgcctgtaatcccagctactcagggggctgaaacaggagaatcgcttgaacccgggaggcggaggttgcgccatcgcactccagcctgggagacaagagcgagacttcgtctcaaaaaaaaaaaattcttcttccaagattcaagttgtgtcatttcaccttaataactggaggttagttaagctgggctgtgttctttgcttaatattaagacaacgttttttccagatggaagaaaactatcttaatgaattgttagcttattaattatgtaatgctaatggcttttaaaagctgagatgttctgactgggtgttgtggctcacacctgtaatcccagtaccttgggaggccaagggggaaggattgcttgaggccaggagtttgggaccatagtgagaccccgcctctatttaaaaaattaaattttgttttgttttgttttgagttggagttttgctcttgttgcccatgctgaagtgcaatggtgcaatctcagctcaccacaacctgtgcctcctgggttcaagcgattctcctgcttcagcctcccgagtagatgggattacaggcgtgcaccaccatgcctggctaattttgtatttttagtagagacagggtttctctatgttggtcaggctggtctcaaactctcgacctcaggtgatctgcccgcctccgcttcccaaagttctgggattataggtgtgagccactgggcctggcctaagaaagtttttttaagccattagacgtttttaaaggaattgggagatgacaattggggaaatatttaaaatttaagtaaaatataaagcttccttatttcatgtaacccagacaatctcagtatacatgatcagttgtgtctgacaggtaaatctatttgaggccttatcacacgttacttttaagaactagaaaggaaaagtcactgatcttaagtatttataatacttcatgtggtctaatactttttacgttttgttttgattcagatttagtccggattcccggtatctggcagtaggttctagtgagaactcagtggatttttatgacctaacgctgggccccactcttaacagaatcagctactgcaaagacattccaagctttgtcattcaaatggacttctctgcagatagcagttatctccaggtacagtaccaatactgtatacccaggtggcaagttcttctgcttttacatttcgtgttagtgaatgcatttaaagttcctgagctccagagctccagcttctcaactcctccctttgtaccttctgacctacagctcccctttcctcccccacttatcagagcttttctcctattaagtttttgtagtgatcttttgcatacttaataatgttagacatgtaaatcaagtagcaatatgctagtattctgtaaaccccctgtggattttgtctctcacctaatggaattcttgtcccattttaatctgatgaaaaaggtctctagtggctgctataaacggcatgtctatgaagtgccttcaggaaaacatcttatggatcatgccgctattgacagaattacttgggctacatggactaggtaaatacttatatattcacaaggcaagaactgactttgaaggccagttagaaaatcctatttctgaactgttagagccattccaataaggaatagtaattgagtttcaagtttttgttaccatattttgaaatggtatgttcatgttgggacccctttttattgaatatatttccatgttttatcagtttccatgatttatcaagttttttttttaaggaaatcaaagttttaactttaaagataccctgatatttttcttaatgctaaatttaatgactggcaaaaaggtattgggtgctgttaagcaactgttattaattctctatctaaaggaatgctatcttgaatctattagaagtcaaagcttccaaatttgttcaaatttcctggctgtatgacaggtaaccatgactatccatttttttggccaatgaaaaatgccatcaaattcctgtatcagccaggcatatagtggctcatgcctgtaatctctgatgtagcaggccgaggtgggaggatcacttgagcctagaagttttgataccagcctgggcaacatagcaagaccccatctctgaaatttttttaattcctatgtcataagtcatttttatttttgtagagatagggatctcacaatattgcccaggctggtctcaaactcttggcctcaagcagtcctcctgcctcagcctcccaaaatgttgggattactggtatgtgctgctggacccagccaagtagcacttttaatttgaaaaatagttctatcagttttcagtcaggcgcggtggctcagcctgtaatcccagcactttgggaggccgagcgggggtgatcacctgaggtcgggagttcgagactagcctgaccaacatggagaaaccctgtctctactaaaaatacaaaataagccgggcatgttagcgcatgcctgtgatcccagctactcgggaggctgaggcaggagaattgcttgaacccaggaggcagaggttgcggtgagccgagatcatgccattgcactccagcctgggtaacaagagcgaaaactccgtctcaaaaaaaaaaaaagaaaaaatagttctatcagttttcataaagtactactttaatcttaaaaagattaatctagaaacccttcaaattataaaatgtcatttttaaaaggcaggagttgatatcctgatgaaattcaggtctccaaacaacttaccataatttacttcctgtattttaagtaacatgatagggtacttagagattaattgccaagaaactttttgaatatagtcaacctgcccgcacttgccatgatgagttttcttttgttccttccctctagtattctaggagatgaggttttgggaatctggtccagacatgctgagaaagctgatgtcaactgtgcctgtgtatctcattcaggaatcagtcttgttacaggagatgactttggcatggttaagttatttgacttcccatgtccagaaaaatttgtaagtttgtgttttgtttactattatcagtttactcctaattttgatgtcttatcatcagcacttttccccatatatttaaaatgttttgtcctaatttctaaatttttccccaaactttctaaatctatttactttgaaataaaagctattagaaacaaatcctctccctcgagtaataccatctttggaaccatcctacaaaagctgtaattagcttttcaccaaacctataatcagttatcaaatttcaaatgcttttccttagagaaaaatggtcagagtacctggagacatctgactgcccacacagcctggttttgcagatccactactcatgctgaaaagcattctaatcactggctgcggtgctaactccctactctctccacagctcttgtcatagagattatagttcctaataagagcctttgacttctgtgtgcaccaaatgccctgagcttgtctgtcattgttttttaggcaaaacacaaaaggttcttgggtcattcgccccatgtgacaaatattcgatttaccagtggtgatcgacatgttgttagtgctggaggtgatgactgcaggttagtaactttctcagcccatgaagagcagactatgttactagttaagagacttaatacaacaactcctacagctttggtttatgaaatcagctagtcaacattagtagaaggtagtataaccagatggctcttcagaatctcatatttatgcaaatacagaataaaaggagttaaagaggaaaaatattacacatgtaacctgaaagcacaactgaaaaatattaaactgttatgaaaatctaaaaacataattaactccctgcaattttcttctctgattgcagcttatttgtctggaaatgtgtacatacacctcactgagagatgctgagatgactacagaaattaactttgagaccagaattacagagaagaaaaaccaaaacccaaccctgcatggtcaagtggtgctaacccaagactgtaacagggagaaatgcccagaatcatcaaaatagtgaaagactgatctgttcaaaatatttgctatatgcactgggtataatccgtaatccatacactgccagataatgccatttcaaggaaggatcgaatacttgatggtaaaggccaagtccccctgtattgggaagtgtgtgatttcggcagacctgctgggaaaatttagggtagagcactctttacagaagaactcaaaaacccaatttggataattttcattatctttttagcaaaatggtttcttaatgtttatattttattttcaaggttcattgtttaatgaaatattttattcttgcatttccataaggaaagggaaagtcatgatcatcctaaaggatcacagtttttaaaaggcaaacattttccctaaggaaacagacacaagctttcctagagaatatgatgttttttaggcattaataaggtccttttttataaaggacacttttctcctagtagttttgaattcaggaacagatccaaagttagcagtatatggctgctacatttccattttcattttcgagccatcagtttatgttcagatgccatctctgtaatcgcacatttaaaacataactgtagcctcactaatggaaaagtagtatgatgaacaatcattcccaatggtgtacaatgtaagggttttagggagcaacagtatttaactggaagaaagaattgcatatttaatgtagtctaatatatacacatttgtttaacatgtaaacaaaagtgttaaattcacatatacaacattatacaatttaatcactcttggaataaaatttttatagccttttttctattgggaaaatttgtttagatgtgtgccactccataggtttatttccaaaatgaatgagcccaactccatttgtaaaaacttgtcagttagaattcctttttttagtggattagggctgaattcttagatccttatttcttttcactttaaatgctgccaaagatcactactcatcattcaggaattcgctgtctagcctatctgtagtttcctgaagattgaaaattatgtagactgctatttaaaaatatatttttctaagtgtgaggtttaagatgctgtattgaccctatgagtttttaatgtgttaattatctttatagcataatagatcgctttaggttcctggaatcccatttggtctgacaggatatatgaagattcttaatacctattttctgtgtctaatacttggttaatactaaaaatagaaatgactaaattacatcacagaaagcataaccagtgattgaacctggtagttttaaagctctaaatagctgtggctgaaggactgattatggggctaagaagcttgaaacgtaagttggtacttgttcatcagtggattctcctaaattaagccaaattttgaaatacatgactattaagtttctactcatgtatttacagtcagtcaataaattaaaggaggaaaaaaatccctgaacaacctgcccataaaaagaaaaatactctacatttgagcctgctgcagttttaaattttccctctgggtcaagtttgccagcttttggctacagagaaattatatttccattacagtgcaggtagaaactctgtaaccttaagcatgtaaactacatagaataaaactgtttccactgcatttctgtccttcaaagtggccaacctgattaagtcagccttaatcactgctgctgtcagtttcacgactaaaggtcatattgactaagtagtcatcagctgaccacctcgctgtatcagccagcaacgaggggaaggtgaagaaacatgataggccatatagaatctgccctatgtttacttttttaacccagataattatttttgtgtgcagtatctaagctcctgattgtgtaacctgggacttctggcaccttttgttccattcattttatgtataaaatgcatgccaaagcacactgtgccctctggtacccttgcttccaatcgccaaccatgctcatttccttcctttttttgtggtccctttttgtggtgatcattttaaaccacgtcatccaacaaatgttttatggtcaaccttagcttgttcataagccatagcaactgaaagattaaactcttaaatatgtgtctgggcagtggctattaaatagcaaaaaacaatcagattttagtattttattatttccttgtaaaatggctgaactaaattaaacccttgtttcccatttgttctataatttatagtgaaactgagaacaaaactatctttataaatgatagctaaaagtatttccagatatttaaacaatttaaaataaatttcttctgcagagatgcaaagcatctcaacactggaatgaacaaatgccttaaattcaatggagtaaacctttagaatgaagaggaactgtcatttcacccaagccgaagacaacagccttatgcacttgtgtgctctgtctttgctgcttctcgtgtttcaagcctttcctgtgggatcagcacagcaaagtgcaacttaccaaatggtttaatgactggttaattctttcttctcccaatggaaaagcaatggcaacacaacagtagactgctggcttgacaatcttaaacgtgagcctttgcacatgtaggtttatcatcatttgagtatacgactaagcaagtcaatgaactttttttttttttttagcagtttaatttggtcctgagaatgttgcagtctttattaccccttttgcattaatccacttttctaaccaccttttaagctttaatttttaacactatacaccaagtctttgaaatcagtgatctgttatttaactctaaagcatttgacacttcttgccttaacagttttaaaaaccacacacaaaaaaactctgtaagtaatacagtaggccaaaagtttcatcctatctatcttgcagtttacctatctgatctgatctctgtaattatagttctgtcatttaaaatatactatttaaatctaatttttacatttcaaaaattatcttcagtagtaactaagtatattttctgtggattctgagaatgttatttttcagaatgtgagaatatatatgtacatttataatcttgtgactttaaagtctgttttcagatacagtatgtaaatacttgtaaaaaaatttgtataattttgtgataatgtagtttcccaaaaaaattatttagaaggcattatgttattagtaaatgagagcactgtatagaactgttcctattttctgcacttgccattccagctgcctccactgtccatacccacctcattcatcctgtcacagaaggcaggaaaactgggaactttaccaaagtagcactcagcctgagaggcctgtataatcatgcttttcaaactaaattcacttaaaaattaaaaagcagaattgaatattttaagcagcctcagtacctttggccaatgctgttttcatggtggattatgaacattatataatctttgggaaaagtgaaagtagtacaatttttagaataatgacaactgcctcactgcatctctccactcacacagcaaccgtgtagccccctaagctgcagtaccatgactaaccatgatgtcaatttcatatgctgatcctcacaacagcagtgcacaaacatgccccaaatattttaacagaatttagctcttccttaagctgtcttttcatagtaaaaacaaaacaaaaacacccaatgttaaaaccacataataaacttacaaacttgaaaaattagacacttcagatagataggcaataaaacttcatattatgaaagcaatatattccaagtttcaaagatttgacaagttctgtagagtatctttcatcagtacatgaaaacttccaaactgcatgatcttctgccaggcaggactgggtgctattcgctggtttgaggtcgaatccatttcaaggcatgtcgtggtgggacattaatggtgggatggtagaatgtgcagtccggtcttgtacattgagtgttaaacctacaatgttttggatgatagaagggacattccatcttcttacaagcagggaagtaacggcagagctgactactggaaggtggtgctggtggtgcaactggttttggagacagtactggaattcttctactcacatgagtgaagggacaatctggtttagtacactttgcatcatatttacaatttgggtgaacaaacaaacatttttcagcaaatttacaattggggaaggctttgcagggtgagatggggtgatggtaggcacactcatccccatttttacaagcaggccagtacttgcagcgctccaaaagtttttctggtttctgtgccacactcagttcactcatctcagcatttgggtcctcaagctgcctgctcagcaagtgcaactgctgtgggtggaggagacctctgagtcccttgtttgaggctgcagtttggtttacgggtttcattccttcaaagcacatgtcctcctcttgatctgacatgtatcctggggggctggggacaccatccagcgtcactataaacttgggacttgcaggtttatctggttgtacaagatctcgtgtctgcataaggtgtcctgaaagtacccgaagggaatctgcagtcttcatccccgactcttggtttggtgccactactacttcctcagacagctttggcttcttcagaataaatgatcttgtgtctgcatggaccatggattccatgtcatagtaatcttgactcatctgcagagtttctgccattactgggtcgatttgcagtcgggataataattgcctctgttgagttccttgatttttttctacagaatctccttttgtttcctcttctttaatggggggacttattctgggggtcctactttgtccctggaccacttctgctagcaattcttcttgagaagttcgagttctgggagcaactggaagtgtctgtttctgtggaactgtagagtagttagttgtttttgttacggattcttgagcttcagatatagccttcaaaatcagattcttgttagcttgtttagaaggtggaagagaaggtctcctttcaggctttgcaggcacagacacactgctggagatgcttcctgttcgagacccgtaatcatcatcttcttcctcctcttctccatcatgattgaatttttttactttaacaactgaacttaccacaggcaactttctcttccgaaagttttcatcctccatactcattttctccgagttgtttctaaagaacggactatacgtttcttctaagctgttaagcacctctggttcacacaaacgtcctgtttcatatacccaactactctgcatatcaagctgcttggcagcatgaatactattctgctgctgttgaaattgcaacctgtttaaatgaacaccactatctgcatttctacttgcaggtggtcgataaatttcaatagaagggcgagaagaaccatatgtaagtgtcactgtaggttttttctgagataagggattctcctgcacaaagttgaggtcttcgtcaatgagatcatctggttctggcttaatatcaatcacatcttcagagggtgctggctccctcaaaggtttcactgttgacattagtcgggttgcagctccatcatcgtaagtctgtctgacatttgtggtttttgactcctgcgaacttgtagaaactctggaatctcttttttcaggtctcgcgctaggaatggcaagtggtggcactgcagcttcatgcctcctctcatctccccgactgaaattgctcttgtttgaaggcacgttactatcaaagatgttggtatcagaagacttcagactagagggttcagttgtaacagagcgaagtttatctaatacaccatgaagccatacggtgaatcgaattgtgttgttccctagaaacagggacagatcctctgtcatttggtcctgacttttcttgttggccaccatcaccataatgtaatcaggaagttcttcatcaacataagctcctaattcttgtaatttccccttaatggcactccggatcttgcggctgatctcggtgccgatctccatggctctgcggcgtgcgggaactcagcactgcgcggcgcttggcttacccggaggctgccgcggactcctaccccgcagccgggacaccaccgcctcc

SEQ ID NO: 17246 - RNA, 14841 nt, Homo sapiens
  source 1..14841: mol_type = other RNA
tcaggccaggcacagtggctcacacctgtaatcttatcactttgggaggctgaggcaggtggatcgcttgagcccaggagttcaagaccagcctgggcaacatggtgaaaccccatcgctataaaaaacaacaattagccgggtgtggtggcacatgcctgtagtccctgctactcaggaggctgaggtgggaggatcacttgagcctggggaggtcaaggctttagtgagctgtgatggtgccactgcactccagcctgggtgacagagtgagaccccatttaaaaaacaaaaacaaaaacaaaaaaaaatgtgacatatagttgactaagaagtacatttcaatacaggattgaaagaacccacatatgttaattaaacacaagcgcagaatttgtgccttttacataaaggaagaatgcacataggcatgctttcagacaagcaattcatctagcagaaaaggaaggaatacatttttcagcccttccaggaataaaatccataaatgggctctatttcgtcctccaacacttgtatttcccacgtcatttactcctgcacacccccactcactagaagcctgctaaactgttccagtgagatattttaacacctgatagggaataaatatgcttctgttttggccttcaaaaataagctctgggccagttgcagtggctcacgcctgtaatcccaacactttgggaggccgaggtgggcggatcacgaggtcaggagtttgggatcagcctggccaatatggtgaaactccatctctactaaaaatacaaaaattagccaggcatggtgcctgtaatcccagctacttgggaggctgaaggagaagaatcgcttgaacctgggaggcacaggttgcagtgagccgagatcacaccactgcactccaggccaggtgacagagcgacactctgtctcaaaaaaataaataaatcaactctgtagcatagcatttgtaattctattattttgccttacatttccattatccttttaataaaattgtttttttacatcttcctaatcaagaagtattatgaggccaggcacagtggctcatacctggaatcccagcactttgggaggccgaggcaggcagatcacctgaggtcaaggtatttgagaccagcctggccaacatggtgaaaccccatctctactaaaaatacagaaattagctgggtgtggtggtgcacacctgtaatgctagctactcgggaggctgaggtaggagaatcgcttgaacctgggaggcagaggttgcaataagcctagatcatgccactgcactcaagcctgggagacagagcgagactacatcttaaaaaaaaaaaaaaaagtattatgagagaggataatgtattgtaatgtattgtagaggctaaataaaattatgctcatgtcagaaaaaaagagtatttctcaaaataaaattcactgaaactggatgtttattttgactgagatatagtatatcctcaaattgccatagaaagtttacaagaatattagaggtaaattataaatatcagggcctttttaaaaaaaaaagattctgcttataacttggtatttgtttataataaaaattatagtagccaataatgaacacttactctggcttggttatttacttaggtcaaaagaaggaggagcggttaaactgtgggatcaggaactgaggcggtgccgtgccttcaggcttgagacaggacaagccacagattgtgttcgttctgtgtgcagaggcaaagtaagatgttccatgagctgatacagtgcagcagaaaacagaaagtggttattactgtgattccctcaccctttgcagcctaatgaacaatacttaataatgcataacgatggatttgcttgccaacattactctgtctttgctgctttctttgccaaagttagcaccagtgtggtgcataagctaggaagctattctgtctaaatactgtatgtaaacctccaatattttctagaatctgccaatttaacaactctagtagacataattgaaagcccttggcagttgactcatattaggacagctgtctccattttttaaaaaaacacacattccctagataaaacgtgcagtaaacaaacaatgaaatactactcagccataaaaaataatgaaattctgtcattcttggtggcaacatggatgagactggaggacatgatgtgaagtgaaataagccaggcacagaaagataaatacatgttctcactcctgtgcagaaactaaaaaagttgatcccacagaggtggagagtagaatagtggttactggaggcggacaagggggagggggagggggatagggaaggactggttaaaggatacaagtttacacagccagataggaatagtatgttttagtattctgtagtactgtaggatgactatagttaagaatcacgtatttatgtattttcaggtatttacaagagaggattttgaaagtttccatcacaaagaaatgataaatgtctgaggtgatggttatgcgtattaccctatgccctatagatatgtataattatgtgtcaatttcaaaataaaaattcaaaactacaactcctatgaaaatttttgagcgtgtttgtacttattaagtgtatttataaatcatacggatattatcttcagcctgcatattaaattgtagttaagcttttactttttaactaaaaaataaattctattattttttcctatatcccactgcactgaccccagtttggaaatcctaagattatcaaataaaaactttgattattgaagaatccaggtgtactgccacagaaaagttctattctgtagcatggactctaatatgtaatctagcccattgtgcttacagatagatgtgtgcctgtagtcatagaaaaatttgcatgagctaatgactgccttgctactagattagctcaaagcaaaaagttctctgaaagcaggtcaatagggtcatttttatattatgaagaagaaaagcagctgttgtattacattcactgtattggtcctgcttgtgtttcagggcaagatccttgttgggacaaggaatgctgaaataatcgaagttggagagaaaaatgcagcttgtaatattttagttaacggtcatgtggatgggccaatctggggactagcaacacatccttccagggattttttcctttctgctgcagaagatgggacagtgagactttgggatattgctgataaagtaagtacagataatttttttaaaagaggttacaacttctaaaaagaaaagttggaagttctaaattgctagtacttaaagaactgccagaattctgttgagcattttgaggggaaactggtataatttagaagtacttcacttaatgtttcctatgactctttttttttttttttttaaatgcagaagatgttaaacaaagtgaatttgggacatgctgctcgtactgtgtgttacagccctgaaggggacatggtggctattggaatgaaaaatggagaatttatcattttactagtgagttctctaaaaatatggggaaagaagagagacaggagatgtgcaatccatgatatcaggttagtgaacaaatggaatagagtttctagtatatacttgatttaacttccatttgtaaaattttccatagccttgccttcaaaaagaggtccccagggcctgtagcatttcccgtattataaattgtatgctaaaatatggctgtttgtatactacttaattcttcttgctaaattataaacccactgggcaccaactataatagcaagtactagtaggtaatgtttgatgaattcatgttaacacttagccatgtccattaagttcatcccaccaagaggtatctcccactgtaatacaagagagctatctgcccttcaaaagttgtcaccctggaaaactaaagttgtgatttcaaacatatcttctcttagtaacctcagtttgggaatatgtagttcattaatttaatcaatacctattgattaaatgttccagaatccaaattaatttaaatgtttcttaaacctttgtttttcagtgcttaagcatttttcaacagtggctaccatttacggagtacttccgtgtgatcagtagataagattattgaatctaggtctgtcaaaagcttgtacacttttcatcagtaaaatccttttacaaatgaaaccttcctcagaacttcaatatataaaatagtaacagtggcttcccttagcttttacatgtctctatcgtacctcagtaagactcatgggccatttcaagagactgaattgtcccatatgactccaaagattgctaggcaaatagcatttcactttgtcttttaaataagttcttcaggccgggcgcggtggctcatgcctgtaatcccagcactttgggaggccgaggcaggcagatcacctgaagtcaggagtactcgaccagcctggccaacatagtgaaaccccatctcaactaaaaatacaaaaatcagccgggcgtggtggcaggcgcctgtaatcccagctactcagggggctgaaacaggagaatcgcttgaacccgggaggcggaggttgcgccatcgcactccagcctgggagacaagagcgagacttcgtctcaaaaaaaaaaaattcttcttccaagattcaagttgtgtcatttcaccttaataactggaggttagttaagctgggctgtgttctttgcttaatattaagacaacgttttttccagatggaagaaaactatcttaatgaattgttagcttattaattatgtaatgctaatggcttttaaaagctgagatgttctgactgggtgttgtggctcacacctgtaatcccagtaccttgggaggccaagggggaaggattgcttgaggccaggagtttgggaccatagtgagaccccgcctctatttaaaaaattaaattttgttttgttttgttttgagttggagttttgctcttgttgcccatgctgaagtgcaatggtgcaatctcagctcaccacaacctgtgcctcctgggttcaagcgattctcctgcttcagcctcccgagtagatgggattacaggcgtgcaccaccatgcctggctaattttgtatttttagtagagacagggtttctctatgttggtcaggctggtctcaaactctcgacctcaggtgatctgcccgcctccgcttcccaaagttctgggattataggtgtgagccactgggcctggcctaagaaagtttttttaagccattagacgtttttaaaggaattgggagatgacaattggggaaatatttaaaatttaagtaaaatataaagcttccttatttcatgtaacccagacaatctcagtatacatgatcagttgtgtctgacaggtaaatctatttgaggccttatcacacgttacttttaagaactagaaaggaaaagtcactgatcttaagtatttataatacttcatgtggtctaatactttttacgttttgttttgattcagatttagtccggattcccggtatctggcagtaggttctagtgagaactcagtggatttttatgacctaacgctgggccccactcttaacagaatcagctactgcaaagacattccaagctttgtcattcaaatggacttctctgcagatagcagttatctccaggtacagtaccaatactgtatacccaggtggcaagttcttctgcttttacatttcgtgttagtgaatgcatttaaagttcctgagctccagagctccagcttctcaactcctccctttgtaccttctgacctacagctcccctttcctcccccacttatcagagcttttctcctattaagtttttgtagtgatcttttgcatacttaataatgttagacatgtaaatcaagtagcaatatgctagtattctgtaaaccccctgtggattttgtctctcacctaatggaattcttgtcccattttaatctgatgaaaaaggtctctagtggctgctataaacggcatgtctatgaagtgccttcaggaaaacatcttatggatcatgccgctattgacagaattacttgggctacatggactaggtaaatacttatatattcacaaggcaagaactgactttgaaggccagttagaaaatcctatttctgaactgttagagccattccaataaggaatagtaattgagtttcaagtttttgttaccatattttgaaatggtatgttcatgttgggacccctttttattgaatatatttccatgttttatcagtttccatgatttatcaagttttttttttaaggaaatcaaagttttaactttaaagataccctgatatttttcttaatgctaaatttaatgactggcaaaaaggtattgggtgctgttaagcaactgttattaattctctatctaaaggaatgctatcttgaatctattagaagtcaaagcttccaaatttgttcaaatttcctggctgtatgacaggtaaccatgactatccatttttttggccaatgaaaaatgccatcaaattcctgtatcagccaggcatatagtggctcatgcctgtaatctctgatgtagcaggccgaggtgggaggatcacttgagcctagaagttttgataccagcctgggcaacatagcaagaccccatctctgaaatttttttaattcctatgtcataagtcatttttatttttgtagagatagggatctcacaatattgcccaggctggtctcaaactcttggcctcaagcagtcctcctgcctcagcctcccaaaatgttgggattactggtatgtgctgctggacccagccaagtagcacttttaatttgaaaaatagttctatcagttttcagtcaggcgcggtggctcagcctgtaatcccagcactttgggaggccgagcgggggtgatcacctgaggtcgggagttcgagactagcctgaccaacatggagaaaccctgtctctactaaaaatacaaaataagccgggcatgttagcgcatgcctgtgatcccagctactcgggaggctgaggcaggagaattgcttgaacccaggaggcagaggttgcggtgagccgagatcatgccattgcactccagcctgggtaacaagagcgaaaactccgtctcaaaaaaaaaaaaagaaaaaatagttctatcagttttcataaagtactactttaatcttaaaaagattaatctagaaacccttcaaattataaaatgtcatttttaaaaggcaggagttgatatcctgatgaaattcaggtctccaaacaacttaccataatttacttcctgtattttaagtaacatgatagggtacttagagattaattgccaagaaactttttgaatatagtcaacctgcccgcacttgccatgatgagttttcttttgttccttccctctagtattctaggagatgaggttttgggaatctggtccagacatgctgagaaagctgatgtcaactgtgcctgtgtatctcattcaggaatcagtcttgttacaggagatgactttggcatggttaagttatttgacttcccatgtccagaaaaatttgtaagtttgtgttttgtttactattatcagtttactcctaattttgatgtcttatcatcagcacttttccccatatatttaaaatgttttgtcctaatttctaaatttttccccaaactttctaaatctatttactttgaaataaaagctattagaaacaaatcctctccctcgagtaataccatctttggaaccatcctacaaaagctgtaattagcttttcaccaaacctataatcagttatcaaatttcaaatgcttttccttagagaaaaatggtcagagtacctggagacatctgactgcccacacagcctggttttgcagatccactactcatgctgaaaagcattctaatcactggctgcggtgctaactccctactctctccacagctcttgtcatagagattatagttcctaataagagcctttgacttctgtgtgcaccaaatgccctgagcttgtctgtcattgttttttaggcaaaacacaaaaggttcttgggtcattcgccccatgtgacaaatattcgatttaccagtggtgatcgacatgttgttagtgctggaggtgatgactgcaggttagtaactttctcagcccatgaagagcagactatgttactagttaagagacttaatacaacaactcctacagctttggtttatgaaatcagctagtcaacattagtagaaggtagtataaccagatggctcttcagaatctcatatttatgcaaatacagaataaaaggagttaaagaggaaaaatattacacatgtaacctgaaagcacaactgaaaaatattaaactgttatgaaaatctaaaaacataattaactccctgcaattttcttctctgattgcagcttatttgtctggaaatgtgtacatacacctcactgagagatgctgagatgactacagaaattaactttgagaccagaattacagagaagaaaaaccaaaacccaaccctgcatggtcaagtggtgctaacccaagactgtaacagggagaaatgcccagaatcatcaaaatagtgaaagactgatctgttcaaaatatttgctatatgcactgggtataatccgtaatccatacactgccagataatgccatttcaaggaaggatcgaatacttgatggtaaaggccaagtccccctgtattgggaagtgtgtgatttcggcagacctgctgggaaaatttagggtagagcactctttacagaagaactcaaaaacccaatttggataattttcattatctttttagcaaaatggtttcttaatgtttatattttattttcaaggttcattgtttaatgaaatattttattcttgcatttccataaggaaagggaaagtcatgatcatcctaaaggatcacagtttttaaaaggcaaacattttccctaaggaaacagacacaagctttcctagagaatatgatgttttttaggcattaataaggtccttttttataaaggacacttttctcctagtagttttgaattcaggaacagatccaaagttagcagtatatggctgctacatttccattttcattttcgagccatcagtttatgttcagatgccatctctgtaatcgcacatttaaaacataactgtagcctcactaatggaaaagtagtatgatgaacaatcattcccaatggtgtacaatgtaagggttttagggagcaacagtatttaactggaagaaagaattgcatatttaatgtagtctaatatatacacatttgtttaacatgtaaacaaaagtgttaaattcacatatacaacattatacaatttaatcactcttggaataaaatttttatagccttttttctattgggaaaatttgtttagatgtgtgccactccataggtttatttccaaaatgaatgagcccaactccatttgtaaaaacttgtcagttagaattcctttttttagtggattagggctgaattcttagatccttatttcttttcactttaaatgctgccaaagatcactactcatcattcaggaattcgctgtctagcctatctgtagtttcctgaagattgaaaattatgtagactgctatttaaaaatatatttttctaagtgtgaggtttaagatgctgtattgaccctatgagtttttaatgtgttaattatctttatagcataatagatcgctttaggttcctggaatcccatttggtctgacaggatatatgaagattcttaatacctattttctgtgtctaatacttggttaatactaaaaatagaaatgactaaattacatcacagaaagcataaccagtgattgaacctggtagttttaaagctctaaatagctgtggctgaaggactgattatggggctaagaagcttgaaacgtaagttggtacttgttcatcagtggattctcctaaattaagccaaattttgaaatacatgactattaagtttctactcatgtatttacagtcagtcaataaattaaaggaggaaaaaaatccctgaacaacctgcccataaaaagaaaaatactctacatttgagcctgctgcagttttaaattttccctctgggtcaagtttgccagcttttggctacagagaaattatatttccattacagtgcaggtagaaactctgtaaccttaagcatgtaaactacatagaataaaactgtttccactgcatttctgtccttcaaagtggccaacctgattaagtcagccttaatcactgctgctgtcagtttcacgactaaaggtcatattgactaagtagtcatcagctgaccacctcgctgtatcagccagcaacgaggggaaggtgaagaaacatgataggccatatagaatctgccctatgtttacttttttaacccagataattatttttgtgtgcagtatctaagctcctgattgtgtaacctgggacttctggcaccttttgttccattcattttatgtataaaatgcatgccaaagcacactgtgccctctggtacccttgcttccaatcgccaaccatgctcatttccttcctttttttgtggtccctttttgtggtgatcattttaaaccacgtcatccaacaaatgttttatggtcaaccttagcttgttcataagccatagcaactgaaagattaaactcttaaatatgtgtctgggcagtggctattaaatagcaaaaaacaatcagattttagtattttattatttccttgtaaaatggctgaactaaattaaacccttgtttcccatttgttctataatttatagtgaaactgagaacaaaactatctttataaatgatagctaaaagtatttccagatatttaaacaatttaaaataaatttcttctgcagagatgcaaagcatctcaacactggaatgaacaaatgccttaaattcaatggagtaaacctttagaatgaagaggaactgtcatttcacccaagccgaagacaacagccttatgcacttgtgtgctctgtctttgctgcttctcgtgtttcaagcctttcctgtgggatcagcacagcaaagtgcaacttaccaaatggtttaatgactggttaattctttcttctcccaatggaaaagcaatggcaacacaacagtagactgctggcttgacaatcttaaacgtgagcctttgcacatgtaggtttatcatcatttgagtatacgactaagcaagtcaatgaactttttttttttttttagcagtttaatttggtcctgagaatgttgcagtctttattaccccttttgcattaatccacttttctaaccaccttttaagctttaatttttaacactatacaccaagtctttgaaatcagtgatctgttatttaactctaaagcatttgacacttcttgccttaacagttttaaaaaccacacacaaaaaaactctgtaagtaatacagtaggccaaaagtttcatcctatctatcttgcagtttacctatctgatctgatctctgtaattatagttctgtcatttaaaatatactatttaaatctaatttttacatttcaaaaattatcttcagtagtaactaagtatattttctgtggattctgagaatgttatttttcagaatgtgagaatatatatgtacatttataatcttgtgactttaaagtctgttttcagatacagtatgtaaatacttgtaaaaaaatttgtataattttgtgataatgtagtttcccaaaaaaattatttagaaggcattatgttattagtaaatgagagcactgtatagaactgttcctattttctgcacttgccattccagctgcctccactgtccatacccacctcattcatcctgtcacagaaggcaggaaaactgggaactttaccaaagtagcactcagcctgagaggcctgtataatcatgcttttcaaactaaattcacttaaaaattaaaaagcagaattgaatattttaagcagcctcagtacctttggccaatgctgttttcatggtggattatgaacattatataatctttgggaaaagtgaaagtagtacaatttttagaataatgacaactgcctcactgcatctctccactcacacagcaaccgtgtagccccctaagctgcagtaccatgactaaccatgatgtcaatttcatatgctgatcctcacaacagcagtgcacaaacatgccccaaatattttaacagaatttagctcttccttaagctgtcttttcatagtaaaaacaaaacaaaaacacccaatgttaaaaccacataataaacttacaaacttgaaaaattagacacttcagatagataggcaataaaacttcatattatgaaagcaatatattccaagtttcaaagatttgacaagttctgtagagtatctttcatcagtacatgaaaacttccaaactgcatgatcttctgccaggcaggactgggtgctattcgctggtttgaggtcgaatccatttcaaggcatgtcgtggtgggacattaatggtgggatggtagaatgtgcagtccggtcttgtacattgagtgttaaacctacaatgttttggatgatagaagggacattccatcttcttacaagcagggaagtaacggcagagctgactactggaaggtggtgctggtggtgcaactggttttggagacagtactggaattcttctactcacatgagtgaagggacaatctggtttagtacactttgcatcatatttacaatttgggtgaacaaacaaacatttttcagcaaatttacaattggggaaggctttgcagggtgagatggggtgatggtaggcacactcatccccatttttacaagcaggccagtacttgcagcgctccaaaagtttttctggtttctgtgccacactcagttcactcatctcagcatttgggtcctcaagctgcctgctcagcaagtgcaactgctgtgggtggaggagacctctgagtcccttgtttgaggctgcagtttggtttacgggtttcattccttcaaagcacatgtcctcctcttgatctgacatgtatcctggggggctggggacaccatccagcgtcactataaacttgggacttgcaggtttatctggttgtacaagatctcgtgtctgcataaggtgtcctgaaagtacccgaagggaatctgcagtcttcatccccgactcttggtttggtgccactactacttcctcagacagctttggcttcttcagaataaatgatcttgtgtctgcatggaccatggattccatgtcatagtaatcttgatttttttctacagaatctccttttgtttcctcttctttaatggggggacttattctgggggtcctactttgtccctggaccacttctgctagcaattcttcttgagaagttcgagttctgggagcaactggaagtgtctgtttctgtggaactgtagagtagttagttgtttttgttacggattcttgagcttcagatatagccttcaaaatcagattcttgttagcttgtttagaaggtggaagagaaggtctcctttcaggctttgcaggcacagacacactgctggagatgcttcctgttcgagacccgtaatcatcatcttcttcctcctcttctccatcatgattgaatttttttactttaacaactgaacttaccacaggcaactttctcttccgaaagttttcatcctccatactcattttctccgagttgtttctaaagaacggactatacgtttcttctaagctgttaagcacctctggttcacacaaacgtcctgtttcatatacccaactactctgcatatcaagctgcttggcagcatgaatactattctgctgctgttgaaattgcaacctgtttaaatgaacaccactatctgcatttctacttgcaggtggtcgataaatttcaatagaagggcgagaagaaccatatgtaagtgtcactgtaggttttttctgagataagggattctcctgcacaaagttgaggtcttcgtcaatgagatcatctggttctggcttaatatcaatcacatcttcagagggtgctggctccctcaaaggtttcactgttgacattagtcgggttgcagctccatcatcgtaagtctgtctgacatttgtggtttttgactcctgcgaacttgtagaaactctggaatctcttttttcaggtctcgcgctaggaatggcaagtggtggcactgcagcttcatgcctcctctcatctccccgactgaaattgctcttgtttgaaggcacgttactatcaaagatgttggtatcagaagacttcagactagagggttcagttgtaacagagcgaagtttatctaatacaccatgaagccatacggtgaatcgaattgtgttgttccctagaaacagggacagatcctctgtcatttggtcctgacttttcttgttggccaccatcaccataatgtaatcaggaagttcttcatcaacataagctcctaattcttgtaatttccccttaatggcactccggatcttgcggctgatctcggtgccgatctccatggctctgcggcgtgcgggaactcagcactgcgcggcgcttggcttacccggaggctgccgcggactcctaccccgcagccgggacaccaccgcctcc

SEQ ID NO: 17247 - RNA, 14816 nt, Homo sapiens
  source 1..14816: mol_type = other RNA
tcaggccaggcacagtggctcacacctgtaatcttatcactttgggaggctgaggcaggtggatcgcttgagcccaggagttcaagaccagcctgggcaacatggtgaaaccccatcgctataaaaaacaacaattagccgggtgtggtggcacatgcctgtagtccctgctactcaggaggctgaggtgggaggatcacttgagcctggggaggtcaaggctttagtgagctgtgatggtgccactgcactccagcctgggtgacagagtgagaccccatttaaaaaacaaaaacaaaaacaaaaaaaaatgtgacatatagttgactaagaagtacatttcaatacaggattgaaagaacccacatatgttaattaaacacaagcgcagaatttgtgccttttacataaaggaagaatgcacataggcatgctttcagacaagcaattcatctagcagaaaaggaaggaatacatttttcagcccttccaggaataaaatccataaatgggctctatttcgtcctccaacacttgtatttcccacgtcatttactcctgcacacccccactcactagaagcctgctaaactgttccagtgagatattttaacacctgatagggaataaatatgcttctgttttggccttcaaaaataagctctgggccagttgcagtggctcacgcctgtaatcccaacactttgggaggccgaggtgggcggatcacgaggtcaggagtttgggatcagcctggccaatatggtgaaactccatctctactaaaaatacaaaaattagccaggcatggtgcctgtaatcccagctacttgggaggctgaaggagaagaatcgcttgaacctgggaggcacaggttgcagtgagccgagatcacaccactgcactccaggccaggtgacagagcgacactctgtctcaaaaaaataaataaatcaactctgtagcatagcatttgtaattctattattttgccttacatttccattatccttttaataaaattgtttttttacatcttcctaatcaagaagtattatgaggccaggcacagtggctcatacctggaatcccagcactttgggaggccgaggcaggcagatcacctgaggtcaaggtatttgagaccagcctggccaacatggtgaaaccccatctctactaaaaatacagaaattagctgggtgtggtggtgcacacctgtaatgctagctactcgggaggctgaggtaggagaatcgcttgaacctgggaggcagaggttgcaataagcctagatcatgccactgcactcaagcctgggagacagagcgagactacatcttaaaaaaaaaaaaaaaagtattatgagagaggataatgtattgtaatgtattgtagaggctaaataaaattatgctcatgtcagaaaaaaagagtatttctcaaaataaaattcactgaaactggatgtttattttgactgagatatagtatatcctcaaattgccatagaaagtttacaagaatattagaggtaaattataaatatcagggcctttttaaaaaaaaaagattctgcttataacttggtatttgtttataataaaaattatagtagccaataatgaacacttactctggcttggttatttacttaggtcaaaagaaggaggagcggttaaactgtgggatcaggaactgaggcggtgccgtgccttcaggcttgagacaggacaagccacagattgtgttcgttctgtgtgcagaggcaaagtaagatgttccatgagctgatacagtgcagcagaaaacagaaagtggttattactgtgattccctcaccctttgcagcctaatgaacaatacttaataatgcataacgatggatttgcttgccaacattactctgtctttgctgctttctttgccaaagttagcaccagtgtggtgcataagctaggaagctattctgtctaaatactgtatgtaaacctccaatattttctagaatctgccaatttaacaactctagtagacataattgaaagcccttggcagttgactcatattaggacagctgtctccattttttaaaaaaacacacattccctagataaaacgtgcagtaaacaaacaatgaaatactactcagccataaaaaataatgaaattctgtcattcttggtggcaacatggatgagactggaggacatgatgtgaagtgaaataagccaggcacagaaagataaatacatgttctcactcctgtgcagaaactaaaaaagttgatcccacagaggtggagagtagaatagtggttactggaggcggacaagggggagggggagggggatagggaaggactggttaaaggatacaagtttacacagccagataggaatagtatgttttagtattctgtagtactgtaggatgactatagttaagaatcacgtatttatgtattttcaggtatttacaagagaggattttgaaagtttccatcacaaagaaatgataaatgtctgaggtgatggttatgcgtattaccctatgccctatagatatgtataattatgtgtcaatttcaaaataaaaattcaaaactacaactcctatgaaaatttttgagcgtgtttgtacttattaagtgtatttataaatcatacggatattatcttcagcctgcatattaaattgtagttaagcttttactttttaactaaaaaataaattctattattttttcctatatcccactgcactgaccccagtttggaaatcctaagattatcaaataaaaactttgattattgaagaatccaggtgtactgccacagaaaagttctattctgtagcatggactctaatatgtaatctagcccattgtgcttacagatagatgtgtgcctgtagtcatagaaaaatttgcatgagctaatgactgccttgctactagattagctcaaagcaaaaagttctctgaaagcaggtcaatagggtcatttttatattatgaagaagaaaagcagctgttgtattacattcactgtattggtcctgcttgtgtttcagggcaagatccttgttgggacaaggaatgctgaaataatcgaagttggagagaaaaatgcagcttgtaatattttagttaacggtcatgtggatgggccaatctggggactagcaacacatccttccagggattttttcctttctgctgcagaagatgggacagtgagactttgggatattgctgataaagtaagtacagataatttttttaaaagaggttacaacttctaaaaagaaaagttggaagttctaaattgctagtacttaaagaactgccagaattctgttgagcattttgaggggaaactggtataatttagaagtacttcacttaatgtttcctatgactctttttttttttttttttaaatgcagaagatgttaaacaaagtgaatttgggacatgctgctcgtactgtgtgttacagccctgaaggggacatggtggctattggaatgaaaaatggagaatttatcattttactagtgagttctctaaaaatatggggaaagaagagagacaggagatgtgcaatccatgatatcaggttagtgaacaaatggaatagagtttctagtatatacttgatttaacttccatttgtaaaattttccatagccttgccttcaaaaagaggtccccagggcctgtagcatttcccgtattataaattgtatgctaaaatatggctgtttgtatactacttaattcttcttgctaaattataaacccactgggcaccaactataatagcaagtactagtaggtaatgtttgatgaattcatgttaacacttagccatgtccattaagttcatcccaccaagaggtatctcccactgtaatacaagagagctatctgcccttcaaaagttgtcaccctggaaaactaaagttgtgatttcaaacatatcttctcttagtaacctcagtttgggaatatgtagttcattaatttaatcaatacctattgattaaatgttccagaatccaaattaatttaaatgtttcttaaacctttgtttttcagtgcttaagcatttttcaacagtggctaccatttacggagtacttccgtgtgatcagtagataagattattgaatctaggtctgtcaaaagcttgtacacttttcatcagtaaaatccttttacaaatgaaaccttcctcagaacttcaatatataaaatagtaacagtggcttcccttagcttttacatgtctctatcgtacctcagtaagactcatgggccatttcaagagactgaattgtcccatatgactccaaagattgctaggcaaatagcatttcactttgtcttttaaataagttcttcaggccgggcgcggtggctcatgcctgtaatcccagcactttgggaggccgaggcaggcagatcacctgaagtcaggagtactcgaccagcctggccaacatagtgaaaccccatctcaactaaaaatacaaaaatcagccgggcgtggtggcaggcgcctgtaatcccagctactcagggggctgaaacaggagaatcgcttgaacccgggaggcggaggttgcgccatcgcactccagcctgggagacaagagcgagacttcgtctcaaaaaaaaaaaattcttcttccaagattcaagttgtgtcatttcaccttaataactggaggttagttaagctgggctgtgttctttgcttaatattaagacaacgttttttccagatggaagaaaactatcttaatgaattgttagcttattaattatgtaatgctaatggcttttaaaagctgagatgttctgactgggtgttgtggctcacacctgtaatcccagtaccttgggaggccaagggggaaggattgcttgaggccaggagtttgggaccatagtgagaccccgcctctatttaaaaaattaaattttgttttgttttgttttgagttggagttttgctcttgttgcccatgctgaagtgcaatggtgcaatctcagctcaccacaacctgtgcctcctgggttcaagcgattctcctgcttcagcctcccgagtagatgggattacaggcgtgcaccaccatgcctggctaattttgtatttttagtagagacagggtttctctatgttggtcaggctggtctcaaactctcgacctcaggtgatctgcccgcctccgcttcccaaagttctgggattataggtgtgagccactgggcctggcctaagaaagtttttttaagccattagacgtttttaaaggaattgggagatgacaattggggaaatatttaaaatttaagtaaaatataaagcttccttatttcatgtaacccagacaatctcagtatacatgatcagttgtgtctgacaggtaaatctatttgaggccttatcacacgttacttttaagaactagaaaggaaaagtcactgatcttaagtatttataatacttcatgtggtctaatactttttacgttttgttttgattcagatttagtccggattcccggtatctggcagtaggttctagtgagaactcagtggatttttatgacctaacgctgggccccactcttaacagaatcagctactgcaaagacattccaagctttgtcattcaaatggacttctctgcagatagcagttatctccaggtacagtaccaatactgtatacccaggtggcaagttcttctgcttttacatttcgtgttagtgaatgcatttaaagttcctgagctccagagctccagcttctcaactcctccctttgtaccttctgacctacagctcccctttcctcccccacttatcagagcttttctcctattaagtttttgtagtgatcttttgcatacttaataatgttagacatgtaaatcaagtagcaatatgctagtattctgtaaaccccctgtggattttgtctctcacctaatggaattcttgtcccattttaatctgatgaaaaaggtctctagtggctgctataaacggcatgtctatgaagtgccttcaggaaaacatcttatggatcatgccgctattgacagaattacttgggctacatggactaggtaaatacttatatattcacaaggcaagaactgactttgaaggccagttagaaaatcctatttctgaactgttagagccattccaataaggaatagtaattgagtttcaagtttttgttaccatattttgaaatggtatgttcatgttgggacccctttttattgaatatatttccatgttttatcagtttccatgatttatcaagttttttttttaaggaaatcaaagttttaactttaaagataccctgatatttttcttaatgctaaatttaatgactggcaaaaaggtattgggtgctgttaagcaactgttattaattctctatctaaaggaatgctatcttgaatctattagaagtcaaagcttccaaatttgttcaaatttcctggctgtatgacaggtaaccatgactatccatttttttggccaatgaaaaatgccatcaaattcctgtatcagccaggcatatagtggctcatgcctgtaatctctgatgtagcaggccgaggtgggaggatcacttgagcctagaagttttgataccagcctgggcaacatagcaagaccccatctctgaaatttttttaattcctatgtcataagtcatttttatttttgtagagatagggatctcacaatattgcccaggctggtctcaaactcttggcctcaagcagtcctcctgcctcagcctcccaaaatgttgggattactggtatgtgctgctggacccagccaagtagcacttttaatttgaaaaatagttctatcagttttcagtcaggcgcggtggctcagcctgtaatcccagcactttgggaggccgagcgggggtgatcacctgaggtcgggagttcgagactagcctgaccaacatggagaaaccctgtctctactaaaaatacaaaataagccgggcatgttagcgcatgcctgtgatcccagctactcgggaggctgaggcaggagaattgcttgaacccaggaggcagaggttgcggtgagccgagatcatgccattgcactccagcctgggtaacaagagcgaaaactccgtctcaaaaaaaaaaaaagaaaaaatagttctatcagttttcataaagtactactttaatcttaaaaagattaatctagaaacccttcaaattataaaatgtcatttttaaaaggcaggagttgatatcctgatgaaattcaggtctccaaacaacttaccataatttacttcctgtattttaagtaacatgatagggtacttagagattaattgccaagaaactttttgaatatagtcaacctgcccgcacttgccatgatgagttttcttttgttccttccctctagtattctaggagatgaggttttgggaatctggtccagacatgctgagaaagctgatgtcaactgtgcctgtgtatctcattcaggaatcagtcttgttacaggagatgactttggcatggttaagttatttgacttcccatgtccagaaaaatttgtaagtttgtgttttgtttactattatcagtttactcctaattttgatgtcttatcatcagcacttttccccatatatttaaaatgttttgtcctaatttctaaatttttccccaaactttctaaatctatttactttgaaataaaagctattagaaacaaatcctctccctcgagtaataccatctttggaaccatcctacaaaagctgtaattagcttttcaccaaacctataatcagttatcaaatttcaaatgcttttccttagagaaaaatggtcagagtacctggagacatctgactgcccacacagcctggttttgcagatccactactcatgctgaaaagcattctaatcactggctgcggtgctaactccctactctctccacagctcttgtcatagagattatagttcctaataagagcctttgacttctgtgtgcaccaaatgccctgagcttgtctgtcattgttttttaggcaaaacacaaaaggttcttgggtcattcgccccatgtgacaaatattcgatttaccagtggtgatcgacatgttgttagtgctggaggtgatgactgcaggttagtaactttctcagcccatgaagagcagactatgttactagttaagagacttaatacaacaactcctacagctttggtttatgaaatcagctagtcaacattagtagaaggtagtataaccagatggctcttcagaatctcatatttatgcaaatacagaataaaaggagttaaagaggaaaaatattacacatgtaacctgaaagcacaactgaaaaatattaaactgttatgaaaatctaaaaacataattaactccctgcaattttcttctctgattgcagcttatttgtctggaaatgtgtacatacacctcactgagagatgctgagatgactacagaaattaactttgagaccagaattacagagaagaaaaaccaaaacccaaccctgcatggtcaagtggtgctaacccaagactgtaacagggagaaatgcccagaatcatcaaaatagtgaaagactgatctgttcaaaatatttgctatatgcactgggtataatccgtaatccatacactgccagataatgccatttcaaggaaggatcgaatacttgatggtaaaggccaagtccccctgtattgggaagtgtgtgatttcggcagacctgctgggaaaatttagggtagagcactctttacagaagaactcaaaaacccaatttggataattttcattatctttttagcaaaatggtttcttaatgtttatattttattttcaaggttcattgtttaatgaaatattttattcttgcatttccataaggaaagggaaagtcatgatcatcctaaaggatcacagtttttaaaaggcaaacattttccctaaggaaacagacacaagctttcctagagaatatgatgttttttaggcattaataaggtccttttttataaaggacacttttctcctagtagttttgaattcaggaacagatccaaagttagcagtatatggctgctacatttccattttcattttcgagccatcagtttatgttcagatgccatctctgtaatcgcacatttaaaacataactgtagcctcactaatggaaaagtagtatgatgaacaatcattcccaatggtgtacaatgtaagggttttagggagcaacagtatttaactggaagaaagaattgcatatttaatgtagtctaatatatacacatttgtttaacatgtaaacaaaagtgttaaattcacatatacaacattatacaatttaatcactcttggaataaaatttttatagccttttttctattgggaaaatttgtttagatgtgtgccactccataggtttatttccaaaatgaatgagcccaactccatttgtaaaaacttgtcagttagaattcctttttttagtggattagggctgaattcttagatccttatttcttttcactttaaatgctgccaaagatcactactcatcattcaggaattcgctgtctagcctatctgtagtttcctgaagattgaaaattatgtagactgctatttaaaaatatatttttctaagtgtgaggtttaagatgctgtattgaccctatgagtttttaatgtgttaattatctttatagcataatagatcgctttaggttcctggaatcccatttggtctgacaggatatatgaagattcttaatacctattttctgtgtctaatacttggttaatactaaaaatagaaatgactaaattacatcacagaaagcataaccagtgattgaacctggtagttttaaagctctaaatagctgtggctgaaggactgattatggggctaagaagcttgaaacgtaagttggtacttgttcatcagtggattctcctaaattaagccaaattttgaaatacatgactattaagtttctactcatgtatttacagtcagtcaataaattaaaggaggaaaaaaatccctgaacaacctgcccataaaaagaaaaatactctacatttgagcctgctgcagttttaaattttccctctgggtcaagtttgccagcttttggctacagagaaattatatttccattacagtgcaggtagaaactctgtaaccttaagcatgtaaactacatagaataaaactgtttccactgcatttctgtccttcaaagtggccaacctgattaagtcagccttaatcactgctgctgtcagtttcacgactaaaggtcatattgactaagtagtcatcagctgaccacctcgctgtatcagccagcaacgaggggaaggtgaagaaacatgataggccatatagaatctgccctatgtttacttttttaacccagataattatttttgtgtgcagtatctaagctcctgattgtgtaacctgggacttctggcaccttttgttccattcattttatgtataaaatgcatgccaaagcacactgtgccctctggtacccttgcttccaatcgccaaccatgctcatttccttcctttttttgtggtccctttttgtggtgatcattttaaaccacgtcatccaacaaatgttttatggtcaaccttagcttgttcataagccatagcaactgaaagattaaactcttaaatatgtgtctgggcagtggctattaaatagcaaaaaacaatcagattttagtattttattatttccttgtaaaatggctgaactaaattaaacccttgtttcccatttgttctataatttatagtgaaactgagaacaaaactatctttataaatgatagctaaaagtatttccagatatttaaacaatttaaaataaatttcttctgcagagatgcaaagcatctcaacactggaatgaacaaatgccttaaattcaatggagtaaacctttagaatgaagaggaactgtcatttcacccaagccgaagacaacagccttatgcacttgtgtgctctgtctttgctgcttctcgtgtttcaagcctttcctgtgggatcagcacagcaaagtgcaacttaccaaatggtttaatgactggttaattctttcttctcccaatggaaaagcaatggcaacacaacagtagactgctggcttgacaatcttaaacgtgagcctttgcacatgtaggtttatcatcatttgagtatacgactaagcaagtcaatgaactttttttttttttttagcagtttaatttggtcctgagaatgttgcagtctttattaccccttttgcattaatccacttttctaaccaccttttaagctttaatttttaacactatacaccaagtctttgaaatcagtgatctgttatttaactctaaagcatttgacacttcttgccttaacagttttaaaaaccacacacaaaaaaactctgtaagtaatacagtaggccaaaagtttcatcctatctatcttgcagtttacctatctgatctgatctctgtaattatagttctgtcatttaaaatatactatttaaatctaatttttacatttcaaaaattatcttcagtagtaactaagtatattttctgtggattctgagaatgttatttttcagaatgtgagaatatatatgtacatttataatcttgtgactttaaagtctgttttcagatacagtatgtaaatacttgtaaaaaaatttgtataattttgtgataatgtagtttcccaaaaaaattatttagaaggcattatgttattagtaaatgagagcactgtatagaactgttcctattttctgcacttgccattccagctgcctccactgtccatacccacctcattcatcctgtcacagaaggcaggaaaactgggaactttaccaaagtagcactcagcctgagaggcctgtataatcatgcttttcaaactaaattcacttaaaaattaaaaagcagaattgaatattttaagcagcctcagtacctttggccaatgctgttttcatggtggattatgaacattatataatctttgggaaaagtgaaagtagtacaatttttagaataatgacaactgcctcactgcatctctccactcacacagcaaccgtgtagccccctaagctgcagtaccatgactaaccatgatgtcaatttcatatgctgatcctcacaacagcagtgcacaaacatgccccaaatattttaacagaatttagctcttccttaagctgtcttttcatagtaaaaacaaaacaaaaacacccaatgttaaaaccacataataaacttacaaacttgaaaaattagacacttcagatagataggcaataaaacttcatattatgaaagcaatatattccaagtttcaaagatttgacaagttctgtagagtatctttcatcagtacatgaaaacttccaaactgcatgatcttctgccaggcaggactgggtgctattcgctggtttgaggtcgaatccatttcaaggcatgtcgtggtgggacattaatggtgggatggtagaatgtgcagtccggtcttgtacattgagtgttaaacctacaatgttttggatgatagaagggacattccatcttcttacaagcagggaagtaacggcagagctgactactggaaggtggtgctggtggtgcaactggttttggagacagtactggaattcttctactcacatgagtgaagggacaatctggtttagtacactttgcatcatatttacaatttgggtgaacaaacaaacatttttcagcaaatttacaattggggaaggctttgcagggtgagatggggtgatggtaggcacactcatccccatttttacaagcaggccagtacttgcagcgctccaaaagtttttctggtttctgtgccacactcagttcactcatctcagcgttagaaaagctaccatttgggtcctcaagctgcctgctcagcaagtgcaactgctgtgggtggaggagacctctgagtcccttgtttgaggctgcagtttggtttacgggtttcattccttcaaagcacatgtcctcctcttgatctgacatgtatcctggggggctggggacaccatccagcgtcactataaacttgggacttgcaggtttatctggttgtacaagatctcgtgtctgcataaggtgtcctgaaagtacccgaagggaatctgcagtcttcatccccgactcttggtttggtgccactactacttcctcagacagctttggcttcttcagaataaatgatcttgtgtctgcatggaccatggattccatgtcatagtaatcttgactcatctgcagagtttctgccattactgggtcgatttgcagtcgggataataattgcctctgttgagttccttgatttttttctacagaatctccttttgtttcctcttctttaatggggggacttattctgggggtcctactttgtccctggaccacttctgctagcaattcttcttgagaagttcgagttctgggagcaactggaagtgtctgtttctgtggaactgtagagtagttagttgtttttgttacggattcttgagcttcagatatagccttcaaaatcagattcttgttagcttgtttagaaggtggaagagaaggtctcctttcaggctttgcaggcacagacacactgctggagatgcttcctgttcgagacccgtaatcatcatcttcttcctcctcttctccatcatgattgaatttttttactttaacaactgaacttaccacaggcaactttctcttccgaaagttttcatcctccatactcattttctccgagttgtttctaaagaacggactatacgtttcttctaagctgttaagcacctctggttcacacaaacgtcctgtttcatatacccaactactctgcatatcaagctgcttggcagcatgaatactattctgctgctgttgaaattgcaacctgtttaaatgaacaccactatctgcatttctacttgcaggtggtcgataaatttcaatagaagggcgagaagaaccatatgtaagtgtcactgtaggttttttctgagataagggattctcctgcacaaagttgaggtcttcgtcaatgagatcatctggttctggcttaatatcaatcacatcttcagagggtgctggctccctcaaaggtttcactgttgacattagtcgggttgcagctccatcatcgtaagtctgtctgacatttgtggtttttgactcctgcgaacttgtagaaactctggaatctcttttttcaggtctcgcgctaggaatggcaagtggtggcactgcagcttcatgcctcctctcatctccccgactgaaattgctcttgtttgaaggcacgttactatcaaagatgttggtatcagaagacttcagactagagggttcagttgtaacagagcgaagtttatctaatacaccatgaagccaacataagctcctaattcttgtaatttccccttaatggcactccggatcttgcggctgatctcggtgccgatctccatggctctgcggcgtgcgggaactcagcactgcgcggcgcttggcttacccggaggctgccgcggactcctaccccgcagccgggacaccaccgcctcc

SEQ ID NO: 17248 - RNA, 14931 nt, Homo sapiens
  source 1..14931: mol_type = other RNA
tcaggccaggcacagtggctcacacctgtaatcttatcactttgggaggctgaggcaggtggatcgcttgagcccaggagttcaagaccagcctgggcaacatggtgaaaccccatcgctataaaaaacaacaattagccgggtgtggtggcacatgcctgtagtccctgctactcaggaggctgaggtgggaggatcacttgagcctggggaggtcaaggctttagtgagctgtgatggtgccactgcactccagcctgggtgacagagtgagaccccatttaaaaaacaaaaacaaaaacaaaaaaaaatgtgacatatagttgactaagaagtacatttcaatacaggattgaaagaacccacatatgttaattaaacacaagcgcagaatttgtgccttttacataaaggaagaatgcacataggcatgctttcagacaagcaattcatctagcagaaaaggaaggaatacatttttcagcccttccaggaataaaatccataaatgggctctatttcgtcctccaacacttgtatttcccacgtcatttactcctgcacacccccactcactagaagcctgctaaactgttccagtgagatattttaacacctgatagggaataaatatgcttctgttttggccttcaaaaataagctctgggccagttgcagtggctcacgcctgtaatcccaacactttgggaggccgaggtgggcggatcacgaggtcaggagtttgggatcagcctggccaatatggtgaaactccatctctactaaaaatacaaaaattagccaggcatggtgcctgtaatcccagctacttgggaggctgaaggagaagaatcgcttgaacctgggaggcacaggttgcagtgagccgagatcacaccactgcactccaggccaggtgacagagcgacactctgtctcaaaaaaataaataaatcaactctgtagcatagcatttgtaattctattattttgccttacatttccattatccttttaataaaattgtttttttacatcttcctaatcaagaagtattatgaggccaggcacagtggctcatacctggaatcccagcactttgggaggccgaggcaggcagatcacctgaggtcaaggtatttgagaccagcctggccaacatggtgaaaccccatctctactaaaaatacagaaattagctgggtgtggtggtgcacacctgtaatgctagctactcgggaggctgaggtaggagaatcgcttgaacctgggaggcagaggttgcaataagcctagatcatgccactgcactcaagcctgggagacagagcgagactacatcttaaaaaaaaaaaaaaaagtattatgagagaggataatgtattgtaatgtattgtagaggctaaataaaattatgctcatgtcagaaaaaaagagtatttctcaaaataaaattcactgaaactggatgtttattttgactgagatatagtatatcctcaaattgccatagaaagtttacaagaatattagaggtaaattataaatatcagggcctttttaaaaaaaaaagattctgcttataacttggtatttgtttataataaaaattatagtagccaataatgaacacttactctggcttggttatttacttaggtcaaaagaaggaggagcggttaaactgtgggatcaggaactgaggcggtgccgtgccttcaggcttgagacaggacaagccacagattgtgttcgttctgtgtgcagaggcaaagtaagatgttccatgagctgatacagtgcagcagaaaacagaaagtggttattactgtgattccctcaccctttgcagcctaatgaacaatacttaataatgcataacgatggatttgcttgccaacattactctgtctttgctgctttctttgccaaagttagcaccagtgtggtgcataagctaggaagctattctgtctaaatactgtatgtaaacctccaatattttctagaatctgccaatttaacaactctagtagacataattgaaagcccttggcagttgactcatattaggacagctgtctccattttttaaaaaaacacacattccctagataaaacgtgcagtaaacaaacaatgaaatactactcagccataaaaaataatgaaattctgtcattcttggtggcaacatggatgagactggaggacatgatgtgaagtgaaataagccaggcacagaaagataaatacatgttctcactcctgtgcagaaactaaaaaagttgatcccacagaggtggagagtagaatagtggttactggaggcggacaagggggagggggagggggatagggaaggactggttaaaggatacaagtttacacagccagataggaatagtatgttttagtattctgtagtactgtaggatgactatagttaagaatcacgtatttatgtattttcaggtatttacaagagaggattttgaaagtttccatcacaaagaaatgataaatgtctgaggtgatggttatgcgtattaccctatgccctatagatatgtataattatgtgtcaatttcaaaataaaaattcaaaactacaactcctatgaaaatttttgagcgtgtttgtacttattaagtgtatttataaatcatacggatattatcttcagcctgcatattaaattgtagttaagcttttactttttaactaaaaaataaattctattattttttcctatatcccactgcactgaccccagtttggaaatcctaagattatcaaataaaaactttgattattgaagaatccaggtgtactgccacagaaaagttctattctgtagcatggactctaatatgtaatctagcccattgtgcttacagatagatgtgtgcctgtagtcatagaaaaatttgcatgagctaatgactgccttgctactagattagctcaaagcaaaaagttctctgaaagcaggtcaatagggtcatttttatattatgaagaagaaaagcagctgttgtattacattcactgtattggtcctgcttgtgtttcagggcaagatccttgttgggacaaggaatgctgaaataatcgaagttggagagaaaaatgcagcttgtaatattttagttaacggtcatgtggatgggccaatctggggactagcaacacatccttccagggattttttcctttctgctgcagaagatgggacagtgagactttgggatattgctgataaagtaagtacagataatttttttaaaagaggttacaacttctaaaaagaaaagttggaagttctaaattgctagtacttaaagaactgccagaattctgttgagcattttgaggggaaactggtataatttagaagtacttcacttaatgtttcctatgactctttttttttttttttttaaatgcagaagatgttaaacaaagtgaatttgggacatgctgctcgtactgtgtgttacagccctgaaggggacatggtggctattggaatgaaaaatggagaatttatcattttactagtgagttctctaaaaatatggggaaagaagagagacaggagatgtgcaatccatgatatcaggttagtgaacaaatggaatagagtttctagtatatacttgatttaacttccatttgtaaaattttccatagccttgccttcaaaaagaggtccccagggcctgtagcatttcccgtattataaattgtatgctaaaatatggctgtttgtatactacttaattcttcttgctaaattataaacccactgggcaccaactataatagcaagtactagtaggtaatgtttgatgaattcatgttaacacttagccatgtccattaagttcatcccaccaagaggtatctcccactgtaatacaagagagctatctgcccttcaaaagttgtcaccctggaaaactaaagttgtgatttcaaacatatcttctcttagtaacctcagtttgggaatatgtagttcattaatttaatcaatacctattgattaaatgttccagaatccaaattaatttaaatgtttcttaaacctttgtttttcagtgcttaagcatttttcaacagtggctaccatttacggagtacttccgtgtgatcagtagataagattattgaatctaggtctgtcaaaagcttgtacacttttcatcagtaaaatccttttacaaatgaaaccttcctcagaacttcaatatataaaatagtaacagtggcttcccttagcttttacatgtctctatcgtacctcagtaagactcatgggccatttcaagagactgaattgtcccatatgactccaaagattgctaggcaaatagcatttcactttgtcttttaaataagttcttcaggccgggcgcggtggctcatgcctgtaatcccagcactttgggaggccgaggcaggcagatcacctgaagtcaggagtactcgaccagcctggccaacatagtgaaaccccatctcaactaaaaatacaaaaatcagccgggcgtggtggcaggcgcctgtaatcccagctactcagggggctgaaacaggagaatcgcttgaacccgggaggcggaggttgcgccatcgcactccagcctgggagacaagagcgagacttcgtctcaaaaaaaaaaaattcttcttccaagattcaagttgtgtcatttcaccttaataactggaggttagttaagctgggctgtgttctttgcttaatattaagacaacgttttttccagatggaagaaaactatcttaatgaattgttagcttattaattatgtaatgctaatggcttttaaaagctgagatgttctgactgggtgttgtggctcacacctgtaatcccagtaccttgggaggccaagggggaaggattgcttgaggccaggagtttgggaccatagtgagaccccgcctctatttaaaaaattaaattttgttttgttttgttttgagttggagttttgctcttgttgcccatgctgaagtgcaatggtgcaatctcagctcaccacaacctgtgcctcctgggttcaagcgattctcctgcttcagcctcccgagtagatgggattacaggcgtgcaccaccatgcctggctaattttgtatttttagtagagacagggtttctctatgttggtcaggctggtctcaaactctcgacctcaggtgatctgcccgcctccgcttcccaaagttctgggattataggtgtgagccactgggcctggcctaagaaagtttttttaagccattagacgtttttaaaggaattgggagatgacaattggggaaatatttaaaatttaagtaaaatataaagcttccttatttcatgtaacccagacaatctcagtatacatgatcagttgtgtctgacaggtaaatctatttgaggccttatcacacgttacttttaagaactagaaaggaaaagtcactgatcttaagtatttataatacttcatgtggtctaatactttttacgttttgttttgattcagatttagtccggattcccggtatctggcagtaggttctagtgagaactcagtggatttttatgacctaacgctgggccccactcttaacagaatcagctactgcaaagacattccaagctttgtcattcaaatggacttctctgcagatagcagttatctccaggtacagtaccaatactgtatacccaggtggcaagttcttctgcttttacatttcgtgttagtgaatgcatttaaagttcctgagctccagagctccagcttctcaactcctccctttgtaccttctgacctacagctcccctttcctcccccacttatcagagcttttctcctattaagtttttgtagtgatcttttgcatacttaataatgttagacatgtaaatcaagtagcaatatgctagtattctgtaaaccccctgtggattttgtctctcacctaatggaattcttgtcccattttaatctgatgaaaaaggtctctagtggctgctataaacggcatgtctatgaagtgccttcaggaaaacatcttatggatcatgccgctattgacagaattacttgggctacatggactaggtaaatacttatatattcacaaggcaagaactgactttgaaggccagttagaaaatcctatttctgaactgttagagccattccaataaggaatagtaattgagtttcaagtttttgttaccatattttgaaatggtatgttcatgttgggacccctttttattgaatatatttccatgttttatcagtttccatgatttatcaagttttttttttaaggaaatcaaagttttaactttaaagataccctgatatttttcttaatgctaaatttaatgactggcaaaaaggtattgggtgctgttaagcaactgttattaattctctatctaaaggaatgctatcttgaatctattagaagtcaaagcttccaaatttgttcaaatttcctggctgtatgacaggtaaccatgactatccatttttttggccaatgaaaaatgccatcaaattcctgtatcagccaggcatatagtggctcatgcctgtaatctctgatgtagcaggccgaggtgggaggatcacttgagcctagaagttttgataccagcctgggcaacatagcaagaccccatctctgaaatttttttaattcctatgtcataagtcatttttatttttgtagagatagggatctcacaatattgcccaggctggtctcaaactcttggcctcaagcagtcctcctgcctcagcctcccaaaatgttgggattactggtatgtgctgctggacccagccaagtagcacttttaatttgaaaaatagttctatcagttttcagtcaggcgcggtggctcagcctgtaatcccagcactttgggaggccgagcgggggtgatcacctgaggtcgggagttcgagactagcctgaccaacatggagaaaccctgtctctactaaaaatacaaaataagccgggcatgttagcgcatgcctgtgatcccagctactcgggaggctgaggcaggagaattgcttgaacccaggaggcagaggttgcggtgagccgagatcatgccattgcactccagcctgggtaacaagagcgaaaactccgtctcaaaaaaaaaaaaagaaaaaatagttctatcagttttcataaagtactactttaatcttaaaaagattaatctagaaacccttcaaattataaaatgtcatttttaaaaggcaggagttgatatcctgatgaaattcaggtctccaaacaacttaccataatttacttcctgtattttaagtaacatgatagggtacttagagattaattgccaagaaactttttgaatatagtcaacctgcccgcacttgccatgatgagttttcttttgttccttccctctagtattctaggagatgaggttttgggaatctggtccagacatgctgagaaagctgatgtcaactgtgcctgtgtatctcattcaggaatcagtcttgttacaggagatgactttggcatggttaagttatttgacttcccatgtccagaaaaatttgtaagtttgtgttttgtttactattatcagtttactcctaattttgatgtcttatcatcagcacttttccccatatatttaaaatgttttgtcctaatttctaaatttttccccaaactttctaaatctatttactttgaaataaaagctattagaaacaaatcctctccctcgagtaataccatctttggaaccatcctacaaaagctgtaattagcttttcaccaaacctataatcagttatcaaatttcaaatgcttttccttagagaaaaatggtcagagtacctggagacatctgactgcccacacagcctggttttgcagatccactactcatgctgaaaagcattctaatcactggctgcggtgctaactccctactctctccacagctcttgtcatagagattatagttcctaataagagcctttgacttctgtgtgcaccaaatgccctgagcttgtctgtcattgttttttaggcaaaacacaaaaggttcttgggtcattcgccccatgtgacaaatattcgatttaccagtggtgatcgacatgttgttagtgctggaggtgatgactgcaggttagtaactttctcagcccatgaagagcagactatgttactagttaagagacttaatacaacaactcctacagctttggtttatgaaatcagctagtcaacattagtagaaggtagtataaccagatggctcttcagaatctcatatttatgcaaatacagaataaaaggagttaaagaggaaaaatattacacatgtaacctgaaagcacaactgaaaaatattaaactgttatgaaaatctaaaaacataattaactccctgcaattttcttctctgattgcagcttatttgtctggaaatgtgtacatacacctcactgagagatgctgagatgactacagaaattaactttgagaccagaattacagagaagaaaaaccaaaacccaaccctgcatggtcaagtggtgctaacccaagactgtaacagggagaaatgcccagaatcatcaaaatagtgaaagactgatctgttcaaaatatttgctatatgcactgggtataatccgtaatccatacactgccagataatgccatttcaaggaaggatcgaatacttgatggtaaaggccaagtccccctgtattgggaagtgtgtgatttcggcagacctgctgggaaaatttagggtagagcactctttacagaagaactcaaaaacccaatttggataattttcattatctttttagcaaaatggtttcttaatgtttatattttattttcaaggttcattgtttaatgaaatattttattcttgcatttccataaggaaagggaaagtcatgatcatcctaaaggatcacagtttttaaaaggcaaacattttccctaaggaaacagacacaagctttcctagagaatatgatgttttttaggcattaataaggtccttttttataaaggacacttttctcctagtagttttgaattcaggaacagatccaaagttagcagtatatggctgctacatttccattttcattttcgagccatcagtttatgttcagatgccatctctgtaatcgcacatttaaaacataactgtagcctcactaatggaaaagtagtatgatgaacaatcattcccaatggtgtacaatgtaagggttttagggagcaacagtatttaactggaagaaagaattgcatatttaatgtagtctaatatatacacatttgtttaacatgtaaacaaaagtgttaaattcacatatacaacattatacaatttaatcactcttggaataaaatttttatagccttttttctattgggaaaatttgtttagatgtgtgccactccataggtttatttccaaaatgaatgagcccaactccatttgtaaaaacttgtcagttagaattcctttttttagtggattagggctgaattcttagatccttatttcttttcactttaaatgctgccaaagatcactactcatcattcaggaattcgctgtctagcctatctgtagtttcctgaagattgaaaattatgtagactgctatttaaaaatatatttttctaagtgtgaggtttaagatgctgtattgaccctatgagtttttaatgtgttaattatctttatagcataatagatcgctttaggttcctggaatcccatttggtctgacaggatatatgaagattcttaatacctattttctgtgtctaatacttggttaatactaaaaatagaaatgactaaattacatcacagaaagcataaccagtgattgaacctggtagttttaaagctctaaatagctgtggctgaaggactgattatggggctaagaagcttgaaacgtaagttggtacttgttcatcagtggattctcctaaattaagccaaattttgaaatacatgactattaagtttctactcatgtatttacagtcagtcaataaattaaaggaggaaaaaaatccctgaacaacctgcccataaaaagaaaaatactctacatttgagcctgctgcagttttaaattttccctctgggtcaagtttgccagcttttggctacagagaaattatatttccattacagtgcaggtagaaactctgtaaccttaagcatgtaaactacatagaataaaactgtttccactgcatttctgtccttcaaagtggccaacctgattaagtcagccttaatcactgctgctgtcagtttcacgactaaaggtcatattgactaagtagtcatcagctgaccacctcgctgtatcagccagcaacgaggggaaggtgaagaaacatgataggccatatagaatctgccctatgtttacttttttaacccagataattatttttgtgtgcagtatctaagctcctgattgtgtaacctgggacttctggcaccttttgttccattcattttatgtataaaatgcatgccaaagcacactgtgccctctggtacccttgcttccaatcgccaaccatgctcatttccttcctttttttgtggtccctttttgtggtgatcattttaaaccacgtcatccaacaaatgttttatggtcaaccttagcttgttcataagccatagcaactgaaagattaaactcttaaatatgtgtctgggcagtggctattaaatagcaaaaaacaatcagattttagtattttattatttccttgtaaaatggctgaactaaattaaacccttgtttcccatttgttctataatttatagtgaaactgagaacaaaactatctttataaatgatagctaaaagtatttccagatatttaaacaatttaaaataaatttcttctgcagagatgcaaagcatctcaacactggaatgaacaaatgccttaaattcaatggagtaaacctttagaatgaagaggaactgtcatttcacccaagccgaagacaacagccttatgcacttgtgtgctctgtctttgctgcttctcgtgtttcaagcctttcctgtgggatcagcacagcaaagtgcaacttaccaaatggtttaatgactggttaattctttcttctcccaatggaaaagcaatggcaacacaacagtagactgctggcttgacaatcttaaacgtgagcctttgcacatgtaggtttatcatcatttgagtatacgactaagcaagtcaatgaactttttttttttttttagcagtttaatttggtcctgagaatgttgcagtctttattaccccttttgcattaatccacttttctaaccaccttttaagctttaatttttaacactatacaccaagtctttgaaatcagtgatctgttatttaactctaaagcatttgacacttcttgccttaacagttttaaaaaccacacacaaaaaaactctgtaagtaatacagtaggccaaaagtttcatcctatctatcttgcagtttacctatctgatctgatctctgtaattatagttctgtcatttaaaatatactatttaaatctaatttttacatttcaaaaattatcttcagtagtaactaagtatattttctgtggattctgagaatgttatttttcagaatgtgagaatatatatgtacatttataatcttgtgactttaaagtctgttttcagatacagtatgtaaatacttgtaaaaaaatttgtataattttgtgataatgtagtttcccaaaaaaattatttagaaggcattatgttattagtaaatgagagcactgtatagaactgttcctattttctgcacttgccattccagctgcctccactgtccatacccacctcattcatcctgtcacagaaggcaggaaaactgggaactttaccaaagtagcactcagcctgagaggcctgtataatcatgcttttcaaactaaattcacttaaaaattaaaaagcagaattgaatattttaagcagcctcagtacctttggccaatgctgttttcatggtggattatgaacattatataatctttgggaaaagtgaaagtagtacaatttttagaataatgacaactgcctcactgcatctctccactcacacagcaaccgtgtagccccctaagctgcagtaccatgactaaccatgatgtcaatttcatatgctgatcctcacaacagcagtgcacaaacatgccccaaatattttaacagaatttagctcttccttaagctgtcttttcatagtaaaaacaaaacaaaaacacccaatgttaaaaccacataataaacttacaaacttgaaaaattagacacttcagatagataggcaataaaacttcatattatgaaagcaatatattccaagtttcaaagatttgacaagttctgtagagtatctttcatcagtacatgaaaacttccaaactgcatgatcttctgccaggcaggactgggtgctattcgctggtttgaggtcgaatccatttcaaggcatgtcgtggtgggacattaatggtgggatggtagaatgtgcagtccggtcttgtacattgagtgttaaacctacaatgttttggatgatagaagggacattccatcttcttacaagcagggaagtaacggcagagctgactactggaaggtggtgctggtggtgcaactggttttggagacagtactggaattcttctactcacatgagtgaagggacaatctggtttagtacactttgcatcatatttacaatttgggtgaacaaacaaacatttttcagcaaatttacaattggggaaggctttgcagggtgagatggggtgatggtaggcacactcatccccatttttacaagcaggccagtacttgcagcgctccaaaagtttttctggtttctgtgccacactcagttcactcatctcagcgttagaaaagctaccatttgggtcctcaagctgcctgctcagcaagtgcaactgctgtgggtggaggagacctctgagtcccttgtttgaggctgcagtttggtttacgggtttcattccttcaaagcacatgtcctcctcttgatctgacatgtatcctggggggctggggacaccatccagcgtcactataaacttgggacttgcaggtttatctggttgtacaagatctcgtgtctgcataaggtgtcctgaaagtacccgaagggaatctgcagtcttcatccccgactcttggtttggtgccactactacttcctcagacagctttggcttcttcagaataaatgatcttgtgtctgcatggaccatggattccatgtcatagtaatcttgactcatctgcagagtttctgccattactgggtcgatttgcagtcgggataataattgcctctgttgagttccttgatttttttctacagaatctccttttgtttcctcttctttaatggggggacttattctgggggtcctactttgtccctggaccacttctgctagcaattcttcttgagaagttcgagttctgggagcaactggaagtgtctgtttctgtggaactgtagagtagttagttgtttttgttacggattcttgagcttcagatatagccttcaaaatcagattcttgttagcttgtttagaaggtggaagagaaggtctcctttcaggctttgcaggcacagacacactgctggagatgcttcctgttcgagacccgtaatcatcatcttcttcctcctcttctccatcatgattgaatttttttactttaacaactgaacttaccacaggcaactttctcttccgaaagttttcatcctccatactcattttctccgagttgtttctaaagaacggactatacgtttcttctaagctgttaagcacctctggttcacacaaacgtcctgtttcatatacccaactactctgcatatcaagctgcttggcagcatgaatactattctgctgctgttgaaattgcaacctgtttaaatgaacaccactatctgcatttctacttgcaggtggtcgataaatttcaatagaagggcgagaagaaccatatgtaagtgtcactgtaggttttttctgagataagggattctcctgcacaaagttgaggtcttcgtcaatgagatcatctggttctggcttaatatcaatcacatcttcagagggtgctggctccctcaaaggtttcactgttgacattagtcgggttgcagctccatcatcgtaagtctgtctgacatttgtggtttttgactcctgcgaacttgtagaaactctggaatctcttttttcaggtctcgcgctaggaatggcaagtggtggcactgcagcttcatgcctcctctcatctccccgactgaaattgctcttgtttgaaggcacgttactatcaaagatgttggtatcagaagacttcagactagagggttcagttgtaacagagcgaagtttatctaatacaccatgaagccatacggtgaatcgaattgtgttgttccctagaaacagggacagatcctctgtcatttggtcctgacttttcttgttggccaccatcaccataatgtaatcaggaagttcttcatcaacataagctcctaattcttgtaatttccccttaatggcactccggatcttgcggctgatctcggtgccgatctccatggctctgcggcgtgcgggaactcagcactgcgcggcgcttggcttacccggaggctgccgcggactcctaccccgcagccgggacaccaccgcctcc

SEQ ID NO: 17249 - RNA, 14907 nt, Homo sapiens
  source 1..14907: mol_type = other RNA
tcaggccaggcacagtggctcacacctgtaatcttatcactttgggaggctgaggcaggtggatcgcttgagcccaggagttcaagaccagcctgggcaacatggtgaaaccccatcgctataaaaaacaacaattagccgggtgtggtggcacatgcctgtagtccctgctactcaggaggctgaggtgggaggatcacttgagcctggggaggtcaaggctttagtgagctgtgatggtgccactgcactccagcctgggtgacagagtgagaccccatttaaaaaacaaaaacaaaaacaaaaaaaaatgtgacatatagttgactaagaagtacatttcaatacaggattgaaagaacccacatatgttaattaaacacaagcgcagaatttgtgccttttacataaaggaagaatgcacataggcatgctttcagacaagcaattcatctagcagaaaaggaaggaatacatttttcagcccttccaggaataaaatccataaatgggctctatttcgtcctccaacacttgtatttcccacgtcatttactcctgcacacccccactcactagaagcctgctaaactgttccagtgagatattttaacacctgatagggaataaatatgcttctgttttggccttcaaaaataagctctgggccagttgcagtggctcacgcctgtaatcccaacactttgggaggccgaggtgggcggatcacgaggtcaggagtttgggatcagcctggccaatatggtgaaactccatctctactaaaaatacaaaaattagccaggcatggtgcctgtaatcccagctacttgggaggctgaaggagaagaatcgcttgaacctgggaggcacaggttgcagtgagccgagatcacaccactgcactccaggccaggtgacagagcgacactctgtctcaaaaaaataaataaatcaactctgtagcatagcatttgtaattctattattttgccttacatttccattatccttttaataaaattgtttttttacatcttcctaatcaagaagtattatgaggccaggcacagtggctcatacctggaatcccagcactttgggaggccgaggcaggcagatcacctgaggtcaaggtatttgagaccagcctggccaacatggtgaaaccccatctctactaaaaatacagaaattagctgggtgtggtggtgcacacctgtaatgctagctactcgggaggctgaggtaggagaatcgcttgaacctgggaggcagaggttgcaataagcctagatcatgccactgcactcaagcctgggagacagagcgagactacatcttaaaaaaaaaaaaaaaagtattatgagagaggataatgtattgtaatgtattgtagaggctaaataaaattatgctcatgtcagaaaaaaagagtatttctcaaaataaaattcactgaaactggatgtttattttgactgagatatagtatatcctcaaattgccatagaaagtttacaagaatattagaggtaaattataaatatcagggcctttttaaaaaaaaaagattctgcttataacttggtatttgtttataataaaaattatagtagccaataatgaacacttactctggcttggttatttacttaggtcaaaagaaggaggagcggttaaactgtgggatcaggaactgaggcggtgccgtgccttcaggcttgagacaggacaagccacagattgtgttcgttctgtgtgcagaggcaaagtaagatgttccatgagctgatacagtgcagcagaaaacagaaagtggttattactgtgattccctcaccctttgcagcctaatgaacaatacttaataatgcataacgatggatttgcttgccaacattactctgtctttgctgctttctttgccaaagttagcaccagtgtggtgcataagctaggaagctattctgtctaaatactgtatgtaaacctccaatattttctagaatctgccaatttaacaactctagtagacataattgaaagcccttggcagttgactcatattaggacagctgtctccattttttaaaaaaacacacattccctagataaaacgtgcagtaaacaaacaatgaaatactactcagccataaaaaataatgaaattctgtcattcttggtggcaacatggatgagactggaggacatgatgtgaagtgaaataagccaggcacagaaagataaatacatgttctcactcctgtgcagaaactaaaaaagttgatcccacagaggtggagagtagaatagtggttactggaggcggacaagggggagggggagggggatagggaaggactggttaaaggatacaagtttacacagccagataggaatagtatgttttagtattctgtagtactgtaggatgactatagttaagaatcacgtatttatgtattttcaggtatttacaagagaggattttgaaagtttccatcacaaagaaatgataaatgtctgaggtgatggttatgcgtattaccctatgccctatagatatgtataattatgtgtcaatttcaaaataaaaattcaaaactacaactcctatgaaaatttttgagcgtgtttgtacttattaagtgtatttataaatcatacggatattatcttcagcctgcatattaaattgtagttaagcttttactttttaactaaaaaataaattctattattttttcctatatcccactgcactgaccccagtttggaaatcctaagattatcaaataaaaactttgattattgaagaatccaggtgtactgccacagaaaagttctattctgtagcatggactctaatatgtaatctagcccattgtgcttacagatagatgtgtgcctgtagtcatagaaaaatttgcatgagctaatgactgccttgctactagattagctcaaagcaaaaagttctctgaaagcaggtcaatagggtcatttttatattatgaagaagaaaagcagctgttgtattacattcactgtattggtcctgcttgtgtttcagggcaagatccttgttgggacaaggaatgctgaaataatcgaagttggagagaaaaatgcagcttgtaatattttagttaacggtcatgtggatgggccaatctggggactagcaacacatccttccagggattttttcctttctgctgcagaagatgggacagtgagactttgggatattgctgataaagtaagtacagataatttttttaaaagaggttacaacttctaaaaagaaaagttggaagttctaaattgctagtacttaaagaactgccagaattctgttgagcattttgaggggaaactggtataatttagaagtacttcacttaatgtttcctatgactctttttttttttttttttaaatgcagaagatgttaaacaaagtgaatttgggacatgctgctcgtactgtgtgttacagccctgaaggggacatggtggctattggaatgaaaaatggagaatttatcattttactagtgagttctctaaaaatatggggaaagaagagagacaggagatgtgcaatccatgatatcaggttagtgaacaaatggaatagagtttctagtatatacttgatttaacttccatttgtaaaattttccatagccttgccttcaaaaagaggtccccagggcctgtagcatttcccgtattataaattgtatgctaaaatatggctgtttgtatactacttaattcttcttgctaaattataaacccactgggcaccaactataatagcaagtactagtaggtaatgtttgatgaattcatgttaacacttagccatgtccattaagttcatcccaccaagaggtatctcccactgtaatacaagagagctatctgcccttcaaaagttgtcaccctggaaaactaaagttgtgatttcaaacatatcttctcttagtaacctcagtttgggaatatgtagttcattaatttaatcaatacctattgattaaatgttccagaatccaaattaatttaaatgtttcttaaacctttgtttttcagtgcttaagcatttttcaacagtggctaccatttacggagtacttccgtgtgatcagtagataagattattgaatctaggtctgtcaaaagcttgtacacttttcatcagtaaaatccttttacaaatgaaaccttcctcagaacttcaatatataaaatagtaacagtggcttcccttagcttttacatgtctctatcgtacctcagtaagactcatgggccatttcaagagactgaattgtcccatatgactccaaagattgctaggcaaatagcatttcactttgtcttttaaataagttcttcaggccgggcgcggtggctcatgcctgtaatcccagcactttgggaggccgaggcaggcagatcacctgaagtcaggagtactcgaccagcctggccaacatagtgaaaccccatctcaactaaaaatacaaaaatcagccgggcgtggtggcaggcgcctgtaatcccagctactcagggggctgaaacaggagaatcgcttgaacccgggaggcggaggttgcgccatcgcactccagcctgggagacaagagcgagacttcgtctcaaaaaaaaaaaattcttcttccaagattcaagttgtgtcatttcaccttaataactggaggttagttaagctgggctgtgttctttgcttaatattaagacaacgttttttccagatggaagaaaactatcttaatgaattgttagcttattaattatgtaatgctaatggcttttaaaagctgagatgttctgactgggtgttgtggctcacacctgtaatcccagtaccttgggaggccaagggggaaggattgcttgaggccaggagtttgggaccatagtgagaccccgcctctatttaaaaaattaaattttgttttgttttgttttgagttggagttttgctcttgttgcccatgctgaagtgcaatggtgcaatctcagctcaccacaacctgtgcctcctgggttcaagcgattctcctgcttcagcctcccgagtagatgggattacaggcgtgcaccaccatgcctggctaattttgtatttttagtagagacagggtttctctatgttggtcaggctggtctcaaactctcgacctcaggtgatctgcccgcctccgcttcccaaagttctgggattataggtgtgagccactgggcctggcctaagaaagtttttttaagccattagacgtttttaaaggaattgggagatgacaattggggaaatatttaaaatttaagtaaaatataaagcttccttatttcatgtaacccagacaatctcagtatacatgatcagttgtgtctgacaggtaaatctatttgaggccttatcacacgttacttttaagaactagaaaggaaaagtcactgatcttaagtatttataatacttcatgtggtctaatactttttacgttttgttttgattcagatttagtccggattcccggtatctggcagtaggttctagtgagaactcagtggatttttatgacctaacgctgggccccactcttaacagaatcagctactgcaaagacattccaagctttgtcattcaaatggacttctctgcagatagcagttatctccaggtacagtaccaatactgtatacccaggtggcaagttcttctgcttttacatttcgtgttagtgaatgcatttaaagttcctgagctccagagctccagcttctcaactcctccctttgtaccttctgacctacagctcccctttcctcccccacttatcagagcttttctcctattaagtttttgtagtgatcttttgcatacttaataatgttagacatgtaaatcaagtagcaatatgctagtattctgtaaaccccctgtggattttgtctctcacctaatggaattcttgtcccattttaatctgatgaaaaaggtctctagtggctgctataaacggcatgtctatgaagtgccttcaggaaaacatcttatggatcatgccgctattgacagaattacttgggctacatggactaggtaaatacttatatattcacaaggcaagaactgactttgaaggccagttagaaaatcctatttctgaactgttagagccattccaataaggaatagtaattgagtttcaagtttttgttaccatattttgaaatggtatgttcatgttgggacccctttttattgaatatatttccatgttttatcagtttccatgatttatcaagttttttttttaaggaaatcaaagttttaactttaaagataccctgatatttttcttaatgctaaatttaatgactggcaaaaaggtattgggtgctgttaagcaactgttattaattctctatctaaaggaatgctatcttgaatctattagaagtcaaagcttccaaatttgttcaaatttcctggctgtatgacaggtaaccatgactatccatttttttggccaatgaaaaatgccatcaaattcctgtatcagccaggcatatagtggctcatgcctgtaatctctgatgtagcaggccgaggtgggaggatcacttgagcctagaagttttgataccagcctgggcaacatagcaagaccccatctctgaaatttttttaattcctatgtcataagtcatttttatttttgtagagatagggatctcacaatattgcccaggctggtctcaaactcttggcctcaagcagtcctcctgcctcagcctcccaaaatgttgggattactggtatgtgctgctggacccagccaagtagcacttttaatttgaaaaatagttctatcagttttcagtcaggcgcggtggctcagcctgtaatcccagcactttgggaggccgagcgggggtgatcacctgaggtcgggagttcgagactagcctgaccaacatggagaaaccctgtctctactaaaaatacaaaataagccgggcatgttagcgcatgcctgtgatcccagctactcgggaggctgaggcaggagaattgcttgaacccaggaggcagaggttgcggtgagccgagatcatgccattgcactccagcctgggtaacaagagcgaaaactccgtctcaaaaaaaaaaaaagaaaaaatagttctatcagttttcataaagtactactttaatcttaaaaagattaatctagaaacccttcaaattataaaatgtcatttttaaaaggcaggagttgatatcctgatgaaattcaggtctccaaacaacttaccataatttacttcctgtattttaagtaacatgatagggtacttagagattaattgccaagaaactttttgaatatagtcaacctgcccgcacttgccatgatgagttttcttttgttccttccctctagtattctaggagatgaggttttgggaatctggtccagacatgctgagaaagctgatgtcaactgtgcctgtgtatctcattcaggaatcagtcttgttacaggagatgactttggcatggttaagttatttgacttcccatgtccagaaaaatttgtaagtttgtgttttgtttactattatcagtttactcctaattttgatgtcttatcatcagcacttttccccatatatttaaaatgttttgtcctaatttctaaatttttccccaaactttctaaatctatttactttgaaataaaagctattagaaacaaatcctctccctcgagtaataccatctttggaaccatcctacaaaagctgtaattagcttttcaccaaacctataatcagttatcaaatttcaaatgcttttccttagagaaaaatggtcagagtacctggagacatctgactgcccacacagcctggttttgcagatccactactcatgctgaaaagcattctaatcactggctgcggtgctaactccctactctctccacagctcttgtcatagagattatagttcctaataagagcctttgacttctgtgtgcaccaaatgccctgagcttgtctgtcattgttttttaggcaaaacacaaaaggttcttgggtcattcgccccatgtgacaaatattcgatttaccagtggtgatcgacatgttgttagtgctggaggtgatgactgcaggttagtaactttctcagcccatgaagagcagactatgttactagttaagagacttaatacaacaactcctacagctttggtttatgaaatcagctagtcaacattagtagaaggtagtataaccagatggctcttcagaatctcatatttatgcaaatacagaataaaaggagttaaagaggaaaaatattacacatgtaacctgaaagcacaactgaaaaatattaaactgttatgaaaatctaaaaacataattaactccctgcaattttcttctctgattgcagcttatttgtctggaaatgtgtacatacacctcactgagagatgctgagatgactacagaaattaactttgagaccagaattacagagaagaaaaaccaaaacccaaccctgcatggtcaagtggtgctaacccaagactgtaacagggagaaatgcccagaatcatcaaaatagtgaaagactgatctgttcaaaatatttgctatatgcactgggtataatccgtaatccatacactgccagataatgccatttcaaggaaggatcgaatacttgatggtaaaggccaagtccccctgtattgggaagtgtgtgatttcggcagacctgctgggaaaatttagggtagagcactctttacagaagaactcaaaaacccaatttggataattttcattatctttttagcaaaatggtttcttaatgtttatattttattttcaaggttcattgtttaatgaaatattttattcttgcatttccataaggaaagggaaagtcatgatcatcctaaaggatcacagtttttaaaaggcaaacattttccctaaggaaacagacacaagctttcctagagaatatgatgttttttaggcattaataaggtccttttttataaaggacacttttctcctagtagttttgaattcaggaacagatccaaagttagcagtatatggctgctacatttccattttcattttcgagccatcagtttatgttcagatgccatctctgtaatcgcacatttaaaacataactgtagcctcactaatggaaaagtagtatgatgaacaatcattcccaatggtgtacaatgtaagggttttagggagcaacagtatttaactggaagaaagaattgcatatttaatgtagtctaatatatacacatttgtttaacatgtaaacaaaagtgttaaattcacatatacaacattatacaatttaatcactcttggaataaaatttttatagccttttttctattgggaaaatttgtttagatgtgtgccactccataggtttatttccaaaatgaatgagcccaactccatttgtaaaaacttgtcagttagaattcctttttttagtggattagggctgaattcttagatccttatttcttttcactttaaatgctgccaaagatcactactcatcattcaggaattcgctgtctagcctatctgtagtttcctgaagattgaaaattatgtagactgctatttaaaaatatatttttctaagtgtgaggtttaagatgctgtattgaccctatgagtttttaatgtgttaattatctttatagcataatagatcgctttaggttcctggaatcccatttggtctgacaggatatatgaagattcttaatacctattttctgtgtctaatacttggttaatactaaaaatagaaatgactaaattacatcacagaaagcataaccagtgattgaacctggtagttttaaagctctaaatagctgtggctgaaggactgattatggggctaagaagcttgaaacgtaagttggtacttgttcatcagtggattctcctaaattaagccaaattttgaaatacatgactattaagtttctactcatgtatttacagtcagtcaataaattaaaggaggaaaaaaatccctgaacaacctgcccataaaaagaaaaatactctacatttgagcctgctgcagttttaaattttccctctgggtcaagtttgccagcttttggctacagagaaattatatttccattacagtgcaggtagaaactctgtaaccttaagcatgtaaactacatagaataaaactgtttccactgcatttctgtccttcaaagtggccaacctgattaagtcagccttaatcactgctgctgtcagtttcacgactaaaggtcatattgactaagtagtcatcagctgaccacctcgctgtatcagccagcaacgaggggaaggtgaagaaacatgataggccatatagaatctgccctatgtttacttttttaacccagataattatttttgtgtgcagtatctaagctcctgattgtgtaacctgggacttctggcaccttttgttccattcattttatgtataaaatgcatgccaaagcacactgtgccctctggtacccttgcttccaatcgccaaccatgctcatttccttcctttttttgtggtccctttttgtggtgatcattttaaaccacgtcatccaacaaatgttttatggtcaaccttagcttgttcataagccatagcaactgaaagattaaactcttaaatatgtgtctgggcagtggctattaaatagcaaaaaacaatcagattttagtattttattatttccttgtaaaatggctgaactaaattaaacccttgtttcccatttgttctataatttatagtgaaactgagaacaaaactatctttataaatgatagctaaaagtatttccagatatttaaacaatttaaaataaatttcttctgcagagatgcaaagcatctcaacactggaatgaacaaatgccttaaattcaatggagtaaacctttagaatgaagaggaactgtcatttcacccaagccgaagacaacagccttatgcacttgtgtgctctgtctttgctgcttctcgtgtttcaagcctttcctgtgggatcagcacagcaaagtgcaacttaccaaatggtttaatgactggttaattctttcttctcccaatggaaaagcaatggcaacacaacagtagactgctggcttgacaatcttaaacgtgagcctttgcacatgtaggtttatcatcatttgagtatacgactaagcaagtcaatgaactttttttttttttttagcagtttaatttggtcctgagaatgttgcagtctttattaccccttttgcattaatccacttttctaaccaccttttaagctttaatttttaacactatacaccaagtctttgaaatcagtgatctgttatttaactctaaagcatttgacacttcttgccttaacagttttaaaaaccacacacaaaaaaactctgtaagtaatacagtaggccaaaagtttcatcctatctatcttgcagtttacctatctgatctgatctctgtaattatagttctgtcatttaaaatatactatttaaatctaatttttacatttcaaaaattatcttcagtagtaactaagtatattttctgtggattctgagaatgttatttttcagaatgtgagaatatatatgtacatttataatcttgtgactttaaagtctgttttcagatacagtatgtaaatacttgtaaaaaaatttgtataattttgtgataatgtagtttcccaaaaaaattatttagaaggcattatgttattagtaaatgagagcactgtatagaactgttcctattttctgcacttgccattccagctgcctccactgtccatacccacctcattcatcctgtcacagaaggcaggaaaactgggaactttaccaaagtagcactcagcctgagaggcctgtataatcatgcttttcaaactaaattcacttaaaaattaaaaagcagaattgaatattttaagcagcctcagtacctttggccaatgctgttttcatggtggattatgaacattatataatctttgggaaaagtgaaagtagtacaatttttagaataatgacaactgcctcactgcatctctccactcacacagcaaccgtgtagccccctaagctgcagtaccatgactaaccatgatgtcaatttcatatgctgatcctcacaacagcagtgcacaaacatgccccaaatattttaacagaatttagctcttccttaagctgtcttttcatagtaaaaacaaaacaaaaacacccaatgttaaaaccacataataaacttacaaacttgaaaaattagacacttcagatagataggcaataaaacttcatattatgaaagcaatatattccaagtttcaaagatttgacaagttctgtagagtatctttcatcagtacatgaaaacttccaaactgcatgatcttctgccaggcaggactgggtgctattcgctggtttgaggtcgaatccatttcaaggcatgtcgtggtgggacattaatggtgggatggtagaatgtgcagtccggtcttgtacattgagtgttaaacctacaatgttttggatgatagaagggacattccatcttcttacaagcagggaagtaacggcagagctgactactggaaggtggtgctggtggtgcaactggttttggagacagtactggaattcttctactcacatgagtgaagggacaatctggtttagtacactttgcatcatatttacaatttgggtgaacaaacaaacatttttcagcaaatttacaattggggaaggctttgcagggtgagatggggtgatggtaggcacactcatccccatttttacaagcaggccagtacttgcagcgctccaaaagtttttctggtttctgtgccacactcagttcactcatctcagcgttagaaaagctaccatttgggtcctcaagctgcctgctcagcaagtgcaactgctgtgggtggaggagacctctgagtcccttgtttgaggctgcagtttggtttacgggtttcattccttcaaagcacatgtcctcctcttgatctgacatgtatcctggggggctggggacaccatccagcgtcactataaacttgggacttgcaggtttatctggttgtacaagatctcgtgtctgcataaggtgtcctgaaagtacccgaagggaatctgcagtcttcatccccgactcttggtttggtgccactactacttcctcagacagctttggcttcttcagaataaatgatcttgtgtctgcatggaccatggattccatgtcatagtaatcttgactcatctgcagagtttctgccattactgggtcgatttgcagtcgggataataattgcctctgttgagttccttgatttttttctacagaatctccttttgtttcctcttctttaatggggggacttattctgggggtcctactttgtccctggaccacttctgctagcaattcttcttgagaagttcgagttctgggagcaactggaagtgtctgtttctgtggaactgtagagtagttagttgtttttgttacggattcttgagcttcagatatagccttcaaaatcagattcttgttagcttgtttagaaggtggaagagaaggtctcctttcaggctttgcaggcacagacacactgctggagatgcttcctgttcgagacccgtaatcatcatcttcttcctcctcttctccatcatgattgaatttttttactttaacaactgaacttaccacaggcaactttctcttccgaaagttttcatcctccatactcattttctccgagttgtttctaaagaacggactatacgtttcttctaagctgttaagcacctctggttcacacaaacgtcctgtttcatatacccaactactctgcatatcaagctgcttggcagcatgaatactattctgctgctgttgaaattgcaacctgtttaaatgaacaccactatctgcatttctacttgcaggtggtcgataaatttcaatagaagggcgagaagaaccatatgtaagtgtcactgtaggttttttctgagataagggattctcctgcacaaagttgaggtcttcgtcaatgagatcatctggttctggcttaatatcaatcacatcttcagagggtgctggctccctcaaaggtttcactgttgacattagtcgggttgcagctccatcatcgtaagtctgtctgacatttgtggtttttgactcctgcgaacttgtagaaactctggaatctcttttttcaggtctcgcgctaggaatggcaagtggtggcactgcagcttcatgcctcctctcatctccccgactgaaattgctcttgtttgaaggcacgttactatcaaagatgttggtatcagaagacttcagactagagggttcagttgtaacagagcgaagtttatctaatacaccatgaagccatacggtgaatcgaattgtgttgttccctagaaacagggacagatcctctgtcatttggtcctgacttttcttgttggccaccatcaccataatgtaatcaggaagttcttcatcaacataagctcctaattcttgtaatttccccttaatggcactctcccgcagcggatccaaagcggcgccgtgcgccgcggtggtggctccagccgggcctgcgcctgtccttccatttcccggcggctacttcagccgcagccacgctccg

SEQ ID NO: 17250 - RNA, 15112 nt, Homo sapiens
  source 1..15112: mol_type = other RNA
tcaggccaggcacagtggctcacacctgtaatcttatcactttgggaggctgaggcaggtggatcgcttgagcccaggagttcaagaccagcctgggcaacatggtgaaaccccatcgctataaaaaacaacaattagccgggtgtggtggcacatgcctgtagtccctgctactcaggaggctgaggtgggaggatcacttgagcctggggaggtcaaggctttagtgagctgtgatggtgccactgcactccagcctgggtgacagagtgagaccccatttaaaaaacaaaaacaaaaacaaaaaaaaatgtgacatatagttgactaagaagtacatttcaatacaggattgaaagaacccacatatgttaattaaacacaagcgcagaatttgtgccttttacataaaggaagaatgcacataggcatgctttcagacaagcaattcatctagcagaaaaggaaggaatacatttttcagcccttccaggaataaaatccataaatgggctctatttcgtcctccaacacttgtatttcccacgtcatttactcctgcacacccccactcactagaagcctgctaaactgttccagtgagatattttaacacctgatagggaataaatatgcttctgttttggccttcaaaaataagctctgggccagttgcagtggctcacgcctgtaatcccaacactttgggaggccgaggtgggcggatcacgaggtcaggagtttgggatcagcctggccaatatggtgaaactccatctctactaaaaatacaaaaattagccaggcatggtgcctgtaatcccagctacttgggaggctgaaggagaagaatcgcttgaacctgggaggcacaggttgcagtgagccgagatcacaccactgcactccaggccaggtgacagagcgacactctgtctcaaaaaaataaataaatcaactctgtagcatagcatttgtaattctattattttgccttacatttccattatccttttaataaaattgtttttttacatcttcctaatcaagaagtattatgaggccaggcacagtggctcatacctggaatcccagcactttgggaggccgaggcaggcagatcacctgaggtcaaggtatttgagaccagcctggccaacatggtgaaaccccatctctactaaaaatacagaaattagctgggtgtggtggtgcacacctgtaatgctagctactcgggaggctgaggtaggagaatcgcttgaacctgggaggcagaggttgcaataagcctagatcatgccactgcactcaagcctgggagacagagcgagactacatcttaaaaaaaaaaaaaaaagtattatgagagaggataatgtattgtaatgtattgtagaggctaaataaaattatgctcatgtcagaaaaaaagagtatttctcaaaataaaattcactgaaactggatgtttattttgactgagatatagtatatcctcaaattgccatagaaagtttacaagaatattagaggtaaattataaatatcagggcctttttaaaaaaaaaagattctgcttataacttggtatttgtttataataaaaattatagtagccaataatgaacacttactctggcttggttatttacttaggtcaaaagaaggaggagcggttaaactgtgggatcaggaactgaggcggtgccgtgccttcaggcttgagacaggacaagccacagattgtgttcgttctgtgtgcagaggcaaagtaagatgttccatgagctgatacagtgcagcagaaaacagaaagtggttattactgtgattccctcaccctttgcagcctaatgaacaatacttaataatgcataacgatggatttgcttgccaacattactctgtctttgctgctttctttgccaaagttagcaccagtgtggtgcataagctaggaagctattctgtctaaatactgtatgtaaacctccaatattttctagaatctgccaatttaacaactctagtagacataattgaaagcccttggcagttgactcatattaggacagctgtctccattttttaaaaaaacacacattccctagataaaacgtgcagtaaacaaacaatgaaatactactcagccataaaaaataatgaaattctgtcattcttggtggcaacatggatgagactggaggacatgatgtgaagtgaaataagccaggcacagaaagataaatacatgttctcactcctgtgcagaaactaaaaaagttgatcccacagaggtggagagtagaatagtggttactggaggcggacaagggggagggggagggggatagggaaggactggttaaaggatacaagtttacacagccagataggaatagtatgttttagtattctgtagtactgtaggatgactatagttaagaatcacgtatttatgtattttcaggtatttacaagagaggattttgaaagtttccatcacaaagaaatgataaatgtctgaggtgatggttatgcgtattaccctatgccctatagatatgtataattatgtgtcaatttcaaaataaaaattcaaaactacaactcctatgaaaatttttgagcgtgtttgtacttattaagtgtatttataaatcatacggatattatcttcagcctgcatattaaattgtagttaagcttttactttttaactaaaaaataaattctattattttttcctatatcccactgcactgaccccagtttggaaatcctaagattatcaaataaaaactttgattattgaagaatccaggtgtactgccacagaaaagttctattctgtagcatggactctaatatgtaatctagcccattgtgcttacagatagatgtgtgcctgtagtcatagaaaaatttgcatgagctaatgactgccttgctactagattagctcaaagcaaaaagttctctgaaagcaggtcaatagggtcatttttatattatgaagaagaaaagcagctgttgtattacattcactgtattggtcctgcttgtgtttcagggcaagatccttgttgggacaaggaatgctgaaataatcgaagttggagagaaaaatgcagcttgtaatattttagttaacggtcatgtggatgggccaatctggggactagcaacacatccttccagggattttttcctttctgctgcagaagatgggacagtgagactttgggatattgctgataaagtaagtacagataatttttttaaaagaggttacaacttctaaaaagaaaagttggaagttctaaattgctagtacttaaagaactgccagaattctgttgagcattttgaggggaaactggtataatttagaagtacttcacttaatgtttcctatgactctttttttttttttttttaaatgcagaagatgttaaacaaagtgaatttgggacatgctgctcgtactgtgtgttacagccctgaaggggacatggtggctattggaatgaaaaatggagaatttatcattttactagtgagttctctaaaaatatggggaaagaagagagacaggagatgtgcaatccatgatatcaggttagtgaacaaatggaatagagtttctagtatatacttgatttaacttccatttgtaaaattttccatagccttgccttcaaaaagaggtccccagggcctgtagcatttcccgtattataaattgtatgctaaaatatggctgtttgtatactacttaattcttcttgctaaattataaacccactgggcaccaactataatagcaagtactagtaggtaatgtttgatgaattcatgttaacacttagccatgtccattaagttcatcccaccaagaggtatctcccactgtaatacaagagagctatctgcccttcaaaagttgtcaccctggaaaactaaagttgtgatttcaaacatatcttctcttagtaacctcagtttgggaatatgtagttcattaatttaatcaatacctattgattaaatgttccagaatccaaattaatttaaatgtttcttaaacctttgtttttcagtgcttaagcatttttcaacagtggctaccatttacggagtacttccgtgtgatcagtagataagattattgaatctaggtctgtcaaaagcttgtacacttttcatcagtaaaatccttttacaaatgaaaccttcctcagaacttcaatatataaaatagtaacagtggcttcccttagcttttacatgtctctatcgtacctcagtaagactcatgggccatttcaagagactgaattgtcccatatgactccaaagattgctaggcaaatagcatttcactttgtcttttaaataagttcttcaggccgggcgcggtggctcatgcctgtaatcccagcactttgggaggccgaggcaggcagatcacctgaagtcaggagtactcgaccagcctggccaacatagtgaaaccccatctcaactaaaaatacaaaaatcagccgggcgtggtggcaggcgcctgtaatcccagctactcagggggctgaaacaggagaatcgcttgaacccgggaggcggaggttgcgccatcgcactccagcctgggagacaagagcgagacttcgtctcaaaaaaaaaaaattcttcttccaagattcaagttgtgtcatttcaccttaataactggaggttagttaagctgggctgtgttctttgcttaatattaagacaacgttttttccagatggaagaaaactatcttaatgaattgttagcttattaattatgtaatgctaatggcttttaaaagctgagatgttctgactgggtgttgtggctcacacctgtaatcccagtaccttgggaggccaagggggaaggattgcttgaggccaggagtttgggaccatagtgagaccccgcctctatttaaaaaattaaattttgttttgttttgttttgagttggagttttgctcttgttgcccatgctgaagtgcaatggtgcaatctcagctcaccacaacctgtgcctcctgggttcaagcgattctcctgcttcagcctcccgagtagatgggattacaggcgtgcaccaccatgcctggctaattttgtatttttagtagagacagggtttctctatgttggtcaggctggtctcaaactctcgacctcaggtgatctgcccgcctccgcttcccaaagttctgggattataggtgtgagccactgggcctggcctaagaaagtttttttaagccattagacgtttttaaaggaattgggagatgacaattggggaaatatttaaaatttaagtaaaatataaagcttccttatttcatgtaacccagacaatctcagtatacatgatcagttgtgtctgacaggtaaatctatttgaggccttatcacacgttacttttaagaactagaaaggaaaagtcactgatcttaagtatttataatacttcatgtggtctaatactttttacgttttgttttgattcagatttagtccggattcccggtatctggcagtaggttctagtgagaactcagtggatttttatgacctaacgctgggccccactcttaacagaatcagctactgcaaagacattccaagctttgtcattcaaatggacttctctgcagatagcagttatctccaggtacagtaccaatactgtatacccaggtggcaagttcttctgcttttacatttcgtgttagtgaatgcatttaaagttcctgagctccagagctccagcttctcaactcctccctttgtaccttctgacctacagctcccctttcctcccccacttatcagagcttttctcctattaagtttttgtagtgatcttttgcatacttaataatgttagacatgtaaatcaagtagcaatatgctagtattctgtaaaccccctgtggattttgtctctcacctaatggaattcttgtcccattttaatctgatgaaaaaggtctctagtggctgctataaacggcatgtctatgaagtgccttcaggaaaacatcttatggatcatgccgctattgacagaattacttgggctacatggactaggtaaatacttatatattcacaaggcaagaactgactttgaaggccagttagaaaatcctatttctgaactgttagagccattccaataaggaatagtaattgagtttcaagtttttgttaccatattttgaaatggtatgttcatgttgggacccctttttattgaatatatttccatgttttatcagtttccatgatttatcaagttttttttttaaggaaatcaaagttttaactttaaagataccctgatatttttcttaatgctaaatttaatgactggcaaaaaggtattgggtgctgttaagcaactgttattaattctctatctaaaggaatgctatcttgaatctattagaagtcaaagcttccaaatttgttcaaatttcctggctgtatgacaggtaaccatgactatccatttttttggccaatgaaaaatgccatcaaattcctgtatcagccaggcatatagtggctcatgcctgtaatctctgatgtagcaggccgaggtgggaggatcacttgagcctagaagttttgataccagcctgggcaacatagcaagaccccatctctgaaatttttttaattcctatgtcataagtcatttttatttttgtagagatagggatctcacaatattgcccaggctggtctcaaactcttggcctcaagcagtcctcctgcctcagcctcccaaaatgttgggattactggtatgtgctgctggacccagccaagtagcacttttaatttgaaaaatagttctatcagttttcagtcaggcgcggtggctcagcctgtaatcccagcactttgggaggccgagcgggggtgatcacctgaggtcgggagttcgagactagcctgaccaacatggagaaaccctgtctctactaaaaatacaaaataagccgggcatgttagcgcatgcctgtgatcccagctactcgggaggctgaggcaggagaattgcttgaacccaggaggcagaggttgcggtgagccgagatcatgccattgcactccagcctgggtaacaagagcgaaaactccgtctcaaaaaaaaaaaaagaaaaaatagttctatcagttttcataaagtactactttaatcttaaaaagattaatctagaaacccttcaaattataaaatgtcatttttaaaaggcaggagttgatatcctgatgaaattcaggtctccaaacaacttaccataatttacttcctgtattttaagtaacatgatagggtacttagagattaattgccaagaaactttttgaatatagtcaacctgcccgcacttgccatgatgagttttcttttgttccttccctctagtattctaggagatgaggttttgggaatctggtccagacatgctgagaaagctgatgtcaactgtgcctgtgtatctcattcaggaatcagtcttgttacaggagatgactttggcatggttaagttatttgacttcccatgtccagaaaaatttgtaagtttgtgttttgtttactattatcagtttactcctaattttgatgtcttatcatcagcacttttccccatatatttaaaatgttttgtcctaatttctaaatttttccccaaactttctaaatctatttactttgaaataaaagctattagaaacaaatcctctccctcgagtaataccatctttggaaccatcctacaaaagctgtaattagcttttcaccaaacctataatcagttatcaaatttcaaatgcttttccttagagaaaaatggtcagagtacctggagacatctgactgcccacacagcctggttttgcagatccactactcatgctgaaaagcattctaatcactggctgcggtgctaactccctactctctccacagctcttgtcatagagattatagttcctaataagagcctttgacttctgtgtgcaccaaatgccctgagcttgtctgtcattgttttttaggcaaaacacaaaaggttcttgggtcattcgccccatgtgacaaatattcgatttaccagtggtgatcgacatgttgttagtgctggaggtgatgactgcaggttagtaactttctcagcccatgaagagcagactatgttactagttaagagacttaatacaacaactcctacagctttggtttatgaaatcagctagtcaacattagtagaaggtagtataaccagatggctcttcagaatctcatatttatgcaaatacagaataaaaggagttaaagaggaaaaatattacacatgtaacctgaaagcacaactgaaaaatattaaactgttatgaaaatctaaaaacataattaactccctgcaattttcttctctgattgcagcttatttgtctggaaatgtgtacatacacctcactgagagatgctgagatgactacagaaattaactttgagaccagaattacagagaagaaaaaccaaaacccaaccctgcatggtcaagtggtgctaacccaagactgtaacagggagaaatgcccagaatcatcaaaatagtgaaagactgatctgttcaaaatatttgctatatgcactgggtataatccgtaatccatacactgccagataatgccatttcaaggaaggatcgaatacttgatggtaaaggccaagtccccctgtattgggaagtgtgtgatttcggcagacctgctgggaaaatttagggtagagcactctttacagaagaactcaaaaacccaatttggataattttcattatctttttagcaaaatggtttcttaatgtttatattttattttcaaggttcattgtttaatgaaatattttattcttgcatttccataaggaaagggaaagtcatgatcatcctaaaggatcacagtttttaaaaggcaaacattttccctaaggaaacagacacaagctttcctagagaatatgatgttttttaggcattaataaggtccttttttataaaggacacttttctcctagtagttttgaattcaggaacagatccaaagttagcagtatatggctgctacatttccattttcattttcgagccatcagtttatgttcagatgccatctctgtaatcgcacatttaaaacataactgtagcctcactaatggaaaagtagtatgatgaacaatcattcccaatggtgtacaatgtaagggttttagggagcaacagtatttaactggaagaaagaattgcatatttaatgtagtctaatatatacacatttgtttaacatgtaaacaaaagtgttaaattcacatatacaacattatacaatttaatcactcttggaataaaatttttatagccttttttctattgggaaaatttgtttagatgtgtgccactccataggtttatttccaaaatgaatgagcccaactccatttgtaaaaacttgtcagttagaattcctttttttagtggattagggctgaattcttagatccttatttcttttcactttaaatgctgccaaagatcactactcatcattcaggaattcgctgtctagcctatctgtagtttcctgaagattgaaaattatgtagactgctatttaaaaatatatttttctaagtgtgaggtttaagatgctgtattgaccctatgagtttttaatgtgttaattatctttatagcataatagatcgctttaggttcctggaatcccatttggtctgacaggatatatgaagattcttaatacctattttctgtgtctaatacttggttaatactaaaaatagaaatgactaaattacatcacagaaagcataaccagtgattgaacctggtagttttaaagctctaaatagctgtggctgaaggactgattatggggctaagaagcttgaaacgtaagttggtacttgttcatcagtggattctcctaaattaagccaaattttgaaatacatgactattaagtttctactcatgtatttacagtcagtcaataaattaaaggaggaaaaaaatccctgaacaacctgcccataaaaagaaaaatactctacatttgagcctgctgcagttttaaattttccctctgggtcaagtttgccagcttttggctacagagaaattatatttccattacagtgcaggtagaaactctgtaaccttaagcatgtaaactacatagaataaaactgtttccactgcatttctgtccttcaaagtggccaacctgattaagtcagccttaatcactgctgctgtcagtttcacgactaaaggtcatattgactaagtagtcatcagctgaccacctcgctgtatcagccagcaacgaggggaaggtgaagaaacatgataggccatatagaatctgccctatgtttacttttttaacccagataattatttttgtgtgcagtatctaagctcctgattgtgtaacctgggacttctggcaccttttgttccattcattttatgtataaaatgcatgccaaagcacactgtgccctctggtacccttgcttccaatcgccaaccatgctcatttccttcctttttttgtggtccctttttgtggtgatcattttaaaccacgtcatccaacaaatgttttatggtcaaccttagcttgttcataagccatagcaactgaaagattaaactcttaaatatgtgtctgggcagtggctattaaatagcaaaaaacaatcagattttagtattttattatttccttgtaaaatggctgaactaaattaaacccttgtttcccatttgttctataatttatagtgaaactgagaacaaaactatctttataaatgatagctaaaagtatttccagatatttaaacaatttaaaataaatttcttctgcagagatgcaaagcatctcaacactggaatgaacaaatgccttaaattcaatggagtaaacctttagaatgaagaggaactgtcatttcacccaagccgaagacaacagccttatgcacttgtgtgctctgtctttgctgcttctcgtgtttcaagcctttcctgtgggatcagcacagcaaagtgcaacttaccaaatggtttaatgactggttaattctttcttctcccaatggaaaagcaatggcaacacaacagtagactgctggcttgacaatcttaaacgtgagcctttgcacatgtaggtttatcatcatttgagtatacgactaagcaagtcaatgaactttttttttttttttagcagtttaatttggtcctgagaatgttgcagtctttattaccccttttgcattaatccacttttctaaccaccttttaagctttaatttttaacactatacaccaagtctttgaaatcagtgatctgttatttaactctaaagcatttgacacttcttgccttaacagttttaaaaaccacacacaaaaaaactctgtaagtaatacagtaggccaaaagtttcatcctatctatcttgcagtttacctatctgatctgatctctgtaattatagttctgtcatttaaaatatactatttaaatctaatttttacatttcaaaaattatcttcagtagtaactaagtatattttctgtggattctgagaatgttatttttcagaatgtgagaatatatatgtacatttataatcttgtgactttaaagtctgttttcagatacagtatgtaaatacttgtaaaaaaatttgtataattttgtgataatgtagtttcccaaaaaaattatttagaaggcattatgttattagtaaatgagagcactgtatagaactgttcctattttctgcacttgccattccagctgcctccactgtccatacccacctcattcatcctgtcacagaaggcaggaaaactgggaactttaccaaagtagcactcagcctgagaggcctgtataatcatgcttttcaaactaaattcacttaaaaattaaaaagcagaattgaatattttaagcagcctcagtacctttggccaatgctgttttcatggtggattatgaacattatataatctttgggaaaagtgaaagtagtacaatttttagaataatgacaactgcctcactgcatctctccactcacacagcaaccgtgtagccccctaagctgcagtaccatgactaaccatgatgtcaatttcatatgctgatcctcacaacagcagtgcacaaacatgccccaaatattttaacagaatttagctcttccttaagctgtcttttcatagtaaaaacaaaacaaaaacacccaatgttaaaaccacataataaacttacaaacttgaaaaattagacacttcagatagataggcaataaaacttcatattatgaaagcaatatattccaagtttcaaagatttgacaagttctgtagagtatctttcatcagtacatgaaaacttccaaactgcatgatcttctgccaggcaggactgggtgctattcgctggtttgaggtcgaatccatttcaaggcatgtcgtggtgggacattaatggtgggatggtagaatgtgcagtccggtcttgtacattgagtgttaaacctacaatgttttggatgatagaagggacattccatcttcttacaagcagggaagtaacggcagagctgactactggaaggtggtgctggtggtgcaactggttttggagacagtactggaattcttctactcacatgagtgaagggacaatctggtttagtacactttgcatcatatttacaatttgggtgaacaaacaaacatttttcagcaaatttacaattggggaaggctttgcagggtgagatggggtgatggtaggcacactcatccccatttttacaagcaggccagtacttgcagcgctccaaaagtttttctggtttctgtgccacactcagttcactcatctcagcgttagaaaagctaccatttgggtcctcaagctgcctgctcagcaagtgcaactgctgtgggtggaggagacctctgagtcccttgtttgaggctgcagtttggtttacgggtttcattccttcaaagcacatgtcctcctcttgatctgacatgtatcctggggggctggggacaccatccagcgtcactataaacttgggacttgcaggtttatctggttgtacaagatctcgtgtctgcataaggtgtcctgaaagtacccgaagggaatctgcagtcttcatccccgactcttggtttggtgccactactacttcctcagacagctttggcttcttcagaataaatgatcttgtgtctgcatggaccatggattccatgtcatagtaatcttgactcatctgcagagtttctgccattactgggtcgatttgcagtcgggataataattgcctctgttgagttccttgatttttttctacagaatctccttttgtttcctcttctttaatggggggacttattctgggggtcctactttgtccctggaccacttctgctagcaattcttcttgagaagttcgagttctgggagcaactggaagtgtctgtttctgtggaactgtagagtagttagttgtttttgttacggattcttgagcttcagatatagccttcaaaatcagattcttgttagcttgtttagaaggtggaagagaaggtctcctttcaggctttgcaggcacagacacactgctggagatgcttcctgttcgagacccgtaatcatcatcttcttcctcctcttctccatcatgattgaatttttttactttaacaactgaacttaccacaggcaactttctcttccgaaagttttcatcctccatactcattttctccgagttgtttctaaagaacggactatacgtttcttctaagctgttaagcacctctggttcacacaaacgtcctgtttcatatacccaactactctgcatatcaagctgcttggcagcatgaatactattctgctgctgttgaaattgcaacctgtttaaatgaacaccactatctgcatttctacttgcaggtggtcgataaatttcaatagaagggcgagaagaaccatatgtaagtgtcactgtaggttttttctgagataagggattctcctgcacaaagttgaggtcttcgtcaatgagatcatctggttctggcttaatatcaatcacatcttcagagggtgctggctccctcaaaggtttcactgttgacattagtcgggttgcagctccatcatcgtaagtctgtctgacatttgtggtttttgactcctgcgaacttgtagaaactctggaatctcttttttcaggtctcgcgctaggaatggcaagtggtggcactgcagcttcatgcctcctctcatctccccgactgaaattgctcttgtttgaaggcacgttactatcaaagatgttggtatcagaagacttcagactagagggttcagttgtaacagagcgaagtttatctaatacaccatgaagccatacggtgaatcgaattgtgttgttccctagaaacagggacagatcctctgtcatttggtcctgacttttcttgttggccaccatcaccataatgtaatcaggaagttcttcatctatttaaaaggaaaggtagatcaaaactttgtttcctcaaaactttcttcttaaagttgatgtgcttgaaaatatagatgtagctctaagctttagagtcgcagagctctactggaattacattggacaagatggcttagctttaatttttttctcttcattccacaggtatttcaaatacaacataagctcctaattcttgtaatttccccttaatggcactccggatcttgcggctgatctcggtgccgatctccatggctctgcggcgtgcgggaactcagcactgcgcggcgcttggcttacccggaggctgccgcggactcctaccccgcagccgggacaccaccgcctcc

SEQ ID NO: 17251 - RNA, 14741 nt, Homo sapiens
  source 1..14741: mol_type = other RNA
tcaggccaggcacagtggctcacacctgtaatcttatcactttgggaggctgaggcaggtggatcgcttgagcccaggagttcaagaccagcctgggcaacatggtgaaaccccatcgctataaaaaacaacaattagccgggtgtggtggcacatgcctgtagtccctgctactcaggaggctgaggtgggaggatcacttgagcctggggaggtcaaggctttagtgagctgtgatggtgccactgcactccagcctgggtgacagagtgagaccccatttaaaaaacaaaaacaaaaacaaaaaaaaatgtgacatatagttgactaagaagtacatttcaatacaggattgaaagaacccacatatgttaattaaacacaagcgcagaatttgtgccttttacataaaggaagaatgcacataggcatgctttcagacaagcaattcatctagcagaaaaggaaggaatacatttttcagcccttccaggaataaaatccataaatgggctctatttcgtcctccaacacttgtatttcccacgtcatttactcctgcacacccccactcactagaagcctgctaaactgttccagtgagatattttaacacctgatagggaataaatatgcttctgttttggccttcaaaaataagctctgggccagttgcagtggctcacgcctgtaatcccaacactttgggaggccgaggtgggcggatcacgaggtcaggagtttgggatcagcctggccaatatggtgaaactccatctctactaaaaatacaaaaattagccaggcatggtgcctgtaatcccagctacttgggaggctgaaggagaagaatcgcttgaacctgggaggcacaggttgcagtgagccgagatcacaccactgcactccaggccaggtgacagagcgacactctgtctcaaaaaaataaataaatcaactctgtagcatagcatttgtaattctattattttgccttacatttccattatccttttaataaaattgtttttttacatcttcctaatcaagaagtattatgaggccaggcacagtggctcatacctggaatcccagcactttgggaggccgaggcaggcagatcacctgaggtcaaggtatttgagaccagcctggccaacatggtgaaaccccatctctactaaaaatacagaaattagctgggtgtggtggtgcacacctgtaatgctagctactcgggaggctgaggtaggagaatcgcttgaacctgggaggcagaggttgcaataagcctagatcatgccactgcactcaagcctgggagacagagcgagactacatcttaaaaaaaaaaaaaaaagtattatgagagaggataatgtattgtaatgtattgtagaggctaaataaaattatgctcatgtcagaaaaaaagagtatttctcaaaataaaattcactgaaactggatgtttattttgactgagatatagtatatcctcaaattgccatagaaagtttacaagaatattagaggtaaattataaatatcagggcctttttaaaaaaaaaagattctgcttataacttggtatttgtttataataaaaattatagtagccaataatgaacacttactctggcttggttatttacttaggtcaaaagaaggaggagcggttaaactgtgggatcaggaactgaggcggtgccgtgccttcaggcttgagacaggacaagccacagattgtgttcgttctgtgtgcagaggcaaagtaagatgttccatgagctgatacagtgcagcagaaaacagaaagtggttattactgtgattccctcaccctttgcagcctaatgaacaatacttaataatgcataacgatggatttgcttgccaacattactctgtctttgctgctttctttgccaaagttagcaccagtgtggtgcataagctaggaagctattctgtctaaatactgtatgtaaacctccaatattttctagaatctgccaatttaacaactctagtagacataattgaaagcccttggcagttgactcatattaggacagctgtctccattttttaaaaaaacacacattccctagataaaacgtgcagtaaacaaacaatgaaatactactcagccataaaaaataatgaaattctgtcattcttggtggcaacatggatgagactggaggacatgatgtgaagtgaaataagccaggcacagaaagataaatacatgttctcactcctgtgcagaaactaaaaaagttgatcccacagaggtggagagtagaatagtggttactggaggcggacaagggggagggggagggggatagggaaggactggttaaaggatacaagtttacacagccagataggaatagtatgttttagtattctgtagtactgtaggatgactatagttaagaatcacgtatttatgtattttcaggtatttacaagagaggattttgaaagtttccatcacaaagaaatgataaatgtctgaggtgatggttatgcgtattaccctatgccctatagatatgtataattatgtgtcaatttcaaaataaaaattcaaaactacaactcctatgaaaatttttgagcgtgtttgtacttattaagtgtatttataaatcatacggatattatcttcagcctgcatattaaattgtagttaagcttttactttttaactaaaaaataaattctattattttttcctatatcccactgcactgaccccagtttggaaatcctaagattatcaaataaaaactttgattattgaagaatccaggtgtactgccacagaaaagttctattctgtagcatggactctaatatgtaatctagcccattgtgcttacagatagatgtgtgcctgtagtcatagaaaaatttgcatgagctaatgactgccttgctactagattagctcaaagcaaaaagttctctgaaagcaggtcaatagggtcatttttatattatgaagaagaaaagcagctgttgtattacattcactgtattggtcctgcttgtgtttcagggcaagatccttgttgggacaaggaatgctgaaataatcgaagttggagagaaaaatgcagcttgtaatattttagttaacggtcatgtggatgggccaatctggggactagcaacacatccttccagggattttttcctttctgctgcagaagatgggacagtgagactttgggatattgctgataaagtaagtacagataatttttttaaaagaggttacaacttctaaaaagaaaagttggaagttctaaattgctagtacttaaagaactgccagaattctgttgagcattttgaggggaaactggtataatttagaagtacttcacttaatgtttcctatgactctttttttttttttttttaaatgcagaagatgttaaacaaagtgaatttgggacatgctgctcgtactgtgtgttacagccctgaaggggacatggtggctattggaatgaaaaatggagaatttatcattttactagtgagttctctaaaaatatggggaaagaagagagacaggagatgtgcaatccatgatatcaggttagtgaacaaatggaatagagtttctagtatatacttgatttaacttccatttgtaaaattttccatagccttgccttcaaaaagaggtccccagggcctgtagcatttcccgtattataaattgtatgctaaaatatggctgtttgtatactacttaattcttcttgctaaattataaacccactgggcaccaactataatagcaagtactagtaggtaatgtttgatgaattcatgttaacacttagccatgtccattaagttcatcccaccaagaggtatctcccactgtaatacaagagagctatctgcccttcaaaagttgtcaccctggaaaactaaagttgtgatttcaaacatatcttctcttagtaacctcagtttgggaatatgtagttcattaatttaatcaatacctattgattaaatgttccagaatccaaattaatttaaatgtttcttaaacctttgtttttcagtgcttaagcatttttcaacagtggctaccatttacggagtacttccgtgtgatcagtagataagattattgaatctaggtctgtcaaaagcttgtacacttttcatcagtaaaatccttttacaaatgaaaccttcctcagaacttcaatatataaaatagtaacagtggcttcccttagcttttacatgtctctatcgtacctcagtaagactcatgggccatttcaagagactgaattgtcccatatgactccaaagattgctaggcaaatagcatttcactttgtcttttaaataagttcttcaggccgggcgcggtggctcatgcctgtaatcccagcactttgggaggccgaggcaggcagatcacctgaagtcaggagtactcgaccagcctggccaacatagtgaaaccccatctcaactaaaaatacaaaaatcagccgggcgtggtggcaggcgcctgtaatcccagctactcagggggctgaaacaggagaatcgcttgaacccgggaggcggaggttgcgccatcgcactccagcctgggagacaagagcgagacttcgtctcaaaaaaaaaaaattcttcttccaagattcaagttgtgtcatttcaccttaataactggaggttagttaagctgggctgtgttctttgcttaatattaagacaacgttttttccagatggaagaaaactatcttaatgaattgttagcttattaattatgtaatgctaatggcttttaaaagctgagatgttctgactgggtgttgtggctcacacctgtaatcccagtaccttgggaggccaagggggaaggattgcttgaggccaggagtttgggaccatagtgagaccccgcctctatttaaaaaattaaattttgttttgttttgttttgagttggagttttgctcttgttgcccatgctgaagtgcaatggtgcaatctcagctcaccacaacctgtgcctcctgggttcaagcgattctcctgcttcagcctcccgagtagatgggattacaggcgtgcaccaccatgcctggctaattttgtatttttagtagagacagggtttctctatgttggtcaggctggtctcaaactctcgacctcaggtgatctgcccgcctccgcttcccaaagttctgggattataggtgtgagccactgggcctggcctaagaaagtttttttaagccattagacgtttttaaaggaattgggagatgacaattggggaaatatttaaaatttaagtaaaatataaagcttccttatttcatgtaacccagacaatctcagtatacatgatcagttgtgtctgacaggtaaatctatttgaggccttatcacacgttacttttaagaactagaaaggaaaagtcactgatcttaagtatttataatacttcatgtggtctaatactttttacgttttgttttgattcagatttagtccggattcccggtatctggcagtaggttctagtgagaactcagtggatttttatgacctaacgctgggccccactcttaacagaatcagctactgcaaagacattccaagctttgtcattcaaatggacttctctgcagatagcagttatctccaggtacagtaccaatactgtatacccaggtggcaagttcttctgcttttacatttcgtgttagtgaatgcatttaaagttcctgagctccagagctccagcttctcaactcctccctttgtaccttctgacctacagctcccctttcctcccccacttatcagagcttttctcctattaagtttttgtagtgatcttttgcatacttaataatgttagacatgtaaatcaagtagcaatatgctagtattctgtaaaccccctgtggattttgtctctcacctaatggaattcttgtcccattttaatctgatgaaaaaggtctctagtggctgctataaacggcatgtctatgaagtgccttcaggaaaacatcttatggatcatgccgctattgacagaattacttgggctacatggactaggtaaatacttatatattcacaaggcaagaactgactttgaaggccagttagaaaatcctatttctgaactgttagagccattccaataaggaatagtaattgagtttcaagtttttgttaccatattttgaaatggtatgttcatgttgggacccctttttattgaatatatttccatgttttatcagtttccatgatttatcaagttttttttttaaggaaatcaaagttttaactttaaagataccctgatatttttcttaatgctaaatttaatgactggcaaaaaggtattgggtgctgttaagcaactgttattaattctctatctaaaggaatgctatcttgaatctattagaagtcaaagcttccaaatttgttcaaatttcctggctgtatgacaggtaaccatgactatccatttttttggccaatgaaaaatgccatcaaattcctgtatcagccaggcatatagtggctcatgcctgtaatctctgatgtagcaggccgaggtgggaggatcacttgagcctagaagttttgataccagcctgggcaacatagcaagaccccatctctgaaatttttttaattcctatgtcataagtcatttttatttttgtagagatagggatctcacaatattgcccaggctggtctcaaactcttggcctcaagcagtcctcctgcctcagcctcccaaaatgttgggattactggtatgtgctgctggacccagccaagtagcacttttaatttgaaaaatagttctatcagttttcagtcaggcgcggtggctcagcctgtaatcccagcactttgggaggccgagcgggggtgatcacctgaggtcgggagttcgagactagcctgaccaacatggagaaaccctgtctctactaaaaatacaaaataagccgggcatgttagcgcatgcctgtgatcccagctactcgggaggctgaggcaggagaattgcttgaacccaggaggcagaggttgcggtgagccgagatcatgccattgcactccagcctgggtaacaagagcgaaaactccgtctcaaaaaaaaaaaaagaaaaaatagttctatcagttttcataaagtactactttaatcttaaaaagattaatctagaaacccttcaaattataaaatgtcatttttaaaaggcaggagttgatatcctgatgaaattcaggtctccaaacaacttaccataatttacttcctgtattttaagtaacatgatagggtacttagagattaattgccaagaaactttttgaatatagtcaacctgcccgcacttgccatgatgagttttcttttgttccttccctctagtattctaggagatgaggttttgggaatctggtccagacatgctgagaaagctgatgtcaactgtgcctgtgtatctcattcaggaatcagtcttgttacaggagatgactttggcatggttaagttatttgacttcccatgtccagaaaaatttgtaagtttgtgttttgtttactattatcagtttactcctaattttgatgtcttatcatcagcacttttccccatatatttaaaatgttttgtcctaatttctaaatttttccccaaactttctaaatctatttactttgaaataaaagctattagaaacaaatcctctccctcgagtaataccatctttggaaccatcctacaaaagctgtaattagcttttcaccaaacctataatcagttatcaaatttcaaatgcttttccttagagaaaaatggtcagagtacctggagacatctgactgcccacacagcctggttttgcagatccactactcatgctgaaaagcattctaatcactggctgcggtgctaactccctactctctccacagctcttgtcatagagattatagttcctaataagagcctttgacttctgtgtgcaccaaatgccctgagcttgtctgtcattgttttttaggcaaaacacaaaaggttcttgggtcattcgccccatgtgacaaatattcgatttaccagtggtgatcgacatgttgttagtgctggaggtgatgactgcaggttagtaactttctcagcccatgaagagcagactatgttactagttaagagacttaatacaacaactcctacagctttggtttatgaaatcagctagtcaacattagtagaaggtagtataaccagatggctcttcagaatctcatatttatgcaaatacagaataaaaggagttaaagaggaaaaatattacacatgtaacctgaaagcacaactgaaaaatattaaactgttatgaaaatctaaaaacataattaactccctgcaattttcttctctgattgcagcttatttgtctggaaatgtgtacatacacctcactgagagatgctgagatgactacagaaattaactttgagaccagaattacagagaagaaaaaccaaaacccaaccctgcatggtcaagtggtgctaacccaagactgtaacagggagaaatgcccagaatcatcaaaatagtgaaagactgatctgttcaaaatatttgctatatgcactgggtataatccgtaatccatacactgccagataatgccatttcaaggaaggatcgaatacttgatggtaaaggccaagtccccctgtattgggaagtgtgtgatttcggcagacctgctgggaaaatttagggtagagcactctttacagaagaactcaaaaacccaatttggataattttcattatctttttagcaaaatggtttcttaatgtttatattttattttcaaggttcattgtttaatgaaatattttattcttgcatttccataaggaaagggaaagtcatgatcatcctaaaggatcacagtttttaaaaggcaaacattttccctaaggaaacagacacaagctttcctagagaatatgatgttttttaggcattaataaggtccttttttataaaggacacttttctcctagtagttttgaattcaggaacagatccaaagttagcagtatatggctgctacatttccattttcattttcgagccatcagtttatgttcagatgccatctctgtaatcgcacatttaaaacataactgtagcctcactaatggaaaagtagtatgatgaacaatcattcccaatggtgtacaatgtaagggttttagggagcaacagtatttaactggaagaaagaattgcatatttaatgtagtctaatatatacacatttgtttaacatgtaaacaaaagtgttaaattcacatatacaacattatacaatttaatcactcttggaataaaatttttatagccttttttctattgggaaaatttgtttagatgtgtgccactccataggtttatttccaaaatgaatgagcccaactccatttgtaaaaacttgtcagttagaattcctttttttagtggattagggctgaattcttagatccttatttcttttcactttaaatgctgccaaagatcactactcatcattcaggaattcgctgtctagcctatctgtagtttcctgaagattgaaaattatgtagactgctatttaaaaatatatttttctaagtgtgaggtttaagatgctgtattgaccctatgagtttttaatgtgttaattatctttatagcataatagatcgctttaggttcctggaatcccatttggtctgacaggatatatgaagattcttaatacctattttctgtgtctaatacttggttaatactaaaaatagaaatgactaaattacatcacagaaagcataaccagtgattgaacctggtagttttaaagctctaaatagctgtggctgaaggactgattatggggctaagaagcttgaaacgtaagttggtacttgttcatcagtggattctcctaaattaagccaaattttgaaatacatgactattaagtttctactcatgtatttacagtcagtcaataaattaaaggaggaaaaaaatccctgaacaacctgcccataaaaagaaaaatactctacatttgagcctgctgcagttttaaattttccctctgggtcaagtttgccagcttttggctacagagaaattatatttccattacagtgcaggtagaaactctgtaaccttaagcatgtaaactacatagaataaaactgtttccactgcatttctgtccttcaaagtggccaacctgattaagtcagccttaatcactgctgctgtcagtttcacgactaaaggtcatattgactaagtagtcatcagctgaccacctcgctgtatcagccagcaacgaggggaaggtgaagaaacatgataggccatatagaatctgccctatgtttacttttttaacccagataattatttttgtgtgcagtatctaagctcctgattgtgtaacctgggacttctggcaccttttgttccattcattttatgtataaaatgcatgccaaagcacactgtgccctctggtacccttgcttccaatcgccaaccatgctcatttccttcctttttttgtggtccctttttgtggtgatcattttaaaccacgtcatccaacaaatgttttatggtcaaccttagcttgttcataagccatagcaactgaaagattaaactcttaaatatgtgtctgggcagtggctattaaatagcaaaaaacaatcagattttagtattttattatttccttgtaaaatggctgaactaaattaaacccttgtttcccatttgttctataatttatagtgaaactgagaacaaaactatctttataaatgatagctaaaagtatttccagatatttaaacaatttaaaataaatttcttctgcagagatgcaaagcatctcaacactggaatgaacaaatgccttaaattcaatggagtaaacctttagaatgaagaggaactgtcatttcacccaagccgaagacaacagccttatgcacttgtgtgctctgtctttgctgcttctcgtgtttcaagcctttcctgtgggatcagcacagcaaagtgcaacttaccaaatggtttaatgactggttaattctttcttctcccaatggaaaagcaatggcaacacaacagtagactgctggcttgacaatcttaaacgtgagcctttgcacatgtaggtttatcatcatttgagtatacgactaagcaagtcaatgaactttttttttttttttagcagtttaatttggtcctgagaatgttgcagtctttattaccccttttgcattaatccacttttctaaccaccttttaagctttaatttttaacactatacaccaagtctttgaaatcagtgatctgttatttaactctaaagcatttgacacttcttgccttaacagttttaaaaaccacacacaaaaaaactctgtaagtaatacagtaggccaaaagtttcatcctatctatcttgcagtttacctatctgatctgatctctgtaattatagttctgtcatttaaaatatactatttaaatctaatttttacatttcaaaaattatcttcagtagtaactaagtatattttctgtggattctgagaatgttatttttcagaatgtgagaatatatatgtacatttataatcttgtgactttaaagtctgttttcagatacagtatgtaaatacttgtaaaaaaatttgtataattttgtgataatgtagtttcccaaaaaaattatttagaaggcattatgttattagtaaatgagagcactgtatagaactgttcctattttctgcacttgccattccagctgcctccactgtccatacccacctcattcatcctgtcacagaaggcaggaaaactgggaactttaccaaagtagcactcagcctgagaggcctgtataatcatgcttttcaaactaaattcacttaaaaattaaaaagcagaattgaatattttaagcagcctcagtacctttggccaatgctgttttcatggtggattatgaacattatataatctttgggaaaagtgaaagtagtacaatttttagaataatgacaactgcctcactgcatctctccactcacacagcaaccgtgtagccccctaagctgcagtaccatgactaaccatgatgtcaatttcatatgctgatcctcacaacagcagtgcacaaacatgccccaaatattttaacagaatttagctcttccttaagctgtcttttcatagtaaaaacaaaacaaaaacacccaatgttaaaaccacataataaacttacaaacttgaaaaattagacacttcagatagataggcaataaaacttcatattatgaaagcaatatattccaagtttcaaagatttgacaagttctgtagagtatctttcatcagtacatgaaaacttccaaactgcatgatcttctgccaggcaggactgggtgctattcgctggtttgaggtcgaatccatttcaaggcatgtcgtggtgggacattaatggtgggatggtagaatgtgcagtccggtcttgtacattgagtgttaaacctacaatgttttggatgatagaagggacattccatcttcttacaagcagggaagtaacggcagagctgactactggaaggtggtgctggtggtgcaactggttttggagacagtactggaattcttctactcacatgagtgaagggacaatctggtttagtacactttgcatcatatttacaatttgggtgaacaaacaaacatttttcagcaaatttacaattggggaaggctttgcagggtgagatggggtgatggtaggcacactcatccccatttttacaagcaggccagtacttgcagcgctccaaaagtttttctggtttctgtgccacactcagttcactcatctcagcgttagaaaagctaccatttgggtcctcaagctgcctgctcagcaagtgcaactgctgtgggtggaggagacctctgagtcccttgtttgaggctgcagtttggtttacgggtttcattccttcaaagcacatgtcctcctcttgatctgacatgtatcctggggggctggggacaccatccagcgtcactataaacttgggacttgcaggtttatctggttgtacaagatctcgtgtctgcataaggtgtcctgaaagtacccgaagggaatctgcagtcttcatccccgactcttggtttggtgccactactacttcctcagacagctttggcttcttcagaataaatgatcttgtgtctgcatggaccatggattccatgtcatagtaatcttgatttttttctacagaatctccttttgtttcctcttctttaatggggggacttattctgggggtcctactttgtccctggaccacttctgctagcaattcttcttgagaagttcgagttctgggagcaactggaagtgtctgtttctgtggaactgtagagtagttagttgtttttgttacggattcttgagcttcagatatagccttcaaaatcagattcttgttagcttgtttagaaggtggaagagaaggtctcctttcaggctttgcaggcacagacacactgctggagatgcttcctgttcgagacccgtaatcatcatcttcttcctcctcttctccatcatgattgaatttttttactttaacaactgaacttaccacaggcaactttctcttccgaaagttttcatcctccatactcattttctccgagttgtttctaaagaacggactatacgtttcttctaagctgttaagcacctctggttcacacaaacgtcctgtttcatatacccaactactctgcatatcaagctgcttggcagcatgaatactattctgctgctgttgaaattgcaacctgtttaaatgaacaccactatctgcatttctacttgcaggtggtcgataaatttcaatagaagggcgagaagaaccatatgtaagtgtcactgtaggttttttctgagataagggattctcctgcacaaagttgaggtcttcgtcaatgagatcatctggttctggcttaatatcaatcacatcttcagagggtgctggctccctcaaaggtttcactgttgacattagtcgggttgcagctccatcatcgtaagtctgtctgacatttgtggtttttgactcctgcgaacttgtagaaactctggaatctcttttttcaggtctcgcgctaggaatggcaagtggtggcactgcagcttcatgcctcctctcatctccccgactgaaattgctcttgtttgaaggcacgttactatcaaagatgttggtatcagaagacttcagactagagggttcagttgtaacagagcgaagtttatctaatacaccatgaagccaacataagctcctaattcttgtaatttccccttaatggcactccggatcttgcggctgatctcggtgccgatctccatggctctgcggcgtgcgggaactcagcactgcgcggcgcttggcttacccggaggctgccgcggactcctaccccgcagccgggacaccaccgcctcc

SEQ ID NO: 17252 - RNA, 14856 nt, Homo sapiens
  source 1..14856: mol_type = other RNA
tcaggccaggcacagtggctcacacctgtaatcttatcactttgggaggctgaggcaggtggatcgcttgagcccaggagttcaagaccagcctgggcaacatggtgaaaccccatcgctataaaaaacaacaattagccgggtgtggtggcacatgcctgtagtccctgctactcaggaggctgaggtgggaggatcacttgagcctggggaggtcaaggctttagtgagctgtgatggtgccactgcactccagcctgggtgacagagtgagaccccatttaaaaaacaaaaacaaaaacaaaaaaaaatgtgacatatagttgactaagaagtacatttcaatacaggattgaaagaacccacatatgttaattaaacacaagcgcagaatttgtgccttttacataaaggaagaatgcacataggcatgctttcagacaagcaattcatctagcagaaaaggaaggaatacatttttcagcccttccaggaataaaatccataaatgggctctatttcgtcctccaacacttgtatttcccacgtcatttactcctgcacacccccactcactagaagcctgctaaactgttccagtgagatattttaacacctgatagggaataaatatgcttctgttttggccttcaaaaataagctctgggccagttgcagtggctcacgcctgtaatcccaacactttgggaggccgaggtgggcggatcacgaggtcaggagtttgggatcagcctggccaatatggtgaaactccatctctactaaaaatacaaaaattagccaggcatggtgcctgtaatcccagctacttgggaggctgaaggagaagaatcgcttgaacctgggaggcacaggttgcagtgagccgagatcacaccactgcactccaggccaggtgacagagcgacactctgtctcaaaaaaataaataaatcaactctgtagcatagcatttgtaattctattattttgccttacatttccattatccttttaataaaattgtttttttacatcttcctaatcaagaagtattatgaggccaggcacagtggctcatacctggaatcccagcactttgggaggccgaggcaggcagatcacctgaggtcaaggtatttgagaccagcctggccaacatggtgaaaccccatctctactaaaaatacagaaattagctgggtgtggtggtgcacacctgtaatgctagctactcgggaggctgaggtaggagaatcgcttgaacctgggaggcagaggttgcaataagcctagatcatgccactgcactcaagcctgggagacagagcgagactacatcttaaaaaaaaaaaaaaaagtattatgagagaggataatgtattgtaatgtattgtagaggctaaataaaattatgctcatgtcagaaaaaaagagtatttctcaaaataaaattcactgaaactggatgtttattttgactgagatatagtatatcctcaaattgccatagaaagtttacaagaatattagaggtaaattataaatatcagggcctttttaaaaaaaaaagattctgcttataacttggtatttgtttataataaaaattatagtagccaataatgaacacttactctggcttggttatttacttaggtcaaaagaaggaggagcggttaaactgtgggatcaggaactgaggcggtgccgtgccttcaggcttgagacaggacaagccacagattgtgttcgttctgtgtgcagaggcaaagtaagatgttccatgagctgatacagtgcagcagaaaacagaaagtggttattactgtgattccctcaccctttgcagcctaatgaacaatacttaataatgcataacgatggatttgcttgccaacattactctgtctttgctgctttctttgccaaagttagcaccagtgtggtgcataagctaggaagctattctgtctaaatactgtatgtaaacctccaatattttctagaatctgccaatttaacaactctagtagacataattgaaagcccttggcagttgactcatattaggacagctgtctccattttttaaaaaaacacacattccctagataaaacgtgcagtaaacaaacaatgaaatactactcagccataaaaaataatgaaattctgtcattcttggtggcaacatggatgagactggaggacatgatgtgaagtgaaataagccaggcacagaaagataaatacatgttctcactcctgtgcagaaactaaaaaagttgatcccacagaggtggagagtagaatagtggttactggaggcggacaagggggagggggagggggatagggaaggactggttaaaggatacaagtttacacagccagataggaatagtatgttttagtattctgtagtactgtaggatgactatagttaagaatcacgtatttatgtattttcaggtatttacaagagaggattttgaaagtttccatcacaaagaaatgataaatgtctgaggtgatggttatgcgtattaccctatgccctatagatatgtataattatgtgtcaatttcaaaataaaaattcaaaactacaactcctatgaaaatttttgagcgtgtttgtacttattaagtgtatttataaatcatacggatattatcttcagcctgcatattaaattgtagttaagcttttactttttaactaaaaaataaattctattattttttcctatatcccactgcactgaccccagtttggaaatcctaagattatcaaataaaaactttgattattgaagaatccaggtgtactgccacagaaaagttctattctgtagcatggactctaatatgtaatctagcccattgtgcttacagatagatgtgtgcctgtagtcatagaaaaatttgcatgagctaatgactgccttgctactagattagctcaaagcaaaaagttctctgaaagcaggtcaatagggtcatttttatattatgaagaagaaaagcagctgttgtattacattcactgtattggtcctgcttgtgtttcagggcaagatccttgttgggacaaggaatgctgaaataatcgaagttggagagaaaaatgcagcttgtaatattttagttaacggtcatgtggatgggccaatctggggactagcaacacatccttccagggattttttcctttctgctgcagaagatgggacagtgagactttgggatattgctgataaagtaagtacagataatttttttaaaagaggttacaacttctaaaaagaaaagttggaagttctaaattgctagtacttaaagaactgccagaattctgttgagcattttgaggggaaactggtataatttagaagtacttcacttaatgtttcctatgactctttttttttttttttttaaatgcagaagatgttaaacaaagtgaatttgggacatgctgctcgtactgtgtgttacagccctgaaggggacatggtggctattggaatgaaaaatggagaatttatcattttactagtgagttctctaaaaatatggggaaagaagagagacaggagatgtgcaatccatgatatcaggttagtgaacaaatggaatagagtttctagtatatacttgatttaacttccatttgtaaaattttccatagccttgccttcaaaaagaggtccccagggcctgtagcatttcccgtattataaattgtatgctaaaatatggctgtttgtatactacttaattcttcttgctaaattataaacccactgggcaccaactataatagcaagtactagtaggtaatgtttgatgaattcatgttaacacttagccatgtccattaagttcatcccaccaagaggtatctcccactgtaatacaagagagctatctgcccttcaaaagttgtcaccctggaaaactaaagttgtgatttcaaacatatcttctcttagtaacctcagtttgggaatatgtagttcattaatttaatcaatacctattgattaaatgttccagaatccaaattaatttaaatgtttcttaaacctttgtttttcagtgcttaagcatttttcaacagtggctaccatttacggagtacttccgtgtgatcagtagataagattattgaatctaggtctgtcaaaagcttgtacacttttcatcagtaaaatccttttacaaatgaaaccttcctcagaacttcaatatataaaatagtaacagtggcttcccttagcttttacatgtctctatcgtacctcagtaagactcatgggccatttcaagagactgaattgtcccatatgactccaaagattgctaggcaaatagcatttcactttgtcttttaaataagttcttcaggccgggcgcggtggctcatgcctgtaatcccagcactttgggaggccgaggcaggcagatcacctgaagtcaggagtactcgaccagcctggccaacatagtgaaaccccatctcaactaaaaatacaaaaatcagccgggcgtggtggcaggcgcctgtaatcccagctactcagggggctgaaacaggagaatcgcttgaacccgggaggcggaggttgcgccatcgcactccagcctgggagacaagagcgagacttcgtctcaaaaaaaaaaaattcttcttccaagattcaagttgtgtcatttcaccttaataactggaggttagttaagctgggctgtgttctttgcttaatattaagacaacgttttttccagatggaagaaaactatcttaatgaattgttagcttattaattatgtaatgctaatggcttttaaaagctgagatgttctgactgggtgttgtggctcacacctgtaatcccagtaccttgggaggccaagggggaaggattgcttgaggccaggagtttgggaccatagtgagaccccgcctctatttaaaaaattaaattttgttttgttttgttttgagttggagttttgctcttgttgcccatgctgaagtgcaatggtgcaatctcagctcaccacaacctgtgcctcctgggttcaagcgattctcctgcttcagcctcccgagtagatgggattacaggcgtgcaccaccatgcctggctaattttgtatttttagtagagacagggtttctctatgttggtcaggctggtctcaaactctcgacctcaggtgatctgcccgcctccgcttcccaaagttctgggattataggtgtgagccactgggcctggcctaagaaagtttttttaagccattagacgtttttaaaggaattgggagatgacaattggggaaatatttaaaatttaagtaaaatataaagcttccttatttcatgtaacccagacaatctcagtatacatgatcagttgtgtctgacaggtaaatctatttgaggccttatcacacgttacttttaagaactagaaaggaaaagtcactgatcttaagtatttataatacttcatgtggtctaatactttttacgttttgttttgattcagatttagtccggattcccggtatctggcagtaggttctagtgagaactcagtggatttttatgacctaacgctgggccccactcttaacagaatcagctactgcaaagacattccaagctttgtcattcaaatggacttctctgcagatagcagttatctccaggtacagtaccaatactgtatacccaggtggcaagttcttctgcttttacatttcgtgttagtgaatgcatttaaagttcctgagctccagagctccagcttctcaactcctccctttgtaccttctgacctacagctcccctttcctcccccacttatcagagcttttctcctattaagtttttgtagtgatcttttgcatacttaataatgttagacatgtaaatcaagtagcaatatgctagtattctgtaaaccccctgtggattttgtctctcacctaatggaattcttgtcccattttaatctgatgaaaaaggtctctagtggctgctataaacggcatgtctatgaagtgccttcaggaaaacatcttatggatcatgccgctattgacagaattacttgggctacatggactaggtaaatacttatatattcacaaggcaagaactgactttgaaggccagttagaaaatcctatttctgaactgttagagccattccaataaggaatagtaattgagtttcaagtttttgttaccatattttgaaatggtatgttcatgttgggacccctttttattgaatatatttccatgttttatcagtttccatgatttatcaagttttttttttaaggaaatcaaagttttaactttaaagataccctgatatttttcttaatgctaaatttaatgactggcaaaaaggtattgggtgctgttaagcaactgttattaattctctatctaaaggaatgctatcttgaatctattagaagtcaaagcttccaaatttgttcaaatttcctggctgtatgacaggtaaccatgactatccatttttttggccaatgaaaaatgccatcaaattcctgtatcagccaggcatatagtggctcatgcctgtaatctctgatgtagcaggccgaggtgggaggatcacttgagcctagaagttttgataccagcctgggcaacatagcaagaccccatctctgaaatttttttaattcctatgtcataagtcatttttatttttgtagagatagggatctcacaatattgcccaggctggtctcaaactcttggcctcaagcagtcctcctgcctcagcctcccaaaatgttgggattactggtatgtgctgctggacccagccaagtagcacttttaatttgaaaaatagttctatcagttttcagtcaggcgcggtggctcagcctgtaatcccagcactttgggaggccgagcgggggtgatcacctgaggtcgggagttcgagactagcctgaccaacatggagaaaccctgtctctactaaaaatacaaaataagccgggcatgttagcgcatgcctgtgatcccagctactcgggaggctgaggcaggagaattgcttgaacccaggaggcagaggttgcggtgagccgagatcatgccattgcactccagcctgggtaacaagagcgaaaactccgtctcaaaaaaaaaaaaagaaaaaatagttctatcagttttcataaagtactactttaatcttaaaaagattaatctagaaacccttcaaattataaaatgtcatttttaaaaggcaggagttgatatcctgatgaaattcaggtctccaaacaacttaccataatttacttcctgtattttaagtaacatgatagggtacttagagattaattgccaagaaactttttgaatatagtcaacctgcccgcacttgccatgatgagttttcttttgttccttccctctagtattctaggagatgaggttttgggaatctggtccagacatgctgagaaagctgatgtcaactgtgcctgtgtatctcattcaggaatcagtcttgttacaggagatgactttggcatggttaagttatttgacttcccatgtccagaaaaatttgtaagtttgtgttttgtttactattatcagtttactcctaattttgatgtcttatcatcagcacttttccccatatatttaaaatgttttgtcctaatttctaaatttttccccaaactttctaaatctatttactttgaaataaaagctattagaaacaaatcctctccctcgagtaataccatctttggaaccatcctacaaaagctgtaattagcttttcaccaaacctataatcagttatcaaatttcaaatgcttttccttagagaaaaatggtcagagtacctggagacatctgactgcccacacagcctggttttgcagatccactactcatgctgaaaagcattctaatcactggctgcggtgctaactccctactctctccacagctcttgtcatagagattatagttcctaataagagcctttgacttctgtgtgcaccaaatgccctgagcttgtctgtcattgttttttaggcaaaacacaaaaggttcttgggtcattcgccccatgtgacaaatattcgatttaccagtggtgatcgacatgttgttagtgctggaggtgatgactgcaggttagtaactttctcagcccatgaagagcagactatgttactagttaagagacttaatacaacaactcctacagctttggtttatgaaatcagctagtcaacattagtagaaggtagtataaccagatggctcttcagaatctcatatttatgcaaatacagaataaaaggagttaaagaggaaaaatattacacatgtaacctgaaagcacaactgaaaaatattaaactgttatgaaaatctaaaaacataattaactccctgcaattttcttctctgattgcagcttatttgtctggaaatgtgtacatacacctcactgagagatgctgagatgactacagaaattaactttgagaccagaattacagagaagaaaaaccaaaacccaaccctgcatggtcaagtggtgctaacccaagactgtaacagggagaaatgcccagaatcatcaaaatagtgaaagactgatctgttcaaaatatttgctatatgcactgggtataatccgtaatccatacactgccagataatgccatttcaaggaaggatcgaatacttgatggtaaaggccaagtccccctgtattgggaagtgtgtgatttcggcagacctgctgggaaaatttagggtagagcactctttacagaagaactcaaaaacccaatttggataattttcattatctttttagcaaaatggtttcttaatgtttatattttattttcaaggttcattgtttaatgaaatattttattcttgcatttccataaggaaagggaaagtcatgatcatcctaaaggatcacagtttttaaaaggcaaacattttccctaaggaaacagacacaagctttcctagagaatatgatgttttttaggcattaataaggtccttttttataaaggacacttttctcctagtagttttgaattcaggaacagatccaaagttagcagtatatggctgctacatttccattttcattttcgagccatcagtttatgttcagatgccatctctgtaatcgcacatttaaaacataactgtagcctcactaatggaaaagtagtatgatgaacaatcattcccaatggtgtacaatgtaagggttttagggagcaacagtatttaactggaagaaagaattgcatatttaatgtagtctaatatatacacatttgtttaacatgtaaacaaaagtgttaaattcacatatacaacattatacaatttaatcactcttggaataaaatttttatagccttttttctattgggaaaatttgtttagatgtgtgccactccataggtttatttccaaaatgaatgagcccaactccatttgtaaaaacttgtcagttagaattcctttttttagtggattagggctgaattcttagatccttatttcttttcactttaaatgctgccaaagatcactactcatcattcaggaattcgctgtctagcctatctgtagtttcctgaagattgaaaattatgtagactgctatttaaaaatatatttttctaagtgtgaggtttaagatgctgtattgaccctatgagtttttaatgtgttaattatctttatagcataatagatcgctttaggttcctggaatcccatttggtctgacaggatatatgaagattcttaatacctattttctgtgtctaatacttggttaatactaaaaatagaaatgactaaattacatcacagaaagcataaccagtgattgaacctggtagttttaaagctctaaatagctgtggctgaaggactgattatggggctaagaagcttgaaacgtaagttggtacttgttcatcagtggattctcctaaattaagccaaattttgaaatacatgactattaagtttctactcatgtatttacagtcagtcaataaattaaaggaggaaaaaaatccctgaacaacctgcccataaaaagaaaaatactctacatttgagcctgctgcagttttaaattttccctctgggtcaagtttgccagcttttggctacagagaaattatatttccattacagtgcaggtagaaactctgtaaccttaagcatgtaaactacatagaataaaactgtttccactgcatttctgtccttcaaagtggccaacctgattaagtcagccttaatcactgctgctgtcagtttcacgactaaaggtcatattgactaagtagtcatcagctgaccacctcgctgtatcagccagcaacgaggggaaggtgaagaaacatgataggccatatagaatctgccctatgtttacttttttaacccagataattatttttgtgtgcagtatctaagctcctgattgtgtaacctgggacttctggcaccttttgttccattcattttatgtataaaatgcatgccaaagcacactgtgccctctggtacccttgcttccaatcgccaaccatgctcatttccttcctttttttgtggtccctttttgtggtgatcattttaaaccacgtcatccaacaaatgttttatggtcaaccttagcttgttcataagccatagcaactgaaagattaaactcttaaatatgtgtctgggcagtggctattaaatagcaaaaaacaatcagattttagtattttattatttccttgtaaaatggctgaactaaattaaacccttgtttcccatttgttctataatttatagtgaaactgagaacaaaactatctttataaatgatagctaaaagtatttccagatatttaaacaatttaaaataaatttcttctgcagagatgcaaagcatctcaacactggaatgaacaaatgccttaaattcaatggagtaaacctttagaatgaagaggaactgtcatttcacccaagccgaagacaacagccttatgcacttgtgtgctctgtctttgctgcttctcgtgtttcaagcctttcctgtgggatcagcacagcaaagtgcaacttaccaaatggtttaatgactggttaattctttcttctcccaatggaaaagcaatggcaacacaacagtagactgctggcttgacaatcttaaacgtgagcctttgcacatgtaggtttatcatcatttgagtatacgactaagcaagtcaatgaactttttttttttttttagcagtttaatttggtcctgagaatgttgcagtctttattaccccttttgcattaatccacttttctaaccaccttttaagctttaatttttaacactatacaccaagtctttgaaatcagtgatctgttatttaactctaaagcatttgacacttcttgccttaacagttttaaaaaccacacacaaaaaaactctgtaagtaatacagtaggccaaaagtttcatcctatctatcttgcagtttacctatctgatctgatctctgtaattatagttctgtcatttaaaatatactatttaaatctaatttttacatttcaaaaattatcttcagtagtaactaagtatattttctgtggattctgagaatgttatttttcagaatgtgagaatatatatgtacatttataatcttgtgactttaaagtctgttttcagatacagtatgtaaatacttgtaaaaaaatttgtataattttgtgataatgtagtttcccaaaaaaattatttagaaggcattatgttattagtaaatgagagcactgtatagaactgttcctattttctgcacttgccattccagctgcctccactgtccatacccacctcattcatcctgtcacagaaggcaggaaaactgggaactttaccaaagtagcactcagcctgagaggcctgtataatcatgcttttcaaactaaattcacttaaaaattaaaaagcagaattgaatattttaagcagcctcagtacctttggccaatgctgttttcatggtggattatgaacattatataatctttgggaaaagtgaaagtagtacaatttttagaataatgacaactgcctcactgcatctctccactcacacagcaaccgtgtagccccctaagctgcagtaccatgactaaccatgatgtcaatttcatatgctgatcctcacaacagcagtgcacaaacatgccccaaatattttaacagaatttagctcttccttaagctgtcttttcatagtaaaaacaaaacaaaaacacccaatgttaaaaccacataataaacttacaaacttgaaaaattagacacttcagatagataggcaataaaacttcatattatgaaagcaatatattccaagtttcaaagatttgacaagttctgtagagtatctttcatcagtacatgaaaacttccaaactgcatgatcttctgccaggcaggactgggtgctattcgctggtttgaggtcgaatccatttcaaggcatgtcgtggtgggacattaatggtgggatggtagaatgtgcagtccggtcttgtacattgagtgttaaacctacaatgttttggatgatagaagggacattccatcttcttacaagcagggaagtaacggcagagctgactactggaaggtggtgctggtggtgcaactggttttggagacagtactggaattcttctactcacatgagtgaagggacaatctggtttagtacactttgcatcatatttacaatttgggtgaacaaacaaacatttttcagcaaatttacaattggggaaggctttgcagggtgagatggggtgatggtaggcacactcatccccatttttacaagcaggccagtacttgcagcgctccaaaagtttttctggtttctgtgccacactcagttcactcatctcagcgttagaaaagctaccatttgggtcctcaagctgcctgctcagcaagtgcaactgctgtgggtggaggagacctctgagtcccttgtttgaggctgcagtttggtttacgggtttcattccttcaaagcacatgtcctcctcttgatctgacatgtatcctggggggctggggacaccatccagcgtcactataaacttgggacttgcaggtttatctggttgtacaagatctcgtgtctgcataaggtgtcctgaaagtacccgaagggaatctgcagtcttcatccccgactcttggtttggtgccactactacttcctcagacagctttggcttcttcagaataaatgatcttgtgtctgcatggaccatggattccatgtcatagtaatcttgatttttttctacagaatctccttttgtttcctcttctttaatggggggacttattctgggggtcctactttgtccctggaccacttctgctagcaattcttcttgagaagttcgagttctgggagcaactggaagtgtctgtttctgtggaactgtagagtagttagttgtttttgttacggattcttgagcttcagatatagccttcaaaatcagattcttgttagcttgtttagaaggtggaagagaaggtctcctttcaggctttgcaggcacagacacactgctggagatgcttcctgttcgagacccgtaatcatcatcttcttcctcctcttctccatcatgattgaatttttttactttaacaactgaacttaccacaggcaactttctcttccgaaagttttcatcctccatactcattttctccgagttgtttctaaagaacggactatacgtttcttctaagctgttaagcacctctggttcacacaaacgtcctgtttcatatacccaactactctgcatatcaagctgcttggcagcatgaatactattctgctgctgttgaaattgcaacctgtttaaatgaacaccactatctgcatttctacttgcaggtggtcgataaatttcaatagaagggcgagaagaaccatatgtaagtgtcactgtaggttttttctgagataagggattctcctgcacaaagttgaggtcttcgtcaatgagatcatctggttctggcttaatatcaatcacatcttcagagggtgctggctccctcaaaggtttcactgttgacattagtcgggttgcagctccatcatcgtaagtctgtctgacatttgtggtttttgactcctgcgaacttgtagaaactctggaatctcttttttcaggtctcgcgctaggaatggcaagtggtggcactgcagcttcatgcctcctctcatctccccgactgaaattgctcttgtttgaaggcacgttactatcaaagatgttggtatcagaagacttcagactagagggttcagttgtaacagagcgaagtttatctaatacaccatgaagccatacggtgaatcgaattgtgttgttccctagaaacagggacagatcctctgtcatttggtcctgacttttcttgttggccaccatcaccataatgtaatcaggaagttcttcatcaacataagctcctaattcttgtaatttccccttaatggcactccggatcttgcggctgatctcggtgccgatctccatggctctgcggcgtgcgggaactcagcactgcgcggcgcttggcttacccggaggctgccgcggactcctaccccgcagccgggacaccaccgcctcc

SEQ ID NO: 17253 - RNA, 14307 nt, Homo sapiens
  source 1..14307: mol_type = other RNA
tcaggccaggcacagtggctcacacctgtaatcttatcactttgggaggctgaggcaggtggatcgcttgagcccaggagttcaagaccagcctgggcaacatggtgaaaccccatcgctataaaaaacaacaattagccgggtgtggtggcacatgcctgtagtccctgctactcaggaggctgaggtgggaggatcacttgagcctggggaggtcaaggctttagtgagctgtgatggtgccactgcactccagcctgggtgacagagtgagaccccatttaaaaaacaaaaacaaaaacaaaaaaaaatgtgacatatagttgactaagaagtacatttcaatacaggattgaaagaacccacatatgttaattaaacacaagcgcagaatttgtgccttttacataaaggaagaatgcacataggcatgctttcagacaagcaattcatctagcagaaaaggaaggaatacatttttcagcccttccaggaataaaatccataaatgggctctatttcgtcctccaacacttgtatttcccacgtcatttactcctgcacacccccactcactagaagcctgctaaactgttccagtgagatattttaacacctgatagggaataaatatgcttctgttttggccttcaaaaataagctctgggccagttgcagtggctcacgcctgtaatcccaacactttgggaggccgaggtgggcggatcacgaggtcaggagtttgggatcagcctggccaatatggtgaaactccatctctactaaaaatacaaaaattagccaggcatggtgcctgtaatcccagctacttgggaggctgaaggagaagaatcgcttgaacctgggaggcacaggttgcagtgagccgagatcacaccactgcactccaggccaggtgacagagcgacactctgtctcaaaaaaataaataaatcaactctgtagcatagcatttgtaattctattattttgccttacatttccattatccttttaataaaattgtttttttacatcttcctaatcaagaagtattatgaggccaggcacagtggctcatacctggaatcccagcactttgggaggccgaggcaggcagatcacctgaggtcaaggtatttgagaccagcctggccaacatggtgaaaccccatctctactaaaaatacagaaattagctgggtgtggtggtgcacacctgtaatgctagctactcgggaggctgaggtaggagaatcgcttgaacctgggaggcagaggttgcaataagcctagatcatgccactgcactcaagcctgggagacagagcgagactacatcttaaaaaaaaaaaaaaaagtattatgagagaggataatgtattgtaatgtattgtagaggctaaataaaattatgctcatgtcagaaaaaaagagtatttctcaaaataaaattcactgaaactggatgtttattttgactgagatatagtatatcctcaaattgccatagaaagtttacaagaatattagaggtaaattataaatatcagggcctttttaaaaaaaaaagattctgcttataacttggtatttgtttataataaaaattatagtagccaataatgaacacttactctggcttggttatttacttaggtcaaaagaaggaggagcggttaaactgtgggatcaggaactgaggcggtgccgtgccttcaggcttgagacaggacaagccacagattgtgttcgttctgtgtgcagaggcaaagtaagatgttccatgagctgatacagtgcagcagaaaacagaaagtggttattactgtgattccctcaccctttgcagcctaatgaacaatacttaataatgcataacgatggatttgcttgccaacattactctgtctttgctgctttctttgccaaagttagcaccagtgtggtgcataagctaggaagctattctgtctaaatactgtatgtaaacctccaatattttctagaatctgccaatttaacaactctagtagacataattgaaagcccttggcagttgactcatattaggacagctgtctccattttttaaaaaaacacacattccctagataaaacgtgcagtaaacaaacaatgaaatactactcagccataaaaaataatgaaattctgtcattcttggtggcaacatggatgagactggaggacatgatgtgaagtgaaataagccaggcacagaaagataaatacatgttctcactcctgtgcagaaactaaaaaagttgatcccacagaggtggagagtagaatagtggttactggaggcggacaagggggagggggagggggatagggaaggactggttaaaggatacaagtttacacagccagataggaatagtatgttttagtattctgtagtactgtaggatgactatagttaagaatcacgtatttatgtattttcaggtatttacaagagaggattttgaaagtttccatcacaaagaaatgataaatgtctgaggtgatggttatgcgtattaccctatgccctatagatatgtataattatgtgtcaatttcaaaataaaaattcaaaactacaactcctatgaaaatttttgagcgtgtttgtacttattaagtgtatttataaatcatacggatattatcttcagcctgcatattaaattgtagttaagcttttactttttaactaaaaaataaattctattattttttcctatatcccactgcactgaccccagtttggaaatcctaagattatcaaataaaaactttgattattgaagaatccaggtgtactgccacagaaaagttctattctgtagcatggactctaatatgtaatctagcccattgtgcttacagatagatgtgtgcctgtagtcatagaaaaatttgcatgagctaatgactgccttgctactagattagctcaaagcaaaaagttctctgaaagcaggtcaatagggtcatttttatattatgaagaagaaaagcagctgttgtattacattcactgtattggtcctgcttgtgtttcagggcaagatccttgttgggacaaggaatgctgaaataatcgaagttggagagaaaaatgcagcttgtaatattttagttaacggtcatgtggatgggccaatctggggactagcaacacatccttccagggattttttcctttctgctgcagaagatgggacagtgagactttgggatattgctgataaagtaagtacagataatttttttaaaagaggttacaacttctaaaaagaaaagttggaagttctaaattgctagtacttaaagaactgccagaattctgttgagcattttgaggggaaactggtataatttagaagtacttcacttaatgtttcctatgactctttttttttttttttttaaatgcagaagatgttaaacaaagtgaatttgggacatgctgctcgtactgtgtgttacagccctgaaggggacatggtggctattggaatgaaaaatggagaatttatcattttactagtgagttctctaaaaatatggggaaagaagagagacaggagatgtgcaatccatgatatcaggttagtgaacaaatggaatagagtttctagtatatacttgatttaacttccatttgtaaaattttccatagccttgccttcaaaaagaggtccccagggcctgtagcatttcccgtattataaattgtatgctaaaatatggctgtttgtatactacttaattcttcttgctaaattataaacccactgggcaccaactataatagcaagtactagtaggtaatgtttgatgaattcatgttaacacttagccatgtccattaagttcatcccaccaagaggtatctcccactgtaatacaagagagctatctgcccttcaaaagttgtcaccctggaaaactaaagttgtgatttcaaacatatcttctcttagtaacctcagtttgggaatatgtagttcattaatttaatcaatacctattgattaaatgttccagaatccaaattaatttaaatgtttcttaaacctttgtttttcagtgcttaagcatttttcaacagtggctaccatttacggagtacttccgtgtgatcagtagataagattattgaatctaggtctgtcaaaagcttgtacacttttcatcagtaaaatccttttacaaatgaaaccttcctcagaacttcaatatataaaatagtaacagtggcttcccttagcttttacatgtctctatcgtacctcagtaagactcatgggccatttcaagagactgaattgtcccatatgactccaaagattgctaggcaaatagcatttcactttgtcttttaaataagttcttcaggccgggcgcggtggctcatgcctgtaatcccagcactttgggaggccgaggcaggcagatcacctgaagtcaggagtactcgaccagcctggccaacatagtgaaaccccatctcaactaaaaatacaaaaatcagccgggcgtggtggcaggcgcctgtaatcccagctactcagggggctgaaacaggagaatcgcttgaacccgggaggcggaggttgcgccatcgcactccagcctgggagacaagagcgagacttcgtctcaaaaaaaaaaaattcttcttccaagattcaagttgtgtcatttcaccttaataactggaggttagttaagctgggctgtgttctttgcttaatattaagacaacgttttttccagatggaagaaaactatcttaatgaattgttagcttattaattatgtaatgctaatggcttttaaaagctgagatgttctgactgggtgttgtggctcacacctgtaatcccagtaccttgggaggccaagggggaaggattgcttgaggccaggagtttgggaccatagtgagaccccgcctctatttaaaaaattaaattttgttttgttttgttttgagttggagttttgctcttgttgcccatgctgaagtgcaatggtgcaatctcagctcaccacaacctgtgcctcctgggttcaagcgattctcctgcttcagcctcccgagtagatgggattacaggcgtgcaccaccatgcctggctaattttgtatttttagtagagacagggtttctctatgttggtcaggctggtctcaaactctcgacctcaggtgatctgcccgcctccgcttcccaaagttctgggattataggtgtgagccactgggcctggcctaagaaagtttttttaagccattagacgtttttaaaggaattgggagatgacaattggggaaatatttaaaatttaagtaaaatataaagcttccttatttcatgtaacccagacaatctcagtatacatgatcagttgtgtctgacaggtaaatctatttgaggccttatcacacgttacttttaagaactagaaaggaaaagtcactgatcttaagtatttataatacttcatgtggtctaatactttttacgttttgttttgattcagatttagtccggattcccggtatctggcagtaggttctagtgagaactcagtggatttttatgacctaacgctgggccccactcttaacagaatcagctactgcaaagacattccaagctttgtcattcaaatggacttctctgcagatagcagttatctccaggtacagtaccaatactgtatacccaggtggcaagttcttctgcttttacatttcgtgttagtgaatgcatttaaagttcctgagctccagagctccagcttctcaactcctccctttgtaccttctgacctacagctcccctttcctcccccacttatcagagcttttctcctattaagtttttgtagtgatcttttgcatacttaataatgttagacatgtaaatcaagtagcaatatgctagtattctgtaaaccccctgtggattttgtctctcacctaatggaattcttgtcccattttaatctgatgaaaaaggtctctagtggctgctataaacggcatgtctatgaagtgccttcaggaaaacatcttatggatcatgccgctattgacagaattacttgggctacatggactaggtaaatacttatatattcacaaggcaagaactgactttgaaggccagttagaaaatcctatttctgaactgttagagccattccaataaggaatagtaattgagtttcaagtttttgttaccatattttgaaatggtatgttcatgttgggacccctttttattgaatatatttccatgttttatcagtttccatgatttatcaagttttttttttaaggaaatcaaagttttaactttaaagataccctgatatttttcttaatgctaaatttaatgactggcaaaaaggtattgggtgctgttaagcaactgttattaattctctatctaaaggaatgctatcttgaatctattagaagtcaaagcttccaaatttgttcaaatttcctggctgtatgacaggtaaccatgactatccatttttttggccaatgaaaaatgccatcaaattcctgtatcagccaggcatatagtggctcatgcctgtaatctctgatgtagcaggccgaggtgggaggatcacttgagcctagaagttttgataccagcctgggcaacatagcaagaccccatctctgaaatttttttaattcctatgtcataagtcatttttatttttgtagagatagggatctcacaatattgcccaggctggtctcaaactcttggcctcaagcagtcctcctgcctcagcctcccaaaatgttgggattactggtatgtgctgctggacccagccaagtagcacttttaatttgaaaaatagttctatcagttttcagtcaggcgcggtggctcagcctgtaatcccagcactttgggaggccgagcgggggtgatcacctgaggtcgggagttcgagactagcctgaccaacatggagaaaccctgtctctactaaaaatacaaaataagccgggcatgttagcgcatgcctgtgatcccagctactcgggaggctgaggcaggagaattgcttgaacccaggaggcagaggttgcggtgagccgagatcatgccattgcactccagcctgggtaacaagagcgaaaactccgtctcaaaaaaaaaaaaagaaaaaatagttctatcagttttcataaagtactactttaatcttaaaaagattaatctagaaacccttcaaattataaaatgtcatttttaaaaggcaggagttgatatcctgatgaaattcaggtctccaaacaacttaccataatttacttcctgtattttaagtaacatgatagggtacttagagattaattgccaagaaactttttgaatatagtcaacctgcccgcacttgccatgatgagttttcttttgttccttccctctagtattctaggagatgaggttttgggaatctggtccagacatgctgagaaagctgatgtcaactgtgcctgtgtatctcattcaggaatcagtcttgttacaggagatgactttggcatggttaagttatttgacttcccatgtccagaaaaatttgtaagtttgtgttttgtttactattatcagtttactcctaattttgatgtcttatcatcagcacttttccccatatatttaaaatgttttgtcctaatttctaaatttttccccaaactttctaaatctatttactttgaaataaaagctattagaaacaaatcctctccctcgagtaataccatctttggaaccatcctacaaaagctgtaattagcttttcaccaaacctataatcagttatcaaatttcaaatgcttttccttagagaaaaatggtcagagtacctggagacatctgactgcccacacagcctggttttgcagatccactactcatgctgaaaagcattctaatcactggctgcggtgctaactccctactctctccacagctcttgtcatagagattatagttcctaataagagcctttgacttctgtgtgcaccaaatgccctgagcttgtctgtcattgttttttaggcaaaacacaaaaggttcttgggtcattcgccccatgtgacaaatattcgatttaccagtggtgatcgacatgttgttagtgctggaggtgatgactgcaggttagtaactttctcagcccatgaagagcagactatgttactagttaagagacttaatacaacaactcctacagctttggtttatgaaatcagctagtcaacattagtagaaggtagtataaccagatggctcttcagaatctcatatttatgcaaatacagaataaaaggagttaaagaggaaaaatattacacatgtaacctgaaagcacaactgaaaaatattaaactgttatgaaaatctaaaaacataattaactccctgcaattttcttctctgattgcagcttatttgtctggaaatgtgtacatacacctcactgagagatgctgagatgactacagaaattaactttgagaccagaattacagagaagaaaaaccaaaacccaaccctgcatggtcaagtggtgctaacccaagactgtaacagggagaaatgcccagaatcatcaaaatagtgaaagactgatctgttcaaaatatttgctatatgcactgggtataatccgtaatccatacactgccagataatgccatttcaaggaaggatcgaatacttgatggtaaaggccaagtccccctgtattgggaagtgtgtgatttcggcagacctgctgggaaaatttagggtagagcactctttacagaagaactcaaaaacccaatttggataattttcattatctttttagcaaaatggtttcttaatgtttatattttattttcaaggttcattgtttaatgaaatattttattcttgcatttccataaggaaagggaaagtcatgatcatcctaaaggatcacagtttttaaaaggcaaacattttccctaaggaaacagacacaagctttcctagagaatatgatgttttttaggcattaataaggtccttttttataaaggacacttttctcctagtagttttgaattcaggaacagatccaaagttagcagtatatggctgctacatttccattttcattttcgagccatcagtttatgttcagatgccatctctgtaatcgcacatttaaaacataactgtagcctcactaatggaaaagtagtatgatgaacaatcattcccaatggtgtacaatgtaagggttttagggagcaacagtatttaactggaagaaagaattgcatatttaatgtagtctaatatatacacatttgtttaacatgtaaacaaaagtgttaaattcacatatacaacattatacaatttaatcactcttggaataaaatttttatagccttttttctattgggaaaatttgtttagatgtgtgccactccataggtttatttccaaaatgaatgagcccaactccatttgtaaaaacttgtcagttagaattcctttttttagtggattagggctgaattcttagatccttatttcttttcactttaaatgctgccaaagatcactactcatcattcaggaattcgctgtctagcctatctgtagtttcctgaagattgaaaattatgtagactgctatttaaaaatatatttttctaagtgtgaggtttaagatgctgtattgaccctatgagtttttaatgtgttaattatctttatagcataatagatcgctttaggttcctggaatcccatttggtctgacaggatatatgaagattcttaatacctattttctgtgtctaatacttggttaatactaaaaatagaaatgactaaattacatcacagaaagcataaccagtgattgaacctggtagttttaaagctctaaatagctgtggctgaaggactgattatggggctaagaagcttgaaacgtaagttggtacttgttcatcagtggattctcctaaattaagccaaattttgaaatacatgactattaagtttctactcatgtatttacagtcagtcaataaattaaaggaggaaaaaaatccctgaacaacctgcccataaaaagaaaaatactctacatttgagcctgctgcagttttaaattttccctctgggtcaagtttgccagcttttggctacagagaaattatatttccattacagtgcaggtagaaactctgtaaccttaagcatgtaaactacatagaataaaactgtttccactgcatttctgtccttcaaagtggccaacctgattaagtcagccttaatcactgctgctgtcagtttcacgactaaaggtcatattgactaagtagtcatcagctgaccacctcgctgtatcagccagcaacgaggggaaggtgaagaaacatgataggccatatagaatctgccctatgtttacttttttaacccagataattatttttgtgtgcagtatctaagctcctgattgtgtaacctgggacttctggcaccttttgttccattcattttatgtataaaatgcatgccaaagcacactgtgccctctggtacccttgcttccaatcgccaaccatgctcatttccttcctttttttgtggtccctttttgtggtgatcattttaaaccacgtcatccaacaaatgttttatggtcaaccttagcttgttcataagccatagcaactgaaagattaaactcttaaatatgtgtctgggcagtggctattaaatagcaaaaaacaatcagattttagtattttattatttccttgtaaaatggctgaactaaattaaacccttgtttcccatttgttctataatttatagtgaaactgagaacaaaactatctttataaatgatagctaaaagtatttccagatatttaaacaatttaaaataaatttcttctgcagagatgcaaagcatctcaacactggaatgaacaaatgccttaaattcaatggagtaaacctttagaatgaagaggaactgtcatttcacccaagccgaagacaacagccttatgcacttgtgtgctctgtctttgctgcttctcgtgtttcaagcctttcctgtgggatcagcacagcaaagtgcaacttaccaaatggtttaatgactggttaattctttcttctcccaatggaaaagcaatggcaacacaacagtagactgctggcttgacaatcttaaacgtgagcctttgcacatgtaggtttatcatcatttgagtatacgactaagcaagtcaatgaactttttttttttttttagcagtttaatttggtcctgagaatgttgcagtctttattaccccttttgcattaatccacttttctaaccaccttttaagctttaatttttaacactatacaccaagtctttgaaatcagtgatctgttatttaactctaaagcatttgacacttcttgccttaacagttttaaaaaccacacacaaaaaaactctgtaagtaatacagtaggccaaaagtttcatcctatctatcttgcagtttacctatctgatctgatctctgtaattatagttctgtcatttaaaatatactatttaaatctaatttttacatttcaaaaattatcttcagtagtaactaagtatattttctgtggattctgagaatgttatttttcagaatgtgagaatatatatgtacatttataatcttgtgactttaaagtctgttttcagatacagtatgtaaatacttgtaaaaaaatttgtataattttgtgataatgtagtttcccaaaaaaattatttagaaggcattatgttattagtaaatgagagcactgtatagaactgttcctattttctgcacttgccattccagctgcctccactgtccatacccacctcattcatcctgtcacagaaggcaggaaaactgggaactttaccaaagtagcactcagcctgagaggcctgtataatcatgcttttcaaactaaattcacttaaaaattaaaaagcagaattgaatattttaagcagcctcagtacctttggccaatgctgttttcatggtggattatgaacattatataatctttgggaaaagtgaaagtagtacaatttttagaataatgacaactgcctcactgcatctctccactcacacagcaaccgtgtagccccctaagctgcagtaccatgactaaccatgatgtcaatttcatatgctgatcctcacaacagcagtgcacaaacatgccccaaatattttaacagaatttagctcttccttaagctgtcttttcatagtaaaaacaaaacaaaaacacccaatgttaaaaccacataataaacttacaaacttgaaaaattagacacttcagatagataggcaataaaacttcatattatgaaagcaatatattccaagtttcaaagatttgacaagttctgtagagtatctttcatcagtacatgaaaacttccaaactgcatgatcttctgccaggcaggactgggtgctattcgctggtttgaggtcgaatccatttcaaggcatgtcgtggtgggacattaatggtgggatggtagaatgtgcagtccggtcttgtacattgagtgttaaacctacaatgttttggatgatagaagggacattccatcttcttacaagcagggaagtaacggcagagctgactactggaaggtggtgctggtggtgcaactggttttggagacagtactggaattcttctactcacatgagtgaagggacaatctggtttagtacactttgcatcatatttacaatttgggtgaacaaacaaacatttttcagcaaatttacaattggggaaggctttgcagggtgagatggggtgatggtaggcacactcatccccatttttacaagcaggccagtacttgcagcgctccaaaagtttttctggtttctgtgccacactcagttcactcatctcagctgtagagtagttagttgtttttgttacggattcttgagcttcagatatagccttcaaaatcagattcttgttagcttgtttagaaggtggaagagaaggtctcctttcaggctttgcaggcacagacacactgctggagatgcttcctgttcgagacccgtaatcatcatcttcttcctcctcttctccatcatgattgaatttttttactttaacaactgaacttaccacaggcaactttctcttccgaaagttttcatcctccatactcattttctccgagttgtttctaaagaacggactatacgtttcttctaagctgttaagcacctctggttcacacaaacgtcctgtttcatatacccaactactctgcatatcaagctgcttggcagcatgaatactattctgctgctgttgaaattgcaacctgtttaaatgaacaccactatctgcatttctacttgcaggtggtcgataaatttcaatagaagggcgagaagaaccatatgtaagtgtcactgtaggttttttctgagataagggattctcctgcacaaagttgaggtcttcgtcaatgagatcatctggttctggcttaatatcaatcacatcttcagagggtgctggctccctcaaaggtttcactgttgacattagtcgggttgcagctccatcatcgtaagtctgtctgacatttgtggtttttgactcctgcgaacttgtagaaactctggaatctcttttttcaggtctcgcgctaggaatggcaagtggtggcactgcagcttcatgcctcctctcatctccccgactgaaattgctcttgtttgaaggcacgttactatcaaagatgttggtatcagaagacttcagactagagggttcagttgtaacagagcgaagtttatctaatacaccatgaagccatacggtgaatcgaattgtgttgttccctagaaacagggacagatcctctgtcatttggtcctgacttttcttgttggccaccatcaccataatgtaatcaggaagttcttcatcaacataagctcctaattcttgtaatttccccttaatggcactccggatcttgcggctgatctcggtgccgatctccatggctctgcggcgtgcgggaactcagcactgcgcggcgcttggcttacccggaggctgccgcggactcctaccccgcagccgggacaccaccgcctcc

SEQ ID NO: 17254 - RNA, 14423 nt, Homo sapiens
  source 1..14423: mol_type = other RNA
tcaggccaggcacagtggctcacacctgtaatcttatcactttgggaggctgaggcaggtggatcgcttgagcccaggagttcaagaccagcctgggcaacatggtgaaaccccatcgctataaaaaacaacaattagccgggtgtggtggcacatgcctgtagtccctgctactcaggaggctgaggtgggaggatcacttgagcctggggaggtcaaggctttagtgagctgtgatggtgccactgcactccagcctgggtgacagagtgagaccccatttaaaaaacaaaaacaaaaacaaaaaaaaatgtgacatatagttgactaagaagtacatttcaatacaggattgaaagaacccacatatgttaattaaacacaagcgcagaatttgtgccttttacataaaggaagaatgcacataggcatgctttcagacaagcaattcatctagcagaaaaggaaggaatacatttttcagcccttccaggaataaaatccataaatgggctctatttcgtcctccaacacttgtatttcccacgtcatttactcctgcacacccccactcactagaagcctgctaaactgttccagtgagatattttaacacctgatagggaataaatatgcttctgttttggccttcaaaaataagctctgggccagttgcagtggctcacgcctgtaatcccaacactttgggaggccgaggtgggcggatcacgaggtcaggagtttgggatcagcctggccaatatggtgaaactccatctctactaaaaatacaaaaattagccaggcatggtgcctgtaatcccagctacttgggaggctgaaggagaagaatcgcttgaacctgggaggcacaggttgcagtgagccgagatcacaccactgcactccaggccaggtgacagagcgacactctgtctcaaaaaaataaataaatcaactctgtagcatagcatttgtaattctattattttgccttacatttccattatccttttaataaaattgtttttttacatcttcctaatcaagaagtattatgaggccaggcacagtggctcatacctggaatcccagcactttgggaggccgaggcaggcagatcacctgaggtcaaggtatttgagaccagcctggccaacatggtgaaaccccatctctactaaaaatacagaaattagctgggtgtggtggtgcacacctgtaatgctagctactcgggaggctgaggtaggagaatcgcttgaacctgggaggcagaggttgcaataagcctagatcatgccactgcactcaagcctgggagacagagcgagactacatcttaaaaaaaaaaaaaaaagtattatgagagaggataatgtattgtaatgtattgtagaggctaaataaaattatgctcatgtcagaaaaaaagagtatttctcaaaataaaattcactgaaactggatgtttattttgactgagatatagtatatcctcaaattgccatagaaagtttacaagaatattagaggtaaattataaatatcagggcctttttaaaaaaaaaagattctgcttataacttggtatttgtttataataaaaattatagtagccaataatgaacacttactctggcttggttatttacttaggtcaaaagaaggaggagcggttaaactgtgggatcaggaactgaggcggtgccgtgccttcaggcttgagacaggacaagccacagattgtgttcgttctgtgtgcagaggcaaagtaagatgttccatgagctgatacagtgcagcagaaaacagaaagtggttattactgtgattccctcaccctttgcagcctaatgaacaatacttaataatgcataacgatggatttgcttgccaacattactctgtctttgctgctttctttgccaaagttagcaccagtgtggtgcataagctaggaagctattctgtctaaatactgtatgtaaacctccaatattttctagaatctgccaatttaacaactctagtagacataattgaaagcccttggcagttgactcatattaggacagctgtctccattttttaaaaaaacacacattccctagataaaacgtgcagtaaacaaacaatgaaatactactcagccataaaaaataatgaaattctgtcattcttggtggcaacatggatgagactggaggacatgatgtgaagtgaaataagccaggcacagaaagataaatacatgttctcactcctgtgcagaaactaaaaaagttgatcccacagaggtggagagtagaatagtggttactggaggcggacaagggggagggggagggggatagggaaggactggttaaaggatacaagtttacacagccagataggaatagtatgttttagtattctgtagtactgtaggatgactatagttaagaatcacgtatttatgtattttcaggtatttacaagagaggattttgaaagtttccatcacaaagaaatgataaatgtctgaggtgatggttatgcgtattaccctatgccctatagatatgtataattatgtgtcaatttcaaaataaaaattcaaaactacaactcctatgaaaatttttgagcgtgtttgtacttattaagtgtatttataaatcatacggatattatcttcagcctgcatattaaattgtagttaagcttttactttttaactaaaaaataaattctattattttttcctatatcccactgcactgaccccagtttggaaatcctaagattatcaaataaaaactttgattattgaagaatccaggtgtactgccacagaaaagttctattctgtagcatggactctaatatgtaatctagcccattgtgcttacagatagatgtgtgcctgtagtcatagaaaaatttgcatgagctaatgactgccttgctactagattagctcaaagcaaaaagttctctgaaagcaggtcaatagggtcatttttatattatgaagaagaaaagcagctgttgtattacattcactgtattggtcctgcttgtgtttcagggcaagatccttgttgggacaaggaatgctgaaataatcgaagttggagagaaaaatgcagcttgtaatattttagttaacggtcatgtggatgggccaatctggggactagcaacacatccttccagggattttttcctttctgctgcagaagatgggacagtgagactttgggatattgctgataaagtaagtacagataatttttttaaaagaggttacaacttctaaaaagaaaagttggaagttctaaattgctagtacttaaagaactgccagaattctgttgagcattttgaggggaaactggtataatttagaagtacttcacttaatgtttcctatgactctttttttttttttttttaaatgcagaagatgttaaacaaagtgaatttgggacatgctgctcgtactgtgtgttacagccctgaaggggacatggtggctattggaatgaaaaatggagaatttatcattttactagtgagttctctaaaaatatggggaaagaagagagacaggagatgtgcaatccatgatatcaggttagtgaacaaatggaatagagtttctagtatatacttgatttaacttccatttgtaaaattttccatagccttgccttcaaaaagaggtccccagggcctgtagcatttcccgtattataaattgtatgctaaaatatggctgtttgtatactacttaattcttcttgctaaattataaacccactgggcaccaactataatagcaagtactagtaggtaatgtttgatgaattcatgttaacacttagccatgtccattaagttcatcccaccaagaggtatctcccactgtaatacaagagagctatctgcccttcaaaagttgtcaccctggaaaactaaagttgtgatttcaaacatatcttctcttagtaacctcagtttgggaatatgtagttcattaatttaatcaatacctattgattaaatgttccagaatccaaattaatttaaatgtttcttaaacctttgtttttcagtgcttaagcatttttcaacagtggctaccatttacggagtacttccgtgtgatcagtagataagattattgaatctaggtctgtcaaaagcttgtacacttttcatcagtaaaatccttttacaaatgaaaccttcctcagaacttcaatatataaaatagtaacagtggcttcccttagcttttacatgtctctatcgtacctcagtaagactcatgggccatttcaagagactgaattgtcccatatgactccaaagattgctaggcaaatagcatttcactttgtcttttaaataagttcttcaggccgggcgcggtggctcatgcctgtaatcccagcactttgggaggccgaggcaggcagatcacctgaagtcaggagtactcgaccagcctggccaacatagtgaaaccccatctcaactaaaaatacaaaaatcagccgggcgtggtggcaggcgcctgtaatcccagctactcagggggctgaaacaggagaatcgcttgaacccgggaggcggaggttgcgccatcgcactccagcctgggagacaagagcgagacttcgtctcaaaaaaaaaaaattcttcttccaagattcaagttgtgtcatttcaccttaataactggaggttagttaagctgggctgtgttctttgcttaatattaagacaacgttttttccagatggaagaaaactatcttaatgaattgttagcttattaattatgtaatgctaatggcttttaaaagctgagatgttctgactgggtgttgtggctcacacctgtaatcccagtaccttgggaggccaagggggaaggattgcttgaggccaggagtttgggaccatagtgagaccccgcctctatttaaaaaattaaattttgttttgttttgttttgagttggagttttgctcttgttgcccatgctgaagtgcaatggtgcaatctcagctcaccacaacctgtgcctcctgggttcaagcgattctcctgcttcagcctcccgagtagatgggattacaggcgtgcaccaccatgcctggctaattttgtatttttagtagagacagggtttctctatgttggtcaggctggtctcaaactctcgacctcaggtgatctgcccgcctccgcttcccaaagttctgggattataggtgtgagccactgggcctggcctaagaaagtttttttaagccattagacgtttttaaaggaattgggagatgacaattggggaaatatttaaaatttaagtaaaatataaagcttccttatttcatgtaacccagacaatctcagtatacatgatcagttgtgtctgacaggtaaatctatttgaggccttatcacacgttacttttaagaactagaaaggaaaagtcactgatcttaagtatttataatacttcatgtggtctaatactttttacgttttgttttgattcagatttagtccggattcccggtatctggcagtaggttctagtgagaactcagtggatttttatgacctaacgctgggccccactcttaacagaatcagctactgcaaagacattccaagctttgtcattcaaatggacttctctgcagatagcagttatctccaggtacagtaccaatactgtatacccaggtggcaagttcttctgcttttacatttcgtgttagtgaatgcatttaaagttcctgagctccagagctccagcttctcaactcctccctttgtaccttctgacctacagctcccctttcctcccccacttatcagagcttttctcctattaagtttttgtagtgatcttttgcatacttaataatgttagacatgtaaatcaagtagcaatatgctagtattctgtaaaccccctgtggattttgtctctcacctaatggaattcttgtcccattttaatctgatgaaaaaggtctctagtggctgctataaacggcatgtctatgaagtgccttcaggaaaacatcttatggatcatgccgctattgacagaattacttgggctacatggactaggtaaatacttatatattcacaaggcaagaactgactttgaaggccagttagaaaatcctatttctgaactgttagagccattccaataaggaatagtaattgagtttcaagtttttgttaccatattttgaaatggtatgttcatgttgggacccctttttattgaatatatttccatgttttatcagtttccatgatttatcaagttttttttttaaggaaatcaaagttttaactttaaagataccctgatatttttcttaatgctaaatttaatgactggcaaaaaggtattgggtgctgttaagcaactgttattaattctctatctaaaggaatgctatcttgaatctattagaagtcaaagcttccaaatttgttcaaatttcctggctgtatgacaggtaaccatgactatccatttttttggccaatgaaaaatgccatcaaattcctgtatcagccaggcatatagtggctcatgcctgtaatctctgatgtagcaggccgaggtgggaggatcacttgagcctagaagttttgataccagcctgggcaacatagcaagaccccatctctgaaatttttttaattcctatgtcataagtcatttttatttttgtagagatagggatctcacaatattgcccaggctggtctcaaactcttggcctcaagcagtcctcctgcctcagcctcccaaaatgttgggattactggtatgtgctgctggacccagccaagtagcacttttaatttgaaaaatagttctatcagttttcagtcaggcgcggtggctcagcctgtaatcccagcactttgggaggccgagcgggggtgatcacctgaggtcgggagttcgagactagcctgaccaacatggagaaaccctgtctctactaaaaatacaaaataagccgggcatgttagcgcatgcctgtgatcccagctactcgggaggctgaggcaggagaattgcttgaacccaggaggcagaggttgcggtgagccgagatcatgccattgcactccagcctgggtaacaagagcgaaaactccgtctcaaaaaaaaaaaaagaaaaaatagttctatcagttttcataaagtactactttaatcttaaaaagattaatctagaaacccttcaaattataaaatgtcatttttaaaaggcaggagttgatatcctgatgaaattcaggtctccaaacaacttaccataatttacttcctgtattttaagtaacatgatagggtacttagagattaattgccaagaaactttttgaatatagtcaacctgcccgcacttgccatgatgagttttcttttgttccttccctctagtattctaggagatgaggttttgggaatctggtccagacatgctgagaaagctgatgtcaactgtgcctgtgtatctcattcaggaatcagtcttgttacaggagatgactttggcatggttaagttatttgacttcccatgtccagaaaaatttgtaagtttgtgttttgtttactattatcagtttactcctaattttgatgtcttatcatcagcacttttccccatatatttaaaatgttttgtcctaatttctaaatttttccccaaactttctaaatctatttactttgaaataaaagctattagaaacaaatcctctccctcgagtaataccatctttggaaccatcctacaaaagctgtaattagcttttcaccaaacctataatcagttatcaaatttcaaatgcttttccttagagaaaaatggtcagagtacctggagacatctgactgcccacacagcctggttttgcagatccactactcatgctgaaaagcattctaatcactggctgcggtgctaactccctactctctccacagctcttgtcatagagattatagttcctaataagagcctttgacttctgtgtgcaccaaatgccctgagcttgtctgtcattgttttttaggcaaaacacaaaaggttcttgggtcattcgccccatgtgacaaatattcgatttaccagtggtgatcgacatgttgttagtgctggaggtgatgactgcaggttagtaactttctcagcccatgaagagcagactatgttactagttaagagacttaatacaacaactcctacagctttggtttatgaaatcagctagtcaacattagtagaaggtagtataaccagatggctcttcagaatctcatatttatgcaaatacagaataaaaggagttaaagaggaaaaatattacacatgtaacctgaaagcacaactgaaaaatattaaactgttatgaaaatctaaaaacataattaactccctgcaattttcttctctgattgcagcttatttgtctggaaatgtgtacatacacctcactgagagatgctgagatgactacagaaattaactttgagaccagaattacagagaagaaaaaccaaaacccaaccctgcatggtcaagtggtgctaacccaagactgtaacagggagaaatgcccagaatcatcaaaatagtgaaagactgatctgttcaaaatatttgctatatgcactgggtataatccgtaatccatacactgccagataatgccatttcaaggaaggatcgaatacttgatggtaaaggccaagtccccctgtattgggaagtgtgtgatttcggcagacctgctgggaaaatttagggtagagcactctttacagaagaactcaaaaacccaatttggataattttcattatctttttagcaaaatggtttcttaatgtttatattttattttcaaggttcattgtttaatgaaatattttattcttgcatttccataaggaaagggaaagtcatgatcatcctaaaggatcacagtttttaaaaggcaaacattttccctaaggaaacagacacaagctttcctagagaatatgatgttttttaggcattaataaggtccttttttataaaggacacttttctcctagtagttttgaattcaggaacagatccaaagttagcagtatatggctgctacatttccattttcattttcgagccatcagtttatgttcagatgccatctctgtaatcgcacatttaaaacataactgtagcctcactaatggaaaagtagtatgatgaacaatcattcccaatggtgtacaatgtaagggttttagggagcaacagtatttaactggaagaaagaattgcatatttaatgtagtctaatatatacacatttgtttaacatgtaaacaaaagtgttaaattcacatatacaacattatacaatttaatcactcttggaataaaatttttatagccttttttctattgggaaaatttgtttagatgtgtgccactccataggtttatttccaaaatgaatgagcccaactccatttgtaaaaacttgtcagttagaattcctttttttagtggattagggctgaattcttagatccttatttcttttcactttaaatgctgccaaagatcactactcatcattcaggaattcgctgtctagcctatctgtagtttcctgaagattgaaaattatgtagactgctatttaaaaatatatttttctaagtgtgaggtttaagatgctgtattgaccctatgagtttttaatgtgttaattatctttatagcataatagatcgctttaggttcctggaatcccatttggtctgacaggatatatgaagattcttaatacctattttctgtgtctaatacttggttaatactaaaaatagaaatgactaaattacatcacagaaagcataaccagtgattgaacctggtagttttaaagctctaaatagctgtggctgaaggactgattatggggctaagaagcttgaaacgtaagttggtacttgttcatcagtggattctcctaaattaagccaaattttgaaatacatgactattaagtttctactcatgtatttacagtcagtcaataaattaaaggaggaaaaaaatccctgaacaacctgcccataaaaagaaaaatactctacatttgagcctgctgcagttttaaattttccctctgggtcaagtttgccagcttttggctacagagaaattatatttccattacagtgcaggtagaaactctgtaaccttaagcatgtaaactacatagaataaaactgtttccactgcatttctgtccttcaaagtggccaacctgattaagtcagccttaatcactgctgctgtcagtttcacgactaaaggtcatattgactaagtagtcatcagctgaccacctcgctgtatcagccagcaacgaggggaaggtgaagaaacatgataggccatatagaatctgccctatgtttacttttttaacccagataattatttttgtgtgcagtatctaagctcctgattgtgtaacctgggacttctggcaccttttgttccattcattttatgtataaaatgcatgccaaagcacactgtgccctctggtacccttgcttccaatcgccaaccatgctcatttccttcctttttttgtggtccctttttgtggtgatcattttaaaccacgtcatccaacaaatgttttatggtcaaccttagcttgttcataagccatagcaactgaaagattaaactcttaaatatgtgtctgggcagtggctattaaatagcaaaaaacaatcagattttagtattttattatttccttgtaaaatggctgaactaaattaaacccttgtttcccatttgttctataatttatagtgaaactgagaacaaaactatctttataaatgatagctaaaagtatttccagatatttaaacaatttaaaataaatttcttctgcagagatgcaaagcatctcaacactggaatgaacaaatgccttaaattcaatggagtaaacctttagaatgaagaggaactgtcatttcacccaagccgaagacaacagccttatgcacttgtgtgctctgtctttgctgcttctcgtgtttcaagcctttcctgtgggatcagcacagcaaagtgcaacttaccaaatggtttaatgactggttaattctttcttctcccaatggaaaagcaatggcaacacaacagtagactgctggcttgacaatcttaaacgtgagcctttgcacatgtaggtttatcatcatttgagtatacgactaagcaagtcaatgaactttttttttttttttagcagtttaatttggtcctgagaatgttgcagtctttattaccccttttgcattaatccacttttctaaccaccttttaagctttaatttttaacactatacaccaagtctttgaaatcagtgatctgttatttaactctaaagcatttgacacttcttgccttaacagttttaaaaaccacacacaaaaaaactctgtaagtaatacagtaggccaaaagtttcatcctatctatcttgcagtttacctatctgatctgatctctgtaattatagttctgtcatttaaaatatactatttaaatctaatttttacatttcaaaaattatcttcagtagtaactaagtatattttctgtggattctgagaatgttatttttcagaatgtgagaatatatatgtacatttataatcttgtgactttaaagtctgttttcagatacagtatgtaaatacttgtaaaaaaatttgtataattttgtgataatgtagtttcccaaaaaaattatttagaaggcattatgttattagtaaatgagagcactgtatagaactgttcctattttctgcacttgccattccagctgcctccactgtccatacccacctcattcatcctgtcacagaaggcaggaaaactgggaactttaccaaagtagcactcagcctgagaggcctgtataatcatgcttttcaaactaaattcacttaaaaattaaaaagcagaattgaatattttaagcagcctcagtacctttggccaatgctgttttcatggtggattatgaacattatataatctttgggaaaagtgaaagtagtacaatttttagaataatgacaactgcctcactgcatctctccactcacacagcaaccgtgtagccccctaagctgcagtaccatgactaaccatgatgtcaatttcatatgctgatcctcacaacagcagtgcacaaacatgccccaaatattttaacagaatttagctcttccttaagctgtcttttcatagtaaaaacaaaacaaaaacacccaatgttaaaaccacataataaacttacaaacttgaaaaattagacacttcagatagataggcaataaaacttcatattatgaaagcaatatattccaagtttcaaagatttgacaagttctgtagagtatctttcatcagtacatgaaaacttccaaactgcatgatcttctgccaggcaggactgggtgctattcgctggtttgaggtcgaatccatttcaaggcatgtcgtggtgggacattaatggtgggatggtagaatgtgcagtccggtcttgtacattgagtgttaaacctacaatgttttggatgatagaagggacattccatcttcttacaagcagggaagtaacggcagagctgactactggaaggtggtgctggtggtgcaactggttttggagacagtactggaattcttctactcacatgagtgaagggacaatctggtttagtacactttgcatcatatttacaatttgggtgaacaaacaaacatttttcagcaaatttacaattggggaaggctttgcagggtgagatggggtgatggtaggcacactcatccccatttttacaagcaggccagtacttgcagcgctccaaaagtttttctggtttctgtgccacactcagttcactcatctcagcttgactcatctgcagagtttctgccattactgggtcgatttgcagtcgggataataattgcctctgttgagttccttgatttttttctacagaatctccttttgtttcctcttctttaatggggggacttattctgggggtcctactttgtccctggaccacttctgctagcaattcttcttgagaagttcgagttctgggagcaactggaagtgtctgtttctgtggaactgtagagtagttagttgtttttgttacggattcttgagcttcagatatagccttcaaaatcagattcttgttagcttgtttagaaggtggaagagaaggtctcctttcaggctttgcaggcacagacacactgctggagatgcttcctgttcgagacccgtaatcatcatcttcttcctcctcttctccatcatgattgaatttttttactttaacaactgaacttaccacaggcaactttctcttccgaaagttttcatcctccatactcattttctccgagttgtttctaaagaacggactatacgtttcttctaagctgttaagcacctctggttcacacaaacgtcctgtttcatatacccaactactctgcatatcaagctgcttggcagcatgaatactattctgctgctgttgaaattgcaacctgtttaaatgaacaccactatctgcatttctacttgcaggtggtcgataaatttcaatagaagggcgagaagaaccatatgtaagtgtcactgtaggttttttctgagataagggattctcctgcacaaagttgaggtcttcgtcaatgagatcatctggttctggcttaatatcaatcacatcttcagagggtgctggctccctcaaaggtttcactgttgacattagtcgggttgcagctccatcatcgtaagtctgtctgacatttgtggtttttgactcctgcgaacttgtagaaactctggaatctcttttttcaggtctcgcgctaggaatggcaagtggtggcactgcagcttcatgcctcctctcatctccccgactgaaattgctcttgtttgaaggcacgttactatcaaagatgttggtatcagaagacttcagactagagggttcagttgtaacagagcgaagtttatctaatacaccatgaagccaacataagctcctaattcttgtaatttccccttaatggcactccggatcttgcggctgatctcggtgccgatctccatggctctgcggcgtgcgggaactcagcactgcgcggcgcttggcttacccggaggctgccgcggactcctaccccgcagccgggacaccaccgcctcc

SEQ ID NO: 17255 - RNA, 13854 nt, Homo sapiens
  source 1..13854: mol_type = other RNA
tcaggccaggcacagtggctcacacctgtaatcttatcactttgggaggctgaggcaggtggatcgcttgagcccaggagttcaagaccagcctgggcaacatggtgaaaccccatcgctataaaaaacaacaattagccgggtgtggtggcacatgcctgtagtccctgctactcaggaggctgaggtgggaggatcacttgagcctggggaggtcaaggctttagtgagctgtgatggtgccactgcactccagcctgggtgacagagtgagaccccatttaaaaaacaaaaacaaaaacaaaaaaaaatgtgacatatagttgactaagaagtacatttcaatacaggattgaaagaacccacatatgttaattaaacacaagcgcagaatttgtgccttttacataaaggaagaatgcacataggcatgctttcagacaagcaattcatctagcagaaaaggaaggaatacatttttcagcccttccaggaataaaatccataaatgggctctatttcgtcctccaacacttgtatttcccacgtcatttactcctgcacacccccactcactagaagcctgctaaactgttccagtgagatattttaacacctgatagggaataaatatgcttctgttttggccttcaaaaataagctctgggccagttgcagtggctcacgcctgtaatcccaacactttgggaggccgaggtgggcggatcacgaggtcaggagtttgggatcagcctggccaatatggtgaaactccatctctactaaaaatacaaaaattagccaggcatggtgcctgtaatcccagctacttgggaggctgaaggagaagaatcgcttgaacctgggaggcacaggttgcagtgagccgagatcacaccactgcactccaggccaggtgacagagcgacactctgtctcaaaaaaataaataaatcaactctgtagcatagcatttgtaattctattattttgccttacatttccattatccttttaataaaattgtttttttacatcttcctaatcaagaagtattatgaggccaggcacagtggctcatacctggaatcccagcactttgggaggccgaggcaggcagatcacctgaggtcaaggtatttgagaccagcctggccaacatggtgaaaccccatctctactaaaaatacagaaattagctgggtgtggtggtgcacacctgtaatgctagctactcgggaggctgaggtaggagaatcgcttgaacctgggaggcagaggttgcaataagcctagatcatgccactgcactcaagcctgggagacagagcgagactacatcttaaaaaaaaaaaaaaaagtattatgagagaggataatgtattgtaatgtattgtagaggctaaataaaattatgctcatgtcagaaaaaaagagtatttctcaaaataaaattcactgaaactggatgtttattttgactgagatatagtatatcctcaaattgccatagaaagtttacaagaatattagaggtaaattataaatatcagggcctttttaaaaaaaaaagattctgcttataacttggtatttgtttataataaaaattatagtagccaataatgaacacttactctggcttggttatttacttaggtcaaaagaaggaggagcggttaaactgtgggatcaggaactgaggcggtgccgtgccttcaggcttgagacaggacaagccacagattgtgttcgttctgtgtgcagaggcaaagtaagatgttccatgagctgatacagtgcagcagaaaacagaaagtggttattactgtgattccctcaccctttgcagcctaatgaacaatacttaataatgcataacgatggatttgcttgccaacattactctgtctttgctgctttctttgccaaagttagcaccagtgtggtgcataagctaggaagctattctgtctaaatactgtatgtaaacctccaatattttctagaatctgccaatttaacaactctagtagacataattgaaagcccttggcagttgactcatattaggacagctgtctccattttttaaaaaaacacacattccctagataaaacgtgcagtaaacaaacaatgaaatactactcagccataaaaaataatgaaattctgtcattcttggtggcaacatggatgagactggaggacatgatgtgaagtgaaataagccaggcacagaaagataaatacatgttctcactcctgtgcagaaactaaaaaagttgatcccacagaggtggagagtagaatagtggttactggaggcggacaagggggagggggagggggatagggaaggactggttaaaggatacaagtttacacagccagataggaatagtatgttttagtattctgtagtactgtaggatgactatagttaagaatcacgtatttatgtattttcaggtatttacaagagaggattttgaaagtttccatcacaaagaaatgataaatgtctgaggtgatggttatgcgtattaccctatgccctatagatatgtataattatgtgtcaatttcaaaataaaaattcaaaactacaactcctatgaaaatttttgagcgtgtttgtacttattaagtgtatttataaatcatacggatattatcttcagcctgcatattaaattgtagttaagcttttactttttaactaaaaaataaattctattattttttcctatatcccactgcactgaccccagtttggaaatcctaagattatcaaataaaaactttgattattgaagaatccaggtgtactgccacagaaaagttctattctgtagcatggactctaatatgtaatctagcccattgtgcttacagatagatgtgtgcctgtagtcatagaaaaatttgcatgagctaatgactgccttgctactagattagctcaaagcaaaaagttctctgaaagcaggtcaatagggtcatttttatattatgaagaagaaaagcagctgttgtattacattcactgtattggtcctgcttgtgtttcagggcaagatccttgttgggacaaggaatgctgaaataatcgaagttggagagaaaaatgcagcttgtaatattttagttaacggtcatgtggatgggccaatctggggactagcaacacatccttccagggattttttcctttctgctgcagaagatgggacagtgagactttgggatattgctgataaagtaagtacagataatttttttaaaagaggttacaacttctaaaaagaaaagttggaagttctaaattgctagtacttaaagaactgccagaattctgttgagcattttgaggggaaactggtataatttagaagtacttcacttaatgtttcctatgactctttttttttttttttttaaatgcagaagatgttaaacaaagtgaatttgggacatgctgctcgtactgtgtgttacagccctgaaggggacatggtggctattggaatgaaaaatggagaatttatcattttactagtgagttctctaaaaatatggggaaagaagagagacaggagatgtgcaatccatgatatcaggttagtgaacaaatggaatagagtttctagtatatacttgatttaacttccatttgtaaaattttccatagccttgccttcaaaaagaggtccccagggcctgtagcatttcccgtattataaattgtatgctaaaatatggctgtttgtatactacttaattcttcttgctaaattataaacccactgggcaccaactataatagcaagtactagtaggtaatgtttgatgaattcatgttaacacttagccatgtccattaagttcatcccaccaagaggtatctcccactgtaatacaagagagctatctgcccttcaaaagttgtcaccctggaaaactaaagttgtgatttcaaacatatcttctcttagtaacctcagtttgggaatatgtagttcattaatttaatcaatacctattgattaaatgttccagaatccaaattaatttaaatgtttcttaaacctttgtttttcagtgcttaagcatttttcaacagtggctaccatttacggagtacttccgtgtgatcagtagataagattattgaatctaggtctgtcaaaagcttgtacacttttcatcagtaaaatccttttacaaatgaaaccttcctcagaacttcaatatataaaatagtaacagtggcttcccttagcttttacatgtctctatcgtacctcagtaagactcatgggccatttcaagagactgaattgtcccatatgactccaaagattgctaggcaaatagcatttcactttgtcttttaaataagttcttcaggccgggcgcggtggctcatgcctgtaatcccagcactttgggaggccgaggcaggcagatcacctgaagtcaggagtactcgaccagcctggccaacatagtgaaaccccatctcaactaaaaatacaaaaatcagccgggcgtggtggcaggcgcctgtaatcccagctactcagggggctgaaacaggagaatcgcttgaacccgggaggcggaggttgcgccatcgcactccagcctgggagacaagagcgagacttcgtctcaaaaaaaaaaaattcttcttccaagattcaagttgtgtcatttcaccttaataactggaggttagttaagctgggctgtgttctttgcttaatattaagacaacgttttttccagatggaagaaaactatcttaatgaattgttagcttattaattatgtaatgctaatggcttttaaaagctgagatgttctgactgggtgttgtggctcacacctgtaatcccagtaccttgggaggccaagggggaaggattgcttgaggccaggagtttgggaccatagtgagaccccgcctctatttaaaaaattaaattttgttttgttttgttttgagttggagttttgctcttgttgcccatgctgaagtgcaatggtgcaatctcagctcaccacaacctgtgcctcctgggttcaagcgattctcctgcttcagcctcccgagtagatgggattacaggcgtgcaccaccatgcctggctaattttgtatttttagtagagacagggtttctctatgttggtcaggctggtctcaaactctcgacctcaggtgatctgcccgcctccgcttcccaaagttctgggattataggtgtgagccactgggcctggcctaagaaagtttttttaagccattagacgtttttaaaggaattgggagatgacaattggggaaatatttaaaatttaagtaaaatataaagcttccttatttcatgtaacccagacaatctcagtatacatgatcagttgtgtctgacaggtaaatctatttgaggccttatcacacgttacttttaagaactagaaaggaaaagtcactgatcttaagtatttataatacttcatgtggtctaatactttttacgttttgttttgattcagatttagtccggattcccggtatctggcagtaggttctagtgagaactcagtggatttttatgacctaacgctgggccccactcttaacagaatcagctactgcaaagacattccaagctttgtcattcaaatggacttctctgcagatagcagttatctccaggtacagtaccaatactgtatacccaggtggcaagttcttctgcttttacatttcgtgttagtgaatgcatttaaagttcctgagctccagagctccagcttctcaactcctccctttgtaccttctgacctacagctcccctttcctcccccacttatcagagcttttctcctattaagtttttgtagtgatcttttgcatacttaataatgttagacatgtaaatcaagtagcaatatgctagtattctgtaaaccccctgtggattttgtctctcacctaatggaattcttgtcccattttaatctgatgaaaaaggtctctagtggctgctataaacggcatgtctatgaagtgccttcaggaaaacatcttatggatcatgccgctattgacagaattacttgggctacatggactaggtaaatacttatatattcacaaggcaagaactgactttgaaggccagttagaaaatcctatttctgaactgttagagccattccaataaggaatagtaattgagtttcaagtttttgttaccatattttgaaatggtatgttcatgttgggacccctttttattgaatatatttccatgttttatcagtttccatgatttatcaagttttttttttaaggaaatcaaagttttaactttaaagataccctgatatttttcttaatgctaaatttaatgactggcaaaaaggtattgggtgctgttaagcaactgttattaattctctatctaaaggaatgctatcttgaatctattagaagtcaaagcttccaaatttgttcaaatttcctggctgtatgacaggtaaccatgactatccatttttttggccaatgaaaaatgccatcaaattcctgtatcagccaggcatatagtggctcatgcctgtaatctctgatgtagcaggccgaggtgggaggatcacttgagcctagaagttttgataccagcctgggcaacatagcaagaccccatctctgaaatttttttaattcctatgtcataagtcatttttatttttgtagagatagggatctcacaatattgcccaggctggtctcaaactcttggcctcaagcagtcctcctgcctcagcctcccaaaatgttgggattactggtatgtgctgctggacccagccaagtagcacttttaatttgaaaaatagttctatcagttttcagtcaggcgcggtggctcagcctgtaatcccagcactttgggaggccgagcgggggtgatcacctgaggtcgggagttcgagactagcctgaccaacatggagaaaccctgtctctactaaaaatacaaaataagccgggcatgttagcgcatgcctgtgatcccagctactcgggaggctgaggcaggagaattgcttgaacccaggaggcagaggttgcggtgagccgagatcatgccattgcactccagcctgggtaacaagagcgaaaactccgtctcaaaaaaaaaaaaagaaaaaatagttctatcagttttcataaagtactactttaatcttaaaaagattaatctagaaacccttcaaattataaaatgtcatttttaaaaggcaggagttgatatcctgatgaaattcaggtctccaaacaacttaccataatttacttcctgtattttaagtaacatgatagggtacttagagattaattgccaagaaactttttgaatatagtcaacctgcccgcacttgccatgatgagttttcttttgttccttccctctagtattctaggagatgaggttttgggaatctggtccagacatgctgagaaagctgatgtcaactgtgcctgtgtatctcattcaggaatcagtcttgttacaggagatgactttggcatggttaagttatttgacttcccatgtccagaaaaatttgtaagtttgtgttttgtttactattatcagtttactcctaattttgatgtcttatcatcagcacttttccccatatatttaaaatgttttgtcctaatttctaaatttttccccaaactttctaaatctatttactttgaaataaaagctattagaaacaaatcctctccctcgagtaataccatctttggaaccatcctacaaaagctgtaattagcttttcaccaaacctataatcagttatcaaatttcaaatgcttttccttagagaaaaatggtcagagtacctggagacatctgactgcccacacagcctggttttgcagatccactactcatgctgaaaagcattctaatcactggctgcggtgctaactccctactctctccacagctcttgtcatagagattatagttcctaataagagcctttgacttctgtgtgcaccaaatgccctgagcttgtctgtcattgttttttaggcaaaacacaaaaggttcttgggtcattcgccccatgtgacaaatattcgatttaccagtggtgatcgacatgttgttagtgctggaggtgatgactgcaggttagtaactttctcagcccatgaagagcagactatgttactagttaagagacttaatacaacaactcctacagctttggtttatgaaatcagctagtcaacattagtagaaggtagtataaccagatggctcttcagaatctcatatttatgcaaatacagaataaaaggagttaaagaggaaaaatattacacatgtaacctgaaagcacaactgaaaaatattaaactgttatgaaaatctaaaaacataattaactccctgcaattttcttctctgattgcagcttatttgtctggaaatgtgtacatacacctcactgagagatgctgagatgactacagaaattaactttgagaccagaattacagagaagaaaaaccaaaacccaaccctgcatggtcaagtggtgctaacccaagactgtaacagggagaaatgcccagaatcatcaaaatagtgaaagactgatctgttcaaaatatttgctatatgcactgggtataatccgtaatccatacactgccagataatgccatttcaaggaaggatcgaatacttgatggtaaaggccaagtccccctgtattgggaagtgtgtgatttcggcagacctgctgggaaaatttagggtagagcactctttacagaagaactcaaaaacccaatttggataattttcattatctttttagcaaaatggtttcttaatgtttatattttattttcaaggttcattgtttaatgaaatattttattcttgcatttccataaggaaagggaaagtcatgatcatcctaaaggatcacagtttttaaaaggcaaacattttccctaaggaaacagacacaagctttcctagagaatatgatgttttttaggcattaataaggtccttttttataaaggacacttttctcctagtagttttgaattcaggaacagatccaaagttagcagtatatggctgctacatttccattttcattttcgagccatcagtttatgttcagatgccatctctgtaatcgcacatttaaaacataactgtagcctcactaatggaaaagtagtatgatgaacaatcattcccaatggtgtacaatgtaagggttttagggagcaacagtatttaactggaagaaagaattgcatatttaatgtagtctaatatatacacatttgtttaacatgtaaacaaaagtgttaaattcacatatacaacattatacaatttaatcactcttggaataaaatttttatagccttttttctattgggaaaatttgtttagatgtgtgccactccataggtttatttccaaaatgaatgagcccaactccatttgtaaaaacttgtcagttagaattcctttttttagtggattagggctgaattcttagatccttatttcttttcactttaaatgctgccaaagatcactactcatcattcaggaattcgctgtctagcctatctgtagtttcctgaagattgaaaattatgtagactgctatttaaaaatatatttttctaagtgtgaggtttaagatgctgtattgaccctatgagtttttaatgtgttaattatctttatagcataatagatcgctttaggttcctggaatcccatttggtctgacaggatatatgaagattcttaatacctattttctgtgtctaatacttggttaatactaaaaatagaaatgactaaattacatcacagaaagcataaccagtgattgaacctggtagttttaaagctctaaatagctgtggctgaaggactgattatggggctaagaagcttgaaacgtaagttggtacttgttcatcagtggattctcctaaattaagccaaattttgaaatacatgactattaagtttctactcatgtatttacagtcagtcaataaattaaaggaggaaaaaaatccctgaacaacctgcccataaaaagaaaaatactctacatttgagcctgctgcagttttaaattttccctctgggtcaagtttgccagcttttggctacagagaaattatatttccattacagtgcaggtagaaactctgtaaccttaagcatgtaaactacatagaataaaactgtttccactgcatttctgtccttcaaagtggccaacctgattaagtcagccttaatcactgctgctgtcagtttcacgactaaaggtcatattgactaagtagtcatcagctgaccacctcgctgtatcagccagcaacgaggggaaggtgaagaaacatgataggccatatagaatctgccctatgtttacttttttaacccagataattatttttgtgtgcagtatctaagctcctgattgtgtaacctgggacttctggcaccttttgttccattcattttatgtataaaatgcatgccaaagcacactgtgccctctggtacccttgcttccaatcgccaaccatgctcatttccttcctttttttgtggtccctttttgtggtgatcattttaaaccacgtcatccaacaaatgttttatggtcaaccttagcttgttcataagccatagcaactgaaagattaaactcttaaatatgtgtctgggcagtggctattaaatagcaaaaaacaatcagattttagtattttattatttccttgtaaaatggctgaactaaattaaacccttgtttcccatttgttctataatttatagtgaaactgagaacaaaactatctttataaatgatagctaaaagtatttccagatatttaaacaatttaaaataaatttcttctgcagagatgcaaagcatctcaacactggaatgaacaaatgccttaaattcaatggagtaaacctttagaatgaagaggaactgtcatttcacccaagccgaagacaacagccttatgcacttgtgtgctctgtctttgctgcttctcgtgtttcaagcctttcctgtgggatcagcacagcaaagtgcaacttaccaaatggtttaatgactggttaattctttcttctcccaatggaaaagcaatggcaacacaacagtagactgctggcttgacaatcttaaacgtgagcctttgcacatgtaggtttatcatcatttgagtatacgactaagcaagtcaatgaactttttttttttttttagcagtttaatttggtcctgagaatgttgcagtctttattaccccttttgcattaatccacttttctaaccaccttttaagctttaatttttaacactatacaccaagtctttgaaatcagtgatctgttatttaactctaaagcatttgacacttcttgccttaacagttttaaaaaccacacacaaaaaaactctgtaagtaatacagtaggccaaaagtttcatcctatctatcttgcagtttacctatctgatctgatctctgtaattatagttctgtcatttaaaatatactatttaaatctaatttttacatttcaaaaattatcttcagtagtaactaagtatattttctgtggattctgagaatgttatttttcagaatgtgagaatatatatgtacatttataatcttgtgactttaaagtctgttttcagatacagtatgtaaatacttgtaaaaaaatttgtataattttgtgataatgtagtttcccaaaaaaattatttagaaggcattatgttattagtaaatgagagcactgtatagaactgttcctattttctgcacttgccattccagctgcctccactgtccatacccacctcattcatcctgtcacagaaggcaggaaaactgggaactttaccaaagtagcactcagcctgagaggcctgtataatcatgcttttcaaactaaattcacttaaaaattaaaaagcagaattgaatattttaagcagcctcagtacctttggccaatgctgttttcatggtggattatgaacattatataatctttgggaaaagtgaaagtagtacaatttttagaataatgacaactgcctcactgcatctctccactcacacagcaaccgtgtagccccctaagctgcagtaccatgactaaccatgatgtcaatttcatatgctgatcctcacaacagcagtgcacaaacatgccccaaatattttaacagaatttagctcttccttaagctgtcttttcatagtaaaaacaaaacaaaaacacccaatgttaaaaccacataataaacttacaaacttgaaaaattagacacttcagatagataggcaataaaacttcatattatgaaagcaatatattccaagtttcaaagatttgacaagttctgtagagtatctttcatcagtacatgaaaacttccaaactgcatgatcttctgccaggcaggactgggtgctattcgctggtttgaggtcgaatccatttcaaggcatgtcgtggtgggacattaatggtgggatggtagaatgtgcagtccggtcttgtacattgagtgttaaacctacaatgttttggatgatagaagggacattccatcttcttacaagcagggaagtaacggcagagctgactactggaaggtggtgctggtggtgcaactggttttggagacagtactggaattcttctactcacatgagtgaagggacaatctggtttagtacactttgcatcatatttacaatttgggtgaacaaacaaacatttttcagcaaatttacaattggggaaggctttgcagggtgagatggggtgatggtaggcacactcatccccatttttacaagcaggccagtacttgcagcgctccaaaagtttttctggtttctgtgccacactcagttcactcatctcagcttgactcatctgcagagtttctgccattactgggtcgatttgcagtcgggataataattgcctctgttgagttcctttctcaacgtttctaaggaagccgattatttttacatcagtagttcttgactgtgattcagtatcttcttcttgatcttcaaactgtctgttgcattcatatgttgttgaatattcattcattttaacctccaaagatgaaatttttgcttcattcttggacactctaacatttagatcaaaaagatttgcttccactgtcaaaatagctgctttcattcctttaatttcattgatatcagctgatattttccttaaaaggtgggaaatattgtctagctcattcagtgaacaagaggagcttgttatggaacctaagtccactggctccggtggaagaaaaattggtagaggtggtgatggaaactttgaagacattctcataaaggtgacaggaacctcaaagacattttcataaaattctctcccttaaaatctgataattttttcttcacagctcattaagttatttcatcgaaagtaaaagcagtgatcaaggctgttaccttaagacgtattaagagcaaataacatcttaaaacctgtaattcaaaagatggggttgtacatttctagagtcagaattcaaaactaaatgtgaaaaagctaaacgtaccagaccaattgctcttcgctacaactaagaagccctaatacgtagggccctacatcctctaagtaccatctgtat

SEQ ID NO: 17256 - RNA, 14348 nt, Homo sapiens
  source 1..14348: mol_type = other RNA
tcaggccaggcacagtggctcacacctgtaatcttatcactttgggaggctgaggcaggtggatcgcttgagcccaggagttcaagaccagcctgggcaacatggtgaaaccccatcgctataaaaaacaacaattagccgggtgtggtggcacatgcctgtagtccctgctactcaggaggctgaggtgggaggatcacttgagcctggggaggtcaaggctttagtgagctgtgatggtgccactgcactccagcctgggtgacagagtgagaccccatttaaaaaacaaaaacaaaaacaaaaaaaaatgtgacatatagttgactaagaagtacatttcaatacaggattgaaagaacccacatatgttaattaaacacaagcgcagaatttgtgccttttacataaaggaagaatgcacataggcatgctttcagacaagcaattcatctagcagaaaaggaaggaatacatttttcagcccttccaggaataaaatccataaatgggctctatttcgtcctccaacacttgtatttcccacgtcatttactcctgcacacccccactcactagaagcctgctaaactgttccagtgagatattttaacacctgatagggaataaatatgcttctgttttggccttcaaaaataagctctgggccagttgcagtggctcacgcctgtaatcccaacactttgggaggccgaggtgggcggatcacgaggtcaggagtttgggatcagcctggccaatatggtgaaactccatctctactaaaaatacaaaaattagccaggcatggtgcctgtaatcccagctacttgggaggctgaaggagaagaatcgcttgaacctgggaggcacaggttgcagtgagccgagatcacaccactgcactccaggccaggtgacagagcgacactctgtctcaaaaaaataaataaatcaactctgtagcatagcatttgtaattctattattttgccttacatttccattatccttttaataaaattgtttttttacatcttcctaatcaagaagtattatgaggccaggcacagtggctcatacctggaatcccagcactttgggaggccgaggcaggcagatcacctgaggtcaaggtatttgagaccagcctggccaacatggtgaaaccccatctctactaaaaatacagaaattagctgggtgtggtggtgcacacctgtaatgctagctactcgggaggctgaggtaggagaatcgcttgaacctgggaggcagaggttgcaataagcctagatcatgccactgcactcaagcctgggagacagagcgagactacatcttaaaaaaaaaaaaaaaagtattatgagagaggataatgtattgtaatgtattgtagaggctaaataaaattatgctcatgtcagaaaaaaagagtatttctcaaaataaaattcactgaaactggatgtttattttgactgagatatagtatatcctcaaattgccatagaaagtttacaagaatattagaggtaaattataaatatcagggcctttttaaaaaaaaaagattctgcttataacttggtatttgtttataataaaaattatagtagccaataatgaacacttactctggcttggttatttacttaggtcaaaagaaggaggagcggttaaactgtgggatcaggaactgaggcggtgccgtgccttcaggcttgagacaggacaagccacagattgtgttcgttctgtgtgcagaggcaaagtaagatgttccatgagctgatacagtgcagcagaaaacagaaagtggttattactgtgattccctcaccctttgcagcctaatgaacaatacttaataatgcataacgatggatttgcttgccaacattactctgtctttgctgctttctttgccaaagttagcaccagtgtggtgcataagctaggaagctattctgtctaaatactgtatgtaaacctccaatattttctagaatctgccaatttaacaactctagtagacataattgaaagcccttggcagttgactcatattaggacagctgtctccattttttaaaaaaacacacattccctagataaaacgtgcagtaaacaaacaatgaaatactactcagccataaaaaataatgaaattctgtcattcttggtggcaacatggatgagactggaggacatgatgtgaagtgaaataagccaggcacagaaagataaatacatgttctcactcctgtgcagaaactaaaaaagttgatcccacagaggtggagagtagaatagtggttactggaggcggacaagggggagggggagggggatagggaaggactggttaaaggatacaagtttacacagccagataggaatagtatgttttagtattctgtagtactgtaggatgactatagttaagaatcacgtatttatgtattttcaggtatttacaagagaggattttgaaagtttccatcacaaagaaatgataaatgtctgaggtgatggttatgcgtattaccctatgccctatagatatgtataattatgtgtcaatttcaaaataaaaattcaaaactacaactcctatgaaaatttttgagcgtgtttgtacttattaagtgtatttataaatcatacggatattatcttcagcctgcatattaaattgtagttaagcttttactttttaactaaaaaataaattctattattttttcctatatcccactgcactgaccccagtttggaaatcctaagattatcaaataaaaactttgattattgaagaatccaggtgtactgccacagaaaagttctattctgtagcatggactctaatatgtaatctagcccattgtgcttacagatagatgtgtgcctgtagtcatagaaaaatttgcatgagctaatgactgccttgctactagattagctcaaagcaaaaagttctctgaaagcaggtcaatagggtcatttttatattatgaagaagaaaagcagctgttgtattacattcactgtattggtcctgcttgtgtttcagggcaagatccttgttgggacaaggaatgctgaaataatcgaagttggagagaaaaatgcagcttgtaatattttagttaacggtcatgtggatgggccaatctggggactagcaacacatccttccagggattttttcctttctgctgcagaagatgggacagtgagactttgggatattgctgataaagtaagtacagataatttttttaaaagaggttacaacttctaaaaagaaaagttggaagttctaaattgctagtacttaaagaactgccagaattctgttgagcattttgaggggaaactggtataatttagaagtacttcacttaatgtttcctatgactctttttttttttttttttaaatgcagaagatgttaaacaaagtgaatttgggacatgctgctcgtactgtgtgttacagccctgaaggggacatggtggctattggaatgaaaaatggagaatttatcattttactagtgagttctctaaaaatatggggaaagaagagagacaggagatgtgcaatccatgatatcaggttagtgaacaaatggaatagagtttctagtatatacttgatttaacttccatttgtaaaattttccatagccttgccttcaaaaagaggtccccagggcctgtagcatttcccgtattataaattgtatgctaaaatatggctgtttgtatactacttaattcttcttgctaaattataaacccactgggcaccaactataatagcaagtactagtaggtaatgtttgatgaattcatgttaacacttagccatgtccattaagttcatcccaccaagaggtatctcccactgtaatacaagagagctatctgcccttcaaaagttgtcaccctggaaaactaaagttgtgatttcaaacatatcttctcttagtaacctcagtttgggaatatgtagttcattaatttaatcaatacctattgattaaatgttccagaatccaaattaatttaaatgtttcttaaacctttgtttttcagtgcttaagcatttttcaacagtggctaccatttacggagtacttccgtgtgatcagtagataagattattgaatctaggtctgtcaaaagcttgtacacttttcatcagtaaaatccttttacaaatgaaaccttcctcagaacttcaatatataaaatagtaacagtggcttcccttagcttttacatgtctctatcgtacctcagtaagactcatgggccatttcaagagactgaattgtcccatatgactccaaagattgctaggcaaatagcatttcactttgtcttttaaataagttcttcaggccgggcgcggtggctcatgcctgtaatcccagcactttgggaggccgaggcaggcagatcacctgaagtcaggagtactcgaccagcctggccaacatagtgaaaccccatctcaactaaaaatacaaaaatcagccgggcgtggtggcaggcgcctgtaatcccagctactcagggggctgaaacaggagaatcgcttgaacccgggaggcggaggttgcgccatcgcactccagcctgggagacaagagcgagacttcgtctcaaaaaaaaaaaattcttcttccaagattcaagttgtgtcatttcaccttaataactggaggttagttaagctgggctgtgttctttgcttaatattaagacaacgttttttccagatggaagaaaactatcttaatgaattgttagcttattaattatgtaatgctaatggcttttaaaagctgagatgttctgactgggtgttgtggctcacacctgtaatcccagtaccttgggaggccaagggggaaggattgcttgaggccaggagtttgggaccatagtgagaccccgcctctatttaaaaaattaaattttgttttgttttgttttgagttggagttttgctcttgttgcccatgctgaagtgcaatggtgcaatctcagctcaccacaacctgtgcctcctgggttcaagcgattctcctgcttcagcctcccgagtagatgggattacaggcgtgcaccaccatgcctggctaattttgtatttttagtagagacagggtttctctatgttggtcaggctggtctcaaactctcgacctcaggtgatctgcccgcctccgcttcccaaagttctgggattataggtgtgagccactgggcctggcctaagaaagtttttttaagccattagacgtttttaaaggaattgggagatgacaattggggaaatatttaaaatttaagtaaaatataaagcttccttatttcatgtaacccagacaatctcagtatacatgatcagttgtgtctgacaggtaaatctatttgaggccttatcacacgttacttttaagaactagaaaggaaaagtcactgatcttaagtatttataatacttcatgtggtctaatactttttacgttttgttttgattcagatttagtccggattcccggtatctggcagtaggttctagtgagaactcagtggatttttatgacctaacgctgggccccactcttaacagaatcagctactgcaaagacattccaagctttgtcattcaaatggacttctctgcagatagcagttatctccaggtacagtaccaatactgtatacccaggtggcaagttcttctgcttttacatttcgtgttagtgaatgcatttaaagttcctgagctccagagctccagcttctcaactcctccctttgtaccttctgacctacagctcccctttcctcccccacttatcagagcttttctcctattaagtttttgtagtgatcttttgcatacttaataatgttagacatgtaaatcaagtagcaatatgctagtattctgtaaaccccctgtggattttgtctctcacctaatggaattcttgtcccattttaatctgatgaaaaaggtctctagtggctgctataaacggcatgtctatgaagtgccttcaggaaaacatcttatggatcatgccgctattgacagaattacttgggctacatggactaggtaaatacttatatattcacaaggcaagaactgactttgaaggccagttagaaaatcctatttctgaactgttagagccattccaataaggaatagtaattgagtttcaagtttttgttaccatattttgaaatggtatgttcatgttgggacccctttttattgaatatatttccatgttttatcagtttccatgatttatcaagttttttttttaaggaaatcaaagttttaactttaaagataccctgatatttttcttaatgctaaatttaatgactggcaaaaaggtattgggtgctgttaagcaactgttattaattctctatctaaaggaatgctatcttgaatctattagaagtcaaagcttccaaatttgttcaaatttcctggctgtatgacaggtaaccatgactatccatttttttggccaatgaaaaatgccatcaaattcctgtatcagccaggcatatagtggctcatgcctgtaatctctgatgtagcaggccgaggtgggaggatcacttgagcctagaagttttgataccagcctgggcaacatagcaagaccccatctctgaaatttttttaattcctatgtcataagtcatttttatttttgtagagatagggatctcacaatattgcccaggctggtctcaaactcttggcctcaagcagtcctcctgcctcagcctcccaaaatgttgggattactggtatgtgctgctggacccagccaagtagcacttttaatttgaaaaatagttctatcagttttcagtcaggcgcggtggctcagcctgtaatcccagcactttgggaggccgagcgggggtgatcacctgaggtcgggagttcgagactagcctgaccaacatggagaaaccctgtctctactaaaaatacaaaataagccgggcatgttagcgcatgcctgtgatcccagctactcgggaggctgaggcaggagaattgcttgaacccaggaggcagaggttgcggtgagccgagatcatgccattgcactccagcctgggtaacaagagcgaaaactccgtctcaaaaaaaaaaaaagaaaaaatagttctatcagttttcataaagtactactttaatcttaaaaagattaatctagaaacccttcaaattataaaatgtcatttttaaaaggcaggagttgatatcctgatgaaattcaggtctccaaacaacttaccataatttacttcctgtattttaagtaacatgatagggtacttagagattaattgccaagaaactttttgaatatagtcaacctgcccgcacttgccatgatgagttttcttttgttccttccctctagtattctaggagatgaggttttgggaatctggtccagacatgctgagaaagctgatgtcaactgtgcctgtgtatctcattcaggaatcagtcttgttacaggagatgactttggcatggttaagttatttgacttcccatgtccagaaaaatttgtaagtttgtgttttgtttactattatcagtttactcctaattttgatgtcttatcatcagcacttttccccatatatttaaaatgttttgtcctaatttctaaatttttccccaaactttctaaatctatttactttgaaataaaagctattagaaacaaatcctctccctcgagtaataccatctttggaaccatcctacaaaagctgtaattagcttttcaccaaacctataatcagttatcaaatttcaaatgcttttccttagagaaaaatggtcagagtacctggagacatctgactgcccacacagcctggttttgcagatccactactcatgctgaaaagcattctaatcactggctgcggtgctaactccctactctctccacagctcttgtcatagagattatagttcctaataagagcctttgacttctgtgtgcaccaaatgccctgagcttgtctgtcattgttttttaggcaaaacacaaaaggttcttgggtcattcgccccatgtgacaaatattcgatttaccagtggtgatcgacatgttgttagtgctggaggtgatgactgcaggttagtaactttctcagcccatgaagagcagactatgttactagttaagagacttaatacaacaactcctacagctttggtttatgaaatcagctagtcaacattagtagaaggtagtataaccagatggctcttcagaatctcatatttatgcaaatacagaataaaaggagttaaagaggaaaaatattacacatgtaacctgaaagcacaactgaaaaatattaaactgttatgaaaatctaaaaacataattaactccctgcaattttcttctctgattgcagcttatttgtctggaaatgtgtacatacacctcactgagagatgctgagatgactacagaaattaactttgagaccagaattacagagaagaaaaaccaaaacccaaccctgcatggtcaagtggtgctaacccaagactgtaacagggagaaatgcccagaatcatcaaaatagtgaaagactgatctgttcaaaatatttgctatatgcactgggtataatccgtaatccatacactgccagataatgccatttcaaggaaggatcgaatacttgatggtaaaggccaagtccccctgtattgggaagtgtgtgatttcggcagacctgctgggaaaatttagggtagagcactctttacagaagaactcaaaaacccaatttggataattttcattatctttttagcaaaatggtttcttaatgtttatattttattttcaaggttcattgtttaatgaaatattttattcttgcatttccataaggaaagggaaagtcatgatcatcctaaaggatcacagtttttaaaaggcaaacattttccctaaggaaacagacacaagctttcctagagaatatgatgttttttaggcattaataaggtccttttttataaaggacacttttctcctagtagttttgaattcaggaacagatccaaagttagcagtatatggctgctacatttccattttcattttcgagccatcagtttatgttcagatgccatctctgtaatcgcacatttaaaacataactgtagcctcactaatggaaaagtagtatgatgaacaatcattcccaatggtgtacaatgtaagggttttagggagcaacagtatttaactggaagaaagaattgcatatttaatgtagtctaatatatacacatttgtttaacatgtaaacaaaagtgttaaattcacatatacaacattatacaatttaatcactcttggaataaaatttttatagccttttttctattgggaaaatttgtttagatgtgtgccactccataggtttatttccaaaatgaatgagcccaactccatttgtaaaaacttgtcagttagaattcctttttttagtggattagggctgaattcttagatccttatttcttttcactttaaatgctgccaaagatcactactcatcattcaggaattcgctgtctagcctatctgtagtttcctgaagattgaaaattatgtagactgctatttaaaaatatatttttctaagtgtgaggtttaagatgctgtattgaccctatgagtttttaatgtgttaattatctttatagcataatagatcgctttaggttcctggaatcccatttggtctgacaggatatatgaagattcttaatacctattttctgtgtctaatacttggttaatactaaaaatagaaatgactaaattacatcacagaaagcataaccagtgattgaacctggtagttttaaagctctaaatagctgtggctgaaggactgattatggggctaagaagcttgaaacgtaagttggtacttgttcatcagtggattctcctaaattaagccaaattttgaaatacatgactattaagtttctactcatgtatttacagtcagtcaataaattaaaggaggaaaaaaatccctgaacaacctgcccataaaaagaaaaatactctacatttgagcctgctgcagttttaaattttccctctgggtcaagtttgccagcttttggctacagagaaattatatttccattacagtgcaggtagaaactctgtaaccttaagcatgtaaactacatagaataaaactgtttccactgcatttctgtccttcaaagtggccaacctgattaagtcagccttaatcactgctgctgtcagtttcacgactaaaggtcatattgactaagtagtcatcagctgaccacctcgctgtatcagccagcaacgaggggaaggtgaagaaacatgataggccatatagaatctgccctatgtttacttttttaacccagataattatttttgtgtgcagtatctaagctcctgattgtgtaacctgggacttctggcaccttttgttccattcattttatgtataaaatgcatgccaaagcacactgtgccctctggtacccttgcttccaatcgccaaccatgctcatttccttcctttttttgtggtccctttttgtggtgatcattttaaaccacgtcatccaacaaatgttttatggtcaaccttagcttgttcataagccatagcaactgaaagattaaactcttaaatatgtgtctgggcagtggctattaaatagcaaaaaacaatcagattttagtattttattatttccttgtaaaatggctgaactaaattaaacccttgtttcccatttgttctataatttatagtgaaactgagaacaaaactatctttataaatgatagctaaaagtatttccagatatttaaacaatttaaaataaatttcttctgcagagatgcaaagcatctcaacactggaatgaacaaatgccttaaattcaatggagtaaacctttagaatgaagaggaactgtcatttcacccaagccgaagacaacagccttatgcacttgtgtgctctgtctttgctgcttctcgtgtttcaagcctttcctgtgggatcagcacagcaaagtgcaacttaccaaatggtttaatgactggttaattctttcttctcccaatggaaaagcaatggcaacacaacagtagactgctggcttgacaatcttaaacgtgagcctttgcacatgtaggtttatcatcatttgagtatacgactaagcaagtcaatgaactttttttttttttttagcagtttaatttggtcctgagaatgttgcagtctttattaccccttttgcattaatccacttttctaaccaccttttaagctttaatttttaacactatacaccaagtctttgaaatcagtgatctgttatttaactctaaagcatttgacacttcttgccttaacagttttaaaaaccacacacaaaaaaactctgtaagtaatacagtaggccaaaagtttcatcctatctatcttgcagtttacctatctgatctgatctctgtaattatagttctgtcatttaaaatatactatttaaatctaatttttacatttcaaaaattatcttcagtagtaactaagtatattttctgtggattctgagaatgttatttttcagaatgtgagaatatatatgtacatttataatcttgtgactttaaagtctgttttcagatacagtatgtaaatacttgtaaaaaaatttgtataattttgtgataatgtagtttcccaaaaaaattatttagaaggcattatgttattagtaaatgagagcactgtatagaactgttcctattttctgcacttgccattccagctgcctccactgtccatacccacctcattcatcctgtcacagaaggcaggaaaactgggaactttaccaaagtagcactcagcctgagaggcctgtataatcatgcttttcaaactaaattcacttaaaaattaaaaagcagaattgaatattttaagcagcctcagtacctttggccaatgctgttttcatggtggattatgaacattatataatctttgggaaaagtgaaagtagtacaatttttagaataatgacaactgcctcactgcatctctccactcacacagcaaccgtgtagccccctaagctgcagtaccatgactaaccatgatgtcaatttcatatgctgatcctcacaacagcagtgcacaaacatgccccaaatattttaacagaatttagctcttccttaagctgtcttttcatagtaaaaacaaaacaaaaacacccaatgttaaaaccacataataaacttacaaacttgaaaaattagacacttcagatagataggcaataaaacttcatattatgaaagcaatatattccaagtttcaaagatttgacaagttctgtagagtatctttcatcagtacatgaaaacttccaaactgcatgatcttctgccaggcaggactgggtgctattcgctggtttgaggtcgaatccatttcaaggcatgtcgtggtgggacattaatggtgggatggtagaatgtgcagtccggtcttgtacattgagtgttaaacctacaatgttttggatgatagaagggacattccatcttcttacaagcagggaagtaacggcagagctgactactggaaggtggtgctggtggtgcaactggttttggagacagtactggaattcttctactcacatgagtgaagggacaatctggtttagtacactttgcatcatatttacaatttgggtgaacaaacaaacatttttcagcaaatttacaattggggaaggctttgcagggtgagatggggtgatggtaggcacactcatccccatttttacaagcaggccagtacttgcagcgctccaaaagtttttctggtttctgtgccacactcagttcactcatctcagcttgatttttttctacagaatctccttttgtttcctcttctttaatggggggacttattctgggggtcctactttgtccctggaccacttctgctagcaattcttcttgagaagttcgagttctgggagcaactggaagtgtctgtttctgtggaactgtagagtagttagttgtttttgttacggattcttgagcttcagatatagccttcaaaatcagattcttgttagcttgtttagaaggtggaagagaaggtctcctttcaggctttgcaggcacagacacactgctggagatgcttcctgttcgagacccgtaatcatcatcttcttcctcctcttctccatcatgattgaatttttttactttaacaactgaacttaccacaggcaactttctcttccgaaagttttcatcctccatactcattttctccgagttgtttctaaagaacggactatacgtttcttctaagctgttaagcacctctggttcacacaaacgtcctgtttcatatacccaactactctgcatatcaagctgcttggcagcatgaatactattctgctgctgttgaaattgcaacctgtttaaatgaacaccactatctgcatttctacttgcaggtggtcgataaatttcaatagaagggcgagaagaaccatatgtaagtgtcactgtaggttttttctgagataagggattctcctgcacaaagttgaggtcttcgtcaatgagatcatctggttctggcttaatatcaatcacatcttcagagggtgctggctccctcaaaggtttcactgttgacattagtcgggttgcagctccatcatcgtaagtctgtctgacatttgtggtttttgactcctgcgaacttgtagaaactctggaatctcttttttcaggtctcgcgctaggaatggcaagtggtggcactgcagcttcatgcctcctctcatctccccgactgaaattgctcttgtttgaaggcacgttactatcaaagatgttggtatcagaagacttcagactagagggttcagttgtaacagagcgaagtttatctaatacaccatgaagccaacataagctcctaattcttgtaatttccccttaatggcactccggatcttgcggctgatctcggtgccgatctccatggctctgcggcgtgcgggaactcagcactgcgcggcgcttggcttacccggaggctgccgcggactcctaccccgcagccgggacaccaccgcctcc

SEQ ID NO: 17257 - RNA, 14463 nt, Homo sapiens
  source 1..14463: mol_type = other RNA
tcaggccaggcacagtggctcacacctgtaatcttatcactttgggaggctgaggcaggtggatcgcttgagcccaggagttcaagaccagcctgggcaacatggtgaaaccccatcgctataaaaaacaacaattagccgggtgtggtggcacatgcctgtagtccctgctactcaggaggctgaggtgggaggatcacttgagcctggggaggtcaaggctttagtgagctgtgatggtgccactgcactccagcctgggtgacagagtgagaccccatttaaaaaacaaaaacaaaaacaaaaaaaaatgtgacatatagttgactaagaagtacatttcaatacaggattgaaagaacccacatatgttaattaaacacaagcgcagaatttgtgccttttacataaaggaagaatgcacataggcatgctttcagacaagcaattcatctagcagaaaaggaaggaatacatttttcagcccttccaggaataaaatccataaatgggctctatttcgtcctccaacacttgtatttcccacgtcatttactcctgcacacccccactcactagaagcctgctaaactgttccagtgagatattttaacacctgatagggaataaatatgcttctgttttggccttcaaaaataagctctgggccagttgcagtggctcacgcctgtaatcccaacactttgggaggccgaggtgggcggatcacgaggtcaggagtttgggatcagcctggccaatatggtgaaactccatctctactaaaaatacaaaaattagccaggcatggtgcctgtaatcccagctacttgggaggctgaaggagaagaatcgcttgaacctgggaggcacaggttgcagtgagccgagatcacaccactgcactccaggccaggtgacagagcgacactctgtctcaaaaaaataaataaatcaactctgtagcatagcatttgtaattctattattttgccttacatttccattatccttttaataaaattgtttttttacatcttcctaatcaagaagtattatgaggccaggcacagtggctcatacctggaatcccagcactttgggaggccgaggcaggcagatcacctgaggtcaaggtatttgagaccagcctggccaacatggtgaaaccccatctctactaaaaatacagaaattagctgggtgtggtggtgcacacctgtaatgctagctactcgggaggctgaggtaggagaatcgcttgaacctgggaggcagaggttgcaataagcctagatcatgccactgcactcaagcctgggagacagagcgagactacatcttaaaaaaaaaaaaaaaagtattatgagagaggataatgtattgtaatgtattgtagaggctaaataaaattatgctcatgtcagaaaaaaagagtatttctcaaaataaaattcactgaaactggatgtttattttgactgagatatagtatatcctcaaattgccatagaaagtttacaagaatattagaggtaaattataaatatcagggcctttttaaaaaaaaaagattctgcttataacttggtatttgtttataataaaaattatagtagccaataatgaacacttactctggcttggttatttacttaggtcaaaagaaggaggagcggttaaactgtgggatcaggaactgaggcggtgccgtgccttcaggcttgagacaggacaagccacagattgtgttcgttctgtgtgcagaggcaaagtaagatgttccatgagctgatacagtgcagcagaaaacagaaagtggttattactgtgattccctcaccctttgcagcctaatgaacaatacttaataatgcataacgatggatttgcttgccaacattactctgtctttgctgctttctttgccaaagttagcaccagtgtggtgcataagctaggaagctattctgtctaaatactgtatgtaaacctccaatattttctagaatctgccaatttaacaactctagtagacataattgaaagcccttggcagttgactcatattaggacagctgtctccattttttaaaaaaacacacattccctagataaaacgtgcagtaaacaaacaatgaaatactactcagccataaaaaataatgaaattctgtcattcttggtggcaacatggatgagactggaggacatgatgtgaagtgaaataagccaggcacagaaagataaatacatgttctcactcctgtgcagaaactaaaaaagttgatcccacagaggtggagagtagaatagtggttactggaggcggacaagggggagggggagggggatagggaaggactggttaaaggatacaagtttacacagccagataggaatagtatgttttagtattctgtagtactgtaggatgactatagttaagaatcacgtatttatgtattttcaggtatttacaagagaggattttgaaagtttccatcacaaagaaatgataaatgtctgaggtgatggttatgcgtattaccctatgccctatagatatgtataattatgtgtcaatttcaaaataaaaattcaaaactacaactcctatgaaaatttttgagcgtgtttgtacttattaagtgtatttataaatcatacggatattatcttcagcctgcatattaaattgtagttaagcttttactttttaactaaaaaataaattctattattttttcctatatcccactgcactgaccccagtttggaaatcctaagattatcaaataaaaactttgattattgaagaatccaggtgtactgccacagaaaagttctattctgtagcatggactctaatatgtaatctagcccattgtgcttacagatagatgtgtgcctgtagtcatagaaaaatttgcatgagctaatgactgccttgctactagattagctcaaagcaaaaagttctctgaaagcaggtcaatagggtcatttttatattatgaagaagaaaagcagctgttgtattacattcactgtattggtcctgcttgtgtttcagggcaagatccttgttgggacaaggaatgctgaaataatcgaagttggagagaaaaatgcagcttgtaatattttagttaacggtcatgtggatgggccaatctggggactagcaacacatccttccagggattttttcctttctgctgcagaagatgggacagtgagactttgggatattgctgataaagtaagtacagataatttttttaaaagaggttacaacttctaaaaagaaaagttggaagttctaaattgctagtacttaaagaactgccagaattctgttgagcattttgaggggaaactggtataatttagaagtacttcacttaatgtttcctatgactctttttttttttttttttaaatgcagaagatgttaaacaaagtgaatttgggacatgctgctcgtactgtgtgttacagccctgaaggggacatggtggctattggaatgaaaaatggagaatttatcattttactagtgagttctctaaaaatatggggaaagaagagagacaggagatgtgcaatccatgatatcaggttagtgaacaaatggaatagagtttctagtatatacttgatttaacttccatttgtaaaattttccatagccttgccttcaaaaagaggtccccagggcctgtagcatttcccgtattataaattgtatgctaaaatatggctgtttgtatactacttaattcttcttgctaaattataaacccactgggcaccaactataatagcaagtactagtaggtaatgtttgatgaattcatgttaacacttagccatgtccattaagttcatcccaccaagaggtatctcccactgtaatacaagagagctatctgcccttcaaaagttgtcaccctggaaaactaaagttgtgatttcaaacatatcttctcttagtaacctcagtttgggaatatgtagttcattaatttaatcaatacctattgattaaatgttccagaatccaaattaatttaaatgtttcttaaacctttgtttttcagtgcttaagcatttttcaacagtggctaccatttacggagtacttccgtgtgatcagtagataagattattgaatctaggtctgtcaaaagcttgtacacttttcatcagtaaaatccttttacaaatgaaaccttcctcagaacttcaatatataaaatagtaacagtggcttcccttagcttttacatgtctctatcgtacctcagtaagactcatgggccatttcaagagactgaattgtcccatatgactccaaagattgctaggcaaatagcatttcactttgtcttttaaataagttcttcaggccgggcgcggtggctcatgcctgtaatcccagcactttgggaggccgaggcaggcagatcacctgaagtcaggagtactcgaccagcctggccaacatagtgaaaccccatctcaactaaaaatacaaaaatcagccgggcgtggtggcaggcgcctgtaatcccagctactcagggggctgaaacaggagaatcgcttgaacccgggaggcggaggttgcgccatcgcactccagcctgggagacaagagcgagacttcgtctcaaaaaaaaaaaattcttcttccaagattcaagttgtgtcatttcaccttaataactggaggttagttaagctgggctgtgttctttgcttaatattaagacaacgttttttccagatggaagaaaactatcttaatgaattgttagcttattaattatgtaatgctaatggcttttaaaagctgagatgttctgactgggtgttgtggctcacacctgtaatcccagtaccttgggaggccaagggggaaggattgcttgaggccaggagtttgggaccatagtgagaccccgcctctatttaaaaaattaaattttgttttgttttgttttgagttggagttttgctcttgttgcccatgctgaagtgcaatggtgcaatctcagctcaccacaacctgtgcctcctgggttcaagcgattctcctgcttcagcctcccgagtagatgggattacaggcgtgcaccaccatgcctggctaattttgtatttttagtagagacagggtttctctatgttggtcaggctggtctcaaactctcgacctcaggtgatctgcccgcctccgcttcccaaagttctgggattataggtgtgagccactgggcctggcctaagaaagtttttttaagccattagacgtttttaaaggaattgggagatgacaattggggaaatatttaaaatttaagtaaaatataaagcttccttatttcatgtaacccagacaatctcagtatacatgatcagttgtgtctgacaggtaaatctatttgaggccttatcacacgttacttttaagaactagaaaggaaaagtcactgatcttaagtatttataatacttcatgtggtctaatactttttacgttttgttttgattcagatttagtccggattcccggtatctggcagtaggttctagtgagaactcagtggatttttatgacctaacgctgggccccactcttaacagaatcagctactgcaaagacattccaagctttgtcattcaaatggacttctctgcagatagcagttatctccaggtacagtaccaatactgtatacccaggtggcaagttcttctgcttttacatttcgtgttagtgaatgcatttaaagttcctgagctccagagctccagcttctcaactcctccctttgtaccttctgacctacagctcccctttcctcccccacttatcagagcttttctcctattaagtttttgtagtgatcttttgcatacttaataatgttagacatgtaaatcaagtagcaatatgctagtattctgtaaaccccctgtggattttgtctctcacctaatggaattcttgtcccattttaatctgatgaaaaaggtctctagtggctgctataaacggcatgtctatgaagtgccttcaggaaaacatcttatggatcatgccgctattgacagaattacttgggctacatggactaggtaaatacttatatattcacaaggcaagaactgactttgaaggccagttagaaaatcctatttctgaactgttagagccattccaataaggaatagtaattgagtttcaagtttttgttaccatattttgaaatggtatgttcatgttgggacccctttttattgaatatatttccatgttttatcagtttccatgatttatcaagttttttttttaaggaaatcaaagttttaactttaaagataccctgatatttttcttaatgctaaatttaatgactggcaaaaaggtattgggtgctgttaagcaactgttattaattctctatctaaaggaatgctatcttgaatctattagaagtcaaagcttccaaatttgttcaaatttcctggctgtatgacaggtaaccatgactatccatttttttggccaatgaaaaatgccatcaaattcctgtatcagccaggcatatagtggctcatgcctgtaatctctgatgtagcaggccgaggtgggaggatcacttgagcctagaagttttgataccagcctgggcaacatagcaagaccccatctctgaaatttttttaattcctatgtcataagtcatttttatttttgtagagatagggatctcacaatattgcccaggctggtctcaaactcttggcctcaagcagtcctcctgcctcagcctcccaaaatgttgggattactggtatgtgctgctggacccagccaagtagcacttttaatttgaaaaatagttctatcagttttcagtcaggcgcggtggctcagcctgtaatcccagcactttgggaggccgagcgggggtgatcacctgaggtcgggagttcgagactagcctgaccaacatggagaaaccctgtctctactaaaaatacaaaataagccgggcatgttagcgcatgcctgtgatcccagctactcgggaggctgaggcaggagaattgcttgaacccaggaggcagaggttgcggtgagccgagatcatgccattgcactccagcctgggtaacaagagcgaaaactccgtctcaaaaaaaaaaaaagaaaaaatagttctatcagttttcataaagtactactttaatcttaaaaagattaatctagaaacccttcaaattataaaatgtcatttttaaaaggcaggagttgatatcctgatgaaattcaggtctccaaacaacttaccataatttacttcctgtattttaagtaacatgatagggtacttagagattaattgccaagaaactttttgaatatagtcaacctgcccgcacttgccatgatgagttttcttttgttccttccctctagtattctaggagatgaggttttgggaatctggtccagacatgctgagaaagctgatgtcaactgtgcctgtgtatctcattcaggaatcagtcttgttacaggagatgactttggcatggttaagttatttgacttcccatgtccagaaaaatttgtaagtttgtgttttgtttactattatcagtttactcctaattttgatgtcttatcatcagcacttttccccatatatttaaaatgttttgtcctaatttctaaatttttccccaaactttctaaatctatttactttgaaataaaagctattagaaacaaatcctctccctcgagtaataccatctttggaaccatcctacaaaagctgtaattagcttttcaccaaacctataatcagttatcaaatttcaaatgcttttccttagagaaaaatggtcagagtacctggagacatctgactgcccacacagcctggttttgcagatccactactcatgctgaaaagcattctaatcactggctgcggtgctaactccctactctctccacagctcttgtcatagagattatagttcctaataagagcctttgacttctgtgtgcaccaaatgccctgagcttgtctgtcattgttttttaggcaaaacacaaaaggttcttgggtcattcgccccatgtgacaaatattcgatttaccagtggtgatcgacatgttgttagtgctggaggtgatgactgcaggttagtaactttctcagcccatgaagagcagactatgttactagttaagagacttaatacaacaactcctacagctttggtttatgaaatcagctagtcaacattagtagaaggtagtataaccagatggctcttcagaatctcatatttatgcaaatacagaataaaaggagttaaagaggaaaaatattacacatgtaacctgaaagcacaactgaaaaatattaaactgttatgaaaatctaaaaacataattaactccctgcaattttcttctctgattgcagcttatttgtctggaaatgtgtacatacacctcactgagagatgctgagatgactacagaaattaactttgagaccagaattacagagaagaaaaaccaaaacccaaccctgcatggtcaagtggtgctaacccaagactgtaacagggagaaatgcccagaatcatcaaaatagtgaaagactgatctgttcaaaatatttgctatatgcactgggtataatccgtaatccatacactgccagataatgccatttcaaggaaggatcgaatacttgatggtaaaggccaagtccccctgtattgggaagtgtgtgatttcggcagacctgctgggaaaatttagggtagagcactctttacagaagaactcaaaaacccaatttggataattttcattatctttttagcaaaatggtttcttaatgtttatattttattttcaaggttcattgtttaatgaaatattttattcttgcatttccataaggaaagggaaagtcatgatcatcctaaaggatcacagtttttaaaaggcaaacattttccctaaggaaacagacacaagctttcctagagaatatgatgttttttaggcattaataaggtccttttttataaaggacacttttctcctagtagttttgaattcaggaacagatccaaagttagcagtatatggctgctacatttccattttcattttcgagccatcagtttatgttcagatgccatctctgtaatcgcacatttaaaacataactgtagcctcactaatggaaaagtagtatgatgaacaatcattcccaatggtgtacaatgtaagggttttagggagcaacagtatttaactggaagaaagaattgcatatttaatgtagtctaatatatacacatttgtttaacatgtaaacaaaagtgttaaattcacatatacaacattatacaatttaatcactcttggaataaaatttttatagccttttttctattgggaaaatttgtttagatgtgtgccactccataggtttatttccaaaatgaatgagcccaactccatttgtaaaaacttgtcagttagaattcctttttttagtggattagggctgaattcttagatccttatttcttttcactttaaatgctgccaaagatcactactcatcattcaggaattcgctgtctagcctatctgtagtttcctgaagattgaaaattatgtagactgctatttaaaaatatatttttctaagtgtgaggtttaagatgctgtattgaccctatgagtttttaatgtgttaattatctttatagcataatagatcgctttaggttcctggaatcccatttggtctgacaggatatatgaagattcttaatacctattttctgtgtctaatacttggttaatactaaaaatagaaatgactaaattacatcacagaaagcataaccagtgattgaacctggtagttttaaagctctaaatagctgtggctgaaggactgattatggggctaagaagcttgaaacgtaagttggtacttgttcatcagtggattctcctaaattaagccaaattttgaaatacatgactattaagtttctactcatgtatttacagtcagtcaataaattaaaggaggaaaaaaatccctgaacaacctgcccataaaaagaaaaatactctacatttgagcctgctgcagttttaaattttccctctgggtcaagtttgccagcttttggctacagagaaattatatttccattacagtgcaggtagaaactctgtaaccttaagcatgtaaactacatagaataaaactgtttccactgcatttctgtccttcaaagtggccaacctgattaagtcagccttaatcactgctgctgtcagtttcacgactaaaggtcatattgactaagtagtcatcagctgaccacctcgctgtatcagccagcaacgaggggaaggtgaagaaacatgataggccatatagaatctgccctatgtttacttttttaacccagataattatttttgtgtgcagtatctaagctcctgattgtgtaacctgggacttctggcaccttttgttccattcattttatgtataaaatgcatgccaaagcacactgtgccctctggtacccttgcttccaatcgccaaccatgctcatttccttcctttttttgtggtccctttttgtggtgatcattttaaaccacgtcatccaacaaatgttttatggtcaaccttagcttgttcataagccatagcaactgaaagattaaactcttaaatatgtgtctgggcagtggctattaaatagcaaaaaacaatcagattttagtattttattatttccttgtaaaatggctgaactaaattaaacccttgtttcccatttgttctataatttatagtgaaactgagaacaaaactatctttataaatgatagctaaaagtatttccagatatttaaacaatttaaaataaatttcttctgcagagatgcaaagcatctcaacactggaatgaacaaatgccttaaattcaatggagtaaacctttagaatgaagaggaactgtcatttcacccaagccgaagacaacagccttatgcacttgtgtgctctgtctttgctgcttctcgtgtttcaagcctttcctgtgggatcagcacagcaaagtgcaacttaccaaatggtttaatgactggttaattctttcttctcccaatggaaaagcaatggcaacacaacagtagactgctggcttgacaatcttaaacgtgagcctttgcacatgtaggtttatcatcatttgagtatacgactaagcaagtcaatgaactttttttttttttttagcagtttaatttggtcctgagaatgttgcagtctttattaccccttttgcattaatccacttttctaaccaccttttaagctttaatttttaacactatacaccaagtctttgaaatcagtgatctgttatttaactctaaagcatttgacacttcttgccttaacagttttaaaaaccacacacaaaaaaactctgtaagtaatacagtaggccaaaagtttcatcctatctatcttgcagtttacctatctgatctgatctctgtaattatagttctgtcatttaaaatatactatttaaatctaatttttacatttcaaaaattatcttcagtagtaactaagtatattttctgtggattctgagaatgttatttttcagaatgtgagaatatatatgtacatttataatcttgtgactttaaagtctgttttcagatacagtatgtaaatacttgtaaaaaaatttgtataattttgtgataatgtagtttcccaaaaaaattatttagaaggcattatgttattagtaaatgagagcactgtatagaactgttcctattttctgcacttgccattccagctgcctccactgtccatacccacctcattcatcctgtcacagaaggcaggaaaactgggaactttaccaaagtagcactcagcctgagaggcctgtataatcatgcttttcaaactaaattcacttaaaaattaaaaagcagaattgaatattttaagcagcctcagtacctttggccaatgctgttttcatggtggattatgaacattatataatctttgggaaaagtgaaagtagtacaatttttagaataatgacaactgcctcactgcatctctccactcacacagcaaccgtgtagccccctaagctgcagtaccatgactaaccatgatgtcaatttcatatgctgatcctcacaacagcagtgcacaaacatgccccaaatattttaacagaatttagctcttccttaagctgtcttttcatagtaaaaacaaaacaaaaacacccaatgttaaaaccacataataaacttacaaacttgaaaaattagacacttcagatagataggcaataaaacttcatattatgaaagcaatatattccaagtttcaaagatttgacaagttctgtagagtatctttcatcagtacatgaaaacttccaaactgcatgatcttctgccaggcaggactgggtgctattcgctggtttgaggtcgaatccatttcaaggcatgtcgtggtgggacattaatggtgggatggtagaatgtgcagtccggtcttgtacattgagtgttaaacctacaatgttttggatgatagaagggacattccatcttcttacaagcagggaagtaacggcagagctgactactggaaggtggtgctggtggtgcaactggttttggagacagtactggaattcttctactcacatgagtgaagggacaatctggtttagtacactttgcatcatatttacaatttgggtgaacaaacaaacatttttcagcaaatttacaattggggaaggctttgcagggtgagatggggtgatggtaggcacactcatccccatttttacaagcaggccagtacttgcagcgctccaaaagtttttctggtttctgtgccacactcagttcactcatctcagcttgatttttttctacagaatctccttttgtttcctcttctttaatggggggacttattctgggggtcctactttgtccctggaccacttctgctagcaattcttcttgagaagttcgagttctgggagcaactggaagtgtctgtttctgtggaactgtagagtagttagttgtttttgttacggattcttgagcttcagatatagccttcaaaatcagattcttgttagcttgtttagaaggtggaagagaaggtctcctttcaggctttgcaggcacagacacactgctggagatgcttcctgttcgagacccgtaatcatcatcttcttcctcctcttctccatcatgattgaatttttttactttaacaactgaacttaccacaggcaactttctcttccgaaagttttcatcctccatactcattttctccgagttgtttctaaagaacggactatacgtttcttctaagctgttaagcacctctggttcacacaaacgtcctgtttcatatacccaactactctgcatatcaagctgcttggcagcatgaatactattctgctgctgttgaaattgcaacctgtttaaatgaacaccactatctgcatttctacttgcaggtggtcgataaatttcaatagaagggcgagaagaaccatatgtaagtgtcactgtaggttttttctgagataagggattctcctgcacaaagttgaggtcttcgtcaatgagatcatctggttctggcttaatatcaatcacatcttcagagggtgctggctccctcaaaggtttcactgttgacattagtcgggttgcagctccatcatcgtaagtctgtctgacatttgtggtttttgactcctgcgaacttgtagaaactctggaatctcttttttcaggtctcgcgctaggaatggcaagtggtggcactgcagcttcatgcctcctctcatctccccgactgaaattgctcttgtttgaaggcacgttactatcaaagatgttggtatcagaagacttcagactagagggttcagttgtaacagagcgaagtttatctaatacaccatgaagccatacggtgaatcgaattgtgttgttccctagaaacagggacagatcctctgtcatttggtcctgacttttcttgttggccaccatcaccataatgtaatcaggaagttcttcatcaacataagctcctaattcttgtaatttccccttaatggcactccggatcttgcggctgatctcggtgccgatctccatggctctgcggcgtgcgggaactcagcactgcgcggcgcttggcttacccggaggctgccgcggactcctaccccgcagccgggacaccaccgcctcc

SEQ ID NO: 17258 - RNA, 14644 nt, Homo sapiens
  source 1..14644: mol_type = other RNA
tcaggccaggcacagtggctcacacctgtaatcttatcactttgggaggctgaggcaggtggatcgcttgagcccaggagttcaagaccagcctgggcaacatggtgaaaccccatcgctataaaaaacaacaattagccgggtgtggtggcacatgcctgtagtccctgctactcaggaggctgaggtgggaggatcacttgagcctggggaggtcaaggctttagtgagctgtgatggtgccactgcactccagcctgggtgacagagtgagaccccatttaaaaaacaaaaacaaaaacaaaaaaaaatgtgacatatagttgactaagaagtacatttcaatacaggattgaaagaacccacatatgttaattaaacacaagcgcagaatttgtgccttttacataaaggaagaatgcacataggcatgctttcagacaagcaattcatctagcagaaaaggaaggaatacatttttcagcccttccaggaataaaatccataaatgggctctatttcgtcctccaacacttgtatttcccacgtcatttactcctgcacacccccactcactagaagcctgctaaactgttccagtgagatattttaacacctgatagggaataaatatgcttctgttttggccttcaaaaataagctctgggccagttgcagtggctcacgcctgtaatcccaacactttgggaggccgaggtgggcggatcacgaggtcaggagtttgggatcagcctggccaatatggtgaaactccatctctactaaaaatacaaaaattagccaggcatggtgcctgtaatcccagctacttgggaggctgaaggagaagaatcgcttgaacctgggaggcacaggttgcagtgagccgagatcacaccactgcactccaggccaggtgacagagcgacactctgtctcaaaaaaataaataaatcaactctgtagcatagcatttgtaattctattattttgccttacatttccattatccttttaataaaattgtttttttacatcttcctaatcaagaagtattatgaggccaggcacagtggctcatacctggaatcccagcactttgggaggccgaggcaggcagatcacctgaggtcaaggtatttgagaccagcctggccaacatggtgaaaccccatctctactaaaaatacagaaattagctgggtgtggtggtgcacacctgtaatgctagctactcgggaggctgaggtaggagaatcgcttgaacctgggaggcagaggttgcaataagcctagatcatgccactgcactcaagcctgggagacagagcgagactacatcttaaaaaaaaaaaaaaaagtattatgagagaggataatgtattgtaatgtattgtagaggctaaataaaattatgctcatgtcagaaaaaaagagtatttctcaaaataaaattcactgaaactggatgtttattttgactgagatatagtatatcctcaaattgccatagaaagtttacaagaatattagaggtaaattataaatatcagggcctttttaaaaaaaaaagattctgcttataacttggtatttgtttataataaaaattatagtagccaataatgaacacttactctggcttggttatttacttaggtcaaaagaaggaggagcggttaaactgtgggatcaggaactgaggcggtgccgtgccttcaggcttgagacaggacaagccacagattgtgttcgttctgtgtgcagaggcaaagtaagatgttccatgagctgatacagtgcagcagaaaacagaaagtggttattactgtgattccctcaccctttgcagcctaatgaacaatacttaataatgcataacgatggatttgcttgccaacattactctgtctttgctgctttctttgccaaagttagcaccagtgtggtgcataagctaggaagctattctgtctaaatactgtatgtaaacctccaatattttctagaatctgccaatttaacaactctagtagacataattgaaagcccttggcagttgactcatattaggacagctgtctccattttttaaaaaaacacacattccctagataaaacgtgcagtaaacaaacaatgaaatactactcagccataaaaaataatgaaattctgtcattcttggtggcaacatggatgagactggaggacatgatgtgaagtgaaataagccaggcacagaaagataaatacatgttctcactcctgtgcagaaactaaaaaagttgatcccacagaggtggagagtagaatagtggttactggaggcggacaagggggagggggagggggatagggaaggactggttaaaggatacaagtttacacagccagataggaatagtatgttttagtattctgtagtactgtaggatgactatagttaagaatcacgtatttatgtattttcaggtatttacaagagaggattttgaaagtttccatcacaaagaaatgataaatgtctgaggtgatggttatgcgtattaccctatgccctatagatatgtataattatgtgtcaatttcaaaataaaaattcaaaactacaactcctatgaaaatttttgagcgtgtttgtacttattaagtgtatttataaatcatacggatattatcttcagcctgcatattaaattgtagttaagcttttactttttaactaaaaaataaattctattattttttcctatatcccactgcactgaccccagtttggaaatcctaagattatcaaataaaaactttgattattgaagaatccaggtgtactgccacagaaaagttctattctgtagcatggactctaatatgtaatctagcccattgtgcttacagatagatgtgtgcctgtagtcatagaaaaatttgcatgagctaatgactgccttgctactagattagctcaaagcaaaaagttctctgaaagcaggtcaatagggtcatttttatattatgaagaagaaaagcagctgttgtattacattcactgtattggtcctgcttgtgtttcagggcaagatccttgttgggacaaggaatgctgaaataatcgaagttggagagaaaaatgcagcttgtaatattttagttaacggtcatgtggatgggccaatctggggactagcaacacatccttccagggattttttcctttctgctgcagaagatgggacagtgagactttgggatattgctgataaagtaagtacagataatttttttaaaagaggttacaacttctaaaaagaaaagttggaagttctaaattgctagtacttaaagaactgccagaattctgttgagcattttgaggggaaactggtataatttagaagtacttcacttaatgtttcctatgactctttttttttttttttttaaatgcagaagatgttaaacaaagtgaatttgggacatgctgctcgtactgtgtgttacagccctgaaggggacatggtggctattggaatgaaaaatggagaatttatcattttactagtgagttctctaaaaatatggggaaagaagagagacaggagatgtgcaatccatgatatcaggttagtgaacaaatggaatagagtttctagtatatacttgatttaacttccatttgtaaaattttccatagccttgccttcaaaaagaggtccccagggcctgtagcatttcccgtattataaattgtatgctaaaatatggctgtttgtatactacttaattcttcttgctaaattataaacccactgggcaccaactataatagcaagtactagtaggtaatgtttgatgaattcatgttaacacttagccatgtccattaagttcatcccaccaagaggtatctcccactgtaatacaagagagctatctgcccttcaaaagttgtcaccctggaaaactaaagttgtgatttcaaacatatcttctcttagtaacctcagtttgggaatatgtagttcattaatttaatcaatacctattgattaaatgttccagaatccaaattaatttaaatgtttcttaaacctttgtttttcagtgcttaagcatttttcaacagtggctaccatttacggagtacttccgtgtgatcagtagataagattattgaatctaggtctgtcaaaagcttgtacacttttcatcagtaaaatccttttacaaatgaaaccttcctcagaacttcaatatataaaatagtaacagtggcttcccttagcttttacatgtctctatcgtacctcagtaagactcatgggccatttcaagagactgaattgtcccatatgactccaaagattgctaggcaaatagcatttcactttgtcttttaaataagttcttcaggccgggcgcggtggctcatgcctgtaatcccagcactttgggaggccgaggcaggcagatcacctgaagtcaggagtactcgaccagcctggccaacatagtgaaaccccatctcaactaaaaatacaaaaatcagccgggcgtggtggcaggcgcctgtaatcccagctactcagggggctgaaacaggagaatcgcttgaacccgggaggcggaggttgcgccatcgcactccagcctgggagacaagagcgagacttcgtctcaaaaaaaaaaaattcttcttccaagattcaagttgtgtcatttcaccttaataactggaggttagttaagctgggctgtgttctttgcttaatattaagacaacgttttttccagatggaagaaaactatcttaatgaattgttagcttattaattatgtaatgctaatggcttttaaaagctgagatgttctgactgggtgttgtggctcacacctgtaatcccagtaccttgggaggccaagggggaaggattgcttgaggccaggagtttgggaccatagtgagaccccgcctctatttaaaaaattaaattttgttttgttttgttttgagttggagttttgctcttgttgcccatgctgaagtgcaatggtgcaatctcagctcaccacaacctgtgcctcctgggttcaagcgattctcctgcttcagcctcccgagtagatgggattacaggcgtgcaccaccatgcctggctaattttgtatttttagtagagacagggtttctctatgttggtcaggctggtctcaaactctcgacctcaggtgatctgcccgcctccgcttcccaaagttctgggattataggtgtgagccactgggcctggcctaagaaagtttttttaagccattagacgtttttaaaggaattgggagatgacaattggggaaatatttaaaatttaagtaaaatataaagcttccttatttcatgtaacccagacaatctcagtatacatgatcagttgtgtctgacaggtaaatctatttgaggccttatcacacgttacttttaagaactagaaaggaaaagtcactgatcttaagtatttataatacttcatgtggtctaatactttttacgttttgttttgattcagatttagtccggattcccggtatctggcagtaggttctagtgagaactcagtggatttttatgacctaacgctgggccccactcttaacagaatcagctactgcaaagacattccaagctttgtcattcaaatggacttctctgcagatagcagttatctccaggtacagtaccaatactgtatacccaggtggcaagttcttctgcttttacatttcgtgttagtgaatgcatttaaagttcctgagctccagagctccagcttctcaactcctccctttgtaccttctgacctacagctcccctttcctcccccacttatcagagcttttctcctattaagtttttgtagtgatcttttgcatacttaataatgttagacatgtaaatcaagtagcaatatgctagtattctgtaaaccccctgtggattttgtctctcacctaatggaattcttgtcccattttaatctgatgaaaaaggtctctagtggctgctataaacggcatgtctatgaagtgccttcaggaaaacatcttatggatcatgccgctattgacagaattacttgggctacatggactaggtaaatacttatatattcacaaggcaagaactgactttgaaggccagttagaaaatcctatttctgaactgttagagccattccaataaggaatagtaattgagtttcaagtttttgttaccatattttgaaatggtatgttcatgttgggacccctttttattgaatatatttccatgttttatcagtttccatgatttatcaagttttttttttaaggaaatcaaagttttaactttaaagataccctgatatttttcttaatgctaaatttaatgactggcaaaaaggtattgggtgctgttaagcaactgttattaattctctatctaaaggaatgctatcttgaatctattagaagtcaaagcttccaaatttgttcaaatttcctggctgtatgacaggtaaccatgactatccatttttttggccaatgaaaaatgccatcaaattcctgtatcagccaggcatatagtggctcatgcctgtaatctctgatgtagcaggccgaggtgggaggatcacttgagcctagaagttttgataccagcctgggcaacatagcaagaccccatctctgaaatttttttaattcctatgtcataagtcatttttatttttgtagagatagggatctcacaatattgcccaggctggtctcaaactcttggcctcaagcagtcctcctgcctcagcctcccaaaatgttgggattactggtatgtgctgctggacccagccaagtagcacttttaatttgaaaaatagttctatcagttttcagtcaggcgcggtggctcagcctgtaatcccagcactttgggaggccgagcgggggtgatcacctgaggtcgggagttcgagactagcctgaccaacatggagaaaccctgtctctactaaaaatacaaaataagccgggcatgttagcgcatgcctgtgatcccagctactcgggaggctgaggcaggagaattgcttgaacccaggaggcagaggttgcggtgagccgagatcatgccattgcactccagcctgggtaacaagagcgaaaactccgtctcaaaaaaaaaaaaagaaaaaatagttctatcagttttcataaagtactactttaatcttaaaaagattaatctagaaacccttcaaattataaaatgtcatttttaaaaggcaggagttgatatcctgatgaaattcaggtctccaaacaacttaccataatttacttcctgtattttaagtaacatgatagggtacttagagattaattgccaagaaactttttgaatatagtcaacctgcccgcacttgccatgatgagttttcttttgttccttccctctagtattctaggagatgaggttttgggaatctggtccagacatgctgagaaagctgatgtcaactgtgcctgtgtatctcattcaggaatcagtcttgttacaggagatgactttggcatggttaagttatttgacttcccatgtccagaaaaatttgtaagtttgtgttttgtttactattatcagtttactcctaattttgatgtcttatcatcagcacttttccccatatatttaaaatgttttgtcctaatttctaaatttttccccaaactttctaaatctatttactttgaaataaaagctattagaaacaaatcctctccctcgagtaataccatctttggaaccatcctacaaaagctgtaattagcttttcaccaaacctataatcagttatcaaatttcaaatgcttttccttagagaaaaatggtcagagtacctggagacatctgactgcccacacagcctggttttgcagatccactactcatgctgaaaagcattctaatcactggctgcggtgctaactccctactctctccacagctcttgtcatagagattatagttcctaataagagcctttgacttctgtgtgcaccaaatgccctgagcttgtctgtcattgttttttaggcaaaacacaaaaggttcttgggtcattcgccccatgtgacaaatattcgatttaccagtggtgatcgacatgttgttagtgctggaggtgatgactgcaggttagtaactttctcagcccatgaagagcagactatgttactagttaagagacttaatacaacaactcctacagctttggtttatgaaatcagctagtcaacattagtagaaggtagtataaccagatggctcttcagaatctcatatttatgcaaatacagaataaaaggagttaaagaggaaaaatattacacatgtaacctgaaagcacaactgaaaaatattaaactgttatgaaaatctaaaaacataattaactccctgcaattttcttctctgattgcagcttatttgtctggaaatgtgtacatacacctcactgagagatgctgagatgactacagaaattaactttgagaccagaattacagagaagaaaaaccaaaacccaaccctgcatggtcaagtggtgctaacccaagactgtaacagggagaaatgcccagaatcatcaaaatagtgaaagactgatctgttcaaaatatttgctatatgcactgggtataatccgtaatccatacactgccagataatgccatttcaaggaaggatcgaatacttgatggtaaaggccaagtccccctgtattgggaagtgtgtgatttcggcagacctgctgggaaaatttagggtagagcactctttacagaagaactcaaaaacccaatttggataattttcattatctttttagcaaaatggtttcttaatgtttatattttattttcaaggttcattgtttaatgaaatattttattcttgcatttccataaggaaagggaaagtcatgatcatcctaaaggatcacagtttttaaaaggcaaacattttccctaaggaaacagacacaagctttcctagagaatatgatgttttttaggcattaataaggtccttttttataaaggacacttttctcctagtagttttgaattcaggaacagatccaaagttagcagtatatggctgctacatttccattttcattttcgagccatcagtttatgttcagatgccatctctgtaatcgcacatttaaaacataactgtagcctcactaatggaaaagtagtatgatgaacaatcattcccaatggtgtacaatgtaagggttttagggagcaacagtatttaactggaagaaagaattgcatatttaatgtagtctaatatatacacatttgtttaacatgtaaacaaaagtgttaaattcacatatacaacattatacaatttaatcactcttggaataaaatttttatagccttttttctattgggaaaatttgtttagatgtgtgccactccataggtttatttccaaaatgaatgagcccaactccatttgtaaaaacttgtcagttagaattcctttttttagtggattagggctgaattcttagatccttatttcttttcactttaaatgctgccaaagatcactactcatcattcaggaattcgctgtctagcctatctgtagtttcctgaagattgaaaattatgtagactgctatttaaaaatatatttttctaagtgtgaggtttaagatgctgtattgaccctatgagtttttaatgtgttaattatctttatagcataatagatcgctttaggttcctggaatcccatttggtctgacaggatatatgaagattcttaatacctattttctgtgtctaatacttggttaatactaaaaatagaaatgactaaattacatcacagaaagcataaccagtgattgaacctggtagttttaaagctctaaatagctgtggctgaaggactgattatggggctaagaagcttgaaacgtaagttggtacttgttcatcagtggattctcctaaattaagccaaattttgaaatacatgactattaagtttctactcatgtatttacagtcagtcaataaattaaaggaggaaaaaaatccctgaacaacctgcccataaaaagaaaaatactctacatttgagcctgctgcagttttaaattttccctctgggtcaagtttgccagcttttggctacagagaaattatatttccattacagtgcaggtagaaactctgtaaccttaagcatgtaaactacatagaataaaactgtttccactgcatttctgtccttcaaagtggccaacctgattaagtcagccttaatcactgctgctgtcagtttcacgactaaaggtcatattgactaagtagtcatcagctgaccacctcgctgtatcagccagcaacgaggggaaggtgaagaaacatgataggccatatagaatctgccctatgtttacttttttaacccagataattatttttgtgtgcagtatctaagctcctgattgtgtaacctgggacttctggcaccttttgttccattcattttatgtataaaatgcatgccaaagcacactgtgccctctggtacccttgcttccaatcgccaaccatgctcatttccttcctttttttgtggtccctttttgtggtgatcattttaaaccacgtcatccaacaaatgttttatggtcaaccttagcttgttcataagccatagcaactgaaagattaaactcttaaatatgtgtctgggcagtggctattaaatagcaaaaaacaatcagattttagtattttattatttccttgtaaaatggctgaactaaattaaacccttgtttcccatttgttctataatttatagtgaaactgagaacaaaactatctttataaatgatagctaaaagtatttccagatatttaaacaatttaaaataaatttcttctgcagagatgcaaagcatctcaacactggaatgaacaaatgccttaaattcaatggagtaaacctttagaatgaagaggaactgtcatttcacccaagccgaagacaacagccttatgcacttgtgtgctctgtctttgctgcttctcgtgtttcaagcctttcctgtgggatcagcacagcaaagtgcaacttaccaaatggtttaatgactggttaattctttcttctcccaatggaaaagcaatggcaacacaacagtagactgctggcttgacaatcttaaacgtgagcctttgcacatgtaggtttatcatcatttgagtatacgactaagcaagtcaatgaactttttttttttttttagcagtttaatttggtcctgagaatgttgcagtctttattaccccttttgcattaatccacttttctaaccaccttttaagctttaatttttaacactatacaccaagtctttgaaatcagtgatctgttatttaactctaaagcatttgacacttcttgccttaacagttttaaaaaccacacacaaaaaaactctgtaagtaatacagtaggccaaaagtttcatcctatctatcttgcagtttacctatctgatctgatctctgtaattatagttctgtcatttaaaatatactatttaaatctaatttttacatttcaaaaattatcttcagtagtaactaagtatattttctgtggattctgagaatgttatttttcagaatgtgagaatatatatgtacatttataatcttgtgactttaaagtctgttttcagatacagtatgtaaatacttgtaaaaaaatttgtataattttgtgataatgtagtttcccaaaaaaattatttagaaggcattatgttattagtaaatgagagcactgtatagaactgttcctattttctgcacttgccattccagctgcctccactgtccatacccacctcattcatcctgtcacagaaggcaggaaaactgggaactttaccaaagtagcactcagcctgagaggcctgtataatcatgcttttcaaactaaattcacttaaaaattaaaaagcagaattgaatattttaagcagcctcagtacctttggccaatgctgttttcatggtggattatgaacattatataatctttgggaaaagtgaaagtagtacaatttttagaataatgacaactgcctcactgcatctctccactcacacagcaaccgtgtagccccctaagctgcagtaccatgactaaccatgatgtcaatttcatatgctgatcctcacaacagcagtgcacaaacatgccccaaatattttaacagaatttagctcttccttaagctgtcttttcatagtaaaaacaaaacaaaaacacccaatgttaaaaccacataataaacttacaaacttgaaaaattagacacttcagatagataggcaataaaacttcatattatgaaagcaatatattccaagtttcaaagatttgacaagttctgtagagtatctttcatcagtacatgaaaacttccaaactgcatgatcttctgccaggcaggactgggtgctattcgctggtttgaggtcgaatccatttcaaggcatgtcgtggtgggacattaatggtgggatggtagaatgtgcagtccggtcttgtacattgagtgttaaacctacaatgttttggatgatagaagggacattccatcttcttacaagcagggaagtaacggcagagctgactactggaaggtggtgctggtggtgcaactggttttggagacagtactggaattcttctactcacatgagtgaagggacaatctggtttagtacactttgcatcatatttacaatttgggtgaacaaacaaacatttttcagcaaatttacaattggggaaggctttgcagggtgagatggggtgatggtaggcacactcatccccatttttacaagcaggccagtacttgcagcgctccaaaagtttttctggtttctgtgccacactcagttcactcatctcagcttgatttttttctacagaatctccttttgtttcctcttctttaatggggggacttattctgggggtcctactttgtccctggaccacttctgctagcaattcttcttgagaagttcgagttctgggagcaactggaagtgtctgtttctgtggaactgtagagtagttagttgtttttgttacggattcttgagcttcagatatagccttcaaaatcagattcttgttagcttgtttagaaggtggaagagaaggtctcctttcaggctttgcaggcacagacacactgctggagatgcttcctgttcgagacccgtaatcatcatcttcttcctcctcttctccatcatgattgaatttttttactttaacaactgaacttaccacaggcaactttctcttccgaaagttttcatcctccatactcattttctccgagttgtttctaaagaacggactatacgtttcttctaagctgttaagcacctctggttcacacaaacgtcctgtttcatatacccaactactctgcatatcaagctgcttggcagcatgaatactattctgctgctgttgaaattgcaacctgtttaaatgaacaccactatctgcatttctacttgcaggtggtcgataaatttcaatagaagggcgagaagaaccatatgtaagtgtcactgtaggttttttctgagataagggattctcctgcacaaagttgaggtcttcgtcaatgagatcatctggttctggcttaatatcaatcacatcttcagagggtgctggctccctcaaaggtttcactgttgacattagtcgggttgcagctccatcatcgtaagtctgtctgacatttgtggtttttgactcctgcgaacttgtagaaactctggaatctcttttttcaggtctcgcgctaggaatggcaagtggtggcactgcagcttcatgcctcctctcatctccccgactgaaattgctcttgtttgaaggcacgttactatcaaagatgttggtatcagaagacttcagactagagggttcagttgtaacagagcgaagtttatctaatacaccatgaagccatacggtgaatcgaattgtgttgttccctagaaacagggacagatcctctgtcatttggtcctgacttttcttgttggccaccatcaccataatgtaatcaggaagttcttcatctatttaaaaggaaaggtagatcaaaactttgtttcctcaaaactttcttcttaaagttgatgtgcttgaaaatatagatgtagctctaagctttagagtcgcagagctctactggaattacattggacaagatggcttagctttaatttttttctcttcattccacaggtatttcaaatacaacataagctcctaattcttgtaatttccccttaatggcactccggatcttgcggctgatctcggtgccgatctccatggctctgcggcgtgcgggaactcagcactgcgcggcgcttggcttacccggaggctgccgcggactcctaccccgcagccgggacaccaccgcctcc

SEQ ID NO: 17259 - RNA, 211 nt, Homo sapiens
  source 1..211: mol_type = other RNA
tcaggccaggcacagtggctcacacctgtgatcgcagcactttgggaggctgaggctggaggattgatcacttaagcccaggagttcaagaccagactgagcaacatagcaagattccatctctatttaaaaaaaaaattgagtcataaaacttacaattatgtaaattatattattattttttgagacagggtctcactctatcacccag

SEQ ID NO: 17260 - RNA, 26 nt, Homo sapiens
  source 1..26: mol_type = other RNA
tcaggccaggcacagtggctcacact

SEQ ID NO: 17261 - RNA, 5321 nt, Homo sapiens
  source 1..5321: mol_type = other RNA
tcaggccaggcacagtggctcacacttgtaatcccagcactttaggaggccgaggccaggagcttgagaccagctggagaacatagtgagatcctgtctctacaaaaaaatttaaaaatacatactttttagacaggtgtggtagatcacacctggtgcctggtggctcccagcattttgggaggctgaggacaggaggatcatctgagcccaggagttcaagaccagcctaggcaacagagcaagactccatctctaaaaaactaaaaacattagccaggtgtagtggcacacacctatagttgcagctacatgggaggccagggcaagaggatcgcctgagcctaggagtttgaggctgcagtgagctacagactgcaccactgcactccagccagtagattagaaatgtttgtgagaaggtaccttaatggatgggcaagatggacagcagctatagtaattattcatagcagcactctagaaataaaaactagatcttatgtggcagggctgtgaaaatgcttttgtcaaaatttaaaattacagattaacacctatgaggctgcaggcacaggggtcacgctgatgaaggcataaaccctgctctcaagtagctcacatccagtgaaaggctcaaaccacaaacagggaagtacgtgagattaattcgttcaaggatcaaacaaatgcctcttttcacccgatgccacatttcattaaatagtttgtagcagtgatactataaaatgtgagctttaaagaactctggtaacattttcaatctcttcctttctccgtactcttctatttccccccaatttctccaatccactcctaattttcacttgtatctttcttctacaaaaaacctaaatatgccaattttactcttcttccttccagttagtaaaatcaatgaaatcacaatttgaaacaaaattataagttgtcacacaatatgaaaaatatgaaattcctgatgattcaagtagttttgatctataaaagcagcaatttcatgattcatcagtcactcccaagtccttgcttttataatttttaaatgtggattttatatatttagaaattaagtacaatggcagcaatatgactatatattggcaagtaacctggtgatttccaatttataaatctgagagctgtttcccatacctgaagcctaacagccaatctgatccaaatccaatctttctgtcactgtcagctacttattaaaataataagatttcatttctacttggaaacaaaatctttaacctgagtttccagtattcaaaatattgctatttagatgtcggatgcttaacatttcatgccaaagtctcacgtgaatgatctgacataagatagaacatactactcagcaacaaaaaaaatgcacaactgacacacagggatcaatctcaaaaatctgcagagaggaagaaggcaaagtacatactacagtattctatttacatgaattctacaatggatagatctaatcggtaaccaaaagcaaatctgtggctgcctagggctaggggtagaggaattgattgggaaagggggtatgagaattttgggggcaatgaaaatatttgtatcttgatcgtgatagtggctgcacagaggtatgaatctgtcaaaacccaataaaatacacacgtaaaaagggtgcaataaatctaagtaaatagtacctcaattcagttgatttacaaaacacaacatgacagtatattttaaattaaatgaaacattaagaccttattttttaaaaaaattaatgttatggataaagctaaagttccctctgaccaccctcccaatcctgatttgcacccctaatctctcatctatacctcctactcgctgttagaactttggtatggattcctctgaacctttaaaaatagatttacgtacattatatagccatagagaatgcatagtattgttttgtacatatatataatttgtatataactttctacaacttgctattttcactgagcattatgtttttgagaccaatccaggttaatatggatctagattatttcttttaactccaatacaataatctatcctatgactacatcatattttaattaggccattcctcttcaatatttagattgtttttccctactacaattcaccagtgtagtggtaaacagtagtcaccactggggtgaggacagaaccgcaggtggtgttctaagggttattagccttatttataagatgtagttataagatgagaatgtattcatgtttaatttacatatgataaatattgacttaaagaattttgagatacatatattagcaaaacgaacaaaacaacatcagttataggaagcaaatcatctaataaaatataaggaaaacaaagttgtagggcctaatagtgtactcatggtttgaagcatatttactggaaaataataagcactaaacagatcataaaaaaaataataagcactaaacagatcataaaaacattctcctatgcaaaggaattccaattaatatatctgtatattggttatcatggcgtaagcataattaatataggtacaagtacttcatttatattttttgctttcttcttttatgactatggtgtctttccccatccctctctttccttcttctcgactcacagtttttatccttatctttgtttctttttcttttatgtgggcttctactcctatcccttctatgtcgtgaacactcagcatccaaatagcttccaccagactgccgtgaatctactgaagctgatcgcctttcttcattcttttcggcatcatcctctgccttctcttgctcttcttgccaatgattgctgagttcttccatgtgcacatttatcacatctcgaatcacctcagtatatgatttcttggttatgtgaacattcttggctctataggactggcgtcttcttttataatctcgtacttctgccaggatttcaaggtaggattttggactttttcgactattgtcttgattgattttggcagccaagtctacaaagagatcgctgtcattttcaataatttgagaatcagagcgctttttctttgtctcctcaactacgaaatcatagagggcaagacgatcagcttgagttagatcacaaacaaaccgtttgtgattcaaaggaacttcaacaggcaatgaagaataaattcctaaagtaaaaataaaatcacaagaataaacaatacatgaagcattgtgaacttaaaatctaataattatctttaaacatgtgctttaataatgcaatattaacacaaacttttttcataatccctaagtatacaaaatatcaatctaagcaataaatgacaaacaattctatcctgaatgttatatccacaaaaaaaaaaaaaatgtattatggatgtttgctattctctccaacaatataaagacagatcccatggaggcaggcaggaataatcataagagacaatttgctctaagaaagccttttgggtaacaatttttatagccatctacaaaagtaggtatctgttgatatgcttttccccatcaaagttgggggaaaaaatgcttttaataagtaatatgcattacagtccctttgaaaataaactatggaaatattaaaaactgtgtaaaaaatatctttttgtatgagacatcaagctagatggtcaatattcaaaatatatcccacttgtgcaaggacttagagctaggggccacaaaataattaagtagcagaaatcccacacctcctcacgccaggaaagcacagattaaattaaactcattttaatttcctgaggaggaagcatagtggcttaaccaaattaattgaaaaaagttaatagcagtgccccccggtagttacagaattttctaaaatctgctcattagtgaaaaaaagtaaatacaataccttgatatgatgtattaaacattgaagaaaatttttgttttgagattcaaattttctcaaataaaaaaatgattggaactgtaaaaaaagcaatttaaaacaattctttctagacttcattactcactaatgcaaacaaagaacatgagctactaaaggaatccttttattgtttgctaacttattctaaagtagtaactggttcatagaacaacataaaatcagtagctctttccagatacttatatttgataaagtctaacctcattaagttcctaggtagaggcaaaaagaattcaaataagagcatactatgaactaagcattacaacaaaaaagaggtactacttgtctacatattaagaggagagctgcagtgaatctgaggccatggtttaacacggctatacataacaatatatggccatttttactcgtcaaagggttttgaattaatggggaaaaaagggttccctttcaagtcaatcaattttattctaattatagtaggcatttcataatacaaaattataaaaacagctttgataagcctaattcctttgaattaggctataaaaatttgggaggaaaacacagattagaaaataatgatgtattacaaacaagcttcatataaacctttgcctgttatttttaaacaaagaaatataatttccttcttaaattattttagccttttcttcaatttattcatcttaaatttctttatgatgaagactgatacttaaattccttgtaattcaaccaaaattccaattcaagactataatatgtgacaggtattaagataaagtttagaaattttacttttaaaaggatatcatttgcaaaaaggatactgcatatctttaaataaggagtacattcaggttcctaattcctctttatactcaccccaattatttgattataacaatcactgtctttcccaactgcagttctagcttgtttaattatctggaattgtgagtccttattcaaagtaatcgaaggtatcttcacattttcatagaaaaactcaggattatacatttcatcctcttcttctttggtatagcccattttcctcaatctacaagatgccatgtgctttgccaaagatgatttaggcatgtgatgattggaatcgtatggacatatcacaacttcatcctccgccgcctcctcttccccgggatccagactatctaggtcccagcccagggacgcggtcacctcctccaacgtccggcagccgctctccacgaactcgttcagctcctcctgcagccgccgccgctcctccacaggtggaggctcgccctccatagctgcagcccacccgccaagaggaagcggccgaact

SEQ ID NO: 17262 - RNA, 3681 nt, Homo sapiens
  source 1..3681: mol_type = other RNA
tcaggccaggcacagtggctcacacttgtaatcccagcactttaggaggccgaggccaggagcttgagaccagctggagaacatagtgagatcctgtctctacaaaaaaatttaaaaatacatactttttagacaggtgtggtagatcacacctggtgcctggtggctcccagcattttgggaggctgaggacaggaggatcatctgagcccaggagttcaagaccagcctaggcaacagagcaagactccatctctaaaaaactaaaaacattagccaggtgtagtggcacacacctatagttgcagctacatgggaggccagggcaagaggatcgcctgagcctaggagtttgaggctgcagtgagctacagactgcaccactgcactccagccagtagattagaaatgtttgtgagaaggtaccttaatggatgggcaagatggacagcagctatagtaattattcatagcagcactctagaaataaaaactagatcttatgtggcagggctgtgaaaatgcttttgtcaaaatttaaaattacagattaacacctatgaggctgcaggcacaggggtcacgctgatgaaggcataaaccctgctctcaagtagctcacatccagtgaaaggctcaaaccacaaacagggaagtacgtgagattaattcgttcaaggatcaaacaaatgcctcttttcacccgatgccacatttcattaaatagtttgtagcagtgatactataaaatgtgagctttaaagaactctggtaacattttcaatctcttcctttctccgtactcttctatttccccccaatttctccaatccactcctaattttcacttgtatctttcttctacaaaaaacctaaatatgccaattttactcttcttccttccagttagtaaaatcaatgaaatcacaatttgaaacaaaattataagttgtcacacaatatgaaaaatatgaaattcctgatgattcaagtagttttgatctataaaagcagcaatttcatgattcatcagtcactcccaagtccttgcttttataatttttaaatgtggattttatatatttagaaattaagtacaatggcagcaatatgactatatattggcaagtaacctggtgatttccaatttataaatctgagagctgtttcccatacctgaagcctaacagccaatctgatccaaatccaatctttctgtcactgtcagctacttattaaaataataagatttcatttctacttggaaacaaaatctttaacctgagtttccagtattcaaaatattgctatttagatgtcggatgcttaacatttcatgccaaagtctcacgtgaatgatctgacataagatagaacatactactcagcaacaaaaaaaatgcacaactgacacacagggatcaatctcaaaaatctgcagagaggaagaaggcaaagtacatactacagtattctatttacatgaattctacaatggatagatctaatcggtaaccaaaagcaaatctgtggctgcctagggctaggggtagaggaattgattgggaaagggggtatgagaattttgggggcaatgaaaatatttgtatcttgatcgtgatagtggctgcacagaggtatgaatctgtcaaaacccaataaaatacacacgtaaaaagggtgcaataaatctaagtaaatagtacctcaattcagttgatttacaaaacacaacatgacagtatattttaaattaaatgaaacattaagaccttattttttaaaaaaattaatgttatggataaagctaaagttccctctgaccaccctcccaatcctgatttgcacccctaatctctcatctatacctcctactcgctgttagaactttggtatggattcctctgaacctttaaaaatagatttacgtacattatatagccatagagaatgcatagtattgttttgtacatatatataatttgtatataactttctacaacttgctattttcactgagcattatgtttttgagaccaatccaggttaatatggatctagattatttcttttaactccaatacaataatctatcctatgactacatcatattttaattaggccattcctcttcaatatttagattgtttttccctactacaattcaccagtgtagtggtaaacagtagtcaccactggggtgaggacagaaccgcaggtggtgttctaagggttattagccttatttataagatgtagttataagatgagaatgtattcatgtttaatttacatatgataaatattgacttaaagaattttgagatacatatattagcaaaacgaacaaaacaacatcagttataggaagcaaatcatctaataaaatataaggaaaacaaagttgtagggcctaatagtgtactcatggtttgaagcatatttactggaaaataataagcactaaacagatcataaaaaaaataataagcactaaacagatcataaaaacattctcctatgcaaaggaattccaattaatatatctgtatattggttatcatggcgtaagcataattaatataggtacaagtacttcatttatattttttgctttcttcttttatgactatggtgtctttccccatccctctctttccttcttctcgactcacagtttttatccttatctttgtttctttttcttttatgtgggcttctactcctatcccttctatgtcgtgaacactcagcatccaaatagcttccaccagactgccgtgaatctactgaagctgatcgcctttcttcattcttttcggcatcatcctctgccttctcttgctcttcttgccaatgattgctgagttcttccatgtgcacatttatcacatctcgaatcacctcagtatatgatttcttggttatgtgaacattcttggctctataggactggcgtcttcttttataatctcgtacttctgccaggatttcaaggtaggattttggactttttcgactattgtcttgattgattttggcagccaagtctacaaagagatcgctgtcattttcaataatttgagaatcagagcgctttttctttgtctcctcaactacgaaatcatagagggcaagacgatcagcttgagttagatcacaaacaaaccgtttgtgattcaaaggaacttcaacaggcaatgaagaataaattctttgattataacaatcactgtctttcccaactgcagttctagcttgtttaattatctggaattgtgagtccttattcaaagtaatcgaaggtatcttcacattttcatagaaaaactcaggattatacatttcatcctcttcttctttggtatagcccattttcctcaatctacaagatgccatgtgctttgccaaagatgatttaggcatgtgatgattggaatcgtatggacatatcacaacttcatcctccgccgcctcctcttccccgggatccagactatctaggtcccagcccagggacgcggtcacctcctccaacgtccggcagccgctctccacgaactcgttcagctcctcctgcagccgccgccgctcctccacaggtggaggctcgccctccatagctgcagcccacccgccaagaggaagcggccgaactgcagaccgcacgcgcaggcctct

SEQ ID NO: 17263 - RNA, 3616 nt, Homo sapiens
  source 1..3616: mol_type = other RNA
tcaggccaggcacagtggctcacacttgtaatcccagcactttaggaggccgaggccaggagcttgagaccagctggagaacatagtgagatcctgtctctacaaaaaaatttaaaaatacatactttttagacaggtgtggtagatcacacctggtgcctggtggctcccagcattttgggaggctgaggacaggaggatcatctgagcccaggagttcaagaccagcctaggcaacagagcaagactccatctctaaaaaactaaaaacattagccaggtgtagtggcacacacctatagttgcagctacatgggaggccagggcaagaggatcgcctgagcctaggagtttgaggctgcagtgagctacagactgcaccactgcactccagccagtagattagaaatgtttgtgagaaggtaccttaatggatgggcaagatggacagcagctatagtaattattcatagcagcactctagaaataaaaactagatcttatgtggcagggctgtgaaaatgcttttgtcaaaatttaaaattacagattaacacctatgaggctgcaggcacaggggtcacgctgatgaaggcataaaccctgctctcaagtagctcacatccagtgaaaggctcaaaccacaaacagggaagtacgtgagattaattcgttcaaggatcaaacaaatgcctcttttcacccgatgccacatttcattaaatagtttgtagcagtgatactataaaatgtgagctttaaagaactctggtaacattttcaatctcttcctttctccgtactcttctatttccccccaatttctccaatccactcctaattttcacttgtatctttcttctacaaaaaacctaaatatgccaattttactcttcttccttccagttagtaaaatcaatgaaatcacaatttgaaacaaaattataagttgtcacacaatatgaaaaatatgaaattcctgatgattcaagtagttttgatctataaaagcagcaatttcatgattcatcagtcactcccaagtccttgcttttataatttttaaatgtggattttatatatttagaaattaagtacaatggcagcaatatgactatatattggcaagtaacctggtgatttccaatttataaatctgagagctgtttcccatacctgaagcctaacagccaatctgatccaaatccaatctttctgtcactgtcagctacttattaaaataataagatttcatttctacttggaaacaaaatctttaacctgagtttccagtattcaaaatattgctatttagatgtcggatgcttaacatttcatgccaaagtctcacgtgaatgatctgacataagatagaacatactactcagcaacaaaaaaaatgcacaactgacacacagggatcaatctcaaaaatctgcagagaggaagaaggcaaagtacatactacagtattctatttacatgaattctacaatggatagatctaatcggtaaccaaaagcaaatctgtggctgcctagggctaggggtagaggaattgattgggaaagggggtatgagaattttgggggcaatgaaaatatttgtatcttgatcgtgatagtggctgcacagaggtatgaatctgtcaaaacccaataaaatacacacgtaaaaagggtgcaataaatctaagtaaatagtacctcaattcagttgatttacaaaacacaacatgacagtatattttaaattaaatgaaacattaagaccttattttttaaaaaaattaatgttatggataaagctaaagttccctctgaccaccctcccaatcctgatttgcacccctaatctctcatctatacctcctactcgctgttagaactttggtatggattcctctgaacctttaaaaatagatttacgtacattatatagccatagagaatgcatagtattgttttgtacatatatataatttgtatataactttctacaacttgctattttcactgagcattatgtttttgagaccaatccaggttaatatggatctagattatttcttttaactccaatacaataatctatcctatgactacatcatattttaattaggccattcctcttcaatatttagattgtttttccctactacaattcaccagtgtagtggtaaacagtagtcaccactggggtgaggacagaaccgcaggtggtgttctaagggttattagccttatttataagatgtagttataagatgagaatgtattcatgtttaatttacatatgataaatattgacttaaagaattttgagatacatatattagcaaaacgaacaaaacaacatcagttataggaagcaaatcatctaataaaatataaggaaaacaaagttgtagggcctaatagtgtactcatggtttgaagcatatttactggaaaataataagcactaaacagatcataaaaaaaataataagcactaaacagatcataaaaacattctcctatgcaaaggaattccaattaatatatctgtatattggttatcatggcgtaagcataattaatataggtacaagtacttcatttatattttttgctttcttcttttatgactatggtgtctttccccatccctctctttccttcttctcgactcacagtttttatccttatctttgtttctttttcttttatgtgggcttctactcctatcccttctatgtcgtgaacactcagcatccaaatagcttccaccagactgccgtgaatctactgaagctgatcgcctttcttcattcttttcggcatcatcctctgccttctcttgctcttcttgccaatgattgctgagttcttccatgtgcacatttatcacatctcgaatcacctcagtatatgatttcttggttatgtgaacattcttggctctataggactggcgtcttcttttataatctcgtacttctgccaggatttcaaggtaggattttggactttttcgactattgtcttgattgattttggcagccaagtctacaaagagatcgctgtcattttcaataatttgagaatcagagcgctttttctttgtctcctcaactacgaaatcatagagggcaagacgatcagcttgagttagatcacaaacaaaccgtttgtgattcaaaggaacttcaacaggcaatgaagaataaattctttgattataacaatcactgtctttcccaactgcagttctagcttgtttaattatctggaattgtgagtccttattcaaagtaatcgaaggtatcttcacattttcatagaaaaactcaggattatacatttcatcctcttcttctttggtatagcccattttcctcaatctacaagatgccatgtgctttgccaaagatgatttaggcatgtgatgattggaatcgtatggacatatcacaacttcatcctcctccaacgtccggcagccgctctccacgaactcgttcagctcctcctgcagccgccgccgctcctccacaggtggaggctcgccctccatagctgcagcccacccgccaagaggaagcggccgaactgcagaccgcacgcgcaggcct

SEQ ID NO: 17264 - RNA, 736 nt, Homo sapiens
  source 1..736: mol_type = other RNA
tcaggccaggcacagtggctcacacttgtaatcccagcactttgggaggctgaggcaggagaatcatttgaacccagaaggcggagattgcagtgagctgagatggcgccactgcactccagcctgggcgacagagcaagagactcaaaaaagagacccagaccaggattacgaatgaggcaatttattaacccagcatggtttgttctaatgcttcttgttggcagctgccacctgtccggcgattctgtccagatctctttgtccctgaggtgtcagtttgcggccgccatcttggtccttttccaccattttcagcccctccagggcttggaggacccggcgggccacactcttggagcctcggctgaagtggctgggcatgacgccgtttctctgacgtcccccatagatcttggtcatggagccaaccccagcgccaccccggaggtacaggtgccgcgctgtggaagcagctcgcgtgtagaaccagttctcatcgtagggagcaagctctttgtgcttggccagcttgacggtatccacccattcggggactttcagcttcccggactttttgaggaaggctgccagagctctgacgaactcctgctggttcacgtcttttacagtaactccaggcatcccgccgctgccccccggggcccacgctcggttcccggacggcgctgaccgggcatgtccgggcctgccgctcgcacgtggccgcggctct

SEQ ID NO: 17265 - RNA, 836 nt, Homo sapiens
  source 1..836: mol_type = other RNA
tcaggccaggcacagtggctcacacttgtaatcccagcactttgggaggctgaggcaggagaatcatttgaacccagaaggcggagattgcagtgagctgagatggcgccactgcactccagcctgggcgacagagcaagagactcaaaaaagagacccagaccaggattacgaatgaggcaatttattaacccagcatggtttgttctaatgcttcttgttggcagctgccacctgtccggcgattctgtccagatctctttgtccctgaggtgtcagtttgcggccgccatcttggtccttttccaccattttcagcccctccagggcttggaggacccggcgggccacactcttggagcctcggctgaagtggctgggcatgacgccgtttctctgacgtcccccatagatcttggtcatggagccaaccccagcgccaccccggaggtacaggtgccgcgctgtggaagcagctcgcgtgtagaaccagttctcatcgtagggagcaagctctttgtgcttggccagcttgacggtatccacccattcggggactttcagcttcccggactttttgaggaaggctgccagagctctgacgaactcctgctggttcacgtcttttacagtaactccaggcatcgggcatgtccgggcctgccgctcgcacgtggccgcggctctagggggcgggacgggcccgcgccgggcgcctcggggccctcaggcacgcgctctgaggcttcggcgtccggccctgccgcctcgcgcccggtccagctcggagcccccgcttaccgtgcggcctccgcgctgccagccaggggaaaggg

SEQ ID NO: 17266 - RNA, 680 nt, Homo sapiens
  source 1..680: mol_type = other RNA
tcaggccaggcacagtggctcacacttgtaatcccagcactttgggaggctgaggcaggagaatcatttgaacccagaaggcggagattgcagtgagctgagatggcgccactgcactccagcctgggcgacagagcaagagactcaaaaaagagacccagaccaggattacgaatgaggcaatttattaacccagcatggtttgttctaatgcttcttgttggcagctgccacctgtccggcgattctgtccagatctctttgtccctgaggtgtcagtttgcggccgccatcttggtccttttccaccattttcagcccctccagggcttggaggacccggcgggccacactcttggagcctcggctgaagtggctgggcatgacgccgtttctctgacgtcccccatagatcttggtcatggagccaaccccagcgccaccccggaggtacaggtgccgcgctgtggaagcagctcgcgtgtagaaccagttctcatcgtagggagcaagctctttgtgcttggccagcttgacggtatccacccattcggggactttcagcttcccggactttttgaggaaggctgccagagctctgacgaactcctgctggttcacgtcttttacagtaactccaggcatcgtgcggcctccgcgctgccagccaggggaaaggg

SEQ ID NO: 17267 - RNA, 693 nt, Homo sapiens
  source 1..693: mol_type = other RNA
tcaggccaggcacagtggctcacacttgtaatcccagcactttgggaggctgaggcaggagaatcatttgaacccagaaggcggagattgcagtgagctgagatggcgccactgcactccagcctgggcgacagagcaagagactcaaaaaagagacccagaccaggattacgaatgaggcaatttattaacccagcatggtttgttctaatgcttcttgttggcagctgccacctgtccggcgattctgtccagatctctttgtccctgaggtgtcagtttgcggccgccatcttggtccttttccaccattttcagcccctccagggcttggaggacccggcgggccacactcttggagcctcggctgaagtggctgggcatgacgccgtttctctgacgtcccccatagatcttggtcatggagccaaccccagcgccaccccggaggtacaggtgccgcgctgtggaagctaagttcctcaccagctcgcgtgtagaaccagttctcatcgtagggagcaagctctttgtgcttggccagcttgacggtatccacccattcggggactttcagcttcccggactttttgaggaaggctgccagagctctgacgaactcctgctggttcacgtcttttacagtaactccaggcatcgtgcggcctccgcgctgccagccaggggaaaggg

SEQ ID NO: 17268 - RNA, 71 nt, Homo sapiens
  source 1..71: mol_type = other RNA
tcaggccaggcacagtggctcacacttgtaatcccagcactttgggaggctgaggcaggcagatcatttga

SEQ ID NO: 17269 - RNA, 289 nt, Homo sapiens
  source 1..289: mol_type = other RNA
tcaggccaggcacagtggctcacacttgtaattccaacactttgggaggccaaggcaggaggagaccagcctgggcagcagagtgagatcccatcttctgttccttcaaattggaatgtccttcagcctccacatctacaacaatggctggaattgtctccgttcttcaaggcctgattataattccatcatcttcatgtaaccttttttttttttcttcatcctactcttcaactgatggagcacaaagtctcaagtgatccgcctgcctcggcctcccaaagtgctg

SEQ ID NO: 17270 - RNA, 353 nt, Homo sapiens
  source 1..353: mol_type = other RNA
tcaggccaggcacagtggctcacagctgtaatcccagcacttagggaagacaaggcaggaatgattgaggccaggagttagagaccagcctgggcaacacagtgagacccatcttataaaataagtttactggtggtaatgtgatggaatttattccggatatctgatgttataaactttagggtccctgaaatatgcaggatccttgtatgtaactggcataaaccccattgtttgagctctcttaattgcttttgtgatttgtttcttcccacaaagacccgcgcgactgtgtccacggatggcacgaaagccaagcgagtccccctgccgagctactcgcgtccgcctcc

SEQ ID NO: 17271 - RNA, 5447 nt, Homo sapiens
  source 1..5447: mol_type = other RNA
tcaggccaggcacagtggctcacagtgcctgtaatcccagcattttgggagcctgaggtgggtggaccacttgaggtcaggagttcgagaccagcctggccaatatgacaaaactttgtctctaccaaaaatacaaaaattagccaggaatggtggcacacacctgcaatcccagctacttgggaggctgaggcaggagaattgcttgaactggggaggtggaggttgcagtgagccaaaattgagccactgcactacagcctgggtgacagggcaagactccatctcaaaaaaacaaataaaataaaataataaaatgtaatatagatttacattaattaaatcagcttgctactgaactaatctcagaagacattgcgccaagtgaaaaaagccaccctcaacaggctatttgctgtatgattctacctatatgacaatcttgaaaaagcaaactctaagagcacagtcagatggctactgtcaaggacaggaaatgggaaggaggaggtgactactgtgggggacaggagcatttttgggttgatgaaactgttctatctctgagatttgataattatataactatgggcatttgtcaacaatccagccaattaccctgaattgttcattatacattctttgcttgcatcaaaacatctccagtacctcataaatatgtgcaactattatatattcataataattaaaaataaattttaaaaaattaaaataataaaaaataaattgctataaaagctcacaaaaccatacactaaagagtcattttttctatatgtaaactgtacttgaaaaatgaaacaaaaagcttaatatttgtactatgaattgattgtagggttctctgaagtgtcaatcttcccttctcccttgtgagtcctgaacaaattcataggtagaattgtgaataggaagagacaaatatcagtattattactggtaaagttgcactggacttaaaaccccaagagtcttcctactactttcccttaattttaaccctgggatccccttaaatagagagtttgcagaacaaacatttagctgggcagagacaaggataattctaaagtgcacattctggctaggcacagtggctcacgcctgtaatcccagcactttgggaggccaacgtgagtggattacctaatgtcaggagttcgagactaccctggccaacatgcccaaaccctgtctctactaaaaatacaaaaatgagccaggcgcagtggtgggcgcctgtaatcccagctactcagggggctgagagaggagaatcacttgaactcgggaggcggaggttgcggtgagcagagattgcgccactgcactccagcctgggcaacagagtgatactccgtctcaaataaataaataaataaaataaattacacattcctccaagagcagaggaccctgacaggaagacagtttgaggtgttaacaaatttgcccatggaaaacaggtgctaccccttaactggggtttagaactgtgtgcctcggctcctctgaaacagcaatactgtaaaacgccgagaacctcatgctcagtctcgtttccaaatttcagtcatctataaatcacatcacgtgcttagaaggagagcaagtgaatggcaggcagaaggagggcggtgcctctactggctgtcagggtgagggtttctgtattatatgcttgatagtagctagcatgttgggagagggaaaaaataactccttctaataaagacagttcacaaatttcacataacaaggggacagggtagattatttttcaaataatactgttttgaaaattagctaaattatttgggaaaaatattgagtagttagtagctttctctggcataagaaatacataatagtagttggtagcttttttcttgacataagaaatacataaataacttacaaataatttatatcacaaattcgtgacaatttgctcaacaaattgtcagtcacatcaaccaatcaataatagccttttaaaaacaaaactctagattatattaaacctatgggtattttcatagtatgtgttcagaaaagagctatttctagttagatataatataaccagcttaaaatataaccagctgaagtctcccccgcctccccccaccccgagcccccaacacacccacccatgcccacctccccgctcagaggctgaaaacaagtgcagcaaggtgtggtaaaaggaaagcaattttattcaaatgcaagcaggtgggggatggccaggctcatgcctttaacagaccattccccgtttgggggctaagtaaaggagtttaagacggaaaagatatgggaaatatgtgggaatagtgcaggaacgtgcaggtctgcgtgttttgttctgaaggttatcttgagtgatggtctgtcctgaggcctgatttgccttttcctgactttggcctggtagtggtgggttaactgtaagtaattcccctctcaagggaggattctgcagccaggtttccctgccttgtttgtttcaaaatcggcccctaggatttctaagcaagtccttaattagataagaaacactgtgtatgaatgtacctggtgggaaagggagacaaagtcttacaacacaaggctacattctgagattcagaaagaaagaaaaaaaaagtttgaaaatgcattttgaggctgggatccttggtcacaataattcaacttgtacacaaaatgttttctccataaaattggttgctcagtatgaaacaactaaggctgatgtgactgtgccctttatgtaacaaatgatctaaaaaataacatgttagagacctagtactcaatgttttatcttctgtctctggaatggcttttctggatactaggtataatatatccaataaaaggcataaagttctttttggatttatgctgaagttgaaagacagtagacatcttctcccatacccagttgccttaaatttgctttagccttcaagtcagttacaggcctagttgcctagattgcaaagagaaatatgaacagagctaagaagggggagataaacttggaatagaagcagtacaatgtacaagttgggacaggaatggtctatgcttactttttttccttcctgtctctcttttaaatttcagcatgacacagttttgaattccaaagagtgtcctatattttctattatatgatcagactacatttgacctacctctctatctcatctctcaacatcatagcccatgacccagctcaatgaaattatgtataggttctccactgtgtcatgcttctatgcattctcaacatactatttctttctcgtggaatgtctttcttttccatctagctgatgctaactataagtggaaaccttcctgccctgccctgattgagatgccattcctgcactctcaaagcaccctgtccatcatgtaacagtgctgttcgtgccatggaacaactgccaatttagtttgctcgatctatccataggctgtaagttccttgaaggcctggctatatcttctggcattctgtaggctcacaaaatatgtgaagaatggtgaacacactgtgtttatggaaaacaacttagtataatttaatacacactaatcagggattacccagaacatgcagttttctagcctgtaaggcacttggataaataaccgtgatgagatgtcatctgtgtgctttctctaaacatagattaccaataacaacaacaaaaaacctaacaataataatgtgttttctgaggtttaagagcatgctaaaataataatgaaagatgcatataaacaaggttgtatagacgaaaaaactaaatcacagggaacttatttattttcttcaaatttgcaccagagaaactgataaaggtgggatttaaatgtatacaagccaaactgtagatattatgtgtttgaccataaaagatcacaaaaaggtgtttgctttttaacaattacatctactatttcctcatatggaacttgaactgttagctggtacacaagttatagtggtttttgccattactttaattttgtcatttactttaatggcaaaaaccgcaatgacttttgcacgaacctgatacattaaaaacgagtttcttaaatgttcaaacaaacaagagagtgtctcttcaaaagtctcatctaaaaagtatgctttaaatttatatgcagagtctttttttaatggctgcttttacctcttgatttcttaatgtataaataataggatttaagagaggtgtgaaaattgtgtaaaacacagaaagaattttatctaccgagtatctgctgaagggccagacgtagataaagacacacggagcaaagaacagagtcacaactgtgatgtgagctgagagagtggagaaagccttagaggatcgactagcagcacggtacctaactgagaatattatgactccataggagacaagcaagaggaggaagcagaccagtgacaggagcccactgtcagcaatgaccaggagctgtaggatgtaggtgtccttgcaggcaagtttaatcacaaggggaaggtcacagaaaaagctgtctataacattgggaccacagaagggcaaagtcaacatgaaagccatttgactagatgagtgcacaaatccaactgcataggaggataacagtagcccagtgagcacccgtgggctcatgatggtcatgtaatggaggggtttgcatatggcaacatacctgtctattgccatggctacaagcaacatcatctcactcccacccaggaggtgcataaagaacatctgggaataacatccccaccatgagatggtcttacgttctcggaggaaatctacaatcatcttaggggtagcaaaagaagccaggatcatatcaatgcaggagaggttgctaagcagaaaatacattggtgtgtgaaggagcgaatcaaaggtcacagtcaccaagatgagcaggtttcctaacacaatccccacgaagaccacagagaatcccaagaagaataaaatctgaagattttgagatttggaaagtcccaacaaaataaattccgataccactgaatggtttgctctttccatatcgtcaactttatcccataatgatcaaaataagtgagaataaggggtagggaaatgatgcatattggaaagaaatgttcatgttgatgtccacatttggtactcagtcaaggcacttgaacttacaaggacccttacttttgtggaattttgtcagtcagtgattttactaatggcccagagaagtatcccaaatagtcagtagaattcagaatataagtttaagacaggggaaaaaaactttcgtgatggcgtcgtacgtgaatcccaggaatggccttttatctccttttcctgtatccccatcagttatctgcaatttac

SEQ ID NO: 17272 - RNA, 5743 nt, Homo sapiens
  source 1..5743: mol_type = other RNA
tcaggccaggcacagtggctcacagtgcctgtaatcccagcattttgggagcctgaggtgggtggaccacttgaggtcaggagttcgagaccagcctggccaatatgacaaaactttgtctctaccaaaaatacaaaaattagccaggaatggtggcacacacctgcaatcccagctacttgggaggctgaggcaggagaattgcttgaactggggaggtggaggttgcagtgagccaaaattgagccactgcactacagcctgggtgacagggcaagactccatctcaaaaaaacaaataaaataaaataataaaatgtaatatagatttacattaattaaatcagcttgctactgaactaatctcagaagacattgcgccaagtgaaaaaagccaccctcaacaggctatttgctgtatgattctacctatatgacaatcttgaaaaagcaaactctaagagcacagtcagatggctactgtcaaggacaggaaatgggaaggaggaggtgactactgtgggggacaggagcatttttgggttgatgaaactgttctatctctgagatttgataattatataactatgggcatttgtcaacaatccagccaattaccctgaattgttcattatacattctttgcttgcatcaaaacatctccagtacctcataaatatgtgcaactattatatattcataataattaaaaataaattttaaaaaattaaaataataaaaaataaattgctataaaagctcacaaaaccatacactaaagagtcattttttctatatgtaaactgtacttgaaaaatgaaacaaaaagcttaatatttgtactatgaattgattgtagggttctctgaagtgtcaatcttcccttctcccttgtgagtcctgaacaaattcataggtagaattgtgaataggaagagacaaatatcagtattattactggtaaagttgcactggacttaaaaccccaagagtcttcctactactttcccttaattttaaccctgggatccccttaaatagagagtttgcagaacaaacatttagctgggcagagacaaggataattctaaagtgcacattctggctaggcacagtggctcacgcctgtaatcccagcactttgggaggccaacgtgagtggattacctaatgtcaggagttcgagactaccctggccaacatgcccaaaccctgtctctactaaaaatacaaaaatgagccaggcgcagtggtgggcgcctgtaatcccagctactcagggggctgagagaggagaatcacttgaactcgggaggcggaggttgcggtgagcagagattgcgccactgcactccagcctgggcaacagagtgatactccgtctcaaataaataaataaataaaataaattacacattcctccaagagcagaggaccctgacaggaagacagtttgaggtgttaacaaatttgcccatggaaaacaggtgctaccccttaactggggtttagaactgtgtgcctcggctcctctgaaacagcaatactgtaaaacgccgagaacctcatgctcagtctcgtttccaaatttcagtcatctataaatcacatcacgtgcttagaaggagagcaagtgaatggcaggcagaaggagggcggtgcctctactggctgtcagggtgagggtttctgtattatatgcttgatagtagctagcatgttgggagagggaaaaaataactccttctaataaagacagttcacaaatttcacataacaaggggacagggtagattatttttcaaataatactgttttgaaaattagctaaattatttgggaaaaatattgagtagttagtagctttctctggcataagaaatacataatagtagttggtagcttttttcttgacataagaaatacataaataacttacaaataatttatatcacaaattcgtgacaatttgctcaacaaattgtcagtcacatcaaccaatcaataatagccttttaaaaacaaaactctagattatattaaacctatgggtattttcatagtatgtgttcagaaaagagctatttctagttagatataatataaccagcttaaaatataaccagctgaagtctcccccgcctccccccaccccgagcccccaacacacccacccatgcccacctccccgctcagaggctgaaaacaagtgcagcaaggtgtggtaaaaggaaagcaattttattcaaatgcaagcaggtgggggatggccaggctcatgcctttaacagaccattccccgtttgggggctaagtaaaggagtttaagacggaaaagatatgggaaatatgtgggaatagtgcaggaacgtgcaggtctgcgtgttttgttctgaaggttatcttgagtgatggtctgtcctgaggcctgatttgccttttcctgactttggcctggtagtggtgggttaactgtaagtaattcccctctcaagggaggattctgcagccaggtttccctgccttgtttgtttcaaaatcggcccctaggatttctaagcaagtccttaattagataagaaacactgtgtatgaatgtacctggtgggaaagggagacaaagtcttacaacacaaggctacattctgagattcagaaagaaagaaaaaaaaagtttgaaaatgcattttgaggctgggatccttggtcacaataattcaacttgtacacaaaatgttttctccataaaattggttgctcagtatgaaacaactaaggctgatgtgactgtgccctttatgtaacaaatgatctaaaaaataacatgttagagacctagtactcaatgttttatcttctgtctctggaatggcttttctggatactaggtataatatatccaataaaaggcataaagttctttttggatttatgctgaagttgaaagacagtagacatcttctcccatacccagttgccttaaatttgctttagccttcaagtcagttacaggcctagttgcctagattgcaaagagaaatatgaacagagctaagaagggggagataaacttggaatagaagcagtacaatgtacaagttgggacaggaatggtctatgcttactttttttccttcctgtctctcttttaaatttcagcatgacacagttttgaattccaaagagtgtcctatattttctattatatgatcagactacatttgacctacctctctatctcatctctcaacatcatagcccatgacccagctcaatgaaattatgtataggttctccactgtgtcatgcttctatgcattctcaacatactatttctttctcgtggaatgtctttcttttccatctagctgatgctaactataagtggaaaccttcctgccctgccctgattgagatgccattcctgcactctcaaagcaccctgtccatcatgtaacagtgctgttcgtgccatggaacaactgccaatttagtttgctcgatctatccataggctgtaagttccttgaaggcctggctatatcttctggcattctgtaggctcacaaaatatgtgaagaatggtgaacacactgtgtttatggaaaacaacttagtataatttaatacacactaatcagggattacccagaacatgcagttttctagcctgtaaggcacttggataaataaccgtgatgagatgtcatctgtgtgctttctctaaacatagattaccaataacaacaacaaaaaacctaacaataataatgtgttttctgaggtttaagagcatgctaaaataataatgaaagatgcatataaacaaggttgtatagacgaaaaaactaaatcacagggaacttatttattttcttcaaatttgcaccagagaaactgataaaggtgggatttaaatgtatacaagccaaactgtagatattatgtgtttgaccataaaagatcacaaaaaggtgtttgctttttaacaattacatctactatttcctcatatggaacttgaactgttagctggtacacaagttatagtggtttttgccattactttaattttgtcatttactttaatggcaaaaaccgcaatgacttttgcacgaacctgatacattaaaaacgagtttcttaaatgttcaaacaaacaagagagtgtctcttcaaaagtctcatctaaaaagtatgctttaaatttatatgcagagtctttttttaatggctgcttttacctcttgatttcttaatgtataaataataggatttaagagaggtgtgaaaattgtgtaaaacacagaaagaattttatctaccgagtatctgctgaagggccagacgtagataaagacacacggagcaaagaacagagtcacaactgtgatgtgagctgagagagtggagaaagccttagaggatcgactagcagcacggtacctaactgagaatattatgactccataggagacaagcaagaggaggaagcagaccagtgacaggagcccactgtcagcaatgaccaggagctgtaggatgtaggtgtccttgcaggcaagtttaatcacaaggggaaggtcacagaaaaagctgtctataacattgggaccacagaagggcaaagtcaacatgaaagccatttgactagatgagtgcacaaatccaactgcataggaggataacagtagcccagtgagcacccgtgggctcatgatggtcatgtaatggaggggtttgcatatggcaacatacctgtctattgccatggctacaagcaacatcatctcactcccacccaggaggtgcataaagaacatctgggaataacatccccaccatgagatggtcttacgttctcggaggaaatctacaatcatcttaggggtagcaaaagaagccaggatcatatcaatgcaggagaggttgctaagcagaaaatacattggtgtgtgaaggagcgaatcaaaggtcacagtcaccaagatgagcaggtttcctaacacaatccccacgaagaccacagagaatcccaagaagaataaaatctgaagattttgagatttggaaagtcccaacaaaataaattccgataccactgaatggtttgctctttccatatcgtcaactttatcccataatgatcaaaataagtgagaataaggggtagggaaatgatgcatattggaaagaaatgttcatgttgatgtccacatttggtactcagtcaaggcacttgaacttacaaggacccttacttttgtggaattttgtcagtcagtgattttactaatggcccagagaagtatcccaaatagtcagtagaattcagaatataagtttctggttattgctatgtagtggttagctggttggcctgtgtatggttgtcataggtttcaaaatgacttagcttgatgtaacatttatgttggtaaaagaaatacagttctttcagtataatctaaatttatgacaaaatttgtcatcggctcatgcttattacaaactggttctattggttcagcttttaaaaaaattgcctccgttgctaatagttttaaattaatctaggtcttacaaaacaccttcagtaaataaagtatttgtagtcatctttttgtgctgttattacttacaagacaggggaaaaaaactttcgtgatggcgtcgtacgtgaatcccaggaatggccttttatctccttttcctgtatccccatcagttatctgcaatttac

SEQ ID NO: 17273 - RNA, 8728 nt, Homo sapiens
  source 1..8728: mol_type = other RNA
tcaggccaggcacagtggctcacatcagagaaataagattatgaatttactgaggcatacaaattggaatctacatttaccatcttgtacaaataggaaagtttctaataacttattaacaaaatcattctgaaacctttacacaaatcagcctgctttaaataaaaaggttagaaacattatgataactatgtacaaagtatatatctgtatactctaacattctaaataaaggtatctttgaaaatttactattatacagtattagtaccatactctataatgagcaaagaaagaatatgagaactcttgggctcagtacagtgtaaatatgttcaaaatgctatacacattttgcctggaaagatttaaaaaatcccacataatcacataaaccactggactgacttttaaaaactttaaaaaagatatttaaagatatggctcattaagcaaacatttagtgatcatatctcactgcagcctcgaactcctgggctcaagtgatcctcctgcctcaattggcaaatgggcaaaagatatgaacagatatttcactgaaaaggataaacagaatggttgaaataagaaatagtgacaacaccaaatgctggcgagcatgcagagaaactggatcactcatacattcctggtgggaatgtaagatggtatagccagtctggaaaacagtttggctgtttcttataaagataagattcatttaaatgggagtctctatatcatttgtttcctaaacatcacgggtatctatctaaacacagccattttataacagatcaaatttatagtaaagtggggaaagacagtagaaatagaataacagagaatttcagaaatatctgattttgcaagcacctgtttctgtccttcccactccaagatcattcctgcattcctctaggaacaagggtcccatgggaatatgatacagccaatgacttaggtgccaatagatgctggtgccaaaatatttatggctatgaggcttcaaaacttaaaaaaaaaaaaaagattccttttacttggaaaggggatttaaaaagaaaaaaccaccaacacgattttgaatcatctatttaacttttttagattacccattttgactggttcgaaccagaagacctggctttgggtttacaataagacgattctgggaccaagtaggttgtaaaggcccaaggtatgtttggggctttctctctctctctctctctctctcttttttttttttgagacagagtctcgctctctcacccaggctggaatgcagtggcccaatctcggctcactgcaacctccacgtcccgggttcaagcaattctcctgtctcagcctcccaagtcgctgggaccacaggcacatgccatcaggactggctaatttttgtatttttagtagagatggggtttcaccatattgatcaggctggtcttgaactcctgacctcaggtgatccacccgccttggcctcccaaagtgctgggattacaggcgtgagccactacacctggcctttttctctctttttttaaattgagatgggtggggtctcactatgttgcctaggctggtctcgaactcctgagctcaagcgatcctcccgccttggcctcacaaattgctgggattacaggtgtgaaccaccacgcttatcctggggcttttaattcttactgaaaatcatagtctaaatttcccaaagggattcagaatcctttggggtacattcaagtcttctaggccatctctgggatgactctagaataacttaaagtcaaagaactccagggtatatctacatctctcctcaaataattacaaaattcttgcaagattcctgggctggactgttttaaattaaagactggtcccttacaggaggggctatttatgaagttccttccctatagcaccagagtgtttcgcactcttaaaattcaatctgttagtcatctgcagtcaaatatataaaacctgtgaagagaaaggcttcaattaaagcttaaaaagttaatatatctatgtgtatttacagacatgtgtctctacacaaatagtttttcaaatatataaacatattaagaattttattttattttattaagacagggccttgccctgttgcccaggctggagtgcagtggcacaatcatagctcatagcaccctcaaactcctgtgttcaagcgattctcctgcttcggtttcctgagtagctgggactacaggggcataccaccacacctggctaatttaaaaaaaatttttttgtagagacaaggtctcactttgctgcccaagctgtaactgaactcctggcttcaagtgatcctctggcctcagcctcccaaagtgctgggattacaggcatgagccactgtacttggccaaaaattttaaataaacaacatgaggattctagctctcactacagagtagttcttcttttgtttttttgtttttgtttttgtttttgtttttttgaaatggagtttaactcttgttgcccaggctggagtgcaatggcgcgatctcggctcaaccgcaacctctgcctcaggggttcaagcggttctcctgcctcagcctcctgactagctgggattacaggcatgtgccacaacgcacagctaatttttttgtagttttaatagagatggggtttctccatgttggtcaggctggtctcaagctactaacctcaggtaatccgtcctccttggcctcccaaagtgctgggaagagtatagttcttcttaatccaacaaaaaagtattttactcacaacaaatataaattgcccccatcaacaaatgtatgtaatatcaaggataacgtgtacaaacaaagttgcactaacaaagtaaaaatttatcccacatacatgaaagcacagtgctaagttctggggaagcagacagtttctgctttcagggagcttccagtctggtagagatttacacagaaggcagattaaagagaatgatgatctcctttgttcagagataaaaaggaagcaaaaaagcaggtcaaatcaaagatgatctgcagaatacattaaccctacactgaaatcatggacctactccagtaattaaggctgcagaggtggggctgggtggatgaaaacatcagaagacaattacagcatgagatattgattgattgattgattgattgattgagacagggtctcactttgccacccaggctagagtacagtgacaccaacttggctcactgcagcctccacctcctggagctcaagtgatcttcccacctcagccccctaattagctgggactatatgtgtgtgtcaccacacccagctaatttgtgtattttttgtagagatagggattcgccaggttgcccaggctggtctcaaactcctgagctgaagtgatccgcctgccttggcctcccaaagtgctaggattacaggtgtgagccactgtgcccagctgagatttattttttctttattaatcagcaaaatagataccctatttatttcaagatacgattaactaatttttttgctaacaaccatttcctaaggtaaaatgaggcagaaagaaaaggagtatgacactatattcactgagtcttcgattttcttctaacagcctgtatcagtggctctcaactgggggcaattttgcctctcagaatggcaatgtttgaagacatttttggccataacaactagggggatggtacttgtagctagagggcagaggtcagggatattgctaaacatcctataaagtacagcatagcatcccaaaataaagatttatccagtccaaaatgtcaatgctgagattaggaaaccatgccatggttggataaaaaagatgaaaaaatcagtatgtctatagtataaaagcaattagtagcactttaagatagattgaacaggaacattctcttcctttatcagacagttgcagaccttctaaaaatatctgatagatctataatgggaaaataaaacatgctgagaagtagcacaaatttttctaaacttcaaatattagcatacaaatgaaaaacaaacttggaagacagaaaggacaagccaggcatggtggctcacgcctgtaatcctagcactttgggaggccgaggtgggtgggtcacaaggtcaggagtttgagaccagcctggccaacatggtaaaaccctgtctctactaaaaatacaaaaatcagctgggcgtagtgacgtatacctgaaatcccagctacttgggaggctgaggcaggaggactgcttgagcccaggagagggaggttgcagtgagccgagatcatgccactgcactccagcctgggcaacagagcatgacaatgtctcaaaaaaaaaaaaaaaaaagaaaggacaattttgttgctcaattgatcttatcaactgtttctgcaaccacaaaagcaaatgtggtcatgtttctgattttagttaagtccaaaaatatttattaaagtcttatcactaaaaatggccacaaatattaaaaataaaatattagtttttagattcacagaagaaaaaaatagccactgacacttgaggagatgctcaattccgatgagggacattcaaagttactttccaacattatctgaaaagtattgatcctttttttttttttttgagacgcagtgtcgctctgttgcccaggctacagtgcagtggcatgatcttggctcactgcaacttccaccccccagattcaagcaattctcctgcctcagcctcccgagtagctgggattacaggcttgcaccaccacatccagctaatttttgtatttttagtggagacagggtttcaccgtgtttgaccaggttggactcctgacctcaaatgatccgcccacttcagcctgccaaagtgctgggattacaggcatgagccactgcacacagcccaaagtatttatcctttattttgtggttatatgttgggaaagaagaacgtggaaaagaagtgaactaacaaattttcaggtattaatattacaattcagtacattctgacaaaaagaattatttcctatgaaattacacccattggctgggtgcagtggttcacggctgcaatcccagcactttgggaggccaaggtgggaggatcacttgaggccaggaattaaagactaccctgggcaacacagcaagaccctgtctctacaaaaaaagaaaaagaaaaaaaaattacacccactgagaaacagaatgtgtaacagtaaaacaacagagcagcttccatgtgattttgataggaaagctttaattggtgactaagctttgtaaaaaggatgtaaacaggggaaagaatgaaaagaataagatttatctacataatgaagtttgactttttacagtaaataaaatacctatttattaatatttccaaatattaattagatttaataatactatatatttgttacaatgccttcatcagaaaatttaataattaagaagatacttgaagttcattcaaatggcacttgcagaaatgcaacttaatttctagttctatcatatctgtctccaaaatggacatatatgacagcaaaaacaaaattctctataaatctctccattagttacattactatgtaactaaaatagctagttctataataaaaggattttatgtgccaaatcctgaccaagagagaaataaagtcattattgctgcaaatccaaatggaacctaacccaaatgtagggaggggcaaataaagtgaaaacatgttggaaggtggggtcaactgccttaggacaattctacatccagcttgacactactcacgacttactcctcctcactgtttcttccaagaaagtctaagcatgtgaaactgtccttgttgctccctgtggatctctggctgagtggctaaagggcaatcctgagcatagacacactctcctcccttctatcagctgtcccccacacatactcacagggatgagtagactgaacaaacatcaaaaagacgcaggaacaaataaaataccccaataaaggcaattcttaagtggtcaataaattagggcacttcttcaaattaagctctgtcaattaggcacttaataaaaacaaaagacatttatacaagcatctaaataacaaagaaagataaagaacaagagaaagacaagatttatgttaactaccagcatgttatacttcagccagaagtttttgaaagaaacgttatttgagaaggaaaataagtagtatttttctgtttcttaaaaatcaatattctttctagttcattaactaaaattagtttttcagtgttttcaacatagaaagaatgctcagattttggttgaacaaggaaaaattaaggcagtgtctttaagaccagtaaaggaaagcattaactatctcataagcttatctgagagggacatattaagctcatatttggatataatattaggaaattatggctttaaacataaaatattaatgtttcaaaattccacattttctcagttattctttctttttagctatatgtacttcaaatagcccacttaaagaattaaagaaatacgtttcacataattttggaacaatatgtgcatggtacttgacccagaactattagcttggatggtaaatcattatgttcctatgtaccactgacccagtataaaaaggaagaggacccataactgtcaaaatgtggttggaaatgactaatgtcctttggaatttgctacaaaatagaagatataaagttttgaggtattgctgccttaccatggtttaggggaaaaaaataagagttttttgttccgttttgtttttttaaaagcaatgcttcttaagttatgaagcttatttaaaattttctcctcttagtcattgtcatatgggttatccctgagcttcatctcatctgcacgtcacataaaccagctacctatggttttgatcatttcatttagtgttatgtcttgttataccaattcatggagcgtttcactgctttggcccagttttccagactcatttcatattcttgacatttcttctgtggcttgaaaaccacttcactttgtctcagtttctttagttcctccttgtcagtccaaaacccaacagcaaggccagctagagaagctgcacccaggcatgacatgtcaatgtcggcaggtctgtctatattctcattaatcaggtctgaagtcatctgcatgacaaaaccattcttacaaactcctccatctgcccggatttttcttacaggaatatgaatctctttcttcatcatctcatataactgtttgtttctgaaagctattgactccaatattgctcgtacaagatggtatttactggtagaaggcttcaaacccataaaagaggcacatgcccaggggtcatttaatggagcctgtaatccactaaaagatggaacaaaacaaactccttcagaatcctccaaacttttggccattttttcagtctcagcagcatctgtgaaaaggtctaactgctgagcccattttatggcagtaccagtgtctcctgcattgctttcagctaagcatacgacttcttgcccaatcttccacccaattaatggataaaagcctccagtagtctgttgaaggctatttccagtgttaatatccaaaaatgtcccagttcccatggttaatttcacatcacctgtctggaagcagcactctccaaacatggctgattgctggtcagcaaccaaggcaactattggtataggcacaccaaatatctcttcatccactgatccaaaattgtggcttgtgtccctcacaggaggtaggagagaaagtggtatcgaaattagagaggtaatcatcccactccaacacatcttatatgggtcaaaaagtccagttgtactagcatttgaaaaatctgtggcatatacagaaccttttgtgagcttatataacaaccaggtatcaatagtcccaaagcagcaattttcttcttcaactgccttttgcacctcagtcaagttctgtaaaatccagaccaatctcaaagaagtctgctgggttgtgaaagtgaacaaactggctgtaaaaagtcgtttacttctagtgaaaaagtgaagcactcggcaagaactgtgaaatatcttcataagaagagaattattccaagattttacaagttcaacagctcttaagtcttgccaacttataaagttgtgaaaatgatttcctgttttcttgttccacgtaataaaagttgctctctgtgttgaaatgccaagaccaacaatttgattcatctgtattcctgcagctttgactgcttcttttattacggcaacaaattgaatccaaagaacatcaggatcaatttctacccagccaatttgaggataaagattttctaccttctgcacgctggagccgcagacccgcgccgcccggtcatagacgtggcagcggatcacagaactgcccacatccagccccagcacgaagccggggtaccgcggctcctgcgctctctgctccgggtccgtgagcagccccgacatcccgatcccgcacgcctctccgctacagccgcctacccagagggcgcgctacaaatcccaatgctccagagtccccgggcggcccaacccgggccccaacccggctcagccggagagcctagagaggcct

SEQ ID NO: 17274 - RNA, 9811 nt, Homo sapiens
  source 1..9811: mol_type = other RNA
tcaggccaggcacagtggctcacatcagagaaataagattatgaatttactgaggcatacaaattggaatctacatttaccatcttgtacaaataggaaagtttctaataacttattaacaaaatcattctgaaacctttacacaaatcagcctgctttaaataaaaaggttagaaacattatgataactatgtacaaagtatatatctgtatactctaacattctaaataaaggtatctttgaaaatttactattatacagtattagtaccatactctataatgagcaaagaaagaatatgagaactcttgggctcagtacagtgtaaatatgttcaaaatgctatacacattttgcctggaaagatttaaaaaatcccacataatcacataaaccactggactgacttttaaaaactttaaaaaagatatttaaagatatggctcattaagcaaacatttagtgatcatatctcactgcagcctcgaactcctgggctcaagtgatcctcctgcctcaattggcaaatgggcaaaagatatgaacagatatttcactgaaaaggataaacagaatggttgaaataagaaatagtgacaacaccaaatgctggcgagcatgcagagaaactggatcactcatacattcctggtgggaatgtaagatggtatagccagtctggaaaacagtttggctgtttcttataaagataagattcatttaaatgggagtctctatatcatttgtttcctaaacatcacgggtatctatctaaacacagccattttataacagatcaaatttatagtaaagtggggaaagacagtagaaatagaataacagagaatttcagaaatatctgattttgcaagcacctgtttctgtccttcccactccaagatcattcctgcattcctctaggaacaagggtcccatgggaatatgatacagccaatgacttaggtgccaatagatgctggtgccaaaatatttatggctatgaggcttcaaaacttaaaaaaaaaaaaaagattccttttacttggaaaggggatttaaaaagaaaaaaccaccaacacgattttgaatcatctatttaacttttttagattacccattttgactggttcgaaccagaagacctggctttgggtttacaataagacgattctgggaccaagtaggttgtaaaggcccaaggtatgtttggggctttctctctctctctctctctctctcttttttttttttgagacagagtctcgctctctcacccaggctggaatgcagtggcccaatctcggctcactgcaacctccacgtcccgggttcaagcaattctcctgtctcagcctcccaagtcgctgggaccacaggcacatgccatcaggactggctaatttttgtatttttagtagagatggggtttcaccatattgatcaggctggtcttgaactcctgacctcaggtgatccacccgccttggcctcccaaagtgctgggattacaggcgtgagccactacacctggcctttttctctctttttttaaattgagatgggtggggtctcactatgttgcctaggctggtctcgaactcctgagctcaagcgatcctcccgccttggcctcacaaattgctgggattacaggtgtgaaccaccacgcttatcctggggcttttaattcttactgaaaatcatagtctaaatttcccaaagggattcagaatcctttggggtacattcaagtcttctaggccatctctgggatgactctagaataacttaaagtcaaagaactccagggtatatctacatctctcctcaaataattacaaaattcttgcaagattcctgggctggactgttttaaattaaagactggtcccttacaggaggggctatttatgaagttccttccctatagcaccagagtgtttcgcactcttaaaattcaatctgttagtcatctgcagtcaaatatataaaacctgtgaagagaaaggcttcaattaaagcttaaaaagttaatatatctatgtgtatttacagacatgtgtctctacacaaatagtttttcaaatatataaacatattaagaattttattttattttattaagacagggccttgccctgttgcccaggctggagtgcagtggcacaatcatagctcatagcaccctcaaactcctgtgttcaagcgattctcctgcttcggtttcctgagtagctgggactacaggggcataccaccacacctggctaatttaaaaaaaatttttttgtagagacaaggtctcactttgctgcccaagctgtaactgaactcctggcttcaagtgatcctctggcctcagcctcccaaagtgctgggattacaggcatgagccactgtacttggccaaaaattttaaataaacaacatgaggattctagctctcactacagagtagttcttcttttgtttttttgtttttgtttttgtttttgtttttttgaaatggagtttaactcttgttgcccaggctggagtgcaatggcgcgatctcggctcaaccgcaacctctgcctcaggggttcaagcggttctcctgcctcagcctcctgactagctgggattacaggcatgtgccacaacgcacagctaatttttttgtagttttaatagagatggggtttctccatgttggtcaggctggtctcaagctactaacctcaggtaatccgtcctccttggcctcccaaagtgctgggaagagtatagttcttcttaatccaacaaaaaagtattttactcacaacaaatataaattgcccccatcaacaaatgtatgtaatatcaaggataacgtgtacaaacaaagttgcactaacaaagtaaaaatttatcccacatacatgaaagcacagtgctaagttctggggaagcagacagtttctgctttcagggagcttccagtctggtagagatttacacagaaggcagattaaagagaatgatgatctcctttgttcagagataaaaaggaagcaaaaaagcaggtcaaatcaaagatgatctgcagaatacattaaccctacactgaaatcatggacctactccagtaattaaggctgcagaggtggggctgggtggatgaaaacatcagaagacaattacagcatgagatattgattgattgattgattgattgattgagacagggtctcactttgccacccaggctagagtacagtgacaccaacttggctcactgcagcctccacctcctggagctcaagtgatcttcccacctcagccccctaattagctgggactatatgtgtgtgtcaccacacccagctaatttgtgtattttttgtagagatagggattcgccaggttgcccaggctggtctcaaactcctgagctgaagtgatccgcctgccttggcctcccaaagtgctaggattacaggtgtgagccactgtgcccagctgagatttattttttctttattaatcagcaaaatagataccctatttatttcaagatacgattaactaatttttttgctaacaaccatttcctaaggtaaaatgaggcagaaagaaaaggagtatgacactatattcactgagtcttcgattttcttctaacagcctgtatcagtggctctcaactgggggcaattttgcctctcagaatggcaatgtttgaagacatttttggccataacaactagggggatggtacttgtagctagagggcagaggtcagggatattgctaaacatcctataaagtacagcatagcatcccaaaataaagatttatccagtccaaaatgtcaatgctgagattaggaaaccatgccatggttggataaaaaagatgaaaaaatcagtatgtctatagtataaaagcaattagtagcactttaagatagattgaacaggaacattctcttcctttatcagacagttgcagaccttctaaaaatatctgatagatctataatgggaaaataaaacatgctgagaagtagcacaaatttttctaaacttcaaatattagcatacaaatgaaaaacaaacttggaagacagaaaggacaagccaggcatggtggctcacgcctgtaatcctagcactttgggaggccgaggtgggtgggtcacaaggtcaggagtttgagaccagcctggccaacatggtaaaaccctgtctctactaaaaatacaaaaatcagctgggcgtagtgacgtatacctgaaatcccagctacttgggaggctgaggcaggaggactgcttgagcccaggagagggaggttgcagtgagccgagatcatgccactgcactccagcctgggcaacagagcatgacaatgtctcaaaaaaaaaaaaaaaaaagaaaggacaattttgttgctcaattgatcttatcaactgtttctgcaaccacaaaagcaaatgtggtcatgtttctgattttagttaagtccaaaaatatttattaaagtcttatcactaaaaatggccacaaatattaaaaataaaatattagtttttagattcacagaagaaaaaaatagccactgacacttgaggagatgctcaattccgatgagggacattcaaagttactttccaacattatctgaaaagtattgatcctttttttttttttttgagacgcagtgtcgctctgttgcccaggctacagtgcagtggcatgatcttggctcactgcaacttccaccccccagattcaagcaattctcctgcctcagcctcccgagtagctgggattacaggcttgcaccaccacatccagctaatttttgtatttttagtggagacagggtttcaccgtgtttgaccaggttggactcctgacctcaaatgatccgcccacttcagcctgccaaagtgctgggattacaggcatgagccactgcacacagcccaaagtatttatcctttattttgtggttatatgttgggaaagaagaacgtggaaaagaagtgaactaacaaattttcaggtattaatattacaattcagtacattctgacaaaaagaattatttcctatgaaattacacccattggctgggtgcagtggttcacggctgcaatcccagcactttgggaggccaaggtgggaggatcacttgaggccaggaattaaagactaccctgggcaacacagcaagaccctgtctctacaaaaaaagaaaaagaaaaaaaaattacacccactgagaaacagaatgtgtaacagtaaaacaacagagcagcttccatgtgattttgataggaaagctttaattggtgactaagctttgtaaaaaggatgtaaacaggggaaagaatgaaaagaataagatttatctacataatgaagtttgactttttacagtaaataaaatacctatttattaatatttccaaatattaattagatttaataatactatatatttgttacaatgccttcatcagaaaatttaataattaagaagatacttgaagttcattcaaatggcacttgcagaaatgcaacttaatttctagttctatcatatctgtctccaaaatggacatatatgacagcaaaaacaaaattctctataaatctctccattagttacattactatgtaactaaaatagctagttctataataaaaggattttatgtgccaaatcctgaccaagagagaaataaagtcattattgctgcaaatccaaatggaacctaacccaaatgtagggaggggcaaataaagtgaaaacatgttggaaggtggggtcaactgccttaggacaattctacatccagcttgacactactcacgacttactcctcctcactgtttcttccaagaaagtctaagcatgtgaaactgtccttgttgctccctgtggatctctggctgagtggctaaagggcaatcctgagcatagacacactctcctcccttctatcagctgtcccccacacatactcacagggatgagtagactgaacaaacatcaaaaagacgcaggaacaaataaaataccccaataaaggcaattcttaagtggtcaataaattagggcacttcttcaaattaagctctgtcaattaggcacttaataaaaacaaaagacatttatacaagcatctaaataacaaagaaagataaagaacaagagaaagacaagatttatgttaactaccagcatgttatacttcagccagaagtttttgaaagaaacgttatttgagaaggaaaataagtagtatttttctgtttcttaaaaatcaatattctttctagttcattaactaaaattagtttttcagtgttttcaacatagaaagaatgctcagattttggttgaacaaggaaaaattaaggcagtgtctttaagaccagtaaaggaaagcattaactatctcataagcttatctgagagggacatattaagctcatatttggatataatattaggaaattatggctttaaacataaaatattaatgtttcaaaattccacattttctcagttattctttctttttagctatatgtacttcaaatagcccacttaaagaattaaagaaatacgtttcacataattttggaacaatatgtgcatggtacttgacccagaactattagcttggatggtaaatcattatgttcctatgtaccactgacccagtataaaaaggaagaggacccataactgtcaaaatgtggttggaaatgactaatgtcctttggaatttgctacaaaatagaagatataaagttttgaggtattgctgccttaccatggtttaggggaaaaaaataagagttttttgttccgttttgtttttttaaaagcaatgcttcttaagttatgaagcttatttaaaattttctcctcttagtcattgtcatatgggttatccctgagcttcatctcatctgcacgtcacataaaccagctacctatggttttgatcatttcatttagtgttatgtcttgttataccaattcatggagcgtttcactgctttggcccagttttccagactcatttcatattcttgacatttcttctgtggcttgaaaaccacttcactttgtctcagtttctttagttcctccttgtcagtccaaaacccaacagcaaggccagctagagaagctgcacccaggcatgacatgtcaatgtcggcaggtctgtctatattctcattaatcaggtctgaagtcatctgcatgacaaaaccattcttacaaactcctccatctgcccggatttttcttacaggaatatgaatctctttcttcatcatctcatataactgtttgtttctgaaagctattgactccaatattgctcgtacaagatggtatttactggtagaaggcttcaaacccataaaagaggcacatgcccaggggtcatttaatggagcctgtaatccactaaaagatggaacaaaacaaactccttcagaatcctccaaacttttggccattttttcagtctcagcagcatctgtgaaaaggtctaactgctgagcccattttatggcagtaccagtgtctcctgcattgctttcagctaagcatacgacttcttgcccaatcttccacccaattaatggataaaagcctccagtagtctgttgaaggctatttccagtgttaatatccaaaaatgtcccagttcccatggttaatttcacatcacctgtctggaagcagcactctccaaacatggctgattgctggtcagcaacctatagtcctagctactcaggaggctgaggcagaagagtcacttgaacccgagaggcggaggtcacagtgagccatcggtgagatcatgccattgcactccagtctgggagacaagagtgaaactccatctcaaaaacaacaacaacaacaacaactcatttaaagaaccctctgtcactaattggtaactcttccagccataccttaatctaaccctgcacctatgcctagattgaataagaccgatcctctctaaatgataatgattttgtaacttggaaattaaattccctttccctcagctgctcccccagctactgtggagactgcacatcttgcaacaggtggtctctacctcctgcttaagctgccacaggaaatcaaaggcaatgtgaaaggactcttaaaaatcaaaaacaggcttggcacagtgactcatgcctgtagtcccagcactttgggaggcaaaggtggcagaaggccccagtctaggagttcgagatcagccaggggaacacagcaaaatcctatgtctaccaaaaatacaaaaaattagccaggtgtcgtggcacacacctgtggtcttggctacttgggaggctggggtggaagaatcacctgagcccaggaagccgaggctgcagtgaggcatgattataccactgcactccagcctgagtgacagagtgagaccctgtctcaaaaaaaaaaaaaaaaatcaaaaatggcaaatatttcattattctacaaacttatttactggtagatgatggctaaggactttattaaatgtacatacaactttctctgctagtttaagttgccctaacactgtttgtggttacacattatcaaacagaacataaatattcgccccatcactgtgttttgtctcagagtaccaaatgtaaactaaataccactcagaattaaaaaaaattttttttaatttaagttttctgataaacaatatacaagcaagtcagaaaaggttataaagtacttccatgatagaatactggctcaatggtccccttcccaaaaatatagcagatattctggtcatatccagggacctttaacaaggcaactattggtataggcacaccaaatatctcttcatccactgatccaaaattgtggcttgtgtccctcacaggaggtaggagagaaagtggtatcgaaattagagaggtaatcatcccactccaacacatcttatatgggtcaaaaagtccagttgtactagcatttgaaaaatctgtggcatatacagaaccttttgtgagcttatataacaaccaggtatcaatagtcccaaagcagcaattttcttcttcaactgccttttgcacctcagtcaagttctgtaaaatccagaccaatctcaaagaagtctgctgggttgtgaaagtgaacaaactggctgtaaaaagtcgtttacttctagtgaaaaagtgaagcactcggcaagaactgtgaaatatcttcataagaagagaattattccaagattttacaagttcaacagctcttaagtcttgccaacttataaagttgtgaaaatgatttcctgttttcttgttccacgtaataaaagttgctctctgtgttgaaatgccaagaccaacaatttgattcatctgtattcctgcagctttgactgcttcttttattacggcaacaaattgaatccaaagaacatcaggatcaatttctacccagccaatttgaggataaagattttctaccttctgcacgctggagccgcagacccgcgccgcccggtcatagacgtggcagcggatcacagaactgcccacatccagccccagcacgaagccggggtaccgcggctcctgcgctctctgctccgggtccgtgagcagccccgacatcccgatcccgcacgcctctccgctacagccgcctacccagagggcgcgctacaaatcccaatgctccagagtccccgggcggcccaacccgggccccaacccggctcagccggagagcctagagaggcct

SEQ ID NO: 17275 - RNA, 5078 nt, Homo sapiens
  source 1..5078: mol_type = other RNA
tcaggccaggcacagtggctcacatctgtaattccagcactttgggaggcccaggtgggaggattgcttgaggacagaagttcaagatcagcctggccaacatagtgagatcctgtctctacaaaaaataaaattaagacaagcctggtggcttacgcctgtagtcccagctactcggggggctaaagtgggaggatcacttcagtccaacaggtcgaggctgcagtgtgctgtgatcatgccactgtactccagcctgagtgacagagaccccgtctcaaaaaaatttttttttcgttgttaaaatacttctcttaacttccattcactggtgctgattccatgctgtgagacccccctaaaactatactctcacctctacttcccctacaagtcttttctataccagattacccacctctcttggcacttagagcagggtttacactgttgttttgacaacaattaatcttctaagaatgcagtggtatgtcagtcagttggggtccactgaaagccaatagtcaagagtgagtgagctgaccactgcaaaagagagcagtgaatgtcatttgcacttccacagggactgcacaaagttctccagtgccgggcttctctctggacttcactgttgtcagtatggtgagagtcagaaagagacactctccaattattcagtcattcacacctgtaatcccagcactttggaagccgaggcaggcgaatcacgaggtcaggagttcgagactagcctggccaacatagtgaaaccccatctctactaaaaatacaaaaaattagctgggtgtggtggtgcacacctgtaatcccagctactcaggaggctgaggcaggagaatcgcttgaacctgggaggcagaggttgcagtaaaccgagattacaccattgcactgcagccctggcaatagtgcgagatgctgtctcaaaaaaaaaaaagaaaagaaaagacattccctcaaccataaatcagcaccatcatcttctcgacatgctgaaaccagtcttgattgctccatattccccaaacccaagagaactgaccattctactacttggtctgaaaaagcttaacagaaaaaattctaggtcttaccatgagtggaaatggaccaaaatgcagatgaattgctaaatgtctaccagactccttccacctttctctaaacctctcattcagaacctcccttttactcccaagccattcggtaaccattctgcttcccttctatctccacattctatctccaccatctgacttctcactgccatctataaagaaggcctgggtcaggtgcggtggctcatgcctgtaatcccaacactttgggaggccgaggcgggtggatcacgaggtcaggagatcgagatcatcctggctaacacggtgaaaccccgtctctactaaaaatacaaaaaatttgccgggtgtggtggcaggcgcctgtaatcccagctactcgggaagctggggcaggagaatggcatgaacctgggaggcagaggttgcagtgagccgagattgtgcgactgcactccagcctgggcaacagagcaagactccatctcaaagaaggcctgaaatgtagggaggaaccagaggaacagtagtacagccagatgcctcttgccacaggaattttcgacattgtcagtcacattgggaaccatttgttcatgtccaagctggtcaaagagaagcccctgggcagcaatgattaaaggaattcttgttgcagagtagccaacacatttatgtaaactctttcttggtaatgataaagacctagggttgcatagatatcttgcagcagacactgttttcttgcaacagacactgcttcaacacacactgttttctgattttgtgttgaaatctggtgagatccacttaacttagaactcaatattagtgtaggttaaaaaaaaattcactacaggaagtaaattggcattctatatatttgagaaactaatgtataaaaattcaagataattacaattggaaggggaccaataattccactttttaatcgaaaataatctatatactcccaataaactcacagtaaaataagcttcaaaaagccttaagacaccaaaagaggaaaaaaagccagtaattagaacaaaatgtgtaatgtggttaatagtatagatatgcttgcctttagacaattcttatatactcaattcttacatgattgaaagattctgtaataatgctctacctttttataaagaaaaaagtaggtttccaaaagaaaattaaacgtttatgactggagttagcggtagtaaggaattagatgtgagtggttgactgctctttgtgccttcgacattttgcagaaaattctgtcttctttttagtccatccaaaatgactgaattattagatcccagactctgtgtccgtggagaatctattccactatctcctgccatgctgtgattttctgtcccttccaagtgactgtgttcatattggacatcctgagccaacactggcatatgtgaagtgttgaaaagttggaacttttgtgggaaatgttttctcatttcctgattctgaggactctgactccagctagctggcttctttcctgtgtcaccaatagtgtcttgtatgacttcagcttcaaaactggcttttcttgcgctatagtaatcaaagattctttcatcagcaggtgctgaggcctgtacacatttagcaacactgggttcttcttcgtagttaaaaccaaactgggcccctgaatttaggccacaactttcagcagagaggttaggttcttggctttcacctggggtagcatgcagcccagtgggtttgtagcattcatttcttttaagcacctgagactcaaccctctccattgtgctgttgtactcggtcagagatctctcaatcactttttgttttcctaaatgatttccctggcttccacctgtgaaggaatactgactgtggccaggcagcatttgacgtaagtcgtcattctcagaaatgtcatcctcctctagatataatgaactacaggcaccatcatcatcttccacttcattctgatacaaggcctggtcatcgttagaaagctgttcattttctaggcttgtagtctctgcatcctggacaaatccttttctcaataattcttctgagtctttgtcttgtcttgcagcttgtcttaaagggttcacgccaactgggtaatccaaaaggccaagattttgaaactggtgtattgtgttatccactaatctacaagcagagggtgttcggtctgaaaaggaggcacctcgtgatggcagactatgcggagtctgtttggtctcccctaatttgtcaaagtgggaatgacttttcctcaagacttcaggaattacctcattttctccaccatacacttcatatctcaacatgctttccataaagggacagcatttaccatcattttgcaacatgctctgttgagggtgactgaagaggtgacctctgaagtcatcattgatgggtttgacagtagggtcatttatgtaaatggattctgcttccattttatcattaggttgttcagcatatggctctttggctttaccatcaaagattcttgaggaatccaaggacctaggcttttggaaaggcttttcctttggtccagtctggctgggtttcagatcactcgtcttctgaattttgtgccctttggatattgtgcttcctcggtgagacaaaccctggaaaggattactgattcgctttttgtaaatcaaatgggaacctagcactgttgtaatctcaccaagtggtttctgacctaccatttcatttgggcttttaattctggggatgggctgtgtagcagggagcttggggtgtttctccagtctaatgcttcctggctgaaactcacttccctgattcctggctttgtgtctatcccttcgagaatggccctgcccttgaggttttgcagacagaccctgccttttcttaaccccctcttttgaaggatacttatgcccgattgtcagcatgtcagtggaagtgccctggctattatattttttctgttcttcgtatttttgcattaggacagtgtgtttgattaaattgtcaacagtcaaaatggggttaattcgtttgattatctcatgttcaacatctcgagggatattgtccaagtcatcttcatctcggacgggccattcttcaggtgggaactgagcagagaaactgctgtgttctgttttgggcttctcctttctagataagctgcgccataagagactaaaaccaaacttcttgcctttttctttatctcttgtgtatggtaaaggtttggtgctctcacaaatgtggtgctccgcagacactgaaactgccccattctgtacccaagatacggattccccaagacctctgtgactcttcctagtcacttctgcagcaactggtgcttcctgaacatcctgagtgtgcatgtcccggaaacactggcaagactgacagtgggatatgggggcagcattctcttgggctgactctgcacagctctccatgctcaccagatatgtcatggaagctggcatcaggcgactttcatctgatggcagcattctcttattttcctgggtggttgtatttgtaatgaagtaagtctgaggagtaactatgaagtatccttctccagtgtgataaatcttcctttctttaatcagcgttcccagagtggtataaagaatatcttccgatggaattgcaatgcctgggtaatgtttcatcaaacgctccaaaagtgattcctgcgttactacaatctgagctgtattcatatcagatatagcacagcaaagaacttcacccaaaggtacgaactgagattgagttattggattcatttgcactggaaagacatcacccaccgccctgatgcggaagccgcgcggcggccgcagggcccggcgccgccaggcatcgcgcagcacctgcaggcaggcggggggcgcgcgcaccagcagcaccccccgccgcagccagccctggaag

SEQ ID NO: 17276 - RNA, 61 nt, Homo sapiens
  source 1..61: mol_type = other RNA
tcaggccaggcacagtggctcacatctgtcatcccagcactttgagaggccaaggcaggat

SEQ ID NO: 17277 - RNA, 70 nt, Homo sapiens
  source 1..70: mol_type = other RNA
tcaggccaggcacagtggctcacccctgtaatcctggagctttgggagggcaaggtgggaggattgcttg

SEQ ID NO: 17278 - RNA, 1609 nt, Homo sapiens
  source 1..1609: mol_type = other RNA
tcaggccaggcacagtggctcacccctgtaatctcagcactttgggagttcaaaaccagcttggatgacatggcaaaaccccatctctacaaaaagatacaaaaattaggcaggcatggaggcacacgcatgtggtcccacctactctggaggctgaagtgggaggctcacctgagctcgggaggtcaaggttgcagtgagccatgattgtgccactgcactccagcctgggtgacagaatgagaccctcccaaaaaagaaaaaaaaaaaagctggaaggctatactaaataggtcactctttcctctatttttccaacttttagaaattcaaatttattcaaaagtttgacatatacaattccataactactatttcatcttcaatctacagaattagctttaagcaactttaaagcttgagctccttctgaatttcccaaagtgtttctgcactcttttgcaagcaggcctcctcttcaagagtcagttttacttttatgaggtctgtgataccattctctcccaggatacatgggacactaaggaatatgtcttcatttattccatagaggcccttacttagggtagaaactggatgcactctcctaagattcttcaaaatactttctgttaaatcagctacagataggctaatgccccaagaagtataacctttcattttgaccatctcatagccactggaaatcacttttttgtggacattttcccactgctcaggatctttatcagttcctatatctgggttcagatccttcagagggacgccagcaatgttcacaccactccacacaggaacacttgagtcgccatgctctccaaggatcagcccatgacagctttcagagtggatgccaagcctttgcccaataaagtaacgaaaacgagcagagtccagattacaaccacttccaataacacggtttttgggaaatccactcaacttccaggctacataagttaagatatccactgagatggagagaagtatggtagaaatgtctttaagtttcctcatacataaagctggattagtaacaataagcagtttgcagtgaggactgtactgggtaatattgggaatcattaatttaaagatggatacatttcgctggactaaatcaaggcgtgtttctccttttttctggcgtgcacctgctgtgataatcactagattggagtttgcagtgaccaggtaatctttgctggagacaatatttggcattttcataaaagggctgccatgttgaagatccattgtctcacccttcagtttgccttcatcaacatccacaaggacaagttcatcactcaaaccttttaataagatgctgatagcacaagccacaccaaccgatccagttcctacaatggagatcttattgtgatgaatggcctcctcttccgcgaaattcttaataagttcactcttgatagttgccatcttggaaacaggggtgaagggccacccgcgcccgagcaggtcacatgccgcctggcggagacacagaaccatccttgggcaaaaacaattcgctcccgcggcgcccgctctctggctgctccccaggactcttgcagcccagctc

SEQ ID NO: 17279 - RNA, 1553 nt, Homo sapiens
  source 1..1553: mol_type = other RNA
tcaggccaggcacagtggctcacccctgtaatctcagcactttgggagttcaaaaccagcttggatgacatggcaaaaccccatctctacaaaaagatacaaaaattaggcaggcatggaggcacacgcatgtggtcccacctactctggaggctgaagtgggaggctcacctgagctcgggaggtcaaggttgcagtgagccatgattgtgccactgcactccagcctgggtgacagaatgagaccctcccaaaaaagaaaaaaaaaaaagctggaaggctatactaaataggtcactctttcctctatttttccaacttttagaaattcaaatttattcaaaagtttgacatatacaattccataactactatttcatcttcaatctacagaattagctttaagcaactttaaagcttgagctccttctgaatttcccaaagtgtttctgcactcttttgcaagcaggcctcctcttcaagagtcagttttacttttatgaggtctgtgataccattctctcccaggatacatgggacactaaggaatatgtcttcatttattccatagaggcccttacttagggtagaaactggatgcactctcctaagattcttcaaaatactttctgttaaatcagctacagataggctaatgccccaagaagtataacctttcattttgaccatctcatagccactggaaatcacttttttgtggacattttcccactgctcaggatctttatcagttcctatatctgggttcagatccttcagagggacgccagcaatgttcacaccactccacacaggaacacttgagtcgccatgctctccaaggatcagcccatgacagctttcagagtggatgccaagcctttgcccaataaagtaacgaaaacgagcagagtccagattacaaccacttccaataacacggtttttgggaaatccactcaacttccaggctacataagttaagatatccactgagatggagagaagtatggtagaaatgtctttaagtttcctcatacataaagctggattagtaacaataagcagtttgcagtgaggactgtactgggtaatattgggaatcattaatttaaagatggatacatttcgctggactaaatcaaggcgtgtttctccttttttctggcgtgcacctgctgtgataatcactagattggagtttgcagtgaccaggtaatctttgctggagacaatatttggcattttcataaaagggctgccatgttgaagatccattgtctcacccttcagtttgccttcatcaacatccacaaggacaagttcatcactcaaaccttttaataagatgctgatagcacaagccacaccaaccgatccagttcctacaatggagatcttattgtgatgaatggcctcctcttccgcgaaattcttaataagttcactcttgatagttgccatcttggaaaccctgctgttcccccaacctccagttctcagctccaggactgcgcccggggtccgcaggtccaggtgagaggtacttctgg

SEQ ID NO: 17280 - RNA, 1535 nt, Homo sapiens
  source 1..1535: mol_type = other RNA
tcaggccaggcacagtggctcacccctgtaatctcagcactttgggagttcaaaaccagcttggatgacatggcaaaaccccatctctacaaaaagatacaaaaattaggcaggcatggaggcacacgcatgtggtcccacctactctggaggctgaagtgggaggctcacctgagctcgggaggtcaaggttgcagtgagccatgattgtgccactgcactccagcctgggtgacagaatgagaccctcccaaaaaagaaaaaaaaaaaagctggaaggctatactaaataggtcactctttcctctatttttccaacttttagaaattcaaatttattcaaaagtttgacatatacaattccataactactatttcatcttcaatctacagaattagctttaagcaactttaaagcttgagctccttctgaatttcccaaagtgtttctgcactcttttgcaagcaggcctcctcttcaagagtcagttttacttttatgaggtctgtgataccattctctcccaggatacatgggacactaaggaatatgtcttcatttattccatagaggcccttacttagggtagaaactggatgcactctcctaagattcttcaaaatactttctgttaaatcagctacagataggctaatgccccaagaagtataacctttcattttgaccatctcatagccactggaaatcacttttttgtggacattttcccactgctcaggatctttatcagttcctatatctgggttcagatccttcagagggacgccagcaatgttcacaccactccacacaggaacacttgagtcgccatgctctccaaggatcagcccatgacagctttcagagtggatgccaagcctttgcccaataaagtaacgaaaacgagcagagtccagattacaaccacttccaataacacggtttttgggaaatccactcaacttccaggctacataagttaagatatccactgagatggagagaagtatggtagaaatgtctttaagtttcctcatacataaagctggattagtaacaataagcagtttgcagtgaggactgtactgggtaatattgggaatcattaatttaaagatggatacatttcgctggactaaatcaaggcgtgtttctccttttttctggcgtgcacctgctgtgataatcactagattggagtttgcagtgaccaggtaatctttgctggagacaatatttggcattttcataaaagggctgccatgttgaagatccattgtctcacccttcagtttgccttcatcaacatccacaaggacaagttcatcactcaaaccttttaataagatgctgatagcacaagccacaccaaccgatccagttcctacaatggagatcttattgtgatgaatggcctcctcttccgcgaaattcttaataagttcactcttgatagttgccatcttggaaacctccagttctcagctccaggactgcgcccggggtccgcaggtccaggtgagaggtacttctg

SEQ ID NO: 17281 - RNA, 1696 nt, Homo sapiens
  source 1..1696: mol_type = other RNA
tcaggccaggcacagtggctcacccctgtaatctcagcactttgggagttcaaaaccagcttggatgacatggcaaaaccccatctctacaaaaagatacaaaaattaggcaggcatggaggcacacgcatgtggtcccacctactctggaggctgaagtgggaggctcacctgagctcgggaggtcaaggttgcagtgagccatgattgtgccactgcactccagcctgggtgacagaatgagaccctcccaaaaaagaaaaaaaaaaaagctggaaggctatactaaataggtcactctttcctctatttttccaacttttagaaattcaaatttattcaaaagtttgacatatacaattccataactactatttcatcttcaatctacagaattagctttaagcaactttaaagcttgagctccttctgaatttcccaaagtgtttctgcactcttttgcaagcaggcctcctcttcaagagtcagttttacttttatgaggtctgtgataccattctctcccaggatacatgggacactaaggaatatgtcttcatttattccatagaggcccttacttagggtagaaactggatgcactctcctaagattcttcaaaatactttctgttaaatcagctacagataggctaatgccccaagaagtataacctttcattttgaccatctcatagccactggaaatcacttttttgtggacattttcccactgctcaggatctttatcagttcctatatctgggttcagatccttcagagggacgccagcaatgttcacaccactccacacaggaacacttgagtcgccatgctctccaaggatcagcccatgacagctttcagagtggatgccaagcctttgcccaataaagtaacgaaaacgagcagagtccagattacaaccacttccaataacacggtttttgggaaatccactcaacttccaggctacataagttaagatatccactgagatggagagaagtatggtagaaatgtctttaagtttcctcatacataaagctggattagtaacaataagcagtttgcagtgaggactgtactgggtaatattgggaatcattaatttaaagatggatacatttcgctggactaaatcaaggcgtgtttctccttttttctggcgtgcacctgctgtgataatcactagattggagtttgcagtgaccaggtaatctttgctggagacaatatttggcattttcataaaagggctgccatgttgaagatccattgtctcacccttcagtttgccttcatcaacatccacaaggacaagttcatcactcaaaccttttaataagatgctgatagcacaagccacaccaaccgatccagttcctacaatggagatcttattgtgatgaatggcctcctcttccgcgaaattcttaataagttcactcttgatagttgccatcttggaaactcaagaggtgaagaaagagaatggaggaaaatggcgttaaagctcatcgaggcacgaaggagatgaaccgccgactaacagacgccgggtcgcccccttactgcagctgcgcggaccgcacccagctcgtgcaggcatcgcaggtgtgatgcttggcaggtgtgatgcttggcaggtgtgatgcttggcaggtgtgatgcttggcaggtgtgaggccggaagc

SEQ ID NO: 17282 - RNA, 1553 nt, Homo sapiens
  source 1..1553: mol_type = other RNA
tcaggccaggcacagtggctcacccctgtaatctcagcactttgggagttcaaaaccagcttggatgacatggcaaaaccccatctctacaaaaagatacaaaaattaggcaggcatggaggcacacgcatgtggtcccacctactctggaggctgaagtgggaggctcacctgagctcgggaggtcaaggttgcagtgagccatgattgtgccactgcactccagcctgggtgacagaatgagaccctcccaaaaaagaaaaaaaaaaaagctggaaggctatactaaataggtcactctttcctctatttttccaacttttagaaattcaaatttattcaaaagtttgacatatacaattccataactactatttcatcttcaatctacagaattagctttaagcaactttaaagcttgagctccttctgaatttcccaaagtgtttctgcactcttttgcaagcaggcctcctcttcaagagtcagttttacttttatgaggtctgtgataccattctctcccaggatacatgggacactaaggaatatgtcttcatttattccatagaggcccttacttagggtagaaactggatgcactctcctaagattcttcaaaatactttctgttaaatcagctacagataggctaatgccccaagaagtataacctttcattttgaccatctcatagccactggaaatcacttttttgtggacattttcccactgctcaggatctttatcagttcctatatctgggttcagatccttcagagggacgccagcaatgttcacaccactccacacaggaacacttgagtcgccatgctctccaaggatcagcccatgacagctttcagagtggatgccaagcctttgcccaataaagtaacgaaaacgagcagagtccagattacaaccacttccaataacacggtttttgggaaatccactcaacttccaggctacataagttaagatatccactggattagtaacaataagcagtttgcagtgaggactgtactgggtaatattgggaatcattaatttaaagatggatacatttcgctggactaaatcaaggcgtgtttctccttttttctggcgtgcacctgctgtgataatcactagattggagtttgcagtgaccaggtaatctttgctggagacaatatttggcattttcataaaagggctgccatgttgaagatccattgtctcacccttcagtttgccttcatcaacatccacaaggacaagttcatcactcaaaccttttaataagatgctgatagcacaagccacaccaaccgatccagttcctacaatggagatcttattgtgatgaatggcctcctcttccgcgaaattcttaataagttcactcttgatagttgccatcttggaaacaggggtgaagggccacccgcgcccgagcaggtcacatgccgcctggcggagacacagaaccatccttgggcaaaaacaattcgctcccgcggcgcccgctctctggctgctccccaggactcttgcagcccagc

SEQ ID NO: 17283 - RNA, 2235 nt, Homo sapiens
  source 1..2235: mol_type = other RNA
tcaggccaggcacagtggctcacccctgtaatctcagcactttgggagttcaaaaccagcttggatgacatggcaaaaccccatctctacaaaaagatacaaaaattaggcaggcatggaggcacacgcatgtggtcccacctactctggaggctgaagtgggaggctcacctgagctcgggaggtcaaggttgcagtgagccatgattgtgccactgcactccagcctgggtgacagaatgagaccctcccaaaaaagaaaaaaaaaaaagctggaaggctatactaaataggtcactctttcctctatttttccaacttttagaaattcaaatttattcaaaagtttgacatatacaattccataactactatttcatcttcaatctacagaattagctttaagcaactttaaagcttgagctccttctgaatttcccaaagtgtttctgcactcttttgcaagcaggcctcctcttcaagagtcagttttacttttatgaggtctgtgataccattctctcccaggatacatgggacactaaggaatatgtcttcatttattccatagaggcccttacttagggtagaaactggatgcactctcctaagattcttcaaaatactttctgttaaatcagctacagataggctaatgccccaagaagtataacctttcattttgaccatctcatagccactggaaatcacttttttgtggacattttcccactgctcaggatctttatcagttcctatatctgggttcagatccttcagagggacgccagcaatgttcacaccactccacacaggaacacttgagtcgccatgctctccaaggatcagcccatgacagctttcagagtggatgccaagcctttgcccaataaagtaacgaaaacgagcagagtccagattacaaccacttccaataacacggtttttgggaaatccactcaacttccaggctacataagttaagatatccactggattagtaacaataagcagtttgcagtgaggactgtactgggtaatattgggaatcattaatttaaagatggatacatttcgctggactaaatcaaggcgtgtttctccttttttctggcgtgcacctgctgtgataatcactagattggagtttgcagtgaccaggtaatctttgctggagacaatatttggcattttcataaaagggctgccatgttgaagatccattgtctcacccttcagtttgccttcatcaacatccacaaggacaagttcatcactcaaaccttttaataagatgctgatagcacaagccacaccaaccgatccagttcctacaatggagatcttattgtgatgaatggcctcctcttccgcgaaattcttaataagttcactcttgatagttgccatcttggaaacctaacagtgaagacaaattgcacagccatttccaagacctggaattggaaatggcttggaattccaagacctgcggtgagagcgcgtatagagaactcctgggcccgtgtggaaggaggtgctgcagacacacaaaagaccgacaaatctgaccagcaaagaagctgggtaggttctggccaggcagctcagcatccatgaagcggaccaggggaaggagaaggaagcgtgagtacagttaagaggaattaagagagagagagaggaaaggaacaggggttgctccaccaaacatgaaactacagctgggacggcactccgtcccgcagctgacccccttttctctcccctttaccctgctgttcccccaacctccagttctcagctccaggactgcgcccggggtccgcaggtccaggtgagaggtacttctggccacactcacaggggtgaagggccacccgcgcccgagcaggtcacatgccgcctggcggagacacagaaccatccttgggcaaaaacaattcgctcccgcggcgcccgctctctggctgctccccaggactcttgcagcccagctcatggccactcactcaagaggtgaagaaagagaatggaggaaaatggcgttaaagctcatcgaggcacgaaggagatgaaccgccgactaacagacgccgggtcgcccccttactgcagctgcgcggaccgcacccagctcgtgcaggcatcgcaggtgtgatgcttggcaggtgtgatgcttggcaggtgtgatgcttggcaggtgtgatgcttggcaggtgtgaggccggaagc

SEQ ID NO: 17284 - RNA, 1642 nt, Homo sapiens
  source 1..1642: mol_type = other RNA
tcaggccaggcacagtggctcacccctgtaatctcagcactttgggagttcaaaaccagcttggatgacatggcaaaaccccatctctacaaaaagatacaaaaattaggcaggcatggaggcacacgcatgtggtcccacctactctggaggctgaagtgggaggctcacctgagctcgggaggtcaaggttgcagtgagccatgattgtgccactgcactccagcctgggtgacagaatgagaccctcccaaaaaagaaaaaaaaaaaagctggaaggctatactaaataggtcactctttcctctatttttccaacttttagaaattcaaatttattcaaaagtttgacatatacaattccataactactatttcatcttcaatctacagaattagctttaagcaactttaaagcttgagctccttctgaatttcccaaagtgtttctgcactcttttgcaagcaggcctcctcttcaagagtcagttttacttttatgaggtctgtgataccattctctcccaggatacatgggacactaaggaatatgtcttcatttattccatagaggcccttacttagggtagaaactggatgcactctcctaagattcttcaaaatactttctgttaaatcagctacagataggctaatgccccaagaagtataacctttcattttgaccatctcatagccactggaaatcacttttttgtggacattttcccactgctcaggatctttatcagttcctatatctgggttcagatccttcagagggacgccagcaatgttcacaccactccacacaggaacacttgagtcgccatgctctccaaggatcagcccatgacagctttcagagtggatgccaagcctttgcccaataaagtaacgaaaacgagcagagtccagattacaaccacttccaataacacggtttttgggaaatccactcaacttccaggctacataagttaagatatccactggattagtaacaataagcagtttgcagtgaggactgtactgggtaatattgggaatcattaatttaaagatggatacatttcgctggactaaatcaaggcgtgtttctccttttttctggcgtgcacctgctgtgataatcactagattggagtttgcagtgaccaggtaatctttgctggagacaatatttggcattttcataaaagggctgccatgttgaagatccattgtctcacccttcagtttgccttcatcaacatccacaaggacaagttcatcactcaaaccttttaataagatgctgatagcacaagccacaccaaccgatccagttcctacaatggagatcttattgtgatgaatggcctcctcttccgcgaaattcttaataagttcactcttgatagttgccatcttggaaactcaagaggtgaagaaagagaatggaggaaaatggcgttaaagctcatcgaggcacgaaggagatgaaccgccgactaacagacgccgggtcgcccccttactgcagctgcgcggaccgcacccagctcgtgcaggcatcgcaggtgtgatgcttggcaggtgtgatgcttggcaggtgtgatgcttggcaggtgtgatgcttggcaggtgtgaggccggaagc

SEQ ID NO: 17285 - RNA, 72 nt, Homo sapiens
  source 1..72: mol_type = other RNA
tcaggccaggcacagtggctcaccgctgtaatcccagcactttgggagacagagacgggaggatggcttgag

SEQ ID NO: 17286 - RNA, 852 nt, Homo sapiens
  source 1..852: mol_type = other RNA
tcaggccaggcacagtggctcaccgctgtaatcccagcactttgggagacagagacgggaggatggcttgagccggagaggtcgaggctgtagtgactcgccactgcactccagcctgggcgacagagcgagaccctctttgtcctgcatcaaccttgggtggaacagcttgcttcattgagggcagttgcaggaaaatccagctgggagccgtcagcagtcctgcccactgcgggtaagagccctgaatcactttctccaagcttccaagtaccagggtccttgccagggtgataaattctatggctggtcacatccaggaagcacccacgagtctggagctgtgggaggtggcagtggataggctgacatattgttcttgaagctggtccagcagattcactgtgcctcaccctgtatctttctctgggcctccttcaccagcttctgggtcaacttctgaggggtcatgacgttcgaactgcttggaattcctgaatacagtgcattatacatatgctctacacgtatctattatagccttacaagttggagttgtttgttatctatttaatgtgtatttgttttgtctccccaactagactggaaacacctagaggacagggacagtatctttctctttctgcaatgctcccagtgcctgggggctaggctaggacgccaagggagctcattaaaagttgttgacagtctctccaccatcctgtgccccaccccgaccactcccctcttcctcggtggccactccacttcctcctcccgggtccccgccccttctcgctccctttagttgaatcctcactggtctcgccccttcttagtggattccat

SEQ ID NO: 17287 - RNA, 71 nt, Homo sapiens
  source 1..71: mol_type = other RNA
tcaggccaggcacagtggctcacctgtaattcagatactttgggaggctgaggtgggaggattacttgagc

SEQ ID NO: 17288 - RNA, 1607 nt, Homo sapiens
  source 1..1607: mol_type = other RNA
tcaggccaggcacagtggctcacgactgtaatcccagcactttgggaagccgaggcaggcggatcacctgaggtcgggagtttgagaccagcttgaccaacatggagaaaccccgtctctactaaaaatagaaaattagccgggcatggtggcacatgcctgtaatcccagctactggggaggctgaagcaggagaatcgcttgaacccgggaggtggaggttgtggtgagccaagatcacgccattgcactccagcctgggcaacaaaagcgaaactccatctcaaaaaaaaaaaaacaaaaaaacccaaaaaaaacagtgtagaagctggtaagtctgtctaccttaggacactgagttaactggccacaatcggggtcccttcacacaaagacagccatgggcagttgtggaggacagaaaccactgcctagtaccaaagcccagtaaggacagagggaaaaaggtatgcctgacttagggattagtctgacttccttggaaaaatccgggcaggttctagccatcttcctaaaacatcggtgtcataggggagcaagggccacagccccagggcaggagagattctgtgacatgtttgaactgtgtagtttgtatagaagggctcaggctttggaatcaaagcagacctggattcaaaccctggatctgatccttactagcttgtgtgactttaggcaaaatgtacaattttctgagtaatgattttcacatttctaaaatgaacccatttccccagaattgttgtgatgattaaatgagataacagcaaaataaaatcctcagcaaagagcctggaatgtgtgtcttctgagatattttcacagagaaacggatatttaaactgagtttctccccatggtaggctacattatcgtctcctggctaataatctctagccaggagacacagtctgcacacccacagacattgtactaatatggtacaatggtttaaaaggccagttcaataatctattattagattacttgctaatctccccttccctataagagcattgtacatcctctcccactgcctggtggcttgcagaggggcatcctttcccatcctactgatgtcagtcttgatcagggggtgctctggccaaaagaatgcaagtgggcaagacatacagtacttcagagaagctttaagaggcattgtgcattcttgctagctctcctgctccttctctctgccacaaagataacatatcccaaacaggagctgctccttcagcatgtatcccctgtccataaagcccaggctgctgggcaccgtaggaacttggaggtggctgaccataggggcccccgggagctgcaccgccatatggtcctcctggagttccagaggggaacatcccaggattggggtgtccatagggccctccaccagctggtggtccataaggccctccaggggcaggacccccataaccaccaccagggggtagcccactaccatactgccctccactattggggggtccagggtagtagctacccggaggggctcctggtgcttgtcctgcagctcctgggcagccctgccggtaaggatagctggccatggtgattct

SEQ ID NO: 17289 - RNA, 2123 nt, Homo sapiens
  source 1..2123: mol_type = other RNA
tcaggccaggcacagtggctcacgccagtaatcacagcactttgggaggccaaggcaggtgaatcacctgaggtcgggagttcaaaaccagcctgaccaacatggagaaatcccatctttactaaaaatacaaaaattagccgggagtggtggtgcgcacctgtaatcccagctactctggaggctgaggcacaagaattgcttgaacccaggaggcagaagttgcgttgagccaagatcgcaccactgcactccagcctggtcaaaaagagaaaaactctgtctcaaaaaaaagaaaaaaaaaaaaaaaaaaagaactcttccagattaaagactaagacgtggcagctaaatgtaatgtgtgatccggaactggatcttggatcagaagaagagcatcagtgggacatcagcaaaatcccagtgaggcctacagagtagctgtcagtattgtgattctccggttttgatcattacattacggttgtatgagatgtaacatttgaggacactgggtgaaggtatttcagaacactgcactatttttgcaacttttttctacatccaacattatttaaaaagttaaaaaataaaaattttttagaaatcgtcaaatgagaatactcatgagcaaaagtttaataaggaataggatgtttacatagcagttttaaagtgtctccccacaaagagaaatagcaattacaaagggaaaagtaaaaactttccagcggaaaactccagcaggcagcaccctcgccaagtgatccaagttaacactacctcttatggggcaaattcacactatgtgcctcctgataagagacactgagaaggacacagcatcacctacttggtatccctgccaaaaatgaataacctgaatctaatcaggaggaaacaccagacaaacctaaagggaggggctttcttcaaagcatctgattatgcccttcaaaaatgtcaaaggcatgaaagataaaaaaagacagaactgtcccaagtcaaaggagactaaagcaatatgataacccagtgcaatgcctaaaccaggatccagtcctcacccagaactttgaccgtttgattatttgtgaaggcattattggtgaaattcaaatggagctggtagattacgttaatattgtatcaatgttaatgtcttagttttgaggactgtactatggctatctacaggggtgtcctgtctttaggaagtgtacactgaaggaatctgaggtaatagggaatcctgtctgcatcttactctcaaatgatttaggaaaaaaaaaatgtgtttaaaaaaatacgttttaaaacaacaaagcaaaacagatgcacacaaagcaaaacagatgcttaaagctacttagcacctacaattttttattttttaactttttaaataatgttggatgtagaaaaaagttgcataatgttaacaactggagaatctgggtaaagggtatatgcaaattcttggtagtattcttgcaacttttctggaagtttgaaattacttcaaaataaaacgtattttaaaaaaacaaaaagtaagaaggttgggtcagaatgtgcatggccatgaatgccaagtaaagatgtgtcacttttattctaataacaacagggagccaccaaaagtttttaaggcaaaacatgatgtaatcaaaggccggcaagatgggacggtctagagttgagcttagtgtcagacaaaagtgaccactaaccagtggaaaagagggacttcgaggtaacttcccagactccagctgatacatgcggagatagacttcagcctgaggtgtggcatcactaacaaagcgaacgactttcagggcatgaaggacatccaagtactgctccttacgatacatcatcaccttggcatgggactcgtggtgtggaggcaagattcccagacggtcatcttttaggagaatttctaatgatttcttttcttcaactccacgaaaccccactttctcataatatactgaacgaaagtttctctgagagtcctcagtcatatttcattctgggacacccgcgcgcgcccagacggcccgggagacaaaactcagcgccgctgccgctgccgctgccgccgccgccggacg

SEQ ID NO: 17290 - RNA, 15352 nt, Homo sapiens
  source 1..15352: mol_type = other RNA
tcaggccaggcacagtggctcacgcccgtaaccccaaccactcaggaggctgaggtgggaggatcacttgagcccaggacttcaagatcagccttggcaatatagcaagactccatctctaaaaaaaaaaaaaaaaaaaaaaccaataagaattaaagaaaagatctggactgtacagtacattctaatataaatgtacacatttagccacagggcctaataaaaagcttaataagaatggtttccctttctattcaggttcaacttaggaaataaatagtgattataatgatattttcatagaaacaaaaacccagttgaggctttacttaactggtattttttttttttgcaccttattttatgaagacacagatttggtttcagaaattcagctactgagctccaactactagggcaggtgaccaccttgaatgtcaggtgaggggagaaattgctccagggtccatcagcagaagagctcatttaattaaccacaaactcaatgcaggacactggcacttaatgatatgggatttcctcatagacatcacaaataaaaatgttgtcttggcagctagtgagagaacacacatgaaacagagagttctggttagacaatgccaacacacagaagggccaaactgaattgcttttcctaccttctgtattatctgaggagtctacagtcaagtccagatgtctatacaacacatagtggcccctatcaacatagccattaatcaaattgacatgtaatattgaacattaattaagtgctaatgtgtaaaaatggacccaagagcggggcctggattcctttcctagataattttataggaaatatgagtggtgcctcttctttagacacggctaaaggtccccagtcaattccttttcttgttggatcatttactataatgatcaccaaccaaatcagcagacatctttattagcaaattcagtaacaggataatctttccaaaatttacaaatatacaatatatttatagtattaccttcagacaacttcagtgcaaagatatacatatagtacattgtgataattatttgtaaaaatatgagacggcataagtaaaaaaagacacacaggatacctccaactataggcaaacagggaaaaatatatttttttcataaagtactgaatgttaacttttttcatctgtttgtaaaaaatatatgtgcaaaagtgtgtttctaattattccctaaatagctggtatagctatacttcagagtcttctttaacaagatttgcggtgtctttaaaagtgtcttctgttgcagaataggttggagttgggtctcttctcgaaggaggcttaggcttagcagggagcgaaggtgatggaggtggtgtcgcagcaacactttccttttgctcgttctccatctgtgcatagattggattttcaaagttggtagtttgtttagattttcgtttgaagagattccattttgtcacctgagttccatcagcagctggtgaagttgggtttgtctctggaactatctcagaagggtttatgggacttccataattcttattatccacattttcagatacagtcacctggattggctgaaccactttgacagcactgtctctggctgagtacattgggttttcaaatattatgggctgcttccccatttccatgacaaagtcttcactcattgccattgacctgtcaatagcagtctcaggtccaaaaccagacactccaatatccatgttaagatctgcccctgatctgaaggtcaccccattcccattttcagagggcttgacgagactgcttaagcttggcagcttgggcagagcaggcaaaagggagccggtccttctatagtggaagaatcctgcaattgccagagctccaattacgacgatcaagaggattgtcaacagcacagctactgcggttgttcctggagagatgccttttgaaaacgccatttcacaatattttccggtgtagccgctaggacacttgcatttggggaggtcagtctcatcaaaatagcaatttcctccgtgcatgcacctgcatggggggggcaggttgataggcagttcgatggctgcatcacactcagtggtgctcccctctataaagctggagccttggggacaggcacagctgtatcctccaggtctcagaaggcagaggtggctgcagatctgtttgcaaaggttgggcactgacttattgtatctgagttgatgaaagattcgaacttgagtgagccaagggttcactaccagcgttttctctttctttccttgcccaaatttattttgtttccatacttctcccttttccttagatatccagtataactggtcttcaaagatgtccaggctgtaagggttcattgcttcctttgcaatgactctcctatcagtcccatcatattttatggtttcaataacgtcctccttgaagtcactccagtagattcggtcattgttcaaataatcgatagaaaggccagttggccaaccaaggtcctcgaaaaccaggatgttgcggtcctctccattcatccaggcagactcgattttaggttcctttccccagtcagtccagaacataagccctagtttgggattcacagcaatagcagctggttggtccaggtcagtggaaatcagccactttctgtaccttccatcaagtttagccacctcaatgcgtttattcttgacatctgaccagtaaatatgccttccaacccagtccactgctattccatctggctgcattacgtatttcagtttcaggtcaacttcctgcacaagattattgcggccggattcaaagttggggatgtaggcacgtttgatagcaccaaacctagagccctcccctcgcacagtgtaatacacaacactgaggcctatgtccttgggatcccaatcataatcaacagcttggatatattcctcatcttgaagatactctgagaacctctcagatgagagattatattttcgaattcggacattgtcaggcagtagcaacaaaggagagctaccctcagctgcacatcgttttccagggcggtcactcatagacgtgaagccatcagcacagacacactcataacttcctttggtatttctgcagtgctggggacaagtcccaaattgttcacattcattgatatctagacaggaggttctgtcaaaaacattggtttcgaacccagctgtacaggagcagataaatcctccttcatttaattgggtacaattttgctcgcatatattttcagcacatgttctttcttttcctttattgcaacccagttcatcggaccagtcaccacagtcatcggcatcatcacacacattgtcatgtggaatgcaatgcccattgccacacttatattcatattctgtacaaggtttaggggtcggttttctacagtgctcctctgtctcatcagttccatctccacagtcatccacaccattgcacacctcatgactataaatgcagcgattgttgtcacaccggaaacggtttggtgaattacagggaacatccaagcacaggtgaagttcttcatctgaaccatcgccacagtcatcatcgccatcacatttccaatatggcgggatacaaacatggtttttgcattcgaacatagtagcctggcagtatgcaccatcaggaaagcgtgtgggacaatcagcttcatcagacgcatccaaacagtcagcggatccatcgcatttcagttcactgtgtacacaatgtccacttgtacactgaaaatattcaggatggcaggtcctcatctcacagtcccgttcatctgagttgtccccacagtcgttgtaatggtcacagatccatcgcgagggaatgcactgctgattgacacatcgaaactcgctctctgtgcactcccggggagcacagttttcctcatctgagttatctccacagtcattttgcccatcacactgccaacgaagagggatgcagtggtgatttttacagcggaaatcccccacaggatggcatgtcctctcctcacagccttgctcatcactgttgtccctgcagtcatctacaccattgcacacggcccactttgggatgcagcggtaatttgttttgcagctgaattctgtgaagttgtcacagagatgggcagagctcatgcattcttcaatgggctcatccgagtggtctccacaatcattatccacatcacacttccaggcctgcgggatgcagcggccattagcacaccgaaactggcccggccggcaggtcctgctggcacagtgggaactgtcttcatctgagttatcctcacagtcgttaaatgtgtcacactgccaggattctgggatgcaacgtttgttggcgcactgccattcattggagtcacagtggtgattctcacaaagaagacggtcttcatcagacccatcagggcaattttggtgagcattgcataaagtctgcgggctggtgcagttgccgtcactgcactggaactgtcccagtcggcagaagcgctgcgggcaaagggccagttcatcagagccatctgagcagtctttctgtccatcacatttccaccagataggaatgcacttttcattgttagcgcacaggaactgggtgctggagcacatgggcatgcagtaggtgctgccactcagctgaagggtgcggaagtcatctggacactcgcaagtgaacccttttcctcctggcttgatgaggcagagatgagaacagccaccattgttggtaccacagggattgctcacaatgggctgcctatatggatggtacacatggatgtcaaatggtctgtgtgttgtgttcaccagtgtctgtctatttgatccatcatatttgtttcccttttccactgtccttgtattccaatctgtccaataaatagtgtcttcaaaaatggtaatagcgaaagggtgaggcagtgccccatcatacaccgtgtgtcgatggtggccctccaaatcagagtactctatgtaacccaggtgggcatctgcccagtagagtagatcattggtgtaatcaatggtgatgccattaggccactctaacttggtggagattatcacagacttgttggttccatccatgcctactctcccaatgtatgcgcggtgaccccagtctgcccagtagaggtacccatattgagggtgaagggcaagtcctctgggattatcaaagcagaaggtgttgttggcatccacacagtgctgggccagcatgcggcggtgtccaccattgaggtcagagacaaagaggccatccaggcgggcatccaaccagtagagctttctggaaacccagtctacagccagactttctgcagctggtagtctgtggtttatgattgtctccttgtttgtcttattcagaaacattctctcaatgacttgcctctgtgtatcaatccaatacaatctcttctctactcggtcaaaatctaatgccacaacattgtccagtccttccaagatgagggagtaaaaatagccatctatagttaaatttctcaaatagtaacggttgctaaaaatgagatagggttcgatgttactgttttgccggcaggtctttccatctggttctcggaggtagcctggggcacacttacagatgtaggagcctattacattctcacacttctggctacagacaaaaggcatctctgtgcattcatcaatatcaacacaagtccgcttgtcagacatgagcttgtaaccaggacgacaggaacaatagaaactggttaaggtgtctgtgcagttgtgatcgcagccactgattgaagggtcatggcattcattaatgccacagcctttctcatcgctgttgtccaaacagtcatctaggtggttgcagagtttcatcatctcgatgcagcgcccattgtcacacttgaactcgtgaggtggacacgtgggttctggggtgtggcacaggtgcatcagctcatcagatccgtctccacagtcattatcctcatcacagacgaaggttttactaatgcagcgcccgttctgacaggtaaactgattctgttggcaagtctggtataagcagcccctctcgtcgctatagtcaccacagtcattgtgccggtcacacctgaatatctttgggatacacagtccgtaaccacaggtgaattcattttcagagcaagttctcctggtgcaattctgattctcatcgtagccgtcagtacaatccacatcgccatcacagacccaagactggggaatgcacctcctgtccggaggtctgtcatttacacagagaaactcggaatccgagcagttttgattctgacactggtgccttttatcctcgtcactcatatccccacagtcattatcaccgtcacagatccattcgcttgggatgcacctcccaccatcacacttgaactcatcagctaggcatgttcgctcagagtgaccacaagaggcaggttcatcagaggcatcaaaacaatctgtttcttgatcacaataccaatgttgaggaatacagcgcccagatgcgcattggaactcactgctgctgcacgtgtgagtggtgcaataagtagggttttcatcactgttatctccacagtcattgtctccgtcacacaaataaacgcgaggaatacaaatatttgaattatgacattttgtgtatccagactggcaagtgcgatcagggcaatttttctcatctgaagtgttattatcatggcagttgtctacaccattgcagataaactcacgaggtatgcaccttctgttattgcacataaactccgtggtggcattgcagtccctgaacaggcaccctgcctcatcactgccatcaccacagtcattgtagtaatcacagcggtaagagtattggacacatcgcccattggcacaggtgaaggctgtcggtgagcaggtgtgaagtgcacagacactttccatctcatcactgccatccccacagtcgttgtcattatcacacttccactcttccgagatgcagcgcccattggagcaggtgaaggaagatgcaccacatcgttcaccattgtccacaatgcagtgcttcctgttgttggccaaataccagttgccctcatgtggacactggcactcggcaccatttggacctggtgcacagatatggctgcagcccccattaaactgttcacaaggattgttacactgttgtttctggttcttcacaacagtgttgattcccctgggctgggagagcaaatttgtggtcattgcaatctgacctgacccgtcatatttgttagctcggtaaattctttgtgtgtacaagtcagtccagtaaatatactggccatagagagtcaagccaaaagcatgaacggctgcattgacaatgacttcacgatccacgcccgtcagagtgctgcgttcaatcctctgcagactagcatccacccagtagagaaggtcctcttcatagtccagagtcagcccactgggcatgaccagactgctgttcacaatgggtacgcggaagtttcctcccaatgtggctctctcgattttggcatgtgtatcccagtcagcccagtacaggtacccttggcagggatctaacacaattgctcttggttttggaacgcgggctatcacagtgcggttagacccatcttcagccatggaattaatcatctggttgaggtagtcactgtaataaattcttctagtaatccagtcaaaggcaatgccatcagcagtccctatacctgaagcaatgacagttggagtatggatccctgaagacagggtggcataggaaatctgtccaactccagaggctaaattttgtgtgaagtagattctatcacttacactgtcatagtctagagacatgacagttctttccacatttattgtttggaaaggtgggctatggttttcagggtccaagtgtaagcttctcaaggaattagacaaggcaaagatgaggaaattttctgttgaaatggcacaattcttgccatcactttgcagggtcccaaaggcacagtcacattttggggtgtgcaatccaggcagagcaaagcagagatgagagcacccaccattgttttccaagcaagggttgttgttgacctctgctggtgaccggggctggacttgcttgtcaaagatggtcacatctcttagccagttgatattgtctcttatcactgtgggtggctctgtgttctctggttccttgctggcttggaagatctttttcaaattcctatctacccatatgatagaattttcaaaaacagtgatgccataaggagttgggtaacgactgccataacgaatcacttcagagttctctccattgatacgaatccttgcaattatatctaaagaatcatcaacccaataaacgtagccatcacttcggtccactgccaagccccgtggtgtgacaatgccctctgacacaagcactgttcgattggtacagtcaaggaaagaacgctcaatctttggtctctgcccatagtcagcccagaagaggtatctgttcttgggatctacaacaatatgcctaggcatgtccactgtgactttaagaagaacacggcggtaagtagtattgatccgcagaacttctatcagtgtttcagaaacaaaggcattggtgaaataaagatttcctgctacccaatccactgcaataccccggactccattttctcctattccatgtgtcacaatgttcatcagagaagatccatctggtttaattctacggatcgcattatcagatgccactgagctgctaaaatcacaccaataaataaagccagaggacacatccacatccacatgcagtgcgtttcgtccttggcctgccaccggcaccatggtttctgaatgatctgacaattccaagctaaagcctctgattgcagacagcattgaaacaacaatgaaagagttatatggagagcaggaccgattatcaggattgagtttaaatccagtggcacaggcgcaggaaaacaatcctcctggtacaggcaggcaaatctgctgacaggcattcatgttgttgctacagccatttgaggattcggcggcattgcgtctgtgataaacttgaagacccctcagatttggaacattatctctcaagactattttgttggccccagtggccttatcaactctttcaatgacctcatactgttcatcagtataataaaggaaagaatcatggactgcaattccccaggggtgggaaagctggtgtaccaggatcattcgatctgttccatccacgtttcctctttcaatcactcctcttccagtgactgcccagtagagtttctgctcttcgatgtcaagagtgacacactccaggtgttcgaggttcccagtaaagagagttttcacagatgtgccatccatgttagcactggcgatcttggcaggaaccccactgtcagttccttggtctgaccagtacagcttcccacgagcaggatcaacagttatgccaattggaaagccaactccaagagctgtcccatcattggcaatcaatgtttttctgtatctgatatctccgtggagtgtcaaaacctcgattgactgagttctaggattggtagaataaaggtttcttgaaatccaatctaaggccaggttcatagaaggccccaccatagatatagaagcaaatactgtcctgttggtgccatctgtcttcactctgtgaatttcacctggattttcaacccaatagatgtattgctcagcatcatcaaattcaacatctaaaccattctgtatccctgctatggggaccatagcatcattgctcttcacctcaggattaagggagattccaaaaattatatgttgccttacagttattaagaaaggttgatcatctctcaagcaattcaggagatcaggagacagactccatcctgaaggacaaacacaggagtaaaaatgaggcccctgtgaggaaagcaggcagagatggctgcagcgggaaaaggcacatggattcacggaatttggttgtttcgaaggatgaaccgcaacaatcccaaggggccattgaatattatacattacaactgactggttccctccatgccacttgttggctcgcataacccgacgagtagcacggtcagtccagtacacagagtcttcaaagagagttagggcataggggtgccgtataatcaaatcactggctatcacctgtctccgatggtgtccattataatcacaaaagtccatgtaatcaagataggagtccatgaagtagagcagtctgttggggtagtcaatagttaagccgcagggccagaagatcttgtcctggacaatgacagtgcgcatgctgccgtccatgctggctcgctcgatgcgagggtggtggccccagtcagaccagaacagtagatgctcattcattctgggatctaatgctagtcctcttggatttgttaggtttttactaatcagcacagtcctgtggctcccatcaattttggagacttcaattgtttccagagcatagtctgtccagtaaagattacgacctacccaatctattgcaatagtttcagtcaagatgatgctactgtcaaataccactcttctgtccgttccattttgaaacgcactccaggttttaccctgagttgcatcagaccaaaagatacgaccactaattgaatcaaaatcaacagctacaatgtaagaaccattctcgaccaatgaatagatattgtggacctgggaggtgacactgtcggcaataattttgttctgacttgccacaagtaacagcagactctcagatgctgtaactttgcaagtcctcccatcactttctaacatgtagcctgtatcacacgagcaccggaaagaacctctcatattgtaacagtgctggctacaagagcctagaatatcacattcatctatgtcttcacaggtcttagaatcattggcaagtaagaatcccaatggacataggcatttagccccaaagggctcttgaacacactcgtgagtacaaccaccattgaaatctgagcagctgttcccattgcaaagtggggactcatctgtcccattggggcagtcaaagatgccatcacacactacactcagattcacacagatgttatggccaagacactgccattgccaactaggacagcgaaagggctgagtagggcagtccttctcatcactcatatccccgcagtcattgtcccgatcacagagccatgccctgtggatgcagtttccgttgtcacagtggaaatatgatgaagggcaagtcttggggacacaggcattgtgctcatcagatccatagaggcagtctggatgcccatcacattcccagaagttcgggatgcagataccatcttcttggcactgaaattcatctgagtggcacataccaggaggcctggttggacagcctgcttcatccgagttgtcactgcaatcaaaaacaccatcacaacgatttgtgacgccaatacatttatccccactggcacacttgaattgagaagcagtacagtttaatacacaaccaacctcatcagatccatcaacacaatccttgtcaccatcacagacaaacgataggtcaatacatcgatgattggggcaattaaactgactaggttggcatgtctctgtcgaattgcagttcttttcatcagatccatccccacaatcattgtctgtgtcacagacccagttctttgagatacactggtgattatcacaggtgtattgggtgtcaaggcaggaagcaggtgcgtgggtggggcagttgtgctcatcactgccatccacacagtcgttgcgtttgtcacagcgccagtgtgcaggaatgcactccccatggccacaggtgaacgccgaagatgaacaggtattattaagtgtgccacatagttgctcatcactgttatcatgacaatcatcgactccatcacagagatagtaattgggcacacatctgccatttttacaggggaaggaaaataagccacactgctctgtgggtggttcattggttgggtccccctcgcatgtcaagtgattggaagccagcctcattccataagggcacccacacactcgctggaaatttggcaccgggaagcagaagtggctgcagtcaccgttaggatgcgtgggttgattacaggcgttagaaccagtctggatgttgacatcatacgatttcaaatgcagtatgtaagcaatgccacttcggataactgtcatttctccaccatctgctttcctgactcgaataatggcacccagtctccagtcagtaaaaaataaatgctctccaaagatggcaagtccaaacggatgtgtcatctgctctatatggcccagtcttcttctgtctaaaccatcaaaggtgctgtgctcaattttatcaaaataggcatctacccagtacaatcgtgaagcagcccaatcgatggccaagccattgggccatccaagagtagtgtttattacaggcaagaggtgagatccgtcactccatgctctcataattttagcaggacggaaccaatcagtgaagaatagatacccggcaaaaggatgaactaccaccgaccgtgggttatttaaatactgaactactgtgcgtctcgttttatcagctagcctcatgacactgatactcttgtaatgagagtctgtccaatagagattctttgaaatccaatcaaaagccaaactttcaacattttccaccctgttagctgcgagaatttctcttcctgtgccatcaatcttttgcttaaaaatcatgtgttttgacatatctgaaaaaaagatagtgctgtcctgggcgtcaaaatcaatcccgacaaagaaagaaggattccccgaaactggaaccatgacatcttcctgggtagacaaggtgaacgggatcccacgaatagcaacttgggatgaaaaaatgaggaaattctgaacagcaatgcagtggcgctcatctgtatccagttggaagccgaatgtgcacttgcaacggaaacccaaaccatcattatctgttctgtggctgaggacacagacctgctcacagcccccattgttatctttacacggattggtagcatagggctgtctgagggaatggtaaacagtcactccatagggcctcagggaagcctggtagtacacttgtgggttggtctctgtgaacttgtttgccttcagcacggccatctttgtccaatctgtaaagaacacctgaccttcaaataagcttactccaaagggatgaggaatgagggagcctccatgaactacagtcttcctttgaattccatcataagttacagtttcaatgtaatcaaaccgagagtcaacccagtaaacacgcttcgatatcatatccagagttaccccagcaggccatcccagctttgttttcaccaagtctttacggttgctgccatccatgaatgccctttccagcttaggttccccagaaaggctctcccaatctgagaaaaataaataaccaacagttgggtccacggcaattcctctaggatgccccaagttttcagttataagggtaacccgatagcttccatccaaatttaccatatctatgcggttgaccttggtttccactagatagattttattattaacccagtccacagccaggttctctggggtttcaacagaaacattgagaacctcttggatatttaaaccattaatgtcaactgaaaaaaccttattttgcacggtgtctgtccaaaaaactctttgcaggtgatagtggaaagccacacccacggccactccacgattctgagactccactaggatccggaagctccttccatgaatatcaccaattaacaaatcccgaccattggagaagataatggaggcctcgccaaaggaatcattagctttgcaatactgtccacgctccaagatatacccttcttcacagtggcacaggtgacggccaggtcggctttcacacttctggtcacaaattccccatatctggcaatcatcaaactcaacacaggtacggctgtcattgtggttgatgatataacctgggggacaaaaacacgctcctccatacggcgtctcatggcactggtactggcagttcaaggcagagcacagagtcatactacagtattttccggtactagtgttgttttcatcttctcttcctgggcaatctaaaatcccatcacaaactttataaatggagatgcatcgtcccgactctgggcaagaccattctcttggggaacatttatgaacatcatgaggaccgctttcacatccatcttcatctccattatctttacagtcatcttctccatcacaaacccagttttgataaatgcatcggccactggggcaagtgaactggtaaccaccgcaggtcggatagttgcaagcatgttcgtcactgccgtcttggcaatcattgtcatggtcacagacataagcacgagggatacactctccattgccacatgaaaactcattgtgcaagcatatctcagtgcagttgatttcatctgaggagtccctgcaatcaactttccaatcacacttctgactggtgttatagcaggccccattgtcacaagtaagctgctcacatgttgggtactggcagtcattctcatcagctccatcggggcagtctctgacgtggtcgcacctgtattcacttgggatacactgaccattggagcatgttatctgatgacttgagcatgtactttgtgagcaatcttgacgttcatctgagccatcatcacagtcttgatcttggtcacacacccaggagttggggatgcattgtccctcactctggcacttgaaatagccctgctggcaggtcacaacagcgcagccaatttcatccgcgtcatctgaacagtctttggtcccatcacacctccagtctgcagggatgcaatgcccacttccacagcgaaaatgcgcactgtcacattcttggccactggccggcgctaggcaggcgacgagagccaggagcagcgtgcacgccactgctgccggcccgcgatccatctccgcgacggtccccggcctcgccgttccttccccgggaggtgggcgcgcgtagcacaccgcaccggcagcgcctctgctagcgaacgctcctttaggtctgcacctccgccagctcctagtggccaaaagcct

SEQ ID NO: 17291 - RNA, 2207 nt, Homo sapiens
  source 1..2207: mol_type = other RNA
tcaggccaggcacagtggctcacgcccgtaatcccaacactctgggaggctgaggccagtgatcacctgaggtcaggaggtcgagaccagcctggccaacatggtgaaaccccatctctactaaaaatacaaaaattagacaggtgcctataatcccagctactagggaggtggaggctgaagcaggagaatcgcttgaatctgggaggcagagggtgcagtgagccgagactgagccactgcaccccagcctgggcaacagagtgagaccctgtctccaaagaaaaagaaaaaaaaaagtgtatgggtgagtgaattttagtatattcacaaagttgtgcgaccatccccagacataactcccaaaccccacatccatcacccatcagtgataacttcccacttttccctccccagcccctggcagccactattctgctttctgcctgcctgggtttgcctgttctagccattttctatcaatggaatcatagaccgtgtggcctttgtggctggcttctttcactcagcatgacattttcaaggttcatccatggggtgctgtggaccagcactctgtgcctgtctgtggctggaaatattccaggacttggtgttacgggctgagcttgagttgtgacctcttcaaactccaatgttgaagtcctaaccctcagaaactcagaatctgactgtgtttggagacaggcaaagaggtaattaaattgaaatcaggtcactagggtgggccctcatcccatctgcctagtgtccttgtgggaggagatgaggacacacacactgagggacaaccacatgaggacccaatgagaagaggccatctgcaaggcaaggagagaggccttagaaggaaccagctccaccaacatcttgatcttggacttccagcctccagaacttcttgaaaattgttttcaattattgtactccatttgtggaactcgtgtcggagtctggtaaacagccgaatgtcttcctcccctacagtttcctctccttgcatgagagcagtgatgtcctgattaaaggcattaactttatctatcaggaagaacattttttcattttcgtcttccggtatgtcgacaccatacttttgtagctcctctgttattctctggtgagtctccttgatttgattttctaacaggggcagagatttacagatatgtgtgatgagctcgctggtaagtttttctgccaggcagggaaccgtggcctttccttcctccagcagatccctgaaatatgggtggttctcaaagaagatcttctctctctgcagggcttcggacaggctcagctggtcctggatctcctgctggccccggcacttgacaatcatgtaacccttcttcaggtggaacacgaggttccgcaccacgtccacaaccttgtcttcagttcctttgtccaccagatcaggcttcgtcaagattccgatggtcctgtctccctcggggtccacctcctgggccatgctgagagcctctgtggtggcgatgtccacattactggggaccaccaccaggctgattgtctcctgcctctggatgtacttcttgatgagtgtcttgatcttatacccaatgtcagcaggctgattgcccacagccactctggttatgccaggaaggtctattagagtcagatccgggacatctcgggagctgatctccagggtgattagctcatgactgattcccattccttccccggcgatggcattctgggctttattaatttccttttctacctctgaagcatccgaaatctcaatctcgtagtcctggtaactgaccttgcctctccacttatcttcgttcacaagtttcttcagtttcagcaccagcgggcatctggtcacgatcccgctgcctctgggaagggcaactcctgacagtgcctccaacacggagctcttgcccgagctctggtccccgatgacggcgatggctggcagggccaggtcctgctccacacctagagcccgcagggagtcaatgaggtcgatgcaggggcgcaccttctcctcatactggctgcacaggttgttctcagccaccgagcctggatttttctgggccacagtagcatctccattcagtaatagagggtgggatgcagcagctggatcagcttttgcgatgtccacttcggaaacaaccatcttccttctttgcaaa

SEQ ID NO: 17292 - RNA, 27 nt, Homo sapiens
  source 1..27: mol_type = other RNA
tcaggccaggcacagtggctcacgcct

SEQ ID NO: 17293 - RNA, 36 nt, Homo sapiens
  source 1..36: mol_type = other RNA
tcaggccaggcacagtggctcacgcctataatccca

SEQ ID NO: 17294 - RNA, 67 nt, Homo sapiens
  source 1..67: mol_type = other RNA
tcaggccaggcacagtggctcacgcctataatcccagcactctgggaggctgaggcgggcagatcac

SEQ ID NO: 17295 - RNA, 4871 nt, Homo sapiens
  source 1..4871: mol_type = other RNA
tcaggccaggcacagtggctcacgcctataatcccagcactttgggaggccaaggcgggcggatcacctgaagtcataagttcgagaccagcctggccaacatggagaaaccccatctactaaaaacacaaaaattagctgtgcatggtggtgggcacttgtaatcccagcgacttgggaggctgaggcaggagaatcgcttgaacccaggaggtggaggttgcagtgagttaagacagtgctactgcactccagcctggttgacagagcaagactgtctcaaaaaataaaaataaaaaaatagaattagaggttatcgctaactaaatcacttttgctgtacctctgtggagatgaatgcagtagtgttgttaatcaccatcttcaaaggaatctgcatggttccctccttctttgtatcactaattttaaaattgaaggcagatgtttcttccttagctgcaaaaggaggctgagaaaacattacctggtactttcaaattctttaggaggaagaaatgctctgcctcattaggtgagggattccttaaacacaggagttaggatactgggcagccaaaagagaaatgacagatgtctgctacagcccattctcttggccattcaatgtcaacacactccttcagctaattcttccaaaactatattcaaggggaaaggacttgacaatataaagtcacagacatgtcacagtcacagacactgttaattgctttctcaatattctttcttcttgctaatactgattttatttgggacagctatgtaccctgctttctttgcaggtaccagtggccatttaactggtcaggcaattaagtcaagggaaaatccatttgggatttctgagaaagctttgctttccctcataaaaggcgatatatatagctggcacaggccatttccattttttcttccttgccttcaacatggccatgacatttggcttggcaacaactttctagcaaacacaagaaaacagcatgagggatgtaagccaatatggtaaggaggcagatttgaaagacagaactgcaccttttcctgtatatagtaagagtcactgattaaacattattcctttcagttgaatcacacatactctcagctacaccattctagaaaataatatctcattagttaagactccatttattgaattcataatactttataagctgtggtgtttcttttgcactaataaaaatagattttgctaatcaagaaccacttgaactcccaacagtatttggcatttaggcatctcaagttagttagtgattaaaaatgtgcttaagactctgtctgggtttgaatcttggttccagtttggacaaataaccacctccttgtgcctgagtatctgcaaaatgaggtacagttaaaatggagtttatataatacagtacctgacaggtagtaaagcactcaatagatggtagctattattggcaataccatacatactttgcttttgtggcaccaaagttttctatttccctcctacccatttattatctctattgaattctcaagtttaaagtccctcttctgtatcttatacatactataatggatttatcacactgcattataattttatatatatacttgtctcctgtaccagactttttcatttttaaattcataagtactaatgaagtggttggcacatagactattttctttttcatcttttagagtgctaactattacacaatggggcctagactagatattttaaaatcagtgtctttaggaattgtttgagatgattagaatacaaattcttgaacttcatcaccaagtttctatttcagtaggtcagggaagcacattttgaagaacactaaaatagaccttcaatgtttgaatccaattatgcataaggtattaatataagaattatacataagatattgatataatactacactaatataaggtactatttgtagagttatacactgctgaatatactgtgctaattacaaagtatttatgactcttgtgaggaccacttgacaaggttgctatatatatgtaaaaaaaccctctgcacttcctcatttgacttactactgagtaaaattagcttatcttctcaaaatgcagtttttgttagaaaatataattttgaactaagatttttgcaaaccaggcaagttcttcatccactcaaggagaaactttaaaatccacttaaaatgaagagcattcctccccgactcaattttctaactacatattatcttcatagcattaacaccagccagaatttatattatgtagagcactaaaagcttcttagacttgtacctcaggcttttaattttgcagggggaaaagttagtatgtcgatttatcctaacacttgagatataaagaactttataaacagctctaaaggaacataaagcacataaagggacaccatattataccttgatttgattacttcatcattttcactgaaatctggccatggtaggtttggccgtggctgccaaatggtatagagtacctgcctcttgaatggatttatggggtcacttaaggtatacttcgaggcagatggctgggctaatagttacttacttactcttgggaaatgaaataaaaaatgctcacacttggaagtgttttttttgtcaaattctatgcaggatatcaaacagaaatttgaaaaattcttaaatgacatatacctattcattaacacccactgctctagatgacatccattagttattactgggatcagatgcttttaggacatctttaaaatattttgttattttaactgtagttctttatagcattacgaaagaaatatcactcacataaagcactaacaactctttttagtactgtgtctctcccatgcagtatggtgcttaatgttactggaaaatattgacaggtttagcattatttcaactaattctgggcaaatctaaatagaatagtataacatgaagaaatttataaatttgaaatgtgagtaaactgggacgggaatgagttgatgagtgaacccagttgaccactgggcatttgaatctcaatgttgcctacacagcattatgagtgtaataattttcattaggtaacaaaactgcttcctcacctttttatatagcttaaacaaaaaaaaagaaaaaagataaaaaaaaaccctgcttctatgtaaacaaaaaaaaagaaagccaactattagtgctaggaatgaaagacatccaatccaagtaagtgatggttcttaactataaaatggaaattgtataaaaattaaaatagaatgtagaactagtaggataacattgaaaaactgactacttatatttgttttttttattttgtgtgtgtttttggctgattatatttaataaaagctacttttagtatttgaactaagtgcacatgtgtgcattcacatacacaggacaagctcctcagctttgaacaatatgaactttggacaatatgacaactatagcatcactgggcaaaaaaaatagctgacttatttccaagtgtgtttcctgggactagcagtaggttctctcaaattaaaagtaaaggcaccaggctataaagtgccaattcttagcaccagagagacttaaaatgtcacaggtgaatgacattacaaatcagagaatctgctgatctagttctgtggaattgtattatttttgtcaaatggaaaaaaaaaatcaaggtttatgccaaatagatttaaacagttaaatctttcctaaaatttcctagaagtgtattttacaatgctatgtaaaataaattgctggcttataaaaaatgctcaaagtttcagagatgtgaaaaataacaaagaactgaaaacatagtttatataaatcaaggtcccagaaatgaaaattaaaagtagtctctttgagaaaggaatggtgaaattcagcatgtagtattcacattaacacatctgagaactgtggacagccaatattgactggaattctaaattgccacctgatacctttaattaagattaaatcaaatctgaggcaagacacttaatggacagtacttgaatgggaagacagtaacttccttccttgatagacaatctccagccatcattcagagttcagttatttgatggcttgggaagcagtgtccattgagttttcctttctggcttgaagagactcactgctgatggacaataattctcgaagttccttattttcaagctctaattgggctaatttttcctgaatcttacaaaactggtcatcatccacctgaactgctttcctcatcacttctcccatttcacagattctgtcaatctgactctcaatttctgcagagtgagactggtgagctttcaggactggttcagcatccaccgcttttttagcaaccattaactgtaacatctgtttccgatatttgctcatgataagttccaaagcatcctggtgttcctccaaggaaatccatagctctctgttttcctgttgcaagtctctaatctgtgtgttctcttgggacagcagaatgtgaggtttgtatttggacatgtccttcatatcggatgcatcctcttgatacctctgcctgacctggtccggaagcgctgtccccgcctcccgcatagctgctacccgccggtgcagcgccgccgactgatccaccagcgactcggcggccgcatcgtgctcccgtagcctctccagcagcgtcttggcgtctgtcaggatcttctcgatggtgcagctcatagcagcagcaccaccccagcccctgccgggctcagctacgcgactcgctcagatcttctgggagtctgtctcagcatt

SEQ ID NO: 17296 - RNA, 4921 nt, Homo sapiens
  source 1..4921: mol_type = other RNA
tcaggccaggcacagtggctcacgcctataatcccagcactttgggaggccaaggcgggcggatcacctgaagtcataagttcgagaccagcctggccaacatggagaaaccccatctactaaaaacacaaaaattagctgtgcatggtggtgggcacttgtaatcccagcgacttgggaggctgaggcaggagaatcgcttgaacccaggaggtggaggttgcagtgagttaagacagtgctactgcactccagcctggttgacagagcaagactgtctcaaaaaataaaaataaaaaaatagaattagaggttatcgctaactaaatcacttttgctgtacctctgtggagatgaatgcagtagtgttgttaatcaccatcttcaaaggaatctgcatggttccctccttctttgtatcactaattttaaaattgaaggcagatgtttcttccttagctgcaaaaggaggctgagaaaacattacctggtactttcaaattctttaggaggaagaaatgctctgcctcattaggtgagggattccttaaacacaggagttaggatactgggcagccaaaagagaaatgacagatgtctgctacagcccattctcttggccattcaatgtcaacacactccttcagctaattcttccaaaactatattcaaggggaaaggacttgacaatataaagtcacagacatgtcacagtcacagacactgttaattgctttctcaatattctttcttcttgctaatactgattttatttgggacagctatgtaccctgctttctttgcaggtaccagtggccatttaactggtcaggcaattaagtcaagggaaaatccatttgggatttctgagaaagctttgctttccctcataaaaggcgatatatatagctggcacaggccatttccattttttcttccttgccttcaacatggccatgacatttggcttggcaacaactttctagcaaacacaagaaaacagcatgagggatgtaagccaatatggtaaggaggcagatttgaaagacagaactgcaccttttcctgtatatagtaagagtcactgattaaacattattcctttcagttgaatcacacatactctcagctacaccattctagaaaataatatctcattagttaagactccatttattgaattcataatactttataagctgtggtgtttcttttgcactaataaaaatagattttgctaatcaagaaccacttgaactcccaacagtatttggcatttaggcatctcaagttagttagtgattaaaaatgtgcttaagactctgtctgggtttgaatcttggttccagtttggacaaataaccacctccttgtgcctgagtatctgcaaaatgaggtacagttaaaatggagtttatataatacagtacctgacaggtagtaaagcactcaatagatggtagctattattggcaataccatacatactttgcttttgtggcaccaaagttttctatttccctcctacccatttattatctctattgaattctcaagtttaaagtccctcttctgtatcttatacatactataatggatttatcacactgcattataattttatatatatacttgtctcctgtaccagactttttcatttttaaattcataagtactaatgaagtggttggcacatagactattttctttttcatcttttagagtgctaactattacacaatggggcctagactagatattttaaaatcagtgtctttaggaattgtttgagatgattagaatacaaattcttgaacttcatcaccaagtttctatttcagtaggtcagggaagcacattttgaagaacactaaaatagaccttcaatgtttgaatccaattatgcataaggtattaatataagaattatacataagatattgatataatactacactaatataaggtactatttgtagagttatacactgctgaatatactgtgctaattacaaagtatttatgactcttgtgaggaccacttgacaaggttgctatatatatgtaaaaaaaccctctgcacttcctcatttgacttactactgagtaaaattagcttatcttctcaaaatgcagtttttgttagaaaatataattttgaactaagatttttgcaaaccaggcaagttcttcatccactcaaggagaaactttaaaatccacttaaaatgaagagcattcctccccgactcaattttctaactacatattatcttcatagcattaacaccagccagaatttatattatgtagagcactaaaagcttcttagacttgtacctcaggcttttaattttgcagggggaaaagttagtatgtcgatttatcctaacacttgagatataaagaactttataaacagctctaaaggaacataaagcacataaagggacaccatattataccttgatttgattacttcatcattttcactgaaatctggccatggtaggtttggccgtggctgccaaatggtatagagtacctgcctcttgaatggatttatggggtcacttaaggtatacttcgaggcagatggctgggctaatagttacttacttactcttgggaaatgaaataaaaaatgctcacacttggaagtgttttttttgtcaaattctatgcaggatatcaaacagaaatttgaaaaattcttaaatgacatatacctattcattaacacccactgctctagatgacatccattagttattactgggatcagatgcttttaggacatctttaaaatattttgttattttaactgtagttctttatagcattacgaaagaaatatcactcacataaagcactaacaactctttttagtactgtgtctctcccatgcagtatggtgcttaatgttactggaaaatattgacaggtttagcattatttcaactaattctgggcaaatctaaatagaatagtataacatgaagaaatttataaatttgaaatgtgagtaaactgggacgggaatgagttgatgagtgaacccagttgaccactgggcatttgaatctcaatgttgcctacacagcattatgagtgtaataattttcattaggtaacaaaactgcttcctcacctttttatatagcttaaacaaaaaaaaagaaaaaagataaaaaaaaaccctgcttctatgtaaacaaaaaaaaagaaagccaactattagtgctaggaatgaaagacatccaatccaagtaagtgatggttcttaactataaaatggaaattgtataaaaattaaaatagaatgtagaactagtaggataacattgaaaaactgactacttatatttgttttttttattttgtgtgtgtttttggctgattatatttaataaaagctacttttagtatttgaactaagtgcacatgtgtgcattcacatacacaggacaagctcctcagctttgaacaatatgaactttggacaatatgacaactatagcatcactgggcaaaaaaaatagctgacttatttccaagtgtgtttcctgggactagcagtaggttctctcaaattaaaagtaaaggcaccaggctataaagtgccaattcttagcaccagagagacttaaaatgtcacaggtgaatgacattacaaatcagagaatctgctgatctagttctgtggaattgtattatttttgtcaaatggaaaaaaaaaatcaaggtttatgccaaatagatttaaacagttaaatctttcctaaaatttcctagaagtgtattttacaatgctatgtaaaataaattgctggcttataaaaaatgctcaaagtttcagagatgtgaaaaataacaaagaactgaaaacatagtttatataaatcaaggtcccagaaatgaaaattaaaagtagtctctttgagaaaggaatggtgaaattcagcatgtagtattcacattaacacatctgagaactgtggacagccaatattgactggaattctaaattgccacctgatacctttaattaagattaaatcaaatctgaggcaagacacttaatggacagtacttgaatgggaagacagtaacttccttccttgatagacaatctccagccatcattcagagttcagttatttgatggcttgggaagcagtgtccattgagttttcctttctggcttgaagagactcactgctgatggacaataattctcgaagttccttattttcaagctctaattgggctaatttttcctgaatcttacaaaactggtcatcatccacctgaactgctttcctcatcacttctcccatttcacagattctgtcaatctgactctcaatttctgcagagtgagactggtgagctttcaggactggttcagcatccaccgcttttttagcaaccattaactgtaacatctgtttccgatatttgctcatgataagttccaaagcatcctggtgttcctccaaggaaatccatagctctctgttttcctgttgcaagtctctaatctgtgtgttctcttgggacagcagaatgtgaggtttgtatttggacatgtccttcatatcggatgcatcctcttgatactcgctctccacccttcagtgcccagaatccgagagcactggactcctaccctctgcctgacctggtccggaagcgctgtccccgcctcccgcatagctgctacccgccggtgcagcgccgccgactgatccaccagcgactcggcggccgcatcgtgctcccgtagcctctccagcagcgtcttggcgtctgtcaggatcttctcgatggtgcagctcatagcagcagcaccaccccagcccctgccgggctcagctacgcgactcgctcagatcttctgggagtctgtctcagcatt

SEQ ID NO: 17297 - RNA, 4859 nt, Homo sapiens
  source 1..4859: mol_type = other RNA
tcaggccaggcacagtggctcacgcctataatcccagcactttgggaggccaaggcgggcggatcacctgaagtcataagttcgagaccagcctggccaacatggagaaaccccatctactaaaaacacaaaaattagctgtgcatggtggtgggcacttgtaatcccagcgacttgggaggctgaggcaggagaatcgcttgaacccaggaggtggaggttgcagtgagttaagacagtgctactgcactccagcctggttgacagagcaagactgtctcaaaaaataaaaataaaaaaatagaattagaggttatcgctaactaaatcacttttgctgtacctctgtggagatgaatgcagtagtgttgttaatcaccatcttcaaaggaatctgcatggttccctccttctttgtatcactaattttaaaattgaaggcagatgtttcttccttagctgcaaaaggaggctgagaaaacattacctggtactttcaaattctttaggaggaagaaatgctctgcctcattaggtgagggattccttaaacacaggagttaggatactgggcagccaaaagagaaatgacagatgtctgctacagcccattctcttggccattcaatgtcaacacactccttcagctaattcttccaaaactatattcaaggggaaaggacttgacaatataaagtcacagacatgtcacagtcacagacactgttaattgctttctcaatattctttcttcttgctaatactgattttatttgggacagctatgtaccctgctttctttgcaggtaccagtggccatttaactggtcaggcaattaagtcaagggaaaatccatttgggatttctgagaaagctttgctttccctcataaaaggcgatatatatagctggcacaggccatttccattttttcttccttgccttcaacatggccatgacatttggcttggcaacaactttctagcaaacacaagaaaacagcatgagggatgtaagccaatatggtaaggaggcagatttgaaagacagaactgcaccttttcctgtatatagtaagagtcactgattaaacattattcctttcagttgaatcacacatactctcagctacaccattctagaaaataatatctcattagttaagactccatttattgaattcataatactttataagctgtggtgtttcttttgcactaataaaaatagattttgctaatcaagaaccacttgaactcccaacagtatttggcatttaggcatctcaagttagttagtgattaaaaatgtgcttaagactctgtctgggtttgaatcttggttccagtttggacaaataaccacctccttgtgcctgagtatctgcaaaatgaggtacagttaaaatggagtttatataatacagtacctgacaggtagtaaagcactcaatagatggtagctattattggcaataccatacatactttgcttttgtggcaccaaagttttctatttccctcctacccatttattatctctattgaattctcaagtttaaagtccctcttctgtatcttatacatactataatggatttatcacactgcattataattttatatatatacttgtctcctgtaccagactttttcatttttaaattcataagtactaatgaagtggttggcacatagactattttctttttcatcttttagagtgctaactattacacaatggggcctagactagatattttaaaatcagtgtctttaggaattgtttgagatgattagaatacaaattcttgaacttcatcaccaagtttctatttcagtaggtcagggaagcacattttgaagaacactaaaatagaccttcaatgtttgaatccaattatgcataaggtattaatataagaattatacataagatattgatataatactacactaatataaggtactatttgtagagttatacactgctgaatatactgtgctaattacaaagtatttatgactcttgtgaggaccacttgacaaggttgctatatatatgtaaaaaaaccctctgcacttcctcatttgacttactactgagtaaaattagcttatcttctcaaaatgcagtttttgttagaaaatataattttgaactaagatttttgcaaaccaggcaagttcttcatccactcaaggagaaactttaaaatccacttaaaatgaagagcattcctccccgactcaattttctaactacatattatcttcatagcattaacaccagccagaatttatattatgtagagcactaaaagcttcttagacttgtacctcaggcttttaattttgcagggggaaaagttagtatgtcgatttatcctaacacttgagatataaagaactttataaacagctctaaaggaacataaagcacataaagggacaccatattataccttgatttgattacttcatcattttcactgaaatctggccatggtaggtttggccgtggctgccaaatggtatagagtacctgcctcttgaatggatttatggggtcacttaaggtatacttcgaggcagatggctgggctaatagttacttacttactcttgggaaatgaaataaaaaatgctcacacttggaagtgttttttttgtcaaattctatgcaggatatcaaacagaaatttgaaaaattcttaaatgacatatacctattcattaacacccactgctctagatgacatccattagttattactgggatcagatgcttttaggacatctttaaaatattttgttattttaactgtagttctttatagcattacgaaagaaatatcactcacataaagcactaacaactctttttagtactgtgtctctcccatgcagtatggtgcttaatgttactggaaaatattgacaggtttagcattatttcaactaattctgggcaaatctaaatagaatagtataacatgaagaaatttataaatttgaaatgtgagtaaactgggacgggaatgagttgatgagtgaacccagttgaccactgggcatttgaatctcaatgttgcctacacagcattatgagtgtaataattttcattaggtaacaaaactgcttcctcacctttttatatagcttaaacaaaaaaaaagaaaaaagataaaaaaaaaccctgcttctatgtaaacaaaaaaaaagaaagccaactattagtgctaggaatgaaagacatccaatccaagtaagtgatggttcttaactataaaatggaaattgtataaaaattaaaatagaatgtagaactagtaggataacattgaaaaactgactacttatatttgttttttttattttgtgtgtgtttttggctgattatatttaataaaagctacttttagtatttgaactaagtgcacatgtgtgcattcacatacacaggacaagctcctcagctttgaacaatatgaactttggacaatatgacaactatagcatcactgggcaaaaaaaatagctgacttatttccaagtgtgtttcctgggactagcagtaggttctctcaaattaaaagtaaaggcaccaggctataaagtgccaattcttagcaccagagagacttaaaatgtcacaggtgaatgacattacaaatcagagaatctgctgatctagttctgtggaattgtattatttttgtcaaatggaaaaaaaaaatcaaggtttatgccaaatagatttaaacagttaaatctttcctaaaatttcctagaagtgtattttacaatgctatgtaaaataaattgctggcttataaaaaatgctcaaagtttcagagatgtgaaaaataacaaagaactgaaaacatagtttatataaatcaaggtcccagaaatgaaaattaaaagtagtctctttgagaaaggaatggtgaaattcagcatgtagtattcacattaacacatctgagaactgtggacagccaatattgactggaattctaaattgccacctgatacctttaattaagattaaatcaaatctgaggcaagacacttaatggacagtacttgaatgggaagacagtaacttccttccttgatagacaatctccagccatcattcagagttcagttatttgatggcttgggaagcagtgtccattgagttttcctttctggcttgaagagactcactgctgatggacaataattctcgaagttccttattttcaagctctaattgggctaatttttcctgaatcttacaaaactggtcatcatccacctgaactgctttcctcatcacttctcccatttcacagattctgtcaatctgactctcaatttctgcagagtgagactggtgagctttcaggactggttcagcatccaccgcttttttagcaaccattaactgtaacatctgtttccgatatttgctcatgataagttccaaagcatcctggtgttcctccaaggaaatccatagctctctgttttcctgttgcaagtctctaatctgtgtgttctcttgggacagcagaatgtgaggtttgtatttggacatgtccttcatatcggatgcatcctcttgatactggtccggaagcgctgtccccgcctcccgcatagctgctacccgccggtgcagcgccgccgactgatccaccagcgactcggcggccgcatcgtgctcccgtagcctctccagcagcgtcttggcgtctgtcaggatcttctcgatggtgcagctcatagcagcagcaccaccccagcccctgccgggctcagctacgcgactcgctcagatcttctgggagtctgtctcagcatt

SEQ ID NO: 17298 - RNA, 4753 nt, Homo sapiens
  source 1..4753: mol_type = other RNA
tcaggccaggcacagtggctcacgcctataatcccagcactttgggaggccaaggcgggcggatcacctgaagtcataagttcgagaccagcctggccaacatggagaaaccccatctactaaaaacacaaaaattagctgtgcatggtggtgggcacttgtaatcccagcgacttgggaggctgaggcaggagaatcgcttgaacccaggaggtggaggttgcagtgagttaagacagtgctactgcactccagcctggttgacagagcaagactgtctcaaaaaataaaaataaaaaaatagaattagaggttatcgctaactaaatcacttttgctgtacctctgtggagatgaatgcagtagtgttgttaatcaccatcttcaaaggaatctgcatggttccctccttctttgtatcactaattttaaaattgaaggcagatgtttcttccttagctgcaaaaggaggctgagaaaacattacctggtactttcaaattctttaggaggaagaaatgctctgcctcattaggtgagggattccttaaacacaggagttaggatactgggcagccaaaagagaaatgacagatgtctgctacagcccattctcttggccattcaatgtcaacacactccttcagctaattcttccaaaactatattcaaggggaaaggacttgacaatataaagtcacagacatgtcacagtcacagacactgttaattgctttctcaatattctttcttcttgctaatactgattttatttgggacagctatgtaccctgctttctttgcaggtaccagtggccatttaactggtcaggcaattaagtcaagggaaaatccatttgggatttctgagaaagctttgctttccctcataaaaggcgatatatatagctggcacaggccatttccattttttcttccttgccttcaacatggccatgacatttggcttggcaacaactttctagcaaacacaagaaaacagcatgagggatgtaagccaatatggtaaggaggcagatttgaaagacagaactgcaccttttcctgtatatagtaagagtcactgattaaacattattcctttcagttgaatcacacatactctcagctacaccattctagaaaataatatctcattagttaagactccatttattgaattcataatactttataagctgtggtgtttcttttgcactaataaaaatagattttgctaatcaagaaccacttgaactcccaacagtatttggcatttaggcatctcaagttagttagtgattaaaaatgtgcttaagactctgtctgggtttgaatcttggttccagtttggacaaataaccacctccttgtgcctgagtatctgcaaaatgaggtacagttaaaatggagtttatataatacagtacctgacaggtagtaaagcactcaatagatggtagctattattggcaataccatacatactttgcttttgtggcaccaaagttttctatttccctcctacccatttattatctctattgaattctcaagtttaaagtccctcttctgtatcttatacatactataatggatttatcacactgcattataattttatatatatacttgtctcctgtaccagactttttcatttttaaattcataagtactaatgaagtggttggcacatagactattttctttttcatcttttagagtgctaactattacacaatggggcctagactagatattttaaaatcagtgtctttaggaattgtttgagatgattagaatacaaattcttgaacttcatcaccaagtttctatttcagtaggtcagggaagcacattttgaagaacactaaaatagaccttcaatgtttgaatccaattatgcataaggtattaatataagaattatacataagatattgatataatactacactaatataaggtactatttgtagagttatacactgctgaatatactgtgctaattacaaagtatttatgactcttgtgaggaccacttgacaaggttgctatatatatgtaaaaaaaccctctgcacttcctcatttgacttactactgagtaaaattagcttatcttctcaaaatgcagtttttgttagaaaatataattttgaactaagatttttgcaaaccaggcaagttcttcatccactcaaggagaaactttaaaatccacttaaaatgaagagcattcctccccgactcaattttctaactacatattatcttcatagcattaacaccagccagaatttatattatgtagagcactaaaagcttcttagacttgtacctcaggcttttaattttgcagggggaaaagttagtatgtcgatttatcctaacacttgagatataaagaactttataaacagctctaaaggaacataaagcacataaagggacaccatattataccttgatttgattacttcatcattttcactgaaatctggccatggtaggtttggccgtggctgccaaatggtatagagtacctgcctcttgaatggatttatggggtcacttaaggtatacttcgaggcagatggctgggctaatagttacttacttactcttgggaaatgaaataaaaaatgctcacacttggaagtgttttttttgtcaaattctatgcaggatatcaaacagaaatttgaaaaattcttaaatgacatatacctattcattaacacccactgctctagatgacatccattagttattactgggatcagatgcttttaggacatctttaaaatattttgttattttaactgtagttctttatagcattacgaaagaaatatcactcacataaagcactaacaactctttttagtactgtgtctctcccatgcagtatggtgcttaatgttactggaaaatattgacaggtttagcattatttcaactaattctgggcaaatctaaatagaatagtataacatgaagaaatttataaatttgaaatgtgagtaaactgggacgggaatgagttgatgagtgaacccagttgaccactgggcatttgaatctcaatgttgcctacacagcattatgagtgtaataattttcattaggtaacaaaactgcttcctcacctttttatatagcttaaacaaaaaaaaagaaaaaagataaaaaaaaaccctgcttctatgtaaacaaaaaaaaagaaagccaactattagtgctaggaatgaaagacatccaatccaagtaagtgatggttcttaactataaaatggaaattgtataaaaattaaaatagaatgtagaactagtaggataacattgaaaaactgactacttatatttgttttttttattttgtgtgtgtttttggctgattatatttaataaaagctacttttagtatttgaactaagtgcacatgtgtgcattcacatacacaggacaagctcctcagctttgaacaatatgaactttggacaatatgacaactatagcatcactgggcaaaaaaaatagctgacttatttccaagtgtgtttcctgggactagcagtaggttctctcaaattaaaagtaaaggcaccaggctataaagtgccaattcttagcaccagagagacttaaaatgtcacaggtgaatgacattacaaatcagagaatctgctgatctagttctgtggaattgtattatttttgtcaaatggaaaaaaaaaatcaaggtttatgccaaatagatttaaacagttaaatctttcctaaaatttcctagaagtgtattttacaatgctatgtaaaataaattgctggcttataaaaaatgctcaaagtttcagagatgtgaaaaataacaaagaactgaaaacatagtttatataaatcaaggtcccagaaatgaaaattaaaagtagtctctttgagaaaggaatggtgaaattcagcatgtagtattcacattaacacatctgagaactgtggacagccaatattgactggaattctaaattgccacctgatacctttaattaagattaaatcaaatctgaggcaagacacttaatggacagtacttgaatgggaagacagtaacttccttccttgatagacaatctccagccatcattcagagttcagttatttgatggcttgggaagcagtgtccattgagttttcctttctggcttgaagagactcactgctgatggacaataattctcgaagttccttattttcaagctctaattgggctaatttttcctgaatcttacaaaactggtcatcatccacctgaactgctttcctcatcacttctcccatttcacagattctgtcaatctgactctcaatttctgcagagtgagactggtgagctttcaggactggttcagcatccaccgcttttttagcaaccattaactgtaacatctgtttccgatatttgctcatgataagttccaaagcatcctggtgttcctccaaggaaatccatagctctggtccggaagcgctgtccccgcctcccgcatagctgctacccgccggtgcagcgccgccgactgatccaccagcgactcggcggccgcatcgtgctcccgtagcctctccagcagcgtcttggcgtctgtcaggatcttctcgatggtgcagctcatagcagcagcaccaccccagcccctgccgggctcagctacgcgactcgctcagatcttctgggagtctgtctcagcatt

SEQ ID NO: 17299 - RNA, 28 nt, Homo sapiens
  source 1..28: mol_type = other RNA
tcaggccaggcacagtggctcacgcctg

SEQ ID NO: 17300 - RNA, 33 nt, Homo sapiens
  source 1..33: mol_type = other RNA
tcaggccaggcacagtggctcacgcctgtaatc

SEQ ID NO: 17301 - RNA, 13009 nt, Homo sapiens
  source 1..13009: mol_type = other RNA
tcaggccaggcacagtggctcacgcctgtaatccaacgactttgggaggccaaggcaggtggatcacctgacgtcaggagttccagaccagcctggccaacatggcgaaaccctgtctctactaaaaatactaaaattagcagggcatgctggtgtgtgcctataatcccagctatggaggggggctgaagcaggaggatcacttgaacctgggaggcggaggttgcagtgagctgagatggtgccactgcactccagcctgggcaacagagcaagattctgtctcaaaaaaaaaaaaaaaaaaaaaggaatgaaagaaaagaaaaagaaatagtgttaaatagctctatgaatgctgcagagagggctaccccataggcagtgtgtggggagtatacaaagcttgttctttggctcctcaggaaggggatcttatcaagaatattattcttttgtggtattgtcagtggaaaggagagatgtaacagcagtctccgagagagggagccttagtctcaggaaagaaaactggatcagctattttaactctatagagaagttttgaaactatagcttttacatttgtagccatgcatctcttcaggggtcagaactacgccttcatttcctataaggaaatctacaaaaaccagggtgtttgaatagttcaaaatttggccagtagcttggttggatgaaatcctgttagcccaggaaatggggcaaaagccaggtctcctatccaagacccatcaacacctgacccagtgaggtgacatggagggcaccttggagctacttagaagaaaccttagtagagagctgatggtataactagagacagtgattcaggtggttacactgtgtaatagatgagataaatgccccatttttactatgaaggggttactaataattttttctggttttaaaaattgccatgggaggccgggcgcggtggctcacgcctgtaatcccagcactttgggaggctgaggtgggcggatcaactgaggtcaggcattcgagaccagcctgaccaacatggagaaaccctgtctctactaaaaatacaaaattagccgggtgtggtggtgcatgcctaaaatctcagctactcgggaggctgaggcaggagaatcgctcgcttgaacccgggaggcggaggttgcggtgagccgagatcgcacattgcactccagcctgggcaacaagagcgaaactccatctcaaaaaaaaaaaaaaaaagaaaagaaaagaataaaggcagtgagaaacagagatgataaagaagaaacagaaaatctttctgatcatgttctatctttgaaattctagtatcctttgaagcccaaactatacttcctacctttggaatctgttaaatactcctattaattataatttccccacttccccttttttgtttaaggtaacctgaatgagtacttcttacttggcagtcttaagccaataataatgctaaaataattgagcattcattatgcatcttgcaccctattagcatgttacatatatttaatgctcaaaactaagattatccccattttacatgtaagggtactgagacccagaaagattaacttgtgtaaggccacacatttaggcaaagccagaatttaatccaggcaatgtgactctagtacttatgctggtggttgccttcacgtaggtccaatgtacacatcgcctatagagtacaggttaaacttgtacttcaatagcagataatctcagtccaaataaaagatttcctaatggtttagtttcagtcatcaaagaatttaagtgaatggaaaaaagtatcttaaggcatacgtaaaggatggggcctttaaagagcccttccaactttggaagaagtaaatctggtcctagtaaaagaccatctgctgtacctgaagtcaaccagttcatctgaagaaaggctaaaattcaatacacttttattagaagcttaaaattgcctgttactactgatattacaatttcctagtgaaatcttttttttgttgagacggagtctcgctctgtcgcccaggctggagtgcagtggcgcgatctcggctcactgccagctccacctcccgggttcacgccattctcctgcctcagcctcccgagtagctgggactacaggcaccccccaccacgccgggctaattttttgtatttttagcagagacggagtttcaccgtgttagccagcatgctctcgatttcctgaccttgtgatccacccccctgggcctcccaaagtgctgggattacaggcctgagccaccgcgcccggcctgaaatcttaaatattagaattcacataggatcaagccaggactccaccttggatttttttttttttttttttagacggagtctcactctgtcgccaggctggagcacagtggcgcaatctcggctcactgcaacctccgcctcccgggttcaagcgattcttctgcctcagcctctggagtagctgggactacaggcgcgcgccactacgcccagctaatttttgtatttttagtagagacggggtttcaccatgttggccaggatggtctccatctcttgatctcgtgatcctcccgtctcagcctctcaaagtactgggattacaggcgtgagtcaccgcgcctggcctttttttttcttttttttgagatggagtctcactctgtcgcccgggggatggagtgcagtggcgcaatctcggctcactgcaacctccacctcccgggttcaagcgattctcttgcctcagcctcccgagtagctgggactacaggcacgtgtcaccatgcccagctaatttttgtatttttagtagaaacagagtttcgccatgttggtcaggctggtctcgaacttctgtcctcaactgttccacctgcctcagcctccgaaagtgctaggattacacgtgtgagccactgtgcccagcgtgtaccttggattttagattacagagagacaaataatctaaaacgatcacctttctctctagaacagtgggttagaggatccagaaacagacccaaatatgttagggaatacattaaaaatggcatttcaaatcagtagaggaaaagaaaacttattaatgatgccaaggcaactagttaaggcaactgaagcataaccttgtccacattcactaaaattccagaaggaacaaatatttaaatgtaagaactgaagctaggggtaaattatttttaaaatattggaattcacaaaaagccattcaaagcataagatccagagcacagaaaaaatgagtaatacatctgactactacataagtactaaaaacatgtccatggcaaaaaaaaaaaaaaaaacccacagaaaaacaacaacaaaacagaaaaaccaccaacaaaatgaaagtaagtgacaaattggagggaatatttgcaacatatttgacaaaggactaatttccttaatatatggagttcaaacagattaatgaacatgatcaacaggctgggtgcagtggctcaagcctgtaatcccagctttttgggaagctgaggtgggcagatggcttgagcccaggagttcaaaaccagcctgggcaacatggcaaaatcccatctctacaaaaaaaattaaaaaatcagctgggtgtggtggtgcatccctgtagttccagttattcgggaggctgaggtgggaggattgtttggacctgagaggcagaagttacagtgaaccaagatgatgccactgcactccagcctgggtgacagagggaggactggtttcaaaaaaaaaagtcaacagcccaatagtaagtggcaaaatacattaaaggccattttcagggaaaaaaattaaaataaaaacagtttatacacatataaaaacaccctaattaaagaaatgcaaatttaaaacaatgatataccatgttgggtgggtgtggtggctcgtgcctgtaatctcaacacttccagaggtcgaagaatcacttgaggccatgaattcaagacaagaggaacaatatagttaagaccctatctcttaaaaaaaatttgtttttttaaattagctgggcatggtagctcatgcctatactcccaactacttgggaggctaaggtgggaggattgcttgacctcaggatattgatggaaccactgcactccagagcttaggcggcagggagaccgtctcaaaacaaaaacaaaaaataaaattatataccatgtttaacctacagcttaacaagcaatatgatataatggttaaaactgctggctctagagtcagaatacttgggattaaatcctggctctactcctcactgtgtattctccagtttccttggttgggttgagaactaaatgagaaaatgtagtaaagcaattagaactgtgcctggcatgtatatagtaactgctcagttaacattagttctactagttcaatcaattagttctattagttcaattctattagttcaattaaaattggtttaaactgaaaaaaaaagaaaaaacgatgatgttgaaaagaaagcagagaactaggcactcatacgccatcatacaccactggtagaagtacaaactggcacaatgtctttcagtggtaatttgacattatctacttattttattttatttatttatttatttttgagacggagtctcgctctgtctcccaggctggactgcagtggcgcgatcgtggctcactgcaagctccgcctcctgggttcacgccattctcctgcctcagcctcctgagtagctgggactacaggcccccgccacacgcccagctaatgttttgtatttttagtagagatggggtttcaccatgttagccaggatggtctcgatctcctgacctcgtgatcgcccgcctcagcctcccaaagtgctgggattacagatgtgagccaccgcacccggcctatctacttattttaaatgcacaaacccttttgactttgcaatgtactttaaaacatttatcctacagatcacatatgtacataaaaatacatacatacatattcataaagatacatagggatttttcattacagcaatgtccttattagcaaaagactataaataaactaaatggtcatccatatgggtctgaacaaactatggtgcatcccaaaatggaatattatgataaaaacataatccccaagatagtcaaaaagcaaatcaaaaagcaatgtggacagctctctcattagtgtttgtatgcagagaagatttctggaaggagacacaagaaatgagtaacagcagttgccctgaggagcaagactgagagttgaaatcaaatggagatttgcttttcactgaacatcctgtaaacatgaaattttttccatgtacattactttttcaattgaacaaaaactggttaacttttaaaaatgagtgcagtcatcatttatcattacattcctatcagaaaggcagagggaggcataccaactgaagacaaattctaagagaaataatgctagcctatcattgcagattaaagggccaaaatggatatcctagagcaaagatagtccttggtccttaaagaactcttctctagagagtgataagaaccacagggactaagctcatgagttatctttccagatctcacattatccaggtattaactccagagcctataaaacaagagctgttcttccctccatctgcagaagcataggagtgctcttatacttggtgtgttggttaagatgaggattttgggggaagaaggaaaagagaagggactgatggatatactttatttattttttattttttgagacggagtctcacgctgtcgcccaggctgaagtgcagtagtagcatgatctctgctcattgcaacctccgcctcccgggttcaagcaattctcctgcctcagcctcccgagtagctgggattagaggcatgcaccaccatgcctggctaattttttgtatttttagtagagacagggtttctccatgttggccaggctggtctcgaactcctgaccttgtgatccgtctgcttcggccacccaaagtgctgggattacaggcatgagccaccgtgcccggcctggatatactttataatggtctcctggtcctaatgatatctttgggcaacttatttcttagtttttccctttcatcttgacaccttatatataaattcactttacaattcacaaagcacagttctacttacttattaattctcctaaccacctcatagatgggtattacaataccattttatgagtttcagaggggtttccttgtcccacacatattaggcttatgtcctggcagccccccattgaactctccaaacctgatcctttccactctgtgattttctctcttcatccctgctcaatctccctgcaccagcacccgattccattttattccagtcaacactaaacgcctgtgttcttaggtgctgattctagacagtgacagaggaaattttttaaggaccaaggacaagatatgtttttccttctggggacagatttgagctagttgctttttaaatattgttcctttgttattctgcctgataagacaaagtagtgggccttataaacaggatctcaccaggattgaatacctactatgctatgatattgtctagacactttattcattttatctcacttaccctgtaaaagcaggctctattatccccacaatacaaatgagttgatagaaatttagtgaagacaagacagttgtttaatgtcatatagctcctatgttcccatgttgaataaggattcaaaccccagtatctggctctacagcctgtggtacattacaccatgttgtccaacaagcatagctctcagggttacatggtttgttaaagtggttaaaaaccccaatcaaaggcccgtggaagttcttaagcaggggtaggttatgccagaaaaaaagtagtggctattcagctaattttctcacatttactcagtctttcccgtctgtaaaataaaaatgaatctaagttccagagaaaacaaatgggggcagtgtgagccaaggaagtgaataataataagcagaagagaaaggcagcctctgctcattggtagtcccaggaggtcggccttctgcagttgccaagcaacgagtgtaaacagcacaagatcatggccactaactacagtgccaaccaggtaagttcccattctccatttctttaacgtttacttttgtttttcagattctatctttggactgtcccctctcataggattctgatctttgaacagatagctgagagtggagtgagataatattttacctcctcagggatagagagagcccaggggcgatccaaaggtatctcttggttaaatttgtagggtgtaaaccagaagttggcaattttttttctgtaaaagggcggagtgtaaaaattttaggctttgcaggccaagtggcaaagtcaaaaatattctgtagctacttgcataattaaagaaaaacatttttccataacatttttgacaaattcaaaatataactgagtacaattttttgtactactaatgaaaataatggaattttgggggttgagaaaacatttcacttaactgggattcaaagttagtgttccatttgactgaatcaattgtaaatgttcatctataaaaatcacccttactctcaggccatccccaaacaggcagcaatatggatatggcccataggccatagtttaccaactcctgatctagaccagtgctgcccaacaaaaagagtgcgacccacaaatgtaattttaaattttctagtagctacatgaaaaaattaaaacataaaatttaaatatattgaatttaacccaataaatccaaatattatttcaacatttaatcagtatttaaaaaattataatcagacattttacgttctttttttgtactaaatctccaaaacctgctgggtgttgtagctcacgtctgtaatcccaacactttgggaggctgaggcacaaggatcgcttgaggccaggggtttgagaccaccctgggcaatatggtgagacctcgtctctacaagtaaatttaaaaattagctggacatggtggcatgcacctgtagtcccagctacctgtgagtctgagggaggaggatcgcttgaacccaggtgtccaaggctgcagtgagctaggatcatgccactgactccaacccaggtggcagaccaagatcctatctcaaaaaaaaaaagaaaagaaaaaaacttaaaaattcagcatatttcatatttacaaagcacctcaatttgaactagtcatatttcaggtgctcaacagctccatgtggctcccggctccatgctggacagcacacatctagaccaaacaaattacacccttgtcatagtgacttaaagcctacatggttggtcaggcctttggtcttcaaatctaaagaattgtgcctagtcttcatttcctgggtttggggccttgaagtctcatagggctacttatctttctctccacagtatgaaaaggctttctcatccaagtatctgcagaactggtctcccactaagccaacaaaagaggtattccatgttcagtgcacctacaagatagcctcatgctctccctgtcaattaactccttttagcattctctaaactcccatatccttctctgaccaagctccccaaatacttccctttttcccctcacaaacctttatctctcccacttgtaccccagagcatctcttctcatgaaggctacactcaaattattgccaacgatcgtggtcatctactgccttctgtgccccgttccaaggtgagatactatcttcactcctatcaagaaagtcaaataattaaggcacagaactgggagatgtgcagtctctcacagccattatcgggaaaattaaagtttaatctaattcatgttgtaatgtgagagcccctgaacttccggccagcttacccagcaggatagagttgtgtttagcacccttcagaagttcttaaattgatcaatgatctgtataaatgaaagccttcaggtgatgacatttgtgcagtgggtactcctttgccacactcggcctaaggatgtggaatttaagttggcagagtaaaggggatgaaaaaattaggcctgcaaagcctaaatgagggagggggataaggaagggtgggaagattatgctttcagtcttgtttcataaccatgcattcctaaaggtaaagaaaggaaataatacagaggtctaagtcagttactgggagtgagaagccctactgaggaatcccttttcatttttaggcaaatccttggggttccttcatgggcacctggcaaatgcctctgaagataccccctgctcgggtgaccctgacctcccgtacaactgctggtgctgcctccctcaccaaatggatacagaaaaatcctgatttactcaaggcctccaatgggctgtgtcctgaaatcttaggcaaggtatctattcttcccatctaacccaaaaccctgtagtctcaatttcttttcaacctcaaaaaatgtctattgttatgccaccactatcccagcatgggggacctctaaccaatttgtcttatcttgactagtccttaatcaccttctgaggcctgaagggatgggctaaggacatcatacccccaacagtagaaaatgatctaatctcaaggtgggggagggtggttagagaaatcaaatttaacttttcttatttgaaacttgatctactgcccatggtatggggagaaagggagttagaatcctgaggtgcattaggaatgatccgggcctgaccagagacatgactatctctcccactcttatcactgacagccccatgatccagacagtcagaagaaactcagaaagaagtctatcacaaagactgtacaacaagcacgaagtccaaccataattccaagctccccagctgccaacctcaattccccagatgaactccaaagctcacacccctctgcaggtcatactccaggtccccaaagaccagccaaatcctaagagcccacctggaagtccacgtatgctagaactctgggcagggcctaatctagctgaggtccagaaatacaaacctggaacttcatatggaccaagtggccacacactgaaaaacccgtatagcgactcagtgaaataaacaagagcccccagtcagaactgtgaaacagggaaattttggggtgggagtaaaagcaaatttggaaaataaacttttttttgttgaatcttttactgatctggattttccattcttgctatggctgcctcttgtaacacaattaggagaaggaaggtaggagaaaataaagtagggaaaagaacatacagtggtttgggtggaacacatttttacaagaattgagtcagttatactccagaaatgaccaagagaaagttggtctgaatcatggaaaaagggcagaacctcaaagaaccagtccctcaaccctacccactcattttttatcctgagcatggacaactaacaactacaaaatcagaaatagaattgagtagagtatgtatatgtgtgtttggagaaggtggggaagaaaaggtagggaaaaccaaagtagaagatactatgcttgtgtaagactttctatctaagcccaagtacaaatatagtttgaaaattgaagatattaaagtgattggaagacagagaagaaaaagacagtaagtagaaatttaaggcagaataacaaacatgatgctctgtcacaccccccacccacccactaccatgcttcaatcacccaaatggtacgaaaccaccaaaaaattcaactgccctacccattttccagcctctaacagctgtttatcattgaccccattttatattttcctggcactggctgttaaatttaatgcccttgccaaacctttcccagtcccaatgacaaagtgttctgtcatgatcacttgtccctcattccaaggacaaagtagagaacagctggtttaaaatggaggaaaggtacaaggacttcccagggcccctctagtaaaaagggaaaaccaatcattacttaaagccaaatactatttgggaccctgaatgaagactgttaaaacagcgggtccccaccttaactaaggtcttcctatccaattgacaccagccagttaacatttcccctcttcgacccacagctttaactggctggccaacaactcgaagtgacagatgagataagtctcttattccagagttcccaaaaactatcaaaacagcatgcctgctaaagcctggcctatatggattttaaaagcagcaagttttctcattaaattatacatttttgccaggttttcaacaatcccttcttttttaaaaaaaaactctatgcttcattcaccccaagcctataacctcaggtcatcatcccctagctgtcaccaacactggtcctctgtgcccctcaatgaatcataatttgctgaactgtaccatgaagcttataatcagtccttaatgggattttggtgcctataacccaaaagcactctacatgcgtcacttcttttctttttctccttccttctctgaggcttttctgtgatatttaaatctctggctaagttctatctgattccctgaaaacttttccaatgatgagatgtaggagaactgtttccctcctggtaaaggtcagattgcggggagagggaggatgtaaatgcctgagacccgagggaagaggaggaaattggttccttcccaacagccattttcttggtttctctagatttcaaggagagtcaaagataaaatgagtatttaattcagtttcagaaaaaaagggtacattacttcgatgagaaagcataaaattaagaggcttttctggaaatccaagaaaaagaaataaccattaatatgttcaatgataattttctagatcttcctcgtgtccaaagctatatattttctcctcaaaagcagctgctccaagaactaactagccctctttatctccctctagctgggacagactaattcccctccacccccacctctcttctttcaataacactgtgtaggtgttaatggcctgggctctcaccaatgaagagaattgtcctttaagccagcaacccacaggcagtggcacccaaagcctcaccaacccaccccccaacccggcccatccccagggcagaagccacagagctggcattgtttccactgtctcaggaagaaggagccaaaagctgaccctcagcacaaatcaaagcccaatatggagagagaataactgcttctaggccgagagtaggcaagctgtgggcaaaaaaggggagtttttgcagccacctcatctttagaaacaaggggaaaactagacccttttccactattatggtctaccaggtactctactgctccaaggagatctgaaaatacaaaaggatctaaacaaataaggagaacttttcccaggctggagataagaatgacaaacagaaagatgggtgaatgtaataatgtgtaggaagatgatgctgggagcctcctttcttcacatggctgccagccccatagaggacaacacagtaagaaccaggacaaccactccagactggtatagctggggaatcttcaggccttttcctaggtcccacatcaagtgtcggatcccattccaggtatgatacatgagagggaagacaagtgcaaacttagctgtgtggatcagtgctggccccagacacagggacttcacaagttccaaataagactcaaagttcccagggagtaacagggccgacatgccaaaaagagagacccctgcactcaaagcaataccagtgccacggtggcagatggacatcgccatgggaagagaccaactcagcaacagcgcagccatcttgggttccggtctggacggaagt

SEQ ID NO: 17302 - RNA, 13195 nt, Homo sapiens
  source 1..13195: mol_type = other RNA
tcaggccaggcacagtggctcacgcctgtaatccaacgactttgggaggccaaggcaggtggatcacctgacgtcaggagttccagaccagcctggccaacatggcgaaaccctgtctctactaaaaatactaaaattagcagggcatgctggtgtgtgcctataatcccagctatggaggggggctgaagcaggaggatcacttgaacctgggaggcggaggttgcagtgagctgagatggtgccactgcactccagcctgggcaacagagcaagattctgtctcaaaaaaaaaaaaaaaaaaaaaggaatgaaagaaaagaaaaagaaatagtgttaaatagctctatgaatgctgcagagagggctaccccataggcagtgtgtggggagtatacaaagcttgttctttggctcctcaggaaggggatcttatcaagaatattattcttttgtggtattgtcagtggaaaggagagatgtaacagcagtctccgagagagggagccttagtctcaggaaagaaaactggatcagctattttaactctatagagaagttttgaaactatagcttttacatttgtagccatgcatctcttcaggggtcagaactacgccttcatttcctataaggaaatctacaaaaaccagggtgtttgaatagttcaaaatttggccagtagcttggttggatgaaatcctgttagcccaggaaatggggcaaaagccaggtctcctatccaagacccatcaacacctgacccagtgaggtgacatggagggcaccttggagctacttagaagaaaccttagtagagagctgatggtataactagagacagtgattcaggtggttacactgtgtaatagatgagataaatgccccatttttactatgaaggggttactaataattttttctggttttaaaaattgccatgggaggccgggcgcggtggctcacgcctgtaatcccagcactttgggaggctgaggtgggcggatcaactgaggtcaggcattcgagaccagcctgaccaacatggagaaaccctgtctctactaaaaatacaaaattagccgggtgtggtggtgcatgcctaaaatctcagctactcgggaggctgaggcaggagaatcgctcgcttgaacccgggaggcggaggttgcggtgagccgagatcgcacattgcactccagcctgggcaacaagagcgaaactccatctcaaaaaaaaaaaaaaaaagaaaagaaaagaataaaggcagtgagaaacagagatgataaagaagaaacagaaaatctttctgatcatgttctatctttgaaattctagtatcctttgaagcccaaactatacttcctacctttggaatctgttaaatactcctattaattataatttccccacttccccttttttgtttaaggtaacctgaatgagtacttcttacttggcagtcttaagccaataataatgctaaaataattgagcattcattatgcatcttgcaccctattagcatgttacatatatttaatgctcaaaactaagattatccccattttacatgtaagggtactgagacccagaaagattaacttgtgtaaggccacacatttaggcaaagccagaatttaatccaggcaatgtgactctagtacttatgctggtggttgccttcacgtaggtccaatgtacacatcgcctatagagtacaggttaaacttgtacttcaatagcagataatctcagtccaaataaaagatttcctaatggtttagtttcagtcatcaaagaatttaagtgaatggaaaaaagtatcttaaggcatacgtaaaggatggggcctttaaagagcccttccaactttggaagaagtaaatctggtcctagtaaaagaccatctgctgtacctgaagtcaaccagttcatctgaagaaaggctaaaattcaatacacttttattagaagcttaaaattgcctgttactactgatattacaatttcctagtgaaatcttttttttgttgagacggagtctcgctctgtcgcccaggctggagtgcagtggcgcgatctcggctcactgccagctccacctcccgggttcacgccattctcctgcctcagcctcccgagtagctgggactacaggcaccccccaccacgccgggctaattttttgtatttttagcagagacggagtttcaccgtgttagccagcatgctctcgatttcctgaccttgtgatccacccccctgggcctcccaaagtgctgggattacaggcctgagccaccgcgcccggcctgaaatcttaaatattagaattcacataggatcaagccaggactccaccttggatttttttttttttttttttagacggagtctcactctgtcgccaggctggagcacagtggcgcaatctcggctcactgcaacctccgcctcccgggttcaagcgattcttctgcctcagcctctggagtagctgggactacaggcgcgcgccactacgcccagctaatttttgtatttttagtagagacggggtttcaccatgttggccaggatggtctccatctcttgatctcgtgatcctcccgtctcagcctctcaaagtactgggattacaggcgtgagtcaccgcgcctggcctttttttttcttttttttgagatggagtctcactctgtcgcccgggggatggagtgcagtggcgcaatctcggctcactgcaacctccacctcccgggttcaagcgattctcttgcctcagcctcccgagtagctgggactacaggcacgtgtcaccatgcccagctaatttttgtatttttagtagaaacagagtttcgccatgttggtcaggctggtctcgaacttctgtcctcaactgttccacctgcctcagcctccgaaagtgctaggattacacgtgtgagccactgtgcccagcgtgtaccttggattttagattacagagagacaaataatctaaaacgatcacctttctctctagaacagtgggttagaggatccagaaacagacccaaatatgttagggaatacattaaaaatggcatttcaaatcagtagaggaaaagaaaacttattaatgatgccaaggcaactagttaaggcaactgaagcataaccttgtccacattcactaaaattccagaaggaacaaatatttaaatgtaagaactgaagctaggggtaaattatttttaaaatattggaattcacaaaaagccattcaaagcataagatccagagcacagaaaaaatgagtaatacatctgactactacataagtactaaaaacatgtccatggcaaaaaaaaaaaaaaaaacccacagaaaaacaacaacaaaacagaaaaaccaccaacaaaatgaaagtaagtgacaaattggagggaatatttgcaacatatttgacaaaggactaatttccttaatatatggagttcaaacagattaatgaacatgatcaacaggctgggtgcagtggctcaagcctgtaatcccagctttttgggaagctgaggtgggcagatggcttgagcccaggagttcaaaaccagcctgggcaacatggcaaaatcccatctctacaaaaaaaattaaaaaatcagctgggtgtggtggtgcatccctgtagttccagttattcgggaggctgaggtgggaggattgtttggacctgagaggcagaagttacagtgaaccaagatgatgccactgcactccagcctgggtgacagagggaggactggtttcaaaaaaaaaagtcaacagcccaatagtaagtggcaaaatacattaaaggccattttcagggaaaaaaattaaaataaaaacagtttatacacatataaaaacaccctaattaaagaaatgcaaatttaaaacaatgatataccatgttgggtgggtgtggtggctcgtgcctgtaatctcaacacttccagaggtcgaagaatcacttgaggccatgaattcaagacaagaggaacaatatagttaagaccctatctcttaaaaaaaatttgtttttttaaattagctgggcatggtagctcatgcctatactcccaactacttgggaggctaaggtgggaggattgcttgacctcaggatattgatggaaccactgcactccagagcttaggcggcagggagaccgtctcaaaacaaaaacaaaaaataaaattatataccatgtttaacctacagcttaacaagcaatatgatataatggttaaaactgctggctctagagtcagaatacttgggattaaatcctggctctactcctcactgtgtattctccagtttccttggttgggttgagaactaaatgagaaaatgtagtaaagcaattagaactgtgcctggcatgtatatagtaactgctcagttaacattagttctactagttcaatcaattagttctattagttcaattctattagttcaattaaaattggtttaaactgaaaaaaaaagaaaaaacgatgatgttgaaaagaaagcagagaactaggcactcatacgccatcatacaccactggtagaagtacaaactggcacaatgtctttcagtggtaatttgacattatctacttattttattttatttatttatttatttttgagacggagtctcgctctgtctcccaggctggactgcagtggcgcgatcgtggctcactgcaagctccgcctcctgggttcacgccattctcctgcctcagcctcctgagtagctgggactacaggcccccgccacacgcccagctaatgttttgtatttttagtagagatggggtttcaccatgttagccaggatggtctcgatctcctgacctcgtgatcgcccgcctcagcctcccaaagtgctgggattacagatgtgagccaccgcacccggcctatctacttattttaaatgcacaaacccttttgactttgcaatgtactttaaaacatttatcctacagatcacatatgtacataaaaatacatacatacatattcataaagatacatagggatttttcattacagcaatgtccttattagcaaaagactataaataaactaaatggtcatccatatgggtctgaacaaactatggtgcatcccaaaatggaatattatgataaaaacataatccccaagatagtcaaaaagcaaatcaaaaagcaatgtggacagctctctcattagtgtttgtatgcagagaagatttctggaaggagacacaagaaatgagtaacagcagttgccctgaggagcaagactgagagttgaaatcaaatggagatttgcttttcactgaacatcctgtaaacatgaaattttttccatgtacattactttttcaattgaacaaaaactggttaacttttaaaaatgagtgcagtcatcatttatcattacattcctatcagaaaggcagagggaggcataccaactgaagacaaattctaagagaaataatgctagcctatcattgcagattaaagggccaaaatggatatcctagagcaaagatagtccttggtccttaaagaactcttctctagagagtgataagaaccacagggactaagctcatgagttatctttccagatctcacattatccaggtattaactccagagcctataaaacaagagctgttcttccctccatctgcagaagcataggagtgctcttatacttggtgtgttggttaagatgaggattttgggggaagaaggaaaagagaagggactgatggatatactttatttattttttattttttgagacggagtctcacgctgtcgcccaggctgaagtgcagtagtagcatgatctctgctcattgcaacctccgcctcccgggttcaagcaattctcctgcctcagcctcccgagtagctgggattagaggcatgcaccaccatgcctggctaattttttgtatttttagtagagacagggtttctccatgttggccaggctggtctcgaactcctgaccttgtgatccgtctgcttcggccacccaaagtgctgggattacaggcatgagccaccgtgcccggcctggatatactttataatggtctcctggtcctaatgatatctttgggcaacttatttcttagtttttccctttcatcttgacaccttatatataaattcactttacaattcacaaagcacagttctacttacttattaattctcctaaccacctcatagatgggtattacaataccattttatgagtttcagaggggtttccttgtcccacacatattaggcttatgtcctggcagccccccattgaactctccaaacctgatcctttccactctgtgattttctctcttcatccctgctcaatctccctgcaccagcacccgattccattttattccagtcaacactaaacgcctgtgttcttaggtgctgattctagacagtgacagaggaaattttttaaggaccaaggacaagatatgtttttccttctggggacagatttgagctagttgctttttaaatattgttcctttgttattctgcctgataagacaaagtagtgggccttataaacaggatctcaccaggattgaatacctactatgctatgatattgtctagacactttattcattttatctcacttaccctgtaaaagcaggctctattatccccacaatacaaatgagttgatagaaatttagtgaagacaagacagttgtttaatgtcatatagctcctatgttcccatgttgaataaggattcaaaccccagtatctggctctacagcctgtggtacattacaccatgttgtccaacaagcatagctctcagggttacatggtttgttaaagtggttaaaaaccccaatcaaaggcccgtggaagttcttaagcaggggtaggttatgccagaaaaaaagtagtggctattcagctaattttctcacatttactcagtctttcccgtctgtaaaataaaaatgaatctaagttccagagaaaacaaatgggggcagtgtgagccaaggaagtgaataataataagcagaagagaaaggcagcctctgctcattggtagtcccaggaggtcggccttctgcagttgccaagcaacgagtgtaaacagcacaagatcatggccactaactacagtgccaaccaggtaagttcccattctccatttctttaacgtttacttttgtttttcagattctatctttggactgtcccctctcataggattctgatctttgaacagatagctgagagtggagtgagataatattttacctcctcagggatagagagagcccaggggcgatccaaaggtatctcttggttaaatttgtagggtgtaaaccagaagttggcaattttttttctgtaaaagggcggagtgtaaaaattttaggctttgcaggccaagtggcaaagtcaaaaatattctgtagctacttgcataattaaagaaaaacatttttccataacatttttgacaaattcaaaatataactgagtacaattttttgtactactaatgaaaataatggaattttgggggttgagaaaacatttcacttaactgggattcaaagttagtgttccatttgactgaatcaattgtaaatgttcatctataaaaatcacccttactctcaggccatccccaaacaggcagcaatatggatatggcccataggccatagtttaccaactcctgatctagaccagtgctgcccaacaaaaagagtgcgacccacaaatgtaattttaaattttctagtagctacatgaaaaaattaaaacataaaatttaaatatattgaatttaacccaataaatccaaatattatttcaacatttaatcagtatttaaaaaattataatcagacattttacgttctttttttgtactaaatctccaaaacctgctgggtgttgtagctcacgtctgtaatcccaacactttgggaggctgaggcacaaggatcgcttgaggccaggggtttgagaccaccctgggcaatatggtgagacctcgtctctacaagtaaatttaaaaattagctggacatggtggcatgcacctgtagtcccagctacctgtgagtctgagggaggaggatcgcttgaacccaggtgtccaaggctgcagtgagctaggatcatgccactgactccaacccaggtggcagaccaagatcctatctcaaaaaaaaaaagaaaagaaaaaaacttaaaaattcagcatatttcatatttacaaagcacctcaatttgaactagtcatatttcaggtgctcaacagctccatgtggctcccggctccatgctggacagcacacatctagaccaaacaaattacacccttgtcatagtgacttaaagcctacatggttggtcaggcctttggtcttcaaatctaaagaattgtgcctagtcttcatttcctgggtttggggccttgaagtctcatagggctacttatctttctctccacagtatgaaaaggctttctcatccaagtatctgcagaactggtctcccactaagccaacaaaagaggtattccatgttcagtgcacctacaagatagcctcatgctctccctgtcaattaactccttttagcattctctaaactcccatatccttctctgaccaagctccccaaatacttccctttttcccctcacaaacctttatctctcccacttgtaccccagagcatctcttctcatgaaggctacactcaaattattgccaacgatcgtggtcatctactgccttctgtgccccgttccaaggtgagatactatcttcactcctatcaagaaagtcaaataattaaggcacagaactgggagatgtgcagtctctcacagccattatcgggaaaattaaagtttaatctaattcatgttgtaatgtgagagcccctgaacttccggccagcttacccagcaggatagagttgtgtttagcacccttcagaagttcttaaattgatcaatgatctgtataaatgaaagccttcaggtgatgacatttgtgcagtgggtactcctttgccacactcggcctaaggatgtggaatttaagttggcagagtaaaggggatgaaaaaattaggcctgcaaagcctaaatgagggagggggataaggaagggtgggaagattatgctttcagtcttgtttcataaccatgcattcctaaaggtaaagaaaggaaataatacagaggtctaagtcagttactgggagtgagaagccctactgaggaatcccttttcatttttaggcaaatccttggggttccttcatgggcacctggcaaatgcctctgaagataccccctgctcgggtgaccctgacctcccgtacaactgctggtgctgcctccctcaccaaatggatacagaaaaatcctgatttactcaaggcctccaatgggctgtgtcctgaaatcttaggcaaggtatctattcttcccatctaacccaaaaccctgtagtctcaatttcttttcaacctcaaaaaatgtctattgttatgccaccactatcccagcatgggggacctctaaccaatttgtcttatcttgactagtccttaatcaccttctgaggcctgaagggatgggctaaggacatcatacccccaacagtagaaaatgatctaatctcaaggtgggggagggtggttagagaaatcaaatttaacttttcttatttgaaacttgatctactgcccatggtatggggagaaagggagttagaatcctgaggtgcattaggaatgatccgggcctgaccagagacatgactatctctcccactcttatcactgacagccccatgatccagacagtcagaagaaactcagaaagaagtctatcacaaagactgtacaacaagcacgaagtccaaccataattccaagctccccagctgccaacctcaattccccagatgaactccaaagctcacacccctctgcaggtcatactccaggtccccaaagaccagccaaatcctaagagcccacctggaagtccacgtatgctagaactctgggcagggcctaatctagctgaggtccagaaatacaaacctggaacttcatatggaccaagtggccacacactgaaaaacccgtatagcgactcagtgaaataaacaagagcccccagtcagaactgtgaaacagggaaattttggggtgggagtaaaagcaaatttggaaaataaacttttttttgttgaatcttttactgatctggattttccattcttgctatggctgcctcttgtaacacaattaggagaaggaaggtaggagaaaataaagtagggaaaagaacatacagtggtttgggtggaacacatttttacaagaattgagtcagttatactccagaaatgaccaagagaaagttggtctgaatcatggaaaaagggcagaacctcaaagaaccagtccctcaaccctacccactcattttttatcctgagcatggacaactaacaactacaaaatcagaaatagaattgagtagagtatgtatatgtgtgtttggagaaggtggggaagaaaaggtagggaaaaccaaagtagaagatactatgcttgtgtaagactttctatctaagcccaagtacaaatatagtttgaaaattgaagatattaaagtgattggaagacagagaagaaaaagacagtaagtagaaatttaaggcagaataacaaacatgatgctctgtcacaccccccacccacccactaccatgcttcaatcacccaaatggtacgaaaccaccaaaaaattcaactgccctacccattttccagcctctaacagctgtttatcattgaccccattttatattttcctggcactggctgttaaatttaatgcccttgccaaacctttcccagtcccaatgacaaagtgttctgtcatgatcacttgtccctcattccaaggacaaagtagagaacagctggtttaaaatggaggaaaggtacaaggacttcccagggcccctctagtaaaaagggaaaaccaatcattacttaaagccaaatactatttgggaccctgaatgaagactgttaaaacagcgggtccccaccttaactaaggtcttcctatccaattgacaccagccagttaacatttcccctcttcgacccacagctttaactggctggccaacaactcgaagtgacagatgagataagtctcttattccagagttcccaaaaactatcaaaacagcatgcctgctaaagcctggcctatatggattttaaaagcagcaagttttctcattaaattatacatttttgccaggttttcaacaatcccttcttttttaaaaaaaaactctatgcttcattcaccccaagcctataacctcaggtcatcatcccctagctgtcaccaacactggtcctctgtgcccctcaatgaatcataatttgctgaactgtaccatgaagcttataatcagtccttaatgggattttggtgcctataacccaaaagcactctacatgcgtcacttcttttctttttctccttccttctctgaggcttttctgtgatatttaaatctctggctaagttctatctgattccctgaaaacttttccaatgatgagatgtaggagaactgtttccctcctggtaaaggtcagattgcggggagagggaggatgtaaatgcctgagacccgagggaagaggaggaaattggttccttcccaacagccattttcttggtttctctagatttcaaggagagtcaaagataaaatgagtatttaattcagtttcagaaaaaaagggtacattacttcgatgagaaagcataaaattaagaggcttttctggaaatccaagaaaaagaaataaccattaatatgttcaatgataattttctagatcttcctcgtgtccaaagctatatattttctcctcaaaagcagctgctccaagaactaactagccctctttatctccctctagctgggacagactaattcccctccacccccacctctcttctttcaataacactgtgtaggtgttaatggcctgggctctcaccaatgaagagaattgtcctttaagccagcaacccacaggcagtggcacccaaagcctcaccaacccaccccccaacccggcccatccccagggcagaagccacagagctggcattgtttccactgtctcaggaagaaggagccaaaagctgaccctcagcacaaatcaaagcccaatatggagagagaataactgcttctaggccgagagtaggcaagctgtgggcaaaaaaggggagtttttgcagccacctcatctttagaaacaaggggaaaactagacccttttccactattatggtctaccaggtactctactgctccaaggagatctgaaaatacaaaaggatctaaacaaataaggagaacttttcccaggctggagataagaatgacaaacagaaagatgggtgaatgtaataatgtgtaggaagatgatgctgggagcctcctttcttcacatggctgccagccccatagaggacaacacagtaagaaccaggacaaccactccagactggtatagctggggaatcttcaggccttttcctaggtcccacatcaagtgtcggatcccattccaggtatgatacatgagagggaagacaagtgcaaacttagctgtgtggatcagtgctggccccagacacagggacttcacaagttccaaataagactcaaagttcccagggagtaacagggccgacatgccaaaaagagagacccctgcactcaaagcaataccagtgccacggtggcagatggacatcgccatgggaagagaccaactttaccagactgcatcactgatagggctgtagatagtaatgtggggagacagaggacggtttgaacctatattcttattccagaaccgctccatctcttctttggccgtggttcccaaaggaacagcatttctgatacagagctgagggctaaagtgggctcggaggcaatgacgaccaacgtgtctcagcaacagcgcagccatcttgggttccggtctggacggaagt

SEQ ID NO: 17303 - RNA, 13066 nt, Homo sapiens
  source 1..13066: mol_type = other RNA
tcaggccaggcacagtggctcacgcctgtaatccaacgactttgggaggccaaggcaggtggatcacctgacgtcaggagttccagaccagcctggccaacatggcgaaaccctgtctctactaaaaatactaaaattagcagggcatgctggtgtgtgcctataatcccagctatggaggggggctgaagcaggaggatcacttgaacctgggaggcggaggttgcagtgagctgagatggtgccactgcactccagcctgggcaacagagcaagattctgtctcaaaaaaaaaaaaaaaaaaaaaggaatgaaagaaaagaaaaagaaatagtgttaaatagctctatgaatgctgcagagagggctaccccataggcagtgtgtggggagtatacaaagcttgttctttggctcctcaggaaggggatcttatcaagaatattattcttttgtggtattgtcagtggaaaggagagatgtaacagcagtctccgagagagggagccttagtctcaggaaagaaaactggatcagctattttaactctatagagaagttttgaaactatagcttttacatttgtagccatgcatctcttcaggggtcagaactacgccttcatttcctataaggaaatctacaaaaaccagggtgtttgaatagttcaaaatttggccagtagcttggttggatgaaatcctgttagcccaggaaatggggcaaaagccaggtctcctatccaagacccatcaacacctgacccagtgaggtgacatggagggcaccttggagctacttagaagaaaccttagtagagagctgatggtataactagagacagtgattcaggtggttacactgtgtaatagatgagataaatgccccatttttactatgaaggggttactaataattttttctggttttaaaaattgccatgggaggccgggcgcggtggctcacgcctgtaatcccagcactttgggaggctgaggtgggcggatcaactgaggtcaggcattcgagaccagcctgaccaacatggagaaaccctgtctctactaaaaatacaaaattagccgggtgtggtggtgcatgcctaaaatctcagctactcgggaggctgaggcaggagaatcgctcgcttgaacccgggaggcggaggttgcggtgagccgagatcgcacattgcactccagcctgggcaacaagagcgaaactccatctcaaaaaaaaaaaaaaaaagaaaagaaaagaataaaggcagtgagaaacagagatgataaagaagaaacagaaaatctttctgatcatgttctatctttgaaattctagtatcctttgaagcccaaactatacttcctacctttggaatctgttaaatactcctattaattataatttccccacttccccttttttgtttaaggtaacctgaatgagtacttcttacttggcagtcttaagccaataataatgctaaaataattgagcattcattatgcatcttgcaccctattagcatgttacatatatttaatgctcaaaactaagattatccccattttacatgtaagggtactgagacccagaaagattaacttgtgtaaggccacacatttaggcaaagccagaatttaatccaggcaatgtgactctagtacttatgctggtggttgccttcacgtaggtccaatgtacacatcgcctatagagtacaggttaaacttgtacttcaatagcagataatctcagtccaaataaaagatttcctaatggtttagtttcagtcatcaaagaatttaagtgaatggaaaaaagtatcttaaggcatacgtaaaggatggggcctttaaagagcccttccaactttggaagaagtaaatctggtcctagtaaaagaccatctgctgtacctgaagtcaaccagttcatctgaagaaaggctaaaattcaatacacttttattagaagcttaaaattgcctgttactactgatattacaatttcctagtgaaatcttttttttgttgagacggagtctcgctctgtcgcccaggctggagtgcagtggcgcgatctcggctcactgccagctccacctcccgggttcacgccattctcctgcctcagcctcccgagtagctgggactacaggcaccccccaccacgccgggctaattttttgtatttttagcagagacggagtttcaccgtgttagccagcatgctctcgatttcctgaccttgtgatccacccccctgggcctcccaaagtgctgggattacaggcctgagccaccgcgcccggcctgaaatcttaaatattagaattcacataggatcaagccaggactccaccttggatttttttttttttttttttagacggagtctcactctgtcgccaggctggagcacagtggcgcaatctcggctcactgcaacctccgcctcccgggttcaagcgattcttctgcctcagcctctggagtagctgggactacaggcgcgcgccactacgcccagctaatttttgtatttttagtagagacggggtttcaccatgttggccaggatggtctccatctcttgatctcgtgatcctcccgtctcagcctctcaaagtactgggattacaggcgtgagtcaccgcgcctggcctttttttttcttttttttgagatggagtctcactctgtcgcccgggggatggagtgcagtggcgcaatctcggctcactgcaacctccacctcccgggttcaagcgattctcttgcctcagcctcccgagtagctgggactacaggcacgtgtcaccatgcccagctaatttttgtatttttagtagaaacagagtttcgccatgttggtcaggctggtctcgaacttctgtcctcaactgttccacctgcctcagcctccgaaagtgctaggattacacgtgtgagccactgtgcccagcgtgtaccttggattttagattacagagagacaaataatctaaaacgatcacctttctctctagaacagtgggttagaggatccagaaacagacccaaatatgttagggaatacattaaaaatggcatttcaaatcagtagaggaaaagaaaacttattaatgatgccaaggcaactagttaaggcaactgaagcataaccttgtccacattcactaaaattccagaaggaacaaatatttaaatgtaagaactgaagctaggggtaaattatttttaaaatattggaattcacaaaaagccattcaaagcataagatccagagcacagaaaaaatgagtaatacatctgactactacataagtactaaaaacatgtccatggcaaaaaaaaaaaaaaaaacccacagaaaaacaacaacaaaacagaaaaaccaccaacaaaatgaaagtaagtgacaaattggagggaatatttgcaacatatttgacaaaggactaatttccttaatatatggagttcaaacagattaatgaacatgatcaacaggctgggtgcagtggctcaagcctgtaatcccagctttttgggaagctgaggtgggcagatggcttgagcccaggagttcaaaaccagcctgggcaacatggcaaaatcccatctctacaaaaaaaattaaaaaatcagctgggtgtggtggtgcatccctgtagttccagttattcgggaggctgaggtgggaggattgtttggacctgagaggcagaagttacagtgaaccaagatgatgccactgcactccagcctgggtgacagagggaggactggtttcaaaaaaaaaagtcaacagcccaatagtaagtggcaaaatacattaaaggccattttcagggaaaaaaattaaaataaaaacagtttatacacatataaaaacaccctaattaaagaaatgcaaatttaaaacaatgatataccatgttgggtgggtgtggtggctcgtgcctgtaatctcaacacttccagaggtcgaagaatcacttgaggccatgaattcaagacaagaggaacaatatagttaagaccctatctcttaaaaaaaatttgtttttttaaattagctgggcatggtagctcatgcctatactcccaactacttgggaggctaaggtgggaggattgcttgacctcaggatattgatggaaccactgcactccagagcttaggcggcagggagaccgtctcaaaacaaaaacaaaaaataaaattatataccatgtttaacctacagcttaacaagcaatatgatataatggttaaaactgctggctctagagtcagaatacttgggattaaatcctggctctactcctcactgtgtattctccagtttccttggttgggttgagaactaaatgagaaaatgtagtaaagcaattagaactgtgcctggcatgtatatagtaactgctcagttaacattagttctactagttcaatcaattagttctattagttcaattctattagttcaattaaaattggtttaaactgaaaaaaaaagaaaaaacgatgatgttgaaaagaaagcagagaactaggcactcatacgccatcatacaccactggtagaagtacaaactggcacaatgtctttcagtggtaatttgacattatctacttattttattttatttatttatttatttttgagacggagtctcgctctgtctcccaggctggactgcagtggcgcgatcgtggctcactgcaagctccgcctcctgggttcacgccattctcctgcctcagcctcctgagtagctgggactacaggcccccgccacacgcccagctaatgttttgtatttttagtagagatggggtttcaccatgttagccaggatggtctcgatctcctgacctcgtgatcgcccgcctcagcctcccaaagtgctgggattacagatgtgagccaccgcacccggcctatctacttattttaaatgcacaaacccttttgactttgcaatgtactttaaaacatttatcctacagatcacatatgtacataaaaatacatacatacatattcataaagatacatagggatttttcattacagcaatgtccttattagcaaaagactataaataaactaaatggtcatccatatgggtctgaacaaactatggtgcatcccaaaatggaatattatgataaaaacataatccccaagatagtcaaaaagcaaatcaaaaagcaatgtggacagctctctcattagtgtttgtatgcagagaagatttctggaaggagacacaagaaatgagtaacagcagttgccctgaggagcaagactgagagttgaaatcaaatggagatttgcttttcactgaacatcctgtaaacatgaaattttttccatgtacattactttttcaattgaacaaaaactggttaacttttaaaaatgagtgcagtcatcatttatcattacattcctatcagaaaggcagagggaggcataccaactgaagacaaattctaagagaaataatgctagcctatcattgcagattaaagggccaaaatggatatcctagagcaaagatagtccttggtccttaaagaactcttctctagagagtgataagaaccacagggactaagctcatgagttatctttccagatctcacattatccaggtattaactccagagcctataaaacaagagctgttcttccctccatctgcagaagcataggagtgctcttatacttggtgtgttggttaagatgaggattttgggggaagaaggaaaagagaagggactgatggatatactttatttattttttattttttgagacggagtctcacgctgtcgcccaggctgaagtgcagtagtagcatgatctctgctcattgcaacctccgcctcccgggttcaagcaattctcctgcctcagcctcccgagtagctgggattagaggcatgcaccaccatgcctggctaattttttgtatttttagtagagacagggtttctccatgttggccaggctggtctcgaactcctgaccttgtgatccgtctgcttcggccacccaaagtgctgggattacaggcatgagccaccgtgcccggcctggatatactttataatggtctcctggtcctaatgatatctttgggcaacttatttcttagtttttccctttcatcttgacaccttatatataaattcactttacaattcacaaagcacagttctacttacttattaattctcctaaccacctcatagatgggtattacaataccattttatgagtttcagaggggtttccttgtcccacacatattaggcttatgtcctggcagccccccattgaactctccaaacctgatcctttccactctgtgattttctctcttcatccctgctcaatctccctgcaccagcacccgattccattttattccagtcaacactaaacgcctgtgttcttaggtgctgattctagacagtgacagaggaaattttttaaggaccaaggacaagatatgtttttccttctggggacagatttgagctagttgctttttaaatattgttcctttgttattctgcctgataagacaaagtagtgggccttataaacaggatctcaccaggattgaatacctactatgctatgatattgtctagacactttattcattttatctcacttaccctgtaaaagcaggctctattatccccacaatacaaatgagttgatagaaatttagtgaagacaagacagttgtttaatgtcatatagctcctatgttcccatgttgaataaggattcaaaccccagtatctggctctacagcctgtggtacattacaccatgttgtccaacaagcatagctctcagggttacatggtttgttaaagtggttaaaaaccccaatcaaaggcccgtggaagttcttaagcaggggtaggttatgccagaaaaaaagtagtggctattcagctaattttctcacatttactcagtctttcccgtctgtaaaataaaaatgaatctaagttccagagaaaacaaatgggggcagtgtgagccaaggaagtgaataataataagcagaagagaaaggcagcctctgctcattggtagtcccaggaggtcggccttctgcagttgccaagcaacgagtgtaaacagcacaagatcatggccactaactacagtgccaaccaggtaagttcccattctccatttctttaacgtttacttttgtttttcagattctatctttggactgtcccctctcataggattctgatctttgaacagatagctgagagtggagtgagataatattttacctcctcagggatagagagagcccaggggcgatccaaaggtatctcttggttaaatttgtagggtgtaaaccagaagttggcaattttttttctgtaaaagggcggagtgtaaaaattttaggctttgcaggccaagtggcaaagtcaaaaatattctgtagctacttgcataattaaagaaaaacatttttccataacatttttgacaaattcaaaatataactgagtacaattttttgtactactaatgaaaataatggaattttgggggttgagaaaacatttcacttaactgggattcaaagttagtgttccatttgactgaatcaattgtaaatgttcatctataaaaatcacccttactctcaggccatccccaaacaggcagcaatatggatatggcccataggccatagtttaccaactcctgatctagaccagtgctgcccaacaaaaagagtgcgacccacaaatgtaattttaaattttctagtagctacatgaaaaaattaaaacataaaatttaaatatattgaatttaacccaataaatccaaatattatttcaacatttaatcagtatttaaaaaattataatcagacattttacgttctttttttgtactaaatctccaaaacctgctgggtgttgtagctcacgtctgtaatcccaacactttgggaggctgaggcacaaggatcgcttgaggccaggggtttgagaccaccctgggcaatatggtgagacctcgtctctacaagtaaatttaaaaattagctggacatggtggcatgcacctgtagtcccagctacctgtgagtctgagggaggaggatcgcttgaacccaggtgtccaaggctgcagtgagctaggatcatgccactgactccaacccaggtggcagaccaagatcctatctcaaaaaaaaaaagaaaagaaaaaaacttaaaaattcagcatatttcatatttacaaagcacctcaatttgaactagtcatatttcaggtgctcaacagctccatgtggctcccggctccatgctggacagcacacatctagaccaaacaaattacacccttgtcatagtgacttaaagcctacatggttggtcaggcctttggtcttcaaatctaaagaattgtgcctagtcttcatttcctgggtttggggccttgaagtctcatagggctacttatctttctctccacagtatgaaaaggctttctcatccaagtatctgcagaactggtctcccactaagccaacaaaagaggtattccatgttcagtgcacctacaagatagcctcatgctctccctgtcaattaactccttttagcattctctaaactcccatatccttctctgaccaagctccccaaatacttccctttttcccctcacaaacctttatctctcccacttgtaccccagagcatctcttctcatgaaggctacactcaaattattgccaacgatcgtggtcatctactgccttctgtgccccgttccaaggtgagatactatcttcactcctatcaagaaagtcaaataattaaggcacagaactgggagatgtgcagtctctcacagccattatcgggaaaattaaagtttaatctaattcatgttgtaatgtgagagcccctgaacttccggccagcttacccagcaggatagagttgtgtttagcacccttcagaagttcttaaattgatcaatgatctgtataaatgaaagccttcaggtgatgacatttgtgcagtgggtactcctttgccacactcggcctaaggatgtggaatttaagttggcagagtaaaggggatgaaaaaattaggcctgcaaagcctaaatgagggagggggataaggaagggtgggaagattatgctttcagtcttgtttcataaccatgcattcctaaaggtaaagaaaggaaataatacagaggtctaagtcagttactgggagtgagaagccctactgaggaatcccttttcatttttaggcaaatccttggggttccttcatgggcacctggcaaatgcctctgaagataccccctgctcgggtgaccctgacctcccgtacaactgctggtgctgcctccctcaccaaatggatacagaaaaatcctgatttactcaaggcctccaatgggctgtgtcctgaaatcttaggcaaggtatctattcttcccatctaacccaaaaccctgtagtctcaatttcttttcaacctcaaaaaatgtctattgttatgccaccactatcccagcatgggggacctctaaccaatttgtcttatcttgactagtccttaatcaccttctgaggcctgaagggatgggctaaggacatcatacccccaacagtagaaaatgatctaatctcaaggtgggggagggtggttagagaaatcaaatttaacttttcttatttgaaacttgatctactgcccatggtatggggagaaagggagttagaatcctgaggtgcattaggaatgatccgggcctgaccagagacatgactatctctcccactcttatcactgacagccccatgatccagacagtcagaagaaactcagaaagaagtctatcacaaagactgtacaacaagcacgaagtccaaccataattccaagctccccagctgccaacctcaattccccagatgaactccaaagctcacacccctctgcaggtcatactccaggtccccaaagaccagccaaatcctaagagcccacctggaagtccacgtatgctagaactctgggcagggcctaatctagctgaggtccagaaatacaaacctggaacttcatatggaccaagtggccacacactgaaaaacccgtatagcgactcagtgaaataaacaagagcccccagtcagaactgtgaaacagggaaattttggggtgggagtaaaagcaaatttggaaaataaacttttttttgttgaatcttttactgatctggattttccattcttgctatggctgcctcttgtaacacaattaggagaaggaaggtaggagaaaataaagtagggaaaagaacatacagtggtttgggtggaacacatttttacaagaattgagtcagttatactccagaaatgaccaagagaaagttggtctgaatcatggaaaaagggcagaacctcaaagaaccagtccctcaaccctacccactcattttttatcctgagcatggacaactaacaactacaaaatcagaaatagaattgagtagagtatgtatatgtgtgtttggagaaggtggggaagaaaaggtagggaaaaccaaagtagaagatactatgcttgtgtaagactttctatctaagcccaagtacaaatatagtttgaaaattgaagatattaaagtgattggaagacagagaagaaaaagacagtaagtagaaatttaaggcagaataacaaacatgatgctctgtcacaccccccacccacccactaccatgcttcaatcacccaaatggtacgaaaccaccaaaaaattcaactgccctacccattttccagcctctaacagctgtttatcattgaccccattttatattttcctggcactggctgttaaatttaatgcccttgccaaacctttcccagtcccaatgacaaagtgttctgtcatgatcacttgtccctcattccaaggacaaagtagagaacagctggtttaaaatggaggaaaggtacaaggacttcccagggcccctctagtaaaaagggaaaaccaatcattacttaaagccaaatactatttgggaccctgaatgaagactgttaaaacagcgggtccccaccttaactaaggtcttcctatccaattgacaccagccagttaacatttcccctcttcgacccacagctttaactggctggccaacaactcgaagtgacagatgagataagtctcttattccagagttcccaaaaactatcaaaacagcatgcctgctaaagcctggcctatatggattttaaaagcagcaagttttctcattaaattatacatttttgccaggttttcaacaatcccttcttttttaaaaaaaaactctatgcttcattcaccccaagcctataacctcaggtcatcatcccctagctgtcaccaacactggtcctctgtgcccctcaatgaatcataatttgctgaactgtaccatgaagcttataatcagtccttaatgggattttggtgcctataacccaaaagcactctacatgcgtcacttcttttctttttctccttccttctctgaggcttttctgtgatatttaaatctctggctaagttctatctgattccctgaaaacttttccaatgatgagatgtaggagaactgtttccctcctggtaaaggtcagattgcggggagagggaggatgtaaatgcctgagacccgagggaagaggaggaaattggttccttcccaacagccattttcttggtttctctagatttcaaggagagtcaaagataaaatgagtatttaattcagtttcagaaaaaaagggtacattacttcgatgagaaagcataaaattaagaggcttttctggaaatccaagaaaaagaaataaccattaatatgttcaatgataattttctagatcttcctcgtgtccaaagctatatattttctcctcaaaagcagctgctccaagaactaactagccctctttatctccctctagctgggacagactaattcccctccacccccacctctcttctttcaataacactgtgtaggtgttaatggcctgggctctcaccaatgaagagaattgtcctttaagccagcaacccacaggcagtggcacccaaagcctcaccaacccaccccccaacccggcccatccccagggcagaagccacagagctggcattgtttccactgtctcaggaagaaggagccaaaagctgaccctcagcacaaatcaaagcccaatatggagagagaataactgcttctaggccgagagtaggcaagctgtgggcaaaaaaggggagtttttgcagccacctcatctttagaaacaaggggaaaactagacccttttccactattatggtctaccaggtactctactgctccaaggagatctgaaaatacaaaaggatctaaacaaataaggagaacttttcccaggctggagataagaatgacaaacagaaagatgggtgaatgtaataatgtgtaggaagatgatgctgggagcctcctttcttcacatggctgccagccccatagaggacaacacagtaagaaccaggacaaccactccagactggtatagctggggaatcttcaggccttttcctaggtcccacatcaagtgtcggatcccattccaggtatgatacatgagagggaagacaagtgcaaacttagctgtgtggatcagtgctggccccagacacagggacttcacaagttccaaataagactcaaagttcccagggagtaacagggccgacatgccaaaaagagagacccctgcactcaaagcaataccagtgccacggtggcagatggacatcgccatgggaagagaccaatttctgatacagagctgagggctaaagtgggctcggaggcaatgacgaccaacgtgtctcagcaacagcgcagccatcttgggttccggtctggacggaagt

SEQ ID NO: 17304 - RNA, 13004 nt, Homo sapiens
  source 1..13004: mol_type = other RNA
tcaggccaggcacagtggctcacgcctgtaatccaacgactttgggaggccaaggcaggtggatcacctgacgtcaggagttccagaccagcctggccaacatggcgaaaccctgtctctactaaaaatactaaaattagcagggcatgctggtgtgtgcctataatcccagctatggaggggggctgaagcaggaggatcacttgaacctgggaggcggaggttgcagtgagctgagatggtgccactgcactccagcctgggcaacagagcaagattctgtctcaaaaaaaaaaaaaaaaaaaaaggaatgaaagaaaagaaaaagaaatagtgttaaatagctctatgaatgctgcagagagggctaccccataggcagtgtgtggggagtatacaaagcttgttctttggctcctcaggaaggggatcttatcaagaatattattcttttgtggtattgtcagtggaaaggagagatgtaacagcagtctccgagagagggagccttagtctcaggaaagaaaactggatcagctattttaactctatagagaagttttgaaactatagcttttacatttgtagccatgcatctcttcaggggtcagaactacgccttcatttcctataaggaaatctacaaaaaccagggtgtttgaatagttcaaaatttggccagtagcttggttggatgaaatcctgttagcccaggaaatggggcaaaagccaggtctcctatccaagacccatcaacacctgacccagtgaggtgacatggagggcaccttggagctacttagaagaaaccttagtagagagctgatggtataactagagacagtgattcaggtggttacactgtgtaatagatgagataaatgccccatttttactatgaaggggttactaataattttttctggttttaaaaattgccatgggaggccgggcgcggtggctcacgcctgtaatcccagcactttgggaggctgaggtgggcggatcaactgaggtcaggcattcgagaccagcctgaccaacatggagaaaccctgtctctactaaaaatacaaaattagccgggtgtggtggtgcatgcctaaaatctcagctactcgggaggctgaggcaggagaatcgctcgcttgaacccgggaggcggaggttgcggtgagccgagatcgcacattgcactccagcctgggcaacaagagcgaaactccatctcaaaaaaaaaaaaaaaaagaaaagaaaagaataaaggcagtgagaaacagagatgataaagaagaaacagaaaatctttctgatcatgttctatctttgaaattctagtatcctttgaagcccaaactatacttcctacctttggaatctgttaaatactcctattaattataatttccccacttccccttttttgtttaaggtaacctgaatgagtacttcttacttggcagtcttaagccaataataatgctaaaataattgagcattcattatgcatcttgcaccctattagcatgttacatatatttaatgctcaaaactaagattatccccattttacatgtaagggtactgagacccagaaagattaacttgtgtaaggccacacatttaggcaaagccagaatttaatccaggcaatgtgactctagtacttatgctggtggttgccttcacgtaggtccaatgtacacatcgcctatagagtacaggttaaacttgtacttcaatagcagataatctcagtccaaataaaagatttcctaatggtttagtttcagtcatcaaagaatttaagtgaatggaaaaaagtatcttaaggcatacgtaaaggatggggcctttaaagagcccttccaactttggaagaagtaaatctggtcctagtaaaagaccatctgctgtacctgaagtcaaccagttcatctgaagaaaggctaaaattcaatacacttttattagaagcttaaaattgcctgttactactgatattacaatttcctagtgaaatcttttttttgttgagacggagtctcgctctgtcgcccaggctggagtgcagtggcgcgatctcggctcactgccagctccacctcccgggttcacgccattctcctgcctcagcctcccgagtagctgggactacaggcaccccccaccacgccgggctaattttttgtatttttagcagagacggagtttcaccgtgttagccagcatgctctcgatttcctgaccttgtgatccacccccctgggcctcccaaagtgctgggattacaggcctgagccaccgcgcccggcctgaaatcttaaatattagaattcacataggatcaagccaggactccaccttggatttttttttttttttttttagacggagtctcactctgtcgccaggctggagcacagtggcgcaatctcggctcactgcaacctccgcctcccgggttcaagcgattcttctgcctcagcctctggagtagctgggactacaggcgcgcgccactacgcccagctaatttttgtatttttagtagagacggggtttcaccatgttggccaggatggtctccatctcttgatctcgtgatcctcccgtctcagcctctcaaagtactgggattacaggcgtgagtcaccgcgcctggcctttttttttcttttttttgagatggagtctcactctgtcgcccgggggatggagtgcagtggcgcaatctcggctcactgcaacctccacctcccgggttcaagcgattctcttgcctcagcctcccgagtagctgggactacaggcacgtgtcaccatgcccagctaatttttgtatttttagtagaaacagagtttcgccatgttggtcaggctggtctcgaacttctgtcctcaactgttccacctgcctcagcctccgaaagtgctaggattacacgtgtgagccactgtgcccagcgtgtaccttggattttagattacagagagacaaataatctaaaacgatcacctttctctctagaacagtgggttagaggatccagaaacagacccaaatatgttagggaatacattaaaaatggcatttcaaatcagtagaggaaaagaaaacttattaatgatgccaaggcaactagttaaggcaactgaagcataaccttgtccacattcactaaaattccagaaggaacaaatatttaaatgtaagaactgaagctaggggtaaattatttttaaaatattggaattcacaaaaagccattcaaagcataagatccagagcacagaaaaaatgagtaatacatctgactactacataagtactaaaaacatgtccatggcaaaaaaaaaaaaaaaaacccacagaaaaacaacaacaaaacagaaaaaccaccaacaaaatgaaagtaagtgacaaattggagggaatatttgcaacatatttgacaaaggactaatttccttaatatatggagttcaaacagattaatgaacatgatcaacaggctgggtgcagtggctcaagcctgtaatcccagctttttgggaagctgaggtgggcagatggcttgagcccaggagttcaaaaccagcctgggcaacatggcaaaatcccatctctacaaaaaaaattaaaaaatcagctgggtgtggtggtgcatccctgtagttccagttattcgggaggctgaggtgggaggattgtttggacctgagaggcagaagttacagtgaaccaagatgatgccactgcactccagcctgggtgacagagggaggactggtttcaaaaaaaaaagtcaacagcccaatagtaagtggcaaaatacattaaaggccattttcagggaaaaaaattaaaataaaaacagtttatacacatataaaaacaccctaattaaagaaatgcaaatttaaaacaatgatataccatgttgggtgggtgtggtggctcgtgcctgtaatctcaacacttccagaggtcgaagaatcacttgaggccatgaattcaagacaagaggaacaatatagttaagaccctatctcttaaaaaaaatttgtttttttaaattagctgggcatggtagctcatgcctatactcccaactacttgggaggctaaggtgggaggattgcttgacctcaggatattgatggaaccactgcactccagagcttaggcggcagggagaccgtctcaaaacaaaaacaaaaaataaaattatataccatgtttaacctacagcttaacaagcaatatgatataatggttaaaactgctggctctagagtcagaatacttgggattaaatcctggctctactcctcactgtgtattctccagtttccttggttgggttgagaactaaatgagaaaatgtagtaaagcaattagaactgtgcctggcatgtatatagtaactgctcagttaacattagttctactagttcaatcaattagttctattagttcaattctattagttcaattaaaattggtttaaactgaaaaaaaaagaaaaaacgatgatgttgaaaagaaagcagagaactaggcactcatacgccatcatacaccactggtagaagtacaaactggcacaatgtctttcagtggtaatttgacattatctacttattttattttatttatttatttatttttgagacggagtctcgctctgtctcccaggctggactgcagtggcgcgatcgtggctcactgcaagctccgcctcctgggttcacgccattctcctgcctcagcctcctgagtagctgggactacaggcccccgccacacgcccagctaatgttttgtatttttagtagagatggggtttcaccatgttagccaggatggtctcgatctcctgacctcgtgatcgcccgcctcagcctcccaaagtgctgggattacagatgtgagccaccgcacccggcctatctacttattttaaatgcacaaacccttttgactttgcaatgtactttaaaacatttatcctacagatcacatatgtacataaaaatacatacatacatattcataaagatacatagggatttttcattacagcaatgtccttattagcaaaagactataaataaactaaatggtcatccatatgggtctgaacaaactatggtgcatcccaaaatggaatattatgataaaaacataatccccaagatagtcaaaaagcaaatcaaaaagcaatgtggacagctctctcattagtgtttgtatgcagagaagatttctggaaggagacacaagaaatgagtaacagcagttgccctgaggagcaagactgagagttgaaatcaaatggagatttgcttttcactgaacatcctgtaaacatgaaattttttccatgtacattactttttcaattgaacaaaaactggttaacttttaaaaatgagtgcagtcatcatttatcattacattcctatcagaaaggcagagggaggcataccaactgaagacaaattctaagagaaataatgctagcctatcattgcagattaaagggccaaaatggatatcctagagcaaagatagtccttggtccttaaagaactcttctctagagagtgataagaaccacagggactaagctcatgagttatctttccagatctcacattatccaggtattaactccagagcctataaaacaagagctgttcttccctccatctgcagaagcataggagtgctcttatacttggtgtgttggttaagatgaggattttgggggaagaaggaaaagagaagggactgatggatatactttatttattttttattttttgagacggagtctcacgctgtcgcccaggctgaagtgcagtagtagcatgatctctgctcattgcaacctccgcctcccgggttcaagcaattctcctgcctcagcctcccgagtagctgggattagaggcatgcaccaccatgcctggctaattttttgtatttttagtagagacagggtttctccatgttggccaggctggtctcgaactcctgaccttgtgatccgtctgcttcggccacccaaagtgctgggattacaggcatgagccaccgtgcccggcctggatatactttataatggtctcctggtcctaatgatatctttgggcaacttatttcttagtttttccctttcatcttgacaccttatatataaattcactttacaattcacaaagcacagttctacttacttattaattctcctaaccacctcatagatgggtattacaataccattttatgagtttcagaggggtttccttgtcccacacatattaggcttatgtcctggcagccccccattgaactctccaaacctgatcctttccactctgtgattttctctcttcatccctgctcaatctccctgcaccagcacccgattccattttattccagtcaacactaaacgcctgtgttcttaggtgctgattctagacagtgacagaggaaattttttaaggaccaaggacaagatatgtttttccttctggggacagatttgagctagttgctttttaaatattgttcctttgttattctgcctgataagacaaagtagtgggccttataaacaggatctcaccaggattgaatacctactatgctatgatattgtctagacactttattcattttatctcacttaccctgtaaaagcaggctctattatccccacaatacaaatgagttgatagaaatttagtgaagacaagacagttgtttaatgtcatatagctcctatgttcccatgttgaataaggattcaaaccccagtatctggctctacagcctgtggtacattacaccatgttgtccaacaagcatagctctcagggttacatggtttgttaaagtggttaaaaaccccaatcaaaggcccgtggaagttcttaagcaggggtaggttatgccagaaaaaaagtagtggctattcagctaattttctcacatttactcagtctttcccgtctgtaaaataaaaatgaatctaagttccagagaaaacaaatgggggcagtgtgagccaaggaagtgaataataataagcagaagagaaaggcagcctctgctcattggtagtcccaggaggtcggccttctgcagttgccaagcaacgagtgtaaacagcacaagatcatggccactaactacagtgccaaccaggtaagttcccattctccatttctttaacgtttacttttgtttttcagattctatctttggactgtcccctctcataggattctgatctttgaacagatagctgagagtggagtgagataatattttacctcctcagggatagagagagcccaggggcgatccaaaggtatctcttggttaaatttgtagggtgtaaaccagaagttggcaattttttttctgtaaaagggcggagtgtaaaaattttaggctttgcaggccaagtggcaaagtcaaaaatattctgtagctacttgcataattaaagaaaaacatttttccataacatttttgacaaattcaaaatataactgagtacaattttttgtactactaatgaaaataatggaattttgggggttgagaaaacatttcacttaactgggattcaaagttagtgttccatttgactgaatcaattgtaaatgttcatctataaaaatcacccttactctcaggccatccccaaacaggcagcaatatggatatggcccataggccatagtttaccaactcctgatctagaccagtgctgcccaacaaaaagagtgcgacccacaaatgtaattttaaattttctagtagctacatgaaaaaattaaaacataaaatttaaatatattgaatttaacccaataaatccaaatattatttcaacatttaatcagtatttaaaaaattataatcagacattttacgttctttttttgtactaaatctccaaaacctgctgggtgttgtagctcacgtctgtaatcccaacactttgggaggctgaggcacaaggatcgcttgaggccaggggtttgagaccaccctgggcaatatggtgagacctcgtctctacaagtaaatttaaaaattagctggacatggtggcatgcacctgtagtcccagctacctgtgagtctgagggaggaggatcgcttgaacccaggtgtccaaggctgcagtgagctaggatcatgccactgactccaacccaggtggcagaccaagatcctatctcaaaaaaaaaaagaaaagaaaaaaacttaaaaattcagcatatttcatatttacaaagcacctcaatttgaactagtcatatttcaggtgctcaacagctccatgtggctcccggctccatgctggacagcacacatctagaccaaacaaattacacccttgtcatagtgacttaaagcctacatggttggtcaggcctttggtcttcaaatctaaagaattgtgcctagtcttcatttcctgggtttggggccttgaagtctcatagggctacttatctttctctccacagtatgaaaaggctttctcatccaagtatctgcagaactggtctcccactaagccaacaaaagaggtattccatgttcagtgcacctacaagatagcctcatgctctccctgtcaattaactccttttagcattctctaaactcccatatccttctctgaccaagctccccaaatacttccctttttcccctcacaaacctttatctctcccacttgtaccccagagcatctcttctcatgaaggctacactcaaattattgccaacgatcgtggtcatctactgccttctgtgccccgttccaaggtgagatactatcttcactcctatcaagaaagtcaaataattaaggcacagaactgggagatgtgcagtctctcacagccattatcgggaaaattaaagtttaatctaattcatgttgtaatgtgagagcccctgaacttccggccagcttacccagcaggatagagttgtgtttagcacccttcagaagttcttaaattgatcaatgatctgtataaatgaaagccttcaggtgatgacatttgtgcagtgggtactcctttgccacactcggcctaaggatgtggaatttaagttggcagagtaaaggggatgaaaaaattaggcctgcaaagcctaaatgagggagggggataaggaagggtgggaagattatgctttcagtcttgtttcataaccatgcattcctaaaggtaaagaaaggaaataatacagaggtctaagtcagttactgggagtgagaagccctactgaggaatcccttttcatttttaggcaaatccttggggttccttcatgggcacctggcaaatgcctctgaagataccccctgctcgggtgaccctgacctcccgtacaactgctggtgctgcctccctcaccaaatggatacagaaaaatcctgatttactcaaggcctccaatgggctgtgtcctgaaatcttaggcaaggtatctattcttcccatctaacccaaaaccctgtagtctcaatttcttttcaacctcaaaaaatgtctattgttatgccaccactatcccagcatgggggacctctaaccaatttgtcttatcttgactagtccttaatcaccttctgaggcctgaagggatgggctaaggacatcatacccccaacagtagaaaatgatctaatctcaaggtgggggagggtggttagagaaatcaaatttaacttttcttatttgaaacttgatctactgcccatggtatggggagaaagggagttagaatcctgaggtgcattaggaatgatccgggcctgaccagagacatgactatctctcccactcttatcactgacagccccatgatccagacagtcagaagaaactcagaaagaagtctatcacaaagactgtacaacaagcacgaagtccaaccataattccaagctccccagctgccaacctcaattccccagatgaactccaaagctcacacccctctgcaggtcatactccaggtccccaaagaccagccaaatcctaagagcccacctggaagtccacgtatgctagaactctgggcagggcctaatctagctgaggtccagaaatacaaacctggaacttcatatggaccaagtggccacacactgaaaaacccgtatagcgactcagtgaaataaacaagagcccccagtcagaactgtgaaacagggaaattttggggtgggagtaaaagcaaatttggaaaataaacttttttttgttgaatcttttactgatctggattttccattcttgctatggctgcctcttgtaacacaattaggagaaggaaggtaggagaaaataaagtagggaaaagaacatacagtggtttgggtggaacacatttttacaagaattgagtcagttatactccagaaatgaccaagagaaagttggtctgaatcatggaaaaagggcagaacctcaaagaaccagtccctcaaccctacccactcattttttatcctgagcatggacaactaacaactacaaaatcagaaatagaattgagtagagtatgtatatgtgtgtttggagaaggtggggaagaaaaggtagggaaaaccaaagtagaagatactatgcttgtgtaagactttctatctaagcccaagtacaaatatagtttgaaaattgaagatattaaagtgattggaagacagagaagaaaaagacagtaagtagaaatttaaggcagaataacaaacatgatgctctgtcacaccccccacccacccactaccatgcttcaatcacccaaatggtacgaaaccaccaaaaaattcaactgccctacccattttccagcctctaacagctgtttatcattgaccccattttatattttcctggcactggctgttaaatttaatgcccttgccaaacctttcccagtcccaatgacaaagtgttctgtcatgatcacttgtccctcattccaaggacaaagtagagaacagctggtttaaaatggaggaaaggtacaaggacttcccagggcccctctagtaaaaagggaaaaccaatcattacttaaagccaaatactatttgggaccctgaatgaagactgttaaaacagcgggtccccaccttaactaaggtcttcctatccaattgacaccagccagttaacatttcccctcttcgacccacagctttaactggctggccaacaactcgaagtgacagatgagataagtctcttattccagagttcccaaaaactatcaaaacagcatgcctgctaaagcctggcctatatggattttaaaagcagcaagttttctcattaaattatacatttttgccaggttttcaacaatcccttcttttttaaaaaaaaactctatgcttcattcaccccaagcctataacctcaggtcatcatcccctagctgtcaccaacactggtcctctgtgcccctcaatgaatcataatttgctgaactgtaccatgaagcttataatcagtccttaatgggattttggtgcctataacccaaaagcactctacatgcgtcacttcttttctttttctccttccttctctgaggcttttctgtgatatttaaatctctggctaagttctatctgattccctgaaaacttttccaatgatgagatgtaggagaactgtttccctcctggtaaaggtcagattgcggggagagggaggatgtaaatgcctgagacccgagggaagaggaggaaattggttccttcccaacagccattttcttggtttctctagatttcaaggagagtcaaagataaaatgagtatttaattcagtttcagaaaaaaagggtacattacttcgatgagaaagcataaaattaagaggcttttctggaaatccaagaaaaagaaataaccattaatatgttcaatgataattttctagatcttcctcgtgtccaaagctatatattttctcctcaaaagcagctgctccaagaactaactagccctctttatctccctctagctgggacagactaattcccctccacccccacctctcttctttcaataacactgtgtaggtgttaatggcctgggctctcaccaatgaagagaattgtcctttaagccagcaacccacaggcagtggcacccaaagcctcaccaacccaccccccaacccggcccatccccagggcagaagccacagagctggcattgtttccactgtctcaggaagaaggagccaaaagctgaccctcagcacaaatcaaagcccaatatggagagagaataactgcttctaggccgagagtaggcaagctgtgggcaaaaaaggggagtttttgcagccacctcatctttagaaacaaggggaaaactagacccttttccactattatggtctaccaggtactctactgctccaaggagatctgaaaatacaaaaggatctaaacaaataaggagaacttttcccaggctggagataagaatgacaaacagaaagatgggtgaatgtaataatgtgtaggaagatgatgctgggagcctcctttcttcacatggctgccagccccatagaggacaacacagtaagaaccaggacaaccactccagactggtatagctggggaatcttcaggccttttcctaggtcccacatctgcactcaaagcaataccagtgccacggtggcagatggacatcgccatgggaagagaccaactgtagatagtaatgtggggagacagaggacggtttgaacctatattcttattccagaaccgctccatctcttctttggccgtggttcccaaaggaacagcatttctgatacagagctgagggctaaagtgggctcggaggcaatgacgaccaacgtgtctcagcaacagcgcagccatcttgggttccggtctggacggaagt

SEQ ID NO: 17305 - RNA, 12902 nt, Homo sapiens
  source 1..12902: mol_type = other RNA
tcaggccaggcacagtggctcacgcctgtaatccaacgactttgggaggccaaggcaggtggatcacctgacgtcaggagttccagaccagcctggccaacatggcgaaaccctgtctctactaaaaatactaaaattagcagggcatgctggtgtgtgcctataatcccagctatggaggggggctgaagcaggaggatcacttgaacctgggaggcggaggttgcagtgagctgagatggtgccactgcactccagcctgggcaacagagcaagattctgtctcaaaaaaaaaaaaaaaaaaaaaggaatgaaagaaaagaaaaagaaatagtgttaaatagctctatgaatgctgcagagagggctaccccataggcagtgtgtggggagtatacaaagcttgttctttggctcctcaggaaggggatcttatcaagaatattattcttttgtggtattgtcagtggaaaggagagatgtaacagcagtctccgagagagggagccttagtctcaggaaagaaaactggatcagctattttaactctatagagaagttttgaaactatagcttttacatttgtagccatgcatctcttcaggggtcagaactacgccttcatttcctataaggaaatctacaaaaaccagggtgtttgaatagttcaaaatttggccagtagcttggttggatgaaatcctgttagcccaggaaatggggcaaaagccaggtctcctatccaagacccatcaacacctgacccagtgaggtgacatggagggcaccttggagctacttagaagaaaccttagtagagagctgatggtataactagagacagtgattcaggtggttacactgtgtaatagatgagataaatgccccatttttactatgaaggggttactaataattttttctggttttaaaaattgccatgggaggccgggcgcggtggctcacgcctgtaatcccagcactttgggaggctgaggtgggcggatcaactgaggtcaggcattcgagaccagcctgaccaacatggagaaaccctgtctctactaaaaatacaaaattagccgggtgtggtggtgcatgcctaaaatctcagctactcgggaggctgaggcaggagaatcgctcgcttgaacccgggaggcggaggttgcggtgagccgagatcgcacattgcactccagcctgggcaacaagagcgaaactccatctcaaaaaaaaaaaaaaaaagaaaagaaaagaataaaggcagtgagaaacagagatgataaagaagaaacagaaaatctttctgatcatgttctatctttgaaattctagtatcctttgaagcccaaactatacttcctacctttggaatctgttaaatactcctattaattataatttccccacttccccttttttgtttaaggtaacctgaatgagtacttcttacttggcagtcttaagccaataataatgctaaaataattgagcattcattatgcatcttgcaccctattagcatgttacatatatttaatgctcaaaactaagattatccccattttacatgtaagggtactgagacccagaaagattaacttgtgtaaggccacacatttaggcaaagccagaatttaatccaggcaatgtgactctagtacttatgctggtggttgccttcacgtaggtccaatgtacacatcgcctatagagtacaggttaaacttgtacttcaatagcagataatctcagtccaaataaaagatttcctaatggtttagtttcagtcatcaaagaatttaagtgaatggaaaaaagtatcttaaggcatacgtaaaggatggggcctttaaagagcccttccaactttggaagaagtaaatctggtcctagtaaaagaccatctgctgtacctgaagtcaaccagttcatctgaagaaaggctaaaattcaatacacttttattagaagcttaaaattgcctgttactactgatattacaatttcctagtgaaatcttttttttgttgagacggagtctcgctctgtcgcccaggctggagtgcagtggcgcgatctcggctcactgccagctccacctcccgggttcacgccattctcctgcctcagcctcccgagtagctgggactacaggcaccccccaccacgccgggctaattttttgtatttttagcagagacggagtttcaccgtgttagccagcatgctctcgatttcctgaccttgtgatccacccccctgggcctcccaaagtgctgggattacaggcctgagccaccgcgcccggcctgaaatcttaaatattagaattcacataggatcaagccaggactccaccttggatttttttttttttttttttagacggagtctcactctgtcgccaggctggagcacagtggcgcaatctcggctcactgcaacctccgcctcccgggttcaagcgattcttctgcctcagcctctggagtagctgggactacaggcgcgcgccactacgcccagctaatttttgtatttttagtagagacggggtttcaccatgttggccaggatggtctccatctcttgatctcgtgatcctcccgtctcagcctctcaaagtactgggattacaggcgtgagtcaccgcgcctggcctttttttttcttttttttgagatggagtctcactctgtcgcccgggggatggagtgcagtggcgcaatctcggctcactgcaacctccacctcccgggttcaagcgattctcttgcctcagcctcccgagtagctgggactacaggcacgtgtcaccatgcccagctaatttttgtatttttagtagaaacagagtttcgccatgttggtcaggctggtctcgaacttctgtcctcaactgttccacctgcctcagcctccgaaagtgctaggattacacgtgtgagccactgtgcccagcgtgtaccttggattttagattacagagagacaaataatctaaaacgatcacctttctctctagaacagtgggttagaggatccagaaacagacccaaatatgttagggaatacattaaaaatggcatttcaaatcagtagaggaaaagaaaacttattaatgatgccaaggcaactagttaaggcaactgaagcataaccttgtccacattcactaaaattccagaaggaacaaatatttaaatgtaagaactgaagctaggggtaaattatttttaaaatattggaattcacaaaaagccattcaaagcataagatccagagcacagaaaaaatgagtaatacatctgactactacataagtactaaaaacatgtccatggcaaaaaaaaaaaaaaaaacccacagaaaaacaacaacaaaacagaaaaaccaccaacaaaatgaaagtaagtgacaaattggagggaatatttgcaacatatttgacaaaggactaatttccttaatatatggagttcaaacagattaatgaacatgatcaacaggctgggtgcagtggctcaagcctgtaatcccagctttttgggaagctgaggtgggcagatggcttgagcccaggagttcaaaaccagcctgggcaacatggcaaaatcccatctctacaaaaaaaattaaaaaatcagctgggtgtggtggtgcatccctgtagttccagttattcgggaggctgaggtgggaggattgtttggacctgagaggcagaagttacagtgaaccaagatgatgccactgcactccagcctgggtgacagagggaggactggtttcaaaaaaaaaagtcaacagcccaatagtaagtggcaaaatacattaaaggccattttcagggaaaaaaattaaaataaaaacagtttatacacatataaaaacaccctaattaaagaaatgcaaatttaaaacaatgatataccatgttgggtgggtgtggtggctcgtgcctgtaatctcaacacttccagaggtcgaagaatcacttgaggccatgaattcaagacaagaggaacaatatagttaagaccctatctcttaaaaaaaatttgtttttttaaattagctgggcatggtagctcatgcctatactcccaactacttgggaggctaaggtgggaggattgcttgacctcaggatattgatggaaccactgcactccagagcttaggcggcagggagaccgtctcaaaacaaaaacaaaaaataaaattatataccatgtttaacctacagcttaacaagcaatatgatataatggttaaaactgctggctctagagtcagaatacttgggattaaatcctggctctactcctcactgtgtattctccagtttccttggttgggttgagaactaaatgagaaaatgtagtaaagcaattagaactgtgcctggcatgtatatagtaactgctcagttaacattagttctactagttcaatcaattagttctattagttcaattctattagttcaattaaaattggtttaaactgaaaaaaaaagaaaaaacgatgatgttgaaaagaaagcagagaactaggcactcatacgccatcatacaccactggtagaagtacaaactggcacaatgtctttcagtggtaatttgacattatctacttattttattttatttatttatttatttttgagacggagtctcgctctgtctcccaggctggactgcagtggcgcgatcgtggctcactgcaagctccgcctcctgggttcacgccattctcctgcctcagcctcctgagtagctgggactacaggcccccgccacacgcccagctaatgttttgtatttttagtagagatggggtttcaccatgttagccaggatggtctcgatctcctgacctcgtgatcgcccgcctcagcctcccaaagtgctgggattacagatgtgagccaccgcacccggcctatctacttattttaaatgcacaaacccttttgactttgcaatgtactttaaaacatttatcctacagatcacatatgtacataaaaatacatacatacatattcataaagatacatagggatttttcattacagcaatgtccttattagcaaaagactataaataaactaaatggtcatccatatgggtctgaacaaactatggtgcatcccaaaatggaatattatgataaaaacataatccccaagatagtcaaaaagcaaatcaaaaagcaatgtggacagctctctcattagtgtttgtatgcagagaagatttctggaaggagacacaagaaatgagtaacagcagttgccctgaggagcaagactgagagttgaaatcaaatggagatttgcttttcactgaacatcctgtaaacatgaaattttttccatgtacattactttttcaattgaacaaaaactggttaacttttaaaaatgagtgcagtcatcatttatcattacattcctatcagaaaggcagagggaggcataccaactgaagacaaattctaagagaaataatgctagcctatcattgcagattaaagggccaaaatggatatcctagagcaaagatagtccttggtccttaaagaactcttctctagagagtgataagaaccacagggactaagctcatgagttatctttccagatctcacattatccaggtattaactccagagcctataaaacaagagctgttcttccctccatctgcagaagcataggagtgctcttatacttggtgtgttggttaagatgaggattttgggggaagaaggaaaagagaagggactgatggatatactttatttattttttattttttgagacggagtctcacgctgtcgcccaggctgaagtgcagtagtagcatgatctctgctcattgcaacctccgcctcccgggttcaagcaattctcctgcctcagcctcccgagtagctgggattagaggcatgcaccaccatgcctggctaattttttgtatttttagtagagacagggtttctccatgttggccaggctggtctcgaactcctgaccttgtgatccgtctgcttcggccacccaaagtgctgggattacaggcatgagccaccgtgcccggcctggatatactttataatggtctcctggtcctaatgatatctttgggcaacttatttcttagtttttccctttcatcttgacaccttatatataaattcactttacaattcacaaagcacagttctacttacttattaattctcctaaccacctcatagatgggtattacaataccattttatgagtttcagaggggtttccttgtcccacacatattaggcttatgtcctggcagccccccattgaactctccaaacctgatcctttccactctgtgattttctctcttcatccctgctcaatctccctgcaccagcacccgattccattttattccagtcaacactaaacgcctgtgttcttaggtgctgattctagacagtgacagaggaaattttttaaggaccaaggacaagatatgtttttccttctggggacagatttgagctagttgctttttaaatattgttcctttgttattctgcctgataagacaaagtagtgggccttataaacaggatctcaccaggattgaatacctactatgctatgatattgtctagacactttattcattttatctcacttaccctgtaaaagcaggctctattatccccacaatacaaatgagttgatagaaatttagtgaagacaagacagttgtttaatgtcatatagctcctatgttcccatgttgaataaggattcaaaccccagtatctggctctacagcctgtggtacattacaccatgttgtccaacaagcatagctctcagggttacatggtttgttaaagtggttaaaaaccccaatcaaaggcccgtggaagttcttaagcaggggtaggttatgccagaaaaaaagtagtggctattcagctaattttctcacatttactcagtctttcccgtctgtaaaataaaaatgaatctaagttccagagaaaacaaatgggggcagtgtgagccaaggaagtgaataataataagcagaagagaaaggcagcctctgctcattggtagtcccaggaggtcggccttctgcagttgccaagcaacgagtgtaaacagcacaagatcatggccactaactacagtgccaaccaggtaagttcccattctccatttctttaacgtttacttttgtttttcagattctatctttggactgtcccctctcataggattctgatctttgaacagatagctgagagtggagtgagataatattttacctcctcagggatagagagagcccaggggcgatccaaaggtatctcttggttaaatttgtagggtgtaaaccagaagttggcaattttttttctgtaaaagggcggagtgtaaaaattttaggctttgcaggccaagtggcaaagtcaaaaatattctgtagctacttgcataattaaagaaaaacatttttccataacatttttgacaaattcaaaatataactgagtacaattttttgtactactaatgaaaataatggaattttgggggttgagaaaacatttcacttaactgggattcaaagttagtgttccatttgactgaatcaattgtaaatgttcatctataaaaatcacccttactctcaggccatccccaaacaggcagcaatatggatatggcccataggccatagtttaccaactcctgatctagaccagtgctgcccaacaaaaagagtgcgacccacaaatgtaattttaaattttctagtagctacatgaaaaaattaaaacataaaatttaaatatattgaatttaacccaataaatccaaatattatttcaacatttaatcagtatttaaaaaattataatcagacattttacgttctttttttgtactaaatctccaaaacctgctgggtgttgtagctcacgtctgtaatcccaacactttgggaggctgaggcacaaggatcgcttgaggccaggggtttgagaccaccctgggcaatatggtgagacctcgtctctacaagtaaatttaaaaattagctggacatggtggcatgcacctgtagtcccagctacctgtgagtctgagggaggaggatcgcttgaacccaggtgtccaaggctgcagtgagctaggatcatgccactgactccaacccaggtggcagaccaagatcctatctcaaaaaaaaaaagaaaagaaaaaaacttaaaaattcagcatatttcatatttacaaagcacctcaatttgaactagtcatatttcaggtgctcaacagctccatgtggctcccggctccatgctggacagcacacatctagaccaaacaaattacacccttgtcatagtgacttaaagcctacatggttggtcaggcctttggtcttcaaatctaaagaattgtgcctagtcttcatttcctgggtttggggccttgaagtctcatagggctacttatctttctctccacagtatgaaaaggctttctcatccaagtatctgcagaactggtctcccactaagccaacaaaagaggtattccatgttcagtgcacctacaagatagcctcatgctctccctgtcaattaactccttttagcattctctaaactcccatatccttctctgaccaagctccccaaatacttccctttttcccctcacaaacctttatctctcccacttgtaccccagagcatctcttctcatgaaggctacactcaaattattgccaacgatcgtggtcatctactgccttctgtgccccgttccaaggtgagatactatcttcactcctatcaagaaagtcaaataattaaggcacagaactgggagatgtgcagtctctcacagccattatcgggaaaattaaagtttaatctaattcatgttgtaatgtgagagcccctgaacttccggccagcttacccagcaggatagagttgtgtttagcacccttcagaagttcttaaattgatcaatgatctgtataaatgaaagccttcaggtgatgacatttgtgcagtgggtactcctttgccacactcggcctaaggatgtggaatttaagttggcagagtaaaggggatgaaaaaattaggcctgcaaagcctaaatgagggagggggataaggaagggtgggaagattatgctttcagtcttgtttcataaccatgcattcctaaaggtaaagaaaggaaataatacagaggtctaagtcagttactgggagtgagaagccctactgaggaatcccttttcatttttaggcaaatccttggggttccttcatgggcacctggcaaatgcctctgaagataccccctgctcgggtgaccctgacctcccgtacaactgctggtgctgcctccctcaccaaatggatacagaaaaatcctgatttactcaaggcctccaatgggctgtgtcctgaaatcttaggcaaggtatctattcttcccatctaacccaaaaccctgtagtctcaatttcttttcaacctcaaaaaatgtctattgttatgccaccactatcccagcatgggggacctctaaccaatttgtcttatcttgactagtccttaatcaccttctgaggcctgaagggatgggctaaggacatcatacccccaacagtagaaaatgatctaatctcaaggtgggggagggtggttagagaaatcaaatttaacttttcttatttgaaacttgatctactgcccatggtatggggagaaagggagttagaatcctgaggtgcattaggaatgatccgggcctgaccagagacatgactatctctcccactcttatcactgacagccccatgatccagacagtcagaagaaactcagaaagaagtctatcacaaagactgtacaacaagcacgaagtccaaccataattccaagctccccagctgccaacctcaattccccagatgaactccaaagctcacacccctctgcaggtcatactccaggtccccaaagaccagccaaatcctaagagcccacctggaagtccacgtatgctagaactctgggcagggcctaatctagctgaggtccagaaatacaaacctggaacttcatatggaccaagtggccacacactgaaaaacccgtatagcgactcagtgaaataaacaagagcccccagtcagaactgtgaaacagggaaattttggggtgggagtaaaagcaaatttggaaaataaacttttttttgttgaatcttttactgatctggattttccattcttgctatggctgcctcttgtaacacaattaggagaaggaaggtaggagaaaataaagtagggaaaagaacatacagtggtttgggtggaacacatttttacaagaattgagtcagttatactccagaaatgaccaagagaaagttggtctgaatcatggaaaaagggcagaacctcaaagaaccagtccctcaaccctacccactcattttttatcctgagcatggacaactaacaactacaaaatcagaaatagaattgagtagagtatgtatatgtgtgtttggagaaggtggggaagaaaaggtagggaaaaccaaagtagaagatactatgcttgtgtaagactttctatctaagcccaagtacaaatatagtttgaaaattgaagatattaaagtgattggaagacagagaagaaaaagacagtaagtagaaatttaaggcagaataacaaacatgatgctctgtcacaccccccacccacccactaccatgcttcaatcacccaaatggtacgaaaccaccaaaaaattcaactgccctacccattttccagcctctaacagctgtttatcattgaccccattttatattttcctggcactggctgttaaatttaatgcccttgccaaacctttcccagtcccaatgacaaagtgttctgtcatgatcacttgtccctcattccaaggacaaagtagagaacagctggtttaaaatggaggaaaggtacaaggacttcccagggcccctctagtaaaaagggaaaaccaatcattacttaaagccaaatactatttgggaccctgaatgaagactgttaaaacagcgggtccccaccttaactaaggtcttcctatccaattgacaccagccagttaacatttcccctcttcgacccacagctttaactggctggccaacaactcgaagtgacagatgagataagtctcttattccagagttcccaaaaactatcaaaacagcatgcctgctaaagcctggcctatatggattttaaaagcagcaagttttctcattaaattatacatttttgccaggttttcaacaatcccttcttttttaaaaaaaaactctatgcttcattcaccccaagcctataacctcaggtcatcatcccctagctgtcaccaacactggtcctctgtgcccctcaatgaatcataatttgctgaactgtaccatgaagcttataatcagtccttaatgggattttggtgcctataacccaaaagcactctacatgcgtcacttcttttctttttctccttccttctctgaggcttttctgtgatatttaaatctctggctaagttctatctgattccctgaaaacttttccaatgatgagatgtaggagaactgtttccctcctggtaaaggtcagattgcggggagagggaggatgtaaatgcctgagacccgagggaagaggaggaaattggttccttcccaacagccattttcttggtttctctagatttcaaggagagtcaaagataaaatgagtatttaattcagtttcagaaaaaaagggtacattacttcgatgagaaagcataaaattaagaggcttttctggaaatccaagaaaaagaaataaccattaatatgttcaatgataattttctagatcttcctcgtgtccaaagctatatattttctcctcaaaagcagctgctccaagaactaactagccctctttatctccctctagctgggacagactaattcccctccacccccacctctcttctttcaataacactgtgtaggtgttaatggcctgggctctcaccaatgaagagaattgtcctttaagccagcaacccacaggcagtggcacccaaagcctcaccaacccaccccccaacccggcccatccccagggcagaagccacagagctggcattgtttccactgtctcaggaagaaggagccaaaagctgaccctcagcacaaatcaaagcccaatatggagagagaataactgcttctaggccgagagtaggcaagctgtgggcaaaaaaggggagtttttgcagccacctcatctttagaaacaaggggaaaactagacccttttccactattatggtctaccaggtactctactgctccaaggagatctgaaaatacaaaaggatctaaacaaataaggagaacttttcccaggctggagataagaatgacaaacagaaagatgggtgaatgtaataatgtgtaggaagatgatgctgggagcctcctttcttcacatggctgccagccccatagaggacaacacagtaagaaccaggacaaccactccagactggtatagctggggaatcttcaggccttttcctaggtcccacatctgcactcaaagcaataccagtgccacggtggcagatggacatcgccatgggaagagaccaatttctgatacagagctgagggctaaagtgggctcggaggcaatgacgaccaacgtgtctcagcaacagcgcagccatcttgggttccggtctggacggaagt

SEQ ID NO: 17306 - RNA, 4911 nt, Homo sapiens
  source 1..4911: mol_type = other RNA
tcaggccaggcacagtggctcacgcctgtaatccagcactttggaaggccgaggtggggggatcacgaggtcaggagttcaagaccagcctggccaacatggtgaaacctcatctctactaaaaatacaaaaactagctgggcatggtggcgggcacctgtaaccccagctacttggagggctgaaggagaattgcttgaatccgggaggcagaggttgcagtgagctgagatggcgccattgcactccagcctggccaacaagagtgaaactccgtctcaaaaacaaacaagcaaacaaacaaaaaatgcttaattttttttttcaatcttgaatgattacatatttaaaagggccatggaattcagggacttagttttatagctgactcagcacttttggtggcatttaaccttcaaacacatcatgtgaaaatggggggctacctgaggaaagagtgccacctactgattataaacataactgtccgtggctacttcttccttgaagttttcatttcaaagtgtcaaaattagtctaatttgtgtgacagctttgagactgtcagattctaaggagattaaggaaggaagaggtggtggtcagaataacctatgttaatcaaaataaactccttagcattagttaaggttctttacctcaatctctcaaaattaatgttattctgaactaaaacttaaaaaaaaaaaaaactaaatctctcagttctacttgtcttattacacatatactcatcttcttttccagaaaaaaataatattcatgtcctaaacttagaaacctaacctgaagttttgatctggatttttaggaagaaggaagtattgatggtttcatcattcttagctctataaaagaacctattaatttttcataacttttagcttagtattatagttggccttttctctgtaagggacattcttaaatattcaagtctaattttctttaaaaagttcgcttgctttctttcttccaggaggatctacctctgaacttcattccaaaaaaaaaaaaaaaaacctaaatacaaattgcataataaatttctctttagattgatattagagtttaaattagtaaggtaccaactatacaaaaggacagagaatccttgctaaaataaagtagattttgtataaggcttccatctatccaaaaaggtttaatatttaaaaatgccagaagaacaatggtactacaccacttccagaagaattagacacactggatgttaaatgaacttcttttaaacctgtaactaacaataagttcaatgatgcagtaaagagttaatttctgttactacattcattctatatattgctattgtatttccttaattttaatttgataggtatacatgtaacactataatttcaaattccaaatcagccggttgtagatattcctattgcagaatttctaactatgagttcatgcaaactaaacatctagtaatgctcaaattgtaaaatttactttttcgtaagtttaagattacctttttttgtatattaaaccttcctttaagaaacaaatctgtttcaacttgtcaaacatgagtatatcagaaatattataattctgctaaaatgacataaaacctcaatttaaagcacagagtgttattttatactgtaatatttttaatgttaaaatgctttttgttaaaaccaacatggattattgaccaattatcttgaccaacagtacttttcaaaataaacaggaaaaactcaaaacagagacacacagatctttaaaagacaatcatgattttaaaaaaatcatggatcatggtataaacagagcacacaaaaggaaaataagaaatgaaaaaaaaactgttgaaattcaaataagttttatacttcagttagtagtattgttctgggctaatatcttactttagataaatgttctacagttatgtaaaacgttaacatgagaggacctgagtaaagggtatgcaaaagaactcttcttggcagggcgcggtggctcacacctgtaatcccggcactttgggaggccgaggcaggcagatcacgaggtcaggagatcgagaccatcctggccaacatggtgaaaccctgtctctactaaaaatactaaaattttgtatttttacaatacagctgggactacaggcgtggtggcgtgcacctgtagtcccagctactcgggaggctgaggcaggagaagcacttgaacccaggaggcagaggctacagtgagccaggattgcgccactgcactccagccttggcgacagagacagactctgtctcaaaaaacaaaaacaacaacaaaaaaactctcttgtacatttctgactcttctataaatctaaaagatctttttaaattataggaaaaaactaacagcttcaaaataaacatgacttcagctgccaaaatttcttgatataattcaagacttcattttttaaaacataattagaaatcaacattatgtttacttaacattatagtcattttattgctctagaaagtttagtttctaaaaccattggattacttacatagtgacaataagactagccacatacacaaaatcaactgtatgaggctgcttctccagcttagtggacaaatattacaaaaatacaaaaatagctgattatagttaagctatcaagtataatttttcatgtatttatcctaagaatatcccctttttatagataaggagatgaacaaaaataaaactaatgttactgataaattactaatgaatgtatttgagaaatccaaattacatgcagacagaaactggtcacaaaaaccattacatttctctatactaaaactgtacaatgttttaaacatttccaatcatgcaacggtaatgaagatcagcatgaattttataagagttgatgggagttcaatgaacaggatttaacacattttacaacccaaatcaaagttgaataatacatccaattcccctaaatttatctatgcgttgagactgaaatgcacattattcccccacaactcctccccctaccccattcccaatcaattaccttacctataaaaccttccatttaaccttttaagtcagatttgatgggtaaacatgtaatctacagtatactctccattattatttcaggatagacacacatatagtcagatgctgaatcttcattacattcctttcaaaaggcatctaaactgttgcaattgtctatgaaaattcaagcctaagaaaccaagaaaactggcagtcaagattctgaactaggtagttctacaaactataatacgaataatctatatgtccacattagtaaaagaaggatttcctgtttgagaaatgtttctcaatggctctttgaagggaaagctgtgtcactactgctttctgctttcaatggctaggtgaccccaaatatttatccaactggctaagaggcttacagttgagccttttaaaaaatactcaaggccacagaagtacttacggaaataaaattttagaagatcatagtttaagatacatagaattcttcttataatggtacattcaaaacacatctgtcctaacaaagcagcataaaaccaattaaaaaaacaatttgaaattaaatacactgagaagtgttaaaatcattaaccaaaattactgaatggtagaatactgtctcaaaatgtactgaattcacatatgtgtatcaccataatgaattcatgccagatataaactcaggttaccaattaggttgaaacaaattttagagctattttttttacatgagaaattaatgtacttcatgatataggcacaacagcatctttttaaaaaaactggtatatttatcactagatacagacttctttaaccattagcaacacagcgcagtaaaattttctcaaaactttttaagcttgatttaacatgccaagaaaatgattatttttccaccgagatgcatttatgtaaattatgtaaattggattgaggtcagtgtaacacctggaatttacaacccctagcagaagtaccagctgctaataatgcttatactatatttgtagcttaactagatgttaaactatggaactgttggtgccaatctgcttataaaggcaatgctctggagacaaagtcttctcacaaacagtgggcaagcaggtttcattattatgtgttcaacaacaatcctcagttcattaaataaggtccgacaatatgggtttcttcgagacgaatatcgaagggtaagaaatctatagtatataaaaggttggagcaaacttccttgaccactaaaaagcataaaaactgtcgcaggcatcaggaatatttcattgcaagcaatgaatttcagaatattttgttgattagcacttaatttgtccaagacagatctcagcagaggtaaactatttgagccccttgcgtcaaggacctttttcgtatatgtggcagcatgaagcaaagagaataacaagactgggaagatactcattgtaactggataggaatttacaaagatgagtgaatacaacaggtagtggcagctgtcctctaacaaagcctgggccaggaatgctctgcttaactggaagtgtggtaatctttgatgcagcctcagagcactggtaagagcatttgccagcaaagcacgttggtaaaagcttgctgcttcatgcaacccaagaagaggcagaacaaacagagcagagcagtaaactgtgaacaagcgagaaagccacattgccgtgtccagtttattggtcatcatgaattgcacagcgcccgccccttgggggccgttcggggtcgtatctgccatgggggctcacactagcgtctgcgacgccgcaaccgcgaagagagaagaaaggggag

SEQ ID NO: 17307 - RNA, 4332 nt, Homo sapiens
  source 1..4332: mol_type = other RNA
tcaggccaggcacagtggctcacgcctgtaatcccaacactttgggaggccgaggccgggggatcacgaggtcaggagatggagaccatcctggctaacacggtgaaaccccatctctactaaaagtacaaaaaattagccgggcgtggtggtgggcgcctgtagtcccaggtactggggaggctgaggcagaagcatggcgtgaaccgggaggcggagcttgcagtgagccgagattgcaccactgcactccagcctgggtgacagagcaagacttcgtctaaaaaaaaaaacaaaaaaaaacaaaaaaaccataaacaatataggagtgtcataggattataaatagatggcatggataataaaatctacaagtttagagaaaattcgtaattataggtgagaagtattaatgaaaggacaaagcttgttcttaaaggatcagaataggccaagatgaaaaaaggcatccatgggaaaagaactgttcatttctataattttaacaaaatagataatctatgttgaataaaatccataaatactatttccaaatttgattaaggtatttactttgaaaacctgaaacaggaacatatttacagtgttaagtgatttgataattttgtagttctgccctaaaaatcaatatccttaattaacccttcatcagtttcttaagtcatctgtcatcctgaaagcaagttaattattctaaatgttaaataattttggtagtgtctaatctataaaacatacatacactaccagttttttttctacctttaacaaattcgttcccataaaagacaattttatcactaacaaaggataactggcaggcataaaatagtgagtagaaaatgattttctaaaatttttcatttctatcattttatagcaagttgcatttatcttaaagataaatattcttcaataaaaataacaattcaaatttttcagttgtagaaattcctggtgatgacatttgatacaaatagtttatccctgaaatccatttaaaatttttaatcaaatcttctgcaattcattgatcaagaatacatacgagactatccagggatatttctagcaaagaaaactgagtcatgcaactcagttcttgaagcaaggaggcaatttaaagtcagaataaaggtttactgggctatcctcaatggacaagtggaggatgtaagtcacctgatttggaacataaaagacttaaaaatgtaagagcaaaacaaatggatggtattgggaaaaataattattaagaaaaaaaaacccaagacaatgaaatgaagaaaacactaatattagattaacagattctatgtaagatctcaacttggatacttaaatttatgcaagcaaaataccatttgatttaatagagaaatactgtgatatgaattgaaacaatttctttgattctataacctggaaaaaaaatggtataaactatatacaagttaaaaccctcaaaggcagtgttgttttcattcactgccatgcatgagatgtctagcataaagctaattagcgcctaataagtcctcaataagggaagaaactaaaaaaacttaaaaattttaaattaaatgacacaataatgccaagactttccaaagcagattgactgtagcagctgcagttacctggacatgcaaaattactagtttaccagtaacatttaagaaagcagacaagaagataattgtgcttctattagcgaattgaaataatggtattttgaaactgagtgaaaaacacattctgagtcatctgtattaacttaaagctgttctgaagattaatgggaaaaataataatgaatagacgattggatttactaaacaatgtttgattaattgtattaatggttataaaatacctatcaaggctgtcttttcttgtccaaaaattcaatacatgaaatatgaaaatttgtaataccatagccaaagccttattgcatagcttctagcttactgatatatttacttattttaatttaaaaagcctgtttttccagccactaggaaataagatttctcacgttttatagtactcaaaaatcatgattaagtatatctaatgctaacctaagtgtaagcaaacagcaaactaaatggtgaattaaaatatccacaccaagcctgacctcagctttcattgaaccttttcttcagaagaaaactaaaaataaatttcactagcatttgctttgcttgacagcataattgagtagcaaccaaagtagccacatgtggtcctttatgtaaggccttctagcctcagaaacacacaccttttgaattagcgtgcctggtacccatttgtgcccaataaatacttgctgaatgaacttttccaatagtgctggatttgctctgagccaaccaaattctcacttttaatgtattttgaaagacagaggacgacaagatgaagaatgcagtttgagactcagaagagcaaacataatcggcccagtatggatatgatcatttgatgcactgtcctcgggcatgctcatttacagaagcctaaaaacaaattttatccctcatttgtgggtttctggtgttgtggagggctttccaatgtttagaagcaatatatttttatagaattctgtaataaacgtgttttaaatcttttataaagctctctgtagcatataagtacatattaaagacagaaatgggggagcatcaaggcccttataatcgcattcattccttaaccacatactacgcatctactgtgtggcattctaggcgggggccgtaacaccagtgcagaaaaacacaacctcttgtcctcttagagcttacattgcactggggaaggagagataagaagataaacaagtatggatatgtagactgtccaaaggataaaatgagaagggggctagggaactttcagtttaaaagtagccgcggaagcaccgagtgacacgagcaaaatcctgaaggtgaaggagcaagccctgtggacgacgctcagggaagagtcctactcgcaaggatgccagggcaggcccgcccccaccctcaacggcgcgcggggacttctgccgcagtcaaggctttggctcactcccctcaagacgggaagccattcgcagggcctagagaaaaggagtgacaggatcttggccccctgagtggcctgaggcaaaaggaataatctaagcaagttttcctacttacttttagcgcactggtacacacacaaatacacaatacaattcatataacacgaatttcgtcccggttgagtaaaattccgcttacctactgcactttttaccgaaaatagcccctttttaatttacacaaacttaatagagaacggtggaacaatggttacttcttgttttacaatttaaaaactacaacaaccatagtactgtacgtataatcacatattgtattccagccttgtccagcgcctcagttttccgaacctaaagaggaaaacgatgtttgaaatcagctggccgcaggcccgcgggtcgcccgcagtcaccggtggctgagtcggggccggcggttctccccgcgcgctcggctccacccacacctagaggggggcgcccgggcagccgcgggcgagcttctcgctcgcgcagcgtcgcctacaggcctttatcctgaccgttagagaagaacccaaacctctgccgacaaaaagcaaaagcagcggagaccgcgtatttccagaaataaacgcatcatcacaaacacgattccaattcaatccagccgacagtcgtcttcacctccaaaggttgcgttcttattcgcagaaataacacgcagtcgggcgtaaggtcccggctctcaaaaggcaaggtgtacgatccatccatccacccggctgcagggacaccatttaaaacgggcatcatcgccatcgaatcgcgggcgtcctctgtggggccgcccggagatcggctccctaaagctaacgacgacctgggacagccagcgcggcctccagccgccgccgtcggcgacctgagagcccgtccgggcctgagtgccccccacgctcacgaccaccaccgaactcgggccccgctcctgtcggcctccaggaaaataaagacagaggagagccggcccgcctgtgtcgcagggcaaacgtcgctctgaagcatcgacaatactggcaacatccacagccgccctgaggggacgggcgtagaggagagctgccgcctcccggctgctgggcccgggtgccgcgcggcgcggccgaggacgcgagcccaagtggcggcagcggcggctgcggcggtggcggaagtggagt

SEQ ID NO: 17308 - RNA, 3963 nt, Homo sapiens
  source 1..3963: mol_type = other RNA
tcaggccaggcacagtggctcacgcctgtaatcccagaactttggaaggtcaaggcggatggatcgcttgaggccaggagttccagaccagtctggccaacatggtgaaaccccgactctactaaaaatacaaaaattagccaggcctggtggcgcacacttgtaatcccagcacttggaaggctgaggcagaatgcttgaacgtgggaggcagaggttgcagtcagcccagatcacgccactgcactccagcctgggcgacagagctagactctgtctttaaaaaaaaaaaaaaaaaaaatagctgggcgtcatggggcacacctgtagtctcagctactggggaggctgaggcatgagaattacttgaaccctggaggcagaggttgcagtaggcccagattgtgccaacgcactccagcctgggcgacagaacgagaccctgtctcaaaaaaaaaaaaaaaaaaagccgggcacagtggtacacacctgtaatcccagcactttgggaggctgaggtgggtggatcgcccctgaggtcagcagttggagaccagcctgaccaacatggtgaaaccccatctctactaaaaatacaaaattagccgggcgtggtggcgtgcgcctgtagtcccagctactcgggagactaaagcaggagaattgcttgaacccgggaggcggaggctgcagtgagccaagattgtgccactgcactccagcctgggtgacacaatgacactccgtctcaaaaaaaaaaaaagaaaagaaaagaaaaagcagctcagctagcaggagagagccagcaccggagcctccacgcctggactttactctctggccccagtgggatcacctcctccaagaagtggcccctggtcctgctgaaggccccactctaagatgcagcgctctccacgctgtgtaagtccctggctaaggctccctgaccacccctgtacttgccggctcagcccaccaggtggcgcccgcgccatgcctcggccctgctggactccgaagccgccacttccctgcgggcgcctcctggtgtttgttcccttgggctcggcctggacagccctgctggttcccggagcctagcccagccccgcgagtgattcacagaactcacacctgacggtgggggaggaaggggagagcagcagccaagaggtgggtccaggctctcccaggggcgagtgacttcagtccagatgtcccctgaacccctggggattccgcatcaggaccagggcctcccatgtccagaccccacattcccgtcagtgtgtcccggggagcacggagggacctccacactgcatttcatggggcgaccgcccttaacacccggacacacacggaaccccacactaccctaaagtctgaaaggtggacacgcgtggcgaagttttagaggaatttcaggacaaaagtcctgaaaccacaaggttcttaccacctgaaaaccagctccgtaacagacaaactagacacttgtgagtttgccggcatttgctttaaaaataacaaggctggtccaagatcttagaagaaaattatattcttttaaagaaaatgaaaatatcctcaagggaaaaacttaatttaagtcaaatcttgtccttttgtcgtggagccccttgccccgcgcgcagacacaggctttcctgaagcgtggccagggcgcccctctcatcgctcctgagcgtgacccggggctggagccgcacggggattttcccgagctgagcaggggggtcggggggcccaagccaggagccctggaagagggagcagggcggcaactggggccgcaaacacccatcaaagtccccaggaccaattcccacagacaccacgtggccacaggcagtgccctttgcaggccccctccccaagggtgtcacccctcaccccctcctgggaccccgcctaaaccaggcacccttccacccaccagcaggaactgcgctaggagatgcaggaacacccatgtccccgccagccccgccttccagaccacaccctgcccgggagtgcgctttgcgaggtcggggtcgggggggagggcgggggccaggcccctgaacaacagacagcagctcccacccagcaatgcagccgggtcacctcgcacccctggccaaggcaggggccctctccagcctggtgacccacggcctaccctgaggctgcagggcacagggggcctccaagtggaaagctggtgatggggtgggtgggaggcagggcccgcagggaagtgacttgagcaggcacagacggtgaataaatagaagcttccacgcgggggtccggcccctgcagacagcagctcggtgggaaactgattggagggagctcccctgacgctgaccagggccacccacgcgggccctccctccacacccacacccaccccggcccagggacgggttttcccctgctcagagctcagtgacgtgcacagtgggtgagggaagaggcccaggttggaggcgccgcaggtggcaacgacgacacagtaggtggcccgccaggggatagcaacggcgtccctcctccccgctcagctgcagcccgcagtcctcacagtggtaacatgccacgtggtagtctctgtccatggacaccacacggatggttgtctcgcagccctgtgcagggaggataggacgggcacaggaggcgcattttggtgcaaaaaccgtgtgatagtctcgcacgcagtagatgttgttctccacgtccacggtgaagggaaccccgtccaggcactcattgcacacggagcaccggaagcagcctgggtggtaggacttgcccagggcctgcaggatcatttccatgatgagatgtccacacacgctgcatttgtcggccgtctgctggaacccggagtacaggaagtcctcctggcagtacactttctcacccacgttgtagaacgccttcccacggagtcgtctcccacacgagtcgcaggtgaagcagtcagtgtgataaagactccccattgcctggcacgcctgctgggctccgtagatgccaagcccacacttgatgcaaatgccgaagtagtcccgcgccgtgcgcgcctcgagcgcccgctccagctcccgggtgagcgcctccagccgccgctcggccgcgcttgggccgccctcccggccagggggcagcgggagtgcaggcagcgggaagggagccggccccgcaggctccggggagcgagcgggcgcggggcaggcgccgggcgggaggaagtcagcgtaggcgccggccgagccccgggagccgaggctggaaacgctggagcgggcgctgcccaccgaaggcggcccgggaccgggacgcgggtccgagcgaccggagcgcgggctgccgtggcgctggtcgtagcccaggctgatgccgctggatcgggcgctgccgccaccgccgccgccgtcggaccccgccaggctggcccgtgggctgcccgcaggctgcgcgctgagctccggaaccgccgcgcgccggggaccccgctccccgcggctcagtccgtccgccccggcctcggggccgccgctgcccttccctctgcggcccagcgcgggcgccgcctcgtctccaggcccaggccgcggcccccgccgcccccgaccgggagagccgcacccgggctccagctcccgcagggccagcccggccaggagtagggccgcctcgtccgcgcccgccctggagcgctgcatggcccggcccgccggccctggcgcgtcacctccgcctccgcttcccgccgccgctccggccgggccgccgcatcgtccgcccgaagcccggagcccgccccgggacccctgggcgcggggcggggcggggccggcgccgggccggggtcgttccggcggccacgcgcgggccgggggacgcggcgccctgctcggcggcgcgcgcggcggaggaatg

SEQ ID NO: 17309 - RNA, 4009 nt, Homo sapiens
  source 1..4009: mol_type = other RNA
tcaggccaggcacagtggctcacgcctgtaatcccagcactctggaaggccaaggcaggtggatcacctgaggtcaggagtttgaggccagcctggccaacatggtgaaactccgtctctactaaaaatacaaaaattagccgggcatggtggcgcgtgtctgtagtgccagctacttgggaggctgaggcaggagaatcacctgaacccaggagctggaggttgcagttagccaagatcgtgctactgcactccagctggggtgacaagagcgaaactccgtctcaaaaaaaaaaaaaaaaaaaaaaagaagaggatgggaagaagagtgatgcaaggggggtcaaccagggaaaaagagaggacccatggcaggggagcaagaaggagtccaatgccagtgtaggtatctgtgtttccatcttcatcactgtcttaggttccagtttaacatcagtttccttacttcctgcctctgtccatggtctgtcaggatccttcaaccccctccaccctgcccttgctccttctgtgacagtccctttcccctcctccatttattgggagctggctcgctccaggatcctcaggtcatagttctttttggccattcgaagtttgaagcgactcacggagttgttgagacgaagggaggcattttgggcagccagggggctggggaacacagccacaatggtgtacaaggcagcgaggtccgagtggcggccattctcagcagtcccactgttgtcccccccaccccctccaggcagcccctgagcatccttgagccactggatcttggcgccagacatggcgagctgcgtgaagagtttgtccgcctcagtacgggtgatgccctcagggagatctgtcacctccagcacccgccccaggacaacatctgctgtccccaggtcagtggaggcagatttgagtgcttgtctcttgccccggtttccatgcttcagtccactctgtccctggtgcaccgtgtaagttgactggccatggagcaagggagggcagatggacagattgtactgtaatggctggcccaaaagggagtagcgcccatcaccctgtgctggacccccaggccgggggaactgtgtgaggacaggcaggggactgagtcctgtgcagacactgctgaggctggtgacaggagagggtgctggagactgggtaggagatgtgacagggctgctgctcatttgtgtgttggcctgggggctgctgtcaggactgtacaggtctccaggcttctgcccccgctggtccatgctgtagtatttacaatgactccactggaccatggatgggttctgagggggctggggtccattagggacattcagctgcatgaccactacacctggtccagaaggtgacactcctgagtactgctgtggcatctgtggtggactgcagggagagggagactgaggcatctggtactgctcagagccagggggttgcagaaaccctacagaagggctcgtaccgttctgctgagcaggtgggatcatgctatagtacactggtacccccgctgctgggaggcctccttgcacagactggctcacagggaccagcatgggttgctggaaaggcggctggaccacattttgcgagtcactacccactggaacttggtaagaaggcagtggagtgtactgaaccaccaggccttgcatctggccccccatgctgctcctctggctgctgagcaggccctggttctgtggctgctggaccccaatcatgccttggtaagccgcctgctgctggttaggcatcatgggctgtaaaccaggctgctgggatggctgaggcagctgctgaccacgttgggggctataggccaccgggtgagagagaggtcgatattgctggttggagttaggatattgtccagggggatagtaagaaacctggatctgttgagggggctgcatgtacccctggggtggcagaacttgctgagtaggtggtgcatggctagaggtggaatagttggaagtggggaggggctgacccgtggaagccatgatgaagctagtctgctgagggtgctgggagataagtggggtctggaatagagctgcagatgggtcagctgcttcagtagaaccttggcgactaaggctcatttgtccaaaggggttgctgaggtcatctgccatgttgtactgctggggcggagagactggcagaaggacttggggacaggagcttggagagaactgaacaggctgcggagagggctgcagagccgggactggctgtgagatcatgtgattattcaagggtggctgttgctgaggcgtgggtgggagagcaggaagttgctgctgctgctgctgctgttgctgctgggcagtacaagggagaagcccccggacagactgggatgaggtgacctggttgcacacttctggggcacctagtgccatacctggcctggagatccttcccgcactgccgcctttactgctgccgatgctgtcacctcgggtaaggatagagattccactgaagctgctagctttggtgacagggggtcgcatgctccggacagagccatcagagtctgtgctgctccaagggcgtggctccagggatttgagttcgctgtctgtgctgctctggcggctgcttgaggtgcggctcagtccttcacggttccccctaaaaatctgccttctcttgtgagagctagaagaaaaggcttctttggagagtctgatgtcatttagatatccgttctggccagtctctcgggcaaatattctctctcggaccctttgatattcctcctctctctcttctattgacttgctcctccttccatcctgcaatggaactctgatctggttatcatctcggtccatactggcatcatctctcttgagaatgaacctctgttgaaattctgtattcttctcatcctttatatgttctgagaacctctgttcagggattcttgtgttactagttttgttgatgatgacagctttcccagtttgatcaacattgtggtccatcccaaaataggcagctacccggtgtaatagcatccggtgatatgaggtcatctgagggaacttcttgaactgattattgttgtcattaataaattccagaatctcctgttctaattttagcagcatcattctgtcccttgggttctttttcagtgtatttacaagaaattcatgtaggtctattccagtggagtccgtatattcctggctggagtctctggacagcatcttccttgggatcttttctttgtttttgtccttgtcttccttttcagagacatcttttgtggacttttcttcctccttgtcagaagggcaactgatgtgcaattgaattatatcctgggtttctaatggcccatcagcaaatggggtggaggactcctcacacactgccaggctacgcaccaactttagcttggaattagacttggctcttttcctggcatgaccatggttagatgtccgcctctgtgtctcctgacgcaaactggtatcttcacattctttctcaatttcttccttacttggagtcttagatataaacttgtttttgtttacagattcttccaccagttttttttctgattctttcattatttccagggtctcttgagtagtgttactgttagacatgttcttcaatagaatacagtggcctctatggactccccagatggatctgtacttacaccaacagcgagctcacattattaatggagacttcattgtaaagatctgttctgccggaattttgccggaagaaattccttctgggaaacctgtgcctcttcccccacccacagccctctcccgcccccttcacccttgaatgaaatgatactgatccttgctgctggagctccagctaactaactgctctgacaagcagctctgaagccgaccatggcccagctgttcagagagatatcatccagagctctgccaacagtcacact

SEQ ID NO: 17310 - RNA, 4110 nt, Homo sapiens
  source 1..4110: mol_type = other RNA
tcaggccaggcacagtggctcacgcctgtaatcccagcactctggaaggccaaggcaggtggatcacctgaggtcaggagtttgaggccagcctggccaacatggtgaaactccgtctctactaaaaatacaaaaattagccgggcatggtggcgcgtgtctgtagtgccagctacttgggaggctgaggcaggagaatcacctgaacccaggagctggaggttgcagttagccaagatcgtgctactgcactccagctggggtgacaagagcgaaactccgtctcaaaaaaaaaaaaaaaaaaaaaaagaagaggatgggaagaagagtgatgcaaggggggtcaaccagggaaaaagagaggacccatggcaggggagcaagaaggagtccaatgccagtgtaggtatctgtgtttccatcttcatcactgtcttaggttccagtttaacatcagtttccttacttcctgcctctgtccatggtctgtcaggatccttcaaccccctccaccctgcccttgctccttctgtgacagtccctttcccctcctccatttattgggagctggctcgctccaggatcctcaggtcatagttctttttggccattcgaagtttgaagcgactcacggagttgttgagacgaagggaggcattttgggcagccagggggctggggaacacagccacaatggtgtacaaggcagcgaggtccgagtggcggccattctcagcagtcccactgttgtcccccccaccccctccaggcagcccctgagcatccttgagccactggatcttggcgccagacatggcgagctgcgtgaagagtttgtccgcctcagtacgggtgatgccctcagggagatctgtcacctccagcacccgccccaggacaacatctgctgtccccaggtcagtggaggcagatttgagtgcttgtctcttgccccggtttccatgcttcagtccactctgtccctggtgcaccgtgtaagttgactggccatggagcaagggagggcagatggacagattgtactgtaatggctggcccaaaagggagtagcgcccatcaccctgtgctggacccccaggccgggggaactgtgtgaggacaggcaggggactgagtcctgtgcagacactgctgaggctggtgacaggagagggtgctggagactgggtaggagatgtgacagggctgctgctcatttgtgtgttggcctgggggctgctgtcaggactgtacaggtctccaggcttctgcccccgctggtccatgctgtagtatttacaatgactccactggaccatggatgggttctgagggggctggggtccattagggacattcagctgcatgaccactacacctggtccagaaggtgacactcctgagtactgctgtggcatctgtggtggactgcagggagagggagactgaggcatctggtactgctcagagccagggggttgcagaaaccctacagaagggctcgtaccgttctgctgagcaggtgggatcatgctatagtacactggtacccccgctgctgggaggcctccttgcacagactggctcacagggaccagcatgggttgctggaaaggcggctggaccacattttgcgagtcactacccactggaacttggtaagaaggcagtggagtgtactgaaccaccaggccttgcatctggccccccatgctgctcctctggctgctgagcaggccctggttctgtggctgctggaccccaatcatgccttggtaagccgcctgctgctggttaggcatcatgggctgtaaaccaggctgctgggatggctgaggcagctgctgaccacgttgggggctataggccaccgggtgagagagaggtcgatattgctggttggagttaggatattgtccagggggatagtaagaaacctggatctgttgagggggctgcatgtacccctggggtggcagaacttgctgagtaggtggtgcatggctagaggtggaatagttggaagtggggaggggctgacccgtggaagccatgatgaagctagtctgctgagggtgctgggagataagtggggtctggaatagagctgcagatgggtcagctgcttcagtagaaccttggcgactaaggctcatttgtccaaaggggttgctgaggtcatctgccatgttgtactgctggggcggagagactggcagaaggacttggggacaggagcttggagagaactgaacaggctgcggagagggctgcagagccgggactggctgtgagatcatgtgattattcaagggtggctgttgctgaggcgtgggtgggagagcaggaagttgctgctgctgctgctgctgttgctgctgggcagtacaagggagaagcccccggacagactgggatgaggtgacctggttgcacacttctggggcacctagtgccatacctggcctggagatccttcccgcactgccgcctttactgctgccgatgctgtcacctcgggtaaggatagagattccactgaagctgctagctttggtgacagggggtcgcatgctccggacagagccatcagagtctgtgctgctccaagggcgtggctccagggatttgagttcgctgtctgtgctgctctggcggctgcttgaggtgcggctcagtccttcacggttccccctaaaaatctgccttctcttgtgagagctagaagaaaaggcttctttggagagtctgatgtcatttagatatccgttctggccagtctctcgggcaaatattctctctcggaccctttgatattcctcctctctctcttctattgacttgctcctccttccatcctgcaatggaactctgatctggttatcatctcggtccatactggcatcatctctcttgagaatgaacctctgttgaaattctgtattcttctcatcctttatatgttctgagaacctctgttcagggattcttgtgttactagttttgttgatgatgacagctttcccagtttgatcaacattgtggtccatcccaaaataggcagctacccggtgtaatagcatccggtgatatgaggtcatctgagggaacttcttgaactgattattgttgtcattaataaattccagaatctcctgttctaattttagcagcatcattctgtcccttgggttctttttcagtgtatttacaagaaattcatgtaggtctattccagtggagtccgtatattcctggctggagtctctggacagcatcttccttgggatcttttctttgtttttgtccttgtcttccttttcagagacatcttttgtggacttttcttcctccttgtcagaagggcaactgatgtgcaattgaattatatcctgggtttctaatggcccatcagcaaatggggtggaggactcctcacacactgccaggctacgcaccaactttagcttggaattagacttggctcttttcctggcatgaccatggttagatgtccgcctctgtgtctcctgacgcaaactggtatcttcacattctttctcaatttcttccttacttggagtcttagatataaacttgtttttgtttacagattcttccaccagttttttttctgattctttcattatttccagggtctcttgagtagtgttactgttagacatgttcttcaatagaatacagtggcctctatggactccgcttcagatggatttttcttcttccttctctccgtcccctccctctcagaagaaaaagactgcaaacaaaatcactacgtcactggaggtagagggaatcccatctctgcactctttagaagccaaggccagcaaataaaaacaagccaattataagaaaaagtaatacaaaataagaataaataaacccagaagaaatccatgtgacaatctcaacacatcaaaaggcattttttagtaaaaaggttttaacaaatgcctcctaggatgttcataatcaaaaaatctccccagacatagcaaaggcttatcacatttaaagactaggggatagttacgtaaagatataggacagacaggcacattcaccagccaggtgcggatagct

SEQ ID NO: 17311 - RNA, 4115 nt, Homo sapiens
  source 1..4115: mol_type = other RNA
tcaggccaggcacagtggctcacgcctgtaatcccagcactctggaaggccaaggcaggtggatcacctgaggtcaggagtttgaggccagcctggccaacatggtgaaactccgtctctactaaaaatacaaaaattagccgggcatggtggcgcgtgtctgtagtgccagctacttgggaggctgaggcaggagaatcacctgaacccaggagctggaggttgcagttagccaagatcgtgctactgcactccagctggggtgacaagagcgaaactccgtctcaaaaaaaaaaaaaaaaaaaaaaagaagaggatgggaagaagagtgatgcaaggggggtcaaccagggaaaaagagaggacccatggcaggggagcaagaaggagtccaatgccagtgtaggtatctgtgtttccatcttcatcactgtcttaggttccagtttaacatcagtttccttacttcctgcctctgtccatggtctgtcaggatccttcaaccccctccaccctgcccttgctccttctgtgacagtccctttcccctcctccatttattgggagctggctcgctccaggatcctcaggtcatagttctttttggccattcgaagtttgaagcgactcacggagttgttgagacgaagggaggcattttgggcagccagggggctggggaacacagccacaatggtgtacaaggcagcgaggtccgagtggcggccattctcagcagtcccactgttgtcccccccaccccctccaggcagcccctgagcatccttgagccactggatcttggcgccagacatggcgagctgcgtgaagagtttgtccgcctcagtacgggtgatgccctcagggagatctgtcacctccagcacccgccccaggacaacatctgctgtccccaggtcagtggaggcagatttgagtgcttgtctcttgccccggtttccatgcttcagtccactctgtccctggtgcaccgtgtaagttgactggccatggagcaagggagggcagatggacagattgtactgtaatggctggcccaaaagggagtagcgcccatcaccctgtgctggacccccaggccgggggaactgtgtgaggacaggcaggggactgagtcctgtgcagacactgctgaggctggtgacaggagagggtgctggagactgggtaggagatgtgacagggctgctgctcatttgtgtgttggcctgggggctgctgtcaggactgtacaggtctccaggcttctgcccccgctggtccatgctgtagtatttacaatgactccactggaccatggatgggttctgagggggctggggtccattagggacattcagctgcatgaccactacacctggtccagaaggtgacactcctgagtactgctgtggcatctgtggtggactgcagggagagggagactgaggcatctggtactgctcagagccagggggttgcagaaaccctacagaagggctcgtaccgttctgctgagcaggtgggatcatgctatagtacactggtacccccgctgctgggaggcctccttgcacagactggctcacagggaccagcatgggttgctggaaaggcggctggaccacattttgcgagtcactacccactggaacttggtaagaaggcagtggagtgtactgaaccaccaggccttgcatctggccccccatgctgctcctctggctgctgagcaggccctggttctgtggctgctggaccccaatcatgccttggtaagccgcctgctgctggttaggcatcatgggctgtaaaccaggctgctgggatggctgaggcagctgctgaccacgttgggggctataggccaccgggtgagagagaggtcgatattgctggttggagttaggatattgtccagggggatagtaagaaacctggatctgttgagggggctgcatgtacccctggggtggcagaacttgctgagtaggtggtgcatggctagaggtggaatagttggaagtggggaggggctgacccgtggaagccatgatgaagctagtctgctgagggtgctgggagataagtggggtctggaatagagctgcagatgggtcagctgcttcagtagaaccttggcgactaaggctcatttgtccaaaggggttgctgaggtcatctgccatgttgtactgctggggcggagagactggcagaaggacttggggacaggagcttggagagaactgaacaggctgcggagagggctgcagagccgggactggctgtgagatcatgtgattattcaagggtggctgttgctgaggcgtgggtgggagagcaggaagttgctgctgctgctgctgctgttgctgctgggcagtacaagggagaagcccccggacagactgggatgaggtgacctggttgcacacttctggggcacctagtgccatacctggcctggagatccttcccgcactgccgcctttactgctgccgatgctgtcacctcgggtaaggatagagattccactgaagctgctagctttggtgacagggggtcgcatgctccggacagagccatcagagtctgtgctgctccaagggcgtggctccagggatttgagttcgctgtctgtgctgctctggcggctgcttgaggtgcggctcagtccttcacggttccccctaaaaatctgccttctcttgtgagagctagaagaaaaggcttctttggagagtctgatgtcatttagatatccgttctggccagtctctcgggcaaatattctctctcggaccctttgatattcctcctctctctcttctattgacttgctcctccttccatcctgcaatggaactctgatctggttatcatctcggtccatactggcatcatctctcttgagaatgaacctctgttgaaattctgtattcttctcatcctttatatgttctgagaacctctgttcagggattcttgtgttactagttttgttgatgatgacagctttcccagtttgatcaacattgtggtccatcccaaaataggcagctacccggtgtaatagcatccggtgatatgaggtcatctgagggaacttcttgaactgattattgttgtcattaataaattccagaatctcctgttctaattttagcagcatcattctgtcccttgggttctttttcagtgtatttacaagaaattcatgtaggtctattccagtggagtccgtatattcctggctggagtctctggacagcatcttccttgggatcttttctttgtttttgtccttgtcttccttttcagagacatcttttgtggacttttcttcctccttgtcagaagggcaactgatgtgcaattgaattatatcctgggtttctaatggcccatcagcaaatggggtggaggactcctcacacactgccaggctacgcaccaactttagcttggaattagacttggctcttttcctggcatgaccatggttagatgtccgcctctgtgtctcctgacgcaaactggtatcttcacattctttctcaatttcttccttacttggagtcttagatataaacttgtttttgtttacagattcttccaccagttttttttctgattctttcattatttccagggtctcttgagtagtgttactgttagacatgttcttcaatagaatacagtggcctctatggactcctgaataaatgctcagcctccatgagtccagtgctggaatggcatcacatataagaaacaagtctaacctctcgcacgggccttggcggggagggcgcccacgtctccgcccgccgcccgggcccacggccgctcggctgcggctcggccccgacggccggcggcggcgcgcttctgggggcgggcttttctcggccggggcttccccggggccgagggctgggaagcaggggggactgggacgggggaggggaaaggggcttgggaaggaggggggagaggggaagaaaaggggggaaccaaacccggaaagggagaaaaggggggaggggaaaatcagaaggggaagaaaagcccagagtccgccccccgctgcggctgcgcgctacgtcac

SEQ ID NO: 17312 - RNA, 3815 nt, Homo sapiens
  source 1..3815: mol_type = other RNA
tcaggccaggcacagtggctcacgcctgtaatcccagcactctggaaggccaaggcaggtggatcacctgaggtcaggagtttgaggccagcctggccaacatggtgaaactccgtctctactaaaaatacaaaaattagccgggcatggtggcgcgtgtctgtagtgccagctacttgggaggctgaggcaggagaatcacctgaacccaggagctggaggttgcagttagccaagatcgtgctactgcactccagctggggtgacaagagcgaaactccgtctcaaaaaaaaaaaaaaaaaaaaaaagaagaggatgggaagaagagtgatgcaaggggggtcaaccagggaaaaagagaggacccatggcaggggagcaagaaggagtccaatgccagtgtaggtatctgtgtttccatcttcatcactgtcttaggttccagtttaacatcagtttccttacttcctgcctctgtccatggtctgtcaggatccttcaaccccctccaccctgcccttgctccttctgtgacagtccctttcccctcctccatttattgggagctggctcgctccaggatcctcaggtcatagttctttttggccattcgaagtttgaagcgactcacggagttgttgagacgaagggaggcattttgggcagccagggggctggggaacacagccacaatggtgtacaaggcagcgaggtccgagtggcggccattctcagcagtcccactgttgtcccccccaccccctccaggcagcccctgagcatccttgagccactggatcttggcgccagacatggcgagctgcgtgaagagtttgtccgcctcagtacgggtgatgccctcagggagatctgtcacctccagcacccgccccaggacaacatctgctgtccccaggtcagtggaggcagatttgagtgcttgtctcttgccccggtttccatgcttcagtccactctgtccctggtgcaccgtgtaagttgactggccatggagcaagggagggcagatggacagattgtactgtaatggctggcccaaaagggagtagcgcccatcaccctgtgctggacccccaggccgggggaactgtgtgaggacaggcaggggactgagtcctgtgcagacactgctgaggctggtgacaggagagggtgctggagactgggtaggagatgtgacagggctgctgctcatttgtgtgttggcctgggggctgctgtcaggactgtacaggtctccaggcttctgcccccgctggtccatgctgtagtatttacaatgactccactggaccatggatgggttctgagggggctggggtccattagggacattcagctgcatgaccactacacctggtccagaaggtgacactcctgagtactgctgtggcatctgtggtggactgcagggagagggagactgaggcatctggtactgctcagagccagggggttgcagaaaccctacagaagggctcgtaccgttctgctgagcaggtgggatcatgctatagtacactggtacccccgctgctgggaggcctccttgcacagactggctcacagggaccagcatgggttgctggaaaggcggctggaccacattttgcgagtcactacccactggaacttggtaagaaggcagtggagtgtactgaaccaccaggccttgcatctggccccccatgctgctcctctggctgctgagcaggccctggttctgtggctgctggaccccaatcatgccttggtaagccgcctgctgctggttaggcatcatgggctgtaaaccaggctgctgggatggctgaggcagctgctgaccacgttgggggctataggccaccgggtgagagagaggtcgatattgctggttggagttaggatattgtccagggggatagtaagaaacctggatctgttgagggggctgcatgtacccctggggtggcagaacttgctgagtaggtggtgcatggctagaggtggaatagttggaagtggggaggggctgacccgtggaagccatgatgaagctagtctgctgagggtgctgggagataagtggggtctggaatagagctgcagatgggtcagctgcttcagtagaaccttggcgactaaggctcatttgtccaaaggggttgctgaggtcatctgccatgttgtactgctggggcggagagactggcagaaggacttggggacaggagcttggagagaactgaacaggctgcggagagggctgcagagccgggactggctgtgagatcatgtgattattcaagggtggctgttgctgaggcgtgggtgggagagcaggaagttgctgctgctgctgctgctgttgctgctgggcagtacaagggagaagcccccggacagactgggatgaggtgacctggttgcacacttctggggcacctagtgccatacctggcctggagatccttcccgcactgccgcctttactgctgccgatgctgtcacctcgggtaaggatagagattccactgaagctgctagctttggtgacagggggtcgcatgctccggacagagccatcagagtctgtgctgctccaagggcgtggctccagggatttgagttcgctgtctgtgctgctctggcggctgcttgaggtgcggctcagtccttcacggttccccctaaaaatctgccttctcttgtgagagctagaagaaaaggcttctttggagagtctgatgtcatttagatatccgttctggccagtctctcgggcaaatattctctctcggaccctttgatattcctcctctctctcttctattgacttgctcctccttccatcctgcaatggaactctgatctggttatcatctcggtccatactggcatcatctctcttgagaatgaacctctgttgaaattctgtattcttctcatcctttatatgttctgagaacctctgttcagggattcttgtgttactagttttgttgatgatgacagctttcccagtttgatcaacattgtggtccatcccaaaataggcagctacccggtgtaatagcatccggtgatatgaggtcatctgagggaacttcttgaactgattattgttgtcattaataaattccagaatctcctgttctaattttagcagcatcattctgtcccttgggttctttttcagtgtatttacaagaaattcatgtaggtctattccagtggagtccgtatattcctggctggagtctctggacagcatcttccttgggatcttttctttgtttttgtccttgtcttccttttcagagacatcttttgtggacttttcttcctccttgtcagaagggcaactgatgtgcaattgaattatatcctgggtttctaatggcccatcagcaaatggggtggaggactcctcacacactgccaggctacgcaccaactttagcttggaattagacttggctcttttcctggcatgaccatggttagatgtccgcctcttgtcaaaaaggaactcataatcctgtgtctcctgacgcaaactggtatcttcacattctttctcaatttcttccttacttggagtcttagatataaacttgtttttgtttacagattcttccaccagttttttttctgattctttcattatttccagggtctcttgagtagtgttactgttagacatgttcttcaatagaatacagtggcctctatggactcctgaataaatgctcagcctccatgagtccagtgctggaatggcatcacatataagaaacaagtctaacct

SEQ ID NO: 17313 - RNA, 3659 nt, Homo sapiens
  source 1..3659: mol_type = other RNA
tcaggccaggcacagtggctcacgcctgtaatcccagcactctggaaggccaaggcaggtggatcacctgaggtcaggagtttgaggccagcctggccaacatggtgaaactccgtctctactaaaaatacaaaaattagccgggcatggtggcgcgtgtctgtagtgccagctacttgggaggctgaggcaggagaatcacctgaacccaggagctggaggttgcagttagccaagatcgtgctactgcactccagctggggtgacaagagcgaaactccgtctcaaaaaaaaaaaaaaaaaaaaaaagaagaggatgggaagaagagtgatgcaaggggggtcaaccagggaaaaagagaggacccatggcaggggagcaagaaggagtccaatgccagtgtaggtatctgtgtttccatcttcatcactgtcttaggttccagtttaacatcagtttccttacttcctgcctctgtccatggtctgtcaggatccttcaaccccctccaccctgcccttgctccttctgtgacagtccctttcccctcctccatttattgggagctggctcgctccaggatcctcaggtcatagttctttttggccattcgaagtttgaagcgactcacggagttgttgagacgaagggaggcattttgggcagccagggggctggggaacacagccacaatggtgtacaaggcagcgaggtccgagtggcggccattctcagcagtcccactgttgtcccccccaccccctccaggcagcccctgagcatccttgagccactggatcttggcgccagacatggcgagctgcgtgaagagtttgtccgcctcagtacgggtgatgccctcagggagatctgtcacctccagcacccgccccaggacaacatctgctgtccccaggtcagtggaggcagatttgagtgcttgtctcttgccccggtttccatgcttcagtccactctgtccctggtgcaccgtgtaagttgactggccatggagcaagggagggcagatggacagattgtactgtaatggctggcccaaaagggagtagcgcccatcaccctgtgctggacccccaggccgggggaactgtgtgaggacaggcaggggactgagtcctgtgcagacactgctgaggctggtgacaggagagggtgctggagactgggtaggagatgtgacagggctgctgctcatttgtgtgttggcctgggggctgctgtcaggactgtacaggtctccaggcttctgcccccgctggtccatgctgtagtatttacaatgactccactggaccatggatgggttctgagggggctggggtccattagggacattcagctgcatgaccactacacctggtccagaaggtgacactcctgagtactgctgtggcatctgtggtggactgcagggagagggagactgaggcatctggtactgctcagagccagggggttgcagaaaccctacagaagggctcgtaccgttctgctgagcaggtgggatcatgctatagtacactggtacccccgctgctgggaggcctccttgcacagactggctcacagggaccagcatgggttgctggaaaggcggctggaccacattttgcgagtcactacccactggaacttggtaagaaggcagtggagtgtactgaaccaccaggccttgcatctggccccccatgctgctcctctggctgctgagcaggccctggttctgtggctgctggaccccaatcatgccttggtaagccgcctgctgctggttaggcatcatgggctgtaaaccaggctgctgggatggctgaggcagctgctgaccacgttgggggctataggccaccgggtgagagagaggtcgatattgctggttggagttaggatattgtccagggggatagtaagaaacctggatctgttgagggggctgcatgtacccctggggtggcagaacttgctgagtaggtggtgcatggctagaggtggaatagttggaagtggggaggggctgacccgtggaagccatgatgaagctagtctgctgagggtgctgggagataagtggggtctggaatagagctgcagatgggtcagctgcttcagtagaaccttggcgactaaggctcatttgtccaaaggggttgctgaggtcatctgccatgttgtactgctggggcggagagactggcagaaggacttggggacaggagcttggagagaactgaacaggctgcggagagggctgcagagccgggactggctgtgagatcatgtgattattcaagggtggctgttgctgaggcgtgggtgggagagcaggaagttgctgctgctgctgctgctgttgctgctgggcagtacaagggagaagcccccggacagactgggatgaggtgacctggttgcacacttctggggcacctagtgccatacctggcctggagatccttcccgcactgccgcctttactgctgccgatgctgtcacctcgggtaaggatagagattccactgaagctgctagctttggtgacagggggtcgcatgctccggacagagccatcagagtctgtgctgctccaagggcgtggctccagggatttgagttcgctgtctgtgctgctctggcggctgcttgaggtgcggctcagtccttcacggttccccctaaaaatctgccttctcttgtgagagctagaagaaaaggcttctttggagagtctgatgtcatttagatatccgttctggccagtctggttatcatctcggtccatactggcatcatctctcttgagaatgaacctctgttgaaattctgtattcttctcatcctttatatgttctgagaacctctgttcagggattcttgtgttactagttttgttgatgatgacagctttcccagtttgatcaacattgtggtccatcccaaaataggcagctacccggtgtaatagcatccggtgatatgaggtcatctgagggaacttcttgaactgattacttgggttctttttcagtgtatttacaagaaattcatgtaggtctattccagtggagtccgtatattcctggctggagtctctggacagcatcttccttgggatcttttctttgtttttgtccttgtcttccttttcagagacatcttttgtggacttttcttcctccttgtcagaagggcaactgatgtgcaattgaattatatcctgggtttctaatggcccatcagcaaatggggtggaggactcctcacacactgccaggctacgcaccaactttagcttggaattagacttggctcttttcctggcatgaccatggttagatgtccgcctcttgtcaaaaaggaactcataatcctgtgtctcctgacgcaaactggtatcttcacattctttctcaatttcttccttacttggagtcttagatataaacttgtttttgtttacagattcttccaccagttttttttctgattctttcattatttccagggtctcttgagtagtgttactgttagacatgttcttcaatagaatacagtggcctctatggactcctgaataaatgctcagcctccatgagtccagtgctggaatggcatcacatataagaaacaagtctaacct

SEQ ID NO: 17314 - RNA, 4014 nt, Homo sapiens
  source 1..4014: mol_type = other RNA
tcaggccaggcacagtggctcacgcctgtaatcccagcactctggaaggccaaggcaggtggatcacctgaggtcaggagtttgaggccagcctggccaacatggtgaaactccgtctctactaaaaatacaaaaattagccgggcatggtggcgcgtgtctgtagtgccagctacttgggaggctgaggcaggagaatcacctgaacccaggagctggaggttgcagttagccaagatcgtgctactgcactccagctggggtgacaagagcgaaactccgtctcaaaaaaaaaaaaaaaaaaaaaaagaagaggatgggaagaagagtgatgcaaggggggtcaaccagggaaaaagagaggacccatggcaggggagcaagaaggagtccaatgccagtgtaggtatctgtgtttccatcttcatcactgtcttaggttccagtttaacatcagtttccttacttcctgcctctgtccatggtctgtcaggatccttcaaccccctccaccctgcccttgctccttctgtgacagtccctttcccctcctccatttattgggagctggctcgctccaggatcctcaggtcatagttctttttggccattcgaagtttgaagcgactcacggagttgttgagacgaagggaggcattttgggcagccagggggctggggaacacagccacaatggtgtacaaggcagcgaggtccgagtggcggccattctcagcagtcccactgttgtcccccccaccccctccaggcagcccctgagcatccttgagccactggatcttggcgccagacatggcgagctgcgtgaagagtttgtccgcctcagtacgggtgatgccctcagggagatctgtcacctccagcacccgccccaggacaacatctgctgtccccaggtcagtggaggcagatttgagtgcttgtctcttgccccggtttccatgcttcagtccactctgtccctggtgcaccgtgtaagttgactggccatggagcaagggagggcagatggacagattgtactgtaatggctggcccaaaagggagtagcgcccatcaccctgtgctggacccccaggccgggggaactgtgtgaggacaggcaggggactgagtcctgtgcagacactgctgaggctggtgacaggagagggtgctggagactgggtaggagatgtgacagggctgctgctcatttgtgtgttggcctgggggctgctgtcaggactgtacaggtctccaggcttctgcccccgctggtccatgctgtagtatttacaatgactccactggaccatggatgggttctgagggggctggggtccattagggacattcagctgcatgaccactacacctggtccagaaggtgacactcctgagtactgctgtggcatctgtggtggactgcagggagagggagactgaggcatctggtactgctcagagccagggggttgcagaaaccctacagaagggctcgtaccgttctgctgagcaggtgggatcatgctatagtacactggtacccccgctgctgggaggcctccttgcacagactggctcacagggaccagcatgggttgctggaaaggcggctggaccacattttgcgagtcactacccactggaacttggtaagaaggcagtggagtgtactgaaccaccaggccttgcatctggccccccatgctgctcctctggctgctgagcaggccctggttctgtggctgctggaccccaatcatgccttggtaagccgcctgctgctggttaggcatcatgggctgtaaaccaggctgctgggatggctgaggcagctgctgaccacgttgggggctataggccaccgggtgagagagaggtcgatattgctggttggagttaggatattgtccagggggatagtaagaaacctggatctgttgagggggctgcatgtacccctggggtggcagaacttgctgagtaggtggtgcatggctagaggtggaatagttggaagtggggaggggctgacccgtggaagccatgatgaagctagtctgctgagggtgctgggagataagtggggtctggaatagagctgcagatgggtcagctgcttcagtagaaccttggcgactaaggctcatttgtccaaaggggttgctgaggtcatctgccatgttgtactgctggggcggagagactggcagaaggacttggggacaggagcttggagagaactgaacaggctgcggagagggctgcagagccgggactggctgtgagatcatgtgattattcaagggtggctgttgctgaggcgtgggtgggagagcaggaagttgctgctgctgctgctgctgttgctgctgggcagtacaagggagaagcccccggacagactgggatgaggtgacctggttgcacacttctggggcacctagtgccatacctggcctggagatccttcccgcactgccgcctttactgctgccgatgctgtcacctcgggtaaggatagagattccactgaagctgctagctttggtgacagggggtcgcatgctccggacagagccatcagagtctgtgctgctccaagggcgtggctccagggatttgagttcgctgtctgtgctgctctggcggctgcttgaggtgcggctcagtccttcacggttccccctaaaaatctgccttctcttgtgagagctagaagaaaaggcttctttggagagtctgatgtcatttagatatccgttctggccagtctggttatcatctcggtccatactggcatcatctctcttgagaatgaacctctgttgaaattctgtattcttctcatcctttatatgttctgagaacctctgttcagggattcttgtgttactagttttgttgatgatgacagctttcccagtttgatcaacattgtggtccatcccaaaataggcagctacccggtgtaatagcatccggtgatatgaggtcatctgagggaacttcttgaactgattattgttgtcattaataaattccagaatctcctgttctaattttagcagcatcattctgtcccttgggttctttttcagtgtatttacaagaaattcatgtaggtctattccagtggagtccgtatattcctggctggagtctctggacagcatcttccttgggatcttttctttgtttttgtccttgtcttccttttcagagacatcttttgtggacttttcttcctccttgtcagaagggcaactgatgtgcaattgaattatatcctgggtttctaatggcccatcagcaaatggggtggaggactcctcacacactgccaggctacgcaccaactttagcttggaattagacttggctcttttcctggcatgaccatggttagatgtccgcctctgtgtctcctgacgcaaactggtatcttcacattctttctcaatttcttccttacttggagtcttagatataaacttgtttttgtttacagattcttccaccagttttttttctgattctttcattatttccagggtctcttgagtagtgttactgttagacatgttcttcaatagaatacagtggcctctatggactccgcttcagatggatttttcttcttccttctctccgtcccctccctctcagaagaaaaagactgcaaacaaaatcactacgtcactggaggtagagggaatcccatctctgcactctttagaagccaaggccagcaaataaaaacaagccaattataagaaaaagtaatacaaaataagaataaataaacccagaagaaatccatgtgacaatctcaacacatcaaaaggcattttttagtaaaaaggttttaacaaatgcctcctaggatgttcataatcaaaaaatctccccagacatagcaaaggcttatcacatttaaagactaggggatagttacgtaaagatataggacagacaggcacattcaccagccaggtgcggatagct

SEQ ID NO: 17315 - RNA, 4019 nt, Homo sapiens
  source 1..4019: mol_type = other RNA
tcaggccaggcacagtggctcacgcctgtaatcccagcactctggaaggccaaggcaggtggatcacctgaggtcaggagtttgaggccagcctggccaacatggtgaaactccgtctctactaaaaatacaaaaattagccgggcatggtggcgcgtgtctgtagtgccagctacttgggaggctgaggcaggagaatcacctgaacccaggagctggaggttgcagttagccaagatcgtgctactgcactccagctggggtgacaagagcgaaactccgtctcaaaaaaaaaaaaaaaaaaaaaaagaagaggatgggaagaagagtgatgcaaggggggtcaaccagggaaaaagagaggacccatggcaggggagcaagaaggagtccaatgccagtgtaggtatctgtgtttccatcttcatcactgtcttaggttccagtttaacatcagtttccttacttcctgcctctgtccatggtctgtcaggatccttcaaccccctccaccctgcccttgctccttctgtgacagtccctttcccctcctccatttattgggagctggctcgctccaggatcctcaggtcatagttctttttggccattcgaagtttgaagcgactcacggagttgttgagacgaagggaggcattttgggcagccagggggctggggaacacagccacaatggtgtacaaggcagcgaggtccgagtggcggccattctcagcagtcccactgttgtcccccccaccccctccaggcagcccctgagcatccttgagccactggatcttggcgccagacatggcgagctgcgtgaagagtttgtccgcctcagtacgggtgatgccctcagggagatctgtcacctccagcacccgccccaggacaacatctgctgtccccaggtcagtggaggcagatttgagtgcttgtctcttgccccggtttccatgcttcagtccactctgtccctggtgcaccgtgtaagttgactggccatggagcaagggagggcagatggacagattgtactgtaatggctggcccaaaagggagtagcgcccatcaccctgtgctggacccccaggccgggggaactgtgtgaggacaggcaggggactgagtcctgtgcagacactgctgaggctggtgacaggagagggtgctggagactgggtaggagatgtgacagggctgctgctcatttgtgtgttggcctgggggctgctgtcaggactgtacaggtctccaggcttctgcccccgctggtccatgctgtagtatttacaatgactccactggaccatggatgggttctgagggggctggggtccattagggacattcagctgcatgaccactacacctggtccagaaggtgacactcctgagtactgctgtggcatctgtggtggactgcagggagagggagactgaggcatctggtactgctcagagccagggggttgcagaaaccctacagaagggctcgtaccgttctgctgagcaggtgggatcatgctatagtacactggtacccccgctgctgggaggcctccttgcacagactggctcacagggaccagcatgggttgctggaaaggcggctggaccacattttgcgagtcactacccactggaacttggtaagaaggcagtggagtgtactgaaccaccaggccttgcatctggccccccatgctgctcctctggctgctgagcaggccctggttctgtggctgctggaccccaatcatgccttggtaagccgcctgctgctggttaggcatcatgggctgtaaaccaggctgctgggatggctgaggcagctgctgaccacgttgggggctataggccaccgggtgagagagaggtcgatattgctggttggagttaggatattgtccagggggatagtaagaaacctggatctgttgagggggctgcatgtacccctggggtggcagaacttgctgagtaggtggtgcatggctagaggtggaatagttggaagtggggaggggctgacccgtggaagccatgatgaagctagtctgctgagggtgctgggagataagtggggtctggaatagagctgcagatgggtcagctgcttcagtagaaccttggcgactaaggctcatttgtccaaaggggttgctgaggtcatctgccatgttgtactgctggggcggagagactggcagaaggacttggggacaggagcttggagagaactgaacaggctgcggagagggctgcagagccgggactggctgtgagatcatgtgattattcaagggtggctgttgctgaggcgtgggtgggagagcaggaagttgctgctgctgctgctgctgttgctgctgggcagtacaagggagaagcccccggacagactgggatgaggtgacctggttgcacacttctggggcacctagtgccatacctggcctggagatccttcccgcactgccgcctttactgctgccgatgctgtcacctcgggtaaggatagagattccactgaagctgctagctttggtgacagggggtcgcatgctccggacagagccatcagagtctgtgctgctccaagggcgtggctccagggatttgagttcgctgtctgtgctgctctggcggctgcttgaggtgcggctcagtccttcacggttccccctaaaaatctgccttctcttgtgagagctagaagaaaaggcttctttggagagtctgatgtcatttagatatccgttctggccagtctggttatcatctcggtccatactggcatcatctctcttgagaatgaacctctgttgaaattctgtattcttctcatcctttatatgttctgagaacctctgttcagggattcttgtgttactagttttgttgatgatgacagctttcccagtttgatcaacattgtggtccatcccaaaataggcagctacccggtgtaatagcatccggtgatatgaggtcatctgagggaacttcttgaactgattattgttgtcattaataaattccagaatctcctgttctaattttagcagcatcattctgtcccttgggttctttttcagtgtatttacaagaaattcatgtaggtctattccagtggagtccgtatattcctggctggagtctctggacagcatcttccttgggatcttttctttgtttttgtccttgtcttccttttcagagacatcttttgtggacttttcttcctccttgtcagaagggcaactgatgtgcaattgaattatatcctgggtttctaatggcccatcagcaaatggggtggaggactcctcacacactgccaggctacgcaccaactttagcttggaattagacttggctcttttcctggcatgaccatggttagatgtccgcctctgtgtctcctgacgcaaactggtatcttcacattctttctcaatttcttccttacttggagtcttagatataaacttgtttttgtttacagattcttccaccagttttttttctgattctttcattatttccagggtctcttgagtagtgttactgttagacatgttcttcaatagaatacagtggcctctatggactcctgaataaatgctcagcctccatgagtccagtgctggaatggcatcacatataagaaacaagtctaacctctcgcacgggccttggcggggagggcgcccacgtctccgcccgccgcccgggcccacggccgctcggctgcggctcggccccgacggccggcggcggcgcgcttctgggggcgggcttttctcggccggggcttccccggggccgagggctgggaagcaggggggactgggacgggggaggggaaaggggcttgggaaggaggggggagaggggaagaaaaggggggaaccaaacccggaaagggagaaaaggggggaggggaaaatcagaaggggaagaaaagcccagagtccgccccccgctgcggctgcgcgctacgtcac

SEQ ID NO: 17316 - RNA, 3719 nt, Homo sapiens
  source 1..3719: mol_type = other RNA
tcaggccaggcacagtggctcacgcctgtaatcccagcactctggaaggccaaggcaggtggatcacctgaggtcaggagtttgaggccagcctggccaacatggtgaaactccgtctctactaaaaatacaaaaattagccgggcatggtggcgcgtgtctgtagtgccagctacttgggaggctgaggcaggagaatcacctgaacccaggagctggaggttgcagttagccaagatcgtgctactgcactccagctggggtgacaagagcgaaactccgtctcaaaaaaaaaaaaaaaaaaaaaaagaagaggatgggaagaagagtgatgcaaggggggtcaaccagggaaaaagagaggacccatggcaggggagcaagaaggagtccaatgccagtgtaggtatctgtgtttccatcttcatcactgtcttaggttccagtttaacatcagtttccttacttcctgcctctgtccatggtctgtcaggatccttcaaccccctccaccctgcccttgctccttctgtgacagtccctttcccctcctccatttattgggagctggctcgctccaggatcctcaggtcatagttctttttggccattcgaagtttgaagcgactcacggagttgttgagacgaagggaggcattttgggcagccagggggctggggaacacagccacaatggtgtacaaggcagcgaggtccgagtggcggccattctcagcagtcccactgttgtcccccccaccccctccaggcagcccctgagcatccttgagccactggatcttggcgccagacatggcgagctgcgtgaagagtttgtccgcctcagtacgggtgatgccctcagggagatctgtcacctccagcacccgccccaggacaacatctgctgtccccaggtcagtggaggcagatttgagtgcttgtctcttgccccggtttccatgcttcagtccactctgtccctggtgcaccgtgtaagttgactggccatggagcaagggagggcagatggacagattgtactgtaatggctggcccaaaagggagtagcgcccatcaccctgtgctggacccccaggccgggggaactgtgtgaggacaggcaggggactgagtcctgtgcagacactgctgaggctggtgacaggagagggtgctggagactgggtaggagatgtgacagggctgctgctcatttgtgtgttggcctgggggctgctgtcaggactgtacaggtctccaggcttctgcccccgctggtccatgctgtagtatttacaatgactccactggaccatggatgggttctgagggggctggggtccattagggacattcagctgcatgaccactacacctggtccagaaggtgacactcctgagtactgctgtggcatctgtggtggactgcagggagagggagactgaggcatctggtactgctcagagccagggggttgcagaaaccctacagaagggctcgtaccgttctgctgagcaggtgggatcatgctatagtacactggtacccccgctgctgggaggcctccttgcacagactggctcacagggaccagcatgggttgctggaaaggcggctggaccacattttgcgagtcactacccactggaacttggtaagaaggcagtggagtgtactgaaccaccaggccttgcatctggccccccatgctgctcctctggctgctgagcaggccctggttctgtggctgctggaccccaatcatgccttggtaagccgcctgctgctggttaggcatcatgggctgtaaaccaggctgctgggatggctgaggcagctgctgaccacgttgggggctataggccaccgggtgagagagaggtcgatattgctggttggagttaggatattgtccagggggatagtaagaaacctggatctgttgagggggctgcatgtacccctggggtggcagaacttgctgagtaggtggtgcatggctagaggtggaatagttggaagtggggaggggctgacccgtggaagccatgatgaagctagtctgctgagggtgctgggagataagtggggtctggaatagagctgcagatgggtcagctgcttcagtagaaccttggcgactaaggctcatttgtccaaaggggttgctgaggtcatctgccatgttgtactgctggggcggagagactggcagaaggacttggggacaggagcttggagagaactgaacaggctgcggagagggctgcagagccgggactggctgtgagatcatgtgattattcaagggtggctgttgctgaggcgtgggtgggagagcaggaagttgctgctgctgctgctgctgttgctgctgggcagtacaagggagaagcccccggacagactgggatgaggtgacctggttgcacacttctggggcacctagtgccatacctggcctggagatccttcccgcactgccgcctttactgctgccgatgctgtcacctcgggtaaggatagagattccactgaagctgctagctttggtgacagggggtcgcatgctccggacagagccatcagagtctgtgctgctccaagggcgtggctccagggatttgagttcgctgtctgtgctgctctggcggctgcttgaggtgcggctcagtccttcacggttccccctaaaaatctgccttctcttgtgagagctagaagaaaaggcttctttggagagtctgatgtcatttagatatccgttctggccagtctggttatcatctcggtccatactggcatcatctctcttgagaatgaacctctgttgaaattctgtattcttctcatcctttatatgttctgagaacctctgttcagggattcttgtgttactagttttgttgatgatgacagctttcccagtttgatcaacattgtggtccatcccaaaataggcagctacccggtgtaatagcatccggtgatatgaggtcatctgagggaacttcttgaactgattattgttgtcattaataaattccagaatctcctgttctaattttagcagcatcattctgtcccttgggttctttttcagtgtatttacaagaaattcatgtaggtctattccagtggagtccgtatattcctggctggagtctctggacagcatcttccttgggatcttttctttgtttttgtccttgtcttccttttcagagacatcttttgtggacttttcttcctccttgtcagaagggcaactgatgtgcaattgaattatatcctgggtttctaatggcccatcagcaaatggggtggaggactcctcacacactgccaggctacgcaccaactttagcttggaattagacttggctcttttcctggcatgaccatggttagatgtccgcctcttgtcaaaaaggaactcataatcctgtgtctcctgacgcaaactggtatcttcacattctttctcaatttcttccttacttggagtcttagatataaacttgtttttgtttacagattcttccaccagttttttttctgattctttcattatttccagggtctcttgagtagtgttactgttagacatgttcttcaatagaatacagtggcctctatggactcctgaataaatgctcagcctccatgagtccagtgctggaatggcatcacatataagaaacaagtctaacct

SEQ ID NO: 17317 - RNA, 3186 nt, Homo sapiens
  source 1..3186: mol_type = other RNA
tcaggccaggcacagtggctcacgcctgtaatcccagcactctggaaggccaaggcaggtggatcacctgaggtcaggagtttgaggccagcctggccaacatggtgaaactccgtctctactaaaaatacaaaaattagccgggcatggtggcgcgtgtctgtagtgccagctacttgggaggctgaggcaggagaatcacctgaacccaggagctggaggttgcagttagccaagatcgtgctactgcactccagctggggtgacaagagcgaaactccgtctcaaaaaaaaaaaaaaaaaaaaaaagaagaggatgggaagaagagtgatgcaaggggggtcaaccagggaaaaagagaggacccatggcaggggagcaagaaggagtccaatgccagtgtaggtatctgtgtttccatcttcatcactgtcttaggttccagtttaacatcagtttccttacttcctgcctctgtccatggtctgtcaggatccttcaaccccctccaccctgcccttgctccttctgtgacagtccctttcccctcctccatttattgggagctggctcgctccaggatcctcaggtcatagttctttttggccattcgaagtttgaagcgactcacggagttgttgagacgaagggaggcattttgggcagccagggggctggggaacacagccacaatggtgtacaaggcagcgaggtccgagtggcggccattctcagcagtcccactgttgtcccccccaccccctccaggcagcccctgagcatccttgagccactggatcttggcgccagacatggcgagctgcgtgaagagtttgtccgcctcagtacgggtgatgccctcagggagatctgtcacctccagcacccgccccaggacaacatctgctgtccccaggtcagtggaggcagatttgagtgcttgtctcttgccccggtttccatgcttcagtccactctgtccctggtgcaccgtgtaagttgactggccatggagcaagggagggcagatggacagattgtactgtaatggctggcccaaaagggagtagcgcccatcaccctgtgctggacccccaggccgggggaactgtgtgaggacaggcaggggactgagtcctgtgcagacactgctgaggctggtgacaggagagggtgctggagactgggtaggagatgtgacagggctgctgctcatttgtgtgttggcctgggggctgctgtcaggactgtacaggtctccaggcttctgcccccgctggtccatgctgtagtatttacaatgactccactggaccatggatgggttctgagggggctggggtccattagggacattcagctgcatgaccactacacctggtccagaaggtgacactcctgagtactgctgtggcatctgtggtggactgcagggagagggagactgaggcatctggtactgctcagagccagggggttgcagaaaccctacagaagggctcgtaccgttctgctgagcaggtgggatcatgctatagtacactggtacccccgctgctgggaggcctccttgcacagactggctcacagggaccagcatgggttgctggaaaggcggctggaccacattttgcgagtcactacccactggaacttggtaagaaggcagtggagtgtactgaaccaccaggccttgcatctggccccccatgctgctcctctggctgctgagcaggccctggttctgtggctgctggaccccaatcatgccttggtaagccgcctgctgctggttaggcatcatgggctgtaaaccaggctgctgggatggctgaggcagctgctgaccacgttgggggctataggccaccgggtgagagagaggtcgatattgctggttggagttaggatattgtccagggggatagtaagaaacctggatctgttgagggggctgcatgtacccctggggtggcagaacttgctgagtaggtggtgcatggctagaggtggaatagttggaagtggggaggggctgacccgtggaagccatgatgaagctagtctgctgagggtgctgggagataagtggggtctggaatagagctgcagatgggtcagctgcttcagtagaaccttggcgactaaggctcatttgtccaaaggggttgctgaggtcatctgccatgttgtactgctggggcggagagactggcagaaggacttggggacaggagcttggagagaactgaacaggctgcggagagggctgcagagccgggactggctgtgagatcatgtgattattcaagggtggctgttgctgaggcgtgggtgggagagcaggaagttgctgctgctgctgctgctgttgctgctgggcagtacaagggagaagcccccggacagactgggatgaggtgacctggttgcacacttctggggcacctagtgccatacctggcctggagatccttcccgcactgccgcctttactgctgccgatgctgtcacctcgggtaaggatagagattccactgaagctgctagctttggtgacagggggtcgcatgctccggacagagccatcagagtctgtgctgctccaagggcgtggctccagggatttgagttcgctgtctgtgctgctctggcggctgcttgaggtgcggctcagtccttcacggttccccctgatgtcatttagatatccgttctggccagtctctcgggcaaatattctctctcggaccctttgatattcctcctctctctcttctattgacttgctcctccttccatcctgcaatggaactctgatctagatcgatgagcagaattaagctagttaagttctcctcgtactgcaagctcactggttatcatctcggtccatactggcatcatctctcttgagaatgaacctctgttgaaattctgtattcttctcatcctttatatgttctgagaacctctgttcagggattcttgtgttactagttttgttgatgatgacagctttcccagtttgatcaacattgtggtccatcccaaaataggcagctacccggtgtaatagcatccggtgatatgaggtcatctgagggaacttcttgaactgattattgttgtcattaataaattccagaatctcctgttctaattttagcagcatcattctgtcc

SEQ ID NO: 17318 - RNA, 3733 nt, Homo sapiens
  source 1..3733: mol_type = other RNA
tcaggccaggcacagtggctcacgcctgtaatcccagcactctggaaggccaaggcaggtggatcacctgaggtcaggagtttgaggccagcctggccaacatggtgaaactccgtctctactaaaaatacaaaaattagccgggcatggtggcgcgtgtctgtagtgccagctacttgggaggctgaggcaggagaatcacctgaacccaggagctggaggttgcagttagccaagatcgtgctactgcactccagctggggtgacaagagcgaaactccgtctcaaaaaaaaaaaaaaaaaaaaaaagaagaggatgggaagaagagtgatgcaaggggggtcaaccagggaaaaagagaggacccatggcaggggagcaagaaggagtccaatgccagtgtaggtatctgtgtttccatcttcatcactgtcttaggttccagtttaacatcagtttccttacttcctgcctctgtccatggtctgtcaggatccttcaaccccctccaccctgcccttgctccttctgtgacagtccctttcccctcctccatttattgggagctggctcgctccaggatcctcaggtcatagttctttttggccattcgaagtttgaagcgactcacggagttgttgagacgaagggaggcattttgggcagccagggggctggggaacacagccacaatggtgtacaaggcagcgaggtccgagtggcggccattctcagcagtcccactgttgtcccccccaccccctccaggcagcccctgagcatccttgagccactggatcttggcgccagacatggcgagctgcgtgaagagtttgtccgcctcagtacgggtgatgccctcagggagatctgtcacctccagcacccgccccaggacaacatctgctgtccccaggtcagtggaggcagatttgagtgcttgtctcttgccccggtttccatgcttcagtccactctgtccctggtgcaccgtgtaagttgactggccatggagcaagggagggcagatggacagattgtactgtaatggctggcccaaaagggagtagcgcccatcaccctgtgctggacccccaggccgggggaactgtgtgaggacaggcaggggactgagtcctgtgcagacactgctgaggctggtgacaggagagggtgctggagactgggtaggagatgtgacagggctgctgctcatttgtgtgttggcctgggggctgctgtcaggactgtacaggtctccaggcttctgcccccgctggtccatgctgtagtatttacaatgactccactggaccatggatgggttctgagggggctggggtccattagggacattcagctgcatgaccactacacctggtccagaaggtgacactcctgagtactgctgtggcatctgtggtggactgcagggagagggagactgaggcatctggtactgctcagagccagggggttgcagaaaccctacagaagggctcgtaccgttctgctgagcaggtgggatcatgctatagtacactggtacccccgctgctgggaggcctccttgcacagactggctcacagggaccagcatgggttgctggaaaggcggctggaccacattttgcgagtcactacccactggaacttggtaagaaggcagtggagtgtactgaaccaccaggccttgcatctggccccccatgctgctcctctggctgctgagcaggccctggttctgtggctgctggaccccaatcatgccttggtaagccgcctgctgctggttaggcatcatgggctgtaaaccaggctgctgggatggctgaggcagctgctgaccacgttgggggctataggccaccgggtgagagagaggtcgatattgctggttggagttaggatattgtccagggggatagtaagaaacctggatctgttgagggggctgcatgtacccctggggtggcagaacttgctgagtaggtggtgcatggctagaggtggaatagttggaagtggggaggggctgacccgtggaagccatgatgaagctagtctgctgagggtgctgggagataagtggggtctggaatagagctgcagatgggtcagctgcttcagtagaaccttggcgactaaggctcatttgtccaaaggggttgctgaggtcatctgccatgttgtactgctggggcggagagactggcagaaggacttggggacaggagcttggagagaactgaacaggctgcggagagggctgcagagccgggactggctgtgagatcatgtgattattcaagggtggctgttgctgaggcgtgggtgggagagcaggaagttgctgctgctgctgctgctgttgctgctgggcagtacaagggagaagcccccggacagactgggatgaggtgacctggttgcacacttctggggcacctagtgccatacctggcctggagatccttcccgcactgccgcctttactgctgccgatgctgtcacctcgggtaaggatagagattccactgaagctgctagctttggtgacagggggtcgcatgctccggacagagccatcagagtctgtgctgctccaagggcgtggctccagggatttgagttcgctgtctgtgctgctctggcggctgcttgaggtgcggctcagtccttcacggttccccctgatgtcatttagatatccgttctggccagtctctcgggcaaatattctctctcggaccctttgatattcctcctctctctcttctattgacttgctcctccttccatcctgcaatggaactctgatctggttatcatctcggtccatactggcatcatctctcttgagaatgaacctctgttgaaattctgtattcttctcatcctttatatgttctgagaacctctgttcagggattcttgtgttactagttttgttgatgatgacagctttcccagtttgatcaacattgtggtccatcccaaaataggcagctacccggtgtaatagcatccggtgatatgaggtcatctgagggaacttcttgaactgattattgttgtcattaataaattccagaatctcctgttctaattttagcagcatcattctgtcccttgggttctttttcagtgtatttacaagaaattcatgtaggtctattccagtggagtccgtatattcctggctggagtctctggacagcatcttccttgggatcttttctttgtttttgtccttgtcttccttttcagagacatcttttgtggacttttcttcctccttgtcagaagggcaactgatgtgcaattgaattatatcctgggtttctaatggcccatcagcaaatggggtggaggactcctcacacactgccaggctacgcaccaactttagcttggaattagacttggctcttttcctggcatgaccatggttagatgtccgcctctgtgtctcctgacgcaaactggtatcttcacattctttctcaatttcttccttacttggagtcttagatataaacttgtttttgtttacagattcttccaccagttttttttctgattctttcattatttccagggtctcttgagtagtgttactgttagacatgttcttcaatagaatacagtggcctctatggactccgcttcagatggatttttcttcttccttctctccgtcccctccctctcagaagaaaaagactgcaa

SEQ ID NO: 17319 - RNA, 3737 nt, Homo sapiens
  source 1..3737: mol_type = other RNA
tcaggccaggcacagtggctcacgcctgtaatcccagcactctggaaggccaaggcaggtggatcacctgaggtcaggagtttgaggccagcctggccaacatggtgaaactccgtctctactaaaaatacaaaaattagccgggcatggtggcgcgtgtctgtagtgccagctacttgggaggctgaggcaggagaatcacctgaacccaggagctggaggttgcagttagccaagatcgtgctactgcactccagctggggtgacaagagcgaaactccgtctcaaaaaaaaaaaaaaaaaaaaaaagaagaggatgggaagaagagtgatgcaaggggggtcaaccagggaaaaagagaggacccatggcaggggagcaagaaggagtccaatgccagtgtaggtatctgtgtttccatcttcatcactgtcttaggttccagtttaacatcagtttccttacttcctgcctctgtccatggtctgtcaggatccttcaaccccctccaccctgcccttgctccttctgtgacagtccctttcccctcctccatttattgggagctggctcgctccaggatcctcaggtcatagttctttttggccattcgaagtttgaagcgactcacggagttgttgagacgaagggaggcattttgggcagccagggggctggggaacacagccacaatggtgtacaaggcagcgaggtccgagtggcggccattctcagcagtcccactgttgtcccccccaccccctccaggcagcccctgagcatccttgagccactggatcttggcgccagacatggcgagctgcgtgaagagtttgtccgcctcagtacgggtgatgccctcagggagatctgtcacctccagcacccgccccaggacaacatctgctgtccccaggtcagtggaggcagatttgagtgcttgtctcttgccccggtttccatgcttcagtccactctgtccctggtgcaccgtgtaagttgactggccatggagcaagggagggcagatggacagattgtactgtaatggctggcccaaaagggagtagcgcccatcaccctgtgctggacccccaggccgggggaactgtgtgaggacaggcaggggactgagtcctgtgcagacactgctgaggctggtgacaggagagggtgctggagactgggtaggagatgtgacagggctgctgctcatttgtgtgttggcctgggggctgctgtcaggactgtacaggtctccaggcttctgcccccgctggtccatgctgtagtatttacaatgactccactggaccatggatgggttctgagggggctggggtccattagggacattcagctgcatgaccactacacctggtccagaaggtgacactcctgagtactgctgtggcatctgtggtggactgcagggagagggagactgaggcatctggtactgctcagagccagggggttgcagaaaccctacagaagggctcgtaccgttctgctgagcaggtgggatcatgctatagtacactggtacccccgctgctgggaggcctccttgcacagactggctcacagggaccagcatgggttgctggaaaggcggctggaccacattttgcgagtcactacccactggaacttggtaagaaggcagtggagtgtactgaaccaccaggccttgcatctggccccccatgctgctcctctggctgctgagcaggccctggttctgtggctgctggaccccaatcatgccttggtaagccgcctgctgctggttaggcatcatgggctgtaaaccaggctgctgggatggctgaggcagctgctgaccacgttgggggctataggccaccgggtgagagagaggtcgatattgctggttggagttaggatattgtccagggggatagtaagaaacctggatctgttgagggggctgcatgtacccctggggtggcagaacttgctgagtaggtggtgcatggctagaggtggaatagttggaagtggggaggggctgacccgtggaagccatgatgaagctagtctgctgagggtgctgggagataagtggggtctggaatagagctgcagatgggtcagctgcttcagtagaaccttggcgactaaggctcatttgtccaaaggggttgctgaggtcatctgccatgttgtactgctggggcggagagactggcagaaggacttggggacaggagcttggagagaactgaacaggctgcggagagggctgcagagccgggactggctgtgagatcatgtgattattcaagggtggctgttgctgaggcgtgggtgggagagcaggaagttgctgctgctgctgctgctgttgctgctgggcagtacaagggagaagcccccggacagactgggatgaggtgacctggttgcacacttctggggcacctagtgccatacctggcctggagatccttcccgcactgccgcctttactgctgccgatgctgtcacctcgggtaaggatagagattccactgaagctgctagctttggtgacagggggtcgcatgctccggacagagccatcagagtctgtgctgctccaagggcgtggctccagggatttgagttcgctgtctgtgctgctctggcggctgcttgaggtgcggctcagtccttcacggttccccctgatgtcatttagatatccgttctggccagtctctcgggcaaatattctctctcggaccctttgatattcctcctctctctcttctattgacttgctcctccttccatcctgcaatggaactctgatctggttatcatctcggtccatactggcatcatctctcttgagaatgaacctctgttgaaattctgtattcttctcatcctttatatgttctgagaacctctgttcagggattcttgtgttactagttttgttgatgatgacagctttcccagtttgatcaacattgtggtccatcccaaaataggcagctacccggtgtaatagcatccggtgatatgaggtcatctgagggaacttcttgaactgattattgttgtcattaataaattccagaatctcctgttctaattttagcagcatcattctgtcccttgggttctttttcagtgtatttacaagaaattcatgtaggtctattccagtggagtccgtatattcctggctggagtctctggacagcatcttccttgggatcttttctttgtttttgtccttgtcttccttttcagagacatcttttgtggacttttcttcctccttgtcagaagggcaactgatgtgcaattgaattatatcctgggtttctaatggcccatcagcaaatggggtggaggactcctcacacactgccaggctacgcaccaactttagcttggaattagacttggctcttttcctggcatgaccatggttagatgtccgcctctgtgtctcctgacgcaaactggtatcttcacattctttctcaatttcttccttacttggagtcttagatataaacttgtttttgtttacagattcttccaccagttttttttctgattctttcattatttccagggtctcttgagtagtgttactgttagacatgttcttcaatagaatacagtggcctctatggactcctgaataaatgctcagcctccatgagtccagtgctggaatggcatcacatataagaaacaagtctaacct

SEQ ID NO: 17320 - RNA, 4137 nt, Homo sapiens
  source 1..4137: mol_type = other RNA
tcaggccaggcacagtggctcacgcctgtaatcccagcactctggaaggccaaggcaggtggatcacctgaggtcaggagtttgaggccagcctggccaacatggtgaaactccgtctctactaaaaatacaaaaattagccgggcatggtggcgcgtgtctgtagtgccagctacttgggaggctgaggcaggagaatcacctgaacccaggagctggaggttgcagttagccaagatcgtgctactgcactccagctggggtgacaagagcgaaactccgtctcaaaaaaaaaaaaaaaaaaaaaaagaagaggatgggaagaagagtgatgcaaggggggtcaaccagggaaaaagagaggacccatggcaggggagcaagaaggagtccaatgccagtgtaggtatctgtgtttccatcttcatcactgtcttaggttccagtttaacatcagtttccttacttcctgcctctgtccatggtctgtcaggatccttcaaccccctccaccctgcccttgctccttctgtgacagtccctttcccctcctccatttattgggagctggctcgctccaggatcctcaggtcatagttctttttggccattcgaagtttgaagcgactcacggagttgttgagacgaagggaggcattttgggcagccagggggctggggaacacagccacaatggtgtacaaggcagcgaggtccgagtggcggccattctcagcagtcccactgttgtcccccccaccccctccaggcagcccctgagcatccttgagccactggatcttggcgccagacatggcgagctgcgtgaagagtttgtccgcctcagtacgggtgatgccctcagggagatctgtcacctccagcacccgccccaggacaacatctgctgtccccaggtcagtggaggcagatttgagtgcttgtctcttgccccggtttccatgcttcagtccactctgtccctggtgcaccgtgtaagttgactggccatggagcaagggagggcagatggacagattgtactgtaatggctggcccaaaagggagtagcgcccatcaccctgtgctggacccccaggccgggggaactgtgtgaggacaggcaggggactgagtcctgtgcagacactgctgaggctggtgacaggagagggtgctggagactgggtaggagatgtgacagggctgctgctcatttgtgtgttggcctgggggctgctgtcaggactgtacaggtctccaggcttctgcccccgctggtccatgctgtagtatttacaatgactccactggaccatggatgggttctgagggggctggggtccattagggacattcagctgcatgaccactacacctggtccagaaggtgacactcctgagtactgctgtggcatctgtggtggactgcagggagagggagactgaggcatctggtactgctcagagccagggggttgcagaaaccctacagaagggctcgtaccgttctgctgagcaggtgggatcatgctatagtacactggtacccccgctgctgggaggcctccttgcacagactggctcacagggaccagcatgggttgctggaaaggcggctggaccacattttgcgagtcactacccactggaacttggtaagaaggcagtggagtgtactgaaccaccaggccttgcatctggccccccatgctgctcctctggctgctgagcaggccctggttctgtggctgctggaccccaatcatgccttggtaagccgcctgctgctggttaggcatcatgggctgtaaaccaggctgctgggatggctgaggcagctgctgaccacgttgggggctataggccaccgggtgagagagaggtcgatattgctggttggagttaggatattgtccagggggatagtaagaaacctggatctgttgagggggctgcatgtacccctggggtggcagaacttgctgagtaggtggtgcatggctagaggtggaatagttggaagtggggaggggctgacccgtggaagccatgatgaagctagtctgctgagggtgctgggagataagtggggtctggaatagagctgcagatgggtcagctgcttcagtagaaccttggcgactaaggctcatttgtccaaaggggttgctgaggtcatctgccatgttgtactgctggggcggagagactggcagaaggacttggggacaggagcttggagagaactgaacaggctgcggagagggctgcagagccgggactggctgtgagatcatgtgattattcaagggtggctgttgctgaggcgtgggtgggagagcaggaagttgctgctgctgctgctgctgttgctgctgggcagtacaagggagaagcccccggacagactgggatgaggtgacctggttgcacacttctggggcacctagtgccatacctggcctggagatccttcccgcactgccgcctttactgctgccgatgctgtcacctcgggtaaggatagagattccactgaagctgctagctttggtgacagggggtcgcatgctccggacagagccatcagagtctgtgctgctccaagggcgtggctccagggatttgagttcgctgtctgtgctgctctggcggctgcttgaggtgcggctcagtccttcacggttccccctgatgtcatttagatatccgttctggccagtctctcgggcaaatattctctctcggaccctttgatattcctcctctctctcttctattgacttgctcctccttccatcctgcaatggaactctgatctggttatcatctcggtccatactggcatcatctctcttgagaatgaacctctgttgaaattctgtattcttctcatcctttatatgttctgagaacctctgttcagggattcttgtgttactagttttgttgatgatgacagctttcccagtttgatcaacattgtggtccatcccaaaataggcagctacccggtgtaatagcatccggtgatatgaggtcatctgagggaacttcttgaactgattattgttgtcattaataaattccagaatctcctgttctaattttagcagcatcattctgtcccttgggttctttttcagtgtatttacaagaaattcatgtaggtctattccagtggagtccgtatattcctggctggagtctctggacagcatcttccttgggatcttttctttgtttttgtccttgtcttccttttcagagacatcttttgtggacttttcttcctccttgtcagaagggcaactgatgtgcaattgaattatatcctgggtttctaatggcccatcagcaaatggggtggaggactcctcacacactgccaggctacgcaccaactttagcttggaattagacttggctcttttcctggcatgaccatggttagatgtccgcctctgtgtctcctgacgcaaactggtatcttcacattctttctcaatttcttccttacttggagtcttagatataaacttgtttttgtttacagattcttccaccagttttttttctgattctttcattatttccagggtctcttgagtagtgttactgttagacatgttcttcaatagaatacagtggcctctatggactcctttaaaacatcccactttggcttcagctctattcaatggcacccagttaccaacatcaagtcacagaaggaagaacgcaccgcttcagatggatttttcttcttccttctctccgtcccctccctctcagaagaaaaagactgcaaacaaaatcactacgtcactggaggtagagggaatcccatctctgcactctttagaagccaaggccagcaaataaaaacaagccaattataagaaaaagtaatacaaaataagaataaataaacccagaagaaatccatgtgacaatctcaacacatcaaaaggcattttttagtaaaaaggttttaacaaatgcctcctaggatgttcataatcaaaaaatctccccagacatagcaaaggcttatcacatttaaagactaggggatagttacgtaaagatataggacagacaggcacattcaccagccaggtgcggatagct

SEQ ID NO: 17321 - RNA, 4186 nt, Homo sapiens
  source 1..4186: mol_type = other RNA
tcaggccaggcacagtggctcacgcctgtaatcccagcactctggaaggccaaggcaggtggatcacctgaggtcaggagtttgaggccagcctggccaacatggtgaaactccgtctctactaaaaatacaaaaattagccgggcatggtggcgcgtgtctgtagtgccagctacttgggaggctgaggcaggagaatcacctgaacccaggagctggaggttgcagttagccaagatcgtgctactgcactccagctggggtgacaagagcgaaactccgtctcaaaaaaaaaaaaaaaaaaaaaaagaagaggatgggaagaagagtgatgcaaggggggtcaaccagggaaaaagagaggacccatggcaggggagcaagaaggagtccaatgccagtgtaggtatctgtgtttccatcttcatcactgtcttaggttccagtttaacatcagtttccttacttcctgcctctgtccatggtctgtcaggatccttcaaccccctccaccctgcccttgctccttctgtgacagtccctttcccctcctccatttattgggagctggctcgctccaggatcctcaggtcatagttctttttggccattcgaagtttgaagcgactcacggagttgttgagacgaagggaggcattttgggcagccagggggctggggaacacagccacaatggtgtacaaggcagcgaggtccgagtggcggccattctcagcagtcccactgttgtcccccccaccccctccaggcagcccctgagcatccttgagccactggatcttggcgccagacatggcgagctgcgtgaagagtttgtccgcctcagtacgggtgatgccctcagggagatctgtcacctccagcacccgccccaggacaacatctgctgtccccaggtcagtggaggcagatttgagtgcttgtctcttgccccggtttccatgcttcagtccactctgtccctggtgcaccgtgtaagttgactggccatggagcaagggagggcagatggacagattgtactgtaatggctggcccaaaagggagtagcgcccatcaccctgtgctggacccccaggccgggggaactgtgtgaggacaggcaggggactgagtcctgtgcagacactgctgaggctggtgacaggagagggtgctggagactgggtaggagatgtgacagggctgctgctcatttgtgtgttggcctgggggctgctgtcaggactgtacaggtctccaggcttctgcccccgctggtccatgctgtagtatttacaatgactccactggaccatggatgggttctgagggggctggggtccattagggacattcagctgcatgaccactacacctggtccagaaggtgacactcctgagtactgctgtggcatctgtggtggactgcagggagagggagactgaggcatctggtactgctcagagccagggggttgcagaaaccctacagaagggctcgtaccgttctgctgagcaggtgggatcatgctatagtacactggtacccccgctgctgggaggcctccttgcacagactggctcacagggaccagcatgggttgctggaaaggcggctggaccacattttgcgagtcactacccactggaacttggtaagaaggcagtggagtgtactgaaccaccaggccttgcatctggccccccatgctgctcctctggctgctgagcaggccctggttctgtggctgctggaccccaatcatgccttggtaagccgcctgctgctggttaggcatcatgggctgtaaaccaggctgctgggatggctgaggcagctgctgaccacgttgggggctataggccaccgggtgagagagaggtcgatattgctggttggagttaggatattgtccagggggatagtaagaaacctggatctgttgagggggctgcatgtacccctggggtggcagaacttgctgagtaggtggtgcatggctagaggtggaatagttggaagtggggaggggctgacccgtggaagccatgatgaagctagtctgctgagggtgctgggagataagtggggtctggaatagagctgcagatgggtcagctgcttcagtagaaccttggcgactaaggctcatttgtccaaaggggttgctgaggtcatctgccatgttgtactgctggggcggagagactggcagaaggacttggggacaggagcttggagagaactgaacaggctgcggagagggctgcagagccgggactggctgtgagatcatgtgattattcaagggtggctgttgctgaggcgtgggtgggagagcaggaagttgctgctgctgctgctgctgttgctgctgggcagtacaagggagaagcccccggacagactgggatgaggtgacctggttgcacacttctggggcacctagtgccatacctggcctggagatccttcccgcactgccgcctttactgctgccgatgctgtcacctcgggtaaggatagagattccactgaagctgctagctttggtgacagggggtcgcatgctccggacagagccatcagagtctgtgctgctccaagggcgtggctccagggatttgagttcgctgtctgtgctgctctggcggctgcttgaggtgcggctcagtccttcacggttccccctgatgtcatttagatatccgttctggccagtctctcgggcaaatattctctctcggaccctttgatattcctcctctctctcttctattgacttgctcctccttccatcctgcaatggaactctgatctggttatcatctcggtccatactggcatcatctctcttgagaatgaacctctgttgaaattctgtattcttctcatcctttatatgttctgagaacctctgttcagggattcttgtgttactagttttgttgatgatgacagctttcccagtttgatcaacattgtggtccatcccaaaataggcagctacccggtgtaatagcatccggtgatatgaggtcatctgagggaacttcttgaactgattattgttgtcattaataaattccagaatctcctgttctaattttagcagcatcattctgtcccttgggttctttttcagtgtatttacaagaaattcatgtaggtctattccagtggagtccgtatattcctggctggagtctctggacagcatcttccttgggatcttttctttgtttttgtccttgtcttccttttcagagacatcttttgtggacttttcttcctccttgtcagaagggcaactgatgtgcaattgaattatatcctgggtttctaatggcccatcagcaaatggggtggaggactcctcacacactgccaggctacgcaccaactttagcttggaattagacttggctcttttcctggcatgaccatggttagatgtccgcctcttgtcaaaaaggaactcataatcctgtgtctcctgacgcaaactggtatcttcacattctttctcaatttcttccttacttggagtcttagatataaacttgtttttgtttacagattcttccaccagttttttttctgattctttcattatttccagggtctcttgagtagtgttactgttagacatgttcttcaatagaatacagtggcctctatggactcctgaataaatgctcagcctccatgagtccagtgctggaatggcatcacatataagaaacaagtctaacctctgtagtcccagctacttgggagccttgagcccaggaggtggagacagcagtgagtcatgatcatgccagtttactccagcctggacaacagagcaagaccctcgcacgggccttggcggggagggcgcccacgtctccgcccgccgcccgggcccacggccgctcggctgcggctcggccccgacggccggcggcggcgcgcttctgggggcgggcttttctcggccggggcttccccggggccgagggctgggaagcaggggggactgggacgggggaggggaaaggggcttgggaaggaggggggagaggggaagaaaaggggggaaccaaacccggaaagggagaaaaggggggaggggaaaatcagaaggggaagaaaagcccagagtccgccccccgctgcggctgcgcgctacgtcac

SEQ ID NO: 17322 - RNA, 3859 nt, Homo sapiens
  source 1..3859: mol_type = other RNA
tcaggccaggcacagtggctcacgcctgtaatcccagcactctggaaggccaaggcaggtggatcacctgaggtcaggagtttgaggccagcctggccaacatggtgaaactccgtctctactaaaaatacaaaaattagccgggcatggtggcgcgtgtctgtagtgccagctacttgggaggctgaggcaggagaatcacctgaacccaggagctggaggttgcagttagccaagatcgtgctactgcactccagctggggtgacaagagcgaaactccgtctcaaaaaaaaaaaaaaaaaaaaaaagaagaggatgggaagaagagtgatgcaaggggggtcaaccagggaaaaagagaggacccatggcaggggagcaagaaggagtccaatgccagtgtaggtatctgtgtttccatcttcatcactgtcttaggttccagtttaacatcagtttccttacttcctgcctctgtccatggtctgtcaggatccttcaaccccctccaccctgcccttgctccttctgtgacagtccctttcccctcctccatttattgggagctggctcgctccaggatcctcaggtcatagttctttttggccattcgaagtttgaagcgactcacggagttgttgagacgaagggaggcattttgggcagccagggggctggggaacacagccacaatggtgtacaaggcagcgaggtccgagtggcggccattctcagcagtcccactgttgtcccccccaccccctccaggcagcccctgagcatccttgagccactggatcttggcgccagacatggcgagctgcgtgaagagtttgtccgcctcagtacgggtgatgccctcagggagatctgtcacctccagcacccgccccaggacaacatctgctgtccccaggtcagtggaggcagatttgagtgcttgtctcttgccccggtttccatgcttcagtccactctgtccctggtgcaccgtgtaagttgactggccatggagcaagggagggcagatggacagattgtactgtaatggctggcccaaaagggagtagcgcccatcaccctgtgctggacccccaggccgggggaactgtgtgaggacaggcaggggactgagtcctgtgcagacactgctgaggctggtgacaggagagggtgctggagactgggtaggagatgtgacagggctgctgctcatttgtgtgttggcctgggggctgctgtcaggactgtacaggtctccaggcttctgcccccgctggtccatgctgtagtatttacaatgactccactggaccatggatgggttctgagggggctggggtccattagggacattcagctgcatgaccactacacctggtccagaaggtgacactcctgagtactgctgtggcatctgtggtggactgcagggagagggagactgaggcatctggtactgctcagagccagggggttgcagaaaccctacagaagggctcgtaccgttctgctgagcaggtgggatcatgctatagtacactggtacccccgctgctgggaggcctccttgcacagactggctcacagggaccagcatgggttgctggaaaggcggctggaccacattttgcgagtcactacccactggaacttggtaagaaggcagtggagtgtactgaaccaccaggccttgcatctggccccccatgctgctcctctggctgctgagcaggccctggttctgtggctgctggaccccaatcatgccttggtaagccgcctgctgctggttaggcatcatgggctgtaaaccaggctgctgggatggctgaggcagctgctgaccacgttgggggctataggccaccgggtgagagagaggtcgatattgctggttggagttaggatattgtccagggggatagtaagaaacctggatctgttgagggggctgcatgtacccctggggtggcagaacttgctgagtaggtggtgcatggctagaggtggaatagttggaagtggggaggggctgacccgtggaagccatgatgaagctagtctgctgagggtgctgggagataagtggggtctggaatagagctgcagatgggtcagctgcttcagtagaaccttggcgactaaggctcatttgtccaaaggggttgctgaggtcatctgccatgttgtactgctggggcggagagactggcagaaggacttggggacaggagcttggagagaactgaacaggctgcggagagggctgcagagccgggactggctgtgagatcatgtgattattcaagggtggctgttgctgaggcgtgggtgggagagcaggaagttgctgctgctgctgctgctgttgctgctgggcagtacaagggagaagcccccggacagactgggatgaggtgacctggttgcacacttctggggcacctagtgccatacctggcctggagatccttcccgcactgccgcctttactgctgccgatgctgtcacctcgggtaaggatagagattccactgaagctgctagctttggtgacagggggtcgcatgctccggacagagccatcagagtctgtgctgctccaagggcgtggctccagggatttgagttcgctgtctgtgctgctctggcggctgcttgaggtgcggctcagtccttcacggttccccctgatgtcatttagatatccgttctggccagtctggttatcatctcggtccatactggcatcatctctcttgagaatgaacctctgttgaaattctgtattcttctcatcctttatatgttctgagaacctctgttcagggattcttgtgttactagttttgttgatgatgacagctttcccagtttgatcaacattgtggtccatcccaaaataggcagctacccggtgtaatagcatccggtgatatgaggtcatctgagggaacttcttgaactgattattgttgtcattaataaattccagaatctcctgttctaattttagcagcatcattctgtcccttgggttctttttcagtgtatttacaagaaattcatgtaggtctattccagtggagtccgtatattcctggctggagtctctggacagcatcttccttgggatcttttctttgtttttgtccttgtcttccttttcagagacatcttttgtggacttttcttcctccttgtcagaagggcaactgatgtgcaattgaattatatcctgggtttctaatggcccatcagcaaatggggtggaggactcctcacacactgccaggctacgcaccaactttagcttggaattagacttggctcttttcctggcatgaccatggttagatgtccgcctctgtgtctcctgacgcaaactggtatcttcacattctttctcaatttcttccttacttggagtcttagatataaacttgtttttgtttacagattcttccaccagttttttttctgattctttcattatttccagggtctcttgagtagtgttactgttagacatgttcttcaatagaatacagtggcctctatggactccccagatggatctgtacttacaccaacagcgagctcacattattaatggagacttcattgtaaagatctgttctgccggaattttgccggaagaaattccttctgggaaacctgtgcctcttcccccacccacagccctctcccgcccccttcacccttgaatgaaatgatactgatccttgctgctggagctccagctaactaactgctctgacaagcagctctgaagccgaccatggcccagctgttcagagagatatcatccagagctctgccaacagtcacact

SEQ ID NO: 17323 - RNA, 3960 nt, Homo sapiens
  source 1..3960: mol_type = other RNA
tcaggccaggcacagtggctcacgcctgtaatcccagcactctggaaggccaaggcaggtggatcacctgaggtcaggagtttgaggccagcctggccaacatggtgaaactccgtctctactaaaaatacaaaaattagccgggcatggtggcgcgtgtctgtagtgccagctacttgggaggctgaggcaggagaatcacctgaacccaggagctggaggttgcagttagccaagatcgtgctactgcactccagctggggtgacaagagcgaaactccgtctcaaaaaaaaaaaaaaaaaaaaaaagaagaggatgggaagaagagtgatgcaaggggggtcaaccagggaaaaagagaggacccatggcaggggagcaagaaggagtccaatgccagtgtaggtatctgtgtttccatcttcatcactgtcttaggttccagtttaacatcagtttccttacttcctgcctctgtccatggtctgtcaggatccttcaaccccctccaccctgcccttgctccttctgtgacagtccctttcccctcctccatttattgggagctggctcgctccaggatcctcaggtcatagttctttttggccattcgaagtttgaagcgactcacggagttgttgagacgaagggaggcattttgggcagccagggggctggggaacacagccacaatggtgtacaaggcagcgaggtccgagtggcggccattctcagcagtcccactgttgtcccccccaccccctccaggcagcccctgagcatccttgagccactggatcttggcgccagacatggcgagctgcgtgaagagtttgtccgcctcagtacgggtgatgccctcagggagatctgtcacctccagcacccgccccaggacaacatctgctgtccccaggtcagtggaggcagatttgagtgcttgtctcttgccccggtttccatgcttcagtccactctgtccctggtgcaccgtgtaagttgactggccatggagcaagggagggcagatggacagattgtactgtaatggctggcccaaaagggagtagcgcccatcaccctgtgctggacccccaggccgggggaactgtgtgaggacaggcaggggactgagtcctgtgcagacactgctgaggctggtgacaggagagggtgctggagactgggtaggagatgtgacagggctgctgctcatttgtgtgttggcctgggggctgctgtcaggactgtacaggtctccaggcttctgcccccgctggtccatgctgtagtatttacaatgactccactggaccatggatgggttctgagggggctggggtccattagggacattcagctgcatgaccactacacctggtccagaaggtgacactcctgagtactgctgtggcatctgtggtggactgcagggagagggagactgaggcatctggtactgctcagagccagggggttgcagaaaccctacagaagggctcgtaccgttctgctgagcaggtgggatcatgctatagtacactggtacccccgctgctgggaggcctccttgcacagactggctcacagggaccagcatgggttgctggaaaggcggctggaccacattttgcgagtcactacccactggaacttggtaagaaggcagtggagtgtactgaaccaccaggccttgcatctggccccccatgctgctcctctggctgctgagcaggccctggttctgtggctgctggaccccaatcatgccttggtaagccgcctgctgctggttaggcatcatgggctgtaaaccaggctgctgggatggctgaggcagctgctgaccacgttgggggctataggccaccgggtgagagagaggtcgatattgctggttggagttaggatattgtccagggggatagtaagaaacctggatctgttgagggggctgcatgtacccctggggtggcagaacttgctgagtaggtggtgcatggctagaggtggaatagttggaagtggggaggggctgacccgtggaagccatgatgaagctagtctgctgagggtgctgggagataagtggggtctggaatagagctgcagatgggtcagctgcttcagtagaaccttggcgactaaggctcatttgtccaaaggggttgctgaggtcatctgccatgttgtactgctggggcggagagactggcagaaggacttggggacaggagcttggagagaactgaacaggctgcggagagggctgcagagccgggactggctgtgagatcatgtgattattcaagggtggctgttgctgaggcgtgggtgggagagcaggaagttgctgctgctgctgctgctgttgctgctgggcagtacaagggagaagcccccggacagactgggatgaggtgacctggttgcacacttctggggcacctagtgccatacctggcctggagatccttcccgcactgccgcctttactgctgccgatgctgtcacctcgggtaaggatagagattccactgaagctgctagctttggtgacagggggtcgcatgctccggacagagccatcagagtctgtgctgctccaagggcgtggctccagggatttgagttcgctgtctgtgctgctctggcggctgcttgaggtgcggctcagtccttcacggttccccctgatgtcatttagatatccgttctggccagtctggttatcatctcggtccatactggcatcatctctcttgagaatgaacctctgttgaaattctgtattcttctcatcctttatatgttctgagaacctctgttcagggattcttgtgttactagttttgttgatgatgacagctttcccagtttgatcaacattgtggtccatcccaaaataggcagctacccggtgtaatagcatccggtgatatgaggtcatctgagggaacttcttgaactgattattgttgtcattaataaattccagaatctcctgttctaattttagcagcatcattctgtcccttgggttctttttcagtgtatttacaagaaattcatgtaggtctattccagtggagtccgtatattcctggctggagtctctggacagcatcttccttgggatcttttctttgtttttgtccttgtcttccttttcagagacatcttttgtggacttttcttcctccttgtcagaagggcaactgatgtgcaattgaattatatcctgggtttctaatggcccatcagcaaatggggtggaggactcctcacacactgccaggctacgcaccaactttagcttggaattagacttggctcttttcctggcatgaccatggttagatgtccgcctctgtgtctcctgacgcaaactggtatcttcacattctttctcaatttcttccttacttggagtcttagatataaacttgtttttgtttacagattcttccaccagttttttttctgattctttcattatttccagggtctcttgagtagtgttactgttagacatgttcttcaatagaatacagtggcctctatggactccgcttcagatggatttttcttcttccttctctccgtcccctccctctcagaagaaaaagactgcaaacaaaatcactacgtcactggaggtagagggaatcccatctctgcactctttagaagccaaggccagcaaataaaaacaagccaattataagaaaaagtaatacaaaataagaataaataaacccagaagaaatccatgtgacaatctcaacacatcaaaaggcattttttagtaaaaaggttttaacaaatgcctcctaggatgttcataatcaaaaaatctccccagacatagcaaaggcttatcacatttaaagactaggggatagttacgtaaagatataggacagacaggcacattcaccagccaggtgcggatagct

SEQ ID NO: 17324 - RNA, 3895 nt, Homo sapiens
  source 1..3895: mol_type = other RNA
tcaggccaggcacagtggctcacgcctgtaatcccagcactctggaaggccaaggcaggtggatcacctgaggtcaggagtttgaggccagcctggccaacatggtgaaactccgtctctactaaaaatacaaaaattagccgggcatggtggcgcgtgtctgtagtgccagctacttgggaggctgaggcaggagaatcacctgaacccaggagctggaggttgcagttagccaagatcgtgctactgcactccagctggggtgacaagagcgaaactccgtctcaaaaaaaaaaaaaaaaaaaaaaagaagaggatgggaagaagagtgatgcaaggggggtcaaccagggaaaaagagaggacccatggcaggggagcaagaaggagtccaatgccagtgtaggtatctgtgtttccatcttcatcactgtcttaggttccagtttaacatcagtttccttacttcctgcctctgtccatggtctgtcaggatccttcaaccccctccaccctgcccttgctccttctgtgacagtccctttcccctcctccatttattgggagctggctcgctccaggatcctcaggtcatagttctttttggccattcgaagtttgaagcgactcacggagttgttgagacgaagggaggcattttgggcagccagggggctggggaacacagccacaatggtgtacaaggcagcgaggtccgagtggcggccattctcagcagtcccactgttgtcccccccaccccctccaggcagcccctgagcatccttgagccactggatcttggcgccagacatggcgagctgcgtgaagagtttgtccgcctcagtacgggtgatgccctcagggagatctgtcacctccagcacccgccccaggacaacatctgctgtccccaggtcagtggaggcagatttgagtgcttgtctcttgccccggtttccatgcttcagtccactctgtccctggtgcaccgtgtaagttgactggccatggagcaagggagggcagatggacagattgtactgtaatggctggcccaaaagggagtagcgcccatcaccctgtgctggacccccaggccgggggaactgtgtgaggacaggcaggggactgagtcctgtgcagacactgctgaggctggtgacaggagagggtgctggagactgggtaggagatgtgacagggctgctgctcatttgtgtgttggcctgggggctgctgtcaggactgtacaggtctccaggcttctgcccccgctggtccatgctgtagtatttacaatgactccactggaccatggatgggttctgagggggctggggtccattagggacattcagctgcatgaccactacacctggtccagaaggtgacactcctgagtactgctgtggcatctgtggtggactgcagggagagggagactgaggcatctggtactgctcagagccagggggttgcagaaaccctacagaagggctcgtaccgttctgctgagcaggtgggatcatgctatagtacactggtacccccgctgctgggaggcctccttgcacagactggctcacagggaccagcatgggttgctggaaaggcggctggaccacattttgcgagtcactacccactggaacttggtaagaaggcagtggagtgtactgaaccaccaggccttgcatctggccccccatgctgctcctctggctgctgagcaggccctggttctgtggctgctggaccccaatcatgccttggtaagccgcctgctgctggttaggcatcatgggctgtaaaccaggctgctgggatggctgaggcagctgctgaccacgttgggggctataggccaccgggtgagagagaggtcgatattgctggttggagttaggatattgtccagggggatagtaagaaacctggatctgttgagggggctgcatgtacccctggggtggcagaacttgctgagtaggtggtgcatggctagaggtggaatagttggaagtggggaggggctgacccgtggaagccatgatgaagctagtctgctgagggtgctgggagataagtggggtctggaatagagctgcagatgggtcagctgcttcagtagaaccttggcgactaaggctcatttgtccaaaggggttgctgaggtcatctgccatgttgtactgctggggcggagagactggcagaaggacttggggacaggagcttggagagaactgaacaggctgcggagagggctgcagagccgggactggctgtgagatcatgtgattattcaagggtggctgttgctgaggcgtgggtgggagagcaggaagttgctgctgctgctgctgctgttgctgctgggcagtacaagggagaagcccccggacagactgggatgaggtgacctggttgcacacttctggggcacctagtgccatacctggcctggagatccttcccgcactgccgcctttactgctgccgatgctgtcacctcgggtaaggatagagattccactgaagctgctagctttggtgacagggggtcgcatgctccggacagagccatcagagtctgtgctgctccaagggcgtggctccagggatttgagttcgctgtctgtgctgctctggcggctgcttgaggtgcggctcagtccttcacggttccccctgatgtcatttagatatccgttctggccagtctggttatcatctcggtccatactggcatcatctctcttgagaatgaacctctgttgaaattctgtattcttctcatcctttatatgttctgagaacctctgttcagggattcttgtgttactagttttgttgatgatgacagctttcccagtttgatcaacattgtggtccatcccaaaataggcagctacccggtgtaatagcatccggtgatatgaggtcatctgagggaacttcttgaactgattattgttgtcattaataaattccagaatctcctgttctaattttagcagcatcattctgtcccttgggttctttttcagtgtatttacaagaaattcatgtaggtctattccagtggagtccgtatattcctggctggagtctctggacagcatcttccttgggatcttttctttgtttttgtccttgtcttccttttcagagacatcttttgtggacttttcttcctccttgtcagaagggcaactgatgtgcaattgaattatatcctgggtttctaatggcccatcagcaaatggggtggaggactcctcacacactgccaggctacgcaccaactttagcttggaattagacttggctcttttcctggcatgaccatggttagatgtccgcctctgtgtctcctgacgcaaactggtatcttcacattctttctcaatttcttccttacttggagtcttagatataaacttgtttttgtttacagattcttccaccagttttttttctgattctttcattatttccagggtctcttgagtagtgttactgttagacatgttcttcaatagaatacagtggcctctatggactcctcgcacgggccttggcggggagggcgcccacgtctccgcccgccgcccgggcccacggccgctcggctgcggctcggccccgacggccggcggcggcgcgcttctgggggcgggcttttctcggccggggcttccccggggccgagggctgggaagcaggggggactgggacgggggaggggaaaggggcttgggaaggaggggggagaggggaagaaaaggggggaaccaaacccggaaagggagaaaaggggggaggggaaaatcagaaggggaagaaaagcccagagtccgccccccgctgcggctgcgcgctacgtcac

SEQ ID NO: 17325 - RNA, 3965 nt, Homo sapiens
  source 1..3965: mol_type = other RNA
tcaggccaggcacagtggctcacgcctgtaatcccagcactctggaaggccaaggcaggtggatcacctgaggtcaggagtttgaggccagcctggccaacatggtgaaactccgtctctactaaaaatacaaaaattagccgggcatggtggcgcgtgtctgtagtgccagctacttgggaggctgaggcaggagaatcacctgaacccaggagctggaggttgcagttagccaagatcgtgctactgcactccagctggggtgacaagagcgaaactccgtctcaaaaaaaaaaaaaaaaaaaaaaagaagaggatgggaagaagagtgatgcaaggggggtcaaccagggaaaaagagaggacccatggcaggggagcaagaaggagtccaatgccagtgtaggtatctgtgtttccatcttcatcactgtcttaggttccagtttaacatcagtttccttacttcctgcctctgtccatggtctgtcaggatccttcaaccccctccaccctgcccttgctccttctgtgacagtccctttcccctcctccatttattgggagctggctcgctccaggatcctcaggtcatagttctttttggccattcgaagtttgaagcgactcacggagttgttgagacgaagggaggcattttgggcagccagggggctggggaacacagccacaatggtgtacaaggcagcgaggtccgagtggcggccattctcagcagtcccactgttgtcccccccaccccctccaggcagcccctgagcatccttgagccactggatcttggcgccagacatggcgagctgcgtgaagagtttgtccgcctcagtacgggtgatgccctcagggagatctgtcacctccagcacccgccccaggacaacatctgctgtccccaggtcagtggaggcagatttgagtgcttgtctcttgccccggtttccatgcttcagtccactctgtccctggtgcaccgtgtaagttgactggccatggagcaagggagggcagatggacagattgtactgtaatggctggcccaaaagggagtagcgcccatcaccctgtgctggacccccaggccgggggaactgtgtgaggacaggcaggggactgagtcctgtgcagacactgctgaggctggtgacaggagagggtgctggagactgggtaggagatgtgacagggctgctgctcatttgtgtgttggcctgggggctgctgtcaggactgtacaggtctccaggcttctgcccccgctggtccatgctgtagtatttacaatgactccactggaccatggatgggttctgagggggctggggtccattagggacattcagctgcatgaccactacacctggtccagaaggtgacactcctgagtactgctgtggcatctgtggtggactgcagggagagggagactgaggcatctggtactgctcagagccagggggttgcagaaaccctacagaagggctcgtaccgttctgctgagcaggtgggatcatgctatagtacactggtacccccgctgctgggaggcctccttgcacagactggctcacagggaccagcatgggttgctggaaaggcggctggaccacattttgcgagtcactacccactggaacttggtaagaaggcagtggagtgtactgaaccaccaggccttgcatctggccccccatgctgctcctctggctgctgagcaggccctggttctgtggctgctggaccccaatcatgccttggtaagccgcctgctgctggttaggcatcatgggctgtaaaccaggctgctgggatggctgaggcagctgctgaccacgttgggggctataggccaccgggtgagagagaggtcgatattgctggttggagttaggatattgtccagggggatagtaagaaacctggatctgttgagggggctgcatgtacccctggggtggcagaacttgctgagtaggtggtgcatggctagaggtggaatagttggaagtggggaggggctgacccgtggaagccatgatgaagctagtctgctgagggtgctgggagataagtggggtctggaatagagctgcagatgggtcagctgcttcagtagaaccttggcgactaaggctcatttgtccaaaggggttgctgaggtcatctgccatgttgtactgctggggcggagagactggcagaaggacttggggacaggagcttggagagaactgaacaggctgcggagagggctgcagagccgggactggctgtgagatcatgtgattattcaagggtggctgttgctgaggcgtgggtgggagagcaggaagttgctgctgctgctgctgctgttgctgctgggcagtacaagggagaagcccccggacagactgggatgaggtgacctggttgcacacttctggggcacctagtgccatacctggcctggagatccttcccgcactgccgcctttactgctgccgatgctgtcacctcgggtaaggatagagattccactgaagctgctagctttggtgacagggggtcgcatgctccggacagagccatcagagtctgtgctgctccaagggcgtggctccagggatttgagttcgctgtctgtgctgctctggcggctgcttgaggtgcggctcagtccttcacggttccccctgatgtcatttagatatccgttctggccagtctggttatcatctcggtccatactggcatcatctctcttgagaatgaacctctgttgaaattctgtattcttctcatcctttatatgttctgagaacctctgttcagggattcttgtgttactagttttgttgatgatgacagctttcccagtttgatcaacattgtggtccatcccaaaataggcagctacccggtgtaatagcatccggtgatatgaggtcatctgagggaacttcttgaactgattattgttgtcattaataaattccagaatctcctgttctaattttagcagcatcattctgtcccttgggttctttttcagtgtatttacaagaaattcatgtaggtctattccagtggagtccgtatattcctggctggagtctctggacagcatcttccttgggatcttttctttgtttttgtccttgtcttccttttcagagacatcttttgtggacttttcttcctccttgtcagaagggcaactgatgtgcaattgaattatatcctgggtttctaatggcccatcagcaaatggggtggaggactcctcacacactgccaggctacgcaccaactttagcttggaattagacttggctcttttcctggcatgaccatggttagatgtccgcctctgtgtctcctgacgcaaactggtatcttcacattctttctcaatttcttccttacttggagtcttagatataaacttgtttttgtttacagattcttccaccagttttttttctgattctttcattatttccagggtctcttgagtagtgttactgttagacatgttcttcaatagaatacagtggcctctatggactcctgaataaatgctcagcctccatgagtccagtgctggaatggcatcacatataagaaacaagtctaacctctcgcacgggccttggcggggagggcgcccacgtctccgcccgccgcccgggcccacggccgctcggctgcggctcggccccgacggccggcggcggcgcgcttctgggggcgggcttttctcggccggggcttccccggggccgagggctgggaagcaggggggactgggacgggggaggggaaaggggcttgggaaggaggggggagaggggaagaaaaggggggaaccaaacccggaaagggagaaaaggggggaggggaaaatcagaaggggaagaaaagcccagagtccgccccccgctgcggctgcgcgctacgtcac

SEQ ID NO: 17326 - RNA, 3665 nt, Homo sapiens
  source 1..3665: mol_type = other RNA
tcaggccaggcacagtggctcacgcctgtaatcccagcactctggaaggccaaggcaggtggatcacctgaggtcaggagtttgaggccagcctggccaacatggtgaaactccgtctctactaaaaatacaaaaattagccgggcatggtggcgcgtgtctgtagtgccagctacttgggaggctgaggcaggagaatcacctgaacccaggagctggaggttgcagttagccaagatcgtgctactgcactccagctggggtgacaagagcgaaactccgtctcaaaaaaaaaaaaaaaaaaaaaaagaagaggatgggaagaagagtgatgcaaggggggtcaaccagggaaaaagagaggacccatggcaggggagcaagaaggagtccaatgccagtgtaggtatctgtgtttccatcttcatcactgtcttaggttccagtttaacatcagtttccttacttcctgcctctgtccatggtctgtcaggatccttcaaccccctccaccctgcccttgctccttctgtgacagtccctttcccctcctccatttattgggagctggctcgctccaggatcctcaggtcatagttctttttggccattcgaagtttgaagcgactcacggagttgttgagacgaagggaggcattttgggcagccagggggctggggaacacagccacaatggtgtacaaggcagcgaggtccgagtggcggccattctcagcagtcccactgttgtcccccccaccccctccaggcagcccctgagcatccttgagccactggatcttggcgccagacatggcgagctgcgtgaagagtttgtccgcctcagtacgggtgatgccctcagggagatctgtcacctccagcacccgccccaggacaacatctgctgtccccaggtcagtggaggcagatttgagtgcttgtctcttgccccggtttccatgcttcagtccactctgtccctggtgcaccgtgtaagttgactggccatggagcaagggagggcagatggacagattgtactgtaatggctggcccaaaagggagtagcgcccatcaccctgtgctggacccccaggccgggggaactgtgtgaggacaggcaggggactgagtcctgtgcagacactgctgaggctggtgacaggagagggtgctggagactgggtaggagatgtgacagggctgctgctcatttgtgtgttggcctgggggctgctgtcaggactgtacaggtctccaggcttctgcccccgctggtccatgctgtagtatttacaatgactccactggaccatggatgggttctgagggggctggggtccattagggacattcagctgcatgaccactacacctggtccagaaggtgacactcctgagtactgctgtggcatctgtggtggactgcagggagagggagactgaggcatctggtactgctcagagccagggggttgcagaaaccctacagaagggctcgtaccgttctgctgagcaggtgggatcatgctatagtacactggtacccccgctgctgggaggcctccttgcacagactggctcacagggaccagcatgggttgctggaaaggcggctggaccacattttgcgagtcactacccactggaacttggtaagaaggcagtggagtgtactgaaccaccaggccttgcatctggccccccatgctgctcctctggctgctgagcaggccctggttctgtggctgctggaccccaatcatgccttggtaagccgcctgctgctggttaggcatcatgggctgtaaaccaggctgctgggatggctgaggcagctgctgaccacgttgggggctataggccaccgggtgagagagaggtcgatattgctggttggagttaggatattgtccagggggatagtaagaaacctggatctgttgagggggctgcatgtacccctggggtggcagaacttgctgagtaggtggtgcatggctagaggtggaatagttggaagtggggaggggctgacccgtggaagccatgatgaagctagtctgctgagggtgctgggagataagtggggtctggaatagagctgcagatgggtcagctgcttcagtagaaccttggcgactaaggctcatttgtccaaaggggttgctgaggtcatctgccatgttgtactgctggggcggagagactggcagaaggacttggggacaggagcttggagagaactgaacaggctgcggagagggctgcagagccgggactggctgtgagatcatgtgattattcaagggtggctgttgctgaggcgtgggtgggagagcaggaagttgctgctgctgctgctgctgttgctgctgggcagtacaagggagaagcccccggacagactgggatgaggtgacctggttgcacacttctggggcacctagtgccatacctggcctggagatccttcccgcactgccgcctttactgctgccgatgctgtcacctcgggtaaggatagagattccactgaagctgctagctttggtgacagggggtcgcatgctccggacagagccatcagagtctgtgctgctccaagggcgtggctccagggatttgagttcgctgtctgtgctgctctggcggctgcttgaggtgcggctcagtccttcacggttccccctgatgtcatttagatatccgttctggccagtctggttatcatctcggtccatactggcatcatctctcttgagaatgaacctctgttgaaattctgtattcttctcatcctttatatgttctgagaacctctgttcagggattcttgtgttactagttttgttgatgatgacagctttcccagtttgatcaacattgtggtccatcccaaaataggcagctacccggtgtaatagcatccggtgatatgaggtcatctgagggaacttcttgaactgattattgttgtcattaataaattccagaatctcctgttctaattttagcagcatcattctgtcccttgggttctttttcagtgtatttacaagaaattcatgtaggtctattccagtggagtccgtatattcctggctggagtctctggacagcatcttccttgggatcttttctttgtttttgtccttgtcttccttttcagagacatcttttgtggacttttcttcctccttgtcagaagggcaactgatgtgcaattgaattatatcctgggtttctaatggcccatcagcaaatggggtggaggactcctcacacactgccaggctacgcaccaactttagcttggaattagacttggctcttttcctggcatgaccatggttagatgtccgcctcttgtcaaaaaggaactcataatcctgtgtctcctgacgcaaactggtatcttcacattctttctcaatttcttccttacttggagtcttagatataaacttgtttttgtttacagattcttccaccagttttttttctgattctttcattatttccagggtctcttgagtagtgttactgttagacatgttcttcaatagaatacagtggcctctatggactcctgaataaatgctcagcctccatgagtccagtgctggaatggcatcacatataagaaacaagtctaacct

SEQ ID NO: 17327 - RNA, 3948 nt, Homo sapiens
  source 1..3948: mol_type = other RNA
tcaggccaggcacagtggctcacgcctgtaatcccagcactctggaaggccaaggcaggtggatcacctgaggtcaggagtttgaggccagcctggccaacatggtgaaactccgtctctactaaaaatacaaaaattagccgggcatggtggcgcgtgtctgtagtgccagctacttgggaggctgaggcaggagaatcacctgaacccaggagctggaggttgcagttagccaagatcgtgctactgcactccagctggggtgacaagagcgaaactccgtctcaaaaaaaaaaaaaaaaaaaaaaagaagaggatgggaagaagagtgatgcaaggggggtcaaccagggaaaaagagaggacccatggcaggggagcaagaaggagtccaatgccagtgtaggtatctgtgtttccatcttcatcactgtcttaggttccagtttaacatcagtttccttacttcctgcctctgtccatggtctgtcaggatccttcaaccccctccaccctgcccttgctccttctgtgacagtccctttcccctcctccatttattgggagctggctcgctccaggatcctcaggtcatagttctttttggccattcgaagtttgaagcgactcacggagttgttgagacgaagggaggcattttgggcagccagggggctggggaacacagccacaatggtgtacaaggcagcgaggtccgagtggcggccattctcagcagtcccactgttgtcccccccaccccctccaggcagcccctgagcatccttgagccactggatcttggcgccagacatggcgagctgcgtgaagagtttgtccgcctcagtacgggtgatgccctcagggagatctgtcacctccagcacccgccccaggacaacatctgctgtccccaggtcagtggaggcagatttgagtgcttgtctcttgccccggtttccatgcttcagtccactctgtccctggtgcaccgtgtaagttgactggccatggagcaagggagggcagatggacagattgtactgtaatggctggcccaaaagggagtagcgcccatcaccctgtgctggacccccaggccgggggaactgtgtgaggacaggcaggggactgagtcctgtgcagacactgctgaggctggtgacaggagagggtgctggagactgggtaggagatgtgacagggctgctgctcatttgtgtgttggcctgggggctgctgtcaggactgtacaggtctccaggcttctgcccccgctggtccatgctgtagtatttacaatgactccactggaccatggatgggttctgagggggctggggtccattagggacattcagctgcatgaccactacacctggtccagaaggtgacactcctgagtactgctgtggcatctgtggtggactgcagggagagggagactgaggcatctggtactgctcagagccagggggttgcagaaaccctacagaagggctcgtaccgttctgctgagcaggtgggatcatgctatagtacactggtacccccgctgctgggaggcctccttgcacagactggctcacagggaccagcatgggttgctggaaaggcggctggaccacattttgcgagtcactacccactggaacttggtaagaaggcagtggagtgtactgaaccaccaggccttgcatctggccccccatgctgctcctctggctgctgagcaggccctggttctgtggctgctggaccccaatcatgccttggtaagccgcctgctgctggttaggcatcatgggctgtaaaccaggctgctgggatggctgaggcagctgctgaccacgttgggggctataggccaccgggtgagagagaggtcgatattgctggttggagttaggatattgtccagggggatagtaagaaacctggatctgttgagggggctgcatgtacccctggggtggcagaacttgctgagtaggtggtgcatggctagaggtggaatagttggaagtggggaggggctgacccgtggaagccatgatgaagctagtctgctgagggtgctgggagataagtggggtctggaatagagctgcagatgggtcagctgcttcagtagaaccttggcgactaaggctcatttgtccaaaggggttgctgaggtcatctgcctgtgagatcatgtgattattcaagggtggctgttgctgaggcgtgggtgggagagcaggaagttgctgctgctgctgctgctgttgctgctgggcagtacaagggagaagcccccggacagactgggatgaggtgacctggttgcacacttctggggcacctagtgccatacctggcctggagatccttcccgcactgccgcctttactgctgccgatgctgtcacctcgggtaaggatagagattccactgaagctgctagctttggtgacagggggtcgcatgctccggacagagccatcagagtctgtgctgctccaagggcgtggctccagggatttgagttcgctgtctgtgctgctctggcggctgcttgaggtgcggctcagtccttcacggttccccctaaaaatctgccttctcttgtgagagctagaagaaaaggcttctttggagagtctgatgtcatttagatatccgttctggccagtctctcgggcaaatattctctctcggaccctttgatattcctcctctctctcttctattgacttgctcctccttccatcctgcaatggaactctgatctggttatcatctcggtccatactggcatcatctctcttgagaatgaacctctgttgaaattctgtattcttctcatcctttatatgttctgagaacctctgttcagggattcttgtgttactagttttgttgatgatgacagctttcccagtttgatcaacattgtggtccatcccaaaataggcagctacccggtgtaatagcatccggtgatatgaggtcatctgagggaacttcttgaactgattacttgggttctttttcagtgtatttacaagaaattcatgtaggtctattccagtggagtccgtatattcctggctggagtctctggacagcatcttccttgggatcttttctttgtttttgtccttgtcttccttttcagagacatcttttgtggacttttcttcctccttgtcagaagggcaactgatgtgcaattgaattatatcctgggtttctaatggcccatcagcaaatggggtggaggactcctcacacactgccaggctacgcaccaactttagcttggaattagacttggctcttttcctggcatgaccatggttagatgtccgcctctgtgtctcctgacgcaaactggtatcttcacattctttctcaatttcttccttacttggagtcttagatataaacttgtttttgtttacagattcttccaccagttttttttctgattctttcattatttccagggtctcttgagtagtgttactgttagacatgttcttcaatagaatacagtggcctctatggactccgcttcagatggatttttcttcttccttctctccgtcccctccctctcagaagaaaaagactgcaaacaaaatcactacgtcactggaggtagagggaatcccatctctgcactctttagaagccaaggccagcaaataaaaacaagccaattataagaaaaagtaatacaaaataagaataaataaacccagaagaaatccatgtgacaatctcaacacatcaaaaggcattttttagtaaaaaggttttaacaaatgcctcctaggatgttcataatcaaaaaatctccccagacatagcaaaggcttatcacatttaaagactaggggatagttacgtaaagatataggacagacaggcacattcaccagccaggtgcggatagct

SEQ ID NO: 17328 - RNA, 3629 nt, Homo sapiens
  source 1..3629: mol_type = other RNA
tcaggccaggcacagtggctcacgcctgtaatcccagcactctggaaggccaaggcaggtggatcacctgaggtcaggagtttgaggccagcctggccaacatggtgaaactccgtctctactaaaaatacaaaaattagccgggcatggtggcgcgtgtctgtagtgccagctacttgggaggctgaggcaggagaatcacctgaacccaggagctggaggttgcagttagccaagatcgtgctactgcactccagctggggtgacaagagcgaaactccgtctcaaaaaaaaaaaaaaaaaaaaaaagaagaggatgggaagaagagtgatgcaaggggggtcaaccagggaaaaagagaggacccatggcaggggagcaagaaggagtccaatgccagtgtaggtatctgtgtttccatcttcatcactgtcttaggttccagtttaacatcagtttccttacttcctgcctctgtccatggtctgtcaggatccttcaaccccctccaccctgcccttgctccttctgtgacagtccctttcccctcctccatttattgggagctggctcgctccaggatcctcaggtcatagttctttttggccattcgaagtttgaagcgactcacggagttgttgagacgaagggaggcattttgggcagccagggggctggggaacacagccacaatggtgtacaaggcagcgaggtccgagtggcggccattctcagcagtcccactgttgtcccccccaccccctccaggcagcccctgagcatccttgagccactggatcttggcgccagacatggcgagctgcgtgaagagtttgtccgcctcagtacgggtgatgccctcagggagatctgtcacctccagcacccgccccaggacaacatctgctgtccccaggtcagtggaggcagatttgagtgcttgtctcttgccccggtttccatgcttcagtccactctgtccctggtgcaccgtgtaagttgactggccatggagcaagggagggcagatggacagattgtactgtaatggctggcccaaaagggagtagcgcccatcaccctgtgctggacccccaggccgggggaactgtgtgaggacaggcaggggactgagtcctgtgcagacactgctgaggctggtgacaggagagggtgctggagactgggtaggagatgtgacagggctgctgctcatttgtgtgttggcctgggggctgctgtcaggactgtacaggtctccaggcttctgcccccgctggtccatgctgtagtatttacaatgactccactggaccatggatgggttctgagggggctggggtccattagggacattcagctgcatgaccactacacctggtccagaaggtgacactcctgagtactgctgtggcatctgtggtggactgcagggagagggagactgaggcatctggtactgctcagagccagggggttgcagaaaccctacagaagggctcgtaccgttctgctgagcaggtgggatcatgctatagtacactggtacccccgctgctgggaggcctccttgcacagactggctcacagggaccagcatgggttgctggaaaggcggctggaccacattttgcgagtcactacccactggaacttggtaagaaggcagtggagtgtactgaaccaccaggccttgcatctggccccccatgctgctcctctggctgctgagcaggccctggttctgtggctgctggaccccaatcatgccttggtaagccgcctgctgctggttaggcatcatgggctgtaaaccaggctgctgggatggctgaggcagctgctgaccacgttgggggctataggccaccgggtgagagagaggtcgatattgctggttggagttaggatattgtccagggggatagtaagaaacctggatctgttgagggggctgcatgtacccctggggtggcagaacttgctgagtaggtggtgcatggctagaggtggaatagttggaagtggggaggggctgacccgtggaagccatgatgaagctagtctgctgagggtgctgggagataagtggggtctggaatagagctgcagatgggtcagctgcttcagtagaaccttggcgactaaggctcatttgtccaaaggggttgctgaggtcatctgcctgtgagatcatgtgattattcaagggtggctgttgctgaggcgtgggtgggagagcaggaagttgctgctgctgctgctgctgttgctgctgggcagtacaagggagaagcccccggacagactgggatgaggtgacctggttgcacacttctggggcacctagtgccatacctggcctggagatccttcccgcactgccgcctttactgctgccgatgctgtcacctcgggtaaggatagagattccactgaagctgctagctttggtgacagggggtcgcatgctccggacagagccatcagagtctgtgctgctccaagggcgtggctccagggatttgagttcgctgtctgtgctgctctggcggctgcttgaggtgcggctcagtccttcacggttccccctaaaaatctgccttctcttgtgagagctagaagaaaaggcttctttggagagtctgatgtcatttagatatccgttctggccagtctctcgggcaaatattctctctcggaccctttgatattcctcctctctctcttctattgacttgctcctccttccatcctgcaatggaactctgatctggttatcatctcggtccatactggcatcatctctcttgagaatgaacctctgttgaaattctgtattcttctcatcctttatatgttctgagaacctctgttcagggattcttgtgttactagttttgttgatgatgacagctttcccagtttgatcaacattgtggtccatcccaaaataggcagctacccggtgtaatagcatccggtgatatgaggtcatctgagggaacttcttgaactgattacttgggttctttttcagtgtatttacaagaaattcatgtaggtctattccagtggagtccgtatattcctggctggagtctctggacagcatcttccttgggatcttttctttgtttttgtccttgtcttccttttcagagacatcttttgtggacttttcttcctccttgtcagaagggcaactgatgtgcaattgaattatatcctgggtttctaatggcccatcagcaaatggggtggaggactcctcacacactgccaggctacgcaccaactttagcttggaattagacttggctcttttcctggcatgaccatggttagatgtccgcctctgtgtctcctgacgcaaactggtatcttcacattctttctcaatttcttccttacttggagtcttagatataaacttgtttttgtttacagattcttccaccagttttttttctgattctttcattatttccagggtctcttgagtagtgttactgttagacatgttcttcaatagaatacagtggcctctatggactcctgaataaatgctcagcctccatgagtccagtgctggaatggcatcacatataagaaacaagtctaacct

SEQ ID NO: 17329 - RNA, 4486 nt, Homo sapiens
  source 1..4486: mol_type = other RNA
tcaggccaggcacagtggctcacgcctgtaatcccagcactctggaaggccaaggcaggtggatcacctgaggtcaggagtttgaggccagcctggccaacatggtgaaactccgtctctactaaaaatacaaaaattagccgggcatggtggcgcgtgtctgtagtgccagctacttgggaggctgaggcaggagaatcacctgaacccaggagctggaggttgcagttagccaagatcgtgctactgcactccagctggggtgacaagagcgaaactccgtctcaaaaaaaaaaaaaaaaaaaaaaagaagaggatgggaagaagagtgatgcaaggggggtcaaccagggaaaaagagaggacccatggcaggggagcaagaaggagtccaatgccagtgtaggtatctgtgtttccatcttcatcactgtcttaggttccagtttaacatcagtttccttacttcctgcctctgtccatggtctgtcaggatccttcaaccccctccaccctgcccttgctccttctgtgacagtccctttcccctcctccatttattgggagctggctcgctccaggatcctcaggtcatagttctttttggccattcgaagtttgaagcgactcacggagttgttgagacgaagggaggcattttgggcagccagggggctggggaacacagccacaatggtgtacaaggcagcgaggtccgagtggcggccattctcagcagtcccactgttgtcccccccaccccctccaggcagcccctgagcatccttgagccactggatcttggcgccagacatggcgagctgcgtgaagagtttgtccgcctcagtacgggtgatgccctcagggagatctgtcacctccagcacccgccccaggacaacatctgctgtccccaggtcagtggaggcagatttgagtgcttgtctcttgccccggtttccatgcttcagtccactctgtccctggtgcaccgtgtaagttgactggccatggagcaagggagggcagatggacagattgtactgtaatggctggcccaaaagggagtagcgcccatcaccctgtgctggacccccaggccgggggaactgtgtgaggacaggcaggggactgagtcctgtgcagacactgctgaggctggtgacaggagagggtgctggagactgggtaggagatgtgacagggctgctgctcatttgtgtgttggcctgggggctgctgtcaggactgtacaggtctccaggcttctgcccccgctggtccatgctgtagtatttacaatgactccactggaccatggatgggttctgagggggctggggtccattagggacattcagctgcatgaccactacacctggtccagaaggtgacactcctgagtactgctgtggcatctgtggtggactgcagggagagggagactgaggcatctggtactgctcagagccagggggttgcagaaaccctacagaagggctcgtaccgttctgctgagcaggtgggatcatgctatagtacactggtacccccgctgctgggaggcctccttgcacagactggctcacagggaccagcatgggttgctggaaaggcggctggaccacattttgcgagtcactacccactggaacttggtaagaaggcagtggagtgtactgaaccaccaggccttgcatctggccccccatgctgctcctctggctgctgagcaggccctggttctgtggctgctggaccccaatcatgccttggtaagccgcctgctgctggttaggcatcatgggctgtaaaccaggctgctgggatggctgaggcagctgctgaccacgttgggggctataggccaccgggtgagagagaggtcgatattgctggttggagttaggatattgtccagggggatagtaagaaacctggatctgttgagggggctgcatgtacccctggggtggcagaacttgctgagtaggtggtgcatggctagaggtggaatagttggaagtggggaggggctgacccgtggaagccatgatgaagctagtctgctgagggtgctgggagataagtggggtctggaatagagctgcagatgggtcagctgcttcagtagaaccttggcgactaaggctcatttgtccaaaggggttgctgaggtcatctgcctgtgagatcatgtgattattcaagggtggctgttgctgaggcgtgggtgggagagcaggaagttgctgctgctgctgctgctgttgctgctgggcagtacaagggagaagcccccggacagactgggatgaggtgacctggttgcacacttctggggcacctagtgccatacctggcctggagatccttcccgcactgccgcctttactgctgccgatgctgtcacctcgggtaaggatagagattccactgaagctgctagctttggtgacagggggtcgcatgctccggacagagccatcagagtctgtgctgctccaagggcgtggctccagggatttgagttcgctgtctgtgctgctctggcggctgcttgaggtgcggctcagtccttcacggttccccctaaaaatctgccttctcttgtgagagctagaagaaaaggcttctttggagagtctgatgtcatttagatatccgttctggccagtctctcgggcaaatattctctctcggaccctttgatattcctcctctctctcttctattgacttgctcctccttccatcctgcaatggaactctgatctggttatcatctcggtccatactggcatcatctctcttgagaatgaacctctgttgaaattctgtattcttctcatcctttatatgttctgagaacctctgttcagggattcttgtgttactagttttgttgatgatgacagctttcccagtttgatcaacattgtggtccatcccaaaataggcagctacccggtgtaatagcatccggtgatatgaggtcatctgagggaacttcttgaactgattattgttgtcattaataaattccagaatctcctgttctaattttagcagcatcattctgtccctgtttaaaaaagattaaaacaaaacaaaacaaaacaaaaagcagccctcccatagacattgaaagtggggattgaaaacacaacttgctcattacagaagctgaaaaaggtatatatccaaacccagtaatgaaccataatgctgctaagcctcacttgcctgttttacaatatttttaaaaagaaaaacaacccgagtatacattttgcaggtcctccaatcatatactttgttataccatatcagaaatctcactgttaacaacatattcatataaacacacgttataaatctaatcgtcattctgtattccatcttgttataaacaattttaaaggaattataatttagcttatgtacaaatcaattattttttccttctgtgctttttattttagctcttcttactatcactcccaatgtgtgctttttaatcagtatactcccaagacttcatatttctttgtttctgcattcttctttcacagaagttttcccaattcttctgaaaacagaaacctcaatgtgagagtattttgaatccctcacagaatataaaactatacctgacaaatactagggggacaggaagatgagcatcctagattctaagaatggaaaaattctgggaagccgtttggcctcttggaatcttgctatcccctaaccccttttcctcttatacccatcatgttattaccttgggttctttttcagtgtatttacaagaaattcatgtaggtctattccagtggagtccgtatattcctggctggagtctctggacagcatcttccttgggatcttttctttgtttttgtccttgtcttccttttcagagacatcttttgtggacttttcttcctccttgtcagaagggcaactgatgtgcaattgaattatatcctgggtttctaatggcccatcagcaaatggggtggaggactcctcacacactgccaggctacgcaccaactttagcttggaattagacttggctcttttcctggcatgaccatggttagatgtccgcctctgtgtctcctgacgcaaactggtatcttcacattctttctcaatttcttccttacttggagtcttagatataaacttgtttttgtttacagattcttccaccagttttttttctgattctttcattatttccagggtctcttgagtagtgttactgttagacatgttcttcaatagaatacagtggcctctatggactcctgaataaatgctcagcctccatgagtccagtgctggaatggcatcacatataagaaacaagtctaacctctcgcacgggccttggcggggagggcgcccacgtctccgcccgccgcccgggcccacggccgctcggctgcggctcggccccgacggccggcggc

SEQ ID NO: 17330 - RNA, 4008 nt, Homo sapiens
  source 1..4008: mol_type = other RNA
tcaggccaggcacagtggctcacgcctgtaatcccagcactctggaaggccaaggcaggtggatcacctgaggtcaggagtttgaggccagcctggccaacatggtgaaactccgtctctactaaaaatacaaaaattagccgggcatggtggcgcgtgtctgtagtgccagctacttgggaggctgaggcaggagaatcacctgaacccaggagctggaggttgcagttagccaagatcgtgctactgcactccagctggggtgacaagagcgaaactccgtctcaaaaaaaaaaaaaaaaaaaaaaagaagaggatgggaagaagagtgatgcaaggggggtcaaccagggaaaaagagaggacccatggcaggggagcaagaaggagtccaatgccagtgtaggtatctgtgtttccatcttcatcactgtcttaggttccagtttaacatcagtttccttacttcctgcctctgtccatggtctgtcaggatccttcaaccccctccaccctgcccttgctccttctgtgacagtccctttcccctcctccatttattgggagctggctcgctccaggatcctcaggtcatagttctttttggccattcgaagtttgaagcgactcacggagttgttgagacgaagggaggcattttgggcagccagggggctggggaacacagccacaatggtgtacaaggcagcgaggtccgagtggcggccattctcagcagtcccactgttgtcccccccaccccctccaggcagcccctgagcatccttgagccactggatcttggcgccagacatggcgagctgcgtgaagagtttgtccgcctcagtacgggtgatgccctcagggagatctgtcacctccagcacccgccccaggacaacatctgctgtccccaggtcagtggaggcagatttgagtgcttgtctcttgccccggtttccatgcttcagtccactctgtccctggtgcaccgtgtaagttgactggccatggagcaagggagggcagatggacagattgtactgtaatggctggcccaaaagggagtagcgcccatcaccctgtgctggacccccaggccgggggaactgtgtgaggacaggcaggggactgagtcctgtgcagacactgctgaggctggtgacaggagagggtgctggagactgggtaggagatgtgacagggctgctgctcatttgtgtgttggcctgggggctgctgtcaggactgtacaggtctccaggcttctgcccccgctggtccatgctgtagtatttacaatgactccactggaccatggatgggttctgagggggctggggtccattagggacattcagctgcatgaccactacacctggtccagaaggtgacactcctgagtactgctgtggcatctgtggtggactgcagggagagggagactgaggcatctggtactgctcagagccagggggttgcagaaaccctacagaagggctcgtaccgttctgctgagcaggtgggatcatgctatagtacactggtacccccgctgctgggaggcctccttgcacagactggctcacagggaccagcatgggttgctggaaaggcggctggaccacattttgcgagtcactacccactggaacttggtaagaaggcagtggagtgtactgaaccaccaggccttgcatctggccccccatgctgctcctctggctgctgagcaggccctggttctgtggctgctggaccccaatcatgccttggtaagccgcctgctgctggttaggcatcatgggctgtaaaccaggctgctgggatggctgaggcagctgctgaccacgttgggggctataggccaccgggtgagagagaggtcgatattgctggttggagttaggatattgtccagggggatagtaagaaacctggatctgttgagggggctgcatgtacccctggggtggcagaacttgctgagtaggtggtgcatggctagaggtggaatagttggaagtggggaggggctgacccgtggaagccatgatgaagctagtctgctgagggtgctgggagataagtggggtctggaatagagctgcagatgggtcagctgcttcagtagaaccttggcgactaaggctcatttgtccaaaggggttgctgaggtcatctgcctgtgagatcatgtgattattcaagggtggctgttgctgaggcgtgggtgggagagcaggaagttgctgctgctgctgctgctgttgctgctgggcagtacaagggagaagcccccggacagactgggatgaggtgacctggttgcacacttctggggcacctagtgccatacctggcctggagatccttcccgcactgccgcctttactgctgccgatgctgtcacctcgggtaaggatagagattccactgaagctgctagctttggtgacagggggtcgcatgctccggacagagccatcagagtctgtgctgctccaagggcgtggctccagggatttgagttcgctgtctgtgctgctctggcggctgcttgaggtgcggctcagtccttcacggttccccctaaaaatctgccttctcttgtgagagctagaagaaaaggcttctttggagagtctgatgtcatttagatatccgttctggccagtctctcgggcaaatattctctctcggaccctttgatattcctcctctctctcttctattgacttgctcctccttccatcctgcaatggaactctgatctggttatcatctcggtccatactggcatcatctctcttgagaatgaacctctgttgaaattctgtattcttctcatcctttatatgttctgagaacctctgttcagggattcttgtgttactagttttgttgatgatgacagctttcccagtttgatcaacattgtggtccatcccaaaataggcagctacccggtgtaatagcatccggtgatatgaggtcatctgagggaacttcttgaactgattattgttgtcattaataaattccagaatctcctgttctaattttagcagcatcattctgtcccttgggttctttttcagtgtatttacaagaaattcatgtaggtctattccagtggagtccgtatattcctggctggagtctctggacagcatcttccttgggatcttttctttgtttttgtccttgtcttccttttcagagacatcttttgtggacttttcttcctccttgtcagaagggcaactgatgtgcaattgaattatatcctgggtttctaatggcccatcagcaaatggggtggaggactcctcacacactgccaggctacgcaccaactttagcttggaattagacttggctcttttcctggcatgaccatggttagatgtccgcctctgtgtctcctgacgcaaactggtatcttcacattctttctcaatttcttccttacttggagtcttagatataaacttgtttttgtttacagattcttccaccagttttttttctgattctttcattatttccagggtctcttgagtagtgttactgttagacatgttcttcaatagaatacagtggcctctatggactccgcttcagatggatttttcttcttccttctctccgtcccctccctctcagaagaaaaagactgcaaacaaaatcactacgtcactggaggtagagggaatcccatctctgcactctttagaagccaaggccagcaaataaaaacaagccaattataagaaaaagtaatacaaaataagaataaataaacccagaagaaatccatgtgacaatctcaacacatcaaaaggcattttttagtaaaaaggttttaacaaatgcctcctaggatgttcataatcaaaaaatctccccagacatagcaaaggcttatcacatttaaagactaggggatagttacgtaaagatataggacagacaggcacattcaccagccaggtgcggatagct

SEQ ID NO: 17331 - RNA, 3689 nt, Homo sapiens
  source 1..3689: mol_type = other RNA
tcaggccaggcacagtggctcacgcctgtaatcccagcactctggaaggccaaggcaggtggatcacctgaggtcaggagtttgaggccagcctggccaacatggtgaaactccgtctctactaaaaatacaaaaattagccgggcatggtggcgcgtgtctgtagtgccagctacttgggaggctgaggcaggagaatcacctgaacccaggagctggaggttgcagttagccaagatcgtgctactgcactccagctggggtgacaagagcgaaactccgtctcaaaaaaaaaaaaaaaaaaaaaaagaagaggatgggaagaagagtgatgcaaggggggtcaaccagggaaaaagagaggacccatggcaggggagcaagaaggagtccaatgccagtgtaggtatctgtgtttccatcttcatcactgtcttaggttccagtttaacatcagtttccttacttcctgcctctgtccatggtctgtcaggatccttcaaccccctccaccctgcccttgctccttctgtgacagtccctttcccctcctccatttattgggagctggctcgctccaggatcctcaggtcatagttctttttggccattcgaagtttgaagcgactcacggagttgttgagacgaagggaggcattttgggcagccagggggctggggaacacagccacaatggtgtacaaggcagcgaggtccgagtggcggccattctcagcagtcccactgttgtcccccccaccccctccaggcagcccctgagcatccttgagccactggatcttggcgccagacatggcgagctgcgtgaagagtttgtccgcctcagtacgggtgatgccctcagggagatctgtcacctccagcacccgccccaggacaacatctgctgtccccaggtcagtggaggcagatttgagtgcttgtctcttgccccggtttccatgcttcagtccactctgtccctggtgcaccgtgtaagttgactggccatggagcaagggagggcagatggacagattgtactgtaatggctggcccaaaagggagtagcgcccatcaccctgtgctggacccccaggccgggggaactgtgtgaggacaggcaggggactgagtcctgtgcagacactgctgaggctggtgacaggagagggtgctggagactgggtaggagatgtgacagggctgctgctcatttgtgtgttggcctgggggctgctgtcaggactgtacaggtctccaggcttctgcccccgctggtccatgctgtagtatttacaatgactccactggaccatggatgggttctgagggggctggggtccattagggacattcagctgcatgaccactacacctggtccagaaggtgacactcctgagtactgctgtggcatctgtggtggactgcagggagagggagactgaggcatctggtactgctcagagccagggggttgcagaaaccctacagaagggctcgtaccgttctgctgagcaggtgggatcatgctatagtacactggtacccccgctgctgggaggcctccttgcacagactggctcacagggaccagcatgggttgctggaaaggcggctggaccacattttgcgagtcactacccactggaacttggtaagaaggcagtggagtgtactgaaccaccaggccttgcatctggccccccatgctgctcctctggctgctgagcaggccctggttctgtggctgctggaccccaatcatgccttggtaagccgcctgctgctggttaggcatcatgggctgtaaaccaggctgctgggatggctgaggcagctgctgaccacgttgggggctataggccaccgggtgagagagaggtcgatattgctggttggagttaggatattgtccagggggatagtaagaaacctggatctgttgagggggctgcatgtacccctggggtggcagaacttgctgagtaggtggtgcatggctagaggtggaatagttggaagtggggaggggctgacccgtggaagccatgatgaagctagtctgctgagggtgctgggagataagtggggtctggaatagagctgcagatgggtcagctgcttcagtagaaccttggcgactaaggctcatttgtccaaaggggttgctgaggtcatctgcctgtgagatcatgtgattattcaagggtggctgttgctgaggcgtgggtgggagagcaggaagttgctgctgctgctgctgctgttgctgctgggcagtacaagggagaagcccccggacagactgggatgaggtgacctggttgcacacttctggggcacctagtgccatacctggcctggagatccttcccgcactgccgcctttactgctgccgatgctgtcacctcgggtaaggatagagattccactgaagctgctagctttggtgacagggggtcgcatgctccggacagagccatcagagtctgtgctgctccaagggcgtggctccagggatttgagttcgctgtctgtgctgctctggcggctgcttgaggtgcggctcagtccttcacggttccccctaaaaatctgccttctcttgtgagagctagaagaaaaggcttctttggagagtctgatgtcatttagatatccgttctggccagtctctcgggcaaatattctctctcggaccctttgatattcctcctctctctcttctattgacttgctcctccttccatcctgcaatggaactctgatctggttatcatctcggtccatactggcatcatctctcttgagaatgaacctctgttgaaattctgtattcttctcatcctttatatgttctgagaacctctgttcagggattcttgtgttactagttttgttgatgatgacagctttcccagtttgatcaacattgtggtccatcccaaaataggcagctacccggtgtaatagcatccggtgatatgaggtcatctgagggaacttcttgaactgattattgttgtcattaataaattccagaatctcctgttctaattttagcagcatcattctgtcccttgggttctttttcagtgtatttacaagaaattcatgtaggtctattccagtggagtccgtatattcctggctggagtctctggacagcatcttccttgggatcttttctttgtttttgtccttgtcttccttttcagagacatcttttgtggacttttcttcctccttgtcagaagggcaactgatgtgcaattgaattatatcctgggtttctaatggcccatcagcaaatggggtggaggactcctcacacactgccaggctacgcaccaactttagcttggaattagacttggctcttttcctggcatgaccatggttagatgtccgcctctgtgtctcctgacgcaaactggtatcttcacattctttctcaatttcttccttacttggagtcttagatataaacttgtttttgtttacagattcttccaccagttttttttctgattctttcattatttccagggtctcttgagtagtgttactgttagacatgttcttcaatagaatacagtggcctctatggactcctgaataaatgctcagcctccatgagtccagtgctggaatggcatcacatataagaaacaagtctaacct

SEQ ID NO: 17332 - RNA, 3713 nt, Homo sapiens
  source 1..3713: mol_type = other RNA
tcaggccaggcacagtggctcacgcctgtaatcccagcactctggaaggccaaggcaggtggatcacctgaggtcaggagtttgaggccagcctggccaacatggtgaaactccgtctctactaaaaatacaaaaattagccgggcatggtggcgcgtgtctgtagtgccagctacttgggaggctgaggcaggagaatcacctgaacccaggagctggaggttgcagttagccaagatcgtgctactgcactccagctggggtgacaagagcgaaactccgtctcaaaaaaaaaaaaaaaaaaaaaaagaagaggatgggaagaagagtgatgcaaggggggtcaaccagggaaaaagagaggacccatggcaggggagcaagaaggagtccaatgccagtgtaggtatctgtgtttccatcttcatcactgtcttaggttccagtttaacatcagtttccttacttcctgcctctgtccatggtctgtcaggatccttcaaccccctccaccctgcccttgctccttctgtgacagtccctttcccctcctccatttattgggagctggctcgctccaggatcctcaggtcatagttctttttggccattcgaagtttgaagcgactcacggagttgttgagacgaagggaggcattttgggcagccagggggctggggaacacagccacaatggtgtacaaggcagcgaggtccgagtggcggccattctcagcagtcccactgttgtcccccccaccccctccaggcagcccctgagcatccttgagccactggatcttggcgccagacatggcgagctgcgtgaagagtttgtccgcctcagtacgggtgatgccctcagggagatctgtcacctccagcacccgccccaggacaacatctgctgtccccaggtcagtggaggcagatttgagtgcttgtctcttgccccggtttccatgcttcagtccactctgtccctggtgcaccgtgtaagttgactggccatggagcaagggagggcagatggacagattgtactgtaatggctggcccaaaagggagtagcgcccatcaccctgtgctggacccccaggccgggggaactgtgtgaggacaggcaggggactgagtcctgtgcagacactgctgaggctggtgacaggagagggtgctggagactgggtaggagatgtgacagggctgctgctcatttgtgtgttggcctgggggctgctgtcaggactgtacaggtctccaggcttctgcccccgctggtccatgctgtagtatttacaatgactccactggaccatggatgggttctgagggggctggggtccattagggacattcagctgcatgaccactacacctggtccagaaggtgacactcctgagtactgctgtggcatctgtggtggactgcagggagagggagactgaggcatctggtactgctcagagccagggggttgcagaaaccctacagaagggctcgtaccgttctgctgagcaggtgggatcatgctatagtacactggtacccccgctgctgggaggcctccttgcacagactggctcacagggaccagcatgggttgctggaaaggcggctggaccacattttgcgagtcactacccactggaacttggtaagaaggcagtggagtgtactgaaccaccaggccttgcatctggccccccatgctgctcctctggctgctgagcaggccctggttctgtggctgctggaccccaatcatgccttggtaagccgcctgctgctggttaggcatcatgggctgtaaaccaggctgctgggatggctgaggcagctgctgaccacgttgggggctataggccaccgggtgagagagaggtcgatattgctggttggagttaggatattgtccagggggatagtaagaaacctggatctgttgagggggctgcatgtacccctggggtggcagaacttgctgagtaggtggtgcatggctagaggtggaatagttggaagtggggaggggctgacccgtggaagccatgatgaagctagtctgctgagggtgctgggagataagtggggtctggaatagagctgcagatgggtcagctgcttcagtagaaccttggcgactaaggctcatttgtccaaaggggttgctgaggtcatctgcctgtgagatcatgtgattattcaagggtggctgttgctgaggcgtgggtgggagagcaggaagttgctgctgctgctgctgctgttgctgctgggcagtacaagggagaagcccccggacagactgggatgaggtgacctggttgcacacttctggggcacctagtgccatacctggcctggagatccttcccgcactgccgcctttactgctgccgatgctgtcacctcgggtaaggatagagattccactgaagctgctagctttggtgacagggggtcgcatgctccggacagagccatcagagtctgtgctgctccaagggcgtggctccagggatttgagttcgctgtctgtgctgctctggcggctgcttgaggtgcggctcagtccttcacggttccccctaaaaatctgccttctcttgtgagagctagaagaaaaggcttctttggagagtctgatgtcatttagatatccgttctggccagtctctcgggcaaatattctctctcggaccctttgatattcctcctctctctcttctattgacttgctcctccttccatcctgcaatggaactctgatctggttatcatctcggtccatactggcatcatctctcttgagaatgaacctctgttgaaattctgtattcttctcatcctttatatgttctgagaacctctgttcagggattcttgtgttactagttttgttgatgatgacagctttcccagtttgatcaacattgtggtccatcccaaaataggcagctacccggtgtaatagcatccggtgatatgaggtcatctgagggaacttcttgaactgattattgttgtcattaataaattccagaatctcctgttctaattttagcagcatcattctgtcccttgggttctttttcagtgtatttacaagaaattcatgtaggtctattccagtggagtccgtatattcctggctggagtctctggacagcatcttccttgggatcttttctttgtttttgtccttgtcttccttttcagagacatcttttgtggacttttcttcctccttgtcagaagggcaactgatgtgcaattgaattatatcctgggtttctaatggcccatcagcaaatggggtggaggactcctcacacactgccaggctacgcaccaactttagcttggaattagacttggctcttttcctggcatgaccatggttagatgtccgcctcttgtcaaaaaggaactcataatcctgtgtctcctgacgcaaactggtatcttcacattctttctcaatttcttccttacttggagtcttagatataaacttgtttttgtttacagattcttccaccagttttttttctgattctttcattatttccagggtctcttgagtagtgttactgttagacatgttcttcaatagaatacagtggcctctatggactcctgaataaatgctcagcctccatgagtccagtgctggaatggcatcacatataagaaacaagtctaacct

SEQ ID NO: 17333 - RNA, 3917 nt, Homo sapiens
  source 1..3917: mol_type = other RNA
tcaggccaggcacagtggctcacgcctgtaatcccagcactctggaaggccaaggcaggtggatcacctgaggtcaggagtttgaggccagcctggccaacatggtgaaactccgtctctactaaaaatacaaaaattagccgggcatggtggcgcgtgtctgtagtgccagctacttgggaggctgaggcaggagaatcacctgaacccaggagctggaggttgcagttagccaagatcgtgctactgcactccagctggggtgacaagagcgaaactccgtctcaaaaaaaaaaaaaaaaaaaaaaagaagaggatgggaagaagagtgatgcaaggggggtcaaccagggaaaaagagaggacccatggcaggggagcaagaaggagtccaatgccagtgtaggtatctgtgtttccatcttcatcactgtcttaggttccagtttaacatcagtttccttacttcctgcctctgtccatggtctgtcaggatccttcaaccccctccaccctgcccttgctccttctgtgacagtccctttcccctcctccatttattgggagctggctcgctccaggatcctcaggtcatagttctttttggccattcgaagtttgaagcgactcacggagttgttgagacgaagggaggcattttgggcagccagggggctggggaacacagccacaatggtgtacaaggcagcgaggtccgagtggcggccattctcagcagtcccactgttgtcccccccaccccctccaggcagcccctgagcatccttgagccactggatcttggcgccagacatggcgagctgcgtgaagagtttgtccgcctcagtacgggtgatgccctcagggagatctgtcacctccagcacccgccccaggacaacatctgctgtccccaggtcagtggaggcagatttgagtgcttgtctcttgccccggtttccatgcttcagtccactctgtccctggtgcaccgtgtaagttgactggccatggagcaagggagggcagatggacagattgtactgtaatggctggcccaaaagggagtagcgcccatcaccctgtgctggacccccaggccgggggaactgtgtgaggacaggcaggggactgagtcctgtgcagacactgctgaggctggtgacaggagagggtgctggagactgggtaggagatgtgacagggctgctgctcatttgtgtgttggcctgggggctgctgtcaggactgtacaggtctccaggcttctgcccccgctggtccatgctgtagtatttacaatgactccactggaccatggatgggttctgagggggctggggtccattagggacattcagctgcatgaccactacacctggtccagaaggtgacactcctgagtactgctgtggcatctgtggtggactgcagggagagggagactgaggcatctggtactgctcagagccagggggttgcagaaaccctacagaagggctcgtaccgttctgctgagcaggtgggatcatgctatagtacactggtacccccgctgctgggaggcctccttgcacagactggctcacagggaccagcatgggttgctggaaaggcggctggaccacattttgcgagtcactacccactggaacttggtaagaaggcagtggagtgtactgaaccaccaggccttgcatctggccccccatgctgctcctctggctgctgagcaggccctggttctgtggctgctggaccccaatcatgccttggtaagccgcctgctgctggttaggcatcatgggctgtaaaccaggctgctgggatggctgaggcagctgctgaccacgttgggggctataggccaccgggtgagagagaggtcgatattgctggttggagttaggatattgtccagggggatagtaagaaacctggatctgttgagggggctgcatgtacccctggggtggcagaacttgctgagtaggtggtgcatggctagaggtggaatagttggaagtggggaggggctgacccgtggaagccatgatgaagctagtctgctgagggtgctgggagataagtggggtctggaatagagctgcagatgggtcagctgcttcagtagaaccttggcgactaaggctcatttgtccaaaggggttgctgaggtcatctgcctgtgagatcatgtgattattcaagggtggctgttgctgaggcgtgggtgggagagcaggaagttgctgctgctgctgctgctgttgctgctgggcagtacaagggagaagcccccggacagactgggatgaggtgacctggttgcacacttctggggcacctagtgccatacctggcctggagatccttcccgcactgccgcctttactgctgccgatgctgtcacctcgggtaaggatagagattccactgaagctgctagctttggtgacagggggtcgcatgctccggacagagccatcagagtctgtgctgctccaagggcgtggctccagggatttgagttcgctgtctgtgctgctctggcggctgcttgaggtgcggctcagtccttcacggttccccctaaaaatctgccttctcttgtgagagctagaagaaaaggcttctttggagagtctgatgtcatttagatatccgttctggccagtctggttatcatctcggtccatactggcatcatctctcttgagaatgaacctctgttgaaattctgtattcttctcatcctttatatgttctgagaacctctgttcagggattcttgtgttactagttttgttgatgatgacagctttcccagtttgatcaacattgtggtccatcccaaaataggcagctacccggtgtaatagcatccggtgatatgaggtcatctgagggaacttcttgaactgattattgttgtcattaataaattccagaatctcctgttctaattttagcagcatcattctgtcccttgggttctttttcagtgtatttacaagaaattcatgtaggtctattccagtggagtccgtatattcctggctggagtctctggacagcatcttccttgggatcttttctttgtttttgtccttgtcttccttttcagagacatcttttgtggacttttcttcctccttgtcagaagggcaactgatgtgcaattgaattatatcctgggtttctaatggcccatcagcaaatggggtggaggactcctcacacactgccaggctacgcaccaactttagcttggaattagacttggctcttttcctggcatgaccatggttagatgtccgcctctgtgtctcctgacgcaaactggtatcttcacattctttctcaatttcttccttacttggagtcttagatataaacttgtttttgtttacagattcttccaccagttttttttctgattctttcattatttccagggtctcttgagtagtgttactgttagacatgttcttcaatagaatacagtggcctctatggactcctgaataaatgctcagcctccatgagtccagtgctggaatggcatcacatataagaaacaagtctaacctctcgcacgggccttggcggggagggcgcccacgtctccgcccgccgcccgggcccacggccgctcggctgcggctcggccccgacggccggcggcggcgcgcttctgggggcgggcttttctcggccggggcttccccggggccgagggctgggaagcaggggggactgggacgggggaggggaaaggggcttgggaaggaggggggagaggggaagaaaaggggggaaccaaacccggaaagggagaaaaggggggaggggaaaatcagaaggggaagaaaagcccagagtccgccccccgctgcggctgcgcgctacgtcac

SEQ ID NO: 17334 - RNA, 3617 nt, Homo sapiens
  source 1..3617: mol_type = other RNA
tcaggccaggcacagtggctcacgcctgtaatcccagcactctggaaggccaaggcaggtggatcacctgaggtcaggagtttgaggccagcctggccaacatggtgaaactccgtctctactaaaaatacaaaaattagccgggcatggtggcgcgtgtctgtagtgccagctacttgggaggctgaggcaggagaatcacctgaacccaggagctggaggttgcagttagccaagatcgtgctactgcactccagctggggtgacaagagcgaaactccgtctcaaaaaaaaaaaaaaaaaaaaaaagaagaggatgggaagaagagtgatgcaaggggggtcaaccagggaaaaagagaggacccatggcaggggagcaagaaggagtccaatgccagtgtaggtatctgtgtttccatcttcatcactgtcttaggttccagtttaacatcagtttccttacttcctgcctctgtccatggtctgtcaggatccttcaaccccctccaccctgcccttgctccttctgtgacagtccctttcccctcctccatttattgggagctggctcgctccaggatcctcaggtcatagttctttttggccattcgaagtttgaagcgactcacggagttgttgagacgaagggaggcattttgggcagccagggggctggggaacacagccacaatggtgtacaaggcagcgaggtccgagtggcggccattctcagcagtcccactgttgtcccccccaccccctccaggcagcccctgagcatccttgagccactggatcttggcgccagacatggcgagctgcgtgaagagtttgtccgcctcagtacgggtgatgccctcagggagatctgtcacctccagcacccgccccaggacaacatctgctgtccccaggtcagtggaggcagatttgagtgcttgtctcttgccccggtttccatgcttcagtccactctgtccctggtgcaccgtgtaagttgactggccatggagcaagggagggcagatggacagattgtactgtaatggctggcccaaaagggagtagcgcccatcaccctgtgctggacccccaggccgggggaactgtgtgaggacaggcaggggactgagtcctgtgcagacactgctgaggctggtgacaggagagggtgctggagactgggtaggagatgtgacagggctgctgctcatttgtgtgttggcctgggggctgctgtcaggactgtacaggtctccaggcttctgcccccgctggtccatgctgtagtatttacaatgactccactggaccatggatgggttctgagggggctggggtccattagggacattcagctgcatgaccactacacctggtccagaaggtgacactcctgagtactgctgtggcatctgtggtggactgcagggagagggagactgaggcatctggtactgctcagagccagggggttgcagaaaccctacagaagggctcgtaccgttctgctgagcaggtgggatcatgctatagtacactggtacccccgctgctgggaggcctccttgcacagactggctcacagggaccagcatgggttgctggaaaggcggctggaccacattttgcgagtcactacccactggaacttggtaagaaggcagtggagtgtactgaaccaccaggccttgcatctggccccccatgctgctcctctggctgctgagcaggccctggttctgtggctgctggaccccaatcatgccttggtaagccgcctgctgctggttaggcatcatgggctgtaaaccaggctgctgggatggctgaggcagctgctgaccacgttgggggctataggccaccgggtgagagagaggtcgatattgctggttggagttaggatattgtccagggggatagtaagaaacctggatctgttgagggggctgcatgtacccctggggtggcagaacttgctgagtaggtggtgcatggctagaggtggaatagttggaagtggggaggggctgacccgtggaagccatgatgaagctagtctgctgagggtgctgggagataagtggggtctggaatagagctgcagatgggtcagctgcttcagtagaaccttggcgactaaggctcatttgtccaaaggggttgctgaggtcatctgcctgtgagatcatgtgattattcaagggtggctgttgctgaggcgtgggtgggagagcaggaagttgctgctgctgctgctgctgttgctgctgggcagtacaagggagaagcccccggacagactgggatgaggtgacctggttgcacacttctggggcacctagtgccatacctggcctggagatccttcccgcactgccgcctttactgctgccgatgctgtcacctcgggtaaggatagagattccactgaagctgctagctttggtgacagggggtcgcatgctccggacagagccatcagagtctgtgctgctccaagggcgtggctccagggatttgagttcgctgtctgtgctgctctggcggctgcttgaggtgcggctcagtccttcacggttccccctaaaaatctgccttctcttgtgagagctagaagaaaaggcttctttggagagtctgatgtcatttagatatccgttctggccagtctggttatcatctcggtccatactggcatcatctctcttgagaatgaacctctgttgaaattctgtattcttctcatcctttatatgttctgagaacctctgttcagggattcttgtgttactagttttgttgatgatgacagctttcccagtttgatcaacattgtggtccatcccaaaataggcagctacccggtgtaatagcatccggtgatatgaggtcatctgagggaacttcttgaactgattattgttgtcattaataaattccagaatctcctgttctaattttagcagcatcattctgtcccttgggttctttttcagtgtatttacaagaaattcatgtaggtctattccagtggagtccgtatattcctggctggagtctctggacagcatcttccttgggatcttttctttgtttttgtccttgtcttccttttcagagacatcttttgtggacttttcttcctccttgtcagaagggcaactgatgtgcaattgaattatatcctgggtttctaatggcccatcagcaaatggggtggaggactcctcacacactgccaggctacgcaccaactttagcttggaattagacttggctcttttcctggcatgaccatggttagatgtccgcctcttgtcaaaaaggaactcataatcctgtgtctcctgacgcaaactggtatcttcacattctttctcaatttcttccttacttggagtcttagatataaacttgtttttgtttacagattcttccaccagttttttttctgattctttcattatttccagggtctcttgagtagtgttactgttagacatgttcttcaatagaatacagtggcctctatggactcctgaataaatgctcagcctccatgagtccagtgctggaatggcatcacatataagaaacaagtctaacct

SEQ ID NO: 17335 - RNA, 2754 nt, Homo sapiens
  source 1..2754: mol_type = other RNA
tcaggccaggcacagtggctcacgcctgtaatcccagcactctggaaggccaaggcaggtggatcacctgaggtcaggagtttgaggccagcctggccaacatggtgaaactccgtctctactaaaaatacaaaaattagccgggcatggtggcgcgtgtctgtagtgccagctacttgggaggctgaggcaggagaatcacctgaacccaggagctggaggttgcagttagccaagatcgtgctactgcactccagctggggtgacaagagcgaaactccgtctcaaaaaaaaaaaaaaaaaaaaaaagaagaggatgggaagaagagtgatgcaaggggggtcaaccagggaaaaagagaggacccatggcaggggagcaagaaggagtccaatgccagtgtaggtatctgtgtttccatcttcatcactgtcttaggttccagtttaacatcagtttccttacttcctgcctctgtccatggtctgtcaggatccttcaaccccctccaccctgcccttgctccttctgtgacagtccctttcccctcctccatttattgggagctggctcgctccaggatcctcaggtcatagttctttttggccattcgaagtttgaagcgactcacggagttgttgagacgaagggaggcattttgggcagccagggggctggggaacacagccacaatggtgtacaaggcagcgaggtccgagtggcggccattctcagcagtcccactgttgtcccccccaccccctccaggcagcccctgagcatccttgagccactggatcttggcgccagacatggcgagctgcgtgaagagtttgtccgcctcagtacgggtgatgccctcagggagatctgtcacctccagcacccgccccaggacaacatctgctgtccccaggtcagtggaggcagatttgagtgcttgtctcttgccccggtttccatgcttcagtccactctgtccctggtgcaccgtgtaagttgactggccatggagcaagggagggcagatggacagattgtactgtaatggctggcccaaaagggagtagcgcccatcaccctgtgctggacccccaggccgggggaactgtgtgaggacaggcaggggactgagtcctgtgcagacactgctgaggctggtgacaggagagggtgctggagactgggtaggagatgtgacagggctgctgctcatttgtgtgttggcctgggggctgctgtcaggactgtacaggtctccaggcttctgcccccgctggtccatgctgtagtatttacaatgactccactggaccatggatgggttctgagggggctggggtccattagggacattcagctgcatgaccactacacctggtccagaaggtgacactcctgagtactgctgtggcatctgtggtggactgcagggagagggagactgaggcatctggtactgctcagagccagggggttgcagaaaccctacagaagggctcgtaccgttctgctgagcaggtgggatcatgctatagtacactggtacccccgctgctgggaggcctccttgcacagactggctcacagggaccagcatgggttgctggaaaggcggctggaccacattttgcgagtcactacccactggaacttggtaagaaggcagtggagtgtactgaaccaccaggccttgcatctggccccccatgctgctcctctggctgctgagcaggccctggttctgtggctgctggaccccaatcatgccttggtaagccgcctgctgctggttaggcatcatgggctgtaaaccaggctgctgggatggctgaggcagctgctgaccacgttgggggctataggccaccgggtgagagagaggtcgatattgctggttggagttaggatattgtccagggggatagtaagaaacctggatctgttgagggggctgcatgtacccctggggtggcagaacttgctgagtaggtggtgcatggctagaggtggaatagttggaagtggggaggggctgacccgtggaagccatgatgaagctagtctgctgagggtgctgggagataagtggggtctggaatagagctgcagatgggtcagctgcttcagtagaaccttggcgactaaggctcatttgtccaaaggggttgctgaggtcatctgcctgtgagatcatgtgattattcaagggtggctgttgctgaggcgtgggtgggagagcaggaagttgctgctgctgctgctgctgttgctgctgggcagtacaagggagaagcccccggacagactgggatgaggtgacctggttgcacacttctggggcacctagtgccatacctggcctggagatccttcccgcactgccgcctttactgctgccgatgctgtcacctcgggtaaggatagagattccactgaagctgctagctttggtgacagggggtcgcatgctccggacagagccatcagagtctgtgctgctccaagggcgtggctccagggatttgagttcgctgtctgtgctgctctggcggctgcttgaggtgcggctcagtccttcacggttccccctctcgggcaaatattctctctcggaccctttgatattcctcctctctctcttctattgacttgctcctccttccatcctgcaatggaactctgatctggttatcatctcggtccatactggcatcatctctcttgagaatgaacctctgttgaaattctgt

SEQ ID NO: 17336 - RNA, 2905 nt, Homo sapiens
  source 1..2905: mol_type = other RNA
tcaggccaggcacagtggctcacgcctgtaatcccagcactctggaaggccaaggcaggtggatcacctgaggtcaggagtttgaggccagcctggccaacatggtgaaactccgtctctactaaaaatacaaaaattagccgggcatggtggcgcgtgtctgtagtgccagctacttgggaggctgaggcaggagaatcacctgaacccaggagctggaggttgcagttagccaagatcgtgctactgcactccagctggggtgacaagagcgaaactccgtctcaaaaaaaaaaaaaaaaaaaaaaagaagaggatgggaagaagagtgatgcaaggggggtcaaccagggaaaaagagaggacccatggcaggggagcaagaaggagtccaatgccagtgtaggtatctgtgtttccatcttcatcactgtcttaggttccagtttaacatcagtttccttacttcctgcctctgtccatggtctgtcaggatccttcaaccccctccaccctgcccttgctccttctgtgacagtccctttcccctcctccatttattgggagctggctcgctccaggatcctcaggtcatagttctttttggccattcgaagtttgaagcgactcacggagttgttgagacgaagggaggcattttgggcagccagggggctggggaacacagccacaatggtgtacaaggcagcgaggtccgagtggcggccattctcagcagtcccactgttgtcccccccaccccctccaggcagcccctgagcatccttgagccactggatcttggcgccagacatggcgagctgcgtgaagagtttgtccgcctcagtacgggtgatgccctcagggagatctgtcacctccagcacccgccccaggacaacatctgctgtccccaggtcagtggaggcagatttgagtgcttgtctcttgccccggtttccatgcttcagtccactctgtccctggtgcaccgtgtaagttgactggccatggagcaagggagggcagatggacagattgtactgtaatggctggcccaaaagggagtagcgcccatcaccctgtgctggacccccaggccgggggaactgtgtgaggacaggcaggggactgagtcctgtgcagacactgctgaggctggtgacaggagagggtgctggagactgggtaggagatgtgacagggctgctgctcatttgtgtgttggcctgggggctgctgtcaggactgtacaggtctccaggcttctgcccccgctggtccatgctgtagtatttacaatgactccactggaccatggatgggttctgagggggctggggtccattagggacattcagctgcatgaccactacacctggtccagaaggtgacactcctgagtactgctgtggcatctgtggtggactgcagggagagggagactgaggcatctggtactgctcagagccagggggttgcagaaaccctacagaagggctcgtaccgttctgctgagcaggtgggatcatgctatagtacactggtacccccgctgctgggaggcctccttgcacagactggctcacagggaccagcatgggttgctggaaaggcggctggaccacattttgcgagtcactacccactggaacttggtaagaaggcagtggagtgtactgaaccaccaggccttgcatctggccccccatgctgctcctctggctgctgagcaggccctggttctgtggctgctggaccccaatcatgccttggtaagccgcctgctgctggttaggcatcatgggctgtaaaccaggctgctgggatggctgaggcagctgctgaccacgttgggggctataggccaccgggtgagagagaggtcgatattgctggttggagttaggatattgtccagggggatagtaagaaacctggatctgttgagggggctgcatgtacccctggggtggcagaacttgctgagtaggtggtgcatggctagaggtggaatagttggaagtggggaggggctgacccgtggaagccatgatgaagctagtctgctgagggtgctgggagataagtggggtctggaatagagctgcagatgggtcagctgcttcagtagaaccttggcgactaaggctcatttgtccaaaggggttgctgaggtcatctgcctgtgagatcatgtgattattcaagggtggctgttgctgaggcgtgggtgggagagcaggaagttgctgctgctgctgctgctgttgctgctgggcagtacaagggagaagcccccggacagactgggatgaggtgacctggttgcacacttctggggcacctagtgccatacctggcctggagatccttcccgcactgccgcctttactgctgccgatgctgtcacctcgggtaaggatagagattccactgaagctgctagctttggtgacagggggtcgcatgctccggacagagccatcagagtctgtgctgctccaagggcgtggctccagggatttgagttcgctgtctgtgctgctctggcggctgcttgaggtgcggctcagtccttcacggttccccctgatgtcatttagatatccgttctggccagtctctcgggcaaatattctctctcggaccctttgatattcctcctctctctcttctattgacttgctcctccttccatcctgcaatggaactctgatctagatcgatgagcagaattaagctagttaagttctcctcgtactgcaagctcactggttatcatctcggtccatactggcatcatctctcttgagaatgaacctctgttgaaattctgtattcttctcatcctttatatgttctgagaacctctgttcagggattcttgtgttactagttttgt

SEQ ID NO: 17337 - RNA, 3599 nt, Homo sapiens
  source 1..3599: mol_type = other RNA
tcaggccaggcacagtggctcacgcctgtaatcccagcactctggaaggccaaggcaggtggatcacctgaggtcaggagtttgaggccagcctggccaacatggtgaaactccgtctctactaaaaatacaaaaattagccgggcatggtggcgcgtgtctgtagtgccagctacttgggaggctgaggcaggagaatcacctgaacccaggagctggaggttgcagttagccaagatcgtgctactgcactccagctggggtgacaagagcgaaactccgtctcaaaaaaaaaaaaaaaaaaaaaaagaagaggatgggaagaagagtgatgcaaggggggtcaaccagggaaaaagagaggacccatggcaggggagcaagaaggagtccaatgccagtgtaggtatctgtgtttccatcttcatcactgtcttaggttccagtttaacatcagtttccttacttcctgcctctgtccatggtctgtcaggatccttcaaccccctccaccctgcccttgctccttctgtgacagtccctttcccctcctccatttattgggagctggctcgctccaggatcctcaggtcatagttctttttggccattcgaagtttgaagcgactcacggagttgttgagacgaagggaggcattttgggcagccagggggctggggaacacagccacaatggtgtacaaggcagcgaggtccgagtggcggccattctcagcagtcccactgttgtcccccccaccccctccaggcagcccctgagcatccttgagccactggatcttggcgccagacatggcgagctgcgtgaagagtttgtccgcctcagtacgggtgatgccctcagggagatctgtcacctccagcacccgccccaggacaacatctgctgtccccaggtcagtggaggcagatttgagtgcttgtctcttgccccggtttccatgcttcagtccactctgtccctggtgcaccgtgtaagttgactggccatggagcaagggagggcagatggacagattgtactgtaatggctggcccaaaagggagtagcgcccatcaccctgtgctggacccccaggccgggggaactgtgtgaggacaggcaggggactgagtcctgtgcagacactgctgaggctggtgacaggagagggtgctggagactgggtaggagatgtgacagggctgctgctcatttgtgtgttggcctgggggctgctgtcaggactgtacaggtctccaggcttctgcccccgctggtccatgctgtagtatttacaatgactccactggaccatggatgggttctgagggggctggggtccattagggacattcagctgcatgaccactacacctggtccagaaggtgacactcctgagtactgctgtggcatctgtggtggactgcagggagagggagactgaggcatctggtactgctcagagccagggggttgcagaaaccctacagaagggctcgtaccgttctgctgagcaggtgggatcatgctatagtacactggtacccccgctgctgggaggcctccttgcacagactggctcacagggaccagcatgggttgctggaaaggcggctggaccacattttgcgagtcactacccactggaacttggtaagaaggcagtggagtgtactgaaccaccaggccttgcatctggccccccatgctgctcctctggctgctgagcaggccctggttctgtggctgctggaccccaatcatgccttggtaagccgcctgctgctggttaggcatcatgggctgtaaaccaggctgctgggatggctgaggcagctgctgaccacgttgggggctataggccaccgggtgagagagaggtcgatattgctggttggagttaggatattgtccagggggatagtaagaaacctggatctgttgagggggctgcatgtacccctggggtggcagaacttgctgagtaggtggtgcatggctagaggtggaatagttggaagtggggaggggctgacccgtggaagccatgatgaagctagtctgctgagggtgctgggagataagtggggtctggaatagagctgcagatgggtcagctgcttcagtagaaccttggcgactaaggctcatttgtccaaaggggttgctgaggtcatctgcctgtgagatcatgtgattattcaagggtggctgttgctgaggcgtgggtgggagagcaggaagttgctgctgctgctgctgctgttgctgctgggcagtacaagggagaagcccccggacagactgggatgaggtgacctggttgcacacttctggggcacctagtgccatacctggcctggagatccttcccgcactgccgcctttactgctgccgatgctgtcacctcgggtaaggatagagattccactgaagctgctagctttggtgacagggggtcgcatgctccggacagagccatcagagtctgtgctgctccaagggcgtggctccagggatttgagttcgctgtctgtgctgctctggcggctgcttgaggtgcggctcagtccttcacggttccccctgatgtcatttagatatccgttctggccagtctctcgggcaaatattctctctcggaccctttgatattcctcctctctctcttctattgacttgctcctccttccatcctgcaatggaactctgatctggttatcatctcggtccatactggcatcatctctcttgagaatgaacctctgttgaaattctgtattcttctcatcctttatatgttctgagaacctctgttcagggattcttgtgttactagttttgttgatgatgacagctttcccagtttgatcaacattgtggtccatcccaaaataggcagctacccggtgtaatagcatccggtgatatgaggtcatctgagggaacttcttgaactgattacttgggttctttttcagtgtatttacaagaaattcatgtaggtctattccagtggagtccgtatattcctggctggagtctctggacagcatcttccttgggatcttttctttgtttttgtccttgtcttccttttcagagacatcttttgtggacttttcttcctccttgtcagaagggcaactgatgtgcaattgaattatatcctgggtttctaatggcccatcagcaaatggggtggaggactcctcacacactgccaggctacgcaccaactttagcttggaattagacttggctcttttcctggcatgaccatggttagatgtccgcctcttgtcaaaaaggaactcataatcctgtgtctcctgacgcaaactggtatcttcacattctttctcaatttcttccttacttggagtcttagatataaacttgtttttgtttacagattcttccaccagttttttttctgattctttcattatttccagggtctcttgagtagtgttactgttagacatgttcttcaatagaatacagtggcctctatggactcctgaataaatgctcagcctccatgagtccagtgctggaatggcatcacatataagaaacaagtctaacct

SEQ ID NO: 17338 - RNA, 4431 nt, Homo sapiens
  source 1..4431: mol_type = other RNA
tcaggccaggcacagtggctcacgcctgtaatcccagcactctggaaggccaaggcaggtggatcacctgaggtcaggagtttgaggccagcctggccaacatggtgaaactccgtctctactaaaaatacaaaaattagccgggcatggtggcgcgtgtctgtagtgccagctacttgggaggctgaggcaggagaatcacctgaacccaggagctggaggttgcagttagccaagatcgtgctactgcactccagctggggtgacaagagcgaaactccgtctcaaaaaaaaaaaaaaaaaaaaaaagaagaggatgggaagaagagtgatgcaaggggggtcaaccagggaaaaagagaggacccatggcaggggagcaagaaggagtccaatgccagtgtaggtatctgtgtttccatcttcatcactgtcttaggttccagtttaacatcagtttccttacttcctgcctctgtccatggtctgtcaggatccttcaaccccctccaccctgcccttgctccttctgtgacagtccctttcccctcctccatttattgggagctggctcgctccaggatcctcaggtcatagttctttttggccattcgaagtttgaagcgactcacggagttgttgagacgaagggaggcattttgggcagccagggggctggggaacacagccacaatggtgtacaaggcagcgaggtccgagtggcggccattctcagcagtcccactgttgtcccccccaccccctccaggcagcccctgagcatccttgagccactggatcttggcgccagacatggcgagctgcgtgaagagtttgtccgcctcagtacgggtgatgccctcagggagatctgtcacctccagcacccgccccaggacaacatctgctgtccccaggtcagtggaggcagatttgagtgcttgtctcttgccccggtttccatgcttcagtccactctgtccctggtgcaccgtgtaagttgactggccatggagcaagggagggcagatggacagattgtactgtaatggctggcccaaaagggagtagcgcccatcaccctgtgctggacccccaggccgggggaactgtgtgaggacaggcaggggactgagtcctgtgcagacactgctgaggctggtgacaggagagggtgctggagactgggtaggagatgtgacagggctgctgctcatttgtgtgttggcctgggggctgctgtcaggactgtacaggtctccaggcttctgcccccgctggtccatgctgtagtatttacaatgactccactggaccatggatgggttctgagggggctggggtccattagggacattcagctgcatgaccactacacctggtccagaaggtgacactcctgagtactgctgtggcatctgtggtggactgcagggagagggagactgaggcatctggtactgctcagagccagggggttgcagaaaccctacagaagggctcgtaccgttctgctgagcaggtgggatcatgctatagtacactggtacccccgctgctgggaggcctccttgcacagactggctcacagggaccagcatgggttgctggaaaggcggctggaccacattttgcgagtcactacccactggaacttggtaagaaggcagtggagtgtactgaaccaccaggccttgcatctggccccccatgctgctcctctggctgctgagcaggccctggttctgtggctgctggaccccaatcatgccttggtaagccgcctgctgctggttaggcatcatgggctgtaaaccaggctgctgggatggctgaggcagctgctgaccacgttgggggctataggccaccgggtgagagagaggtcgatattgctggttggagttaggatattgtccagggggatagtaagaaacctggatctgttgagggggctgcatgtacccctggggtggcagaacttgctgagtaggtggtgcatggctagaggtggaatagttggaagtggggaggggctgacccgtggaagccatgatgaagctagtctgctgagggtgctgggagataagtggggtctggaatagagctgcagatgggtcagctgcttcagtagaaccttggcgactaaggctcatttgtccaaaggggttgctgaggtcatctgcctgtgagatcatgtgattattcaagggtggctgttgctgaggcgtgggtgggagagcaggaagttgctgctgctgctgctgctgttgctgctgggcagtacaagggagaagcccccggacagactgggatgaggtgacctggttgcacacttctggggcacctagtgccatacctggcctggagatccttcccgcactgccgcctttactgctgccgatgctgtcacctcgggtaaggatagagattccactgaagctgctagctttggtgacagggggtcgcatgctccggacagagccatcagagtctgtgctgctccaagggcgtggctccagggatttgagttcgctgtctgtgctgctctggcggctgcttgaggtgcggctcagtccttcacggttccccctgatgtcatttagatatccgttctggccagtctctcgggcaaatattctctctcggaccctttgatattcctcctctctctcttctattgacttgctcctccttccatcctgcaatggaactctgatctggttatcatctcggtccatactggcatcatctctcttgagaatgaacctctgttgaaattctgtattcttctcatcctttatatgttctgagaacctctgttcagggattcttgtgttactagttttgttgatgatgacagctttcccagtttgatcaacattgtggtccatcccaaaataggcagctacccggtgtaatagcatccggtgatatgaggtcatctgagggaacttcttgaactgattattgttgtcattaataaattccagaatctcctgttctaattttagcagcatcattctgtccctgtttaaaaaagattaaaacaaaacaaaacaaaacaaaaagcagccctcccatagacattgaaagtggggattgaaaacacaacttgctcattacagaagctgaaaaaggtatatatccaaacccagtaatgaaccataatgctgctaagcctcacttgcctgttttacaatatttttaaaaagaaaaacaacccgagtatacattttgcaggtcctccaatcatatactttgttataccatatcagaaatctcactgttaacaacatattcatataaacacacgttataaatctaatcgtcattctgtattccatcttgttataaacaattttaaaggaattataatttagcttatgtacaaatcaattattttttccttctgtgctttttattttagctcttcttactatcactcccaatgtgtgctttttaatcagtatactcccaagacttcatatttctttgtttctgcattcttctttcacagaagttttcccaattcttctgaaaacagaaacctcaatgtgagagtattttgaatccctcacagaatataaaactatacctgacaaatactagggggacaggaagatgagcatcctagattctaagaatggaaaaattctgggaagccgtttggcctcttggaatcttgctatcccctaaccccttttcctcttatacccatcatgttattaccttgggttctttttcagtgtatttacaagaaattcatgtaggtctattccagtggagtccgtatattcctggctggagtctctggacagcatcttccttgggatcttttctttgtttttgtccttgtcttccttttcagagacatcttttgtggacttttcttcctccttgtcagaagggcaactgatgtgcaattgaattatatcctgggtttctaatggcccatcagcaaatggggtggaggactcctcacacactgccaggctacgcaccaactttagcttggaattagacttggctcttttcctggcatgaccatggttagatgtccgcctctgtgtctcctgacgcaaactggtatcttcacattctttctcaatttcttccttacttggagtcttagatataaacttgtttttgtttacagattcttccaccagttttttttctgattctttcattatttccagggtctcttgagtagtgttactgttagacatgttcttcaatagaatacagtggcctctatggactcctgaataaatgctcagcctccatgagtccagtgctggaatggcatcacatataagaaacaagtctaacctctcgcacgggccttggcggggagggcgcccacgtctccgcccgccgcccgggcccacggccgctcggctgcggctcggccccgacggccggcgg

SEQ ID NO: 17339 - RNA, 3983 nt, Homo sapiens
  source 1..3983: mol_type = other RNA
tcaggccaggcacagtggctcacgcctgtaatcccagcactctggaaggccaaggcaggtggatcacctgaggtcaggagtttgaggccagcctggccaacatggtgaaactccgtctctactaaaaatacaaaaattagccgggcatggtggcgcgtgtctgtagtgccagctacttgggaggctgaggcaggagaatcacctgaacccaggagctggaggttgcagttagccaagatcgtgctactgcactccagctggggtgacaagagcgaaactccgtctcaaaaaaaaaaaaaaaaaaaaaaagaagaggatgggaagaagagtgatgcaaggggggtcaaccagggaaaaagagaggacccatggcaggggagcaagaaggagtccaatgccagtgtaggtatctgtgtttccatcttcatcactgtcttaggttccagtttaacatcagtttccttacttcctgcctctgtccatggtctgtcaggatccttcaaccccctccaccctgcccttgctccttctgtgacagtccctttcccctcctccatttattgggagctggctcgctccaggatcctcaggtcatagttctttttggccattcgaagtttgaagcgactcacggagttgttgagacgaagggaggcattttgggcagccagggggctggggaacacagccacaatggtgtacaaggcagcgaggtccgagtggcggccattctcagcagtcccactgttgtcccccccaccccctccaggcagcccctgagcatccttgagccactggatcttggcgccagacatggcgagctgcgtgaagagtttgtccgcctcagtacgggtgatgccctcagggagatctgtcacctccagcacccgccccaggacaacatctgctgtccccaggtcagtggaggcagatttgagtgcttgtctcttgccccggtttccatgcttcagtccactctgtccctggtgcaccgtgtaagttgactggccatggagcaagggagggcagatggacagattgtactgtaatggctggcccaaaagggagtagcgcccatcaccctgtgctggacccccaggccgggggaactgtgtgaggacaggcaggggactgagtcctgtgcagacactgctgaggctggtgacaggagagggtgctggagactgggtaggagatgtgacagggctgctgctcatttgtgtgttggcctgggggctgctgtcaggactgtacaggtctccaggcttctgcccccgctggtccatgctgtagtatttacaatgactccactggaccatggatgggttctgagggggctggggtccattagggacattcagctgcatgaccactacacctggtccagaaggtgacactcctgagtactgctgtggcatctgtggtggactgcagggagagggagactgaggcatctggtactgctcagagccagggggttgcagaaaccctacagaagggctcgtaccgttctgctgagcaggtgggatcatgctatagtacactggtacccccgctgctgggaggcctccttgcacagactggctcacagggaccagcatgggttgctggaaaggcggctggaccacattttgcgagtcactacccactggaacttggtaagaaggcagtggagtgtactgaaccaccaggccttgcatctggccccccatgctgctcctctggctgctgagcaggccctggttctgtggctgctggaccccaatcatgccttggtaagccgcctgctgctggttaggcatcatgggctgtaaaccaggctgctgggatggctgaggcagctgctgaccacgttgggggctataggccaccgggtgagagagaggtcgatattgctggttggagttaggatattgtccagggggatagtaagaaacctggatctgttgagggggctgcatgtacccctggggtggcagaacttgctgagtaggtggtgcatggctagaggtggaatagttggaagtggggaggggctgacccgtggaagccatgatgaagctagtctgctgagggtgctgggagataagtggggtctggaatagagctgcagatgggtcagctgcttcagtagaaccttggcgactaaggctcatttgtccaaaggggttgctgaggtcatctgcctgtgagatcatgtgattattcaagggtggctgttgctgaggcgtgggtgggagagcaggaagttgctgctgctgctgctgctgttgctgctgggcagtacaagggagaagcccccggacagactgggatgaggtgacctggttgcacacttctggggcacctagtgccatacctggcctggagatccttcccgcactgccgcctttactgctgccgatgctgtcacctcgggtaaggatagagattccactgaagctgctagctttggtgacagggggtcgcatgctccggacagagccatcagagtctgtgctgctccaagggcgtggctccagggatttgagttcgctgtctgtgctgctctggcggctgcttgaggtgcggctcagtccttcacggttccccctgatgtcatttagatatccgttctggccagtctctcgggcaaatattctctctcggaccctttgatattcctcctctctctcttctattgacttgctcctccttccatcctgcaatggaactctgatctggttatcatctcggtccatactggcatcatctctcttgagaatgaacctctgttgaaattctgtattcttctcatcctttatatgttctgagaacctctgttcagggattcttgtgttactagttttgttgatgatgacagctttcccagtttgatcaacattgtggtccatcccaaaataggcagctacccggtgtaatagcatccggtgatatgaggtcatctgagggaacttcttgaactgattattgttgtcattaataaattccagaatctcctgttctaattttagcagcatcattctgtcccttgggttctttttcagtgtatttacaagaaattcatgtaggtctattccagtggagtccgtatattcctggctggagtctctggacagcatcttccttgggatcttttctttgtttttgtccttgtcttccttttcagagacatcttttgtggacttttcttcctccttgtcagaagggcaactgatgtgcaattgaattatatcctgggtttctaatggcccatcagcaaatggggtggaggactcctcacacactgccaggctacgcaccaactttagcttggaattagacttggctcttttcctggcatgaccatggttagatgtccgcctcttgtcaaaaaggaactcataatcctgtgtctcctgacgcaaactggtatcttcacattctttctcaatttcttccttacttggagtcttagatataaacttgtttttgtttacagattcttccaccagttttttttctgattctttcattatttccagggtctcttgagtagtgttactgttagacatgttcttcaatagaatacagtggcctctatggactcctgaataaatgctcagcctccatgagtccagtgctggaatggcatcacatataagaaacaagtctaacctctcgcacgggccttggcggggagggcgcccacgtctccgcccgccgcccgggcccacggccgctcggctgcggctcggccccgacggccggcggcggcgcgcttctgggggcgggcttttctcggccggggcttccccggggccgagggctgggaagcaggggggactgggacgggggaggggaaaggggcttgggaaggaggggggagaggggaagaaaaggggggaaccaaacccggaaagggagaaaaggggggaggggaaaatcagaaggggaagaaaagcccagagtccgccccccgctgcggctgcgcgctacgtcac

SEQ ID NO: 17340 - RNA, 3616 nt, Homo sapiens
  source 1..3616: mol_type = other RNA
tcaggccaggcacagtggctcacgcctgtaatcccagcactctggaaggccaaggcaggtggatcacctgaggtcaggagtttgaggccagcctggccaacatggtgaaactccgtctctactaaaaatacaaaaattagccgggcatggtggcgcgtgtctgtagtgccagctacttgggaggctgaggcaggagaatcacctgaacccaggagctggaggttgcagttagccaagatcgtgctactgcactccagctggggtgacaagagcgaaactccgtctcaaaaaaaaaaaaaaaaaaaaaaagaagaggatgggaagaagagtgatgcaaggggggtcaaccagggaaaaagagaggacccatggcaggggagcaagaaggagtccaatgccagtgtaggtatctgtgtttccatcttcatcactgtcttaggttccagtttaacatcagtttccttacttcctgcctctgtccatggtctgtcaggatccttcaaccccctccaccctgcccttgctccttctgtgacagtccctttcccctcctccatttattgggagctggctcgctccaggatcctcaggtcatagttctttttggccattcgaagtttgaagcgactcacggagttgttgagacgaagggaggcattttgggcagccagggggctggggaacacagccacaatggtgtacaaggcagcgaggtccgagtggcggccattctcagcagtcccactgttgtcccccccaccccctccaggcagcccctgagcatccttgagccactggatcttggcgccagacatggcgagctgcgtgaagagtttgtccgcctcagtacgggtgatgccctcagggagatctgtcacctccagcacccgccccaggacaacatctgctgtccccaggtcagtggaggcagatttgagtgcttgtctcttgccccggtttccatgcttcagtccactctgtccctggtgcaccgtgtaagttgactggccatggagcaagggagggcagatggacagattgtactgtaatggctggcccaaaagggagtagcgcccatcaccctgtgctggacccccaggccgggggaactgtgtgaggacaggcaggggactgagtcctgtgcagacactgctgaggctggtgacaggagagggtgctggagactgggtaggagatgtgacagggctgctgctcatttgtgtgttggcctgggggctgctgtcaggactgtacaggtctccaggcttctgcccccgctggtccatgctgtagtatttacaatgactccactggaccatggatgggttctgagggggctggggtccattagggacattcagctgcatgaccactacacctggtccagaaggtgacactcctgagtactgctgtggcatctgtggtggactgcagggagagggagactgaggcatctggtactgctcagagccagggggttgcagaaaccctacagaagggctcgtaccgttctgctgagcaggtgggatcatgctatagtacactggtacccccgctgctgggaggcctccttgcacagactggctcacagggaccagcatgggttgctggaaaggcggctggaccacattttgcgagtcactacccactggaacttggtaagaaggcagtggagtgtactgaaccaccaggccttgcatctggccccccatgctgctcctctggctgctgagcaggccctggttctgtggctgctggaccccaatcatgccttggtaagccgcctgctgctggttaggcatcatgggctgtaaaccaggctgctgggatggctgaggcagctgctgaccacgttgggggctataggccaccgggtgagagagaggtcgatattgctggttggagttaggatattgtccagggggatagtaagaaacctggatctgttgagggggctgcatgtacccctggggtggcagaacttgctgagtaggtggtgcatggctagaggtggaatagttggaagtggggaggggctgacccgtggaagccatgatgaagctagtctgctgagggtgctgggagataagtggggtctggaatagagctgcagatgggtcagctgcttcagtagaaccttggcgactaaggctcatttgtccaaaggggttgctgaggtcatctgcctgtgagatcatgtgattattcaagggtggctgttgctgaggcgtgggtgggagagcaggaagttgctgctgctgctgctgctgttgctgctgggcagtacaagggagaagcccccggacagactgggatgaggtgacctggttgcacacttctggggcacctagtgccatacctggcctggagatccttcccgcactgccgcctttactgctgccgatgctgtcacctcgggtaaggatagagattccactgaagctgctagctttggtgacagggggtcgcatgctccggacagagccatcagagtctgtgctgctccaagggcgtggctccagggatttgagttcgctgtctgtgctgctctggcggctgcttgaggtgcggctcagtccttcacggttccccctgatgtcatttagatatccgttctggccagtctggttatcatctcggtccatactggcatcatctctcttgagaatgaacctctgttgaaattctgtattcttctcatcctttatatgttctgagaacctctgttcagggattcttgtgttactagttttgttgatgatgacagctttcccagtttgatcaacattgtggtccatcccaaaataggcagctacccggtgtaatagcatccggtgatatgaggtcatctgagggaacttcttgaactgattacttgggttctttttcagtgtatttacaagaaattcatgtaggtctattccagtggagtccgtatattcctggctggagtctctggacagcatcttccttgggatcttttctttgtttttgtccttgtcttccttttcagagacatcttttgtggacttttcttcctccttgtcagaagggcaactgatgtgcaattgaattatatcctgggtttctaatggcccatcagcaaatggggtggaggactcctcacacactgccaggctacgcaccaactttagcttggaattagacttggctcttttcctggcatgaccatggttagatgtccgcctctgtgtctcctgacgcaaactggtatcttcacattctttctcaatttcttccttacttggagtcttagatataaacttgtttttgtttacagattcttccaccagttttttttctgattctttcattatttccagggtctcttgagtagtgttactgttagacatgttcttcaatagaatacagtggcctctatggactcctgaataaatgctcagcctccatgagtccagtgctggaatggcatcacatataagaaacaagtctaacctctgtaattccagctactcaggaggctgaagcaggaaatcgcttgaaactggtggtgggggtgggcaggggagaggggcagaggttgtaatgagccgaaatcatgccacttcactccagcagcctaggcaaaagagcg

SEQ ID NO: 17341 - RNA, 3503 nt, Homo sapiens
  source 1..3503: mol_type = other RNA
tcaggccaggcacagtggctcacgcctgtaatcccagcactctggaaggccaaggcaggtggatcacctgaggtcaggagtttgaggccagcctggccaacatggtgaaactccgtctctactaaaaatacaaaaattagccgggcatggtggcgcgtgtctgtagtgccagctacttgggaggctgaggcaggagaatcacctgaacccaggagctggaggttgcagttagccaagatcgtgctactgcactccagctggggtgacaagagcgaaactccgtctcaaaaaaaaaaaaaaaaaaaaaaagaagaggatgggaagaagagtgatgcaaggggggtcaaccagggaaaaagagaggacccatggcaggggagcaagaaggagtccaatgccagtgtaggtatctgtgtttccatcttcatcactgtcttaggttccagtttaacatcagtttccttacttcctgcctctgtccatggtctgtcaggatccttcaaccccctccaccctgcccttgctccttctgtgacagtccctttcccctcctccatttattgggagctggctcgctccaggatcctcaggtcatagttctttttggccattcgaagtttgaagcgactcacggagttgttgagacgaagggaggcattttgggcagccagggggctggggaacacagccacaatggtgtacaaggcagcgaggtccgagtggcggccattctcagcagtcccactgttgtcccccccaccccctccaggcagcccctgagcatccttgagccactggatcttggcgccagacatggcgagctgcgtgaagagtttgtccgcctcagtacgggtgatgccctcagggagatctgtcacctccagcacccgccccaggacaacatctgctgtccccaggtcagtggaggcagatttgagtgcttgtctcttgccccggtttccatgcttcagtccactctgtccctggtgcaccgtgtaagttgactggccatggagcaagggagggcagatggacagattgtactgtaatggctggcccaaaagggagtagcgcccatcaccctgtgctggacccccaggccgggggaactgtgtgaggacaggcaggggactgagtcctgtgcagacactgctgaggctggtgacaggagagggtgctggagactgggtaggagatgtgacagggctgctgctcatttgtgtgttggcctgggggctgctgtcaggactgtacaggtctccaggcttctgcccccgctggtccatgctgtagtatttacaatgactccactggaccatggatgggttctgagggggctggggtccattagggacattcagctgcatgaccactacacctggtccagaaggtgacactcctgagtactgctgtggcatctgtggtggactgcagggagagggagactgaggcatctggtactgctcagagccagggggttgcagaaaccctacagaagggctcgtaccgttctgctgagcaggtgggatcatgctatagtacactggtacccccgctgctgggaggcctccttgcacagactggctcacagggaccagcatgggttgctggaaaggcggctggaccacattttgcgagtcactacccactggaacttggtaagaaggcagtggagtgtactgaaccaccaggccttgcatctggccccccatgctgctcctctggctgctgagcaggccctggttctgtggctgctggaccccaatcatgccttggtaagccgcctgctgctggttaggcatcatgggctgtaaaccaggctgctgggatggctgaggcagctgctgaccacgttgggggctataggccaccgggtgagagagaggtcgatattgctggttggagttaggatattgtccagggggatagtaagaaacctggatctgttgagggggctgcatgtacccctggggtggcagaacttgctgagtaggtggtgcatggctagaggtggaatagttggaagtggggaggggctgacccgtggaagccatgatgaagctagtctgctgagggtgctgggagataagtggggtctggaatagagctgcagatgggtcagctgcttcagtagaaccttggcgactaaggctcatttgtccaaaggggttgctgaggtcatctgcctgtgagatcatgtgattattcaagggtggctgttgctgaggcgtgggtgggagagcaggaagttgctgctgctgctgctgctgttgctgctgggcagtacaagggagaagcccccggacagactgggatgaggtgacctggttgcacacttctggggcacctagtgccatacctggcctggagatccttcccgcactgccgcctttactgctgccgatgctgtcacctcgggtaaggatagagattccactgaagctgctagctttggtgacagggggtcgcatgctccggacagagccatcagagtctgtgctgctccaagggcgtggctccagggatttgagttcgctgtctgtgctgctctggcggctgcttgaggtgcggctcagtccttcacggttccccctgatgtcatttagatatccgttctggccagtctggttatcatctcggtccatactggcatcatctctcttgagaatgaacctctgttgaaattctgtattcttctcatcctttatatgttctgagaacctctgttcagggattcttgtgttactagttttgttgatgatgacagctttcccagtttgatcaacattgtggtccatcccaaaataggcagctacccggtgtaatagcatccggtgatatgaggtcatctgagggaacttcttgaactgattacttgggttctttttcagtgtatttacaagaaattcatgtaggtctattccagtggagtccgtatattcctggctggagtctctggacagcatcttccttgggatcttttctttgtttttgtccttgtcttccttttcagagacatcttttgtggacttttcttcctccttgtcagaagggcaactgatgtgcaattgaattatatcctgggtttctaatggcccatcagcaaatggggtggaggactcctcacacactgccaggctacgcaccaactttagcttggaattagacttggctcttttcctggcatgaccatggttagatgtccgcctcttgtcaaaaaggaactcataatcctgtgtctcctgacgcaaactggtatcttcacattctttctcaatttcttccttacttggagtcttagatataaacttgtttttgtttacagattcttccaccagttttttttctgattctttcattatttccagggtctcttgagtagtgttactgttagacatgttcttcaatagaatacagtggcctctatggactcctgaataaatgctcagcctccatgagtccagtgctggaatggcatcacatataagaaacaagtctaacct

SEQ ID NO: 17342 - RNA, 3793 nt, Homo sapiens
  source 1..3793: mol_type = other RNA
tcaggccaggcacagtggctcacgcctgtaatcccagcactctggaaggccaaggcaggtggatcacctgaggtcaggagtttgaggccagcctggccaacatggtgaaactccgtctctactaaaaatacaaaaattagccgggcatggtggcgcgtgtctgtagtgccagctacttgggaggctgaggcaggagaatcacctgaacccaggagctggaggttgcagttagccaagatcgtgctactgcactccagctggggtgacaagagcgaaactccgtctcaaaaaaaaaaaaaaaaaaaaaaagaagaggatgggaagaagagtgatgcaaggggggtcaaccagggaaaaagagaggacccatggcaggggagcaagaaggagtccaatgccagtgtaggtatctgtgtttccatcttcatcactgtcttaggttccagtttaacatcagtttccttacttcctgcctctgtccatggtctgtcaggatccttcaaccccctccaccctgcccttgctccttctgtgacagtccctttcccctcctccatttattgggagctggctcgctccaggatcctcaggtcatagttctttttggccattcgaagtttgaagcgactcacggagttgttgagacgaagggaggcattttgggcagccagggggctggggaacacagccacaatggtgtacaaggcagcgaggtccgagtggcggccattctcagcagtcccactgttgtcccccccaccccctccaggcagcccctgagcatccttgagccactggatcttggcgccagacatggcgagctgcgtgaagagtttgtccgcctcagtacgggtgatgccctcagggagatctgtcacctccagcacccgccccaggacaacatctgctgtccccaggtcagtggaggcagatttgagtgcttgtctcttgccccggtttccatgcttcagtccactctgtccctggtgcaccgtgtaagttgactggccatggagcaagggagggcagatggacagattgtactgtaatggctggcccaaaagggagtagcgcccatcaccctgtgctggacccccaggccgggggaactgtgtgaggacaggcaggggactgagtcctgtgcagacactgctgaggctggtgacaggagagggtgctggagactgggtaggagatgtgacagggctgctgctcatttgtgtgttggcctgggggctgctgtcaggactgtacaggtctccaggcttctgcccccgctggtccatgctgtagtatttacaatgactccactggaccatggatgggttctgagggggctggggtccattagggacattcagctgcatgaccactacacctggtccagaaggtgacactcctgagtactgctgtggcatctgtggtggactgcagggagagggagactgaggcatctggtactgctcagagccagggggttgcagaaaccctacagaagggctcgtaccgttctgctgagcaggtgggatcatgctatagtacactggtacccccgctgctgggaggcctccttgcacagactggctcacagggaccagcatgggttgctggaaaggcggctggaccacattttgcgagtcactacccactggaacttggtaagaaggcagtggagtgtactgaaccaccaggccttgcatctggccccccatgctgctcctctggctgctgagcaggccctggttctgtggctgctggaccccaatcatgccttggtaagccgcctgctgctggttaggcatcatgggctgtaaaccaggctgctgggatggctgaggcagctgctgaccacgttgggggctataggccaccgggtgagagagaggtcgatattgctggttggagttaggatattgtccagggggatagtaagaaacctggatctgttgagggggctgcatgtacccctggggtggcagaacttgctgagtaggtggtgcatggctagaggtggaatagttggaagtggggaggggctgacccgtggaagccatgatgaagctagtctgctgagggtgctgggagataagtggggtctggaatagagctgcagatgggtcagctgcttcagtagaaccttggcgactaaggctcatttgtccaaaggggttgctgaggtcatctgcctgtgagatcatgtgattattcaagggtggctgttgctgaggcgtgggtgggagagcaggaagttgctgctgctgctgctgctgttgctgctgggcagtacaagggagaagcccccggacagactgggatgaggtgacctggttgcacacttctggggcacctagtgccatacctggcctggagatccttcccgcactgccgcctttactgctgccgatgctgtcacctcgggtaaggatagagattccactgaagctgctagctttggtgacagggggtcgcatgctccggacagagccatcagagtctgtgctgctccaagggcgtggctccagggatttgagttcgctgtctgtgctgctctggcggctgcttgaggtgcggctcagtccttcacggttccccctgatgtcatttagatatccgttctggccagtctggttatcatctcggtccatactggcatcatctctcttgagaatgaacctctgttgaaattctgtattcttctcatcctttatatgttctgagaacctctgttcagggattcttgtgttactagttttgttgatgatgacagctttcccagtttgatcaacattgtggtccatcccaaaataggcagctacccggtgtaatagcatccggtgatatgaggtcatctgagggaacttcttgaactgattattgttgtcattaataaattccagaatctcctgttctaattttagcagcatcattctgtcccttgggttctttttcagtgtatttacaagaaattcatgtaggtctattccagtggagtccgtatattcctggctggagtctctggacagcatcttccttgggatcttttctttgtttttgtccttgtcttccttttcagagacatcttttgtggacttttcttcctccttgtcagaagggcaactgatgtgcaattgaattatatcctgggtttctaatggcccatcagcaaatggggtggaggactcctcacacactgccaggctacgcaccaactttagcttggaattagacttggctcttttcctggcatgaccatggttagatgtccgcctctgtgtctcctgacgcaaactggtatcttcacattctttctcaatttcttccttacttggagtcttagatataaacttgtttttgtttacagattcttccaccagttttttttctgattctttcattatttccagggtctcttgagtagtgttactgttagacatgttcttcaatagaatacagtggcctctatggactcctcgcacgggccttggcggggagggcgcccacgtctccgcccgccgcccgggcccacggccgctcggctgcggctcggccccgacggccggcggcggcgcgcttctgggggcgggcttttctcggccggggcttccccggggccgagggctgggaagcaggggggactgggacgggggaggggaaaggggcttgggaaggaggggggagaggggaagaaaaggggggaaccaaacccggaaagggagaaaaggggggaggggaaaatcagaaggggaagaaaagcccagagtccgccccccgctgcggctgcgcgctacgtcac

SEQ ID NO: 17343 - RNA, 3863 nt, Homo sapiens
  source 1..3863: mol_type = other RNA
tcaggccaggcacagtggctcacgcctgtaatcccagcactctggaaggccaaggcaggtggatcacctgaggtcaggagtttgaggccagcctggccaacatggtgaaactccgtctctactaaaaatacaaaaattagccgggcatggtggcgcgtgtctgtagtgccagctacttgggaggctgaggcaggagaatcacctgaacccaggagctggaggttgcagttagccaagatcgtgctactgcactccagctggggtgacaagagcgaaactccgtctcaaaaaaaaaaaaaaaaaaaaaaagaagaggatgggaagaagagtgatgcaaggggggtcaaccagggaaaaagagaggacccatggcaggggagcaagaaggagtccaatgccagtgtaggtatctgtgtttccatcttcatcactgtcttaggttccagtttaacatcagtttccttacttcctgcctctgtccatggtctgtcaggatccttcaaccccctccaccctgcccttgctccttctgtgacagtccctttcccctcctccatttattgggagctggctcgctccaggatcctcaggtcatagttctttttggccattcgaagtttgaagcgactcacggagttgttgagacgaagggaggcattttgggcagccagggggctggggaacacagccacaatggtgtacaaggcagcgaggtccgagtggcggccattctcagcagtcccactgttgtcccccccaccccctccaggcagcccctgagcatccttgagccactggatcttggcgccagacatggcgagctgcgtgaagagtttgtccgcctcagtacgggtgatgccctcagggagatctgtcacctccagcacccgccccaggacaacatctgctgtccccaggtcagtggaggcagatttgagtgcttgtctcttgccccggtttccatgcttcagtccactctgtccctggtgcaccgtgtaagttgactggccatggagcaagggagggcagatggacagattgtactgtaatggctggcccaaaagggagtagcgcccatcaccctgtgctggacccccaggccgggggaactgtgtgaggacaggcaggggactgagtcctgtgcagacactgctgaggctggtgacaggagagggtgctggagactgggtaggagatgtgacagggctgctgctcatttgtgtgttggcctgggggctgctgtcaggactgtacaggtctccaggcttctgcccccgctggtccatgctgtagtatttacaatgactccactggaccatggatgggttctgagggggctggggtccattagggacattcagctgcatgaccactacacctggtccagaaggtgacactcctgagtactgctgtggcatctgtggtggactgcagggagagggagactgaggcatctggtactgctcagagccagggggttgcagaaaccctacagaagggctcgtaccgttctgctgagcaggtgggatcatgctatagtacactggtacccccgctgctgggaggcctccttgcacagactggctcacagggaccagcatgggttgctggaaaggcggctggaccacattttgcgagtcactacccactggaacttggtaagaaggcagtggagtgtactgaaccaccaggccttgcatctggccccccatgctgctcctctggctgctgagcaggccctggttctgtggctgctggaccccaatcatgccttggtaagccgcctgctgctggttaggcatcatgggctgtaaaccaggctgctgggatggctgaggcagctgctgaccacgttgggggctataggccaccgggtgagagagaggtcgatattgctggttggagttaggatattgtccagggggatagtaagaaacctggatctgttgagggggctgcatgtacccctggggtggcagaacttgctgagtaggtggtgcatggctagaggtggaatagttggaagtggggaggggctgacccgtggaagccatgatgaagctagtctgctgagggtgctgggagataagtggggtctggaatagagctgcagatgggtcagctgcttcagtagaaccttggcgactaaggctcatttgtccaaaggggttgctgaggtcatctgcctgtgagatcatgtgattattcaagggtggctgttgctgaggcgtgggtgggagagcaggaagttgctgctgctgctgctgctgttgctgctgggcagtacaagggagaagcccccggacagactgggatgaggtgacctggttgcacacttctggggcacctagtgccatacctggcctggagatccttcccgcactgccgcctttactgctgccgatgctgtcacctcgggtaaggatagagattccactgaagctgctagctttggtgacagggggtcgcatgctccggacagagccatcagagtctgtgctgctccaagggcgtggctccagggatttgagttcgctgtctgtgctgctctggcggctgcttgaggtgcggctcagtccttcacggttccccctgatgtcatttagatatccgttctggccagtctggttatcatctcggtccatactggcatcatctctcttgagaatgaacctctgttgaaattctgtattcttctcatcctttatatgttctgagaacctctgttcagggattcttgtgttactagttttgttgatgatgacagctttcccagtttgatcaacattgtggtccatcccaaaataggcagctacccggtgtaatagcatccggtgatatgaggtcatctgagggaacttcttgaactgattattgttgtcattaataaattccagaatctcctgttctaattttagcagcatcattctgtcccttgggttctttttcagtgtatttacaagaaattcatgtaggtctattccagtggagtccgtatattcctggctggagtctctggacagcatcttccttgggatcttttctttgtttttgtccttgtcttccttttcagagacatcttttgtggacttttcttcctccttgtcagaagggcaactgatgtgcaattgaattatatcctgggtttctaatggcccatcagcaaatggggtggaggactcctcacacactgccaggctacgcaccaactttagcttggaattagacttggctcttttcctggcatgaccatggttagatgtccgcctctgtgtctcctgacgcaaactggtatcttcacattctttctcaatttcttccttacttggagtcttagatataaacttgtttttgtttacagattcttccaccagttttttttctgattctttcattatttccagggtctcttgagtagtgttactgttagacatgttcttcaatagaatacagtggcctctatggactcctgaataaatgctcagcctccatgagtccagtgctggaatggcatcacatataagaaacaagtctaacctctcgcacgggccttggcggggagggcgcccacgtctccgcccgccgcccgggcccacggccgctcggctgcggctcggccccgacggccggcggcggcgcgcttctgggggcgggcttttctcggccggggcttccccggggccgagggctgggaagcaggggggactgggacgggggaggggaaaggggcttgggaaggaggggggagaggggaagaaaaggggggaaccaaacccggaaagggagaaaaggggggaggggaaaatcagaaggggaagaaaagcccagagtccgccccccgctgcggctgcgcgctacgtcac

SEQ ID NO: 17344 - RNA, 3887 nt, Homo sapiens
  source 1..3887: mol_type = other RNA
tcaggccaggcacagtggctcacgcctgtaatcccagcactctggaaggccaaggcaggtggatcacctgaggtcaggagtttgaggccagcctggccaacatggtgaaactccgtctctactaaaaatacaaaaattagccgggcatggtggcgcgtgtctgtagtgccagctacttgggaggctgaggcaggagaatcacctgaacccaggagctggaggttgcagttagccaagatcgtgctactgcactccagctggggtgacaagagcgaaactccgtctcaaaaaaaaaaaaaaaaaaaaaaagaagaggatgggaagaagagtgatgcaaggggggtcaaccagggaaaaagagaggacccatggcaggggagcaagaaggagtccaatgccagtgtaggtatctgtgtttccatcttcatcactgtcttaggttccagtttaacatcagtttccttacttcctgcctctgtccatggtctgtcaggatccttcaaccccctccaccctgcccttgctccttctgtgacagtccctttcccctcctccatttattgggagctggctcgctccaggatcctcaggtcatagttctttttggccattcgaagtttgaagcgactcacggagttgttgagacgaagggaggcattttgggcagccagggggctggggaacacagccacaatggtgtacaaggcagcgaggtccgagtggcggccattctcagcagtcccactgttgtcccccccaccccctccaggcagcccctgagcatccttgagccactggatcttggcgccagacatggcgagctgcgtgaagagtttgtccgcctcagtacgggtgatgccctcagggagatctgtcacctccagcacccgccccaggacaacatctgctgtccccaggtcagtggaggcagatttgagtgcttgtctcttgccccggtttccatgcttcagtccactctgtccctggtgcaccgtgtaagttgactggccatggagcaagggagggcagatggacagattgtactgtaatggctggcccaaaagggagtagcgcccatcaccctgtgctggacccccaggccgggggaactgtgtgaggacaggcaggggactgagtcctgtgcagacactgctgaggctggtgacaggagagggtgctggagactgggtaggagatgtgacagggctgctgctcatttgtgtgttggcctgggggctgctgtcaggactgtacaggtctccaggcttctgcccccgctggtccatgctgtagtatttacaatgactccactggaccatggatgggttctgagggggctggggtccattagggacattcagctgcatgaccactacacctggtccagaaggtgacactcctgagtactgctgtggcatctgtggtggactgcagggagagggagactgaggcatctggtactgctcagagccagggggttgcagaaaccctacagaagggctcgtaccgttctgctgagcaggtgggatcatgctatagtacactggtacccccgctgctgggaggcctccttgcacagactggctcacagggaccagcatgggttgctggaaaggcggctggaccacattttgcgagtcactacccactggaacttggtaagaaggcagtggagtgtactgaaccaccaggccttgcatctggccccccatgctgctcctctggctgctgagcaggccctggttctgtggctgctggaccccaatcatgccttggtaagccgcctgctgctggttaggcatcatgggctgtaaaccaggctgctgggatggctgaggcagctgctgaccacgttgggggctataggccaccgggtgagagagaggtcgatattgctggttggagttaggatattgtccagggggatagtaagaaacctggatctgttgagggggctgcatgtacccctggggtggcagaacttgctgagtaggtggtgcatggctagaggtggaatagttggaagtggggaggggctgacccgtggaagccatgatgaagctagtctgctgagggtgctgggagataagtggggtctggaatagagctgcagatgggtcagctgcttcagtagaaccttggcgactaaggctcatttgtccaaaggggttgctgaggtcatctgcctgtgagatcatgtgattattcaagggtggctgttgctgaggcgtgggtgggagagcaggaagttgctgctgctgctgctgctgttgctgctgggcagtacaagggagaagcccccggacagactgggatgaggtgacctggttgcacacttctggggcacctagtgccatacctggcctggagatccttcccgcactgccgcctttactgctgccgatgctgtcacctcgggtaaggatagagattccactgaagctgctagctttggtgacagggggtcgcatgctccggacagagccatcagagtctgtgctgctccaagggcgtggctccagggatttgagttcgctgtctgtgctgctctggcggctgcttgaggtgcggctcagtccttcacggttccccctgatgtcatttagatatccgttctggccagtctggttatcatctcggtccatactggcatcatctctcttgagaatgaacctctgttgaaattctgtattcttctcatcctttatatgttctgagaacctctgttcagggattcttgtgttactagttttgttgatgatgacagctttcccagtttgatcaacattgtggtccatcccaaaataggcagctacccggtgtaatagcatccggtgatatgaggtcatctgagggaacttcttgaactgattattgttgtcattaataaattccagaatctcctgttctaattttagcagcatcattctgtcccttgggttctttttcagtgtatttacaagaaattcatgtaggtctattccagtggagtccgtatattcctggctggagtctctggacagcatcttccttgggatcttttctttgtttttgtccttgtcttccttttcagagacatcttttgtggacttttcttcctccttgtcagaagggcaactgatgtgcaattgaattatatcctgggtttctaatggcccatcagcaaatggggtggaggactcctcacacactgccaggctacgcaccaactttagcttggaattagacttggctcttttcctggcatgaccatggttagatgtccgcctcttgtcaaaaaggaactcataatcctgtgtctcctgacgcaaactggtatcttcacattctttctcaatttcttccttacttggagtcttagatataaacttgtttttgtttacagattcttccaccagttttttttctgattctttcattatttccagggtctcttgagtagtgttactgttagacatgttcttcaatagaatacagtggcctctatggactcctgaataaatgctcagcctccatgagtccagtgctggaatggcatcacatataagaaacaagtctaacctctcgcacgggccttggcggggagggcgcccacgtctccgcccgccgcccgggcccacggccgctcggctgcggctcggccccgacggccggcggcggcgcgcttctgggggcgggcttttctcggccggggcttccccggggccgagggctgggaagcaggggggactgggacgggggaggggaaaggggcttgggaaggaggggggagaggggaagaaaaggggggaaccaaacccggaaagggagaaaaggggggaggggaaaatcagaaggggaagaaaagcccagagtccgccccccgctgcggctgcgcgctacgtcac

SEQ ID NO: 17345 - RNA, 2775 nt, Homo sapiens
  source 1..2775: mol_type = other RNA
tcaggccaggcacagtggctcacgcctgtaatcccagcactctggaaggccaaggcaggtggatcacctgaggtcaggagtttgaggccagcctggccaacatggtgaaactccgtctctactaaaaatacaaaaattagccgggcatggtggcgcgtgtctgtagtgccagctacttgggaggctgaggcaggagaatcacctgaacccaggagctggaggttgcagttagccaagatcgtgctactgcactccagctggggtgacaagagcgaaactccgtctcaaaaaaaaaaaaaaaaaaaaaaagaagaggatgggaagaagagtgatgcaaggggggtcaaccagggaaaaagagaggacccatggcaggggagcaagaaggagtccaatgccagtgtaggtatctgtgtttccatcttcatcactgtcttaggttccagtttaacatcagtttccttacttcctgcctctgtccatggtctgtcaggatccttcaaccccctccaccctgcccttgctccttctgtgacagtccctttcccctcctccatttattgggagctggctcgctccaggatcctcaggtcatagttctttttggccattcgaagtttgaagcgactcacggagttgttgagacgaagggaggcattttgggcagccagggggctggggaacacagccacaatggtgtacaaggcagcgaggtccgagtggcggccattctcagcagtcccactgttgtcccccccaccccctccaggcagcccctgagcatccttgagccactggatcttggcgccagacatggcgagctgcgtgaagagtttgtccgcctcagtacgggtgatgccctcagggagatctgtcacctccagcacccgccccaggacaacatctgctgtccccaggtcagtggaggcagatttgagtgcttgtctcttgccccggtttccatgcttcagtccactctgtccctggtgcaccgtgtaagttgactggccatggagcaagggagggcagatggacagattgtactgtaatggctggcccaaaagggagtagcgcccatcaccctgtgctggacccccaggccgggggaactgtgtgaggacaggcaggggactgagtcctgtgcagacactgctgaggctggtgacaggagagggtgctggagactgggtaggagatgtgacagggctgctgctcatttgtgtgttggcctgggggctgctgtcaggactgtacaggtctccaggcttctgcccccgctggtccatgctgtagtatttacaatgactccactggaccatggatgggttctgagggggctggggtccattagggacattcagctgcatgaccactacacctggtccagaaggtgacactcctgagtactgctgtggcatctgtggtggactgcagggagagggagactgaggcatctggtactgctcagagccagggggttgcagaaaccctacagaagggctcgtaccgttctgctgagcaggtgggatcatgctatagtacactggtacccccgctgctgggaggcctccttgcacagactggctcacagggaccagcatgggttgctggaaaggcggctggaccacattttgcgagtcactacccactggaacttggtaagaaggcagtggagtgtactgaaccaccaggccttgcatctggccccccatgctgctcctctggctgctgagcaggccctggttctgtggctgctggaccccaatcatgccttggtaagccgcctgctgctggttaggcatcatgggctgtaaaccaggctgctgggatggctgaggcagctgctgaccacgttgggggctataggccaccgggtgagagagaggtcgatattgctggttggagttaggatattgtccagggggatagtaagaaacctggatctgttgagggggctgcatgtacccctggggtggcagaacttgctgagtaggtggtgcatggctagaggtggaatagttggaagtggggaggggctgacccgtggaagccatgatgaagctagtctgctgagggtgctgggagataagtggggtctggaatagagctgcagatgggtcagctgcttcagtagaaccttggcgactaaggctcatttgtccaaaggggttgctgaggtcatctgcctgtgagatcatgtgattattcaagggtggctgttgctgaggcgtgggtgggagagcaggaagttgctgctgctgctgctgctgttgctgctgggcagtacaagggagaagcccccggacagactgggatgaggtgacctggttgcacacttctggggcacctagtgccatacctggcctggagatccttcccgcactgccgcctttactgctgccgatgctgtcacctcgggtaaggatagagattccactgaagctgctagctttggtgacagggggtcgcatgctccggacagagccatcagagtctgtgctgctccaagggcgtggctccagggatttgagttcgctgtctgtgctgctctggcggctgcttgaggtgcggctcagtccttcacggttccccctggttatcatctcggtccatactggcatcatctctcttgagaatgaacctctgttgaaattctgtattcttctcatcctttatatgttctgagaacctctgttcagggattcttgtgttactagttttgttgatgatgacagctttcccagtttgatcaacattgtggtccatcccaaaata

SEQ ID NO: 17346 - RNA, 3979 nt, Homo sapiens
  source 1..3979: mol_type = other RNA
tcaggccaggcacagtggctcacgcctgtaatcccagcactctggaaggccaaggcaggtggatcacctgaggtcaggagtttgaggccagcctggccaacatggtgaaactccgtctctactaaaaatacaaaaattagccgggcatggtggcgcgtgtctgtagtgccagctacttgggaggctgaggcaggagaatcacctgaacccaggagctggaggttgcagttagccaagatcgtgctactgcactccagctggggtgacaagagcgaaactccgtctcaaaaaaaaaaaaaaaaaaaaaaagaagaggatgggaagaagagtgatgcaaggggggtcaaccagggaaaaagagaggacccatggcaggggagcaagaaggagtccaatgccagtgtaggtatctgtgtttccatcttcatcactgtcttaggttccagtttaacatcagtttccttacttcctgcctctgtccatggtctgtcaggatccttcaaccccctccaccctgcccttgctccttctgtgacagtccctttcccctcctccatttattgggagctggctcgctccaggatcctcaggtcatagttctttttggccattcgaagtttgaagcgactcacggagttgttgagacgaagggaggcattttgggcagccagggggctggggaacacagccacaatggtgtacaaggcagcgaggtccgagtggcggccattctcagcagtcccactgttgtcccccccaccccctccaggcagcccctgagcatccttgagccactggatcttggcgccagacatggcgagctgcgtgaagagtttgtccgcctcagtacgggtgatgccctcagggagatctgtcacctccagcacccgccccaggacaacatctgctgtccccaggtcagtggaggcagatttgagtgcttgtctcttgccccggtttccatgcttcagtccactctgtcccttcaacatttgaaagacgactctcatcccatgtaaacaacattgactgccttgcatcagaatgtctgcctggtgcaccgtgtaagttgactggccatggagcaagggagggcagatggacagattgtactgtaatggctggcccaaaagggagtagcgcccatcaccctgtgctggacccccaggccgggggaactgtgtgaggacaggcaggggactgagtcctgtgcagacactgctgaggctggtgacaggagagggtgctggagactgggtaggagatgtgacagggctgctgctcatttgtgtgttggcctgggggctgctgtcaggactgtacaggtctccaggcttctgcccccgctggtccatgctgtagtatttacaatgactccactggaccatggatgggttctgagggggctggggtccattagggacattcagctgcatgaccactacacctggtccagaaggtgacactcctgagtactgctgtggcatctgtggtggactgcagggagagggagactgaggcatctggtactgctcagagccagggggttgcagaaaccctacagaagggctcgtaccgttctgctgagcaggtgggatcatgctatagtacactggtacccccgctgctgggaggcctccttgcacagactggctcacagggaccagcatgggttgctggaaaggcggctggaccacattttgcgagtcactacccactggaacttggtaagaaggcagtggagtgtactgaaccaccaggccttgcatctggccccccatgctgctcctctggctgctgagcaggccctggttctgtggctgctggaccccaatcatgccttggtaagccgcctgctgctggttaggcatcatgggctgtaaaccaggctgctgggatggctgaggcagctgctgaccacgttgggggctataggccaccgggtgagagagaggtcgatattgctggttggagttaggatattgtccagggggatagtaagaaacctggatctgttgagggggctgcatgtacccctggggtggcagaacttgctgagtaggtggtgcatggctagaggtggaatagttggaagtggggaggggctgacccgtggaagccatgatgaagctagtctgctgagggtgctgggagataagtggggtctggaatagagctgcagatgggtcagctgcttcagtagaaccttggcgactaaggctcatttgtccaaaggggttgctgaggtcatctgccatgttgtactgctggggcggagagactggcagaaggacttggggacaggagcttggagagaactgaacaggctgcggagagggctgcagagccgggactggctgtgagatcatgtgattattcaagggtggctgttgctgaggcgtgggtgggagagcaggaagttgctgctgctgctgctgctgttgctgctgggcagtacaagggagaagcccccggacagactgggatgaggtgacctggttgcacacttctggggcacctagtgccatacctggcctggagatccttcccgcactgccgcctttactgctgccgatgctgtcacctcgggtaaggatagagattccactgaagctgctagctttggtgacagggggtcgcatgctccggacagagccatcagagtctgtgctgctccaagggcgtggctccagggatttgagttcgctgtctgtgctgctctggcggctgcttgaggtgcggctcagtccttcacggttccccctaaaaatctgccttctcttgtgagagctagaagaaaaggcttctttggagagtctgatgtcatttagatatccgttctggccagtctctcgggcaaatattctctctcggaccctttgatattcctcctctctctcttctattgacttgctcctccttccatcctgcaatggaactctgatctggttatcatctcggtccatactggcatcatctctcttgagaatgaacctctgttgaaattctgtattcttctcatcctttatatgttctgagaacctctgttcagggattcttgtgttactagttttgttgatgatgacagctttcccagtttgatcaacattgtggtccatcccaaaataggcagctacccggtgtaatagcatccggtgatatgaggtcatctgagggaacttcttgaactgattattgttgtcattaataaattccagaatctcctgttctaattttagcagcatcattctgtcccttgggttctttttcagtgtatttacaagaaattcatgtaggtctattccagtggagtccgtatattcctggctggagtctctggacagcatcttccttgggatcttttctttgtttttgtccttgtcttccttttcagagacatcttttgtggacttttcttcctccttgtcagaagggcaactgatgtgcaattgaattatatcctgggtttctaatggcccatcagcaaatggggtggaggactcctcacacactgccaggctacgcaccaactttagcttggaattagacttggctcttttcctggcatgaccatggttagatgtccgcctcagcatggccttgggtaggtgaggatttctcttttcttggtcttcttcactagttagcaaataacacggccacaatgcaaaatggagaactgggaaggtggatggaaagaataagaaatgatggtggatctgctcagtggtaagatctgttgcagtaagggaagattcatagtccagaaatatgaagcagtatttgtcactactttttcaaacaggcaatacatacaacatggcacaaagattcaaaaggcataatggggatatatatagaacagtaagtctcctttcataattgtcccccagatacttggttctctcctaaatggtcaaccagtattaaagttcttttggatatatccaggtatcttttaggcatatataagcttagt

SEQ ID NO: 17347 - RNA, 3860 nt, Homo sapiens
  source 1..3860: mol_type = other RNA
tcaggccaggcacagtggctcacgcctgtaatcccagcactctggaaggccaaggcaggtggatcacctgaggtcaggagtttgaggccagcctggccaacatggtgaaactccgtctctactaaaaatacaaaaattagccgggcatggtggcgcgtgtctgtagtgccagctacttgggaggctgaggcaggagaatcacctgaacccaggagctggaggttgcagttagccaagatcgtgctactgcactccagctggggtgacaagagcgaaactccgtctcaaaaaaaaaaaaaaaaaaaaaaagaagaggatgggaagaagagtgatgcaaggggggtcaaccagggaaaaagagaggacccatggcaggggagcaagaaggagtccaatgccagtgtaggtatctgtgtttccatcttcatcactgtcttaggttccagtttaacatcagtttccttacttcctgcctctgtccatggtctgtcaggatccttcaaccccctccaccctgcccttgctccttctgtgacagtccctttcccctcctccatttattgggagctggctcgctccaggatcctcaggtcatagttctttttggccattcgaagtttgaagcgactcacggagttgttgagacgaagggaggcattttgggcagccagggggctggggaacacagccacaatggtgtacaaggcagcgaggtccgagtggcggccattctcagcagtcccactgttgtcccccccaccccctccaggcagcccctgagcatccttgagccactggatcttggcgccagacatggcgagctgcgtgaagagtttgtccgcctcagtacgggtgatgccctcagggagatctgtcacctccagcacccgccccaggacaacatctgctgtccccaggtcagtggaggcagatttgagtgcttgtctcttgccccggtttccatgcttcagtccactctgtcccttcaacatttgaaagacgactctcatcccatgtaaacaacattgactgccttgcatcagaatgtctgcctggtgcaccgtgtaagttgactggccatggagcaagggagggcagatggacagattgtactgtaatggctggcccaaaagggagtagcgcccatcaccctgtgctggacccccaggccgggggaactgtgtgaggacaggcaggggactgagtcctgtgcagacactgctgaggctggtgacaggagagggtgctggagactgggtaggagatgtgacagggctgctgctcatttgtgtgttggcctgggggctgctgtcaggactgtacaggtctccaggcttctgcccccgctggtccatgctgtagtatttacaatgactccactggaccatggatgggttctgagggggctggggtccattagggacattcagctgcatgaccactacacctggtccagaaggtgacactcctgagtactgctgtggcatctgtggtggactgcagggagagggagactgaggcatctggtactgctcagagccagggggttgcagaaaccctacagaagggctcgtaccgttctgctgagcaggtgggatcatgctatagtacactggtacccccgctgctgggaggcctccttgcacagactggctcacagggaccagcatgggttgctggaaaggcggctggaccacattttgcgagtcactacccactggaacttggtaagaaggcagtggagtgtactgaaccaccaggccttgcatctggccccccatgctgctcctctggctgctgagcaggccctggttctgtggctgctggaccccaatcatgccttggtaagccgcctgctgctggttaggcatcatgggctgtaaaccaggctgctgggatggctgaggcagctgctgaccacgttgggggctataggccaccgggtgagagagaggtcgatattgctggttggagttaggatattgtccagggggatagtaagaaacctggatctgttgagggggctgcatgtacccctggggtggcagaacttgctgagtaggtggtgcatggctagaggtggaatagttggaagtggggaggggctgacccgtggaagccatgatgaagctagtctgctgagggtgctgggagataagtggggtctggaatagagctgcagatgggtcagctgcttcagtagaaccttggcgactaaggctcatttgtccaaaggggttgctgaggtcatctgccatgttgtactgctggggcggagagactggcagaaggacttggggacaggagcttggagagaactgaacaggctgcggagagggctgcagagccgggactggctgtgagatcatgtgattattcaagggtggctgttgctgaggcgtgggtgggagagcaggaagttgctgctgctgctgctgctgttgctgctgggcagtacaagggagaagcccccggacagactgggatgaggtgacctggttgcacacttctggggcacctagtgccatacctggcctggagatccttcccgcactgccgcctttactgctgccgatgctgtcacctcgggtaaggatagagattccactgaagctgctagctttggtgacagggggtcgcatgctccggacagagccatcagagtctgtgctgctccaagggcgtggctccagggatttgagttcgctgtctgtgctgctctggcggctgcttgaggtgcggctcagtccttcacggttccccctaaaaatctgccttctcttgtgagagctagaagaaaaggcttctttggagagtctgatgtcatttagatatccgttctggccagtctctcgggcaaatattctctctcggaccctttgatattcctcctctctctcttctattgacttgctcctccttccatcctgcaatggaactctgatctggttatcatctcggtccatactggcatcatctctcttgagaatgaacctctgttgaaattctgtattcttctcatcctttatatgttctgagaacctctgttcagggattcttgtgttactagttttgttgatgatgacagctttcccagtttgatcaacattgtggtccatcccaaaataggcagctacccggtgtaatagcatccggtgatatgaggtcatctgagggaacttcttgaactgattattgttgtcattaataaattccagaatctcctgttctaattttagcagcatcattctgtcccttgggttctttttcagtgtatttacaagaaattcatgtaggtctattccagtggagtccgtatattcctggctggagtctctggacagcatcttccttgggatcttttctttgtttttgtccttgtcttccttttcagagacatcttttgtggacttttcttcctccttgtcagaagggcaactgatgtgcaattgaattatatcctgggtttctaatggcccatcagcaaatggggtggaggactcctcacacactgccaggctacgcaccaactttagcttggaattagacttggctcttttcctggcatgaccatggttagatgtccgcctctgtgtctcctgacgcaaactggtatcttcacattctttctcaatttcttccttacttggagtcttagatataaacttgtttttgtttacagattcttccaccagttttttttctgattctttcattatttccagggtctcttgagtagtgttactgttagacatgttcttcaatagaatacagtggcctctatggactcctgaataaatgctcagcctccatgagtccagtgctggaatggcatcacatataagaaacaagtctaacct

SEQ ID NO: 17348 - RNA, 3980 nt, Homo sapiens
  source 1..3980: mol_type = other RNA
tcaggccaggcacagtggctcacgcctgtaatcccagcactctggaaggccaaggcaggtggatcacctgaggtcaggagtttgaggccagcctggccaacatggtgaaactccgtctctactaaaaatacaaaaattagccgggcatggtggcgcgtgtctgtagtgccagctacttgggaggctgaggcaggagaatcacctgaacccaggagctggaggttgcagttagccaagatcgtgctactgcactccagctggggtgacaagagcgaaactccgtctcaaaaaaaaaaaaaaaaaaaaaaagaagaggatgggaagaagagtgatgcaaggggggtcaaccagggaaaaagagaggacccatggcaggggagcaagaaggagtccaatgccagtgtaggtatctgtgtttccatcttcatcactgtcttaggttccagtttaacatcagtttccttacttcctgcctctgtccatggtctgtcaggatccttcaaccccctccaccctgcccttgctccttctgtgacagtccctttcccctcctccatttattgggagctggctcgctccaggatcctcaggtcatagttctttttggccattcgaagtttgaagcgactcacggagttgttgagacgaagggaggcattttgggcagccagggggctggggaacacagccacaatggtgtacaaggcagcgaggtccgagtggcggccattctcagcagtcccactgttgtcccccccaccccctccaggcagcccctgagcatccttgagccactggatcttggcgccagacatggcgagctgcgtgaagagtttgtccgcctcagtacgggtgatgccctcagggagatctgtcacctccagcacccgccccaggacaacatctgctgtccccaggtcagtggaggcagatttgagtgcttgtctcttgccccggtttccatgcttcagtccactctgtcccttcaacatttgaaagacgactctcatcccatgtaaacaacattgactgccttgcatcagaatgtctgcctggtgcaccgtgtaagttgactggccatggagcaagggagggcagatggacagattgtactgtaatggctggcccaaaagggagtagcgcccatcaccctgtgctggacccccaggccgggggaactgtgtgaggacaggcaggggactgagtcctgtgcagacactgctgaggctggtgacaggagagggtgctggagactgggtaggagatgtgacagggctgctgctcatttgtgtgttggcctgggggctgctgtcaggactgtacaggtctccaggcttctgcccccgctggtccatgctgtagtatttacaatgactccactggaccatggatgggttctgagggggctggggtccattagggacattcagctgcatgaccactacacctggtccagaaggtgacactcctgagtactgctgtggcatctgtggtggactgcagggagagggagactgaggcatctggtactgctcagagccagggggttgcagaaaccctacagaagggctcgtaccgttctgctgagcaggtgggatcatgctatagtacactggtacccccgctgctgggaggcctccttgcacagactggctcacagggaccagcatgggttgctggaaaggcggctggaccacattttgcgagtcactacccactggaacttggtaagaaggcagtggagtgtactgaaccaccaggccttgcatctggccccccatgctgctcctctggctgctgagcaggccctggttctgtggctgctggaccccaatcatgccttggtaagccgcctgctgctggttaggcatcatgggctgtaaaccaggctgctgggatggctgaggcagctgctgaccacgttgggggctataggccaccgggtgagagagaggtcgatattgctggttggagttaggatattgtccagggggatagtaagaaacctggatctgttgagggggctgcatgtacccctggggtggcagaacttgctgagtaggtggtgcatggctagaggtggaatagttggaagtggggaggggctgacccgtggaagccatgatgaagctagtctgctgagggtgctgggagataagtggggtctggaatagagctgcagatgggtcagctgcttcagtagaaccttggcgactaaggctcatttgtccaaaggggttgctgaggtcatctgccatgttgtactgctggggcggagagactggcagaaggacttggggacaggagcttggagagaactgaacaggctgcggagagggctgcagagccgggactggctgtgagatcatgtgattattcaagggtggctgttgctgaggcgtgggtgggagagcaggaagttgctgctgctgctgctgctgttgctgctgggcagtacaagggagaagcccccggacagactgggatgaggtgacctggttgcacacttctggggcacctagtgccatacctggcctggagatccttcccgcactgccgcctttactgctgccgatgctgtcacctcgggtaaggatagagattccactgaagctgctagctttggtgacagggggtcgcatgctccggacagagccatcagagtctgtgctgctccaagggcgtggctccagggatttgagttcgctgtctgtgctgctctggcggctgcttgaggtgcggctcagtccttcacggttccccctaaaaatctgccttctcttgtgagagctagaagaaaaggcttctttggagagtctgatgtcatttagatatccgttctggccagtctctcgggcaaatattctctctcggaccctttgatattcctcctctctctcttctattgacttgctcctccttccatcctgcaatggaactctgatctggttatcatctcggtccatactggcatcatctctcttgagaatgaacctctgttgaaattctgtattcttctcatcctttatatgttctgagaacctctgttcagggattcttgtgttactagttttgttgatgatgacagctttcccagtttgatcaacattgtggtccatcccaaaataggcagctacccggtgtaatagcatccggtgatatgaggtcatctgagggaacttcttgaactgattattgttgtcattaataaattccagaatctcctgttctaattttagcagcatcattctgtcccttgggttctttttcagtgtatttacaagaaattcatgtaggtctattccagtggagtccgtatattcctggctggagtctctggacagcatcttccttgggatcttttctttgtttttgtccttgtcttccttttcagagacatcttttgtggacttttcttcctccttgtcagaagggcaactgatgtgcaattgaattatatcctgggtttctaatggcccatcagcaaatggggtggaggactcctcacacactgccaggctacgcaccaactttagcttggaattagacttggctcttttcctggcatgaccatggttagatgtccgcctcttgtcaaaaaggaactcataatcctgtgtctcctgacgcaaactggtatcttcacattctttctcaatttcttccttacttggagtcttagatataaacttgtttttgtttacagattcttccaccagttttttttctgattctttcattatttccagggtctcttgagtagtgttactgttagacatgttcttcaatagaatacagtggcctctatggactcctgaataaatgctcagcctccatgagtccagtgctggaatggcatcacatataagaaacaagtctaacctctcgcacgggccttggcggggagggcgcccacgtctccgcccgccgcccgggcccacggccgctcggctgcggctcggccccgacggccggcggcg

SEQ ID NO: 17349 - RNA, 3903 nt, Homo sapiens
  source 1..3903: mol_type = other RNA
tcaggccaggcacagtggctcacgcctgtaatcccagcactctggaaggccaaggcaggtggatcacctgaggtcaggagtttgaggccagcctggccaacatggtgaaactccgtctctactaaaaatacaaaaattagccgggcatggtggcgcgtgtctgtagtgccagctacttgggaggctgaggcaggagaatcacctgaacccaggagctggaggttgcagttagccaagatcgtgctactgcactccagctggggtgacaagagcgaaactccgtctcaaaaaaaaaaaaaaaaaaaaaaagaagaggatgggaagaagagtgatgcaaggggggtcaaccagggaaaaagagaggacccatggcaggggagcaagaaggagtccaatgccagtgtaggtatctgtgtttccatcttcatcactgtcttaggttccagtttaacatcagtttccttacttcctgcctctgtccatggtctgtcaggatccttcaaccccctccaccctgcccttgctccttctgtgacagtccctttcccctcctccatttattgggagctggctcgctccaggatcctcaggtcatagttctttttggccattcgaagtttgaagcgactcacggagttgttgagacgaagggaggcattttgggcagccagggggctggggaacacagccacaatggtgtacaaggcagcgaggtccgagtggcggccattctcagcagtcccactgttgtcccccccaccccctccaggcagcccctgagcatccttgagccactggatcttggcgccagacatggcgagctgcgtgaagagtttgtccgcctcagtacgggtgatgccctcagggagatctgtcacctccagcacccgccccaggacaacatctgctgtccccaggtcagtggaggcagatttgagtgcttgtctcttgccccggtttccatgcttcagtccactctgtcccttcaacatttgaaagacgactctcatcccatgtaaacaacattgactgccttgcatcagaatgtctgcctggtgcaccgtgtaagttgactggccatggagcaagggagggcagatggacagattgtactgtaatggctggcccaaaagggagtagcgcccatcaccctgtgctggacccccaggccgggggaactgtgtgaggacaggcaggggactgagtcctgtgcagacactgctgaggctggtgacaggagagggtgctggagactgggtaggagatgtgacagggctgctgctcatttgtgtgttggcctgggggctgctgtcaggactgtacaggtctccaggcttctgcccccgctggtccatgctgtagtatttacaatgactccactggaccatggatgggttctgagggggctggggtccattagggacattcagctgcatgaccactacacctggtccagaaggtgacactcctgagtactgctgtggcatctgtggtggactgcagggagagggagactgaggcatctggtactgctcagagccagggggttgcagaaaccctacagaagggctcgtaccgttctgctgagcaggtgggatcatgctatagtacactggtacccccgctgctgggaggcctccttgcacagactggctcacagggaccagcatgggttgctggaaaggcggctggaccacattttgcgagtcactacccactggaacttggtaagaaggcagtggagtgtactgaaccaccaggccttgcatctggccccccatgctgctcctctggctgctgagcaggccctggttctgtggctgctggaccccaatcatgccttggtaagccgcctgctgctggttaggcatcatgggctgtaaaccaggctgctgggatggctgaggcagctgctgaccacgttgggggctataggccaccgggtgagagagaggtcgatattgctggttggagttaggatattgtccagggggatagtaagaaacctggatctgttgagggggctgcatgtacccctggggtggcagaacttgctgagtaggtggtgcatggctagaggtggaatagttggaagtggggaggggctgacccgtggaagccatgatgaagctagtctgctgagggtgctgggagataagtggggtctggaatagagctgcagatgggtcagctgcttcagtagaaccttggcgactaaggctcatttgtccaaaggggttgctgaggtcatctgccatgttgtactgctggggcggagagactggcagaaggacttggggacaggagcttggagagaactgaacaggctgcggagagggctgcagagccgggactggctgtgagatcatgtgattattcaagggtggctgttgctgaggcgtgggtgggagagcaggaagttgctgctgctgctgctgctgttgctgctgggcagtacaagggagaagcccccggacagactgggatgaggtgacctggttgcacacttctggggcacctagtgccatacctggcctggagatccttcccgcactgccgcctttactgctgccgatgctgtcacctcgggtaaggatagagattccactgaagctgctagctttggtgacagggggtcgcatgctccggacagagccatcagagtctgtgctgctccaagggcgtggctccagggatttgagttcgctgtctgtgctgctctggcggctgcttgaggtgcggctcagtccttcacggttccccctaaaaatctgccttctcttgtgagagctagaagaaaaggcttctttggagagtctgatgtcatttagatatccgttctggccagtctctcgggcaaatattctctctcggaccctttgatattcctcctctctctcttctattgacttgctcctccttccatcctgcaatggaactctgatctggttatcatctcggtccatactggcatcatctctcttgagaatgaacctctgttgaaattctgtattcttctcatcctttatatgttctgagaacctctgttcagggattcttgtgttactagttttgttgatgatgacagctttcccagtttgatcaacattgtggtccatcccaaaataggcagctacccggtgtaatagcatccggtgatatgaggtcatctgagggaacttcttgaactgattattgttgtcattaataaattccagaatctcctgttctaattttagcagcatcattctgtcccttgggttctttttcagtgtatttacaagaaattcatgtaggtctattccagtggagtccgtatattcctggctggagtctctggacagcatcttccttgggatcttttctttgtttttgtccttgtcttccttttcagagacatcttttgtggacttttcttcctccttgtcagaagggcaactgatgtgcaattgaattatatcctgggtttctaatggcccatcagcaaatggggtggaggactcctcacacactgccaggctacgcaccaactttagcttggaattagacttggctcttttcctggcatgaccatggttagatgtccgcctcttgtcaaaaaggaactcataatcctgtgtctcctgacgcaaactggtatcttcacattctttctcaatttcttccttacttggagtcttagatataaacttgtttttgtttacagattcttccaccagttttttttctgattctttcattatttccagggtctcttgagtagtgttactgttagacatgttcttcaatagaatacagtggcctctatggactcctgaataaatgctcagcctccatgagtccagtgctggaatggcatcacatataagaaacaagtctaacctctgtaattccagctactca

SEQ ID NO: 17350 - RNA, 3760 nt, Homo sapiens
  source 1..3760: mol_type = other RNA
tcaggccaggcacagtggctcacgcctgtaatcccagcactctggaaggccaaggcaggtggatcacctgaggtcaggagtttgaggccagcctggccaacatggtgaaactccgtctctactaaaaatacaaaaattagccgggcatggtggcgcgtgtctgtagtgccagctacttgggaggctgaggcaggagaatcacctgaacccaggagctggaggttgcagttagccaagatcgtgctactgcactccagctggggtgacaagagcgaaactccgtctcaaaaaaaaaaaaaaaaaaaaaaagaagaggatgggaagaagagtgatgcaaggggggtcaaccagggaaaaagagaggacccatggcaggggagcaagaaggagtccaatgccagtgtaggtatctgtgtttccatcttcatcactgtcttaggttccagtttaacatcagtttccttacttcctgcctctgtccatggtctgtcaggatccttcaaccccctccaccctgcccttgctccttctgtgacagtccctttcccctcctccatttattgggagctggctcgctccaggatcctcaggtcatagttctttttggccattcgaagtttgaagcgactcacggagttgttgagacgaagggaggcattttgggcagccagggggctggggaacacagccacaatggtgtacaaggcagcgaggtccgagtggcggccattctcagcagtcccactgttgtcccccccaccccctccaggcagcccctgagcatccttgagccactggatcttggcgccagacatggcgagctgcgtgaagagtttgtccgcctcagtacgggtgatgccctcagggagatctgtcacctccagcacccgccccaggacaacatctgctgtccccaggtcagtggaggcagatttgagtgcttgtctcttgccccggtttccatgcttcagtccactctgtcccttcaacatttgaaagacgactctcatcccatgtaaacaacattgactgccttgcatcagaatgtctgcctggtgcaccgtgtaagttgactggccatggagcaagggagggcagatggacagattgtactgtaatggctggcccaaaagggagtagcgcccatcaccctgtgctggacccccaggccgggggaactgtgtgaggacaggcaggggactgagtcctgtgcagacactgctgaggctggtgacaggagagggtgctggagactgggtaggagatgtgacagggctgctgctcatttgtgtgttggcctgggggctgctgtcaggactgtacaggtctccaggcttctgcccccgctggtccatgctgtagtatttacaatgactccactggaccatggatgggttctgagggggctggggtccattagggacattcagctgcatgaccactacacctggtccagaaggtgacactcctgagtactgctgtggcatctgtggtggactgcagggagagggagactgaggcatctggtactgctcagagccagggggttgcagaaaccctacagaagggctcgtaccgttctgctgagcaggtgggatcatgctatagtacactggtacccccgctgctgggaggcctccttgcacagactggctcacagggaccagcatgggttgctggaaaggcggctggaccacattttgcgagtcactacccactggaacttggtaagaaggcagtggagtgtactgaaccaccaggccttgcatctggccccccatgctgctcctctggctgctgagcaggccctggttctgtggctgctggaccccaatcatgccttggtaagccgcctgctgctggttaggcatcatgggctgtaaaccaggctgctgggatggctgaggcagctgctgaccacgttgggggctataggccaccgggtgagagagaggtcgatattgctggttggagttaggatattgtccagggggatagtaagaaacctggatctgttgagggggctgcatgtacccctggggtggcagaacttgctgagtaggtggtgcatggctagaggtggaatagttggaagtggggaggggctgacccgtggaagccatgatgaagctagtctgctgagggtgctgggagataagtggggtctggaatagagctgcagatgggtcagctgcttcagtagaaccttggcgactaaggctcatttgtccaaaggggttgctgaggtcatctgccatgttgtactgctggggcggagagactggcagaaggacttggggacaggagcttggagagaactgaacaggctgcggagagggctgcagagccgggactggctgtgagatcatgtgattattcaagggtggctgttgctgaggcgtgggtgggagagcaggaagttgctgctgctgctgctgctgttgctgctgggcagtacaagggagaagcccccggacagactgggatgaggtgacctggttgcacacttctggggcacctagtgccatacctggcctggagatccttcccgcactgccgcctttactgctgccgatgctgtcacctcgggtaaggatagagattccactgaagctgctagctttggtgacagggggtcgcatgctccggacagagccatcagagtctgtgctgctccaagggcgtggctccagggatttgagttcgctgtctgtgctgctctggcggctgcttgaggtgcggctcagtccttcacggttccccctaaaaatctgccttctcttgtgagagctagaagaaaaggcttctttggagagtctgatgtcatttagatatccgttctggccagtctggttatcatctcggtccatactggcatcatctctcttgagaatgaacctctgttgaaattctgtattcttctcatcctttatatgttctgagaacctctgttcagggattcttgtgttactagttttgttgatgatgacagctttcccagtttgatcaacattgtggtccatcccaaaataggcagctacccggtgtaatagcatccggtgatatgaggtcatctgagggaacttcttgaactgattattgttgtcattaataaattccagaatctcctgttctaattttagcagcatcattctgtcccttgggttctttttcagtgtatttacaagaaattcatgtaggtctattccagtggagtccgtatattcctggctggagtctctggacagcatcttccttgggatcttttctttgtttttgtccttgtcttccttttcagagacatcttttgtggacttttcttcctccttgtcagaagggcaactgatgtgcaattgaattatatcctgggtttctaatggcccatcagcaaatggggtggaggactcctcacacactgccaggctacgcaccaactttagcttggaattagacttggctcttttcctggcatgaccatggttagatgtccgcctctgtgtctcctgacgcaaactggtatcttcacattctttctcaatttcttccttacttggagtcttagatataaacttgtttttgtttacagattcttccaccagttttttttctgattctttcattatttccagggtctcttgagtagtgttactgttagacatgttcttcaatagaatacagtggcctctatggactccgcttcagatggatttttcttcttccttctctccgtcccctccctctcagaagaaaaagactgcaa

SEQ ID NO: 17351 - RNA, 3764 nt, Homo sapiens
  source 1..3764: mol_type = other RNA
tcaggccaggcacagtggctcacgcctgtaatcccagcactctggaaggccaaggcaggtggatcacctgaggtcaggagtttgaggccagcctggccaacatggtgaaactccgtctctactaaaaatacaaaaattagccgggcatggtggcgcgtgtctgtagtgccagctacttgggaggctgaggcaggagaatcacctgaacccaggagctggaggttgcagttagccaagatcgtgctactgcactccagctggggtgacaagagcgaaactccgtctcaaaaaaaaaaaaaaaaaaaaaaagaagaggatgggaagaagagtgatgcaaggggggtcaaccagggaaaaagagaggacccatggcaggggagcaagaaggagtccaatgccagtgtaggtatctgtgtttccatcttcatcactgtcttaggttccagtttaacatcagtttccttacttcctgcctctgtccatggtctgtcaggatccttcaaccccctccaccctgcccttgctccttctgtgacagtccctttcccctcctccatttattgggagctggctcgctccaggatcctcaggtcatagttctttttggccattcgaagtttgaagcgactcacggagttgttgagacgaagggaggcattttgggcagccagggggctggggaacacagccacaatggtgtacaaggcagcgaggtccgagtggcggccattctcagcagtcccactgttgtcccccccaccccctccaggcagcccctgagcatccttgagccactggatcttggcgccagacatggcgagctgcgtgaagagtttgtccgcctcagtacgggtgatgccctcagggagatctgtcacctccagcacccgccccaggacaacatctgctgtccccaggtcagtggaggcagatttgagtgcttgtctcttgccccggtttccatgcttcagtccactctgtcccttcaacatttgaaagacgactctcatcccatgtaaacaacattgactgccttgcatcagaatgtctgcctggtgcaccgtgtaagttgactggccatggagcaagggagggcagatggacagattgtactgtaatggctggcccaaaagggagtagcgcccatcaccctgtgctggacccccaggccgggggaactgtgtgaggacaggcaggggactgagtcctgtgcagacactgctgaggctggtgacaggagagggtgctggagactgggtaggagatgtgacagggctgctgctcatttgtgtgttggcctgggggctgctgtcaggactgtacaggtctccaggcttctgcccccgctggtccatgctgtagtatttacaatgactccactggaccatggatgggttctgagggggctggggtccattagggacattcagctgcatgaccactacacctggtccagaaggtgacactcctgagtactgctgtggcatctgtggtggactgcagggagagggagactgaggcatctggtactgctcagagccagggggttgcagaaaccctacagaagggctcgtaccgttctgctgagcaggtgggatcatgctatagtacactggtacccccgctgctgggaggcctccttgcacagactggctcacagggaccagcatgggttgctggaaaggcggctggaccacattttgcgagtcactacccactggaacttggtaagaaggcagtggagtgtactgaaccaccaggccttgcatctggccccccatgctgctcctctggctgctgagcaggccctggttctgtggctgctggaccccaatcatgccttggtaagccgcctgctgctggttaggcatcatgggctgtaaaccaggctgctgggatggctgaggcagctgctgaccacgttgggggctataggccaccgggtgagagagaggtcgatattgctggttggagttaggatattgtccagggggatagtaagaaacctggatctgttgagggggctgcatgtacccctggggtggcagaacttgctgagtaggtggtgcatggctagaggtggaatagttggaagtggggaggggctgacccgtggaagccatgatgaagctagtctgctgagggtgctgggagataagtggggtctggaatagagctgcagatgggtcagctgcttcagtagaaccttggcgactaaggctcatttgtccaaaggggttgctgaggtcatctgccatgttgtactgctggggcggagagactggcagaaggacttggggacaggagcttggagagaactgaacaggctgcggagagggctgcagagccgggactggctgtgagatcatgtgattattcaagggtggctgttgctgaggcgtgggtgggagagcaggaagttgctgctgctgctgctgctgttgctgctgggcagtacaagggagaagcccccggacagactgggatgaggtgacctggttgcacacttctggggcacctagtgccatacctggcctggagatccttcccgcactgccgcctttactgctgccgatgctgtcacctcgggtaaggatagagattccactgaagctgctagctttggtgacagggggtcgcatgctccggacagagccatcagagtctgtgctgctccaagggcgtggctccagggatttgagttcgctgtctgtgctgctctggcggctgcttgaggtgcggctcagtccttcacggttccccctaaaaatctgccttctcttgtgagagctagaagaaaaggcttctttggagagtctgatgtcatttagatatccgttctggccagtctggttatcatctcggtccatactggcatcatctctcttgagaatgaacctctgttgaaattctgtattcttctcatcctttatatgttctgagaacctctgttcagggattcttgtgttactagttttgttgatgatgacagctttcccagtttgatcaacattgtggtccatcccaaaataggcagctacccggtgtaatagcatccggtgatatgaggtcatctgagggaacttcttgaactgattattgttgtcattaataaattccagaatctcctgttctaattttagcagcatcattctgtcccttgggttctttttcagtgtatttacaagaaattcatgtaggtctattccagtggagtccgtatattcctggctggagtctctggacagcatcttccttgggatcttttctttgtttttgtccttgtcttccttttcagagacatcttttgtggacttttcttcctccttgtcagaagggcaactgatgtgcaattgaattatatcctgggtttctaatggcccatcagcaaatggggtggaggactcctcacacactgccaggctacgcaccaactttagcttggaattagacttggctcttttcctggcatgaccatggttagatgtccgcctctgtgtctcctgacgcaaactggtatcttcacattctttctcaatttcttccttacttggagtcttagatataaacttgtttttgtttacagattcttccaccagttttttttctgattctttcattatttccagggtctcttgagtagtgttactgttagacatgttcttcaatagaatacagtggcctctatggactcctgaataaatgctcagcctccatgagtccagtgctggaatggcatcacatataagaaacaagtctaacct

SEQ ID NO: 17352 - RNA, 3788 nt, Homo sapiens
  source 1..3788: mol_type = other RNA
tcaggccaggcacagtggctcacgcctgtaatcccagcactctggaaggccaaggcaggtggatcacctgaggtcaggagtttgaggccagcctggccaacatggtgaaactccgtctctactaaaaatacaaaaattagccgggcatggtggcgcgtgtctgtagtgccagctacttgggaggctgaggcaggagaatcacctgaacccaggagctggaggttgcagttagccaagatcgtgctactgcactccagctggggtgacaagagcgaaactccgtctcaaaaaaaaaaaaaaaaaaaaaaagaagaggatgggaagaagagtgatgcaaggggggtcaaccagggaaaaagagaggacccatggcaggggagcaagaaggagtccaatgccagtgtaggtatctgtgtttccatcttcatcactgtcttaggttccagtttaacatcagtttccttacttcctgcctctgtccatggtctgtcaggatccttcaaccccctccaccctgcccttgctccttctgtgacagtccctttcccctcctccatttattgggagctggctcgctccaggatcctcaggtcatagttctttttggccattcgaagtttgaagcgactcacggagttgttgagacgaagggaggcattttgggcagccagggggctggggaacacagccacaatggtgtacaaggcagcgaggtccgagtggcggccattctcagcagtcccactgttgtcccccccaccccctccaggcagcccctgagcatccttgagccactggatcttggcgccagacatggcgagctgcgtgaagagtttgtccgcctcagtacgggtgatgccctcagggagatctgtcacctccagcacccgccccaggacaacatctgctgtccccaggtcagtggaggcagatttgagtgcttgtctcttgccccggtttccatgcttcagtccactctgtcccttcaacatttgaaagacgactctcatcccatgtaaacaacattgactgccttgcatcagaatgtctgcctggtgcaccgtgtaagttgactggccatggagcaagggagggcagatggacagattgtactgtaatggctggcccaaaagggagtagcgcccatcaccctgtgctggacccccaggccgggggaactgtgtgaggacaggcaggggactgagtcctgtgcagacactgctgaggctggtgacaggagagggtgctggagactgggtaggagatgtgacagggctgctgctcatttgtgtgttggcctgggggctgctgtcaggactgtacaggtctccaggcttctgcccccgctggtccatgctgtagtatttacaatgactccactggaccatggatgggttctgagggggctggggtccattagggacattcagctgcatgaccactacacctggtccagaaggtgacactcctgagtactgctgtggcatctgtggtggactgcagggagagggagactgaggcatctggtactgctcagagccagggggttgcagaaaccctacagaagggctcgtaccgttctgctgagcaggtgggatcatgctatagtacactggtacccccgctgctgggaggcctccttgcacagactggctcacagggaccagcatgggttgctggaaaggcggctggaccacattttgcgagtcactacccactggaacttggtaagaaggcagtggagtgtactgaaccaccaggccttgcatctggccccccatgctgctcctctggctgctgagcaggccctggttctgtggctgctggaccccaatcatgccttggtaagccgcctgctgctggttaggcatcatgggctgtaaaccaggctgctgggatggctgaggcagctgctgaccacgttgggggctataggccaccgggtgagagagaggtcgatattgctggttggagttaggatattgtccagggggatagtaagaaacctggatctgttgagggggctgcatgtacccctggggtggcagaacttgctgagtaggtggtgcatggctagaggtggaatagttggaagtggggaggggctgacccgtggaagccatgatgaagctagtctgctgagggtgctgggagataagtggggtctggaatagagctgcagatgggtcagctgcttcagtagaaccttggcgactaaggctcatttgtccaaaggggttgctgaggtcatctgccatgttgtactgctggggcggagagactggcagaaggacttggggacaggagcttggagagaactgaacaggctgcggagagggctgcagagccgggactggctgtgagatcatgtgattattcaagggtggctgttgctgaggcgtgggtgggagagcaggaagttgctgctgctgctgctgctgttgctgctgggcagtacaagggagaagcccccggacagactgggatgaggtgacctggttgcacacttctggggcacctagtgccatacctggcctggagatccttcccgcactgccgcctttactgctgccgatgctgtcacctcgggtaaggatagagattccactgaagctgctagctttggtgacagggggtcgcatgctccggacagagccatcagagtctgtgctgctccaagggcgtggctccagggatttgagttcgctgtctgtgctgctctggcggctgcttgaggtgcggctcagtccttcacggttccccctaaaaatctgccttctcttgtgagagctagaagaaaaggcttctttggagagtctgatgtcatttagatatccgttctggccagtctggttatcatctcggtccatactggcatcatctctcttgagaatgaacctctgttgaaattctgtattcttctcatcctttatatgttctgagaacctctgttcagggattcttgtgttactagttttgttgatgatgacagctttcccagtttgatcaacattgtggtccatcccaaaataggcagctacccggtgtaatagcatccggtgatatgaggtcatctgagggaacttcttgaactgattattgttgtcattaataaattccagaatctcctgttctaattttagcagcatcattctgtcccttgggttctttttcagtgtatttacaagaaattcatgtaggtctattccagtggagtccgtatattcctggctggagtctctggacagcatcttccttgggatcttttctttgtttttgtccttgtcttccttttcagagacatcttttgtggacttttcttcctccttgtcagaagggcaactgatgtgcaattgaattatatcctgggtttctaatggcccatcagcaaatggggtggaggactcctcacacactgccaggctacgcaccaactttagcttggaattagacttggctcttttcctggcatgaccatggttagatgtccgcctcttgtcaaaaaggaactcataatcctgtgtctcctgacgcaaactggtatcttcacattctttctcaatttcttccttacttggagtcttagatataaacttgtttttgtttacagattcttccaccagttttttttctgattctttcattatttccagggtctcttgagtagtgttactgttagacatgttcttcaatagaatacagtggcctctatggactcctgaataaatgctcagcctccatgagtccagtgctggaatggcatcacatataagaaacaagtctaacct

SEQ ID NO: 17353 - RNA, 3806 nt, Homo sapiens
  source 1..3806: mol_type = other RNA
tcaggccaggcacagtggctcacgcctgtaatcccagcactctggaaggccaaggcaggtggatcacctgaggtcaggagtttgaggccagcctggccaacatggtgaaactccgtctctactaaaaatacaaaaattagccgggcatggtggcgcgtgtctgtagtgccagctacttgggaggctgaggcaggagaatcacctgaacccaggagctggaggttgcagttagccaagatcgtgctactgcactccagctggggtgacaagagcgaaactccgtctcaaaaaaaaaaaaaaaaaaaaaaagaagaggatgggaagaagagtgatgcaaggggggtcaaccagggaaaaagagaggacccatggcaggggagcaagaaggagtccaatgccagtgtaggtatctgtgtttccatcttcatcactgtcttaggttccagtttaacatcagtttccttacttcctgcctctgtccatggtctgtcaggatccttcaaccccctccaccctgcccttgctccttctgtgacagtccctttcccctcctccatttattgggagctggctcgctccaggatcctcaggtcatagttctttttggccattcgaagtttgaagcgactcacggagttgttgagacgaagggaggcattttgggcagccagggggctggggaacacagccacaatggtgtacaaggcagcgaggtccgagtggcggccattctcagcagtcccactgttgtcccccccaccccctccaggcagcccctgagcatccttgagccactggatcttggcgccagacatggcgagctgcgtgaagagtttgtccgcctcagtacgggtgatgccctcagggagatctgtcacctccagcacccgccccaggacaacatctgctgtccccaggtcagtggaggcagatttgagtgcttgtctcttgccccggtttccatgcttcagtccactctgtcccttcaacatttgaaagacgactctcatcccatgtaaacaacattgactgccttgcatcagaatgtctgcctggtgcaccgtgtaagttgactggccatggagcaagggagggcagatggacagattgtactgtaatggctggcccaaaagggagtagcgcccatcaccctgtgctggacccccaggccgggggaactgtgtgaggacaggcaggggactgagtcctgtgcagacactgctgaggctggtgacaggagagggtgctggagactgggtaggagatgtgacagggctgctgctcatttgtgtgttggcctgggggctgctgtcaggactgtacaggtctccaggcttctgcccccgctggtccatgctgtagtatttacaatgactccactggaccatggatgggttctgagggggctggggtccattagggacattcagctgcatgaccactacacctggtccagaaggtgacactcctgagtactgctgtggcatctgtggtggactgcagggagagggagactgaggcatctggtactgctcagagccagggggttgcagaaaccctacagaagggctcgtaccgttctgctgagcaggtgggatcatgctatagtacactggtacccccgctgctgggaggcctccttgcacagactggctcacagggaccagcatgggttgctggaaaggcggctggaccacattttgcgagtcactacccactggaacttggtaagaaggcagtggagtgtactgaaccaccaggccttgcatctggccccccatgctgctcctctggctgctgagcaggccctggttctgtggctgctggaccccaatcatgccttggtaagccgcctgctgctggttaggcatcatgggctgtaaaccaggctgctgggatggctgaggcagctgctgaccacgttgggggctataggccaccgggtgagagagaggtcgatattgctggttggagttaggatattgtccagggggatagtaagaaacctggatctgttgagggggctgcatgtacccctggggtggcagaacttgctgagtaggtggtgcatggctagaggtggaatagttggaagtggggaggggctgacccgtggaagccatgatgaagctagtctgctgagggtgctgggagataagtggggtctggaatagagctgcagatgggtcagctgcttcagtagaaccttggcgactaaggctcatttgtccaaaggggttgctgaggtcatctgccatgttgtactgctggggcggagagactggcagaaggacttggggacaggagcttggagagaactgaacaggctgcggagagggctgcagagccgggactggctgtgagatcatgtgattattcaagggtggctgttgctgaggcgtgggtgggagagcaggaagttgctgctgctgctgctgctgttgctgctgggcagtacaagggagaagcccccggacagactgggatgaggtgacctggttgcacacttctggggcacctagtgccatacctggcctggagatccttcccgcactgccgcctttactgctgccgatgctgtcacctcgggtaaggatagagattccactgaagctgctagctttggtgacagggggtcgcatgctccggacagagccatcagagtctgtgctgctccaagggcgtggctccagggatttgagttcgctgtctgtgctgctctggcggctgcttgaggtgcggctcagtccttcacggttccccctgatgtcatttagatatccgttctggccagtctctcgggcaaatattctctctcggaccctttgatattcctcctctctctcttctattgacttgctcctccttccatcctgcaatggaactctgatctggttatcatctcggtccatactggcatcatctctcttgagaatgaacctctgttgaaattctgtattcttctcatcctttatatgttctgagaacctctgttcagggattcttgtgttactagttttgttgatgatgacagctttcccagtttgatcaacattgtggtccatcccaaaataggcagctacccggtgtaatagcatccggtgatatgaggtcatctgagggaacttcttgaactgattattgttgtcattaataaattccagaatctcctgttctaattttagcagcatcattctgtcccttgggttctttttcagtgtatttacaagaaattcatgtaggtctattccagtggagtccgtatattcctggctggagtctctggacagcatcttccttgggatcttttctttgtttttgtccttgtcttccttttcagagacatcttttgtggacttttcttcctccttgtcagaagggcaactgatgtgcaattgaattatatcctgggtttctaatggcccatcagcaaatggggtggaggactcctcacacactgccaggctacgcaccaactttagcttggaattagacttggctcttttcctggcatgaccatggttagatgtccgcctctgtgtctcctgacgcaaactggtatcttcacattctttctcaatttcttccttacttggagtcttagatataaacttgtttttgtttacagattcttccaccagttttttttctgattctttcattatttccagggtctcttgagtagtgttactgttagacatgttcttcaatagaatacagtggcctctatggactcctgaataaatgctcagcctccatgagtccagtgctggaatggcatcacatataagaaacaagtctaacct

SEQ ID NO: 17354 - RNA, 3830 nt, Homo sapiens
  source 1..3830: mol_type = other RNA
tcaggccaggcacagtggctcacgcctgtaatcccagcactctggaaggccaaggcaggtggatcacctgaggtcaggagtttgaggccagcctggccaacatggtgaaactccgtctctactaaaaatacaaaaattagccgggcatggtggcgcgtgtctgtagtgccagctacttgggaggctgaggcaggagaatcacctgaacccaggagctggaggttgcagttagccaagatcgtgctactgcactccagctggggtgacaagagcgaaactccgtctcaaaaaaaaaaaaaaaaaaaaaaagaagaggatgggaagaagagtgatgcaaggggggtcaaccagggaaaaagagaggacccatggcaggggagcaagaaggagtccaatgccagtgtaggtatctgtgtttccatcttcatcactgtcttaggttccagtttaacatcagtttccttacttcctgcctctgtccatggtctgtcaggatccttcaaccccctccaccctgcccttgctccttctgtgacagtccctttcccctcctccatttattgggagctggctcgctccaggatcctcaggtcatagttctttttggccattcgaagtttgaagcgactcacggagttgttgagacgaagggaggcattttgggcagccagggggctggggaacacagccacaatggtgtacaaggcagcgaggtccgagtggcggccattctcagcagtcccactgttgtcccccccaccccctccaggcagcccctgagcatccttgagccactggatcttggcgccagacatggcgagctgcgtgaagagtttgtccgcctcagtacgggtgatgccctcagggagatctgtcacctccagcacccgccccaggacaacatctgctgtccccaggtcagtggaggcagatttgagtgcttgtctcttgccccggtttccatgcttcagtccactctgtcccttcaacatttgaaagacgactctcatcccatgtaaacaacattgactgccttgcatcagaatgtctgcctggtgcaccgtgtaagttgactggccatggagcaagggagggcagatggacagattgtactgtaatggctggcccaaaagggagtagcgcccatcaccctgtgctggacccccaggccgggggaactgtgtgaggacaggcaggggactgagtcctgtgcagacactgctgaggctggtgacaggagagggtgctggagactgggtaggagatgtgacagggctgctgctcatttgtgtgttggcctgggggctgctgtcaggactgtacaggtctccaggcttctgcccccgctggtccatgctgtagtatttacaatgactccactggaccatggatgggttctgagggggctggggtccattagggacattcagctgcatgaccactacacctggtccagaaggtgacactcctgagtactgctgtggcatctgtggtggactgcagggagagggagactgaggcatctggtactgctcagagccagggggttgcagaaaccctacagaagggctcgtaccgttctgctgagcaggtgggatcatgctatagtacactggtacccccgctgctgggaggcctccttgcacagactggctcacagggaccagcatgggttgctggaaaggcggctggaccacattttgcgagtcactacccactggaacttggtaagaaggcagtggagtgtactgaaccaccaggccttgcatctggccccccatgctgctcctctggctgctgagcaggccctggttctgtggctgctggaccccaatcatgccttggtaagccgcctgctgctggttaggcatcatgggctgtaaaccaggctgctgggatggctgaggcagctgctgaccacgttgggggctataggccaccgggtgagagagaggtcgatattgctggttggagttaggatattgtccagggggatagtaagaaacctggatctgttgagggggctgcatgtacccctggggtggcagaacttgctgagtaggtggtgcatggctagaggtggaatagttggaagtggggaggggctgacccgtggaagccatgatgaagctagtctgctgagggtgctgggagataagtggggtctggaatagagctgcagatgggtcagctgcttcagtagaaccttggcgactaaggctcatttgtccaaaggggttgctgaggtcatctgccatgttgtactgctggggcggagagactggcagaaggacttggggacaggagcttggagagaactgaacaggctgcggagagggctgcagagccgggactggctgtgagatcatgtgattattcaagggtggctgttgctgaggcgtgggtgggagagcaggaagttgctgctgctgctgctgctgttgctgctgggcagtacaagggagaagcccccggacagactgggatgaggtgacctggttgcacacttctggggcacctagtgccatacctggcctggagatccttcccgcactgccgcctttactgctgccgatgctgtcacctcgggtaaggatagagattccactgaagctgctagctttggtgacagggggtcgcatgctccggacagagccatcagagtctgtgctgctccaagggcgtggctccagggatttgagttcgctgtctgtgctgctctggcggctgcttgaggtgcggctcagtccttcacggttccccctgatgtcatttagatatccgttctggccagtctctcgggcaaatattctctctcggaccctttgatattcctcctctctctcttctattgacttgctcctccttccatcctgcaatggaactctgatctggttatcatctcggtccatactggcatcatctctcttgagaatgaacctctgttgaaattctgtattcttctcatcctttatatgttctgagaacctctgttcagggattcttgtgttactagttttgttgatgatgacagctttcccagtttgatcaacattgtggtccatcccaaaataggcagctacccggtgtaatagcatccggtgatatgaggtcatctgagggaacttcttgaactgattattgttgtcattaataaattccagaatctcctgttctaattttagcagcatcattctgtcccttgggttctttttcagtgtatttacaagaaattcatgtaggtctattccagtggagtccgtatattcctggctggagtctctggacagcatcttccttgggatcttttctttgtttttgtccttgtcttccttttcagagacatcttttgtggacttttcttcctccttgtcagaagggcaactgatgtgcaattgaattatatcctgggtttctaatggcccatcagcaaatggggtggaggactcctcacacactgccaggctacgcaccaactttagcttggaattagacttggctcttttcctggcatgaccatggttagatgtccgcctcttgtcaaaaaggaactcataatcctgtgtctcctgacgcaaactggtatcttcacattctttctcaatttcttccttacttggagtcttagatataaacttgtttttgtttacagattcttccaccagttttttttctgattctttcattatttccagggtctcttgagtagtgttactgttagacatgttcttcaatagaatacagtggcctctatggactcctgaataaatgctcagcctccatgagtccagtgctggaatggcatcacatataagaaacaagtctaacct

SEQ ID NO: 17355 - RNA, 3734 nt, Homo sapiens
  source 1..3734: mol_type = other RNA
tcaggccaggcacagtggctcacgcctgtaatcccagcactctggaaggccaaggcaggtggatcacctgaggtcaggagtttgaggccagcctggccaacatggtgaaactccgtctctactaaaaatacaaaaattagccgggcatggtggcgcgtgtctgtagtgccagctacttgggaggctgaggcaggagaatcacctgaacccaggagctggaggttgcagttagccaagatcgtgctactgcactccagctggggtgacaagagcgaaactccgtctcaaaaaaaaaaaaaaaaaaaaaaagaagaggatgggaagaagagtgatgcaaggggggtcaaccagggaaaaagagaggacccatggcaggggagcaagaaggagtccaatgccagtgtaggtatctgtgtttccatcttcatcactgtcttaggttccagtttaacatcagtttccttacttcctgcctctgtccatggtctgtcaggatccttcaaccccctccaccctgcccttgctccttctgtgacagtccctttcccctcctccatttattgggagctggctcgctccaggatcctcaggtcatagttctttttggccattcgaagtttgaagcgactcacggagttgttgagacgaagggaggcattttgggcagccagggggctggggaacacagccacaatggtgtacaaggcagcgaggtccgagtggcggccattctcagcagtcccactgttgtcccccccaccccctccaggcagcccctgagcatccttgagccactggatcttggcgccagacatggcgagctgcgtgaagagtttgtccgcctcagtacgggtgatgccctcagggagatctgtcacctccagcacccgccccaggacaacatctgctgtccccaggtcagtggaggcagatttgagtgcttgtctcttgccccggtttccatgcttcagtccactctgtcccttcaacatttgaaagacgactctcatcccatgtaaacaacattgactgccttgcatcagaatgtctgcctggtgcaccgtgtaagttgactggccatggagcaagggagggcagatggacagattgtactgtaatggctggcccaaaagggagtagcgcccatcaccctgtgctggacccccaggccgggggaactgtgtgaggacaggcaggggactgagtcctgtgcagacactgctgaggctggtgacaggagagggtgctggagactgggtaggagatgtgacagggctgctgctcatttgtgtgttggcctgggggctgctgtcaggactgtacaggtctccaggcttctgcccccgctggtccatgctgtagtatttacaatgactccactggaccatggatgggttctgagggggctggggtccattagggacattcagctgcatgaccactacacctggtccagaaggtgacactcctgagtactgctgtggcatctgtggtggactgcagggagagggagactgaggcatctggtactgctcagagccagggggttgcagaaaccctacagaagggctcgtaccgttctgctgagcaggtgggatcatgctatagtacactggtacccccgctgctgggaggcctccttgcacagactggctcacagggaccagcatgggttgctggaaaggcggctggaccacattttgcgagtcactacccactggaacttggtaagaaggcagtggagtgtactgaaccaccaggccttgcatctggccccccatgctgctcctctggctgctgagcaggccctggttctgtggctgctggaccccaatcatgccttggtaagccgcctgctgctggttaggcatcatgggctgtaaaccaggctgctgggatggctgaggcagctgctgaccacgttgggggctataggccaccgggtgagagagaggtcgatattgctggttggagttaggatattgtccagggggatagtaagaaacctggatctgttgagggggctgcatgtacccctggggtggcagaacttgctgagtaggtggtgcatggctagaggtggaatagttggaagtggggaggggctgacccgtggaagccatgatgaagctagtctgctgagggtgctgggagataagtggggtctggaatagagctgcagatgggtcagctgcttcagtagaaccttggcgactaaggctcatttgtccaaaggggttgctgaggtcatctgccatgttgtactgctggggcggagagactggcagaaggacttggggacaggagcttggagagaactgaacaggctgcggagagggctgcagagccgggactggctgtgagatcatgtgattattcaagggtggctgttgctgaggcgtgggtgggagagcaggaagttgctgctgctgctgctgctgttgctgctgggcagtacaagggagaagcccccggacagactgggatgaggtgacctggttgcacacttctggggcacctagtgccatacctggcctggagatccttcccgcactgccgcctttactgctgccgatgctgtcacctcgggtaaggatagagattccactgaagctgctagctttggtgacagggggtcgcatgctccggacagagccatcagagtctgtgctgctccaagggcgtggctccagggatttgagttcgctgtctgtgctgctctggcggctgcttgaggtgcggctcagtccttcacggttccccctgatgtcatttagatatccgttctggccagtctggttatcatctcggtccatactggcatcatctctcttgagaatgaacctctgttgaaattctgtattcttctcatcctttatatgttctgagaacctctgttcagggattcttgtgttactagttttgttgatgatgacagctttcccagtttgatcaacattgtggtccatcccaaaataggcagctacccggtgtaatagcatccggtgatatgaggtcatctgagggaacttcttgaactgattattgttgtcattaataaattccagaatctcctgttctaattttagcagcatcattctgtcccttgggttctttttcagtgtatttacaagaaattcatgtaggtctattccagtggagtccgtatattcctggctggagtctctggacagcatcttccttgggatcttttctttgtttttgtccttgtcttccttttcagagacatcttttgtggacttttcttcctccttgtcagaagggcaactgatgtgcaattgaattatatcctgggtttctaatggcccatcagcaaatggggtggaggactcctcacacactgccaggctacgcaccaactttagcttggaattagacttggctcttttcctggcatgaccatggttagatgtccgcctcttgtcaaaaaggaactcataatcctgtgtctcctgacgcaaactggtatcttcacattctttctcaatttcttccttacttggagtcttagatataaacttgtttttgtttacagattcttccaccagttttttttctgattctttcattatttccagggtctcttgagtagtgttactgttagacatgttcttcaatagaatacagtggcctctatggactcctgaataaatgctcagcctccatgagtccagtgctggaatggcatcacatataagaaacaagtctaacct

SEQ ID NO: 17356 - RNA, 3782 nt, Homo sapiens
  source 1..3782: mol_type = other RNA
tcaggccaggcacagtggctcacgcctgtaatcccagcactctggaaggccaaggcaggtggatcacctgaggtcaggagtttgaggccagcctggccaacatggtgaaactccgtctctactaaaaatacaaaaattagccgggcatggtggcgcgtgtctgtagtgccagctacttgggaggctgaggcaggagaatcacctgaacccaggagctggaggttgcagttagccaagatcgtgctactgcactccagctggggtgacaagagcgaaactccgtctcaaaaaaaaaaaaaaaaaaaaaaagaagaggatgggaagaagagtgatgcaaggggggtcaaccagggaaaaagagaggacccatggcaggggagcaagaaggagtccaatgccagtgtaggtatctgtgtttccatcttcatcactgtcttaggttccagtttaacatcagtttccttacttcctgcctctgtccatggtctgtcaggatccttcaaccccctccaccctgcccttgctccttctgtgacagtccctttcccctcctccatttattgggagctggctcgctccaggatcctcaggtcatagttctttttggccattcgaagtttgaagcgactcacggagttgttgagacgaagggaggcattttgggcagccagggggctggggaacacagccacaatggtgtacaaggcagcgaggtccgagtggcggccattctcagcagtcccactgttgtcccccccaccccctccaggcagcccctgagcatccttgagccactggatcttggcgccagacatggcgagctgcgtgaagagtttgtccgcctcagtacgggtgatgccctcagggagatctgtcacctccagcacccgccccaggacaacatctgctgtccccaggtcagtggaggcagatttgagtgcttgtctcttgccccggtttccatgcttcagtccactctgtcccttcaacatttgaaagacgactctcatcccatgtaaacaacattgactgccttgcatcagaatgtctgcctggtgcaccgtgtaagttgactggccatggagcaagggagggcagatggacagattgtactgtaatggctggcccaaaagggagtagcgcccatcaccctgtgctggacccccaggccgggggaactgtgtgaggacaggcaggggactgagtcctgtgcagacactgctgaggctggtgacaggagagggtgctggagactgggtaggagatgtgacagggctgctgctcatttgtgtgttggcctgggggctgctgtcaggactgtacaggtctccaggcttctgcccccgctggtccatgctgtagtatttacaatgactccactggaccatggatgggttctgagggggctggggtccattagggacattcagctgcatgaccactacacctggtccagaaggtgacactcctgagtactgctgtggcatctgtggtggactgcagggagagggagactgaggcatctggtactgctcagagccagggggttgcagaaaccctacagaagggctcgtaccgttctgctgagcaggtgggatcatgctatagtacactggtacccccgctgctgggaggcctccttgcacagactggctcacagggaccagcatgggttgctggaaaggcggctggaccacattttgcgagtcactacccactggaacttggtaagaaggcagtggagtgtactgaaccaccaggccttgcatctggccccccatgctgctcctctggctgctgagcaggccctggttctgtggctgctggaccccaatcatgccttggtaagccgcctgctgctggttaggcatcatgggctgtaaaccaggctgctgggatggctgaggcagctgctgaccacgttgggggctataggccaccgggtgagagagaggtcgatattgctggttggagttaggatattgtccagggggatagtaagaaacctggatctgttgagggggctgcatgtacccctggggtggcagaacttgctgagtaggtggtgcatggctagaggtggaatagttggaagtggggaggggctgacccgtggaagccatgatgaagctagtctgctgagggtgctgggagataagtggggtctggaatagagctgcagatgggtcagctgcttcagtagaaccttggcgactaaggctcatttgtccaaaggggttgctgaggtcatctgcctgtgagatcatgtgattattcaagggtggctgttgctgaggcgtgggtgggagagcaggaagttgctgctgctgctgctgctgttgctgctgggcagtacaagggagaagcccccggacagactgggatgaggtgacctggttgcacacttctggggcacctagtgccatacctggcctggagatccttcccgcactgccgcctttactgctgccgatgctgtcacctcgggtaaggatagagattccactgaagctgctagctttggtgacagggggtcgcatgctccggacagagccatcagagtctgtgctgctccaagggcgtggctccagggatttgagttcgctgtctgtgctgctctggcggctgcttgaggtgcggctcagtccttcacggttccccctaaaaatctgccttctcttgtgagagctagaagaaaaggcttctttggagagtctgatgtcatttagatatccgttctggccagtctctcgggcaaatattctctctcggaccctttgatattcctcctctctctcttctattgacttgctcctccttccatcctgcaatggaactctgatctggttatcatctcggtccatactggcatcatctctcttgagaatgaacctctgttgaaattctgtattcttctcatcctttatatgttctgagaacctctgttcagggattcttgtgttactagttttgttgatgatgacagctttcccagtttgatcaacattgtggtccatcccaaaataggcagctacccggtgtaatagcatccggtgatatgaggtcatctgagggaacttcttgaactgattattgttgtcattaataaattccagaatctcctgttctaattttagcagcatcattctgtcccttgggttctttttcagtgtatttacaagaaattcatgtaggtctattccagtggagtccgtatattcctggctggagtctctggacagcatcttccttgggatcttttctttgtttttgtccttgtcttccttttcagagacatcttttgtggacttttcttcctccttgtcagaagggcaactgatgtgcaattgaattatatcctgggtttctaatggcccatcagcaaatggggtggaggactcctcacacactgccaggctacgcaccaactttagcttggaattagacttggctcttttcctggcatgaccatggttagatgtccgcctcttgtcaaaaaggaactcataatcctgtgtctcctgacgcaaactggtatcttcacattctttctcaatttcttccttacttggagtcttagatataaacttgtttttgtttacagattcttccaccagttttttttctgattctttcattatttccagggtctcttgagtagtgttactgttagacatgttcttcaatagaatacagtggcctctatggactcctgaataaatgctcagcctccatgagtccagtgctggaatggcatcacatataagaaacaagtctaacct

SEQ ID NO: 17357 - RNA, 3728 nt, Homo sapiens
  source 1..3728: mol_type = other RNA
tcaggccaggcacagtggctcacgcctgtaatcccagcactctggaaggccaaggcaggtggatcacctgaggtcaggagtttgaggccagcctggccaacatggtgaaactccgtctctactaaaaatacaaaaattagccgggcatggtggcgcgtgtctgtagtgccagctacttgggaggctgaggcaggagaatcacctgaacccaggagctggaggttgcagttagccaagatcgtgctactgcactccagctggggtgacaagagcgaaactccgtctcaaaaaaaaaaaaaaaaaaaaaaagaagaggatgggaagaagagtgatgcaaggggggtcaaccagggaaaaagagaggacccatggcaggggagcaagaaggagtccaatgccagtgtaggtatctgtgtttccatcttcatcactgtcttaggttccagtttaacatcagtttccttacttcctgcctctgtccatggtctgtcaggatccttcaaccccctccaccctgcccttgctccttctgtgacagtccctttcccctcctccatttattgggagctggctcgctccaggatcctcaggtcatagttctttttggccattcgaagtttgaagcgactcacggagttgttgagacgaagggaggcattttgggcagccagggggctggggaacacagccacaatggtgtacaaggcagcgaggtccgagtggcggccattctcagcagtcccactgttgtcccccccaccccctccaggcagcccctgagcatccttgagccactggatcttggcgccagacatggcgagctgcgtgaagagtttgtccgcctcagtacgggtgatgccctcagggagatctgtcacctccagcacccgccccaggacaacatctgctgtccccaggtcagtggaggcagatttgagtgcttgtctcttgccccggtttccatgcttcagtccactctgtcccttcaacatttgaaagacgactctcatcccatgtaaacaacattgactgccttgcatcagaatgtctgcctggtgcaccgtgtaagttgactggccatggagcaagggagggcagatggacagattgtactgtaatggctggcccaaaagggagtagcgcccatcaccctgtgctggacccccaggccgggggaactgtgtgaggacaggcaggggactgagtcctgtgcagacactgctgaggctggtgacaggagagggtgctggagactgggtaggagatgtgacagggctgctgctcatttgtgtgttggcctgggggctgctgtcaggactgtacaggtctccaggcttctgcccccgctggtccatgctgtagtatttacaatgactccactggaccatggatgggttctgagggggctggggtccattagggacattcagctgcatgaccactacacctggtccagaaggtgacactcctgagtactgctgtggcatctgtggtggactgcagggagagggagactgaggcatctggtactgctcagagccagggggttgcagaaaccctacagaagggctcgtaccgttctgctgagcaggtgggatcatgctatagtacactggtacccccgctgctgggaggcctccttgcacagactggctcacagggaccagcatgggttgctggaaaggcggctggaccacattttgcgagtcactacccactggaacttggtaagaaggcagtggagtgtactgaaccaccaggccttgcatctggccccccatgctgctcctctggctgctgagcaggccctggttctgtggctgctggaccccaatcatgccttggtaagccgcctgctgctggttaggcatcatgggctgtaaaccaggctgctgggatggctgaggcagctgctgaccacgttgggggctataggccaccgggtgagagagaggtcgatattgctggttggagttaggatattgtccagggggatagtaagaaacctggatctgttgagggggctgcatgtacccctggggtggcagaacttgctgagtaggtggtgcatggctagaggtggaatagttggaagtggggaggggctgacccgtggaagccatgatgaagctagtctgctgagggtgctgggagataagtggggtctggaatagagctgcagatgggtcagctgcttcagtagaaccttggcgactaaggctcatttgtccaaaggggttgctgaggtcatctgcctgtgagatcatgtgattattcaagggtggctgttgctgaggcgtgggtgggagagcaggaagttgctgctgctgctgctgctgttgctgctgggcagtacaagggagaagcccccggacagactgggatgaggtgacctggttgcacacttctggggcacctagtgccatacctggcctggagatccttcccgcactgccgcctttactgctgccgatgctgtcacctcgggtaaggatagagattccactgaagctgctagctttggtgacagggggtcgcatgctccggacagagccatcagagtctgtgctgctccaagggcgtggctccagggatttgagttcgctgtctgtgctgctctggcggctgcttgaggtgcggctcagtccttcacggttccccctgatgtcatttagatatccgttctggccagtctctcgggcaaatattctctctcggaccctttgatattcctcctctctctcttctattgacttgctcctccttccatcctgcaatggaactctgatctggttatcatctcggtccatactggcatcatctctcttgagaatgaacctctgttgaaattctgtattcttctcatcctttatatgttctgagaacctctgttcagggattcttgtgttactagttttgttgatgatgacagctttcccagtttgatcaacattgtggtccatcccaaaataggcagctacccggtgtaatagcatccggtgatatgaggtcatctgagggaacttcttgaactgattattgttgtcattaataaattccagaatctcctgttctaattttagcagcatcattctgtcccttgggttctttttcagtgtatttacaagaaattcatgtaggtctattccagtggagtccgtatattcctggctggagtctctggacagcatcttccttgggatcttttctttgtttttgtccttgtcttccttttcagagacatcttttgtggacttttcttcctccttgtcagaagggcaactgatgtgcaattgaattatatcctgggtttctaatggcccatcagcaaatggggtggaggactcctcacacactgccaggctacgcaccaactttagcttggaattagacttggctcttttcctggcatgaccatggttagatgtccgcctcttgtcaaaaaggaactcataatcctgtgtctcctgacgcaaactggtatcttcacattctttctcaatttcttccttacttggagtcttagatataaacttgtttttgtttacagattcttccaccagttttttttctgattctttcattatttccagggtctcttgagtagtgttactgttagacatgttcttcaatagaatacagtggcctctatggactcctgaataaatgctcagcctccatgagtccagtgctggaatggcatcacatataagaaacaagtctaacct

SEQ ID NO: 17358 - RNA, 3632 nt, Homo sapiens
  source 1..3632: mol_type = other RNA
tcaggccaggcacagtggctcacgcctgtaatcccagcactctggaaggccaaggcaggtggatcacctgaggtcaggagtttgaggccagcctggccaacatggtgaaactccgtctctactaaaaatacaaaaattagccgggcatggtggcgcgtgtctgtagtgccagctacttgggaggctgaggcaggagaatcacctgaacccaggagctggaggttgcagttagccaagatcgtgctactgcactccagctggggtgacaagagcgaaactccgtctcaaaaaaaaaaaaaaaaaaaaaaagaagaggatgggaagaagagtgatgcaaggggggtcaaccagggaaaaagagaggacccatggcaggggagcaagaaggagtccaatgccagtgtaggtatctgtgtttccatcttcatcactgtcttaggttccagtttaacatcagtttccttacttcctgcctctgtccatggtctgtcaggatccttcaaccccctccaccctgcccttgctccttctgtgacagtccctttcccctcctccatttattgggagctggctcgctccaggatcctcaggtcatagttctttttggccattcgaagtttgaagcgactcacggagttgttgagacgaagggaggcattttgggcagccagggggctggggaacacagccacaatggtgtacaaggcagcgaggtccgagtggcggccattctcagcagtcccactgttgtcccccccaccccctccaggcagcccctgagcatccttgagccactggatcttggcgccagacatggcgagctgcgtgaagagtttgtccgcctcagtacgggtgatgccctcagggagatctgtcacctccagcacccgccccaggacaacatctgctgtccccaggtcagtggaggcagatttgagtgcttgtctcttgccccggtttccatgcttcagtccactctgtcccttcaacatttgaaagacgactctcatcccatgtaaacaacattgactgccttgcatcagaatgtctgcctggtgcaccgtgtaagttgactggccatggagcaagggagggcagatggacagattgtactgtaatggctggcccaaaagggagtagcgcccatcaccctgtgctggacccccaggccgggggaactgtgtgaggacaggcaggggactgagtcctgtgcagacactgctgaggctggtgacaggagagggtgctggagactgggtaggagatgtgacagggctgctgctcatttgtgtgttggcctgggggctgctgtcaggactgtacaggtctccaggcttctgcccccgctggtccatgctgtagtatttacaatgactccactggaccatggatgggttctgagggggctggggtccattagggacattcagctgcatgaccactacacctggtccagaaggtgacactcctgagtactgctgtggcatctgtggtggactgcagggagagggagactgaggcatctggtactgctcagagccagggggttgcagaaaccctacagaagggctcgtaccgttctgctgagcaggtgggatcatgctatagtacactggtacccccgctgctgggaggcctccttgcacagactggctcacagggaccagcatgggttgctggaaaggcggctggaccacattttgcgagtcactacccactggaacttggtaagaaggcagtggagtgtactgaaccaccaggccttgcatctggccccccatgctgctcctctggctgctgagcaggccctggttctgtggctgctggaccccaatcatgccttggtaagccgcctgctgctggttaggcatcatgggctgtaaaccaggctgctgggatggctgaggcagctgctgaccacgttgggggctataggccaccgggtgagagagaggtcgatattgctggttggagttaggatattgtccagggggatagtaagaaacctggatctgttgagggggctgcatgtacccctggggtggcagaacttgctgagtaggtggtgcatggctagaggtggaatagttggaagtggggaggggctgacccgtggaagccatgatgaagctagtctgctgagggtgctgggagataagtggggtctggaatagagctgcagatgggtcagctgcttcagtagaaccttggcgactaaggctcatttgtccaaaggggttgctgaggtcatctgcctgtgagatcatgtgattattcaagggtggctgttgctgaggcgtgggtgggagagcaggaagttgctgctgctgctgctgctgttgctgctgggcagtacaagggagaagcccccggacagactgggatgaggtgacctggttgcacacttctggggcacctagtgccatacctggcctggagatccttcccgcactgccgcctttactgctgccgatgctgtcacctcgggtaaggatagagattccactgaagctgctagctttggtgacagggggtcgcatgctccggacagagccatcagagtctgtgctgctccaagggcgtggctccagggatttgagttcgctgtctgtgctgctctggcggctgcttgaggtgcggctcagtccttcacggttccccctgatgtcatttagatatccgttctggccagtctggttatcatctcggtccatactggcatcatctctcttgagaatgaacctctgttgaaattctgtattcttctcatcctttatatgttctgagaacctctgttcagggattcttgtgttactagttttgttgatgatgacagctttcccagtttgatcaacattgtggtccatcccaaaataggcagctacccggtgtaatagcatccggtgatatgaggtcatctgagggaacttcttgaactgattattgttgtcattaataaattccagaatctcctgttctaattttagcagcatcattctgtcccttgggttctttttcagtgtatttacaagaaattcatgtaggtctattccagtggagtccgtatattcctggctggagtctctggacagcatcttccttgggatcttttctttgtttttgtccttgtcttccttttcagagacatcttttgtggacttttcttcctccttgtcagaagggcaactgatgtgcaattgaattatatcctgggtttctaatggcccatcagcaaatggggtggaggactcctcacacactgccaggctacgcaccaactttagcttggaattagacttggctcttttcctggcatgaccatggttagatgtccgcctcttgtcaaaaaggaactcataatcctgtgtctcctgacgcaaactggtatcttcacattctttctcaatttcttccttacttggagtcttagatataaacttgtttttgtttacagattcttccaccagttttttttctgattctttcattatttccagggtctcttgagtagtgttactgttagacatgttcttcaatagaatacagtggcctctatggactcctgaataaatgctcagcctccatgagtccagtgctggaatggcatcacatataagaaacaagtctaacct

SEQ ID NO: 17359 - RNA, 754 nt, Homo sapiens
  source 1..754: mol_type = other RNA
tcaggccaggcacagtggctcacgcctgtaatcccagcactctggcaaagctgagatgggtgaatcacttgaggccaggagttcgagaccagcctggccaacatggcgaaaccccgtctccactaaaaatacaaaaaattagcagggcacggtggtgcgcacctgtaatcccagttacttgggaggctgaggcaggagaatcgcttgaacccggaaggcagaggttgccatgagccaagatcgtgccactgcactgcagcctgggcgacagagcaagactctgtctcaaaagagaaaaaggaaaaaaaaagaaggaaaaacaacccaaccaactattggttcctctcttaggaatgaagacagtcccaggcaacaactgtaaaactctctggcatttcgctttttattcccaccacacctctttcacagtctctgccaggtgctcctcctccgaggtaaagagcttgtactcaatcttctgttggatggcctccaagatcaactggttatgcctcaggattgtttctaaagtggcatgttctggggtggtcactgcccggaagaaagcatcggcaccaggctcccttcgtatttcctccatgagcaggtccaatggacaggtctttgtctcctgaaccaccagcagcagttgccaaatggctgtggcagagagagtctgcttttctagaactgctgatatcagagaattgaaaccacctgaaccagagtcacgtttcacaagcttctccatgac

SEQ ID NO: 17360 - RNA, 2089 nt, Homo sapiens
  source 1..2089: mol_type = other RNA
tcaggccaggcacagtggctcacgcctgtaatcccagcactttagaaggccaagacaggtggatcgcctgaggtcaggagttggagaccagcctggccaacacggtgaaaccctgtcattactaaaaatgcaaaaattagccgggtgtggtggcgggcacctgtagtcccacctacttgggaggctgaggcaggagaattgcttgaacctgggaggcggaggttgcggtgagccgagatcacgccattgcactccagtctaggtgacaagagtgaaactccatctcaaaaaaacaaaacaaacacaaaaacaaaacaagtaaatcatcttaagctgcatcgtcatcatcatcatccactgcagcgtaaatggcttgattcctcctcttaattttctttctttgttcaggttcatgttcatcactcagcctcttcaatggcaccttggttaagtcctctccattccctgactccacagtcccaccaggtttcccctctctatcaattgtggaatccaccgtatcatcagaagatacaatcatagagcctggcaagatcctgacatcagagaaacttgcagaaaactcagaagcttgatcagaaggttctaccgatggtgtattcatgccactatgtgcacttacaatactatcttcatcttcttcttcatctaacattatttcatctggattaatagaagacagagcagatgtgtctgtattatattcactctggtcttctccagagtcattactctccacatcatcctgttcttcatattcaccacacacatgatgttcttccttggacttctgaagcctaacattgatgtctatgatgccaagttgggcacaaaattcagttgtctgaggattgatcctatgaatcagctgcatttgtgtctgtggcttgctaggatcataacaagcagctgttacactaaagttacatggaaccttgagatcatgattcaatttttccaatacttctttcataccttcttctgttgcactataatcccaccttgcatgcaggccattattttctggcatattccacaggcgcccagtcacattaataagatcatccgtagccctgagaatagtgagccattcaatatcatattccaagtaatcaggagcactggggtcatgttctatctctaatatctgaagaaaatctctatgtggtaagcatttgtccaaggctaaaaatttggttgctctggctgtctgtcctttatcctttgcctgatgctgcatcaaggcggcaaacttcacatgaaggtgggcagaaaaccaataagtaggtttgagatgctctaaaagctctgaggcagctggacttcctaatgtgttattttccacttcttgtcggaaaaaagatttagtcttaagaagttgcttcttatttccataatgatatatacttcttggccaatcatgagacaagaatatatctataggctgcttcagctgttttaatttatagacttcaatatttctcacatgatatatactcctgattgtagatgaattataaggggggcactcaaaatgaccttttcgatagtcatgagatttaaagataccagagattccaccgatccttacacctcggtattttaccacaccagccaaacctaaataataaatgtttggtgccacccagccaccatagggtaactcttgcaaatgatttgaggcttcatggtttcccccaatgaagagcgtgagaactggagcctttttctctccagagtaatacctgtagaaggtttgcatgtgacgatacttgggcggcacggccatgcagcgtagatccgcctcgttgcgcaccgcctggaagtcgccgcagcacagcaagaggtcgacaggccccgggccgcgccgctctgccagcgccagcgtctcatagatcttatccagctcgccgtggcagcagccagccacagccacccgcattctgccggcctgaggaggtgagcgctgcctgcaacgccctacaccacagccagcccaggaccgactgatcgctcagctcccgccaactttaataagtatagccaccgcctgggtgtagactcctgc

SEQ ID NO: 17361 - RNA, 5237 nt, Homo sapiens
  source 1..5237: mol_type = other RNA
tcaggccaggcacagtggctcacgcctgtaatcccagcactttaggaggtcgaggcacgtggatcatctaaggtcaggagttcgaaaccagcctggccaacatggtgaaaccccgtctctactaaaaatacaaaaattagccaggcatggtggtgcacacctataatcacagctactcaggaggctgaggtaggagaatcacttgaacccaggaggtggaggttgcagtgagccgagatcgcgccattgcactccagcctgggcaacaaaaacaaaactccgtctcaaaaaaaaaaaaaaaaaaaaaaatctcatcagaccagaccagtagttaacatttggaatttgatttataatggacaaacatggttgtcttcatttgagaagtttattgagcatttacgtgccaggagtgggctacgagatccagtcaacaaacaaacaatacatactcccagtaataaattaattccaatccattagccaaagtatttttctccaaagtagtaatcaccactgacactaggtataaaatgctccaacaagccgggcgcagtggctcacccctgtaatcccagtactttgggaggccggtggaccacctaaggtcaggagtttgagaccagcctgaccaacatggagaaaccccatctctactaaaaatacaaaattagccaggcgtggtggtgcatgcctgtaatcccagctactcaggagcctgaggcaggagaattgcttgaccccaggaggcggtggttgtggtgagccgagatcgtgccattgcactccagcctgggcaacaagagcaaaactctcaaaaaaaaaaaacaaaaaaaaaaaaaaaaaaaaaaaacgaaatgtgcagaaccttctaactaaaagtaacttccttatttcagaaaaggaaaatcagatctagaagttatttctcaagtagctagaaagcaagagttgatcagaaatgaccaactgctatcaagtttagtgttcctctaagtactgaaaaggacttatgagtactttaagaactctccttttcctaccaaagatattggagcccacatatgtaaatatattttgacttactggagacagagagatggataagaatgaagtttcggtacagcaaatccccatcaacaaaataaaatggcaaggaagggggaaccctaggaaaaatattttagaacatgaccatgtatgacccttacagacaaaagcctttatatatcagtaaaaaaaaaaaaaaaaaaaagaggccgggcgcggtggctcaagcctgtaatcccagcactttgggaggccgaggtaagtggatcatgaggtcaggagatcgagaccatcctggcgaacatggtgaaaccccgtctctactaaaaatacaaaaaaaaaaaaattagctgggcgtgatggcaggcgcctgtagtaccagctaatcgggaggctgaggcaggagaacggcgcaaacccagggggcagagcttgcagtgagccgacatcgcaccactgcactccagcctgggagacagtgagactccgtctcaaaaaaaaaaaaaaaaggccaggtgtggtggctcacacctgtaatcccagcactgtgggaggccaaggcaggcagatcacaaggtcaggagttcgagaccagcctggccaatatggtgaaaccccgcctctactaaaaatacaaaaattagcagggcatggtggtgggtgcctgtagttccagcttctcgggaggctgaggcaggagaattgcttgaacctggaggcagaggttgcagtgagccaagatcaggtcactgcactccagcctggacgacggagactccatctcaaataaataaataactaagtaaaaaaaaaggtaacacattaagaatgagcaaaggctatgaaaaattaaaagtaaataaataaatcagtaggctgggcgtggtggctcacacctgtaatcccagcactttgggaagctgaggcgggcagaccacgaggtcaggagctcaagagcagcatggccaacatggtgaaaccttgtctctactaaaaatacaaaatgttagccgggtgtggtggcatgggcctgtggtcccagctaattgggaggctaaggcaggagaatcgcttgaacccaggaggtgaaaggtgcagtgagctgagattacgccactgctctccagcctaggtgacagagcaagactctgtctcaaaaaaataaataaatcagtaaaaaaaatttaatgcagtaagaatgagcaaaggctatgaaaagctagtaacagaggaaataaagtagctgtgaaaatattaaaagatggccgggcatggtagttcacacctgtaatcccagcactttgggagaccaaggcaggaggatcacttgagccaaggagttcatcatcagcctggacaacatggcaagaccctccctctacaaaaagtagaaaaattggctgggcgtggtggtatgtgcctgtaaccccagctactcaggaggctgaggtggaagaatcaattgaacccaggtggcagaagctgcagtgagctgagatcacaccactgtactccagcctgggtgagagagatggagaccctgtcacaaaacaaacaaaagagatattgacaagttttcataatcctatgcattctatcttctcagcttttgttccagcaattttttcatttccctgagaattttaactgtcctattattttcctgcctacagtacctctttatgcaggtacatcctctgggcagagaagccagctatgctcttcagtattgtcagcctgccacatatatccagtttaggaatttctcttaaacacaaagtactctagaaacttacaaagagcagccgggtgcggtggctcacacctgtaatcccagcactgtggtaggtaggccaaggcaggtggatcacctgaggtcaggagttcgtgaccggcctggccaacatggtgaaaccccgtctctactaaaaatactaaaaaactagccaggcgtggtggtgggcacctgtaatcccagctacgtgggaggctgaggcaagagaattgcttgaacccggagacggaggttgcagtgggccgacagggtgccactgcactccagcctcagtgacagagtgagaatcagtctcaaaaaaaaaaacaaaaaaaaaacttacaaagagctcagccttgaattatctagcccagttgactgtaccaatattcaagtaaaatagatcaagaagcatttgcttaccaatttctcaatttgatcttggttttaaagaataacacaaatgacagaaaacaactatgcattatggaacctttatttttcatgtgatttctgtacataaggagtatgagagtaacccttttacaaatggaactaatttactagaacaatgacaaaactgaactggtatttgatgtgaatccacaggagtttaagcttcaaatccagccaagaaatttgttacaatctctttcagctttgcatctgattgttctgagatctttccatcagccctgatagtgcccaacaaggcttggtgctggctgacgacatgagacaagaaagcattctcaaactttgtaatcttgctgggctccagtttatcaagatatccccttacacccgcatagataacagccacttgttcttcaatagccatgggagaatactgtccttgcttcagcaactcagttagacgcacgccacgactcaaaagttgttgagtggcagcatcgaggtcagaaccgaactgggcaaaagcagcaacctcacgatactgagccaattccagcttcatggtacctgctacctgcttcatagccctggtttgggcagcggatccgacacgagatacagacagaccaacgttaattgcagggcggatacctttgtagaacaattctgtttccaagaagatctgtccgtcagtgatggaaatgacatttgttggaatgtaagcagacacatcaccagcctgtgtttctatgactggcaaagcagtcaaggagccaccaccaaaagcatcgttcattttggctgctctctccagcaaccgggagtgtaggtagaacacatcaccaggataggcctcacgaccagggggtcggcggagcaacagagacatctgacggtaagcaacagcctgtttggataagtcgtcatagatgatcaaagcatgtttgccattgtctctaaaatactctcccatggaacagccagagtaaggagccaggtactgaagtggggcagcatccgaggccgtagccgacaccacaatggtgtacttcatggcatctgcatctgtaagtctcttcaccaactgggcaacagtggatctcttttgaccaatagcaacataaatacagtacagcttcttcttttcatcagatccatcattgaaacgtttctggttaatgattgtgtcaatagcaattgaggttttcccagtctgtcggtcaccaataatcagttcacgctgaccacgaccaattggcaccaagctatccacagccttaatgccagtctgcattggttcccgcactgaaattcgaggaatgataccgggggctttcagaccaactcgcctacgcgtcttggaaccaattggaccctttccatcaatagcattaccaagggcatcaactacacgacccaacagctcctcaccaactggaacgtccacaatggctcctgtcctcttcactatatctccttccttaattagtttatcatttccaaacacgacaacaccaacattgtcaggttccaagttcaaggacataccctttaagcctgaagaaaactctaccatttcttctgcttgaacattcctcagcccatgtacgcgggcaataccatcaccaatacttaagacacgcccagtttcttcaagatcaacagaggtatcagctccaagaatacgctcttcaagaatagaggacatctcagcagtcccacagttatacgatgtatgtaatttatatcttcatctagtaagtgcggcgtagactgagaaataataacttaccagtcttttgaagatgagtgttagaggcatggaagttccttgcagcaatgaaagatgaacccaaagcatttctggagaccagtccggcccgccgaggaagggcgcggaccacggccgcagcaacgcgcacggacagcatctttgcagttactccgcaggcggtacttctgcagccgcagcctccggactgactgggacaaaatg

SEQ ID NO: 17362 - RNA, 5164 nt, Homo sapiens
  source 1..5164: mol_type = other RNA
tcaggccaggcacagtggctcacgcctgtaatcccagcactttaggaggtcgaggcacgtggatcatctaaggtcaggagttcgaaaccagcctggccaacatggtgaaaccccgtctctactaaaaatacaaaaattagccaggcatggtggtgcacacctataatcacagctactcaggaggctgaggtaggagaatcacttgaacccaggaggtggaggttgcagtgagccgagatcgcgccattgcactccagcctgggcaacaaaaacaaaactccgtctcaaaaaaaaaaaaaaaaaaaaaaatctcatcagaccagaccagtagttaacatttggaatttgatttataatggacaaacatggttgtcttcatttgagaagtttattgagcatttacgtgccaggagtgggctacgagatccagtcaacaaacaaacaatacatactcccagtaataaattaattccaatccattagccaaagtatttttctccaaagtagtaatcaccactgacactaggtataaaatgctccaacaagccgggcgcagtggctcacccctgtaatcccagtactttgggaggccggtggaccacctaaggtcaggagtttgagaccagcctgaccaacatggagaaaccccatctctactaaaaatacaaaattagccaggcgtggtggtgcatgcctgtaatcccagctactcaggagcctgaggcaggagaattgcttgaccccaggaggcggtggttgtggtgagccgagatcgtgccattgcactccagcctgggcaacaagagcaaaactctcaaaaaaaaaaaacaaaaaaaaaaaaaaaaaaaaaaaacgaaatgtgcagaaccttctaactaaaagtaacttccttatttcagaaaaggaaaatcagatctagaagttatttctcaagtagctagaaagcaagagttgatcagaaatgaccaactgctatcaagtttagtgttcctctaagtactgaaaaggacttatgagtactttaagaactctccttttcctaccaaagatattggagcccacatatgtaaatatattttgacttactggagacagagagatggataagaatgaagtttcggtacagcaaatccccatcaacaaaataaaatggcaaggaagggggaaccctaggaaaaatattttagaacatgaccatgtatgacccttacagacaaaagcctttatatatcagtaaaaaaaaaaaaaaaaaaaagaggccgggcgcggtggctcaagcctgtaatcccagcactttgggaggccgaggtaagtggatcatgaggtcaggagatcgagaccatcctggcgaacatggtgaaaccccgtctctactaaaaatacaaaaaaaaaaaaattagctgggcgtgatggcaggcgcctgtagtaccagctaatcgggaggctgaggcaggagaacggcgcaaacccagggggcagagcttgcagtgagccgacatcgcaccactgcactccagcctgggagacagtgagactccgtctcaaaaaaaaaaaaaaaaggccaggtgtggtggctcacacctgtaatcccagcactgtgggaggccaaggcaggcagatcacaaggtcaggagttcgagaccagcctggccaatatggtgaaaccccgcctctactaaaaatacaaaaattagcagggcatggtggtgggtgcctgtagttccagcttctcgggaggctgaggcaggagaattgcttgaacctggaggcagaggttgcagtgagccaagatcaggtcactgcactccagcctggacgacggagactccatctcaaataaataaataactaagtaaaaaaaaaggtaacacattaagaatgagcaaaggctatgaaaaattaaaagtaaataaataaatcagtaggctgggcgtggtggctcacacctgtaatcccagcactttgggaagctgaggcgggcagaccacgaggtcaggagctcaagagcagcatggccaacatggtgaaaccttgtctctactaaaaatacaaaatgttagccgggtgtggtggcatgggcctgtggtcccagctaattgggaggctaaggcaggagaatcgcttgaacccaggaggtgaaaggtgcagtgagctgagattacgccactgctctccagcctaggtgacagagcaagactctgtctcaaaaaaataaataaatcagtaaaaaaaatttaatgcagtaagaatgagcaaaggctatgaaaagctagtaacagaggaaataaagtagctgtgaaaatattaaaagatggccgggcatggtagttcacacctgtaatcccagcactttgggagaccaaggcaggaggatcacttgagccaaggagttcatcatcagcctggacaacatggcaagaccctccctctacaaaaagtagaaaaattggctgggcgtggtggtatgtgcctgtaaccccagctactcaggaggctgaggtggaagaatcaattgaacccaggtggcagaagctgcagtgagctgagatcacaccactgtactccagcctgggtgagagagatggagaccctgtcacaaaacaaacaaaagagatattgacaagttttcataatcctatgcattctatcttctcagcttttgttccagcaattttttcatttccctgagaattttaactgtcctattattttcctgcctacagtacctctttatgcaggtacatcctctgggcagagaagccagctatgctcttcagtattgtcagcctgccacatatatccagtttaggaatttctcttaaacacaaagtactctagaaacttacaaagagcagccgggtgcggtggctcacacctgtaatcccagcactgtggtaggtaggccaaggcaggtggatcacctgaggtcaggagttcgtgaccggcctggccaacatggtgaaaccccgtctctactaaaaatactaaaaaactagccaggcgtggtggtgggcacctgtaatcccagctacgtgggaggctgaggcaagagaattgcttgaacccggagacggaggttgcagtgggccgacagggtgccactgcactccagcctcagtgacagagtgagaatcagtctcaaaaaaaaaaacaaaaaaaaaacttacaaagagctcagccttgaattatctagcccagttgactgtaccaatattcaagtaaaatagatcaagaagcatttgcttaccaatttctcaatttgatcttggttttaaagaataacacaaatgacagaaaacaactatgcattatggaacctttatttttcatgtgatttctgtacataaggagtatgagagtaacccttttacaaatggaactaatttactagaacaatgacaaaactgaactggtatttgatgtgaatccacaggagtttaagcttcaaatccagccaagaaatttgttacaatctctttcagctttgcatctgattgttctgagatctttccatcagccctgatagtgcccaacaaggcttggtgctggctgacgacatgagacaagaaagcattctcaaactttgtaatcttgctgggctccagtttatcaagatatccccttacacccgcatagataacagccacttgttcttcaatagccatgggagaatactgtccttgcttcagcaactcagttagacgcacgccacgactcaaaagttgttgagtggcagcatcgaggtcagaaccgaactgggcaaaagcagcaacctcacgatactgagccaattccagcttcatggtacctgctacctgcttcatagccctggtttgggcagcggatccgacacgagatacagacagaccaacgttaattgcagggcggatacctttgtagaacaattctgtttccaagaagatctgtccgtcagtgatggaaatgacatttgttggaatgtaagcagacacatcaccagcctgtgtttctatgactggcaaagcagtcaaggagccaccaccaaaagcatcgttcattttggctgctctctccagcaaccgggagtgtaggtagaacacatcaccaggataggcctcacgaccagggggtcggcggagcaacagagacatctgacggtaagcaacagcctgtttggataagtcgtcatagatgatcaaagcatgtttgccattgtctctaaaatactctcccatggaacagccagagtaaggagccaggtactgaagtggggcagcatccgaggccgtagccgacaccacaatggtgtacttcatggcatctgcatctgtaagtctcttcaccaactgggcaacagtggatctcttttgaccaatagcaacataaatacagtacagcttcttcttttcatcagatccatcattgaaacgtttctggttaatgattgtgtcaatagcaattgaggttttcccagtctgtcggtcaccaataatcagttcacgctgaccacgaccaattggcaccaagctatccacagccttaatgccagtctgcattggttcccgcactgaaattcgaggaatgataccgggggctttcagaccaactcgcctacgcgtcttggaaccaattggaccctttccatcaatagcattaccaagggcatcaactacacgacccaacagctcctcaccaactggaacgtccacaatggctcctgtcctcttcactatatctccttccttaattagtttatcatttccaaacacgacaacaccaacattgtcaggttccaagttcaaggacataccctttaagcctgaagaaaactctaccatttcttctgcttgaacattcctcagcccatgtacgcgggcaataccatcaccaatacttaagacacgcccagtttcttcaagatcaacagaggtatcagctccaagaatacgctcttcaagaatagaggacatctcagcagtcccagtcttttgaagatgagtgttagaggcatggaagttccttgcagcaatgaaagatgaacccaaagcatttctggagaccagtccggcccgccgaggaagggcgcggaccacggccgcagcaacgcgcacggacagcatctttgcagttactccgcaggcggtacttctgcagccgcagcctccggactgactgggacaaaatg

SEQ ID NO: 17363 - RNA, 5238 nt, Homo sapiens
  source 1..5238: mol_type = other RNA
tcaggccaggcacagtggctcacgcctgtaatcccagcactttaggaggtcgaggcacgtggatcatctaaggtcaggagttcgaaaccagcctggccaacatggtgaaaccccgtctctactaaaaatacaaaaattagccaggcatggtggtgcacacctataatcacagctactcaggaggctgaggtaggagaatcacttgaacccaggaggtggaggttgcagtgagccgagatcgcgccattgcactccagcctgggcaacaaaaacaaaactccgtctcaaaaaaaaaaaaaaaaaaaaaaatctcatcagaccagaccagtagttaacatttggaatttgatttataatggacaaacatggttgtcttcatttgagaagtttattgagcatttacgtgccaggagtgggctacgagatccagtcaacaaacaaacaatacatactcccagtaataaattaattccaatccattagccaaagtatttttctccaaagtagtaatcaccactgacactaggtataaaatgctccaacaagccgggcgcagtggctcacccctgtaatcccagtactttgggaggccggtggaccacctaaggtcaggagtttgagaccagcctgaccaacatggagaaaccccatctctactaaaaatacaaaattagccaggcgtggtggtgcatgcctgtaatcccagctactcaggagcctgaggcaggagaattgcttgaccccaggaggcggtggttgtggtgagccgagatcgtgccattgcactccagcctgggcaacaagagcaaaactctcaaaaaaaaaaaacaaaaaaaaaaaaaaaaaaaaaaaacgaaatgtgcagaaccttctaactaaaagtaacttccttatttcagaaaaggaaaatcagatctagaagttatttctcaagtagctagaaagcaagagttgatcagaaatgaccaactgctatcaagtttagtgttcctctaagtactgaaaaggacttatgagtactttaagaactctccttttcctaccaaagatattggagcccacatatgtaaatatattttgacttactggagacagagagatggataagaatgaagtttcggtacagcaaatccccatcaacaaaataaaatggcaaggaagggggaaccctaggaaaaatattttagaacatgaccatgtatgacccttacagacaaaagcctttatatatcagtaaaaaaaaaaaaaaaaaaaagaggccgggcgcggtggctcaagcctgtaatcccagcactttgggaggccgaggtaagtggatcatgaggtcaggagatcgagaccatcctggcgaacatggtgaaaccccgtctctactaaaaatacaaaaaaaaaaaaattagctgggcgtgatggcaggcgcctgtagtaccagctaatcgggaggctgaggcaggagaacggcgcaaacccagggggcagagcttgcagtgagccgacatcgcaccactgcactccagcctgggagacagtgagactccgtctcaaaaaaaaaaaaaaaaggccaggtgtggtggctcacacctgtaatcccagcactgtgggaggccaaggcaggcagatcacaaggtcaggagttcgagaccagcctggccaatatggtgaaaccccgcctctactaaaaatacaaaaattagcagggcatggtggtgggtgcctgtagttccagcttctcgggaggctgaggcaggagaattgcttgaacctggaggcagaggttgcagtgagccaagatcaggtcactgcactccagcctggacgacggagactccatctcaaataaataaataactaagtaaaaaaaaaggtaacacattaagaatgagcaaaggctatgaaaaattaaaagtaaataaataaatcagtaggctgggcgtggtggctcacacctgtaatcccagcactttgggaagctgaggcgggcagaccacgaggtcaggagctcaagagcagcatggccaacatggtgaaaccttgtctctactaaaaatacaaaatgttagccgggtgtggtggcatgggcctgtggtcccagctaattgggaggctaaggcaggagaatcgcttgaacccaggaggtgaaaggtgcagtgagctgagattacgccactgctctccagcctaggtgacagagcaagactctgtctcaaaaaaataaataaatcagtaaaaaaaatttaatgcagtaagaatgagcaaaggctatgaaaagctagtaacagaggaaataaagtagctgtgaaaatattaaaagatggccgggcatggtagttcacacctgtaatcccagcactttgggagaccaaggcaggaggatcacttgagccaaggagttcatcatcagcctggacaacatggcaagaccctccctctacaaaaagtagaaaaattggctgggcgtggtggtatgtgcctgtaaccccagctactcaggaggctgaggtggaagaatcaattgaacccaggtggcagaagctgcagtgagctgagatcacaccactgtactccagcctgggtgagagagatggagaccctgtcacaaaacaaacaaaagagatattgacaagttttcataatcctatgcattctatcttctcagcttttgttccagcaattttttcatttccctgagaattttaactgtcctattattttcctgcctacagtacctctttatgcaggtacatcctctgggcagagaagccagctatgctcttcagtattgtcagcctgccacatatatccagtttaggaatttctcttaaacacaaagtactctagaaacttacaaagagcagccgggtgcggtggctcacacctgtaatcccagcactgtggtaggtaggccaaggcaggtggatcacctgaggtcaggagttcgtgaccggcctggccaacatggtgaaaccccgtctctactaaaaatactaaaaaactagccaggcgtggtggtgggcacctgtaatcccagctacgtgggaggctgaggcaagagaattgcttgaacccggagacggaggttgcagtgggccgacagggtgccactgcactccagcctcagtgacagagtgagaatcagtctcaaaaaaaaaaacaaaaaaaaaacttacaaagagctcagccttgaattatctagcccagttgactgtaccaatattcaagtaaaatagatcaagaagcatttgcttaccaatttctcaatttgatcttggttttaaagaataacacaaatgacagaaaacaactatgcattatggaacctttatttttcatgtgatttctgtacataaggagtatgagagtaacccttttacaaatggaactaatttactagaacaatgacaaaactgaactggtatttgatgtgaatccacaggagtttaagcttcaaatccagccaagaaatttgttacaatctctttcagctttgcatctgattgttctgagatctttccatcagccctgatagtgcccaacaaggcttggtgctggctgacgacatgagacaagaaagcattctcaaactttgtaatcttgctgggctccagtttatcaagatatccccttacacccgcatagataacagccacttgttcttcaatagccatgggagaatactgtccttgcttcagcaactcagttagacgcacgccacgactcaaaagttgttgagtggcagcatcgaggtcagaaccgaactgggcaaaagcagcaacctcacgatactgagccaattccagcttcatggtacctgctacctgcttcatagccctggtttgggcagcggatccgacacgagatacagacagaccaacgttaattgcagggcggatacctttgtagaacaattctgtttccaagaagatctgtccgtcagtgatggaaatgacatttgttggaatgtaagcagacacatcaccagcctgtgtttctatgactggcaaagcagtcaaggagccaccaccaaaagcatcgttcattttggctgctctctccagcaaccgggagtgtaggtagaacacatcaccaggataggcctcacgaccagggggtcggcggagcaacagagacatctgacggtaagcaacagcctgtttggataagtcgtcatagatgatcaaagcatgtttgccattgtctctaaaatactctcccatggaacagccagagtaaggagccaggtactgaagtggggcagcatccgaggccgtagccgacaccacaatggtgtacttcatggcatctgcatctgtaagtctcttcaccaactgggcaacagtggatctcttttgaccaatagcaacataaatacagtacagcttcttcttttcatcagatccatcattgaaacgtttctggttaatgattgtgtcaatagcaattgaggttttcccagtctgtcggtcaccaataatcagttcacgctgaccacgaccaattggcaccaagctatccacagccttaatgccagtctgcattggttcccgcactgaaattcgaggaatgataccgggggctttcagaccaactcgcctacgcgtcttggaaccaattggaccctttccatcaatagcattaccaagggcatcaactacacgacccaacagctcctcaccaactggaacgtccacaatggctcctgtcctcttcactatatctccttccttaattagtttatcatttccaaacacgacaacaccaacattgtcaggttccaagttcaaggacataccctttaagcctgaagaaaactctaccatttcttctgcttgaacattcctcagcccatgtacgcgggcaataccatcaccaatacttaagacacgcccagtttcttcaagatcaacagaggtatcagctccaagaatacgctcttcaagaatagaggacatctcagcagtcccagtcttttgaagatgagtgttagaggcatggaagttccttgcagcaatgaaagatgaacccaaagcatttctggagaccagtccggcccgccgaggaagggcgcggaccacggccgcagcaacgcgcacggacagcatctttgcagttactccgcaggcggtacttctgcagccgcagcctccggactggttctaggcggctctatctctcgtagtgttgattataccgcggaaggcgggaagagctgggaagtggcaacgaagcgaggcttgcaat

SEQ ID NO: 17364 - RNA, 5500 nt, Homo sapiens
  source 1..5500: mol_type = other RNA
tcaggccaggcacagtggctcacgcctgtaatcccagcactttaggaggtcgaggcacgtggatcatctaaggtcaggagttcgaaaccagcctggccaacatggtgaaaccccgtctctactaaaaatacaaaaattagccaggcatggtggtgcacacctataatcacagctactcaggaggctgaggtaggagaatcacttgaacccaggaggtggaggttgcagtgagccgagatcgcgccattgcactccagcctgggcaacaaaaacaaaactccgtctcaaaaaaaaaaaaaaaaaaaaaaatctcatcagaccagaccagtagttaacatttggaatttgatttataatggacaaacatggttgtcttcatttgagaagtttattgagcatttacgtgccaggagtgggctacgagatccagtcaacaaacaaacaatacatactcccagtaataaattaattccaatccattagccaaagtatttttctccaaagtagtaatcaccactgacactaggtataaaatgctccaacaagccgggcgcagtggctcacccctgtaatcccagtactttgggaggccggtggaccacctaaggtcaggagtttgagaccagcctgaccaacatggagaaaccccatctctactaaaaatacaaaattagccaggcgtggtggtgcatgcctgtaatcccagctactcaggagcctgaggcaggagaattgcttgaccccaggaggcggtggttgtggtgagccgagatcgtgccattgcactccagcctgggcaacaagagcaaaactctcaaaaaaaaaaaacaaaaaaaaaaaaaaaaaaaaaaaacgaaatgtgcagaaccttctaactaaaagtaacttccttatttcagaaaaggaaaatcagatctagaagttatttctcaagtagctagaaagcaagagttgatcagaaatgaccaactgctatcaagtttagtgttcctctaagtactgaaaaggacttatgagtactttaagaactctccttttcctaccaaagatattggagcccacatatgtaaatatattttgacttactggagacagagagatggataagaatgaagtttcggtacagcaaatccccatcaacaaaataaaatggcaaggaagggggaaccctaggaaaaatattttagaacatgaccatgtatgacccttacagacaaaagcctttatatatcagtaaaaaaaaaaaaaaaaaaaagaggccgggcgcggtggctcaagcctgtaatcccagcactttgggaggccgaggtaagtggatcatgaggtcaggagatcgagaccatcctggcgaacatggtgaaaccccgtctctactaaaaatacaaaaaaaaaaaaattagctgggcgtgatggcaggcgcctgtagtaccagctaatcgggaggctgaggcaggagaacggcgcaaacccagggggcagagcttgcagtgagccgacatcgcaccactgcactccagcctgggagacagtgagactccgtctcaaaaaaaaaaaaaaaaggccaggtgtggtggctcacacctgtaatcccagcactgtgggaggccaaggcaggcagatcacaaggtcaggagttcgagaccagcctggccaatatggtgaaaccccgcctctactaaaaatacaaaaattagcagggcatggtggtgggtgcctgtagttccagcttctcgggaggctgaggcaggagaattgcttgaacctggaggcagaggttgcagtgagccaagatcaggtcactgcactccagcctggacgacggagactccatctcaaataaataaataactaagtaaaaaaaaaggtaacacattaagaatgagcaaaggctatgaaaaattaaaagtaaataaataaatcagtaggctgggcgtggtggctcacacctgtaatcccagcactttgggaagctgaggcgggcagaccacgaggtcaggagctcaagagcagcatggccaacatggtgaaaccttgtctctactaaaaatacaaaatgttagccgggtgtggtggcatgggcctgtggtcccagctaattgggaggctaaggcaggagaatcgcttgaacccaggaggtgaaaggtgcagtgagctgagattacgccactgctctccagcctaggtgacagagcaagactctgtctcaaaaaaataaataaatcagtaaaaaaaatttaatgcagtaagaatgagcaaaggctatgaaaagctagtaacagaggaaataaagtagctgtgaaaatattaaaagatggccgggcatggtagttcacacctgtaatcccagcactttgggagaccaaggcaggaggatcacttgagccaaggagttcatcatcagcctggacaacatggcaagaccctccctctacaaaaagtagaaaaattggctgggcgtggtggtatgtgcctgtaaccccagctactcaggaggctgaggtggaagaatcaattgaacccaggtggcagaagctgcagtgagctgagatcacaccactgtactccagcctgggtgagagagatggagaccctgtcacaaaacaaacaaaagagatattgacaagttttcataatcctatgcattctatcttctcagcttttgttccagcaattttttcatttccctgagaattttaactgtcctattattttcctgcctacagtacctctttatgcaggtacatcctctgggcagagaagccagctatgctcttcagtattgtcagcctgccacatatatccagtttaggaatttctcttaaacacaaagtactctagaaacttacaaagagcagccgggtgcggtggctcacacctgtaatcccagcactgtggtaggtaggccaaggcaggtggatcacctgaggtcaggagttcgtgaccggcctggccaacatggtgaaaccccgtctctactaaaaatactaaaaaactagccaggcgtggtggtgggcacctgtaatcccagctacgtgggaggctgaggcaagagaattgcttgaacccggagacggaggttgcagtgggccgacagggtgccactgcactccagcctcagtgacagagtgagaatcagtctcaaaaaaaaaaacaaaaaaaaaacttacaaagagctcagccttgaattatctagcccagttgactgtaccaatattcaagtaaaatagatcaagaagcatttgcttaccaatttctcaatttgatcttggttttaaagaataacacaaatgacagaaaacaactatgcattatggaacctttatttttcatgtgatttctgtacataaggagtatgagagtaacccttttacaaatggaactaatttactagaacaatgacaaaactgaactggtatttgatgtgaatccacaggagtttaagcttcaaatccagccaagaaatttgttacaatctctttcagctttgcatctgattgttctgagatctttccatcagccctgatagtgcccaacaaggcttggtgctggctgacgacatgagacaagaaagcattctcaaactttgtaatcttgctgggctccagtttatcaagatatccccttacacccgcatagataacagccacttgttcttcaatagccatgggagaatactgtccttgcttcagcaactcagttagacgcacgccacgactcaaaagttgttgagtggcagcatcgaggtcagaaccgaactgggcaaaagcagcaacctcacgatactgagccaattccagcttcatggtacctgctacctgcttcatagccctggtttgggcagcggatccgacacgagatacagacagaccaacgttaattgcagggcggatacctttgtagaacaattctgtttccaagaagatctgtccgtcagtgatggaaatgacatttgttggaatgtaagcagacacatcaccagcctgtgtttctatgactggcaaagcagtcaaggagccaccaccaaaagcatcgttcattttggctgctctctccagcaaccgggagtgtaggtagaacacatcaccaggataggcctcacgaccagggggtcggcggagcaacagagacatctgacggtaagcaacagcctgtttggataagtcgtcatagatgatcaaagcatgtttgccattgtctctaaaatactctcccatggaacagccagagtaaggagccaggtactgaagtggggcagcatccgaggccgtagccgacaccacaatggtgtacttcatggcatctgcatctgtaagtctcttcaccaactgggcaacagtggatctcttttgaccaatagcaacataaatacagtacagcttcttcttttcatcagatccatcattgaaacgtttctggttaatgattgtgtcaatagcaattgaggttttcccagtctgtcggtcaccaataatcagttcacgctgaccacgaccaattggcaccaagctatccacagccttaatgccagtctgcattggttcccgcactgaaattcgaggaatgataccgggggctttcagaccaactcgcctacgcgtcttggaaccaattggaccctttccatcaatagcattaccaagggcatcaactacacgacccaacagctcctcaccaactggaacgtccacaatggctcctgtcctcttcactatatctccttccttaattagtttatcatttccaaacacgacaacaccaacattgtcaggttccaagttcaaggacataccctttaagcctgaagaaaactctaccatttcttctgcttgaacattcctcagcccatgtacgcgggcaataccatcaccaatacttaagacacgcccagtttcttcaagatcaacagaggtatcagctccaagaatacgctcttcaagaatagaggacatctcagcagtcccagtcttttgaagatgagtgttagaggcatggaagttccttgcagcaatgaaagatgaacccaaagcatttctggagaccgattcagaacaggcctcggagagctagcgcccaagccctgaccttcacccaagatcccccttctagggccgctgtcagccgaagacaggaatcttgaggccctgtctctggacaccatcgagttaactgtctgccctgtaccattctgcctctgcgcaggtgacgagcaaaagggcacctgtgtcgcctgctctgtccagccggagaagccacgggtgcaagatggcggcattcgccacagcccctcgccctcctgcagagagcgcccgagccggcgcaccaccaccctgcagccccacccggccgcctgcatcatgccggccttcggtgctcaccagtccggcccgccgaggaagggcgcggaccacggccgcagcaacgcgcacggacagcatctttgcagttactccgcaggcggtacttctgcagccgcagcctccggactgactgggacaaaatg

SEQ ID NO: 17365 - RNA, 5098 nt, Homo sapiens
  source 1..5098: mol_type = other RNA
tcaggccaggcacagtggctcacgcctgtaatcccagcactttaggaggtcgaggcacgtggatcatctaaggtcaggagttcgaaaccagcctggccaacatggtgaaaccccgtctctactaaaaatacaaaaattagccaggcatggtggtgcacacctataatcacagctactcaggaggctgaggtaggagaatcacttgaacccaggaggtggaggttgcagtgagccgagatcgcgccattgcactccagcctgggcaacaaaaacaaaactccgtctcaaaaaaaaaaaaaaaaaaaaaaatctcatcagaccagaccagtagttaacatttggaatttgatttataatggacaaacatggttgtcttcatttgagaagtttattgagcatttacgtgccaggagtgggctacgagatccagtcaacaaacaaacaatacatactcccagtaataaattaattccaatccattagccaaagtatttttctccaaagtagtaatcaccactgacactaggtataaaatgctccaacaagccgggcgcagtggctcacccctgtaatcccagtactttgggaggccggtggaccacctaaggtcaggagtttgagaccagcctgaccaacatggagaaaccccatctctactaaaaatacaaaattagccaggcgtggtggtgcatgcctgtaatcccagctactcaggagcctgaggcaggagaattgcttgaccccaggaggcggtggttgtggtgagccgagatcgtgccattgcactccagcctgggcaacaagagcaaaactctcaaaaaaaaaaaacaaaaaaaaaaaaaaaaaaaaaaaacgaaatgtgcagaaccttctaactaaaagtaacttccttatttcagaaaaggaaaatcagatctagaagttatttctcaagtagctagaaagcaagagttgatcagaaatgaccaactgctatcaagtttagtgttcctctaagtactgaaaaggacttatgagtactttaagaactctccttttcctaccaaagatattggagcccacatatgtaaatatattttgacttactggagacagagagatggataagaatgaagtttcggtacagcaaatccccatcaacaaaataaaatggcaaggaagggggaaccctaggaaaaatattttagaacatgaccatgtatgacccttacagacaaaagcctttatatatcagtaaaaaaaaaaaaaaaaaaaagaggccgggcgcggtggctcaagcctgtaatcccagcactttgggaggccgaggtaagtggatcatgaggtcaggagatcgagaccatcctggcgaacatggtgaaaccccgtctctactaaaaatacaaaaaaaaaaaaattagctgggcgtgatggcaggcgcctgtagtaccagctaatcgggaggctgaggcaggagaacggcgcaaacccagggggcagagcttgcagtgagccgacatcgcaccactgcactccagcctgggagacagtgagactccgtctcaaaaaaaaaaaaaaaaggccaggtgtggtggctcacacctgtaatcccagcactgtgggaggccaaggcaggcagatcacaaggtcaggagttcgagaccagcctggccaatatggtgaaaccccgcctctactaaaaatacaaaaattagcagggcatggtggtgggtgcctgtagttccagcttctcgggaggctgaggcaggagaattgcttgaacctggaggcagaggttgcagtgagccaagatcaggtcactgcactccagcctggacgacggagactccatctcaaataaataaataactaagtaaaaaaaaaggtaacacattaagaatgagcaaaggctatgaaaaattaaaagtaaataaataaatcagtaggctgggcgtggtggctcacacctgtaatcccagcactttgggaagctgaggcgggcagaccacgaggtcaggagctcaagagcagcatggccaacatggtgaaaccttgtctctactaaaaatacaaaatgttagccgggtgtggtggcatgggcctgtggtcccagctaattgggaggctaaggcaggagaatcgcttgaacccaggaggtgaaaggtgcagtgagctgagattacgccactgctctccagcctaggtgacagagcaagactctgtctcaaaaaaataaataaatcagtaaaaaaaatttaatgcagtaagaatgagcaaaggctatgaaaagctagtaacagaggaaataaagtagctgtgaaaatattaaaagatggccgggcatggtagttcacacctgtaatcccagcactttgggagaccaaggcaggaggatcacttgagccaaggagttcatcatcagcctggacaacatggcaagaccctccctctacaaaaagtagaaaaattggctgggcgtggtggtatgtgcctgtaaccccagctactcaggaggctgaggtggaagaatcaattgaacccaggtggcagaagctgcagtgagctgagatcacaccactgtactccagcctgggtgagagagatggagaccctgtcacaaaacaaacaaaagagatattgacaagttttcataatcctatgcattctatcttctcagcttttgttccagcaattttttcatttccctgagaattttaactgtcctattattttcctgcctacagtacctctttatgcaggtacatcctctgggcagagaagccagctatgctcttcagtattgtcagcctgccacatatatccagtttaggaatttctcttaaacacaaagtactctagaaacttacaaagagcagccgggtgcggtggctcacacctgtaatcccagcactgtggtaggtaggccaaggcaggtggatcacctgaggtcaggagttcgtgaccggcctggccaacatggtgaaaccccgtctctactaaaaatactaaaaaactagccaggcgtggtggtgggcacctgtaatcccagctacgtgggaggctgaggcaagagaattgcttgaacccggagacggaggttgcagtgggccgacagggtgccactgcactccagcctcagtgacagagtgagaatcagtctcaaaaaaaaaaacaaaaaaaaaacttacaaagagctcagccttgaattatctagcccagttgactgtaccaatattcaagtaaaatagatcaagaagcatttgcttaccaatttctcaatttgatcttggttttaaagaataacacaaatgacagaaaacaactatgcattatggaacctttatttttcatgtgatttctgtacataaggagtatgagagtaacccttttacaaatggaactaatttactagaacaatgacaaaactgaactggtatttgatgtgaatccacaggagtttaagcttcaaatccagccaagaaatttgttacaatctctttcagctttgcatctgattgttctgagatctttccatcagccctgatagtgcccaacaaggcttggtgctggctgacgacatgagacaagaaagcattctcaaactttgtaatcttgctgggctccagtttatcaagatatccccttacacccgcatagataacagccacttgttcttcaatagccatgggagaatactgtccttgcttcagcaactcagttagacgcacgccacgactcaaaagttgttgagtggcagcatcgaggtcagaaccgaactgggcaaaagcagcaacctcacgatactgagccaattccagcttcatggtacctgctacctgcttcatagccctggtttgggcagcggatccgacacgagatacagacagaccaacgttaattgcagggcggatacctttgtagaacaattctgtttccaagaagatctgtccgtcagtgatggaaatgacatttgttggaatgtaagcagacacatcaccagcctgtgtttctatgactggcaaagcagtcaaggagccaccaccaaaagcatcgttcattttggctgctctctccagcaaccgggagtgtaggtagaacacatcaccaggataggcctcacgaccagggggtcggcggagcaacagagacatctgacggtaagcaacagcctgtttggataagtcgtcatagatgatcaaagcatgtttgccattgtctctaaaatactctcccatggaacagccagagtaaggagccaggtactgaagtggggcagcatccgaggccgtagccgacaccacaatggtgtacttcatggcatctgcatctgtaagtctcttcaccaactgggcaacagtggatctcttttgaccaatagcaacataaatacagtacagcttcttcttttcatcagatccatcattgaaacgtttctggttaatgattgtgtcaatagcaattgaggttttcccagtctgtcggtcaccaataatcagttcacgctgaccacgaccaattggcaccaagctatccacagccttaatgccagtctgcattggttcccgcactgaaattcgaggaatgataccgggggctttcagaccaactcgcctacgcgtcttggaaccaattggaccgtccacaatggctcctgtcctcttcactatatctccttccttaattagtttatcatttccaaacacgacaacaccaacattgtcaggttccaagttcaaggacataccctttaagcctgaagaaaactctaccatttcttctgcttgaacattcctcagcccatgtacgcgggcaataccatcaccaatacttaagacacgcccagtttcttcaagatcaacagaggtatcagctccaagaatacgctcttcaagaatagaggacatctcagcagtcccagtcttttgaagatgagtgttagaggcatggaagttccttgcagcaatgaaagatgaacccaaagcatttctggagaccagtccggcccgccgaggaagggcgcggaccacggccgcagcaacgcgcacggacagcatctttgcagttactccgcaggcggtacttctgcagccgcagcctccggactgactgggacaaaatg

SEQ ID NO: 17366 - RNA, 2118 nt, Homo sapiens
  source 1..2118: mol_type = other RNA
tcaggccaggcacagtggctcacgcctgtaatcccagcactttgggaagctgaggccagcggatcatgaggtcaggagtttgagaccagcctgaccaacatggtgaaaccctgtctctactaaaaatacaaaaattaacctggcgtggtggaacatgcctataatcccagctactcaggaggccgaggcaggagaatcacttgaacccaggaggcggaggttgcagtgagctgagatcgcaccactgcactccagcctgggctattgagtgagaatccatcttcagaaaacaaacaaacaaacaaaaaagaaagaaatccctatcctagccgagttaatagcttaactctggagcctgataatatatgttttttaactgagtttttcttgtaaggcccaatgaatttcctctgagttctcagcagtcacaggagtaatattgcatttataggataaactaggccttttggtaattatcccatcttcccaaataatttctcccagatgcaaaatgcaaagacactcgtggccattatatagtatcaaagtcttattatgaagtacccgttgaagggcacagattgaatttccagtgtttagtgtacatggctctaatagttttaagtctggaggacaaagccaacttttgggccatttcttacctcggtccaaaccagtagttatattattataacagttaactaaataaccatagataacaggcatatccacctttgtttatctatccatagtaggactggagaaaacttctattctcaagttaatcgattgacattagagctgtcttctgaggtctctatccataaatgccagacacttaattagatgcatttcttttctatactatacttccaatcaaaccagttaacaaatttttttgtgtgaaatttagggctttggtttctggatgcatagtagttacttttactttgatattaaaacatagtaatgaacatggtcttgtgtttatttggccaataatcagactgttggattcataaatgcaggcccagcatttctgtactgggaatacaattcagaggagagaggaaatgtgactgtaggaaccattattgggagtacagaaagaaaaagtggtgtaacaaataacatgtttattttctaataaaatgtgattcttatagtaattgaacaaaacactattgcaactaggacagcaaggtagtcagaataatacattccttagaatacctcctttcagttgagttcattaccaatattagtcactctaggaaattaaacttcaaatcctttgtggaaactgcagtctagtcctcctgaggagctggcttcacatggaaagcatgaaaccatctggtttttctttcactctgatacccatatgagtgatcgtggcacttgaaagggtcccatccagcctggtgacaatgcatgtttcctccagaacactcatatttaaacaaaattgcccagtttaataggggtgatatttcttccagtagttccttctaggtccttttcactttatgtctcaggatgtcacaagtcgggaatcttgtacagagatggcatagacaaggtatgaggccacatttcccaaggggcttttattggctctacaagtcaactttgattctttaaagaagcatgccattccagtcaaagccttggtgaaataactagtttctccagttgtgtcctttgccatccggggctgaggtttcattttctttggttattccccaggccagtaccatttgctttttactttccagaagttctgtaaagattgttgatggtaccctttcttagcttttttttttttttttggtcttgatatagtcctattcttctaaaaaatcttttcatttgtctccgtcagactttgatggagaggaggggagatattgtttacatttgttaaaaatggcttttaagttaaattctaactaagggtctattaggaaataaaattgccttctgactccttttgatttattttgcagaattgcatatatccaaagctctgggtaattattaaacattagaagtatagaacaaacaggccagccaggcccggcgaggccgcggcgggtccggcgccccggacctccg

SEQ ID NO: 17367 - RNA, 2249 nt, Homo sapiens
  source 1..2249: mol_type = other RNA
tcaggccaggcacagtggctcacgcctgtaatcccagcactttgggaagctgaggccagcggatcatgaggtcaggagtttgagaccagcctgaccaacatggtgaaaccctgtctctactaaaaatacaaaaattaacctggcgtggtggaacatgcctataatcccagctactcaggaggccgaggcaggagaatcacttgaacccaggaggcggaggttgcagtgagctgagatcgcaccactgcactccagcctgggctattgagtgagaatccatcttcagaaaacaaacaaacaaacaaaaaagaaagaaatccctatcctagccgagttaatagcttaactctggagcctgataatatatgttttttaactgagtttttcttgtaaggcccaatgaatttcctctgagttctcagcagtcacaggagtaatattgcatttataggataaactaggccttttggtaattatcccatcttcccaaataatttctcccagatgcaaaatgcaaagacactcgtggccattatatagtatcaaagtcttattatgaagtacccgttgaagggcacagattgaatttccagtgtttagtgtacatggctctaatagttttaagtctggaggacaaagccaacttttgggccatttcttacctcggtccaaaccagtagttatattattataacagttaactaaataaccatagataacaggcatatccacctttgtttatctatccatagtaggactggagaaaacttctattctcaagttaatcgattgacattagagctgtcttctgaggtctctatccataaatgccagacacttaattagatgcatttcttttctatactatacttccaatcaaaccagttaacaaatttttttgtgtgaaatttagggctttggtttctggatgcatagtagttacttttactttgatattaaaacatagtaatgaacatggtcttgtgtttatttggccaataatcagactgttggattcataaatgcaggcccagcatttctgtactgggaatacaattcagaggagagaggaaatgtgactgtaggaaccattattgggagtacagaaagaaaaagtggtgtaacaaataacatgtttattttctaataaaatgtgattcttatagtaattgaacaaaacactattgcaactaggacagcaaggtagtcagaataatacattccttagaatacctcctttcagttgagttcattaccaatattagtcactctaggaaattaaacttcaaatcctttgtggaaactgcagtctagtcctcctgaggagctggcttcacatggaaagcatgaaaccatctggtttttctttcactctgatacccatatgagtgatcgtggcacttgaaagggtcccatccagcctggtgacaatgcatgtttcctccagaacactcatatttaaacaaaattgcccagtttaataggggtgatatttcttccagtagttccttctaggtccttttcactttatgtctcaggatgtctacttgtgccaacttaattccagacaaaacataagcttccaagagctcatgatcagacaccacagcataagaaaccttcagttggccaatttatcccaagtacatggtccatcagtaaacactatgaaatcacaagtcgggaatcttgtacagagatggcatagacaaggtatgaggccacatttcccaaggggcttttattggctctacaagtcaactttgattctttaaagaagcatgccattccagtcaaagccttggtgaaataactagtttctccagttgtgtcctttgccatccggggctgaggtttcattttctttggttattccccaggccagtaccatttgctttttactttccagaagttctgtaaagattgttgatggtaccctttcttagcttttttttttttttttggtcttgatatagtcctattcttctaaaaaatcttttcatttgtctccgtcagactttgatggagaggaggggagatattgtttacatttgttaaaaatggcttttaagttaaattctaactaagggtctattaggaaataaaattgccttctgactccttttgatttattttgcagaattgcatatatccaaagctctgggtaattattaaacattagaagtatagaacaaacaggccagccaggcccggcgaggccgcggcgggtccggcgccccggacctccg

SEQ ID NO: 17368 - RNA, 6165 nt, Homo sapiens
  source 1..6165: mol_type = other RNA
tcaggccaggcacagtggctcacgcctgtaatcccagcactttgggaggcagaggtgggtggattgcttgagcccaggagtttgagaccagcatgagcaacatgggaaaaaaaaataaaagttttgtctctacaaaaaaatataaaaaattagctggcagggtggcacacacctgtagccccagctactcgggaggctcagatgggacctgagcctgggaggtcaaggctgcagtaagctgtgatcctgccactgcactccaccctgggcaaccctgtctcaaaaaataaaaaagacagtaaaaatatccctatactggggcaggaactttacaaggtatcctgtggcaaagggagcagagatggggggaaaggggtgctaaaagtttgattggaaagggacttttccatggttacaacaccaactgacatggaagctgcacctctgagagggccctggtcctagaggtcaaccacctgatggagagccttggtaaaccaagccctctttcaccaatctcaggaatcaggtagcacagccaagcactctaacttcacacataaggaaattgatgcagaggttcattgacttgctcaagatcaatcctgccaagaaaaggcacaccatgcctggaacccagatctgatgactccaagacccttcctatgactctggcccccctgcccagccacttctagtgccagttttgggacagtgaagggacatcttcagtgccatgaacagctgctgccgtaggaaggcaagaggatggcagaaccaagatgaccaaaccttcctgaggacaaagctgaacaggcatcagaacaccaacaggagacttctgccccgcccccaccatcctgtgacaccaccacacaatatcagagccttcattttcacctgctcatggcaatccagagcaggtaagattattccatactctactgaaaaagacatcttccaggttggtttcttctcatttcaagaaatgaccagctccatgaacgggcccctatagtcaggacactgctctactattaaaacattttatcctttcattcataatctgacctcttcaataatcagaagcaatgattactcacatgctttagcaatatcactcctttgcctttaagtaattgattcttgctttttgcttcaacacaagtgggtgggccagtgagggagctcctcccagaacaggctgccttttctcctgagagcagcaggcacatgcacttgttccttcgggttgaatctgattgctagcaccagatctcatacatggagaggggtatgtgaagctgagaggggcctgcagtgtgcaggggctagagacatgaacacaacaatggtaagcgtttatatctgctgaggccgaggatcctatagaaaattcagaaacggagtggggaggagtctgatttatgggaactggcagcaaggctaactgcatgagaagcctttcacccttttactgagtccttggatctgtggttaacccttataaaatataattcagattcaaaccacatcactcctcaactcaaaattgtccaaaagctccctgcctccctctgagccagctcaagcccccgtaatgacccatgatgctcatatggccgggcctgtggcctccctggcccctctccttcccttccagctggctccctgcactccatcccaggggcttccttcctgaggacaccagtcaagacccaatctcctctgcctgcaactctccctagagagctacctgctacctccctggcttccttcacgtctttgctcacatttcaccttctcagttgaggccctccctgaccagactatctaaaatcacgactgatctcccaatccagcactccctctgctcttctctgattcactttgtccactacacacatcaccatccagaatactgcgtatcccatttgtttgtcatctgtaaagatccaagatggcaggattttcatctgttctggtccctgctgggtctctggcaaacacaccagcgcctggtgtatgggagtgctcagcacatttctgttaaacagatggaccgctgctgcctatgcaggcctgtgggatggggatggcaacagggtactggtagagatccacacgccaagcgcttgagcccagcatcctgctctcctccacctgccgctgagaccactctaaccccctagcagatatccaaaagccagccaggaaggctgaagccccagccagaactccccagggggcatttgggaaggctaggagttcttgatgctgctgcttttaaagtcaacagaataggcatggccacaggccaaacttgaagacaaatctaggatcccactggcccctttccagcagccatagcccatgatgccacagatattctgtccaaccacaaagggcagtggtctctctcttcagagttgtggaaggagacctgaataggggagccgcaggctatggtgcagaggccactcctaggggccggagtctccagaagggctccaaaggacatggtgctgcacttccccagcgtcacatcctagcaggcaggctggggactccccgagctttcaaatccttgggattctgtcactagcttccaaaacagaaagggctgggccctttatcaaagttactccacaatgcctataattaagggttctctagcaggggactgagaacccacccccactgtcactgtcaggtcccaggctaatctctaatatggtttttcatatgccgagccaggttcgaagaccacctgaaggtctttccacacttgctgcatttgaagggcctctctcgagtatgaaatctcttgtggctaatgagttgtgaactcttgttaaaagttttcccacatatgctgcatttgtggcactttttcccaatgcttatgtcctggagtccagtgagcctggagctctggctgcaagcttctttgcagtcttcgaggggcatctcttcacttggttttagcttctgtaatctcaactttgtgtcctgagaggaagaccgtgcaggcgggctacgttcagcctgtgctgctctggtgtgtttcctctggtgactggaaagggtatgtctcccaatgaactctttcccacaccactgacatttgaaaggtctctctgtagagtggatcctctgatggttaacaaggcgatagtttctatcataagatttcccacatagattacatttatagcgcttctctccactgtgtattcccttatgatctaaaagggttcttttacgtgtaaaggttttcccacattcttgacaccaaaaacgtttctcaccagtgaggatttttggctccacatttggagtcttttcactttcatggcaatcatactgtttttgaagagagtgaatcctctgatgtcggtagagattggaactccatctgaaggctttcccacactccctgcacttatatggcttctctccagtgtgaactctctgatggatgaggaggaatgagtgattgcggaaggccttgccacactggctgcatttgtagggctcctctttggagtgactgctctgaggaacctggaacactgtgtcctgactaaaagatggcccgccctcaggttttcttttcatggcatgcttcttcttatgaacaataaaggctgacctataggcaaagtccttcccacaatcgctacactggtaaggtttctcacctgtgtgaattctctggtggtcaacgagagttttctttctagtaaaagttttcccacactgctgacacagaaatgttttctccacagcgggagcaccctggggctgactgcagtcaggagattgcctgaagccttcacgacattcatcttgtttgtagaatttttcctcctcatgcaacctcatatgacgagtaaagtttgatctccatctaaaggttttcctacatttggtacatttatagggcttctcctgggtgtgaatcctttgatgttcaagaacatatgacttacagtggaaggatttcctgcactggctgcagtcaaagagtttctccccactttggtctcccaaatgatgatcaaaccctgagctgtaggtgagagctgccctatactgattcaattcaagaaatttcttcttagcatgggtttctcggtgcagacggtaggctgacaggcgtcggaaagctttctcacataaatcgcatttataaggcttcactccagtgtgaattttctcatgccgcgcacagttggaactccaccggaaggctttcccacacaccctacatttaaatgctttctcttgagtgtgaagtctctgatgatacgcaagatgggagctatgactgaaagtccttccacagtcactgcacttaaatgacactcccactgtgtgaagactctgcccacgttggtgatgagagctaaggctgaagtcttttccacacacgtcctttttgttccctttcagtccactatgaattctctgatgtaggctgaagcccccaatcatgtgtctgagccccttcccatatttcttgtagtcatagtggtgtgaactcattctgaagtgtttgccacagccatgtttaagggattcctttcttccagaaactctcaaatatgtaacatgttttaagtcaagactattacttcctgatacttcagagtcttttcctgtcctgtgactgaaattggtctcttctttcttaactcttacttgtatgggattttcacattgatccttctgcctgctcttctgttgaaaagattctctgagcccaattccctcagaaacacttgtcgcaggacatcctgatgacacagctaaggtttctgcttcttccaaaggttcctgatttaagatgaatttgtttgttttactctggaggtcatctcctgtaggagcagcaactggattccccttaggctgagctgcctgcatgttcaggccccatggctcccttgcttccaaccaggagatcagagcaggtttggtgaatggtcccaccagggaagccatgttcctataattctccagcatcacatccctgtacaggttcctctgagcagagtccagccacccccactcgtcctgggagaaggtcacctccacatccttgaaagtcatggtctcctggagctgggctgtcagggacctggttggtgttacctggtctcccgggcacccctctctcgggaaaagggcaggcatctgggcagcaggagtatcggattgcccagccaggaagtcacgtgcttctatttcatagggaggctccaggtggtcccccagagcagagctgctcctgagaggtgaagcaagggaccatatctgtgcagatcgcagggctcctgtacccatccaatgcacatctgggctctgggcagggcccgggtccctccaggatgtcccatcaaggtccctctgcagctcctccagcaaggccacagcctcctcgccactctcagggttatgaagctgcacccaaacccggagctccccaggcaggatgctcaggaactgttccagcaccagcagctctaggatctgtgccttggagagaacgtcaggcctcagccaccagcgacagagttcccggagccggctcagagtttctaggggccctgaagactcatggtagcgaagctgtctgaagagctggcggaacagctcctggccagggcggttgagagtctgtggcctggcagcctgcactggagtatagctttcatcctcttcttccttctttactgtctgaagccgccctcgctccctcgaagactgggcctgagctggataggcagcatgccacctgcctggaggcatcactcctgttcagggactaaccagaagagtgcgaaccaagtccaccttagacgtgggtcctcagaagtatcttctcagcagtcaacaatgccaacatttgctgggacatcagaagtcatcagcaagtgactgaaattaccagcatttctgtagtcccagctactcgggaggctgaggcagaagaatcacttgaacccaggaggcggaggctgcagtgagccgagatcatgccattgcactccagccttgcgaaagagcgagactccaccgactcccgccgccgagcgacaatcggtccacccgccgccaccgcagccgcccgtcccgcgcctacctcccggcggctcc

SEQ ID NO: 17369 - RNA, 6008 nt, Homo sapiens
  source 1..6008: mol_type = other RNA
tcaggccaggcacagtggctcacgcctgtaatcccagcactttgggaggcagaggtgggtggattgcttgagcccaggagtttgagaccagcatgagcaacatgggaaaaaaaaataaaagttttgtctctacaaaaaaatataaaaaattagctggcagggtggcacacacctgtagccccagctactcgggaggctcagatgggacctgagcctgggaggtcaaggctgcagtaagctgtgatcctgccactgcactccaccctgggcaaccctgtctcaaaaaataaaaaagacagtaaaaatatccctatactggggcaggaactttacaaggtatcctgtggcaaagggagcagagatggggggaaaggggtgctaaaagtttgattggaaagggacttttccatggttacaacaccaactgacatggaagctgcacctctgagagggccctggtcctagaggtcaaccacctgatggagagccttggtaaaccaagccctctttcaccaatctcaggaatcaggtagcacagccaagcactctaacttcacacataaggaaattgatgcagaggttcattgacttgctcaagatcaatcctgccaagaaaaggcacaccatgcctggaacccagatctgatgactccaagacccttcctatgactctggcccccctgcccagccacttctagtgccagttttgggacagtgaagggacatcttcagtgccatgaacagctgctgccgtaggaaggcaagaggatggcagaaccaagatgaccaaaccttcctgaggacaaagctgaacaggcatcagaacaccaacaggagacttctgccccgcccccaccatcctgtgacaccaccacacaatatcagagccttcattttcacctgctcatggcaatccagagcaggtaagattattccatactctactgaaaaagacatcttccaggttggtttcttctcatttcaagaaatgaccagctccatgaacgggcccctatagtcaggacactgctctactattaaaacattttatcctttcattcataatctgacctcttcaataatcagaagcaatgattactcacatgctttagcaatatcactcctttgcctttaagtaattgattcttgctttttgcttcaacacaagtgggtgggccagtgagggagctcctcccagaacaggctgccttttctcctgagagcagcaggcacatgcacttgttccttcgggttgaatctgattgctagcaccagatctcatacatggagaggggtatgtgaagctgagaggggcctgcagtgtgcaggggctagagacatgaacacaacaatggtaagcgtttatatctgctgaggccgaggatcctatagaaaattcagaaacggagtggggaggagtctgatttatgggaactggcagcaaggctaactgcatgagaagcctttcacccttttactgagtccttggatctgtggttaacccttataaaatataattcagattcaaaccacatcactcctcaactcaaaattgtccaaaagctccctgcctccctctgagccagctcaagcccccgtaatgacccatgatgctcatatggccgggcctgtggcctccctggcccctctccttcccttccagctggctccctgcactccatcccaggggcttccttcctgaggacaccagtcaagacccaatctcctctgcctgcaactctccctagagagctacctgctacctccctggcttccttcacgtctttgctcacatttcaccttctcagttgaggccctccctgaccagactatctaaaatcacgactgatctcccaatccagcactccctctgctcttctctgattcactttgtccactacacacatcaccatccagaatactgcgtatcccatttgtttgtcatctgtaaagatccaagatggcaggattttcatctgttctggtccctgctgggtctctggcaaacacaccagcgcctggtgtatgggagtgctcagcacatttctgttaaacagatggaccgctgctgcctatgcaggcctgtgggatggggatggcaacagggtactggtagagatccacacgccaagcgcttgagcccagcatcctgctctcctccacctgccgctgagaccactctaaccccctagcagatatccaaaagccagccaggaaggctgaagccccagccagaactccccagggggcatttgggaaggctaggagttcttgatgctgctgcttttaaagtcaacagaataggcatggccacaggccaaacttgaagacaaatctaggatcccactggcccctttccagcagccatagcccatgatgccacagatattctgtccaaccacaaagggcagtggtctctctcttcagagttgtggaaggagacctgaataggggagccgcaggctatggtgcagaggccactcctaggggccggagtctccagaagggctccaaaggacatggtgctgcacttccccagcgtcacatcctagcaggcaggctggggactccccgagctttcaaatccttgggattctgtcactagcttccaaaacagaaagggctgggccctttatcaaagttactccacaatgcctataattaagggttctctagcaggggactgagaacccacccccactgtcactgtcaggtcccaggctaatctctaatatggtttttcatatgccgagccaggttcgaagaccacctgaaggtctttccacacttgctgcatttgaagggcctctctcgagtatgaaatctcttgtggctaatgagttgtgaactcttgttaaaagttttcccacatatgctgcatttgtggcactttttcccaatgcttatgtcctggagtccagtgagcctggagctctggctgcaagcttctttgcagtcttcgaggggcatctcttcacttggttttagcttctgtaatctcaactttgtgtcctgagaggaagaccgtgcaggcgggctacgttcagcctgtgctgctctggtgtgtttcctctggtgactggaaagggtatgtctcccaatgaactctttcccacaccactgacatttgaaaggtctctctgtagagtggatcctctgatggttaacaaggcgatagtttctatcataagatttcccacatagattacatttatagcgcttctctccactgtgtattcccttatgatctaaaagggttcttttacgtgtaaaggttttcccacattcttgacaccaaaaacgtttctcaccagtgaggatttttggctccacatttggagtcttttcactttcatggcaatcatactgtttttgaagagagtgaatcctctgatgtcggtagagattggaactccatctgaaggctttcccacactccctgcacttatatggcttctctccagtgtgaactctctgatggatgaggaggaatgagtgattgcggaaggccttgccacactggctgcatttgtagggctcctctttggagtgactgctctgaggaacctggaacactgtgtcctgactaaaagatggcccgccctcaggttttcttttcatggcatgcttcttcttatgaacaataaaggctgacctataggcaaagtccttcccacaatcgctacactggtaaggtttctcacctgtgtgaattctctggtggtcaacgagagttttctttctagtaaaagttttcccacactgctgacacagaaatgttttctccacagcgggagcaccctggggctgactgcagtcaggagattgcctgaagccttcacgacattcatcttgtttgtagaatttttcctcctcatgcaacctcatatgacgagtaaagtttgatctccatctaaaggttttcctacatttggtacatttatagggcttctcctgggtgtgaatcctttgatgttcaagaacatatgacttacagtggaaggatttcctgcactggctgcagtcaaagagtttctccccactttggtctcccaaatgatgatcaaaccctgagctgtaggtgagagctgccctatactgattcaattcaagaaatttcttcttagcatgggtttctcggtgcagacggtaggctgacaggcgtcggaaagctttctcacataaatcgcatttataaggcttcactccagtgtgaattttctcatgccgcgcacagttggaactccaccggaaggctttcccacacaccctacatttaaatgctttctcttgagtgtgaagtctctgatgatacgcaagatgggagctatgactgaaagtccttccacagtcactgcacttaaatgacactcccactgtgtgaagactctgcccacgttggtgatgagagctaaggctgaagtcttttccacacacgtcctttttgttccctttcagtccactatgaattctctgatgtaggctgaagcccccaatcatgtgtctgagccccttcccatatttcttgtagtcatagtggtgtgaactcattctgaagtgtttgccacagccatgtttaagggattcctttcttccagaaactctcaaatatgtaacatgttttaagtcaagactattacttcctgatacttcagagtcttttcctgtcctgtgactgaaattggtctcttctttcttaactcttacttgtatgggattttcacattgatccttctgcctgctcttctgttgaaaagattctctgagcccaattccctcagaaacacttgtcgcaggacatcctgatgacacagctaaggtttctgcttcttccaaaggttcctgatttaagatgaatttgtttgttttactctggaggtcatctcctgtaggagcagcaactggattccccttaggctgagctgcctgcatgttcaggccccatggctcccttgcttccaaccaggagatcagagcaggtttggtgaatggtcccaccagggaagccatgttcctataattctccagcatcacatccctgtacaggttcctctgagcagagtccagccacccccactcgtcctgggagaaggtcacctccacatccttgaaagtcatggtctcctggtctcccgggcacccctctctcgggaaaagggcaggcatctgggcagcaggagtatcggattgcccagccaggaagtcacgtgcttctatttcatagggaggctccaggtggtcccccagagcagagctgctcctgagaggtgaagcaagggaccatatctgtgcagatcgcagggctcctgtacccatccaatgcacatctgggctctgggcagggcccgggtccctccaggatgtcccatcaaggtccctctgcagctcctccagcaaggccacagcctcctcgccactctcagggttatgaagctgcacccaaacccggagctccccaggcaggatgctcaggaactgttccagcaccagcagctctaggatctgtgccttggagagaacgtcaggcctcagccaccagcgacagagttcccggagccggctcagagtttctaggggccctgaagactcatggtagcgaagctgtctgaagagctggcggaacagctcctggccagggcggttgagagtctgtggcctggcagcctgcactggagtatagctttcatcctcttcttccttctttactgtctgaagccgccctcgctccctcgaagactgggcctgagctggataggcagcatgccacctgcctggaggcatcactcctgttcagggactaaccagaagagtgcgaaccaagtccaccttagacgtgggtcctcagaagtatcttctcagcagtcaacaatgccaacatttgctgggacatcagaagtcatcagcaagtgactgaaattaccagcatttcgactcccgccgccgagcgacaatcggtccacccgccgccaccgcagccgcccgtcccgcgcctacctcccggcggctcc

SEQ ID NO: 17370 - RNA, 4347 nt, Homo sapiens
  source 1..4347: mol_type = other RNA
tcaggccaggcacagtggctcacgcctgtaatcccagcactttgggaggccaacgtgagtggattacctaatgtcaggagttcgagactaccctggccaacatgcccaaaccctgtctctactaaaaatacaaaaatgagccaggcgcagtggtgggcgcctgtaatcccagctactcagggggctgagagaggagaatcacttgaactcgggaggcggaggttgcggtgagcagagattgcgccactgcactccagcctgggcaacagagtgatactccgtctcaaataaataaataaataaaataaattacacattcctccaagagcagaggaccctgacaggaagacagtttgaggtgttaacaaatttgcccatggaaaacaggtgctaccccttaactggggtttagaactgtgtgcctcggctcctctgaaacagcaatactgtaaaacgccgagaacctcatgctcagtctcgtttccaaatttcagtcatctataaatcacatcacgtgcttagaaggagagcaagtgaatggcaggcagaaggagggcggtgcctctactggctgtcagggtgagggtttctgtattatatgcttgatagtagctagcatgttgggagagggaaaaaataactccttctaataaagacagttcacaaatttcacataacaaggggacagggtagattatttttcaaataatactgttttgaaaattagctaaattatttgggaaaaatattgagtagttagtagctttctctggcataagaaatacataatagtagttggtagcttttttcttgacataagaaatacataaataacttacaaataatttatatcacaaattcgtgacaatttgctcaacaaattgtcagtcacatcaaccaatcaataatagccttttaaaaacaaaactctagattatattaaacctatgggtattttcatagtatgtgttcagaaaagagctatttctagttagatataatataaccagcttaaaatataaccagctgaagtctcccccgcctccccccaccccgagcccccaacacacccacccatgcccacctccccgctcagaggctgaaaacaagtgcagcaaggtgtggtaaaaggaaagcaattttattcaaatgcaagcaggtgggggatggccaggctcatgcctttaacagaccattccccgtttgggggctaagtaaaggagtttaagacggaaaagatatgggaaatatgtgggaatagtgcaggaacgtgcaggtctgcgtgttttgttctgaaggttatcttgagtgatggtctgtcctgaggcctgatttgccttttcctgactttggcctggtagtggtgggttaactgtaagtaattcccctctcaagggaggattctgcagccaggtttccctgccttgtttgtttcaaaatcggcccctaggatttctaagcaagtccttaattagataagaaacactgtgtatgaatgtacctggtgggaaagggagacaaagtcttacaacacaaggctacattctgagattcagaaagaaagaaaaaaaaagtttgaaaatgcattttgaggctgggatccttggtcacaataattcaacttgtacacaaaatgttttctccataaaattggttgctcagtatgaaacaactaaggctgatgtgactgtgccctttatgtaacaaatgatctaaaaaataacatgttagagacctagtactcaatgttttatcttctgtctctggaatggcttttctggatactaggtataatatatccaataaaaggcataaagttctttttggatttatgctgaagttgaaagacagtagacatcttctcccatacccagttgccttaaatttgctttagccttcaagtcagttacaggcctagttgcctagattgcaaagagaaatatgaacagagctaagaagggggagataaacttggaatagaagcagtacaatgtacaagttgggacaggaatggtctatgcttactttttttccttcctgtctctcttttaaatttcagcatgacacagttttgaattccaaagagtgtcctatattttctattatatgatcagactacatttgacctacctctctatctcatctctcaacatcatagcccatgacccagctcaatgaaattatgtataggttctccactgtgtcatgcttctatgcattctcaacatactatttctttctcgtggaatgtctttcttttccatctagctgatgctaactataagtggaaaccttcctgccctgccctgattgagatgccattcctgcactctcaaagcaccctgtccatcatgtaacagtgctgttcgtgccatggaacaactgccaatttagtttgctcgatctatccataggctgtaagttccttgaaggcctggctatatcttctggcattctgtaggctcacaaaatatgtgaagaatggtgaacacactgtgtttatggaaaacaacttagtataatttaatacacactaatcagggattacccagaacatgcagttttctagcctgtaaggcacttggataaataaccgtgatgagatgtcatctgtgtgctttctctaaacatagattaccaataacaacaacaaaaaacctaacaataataatgtgttttctgaggtttaagagcatgctaaaataataatgaaagatgcatataaacaaggttgtatagacgaaaaaactaaatcacagggaacttatttattttcttcaaatttgcaccagagaaactgataaaggtgggatttaaatgtatacaagccaaactgtagatattatgtgtttgaccataaaagatcacaaaaaggtgtttgctttttaacaattacatctactatttcctcatatggaacttgaactgttagctggtacacaagttatagtggtttttgccattactttaattttgtcatttactttaatggcaaaaaccgcaatgacttttgcacgaacctgatacattaaaaacgagtttcttaaatgttcaaacaaacaagagagtgtctcttcaaaagtctcatctaaaaagtatgctttaaatttatatgcagagtctttttttaatggctgcttttacctcttgatttcttaatgtataaataataggatttaagagaggtgtgaaaattgtgtaaaacacagaaagaattttatctaccgagtatctgctgaagggccagacgtagataaagacacacggagcaaagaacagagtcacaactgtgatgtgagctgagagagtggagaaagccttagaggatcgactagcagcacggtacctaactgagaatattatgactccataggagacaagcaagaggaggaagcagaccagtgacaggagcccactgtcagcaatgaccaggagctgtaggatgtaggtgtccttgcaggcaagtttaatcacaaggggaaggtcacagaaaaagctgtctataacattgggaccacagaagggcaaagtcaacatgaaagccatttgactagatgagtgcacaaatccaactgcataggaggataacagtagcccagtgagcacccgtgggctcatgatggtcatgtaatggaggggtttgcatatggcaacatacctgtctattgccatggctacaagcaacatcatctcactcccacccaggaggtgcataaagaacatctgggaataacatccccaccatgagatggtcttacgttctcggaggaaatctacaatcatcttaggggtagcaaaagaagccaggatcatatcaatgcaggagaggttgctaagcagaaaatacattggtgtgtgaaggagcgaatcaaaggtcacagtcaccaagatgagcaggtttcctaacacaatccccacgaagaccacagagaatcccaagaagaataaaatctgaagattttgagatttggaaagtcccaacaaaataaattccgataccactgaatggtttgctctttccatatcgtcaactttatcccataatgatcaaaataagtgagaataaggggtagggaaatgatgcatattggaaagaaatgttcatgttgatgtccacatttggtactcagtcaaggcacttgaacttacaaggacccttacttttgtggaattttgtcagtcagtgattttactaatggcccagagaagtatcccaaatagtcagtagaattcagaatataagtttaagacaggggaaaaaaactttcgtgatggcgtcgtacgtgaatcccaggaatggccttttatctccttttcctgtatccccatcagttatctgcaatttac

SEQ ID NO: 17371 - RNA, 4643 nt, Homo sapiens
  source 1..4643: mol_type = other RNA
tcaggccaggcacagtggctcacgcctgtaatcccagcactttgggaggccaacgtgagtggattacctaatgtcaggagttcgagactaccctggccaacatgcccaaaccctgtctctactaaaaatacaaaaatgagccaggcgcagtggtgggcgcctgtaatcccagctactcagggggctgagagaggagaatcacttgaactcgggaggcggaggttgcggtgagcagagattgcgccactgcactccagcctgggcaacagagtgatactccgtctcaaataaataaataaataaaataaattacacattcctccaagagcagaggaccctgacaggaagacagtttgaggtgttaacaaatttgcccatggaaaacaggtgctaccccttaactggggtttagaactgtgtgcctcggctcctctgaaacagcaatactgtaaaacgccgagaacctcatgctcagtctcgtttccaaatttcagtcatctataaatcacatcacgtgcttagaaggagagcaagtgaatggcaggcagaaggagggcggtgcctctactggctgtcagggtgagggtttctgtattatatgcttgatagtagctagcatgttgggagagggaaaaaataactccttctaataaagacagttcacaaatttcacataacaaggggacagggtagattatttttcaaataatactgttttgaaaattagctaaattatttgggaaaaatattgagtagttagtagctttctctggcataagaaatacataatagtagttggtagcttttttcttgacataagaaatacataaataacttacaaataatttatatcacaaattcgtgacaatttgctcaacaaattgtcagtcacatcaaccaatcaataatagccttttaaaaacaaaactctagattatattaaacctatgggtattttcatagtatgtgttcagaaaagagctatttctagttagatataatataaccagcttaaaatataaccagctgaagtctcccccgcctccccccaccccgagcccccaacacacccacccatgcccacctccccgctcagaggctgaaaacaagtgcagcaaggtgtggtaaaaggaaagcaattttattcaaatgcaagcaggtgggggatggccaggctcatgcctttaacagaccattccccgtttgggggctaagtaaaggagtttaagacggaaaagatatgggaaatatgtgggaatagtgcaggaacgtgcaggtctgcgtgttttgttctgaaggttatcttgagtgatggtctgtcctgaggcctgatttgccttttcctgactttggcctggtagtggtgggttaactgtaagtaattcccctctcaagggaggattctgcagccaggtttccctgccttgtttgtttcaaaatcggcccctaggatttctaagcaagtccttaattagataagaaacactgtgtatgaatgtacctggtgggaaagggagacaaagtcttacaacacaaggctacattctgagattcagaaagaaagaaaaaaaaagtttgaaaatgcattttgaggctgggatccttggtcacaataattcaacttgtacacaaaatgttttctccataaaattggttgctcagtatgaaacaactaaggctgatgtgactgtgccctttatgtaacaaatgatctaaaaaataacatgttagagacctagtactcaatgttttatcttctgtctctggaatggcttttctggatactaggtataatatatccaataaaaggcataaagttctttttggatttatgctgaagttgaaagacagtagacatcttctcccatacccagttgccttaaatttgctttagccttcaagtcagttacaggcctagttgcctagattgcaaagagaaatatgaacagagctaagaagggggagataaacttggaatagaagcagtacaatgtacaagttgggacaggaatggtctatgcttactttttttccttcctgtctctcttttaaatttcagcatgacacagttttgaattccaaagagtgtcctatattttctattatatgatcagactacatttgacctacctctctatctcatctctcaacatcatagcccatgacccagctcaatgaaattatgtataggttctccactgtgtcatgcttctatgcattctcaacatactatttctttctcgtggaatgtctttcttttccatctagctgatgctaactataagtggaaaccttcctgccctgccctgattgagatgccattcctgcactctcaaagcaccctgtccatcatgtaacagtgctgttcgtgccatggaacaactgccaatttagtttgctcgatctatccataggctgtaagttccttgaaggcctggctatatcttctggcattctgtaggctcacaaaatatgtgaagaatggtgaacacactgtgtttatggaaaacaacttagtataatttaatacacactaatcagggattacccagaacatgcagttttctagcctgtaaggcacttggataaataaccgtgatgagatgtcatctgtgtgctttctctaaacatagattaccaataacaacaacaaaaaacctaacaataataatgtgttttctgaggtttaagagcatgctaaaataataatgaaagatgcatataaacaaggttgtatagacgaaaaaactaaatcacagggaacttatttattttcttcaaatttgcaccagagaaactgataaaggtgggatttaaatgtatacaagccaaactgtagatattatgtgtttgaccataaaagatcacaaaaaggtgtttgctttttaacaattacatctactatttcctcatatggaacttgaactgttagctggtacacaagttatagtggtttttgccattactttaattttgtcatttactttaatggcaaaaaccgcaatgacttttgcacgaacctgatacattaaaaacgagtttcttaaatgttcaaacaaacaagagagtgtctcttcaaaagtctcatctaaaaagtatgctttaaatttatatgcagagtctttttttaatggctgcttttacctcttgatttcttaatgtataaataataggatttaagagaggtgtgaaaattgtgtaaaacacagaaagaattttatctaccgagtatctgctgaagggccagacgtagataaagacacacggagcaaagaacagagtcacaactgtgatgtgagctgagagagtggagaaagccttagaggatcgactagcagcacggtacctaactgagaatattatgactccataggagacaagcaagaggaggaagcagaccagtgacaggagcccactgtcagcaatgaccaggagctgtaggatgtaggtgtccttgcaggcaagtttaatcacaaggggaaggtcacagaaaaagctgtctataacattgggaccacagaagggcaaagtcaacatgaaagccatttgactagatgagtgcacaaatccaactgcataggaggataacagtagcccagtgagcacccgtgggctcatgatggtcatgtaatggaggggtttgcatatggcaacatacctgtctattgccatggctacaagcaacatcatctcactcccacccaggaggtgcataaagaacatctgggaataacatccccaccatgagatggtcttacgttctcggaggaaatctacaatcatcttaggggtagcaaaagaagccaggatcatatcaatgcaggagaggttgctaagcagaaaatacattggtgtgtgaaggagcgaatcaaaggtcacagtcaccaagatgagcaggtttcctaacacaatccccacgaagaccacagagaatcccaagaagaataaaatctgaagattttgagatttggaaagtcccaacaaaataaattccgataccactgaatggtttgctctttccatatcgtcaactttatcccataatgatcaaaataagtgagaataaggggtagggaaatgatgcatattggaaagaaatgttcatgttgatgtccacatttggtactcagtcaaggcacttgaacttacaaggacccttacttttgtggaattttgtcagtcagtgattttactaatggcccagagaagtatcccaaatagtcagtagaattcagaatataagtttctggttattgctatgtagtggttagctggttggcctgtgtatggttgtcataggtttcaaaatgacttagcttgatgtaacatttatgttggtaaaagaaatacagttctttcagtataatctaaatttatgacaaaatttgtcatcggctcatgcttattacaaactggttctattggttcagcttttaaaaaaattgcctccgttgctaatagttttaaattaatctaggtcttacaaaacaccttcagtaaataaagtatttgtagtcatctttttgtgctgttattacttacaagacaggggaaaaaaactttcgtgatggcgtcgtacgtgaatcccaggaatggccttttatctccttttcctgtatccccatcagttatctgcaatttac

SEQ ID NO: 17372 - RNA, 1080 nt, Homo sapiens
  source 1..1080: mol_type = other RNA
tcaggccaggcacagtggctcacgcctgtaatcccagcactttgggaggccgaggcaggcagatcccttgagctcaggagttcaagagaagcctgggcaacatggcaaaaccccatctctactaaaaatacaaaaaactagctgggtgtggtggcacaggcctgtagtctcagctacttggaaagctgaggtgggaggatggcttgaccccaacaggttgaggctgcagtgagccaagattgcaccactgctctccagcctgggcaacagggcaagaccctgtctcaaaacaacaacaacaacaaaatcacagatgagtaagacacaggtctttccctaaacaaggttacagtctaatgggcagaagggctaggacagggactcagatgaaataatgccaggtagaatgtgatcagtgcccctggaggtgtggcaagccaacactgtgaggaatcagcggcaggaagatcatatcaaatcacgaggctccagaaaaactacgagggtccaggaatggtggctcacgcttgtaatctcaacgctttgggaggcagaggtgggctgattgcttgagcccaggagttcaagaccagcctggacaacatgatgaaaccctgtgtgtacagaaaatacaaaaattagctgggcatagtgagctgtgcctgtagtcccagttactcaggaggctgaggtgagaggatcgttgagctagggaggctgacggaggtcgaggcagcagtgagctgtgatcatgccactgcattctcctgggctaaagggcaagcccctgcctcaattaaataaaacaacaacaacaacaaaataaaaaactaccaggaagggccatgaggcacagaaggattgcatcaggcggagataggagatgagaagagagacatttcaaggtgatatataaagaactaccagggggtgaggaagcatatggggagatgtgtggagacacagcctgaaagtcttgaagtcacatcacggagccttgaatgaccgaccgaggcgctgacactcaagagaggcaatgggaagccagtgaaggtttgtgtgtgtgtgtgtgcgtgtgtg

SEQ ID NO: 17373 - RNA, 412 nt, Homo sapiens
  source 1..412: mol_type = other RNA
tcaggccaggcacagtggctcacgcctgtaatcccagcactttgggaggccgaggtgggcggatcacgaggtcaggagatcaagaccatcctggctaacacggtgaaaccccgtctctattaaaaatacaaaaaattagccaggcgtggtggcggccgcctgtaatcccagctactcgggaggctggggcaggagaatggcatgaacctgggagatgcagcttgcagactgcaccactgcactccagcctgggagacagtgcgagactccgtctcaaaaactctgcaagagagcagaacaaggttcttatgaattattcaaatggttatatcttgtatgttaaaaatttttttataaaatccatatatatctagtctgtttcatcctataatcacctacctgtgaaacttga

SEQ ID NO: 17374 - RNA, 1084 nt, Homo sapiens
  source 1..1084: mol_type = other RNA
tcaggccaggcacagtggctcacgcctgtaatcccagcactttgggaggccgaggtgggcggatcatgaggtcaggagatagaaaccattctggctaacgcggtgaaaccccgtctctaacgttgctggtgggaatataaaacagttcagcctccatggaataagcttctcagttcctcaaatgaattgccatatgacccagcaactccactccttttgtgtttccatatataatcttgtaacatctcaagtcttccatctgtcagcgccggctcgtgctagctttctacattaggtggaagtctcagctctgtgtttggagtgcagggaaagcgaggacaaccagagacaaagggaggaggcaggacttcaatccccagccctggaaactctgctctgtaacttgatcaaagaagatgccagatcagagtggttactcagcagcaccagctgtaggagatgcattccacagatcctcttggcacaaacctttagccggcctttcacactgccaggatatccgctttgggacctcccccatttgagaagggcatcactctgatgagtttctagagtggaggcaaacctgggcttaaggtgccatcaagttccaaaagggagacagtgactgtactgagtgggcatttatttagttatttcacagtgaagatatcttttctggaaaattcctcataagaaaactgaaattcaagctcctgctcgttcttcagccaccgctactcgttcctgctttttgtgcccataggttcttctgcccaaaacaaaagctgttaaatcaccgcggcggcgctgacgtcagggagcagggccgcgaggccccaccaggtcgccaatgaagcctcccctcggctctgccgggggctttgcggggcgcatagaggctcccaggcggatagaggctcccaggcggaggagtccgggaacccctaaagaccctttaggaagcaaggtccggaaaaccaagcacgagcaagaggccccgggcggctgtatccctgcccggcgaattcagagggagcgggcgccgcggccacccaagagcaacgaagacggcggcgcggag

SEQ ID NO: 17375 - RNA, 1809 nt, Homo sapiens
  source 1..1809: mol_type = other RNA
tcaggccaggcacagtggctcacgcctgtaatcccagcactttgggaggctgaggcaggcagatcacgaggtcagaagatgaagaccatcctggctaacacggtgaaaccctgtctctacaaaaaatataaaaaattagtcggtcccagctaattgggaggccgaggcaggagaatcgtttgaacctgggaggtggaggttgcagtgagccgaagtcacgccactgcactccagcctgggcgacagagtaagaatctgtcttaaaaaaaaaagaaagaaaaaaaaaaagtggcctggtaggaggatcgcttgagcccaggagtttgaggctgtagtgagccatgatcagaccactgtacttcaacctgggtgacagagcgagaccctatctcaaaaaaaaaaaaaaaaaagttcataatttaaaacccacctcaagtgataatcttggaaccttggttttctcacctgtaaaatagggatgataatactaccgatcttgtagggctgttataggattaaatgagttaacacagtgacgtgcttagaaactgtgcctcgtacacagcctacgcccaataaaatgtttgatgtttttatctcgccttcacatttgcccagagacaaagcagcacacggatttgagatttcccaggactggctttaatttgaaaaatctgattggggtctcttcccgtatcagagaaggaacagcccaagctatgaccccagggccagggaattcagtccccaccagaccctgtcattccatcactagggggtaattccaggctccccctgccagccctgagacaggaggacggatgtgaagttgcccaggactagattctgtctctccaaagtggcccaagccctgttctctgtactagggaagccagctgtgtcttttcgaggacagttggtccagccagcaggctcagttcagataccagacaaccattccagcacgagggctcagcgccctggccccggcggtcgctccagtgcctgtgtgcccaccagcacatccatgaggtagtccaattcggcctcgtccagctccggagcttcctccttgcccggcccatcctcagggcctggtttgaggccctcagaggctggtgcccaaagttcattgtcatacatagaggtgtcaatatcctcaaacaggccctcaagcccatcgtccagtagacagccagtggctgggcccagcaggtccaaggcacccaggctgggcgctgctcccccgatgctacggcctggtggcccctcgtctgccaagggttggggagcctgactcaggccctcaatgtggctgaggtcctccaggaggctggccatggaggctgaaagggcagcgtccgagcttgccagtaagttgtcagccacactgggggctgcaggtgggctaggcacaggtggcagggcagccgcgggtgccatggacgcctggatgcgccgcagagtgttcacgaccagcaccaggtgccgcaggtccggctcactctgctgcaggctgtggtggagcttgagcactgagaggtcaaagagggagctagaggccacggccgggggtgcctgtgccaccgctgtgtggccaggatctagccaccaggagtcgactgccagaggttccttctcctcctcctcctcccgtttccgcttcagacccttgctcagcatcttgctcactagcggccaatcagaacgaagaggtagccacccacaaccaatcaggaaacggcggcggcagcatcgcttgttggctgtcctccggaaacccgcgcctgggtcgcgagacgcagttct

SEQ ID NO: 17376 - RNA, 9588 nt, Homo sapiens
  source 1..9588: mol_type = other RNA
tcaggccaggcacagtggctcacgcctgtaatcccagcactttgggaggctgaggcaggcagatcacgaggtcaggagatcaagaccatcctggtcaacatggtgacacgccatctcttataaaatacaaaaaattagctgggcgtggtggcacacgcctgtagtgccagctactcgggaggctgaggcaggggaatcacttgaacctgggatacggaggttgcagtgagccaagatcgcgccactgcactccagcctggcgacagagtgagagtctgtcaaaaaaacaaaaaaaacaaacctgatgcatatttcctaaagactacaacattctgatattctatgtatagtatatatttttgcataactgaataaaacacataatttaaacactgttagtgaccaaagccaccatgtttgagaaaaggcaataaatttcagcaactgtttaaactgcttataaatatagtatgccaaagctggaagtttactggataggaagagtagcttagacagaaagcgtctctgaggctctatgactggctaggtacccgacccacgcgttctcagagtaccctgtgcttgtccctgttgtcacacccaacatgccgtgttataactgccagtctctgtgattacacactgcaggatccttgagggcagggatggtgctggttcactgaagtacccttcgtgcttgacatacagtaaagactccataaataattgtttgataactactgaatgagtaaccagccatcttcactcattgatctgctgggagcaacagaagcaggcaagagtagcaccacatgacacaggaataagaggcacggtttccaagagcaggccggacgcagtgactcacgcctgtaatcccagcactttgggaggcagaggcggattgcctgaggtcaggccgagatcagcctgaccaacatggtgaaaccctatctctactaaaaatacaaaaattagccgggcgtggtggcgggcgcctgtaatcccagctactcaggaggctgagacaggagaatcgcttcaatccaggaggcggaggttgtggtgagccgagattgcaccactgcactccagcctggcaacaagagtgaaactccatctttaaaaaaaaaaaaaaaaaaaaaaaggcacggttaccaagagcctgtgtttggtgtttgccagatggccaaaggctcccatcaaaatatgactgatggaatactcagacatgtccattcaataatgtccctacagtacgacatactatactcacctattatgagtgacaccaaaggatacatgatattttggctaggatcattttgactgttaagccaactcttacacacaccttaccaaaatttgcaaactgtctattaatcacaagcaactaagcaccaacaacactattcaagaaaggaaaaatgagttagggtgggttatattttactaggaaattcctctggctatattctataggaattaggtgtaatatctgttatgcaattgcttagcatagtgtttggcaaagtattaacaaagcctctttcccttctgcatgagaattttacctttgttaactttctagctctgttcccctggcaacctaataaaaattcatatgtcaactgctaggcaatgttacatatggtagacatgatgcccaattggtaaactgcatctggactgggagaactataaatgcctgataggaagcctcagctctgggcatccctaagtacagtgacgcttggaacaggcatgtcttttatagggacactggaggccatgtctatgaagctgttataagagatacttgttcctgtgggacaaggggctcttaagccggggaagcttccatacttgccccatgtagatctgtctccttgcacctgcactatgccacacagacagctgcagagactttcagagaagagcaactggttctgccttgctagtaagcagtgcttcccattctatatccttttaagtgaatctgatgccaagtgtggcagtttataaatttgaatgtttctaaaccttcagttgggcctaagacccttggagggcactgcagtattatttgcatgtttttctgatggcagtagatgctcctcaggggctatggatggtaaaagatgtgaaactgtttggtatgtttttctacttccaaaaaaatcctgaccatacccttcactgtatgcatgacagataatccatatccattacatgtcaccaagacctgtatatgaaattgatgccttccttcaaaatccccaagcttgttactactaaaccttcctcatcaaagcacataatccctgccctaacctccactgattaactgacaaaggtccagaaatcaaatgatggatataaaaattgccccccctaaaaccacaattgtcaatgaagaattggcagtagtaaaataatctacctggagggtcaagacggatgctaaatgttctccttcagttatgaagtttccatgtcatccgatcatgcagtcatgtgagttactgtcaccttttaaaactaggatatatttaggccgggcgcggtggctcacgcctgtaatcctagcactttgggaggccgaggcgggtggatcacaaggtcaggatattgagactatcctggctaacacggtgaaaccccgtctctactaaaaatacaaaaaattagctgggcatggtggcgggtgcctgtagtcccagctactcaggaggctgaggcaggagaatggcatgaacccaggaggcggagcttgcagtgagccgagattgtgccactgcactccagcctgggcaacagagcgagactccgtctcagaaaaaaaaagaaaagaaaaacaacaacaacaacaaaaactaggacatgtttaggaaccaaccaaactactctgaccccaaaacacttttcgtttttctctacagaaacatcatttgaagaaaagaattcaaatttccagcactacaatgaaaggtttgtggaacacagtactgttgagtggagagaactacaaaagcaacagaaatcaatgaaaacagtgcccatcatatgcacctgaataaagtgtccctttatcaggttagaagatagtgtgatcacatgaaaacacaaggcaagctacaagagaccagcaacaacaggaagcacagtgggaatgctcaaaacagagcataataggaacttctcacccatcccaaccctttgcccctccctaccccattacactagacttcacagagatcattctcttaatgcacaagggacacacacaagaaaaatctagagttccaaataaaacagtctgagttcagttaaccaaaggccactccactctttcctacggctcccagaatcagtgcatgcagccctacctgttgcctttctctccctggggtttgtcacgacatcaatgaacaataacaaaaaaaacccatctcagtattccaaaccaccagaatactcaattccataacatgttgcagaacactaggtcagcagcttccttaaggaatattcaaagtctggtggccaccaaaatatttacatcagaacggcatctttctgccaaatgatcagaatcatgatgcactatgtcatttcttaattattataggtaaggccctatttacattccttctcaacttttgagaagggggtcctcatcccccaagagaaataacttcccaagaatgccattttggaattccattacaagtaagagtcctgttcccattcatgcaatacatctaatatgagacgaaaatatccctttgtgaacttgggtggaatgtgccagaatagaaactaaaccactaacggtctgtgttgggctcaactgtaaatttacttagtataaaaataccaccaaccccacaaattaaacctcaaagacactgtgattataaatactgaccacctaaaggggaccaatttatgatctgatagtctagacagaggaagtatctcctttaaaagtgatagaactcagtgatccagttattgccagtgcctatacacaaactccaaatagtccaccagaaatgcaacaatctgagatattacgaaagaaagagaatcatttaaacattaggtgtcacattctgttttcttcccagtgattctgctactttaaaaattaacaaaatgatcagaacctagtaacgattctgggtgtatgaatgagtcagaattttctaagtttccacattataaacctaaatcagatcttgggcaagctatgaaccatctggcctcagcgcttcattttactaatccactattttctaaaatttgcgagagtataaggggctactaaatattatgaaggtcagccaggcacggtggctcacgcctgtaatcccagcactttgggaggctgaggcaggcggatcacttgaggtcaggagttcaagaccagcctggccaacatggtgaaaccccatttctactaaaaatacaaaaattggccaggcgtggtggcgcgtgcctataatcccaactactcaagaggctgagacagaagaatctcttgaacctgggaggtggaggttgcagtgagccgagatcacgccattgcactccagcctgggtgacaaagatgaaactccatctcaaaataaataaataaatacataaaataaaattaaaaataaataaatattatgcaggtaaaaggtagcttaaaatagaacacaaaattaagtccactcattaaagatcctttaaaaaatcctactttatcttacagcagagtttctcaacattggtattactgacattttgaattggagaattcattgttgtggggactgtcctgtgcatttcaggatgtttggcagcttccctggcctctacccactagatgccagtagccacctgcaaggcacgaaatcacccccaactgagaatcactgtcctacagtgaaatctctaatgtaaaatgttttacccagggatatgaagaggtcacggaatcactgaagaggatcatagctccactggagaaagcaggcaaagaggctgaactatgaggtagaaaagtcattaaaacatcagagataatttaaacagagaaagcaaaaatatcaaacactgttcctggccaagtaaatcttctacacatccatttaggtttcctttttgctgagatccctcttttaaaataacagcaaatatatgtatacatttttggagacagtttcgctcttgttgcccaggctggagtgcagtggtgtgatgtcggctcacagcaacctccgcctcctgggttcaagcgattctcctgcttcagcctcctgagtagctggaattacaggcatgcgccaccatgcctggctaattttgtatttttagtagagacggggtttctccatgttggccaggctggtcttgaactcccgacctcaggtgatccacctgccttggcctcccaaagtgttgggattacaggcgtgagccactgcgcctggccacagctagtatttttatttcagataagacaaatatctctggtccctgataattttcaatgagtaactcttgatctagaatatttttcttttatttatttattttattattatttttttgagacaaggtctcacactgttgcccaggctggagtggagtggcacgattccagctcactgcaaccttttccaggctcaagtgttcctctcgccacagcctcctgagtagctgggattacaggcacatgccaccactcctgactaatttttgtatttttgctagagacggggtttcgccatgttggtcaggctggtatcgaactcctgacctcaagtgttccatctgccttggcctcccaaagtgctgggattataggcgtgagccaccgcacacagccaagaatgatatttatcgaactacctgtgataagagaagttttaaattttccattctactgcagaccaatacgtggtcctgctgtacaggctggtatccaacctctgcaccatgtggccctctagctgaccagaactgaactggtccatacctcactcaagaagacaaagccatgagtcacagcaatgtcaaagtgttatcaacatttctatatgtgtattcttaatttctgactttccttgtagcagactggtagaaaacagtttacagaacagggcctctctgtgggccagagtttgagttgcactgttccagttttaactactattgagaagtacgacttaaacacctgtctaatgctttggctaacatttacaagccaatttataatgtttttgacttttttgttgttcaagaggtagaaataaaagtgacttttaccaccttttgaaagacaactacacttaaaggaagacaagaagatttcttttaaaatccattttggatattttaacataagacaaaattatggaaattgccttcaattacattccgaattcctaacactgcctgccctttagccctttaaagagttcagcctcttttgttacaataattgtgtggctggaaagtgggcgaaaggtagactgcttttaaaaacctgttctgctactaaccttccctttccctcatgaagatcttttaaaagatgaacattttagaaatgttacttggcattatgggcttatactttccctccaattaaagttctaggcaaggaggtagaaggcaggactcaactccaaaggccggactcggacatggaccaaattgaggactagctaaaacagggcggtggtgggagggtggtgcaggaagcagatttccataagaaacacttatcactgtgccatgtcaattaccattgccatggcaacacctggaagtcactgccccttatcatggcaaccacccagcggcttggaagttaccaccattttcctaaatattgctgcataatctgccccttaatttgcatgtaactaaaagtgggtataaatataagtgccgacctgcctctgagctactactctgggcacactgcctatggtgtagccctgctccacgaggagcggccccttagctgctgttgggcactgctgcttcaatacaagctgctgtctaacaccactggcttgcccttgaattctttcctgggtgaagccaagaactcctctgggctaagccccaatttttgggctcacctgccctacatcagcataaactaagtaaaagaatgccagaggcagctacatttccaagttacacagctccagcttttggaaattgctggaaaaagtaggggagcattttgagttttgcccaaatgagttgttttatgataacagaacaggttgtatgtgtagaatcgtcaaatgccaaaccagacagggaaaccatccagacctggggtcatagcctcccttctcagggctaacttaaaatttaattcaactgggcaagtcaggatgccataatgagcctttcagatcattcccatgttcgtctgcccataagtattccaagcctttaaaattgttctagatttagggagtaccttttatgatcatgtagccagaccgccctgcctgctttatatcaatgaaggtttctctttaatactttgccagaaaatttaatgtggaattcattaggaaaggcttggcaaaggtaaacttgatcccaaaacttaatggtttttagagaaagaggatgataacaaaggaatgcagaggactgaatcaatataaaaacaagcctggagattttcttatctttctcctaaccagagtttggacacacagcaagaaaaacaggagacctcagggcctgctttgactcactcagaattaaggagtggccagcaaagccctcagaaaccaagggcaccacacaaaaaggttatctgtcctttgagtcacaaaatccaacctctatcagatagtctaataaaaatgcacatataataacagtgaaaaaatgttcctctcagggttccacaaaattggacaaatggtatctttcaacaacagaacgagcactaacaagttttaaaacctcctcttccccaccaatttattgctacgtaagtgtctctcggtctgataagttaggctgaatttgtggtttgtcatcagaatcatctccagcagggtcattttcctcacccgactccacatagattggccagtcattgtctgtgtcgctcttttcttggctttcagatgaagcctccaccaagctaaggttgatgggcatcaaatcatcatcatcatcgggtgtgtctgtaacgcaggtgcagctgtcacacagcccgaagcgccgcagcccctgggacaggtgactcgtgaatgttctcctgcagcccttgcagatgattggacggttggatctgtggacactcagtgcgtggctccgcaggtgctcttgtcgagtgaacctcttgccgcaggtctcacaggggtagggccgctcgcctgtgtgtgaacggatgtgccgcttgaggatgcccttctgtttggcagtgtaagggcagaaaggacacttgtggagcttgatggggaccaccagcacatcacctgagtcctctccataccagtcagcctggacatccatcatggaactcatggctactcctgcaccttctggtcttccttccaaactcctagaaaagtgatggtctgcatcatccttgctcggggcagcgctgttgcgcaagagcgcctccaggaactgcttcacgtggtagttgctgtaagccaagtcaaccgcctggccgcttggcaaggcctcctccacgtgggccaggttcagcggggcagcatactgctgcagctgttcaccaacgtccacctccacttcatcagcatcaaattccaccttgggctctatccgtttgggtggagtagagaggttgctgtcagccgagccaccgccaaggctgtctctcaccaccagttccaaggggtggcagtctccgcagtcaccgcaaggggactctctcaggcactccacgctcttttctccctcggctggagaggagaccaagctcttggtaccacaggaggtcccctcccggcctgaactggggctttcactgtcaacctgatgagccgccgctgctgccgccgctgcagccgccgccgctgccgccgccactgctgcagccacagcagcctccttctccatctttcggcaaatgtcgagggatgacctaatgtatgtcttgcagaagttcaccacgtcattcatctgcaggtagctggcagccgacatcacttcaatcacattctccccacacaaatccaacttcccagaatagaggaaatctaagatgatggagaaggcatcagaggtgacaatgtccaaggaggcggtgctatgccgcccgctgtcctggatatagtgaatgagcagggctcggaagtagccgctgttagcaaacaaaatgttcctgtgggccttgaagatccgcccttccacaatgatgctgcagtcacagaaaaagtccctctttctctgttcattcagctcccccaaaagcttggcataataggattgcatctccattgctccgccagctgctgctgctccagagcaaacctgtatctcttccagcgggttccagcagcgcagccacggagc

SEQ ID NO: 17377 - RNA, 9732 nt, Homo sapiens
  source 1..9732: mol_type = other RNA
tcaggccaggcacagtggctcacgcctgtaatcccagcactttgggaggctgaggcgggcagatcacttgaggtaaggagtttgagaccagccgggccaacatgatgaaactgtgtctctaccaaaaatataaaaaattagctggttgtggtggcgcatgcctataatcccagctactcagaaggctgaggcaggagaattgcttgaacccagaggcagaggttgcagtgagccaagatcatgccactacactccagcctgggcaacagagcaagactccgtctcaaaaaataaataaataaaaataaataataattaaaaaaaaagactgggccaggcgtggtggctcatgcctgtgatcccagcactttgagaggccaagactggtggatcacttgaggccaggagttcaagatcagcttggccaacatggtcaaaccctgtctctaccaaaaaaatacaaaaattagctgggtgtggtggcacacacctgtagttccagctactcaggaagctaaggtgggagaattgcttgaacctgggaggcggaggctgctgtgagctgatagcgccactgcacttcagcctgagcgacaaagtgagactgtctcaaaaaaataaataaaaaacaggctgagcacggtggctcacgcctgtaaccccaacacttttggaggttgaggcgggtggatcacctggggtcaggagttcaagatcagcctgatcaacatggtgaaaccccgtctctagtaaatacaataaattagctgggtgtggtggcacgtgcctgtaagcccagctacttgggagtctgaggcaggagaatcacttgaacctgggaggcagaggttgcagtgatccgagattgcaccattacactccagcctgggcaacaagaatgaagactctgtctcaaacaaaaacaacaacaaattaaaaaaaaaaaaaaagaatggctatgcagttacttttctggttacagaaaaaatcctgcagacctttataggaataaattattgatcaatccaaactttcaccatgaagtaatcttgtaagtctggaggactcttaaagttatgaattattatggaaacatggagctcctaagttgccataatctgtcttcacattgcttgggctgagggtggggacaaaaaagagcaggtgggctgtctaccaaaagagatataacccataaggtgcattcttcctaatgcagtcatggaatacttctgccacacctgtttaacgggtgacagcatctgtaaaagtgacatttggatggatgtcaggaagccatcaacaagcagttaacaaagcacccactgtaggcctacaactaggcttgtttctatggcaagtataaaaataaggagatacatgtgggtcctgtctccaaaagcataaaatattattttaaatgtgctttttgtttcttattttaaaattagaaattctaagtactatgtagatgttaacttttcttgggtctgtatcctttccaggaaaggcaggataatagggagggctttgtcacaactggcagatactgctgataaatgacataaatgacatactcaaacacaaaactccagcaatatagtgactggtagctgccaaaactttctgcaaaccacatgaaactgcttggggagaaggcattatgtaaatgctaaggtgtaacacctaagaaaatagctttgaactcttaggccgtttggttatatatgtcaaaacttggatttcctaaactaagtcttatttaaactataattatagtttacaaatgcttatatattttactggacttaattttgaacataatgtcatcaagtgctgccaaaccatttttgaaaagataattcaagaaattaacagaaagctcaattattgaagcttgcggggtgggggaccctatcagtggactgcatgactgcagaccacccccaccaaggtacagccttcaacacagtccaaccctccaaaaacatcagggaaaacatctccaccacagattctatgtcatgcaaatgaagagattctgacagcctctttaagatctcatatcctggtccctaggagcttcctaacttctagtggccattaattaaagaaacataatacctttatgaagtaagtagtctttcaggaagaccgcagtgtgacatgcctgaagaaatacatattacagactgggtgtgaatatatctgttgtttctaagagctggtggctcttatattgaatgagctggccactttgcctaaacatgctatgatttaaacaaacacaccatgcaccatgaactgtcatagcatttttaaccctccatcaatatccaacctgtatagaatgtgcagagaagtcagatcttgaagaggcccaagtctatatagctctaaggcagggaagtcctgtcttcctgatactcatgtagttaaggaaattgctaacttgatgggttaatattcactcaacctctcaggaaattctactgttgtgtcaccagtgcatgtcatctgaagcttcgtaaaattgctaaaccatacaaaccataccatgttattttggaatttgtacaacttaatgcaccctaatgggagcataatgattatgttcattcaagttataaagcaattttatatttacaaatactttacaaaaataattcattctttacatcaaatgtgatcaataaaaattaacccaatttcacagataagcaactagatactgatataaattacacagaaatcaattcagaacaaaaaatatgaatttattctctttaaacttccagcccttgtaagtccttcctacctctaattaattcagcagagtagctgagctaaaagttcacacaggatttactactcaactcttcttccagcttaaagtaagtaggaggaacactactctttaaagttccatggctaaaggataaacagaaacataagcgcacatcatttcacaattaggctctttcggttgcagcctaatttgggggtttgaaacattcagctgggaaatagagggtccatatagaaacagacccaattgttgaaatagagtttgaaatcactccaacatctgatttgtgttcaaggttcacaatgaggtcttaaccaagatatgagacagcagttgctgaatctcaattgtcatgatcttctgtgtgttccatttcaaccccctgctatatccactgtattcatcatcacagtaaacaggtatagaatttccatcacaaacagtatgaatagctaagttacatctcattggatgagcctatccatactcttaagactcaagttatttctgttatctctaaatgtgtggcttctaagaacaggaacgtaacttacttttcaatctaacagtgcaaatcaaattacatggattctaaaaacaccaattgacctaaaagaagaggtattcattgggggaaaatggctacttattcaatttgtatgagaaaatgggaaaaaagaagaaaaataaactatgtttacaggatatgacagaatatcccataaactaacgttatcacaataaaaatgctgcataataaataagttattttaaacataaacattttcatataaaatatattgtcaaatttgaaactaagttcaaactttcttgtaaaatagcctctagaacaccaattgaggtaacagggactcaagaatactgaataaatgaacattacataatttgcattaataacttttaaacctgactctttaataaatcttggaatatctcttttagttgtaaaaaagatattcggttaagagtttggattctattttgatgtttagcaagccaaattatcttttttgtatgatgcttaaaatgtaaacagcactgcttgacacaataattataaactacatgaatgaaagatttgctaaaaatttcatttactaaaatcagccatttttctgattttatcctgacaaaagagtaaattacaccttgggatatatatatatgttttttttctgtcagtttaatccattttattgacttctcaattaacaacaaaattcatttggacagtaaatcagaaaatactttctatggtggctttaaattacattttttaacccaaaaatgttatccagagccattttagacaacaaatgtatcttaagtacaaacggtaaaaattcacattcccttcagtaactctccttccacttagaacacaatgaacttcttaggtaggcagagttctcgttcacttaaccacaaccccattttagcacagaactgcagcaaaaagaattgaagaagtgattagaaaggatatgcattattaataaaccatatgctatgtgagtgttaggttcccacgaaatattttactgtatatttaaaaaaaaatcccttctcaagggcactgctttcattcaaggactgatttcattacctacttcattatcttttatagtgaaatgctccttttcaagttattaatacacattggagttgttaccagcaaacactgtcctacacctgcagttcaaaatatgagtagcagtctaatacttagattcagttataaattatatatgtataaaacaaagagttgccattatttatatattgtaataaatacacaagaatgaatacaagttatttttcataaaatacaatttctaatcaatttaggggatttccacactatgaggacattaaatacttaaaacaccaggtaatcccctctgttacagaatgccagccgggtgagatcttaaagagattctttattgatagccaaatactgttgactatactagcaatctgtattttcttgctatttaagaaaaaaatacagaacctagacatttaaaacattatccgtgtaataatcactacagactctcactgggtctttaaaaattttgttaaaaatcgccaaagtcatgatgaacacaattaatgcagctacatcatttgaaaaagcaatataaattatgctgttaaagacaaaaacattgacatacataaacatcacaatgtaacacagcagtaactaattgctatttcatatgaaaaattaaatgtaaaaagttatgctagagaacttggaaatttttcactttagcaaaatgttctatttatatacctccaacttctatgatacagtatacaataaaatactttaaaaagatatgacattcaaatgcttcatttacacaaataatattgccaatactaataaaagtgatgcccttaaacatgaactgctctgctaattgtaattttaaaatgttttctttacttgattttacattttaattagcaggtagcattacatattaatcagttctgtgctgacaaataagagaggtcctagtcaaaatactgtttctcaaaagtaatgtacatcatattgcttgaaactaaacaaccatataaaaagtggcaatcatttatctaaacattgattatgaaagacaactggcatatattcaggcagagtgttgagttcatgattgtttatttacaataaaagtacttttactgaagctaacataagtttttaggtcaattactacagtctcttaaagttataaaaatattatataaaataccacaggctttagaggctataacttcatgtggttctgatactagcagctgaaaagtgtttataatttaaaaataaataaactatagaggtaaaccagttacaaaacagcagaggactgagatagtcacaagagtgaaaagaattgctcagttacacaatagctaacaaaatggtgaagcagttggatcaaaagttttaaaaacctctttcagagatttgtcatctgtttctctaccgggatcattatctggggtcgggctcccctgtcctggctgccttgcctgccttggatcactgtactgtggcctaattaagcctgttaatgcctgaacaggaaggctgtgcactgctgggacctgaaccttaccagaactcctgggaacgtccgcctgtgggtcagctggcccctcaagagtgactcccacgtttggactgggtttttgtggaaggatggcttctccaggagaaggttcagttttgtcactactttttaagccaccactttttttctggttctttgagttttctcctgaagaagctgttgctagctctgatgtggatgatgaaccgtgatccctagggtcatacaaactaataccactaagaactgaagtggaagttcccagtggaaggccagctgaggaagagagtttaggggcatatggaggcagagccccggaaccagaattgctagttcctgcccctgagggctgtgatgaaccagggtttgatctgggtaagtgaggggcaccctttgatgcatgtgaatccttcataaccacttgatgagactctgtattgggcagtctgtgaagcctaggatcaaaatttttttgtagtctaggatctcctaatttagctcctgaaccgtgtgagtctccaaattgttctaggtagccttctctgtttgttgtgttaattttggctttggctgctaattttggatcaatggacactgtattttgatgaagatcactttttgtattccataatctatttagcctctggtcagctataagtgggggcagaggtaaattgattgaagacactggatcaggtttaggtaaaggtactggaagtaagtcttcgggagcccacacgatgtgttttgcaaagttgggtttggttagagtaatgtccattttaatgtgactgaactgtctcaattgtgaccttggatcctggagcattatgccaggtgaggcatccaaaggtattaagaaagctttttctctcagttctctttctgtatcttcatcatcatcatcgcctcttttgtgtttgacattagtgccagcatttgcatgatgcaaatcaaactttgctccaccaacagaagagcctatgtgaccacttccattccctctcaatttcctgggatcccacgcaagtctaagatccagtggggcagactcagaaggctttctaatgtcttgccttgggatagtcctaagcctagggtcaaccacttggtttcctttacttttctctttagcaagtcttggatcagtaggagtgctgagttctgtggaaggttgttgctgattccttaaagtttctgtttgtttctgtaatgttttcagtattgatttgacactgcttccttcttcctcttcactactggaataccagttaactgtatcatcttcttccttgcttggtgccctatgaggttgggtgctggtttgttcttcatcttcttggtatctctgagtaagtcttacaaaaagagctctttgcactgcagggaggaggcctggtacaggcagagggccatggcctgtcctagtgctgctgccatcagacccactcccatggttaggtgagtcttgaacaacaggaggctgctgctgggcaaattcaccatgccacatcccatcaccagagttattgggtggctgaaaattatgtatagaatgctgtgcatagtaattatcgtaaaactcagctgggttttgcagggactcataattggtgttgagctgcatttcaccaggactttgctggtatgatgaacctggagaacagtgattctctctgggtactttcatcacatgtcctggaaagcctggggagtggtaagccccacccatacttggtggtgtcaaagatgtgtctggttgaacaagcactccagcttgattttgaggacctacaatttcaggtggaccaggtggtaaaggtgggctctgtggcactggtagaccaggaggtcctgcacatgggtgatgtccaggggagcctgggtgcatcacaggactactgtgtccctgagacatgttaggtccaggacctggacttgacccagaactatagatatgttgagggtgtggactgcttccctgaaattgtggtcctggtggtgaggcactggtataaaatgctggtggcttcctcccaattttatgcgctaaatccacagtaggttttacaactatttcaaaaagagatggaattttcctaaaatcatcagagaaatctgtctgaaaatcgtcttcaggatcagaaaagggaaaatgctctggaggggttggcagaagcccaacccctggaggtggtttgggaagaggagttatgccacgctttctaagttcctctaattctctttcatcttcatttatgagttcttcatcagtattcaacactttgtccaaaagtttctttgtttctttagttagatcatcatgggaaaatttacagttgtctccctggtaacattttgctccactatgatagaacttgcatggaaattcattatgcatataaatgcagttctctcctttggtacaatatccttgtaaataaaatttgcagatctcttttcttttctccaactctgcatcatgatcaaatttacactgatctcccttaatacacctcccttccaggaagtatttacagatttgttttcctttgtgttccactgtgtgctgattaataaattcctgagtcataaccttccattttttccctggtttattatactcttgaaagtcatccgatactgaaaacacattaggccctttattggttcttcccccacgttcttttcgtttgattttcttcggcaagccacgtccacgaccaacattaaaacttttaactctctgttcaataccttgctgaactcctttcattctctgtttttttcctgattctttagaaaatgatgaccctaaagcaatatttgaggtttctttagcttgcctgtattgtttcagctgattggcaaaatcttcctctgtttcctgaccgtagttaccaaagttgtcatcactgtagttaccgaagttgtcatcactgtaggtgctgtactcatcatattctttacttttaaattttttgttatgttgacccttctttgatgttatgtagcttcctgatatatgtccacgctgagtaaatggaatgtcataatccctgtagaaaccagttctttttttatgggaactttctgtatgttcaacatctgaatcaaggctgtagtccgaactatcatcactagatggggaattatgcttatgtttctcacgttttctccttttggattttttcttctctctctctttcttatgtttttttcttgattttctgtaggctttctcacttttctgcttttcattctcttttgcttctttttcttgtatttcttcaaatcctgcatcgtctatttcaccatcttctaattcgccatcttctctgtcgtgccctgcatgttcagagtctgtcatgtttggtcaagaacggggcggggctggagggcaggtctgcgaggccggcggcggcggggcgcggggaagaccccccgcgccgcctgcgggaacctgctcccggccgccgccgacaggtgacgaagtggtaaaaactcacggttactagtgagcgacacagacacagactttccagtctattaacaaccacgccagagagatggggctctaactgcaaacactgggcaacggccccgcgctgccggcgctgccgctctagtctctattcgccgccggtggctgtggcgtgggagcgggcgggcggcgtgcagcgacgcggggatttggacagtggccgtaacggtgatttctcctcaccaacatggcggcacccgaaacaggcggctcgagaaaatggc

SEQ ID NO: 17378 - RNA, 3309 nt, Homo sapiens
  source 1..3309: mol_type = other RNA
tcaggccaggcacagtggctcacgcctgtaatcccagcactttgtggggggccaaggtgggtggatcacttgaggtcaggagttcaagaccagcctggccaacatggtgaaaccccgtctctactaaaaatataaaaattagagacgggcatggtggtggcacacctgtaatccccactactcaggagggtgaggcaggagaattgcttgaacctgagaggtagaggctgcagtgaaccgagattgtgccactgcattccagcctgggtgacagggtgagactccatctcaaaaaaaataaaataaagataaaatcataaacactcataattcagttataccttttttcaagtaactaaagttcaaacttacttaggggaacaggctttcctgggtgccacctgcttctcaagtcctgtgctttccacaccacagaatagtaaactgggtgcactgagtgcctggttcccctcagcccttaaccagtgctggcttgtccgagtttagaatcccagggctgactttgttggtggaatgctagctcccattcatttcccacctgcactggacgttttctgaatctccttgaagtccgggagatcttcattccaaagctcttcacttttctgcagcattgtgaccccatctggctggggaactggaagtcctgctcagagaaaagcaggaggggacatggagttctgaaattcactttctgctcccatgtctggaagtgacaggtgaaatgagaatgatagtgcctctcaagaaggtctagttcccagaagagaaagtttaatgactcattttcccccttttactcctttgagggtacaggataatgcccttatctattttcataataattataatgatgatgataatgaaaactaacgtttgccaagtgctaatactgtgtcaggatcctcataacagcccagggaggtagaaaccatcacaatgtccactgtccagatgagaaaatggaggctaagggtatttaaagaggttgcccaagaacaacaaaccttttaaatggcagactggtgtgtataatctacgcagggttcacatctatggaacactttattttaaattcttttaataatattattatttttcagctgagtctgggtctcactctgtcgcccaggctggaatgcagtggcatgatcacagctcactgcggcctccaactcctgggctcaagtgattctcctgccccagcctcccgagtagctgggactacaggcttgcgccaccatgcccggcttatagggcactttagatggaaacaaatgactggatctttaactcctacctttctctcctctcttcctgtaatgttgttactgaaggcaggaagggagactccttggctaaagagcagagcaagagcctcaaagtggtctttgtgagccaccctggactactggttcagtagagggttgagtcaagcaatatttgaggacgggatataaacagtatttcttaaagttgtcaccaatttttcccccgatgaggccattccagacccaaattagtcataacagagccaggacaataatcacatctcctgattctgagcctgaatgcttcccacaggactgcgtcgctcccactgctctgaggtccattgtgggggagagttgccactgggattccacctcaaggcctggggaccaagcctccaggattcctcttgagactcctccactatttcattaccatcccgccacatcttctagtgctatgccctggttccctttggaatcctctcaatcccaaagaaggcctcctaccacctctaaggcatcaaaggtgttagaaagtgccccaagactcaacagggcatccatctcatcatagaagacactggtgcctggtgtgtaggtgctcctggctttgcagtagtcggtcaggaggtttttgaaccgatagcaacattgctccagggtccacaggaagccatgttctcacagctgctcagccataatccggtacacctggtggtttcgatggcaggtgcggagtttttcgtggatccaggcctctgagaattcccagaaaaatcttggtttctttgtatccccagtgcactcctgccaccttctcatcctccagggcctgccactccagctcgctccaggtcttggcttttctccagattagcacctggccagacttgactctcaccccagccactgagcagtctttcacactctctttttctccagaatttgaagatctagatgctgtgggttttcatcctactccacgtgggagttcactttgggcctatggattggaaaatccagcgtgacctcattttcagaattctgctgagttatttctaggtggttcttcagtccaggttctggatccctccatgcctcctgggagctgctcactatctcctggccacccctgctcttctctgcaggaattcccagagccacatcaggcagggctccagcctctgtcttccaggttctttctgcaagtcttccaccagggccactgcctcctctccactctccggatgctgctgtctgacccagatctggatctcctggagaaggacagtcgggaactgttctaggaccagcaactccaggatctgctcttttgtacacttctctggccttagccactgacaacagagcttctggagctggaggagggcctctcggggtcgtgatgcttcttggtaacggaaatgccaaaagctctggcaggatgtctctggtccagggtaattcccttgaagggaaatttcctgctcccagtgggaatcttcttccagtttaactatttggagatcttgtactgaaggagtctggatttgttggtccacagctacagccattgttcaggtcagagaagagctttgcaaccgcactctaaagctcaaacctcttcatcacctcactgggaagccatcttagaacttccacttaggagtcactaagtggaacttctcttgaaattctagagtcagagacatacattacaaagttaactctagtaaaaatcgcaagtgttagcccagcaggcttgaggtgaagaagagagccttcctgtcccagccctgttgcatgccctggtgcctgtggagtcactggtggggtggcagttccggaagtttgataagaggagtcaagggctagtgacctggttgaaaagtagaggagcttgaagctgagagaatacggacgattcggccccgtgacatgttcttagcggggacgcaagaagcccgagcccaggtcccaaacacggctattcggctagccactgagcaccgga

SEQ ID NO: 17379 - RNA, 3867 nt, Homo sapiens
  source 1..3867: mol_type = other RNA
tcaggccaggcacagtggctcacgcctgtaatcccagcactttgtggggggccaaggtgggtggatcacttgaggtcaggagttcaagaccagcctggccaacatggtgaaaccccgtctctactaaaaatataaaaattagagacgggcatggtggtggcacacctgtaatccccactactcaggagggtgaggcaggagaattgcttgaacctgagaggtagaggctgcagtgaaccgagattgtgccactgcattccagcctgggtgacagggtgagactccatctcaaaaaaaataaaataaagataaaatcataaacactcataattcagttataccttttttcaagtaactaaagttcaaacttacttaggggaacaggctttcctgggtgccacctgcttctcaagtcctgtgctttccacaccacagaatagtaaactgggtgcactgagtgcctggttcccctcagcccttaaccagtgctggcttgtccgagtttagaatcccagggctgactttgttggtggaatgctagctcccattcatttcccacctgcactggacgttttctgaatctccttgaagtccgggagatcttcattccaaagctcttcacttttctgcagcattgtgaccccatctggctggggaactggaagtcctgctcagagaaaagcaggaggggacatggagttctgaaattcactttctgctcccatgtctggaagtgacaggtgaaatgagaatgatagtgcctctcaagaaggtctagttcccagaagagaaagtttaatgactcattttcccccttttactcctttgagggtacaggataatgcccttatctattttcataataattataatgatgatgataatgaaaactaacgtttgccaagtgctaatactgtgtcaggatcctcataacagcccagggaggtagaaaccatcacaatgtccactgtccagatgagaaaatggaggctaagggtatttaaagaggttgcccaagaacaacaaaccttttaaatggcagactggtgtgtataatctacgcagggttcacatctatggaacactttattttaaattcttttaataatattattatttttcagctgagtctgggtctcactctgtcgcccaggctggaatgcagtggcatgatcacagctcactgcggcctccaactcctgggctcaagtgattctcctgccccagcctcccgagtagctgggactacaggcttgcgccaccatgcccggcttatagggcactttagatggaaacaaatgactggatctttaactcctacctttctctcctctcttcctgtaatgttgttactgaaggcaggaagggagactccttggctaaagagcagagcaagagcctcaaagtggtctttgtgagccaccctggactactggttcagtagagggttgagtcaagcaatatttgaggacgggatataaacagtatttcttaaagttgtcaccaatttttcccccgatgaggccattccagacccaaattagtcataacagagccaggacaataatcacatctcctgattctgagcctgaatgcttcccacaggactgcgtcgctcccactgctctgaggtccattgtgggggagagttgccactgggattccacctcaaggcctggggaccaagcctccaggattcctcttgagactcctccactatttcattaccatcccgccacatcttctagtgctatgccctggttccctttggaatcctctcaatcccaaagaaggcctcctaccacctctaaggcatcaaaggtgttagaaagtgccccaagactcaacagggcatccatctcatcatagaagacactggtgcctggtgtgtaggtgctcctggctttgcagtagtcggtcaggaggtttttgaaccgatagcaacattgctccagggtccacaggaagccatgttctcacagctgctcagccataatccggtacacctggtggtttcgatggcaggtgcggagtttttcgtggatccaggcctctgagaattcccagaaaaatcttggtttctttgtatccccagtgcactcctgccaccttctcatcctccagggcctgccactccagctcgctccaggtcttggcttttctccagattagcacctggccagacttgactctcaccccagccactgagcagtctttcacactctctttttctccagaatttgaagatctagatgctgtgggttttcatcctactccacgtgggagttcactttgggcctatggattggaaaatccagcgtgacctcattttcagaattctgctgagttatttctaggtggttcttcagtccaggttctggatccctccatgcctcctgggagctgctcactatctcctggccacccctgctcttctctgcaggaattcccagagccacatcaggcagggcttggcatcccgttctttaacgtaatgtaatacatttcacacgtcttccgtctccatttggattatcaacatgacgtacataacccgttccattgaccggataacaagcagccatggcttttgtccggcccggggacgcgcgaggcggggacgcggccgccgcggggtcggccgcggacttggcctttgccttggctgcgtccccggaggcgctgtcccggcgcctcgctgccttcctggcctccagggcccggtccctggacggcggcgctgcagcgggcggcgcggggccggagtcctggtgagggccccctccgtggccgagggcgccctcgctgccctggcacacgagcttgtgcttcttccagtcctggcgctggcgctccttgcagcagaaggagctgcggctgcagcgcagcaggttctccatcttcccgcacagctcgcagtactgccggtctcgctcgctcgagctcggctcgccgggcccgcagctgtcattggccatggcgaccgcagctgagcaggaggggtgcggccggacggcctcgcccgaggctccagcctctgtcttccaggttctttctgcaagtcttccaccagggccactgcctcctctccactctccggatgctgctgtctgacccagatctggatctcctggagaaggacagtcgggaactgttctaggaccagcaactccaggatctgctcttttgtacacttctctggccttagccactgacaacagagcttctggagctggaggagggcctctcggggtcgtgatgcttcttggtaacggaaatgccaaaagctctggcaggatgtctctggtccagggtaattcccttgaagggaaatttcctgctcccagtgggaatcttcttccagtttaactatttggagatcttgtactgaaggagtctggatttgttggtccacagctacagccattgttcaggtcagagaagagctttgcaaccgcactctaaagctcaaacctcttcatcacctcactgggaagccatcttagaacttccacttaggagtcactaagtggaacttctcttgaaattctagagtcagagacatacattacaaagttaactctagtaaaaatcgcaagtgttagcccagcaggcttgaggtgaagaagagagccttcctgtcccagccctgttgcatgccctggtgcctgtggagtcactggtggggtggcagttccggaagtttgataagaggagtcaagggctagtgacctggttgaaaagtagaggagcttgaagctgagagaatacggacgattcggccccgtgacatgttcttagcggggacgcaagaagcccgagcccaggtcccaaacacggctattcggctagccactgagcaccgga

SEQ ID NO: 17380 - RNA, 2090 nt, Homo sapiens
  source 1..2090: mol_type = other RNA
tcaggccaggcacagtggctcacgcctgtaatcccagcatttcgggaggctgaggcgggtggatcatgaggtcagaagttcgagaccagcctgaccaacatggtgagaccctgtctctattaaaaatacaaaaattagctgggtgtggtggcgggcacctgtaataatcccagctacttgggaggctgaggcaggagaatcgcttgaaaccggaaggctgaggttgcagtgagccgagatcatgccactacactccagcctaagcgaaagagcgaaactctgtctcaaaaaacaaacaataaatgttttcgaatcactggtttctatccttgcattttatagataaacagactgaggcccagaaaaggggaagatttttccaagggtctaactagaactattttgtttagtttatttgtgtgccatagccctttacttagtaaacatttaggaaattggagtaacagtttaaaccgacacacaagagcagggagtggcgtgacttgggagttagagaagaccactgcctgcagctcaaggcatgcctttcctagcccaaaaccagcctgtcaaaactctctgctaacacattctgcatttagcacatattgacatagaagttttttggtctaccttccaactaaactgcaagcccctgaagggcagaggccaaatcctataaaatgttttgttgacacatttgataaaccaagactttacacacagacaccacataaatagttgttgattaaatcatcatttaaataaaagaattcaatcatataagtagacagaagacttcagttaggaaggcggccaacaaaggactctcagacaaactttttaaaaggctgttaataaccacacatctgacaagggttaatgaccagaatatgtaagaaactcaaatgacccaattaaaaaatgggcaaaccatgtgaacagacatttctccaaagaaaacatacagggccaggtgcagtggctcacacctgtaatcccaatactttgggaggctgaggtgagatgaacacttgagcccagtagtttgagaccagccttggcaacatagtgagacccctctctacaaaaaattggctgggcgcggtggctcatgcctgtaatcctagcactttgggaggccaaggcgggtggatcacttgaggtcaggagttcaaaaccagcctggccaacatggtgaaaactcgtctctactaaaaatacaaaaattagccaggcatggtggcgtgtgcctgtaatcccagctactcaggaagctgaggcaggagaatcgcttgaaccttggaggcagaggttgcagtgagccgagattgcaccactgcactccagcctgggtgacagagcgagactgtgtctcaaaataataataataataattaaaaattagccaggtgtggtggtgtgtgctcgtactcccagctacttggaaacccgcagtgagtgaagatcgtatcactgcactccagcctgtgagagagagcgagaccttgcacaggtataggaagagaggctccaagtcagcgcactcacagttcctgagtctctcgtcttccacagacactggagctgtgcaaacttactggccgcgctgatgaaagtacatagattcatggccaggtctatgatccacttctgcagggcaaggatgaaccaagaagacaccaatacagcgatgtaaggagtggcctgcttcacgttcccgttaaaatgaaagatacagagcaggaggatgacatcttgcgcgatgaggatggggtactccaggtaggtcagcggcggatacccatagtaacactggtaccgcagaaacaccaggaatcctgccagctccagaagtaaactcggaaggctgaggccccgcgcgctgcgcgccgctagcacagcggagatctgcggcagcttcagcgcggcgcacacgcccagcgtgctccagttacacagccccagcagcgccgcctccatagcgccacgggcgcgggcacctgggcggccgcagcgagaagggaccgctcagcctcggcggcgcagctctgccgaagccttccgccttcccgggatccgcccgggac

SEQ ID NO: 17381 - RNA, 4876 nt, Homo sapiens
  source 1..4876: mol_type = other RNA
tcaggccaggcacagtggctcacgcctgtaatcccagccctttgggaggctgaggcgggcggatcacctgaggtcaggagtttgagaccagcctggccaacatggcaaaaccccatctccactaaaaatacaaaaatttgcaaggcgtgctggcaggtgcctgtaatgcagctactcaggaggctgaggcaggagaaatccttgaacctgggaggcggaggttgcagtgagccatgatcactccactgcactccagcctgggtgacaaagtgagactccttctggaaaaaaaaaaaaaaaagatgcaaaactttgacacagcagtccagtgtggtggctcatgcctgtaatcccagcactttgggaggccgaggtgggtggattccttgagctcaggagttagagaccagcatgggcaacatggtgaaaccctgtctctacaaaaaacacaaaaattagccaggtgtaccgaggtgcacctgtggtcccagctacttaggaggctgaggtgggaggattgcttgagccccgaagttcaggctacagtgagttgtgattgcaccactgcactccagcctgggtagcagagcaagaccttgtctcaaaaaattaaaaataaaaatactttgacatagtcaaagtttgtgctctctttaatttttttcattatcaaaagagaatattctatatggaattgtctgtcctaccaaaggtatgaccttgtaaatgtgtatttgtcttttcaatccaattctccttttatatccatattttactcatttcttaattgtaataaagtggaaaactgatctaattatatataaaaccttgtgtcaaaatagatttaatgattaacactaatcaattgccaggagacaaaacacaaacaaaacagataaaccaaacaaaactaaatctaccaccaaacttacaacaggaatagaaaatggtgaaagcaacagaaatatatgtgactgatacaatgttgagatactttcccttcaatcattataagcatttgtcaataacagttctatcatattttcctttttatatttaaagtatcatgatctccacattggatgctctataaatatcacaatcttaatgatgaattctagactcattcaagttagagcaactgctttacacaaaatgatagcagtagacaaatctaggcagctgcttgggtggggtggggttctcacaggttctgaagctagcttgcagttagaattttgggagtcaatagaagtaaatgaattcatgaaatatttcaaattatgattcagtgcaagatacatacatatcttataattctattcatcataaatattttcatatgtatatgagaatacatctaaatatatgtaacatgtacatatataaatgtatgtatatatgagaaatgcttgtaaatttctgtcccaaacttagaattatgtacaagatccctgaatttcataattcgaggcagtgtaattttataggcatgacatgggactagaaaagtgtgctcactcattctaaacccagttgtcaccaacctgctagattctgggcaagttgttcttccatgccttagtgtgattatggcaaagtagaatttgcctgtagccctttaaagaggattaaaataagtgcaaagtgcaaagtcacatgagcaaaagtgcttatgtaaagccaagacacaaggaatagcaagatttttatatgcaacgtgggtaacttttaaaagcaagttagatttcctaattaaatgtaaatgttgctagatgatttatttgcaacaagcaacaaagagactgagaatctaaaaggataaagtctttggcagtctgtaatgattaaggacttacttttatctgccttaagatgatgcatcttaaaagagagacatacactcacatatgcactgtaatatgatttatgctttctaaacttttaatttggtaggaactatcaaacatgtgggtttgcagtctcactcctgtaaaaattataaaacaaaataaacaatgatcattttataagtgatcctaaatgataagaaaatgtaatagcctggcaaaaacataaagcacagaaatttctattctatttttcaggagtatgttatttcttgagctcctggaagaggaaacaaactcacatatacctacatacccacccagataaatttgtgtgcatatactccagaaatttatagcttatatgctgctacattcttaaggaaaaactggttatacatatgatttagaagaagagacaaagaatgggtttatatgattatggtgttttccttttgtgttcagacatattaagagatgcaaaaggtttctggtaacattaatcaatattattttaagagcagaaaagcaaattactttttccacattctcaaactattacttatgaagtttaacaaatttcaaaataatcatatgtagttatacagagagataattttgcaacgaagatgggagtatttactaatcagtaacaggggcaacttcattaagttctagtgtctcctagattttaggtctgtttatttgatagcataacaacccttgcaaatccttttcattgcaaacttgtatcttctgaagaactaacttcatagcaaatagtattttttagaagaagaaaactactgaccccactacctataataaaacatgactgacagcaagagttaagaactaaactctgcaaaatatgatgactgctgtgcaataatttaacatataaaaccaagtgattatattaaggtcacagatttatactgaaatgtcaaattctgtgaagtatttctaaccccccgccaaaaaaatcctaagaaagagtaggtccaatatctttttggataatctttttttttttttttttttttgagatggagtctcactctgtcgcccaggttggagtgcaatggcacaatctcgcctcactacaacctccacctcccgagttcaagcgattctcccacctcagcctccccagtagctgggattagaggcacccgccatcatgtctggctaatttcttttgtatttttgtagagacggggttttgccatgttggccaggctggtctcaaactcctgacctcaggtgatccgcccacctatccctcccaaagtgctgggattacaggcgtgagccactgcgcccagcctgactttggataatcttaatggttagacatccttgcttttttaatattcaacacaagaaatctataacctttatctgtacaaaggatccaaagagttcactaattctacctatgctctttataagaaagattttttttgaaccattaaaacaaacattacaaaaaagtgctttcttcttaactgcaaggatatagagtcaaaaagtctcttatcaagctgataatgatcaagttcaggtccaagatgcagacagaacttctgtggtacagtacatggacttattcttcctttattccttgcagtttgtcataaaaagttggatagtcatgtcttttgtggtcttcttcttcttcttcttctccttctcctcctcctcctccttcatctccttctccttcttctcttttcttcttcttttctttctttctttttttattttatttttgagatggagtcttgctctgtcgcccaggctggaatgcagtggcgtgatctcagcttactgcaacctctgcctcccaggttcgagcaattctcctgcttcagcctcccaagtaggtgggactacaggcatgccccatgacgcctaggtaatttttgaatttttagtagagaccgggtttcaccatgttggccaggctggtctcgaactcctggcctcccaaagtgctgggattacaggcatgagccaccatgcccggcctatcaaataacacaaatttcttataccaaaatgacaaggtagtcagtgagatgggagagacatagattttttaaataccctaaatccttttgtgtgcccaggatatggtggtggtggtgaaacactgtgttttctggtcagcgccactgcctgttcataagaaggtaatcctgcatcctccacagaaggcggcaatggagacaaggcagcctcctcaggtcttctgaaaatgatggagggagtgtgcctccccctttcatagacggctgaagagcatggatgttgtagcctattacacttagtgatacaaagatagtagccaagtaatccaaaaataaccaaaaatactccagcagcaattaatccagtcagaaggcccataacatctattttctctctgttgccatctgattttgtggttggtcctttagctgaatattcctgccaaaatgcaatcgttttatcttcatccacaaaaatctctctggcttcctcataattgcaaagttcttcattgcactctctttctaggttgccgggagtgaagagctccagatcaaatctattatacagaaggcgtctatgtatgaaaaagtttgcttcttcttttgatgtaaacacttcttctcccgcatgcttagaagcctttggacctcttgcgcaatgaggaaaccccagggtaactgtgggcagttggctgagtagaaccagaagcgtaaacatagtctggcaactgtcaaacaaactgtgtccccccgcacatgttccagcagcccccgggccagaggctcttcttggggcggttccttcggccgccaggccctcggtctccggcgccctcaaacctcggcgacgctccgggcctcgctctccgcagggtctggatggcccccgcgcgcaaacctgggaagggcctggggttcgcagaggggcgcccggggaacacgcgcggggtgaggtcctgcctcggtccggggaggcggccgacggag

SEQ ID NO: 17382 - RNA, 124 nt, Homo sapiens
  source 1..124: mol_type = other RNA
tcaggccaggcacagtggctcacgcctgtaatcccagcgctttgggaggccatagcaggtggatcgcttgaggtcaggagtttaagagcagcctggccaacatggtgaaaccccatctcttcta

SEQ ID NO: 17383 - RNA, 5370 nt, Homo sapiens
  source 1..5370: mol_type = other RNA
tcaggccaggcacagtggctcacgcctgtaatcccagctttgggaggccgaggtgggcggattacgagctcccatcctggctaacaaagtgaaaccctgtctctactaaaaatacaaaaaattggccaggcgtggtggcggagattagaatcccagctactcaggaggctgaggtaggagaatggcatgaacccaggaggcgaagcttgcagtgagccgagatggcgccactgcactccagcctgggcaacatagtgagactccatctcaaaaaaaaaaaaaaaaaaaaaaagatacagcatagtaaagaatctcaatattaatatgcatagtaaataacattttttctgtaaagtcataagcagacatggagaacatggagactaagaaatcaacctggtatttgaaatgtacaatgagtcttgaataatgaaaacagatttcaaaatttggagatctggtcaggatgctgtagacagaggggaatattctagcagatggcaagtataaattgaaatgtaatctcggcacctgaacttttgtggaatcacacattagctaaaactcaactataaaatctaattacatttcttttgaaaccttcttttaaaatgttgatcagttattaataatttaatatgtgtaactactaggaatagtaggtaaagactcagtgcagtaaaactcactataaagtgtgtgtggctcatctgttcagccatcacgctcaagaaaatgtgctcaagttcatttgtgactaactggcaaagttctcatcacaaaacaaaagctccaaactgaaaaatgttcttaactgtctcttaactggactcaattgcttctctgccatgaaatcttttttttttaagcaaaacattgcttaatcattttcttttattgttatgcttaagaataaaaacacataaaactgatcaatatggcaatcaagttaattcaataagacacttttttatttgtttaccacctgtaagtgccacagagactaccactacaggaaaagacaatagaggaggaagctctaaggtaaggtttgagttaattttctatatttaaagtttctttagaaaaatgtcctttggtttgtagacacagttcatataccattagttgaagctgtgcatagttatacagggcggaaatgtctcctttaaggttaacgtcgttttacacttacaatgtgacttctttatttgaaatgtggctagtttcatccagtctaaattggagatacgtatcattgtctctttttgcctcaggacagtactggaaatgagatgtttcatttcaatgcatttttctcagtggaaacacagttgagcaatcagaaagtcacttggttaagtagcagctttgggctggtcctcgtgcagtggtgtttacaactaattgatcataaccggttacagatttctttgatccttttccactcccactgctttatttgactagccattcagcttcctcttctttcaaataatactgggttctttagagttttcaagcaggtcatctttttcatccctttaatcactgtggttggtcttttctgaaaaaaacagtttttccacatccttctcaggtaattttcatgactttacaatggcttgtgtttaatggcagagtgagccaaaggatcagagatttatttggctcttattagcttgtattacaatagtgagagaatgttctggcttatagacaaggaggaagcaataaatatagcatgtcttaccttcaggaaaggttttgattctattatgagtaccattttactcagcaagccagaaagttaatcatcttcattacataacaaacgggggttcatggaacctcacccttctaattcttataatgctgaaccaaataaagtggcccttgtactcacttgtatacctttgagggggcaggggcaatctagttgatgtcctattttgatgctctcctgcagcctattaggtcctgagttcctctggcttatcagtcaatgaaccagggttcacttttccagactgtacctttctgttactcttccttatactagtataacatttttatagggttgatataagctttgctcataaaaatacgggaagaaaaatcagagaatataacaaatggagacattttaaaatcacagagaattagtgttctcactgtccctggaaattcactcactgatttaagttcctaagttaattatcataagttttagttgctatcttgatctgcacctaaaacactcccctttggtatcattaatgttccaagatcagctactgagaagcaacataggtgaggtattgaataggaaaacaggctgggagggtcttttttctcctgggaatgctgaataaactgtgggttgtatgcctgcattttgactgaaactcattacataaggtcacatgtggaattttccatttttatcatgttggtgctcaaatactttcagattttggaggatttctgattttagattttccgattagggatgctcaacctgttcttctaaaagcttagctaactatatgggtcctcttcagtttaaaacatggattatgtgtccttcagcatgttccattccacctcacatgagtaatgctctgggaggtgtacaagcttatatttcacgctcttaagatctactgatcaaaaatctagcccgaaagtccatgagggcaaggattatgtcttatacctctttatagccctctttgtgcttggcattgttcattttaccctgaacttactcaataattgagggacagagcaggatttatacttaggatgctggacccagagtttatacctgggtcactgcccctaggctgggatggagccaggttttcaccagccagtctagacaaggaatgaagtctcatctgtagatacagtgaaacccctttgtcctaccataagctaattaatgaaatgaaactttttgaaaattaatagaatttagatgcaataccagaatttatagtataaataattaggataaaaacataactttttaactcacgaagtgcatatggtgtggcagagattgttcggcaagtttgctgcttcacttgtctttgtttcctaaagataaatttagtatcatgcaagaaatgcacattacatcctttcggtgcaataatatttcacataaatttgatttgcctgaagccaatactgtaaataaagcaaacatattctgtgtttcattttttaaaaagagtgatgaacgcagttcctgggcttatttaagcttcctgcgttttataactttttcagtgggatgaattagcatgatgtggtgaaacaggctggcagatgccagaggaaattaagacttcctgggcatacaagtaagagaactccacatatagcagagaaataagaacaatctgattttcaaagcagttgctaatcttatttctgctcatatctactctacatgtttctcctgatgtgaaacttttatgaagttccagttttagggttcactgaagaaaagactgccaataatcctgaaccctgccatattttatcaaagcttagacagacaaatggtcataaggaactgaaataaaaggaatttagtatctcagtggactgctgtaagtaggattcctaacccaaagaccaaatactgagaagtcaaacgtaaatatgtgtgtgtttgcatgtatgcgcatagacatatatgtgcatacgcatatatgtgtacgtggagagaggaagaaacgaagaagaaagaatgagagaggggtaggggagattcagagactaaattgggaagagtaaaagtagaagagtagcttcaaatagatttggtctgaaggctaatttgtgaaagtacaattagagaaagacaatgactgcaattataaacctcattatctttaacagttaagcaattgttaaaagacacaaaaagtaatttaagctttatgtgctatcaaccatgcaaaagttattaaattcatcatttgtacatatgtggaaatatagacatatgttaacatcttatatttaaggatatgttgagcaggtatgcattctatagtaaataaatatataatgaaaaatagatatagaaaccagtgattgaataacatgactttgtaaaccaagcaaaaggaaaaaacacctcctctctttctctagctgatattctcattgtcactgacaggttagtataatagtaaaaatgtcagcaattattttaaaccaagaagcaatacaatttcattttttctagccaagaaaataaatcactatatctaaaaatataattaaaaaatgattaaaattgatagctggtaatgctttttattcattaaaccattaaattctcactgtaaccccatttgattggaaaggaaagtaaggcttcaagatgttgagtaacttgtccagtcacaaagtaaatggtagatatgggatgtgaattcagtttcctgttgttccagagcaggagtagcaaaccctacagttaccctacagcaaattcattgggaaaatgggctctcattgtccagtcaaatgttttaaaagaataaagccttttagcagggcaggtatatatgctctgttgaccctattctgattcttgattactacatttaaaactacctcaaaatgtcgtggcataaaatctctactattttattgggctcacatttttatatgttaggaagtcaggaagtactcaggtggggggttcatctctaatccatctgctattaactggggtcagctggtgctgaaagattggcttccaacttggcttcttcatttgcaggtctggcacttttgttttccctgggctttctgtttctagcacagcctctcagcctccaagccctctccacatgggcttgggtgggagtagtcacacttattaaatggtggttagcttccaacagggaggaagtacaagtttccaggccagttaagggctgtgcctgttactggcagtatcagttctgcatactgtattggtcaaagcagtctggggctgctgtctcagattcaagtaggtggcaaagtaaactttacctcttgatggaagagttataacagctcaatgcagatgagagatgttgtgctcgtctttggaaaagacaatctgtcacaagccctgtaactccaaattgctttaaatctagtatcttcagatattgaaaatacttgccaaccacacaaggactagagtttatgtctatacagtagagcttatttttataactaccattaaatcatcttctcctaatcttaaatactaattatatacagataacaaaagaaagtcaacactgaaaataaatataaaacaaatatgcacaaaattacaagaag

SEQ ID NO: 17384 - RNA, 6188 nt, Homo sapiens
  source 1..6188: mol_type = other RNA
tcaggccaggcacagtggctcacgcctgtaatcccagctttgggaggccgaggtgggcggattacgagctcccatcctggctaacaaagtgaaaccctgtctctactaaaaatacaaaaaattggccaggcgtggtggcggagattagaatcccagctactcaggaggctgaggtaggagaatggcatgaacccaggaggcgaagcttgcagtgagccgagatggcgccactgcactccagcctgggcaacatagtgagactccatctcaaaaaaaaaaaaaaaaaaaaaaagatacagcatagtaaagaatctcaatattaatatgcatagtaaataacattttttctgtaaagtcataagcagacatggagaacatggagactaagaaatcaacctggtatttgaaatgtacaatgagtcttgaataatgaaaacagatttcaaaatttggagatctggtcaggatgctgtagacagaggggaatattctagcagatggcaagtataaattgaaatgtaatctcggcacctgaacttttgtggaatcacacattagctaaaactcaactataaaatctaattacatttcttttgaaaccttcttttaaaatgttgatcagttattaataatttaatatgtgtaactactaggaatagtaggtaaagactcagtgcagtaaaactcactataaagtgtgtgtggctcatctgttcagccatcacgctcaagaaaatgtgctcaagttcatttgtgactaactggcaaagttctcatcacaaaacaaaagctccaaactgaaaaatgttcttaactgtctcttaactggactcaattgcttctctgccatgaaatcttttttttttaagcaaaacattgcttaatcattttcttttattgttatgcttaagaataaaaacacataaaactgatcaatatggcaatcaagttaattcaataagacacttttttatttgtttaccacctgtaagtgccacagagactaccactacaggaaaagacaatagaggaggaagctctaaggtaaggtttgagttaattttctatatttaaagtttctttagaaaaatgtcctttggtttgtagacacagttcatataccattagttgaagctgtgcatagttatacagggcggaaatgtctcctttaaggttaacgtcgttttacacttacaatgtgacttctttatttgaaatgtggctagtttcatccagtctaaattggagatacgtatcattgtctctttttgcctcaggacagtactggaaatgagatgtttcatttcaatgcatttttctcagtggaaacacagttgagcaatcagaaagtcacttggttaagtagcagctttgggctggtcctcgtgcagtggtgtttacaactaattgatcataaccggttacagatttctttgatccttttccactcccactgctttatttgactagcctgtaagaaacgtattaaaatgtatcagaaggtgctccccatgagaaatctgctcctcagcatctttaaaaaacaatctgacaggtttggtcaccatctagttttggcaatatgagtggcatcaccagggataggagggaagttaattttaggtcaacataaagaagatatttctaatgattatgctatttttaaatggtattataatttcctcagctcactaaattgttaaagcagagattaaatgataaatttgaggaatagtttaggatgatgcatgtatcatgaaaaaaacaggttagaaattgagcaaatctatgctttttacccacttacggcttagttgcctcttacataaaaatgatcatagtaaggttatcgaaaggcagaggactacaacattcattttaagaaccatgactctttgacctcctctggtcaatgaattcgtctcatgaattaccatgaattaaacttagtttactttttcaactgatgttaatgataccacattccatggttgttatagattaaatgaagtactaacacttcatttgaaaatgaaaactgaaactattaaactaaagctaagtagaaagcccttagcccttcattgtaatttttttcatcatttaataacacaaactcactaaataaattgatttttgaaaataaaaataataaataggttattttaatttttatatcccttcacaccttacctgcttgtagcctccagctatacataatcttcatagctgtttgtattgttgttactgttgttcaggttagttcttattccagagaaggacagagggcattcagcttcctcttctttcaaataatactgggttctttagagttttcaagcaggtcatctttttcatccctttaatcactgtggttggtcttttctgaaaaaaacagtttttccacatccttctcaggtaattttcatgactttacaatggcttgtgtttaatggcagagtgagccaaaggatcagagatttatttggctcttattagcttgtattacaatagtgagagaatgttctggcttatagacaaggaggaagcaataaatatagcatgtcttaccttcaggaaaggttttgattctattatgagtaccattttactcagcaagccagaaagttaatcatcttcattacataacaaacgggggttcatggaacctcacccttctaattcttataatgctgaaccaaataaagtggcccttgtactcacttgtatacctttgagggggcaggggcaatctagttgatgtcctattttgatgctctcctgcagcctattaggtcctgagttcctctggcttatcagtcaatgaaccagggttcacttttccagactgtacctttctgttactcttccttatactagtataacatttttatagggttgatataagctttgctcataaaaatacgggaagaaaaatcagagaatataacaaatggagacattttaaaatcacagagaattagtgttctcactgtccctggaaattcactcactgatttaagttcctaagttaattatcataagttttagttgctatcttgatctgcacctaaaacactcccctttggtatcattaatgttccaagatcagctactgagaagcaacataggtgaggtattgaataggaaaacaggctgggagggtcttttttctcctgggaatgctgaataaactgtgggttgtatgcctgcattttgactgaaactcattacataaggtcacatgtggaattttccatttttatcatgttggtgctcaaatactttcagattttggaggatttctgattttagattttccgattagggatgctcaacctgttcttctaaaagcttagctaactatatgggtcctcttcagtttaaaacatggattatgtgtccttcagcatgttccattccacctcacatgagtaatgctctgggaggtgtacaagcttatatttcacgctcttaagatctactgatcaaaaatctagcccgaaagtccatgagggcaaggattatgtcttatacctctttatagccctctttgtgcttggcattgttcattttaccctgaacttactcaataattgagggacagagcaggatttatacttaggatgctggacccagagtttatacctgggtcactgcccctaggctgggatggagccaggttttcaccagccagtctagacaaggaatgaagtctcatctgtagatacagtgaaacccctttgtcctaccataagctaattaatgaaatgaaactttttgaaaattaatagaatttagatgcaataccagaatttatagtataaataattaggataaaaacataactttttaactcacgaagtgcatatggtgtggcagagattgttcggcaagtttgctgcttcacttgtctttgtttcctaaagataaatttagtatcatgcaagaaatgcacattacatcctttcggtgcaataatatttcacataaatttgatttgcctgaagccaatactgtaaataaagcaaacatattctgtgtttcattttttaaaaagagtgatgaacgcagttcctgggcttatttaagcttcctgcgttttataactttttcagtgggatgaattagcatgatgtggtgaaacaggctggcagatgccagaggaaattaagacttcctgggcatacaagtaagagaactccacatatagcagagaaataagaacaatctgattttcaaagcagttgctaatcttatttctgctcatatctactctacatgtttctcctgatgtgaaacttttatgaagttccagttttagggttcactgaagaaaagactgccaataatcctgaaccctgccatattttatcaaagcttagacagacaaatggtcataaggaactgaaataaaaggaatttagtatctcagtggactgctgtaagtaggattcctaacccaaagaccaaatactgagaagtcaaacgtaaatatgtgtgtgtttgcatgtatgcgcatagacatatatgtgcatacgcatatatgtgtacgtggagagaggaagaaacgaagaagaaagaatgagagaggggtaggggagattcagagactaaattgggaagagtaaaagtagaagagtagcttcaaatagatttggtctgaaggctaatttgtgaaagtacaattagagaaagacaatgactgcaattataaacctcattatctttaacagttaagcaattgttaaaagacacaaaaagtaatttaagctttatgtgctatcaaccatgcaaaagttattaaattcatcatttgtacatatgtggaaatatagacatatgttaacatcttatatttaaggatatgttgagcaggtatgcattctatagtaaataaatatataatgaaaaatagatatagaaaccagtgattgaataacatgactttgtaaaccaagcaaaaggaaaaaacacctcctctctttctctagctgatattctcattgtcactgacaggttagtataatagtaaaaatgtcagcaattattttaaaccaagaagcaatacaatttcattttttctagccaagaaaataaatcactatatctaaaaatataattaaaaaatgattaaaattgatagctggtaatgctttttattcattaaaccattaaattctcactgtaaccccatttgattggaaaggaaagtaaggcttcaagatgttgagtaacttgtccagtcacaaagtaaatggtagatatgggatgtgaattcagtttcctgttgttccagagcaggagtagcaaaccctacagttaccctacagcaaattcattgggaaaatgggctctcattgtccagtcaaatgttttaaaagaataaagccttttagcagggcaggtatatatgctctgttgaccctattctgattcttgattactacatttaaaactacctcaaaatgtcgtggcataaaatctctactattttattgggctcacatttttatatgttaggaagtcaggaagtactcaggtggggggttcatctctaatccatctgctattaactggggtcagctggtgctgaaagattggcttccaacttggcttcttcatttgcaggtctggcacttttgttttccctgggctttctgtttctagcacagcctctcagcctccaagccctctccacatgggcttgggtgggagtagtcacacttattaaatggtggttagcttccaacagggaggaagtacaagtttccaggccagttaagggctgtgcctgttactggcagtatcagttctgcatactgtattggtcaaagcagtctggggctgctgtctcagattcaagtaggtggcaaagtaaactttacctcttgatggaagagttataacagctcaatgcagatgagagatgttgtgctcgtctttggaaaagacaatctgtcacaagccctgtaactccaaattgctttaaatctagtatcttcagatattgaaaatacttgccaaccacacaaggactagagtttatgtctatacagtagagcttatttttataactaccattaaatcatcttctcctaatcttaaatactaattatatacagataacaaaagaaagtcaacactgaaaataaatataaaacaaatatgcacaaaattacaagaag

SEQ ID NO: 17385 - RNA, 4712 nt, Homo sapiens
  source 1..4712: mol_type = other RNA
tcaggccaggcacagtggctcacgcctgtaatcccagctttgggaggccgaggtgggcggattacgagctcccatcctggctaacaaagtgaaaccctgtctctactaaaaatacaaaaaattggccaggcgtggtggcggagattagaatcccagctactcaggaggctgaggtaggagaatggcatgaacccaggaggcgaagcttgcagtgagccgagatggcgccactgcactccagcctgggcaacatagtgagactccatctcaaaaaaaaaaaaaaaaaaaaaaagatacagcatagtaaagaatctcaatattaatatgcatagtaaataacattttttctgtaaagtcataagcagacatggagaacatggagactaagaaatcaacctggtatttgaaatgtacaatgagtcttgaataatgaaaacagatttcaaaatttggagatctggtcaggatgctgtagacagaggggaatattctagcagatggcaagtataaattgaaatgtaatctcggcacctgaacttttgtggaatcacacattagctaaaactcaactataaaatctaattacatttcttttgaaaccttcttttaaaatgttgatcagttattaataatttaatatgtgtaactactaggaatagtaggtaaagactcagtgcagtaaaactcactataaagtgtgtgtggctcatctgttcagccatcacgctcaagaaaatgtgctcaagttcatttgtgactaactggcaaagttctcatcacaaaacaaaagctccaaactgaaaaatgttcttaactgtctcttaactggactcaattgcttctctgccatgaaatcttttttttttaagcaaaacattgcttaatcattttcttttattgttatgcttaagaataaaaacacataaaactgatcaatatggcaatcaagttaattcaataagacacttttttatttgtttaccacctgtaagtgccacagagactaccactacaggaaaagacaatagaggaggaagctctaaggtaaggtttgagttaattttctatatttaaagtttctttagaaaaatgtcctttggtttgtagacacagttcatataccattagttgaagctgtgcatagttatacagggcggaaatgtctcctttaaggttaacgtcgttttacacttacaatgtgacttctttatttgaaatgtggctagtttcatccagtctaaattggagatacgtatcattgtctctttttgcctcaggacagtactggaaatgagatgtttcatttcaatgcatttttctcagtggaaacacagttgagcaatcagaaagtcacttggttaagtagcagctttgggctggtcctcgtgcagtggtgtttacaactaattgatcataaccggttacagatttctttgatccttttccactcccactgctttatttgactagcctgtaagaaacgtattaaaatgtatcagaaggtgctccccatgagaaatctgctcctcagcatctttaaaaaacaatctgacaggtttggtcaccatctagttttggcaatatgagtggcatcaccagggataggagggaagttaattttaggtcaacataaagaagatatttctaatgattatgctatttttaaatggtattataatttcctcagctcactaaattgttaaagcagagattaaatgataaatttgaggaatagtttaggatgatgcatgtatcatgaaaaaaacaggttagaaattgagcaaatctatgctttttacccacttacggcttagttgcctcttacataaaaatgatcatagtaaggttatcgaaaggcagaggactacaacattcattttaagaaccatgactctttgacctcctctggtcaatgaattcgtctcatgaattaccatgaattaaacttagtttactttttcaactgatgttaatgataccacattccatggttgttatagattaaatgaagtactaacacttcatttgaaaatgaaaactgaaactattaaactaaagctaagtagaaagcccttagcccttcattgtaatttttttcatcatttaataacacaaactcactaaataaattgatttttgaaaataaaaataataaataggttattttaatttttatatcccttcacaccttacctgcttgtagcctccagctatacataatcttcatagctgtttgtattgttgttactgttgttcaggttagttcttattccagagaaggacagagggcattcagcttcctcttctttcaaataatactgggttctttagagttttcaagcaggtcatctttttcatccctttaatcactgtggttggtcttttgaagtgcatatggtgtggcagagattgttcggcaagtttgctgcttcacttgtctttgtttcctaaagataaatttagtatcatgcaagaaatgcacattacatcctttcggtgcaataatatttcacataaatttgatttgcctgaagccaatactgtaaataaagcaaacatattctgtgtttcattttttaaaaagagtgatgaacgcagttcctgggcttatttaagcttcctgcgttttataactttttcagtgggatgaattagcatgatgtggtgaaacaggctggcagatgccagaggaaattaagacttcctgggcatacaagtaagagaactccacatatagcagagaaataagaacaatctgattttcaaagcagttgctaatcttatttctgctcatatctactctacatgtttctcctgatgtgaaacttttatgaagttccagttttagggttcactgaagaaaagactgccaataatcctgaaccctgccatattttatcaaagcttagacagacaaatggtcataaggaactgaaataaaaggaatttagtatctcagtggactgctgtaagtaggattcctaacccaaagaccaaatactgagaagtcaaacgtaaatatgtgtgtgtttgcatgtatgcgcatagacatatatgtgcatacgcatatatgtgtacgtggagagaggaagaaacgaagaagaaagaatgagagaggggtaggggagattcagagactaaattgggaagagtaaaagtagaagagtagcttcaaatagatttggtctgaaggctaatttgtgaaagtacaattagagaaagacaatgactgcaattataaacctcattatctttaacagttaagcaattgttaaaagacacaaaaagtaatttaagctttatgtgctatcaaccatgcaaaagttattaaattcatcatttgtacatatgtggaaatatagacatatgttaacatcttatatttaaggatatgttgagcaggtatgcattctatagtaaataaatatataatgaaaaatagatatagaaaccagtgattgaataacatgactttgtaaaccaagcaaaaggaaaaaacacctcctctctttctctagctgatattctcattgtcactgacaggttagtataatagtaaaaatgtcagcaattattttaaaccaagaagcaatacaatttcattttttctagccaagaaaataaatcactatatctaaaaatataattaaaaaatgattaaaattgatagctggtaatgctttttattcattaaaccattaaattctcactgtaaccccatttgattggaaaggaaagtaaggcttcaagatgttgagtaacttgtccagtcacaaagtaaatggtagatatgggatgtgaattcagtttcctgttgttccagagcaggagtagcaaaccctacagttaccctacagcaaattcattgggaaaatgggctctcattgtccagtcaaatgttttaaaagaataaagccttttagcagggcaggtatatatgctctgttgaccctattctgattcttgattactacatttaaaactacctcaaaatgtcgtggcataaaatctctactattttattgggctcacatttttatatgttaggaagtcaggaagtactcaggtggggggttcatctctaatccatctgctattaactggggtcagctggtgctgaaagattggcttccaacttggcttcttcatttgcaggtctggcacttttgttttccctgggctttctgtttctagcacagcctctcagcctccaagccctctccacatgggcttgggtgggagtagtcacacttattaaatggtggttagcttccaacagggaggaagtacaagtttccaggccagttaagggctgtgcctgttactggcagtatcagttctgcatactgtattggtcaaagcagtctggggctgctgtctcagattcaagtaggtggcaaagtaaactttacctcttgatggaagagttataacagctcaatgcagatgagagatgttgtgctcgtctttggaaaagacaatctgtcacaagccctgtaactccaaattgctttaaatctagtatcttcagatattgaaaatacttgccaaccacacaaggactagagtttatgtctatacagtagagcttatttttataactaccattaaatcatcttctcctaatcttaaatactaattatatacagataacaaaagaaagtcaacactgaaaataaatataaaacaaatatgcacaaaattacaagaag

SEQ ID NO: 17386 - RNA, 2479 nt, Homo sapiens
  source 1..2479: mol_type = other RNA
tcaggccaggcacagtggctcacgcctgtaatcccagctttgggaggccgaggtgggcggattacgagctcccatcctggctaacaaagtgaaaccctgtctctactaaaaatacaaaaaattggccaggcgtggtggcggagattagaatcccagctactcaggaggctgaggtaggagaatggcatgaacccaggaggcgaagcttgcagtgagccgagatggcgccactgcactccagcctgggcaacatagtgagactccatctcaaaaaaaaaaaaaaaaaaaaaaagatacagcatagtaaagaatctcaatattaatatgcatagtaaataacattttttctgtaaagtcataagcagacatggagaacatggagactaagaaatcaacctggtatttgaaatgtacaatgagtcttgaataatgaaaacagatttcaaaatttggagatctggtcaggatgctgtagacagaggggaatattctagcagatggcaagtataaattgaaatgtaatctcggcacctgaacttttgtggaatcacacattagctaaaactcaactataaaatctaattacatttcttttgaaaccttcttttaaaatgttgatcagttattaataatttaatatgtgtaactactaggaatagtaggtaaagactcagtgcagtaaaactcactataaagtgtgtgtggctcatctgttcagccatcacgctcaagaaaatgtgctcaagttcatttgtgactaactggcaaagttctcatcacaaaacaaaagctccaaactgaaaaatgttcttaactgtctcttaactggactcaattgcttctctgccatgaaatcttttttttttaagcaaaacattgcttaatcattttcttttattgttatgcttaagaataaaaacacataaaactgatcaatatggcaatcaagttaattcaataagacacttttttatttgtttaccacctgtaagtgccacagagactaccactacaggaaaagacaatagaggaggaagctctaaggtaaggtttgagttaattttctatatttaaagtttctttagaaaaatgtcctttggtttgtagacacagttcatataccattagttgaagctgtgcatagttatacagggcggaaatgtctcctttaaggttaacgtcgttttacacttacaatgtgacttctttatttgaaatgtggctagtttcatccagtctaaattggagatacgtatcattgtctctttttgcctcaggacagtactggaaatgagatgtttcatttcaatgcatttttctcagtggaaacacagttgagcaatcagaaagtcacttggttaagtagcagctttgggctggtcctcgtgcagtggtgtttacaactaattgatcataaccggttacagatttctttgatccttttccactcccactgctttatttgactagcctgtaagaaacgtattaaaatgtatcagaaggtgctccccatgagaaatctgctcctcagcatctttaaaaaacaatctgacaggtttggtcaccatctagttttggcaatatgagtggcatcaccagggataggagggaagttaattttaggtcaacataaagaagatatttctaatgattatgctatttttaaatggtattataatttcctcagctcactaaattgttaaagcagagattaaatgataaatttgaggaatagtttaggatgatgcatgtatcatgaaaaaaacaggttagaaattgagcaaatctatgctttttacccacttacggcttagttgcctcttacataaaaatgatcatagtaaggttatcgaaaggcagaggactacaacattcattttaagaaccatgactctttgacctcctctggtcaatgaattcgtctcatgaattaccatgaattaaacttagtttactttttcaactgatgttaatgataccacattccatggttgttatagattaaatgaagtactaacacttcatttgaaaatgaaaactgaaactattaaactaaagctaagtagaaagcccttagcccttcattgtaatttttttcatcatttaataacacaaactcactaaataaattgatttttgaaaataaaaataataaataggttattttaatttttatatcccttcacaccttacctgcttgtagcctccagctatacataatcttcatagctgtttgtattgttgttactgttgttcaggttagttcttattccagagaaggacagagggcattcagcttcctcttctttcaaataatactgggttctttagagttttcaagcaggtcatctttttcatccctttaatcactgtggttggtcttttgaagtgcatatggtgtggcagagattgttcggcaagtttgctgcttcacttgtctttgtttcctgtattcccattactttgggaagctgagcag

SEQ ID NO: 17387 - RNA, 5563 nt, Homo sapiens
  source 1..5563: mol_type = other RNA
tcaggccaggcacagtggctcacgcctgtaatcccagctttgggaggccgaggtgggcggattacgagctcccatcctggctaacaaagtgaaaccctgtctctactaaaaatacaaaaaattggccaggcgtggtggcggagattagaatcccagctactcaggaggctgaggtaggagaatggcatgaacccaggaggcgaagcttgcagtgagccgagatggcgccactgcactccagcctgggcaacatagtgagactccatctcaaaaaaaaaaaaaaaaaaaaaaagatacagcatagtaaagaatctcaatattaatatgcatagtaaataacattttttctgtaaagtcataagcagacatggagaacatggagactaagaaatcaacctggtatttgaaatgtacaatgagtcttgaataatgaaaacagatttcaaaatttggagatctggtcaggatgctgtagacagaggggaatattctagcagatggcaagtataaattgaaatgtaatctcggcacctgaacttttgtggaatcacacattagctaaaactcaactataaaatctaattacatttcttttgaaaccttcttttaaaatgttgatcagttattaataatttaatatgtgtaactactaggaatagtaggtaaagactcagtgcagtaaaactcactataaagtgtgtgtggctcatctgttcagccatcacgctcaagaaaatgtgctcaagttcatttgtgactaactggcaaagttctcatcacaaaacaaaagctccaaactgaaaaatgttcttaactgtctcttaactggactcaattgcttctctgccatgaaatcttttttttttaagcaaaacattgcttaatcattttcttttattgttatgcttaagaataaaaacacataaaactgatcaatatggcaatcaagttaattcaataagacacttttttatttgtttaccacctgtaagtgccacagagactaccactacaggaaaagacaatagaggaggaagctctaaggtaaggtttgagttaattttctatatttaaagtttctttagaaaaatgtcctttggtttgtagacacagttcatataccattagttgaagctgtgcatagttatacagggcggaaatgtctcctttaaggttaacgtcgttttacacttacaatgtgacttctttatttgaaatgtggctagtttcatccagtctaaattggagatacgtatcattgtctctttttgcctcaggacagtactggaaatgagatgtttcatttcaatgcatttttctcagtggaaacacagttgagcaatcagaaagtcacttggttaagtagcagctttgggctggtcctcgtgcagtggtgtttacaactaattgatcataaccggttacagatttctttgatccttttccactcccactgctttatttgactagcctgtaagaaacgtattaaaatgtatcagaaggtgctccccatgagaaatctgctcctcagcatctttaaaaaacaatctgacaggtttggtcaccatctgcttgtagcctccagctatacataatcttcatagctgtttgtattgttgttactgttgttcaggttagttcttattccagagaaggacagagggcattcagcttcctcttctttcaaataatactgggttctttagagttttcaagcaggtcatctttttcatccctttaatcactgtggttggtcttttctgaaaaaaacagtttttccacatccttctcaggtaattttcatgactttacaatggcttgtgtttaatggcagagtgagccaaaggatcagagatttatttggctcttattagcttgtattacaatagtgagagaatgttctggcttatagacaaggaggaagcaataaatatagcatgtcttaccttcaggaaaggttttgattctattatgagtaccattttactcagcaagccagaaagttaatcatcttcattacataacaaacgggggttcatggaacctcacccttctaattcttataatgctgaaccaaataaagtggcccttgtactcacttgtatacctttgagggggcaggggcaatctagttgatgtcctattttgatgctctcctgcagcctattaggtcctgagttcctctggcttatcagtcaatgaaccagggttcacttttccagactgtacctttctgttactcttccttatactagtataacatttttatagggttgatataagctttgctcataaaaatacgggaagaaaaatcagagaatataacaaatggagacattttaaaatcacagagaattagtgttctcactgtccctggaaattcactcactgatttaagttcctaagttaattatcataagttttagttgctatcttgatctgcacctaaaacactcccctttggtatcattaatgttccaagatcagctactgagaagcaacataggtgaggtattgaataggaaaacaggctgggagggtcttttttctcctgggaatgctgaataaactgtgggttgtatgcctgcattttgactgaaactcattacataaggtcacatgtggaattttccatttttatcatgttggtgctcaaatactttcagattttggaggatttctgattttagattttccgattagggatgctcaacctgttcttctaaaagcttagctaactatatgggtcctcttcagtttaaaacatggattatgtgtccttcagcatgttccattccacctcacatgagtaatgctctgggaggtgtacaagcttatatttcacgctcttaagatctactgatcaaaaatctagcccgaaagtccatgagggcaaggattatgtcttatacctctttatagccctctttgtgcttggcattgttcattttaccctgaacttactcaataattgagggacagagcaggatttatacttaggatgctggacccagagtttatacctgggtcactgcccctaggctgggatggagccaggttttcaccagccagtctagacaaggaatgaagtctcatctgtagatacagtgaaacccctttgtcctaccataagctaattaatgaaatgaaactttttgaaaattaatagaatttagatgcaataccagaatttatagtataaataattaggataaaaacataactttttaactcacgaagtgcatatggtgtggcagagattgttcggcaagtttgctgcttcacttgtctttgtttcctaaagataaatttagtatcatgcaagaaatgcacattacatcctttcggtgcaataatatttcacataaatttgatttgcctgaagccaatactgtaaataaagcaaacatattctgtgtttcattttttaaaaagagtgatgaacgcagttcctgggcttatttaagcttcctgcgttttataactttttcagtgggatgaattagcatgatgtggtgaaacaggctggcagatgccagaggaaattaagacttcctgggcatacaagtaagagaactccacatatagcagagaaataagaacaatctgattttcaaagcagttgctaatcttatttctgctcatatctactctacatgtttctcctgatgtgaaacttttatgaagttccagttttagggttcactgaagaaaagactgccaataatcctgaaccctgccatattttatcaaagcttagacagacaaatggtcataaggaactgaaataaaaggaatttagtatctcagtggactgctgtaagtaggattcctaacccaaagaccaaatactgagaagtcaaacgtaaatatgtgtgtgtttgcatgtatgcgcatagacatatatgtgcatacgcatatatgtgtacgtggagagaggaagaaacgaagaagaaagaatgagagaggggtaggggagattcagagactaaattgggaagagtaaaagtagaagagtagcttcaaatagatttggtctgaaggctaatttgtgaaagtacaattagagaaagacaatgactgcaattataaacctcattatctttaacagttaagcaattgttaaaagacacaaaaagtaatttaagctttatgtgctatcaaccatgcaaaagttattaaattcatcatttgtacatatgtggaaatatagacatatgttaacatcttatatttaaggatatgttgagcaggtatgcattctatagtaaataaatatataatgaaaaatagatatagaaaccagtgattgaataacatgactttgtaaaccaagcaaaaggaaaaaacacctcctctctttctctagctgatattctcattgtcactgacaggttagtataatagtaaaaatgtcagcaattattttaaaccaagaagcaatacaatttcattttttctagccaagaaaataaatcactatatctaaaaatataattaaaaaatgattaaaattgatagctggtaatgctttttattcattaaaccattaaattctcactgtaaccccatttgattggaaaggaaagtaaggcttcaagatgttgagtaacttgtccagtcacaaagtaaatggtagatatgggatgtgaattcagtttcctgttgttccagagcaggagtagcaaaccctacagttaccctacagcaaattcattgggaaaatgggctctcattgtccagtcaaatgttttaaaagaataaagccttttagcagggcaggtatatatgctctgttgaccctattctgattcttgattactacatttaaaactacctcaaaatgtcgtggcataaaatctctactattttattgggctcacatttttatatgttaggaagtcaggaagtactcaggtggggggttcatctctaatccatctgctattaactggggtcagctggtgctgaaagattggcttccaacttggcttcttcatttgcaggtctggcacttttgttttccctgggctttctgtttctagcacagcctctcagcctccaagccctctccacatgggcttgggtgggagtagtcacacttattaaatggtggttagcttccaacagggaggaagtacaagtttccaggccagttaagggctgtgcctgttactggcagtatcagttctgcatactgtattggtcaaagcagtctggggctgctgtctcagattcaagtaggtggcaaagtaaactttacctcttgatggaagagttataacagctcaatgcagatgagagatgttgtgctcgtctttggaaaagacaatctgtcacaagccctgtaactccaaattgctttaaatctagtatcttcagatattgaaaatacttgccaaccacacaaggactagagtttatgtctatacagtagagcttatttttataactaccattaaatcatcttctcctaatcttaaatactaattatatacagataacaaaagaaagtcaacactgaaaataaatataaaacaaatatgcacaaaattacaagaag

SEQ ID NO: 17388 - RNA, 1639 nt, Homo sapiens
  source 1..1639: mol_type = other RNA
tcaggccaggcacagtggctcacgcctgtaatcccagtactttgggaggccaaggcgggtggatcacgacgtcaggagtccaagaccagcttgacatggtgaaaccctgtctctactaaaaatacaaaaattagccgagcgtggtgacacacgcctgtaatcccagctactcaggaggcaaggcaggagaattgcttgaaccagggaggcggaggttgcagtgagcccagatcgcgctattgcactccagcctggacaagagagcgagactctgactccaaaaaaaaaaaaaagaaagaaaactcattctatttttctctttggagcagaggttgcaaaactgtgatgcctaacaaaaacgttgtgtataaaagctccaaaaccaagcattagcctaaattggctataactgcaacttaaatcaaaaactatatccaactagatcttcgttgtggctatgcaactttttgctttgtggcctgaaggtttttactgaggtaacaacctcttatctcttgtccttccctcaaccacaaaagcaaaaataaacaacaacaaaaaacacctctacagcttccttcttcatggctgtctttggcaatgcttccaaatcttgaaagcaaaagaacctgctgaagtatatgaggaggatgaaaacactaaacatgacatatgaaaaccaatctaagcgtatgaattgagaaagaaaatactagaaggaaggcagagcagcagtcggccctcaacagaaaacaaaaaagaaggagggctgtaactgctctggcccttcttccatattatctcccaattagaagagcgtggaaccgaaaacttaaactctgaaaaggtaataactttcaaggaggagctacggaagtgaataaatgataaagaagaacagcagtagctttagctgtcaatgagtttctttgctctggcattggcaatatcaatacgatctctgttggtgtcagccttgtctgtgattcgttttatttgtggattttgagcatcaatctcattgcctatgttcagggccatgtcttttagatttcccaggatactgcccacttgagtcaggttctcttccatttcatcttctctggcatcattagttatgcgtttaatgtatccaccactggctgctcccgttgttggttgctgaagctgaccatttgtcaccgggcctggctgtttagatactacattgcaaggtgagttttctccaccatctccccatgttgtcttataagccttgccagactcaaagttctttgttctattacatgggcagacacaaaggccacagcatttgttgagttctgttaaagtcttctctgtctctctcatgtccttatttatttggtccaagccttcttctatgcggtttagttgttccttttgttcatccagcatagtgatggtcttgattcctgcatcctgagactcaatggctaaacccaggattctcctcgtactttccagagactcatcagtaatctggtgagctctctgttgaatttcttctgatgacagattatccatgatgaatcaaaactcaagcgggcgaggccactcctctccggcggcaactcggacaccccaacaccggacctggcgctgcaccctagtcgcgcct

SEQ ID NO: 17389 - RNA, 2000 nt, Homo sapiens
  source 1..2000: mol_type = other RNA
tcaggccaggcacagtggctcacgcctgtaatcccagtactttgggaggccaaggcgggtggatcacgacgtcaggagtccaagaccagcttgacatggtgaaaccctgtctctactaaaaatacaaaaattagccgagcgtggtgacacacgcctgtaatcccagctactcaggaggcaaggcaggagaattgcttgaaccagggaggcggaggttgcagtgagcccagatcgcgctattgcactccagcctggacaagagagcgagactctgactccaaaaaaaaaaaaaagaaagaaaactcattctatttttctctttggagcagaggttgcaaaactgtgatgcctaacaaaaacgttgtgtataaaagctccaaaaccaagcattagcctaaattggctataactgcaacttaaatcaaaaactatatccaactagatcttcgttgtggctatgcaactttttgctttgtggcctgaaggtttttactgaggtaacaacctcttatctcttgtccttccctcaaccacaaaagcaaaaataaacaacaacaaaaaacacctctacagcttccttcttcatggctgtctttggcaatgcttccaaatcttgaaagcaaaagaacctgctgaagtatatgaggaggatgaaaacactaaacatgacatatgaaaaccaatctaagcgtatgaattgagaaagaaaatactagaaggaaggcagagcagcagtcggccctcaacagaaaacaaaaaagaaggagggctgtaactgctctggcccttcttccatattatctcccaattagaagagcgtggaaccgaaaacttaaactctgaaaaggtaataactttcaaggaggagctacggaagtgaataaatgataaagaagaacagcagtagctttagctgtcaatgagtttctttgctctggcattggcaatatcaatacgatctctgttggtgtcagccttgtctgtgattcgttttatttgtggattttgagcatcaatctcattgcctatgttcagggccatgtcttttagatttcccaggatactgcccacttgagtcaggttctcttccatttcatcttctctggcatcattagttatgcgtttaatgtatccaccactggctgctcccgttgttggttgctgaagctgaccatttgtcaccgggcctggctgtttagatactacattgcaaggtgagttttctccaccatctccccatgttgtcttataagccttgccagactcaaagttctttgttctggtttcatagaaacaaccaacatctgagaatctattacatgggcagacacaaaggccacagcatttgttgagttctgttaaagtcttctctgtctctctcatgtccttatttatttggtccaagccttcttctatgcggtttagttgttccttttgttcatccagcatagtgatggtcttgattcctgcatcctgagactcaatggctaaacccaggattctcctcgtactttccagagactcatcagtaatctggtgagctctctgttgaatttcttctgatgacagattatccatgatgaatcaaaactcaagcgggcgaggccactcctctccggcggcaactcggacaccccaacaccggacctggcgctgcaccctagtcgcgcctgcgcgcgccgagcccgcgcgcctgctcacttcccgttcgccgcggacacagacacacccctgcagctggagccaatcacggtgctgggggtttaaatgtccctgccacgcagacggagagtctgggaattcactagttaaccggatagatttcagtcctgcccgaagctgggaggtgttcatgcaataaacatttactgagggcaaaccgtatgccaggcactgtgctggatgaacgctgaagaaaagaaagcgaatacagtgctttccctgctcttcatcgcctttcaatatgtctagactaagatatagatatgtaaacaaattat

SEQ ID NO: 17390 - RNA, 1480 nt, Homo sapiens
  source 1..1480: mol_type = other RNA
tcaggccaggcacagtggctcacgcctgtaatcccagtactttgggaggccaaggcgggtggatcacgacgtcaggagtccaagaccagcttgacatggtgaaaccctgtctctactaaaaatacaaaaattagccgagcgtggtgacacacgcctgtaatcccagctactcaggaggcaaggcaggagaattgcttgaaccagggaggcggaggttgcagtgagcccagatcgcgctattgcactccagcctggacaagagagcgagactctgactccaaaaaaaaaaaaaagaaagaaaactcattctatttttctctttggagcagaggttgcaaaactgtgatgcctaacaaaaacgttgtgtataaaagctccaaaaccaagcattagcctaaattggctataactgcaacttaaatcaaaaactatatccaactagatcttcgttgtggctatgcaactttttgctttgtggcctgaaggtttttactgaggtaacaacctcttatctcttgtccttccctcaaccacaaaagcaaaaataaacaacaacaaaaaacacctctacagcttccttcttcatggctgtctttggcaatgcttccaaatcttgaaagcaaaagaacctgctgaagtatatgaggaggatgaaaacactaaacatgacatatgaaaaccaatctaagcgtatgaattgagaaagaaaatactagaaggaaggcagagcagcagtcggccctcaacagaaaacaaaaaagaaggagggctgtaactgctctggcccttcttccatattatctcccaattagaagagcgtggaaccgaaaacttaaactctgaaaaggtaataactttcaaggaggagctacggaagtgaataaatgataaagaagaacagcagtagctttagctgtcaatgagtttctttgctctggcattggcaatatcaatacgatctctgttggtgtcagccttgtctgtgattcgttttatttgtggattttgagcatcaatctcattgcctatgttcagggccatgtcttttagatttcccaggatactgcccacttgagtcaggttctcttccatttcatcttctctggcatcattagttatgctattacatgggcagacacaaaggccacagcatttgttgagttctgttaaagtcttctctgtctctctcatgtccttatttatttggtccaagccttcttctatgcggtttagttgttccttttgttcatccagcatagtgatggtcttgattcctgcatcctgagactcaatggctaaacccaggattctcctcgtactttccagagactcatcagtaatctggtgagctctctgttgaatttcttctgatgacagattatccatgatgaatcaaaactcaagcgggcgaggccactcctctccggcggcaactcggacaccccaacaccggacctggcgctgcaccctagtcgcgcct

SEQ ID NO: 17391 - RNA, 34 nt, Homo sapiens
  source 1..34: mol_type = other RNA
tcaggccaggcacagtggctcacgcctgtaatct

SEQ ID NO: 17392 - RNA, 6007 nt, Homo sapiens
  source 1..6007: mol_type = other RNA
tcaggccaggcacagtggctcacgcctgtaatctcagcactttgggaggccaaggtgggcagatcgttggagcccaggagtttgagatcagcctgagcaacatggcgaaaccccatttctacaaaatacaaaaaaaattagctaggcattgtggtgcacaactgtagtcccagctacttgggaggctgagatgggaggatcacttgaatctggagaggttgaggctgcagtgaactgtgattgtgccactgcactccagcctgggtgacagagcaagaccctgtctcaaaaaaagaaaaagaacttcacataaaagatggtacctgtactattatttgcaacgtacttagttgttttaagatttatcagcaaataaagaagcagtcgtagtgagggaaaagtgtatttcacagtcattacaaaagtacatatatctaataatggtgacataaatatagtccttacttatgaccaaatcatacaattaaaatggacatttcctcctagacttcacacaatgacagtccagtcaatttctgtcagtaactacagggtgactggaatcacaggcacagactgaggaagacagtcacggtcgaacagacaacatgcttcggacttaccaaagggagagtcgagctttccatataaatataataaaataataaagaatctaacatttctcctttcactcggtttcatagatttgtcaggtgctcacacacacacacacacacaaatacagctgatcccctttcatcactccccctcacctctcactgggtttagaataaacctgagttcagagtccaggtcgccaatggcaacgcggtcagttagcggcacatgtgcagctgttcttgaagcctgccaggaataagaagcacgttctccacaagctaacggcaaggcggaagtacccctgctctcaaggaaaatgcatcaggggttccagcaagttcccaatgcgcaggtatacaccctgcaagcctgcaaagtggagccgttgcagctggaaaccgtctttagaaaaggtacacttcatgtcgaatggagagatggtcttagatgattattttcttctctctgcttataaagctctattttctttttttggagacagggtctcactttgccacctaagctggagtgcagtagcatgatcttggctcactgcagcctcgacctcctaggttcaagtgatcctcccacctcagtccccgaagtagctgggactacaggcacgtaccaccacacccagctatttttttttgtatttttcggtagagacgggctttcaccatgttgcccaggctgctctcgaactcctgagctcaagcgatccacctgcctcggcctcccaaagtgctgggattacaggtgtgagccaccacacctggcctaaaagctctgttttcaatggtaagttctggaacccagtctgaagctatacaaaaaataacaccaatggccaaggggtctgacctcatcctagaatgccctagagccgtggtgatcccctagggaagaaacaggcagctccaggtctcaccaaggtcagccaaatatccattctgtcccgctctgtcagagatgtgagggactgaaggatgtcaccactggtgaatgagagaatgattcagaactgcctctctgccttctggcaaggctgcctgccagggaaataaaggctggctttgcaattctagatttgtgttttgggatccttggactgagatgactatctgaggtggccacagaggtggtctctggtcacacctgcaccggtcaaaagttgaagactccaggccattctgtaactggtctcctacactaacccctatccaacctgtgctgatgggtcttctttttctgattcttctcaccaatgactgcaccctgtcaagtgccagctggatacagtcagacaacacggctgtccacaaaacacacacaggggcacagacacaatactggagacacatctttggttcgatccttggagaaaggtgtgaaaacacaacgtggactgaaccctgtttgaggagcttggctttcctcgaagaagaaactggcctgtatctgaacaggttctctgccaggcaagcctgctcccagctcccagcaaactcgccgagctctgagccgcaccagttctgtgggcagcttgaaatcagcatcgcacagagataatgctgccttctcgccatctgagttatgctctgaattgtcacaatcatcttttccctctttctacagaaccagctgtaaccgtgttctatgccttccagaaggatcagggctatgccttaaacaacaggatgaacacagggccaccgagacttgccctgcctgtgggccacagcactcagcaaatcaccacagtcagcttttttgctctccacactgaaccctcctgtgaaaacatgagtttggtggaattgcttctcatctctccatccaagttttaaaaaattatgttatttcaatttaccgacatcacatttaaaaaaaatctttggaaaagataattcaatcattagcatgtttcaacaacaacaacaacaaaaatctatcaaaatcttgcttgggaaatgagtgtctccttcagtctttctcttctgttggggtccccactgtttggtttgatcttggtccgaagctcctctccatcttcctctgaggatcctgggcctgcccccggctcctgctggccttcaggtaatccctgctatgaaaggcagggctgctacactccgcagaggaaacgtggcctggatgaatgactgtgatattgttctctccctgtaactgtggccaactgctgtgagaggcacacatgtagcacagcgtgaagaaagatctggtaacagtccataatctgagtgccccagaaggctcatgccctgttttccccccaagcctgggggaagtgggaagtggaaggggttggtgagtacttgggaggaaggaagatctgaatgataggaattggctgcccctggagccaaccctcctagcgattccagcatctctgggggtccctaagcgaggttgggttgtgcaggctttgggtctgtggattcagctacaggtgggactaaggatgctccacgcgaggccttggagtgctcacaccctgacagatgtgtggagctctgttcagttgctgttttctagagataccccaaaccccgctggcccaagttagcactgggtcttgaccccatcggccatgtcaaaggcaaggttcacaggggctaggggctgcagtgggggcaggctggcctccaggggcctatctgcagatggctgcagactctgatggcgcttccttaacatctgtccgatgcccatcatagggaaccggcctcggcttttcacacaattggggctccccagaggctgcatggggccattgctgggaaccggaggtgggcaacacaggccctcctcttttggggggctgttcttatcttcgtgagcaaaagagaccagagttggatgcaaaggagtatggagaggcgacatgcttccggatggcagacccggggacagcgtcctctcgctggaatttctgcgagccaagctgaccggggagttcagaatcctgtagtgatgagagggagacagcacttctacgtggtcgtcgcgatccacagactcgaaggagcgcaccatgtccagcatcagggggtcttccttgtgggggatgccagtgcttccgggccctggctgatggggctccggtttcttcacaatcctcggggtcctgggcggtggcacggggatgaactccatggaagaagaagccacacaattggaatctgaggttttgcggaaaatattgcggcagccaaaggaatctttgtcggggaagctggacttggaggccttccggtccttcaggagggctttggtgttctgaatctgtgtcataagcgagcctgagggctgtttgtgcgagggcaggttcttgtccaacttcttggagaatggtcgatgaagaaaatcccctcttttttcttgttctttgggctttttatcctgcacggcatggaattcaagatctcgtgtccaggtgtccagagaggcctcataggactccttgggggccctgtacttttctatctggtagagccgggtcttgtagcagaggctgtcctggatgtcagatttccctgacaaatagcgctccagtttcttgtttaagaggaagtagatggccaggatgtggcaggcgcggttggagagcacagtgttgatcacgtcgctgttcttgtaacccagcttctcggtcatgtgcagcacgacgctcgggctcagatcttccagagaaatcctgttgggataggtgacattacagggcactttgcccgtgtaattctcattaagccagcgattcgccagtgcctgctgaatatttggcctcttcacaggatccggttccaggagagagcgcaggaaactgatggcacctgtggagagctgagtggggagggggttcatttctttgtctaccatcttctggtacaaagccctcaggctgaaaggctccaccgtgaaaggcagcgtcccggtcaacatggcatacatgttcacacctatggaccagacatcgattttggggccgtatttcttcctggcgagcagttcaggtgcagcgtaggcagggctgccacactgtgtgctgaacggatccgagtaacccaggatccctgcgcagttgctcaaaccaaagtcaatcagcttgatattattgtcttcatctagtagcaaattctctatcttcaagtctctgtggaccaccccggcccggtgcaggtgctctacggcagagatgagctgtcggatgtatctgcgggcttcggactcctccagccgcttcttctcatagatcttgtgcatcaggttgcccccagggcacagctccatgaccaggtagtagctgttttccgtttctaaaatatcaaggagctgagtgatattggggtggcggatcatctgctggatctgaccctctcgccgcaggtttttggtgacataggtgtcctttttggctctcttcttatcaatgacttttatggccaccttctccccggtcagcacgtgcagcccctcgcgcaccttggcaaaggagccctcgcccagcttcctgctgccgatgaggtagttgcccacgcgcttgtggtgctggaagtcgcggagccgctcgcggggcacgccgctcacccaggcaggcaggaaacttccctcgcaggccgccgcgggcctggccgcgtcctccgcgccgccgccgcccccaggcgccgccggctcccccaggagcccgtcccccgccgccgccggcatcgcgctcgccgcggcccgcgcggctcctgctcgtctcccgcgctcgcagctcctcctccccaggctcttcggcttccccggcttctcccgccgccgccctgggcccagccccgcctgggtctccgcacccagagcccggggccgccgcgatcacgccccccgcgccgcccagcgaggcgcgtagacaatagcggctgcccaggggacgcgggaccggggaccccgcccccaaaagttcttcctcttagggtcgcccgggcccctttcaggacaccaggatcccgccccgggtcccgtccaggaagctaatgacagtcgccctgctcgggcgcgcggggtggggcgcggtccggcggcgcctgggtcccggggtccgggtgcctgggtccgggagcccgggtgcctccgcagcctccgcctcgccgccgccgtctggcccgcacgggcttgggtcgggctcccgcgatcgctcctagccgtgcgctgggcggccgctcccgccggagagaagcgcgcggcgggctgccggcgccctctggaaggcagcagaagaaagccccattcagtttgaatttgcagaaatttaatccgctcgcgggcggcgggaacagatgcgagctccactccgcagcccgtgcactttcaaatccctagt

SEQ ID NO: 17393 - RNA, 2812 nt, Homo sapiens
  source 1..2812: mol_type = other RNA
tcaggccaggcacagtggctcacgcctgtaattccagcactttgggagaccgcagtgggcggatcacgaggtcaggagttggagaccagcccggccaacatagtgaaaccctgtctctactaaaactacaaaaattggccaggcatagtggcatgtgcctgtagtcccagctacctgggaggctgaggcagaagaattgcttgaatccaggaggcagaggttttagtgagccgagattatgccactgcactccagcttgggtgacagagtgagacttcacctcaaaaaaaaaaataaataaataaaagaaaagaaaaaacaatcctgaaactcatatggaaccgcaaaaaaccccaaacagccaacagataactgtgaaagaaaaagttggaggcatcacacctcttgatttaaaattgtattacaaagctatagtaatcaaaacagtatggtgctggcataaaaacaaaaaaatagaccaatggaacagaacagagacctttgaaataaatccaaacatatactgtcaactaatttttgacaagggcaaacaagacaacacaatggtaaaaaagatagtttcttcaataataggattttcacatgcaaaagaataaaattcgaccctgatcatacaccatacacaaaaatcaactcaaaacagatacaagaccaaagacccaaataagacctgaaaccataaaactcctagaagaaaacatagggggaaagcctcttgacattggccttagcaataattttttggatatcgcaccacaagccaggctacaaatgtaaacataaacaaggaggactgcatcaaactaaaaagcttctgcacagcaaaggaacaaccaacaaaatgaaaggggaacctatagactggaagaaatatttgcaaaccacatatctgataaagtgttaatatccaaaaatcagtaaagaactcttacaacttaatagcagaaaaacaacccagttgaaaaatgggccaaataggaaatgaccagtaggaaatggggagatgtacattaaaataatacaaagtagcagacatgtaggatgaacaagttagagatctagtgtacatcatgagggctatagttaataaaaatatattgtctttgggatttttgttaaataagtagattttagctgttcctgtcacacaaacaaaaatctaactatgtgagatggtagctatgttaatttgcttcactatagtaaccagtttactatctatatttatcctttaagatcatgttgtcaacctcaaatatataaaataaaatttattttaaaaaagaaaagtttgtcttcaatccagaaagaaccactattaccattttttggtgttccattccaaaatatcccacaaatatacaattgttcaatcaaatttaacattagactttatacttgaacattcaaagtacgtaagaaattatagaaaagtgtctgcgtgactccctgtctgtagggcacaggcttcatctccactaacacacacacgaccagtaccttatacagagagtccttgtttgtctttagtctgacaccatgggcgagcccgaggtggcccgtggtccacattcctgaccaggtgtctttctcacccactggtttcaacaaagatgttactgggttatagaaggctgggatggaaacaggataccaagttcgcatgaagacaatatcgctcatccacagcttatcctcaaagctagcctggaaagctccttctggagctcagagtgctctcttgatctgcccccttatcccactgacagttcgaatcacagcatcttcaaatttggccacttccaaggcagaattaaacattcccttaataaatgaagtgttcttgaaaattttatatggaaaaccagttagctttaatttcttcacaatttttatggatttatccagatcaaggacaactcctgtggcagctatccgaaaatcaggcattatgccactgacagactgtattgccaagaaaccagttccctgtggagtgatagggtcccaaaaggctgctccacaatgcatgtgctgtggggtatactttagaagcctttgtcttccattgtggtcttcaatataatagagcaggatggtctgaaacctcctccaccctacagaaaatatgattggatcttgggacttgaggattttcttataccagcgatgtttcttcagacgcatctgcacgtgtccaacatttccctcgctgttgcccaagccacccaggataatggggtaatgggggtcaaagttctgcacaaattcacagggaacattttcaatctcaacgcggacgtacatcccaggtcgaaaaccatcatactgaactctggcttcatcatcttgatcttcaaattctacgtgattcagctcaaaaccttttgattccacttcttccaccaaaaactgcttcatttctctgcttctctctgtgcttctttctgcatttctcctttaagatcatcaaaatatgtgctttctccttcatcatattccgcatcaaacatctccttcaattttctcttcttatccaaatgctttttcttggcactttcttcttcgtcggggtcaatttcttccttgtttctctatatcttcattctgagtgtcggggcccgattttcccttgtgcatgtcccctgtttccaagtcttcaaagtcaccgtagagctcctcctttcacagctggggagtggacctgggcctgcgcctctccgcgccagcgcctgcgctgtgcgcctctccgcgcctgcgccgccgctgtgcgcctctccgccgctgtgcg

SEQ ID NO: 17394 - RNA, 2755 nt, Homo sapiens
  source 1..2755: mol_type = other RNA
tcaggccaggcacagtggctcacgcctgtaattccagcactttgggagaccgcagtgggcggatcacgaggtcaggagttggagaccagcccggccaacatagtgaaaccctgtctctactaaaactacaaaaattggccaggcatagtggcatgtgcctgtagtcccagctacctgggaggctgaggcagaagaattgcttgaatccaggaggcagaggttttagtgagccgagattatgccactgcactccagcttgggtgacagagtgagacttcacctcaaaaaaaaaaataaataaataaaagaaaagaaaaaacaatcctgaaactcatatggaaccgcaaaaaaccccaaacagccaacagataactgtgaaagaaaaagttggaggcatcacacctcttgatttaaaattgtattacaaagctatagtaatcaaaacagtatggtgctggcataaaaacaaaaaaatagaccaatggaacagaacagagacctttgaaataaatccaaacatatactgtcaactaatttttgacaagggcaaacaagacaacacaatggtaaaaaagatagtttcttcaataataggattttcacatgcaaaagaataaaattcgaccctgatcatacaccatacacaaaaatcaactcaaaacagatacaagaccaaagacccaaataagacctgaaaccataaaactcctagaagaaaacatagggggaaagcctcttgacattggccttagcaataattttttggatatcgcaccacaagccaggctacaaatgtaaacataaacaaggaggactgcatcaaactaaaaagcttctgcacagcaaaggaacaaccaacaaaatgaaaggggaacctatagactggaagaaatatttgcaaaccacatatctgataaagtgttaatatccaaaaatcagtaaagaactcttacaacttaatagcagaaaaacaacccagttgaaaaatgggccaaataggaaatgaccagtaggaaatggggagatgtacattaaaataatacaaagtagcagacatgtaggatgaacaagttagagatctagtgtacatcatgagggctatagttaataaaaatatattgtctttgggatttttgttaaataagtagattttagctgttcctgtcacacaaacaaaaatctaactatgtgagatggtagctatgttaatttgcttcactatagtaaccagtttactatctatatttatcctttaagatcatgttgtcaacctcaaatatataaaataaaatttattttaaaaaagaaaagtttgtcttcaatccagaaagaaccactattaccattttttggtgttccattccaaaatatcccacaaatatacaattgttcaatcaaatttaacattagactttatacttgaacattcaaagtacgtaagaaattatagaaaagtgtctgcgtgactccctgtctgtagggcacaggcttcatctccactaacacacacacgaccagtaccttatacagagagtccttgtttgtctttagtctgacaccatgggcgagcccgaggtggcccgtggtccacattcctgaccaggtgtctttctcacccactggtttcaacaaagatgttactgggttatagaaggctgggatggaaacaggataccaagttcgcatgaagacaatatcttaataaatgaagtgttcttgaaaattttatatggaaaaccagttagctttaatttcttcacaatttttatggatttatccagatcaaggacaactcctgtggcagctatccgaaaatcaggcattatgccactgacagactgtattgccaagaaaccagttccctgtggagtgatagggtcccaaaaggctgctccacaatgcatgtgctgtggggtatactttagaagcctttgtcttccattgtggtcttcaatataatagagcaggatggtctgaaacctcctccaccctacagaaaatatgattggatcttgggacttgaggattttcttataccagcgatgtttcttcagacgcatctgcacgtgtccaacatttccctcgctgttgcccaagccacccaggataatggggtaatgggggtcaaagttctgcacaaattcacagggaacattttcaatctcaacgcggacgtacatcccaggtcgaaaaccatcatactgaactctggcttcatcatcttgatcttcaaattctacgtgattcagcatcaactgtacacacgtttctgtgtctgtctccttcagagtgacatcactgtctccagcaacctgctcagcaaccccaggcaggagggccacaccatctccctttatctccgcatctgaccttatactccacgtgtccttctgaactctgaccaggatgagttttcagagcacttcccctgggagctctggtgtgtccataagccacacgggccactgatcacctgtgcttctttctgcatttctcctttaagatcatcaaaatatgtgctttctccttcatcatattccgcatcaaacatctccttcaattttctcttcttatccaaatgctttttcttggcactttcttcttcgtcggggtcaatttcttccttgtttctctatatcttcattcctttcacagctggggagtggacctgggcctgcgcctctccgcgccagcgcctgcgctgtgcgcctctccgcgcctgcgccgccgctgtgcgcctctccgccgctgtgcg

SEQ ID NO: 17395 - RNA, 2829 nt, Homo sapiens
  source 1..2829: mol_type = other RNA
tcaggccaggcacagtggctcacgcctgtaattccagcactttgggagaccgcagtgggcggatcacgaggtcaggagttggagaccagcccggccaacatagtgaaaccctgtctctactaaaactacaaaaattggccaggcatagtggcatgtgcctgtagtcccagctacctgggaggctgaggcagaagaattgcttgaatccaggaggcagaggttttagtgagccgagattatgccactgcactccagcttgggtgacagagtgagacttcacctcaaaaaaaaaaataaataaataaaagaaaagaaaaaacaatcctgaaactcatatggaaccgcaaaaaaccccaaacagccaacagataactgtgaaagaaaaagttggaggcatcacacctcttgatttaaaattgtattacaaagctatagtaatcaaaacagtatggtgctggcataaaaacaaaaaaatagaccaatggaacagaacagagacctttgaaataaatccaaacatatactgtcaactaatttttgacaagggcaaacaagacaacacaatggtaaaaaagatagtttcttcaataataggattttcacatgcaaaagaataaaattcgaccctgatcatacaccatacacaaaaatcaactcaaaacagatacaagaccaaagacccaaataagacctgaaaccataaaactcctagaagaaaacatagggggaaagcctcttgacattggccttagcaataattttttggatatcgcaccacaagccaggctacaaatgtaaacataaacaaggaggactgcatcaaactaaaaagcttctgcacagcaaaggaacaaccaacaaaatgaaaggggaacctatagactggaagaaatatttgcaaaccacatatctgataaagtgttaatatccaaaaatcagtaaagaactcttacaacttaatagcagaaaaacaacccagttgaaaaatgggccaaataggaaatgaccagtaggaaatggggagatgtacattaaaataatacaaagtagcagacatgtaggatgaacaagttagagatctagtgtacatcatgagggctatagttaataaaaatatattgtctttgggatttttgttaaataagtagattttagctgttcctgtcacacaaacaaaaatctaactatgtgagatggtagctatgttaatttgcttcactatagtaaccagtttactatctatatttatcctttaagatcatgttgtcaacctcaaatatataaaataaaatttattttaaaaaagaaaagtttgtcttcaatccagaaagaaccactattaccattttttggtgttccattccaaaatatcccacaaatatacaattgttcaatcaaatttaacattagactttatacttgaacattcaaagtacgtaagaaattatagaaaagtgtctgcgtgactccctgtctgtagggcacaggcttcatctccactaacacacacacgaccagtaccttatacagagagtccttgtttgtctttagtctgacaccatgggcgagcccgaggtggcccgtggtccacattcctgaccaggtgtctttctcacccactggtttcaacaaagatgttactgggttatagaaggctgggatggaaacaggataccaagttcgcatgaagacaatatcttaataaatgaagtgttcttgaaaattttatatggaaaaccagttagctttaatttcttcacaatttttatggatttatccagatcaaggacaactcctgtggcagctatccgaaaatcaggcattatgccactgacagactgtattgccaagaaaccagttccctgtggagtgatagggtcccaaaaggctgctccacaatgcatgtgctgtggggtatactttagaagcctttgtcttccattgtggtcttcaatataatagagcaggatggtctgaaacctcctccaccctacagaaaatatgattggatcttgggacttgaggattttcttataccagcgatgtttcttcagacgcatctgcacgtgtccaacatttccctcgctgttgcccaagccacccaggataatggggtaatgggggtcaaagttctgcacaaattcacagggaacattttcaatctcaacgcggacgtacatcccaggtcgaaaaccatcatactgaactctggcttcatcatcttgatcttcaaattctacgtgattcagcatcaactgtacacacgtttctgtgtctgtctccttcagagtgacatcactgtctccagcaacctgctcagcaaccccaggcaggagggccacaccatctccctttatctccgcatctgaccttatactccacgtgtccttctgaactctgaccaggatgagttttcagagcacttcccctgggagctctggtgtgtccataagccacacgggccactgatcacctgtgcttctttctgcatttctcctttaagatcatcaaaatatgtgctttctccttcatcatattccgcatcaaacatctccttcaattttctcttcttatccaaatgctttttcttggcactttcttcttcgtcggggtcaatttcttccttgtttctctatatcttcattctgagtgtcggggcccgattttcccttgtgcatgtcccctgtttccaagtcttcaaagtcaccgtagagctcctcctttcacagctggggagtggacctgggcctgcgcctctccgcgccagcgcctgcgctgtgcgcctctccgcgcctgcgccgccgctgtgcgcctctccgccgctgtgcg

SEQ ID NO: 17396 - RNA, 2531 nt, Homo sapiens
  source 1..2531: mol_type = other RNA
tcaggccaggcacagtggctcacgcctgtaattccagcactttgggagaccgcagtgggcggatcacgaggtcaggagttggagaccagcccggccaacatagtgaaaccctgtctctactaaaactacaaaaattggccaggcatagtggcatgtgcctgtagtcccagctacctgggaggctgaggcagaagaattgcttgaatccaggaggcagaggttttagtgagccgagattatgccactgcactccagcttgggtgacagagtgagacttcacctcaaaaaaaaaaataaataaataaaagaaaagaaaaaacaatcctgaaactcatatggaaccgcaaaaaaccccaaacagccaacagataactgtgaaagaaaaagttggaggcatcacacctcttgatttaaaattgtattacaaagctatagtaatcaaaacagtatggtgctggcataaaaacaaaaaaatagaccaatggaacagaacagagacctttgaaataaatccaaacatatactgtcaactaatttttgacaagggcaaacaagacaacacaatggtaaaaaagatagtttcttcaataataggattttcacatgcaaaagaataaaattcgaccctgatcatacaccatacacaaaaatcaactcaaaacagatacaagaccaaagacccaaataagacctgaaaccataaaactcctagaagaaaacatagggggaaagcctcttgacattggccttagcaataattttttggatatcgcaccacaagccaggctacaaatgtaaacataaacaaggaggactgcatcaaactaaaaagcttctgcacagcaaaggaacaaccaacaaaatgaaaggggaacctatagactggaagaaatatttgcaaaccacatatctgataaagtgttaatatccaaaaatcagtaaagaactcttacaacttaatagcagaaaaacaacccagttgaaaaatgggccaaataggaaatgaccagtaggaaatggggagatgtacattaaaataatacaaagtagcagacatgtaggatgaacaagttagagatctagtgtacatcatgagggctatagttaataaaaatatattgtctttgggatttttgttaaataagtagattttagctgttcctgtcacacaaacaaaaatctaactatgtgagatggtagctatgttaatttgcttcactatagtaaccagtttactatctatatttatcctttaagatcatgttgtcaacctcaaatatataaaataaaatttattttaaaaaagaaaagtttgtcttcaatccagaaagaaccactattaccattttttggtgttccattccaaaatatcccacaaatatacaattgttcaatcaaatttaacattagactttatacttgaacattcaaagtacgtaagaaattatagaaaagtgtctgcgtgactccctgtctgtagggcacaggcttcatctccactaacacacacacgaccagtaccttatacagagagtccttgtttgtctttagtctgacaccatgggcgagcccgaggtggcccgtggtccacattcctgaccaggtgtctttctcacccactggtttcaacaaagatgttactgggttatagaaggctgggatggaaacaggataccaagttcgcatgaagacaatatcttaataaatgaagtgttcttgaaaattttatatggaaaaccagttagctttaatttcttcacaatttttatggatttatccagatcaaggacaactcctgtggcagctatccgaaaatcaggcattatgccactgacagactgtattgccaagaaaccagttccctgtggagtgatagggtcccaaaaggctgctccacaatgcatgtgctgtggggtatactttagaagcctttgtcttccattgtggtcttcaatataatagagcaggatggtctgaaacctcctccaccctacagaaaatatgattggatcttgggacttgaggattttcttataccagcgatgtttcttcagacgcatctgcacgtgtccaacatttccctcgctgttgcccaagccacccaggataatggggtaatgggggtcaaagttctgcacaaattcacagggaacattttcaatctcaacgcggacgtacatcccaggtcgaaaaccatcatactgaactctggcttcatcatcttgatcttcaaattctacgtgattcagctgtgcttctttctgcatttctcctttaagatcatcaaaatatgtgctttctccttcatcatattccgcatcaaacatctccttcaattttctcttcttatccaaatgctttttcttggcactttcttcttcgtcggggtcaatttcttccttgtttctctatatcttcattcctttcacagctggggagtggacctgggcctgcgcctctccgcgccagcgcctgcgctgtgcgcctctccgcgcctgcgccgccgctgtgcgcctctccgccgctgtgcg

SEQ ID NO: 17397 - RNA, 2605 nt, Homo sapiens
  source 1..2605: mol_type = other RNA
tcaggccaggcacagtggctcacgcctgtaattccagcactttgggagaccgcagtgggcggatcacgaggtcaggagttggagaccagcccggccaacatagtgaaaccctgtctctactaaaactacaaaaattggccaggcatagtggcatgtgcctgtagtcccagctacctgggaggctgaggcagaagaattgcttgaatccaggaggcagaggttttagtgagccgagattatgccactgcactccagcttgggtgacagagtgagacttcacctcaaaaaaaaaaataaataaataaaagaaaagaaaaaacaatcctgaaactcatatggaaccgcaaaaaaccccaaacagccaacagataactgtgaaagaaaaagttggaggcatcacacctcttgatttaaaattgtattacaaagctatagtaatcaaaacagtatggtgctggcataaaaacaaaaaaatagaccaatggaacagaacagagacctttgaaataaatccaaacatatactgtcaactaatttttgacaagggcaaacaagacaacacaatggtaaaaaagatagtttcttcaataataggattttcacatgcaaaagaataaaattcgaccctgatcatacaccatacacaaaaatcaactcaaaacagatacaagaccaaagacccaaataagacctgaaaccataaaactcctagaagaaaacatagggggaaagcctcttgacattggccttagcaataattttttggatatcgcaccacaagccaggctacaaatgtaaacataaacaaggaggactgcatcaaactaaaaagcttctgcacagcaaaggaacaaccaacaaaatgaaaggggaacctatagactggaagaaatatttgcaaaccacatatctgataaagtgttaatatccaaaaatcagtaaagaactcttacaacttaatagcagaaaaacaacccagttgaaaaatgggccaaataggaaatgaccagtaggaaatggggagatgtacattaaaataatacaaagtagcagacatgtaggatgaacaagttagagatctagtgtacatcatgagggctatagttaataaaaatatattgtctttgggatttttgttaaataagtagattttagctgttcctgtcacacaaacaaaaatctaactatgtgagatggtagctatgttaatttgcttcactatagtaaccagtttactatctatatttatcctttaagatcatgttgtcaacctcaaatatataaaataaaatttattttaaaaaagaaaagtttgtcttcaatccagaaagaaccactattaccattttttggtgttccattccaaaatatcccacaaatatacaattgttcaatcaaatttaacattagactttatacttgaacattcaaagtacgtaagaaattatagaaaagtgtctgcgtgactccctgtctgtagggcacaggcttcatctccactaacacacacacgaccagtaccttatacagagagtccttgtttgtctttagtctgacaccatgggcgagcccgaggtggcccgtggtccacattcctgaccaggtgtctttctcacccactggtttcaacaaagatgttactgggttatagaaggctgggatggaaacaggataccaagttcgcatgaagacaatatcttaataaatgaagtgttcttgaaaattttatatggaaaaccagttagctttaatttcttcacaatttttatggatttatccagatcaaggacaactcctgtggcagctatccgaaaatcaggcattatgccactgacagactgtattgccaagaaaccagttccctgtggagtgatagggtcccaaaaggctgctccacaatgcatgtgctgtggggtatactttagaagcctttgtcttccattgtggtcttcaatataatagagcaggatggtctgaaacctcctccaccctacagaaaatatgattggatcttgggacttgaggattttcttataccagcgatgtttcttcagacgcatctgcacgtgtccaacatttccctcgctgttgcccaagccacccaggataatggggtaatgggggtcaaagttctgcacaaattcacagggaacattttcaatctcaacgcggacgtacatcccaggtcgaaaaccatcatactgaactctggcttcatcatcttgatcttcaaattctacgtgattcagctgtgcttctttctgcatttctcctttaagatcatcaaaatatgtgctttctccttcatcatattccgcatcaaacatctccttcaattttctcttcttatccaaatgctttttcttggcactttcttcttcgtcggggtcaatttcttccttgtttctctatatcttcattctgagtgtcggggcccgattttcccttgtgcatgtcccctgtttccaagtcttcaaagtcaccgtagagctcctcctttcacagctggggagtggacctgggcctgcgcctctccgcgccagcgcctgcgctgtgcgcctctccgcgcctgcgccgccgctgtgcgcctctccgccgctgtgcg

SEQ ID NO: 17398 - RNA, 2546 nt, Homo sapiens
  source 1..2546: mol_type = other RNA
tcaggccaggcacagtggctcacgcctgtaattccagcactttgggagaccgcagtgggcggatcacgaggtcaggagttggagaccagcccggccaacatagtgaaaccctgtctctactaaaactacaaaaattggccaggcatagtggcatgtgcctgtagtcccagctacctgggaggctgaggcagaagaattgcttgaatccaggaggcagaggttttagtgagccgagattatgccactgcactccagcttgggtgacagagtgagacttcacctcaaaaaaaaaaataaataaataaaagaaaagaaaaaacaatcctgaaactcatatggaaccgcaaaaaaccccaaacagccaacagataactgtgaaagaaaaagttggaggcatcacacctcttgatttaaaattgtattacaaagctatagtaatcaaaacagtatggtgctggcataaaaacaaaaaaatagaccaatggaacagaacagagacctttgaaataaatccaaacatatactgtcaactaatttttgacaagggcaaacaagacaacacaatggtaaaaaagatagtttcttcaataataggattttcacatgcaaaagaataaaattcgaccctgatcatacaccatacacaaaaatcaactcaaaacagatacaagaccaaagacccaaataagacctgaaaccataaaactcctagaagaaaacatagggggaaagcctcttgacattggccttagcaataattttttggatatcgcaccacaagccaggctacaaatgtaaacataaacaaggaggactgcatcaaactaaaaagcttctgcacagcaaaggaacaaccaacaaaatgaaaggggaacctatagactggaagaaatatttgcaaaccacatatctgataaagtgttaatatccaaaaatcagtaaagaactcttacaacttaatagcagaaaaacaacccagttgaaaaatgggccaaataggaaatgaccagtaggaaatggggagatgtacattaaaataatacaaagtagcagacatgtaggatgaacaagttagagatctagtgtacatcatgagggctatagttaataaaaatatattgtctttgggatttttgttaaataagtagattttagctgttcctgtcacacaaacaaaaatctaactatgtgagatggtagctatgttaatttgcttcactatagtaaccagtttactatctatatttatcctttaagatcatgttgtcaacctcaaatatataaaataaaatttattttaaaaaagaaaagtttgtcttcaatccagaaagaaccactattaccattttttggtgttccattccaaaatatcccacaaatatacaattgttcaatcaaatttaacattagactttatacttgaacattcaaagtacgtaagaaattatagaaaagtgtctgcgtgactccctgtctgtagggcacaggcttcatctccactaacacacacacgaccagtaccttatacagagagtccttgtttgtctttagtctgacaccatgggcgagcccgaggtggcccgtggtccacattcctgaccaggtgtctttctcacccactggtttcaacaaagatgttactgggttatagaaggctgggatggaaacaggataccaagttcgcatgaagacaatatcttaataaatgaagtgttcttgaaaattttatatggaaaaccagttagctttaatttcttcacaatttttatggatttatccagatcaaggacaactcctgtggcagctatccgaaaatcaggcccaaaaggctgctccacaatgcatgtgctgtggggtatactttagaagcctttgtcttccattgtggtcttcaatataatagagcaggatggtctgaaacctcctccaccctacagaaaatatgattggatcttgggacttgaggattttcttataccagcgatgtttcttcagacgcatctgcacgtgtccaacatttccctcgctgttgcccaagccacccaggataatggggtaatgggggtcaaagttctgcacaaattcacagggaacattttcaatctcaacgcggacgtacatcccaggtcgaaaaccatcatactgaactctggcttcatcatcttgatcttcaaattctacgtgattcagctgtgcttctttctgcatttctcctttaagatcatcaaaatatgtgctttctccttcatcatattccgcatcaaacatctccttcaattttctcttcttatccaaatgctttttcttggcactttcttcttcgtcggggtcaatttcttccttgtttctctatatcttcattctgagtgtcggggcccgattttcccttgtgcatgtcccctgtttccaagtcttcaaagtcaccgtagagctcctcctttcacagctggggagtggacctgggcctgcgcctctccgcgccagcgcctgcgctgtgcgcctctccgcgcctgcgccgccgctgtgcgcctctccgccgctgtgcg

SEQ ID NO: 17399 - RNA, 31 nt, Homo sapiens
  source 1..31: mol_type = other RNA
tcaggccaggcacagtggctcacgcctgtag

SEQ ID NO: 17400 - RNA, 3578 nt, Homo sapiens
  source 1..3578: mol_type = other RNA
tcaggccaggcacagtggctcacgcttgtaatcccagcactttgggaggctgaggtgggtggatcacctgaggtcaggagtttgagaccagcccggccaacacggtgaaaccccgtctctactaaaaaatacaaaaattagctgggcatagtggcgggcacctgtagttccagctactctggaggctgaggcaggagaattgcttgaacccaggaggcagaggttgcagtgagccaagatcgtgccattgcactccagcctgggcaacaagagtgaaactccctctcaaaaaaaaaagtacagtgggatgatgaaattgtcttcaatcaccacactccgaaaatagttaactgtaaccaaacgtaaatgttgaaagcagcaataaagacaaaagcgatacagaataaaagcatggcggggctcaccatatccaggggattgggcaagtcagatgcttgccgacccctcagcaacctgtcttgtgcaaaaatgatcagggactccatcattaagccccaggttaccttcaccagcacctgcaggggaacaccccagaagacgagccccatggcttcagaacacacatttcagaggaccaaaagatgaggaagagatccacttcactccccaaagtctcttgcggagccctaactcaatcactcagtgaccaagagctggcaatgtactgaatattcacaactgcagcaaaaggtaccctcaaacataaggcccagaaactcttgctgaatttcaaagtagaaacgcttgaatgttaacctcgggagcagacatgttattgcgactgcatactgagtcggacctgtttctcctgcgggttttgagtctaagtccacaaggggcctgggaggcaagctgtcctcctagtcgtctctccaaggagtttgaacacagagagagcccatcatccctccgcctttcattgccatcttcagcgattccaacggctggagggagagtctgggaagcacacaggccccaaacctgacagggccgagcccagccctgatggtttcccttccttgctgggacacagctccttccagcagttgagaaactcaagggacagtccctctcacggggctggaggatcctgtggacagccatccctgtctttaggcaggtgtgtgtgacgggtcagttccgagactccgaggctgtggggctgcggaccgtggacatgaggtgtgacttgtaggtcttgctcaggccagtcatccagaacttcagcagcttgacattgtcctcctcggacgcacccaggatgctcagcagcttctgtgtgtcctctttgggtcgactgtccaccttggtgaacttaaaaagcaccttcactttgttcatccactcctccttgaggcagacgaggcactggtccaccacatccacagacaggttctggttggtcagagccgcttcaatcttattcaggatggtggggcccactcggtctgcagctacagggctcccactggtcaccacaaactcgtacttgctgagagactggtcatcctcacaccccacagggtggagggtggaacgtgcggctgcgtggacctccacgatgacagcaaactctgaggagagcacgtggggggggatctgcacgtgcgggctgagccccaggaagttgcaccgataggcctcctcgtactggctgctgtatgggatgatgcggacgcagcccacgggaagcatggtccgaagtacttcaaaagctgactggacgaggtccacgtctctgcttttccagatcacctggttccccatgagaacgtgccaggccagcatgcggaaagaaggggcacccaggacctgcctcatgtgccggagggacttgaagactggcagcttccggggctgccagctcccacagcctgagagagaggaggactctgccgggccctgggtcagctcccgcccttctgtactctctggcaacacaggggctttctcctcctcttcagcctcagagttgtcccagctttctgattcctcttctaaatcagcgagcttctccatctggaccaaggtatcctcggtcggagcaccttccaggagcttctcggtcagccggctgccacacgccttcaggagccaggcaaaggaggtgtgcaggcacgcccacaggttgtcatcacttgtcagcgatgtcagcgagcgggcggcgttgccgttcctctggtgtaggaatggcgtgaaggctgtgttcatcctctgagcacgctgtgggcatccaaactgctctgcctcaaacaccttgagcgccttgccctggagctcatcgatgattccccggaccttccccagcaggaagggccaggagttgatgaggtagatccggtccatcatgatggtgatgatgctgtaccagcgctggaagcccctggccaggctgtccttgatgaagaaggtgtggctgaacacaaagccgtgctgctcatctccgaagaagatggggccttcacggccagggcagacctcacagctcaggctccggacacaggcctggcggacaatgctgaagagctgggggtggctggggtgctggtggctgacgtatttaatggaggtctctttatcatggctgatatatcccgggtgccctgcagcaagtgaccggcagccctcgcacatgtccgactttttgggccccgggctgctggactcgacgctggccccctctgcggggctgtgcgcacgcatccgactgttcatctgaatgccaccttcctcttcttccgcctgctcaccctggccaggactgtcctcattcccatccccttgaggaagtggggcgtgcagcacctccgtgcagaagagagtgcgggggccgtggagctcgcagaagtggcagagagccacgatggcattcatggtgccttggagactgcaacaggcctcctgcagggggtcggcgggggacacaggaaaactgcttcctgcgagaggcccacgcagggaatgaccagaggaggcaggagcctggaaggactggcttacggggccaagcaagagttgaagggcagggtgggtgctgtactgtctgaggggtgtgtaaggtccggtgtccaaagagcagcagcagacagggtggaggctgacgtttctgcagttggctgcttagctgcacgagctgctccggcacctgtcctcctgctgagatacggctgagcacgagtggtcacactgacactcagcagaatcacgcttccaccgtccacaccagaccaccacacacgaggctgctgccaaatgggtcaggcatggtggtggcagacacccttgaagacctggcgttttctgctccccaaatcgaggcccgcgggacacctggactcggcagccggggtcccgctctgggtcccagccccgcccctgactgcgctgggtaggtggtcgctgcgggacccggaccggcggaatcacacccagagcccccaagcccacggcagggatgtcacccggggtggcgaggctctcaagcccgggttcaggctctcaggggagctggcagaaccaggagcgaccacactcactcgcggtcccgcagccccgcc

SEQ ID NO: 17401 - RNA, 3662 nt, Homo sapiens
  source 1..3662: mol_type = other RNA
tcaggccaggcacagtggctcacgcttgtaatcccagcactttgggaggctgaggtgggtggatcacctgaggtcaggagtttgagaccagcccggccaacacggtgaaaccccgtctctactaaaaaatacaaaaattagctgggcatagtggcgggcacctgtagttccagctactctggaggctgaggcaggagaattgcttgaacccaggaggcagaggttgcagtgagccaagatcgtgccattgcactccagcctgggcaacaagagtgaaactccctctcaaaaaaaaaagtacagtgggatgatgaaattgtcttcaatcaccacactccgaaaatagttaactgtaaccaaacgtaaatgttgaaagcagcaataaagacaaaagcgatacagaataaaagcatggcggggctcaccatatccaggggattgggcaagtcagatgcttgccgacccctcagcaacctgtcttgtgcaaaaatgatcagggactccatcattaagccccaggttaccttcaccagcacctgcaggggaacaccccagaagacgagccccatggcttcagaacacacatttcagaggaccaaaagatgaggaagagatccacttcactccccaaagtctcttgcggagccctaactcaatcactcagtgaccaagagctggcaatgtactgaatattcacaactgcagcaaaaggtaccctcaaacataaggcccagaaactcttgctgaatttcaaagtagaaacgcttgaatgttaacctcgggagcagacatgttattgcgactgcatactgagtcggacctgtttctcctgcgggttttgagtctaagtccacaaggggcctgggaggcaagctgtcctcctagtcgtctctccaaggagtttgaacacagagagagcccatcatccctccgcctttcattgccatcttcagcgattccaacggctggagggagagtctgggaagcacacaggccccaaacctgacagggccgagcccagccctgatggtttcccttccttgctgggacacagctccttccagcagttgagaaactcaagggacagtccctctcacggggctggaggatcctgtggacagccatccctgtctttaggcaggtgtgtgtgacgggtcagttccgagactccgaggctgtggggctgcggaccgtggacatgaggtgtgacttgtaggtcttgctcaggccagtcatccagaacttcagcagcttgacattgtcctcctcggacgcacccaggatgctcagcagcttctgtgtgtcctctttgggtcgactgtccaccttggtgaacttaaaaagcaccttcactttgttcatccactcctccttgaggcagacgaggcactggtccaccacatccacagacaggttctggttggtcagagccgcttcaatcttattcaggatggtggggcccactcggtctgcagctacagggctcccactggtcaccacaaactcgtacttgctgagagactggtcatcctcacaccccacagggtggagggtggaacgtgcggctgcgtggacctccacgatgacagcaaactctgaggagagcacgtggggggggatctgcacgtgcgggctgagccccaggaagttgcaccgataggcctcctcgtactggctgctgtatgggatgatgcggacgcagcccacgggaagcatggtccgaagtacttcaaaagctgactggacgaggtccacgtctctgcttttccagatcacctggttccccatgagaacgtgccaggccagcatgcggaaagaaggggcacccaggacctgcctcatgtgccggagggacttgaagactggcagcttccggggctgccagctcccacagcctgagagagaggaggactctgccgggccctgggtcagctcccgcccttctgtactctctggcaacacaggggctttctcctcctcttcagcctcagagttgtcccagctttctgattcctcttctaaatcagcgagcttctccatctggaccaaggtatcctcggtcggagcaccttccaggagcttctcggtcagccggctgccacacgccttcaggagccaggcaaaggaggtgtgcaggcacgcccacaggttgtcatcacttgtcagcgatgtcagcgagcgggcggcgttgccgttcctctggtgtaggaatggcgtgaaggctgtgttcatcctctgagcacgctgtgggcatccaaactgctctgcctcaaacaccttgagcgccttgccctggagctcatcgatgattccccggaccttccccagcaggaagggccaggagttgatgaggtagatccggtccatcatgatggtgatgatgctgtaccagcgctggaagcccctggccaggctgtccttgatgaagaaggtgtggctgaacacaaagccgtgctgctcatctccgaagaagatggggccttcacggccagggcagacctcacagctcaggctccggacacaggcctggcggacaatgctgaagagctgggggtggctggggtgctggtggctgacgtatttaatggaggtctctttatcatggctgatatatcccgggtgccctgcagcaagtgaccggcagccctcgcacatgtccgactttttgggccccgggctgctggactcgacgctggccccctctgcggggctgtgcgcacgcatccgactgttcatctgaatgccaccttcctcttcttccgcctgctcaccctggccaggactgtcctcattcccatccccttgaggaagtggggcgtgcagcacctccgtgcagaagagagtgcgggggccgtggagctcgcagaagtggcagagagccacgatggcattcatggtgccttggagactgcaacaggcctcctgcagggggtcggcgggggacacaggaaaactgcttcctgcgagaggcccacgcagggaatgaccagaggaggcaggagcctggaaggactggcttacggggccaagcaagagttgaagggcagggtgggtgctgtactgtctgaggggtgtgtaaggtccggtgtccaaagagcagcagcagacagggtggaggctgtaggaagcagatcttatagctcctccaggccaccgaaagaccctggatgtgttatcagagactggggaggctttgggggttctgacgtttctgcagttggctgcttagctgcacgagctgctccggcacctgtcctcctgctgagatacggctgagcacgagtggtcacactgacactcagcagaatcacgcttccaccgtccacaccagaccaccacacacgaggctgctgccaaatgggtcaggcatggtggtggcagacacccttgaagacctggcgttttctgctccccaaatcgaggcccgcgggacacctggactcggcagccggggtcccgctctgggtcccagccccgcccctgactgcgctgggtaggtggtcgctgcgggacccggaccggcggaatcacacccagagcccccaagcccacggcagggatgtcacccggggtggcgaggctctcaagcccgggttcaggctctcaggggagctggcagaaccaggagcgaccacactcactcgcggtcccgcagccccgcc

SEQ ID NO: 17402 - RNA, 3379 nt, Homo sapiens
  source 1..3379: mol_type = other RNA
tcaggccaggcacagtggctcacgcttgtaatcccagcactttgggaggctgaggtgggtggatcacctgaggtcaggagtttgagaccagcccggccaacacggtgaaaccccgtctctactaaaaaatacaaaaattagctgggcatagtggcgggcacctgtagttccagctactctggaggctgaggcaggagaattgcttgaacccaggaggcagaggttgcagtgagccaagatcgtgccattgcactccagcctgggcaacaagagtgaaactccctctcaaaaaaaaaagtacagtgggatgatgaaattgtcttcaatcaccacactccgaaaatagttaactgtaaccaaacgtaaatgttgaaagcagcaataaagacaaaagcgatacagaataaaagcatggcggggctcaccatatccaggggattgggcaagtcagatgcttgccgacccctcagcaacctgtcttgtgcaaaaatgatcagggactccatcattaagccccaggttaccttcaccagcacctgcaggggaacaccccagaagacgagccccatggcttcagaacacacatttcagaggaccaaaagatgaggaagagatccacttcactccccaaagtctcttgcggagccctaactcaatcactcagtgaccaagagctggcaatgtactgaatattcacaactgcagcaaaaggtaccctcaaacataaggcccagaaactcttgctgaatttcaaagtagaaacgcttgaatgttaacctcgggagcagacatgttattgcgactgcatactgagtcggacctgtttctcctgcgggttttgagtctaagtccacaaggggcctgggaggcaagctgtcctcctagtcgtctctccaaggagtttgaacacagagagagcccatcatccctccgcctttcattgccatcttcagcgattccaacggctggagggagagtctgggaagcacacaggccccaaacctgacagggccgagcccagccctgatggtttcccttccttgctgggacacagctccttccagcagttgagaaactcaagggacagtccctctcacggggctggaggatcctgtggacagccatccctgtctttaggcaggtgtgtgtgacgggtcagttccgagactccgaggctgtggggctgcggaccgtggacatgaggtgtgacttgtaggtcttgctcaggccagtcatccagaacttcagcagcttgacattgtcctcctcggacgcacccaggatgctcagcagcttctgtgtgtcctctttgggtcgactgtccaccttggtgaacttaaaaagcaccttcactttgttcatccactcctccttgaggcagacgaggcactggtccaccacatccacagacaggttctggttggtcagagccgcttcaatcttattcaggatggtggggcccactcggtctgcagctacagggctcccactggtcaccacaaactcgtacttgctgagagactggtcatcctcacaccccacagggtggagggtggaacgtgcggctgcgtggacctccacgatgacagcaaactctgaggagagcacgtggggggggatctgcacgtgcgggctgagccccaggaagttgcaccgataggcctcctcgtactggctgctgtatgggatgatgcggacgcagcccacgggaagcatggtccgaagtacttcaaaagctgactggacgaggtccacgtctctgcttttccagatcacctggttccccatgagaacgtgccaggccagcatgcggaaagaaggggcacccaggacctgcctcatgtgccggagggacttgaagactggcagcttccggggctgccagctcccacagcctgagagagaggaggactctgccgggccctgggtcagctcccgcccttctgtactctctggcaacacaggggctttctcctcctcttcagcctcagagttgtcccagctttctgattcctcttctaaatcagcgagcttctccatctggaccaaggtatcctcggtcggagcaccttccaggagcttctcggtcagccggctgccacacgccttcaggagccaggcaaaggaggtgtgcaggcacgcccacaggttgtcatcacttgtcagcgatgtcagcgagcgggcggcgttgccgttcctctggtgtaggaatggcgtgaaggctgtgttcatcctctgagcacgctgtgggcatccaaactgctctgcctcaaacaccttgagcgccttgccctggagctcatcgatgattccccggaccttccccagcaggaagggccaggagttgatgaggtagatccggtccatcatgatggtgatgatgctgtaccagcgctggaagcccctggccaggctgtccttgatgaagaaggtgtggctgaacacaaagccgtgctgctcatctccgaagaagatggggccttcacggccagggcagacctcacagctcaggctccggacacaggcctggcggacaatgctgaagagctgggggtggctggggtgctggtggctgacgtatttaatggaggtctctttatcatggctgatatatcccgggtgccctgcagcaagtgaccggcagccctcgcacatgtccgactttttgggccccgggctgctggactcgacgctggccccctctgcggggctgtgcgcacgcatccgactgttcatctgaatgccaccttcctcttcttccgcctgctcaccctggccaggactgtcctcattcccatccccttgaggaagtggggcgtgcagcacctccgtgcagaagagagtgcgggggccgtggagctcgcagaagtggcagagagccacgatggcattcatggtgccttggagactgcaacaggcctgacgtttctgcagttggctgcttagctgcacgagctgctccggcacctgtcctcctgctgagatacggctgagcacgagtggtcacactgacactcagcagaatcacgcttccaccgtccacaccagaccaccacacacgaggctgctgccaaatgggtcaggcatggtggtggcagacacccttgaagacctggcgttttctgctccccaaatcgaggcccgcgggacacctggactcggcagccggggtcccgctctgggtcccagccccgcccctgactgcgctgggtaggtggtcgctgcgggacccggaccggcggaatcacacccagagcccccaagcccacggcagggatgtcacccggggtggcgaggctctcaagcccgggttcaggctctcaggggagctggcagaaccaggagcgaccacactcactcgcggtcccgcagccccgcc

SEQ ID NO: 17403 - RNA, 3641 nt, Homo sapiens
  source 1..3641: mol_type = other RNA
tcaggccaggcacagtggctcacgcttgtaatcccagcactttgggaggctgaggtgggtggatcacctgaggtcaggagtttgagaccagcccggccaacacggtgaaaccccgtctctactaaaaaatacaaaaattagctgggcatagtggcgggcacctgtagttccagctactctggaggctgaggcaggagaattgcttgaacccaggaggcagaggttgcagtgagccaagatcgtgccattgcactccagcctgggcaacaagagtgaaactccctctcaaaaaaaaaagtacagtgggatgatgaaattgtcttcaatcaccacactccgaaaatagttaactgtaaccaaacgtaaatgttgaaagcagcaataaagacaaaagcgatacagaataaaagcatggcggggctcaccatatccaggggattgggcaagtcagatgcttgccgacccctcagcaacctgtcttgtgcaaaaatgatcagggactccatcattaagccccaggttaccttcaccagcacctgcaggggaacaccccagaagacgagccccatggcttcagaacacacatttcagaggaccaaaagatgaggaagagatccacttcactccccaaagtctcttgcggagccctaactcaatcactcagtgaccaagagctggcaatgtactgaatattcacaactgcagcaaaaggtaccctcaaacataaggcccagaaactcttgctgaatttcaaagtagaaacgcttgaatgttaacctcgggagcagacatgttattgcgactgcatactgagtcggacctgtttctcctgcgggttttgagtctaagtccacaaggggcctgggaggcaagctgtcctcctagtcgtctctccaaggagtttgaacacagagagagcccatcatccctccgcctttcattgccatcttcagcgattccaacggctggagggagagtctgggaagcacacaggccccaaacctgacagggccgagcccagccctgatggtttcccttccttgctgggacacagctccttccagcagttgagaaactcaagggacagtccctctcacggggctggaggatcctgtggacagccatccctgtctttaggcaggtgtgtgtgacgggtcagttccgagactccgaggctgtggggctgcggaccgtggacatgaggtgtgacttgtaggtcttgctcaggccagtcatccagaacttcagcagcttgacattgtcctcctcggacgcacccaggatgctcagcagcttctgtgtgtcctctttgggtcgactgtccaccttggtgaacttaaaaagcaccttcactttgttcatccactcctccttgaggcagacgaggcactggtccaccacatccacagacaggttctggttggtcagagccgcttcaatcttattcaggatggtggggcccactcggtctgcagctacagggctcccactggtcaccacaaactcgtacttgctgagagactggtcatcctcacaccccacagggtggagggtggaacgtgcggctgcgtggacctccacgatgacagcaaactctgaggagagcacgtggggggggatctgcacgtgcgggctgagccccaggaagttgcaccgataggcctcctcgtactggctgctgtatgggatgatgcggacgcagcccacgggaagcatggtccgaagtacttcaaaagctgactggacgaggtccacgtctctgcttttccagatcacctggttccccatgagaacgtgccaggccagcatgcggaaagaaggggcacccaggacctgcctcatgtgccggagggacttgaagactggcagcttccggggctgccagctcccacagcctgagagagaggaggactctgccgggccctgggtcagctcccgcccttctgtactctctggcaacacaggggctttctcctcctcttcagcctcagagttgtcccagctttctgattcctcttctaaatcagcgagcttctccatctggaccaaggtatcctcggtcggagcaccttccaggagcttctcggtcagccggctgccacacgccttcaggagccaggcaaaggaggtgtgcaggcacgcccacaggttgtcatcacttgtcagcgatgtcagcgagcgggcggcgttgccgttcctctggtgtaggaatggcgtgaaggctgtgttcatcctctgagcacgctgtgggcatccaaactgctctgcctcaaacaccttgagcgccttgccctggagctcatcgatgattccccggaccttccccagcaggaagggccaggagttgatgaggtagatccggtccatcatgatggtgatgatgctgtaccagcgctggaagcccctggccaggctgtccttgatgaagaaggtgtggctgaacacaaagccgtgctgctcatctccgaagaagatggggccttcacggccagggcagacctggagcatgcagaagaaccagcaggtcagagcagccactgcactctccctgcactcacagctcaggctccggacacaggcctggcggacaatgctgaagagctgggggtggctggggtgctggtggctgacgtatttaatggaggtctctttatcatggctgatatatcccgggtgccctgcagcaagtgaccggcagccctcgcacatgtccgactttttgggccccgggctgctggactcgacgctggccccctctgcggggctgtgcgcacgcatccgactgttcatctgaatgccaccttcctcttcttccgcctgctcaccctggccaggactgtcctcattcccatccccttgaggaagtggggcgtgcagcacctccgtgcagaagagagtgcgggggccgtggagctcgcagaagtggcagagagccacgatggcattcatggtgccttggagactgcaacaggcctgacgtttctgcagttggctgcttagctgcacgagctgctccggcacctgtcctcctgctgagatacggctgagcacgagtggtcacactgacactcagcagaatcacgcttccaccgtccacaccagaccaccacacacgaggctgctgccaaatgggtcaggcatggtggtggcagacacccttgaagacctggcgttttcttggacttcaatccacaagccaatccattctttccaggagacaaggacgcgactgacagtactctcaactggagagaagcgcggtcttccaccctccctggaggacacggtgctaccctattagcgcatcagaggaccctcctgaacgccaaactgggagaagaggatgacacacaccctctcctccaaacagagcgaagacaaaacctgctccccaaatcgaggcccgcgggacacctggactcggcagccggggtcccgctctgggtcccagccccgcccctgactgcgctgggtaggtggtcgctgcgggacccggaccggcggaatcacacccagagcccccaagcccacggcagggatgtcacccggggtggcgaggctctcaagcccgggttcaggctctcaggggagctggcagaaccaggagcgaccacactcactcgcggtcccgcagccccgcc

SEQ ID NO: 17404 - RNA, 5456 nt, Homo sapiens
  source 1..5456: mol_type = other RNA
tcaggccaggcacagtggctcacggctataatttcagcactttaggaggccgaggtgggagggtggcttgagcccaagagttcaagaccagcctgggcaacatagtgagaacccatctctacaaaaacataatacggttagtcaggtgttgtggcacatgtctgtggtcccagctactcaggaggctgaggtgagaggatcactagagcccaggaggtcgaggctgcaggctccagtctaggcaacagagagagactctgtctcaaaaaaaaaaaaatttcctatataagtaggatgtgtaatgtactagtcacttaatgagtgccatacccatctctgttctgaccagactaatccccaaatgtcatccttggttcccaggacaatccacagaaaactgctgccacgataagaggagatttttatgtcactggagacagaggagtgatggacagtgatgggtatttctggtttgtcggcagagctgatgatgtcattatatcctctgggtttgtatatttgccactctgaagaggtaacaattcgacagggagggagatctctaacttggaggatgtggtggtcaaaaacttcttttcctcttcaggtaccgtattgggccatttgaagtggagagtgcactcattgagcatccagcagttgttgaatcggctgttgtcagtagtccagatcaaatccgcggagaggtagatgaatgtcatttattaaagaagcaacatcatattttcaagttctgtccatttgaccactgtaaaggctgaaaatattctgaaaaacctcactttgtaattgtatccaagctttgttcagaggtaacctctggcatttgcagtcatcacacaaactgttattaataaatagtaagcacctgtgttcagcatttgttgcaaatccttgatgtgtctgcagcagaaaaactgatcacactgtaggatttccctagttcctttgaccgctgctcttcatggtgagttttcaacttgctgggtcaggagggcttaacatcacccacatatcaagattctggtgagccctggaagtctaaagtcattttgtggcttcagaggcaggaagaactcccaacagcgatgtgtcgctagcatcttcacaaccatggttgggggtgtcatctgaggttcttgtcccatgtgggtcctctctcttgaggcaggtctccatctcatggaataaattctcctcgagagaacccctccttctggttgaaactctgaggggcagatgtttttgtttctgaactcggcaccacgtgagaaatagaataaacagaaccaggagaaggagcccaaagatactggataaaataagtgctaaatgacctgaggaggcattcagtgatttcagcgactgtccagagcacctcacgccagcatcttccttgtgtccacagtcactctgtccccagggtttggcgtgacagtcccatagaaatgactcatttcctttgcaccgcatgtcatccaaccagatggttccagttccctggccaaacgaagcgtccctcagggcagccagagcagagccacagcccagctgctgacacaccacttccgcctcggccaggtcccaggagtcatcacacactgtgccccaggagcctgcgtgccagatctccactctcccagagcactcggtgtctcctccacgcactcttattctatcttcacatgtgatccaggtctcttctgctgggctggagattcttcgctcccatggggcagacaggcactgccatatggagatatgcgttttaggacactgaatgtcatccacccacatgaaaccagagcctgtcttagataaaggggcgaggctgacaactccattctccccacagcccagctgcctgcacacaatgcctgctatggctgtggtgatgttcctcctgccgacgctgccccaggtcccgttatagaagacttccaatctcccagcacagctctctgtttcagtttcactgtagagcctcaaggctgtgaattctgagcagatgacccctgcgtcctccttgtgcctgcagtcgtgctgcccccagccgcgggaagggcactgccacaagtgggactccattcctgtgcagttcaggtcatccagccagatgggccctgacccctccccaaagtgagcagagaccgtggcattgaaggccactccacagcccagcttttgacacaccacgtgggcatcgctcaggtcccagccgtcatcacagatggtgccccagaagccgtcgtgatagatctctactctcccggcacagcggctgtccccatccactaggcggagccgtttgtcctctaagcagatcaaagcactgccctctggaactgcagacaaatatgggtcagatacatttgcgaggcatggaaacagtggctgggtcaggcttcctgtgcagatcacagagacagtatttccatggatacagggaggtgctccaagaactgtcatttgacagttatccagaagtgactcattccctaagcaatgaaacctgtgtccccacacacgaacacttctttctccaatatattttcctcctgtggttgagagagcagtcccacagctgagctgtctgcatagaacacgggcatcttctgggtcccagtgggtgtcacacagtgagccccagtgtccaagcacgttgatctccacttgcccgtcacactgggatttgccattcacaagtcggacatctgtatatcgggaacagacaactccaacttctctgctgtggatacaagtgtcttccggatgttgaacaatggggcataatgcaaggtgagtttcactcccttcacactggaacttttcggcccaagttagaccattcccttttccaaagtgatctcccacagaaagagatatggcatctccacagtttaattctctgcacagcacattggcagcatgaagagagaaatcagaatcacagacagagcgccatgtgtctgcatgtttcacttcaacacgtccagagcagggcatatcagctccaaccagcctgggctgcctgtgggctgagcagatcaaacttgcttccatatttaaatgacacgcagtctgtttccactcccatcgtatacaatcccagagagaggcttcccctccagtgcagccagaattcgacattaagatgtgtaatgttctttctgtgaaatgaggctctctggagaccctgattgcagacccacattcaagttgcctgcaaacaacttcagcaatgttcattccccagccattagcacacagaattcccacggcaccctggacattcacctcaacttttccagcacacctgctgcttccacccacaagcctcagctccatatccgatgcatcagaacagatcactccaacatcttcactgtgactgcagtcattatttccccacccactgttcctgcatgaccagagatctgactcatctccatcacaggaaacatcatcgagccaaatttttccatatcctgtagaagcgtttcccagacccatgccaatgatagaagatgggcagtccagctggctacacaccacagctgcagctttactgttccagccgtcatcacacactgtgccccaccgtccttgaaagtacacctccagtcttcccgagcagcggttgctgccgcccaccagcctcaggccccatgttgcatcacctgagcaggttacaatcacatcctctctgtgtacacaattatgctttccccatccactgtgttcacagtcccagatatttgactcatttccaatgcaagaaacgtcatccagccaaataggtcctgatgcttctttaaaataggtcataccaaacacatgcaaaggctttccacatcccaattgtttacaaacaacagctgcattccttgtgctccatctgtcatgacacacagtcccccactctccttggtatttcacctccaatctcccataacaggggctatgagccccgacaagccttaggtccagatctgccttatcagaacaaattactccagcatctgatcttcggaagcatgttcgctttgcttttccatcatatgtgcagtcccagagagctgactcattcccagtgcaagatatgctgtttatccaaatgtctctagcttcattactaggtttagcacgacgactgccaaagacgctgaacggacatcctagctgcttacaaaccacaagggcttgttcattcttccagttctggtcacatattgtccaccactgttcatgaattctcacctctactctccctgaacaattgttacttccatctgctagtcgcagttccaaatctgctccatctgagcagatcacagacacatcgttttgatgaagacagtcaaaattgacggttccggaatgtctgcagtcccaaagaaaagattcattaccggagcaggagacaccatcaagccatacaacatcagaccctgactgcaaatgaggcaagccagcgaagtgaagtgcggttccacatcccaactgcttgcatacgacatcagctgcagcattgttccacttatggtggcatacggtcccccaccttccttggattttcagctctactctccccatacagcggttagttccacctacaagccttagttcaagatcactactatcataacaagttaatgtgacatcctcattgtgactgcagtcatgatttccccatccacgatgtctgcaattccagagtgccaactcattcccctggcataaaatgtcatccagccaaatggggcgcaatacagcagggctattaacaactccagaagaaataaaagaagatggacatcctagttgcctgcacaccacggcagcagtattcaagttccacccatcatcacatatagttccccacctttcttggaatttcacctccactctccctgaacaggagttgtttccatccactagcctcaaacccagattggcttcaccataacagttcacaccaacatcttctccatgataacagttatggcttccccattcccggtgttgacattcccagagagctgactcatttccataacaggaaacatcatcaagccaaatttttccatgtctagtcacggcttgtccaaaacgaaacatggcgaaagaaaatggacatccaagctgtttgcacacgacagttgaggcagtagtgttccacccatcatcacacacagtcccccactgtccctggaatttcacctccactgtcccagagcagggaccgtctccattgaccagcctcaactccaaatctgttccattaaaactgctgatgagaaagcaggaattcaggagcaggatgcaagttaccacagcagagaaaaggttctgatgacagcagcatcttccaaaatcaatatgccacgagttttgaggcagcatcattatgggtctatctcttcctgagtcct

SEQ ID NO: 17405 - RNA, 1597 nt, Homo sapiens
  source 1..1597: mol_type = other RNA
tcaggccaggcacagtggctcacggctgtggtcccagcatgttgagaggctgagatggaacagtcccttgaggtcaggagtttgacatcagcctgggcaacatagtgagacccccatctcttgattcccagttcaatattttctcctccgtatacatccatgccaggatccagaagaccaatttcaccgaagaacttcctgttgaccacgaacgagcagcctatcatggctggggtcctgatggggagagaagggtctccggcgtcccaccagtcttttggggggctgatgtacatgcaccacagctcccagctgtacccgtgggccgagttctcgtaccgctgcacctcaaagttgtcctgtttgatgttgtcaatggaggggaggatcacacgcttccggttttcctggatgcgggatagaaccggctcagcccagccagcggtgaattccacgtgggcatcaaagaagccagtgacctgcccggtagccaccttccagccctcaatgcgagcgcggatcaggccttccctcttctgatttcttaccaccttcaccagcccggggtagcgtttgtggacatactcctctagggggaccttcagctcctcttcgtcgctgttgtcatccaccagaatgatttccttcagcaggtgtgtgggcgtgtgattgacggcactgtgcacggaccgcaggatcaccgacagggcctcgttcacgaagatgaatatgatggatatctggggcaggtccttggagtacttgagctccttacacttggtgggacgataatccggaatggaacggtccagtgaaattttttcactgaggtatgaattgtagccatacttctcatggggtcccttagccttttcttcttcagccggggaaagagtagccggaaggccccctttaccccgcccaccataaccttcaatgagcccaagggatttggataagccattcagctgccggtacacgatgtcctccagcagcgacaggcgcttcaggaccgcatcctggatggggctggcgctgtgcgcgctgaggttggccacctcggcgcgcggccggatctcgtggaaggcgtctccgctgcgcaccgcgatgggccggcacttggccaggaagagcacgaagccggctaccgcgatcaagttcaacaccaacagcactttgactcttctcagtgaagccatcaaacagcccggccggccctcgccccggacctgcgccccctcgggctccggcgaggcgcggggcagccaggggccgtgcaagcctcacacaccagacggccggcagggatccaagcccctgctcgtcccacctcaaggatgctcgggcggcggagacggctgggaggtcggattggtggtggggagaacggaatcgctcacatggaagtcctcgctctgcagaagtgctccccgagacgcctgctcagtccacggcgcacggccccgtccaggcgtctccgcgaaaggccagggatttgagggtttctcttctgcaccagcaagtggttcgcctctggacctctagccgccggcgccgcggactccgaggccggcaggcggggctgcccgggaggcac

SEQ ID NO: 17406 - RNA, 4134 nt, Homo sapiens
  source 1..4134: mol_type = other RNA
tcaggccaggcacagtggctcacgtctgtaatcccagaactttgggaggctgaggcgggcagatcacgaggtcaggagttcgagaccagcttggccaacatgttgaaaccctgtctctactaaaaatataaaaatcagctgggtgtggtggtgcacgccggtaatcctagctactcaggaaactgaggcaggagaatcacttgaacctgggaggcggaagttgcagtgagtggagattgtgccactgtactccagccggggcaaaagaggagactctgtctcaaaaaaataaaaataaaataaataataataataatgatgataataaaaaatgctgtaaaatagtgaggacagttttacttttctccctccaaacagtaaagaacagtaaactcttctatcttctgtaactagggtaaaaaaataagagactgaccaactgacttatatgaagtattaatagaactgaacgatctttccaatacatcatgtaaaactgtaactatgcttattgtttgacaaaataaatttaacaatgaccatgtataagaaatataacgaatagatcccattttgacatataaccgattttaactaaagggcttctgaacctttcaaaagtgacacgaattctctcttcactcccagaatgaaatttgtcatctttttcattgaaatacatttcaacacactgctcttcaaaatcatgaagtttcttttgatcttcttctgttaagaaaagttttggtccatcggaagtcttatctttctttcttctcttacatatgcagcaaaacagagaaactatatggctaagaatgataagtggaggaggcagaactggtttctcatgataagccataataaaatgataacgctggtacttccatacaatattggaaattgccttcacttgtaaatacacattgcatcaatttcgtatgcataaacttcaccaaaaatcatccagtatgggtgaaaaactatatctttagcaagagtccaagatggtgcttcatgaggataaagtattgcctttctgggaacaccaaaactaagtaatacaagagccataatcactacaatgtagaacatattggccaccatttttccaatcatcattacataaggtcctgcctgttgatttacagctagaaaatctagcaaacgcacataccaaaatattatgttaagacagtaaattaatcttccagccacaaaaacatgattatcatatgcatttgcaaagttccattttgctccaaatcttagtccaaatccaatgaagaaagaaattatggcaattgtatcactgatgttgaagtaatcactaaaccatactttaatcttctggtttactttcccagcttcagacataaagatctcacggactttctcaatggcataagtaaaaatataagcaataacaatccattcttgaactgaaggtaactgttccatttgtacaagaaccacaaatgtataaagcatcagaaatcctaaatatgccaacgtgttaaaccagaattttacaattggtgcatgataaaaggcataaaactttcgcgtaattggaagcttttttgatttcatttgtatctccatctcattctttccttcattactatccaaaatccgtacttctttaaacacttccatggggatctcttctgttatgttctgaaagttgttttcgctgtcatccattgtcatctgatgagcatcttgagattgtgggatatgggacatttcagccttagttttatactctaacagcaatatggcaggtggaactaaaatgcttagtatgaccttgtaccaggaatttttcctcatattcagccttcccatccacatatcagataacaacatttgtgtacaggtgtgagctacaaaaggtctaagtcttgaagaaactgctaacttaaggcaggttgaattactccagttcttcagttcataagtgagcaatttcatagccatggtttcatcttgtctgaaggactgttctaataattcaacggccaactgaccaaaatcattggaatactgttttagttcttctgaagtatcatctaccaggtcactctgctttgcttcatatgccattgaacgatagatcttacaggcaactaatgctttagccattgattcttcaccatgttgccataaaaaacgggccatgacctgcctcttcataaggcaagcccaaattaaaagttcattaagtggataaggaaagcgcttggtttctggatcatcaatgtctacaatttcatctttggttcttttcttctttccttcttccataactgtatcaatctttggtcggtagggctgtgctgtcttaatgaaatggttatgcctcattttttcctttttatctgccctattgccaaaagattcatgactctttcgcaactgaggagtgctgctggaggtatttcggccagacctccgattatttccaccaagactattatatattaatcgaaaacgtttcctagtataggtgcatctgtaggttcctcccatgagatattcaataacaagtcctatatcaatcagagtgatcttatatcctggaggaagatttccctgtttgacgtctcgaacaagatgaaacagcattggattagttggaccttgtttagtgttgtaaagttcttccagtctcggaatggtaaggaatttatgcatgcttactccattttcaataagaagttttacaaatgcaactctatccattacaagagcatcaagcatagcttgttccaaggatccaaccagccactgctgtccataaacaaatacatgatttttggcaatgtcaactctatcccatgccaatgtaaggataagctggtcaaatgcagatgcattagtaccttttagcagtgcagtaagtattgctacatctatatcttgatgttcatctgacccaatatggaaaacagtgataagctcctttcttttcatgcactccatcagtgtttgaaataaatgaagtgcttcattctggccaaagttaaatgtttttttgatagtggaaataatatcgggctctgctgcatcaggaagattccctccttcttctgtttgtttatgaatatacgctagcagatctgcagctctgcctgttccttcacacacaactactggaacaggggggctttcctgaaggtattcaagaactgtgaggataacatttggcccaccctcaaatataagtgccaccacagggacaccctggccaatcctagcatgaattctttgctgattaatagttttttcaagttctcttctcagtctgacttccgccccatactttccaacagtgccatcatccaccaatatgaaatgggaatgcagattattcaaaacattcaatttgctcagggggttcaataaggtttgataaggagcaaccacatctctcccaacaagatcatttctgttttcaatcactccccatggagctattccgatagtgcaaatctttcgagatgatctggaagcatgttctttgagggcatctccaacatgttttgccacacctgtgtttactcctccagttaaaatccaggctccagttgtaactgcagctttaataagaccttttccaagcaactgcttgattcgtgggtgaagctcaaatttctgcatgcccccatgtacagagataacaagtttgggtaactccatttgccattctttaagcagaagttgcagaatgacttcaggtttggtgtcatatgatagcctcacatacttagctctgtaggaatgagaacccccttgaaaatttatgactccataagcatccgttgggctctgttctgtatgcttttccacagaccattcttctattgcctgattaaaatggtcacccaatttcacatctgagtatttcatggcaagacttgcagtaaaacaagcatgttgcttgaccaagcgaccacaaaaacacctgacgagttgctgacaaatttgacatcctggaaggcatctgtgagggtccttggaacttggtataatatatacacattccctcttggtcaaagtgctttctatccaggatttctgggactgcaatccgagtactttaggaggcctcatggatcacctgaggcc

SEQ ID NO: 17407 - RNA, 1029 nt, Homo sapiens
  source 1..1029: mol_type = other RNA
tcaggccaggcacagtggctcacgtctgtaatcccagcactttgggaggttgaggggggcggatcacttcaggtcaggagttggagtccagcctggccaacatgatgaaaccccatctctgctaaaaatacaaaaattagcaaggcatggtggtgcacacctgtgactctagctactcgggaggcggaggcaggagaattgcttgaaccctggaggcagaggttgcagtgaattgagaccacaccactgcactccagcctgggtgacagagtgagaccctgcctcaaaacaaaacaaaacaaccatcctgcacaattatgagtgagagtaaatccaacacatctcacagcatcttgggaaaatgataaggctcactttcttctttcccttcagtgtgaactcatgtaataacttcagagaaaggcatttccctgctgtctggaagttgaactccttctacaaactggtggagcttgctgcccagtcctgtgccctccgagctgaggggaaggcgtggggattttctgttctactgaaatggcaggattatgtcatagcagtggttttgagtgtttagaggtagtgttattttaattatttttctaactctggtttaaataaaaacttacaaatcaggaaagaactggctatctgtatgttaaaaaaattaagagagggctgggtgcagtgtctcacgcctgtaatcccaacactttgggaggccgaggtgggtggatcacgaagtcaggagatcgagaccatcctggccaaccaacatggtgaaaccccgtctctactaaaaatacaaaaattagctgggcgtggtggcgtgcgcctgtaatcccagctacgcaggaggctgaggcaggagaatcgcttgaacctgggaggcggaggttgcagtgaaccgagattgtgccagtgcactccagcctggccaacagaacaagactccgtcttaaaaaaaaaaaaaggagagagagagagggaacattgactcttaccttgtaccatcccaaaaattcattt

SEQ ID NO: 17408 - RNA, 5738 nt, Homo sapiens
  source 1..5738: mol_type = other RNA
tcaggccaggcacagtggctcactcattctaagtgtgctgcaaagcccctttagtgaagaaatctacttctcaaacataatggtcagaataatgaagggtaacatgattattcacatttaatcgacttcatttacatagataaagcctaaaggaaaaatccaatctgtatttatgtgcatgcactgatgtttaaaaatccactggaggaaaaggaaaatttagtcagcaaaatcttttctagataaatgctagaaatcattattccaagaaaagaatcctccacttttactatatgtgtgtgtgtgtgtgtgtgtgtgtgtgtgtgtgtgtactcattaaaaaatacataagagctcctccatggcttgagaatattttatgaagttataaaaatcagtattacctgtcaagtactatgttacatgtgcaatcaaaactgttgaggttacctgaataaaaaaaatccctgatgtctattacagaaagcttttaacagaacttgccttggcaatttactcctaaatcttctttttcctccagctcaatataatattgctacctaatattgtgactgcacaaaaccattttaggtaccacttgggaataagtattaagagttcaagtaaggctgggtacagtggccaacgcctgtaatcccaacactttgggaggccaaggtggaaggactgcttggggccaggagttcaagaccagcctgggtaacagagcaagaccttcaactccacaaatataaaaataaaaaattagatgtggtgacacgagcctatagtcccagctaatttgggaggctgaggtgggaaggttggttgagcccaagagttcaaggctgcagtgagctgtgatcacaccactgcactccagcctgggtgatagagcaagattctgtctaaaaaagggttcaagtaaatgcaaatgatgttttggcaaccttttctcaaaagattctgcattggaatacagactgtaatattaaactactatgtgtatattgtttctacagttgtatacaccgtagtgtcttttacaggtatataaggtcaatggccctagtctaattcagatttaaactagtgcttgccttgtaactctgcaagtgatcaataatctcttaatactgaaaatcacaaaataggataaaacgttctgttgctagtcccataaagcttactacattttttccccattctccccaaacttaggagaaacttgactaaagatgtgagataaaattatttattgtaaaaagtaaatgatcatctccccagccccattcccaaagtcacttgagcctttgcaatccaatttgagatcactttaaaaaaccttcccccgtaacatgtccttgtgtttttgttttttcctccaattaaagtgattaattggaaaggggagcattaggtgacattccttgccttgagacagctggtggtttcctacaccctgtggtggtaactccagacatggagcagctagagctgcggacagttactgctgcagacagggctgtgtcccgtgactcattatggttcagttcggtttctaaatctcccccagtaaaaatcctccccctggaaccatctgctctttggacaagcttctgccccctgaacctggtgcaatcagggtctggtctaggctttgcagagctgggaggaaatccctgggcctccagctaacgctgtccaaggtgctgaataccgtactcagtgtgttgccactggctgagctggtgcaacctttcacctctgagaaacgttttccaagacaggacagtgttatggagcatggactcaagccttgggccatctacatccgttctttctccaccaagatgagttaggcgaccttggccacgtgacccccacctttctgagccaaagcacttaaaacacataataaacattcaaaaccatagcacttagaatcaggaagtccttttatcgtttttcacagtataaggcacttattttttgatatcattctctttttttaaaggcaaaggaattacaagtgaacacactagtcatggcccatcagaatgatagatgcttatctacaaaaacatttcctgacttcttgctgaacctcttgcctctgggaaatactgctgtttgcttacttaaaaagtggtgagaaattaatatgattctctcttcccttttaaaaaattaaatttgtataaatataaggcgtacaagtgcagttttgttacacggatatattgcgaagtggtgaagtccaggcttttcctgcaaccaacaccagaaaagtgtacactgtacccatcaggtactttctcatcccttaccctcctcccacccttctgagtctccaatgtttgttccacactctatgttcatgggtacactttatgtagctcccatttatgagtgagaacatgaagtattcgactttctacttctaagttatttcacttaagataacagcctccagttccatccaggttgctgcaaaagacatggtttcattctttttagtggctgaatagtattccattatgtatacataccacatgttctttatccaatcatctgttgatgtgattcccttttctttgcatattcttggggtacttttgaatcagttcttttaagtttttggggaaggagatttggtttcattttcattactttcaattatctccattatccttctgcaaacccatgtgccacaattcagagcattgtgcatacgtaagaacagagtgagagctccttttcatttccccctggaggaacccccatcctggaatcgaagccctctgtttatgatccaagtgtcaccacatctcaagtctcaatgtgtgtgtgtgtggttttttttttttttttttgagacagagtcttgctctgttgcccaggctggagtgcagtggcatgatcttggctcactgcaacctctgcctcctgagttccagcgatctcctgcctcagcctcccgagtagctgggattacaggtgtgcaccagcatgcctggctaatttttgtatttttagtagagatggagtttcaccatgttggccaggctgttctcaaactcctgatctcaggtgatctgcccgtctcagcctcccaaagtgctgggattacaggcgtaagccactgtgcctggcccaatgtgtggttgttattagctatgccctttaccgaactccttttcttgacctcctatacctacacctgttgtaaagaaacaaatacaaaacaggatttcagcaaaacactaaaagaagagcgttctagttttttaaaaaatttaattttcttgtggcacataacaatgaactctggtgtcaccagcctattgtataattaacttctcgtcttttgttccttatgaatttacatatttaattatctttccatttaatttcccatggttttgctacgttgactaaactctgtaatgagaaagtcttttaatttaatagactttgcaggtcatgtgtaaccagctttggaaatcattttaggattactgagtgctgtttcataatgctgtatatttttcctgccaggatttggagtacctaggttatttgtccaccagaacaatggctgtaaaggagaaaattgagcagtggtcagaagctgctgagaagatgcggtaaaacaggttacataaaaaacaatgctggtttgaaataacctatgcgcttttgtcaagggattttgcattagtgcatttagtccaagtcagggccaattcagaggatgtggctgaaggcaccgttttggccttttttgtttcttttgagagctctgcatacattcccacttttcctgtcaaagtggacaaaatgaagagtctcatgagtggaggggcattctgatcccaagagaccacccatctgtggagtggctacacagccagaatgtggatgtgaaccaactcaacgtgctccccagagactgaagaagcggcgttttagagctttggtttcagtctcttggaggagattttcagaaatggccaatttatgtgcaaaggtgacttttctaggcacccaggaaggcaaatttaagctccgagctgtatcaactgcattctgttcctatcatcagaagtctcagaattgaacagtaaatggtgcctacttggctccttgtcaaaataagtctgcatggctctcacaacaagggagacagctgttcgttccgctggaaaggaaaggagatgaactttgttttgcctagcgttttgggaatcgtgaccacaatttaatacaatcaggtgtagtttgtttaaggaattatcaaagatcatacttggctgtcagattggaattgaggtcgataggcagactttgaccatatgctaaccagaatacaatccaattcaaaagtggagttgagaaacacagcattaggagaatttattcaaacatccatgcagagatagtctaatattttaaaaactgatttccaggatcattcgctccattttaaaggaaatgcagttctattttgaatataattcaggacagggccccagctctctgatttatgcaaaaggacataaattcacaaacctgcctgggctatttttatatttcagcaagaggttgtgtgcagctgctgtttctggcaaaataaaaaaatagtgcaagtgaaaagtgaacgggaacgggaaggagcgtcattttttcttgatcaaatccatgagatcgtcttctattcctttctcactcagctcatctagactgtagtatcggtgaacaattttctcggcggtgaccaccacgactcggagcccgtgggggtctctgcccagctggcatccaatggcagatgacaccaccatgtcgaggttctggtaggtacccccggcattcctgtggtagtggcctgagaacacgactttgacacctgcgtggatgaacttgtctgccaacttcttccgagtggacttgctgaggttgaagtagtagtcgtcgtcctcgtcgatgctctccaggaacagcgggatgtgctggaagacgatggcatgctggcagtgccgctgcctcgcgatgctcagctgctcgtccagccactggtcctgagcctgcttcaggctggggcatttggaggggttctcgtagaactgggagttgaggaccaggaacaggacgcccccgacccagaagctgaagtagtcatctccccaagtccggcagaactcctcgacggtctcggccgtgggggtgttgccaatgtcatggttgccgctgacaaggaccagtgggatggccctgtccactgccctaagcactcgcttcaggtcctccgtctgctccgtccgccacggcttccctggcatggcgtggatgaggtcgccgcacagaacgaagaatttgggtttggggttcagcttgttgatggcctggacggcttgctcagttagacggatctcctgttcccattcgtcaccgccattgtcacagtccccagtggaccaggccttgatcagcccaaactgtgggtctgcgcccaggatgaagtagaatgggcctttccattcgctttccttttctgcgggaaacgcggccagggtcctgcccctggctctgtggaaaacaccccccgcctctgcagccgacatggcgagcgagtttctggccttcacttagaacactgcgtgggtggaagccgcgcgacttcacacagaacaaccgctggacctgtcccgctttgggcgacgccctttgatctc

SEQ ID NO: 17409 - RNA, 5312 nt, Homo sapiens
  source 1..5312: mol_type = other RNA
tcaggccaggcacagtggctcactcattctaagtgtgctgcaaagcccctttagtgaagaaatctacttctcaaacataatggtcagaataatgaagggtaacatgattattcacatttaatcgacttcatttacatagataaagcctaaaggaaaaatccaatctgtatttatgtgcatgcactgatgtttaaaaatccactggaggaaaaggaaaatttagtcagcaaaatcttttctagataaatgctagaaatcattattccaagaaaagaatcctccacttttactatatgtgtgtgtgtgtgtgtgtgtgtgtgtgtgtgtgtgtactcattaaaaaatacataagagctcctccatggcttgagaatattttatgaagttataaaaatcagtattacctgtcaagtactatgttacatgtgcaatcaaaactgttgaggttacctgaataaaaaaaatccctgatgtctattacagaaagcttttaacagaacttgccttggcaatttactcctaaatcttctttttcctccagctcaatataatattgctacctaatattgtgactgcacaaaaccattttaggtaccacttgggaataagtattaagagttcaagtaaggctgggtacagtggccaacgcctgtaatcccaacactttgggaggccaaggtggaaggactgcttggggccaggagttcaagaccagcctgggtaacagagcaagaccttcaactccacaaatataaaaataaaaaattagatgtggtgacacgagcctatagtcccagctaatttgggaggctgaggtgggaaggttggttgagcccaagagttcaaggctgcagtgagctgtgatcacaccactgcactccagcctgggtgatagagcaagattctgtctaaaaaagggttcaagtaaatgcaaatgatgttttggcaaccttttctcaaaagattctgcattggaatacagactgtaatattaaactactatgtgtatattgtttctacagttgtatacaccgtagtgtcttttacaggtatataaggtcaatggccctagtctaattcagatttaaactagtgcttgccttgtaactctgcaagtgatcaataatctcttaatactgaaaatcacaaaataggataaaacgttctgttgctagtcccataaagcttactacattttttccccattctccccaaacttaggagaaacttgactaaagatgtgagataaaattatttattgtaaaaagtaaatgatcatctccccagccccattcccaaagtcacttgagcctttgcaatccaatttgagatcactttaaaaaaccttcccccgtaacatgtccttgtgtttttgttttttcctccaattaaagtgattaattggaaaggggagcattaggtgacattccttgccttgagacagctggtggtttcctacaccctgtggtggtaactccagacatggagcagctagagctgcggacagttactgctgcagacagggctgtgtcccgtgactcattatggttcagttcggtttctaaatctcccccagtaaaaatcctccccctggaaccatctgctctttggacaagcttctgccccctgaacctggtgcaatcagggtctggtctaggctttgcagagctgggaggaaatccctgggcctccagctaacgctgtccaaggtgctgaataccgtactcagtgtgttgccactggctgagctggtgcaacctttcacctctgagaaacgttttccaagacaggacagtgttatggagcatggactcaagccttgggccatctacatccgttctttctccaccaagatgagttaggcgaccttggccacgtgacccccacctttctgagccaaagcacttaaaacacataataaacattcaaaaccatagcacttagaatcaggaagtccttttatcgtttttcacagtataaggcacttattttttgatatcattctctttttttaaaggcaaaggaattacaagtgaacacactagtcatggcccatcagaatgatagatgcttatctacaaaaacatttcctgacttcttgctgaacctcttgcctctgggaaatactgctgtttgcttacttaaaaagtggtgagaaattaatatgattctctcttcccttttaaaaaattaaatttgtataaatataaggcgtacaagtgcagttttgttacacggatatattgcgaagtggtgaagtccaggcttttcctgcaaccaacaccagaaaagtgtacactgtacccatcaggtactttctcatcccttaccctcctcccacccttctgagtctccaatgtttgttccacactctatgttcatgggtacactttatgtagctcccatttatgagtgagaacatgaagtattcgactttctacttctaagttatttcacttaagataacagcctccagttccatccaggttgctgcaaaagacatggtttcattctttttagtggctgaatagtattccattatgtatacataccacatgttctttatccaatcatctgttgatgtgattcccttttctttgcatattcttggggtacttttgaatcagttcttttaagtttttggggaaggagatttggtttcattttcattactttcaattatctccattatccttctgcaaacccatgtgccacaattcagagcattgtgcatacgtaagaacagagtgagagctccttttcatttccccctggaggaacccccatcctggaatcgaagccctctgtttatgatccaagtgtcaccacatctcaagtctcaatgtgtgtgtgtgtggttttttttttttttttttgagacagagtcttgctctgttgcccaggctggagtgcagtggcatgatcttggctcactgcaacctctgcctcctgagttccagcgatctcctgcctcagcctcccgagtagctgggattacaggtgtgcaccagcatgcctggctaatttttgtatttttagtagagatggagtttcaccatgttggccaggctgttctcaaactcctgatctcaggtgatctgcccgtctcagcctcccaaagtgctgggattacaggcgtaagccactgtgcctggcccaatgtgtggttgttattagctatgccctttaccgaactccttttcttgacctcctatacctacacctgttgtaaagaaacaaatacaaaacaggatttcagcaaaacactaaaagaagagcgttctagttttttaaaaaatttaattttcttgtggcacataacaatgaactctggtgtcaccagcctattgtataattaacttctcgtcttttgttccttatgaatttacatatttaattatctttccatttaatttcccatggttttgctacgttgactaaactctgtaatgagaaagtcttttaatttaatagactttgcaggtcatgtgtaaccagctttggaaatcattttaggattactgagtgctgtttcataatgctgtatatttttcctgccaggatttggagtacctaggttatttgtccaccagaacaatggctgtaaaggagaaaattgagcagtggtcagaagctgctgagaagatgcggtaaaacaggttacataaaaaacaatgctggtttgaaataacctatgcgcttttgtcaagggattttgcattagtgcatttagtccaagtcagggccaattcagaggatgtggctgaaggcaccgttttggccttttttgtttcttttgagagctctgcatacattcccacttttcctgtcaaagtggacaaaatgaagagtctcatgagtggaggggcattctgatcccaagagaccacccatctgtggagtggctacacagccagaatgtggatgtgaaccaactcaacgtgctccccagagactgaagaagcggcgttttagagctttggtttcagtctcttggaggagattttcagaaatggccaatttatgtgcaaaggtgacttttctaggcacccaggaaggcaaatttaagctccgagctgtatcaactgcattctgttcctatcatcagaagtctcagaattgaacagtaaatggtgcctacttggctccttgtcaaaataagtctgcatggctctcacaacaagggagacagctgttcgttccgctggaaaggaaaggagatgaactttgttttgcctagcgttttgggaatcgtgaccacaatttaatacaatcaggtgtagtttgtttaaggaattatcaaagatcatacttggctgtcagattggaattgaggtcgataggcagactttgaccatatgctaaccagaatacaatccaattcaaaagtggagttgagaaacacagcattaggagaatttattcaaacatccatgcagagatagtctaatattttaaaaactgatttccaggatcattcgctccattttaaaggaaatgcagttctattttgaatataattcaggacagggccccagctctctgatttatgcaaaaggacataaattcacaaacctgcctgggctatttttatatttcagcaagaggttgtgtgcagctgctgtttctggcaaaataaaaaaatagtgcaagtgaaaagtgaacgggaacgggaaggagcgtcattttttcttgatcaaatccatgagatcgtcttctattcctttctcactcagctcatctagactgtagtatcggtgaacaattttctcggcggtgaccaccacgactcggagcccgtgggggtctctgcccagctggcatccaatggcagatgacaccaccatgtcgaggttctggtaggtacccccggcattcctgtggtagtggcctgagaacacgactttgacacctggcatggcgtggatgaggtcgccgcacagaacgaagaatttgggtttggggttcagcttgttgatggcctggacggcttgctcagttagacggatctcctgttcccattcgtcaccgccattgtcacagtccccagtggaccaggccttgatcagcccaaactgtgggtctgcgcccaggatgaagtagaatgggcctttccattcgctttccttttctgcgggaaacgcggccagggtcctgcccctggctctgtggaaaacaccccccgcctctgcagccgacatggcgagcgagtttctggccttcacttagaacactgcgtgggtggaagccgcgcgacttcacacagaacaaccgctggacctgtcccgctttgggcgacgccctttgatctc

SEQ ID NO: 17410 - RNA, 1829 nt, Homo sapiens
  source 1..1829: mol_type = other RNA
tcaggccaggcacagtggctcactcctacaatcctagcactttgggaggctgagacaggtagatcacttgaggccagagttcaagaccagcctggccaacacggcgaaaccccgtctctactaaaattacaaaagtagccaggcatggtggtgcgtgcctgtaatcccagctactccagaggctaaggcacaagaatcacctgaacctgggaggcggaggttccaacgagccaagattacaccactgcactccagcctgagcaacagagtgcgactctgactcaaaaataataaaatcaatgatgatggctaggttaatagatcacaaaagaacatacatgaaatcaaatctcaccatggcaacaacctccagaaacaaggactataggtagatttatctctgtgattaacacagtgtcttacccacagtaggtgcttaataaatattttttattcattgctctctaatcctattttctttagtgccagtgacaacgtctcagtataaacatttccatcctttaatactgtatttatttccttagcagttttccttttcttccattctatcttctgacccaatgcaatgaaaacttctcaaaatatcagtcaaaacttcgttgtttttacttcaacactgaaattacagccagtaagagtaaggctaggcctacctcttgagacataaacacaagcatgaggattatggacagaaacaaatccgtattccaggaacagccgttgattatcgtgagggccgtaacagatgaatacctcttcatgctttctccaacgtgaagtcgttctaatttcgtaagaatgagtttcttcattaaacgctgcttttacctggacatgtgggctatgattcagcaggtccaggtacggagcgagtgcacaggtgtccggctctgcagaaaggcattcccgctgcctgggcctcaggtacacggctctggtgttgacggtgcaccaagcccacagcagggcactgtagctgaagatgctgtcaacagcctccgcaaacagaggctgcagagaagagaaaaagtctctggaggaagcaaagaactcctgcacgtgggctctctgctcttcagcctttgcttttaaagatttgggaagaaggttcaccacttccggctccaaacaaacagggcaggtatacgccttgggtaaaatctccaggtaaggcttccaaagagatcggtgcccagcatgcttttctgaaactaaaaaggtgcacagcgccagcagaggagatggaggaggcttccacttagtaatgtatgcccctaagtagcttcgaatcactgtgtccgtggtgagcaggcaactctcaggcaacgaaataatcatctgtccctcctgcagggatgtttgactcatcagccctcttcctgtacctggaaaacaagcaggcgctaagtttgaatcttgaaacttcctagctttcagccacttcctcagctctataaattcagacttgtggctctcattcactcctcttgattcagaacttccgcagagttttcgtcttctgatccggcttgttctcccttttcctttctgcatgctaaaactgtagtttcttttttctgaaatacagttctattttttcaaaaaggacaaaactgtaatttctgtggaaatgctcaatctaggcgccggcggccgcttccaagatggaggctgcagtgggcgggcccaaggcacgtggaaataccaaacagccccagatgaaggcaagttaaaggaaccggccaaaactgcagagggagaggctgaaggctgtcgcgcctgcctggtgtccttaagcaatccaagtc

SEQ ID NO: 17411 - RNA, 5866 nt, Homo sapiens
  source 1..5866: mol_type = other RNA
tcaggccaggcacagtggctcactcctgtaatcccagcactttgggaggccgaggcaggcggatcacctgaggtcaggagttcgagaccagcctgaccaacacggcgaaaccccatctctactaaaaatacaaaaaaattgccaggcgtggtggtacacacctgtaatcccagctactcgggaggctgaagcaggagaattgcttgaacccaggaggtggaggttgcagtgagctgagattgcaccactgcactccggggcacctgagcaagactccgtctcaaaacaacgacgacaacaacaacaacaacaaaaaacaagtgatatagagaacttgtgcttgctgttaagggaatgcaatactttgggccagtgaaaaatacctagaaattgatcaatatgaaatgtagcccaaaggagtcatatatcttcaaaatctaatgagatcaccctgtttttggcttattcccaaagctgtctctgtgtttacagttggagagaaaaggttagtggagtggcttttataaataagattaattattacagctataactgaagtctccaggcaggaggctttacaactcagtcagtgctatattgtgcctccattttacttccaggacctgactggcataccgttcttgatgctttctacaaatataaaaatctctgcaactgtttagataaaattggaagaaaaaaaaaaggcaaagctgaccataaaaacaacagggggttgggggaggcagagaaaaaggacaagtatacattacatagtttaggaaagtccaggattattgcagaaattaaaatgaacaaggaaaagggcaggcaccaataaaagcacctaaagctagcaaatgcctaaactggtttatttagagtccctccccacaatgttcataggggaggaaaataatgtaatttgaaaagcatcaaaactaaacaaatgcacactgaccttagaaaataagattttgaatttcatcatgatacccttttttcctataaaatttactttttcactctgaaagacttcttcatggtggatttgcccttgcccggcaattttacttcctttcttgcactggttgcaggcttctttgaggagccaccactaggtttcttgatgactgtggatgagggtctggtcttcttggcaggcgttttggccttaggaggtgctttcttaggcaagggcctagctttcccccgctgggcagctgagactttaggtgcaggtttggaccctctctgcttcacagatgcggccttccctggggacttggctggggttttcttctgcaaccttctcttaggtggcggctcttcatcctcagagtcttcttctgatgactcatcttcatcttcatcctcatctctagaatcatctggctctttcttcggaaacagaactcctgggctgggataatagggaaaacagagctggaaggtgccactgaaccctttcccagagatctgttccatccacccattcttttcgcatttctgcagggtttttttcagcaaatgcatttgatagttagaattggttcctgggtgattctctaggacatacttcttcagagcagtggtagagcaggtcttcggctcattcatggcagcaatggcagacaagattgcatattccatcaggcttccaccaagcaggggtttctcccctgatttcttcagctggaatgtccccgaagcacctttgccagttatctgttctaactggcccctctctactgctctctgcagagcgttcttcaacagctgaggcctgatgtccactctaagcttaggataatactgagacacatatttcctgatgagactgtaggaagcttctttaggttcacaaaggcgagtaaaggccagtgggaggacatcctccaattttacttgtggttctggatccactgcagagctcctattctttctgtttctggatttctgaggtgtttttcttgatttctgaaccacaacaaaacttccagaagcaccttttcctttaacctgtttgatgactcctctatttaattctcttttcagtgcttgtttaaggagataaccccttctctccagctccagagaaggatacttatggatgatgtattttcgaatagcaaccactgatgcaccactcttctggaagcatgccttaatggcctcagttaagattgcatccatcttgggacgtggggaagaagccatcggtgtttgtttctgggccctggctagctggctggcagaaagggtagcccaggaaggaattgtttttttcactttcttctccttttctttagactgatctttctcactttaaaacaaagaattgttattatagaagataagctctctagaaagacgtataaagtcagaaggaggaaaagaccagggagggataaaaattaatgctttaatttatttacaggctaagatgacatgtaccataagcaaaattttacaaaataaatcttctttaaaaactgggtactataaatgaattaaaaaggtatttttctcttagctgcaggagaaaggagtcacataaattagcactggtataagggctcagtacataagacaaatgagaattttaaaatgcacattagttaacaattacaacagatgcaatatggtatagtggaaaaaactcaagctcttaaagtcagaaaacctttgtttgtattttcactcaaacatttactagctagctatatgatcttagtaaatgatgtgagtctttctcctcagctataaaacagtaatatagaaccaactatttcccaaggtgttgcaagaattataagagtatgtttatcaaaacaattttgtgagatttaaagcattatgtaaattttattctgagtatataacagtactctgtgcacctaataggtgcattagaacatttaacaacagacgataggctgggtgcagtggctcatgcctgtaatcccagcaatttaggaggctgaggagggaggacagcttgaggccaggagttcaagcccaacctagccaacatagtgagacgccatctccattaaacacacacacacacacacaaacacacccacacccacacacgatagttgctataaattccacagaccttagctatacttatgaaactcagataaagaataccctgaagattatagctagaaggtatagttattactaagttattcttttatggtcatgtgctgtgtaacaatatttggtcaacagaccacatatacaatggtggtcccttaagattataatggaactgaaaacctcctattacctggttaacatgatagctgtggtaatatcacagcgcagcacgttactcacttgtttgtggtgacattggtgtaaacaaacctacagtgctgccagtcatacaaaaatatagcatattggctgggcgcggtgactcatgcctgtaatcccagcactttgggaggccaaggtgggcggatcacaaggtcaaaagattgagaccatcctggccaacatggtgaaacccccgtctctcctgaaaatacaaaaattagctaggtgtggaggtgcacgcctgtagtcccagctacttggcaggttgaggcaggagaatcgcttgaacctgggaggtggaggttgcagtgagcccagatcgcgccactgcactccacactccaacctgggtgacagagtaagactccatctcaaaaaaaaaaaaaaagcacattacaattatacataatacctgataataaacagctatgctactagtttatgtgtttactatactatactttttatcattagagtatatgttttctacctacaaaaaaaaagttaactgtaaaacagcctcaagcaggtccttcagaaggtattccaaaagacagcactgttatcataggaaatgacaggtccatgtgtgttgctgcccctgaaggccttgagtgggacaagatctggaggtggaagacagtgatattgatgaccctgaccttgtgcaggcctaggttaaggtgtgtgtatgtgtcttagttttgtttttttataaatatgaggtctcacaacgttgcccaatctagattcaaatttcaggactcaagcaatccccccacctcagcttcctaagtagctagggctacagctgtgcaccattgcgtccggcttgtgtctttgtttttggtaaagttttaaaagtttttaaaaataaaaactttttagttttaaaagttgctaaaaataaaaactttttagttttaaaagttgcacacagtagtcctaggcctttgcattcacttaccactcactcactcacccaaacaacttccaatcctttaaggtccattcatggtaggtgtcctacacaggtataccattttttatcttttatattatatttttactgtaccttttctatgtttaaatacacaaatacttaccgttgtgttataactgcctacagtatttagtacagtaacatgctgtacaggtttgtagcctagaagcaacagactatcccataaagcctaggtatgtagtaggctgtaccacgtaggtttgtgtaagtacactttatgatgttggcacgatgatgaaatcgcctaaagatgtatctctcagaatgtatacccattgttaagcaatgcatgactatagttaaaagcaatttctaactgttctgaccaattatgaaaagagtggaatgaatactatcagctctcctgcaaaaaaaaaaaaaaaaaaattaaaaattaaaaagtaactgccatcactttatatagatacacatcaatagcaaattttactttcagattctcaaagccaattcttcaactgaatatttcatcaaacatatatagacttttaggtcacactaccaatggcttgatacaaatcaatgccttctaacataagcacacaaaaacaacccactcctggcacagaagtaggaataaaatagtgaaatgtcttctaggtcagatttttatagttatgtttcatttcttattgaagtcttgccaatgcttaaaatatcagatactcccacaataaattacaagctcaaaaacacattccaaagccaatgacaaagacttttggattattcaaaccattgtgttctgctaactacagcatattctaacaggtcaaacaactatataataaacctatttcaaatggtaattctaaaaattaaatccaaatagcaaatacctagcataaaccaatgttataacactttaaaacaatctaatctaaagtccttttacacattcttcaaatataaatagcaagaagacataactccttactcctttttggtttcctcagaagacttattttcttccttctcttcattctcaggttccccctttggctgctctgcctcactcgaagtagcaggtggagtttcattctcttgttcttctacagtggagacagattcctctgaacttatgtctggttctggcttttcttcctccccttcagcaagcttgcttttgggaggagtttcccgggtagaattcacagttcgacgaatcggcatggtgctatcttctaccttctaacttgtccgcgtggatcagctgagctcctactataagtgggagtgccttaggatggacgagttcaccttgagacgtatcagtcgccattttaaataatttctaggcccgagtacaggttacactctgaagcctctgctgttaaccacaaggatttttcctaatggtttcagtgtggtgaagaatcaacctctgcgttcggccggtcctggcgcccgcgtcccgcacggcctctcggcgccgctcccgccgccgctagtcgcctccgccaccgctgtcctccagtcccagccgccgag

SEQ ID NO: 17412 - RNA, 5046 nt, Homo sapiens
  source 1..5046: mol_type = other RNA
tcaggccaggcacagtggctcactcctgtaatcccagcactttgggaggccgaggcaggcggatcacctgaggtcaggagttcgagaccagcctgaccaacacggcgaaaccccatctctactaaaaatacaaaaaaattgccaggcgtggtggtacacacctgtaatcccagctactcgggaggctgaagcaggagaattgcttgaacccaggaggtggaggttgcagtgagctgagattgcaccactgcactccggggcacctgagcaagactccgtctcaaaacaacgacgacaacaacaacaacaacaaaaaacaagtgatatagagaacttgtgcttgctgttaagggaatgcaatactttgggccagtgaaaaatacctagaaattgatcaatatgaaatgtagcccaaaggagtcatatatcttcaaaatctaatgagatcaccctgtttttggcttattcccaaagctgtctctgtgtttacagttggagagaaaaggttagtggagtggcttttataaataagattaattattacagctataactgaagtctccaggcaggaggctttacaactcagtcagtgctatattgtgcctccattttacttccaggacctgactggcataccgttcttgatgctttctacaaatataaaaatctctgcaactgtttagataaaattggaagaaaaaaaaaaggcaaagctgaccataaaaacaacagggggttgggggaggcagagaaaaaggacaagtatacattacatagtttaggaaagtccaggattattgcagaaattaaaatgaacaaggaaaagggcaggcaccaataaaagcacctaaagctagcaaatgcctaaactggtttatttagagtccctccccacaatgttcataggggaggaaaataatgtaatttgaaaagcatcaaaactaaacaaatgcacactgaccttagaaaataagattttgaatttcatcatgatacccttttttcctataaaatttactttttcactctgaaagacttcttcatggtggatttgcccttgcccggcaattttacttcctttcttgcactggttgcaggcttctttgaggagccaccactaggtttcttgatgactgtggatgagggtctggtcttcttggcaggcgttttggccttaggaggtgctttcttaggcaagggcctagctttcccccgctgggcagctgagactttaggtgcaggtttggaccctctctgcttcacagatgcggccttccctggggacttggctggggttttcttctgcaaccttctcttaggtggcggctcttcatcctcagagtcttcttctgatgactcatcttcatcttcatcctcatctctagaatcatctggctctttcttcggaaacagaactcctgggctgggataatagggaaaacagagctggaaggtgccactgaaccctttcccagagatctgttccatccacccattcttttcgcatttctgcagggtttttttcagcaaatgcatttgatagttagaattggttcctgggtgattctctaggacatacttcttcagagcagtggtagagcaggtcttcggctcattcatggcagcaatggcagacaagattgcatattccatcaggcttccaccaagcaggggtttctcccctgatttcttcagctggaatgtccccgaagcacctttgccagttatctgttctaactggcccctctctactgctctctgcagagcgttcttcaacagctgaggcctgatgtccactctaagcttaggataatactgagacacatatttcctgatgagactgtaggaagcttctttaggttcacaaaggcgagtaaaggccagtgggaggacatcctccaattttacttgtggttctggatccactgcagagctcctattctttctgtttctggatttctgaggtgtttttcttgatttctgaaccacaacaaaacttccagaagcaccttttcctttaacctgtttgatgactcctctatttaattctcttttcagtgcttgtttaaggagataaccccttctctccagctccagagaaggatacttatggatgatgtattttcgaatagcaaccactgatgcaccactcttctggaagcatgccttaatggcctcagttaagattgcatccatcttgggacgtggggaagaagccatcggtgtttgtttctgggccctggctagctggctggcagaaagggtagcccaggaaggaattgtttttttcactttcttctccttttctttagactgatctttctcactttaaaacaaagaattgttattatagaagataagctctctagaaagacgtataaagtcagaaggaggaaaagaccagggagggataaaaattaatgctttaatttatttacaggctaagatgacatgtaccataagcaaaattttacaaaataaatcttctttaaaaactgggtactataaatgaattaaaaaggtatttttctcttagctgcaggagaaaggagtcacataaattagcactggtataagggctcagtacataagacaaatgagaattttaaaatgcacattagttaacaattacaacagatgcaatatggtatagtggaaaaaactcaagctcttaaagtcagaaaacctttgtttgtattttcactcaaacatttactagctagctatatgatcttagtaaatgatgtgagtctttctcctcagctataaaacagtaatatagaaccaactatttcccaaggtgttgcaagaattataagagtatgtttatcaaaacaattttgtgagatttaaagcattatgtaaattttattctgagtatataacagtactctgtgcacctaataggtgcattagaacatttaacaacagacgataggctgggtgcagtggctcatgcctgtaatcccagcaatttaggaggctgaggagggaggacagcttgaggccaggagttcaagcccaacctagccaacatagtgagacgccatctccattaaacacacacacacacacacaaacacacccacacccacacacgatagttgctataaattccacagaccttagctatacttatgaaactcagataaagaataccctgaagattatagctagaaggtatagttattactaagttattcttttatggtcatgtgctgtgtaacaatatttggtcaacagaccacatatacaatggtggtcccttaagattataatggaactgaaaacctcctattacctggttaacatgatagctgtggtaatatcacagcgcagcacgttactcacttgtttgtggtgacattggtgtaaacaaacctacagtgctgccagtcatacaaaaatatagcatattggctgggcgcggtgactcatgcctgtaatcccagcactttgggaggccaaggtgggcggatcacaaggtcaaaagattgagaccatcctggccaacatggtgaaacccccgtctctcctgaaaatacaaaaattagctaggtgtggaggtgcacgcctgtagtcccagctacttggcaggttgaggcaggagaatcgcttgaacctgggaggtggaggttgcagtgagcccagatcgcgccactgcactccacactccaacctgggtgacagagtaagactccatctcaaaaaaaaaaaaaaagcacattacaattatacataatacctgataataaacagctatgctactagtttatgtgtttactatactatactttttatcattagagtatatgttttctacctacaaaaaaaaagttaactgtaaaacagcctcaagcaggtccttcagaaggtattccaaaagacagcactgttatcataggaaatgacaggtccatgtgtgttgctgcccctgaaggccttgagtgggacaagatctggaggtggaagacagtgatattgatgaccctgaccttgtgcaggcctaggttaaggtgtgtgtatgtgtcttagttttgtttttttataaatatgaggtctcacaacgttgcccaatctagattcaaatttcaggactcaagcaatccccccacctcagcttcctaagtagctagggctacagctgtgcaccattgcgtccggcttgtgtctttgtttttggtaaagttttaaaagtttttaaaaataaaaactttttagttttaaaagttgctaaaaataaaaactttttagttttaaaagttgcacacagtagtcctaggcctttgcattcacttaccactcactcactcacccaaacaacttccaatcctttaaggtccattcatggtaggtgtcctacacaggtataccattttttatcttttatattatatttttactgtaccttttctatgtttaaatacacaaatacttaccgttgtgttataactgcctacagtatttagtacagtaacatgctgtacaggtttgtagcctagaagcaacagactatcccataaagcctaggtatgtagtaggctgtaccacgtaggtttgtgtaagtacactttatgatgttggcacgatgatgaaatcgcctaaagatgtatctctcagaatgtatacccattgttaagcaatgcatgactatagttaaaagcaatttctaactgttctgaccaattatgaaaagagtggaatgaatactatcagctctctcctttttggtttcctcagaagacttattttcttccttctcttcattctcaggttccccctttggctgctctgcctcactcgaagtagcaggtggagtttcattctcttgttcttctacagtggagacagattcctctgaacttatgtctggttctggcttttcttcctccccttcagcaagcttgcttttgggaggagtttcccgggtagaattcacagttcgacgaatcggcatggtgctatcttctaccttctctgcgttcggccggtcctggcgcccgcgtcccgcacggcctctcggcgccgctcccgccgccgctagtc

SEQ ID NO: 17413 - RNA, 2598 nt, Homo sapiens
  source 1..2598: mol_type = other RNA
tcaggccaggcacagtggctcactcctgtaatcccagcactttgggaggccgaggcaggcggatcacctgaggtcaggagttcgagaccagcctgaccaacacggcgaaaccccatctctactaaaaatacaaaaaaattgccaggcgtggtggtacacacctgtaatcccagctactcgggaggctgaagcaggagaattgcttgaacccaggaggtggaggttgcagtgagctgagattgcaccactgcactccggggcacctgagcaagactccgtctcaaaacaacgacgacaacaacaacaacaacaaaaaacaagtgatatagagaacttgtgcttgctgttaagggaatgcaatactttgggccagtgaaaaatacctagaaattgatcaatatgaaatgtagcccaaaggagtcatatatcttcaaaatctaatgagatcaccctgtttttggcttattcccaaagctgtctctgtgtttacagttggagagaaaaggttagtggagtggcttttataaataagattaattattacagctataactgaagtctccaggcaggaggctttacaactcagtcagtgctatattgtgcctccattttacttccaggacctgactggcataccgttcttgatgctttctacaaatataaaaatctctgcaactgtttagataaaattggaagaaaaaaaaaaggcaaagctgaccataaaaacaacagggggttgggggaggcagagaaaaaggacaagtatacattacatagtttaggaaagtccaggattattgcagaaattaaaatgaacaaggaaaagggcaggcaccaataaaagcacctaaagctagcaaatgcctaaactggtttatttagagtccctccccacaatgttcataggggaggaaaataatgtaatttgaaaagcatcaaaactaaacaaatgcacactgaccttagaaaataagattttgaatttcatcatgatacccttttttcctataaaatttactttttcactctgaaagacttcttcatggtggatttgcccttgcccggcaattttacttcctttcttgcactggttgcaggcttctttgaggagccaccactaggtttcttgatgactgtggatgagggtctggtcttcttggcaggcgttttggccttaggaggtgctttcttaggcaagggcctagctttcccccgctgggcagctgagactttaggtgcaggtttggaccctctctgcttcacagatgcggccttccctggggacttggctggggttttcttctgcaaccttctcttaggtggcggctcttcatcctcagagtcttcttctgatgactcatcttcatcttcatcctcatctctagaatcatctggctctttcttcggaaacagaactcctgggctgggataatagggaaaacagagctggaaggtgccactgaaccctttcccagagatctgttccatccacccattcttttcgcatttctgcagggtttttttcagcaaatgcatttgatagttagaattggttcctgggtgattctctaggacatacttcttcagagcagtggtagagcaggtcttcggctcattcatggcagcaatggcagacaagattgcatattccatcaggcttccaccaagcaggggtttctcccctgatttcttcagctggaatgtccccgaagcacctttgccagttatctgttctaactggcccctctctactgctctctgcagagcgttcttcaacagctgaggcctgatgtccactctaagcttaggataatactgagacacatatttcctgatgagactgtaggaagcttctttaggttcacaaaggcgagtaaaggccagtgggaggacatcctccaattttacttgtggttctggatccactgcagagctcctattctttctgtttctggatttctgaggtgtttttcttgatttctgaaccacaacaaaacttccagaagcaccttttcctttaacctgtttgatgactcctctatttaattctcttttcagtgcttgtttaaggagataaccccttctctccagctccagagaaggatacttatggatgatgtattttcgaatagcaaccactgatgcaccactcttctggaagcatgccttaatggcctcagttaagattgcatccatcttgggacgtggggaagaagccatcggtgtttgtttctgggccctggctagctggctggcagaaagggtagcccaggaaggaattgtttttttcactttcttctccttttctttagactgatctttctcatcctttttggtttcctcagaagacttattttcttccttctcttcattctcaggttccccctttggctgctctgcctcactcgaagtagcaggtggagtttcattctcttgttcttctacagtggagacagattcctctgaacttatgtctggttctggcttttcttcctccccttcagcaagcttgcttttgggaggagtttcccgggtagaattcacagttcgacgaatcggcatggtgctatcttctaccttcactgggagctccgtaat

SEQ ID NO: 17414 - RNA, 2980 nt, Homo sapiens
  source 1..2980: mol_type = other RNA
tcaggccaggcacagtggctcactcctgtaatcccagcactttgggaggccgaggcaggcggatcacctgaggtcaggagttcgagaccagcctgaccaacacggcgaaaccccatctctactaaaaatacaaaaaaattgccaggcgtggtggtacacacctgtaatcccagctactcgggaggctgaagcaggagaattgcttgaacccaggaggtggaggttgcagtgagctgagattgcaccactgcactccggggcacctgagcaagactccgtctcaaaacaacgacgacaacaacaacaacaacaaaaaacaagtgatatagagaacttgtgcttgctgttaagggaatgcaatactttgggccagtgaaaaatacctagaaattgatcaatatgaaatgtagcccaaaggagtcatatatcttcaaaatctaatgagatcaccctgtttttggcttattcccaaagctgtctctgtgtttacagttggagagaaaaggttagtggagtggcttttataaataagattaattattacagctataactgaagtctccaggcaggaggctttacaactcagtcagtgctatattgtgcctccattttacttccaggacctgactggcataccgttcttgatgctttctacaaatataaaaatctctgcaactgtttagataaaattggaagaaaaaaaaaaggcaaagctgaccataaaaacaacagggggttgggggaggcagagaaaaaggacaagtatacattacatagtttaggaaagtccaggattattgcagaaattaaaatgaacaaggaaaagggcaggcaccaataaaagcacctaaagctagcaaatgcctaaactggtttatttagagtccctccccacaatgttcataggggaggaaaataatgtaatttgaaaagcatcaaaactaaacaaatgcacactgaccttagaaaataagattttgaatttcatcatgatacccttttttcctataaaatttactttttcactctgaaagacttcttcatggtggatttgcccttgcccggcaattttacttcctttcttgcactggttgcaggcttctttgaggagccaccactaggtttcttgatgactgtggatgagggtctggtcttcttggcaggcgttttggccttaggaggtgctttcttaggcaagggcctagctttcccccgctgggcagctgagactttaggtgcaggtttggaccctctctgcttcacagatgcggccttccctggggacttggctggggttttcttctgcaaccttctcttaggtggcggctcttcatcctcagagtcttcttctgatgactcatcttcatcttcatcctcatctctagaatcatctggctctttcttcggaaacagaactcctgggctgggataatagggaaaacagagctggaaggtgccactgaaccctttcccagagatctgttccatccacccattcttttcgcatttctgcagggtttttttcagcaaatgcatttgatagttagaattggttcctgggtgattctctaggacatacttcttcagagcagtggtagagcaggtcttcggctcattcatggcagcaatggcagacaagattgcatattccatcaggcttccaccaagcaggggtttctcccctgatttcttcagctggaatgtccccgaagcacctttgccagttatctgttctaactggcccctctctactgctctctgcagagcgttcttcaacagctgaggcctgatgtccactctaagcttaggataatactgagacacatatttcctgatgagactgtaggaagcttctttaggttcacaaaggcgagtaaaggccagtgggaggacatcctccaattttacttgtggttctggatccactgcagagctcctattctttctgtttctggatttctgaggtgtttttcttgatttctgaaccacaacaaaacttccagaagcaccttttcctttaacctgtttgatgactcctctatttaattctcttttcagtgcttgtttaaggagataaccccttctctccagctccagagaaggatacttatggatgatgtattttcgaatagcaaccactgatgcaccactcttctggaagcatgccttaatggcctcagttaagattgcatccatcttgggacgtggggaagaagccatcggtgtttgtttctgggccctggctagctggctggcagaaagggtagcccaggaaggaattgtttttttcactttcttctccttttctttagactgatctttctcatcctttttggtttcctcagaagacttattttcttccttctcttcattctcaggttccccctttggctgctctgcctcactcgaagtagcaggtggagtttcattctcttgttcttctacagtggagacagattcctctgaacttatgtctggttctggcttttcttcctccccttcagcaagcttgcttttgggaggagtttcccgggtagaattcacagttcgacgaatcggcatggtgctatcttctaccttcgaggcaccgctctcattcaaaccccaccgcctaaggtggcgagtaaccagttctacgtttcccaccgggggagcgagactcaaggccgccgtcgcggagcagcaaagcgacagccgacagccccgcccgcagaaggccgcgggaaggacggcaagagcagcggagacaaagcagcgaggcgaggtagctacaggccacagcggcgaacgcgcacggcgggggagagcgcgggccgccagcgaggcggggaaagctcggaccgcggacaccgacggatgaggctggggctcggcgcggtgacagttcggggctcacgctcggcagggacaccgcggcgcccgccccggcgacggaagcagcggcggaacgcgagcctcggcgctccgcacactcaccact

SEQ ID NO: 17415 - RNA, 3105 nt, Homo sapiens
  source 1..3105: mol_type = other RNA
tcaggccaggcacagtggctcactcctgtaatcccagcactttgggaggccgaggcaggcggatcacctgaggtcaggagttcgagaccagcctgaccaacacggcgaaaccccatctctactaaaaatacaaaaaaattgccaggcgtggtggtacacacctgtaatcccagctactcgggaggctgaagcaggagaattgcttgaacccaggaggtggaggttgcagtgagctgagattgcaccactgcactccggggcacctgagcaagactccgtctcaaaacaacgacgacaacaacaacaacaacaaaaaacaagtgatatagagaacttgtgcttgctgttaagggaatgcaatactttgggccagtgaaaaatacctagaaattgatcaatatgaaatgtagcccaaaggagtcatatatcttcaaaatctaatgagatcaccctgtttttggcttattcccaaagctgtctctgtgtttacagttggagagaaaaggttagtggagtggcttttataaataagattaattattacagctataactgaagtctccaggcaggaggctttacaactcagtcagtgctatattgtgcctccattttacttccaggacctgactggcataccgttcttgatgctttctacaaatataaaaatctctgcaactgtttagataaaattggaagaaaaaaaaaaggcaaagctgaccataaaaacaacagggggttgggggaggcagagaaaaaggacaagtatacattacatagtttaggaaagtccaggattattgcagaaattaaaatgaacaaggaaaagggcaggcaccaataaaagcacctaaagctagcaaatgcctaaactggtttatttagagtccctccccacaatgttcataggggaggaaaataatgtaatttgaaaagcatcaaaactaaacaaatgcacactgaccttagaaaataagattttgaatttcatcatgatacccttttttcctataaaatttactttttcactctgaaagacttcttcatggtggatttgcccttgcccggcaattttacttcctttcttgcactggttgcaggcttctttgaggagccaccactaggtttcttgatgactgtggatgagggtctggtcttcttggcaggcgttttggccttaggaggtgctttcttaggcaagggcctagctttcccccgctgggcagctgagactttaggtgcaggtttggaccctctctgcttcacagatgcggccttccctggggacttggctggggttttcttctgcaaccttctcttaggtggcggctcttcatcctcagagtcttcttctgatgactcatcttcatcttcatcctcatctctagaatcatctggctctttcttcggaaacagaactcctgggctgggataatagggaaaacagagctggaaggtgccactgaaccctttcccagagatctgttccatccacccattcttttcgcatttctgcagggtttttttcagcaaatgcatttgatagttagaattggttcctgggtgattctctaggacatacttcttcagagcagtggtagagcaggtcttcggctcattcatggcagcaatggcagacaagattgcatattccatcaggcttccaccaagcaggggtttctcccctgatttcttcagctggaatgtccccgaagcacctttgccagttatctgttctaactggcccctctctactgctctctgcagagcgttcttcaacagctgaggcctgatgtccactctaagcttaggataatactgagacacatatttcctgatgagactgtaggaagcttctttaggttcacaaaggcgagtaaaggccagtgggaggacatcctccaattttacttgtggttctggatccactgcagagctcctattctttctgtttctggatttctgaggtgtttttcttgatttctgaaccacaacaaaacttccagaagcaccttttcctttaacctgtttgatgactcctctatttaattctcttttcagtgcttgtttaaggagataaccccttctctccagctccagagaaggatacttatggatgatgtattttcgaatagcaaccactgatgcaccactcttctggaagcatgccttaatggcctcagttaagattgcatccatcttgggacgtggggaagaagccatcggtgtttgtttctgggccctggctagctggctggcagaaagggtagcccaggaaggaattgtttttttcactttcttctccttttctttagactgatctttctcatcctttttggtttcctcagaagacttattttcttccttctcttcattctcaggttccccctttggctgctctgcctcactcgaagtagcaggtggagtttcattctcttgttcttctacagtggagacagattcctctgaacttatgtctggttctggcttttcttcctccccttcagcaagcttgcttttgggaggagtttcccgggtagaattcacagttcgacgaatcggcatggtgctatcttctaccttctaacttgtccgcgtggatcagctgagctcctactataagtgggagtgccttaggatggacgagttcaccttgagacgtatcagtcgccattttaaataatttctaggcccgagtacaggttacactctgaagcctctgctgttaaccacaaggatttttcctaatggtttcagtgtggtgaagaatcaaccactgggagctccgtaatggcggcggcgggggcggagaacccggggggcgggcccgccgcagccagtcaccgccgccggcatctttcgaaccggctccgaaaaccgctgagggagtggggtgaggggagggcgcgggcggacgccggaccgcggcgggcctcggagcatgcgcagccctcagccaatcggggcgggcagaggacgccgacgcaggcgcgctgggacgcagggtcgcacggccagagaagagctccccctcctcccccaaatccaaacaaaacaagggcgggagcgcgcgcgccggagggcccctgaggaggagtccaccaaaag

SEQ ID NO: 17416 - RNA, 2908 nt, Homo sapiens
  source 1..2908: mol_type = other RNA
tcaggccaggcacagtggctcactcctgtaatcccagcactttgggaggccgaggcaggcggatcacctgaggtcaggagttcgagaccagcctgaccaacacggcgaaaccccatctctactaaaaatacaaaaaaattgccaggcgtggtggtacacacctgtaatcccagctactcgggaggctgaagcaggagaattgcttgaacccaggaggtggaggttgcagtgagctgagattgcaccactgcactccggggcacctgagcaagactccgtctcaaaacaacgacgacaacaacaacaacaacaaaaaacaagtgatatagagaacttgtgcttgctgttaagggaatgcaatactttgggccagtgaaaaatacctagaaattgatcaatatgaaatgtagcccaaaggagtcatatatcttcaaaatctaatgagatcaccctgtttttggcttattcccaaagctgtctctgtgtttacagttggagagaaaaggttagtggagtggcttttataaataagattaattattacagctataactgaagtctccaggcaggaggctttacaactcagtcagtgctatattgtgcctccattttacttccaggacctgactggcataccgttcttgatgctttctacaaatataaaaatctctgcaactgtttagataaaattggaagaaaaaaaaaaggcaaagctgaccataaaaacaacagggggttgggggaggcagagaaaaaggacaagtatacattacatagtttaggaaagtccaggattattgcagaaattaaaatgaacaaggaaaagggcaggcaccaataaaagcacctaaagctagcaaatgcctaaactggtttatttagagtccctccccacaatgttcataggggaggaaaataatgtaatttgaaaagcatcaaaactaaacaaatgcacactgaccttagaaaataagattttgaatttcatcatgatacccttttttcctataaaatttactttttcactctgaaagacttcttcatggtggatttgcccttgcccggcaattttacttcctttcttgcactggttgcaggcttctttgaggagccaccactaggtttcttgatgactgtggatgagggtctggtcttcttggcaggcgttttggccttaggaggtgctttcttaggcaagggcctagctttcccccgctgggcagctgagactttaggtgcaggtttggaccctctctgcttcacagatgcggccttccctggggacttggctggggttttcttctgcaaccttctcttaggtggcggctcttcatcctcagagtcttcttctgatgactcatcttcatcttcatcctcatctctagaatcatctggctctttcttcggaaacagaactcctgggctgggataatagggaaaacagagctggaaggtgccactgaaccctttcccagagatctgttccatccacccattcttttcgcatttctgcagggtttttttcagcaaatgcatttgatagttagaattggttcctgggtgattctctaggacatacttcttcagagcagtggtagagcaggtcttcggctcattcatggcagcaatggcagacaagattgcatattccatcaggcttccaccaagcaggggtttctcccctgatttcttcagctggaatgtccccgaagcacctttgccagttatctgttctaactggcccctctctactgctctctgcagagcgttcttcaacagctgaggcctgatgtccactctaagcttaggataatactgagacacatatttcctgatgagactgtaggaagcttctttaggttcacaaaggcgagtaaaggccagtgggaggacatcctccaattttacttgtggttctggatccactgcagagctcctattctttctgtttctggatttctgaggtgtttttcttgatttctgaaccacaacaaaacttccagaagcaccttttcctttaacctgtttgatgactcctctatttaattctcttttcagtgcttgtttaaggagataaccccttctctccagctccagagaaggatacttatggatgatgtattttcgaatagcaaccactgatgcaccactcttctggaagcatgccttaatggcctcagttaagattgcatccatcttgggacgtggggaagaagccatcggtgtttgtttctgggccctggctagctggctggcagaaagggtagcccaggaaggaattgtttttttcactttcttctccttttctttagactgatctttctcatcctttttggtttcctcagaagacttattttcttccttctcttcattctcaggttccccctttggctgctctgcctcactcgaagtagcaggtggagtttcattctcttgttcttctacagtggagacagattcctctgaacttatgtctggttctggcttttcttcctccccttcagcaagcttgcttttgggaggagtttcccgggtagaattcacagttcgacgaatcggcatggtgctatcttctaccttctaacttgtccgcgtggatcagctgagctcctactataagtgggagtgccttaggatggacgagttcaccttgagacgtatcagtcgccattttaaataatttctaggcccgagtacaggttacactctgaagcctctgctgttaaccacaaggatttttcctaatggtttcagtgtggtgaagaatcaaccgcggacaccgacggatgaggctggggctcggcgcggtgacagttcggggctcacgctcggcagggacaccgcggcgcccgccccggcgacggaagcagcggcggaacgcgagcctcggcgctccgcacactcacca

SEQ ID NO: 17417 - RNA, 3238 nt, Homo sapiens
  source 1..3238: mol_type = other RNA
tcaggccaggcacagtggctcactcctgtaatcccagcactttgggaggccgaggcaggcggatcacctgaggtcaggagttcgagaccagcctgaccaacacggcgaaaccccatctctactaaaaatacaaaaaaattgccaggcgtggtggtacacacctgtaatcccagctactcgggaggctgaagcaggagaattgcttgaacccaggaggtggaggttgcagtgagctgagattgcaccactgcactccggggcacctgagcaagactccgtctcaaaacaacgacgacaacaacaacaacaacaaaaaacaagtgatatagagaacttgtgcttgctgttaagggaatgcaatactttgggccagtgaaaaatacctagaaattgatcaatatgaaatgtagcccaaaggagtcatatatcttcaaaatctaatgagatcaccctgtttttggcttattcccaaagctgtctctgtgtttacagttggagagaaaaggttagtggagtggcttttataaataagattaattattacagctataactgaagtctccaggcaggaggctttacaactcagtcagtgctatattgtgcctccattttacttccaggacctgactggcataccgttcttgatgctttctacaaatataaaaatctctgcaactgtttagataaaattggaagaaaaaaaaaaggcaaagctgaccataaaaacaacagggggttgggggaggcagagaaaaaggacaagtatacattacatagtttaggaaagtccaggattattgcagaaattaaaatgaacaaggaaaagggcaggcaccaataaaagcacctaaagctagcaaatgcctaaactggtttatttagagtccctccccacaatgttcataggggaggaaaataatgtaatttgaaaagcatcaaaactaaacaaatgcacactgaccttagaaaataagattttgaatttcatcatgatacccttttttcctataaaatttactttttcactctgaaagacttcttcatggtggatttgcccttgcccggcaattttacttcctttcttgcactggttgcaggcttctttgaggagccaccactaggtttcttgatgactgtggatgagggtctggtcttcttggcaggcgttttggccttaggaggtgctttcttaggcaagggcctagctttcccccgctgggcagctgagactttaggtgcaggtttggaccctctctgcttcacagatgcggccttccctggggacttggctggggttttcttctgcaaccttctcttaggtggcggctcttcatcctcagagtcttcttctgatgactcatcttcatcttcatcctcatctctagaatcatctggctctttcttcggaaacagaactcctgggctgggataatagggaaaacagagctggaaggtgccactgaaccctttcccagagatctgttccatccacccattcttttcgcatttctgcagggtttttttcagcaaatgcatttgatagttagaattggttcctgggtgattctctaggacatacttcttcagagcagtggtagagcaggtcttcggctcattcatggcagcaatggcagacaagattgcatattccatcaggcttccaccaagcaggggtttctcccctgatttcttcagctggaatgtccccgaagcacctttgccagttatctgttctaactggcccctctctactgctctctgcagagcgttcttcaacagctgaggcctgatgtccactctaagcttaggataatactgagacacatatttcctgatgagactgtaggaagcttctttaggttcacaaaggcgagtaaaggccagtgggaggacatcctccaattttacttgtggttctggatccactgcagagctcctattctttctgtttctggatttctgaggtgtttttcttgatttctgaaccacaacaaaacttccagaagcaccttttcctttaacctgtttgatgactcctctatttaattctcttttcagtgcttgtttaaggagataaccccttctctccagctccagagaaggatacttatggatgatgtattttcgaatagcaaccactgatgcaccactcttctggaagcatgccttaatggcctcagttaagattgcatccatcttgggacgtggggaagaagccatcggtgtttgtttctgggccctggctagctggctggcagaaagggtagcccaggaaggaattgtttttttcactttcttctccttttctttagactgatctttctcatcctttttggtttcctcagaagacttattttcttccttctcttcattctcaggttccccctttggctgctctgcctcactcgaagtagcaggtggagtttcattctcttgttcttctacagtggagacagattcctctgaacttatgtctggttctggcttttcttcctccccttcagcaagcttgcttttgggaggagtttcccgggtagaattcacagttcgacgaatcggcatggtgctatcttctaccttctaacttgtccgcgtggatcagctgagctcctactataagtgggagtgccttaggatggacgagttcaccttgagacgtatcagtcgccattttaaataatttctaggcccgagtacaggttacactctgaagcctctgctgttaaccacaaggatttttcctaatggtttcagtgtggtgaagaatcaacctcaccactcctgcctccatctcttacaaacgctcagatgggcgactgtaactttctgacgacctaccgaggcaccgctctcattcaaaccccaccgcctaaggtggcgagtaaccagttctacgtttcccaccgggggagcgagactcaaggccgccgtcgcggagcagcaaagcgacagccgacagccccgcccgcagaaggccgcgggaaggacggcaagagcagcggagacaaagcagcgaggcgaggtagctacaggccacagcggcgaacgcgcacggcgggggagagcgcgggccgccagcgaggcggggaaagctcggaccgcggacaccgacggatgaggctggggctcggcgcggtgacagttcggggctcacgctcggcagggacaccgcggcgcccgccccggcgacggaagcagcggcggaacgcgagcctcggcgctccgcacactcaccact

SEQ ID NO: 17418 - RNA, 2800 nt, Homo sapiens
  source 1..2800: mol_type = other RNA
tcaggccaggcacagtggctcactcctgtaatcccagcactttgggaggccgaggcaggcggatcacctgaggtcaggagttcgagaccagcctgaccaacacggcgaaaccccatctctactaaaaatacaaaaaaattgccaggcgtggtggtacacacctgtaatcccagctactcgggaggctgaagcaggagaattgcttgaacccaggaggtggaggttgcagtgagctgagattgcaccactgcactccggggcacctgagcaagactccgtctcaaaacaacgacgacaacaacaacaacaacaaaaaacaagtgatatagagaacttgtgcttgctgttaagggaatgcaatactttgggccagtgaaaaatacctagaaattgatcaatatgaaatgtagcccaaaggagtcatatatcttcaaaatctaatgagatcaccctgtttttggcttattcccaaagctgtctctgtgtttacagttggagagaaaaggttagtggagtggcttttataaataagattaattattacagctataactgaagtctccaggcaggaggctttacaactcagtcagtgctatattgtgcctccattttacttccaggacctgactggcataccgttcttgatgctttctacaaatataaaaatctctgcaactgtttagataaaattggaagaaaaaaaaaaggcaaagctgaccataaaaacaacagggggttgggggaggcagagaaaaaggacaagtatacattacatagtttaggaaagtccaggattattgcagaaattaaaatgaacaaggaaaagggcaggcaccaataaaagcacctaaagctagcaaatgcctaaactggtttatttagagtccctccccacaatgttcataggggaggaaaataatgtaatttgaaaagcatcaaaactaaacaaatgcacactgaccttagaaaataagattttgaatttcatcatgatacccttttttcctataaaatttactttttcactctgaaagacttcttcatggtggatttgcccttgcccggcaattttacttcctttcttgcactggttgcaggcttctttgaggagccaccactaggtttcttgatgactgtggatgagggtctggtcttcttggcaggcgttttggccttaggaggtgctttcttaggcaagggcctagctttcccccgctgggcagctgagactttaggtgcaggtttggaccctctctgcttcacagatgcggccttccctggggacttggctggggttttcttctgcaaccttctcttaggtggcggctcttcatcctcagagtcttcttctgatgactcatcttcatcttcatcctcatctctagaatcatctggctctttcttcggaaacagaactcctgggctgggataatagggaaaacagagctggaaggtgccactgaaccctttcccagagatctgttccatccacccattcttttcgcatttctgcagggtttttttcagcaaatgcatttgatagttagaattggttcctgggtgattctctaggacatacttcttcagagcagtggtagagcaggtcttcggctcattcatggcagcaatggcagacaagattgcatattccatcaggcttccaccaagcaggggtttctcccctgatttcttcagctggaatgtccccgaagcacctttgccagttatctgttctaactggcccctctctactgctctctgcagagcgttcttcaacagctgaggcctgatgtccactctaagcttaggataatactgagacacatatttcctgatgagactgtaggaagcttctttaggttcacaaaggcgagtaaaggccagtgggaggacatcctccaattttacttgtggttctggatccactgcagagctcctattctttctgtttctggatttctgaggtgtttttcttgatttctgaaccacaacaaaacttccagaagcaccttttcctttaacctgtttgatgactcctctatttaattctcttttcagtgcttgtttaaggagataaccccttctctccagctccagagaaggatacttatggatgatgtattttcgaatagcaaccactgatgcaccactcttctggaagcatgccttaatggcctcagttaagattgcatccatcttgggacgtggggaagaagccatcggtgtttgtttctgggccctggctagctggctggcagaaagggtagcccaggaaggaattgtttttttcactttcttctccttttctttagactgatctttctcatcctttttggtttcctcagaagacttattttcttccttctcttcattctcaggttccccctttggctgctctgcctcactcgaagtagcaggtggagtttcattctcttgttcttctacagtggagacagattcctctgaacttatgtctggttctggcttttcttcctccccttcagcaagcttgcttttgggaggagtttcccgggtagaattcacagttcgacgaatcggcatggtgctatcttctaccttctcacctaacttgtccgcgtggatcagctgagctcctactataagtgggagtgccttaggatggacgagttcaccttgagacgtatcagtcgccattttaaataatttctaggcccgagtacaggttacactctgaagcctctgctgttaaccacaaggatttttcctaatggtttcagtgtggtgaagaatcaaccactgggagctccgtaatggcggc

SEQ ID NO: 17419 - RNA, 3176 nt, Homo sapiens
  source 1..3176: mol_type = other RNA
tcaggccaggcacagtggctcactcctgtaatcccagcactttgggaggccgaggcaggcggatcacctgaggtcaggagttcgagaccagcctgaccaacacggcgaaaccccatctctactaaaaatacaaaaaaattgccaggcgtggtggtacacacctgtaatcccagctactcgggaggctgaagcaggagaattgcttgaacccaggaggtggaggttgcagtgagctgagattgcaccactgcactccggggcacctgagcaagactccgtctcaaaacaacgacgacaacaacaacaacaacaaaaaacaagtgatatagagaacttgtgcttgctgttaagggaatgcaatactttgggccagtgaaaaatacctagaaattgatcaatatgaaatgtagcccaaaggagtcatatatcttcaaaatctaatgagatcaccctgtttttggcttattcccaaagctgtctctgtgtttacagttggagagaaaaggttagtggagtggcttttataaataagattaattattacagctataactgaagtctccaggcaggaggctttacaactcagtcagtgctatattgtgcctccattttacttccaggacctgactggcataccgttcttgatgctttctacaaatataaaaatctctgcaactgtttagataaaattggaagaaaaaaaaaaggcaaagctgaccataaaaacaacagggggttgggggaggcagagaaaaaggacaagtatacattacatagtttaggaaagtccaggattattgcagaaattaaaatgaacaaggaaaagggcaggcaccaataaaagcacctaaagctagcaaatgcctaaactggtttatttagagtccctccccacaatgttcataggggaggaaaataatgtaatttgaaaagcatcaaaactaaacaaatgcacactgaccttagaaaataagattttgaatttcatcatgatacccttttttcctataaaatttactttttcactctgaaagacttcttcatggtggatttgcccttgcccggcaattttacttcctttcttgcactggttgcaggcttctttgaggagccaccactaggtttcttgatgactgtggatgagggtctggtcttcttggcaggcgttttggccttaggaggtgctttcttaggcaagggcctagctttcccccgctgggcagctgagactttaggtgcaggtttggaccctctctgcttcacagatgcggccttccctggggacttggctggggttttcttctgcaaccttctcttaggtggcggctcttcatcctcagagtcttcttctgatgactcatcttcatcttcatcctcatctctagaatcatctggctctttcttcggaaacagaactcctgggctgggataatagggaaaacagagctggaaggtgccactgaaccctttcccagagatctgttccatccacccattcttttcgcatttctgcagggtttttttcagcaaatgcatttgatagttagaattggttcctgggtgattctctaggacatacttcttcagagcagtggtagagcaggtcttcggctcattcatggcagcaatggcagacaagattgcatattccatcaggcttccaccaagcaggggtttctcccctgatttcttcagctggaatgtccccgaagcacctttgccagttatctgttctaactggcccctctctactgctctctgcagagcgttcttcaacagctgaggcctgatgtccactctaagcttaggataatactgagacacatatttcctgatgagactgtaggaagcttctttaggttcacaaaggcgagtaaaggccagtgggaggacatcctccaattttacttgtggttctggatccactgcagagctcctattctttctgtttctggatttctgaggtgtttttcttgatttctgaaccacaacaaaacttccagaagcaccttttcctttaacctgtttgatgactcctctatttaattctcttttcagtgcttgtttaaggagataaccccttctctccagctccagagaaggatacttatggatgatgtattttcgaatagcaaccactgatgcaccactcttctggaagcatgccttaatggcctcagttaagattgcatccatcttgggacgtggggaagaagccatcggtgtttgtttctgggccctggctagctggctggcagaaagggtagcccaggaaggaattgtttttttcactttcttctccttttctttagactgatctttctcatcctttttggtttcctcagaagacttattttcttccttctcttcattctcaggttccccctttggctgctctgcctcactcgaagtagcaggtggagtttcattctcttgttcttctacagtggagacagattcctctgaacttatgtctggttctggcttttcttcctccccttcagcaagcttgcttttgggaggagtttcccgggtagaattcacagttcgacgaatcggcatggtgctatcttctaccttctcacctaacttgtccgcgtggatcagctgagctcctactataagtgggagtgccttaggatggacgagttcaccttgagacgtatcagtcgccattttaaataatttctaggcccgagtacaggttacactctgaagcctctgctgttaaccacaaggatttttcctaatggtttcagtgtggtgaagaatcaaccgaggcaccgctctcattcaaaccccaccgcctaaggtggcgagtaaccagttctacgtttcccaccgggggagcgagactcaaggccgccgtcgcggagcagcaaagcgacagccgacagccccgcccgcagaaggccgcgggaaggacggcaagagcagcggagacaaagcagcgaggcgaggtagctacaggccacagcggcgaacgcgcacggcgggggagagcgcgggccgccagcgaggcggggaaagctcggaccgcggacaccgacggatgaggctggggctcggcgcggtgacagttcggggctcacgctcggcagggacaccgcggcgcccgccccggcgacggaagcagcggcggaacgcgagcctcggcgctccgcacactcaccact

SEQ ID NO: 17420 - RNA, 2915 nt, Homo sapiens
  source 1..2915: mol_type = other RNA
tcaggccaggcacagtggctcactcctgtaatcccagcactttgggaggccgaggcaggcggatcacctgaggtcaggagttcgagaccagcctgaccaacacggcgaaaccccatctctactaaaaatacaaaaaaattgccaggcgtggtggtacacacctgtaatcccagctactcgggaggctgaagcaggagaattgcttgaacccaggaggtggaggttgcagtgagctgagattgcaccactgcactccggggcacctgagcaagactccgtctcaaaacaacgacgacaacaacaacaacaacaaaaaacaagtgatatagagaacttgtgcttgctgttaagggaatgcaatactttgggccagtgaaaaatacctagaaattgatcaatatgaaatgtagcccaaaggagtcatatatcttcaaaatctaatgagatcaccctgtttttggcttattcccaaagctgtctctgtgtttacagttggagagaaaaggttagtggagtggcttttataaataagattaattattacagctataactgaagtctccaggcaggaggctttacaactcagtcagtgctatattgtgcctccattttacttccaggacctgactggcataccgttcttgatgctttctacaaatataaaaatctctgcaactgtttagataaaattggaagaaaaaaaaaaggcaaagctgaccataaaaacaacagggggttgggggaggcagagaaaaaggacaagtatacattacatagtttaggaaagtccaggattattgcagaaattaaaatgaacaaggaaaagggcaggcaccaataaaagcacctaaagctagcaaatgcctaaactggtttatttagagtccctccccacaatgttcataggggaggaaaataatgtaatttgaaaagcatcaaaactaaacaaatgcacactgaccttagaaaataagattttgaatttcatcatgatacccttttttcctataaaatttactttttcactctgaaagacttcttcatggtggatttgcccttgcccggcaattttacttcctttcttgcactggttgcaggcttctttgaggagccaccactaggtttcttgatgactgtggatgagggtctggtcttcttggcaggcgttttggccttaggaggtgctttcttaggcaagggcctagctttcccccgctgggcagctgagactttaggtgcaggtttggaccctctctgcttcacagatgcggccttccctggggacttggctggggttttcttctgcaaccttctcttaggtggcggctcttcatcctcagagtcttcttctgatgactcatcttcatcttcatcctcatctctagaatcatctggctctttcttcggaaacagaactcctgggctgggataatagggaaaacagagctggaaggtgccactgaaccctttcccagagatctgttccatccacccattcttttcgcatttctgcagggtttttttcagcaaatgcatttgatagttagaattggttcctgggtgattctctaggacatacttcttcagagcagtggtagagcaggtcttcggctcattcatggcagcaatggcagacaagattgcatattccatcaggcttccaccaagcaggggtttctcccctgatttcttcagctggaatgtccccgaagcacctttgccagttatctgttctaactggcccctctctactgctctctgcagagcgttcttcaacagctgaggcctgatgtccactctaagcttaggataatactgagacacatatttcctgatgagactgtaggaagcttctttaggttcacaaaggcgagtaaaggccagtgggaggacatcctccaattttacttgtggttctggatccactgcagagctcctattctttctgtttctggatttctgaggtgtttttcttgatttctgaaccacaacaaaacttccagaagcaccttttcctttaacctgtttgatgactcctctatttaattctcttttcagtgcttgtttaaggagataaccccttctctccagctccagagaaggatacttatggatgatgtattttcgaatagcaaccactgatgcaccactcttctggaagcatgccttaatggcctcagttaagattgcatccatcttgggacgtggggaagaagccatcggtgtttgtttctgggccctggctagctggctggcagaaagggtagcccaggaaggaattgtttttttcactttcttctccttttctttagactgatctttctcatcctttttggtttcctcagaagacttattttcttccttctcttcattctcaggttccccctttggctgctctgcctcactcgaagtagcaggtggagtttcattctcttgttcttctacagtggagacagattcctctgaacttatgtctggttctggcttttcttcctccccttcagcaagcttgcttttgggaggagtttcccgggtagaattcacagttcgacgaatcggcatggtgctatcttctaccttctcacctaacttgtccgcgtggatcagctgagctcctactataagtgggagtgccttaggatggacgagttcaccttgagacgtatcagtcgccattttaaataatttctaggcccgagtacaggttacactctgaagcctctgctgttaaccacaaggatttttcctaatggtttcagtgtggtgaagaatcaaccgcggacaccgacggatgaggctggggctcggcgcggtgacagttcggggctcacgctcggcagggacaccgcggcgcccgccccggcgacggaagcagcggcggaacgcgagcctcggcgctccgcacactcaccact

SEQ ID NO: 17421 - RNA, 3243 nt, Homo sapiens
  source 1..3243: mol_type = other RNA
tcaggccaggcacagtggctcactcctgtaatcccagcactttgggaggccgaggcaggcggatcacctgaggtcaggagttcgagaccagcctgaccaacacggcgaaaccccatctctactaaaaatacaaaaaaattgccaggcgtggtggtacacacctgtaatcccagctactcgggaggctgaagcaggagaattgcttgaacccaggaggtggaggttgcagtgagctgagattgcaccactgcactccggggcacctgagcaagactccgtctcaaaacaacgacgacaacaacaacaacaacaaaaaacaagtgatatagagaacttgtgcttgctgttaagggaatgcaatactttgggccagtgaaaaatacctagaaattgatcaatatgaaatgtagcccaaaggagtcatatatcttcaaaatctaatgagatcaccctgtttttggcttattcccaaagctgtctctgtgtttacagttggagagaaaaggttagtggagtggcttttataaataagattaattattacagctataactgaagtctccaggcaggaggctttacaactcagtcagtgctatattgtgcctccattttacttccaggacctgactggcataccgttcttgatgctttctacaaatataaaaatctctgcaactgtttagataaaattggaagaaaaaaaaaaggcaaagctgaccataaaaacaacagggggttgggggaggcagagaaaaaggacaagtatacattacatagtttaggaaagtccaggattattgcagaaattaaaatgaacaaggaaaagggcaggcaccaataaaagcacctaaagctagcaaatgcctaaactggtttatttagagtccctccccacaatgttcataggggaggaaaataatgtaatttgaaaagcatcaaaactaaacaaatgcacactgaccttagaaaataagattttgaatttcatcatgatacccttttttcctataaaatttactttttcactctgaaagacttcttcatggtggatttgcccttgcccggcaattttacttcctttcttgcactggttgcaggcttctttgaggagccaccactaggtttcttgatgactgtggatgagggtctggtcttcttggcaggcgttttggccttaggaggtgctttcttaggcaagggcctagctttcccccgctgggcagctgagactttaggtgcaggtttggaccctctctgcttcacagatgcggccttccctggggacttggctggggttttcttctgcaaccttctcttaggtggcggctcttcatcctcagagtcttcttctgatgactcatcttcatcttcatcctcatctctagaatcatctggctctttcttcggaaacagaactcctgggctgggataatagggaaaacagagctggaaggtgccactgaaccctttcccagagatctgttccatccacccattcttttcgcatttctgcagggtttttttcagcaaatgcatttgatagttagaattggttcctgggtgattctctaggacatacttcttcagagcagtggtagagcaggtcttcggctcattcatggcagcaatggcagacaagattgcatattccatcaggcttccaccaagcaggggtttctcccctgatttcttcagctggaatgtccccgaagcacctttgccagttatctgttctaactggcccctctctactgctctctgcagagcgttcttcaacagctgaggcctgatgtccactctaagcttaggataatactgagacacatatttcctgatgagactgtaggaagcttctttaggttcacaaaggcgagtaaaggccagtgggaggacatcctccaattttacttgtggttctggatccactgcagagctcctattctttctgtttctggatttctgaggtgtttttcttgatttctgaaccacaacaaaacttccagaagcaccttttcctttaacctgtttgatgactcctctatttaattctcttttcagtgcttgtttaaggagataaccccttctctccagctccagagaaggatacttatggatgatgtattttcgaatagcaaccactgatgcaccactcttctggaagcatgccttaatggcctcagttaagattgcatccatcttgggacgtggggaagaagccatcggtgtttgtttctgggccctggctagctggctggcagaaagggtagcccaggaaggaattgtttttttcactttcttctccttttctttagactgatctttctcatcctttttggtttcctcagaagacttattttcttccttctcttcattctcaggttccccctttggctgctctgcctcactcgaagtagcaggtggagtttcattctcttgttcttctacagtggagacagattcctctgaacttatgtctggttctggcttttcttcctccccttcagcaagcttgcttttgggaggagtttcccgggtagaattcacagttcgacgaatcggcatggtgctatcttctaccttctcacctaacttgtccgcgtggatcagctgagctcctactataagtgggagtgccttaggatggacgagttcaccttgagacgtatcagtcgccattttaaataatttctaggcccgagtacaggttacactctgaagcctctgctgttaaccacaaggatttttcctaatggtttcagtgtggtgaagaatcaacctcaccactcctgcctccatctcttacaaacgctcagatgggcgactgtaactttctgacgacctaccgaggcaccgctctcattcaaaccccaccgcctaaggtggcgagtaaccagttctacgtttcccaccgggggagcgagactcaaggccgccgtcgcggagcagcaaagcgacagccgacagccccgcccgcagaaggccgcgggaaggacggcaagagcagcggagacaaagcagcgaggcgaggtagctacaggccacagcggcgaacgcgcacggcgggggagagcgcgggccgccagcgaggcggggaaagctcggaccgcggacaccgacggatgaggctggggctcggcgcggtgacagttcggggctcacgctcggcagggacaccgcggcgcccgccccggcgacggaagcagcggcggaacgcgagcctcggcgctccgcacactcaccact

SEQ ID NO: 17422 - RNA, 2889 nt, Homo sapiens
  source 1..2889: mol_type = other RNA
tcaggccaggcacagtggctcactcctgtaatcccagcactttgggaggccgaggcaggcggatcacctgaggtcaggagttcgagaccagcctgaccaacacggcgaaaccccatctctactaaaaatacaaaaaaattgccaggcgtggtggtacacacctgtaatcccagctactcgggaggctgaagcaggagaattgcttgaacccaggaggtggaggttgcagtgagctgagattgcaccactgcactccggggcacctgagcaagactccgtctcaaaacaacgacgacaacaacaacaacaacaaaaaacaagtgatatagagaacttgtgcttgctgttaagggaatgcaatactttgggccagtgaaaaatacctagaaattgatcaatatgaaatgtagcccaaaggagtcatatatcttcaaaatctaatgagatcaccctgtttttggcttattcccaaagctgtctctgtgtttacagttggagagaaaaggttagtggagtggcttttataaataagattaattattacagctataactgaagtctccaggcaggaggctttacaactcagtcagtgctatattgtgcctccattttacttccaggacctgactggcataccgttcttgatgctttctacaaatataaaaatctctgcaactgtttagataaaattggaagaaaaaaaaaaggcaaagctgaccataaaaacaacagggggttgggggaggcagagaaaaaggacaagtatacattacatagtttaggaaagtccaggattattgcagaaattaaaatgaacaaggaaaagggcaggcaccaataaaagcacctaaagctagcaaatgcctaaactggtttatttagagtccctccccacaatgttcataggggaggaaaataatgtaatttgaaaagcatcaaaactaaacaaatgcacactgaccttagaaaataagattttgaatttcatcatgatacccttttttcctataaaatttactttttcactctgaaagacttcttcatggtggatttgcccttgcccggcaattttacttcctttcttgcactggttgcaggcttctttgaggagccaccactaggtttcttgatgactgtggatgagggtctggtcttcttggcaggcgttttggccttaggaggtgctttcttaggcaagggcctagctttcccccgctgggcagctgagactttaggtgcaggtttggaccctctctgcttcacagatgcggccttccctggggacttggctggggttttcttctgcaaccttctcttaggtggcggctcttcatcctcagagtcttcttctgatgactcatcttcatcttcatcctcatctctagaatcatctggctctttcttcggaaacagaactcctgggctgggataatagggaaaacagagctggaaggtgccactgaaccctttcccagagatctgttccatccacccattcttttcgcatttctgcagggtttttttcagcaaatgcatttgatagttagaattggttcctgggtgattctctaggacatacttcttcagagcagtggtagagcaggtcttcggctcattcatggcagcaatggcagacaagattgcatattccatcaggcttccaccaagcaggggtttctcccctgatttcttcagctggaatgtccccgaagcacctttgccagttatctgttctaactggcccctctctactgctctctgcagagcgttcttcaacagctgaggcctgatgtccactctaagcttaggataatactgagacacatatttcctgatgagactgtaggaagcttctttaggttcacaaaggcgagtaaaggccagtgggaggacatcctccaattttacttgtggttctggatccactgcagagctcctattctttctgtttctggatttctgaggtgtttttcttgatttctgaaccacaacaaaacttccagaagcaccttttcctttaacctgtttgatgactcctctatttaattctcttttcagtgcttgtttaaggagataaccccttctctccagctccagagaaggatacttatggatgatgtattttcgaatagcaaccactgatgcaccactcttctggaagcatgccttaatggcctcagttaagattgcatccatcttgggacgtggggaagaagccatcggtgtttgtttctgggccctggctagctggctggcagaaagggtagcccaggaaggaattgtttttttcactttcttctccttttctttagactgatctttctcatcctttttggtttcctcagaagacttattttcttccttctcttcattctcaggttccccctttggctgctctgcctcactcgaagtagcaggtggagtttcattctcttgttcttctacagtggagacagattcctctgaacttatgtctggttctggcttttcttcctccccttcagcaagcttgcttttgggaggagtttcccgggtagaattcacagttcgacgaatcggcatggtgctatcttctaccttctcacctaacttgtccgcgtggatcagctgagctcctactataagtgggagtgccttaggatggacgagttcaccttgagacgtatcagtcgccattttaaataatttctaggcccgagtacaggttacactctgaagcctctgctgttaaccacaaggatttttcctaatggtttcagtgtggtgaagaatcaacctctgcgttcggccggtcctggcgcccgcgtcccgcacggcctctcggcgccgctcccgccgccgctagtcgcctccgccaccgctgtcctccagtcccagccgccgagctct

SEQ ID NO: 17423 - RNA, 2860 nt, Homo sapiens
  source 1..2860: mol_type = other RNA
tcaggccaggcacagtggctcactcctgtaatcccagcactttgggaggccgaggcaggcggatcacctgaggtcaggagttcgagaccagcctgaccaacacggcgaaaccccatctctactaaaaatacaaaaaaattgccaggcgtggtggtacacacctgtaatcccagctactcgggaggctgaagcaggagaattgcttgaacccaggaggtggaggttgcagtgagctgagattgcaccactgcactccggggcacctgagcaagactccgtctcaaaacaacgacgacaacaacaacaacaacaaaaaacaagtgatatagagaacttgtgcttgctgttaagggaatgcaatactttgggccagtgaaaaatacctagaaattgatcaatatgaaatgtagcccaaaggagtcatatatcttcaaaatctaatgagatcaccctgtttttggcttattcccaaagctgtctctgtgtttacagttggagagaaaaggttagtggagtggcttttataaataagattaattattacagctataactgaagtctccaggcaggaggctttacaactcagtcagtgctatattgtgcctccattttacttccaggacctgactggcataccgttcttgatgctttctacaaatataaaaatctctgcaactgtttagataaaattggaagaaaaaaaaaaggcaaagctgaccataaaaacaacagggggttgggggaggcagagaaaaaggacaagtatacattacatagtttaggaaagtccaggattattgcagaaattaaaatgaacaaggaaaagggcaggcaccaataaaagcacctaaagctagcaaatgcctaaactggtttatttagagtccctccccacaatgttcataggggaggaaaataatgtaatttgaaaagcatcaaaactaaacaaatgcacactgaccttagaaaataagattttgaatttcatcatgatacccttttttcctataaaatttactttttcactctgaaagacttcttcatggtggatttgcccttgcccggcaattttacttcctttcttgcactggttgcaggcttctttgaggagccaccactaggtttcttgatgactgtggatgagggtctggtcttcttggcaggcgttttggccttaggaggtgctttcttaggcaagggcctagctttcccccgctgggcagctgagactttaggtgcaggtttggaccctctctgcttcacagatgcggccttccctggggacttggctggggttttcttctgcaaccttctcttaggtggcggctcttcatcctcagagtcttcttctgatgactcatcttcatcttcatcctcatctctagaatcatctggctctttcttcggaaacagaactcctgggctgggataatagggaaaacagagctggaaggtgccactgaaccctttcccagagatctgttccatccacccattcttttcgcatttctgcagggtttttttcagcaaatgcatttgatagttagaattggttcctgggtgattctctaggacatacttcttcagagcagtggtagagcaggtcttcggctcattcatggcagcaatggcagacaagattgcatattccatcaggcttccaccaagcaggggtttctcccctgatttcttcagctggaatgtccccgaagcacctttgccagttatctgttctaactggcccctctctactgctctctgcagagcgttcttcaacagctgaggcctgatgtccactctaagcttaggataatactgagacacatatttcctgatgagactgtaggaagcttctttaggttcacaaaggcgagtaaaggccagtgggaggacatcctccaattttacttgtggttctggatccactgcagagctcctattctttctgtttctggatttctgaggtgtttttcttgatttctgaaccacaacaaaacttccagaagcaccttttcctttaacctgtttgatgactcctctatttaattctcttttcagtgcttgtttaaggagataaccccttctctccagctccagagaaggatacttatggatgatgtattttcgaatagcaaccactgatgcaccactcttctggaagcatgccttaatggcctcagttaagattgcatccatcttgggacgtggggaagaagccatcggtgtttgtttctgggccctggctagctggctggcagaaagggtagcccaggaaggaattgtttttttcactttcttctccttttctttagactgatctttctcatcctttttggtttcctcagaagacttattttcttccttctcttcattctcaggttccccctttggctgctctgcctcactcgaagtagcaggtggagtttcattctcttgttcttctacagtggagacagattcctctgaacttatgtctggttctggcttttcttcctccccttcagcaagcttgcttttgggaggagtttcccgggtagaattcacagttcgacgaatcggcatggtgctatcttctaccttctcacctaacttgtccgcgtggatcagctgagctcctactataagtgggagtgccttaggatggacgagttcaccttgagacgtatcagtcgccattttaaataatttctaggcccgagtacaggttacactctgaagcctctgctgttaaccacaaggatttttcctaatggtttcagtgtggtgaagaatcaacgctcggcagggacaccgcggcgcccgccccggcgacggaagcagcggcggaacgcgagcctcggcgctccgcacactcaccact

SEQ ID NO: 17424 - RNA, 2693 nt, Homo sapiens
  source 1..2693: mol_type = other RNA
tcaggccaggcacagtggctcactcctgtaatcccagcactttgggaggccgaggcaggcggatcacctgaggtcaggagttcgagaccagcctgaccaacacggcgaaaccccatctctactaaaaatacaaaaaaattgccaggcgtggtggtacacacctgtaatcccagctactcgggaggctgaagcaggagaattgcttgaacccaggaggtggaggttgcagtgagctgagattgcaccactgcactccggggcacctgagcaagactccgtctcaaaacaacgacgacaacaacaacaacaacaaaaaacaagtgatatagagaacttgtgcttgctgttaagggaatgcaatactttgggccagtgaaaaatacctagaaattgatcaatatgaaatgtagcccaaaggagtcatatatcttcaaaatctaatgagatcaccctgtttttggcttattcccaaagctgtctctgtgtttacagttggagagaaaaggttagtggagtggcttttataaataagattaattattacagctataactgaagtctccaggcaggaggctttacaactcagtcagtgctatattgtgcctccattttacttccaggacctgactggcataccgttcttgatgctttctacaaatataaaaatctctgcaactgtttagataaaattggaagaaaaaaaaaaggcaaagctgaccataaaaacaacagggggttgggggaggcagagaaaaaggacaagtatacattacatagtttaggaaagtccaggattattgcagaaattaaaatgaacaaggaaaagggcaggcaccaataaaagcacctaaagctagcaaatgcctaaactggtttatttagagtccctccccacaatgttcataggggaggaaaataatgtaatttgaaaagcatcaaaactaaacaaatgcacactgaccttagaaaataagattttgaatttcatcatgatacccttttttcctataaaatttactttttcactctgaaagacttcttcatggtggatttgcccttgcccggcaattttacttcctttcttgcactggttgcaggcttctttgaggagccaccactaggtttcttgatgactgtggatgagggtctggtcttcttggcaggcgttttggccttaggaggtgctttcttaggcaagggcctagctttcccccgctgggcagctgagactttaggtgcaggtttggaccctctctgcttcacagatgcggccttccctggggacttggctggggttttcttctgcaaccttctcttaggtggcggctcttcatcctcagagtcttcttctgatgactcatcttcatcttcatcctcatctctagaatcatctggctctttcttcggaaacagaactcctgggctgggataatagggaaaacagagctggaaggtgccactgaaccctttcccagagatctgttccatccacccattcttttcgcatttctgcagggtttttttcagcaaatgcatttgatagttagaattggttcctgggtgattctctaggacatacttcttcagagcagtggtagagcaggtcttcggctcattcatggcagcaatggcagacaagattgcatattccatcaggcttccaccaagcaggggtttctcccctgatttcttcagctggaatgtccccgaagcacctttgccagttatctgttctaactggcccctctctactgctctctgcagagcgttcttcaacagctgaggcctgatgtccactctaagcttaggataatactgagacacatatttcctgatgagactgtaggaagcttctttaggttcacaaaggcgagtaaaggccagtgggaggacatcctccaattttacttgtggttctggatccactgcagagctcctattctttctgtttctggatttctgaggtgtttttcttgatttctgaaccacaacaaaacttccagaagcaccttttcctttaacctgtttgatgactcctctatttaattctcttttcagtgcttgtttaaggagataaccccttctctccagctccagagaaggatacttatggatgatgtattttcgaatagcaaccactgatgcaccactcttctggaagcatgccttaatggcctcagttaagattgcatccatcttgggacgtggggaagaagccatcggtgtttgtttctgggccctggctagctggctggcagaaagggtagcccaggaaggaattgtttttttcactttcttctccttttctttagactgatctttctcatcctttttggtttcctcagaagacttattttcttccttctcttcattctcaggttccccctttggctgctctgcctcactcgaagtagcaggtggagtttcattctcttgttcttctacagtggagacagattcctctgaacttatgtctggttctggcttttcttcctccccttcagcaagcttgcttttgggaggagtttcccgggtagaattcacagttcgacgaatcggcatggtgctatcttctaccttctctgcgttcggccggtcctggcgcccgcgtcccgcacggcctctcggcgccgctcccgccgccgctagtcgcctccgccaccgctgtcctccagtcccagccgccgagctct

SEQ ID NO: 17425 - RNA, 2982 nt, Homo sapiens
  source 1..2982: mol_type = other RNA
tcaggccaggcacagtggctcactcctgtaatcccagcactttgggaggccgaggcaggcggatcacctgaggtcaggagttcgagaccagcctgaccaacacggcgaaaccccatctctactaaaaatacaaaaaaattgccaggcgtggtggtacacacctgtaatcccagctactcgggaggctgaagcaggagaattgcttgaacccaggaggtggaggttgcagtgagctgagattgcaccactgcactccggggcacctgagcaagactccgtctcaaaacaacgacgacaacaacaacaacaacaaaaaacaagtgatatagagaacttgtgcttgctgttaagggaatgcaatactttgggccagtgaaaaatacctagaaattgatcaatatgaaatgtagcccaaaggagtcatatatcttcaaaatctaatgagatcaccctgtttttggcttattcccaaagctgtctctgtgtttacagttggagagaaaaggttagtggagtggcttttataaataagattaattattacagctataactgaagtctccaggcaggaggctttacaactcagtcagtgctatattgtgcctccattttacttccaggacctgactggcataccgttcttgatgctttctacaaatataaaaatctctgcaactgtttagataaaattggaagaaaaaaaaaaggcaaagctgaccataaaaacaacagggggttgggggaggcagagaaaaaggacaagtatacattacatagtttaggaaagtccaggattattgcagaaattaaaatgaacaaggaaaagggcaggcaccaataaaagcacctaaagctagcaaatgcctaaactggtttatttagagtccctccccacaatgttcataggggaggaaaataatgtaatttgaaaagcatcaaaactaaacaaatgcacactgaccttagaaaataagattttgaatttcatcatgatacccttttttcctataaaatttactttttcactctgaaagacttcttcatggtggatttgcccttgcccggcaattttacttcctttcttgcactggttgcaggcttctttgaggagccaccactaggtttcttgatgactgtggatgagggtctggtcttcttggcaggcgttttggccttaggaggtgctttcttaggcaagggcctagctttcccccgctgggcagctgagactttaggtgcaggtttggaccctctctgcttcacagatgcggccttccctggggacttggctggggttttcttctgcaaccttctcttaggtggcggctcttcatcctcagagtcttcttctgatgactcatcttcatcttcatcctcatctctagaatcatctggctctttcttcggaaacagaactcctgggctgggataatagggaaaacagagctggaaggtgccactgaaccctttcccagagatctgttccatccacccattcttttcgcatttctgcagggtttttttcagcaaatgcatttgatagttagaattggttcctgggtgattctctaggacatacttcttcagagcagtggtagagcaggtcttcggctcattcatggcagcaatggcagacaagattgcatattccatcaggcttccaccaagcaggggtttctcccctgatttcttcagctgttttccaaggaggaagagaaaagcatcaagacaacactctcccaaagcaggtcaagacaagactcctctgcaccaggtgggtcggagttcctggaatgtccccgaagcacctttgccagttatctgttctaactggcccctctctactgctctctgcagagcgttcttcaacagctgaggcctgatgtccactctaagcttaggataatactgagacacatatttcctgatgagactgtaggaagcttctttaggttcacaaaggcgagtaaaggccagtgggaggacatcctccaattttacttgtggttctggatccactgcagagctcctattctttctgtttctggatttctgaggtgtttttcttgatttctgaaccacaacaaaacttccagaagcaccttttcctttaacctgtttgatgactcctctatttaattctcttttcagtgcttgtttaaggagataaccccttctctccagctccagagaaggatacttatggatgatgtattttcgaatagcaaccactgatgcaccactcttctggaagcatgccttaatggcctcagttaagattgcatccatcttgggacgtggggaagaagccatcggtgtttgtttctgggccctggctagctggctggcagaaagggtagcccaggaaggaattgtttttttcactttcttctccttttctttagactgatctttctcatcctttttggtttcctcagaagacttattttcttccttctcttcattctcaggttccccctttggctgctctgcctcactcgaagtagcaggtggagtttcattctcttgttcttctacagtggagacagattcctctgaacttatgtctggttctggcttttcttcctccccttcagcaagcttgcttttgggaggagtttcccgggtagaattcacagttcgacgaatcggcatggtgctatcttctaccttctcacctaacttgtccgcgtggatcagctgagctcctactataagtgggagtgccttaggatggacgagttcaccttgagacgtatcagtcgccattttaaataatttctaggcccgagtacaggttacactctgaagcctctgctgttaaccacaaggatttttcctaatggtttcagtgtggtgaagaatcaacctctgcgttcggccggtcctggcgcccgcgtcccgcacggcctctcggcgccgctcccgccgccgctagtcgcctccgccaccgctgtcctccagtcccagccgccgagctct

SEQ ID NO: 17426 - RNA, 2786 nt, Homo sapiens
  source 1..2786: mol_type = other RNA
tcaggccaggcacagtggctcactcctgtaatcccagcactttgggaggccgaggcaggcggatcacctgaggtcaggagttcgagaccagcctgaccaacacggcgaaaccccatctctactaaaaatacaaaaaaattgccaggcgtggtggtacacacctgtaatcccagctactcgggaggctgaagcaggagaattgcttgaacccaggaggtggaggttgcagtgagctgagattgcaccactgcactccggggcacctgagcaagactccgtctcaaaacaacgacgacaacaacaacaacaacaaaaaacaagtgatatagagaacttgtgcttgctgttaagggaatgcaatactttgggccagtgaaaaatacctagaaattgatcaatatgaaatgtagcccaaaggagtcatatatcttcaaaatctaatgagatcaccctgtttttggcttattcccaaagctgtctctgtgtttacagttggagagaaaaggttagtggagtggcttttataaataagattaattattacagctataactgaagtctccaggcaggaggctttacaactcagtcagtgctatattgtgcctccattttacttccaggacctgactggcataccgttcttgatgctttctacaaatataaaaatctctgcaactgtttagataaaattggaagaaaaaaaaaaggcaaagctgaccataaaaacaacagggggttgggggaggcagagaaaaaggacaagtatacattacatagtttaggaaagtccaggattattgcagaaattaaaatgaacaaggaaaagggcaggcaccaataaaagcacctaaagctagcaaatgcctaaactggtttatttagagtccctccccacaatgttcataggggaggaaaataatgtaatttgaaaagcatcaaaactaaacaaatgcacactgaccttagaaaataagattttgaatttcatcatgatacccttttttcctataaaatttactttttcactctgaaagacttcttcatggtggatttgcccttgcccggcaattttacttcctttcttgcactggttgcaggcttctttgaggagccaccactaggtttcttgatgactgtggatgagggtctggtcttcttggcaggcgttttggccttaggaggtgctttcttaggcaagggcctagctttcccccgctgggcagctgagactttaggtgcaggtttggaccctctctgcttcacagatgcggccttccctggggacttggctggggttttcttctgcaaccttctcttaggtggcggctcttcatcctcagagtcttcttctgatgactcatcttcatcttcatcctcatctctagaatcatctggctctttcttcggaaacagaactcctgggctgggataatagggaaaacagagctggaaggtgccactgaaccctttcccagagatctgttccatccacccattcttttcgcatttctgcagggtttttttcagcaaatgcatttgatagttagaattggttcctgggtgattctctaggacatacttcttcagagcagtggtagagcaggtcttcggctcattcatggcagcaatggcagacaagattgcatattccatcaggcttccaccaagcaggggtttctcccctgatttcttcagctgttttccaaggaggaagagaaaagcatcaagacaacactctcccaaagcaggtcaagacaagactcctctgcaccaggtgggtcggagttcctggaatgtccccgaagcacctttgccagttatctgttctaactggcccctctctactgctctctgcagagcgttcttcaacagctgaggcctgatgtccactctaagcttaggataatactgagacacatatttcctgatgagactgtaggaagcttctttaggttcacaaaggcgagtaaaggccagtgggaggacatcctccaattttacttgtggttctggatccactgcagagctcctattctttctgtttctggatttctgaggtgtttttcttgatttctgaaccacaacaaaacttccagaagcaccttttcctttaacctgtttgatgactcctctatttaattctcttttcagtgcttgtttaaggagataaccccttctctccagctccagagaaggatacttatggatgatgtattttcgaatagcaaccactgatgcaccactcttctggaagcatgccttaatggcctcagttaagattgcatccatcttgggacgtggggaagaagccatcggtgtttgtttctgggccctggctagctggctggcagaaagggtagcccaggaaggaattgtttttttcactttcttctccttttctttagactgatctttctcatcctttttggtttcctcagaagacttattttcttccttctcttcattctcaggttccccctttggctgctctgcctcactcgaagtagcaggtggagtttcattctcttgttcttctacagtggagacagattcctctgaacttatgtctggttctggcttttcttcctccccttcagcaagcttgcttttgggaggagtttcccgggtagaattcacagttcgacgaatcggcatggtgctatcttctaccttctctgcgttcggccggtcctggcgcccgcgtcccgcacggcctctcggcgccgctcccgccgccgctagtcgcctccgccaccgctgtcctccagtcccagccgccgagctct

SEQ ID NO: 17427 - RNA, 3702 nt, Homo sapiens
  source 1..3702: mol_type = other RNA
tcaggccaggcacagtggctcactcctgtaatctcagcactttgggaggtggagtcgggtggatcataaagtcagaagatagagaccattctggctaacacggtgaaacccagtctctactaaaaacacaaaaaattacccaggtgtggtggcacacaactgtagtgtcagctacttgggagactgaggcaggagaattgcttgaacctgggaggaggaggttgcagtgagctgagatcgtgccactgcactccaacctgggcgacagagcaagactccatctcaaaaaaaaaacaagaaaaagaaaataaaggctgggaaaagtagctcccatctgttggctaggctgttctcaaactcgtgagctccagtgacctacctgtctttgcctctcaaagtgctggaattacaggcatgagccatggcccccagtgcaatcctcttaacataaacagtttaatggcaattaatgcttgaaatcaatgttaaatcaacaaactcaggtcaaggctgatttgactctaatgtcaattaatgcttgatggtttgctatactcactgcatttgaaacaactgtctccaaaaggaattgtctgatggtctgcaaggagtgaccttggactgaagacccttccacactgatgacatttgtaagatttctgtccagcatggattctctgatgtctaatgaggtgtgaatgtgaagtaaacgctttgccacaatcatcacacttgtgaggtttctctcctgtatgaatcctcctatgttttgcataggatgaagcttgactgaagaccttgcctcaatcatgacatttataaggtttctctccagcatgagttcaccagtgaaatgcaaggcatgaacgatgtctgaaaaatttgccacatttattacacttgtaagatctcttcactgtggattctccaatgatgtgcaatggttgtagcattactgaaaactttgtgacaatcattacattagtcaagtttccctataccatggattgcttgatggtgaataagtggtgactgcccactaaagggtttgccacactcattgcacttgtaaggtttctctccagtgtgaattctagtatggggtgccacgtgtgaatcattcccgaaagccttgtcacaaaccttacatttctatggcttttctccagtgtgaattctcctatgtatttgaagctggatttgtgaatgaaaactttgtcacattgttcacgtttgtaagatttctatgcagtatgaagtctatgatgacttgcaaggtgtgattgttgattaaaaaccatgtcacattcattgtgcttgtaaggtttctctccactatgaattacaaggtgtgaattttgaccttttaattacaaggtgtgaattttgaccaacggtcttgccacactcattacacttataatgagtttctctccagtgtgaattctagtatgttttgccagatatgcattatatgcaaaaaccttgtcacaaaccttacctctgtatggtttctcttcaatgtgaattttcttatgtgttttaaggtttgatttacaactgaaaacttttgtcacattcctcccatttgtaaggtttctctccagtatgaagtctatggtgatgtgcaaaggttgctttttgattaaaaaccttgccacattcattatgcttgtaaggtttctctccagtatgaattgccttatgacttacagggttgaattgtgatggaaggtcttgccacactcattacactattaaggcttctctccactatgaagcctatgatggtatacaagggatgacatctgactgaaggtcttgccacactcattacacttgtaaggtttctctccagtatgaagcctacgatggattataagcgatgatgtctgaccgaaggtcttgccacactcattacacttgtaaggtttctctccagtatgaactctctgatgttgtgccaggtgtgaatccctctggaaagccttgtcacaaaccttacatttgtatggtttctctccagtatgaatcctcctgtgtctttccaggtttgatttgcgactgaaaactttgcaacattcttcacatttgtaaggtttctctccactatgaatcctcctatgtctttcaaggtgtgatttgcgactgaaaactttgtcacactcttcacatttgtaaggtttctctccagtatgaagtctatgatggcgtgcaagggttgatagtcgattaaaaactttgccacattcattacatgtgtaaggtttctctccagtgtgaagtatagtatgttttgccagatatgaattatatgcgaaagcctcatcacaaaccttacatttgtatggtttctctccagtatgaatcctcttatgtctttcaaggtgtgatttgcgactgaaaactttgtcacattcttcacattcataaggtttctctccagtatgaagcgctttgtgaatgaagagggatgaattatgaccaaaggtcttgccacactcattacacttgtaaggtttctcaccagtgtgacatctacgatggcaggcaaggtatcgcttctgattaaagaccttgccacatacatcacatttacattgtttctcttctaagtgaattatctgatgtttttttaagagtgagctgcaattaaaggatttgaagctctgtatacattcaaaagatttttctctcatgtgtacttcccatttttgtgtgagtaatgaagaatggagggaattatttccatacttattagaaatatgggttttgggcctacaacaaattctttgggatgttgaaactgaggaagcattgttgatagacttctcaacttgattaccaattttcccttcagactgaaatatgtgcggttcaggcagatgcaaatgaaagcttgatccaagctgatctttaatacgcttgtttccagcatgcctttgatcatgttggcctgtactaccagccaactctttgatttctgtcatgggtgctgcatggccatttgtttcatcttctttccactgaaactcgaagccatgaatgtctttctcaatttcatggaaacaaaattctccaatgtgatgacttgcttgtctgtgcaatgtccctgtgtggatcacttctgtattgccttgccctgttgacgacaacgtcttcaacatgcatttggaagagatatccagggagacgaggttcctataattctccagcatcacgtccctgtataaagtcctctgagcagggtccaggcatttccactcctcctgagagaattctatggccacgtccctgaatgtcaatagacccacgtacttcgtgcatattaatacgtgactcccattggcagctgctccaatcctggtccacagtgagctgacagtgcatccagatgtggcccctgaacaatccctgctgcccaagagcactgacaccacaggaccctcaccccgtgtccatccatgtcggggtgtgagcccttcccaggacctgcccagtgcagcctcttcccaagttcatgacactgggtcacgagagacggaacctaagcgagatgagagggactgaggaagagccatccctgactcctttgctttcctcttcctcttctgggtttctttctcacgtaccaacagtctttagaagtcaatccgcccgccgcggcgtgaccgtcattccacgggatccacttcctggtct

SEQ ID NO: 17428 - RNA, 3447 nt, Homo sapiens
  source 1..3447: mol_type = other RNA
tcaggccaggcacagtggctcactcctgtaatctcagcactttgggaggtggagtcgggtggatcataaagtcagaagatagagaccattctggctaacacggtgaaacccagtctctactaaaaacacaaaaaattacccaggtgtggtggcacacaactgtagtgtcagctacttgggagactgaggcaggagaattgcttgaacctgggaggaggaggttgcagtgagctgagatcgtgccactgcactccaacctgggcgacagagcaagactccatctcaaaaaaaaaacaagaaaaagaaaataaaggctgggaaaagtagctcccatctgttggctaggctgttctcaaactcgtgagctccagtgacctacctgtctttgcctctcaaagtgctggaattacaggcatgagccatggcccccagtgcaatcctcttaacataaacagtttaatggcaattaatgcttgaaatcaatgttaaatcaacaaactcaggtcaaggctgatttgactctaatgtcaattaatgcttgatggtttgctatactcactgcatttgaaacaactgtctccaaaaggaattgtctgatggtctgcaaggagtgaccttggactgaagacccttccacactgatgacatttgtaagatttctgtccagcatggattctctgatgtctaatgaggtgtgaatgtgaagtaaacgctttgccacaatcatcacacttgtgaggtttctctcctgtatgaatcctcctatgttttgcataggatgaagcttgactgaagaccttgcctcaatcatgacatttataaggtttctctccagcatgagttcaccagtgaaatgcaaggcatgaacgatgtctgaaaaatttgccacatttattacacttgtaagatctcttcactgtggattctccaatgatgtgcaatggttgtagcattactgaaaactttgtgacaatcattacattagtcaagtttccctataccatggattgcttgatggtgaataagtggtgactgcccactaaagggtttgccacactcattgcacttgtaaggtttctctccagtgtgaattctagtatggggtgccacgtgtgaatcattcccgaaagccttgtcacaaaccttacatttctatggcttttctccagtgtgaattctcctatgtatttgaagctggatttgtgaatgaaaactttgtcacattgttcacgtttgtaagatttctatgcagtatgaagtctatgatgacttgcaaggtgtgattgttgattaaaaaccatgtcacattcattgtgcttgtaaggtttctctccactatgaattacaaggtgtgaattttgaccttttaattacaaggtgtgaattttgaccaacggtcttgccacactcattacacttataatgagtttctctccagtgtgaattctagtatgttttgccagatatgcattatatgcaaaaaccttgtcacaaaccttacctctgtatggtttctcttcaatgtgaattttcttatgtgttttaaggtttgatttacaactgaaaacttttgtcacattcctcccatttgtaaggtttctctccagtatgaagtctatggtgatgtgcaaaggttgctttttgattaaaaaccttgccacattcattatgcttgtaaggtttctctccagtatgaattgccttatgacttacagggttgaattgtgatggaaggtcttgccacactcattacactattaaggcttctctccactatgaagcctatgatggtatacaagggatgacatctgactgaaggtcttgccacactcattacacttgtaaggtttctctccagtatgaagcctacgatggattataagcgatgatgtctgaccgaaggtcttgccacactcattacacttgtaaggtttctctccagtatgaactctctgatgttgtgccaggtgtgaatccctctggaaagccttgtcacaaaccttacatttgtatggtttctctccagtatgaatcctcctgtgtctttccaggtttgatttgcgactgaaaactttgcaacattcttcacatttgtaaggtttctctccactatgaatcctcctatgtctttcaaggtgtgatttgcgactgaaaactttgtcacactcttcacatttgtaaggtttctctccagtatgaagtctatgatggcgtgcaagggttgatagtcgattaaaaactttgccacattcattacatgtgtaaggtttctctccagtgtgaagtatagtatgttttgccagatatgaattatatgcgaaagcctcatcacaaaccttacatttgtatggtttctctccagtatgaatcctcttatgtctttcaaggtgtgatttgcgactgaaaactttgtcacattcttcacattcataaggtttctctccagtatgaagcgctttgtgaatgaagagggatgaattatgaccaaaggtcttgccacactcattacacttgtaaggtttctcaccagtgtgacatctacgatggcaggcaaggtatcgcttctgattaaagaccttgccacatacatcacatttacattgtttctcttctaagtgaattatctgatgtttttttaagagtgagctgcaattaaaggatttgaagctctgtatacattcaaaagatttttctctcatgtgtacttcccatttttgtgtgagtaatgaagaatggagggaattatttccatacttattagaaatatgggttttgggcctacaacaaattctttgggatgttgaaactgaggaagcattgttgatagacttctcaacttgattaccaattttcccttcagactgaaatatgtgcggttcaggcagatgcaaatgaaagcttgatccaagctgatctttaatacgcttgtttccagcatgcctttgatcatgttggcctgtactaccagccaactctttgatttctgtcatgggtgctgcatggccatttgtttcatcttctttccactgaaactcgaagccatgaatgtctttctcaatttcatggaaacaaaattctccaatgtgatgacttgcttgtctgtgcaatgtccctgtgtggatcacttctgtattgccttgccctgttgacgacaacgtcttcaacatgcatttggaagagatatccagggagacgaggttcctataattctccagcatcacgtccctgtataaagtcctctgagcagggtccaggcatttccactcctcctgagagaattctatggccacgtccctgaatgtcaatagaccctgaggaagagccatccctgactcctttgctttcctcttcctcttctgggtttctttctcacgtaccaacagtctttagaagtcaatccgcccgccgcggcgtgaccgtcattccacgggatccacttcctggtct

SEQ ID NO: 17429 - RNA, 3692 nt, Homo sapiens
  source 1..3692: mol_type = other RNA
tcaggccaggcacagtggctcactcctgtaatctcagcactttgggaggtggagtcgggtggatcataaagtcagaagatagagaccattctggctaacacggtgaaacccagtctctactaaaaacacaaaaaattacccaggtgtggtggcacacaactgtagtgtcagctacttgggagactgaggcaggagaattgcttgaacctgggaggaggaggttgcagtgagctgagatcgtgccactgcactccaacctgggcgacagagcaagactccatctcaaaaaaaaaacaagaaaaagaaaataaaggctgggaaaagtagctcccatctgttggctaggctgttctcaaactcgtgagctccagtgacctacctgtctttgcctctcaaagtgctggaattacaggcatgagccatggcccccagtgcaatcctcttaacataaacagtttaatggcaattaatgcttgaaatcaatgttaaatcaacaaactcaggtcaaggctgatttgactctaatgtcaattaatgcttgatggtttgctatactcactgcatttgaaacaactgtctccaaaaggaattgtctgatggtctgcaaggagtgaccttggactgaagacccttccacactgatgacatttgtaagatttctgtccagcatggattctctgatgtctaatgaggtgtgaatgtgaagtaaacgctttgccacaatcatcacacttgtgaggtttctctcctgtatgaatcctcctatgttttgcataggatgaagcttgactgaagaccttgcctcaatcatgacatttataaggtttctctccagcatgagttcaccagtgaaatgcaaggcatgaacgatgtctgaaaaatttgccacatttattacacttgtaagatctcttcactgtggattctccaatgatgtgcaatggttgtagcattactgaaaactttgtgacaatcattacattagtcaagtttccctataccatggattgcttgatggtgaataagtggtgactgcccactaaagggtttgccacactcattgcacttgtaaggtttctctccagtgtgaattctagtatggggtgccacgtgtgaatcattcccgaaagccttgtcacaaaccttacatttctatggcttttctccagtgtgaattctcctatgtatttgaagctggatttgtgaatgaaaactttgtcacattgttcacgtttgtaagatttctatgcagtatgaagtctatgatgacttgcaaggtgtgattgttgattaaaaaccatgtcacattcattgtgcttgtaaggtttctctccactatgaattacaaggtgtgaattttgaccttttaattacaaggtgtgaattttgaccaacggtcttgccacactcattacacttataatgagtttctctccagtgtgaattctagtatgttttgccagatatgcattatatgcaaaaaccttgtcacaaaccttacctctgtatggtttctcttcaatgtgaattttcttatgtgttttaaggtttgatttacaactgaaaacttttgtcacattcctcccatttgtaaggtttctctccagtatgaagtctatggtgatgtgcaaaggttgctttttgattaaaaaccttgccacattcattatgcttgtaaggtttctctccagtatgaattgccttatgacttacagggttgaattgtgatggaaggtcttgccacactcattacactattaaggcttctctccactatgaagcctatgatggtatacaagggatgacatctgactgaaggtcttgccacactcattacacttgtaaggtttctctccagtatgaagcctacgatggattataagcgatgatgtctgaccgaaggtcttgccacactcattacacttgtaaggtttctctccagtatgaactctctgatgttgtgccaggtgtgaatccctctggaaagccttgtcacaaaccttacatttgtatggtttctctccagtatgaatcctcctgtgtctttccaggtttgatttgcgactgaaaactttgcaacattcttcacatttgtaaggtttctctccactatgaatcctcctatgtctttcaaggtgtgatttgcgactgaaaactttgtcacactcttcacatttgtaaggtttctctccagtatgaagtctatgatggcgtgcaagggttgatagtcgattaaaaactttgccacattcattacatgtgtaaggtttctctccagtgtgaagtatagtatgttttgccagatatgaattatatgcgaaagcctcatcacaaaccttacatttgtatggtttctctccagtatgaatcctcttatgtctttcaaggtgtgatttgcgactgaaaactttgtcacattcttcacattcataaggtttctctccagtatgaagcgctttgtgaatgaagagggatgaattatgaccaaaggtcttgccacactcattacacttgtaaggtttctcaccagtgtgacatctacgatggcaggcaaggtatcgcttctgattaaagaccttgccacatacatcacatttacattgtttctcttctaagtgaattatctgatgtttttttaagagtgagctgcaattaaaggatttgaagctctgtatacattcaaaagatttttctctcatgtgtacttcccatttttgtgtgagtaatgaagaatggagggaattatttccatacttattagaaatatgggttttgggcctacaacaaattctttgggatgttgaaactgaggaagcattgttgatagacttctcaacttgattaccaattttcccttcagactgaaatatgtgcggttcaggcagatgcaaatgaaagcttgatccaagctgatctttaatacgcttgtttccagcatgcctttgatcatgttggcctgtactaccagccaactctttgatttctgtcatgggtgctgcatggccatttgtttcatcttctttccactgaaactcgaagccatgaatgtctttctcaatttcatggaaacaaaattctccaatgtgatgacttgcttgtctgtgcaatgtccctgtgtggatcacttctgtattgccttgccctgttgacgacaacgtcttcaacatgcatttggaagagatatccagggagacgaggttcctataattctccagcatcacgtccctgtataaagtcctctgagcagggtccaggcatttccactcctcctgagagaattctatggccacgtccctgaatgtcaatagaccttcgtgcatattaatacgtgactcccattggcagctgctccaatcctggtccacagtgagctgacagtgcatccagatgtggcccctgaacaatccctgctgcccaagagcactgacaccacaggaccctcaccccgtgtccatccatgtcggggtgtgagcccttcccaggacctgcccagtgcagcctcttcccaagttcatgacactgggtcacgagagacggaacctaagcgagatgagagggactgaggaagagccatccctgactcctttgctttcctcttcctcttctgggtttctttctcacgtaccaacagtctttagaagtcaatccgcccgccgcggcgtgaccgtcattccacgggatccacttcctgg

SEQ ID NO: 17430 - RNA, 3820 nt, Homo sapiens
  source 1..3820: mol_type = other RNA
tcaggccaggcacagtggctcactcctgtaatctcagcactttgggaggtggagtcgggtggatcataaagtcagaagatagagaccattctggctaacacggtgaaacccagtctctactaaaaacacaaaaaattacccaggtgtggtggcacacaactgtagtgtcagctacttgggagactgaggcaggagaattgcttgaacctgggaggaggaggttgcagtgagctgagatcgtgccactgcactccaacctgggcgacagagcaagactccatctcaaaaaaaaaacaagaaaaagaaaataaaggctgggaaaagtagctcccatctgttggctaggctgttctcaaactcgtgagctccagtgacctacctgtctttgcctctcaaagtgctggaattacaggcatgagccatggcccccagtgcaatcctcttaacataaacagtttaatggcaattaatgcttgaaatcaatgttaaatcaacaaactcaggtcaaggctgatttgactctaatgtcaattaatgcttgatggtttgctatactcactgcatttgaaacaactgtctccaaaaggaattgtctgatggtctgcaaggagtgaccttggactgaagacccttccacactgatgacatttgtaagatttctgtccagcatggattctctgatgtctaatgaggtgtgaatgtgaagtaaacgctttgccacaatcatcacacttgtgaggtttctctcctgtatgaatcctcctatgttttgcataggatgaagcttgactgaagaccttgcctcaatcatgacatttataaggtttctctccagcatgagttcaccagtgaaatgcaaggcatgaacgatgtctgaaaaatttgccacatttattacacttgtaagatctcttcactgtggattctccaatgatgtgcaatggttgtagcattactgaaaactttgtgacaatcattacattagtcaagtttccctataccatggattgcttgatggtgaataagtggtgactgcccactaaagggtttgccacactcattgcacttgtaaggtttctctccagtgtgaattctagtatggggtgccacgtgtgaatcattcccgaaagccttgtcacaaaccttacatttctatggcttttctccagtgtgaattctcctatgtatttgaagctggatttgtgaatgaaaactttgtcacattgttcacgtttgtaagatttctatgcagtatgaagtctatgatgacttgcaaggtgtgattgttgattaaaaaccatgtcacattcattgtgcttgtaaggtttctctccactatgaattacaaggtgtgaattttgaccttttaattacaaggtgtgaattttgaccaacggtcttgccacactcattacacttataatgagtttctctccagtgtgaattctagtatgttttgccagatatgcattatatgcaaaaaccttgtcacaaaccttacctctgtatggtttctcttcaatgtgaattttcttatgtgttttaaggtttgatttacaactgaaaacttttgtcacattcctcccatttgtaaggtttctctccagtatgaagtctatggtgatgtgcaaaggttgctttttgattaaaaaccttgccacattcattatgcttgtaaggtttctctccagtatgaattgccttatgacttacagggttgaattgtgatggaaggtcttgccacactcattacactattaaggcttctctccactatgaagcctatgatggtatacaagggatgacatctgactgaaggtcttgccacactcattacacttgtaaggtttctctccagtatgaagcctacgatggattataagcgatgatgtctgaccgaaggtcttgccacactcattacacttgtaaggtttctctccagtatgaactctctgatgttgtgccaggtgtgaatccctctggaaagccttgtcacaaaccttacatttgtatggtttctctccagtatgaatcctcctgtgtctttccaggtttgatttgcgactgaaaactttgcaacattcttcacatttgtaaggtttctctccactatgaatcctcctatgtctttcaaggtgtgatttgcgactgaaaactttgtcacactcttcacatttgtaaggtttctctccagtatgaagtctatgatggcgtgcaagggttgatagtcgattaaaaactttgccacattcattacatgtgtaaggtttctctccagtgtgaagtatagtatgttttgccagatatgaattatatgcgaaagcctcatcacaaaccttacatttgtatggtttctctccagtatgaatcctcttatgtctttcaaggtgtgatttgcgactgaaaactttgtcacattcttcacattcataaggtttctctccagtatgaagcgctttgtgaatgaagagggatgaattatgaccaaaggtcttgccacactcattacacttgtaaggtttctcaccagtgtgacatctacgatggcaggcaaggtatcgcttctgattaaagaccttgccacatacatcacatttacattgtttctcttctaagtgaattatctgatgtttttttaagagtgagctgcaattaaaggatttgaagctctgtatacattcaaaagatttttctctcatgtgtacttcccatttttgtgtgagtaatgaagaatggagggaattatttccatacttattagaaatatgggttttgggcctacaacaaattctttgggatgttgaaactgaggaagcattgttgatagacttctcaacttgattaccaattttcccttcagactgaaatatgtgcggttcaggcagatgcaaatgaaagcttgatccaagctgatctttaatacgcttgtttccagcatgcctttgatcatgttggcctgtactaccagccaactctttgatttctgtcatgggtgctgcatggccatttgtttcatcttctttccactgaaactcgaagccatgaatgtctttctcaatttcatggaaacaaaattctccaatgtgatgacttgcttgtctgtgcaatgtccctgtgtggatcacttctgtattgccttgccctgttgacgacaacgtcttcaacatgcatttggaagagatatctgtagtcccaggtacttggaaggctgaggcaggagaattgcttgaacctgggaagtggaggttgcagtgagcggagatgacaccactgtactttagccgggatgacagaccaaaactccagggagacgaggttcctataattctccagcatcacgtccctgtataaagtcctctgagcagggtccaggcatttccactcctcctgagagaattctatggccacgtccctgaatgtcaatagacccacgtacttcgtgcatattaatacgtgactcccattggcagctgctccaatcctggtccacagtgagctgacagtgcatccagatgtggcccctgaacaatccctgctgcccaagagcactgacaccacaggaccctcaccccgtgtccatccatgtcggggtgtgagcccttcccaggacctgcccagtgcagcctcttcccaagttcatgacactgggtcacgagagacggaacctaagcgagatgagagggactgaggaagagccatccctgactcctttgctttcctcttcctcttctgggtttctttctcacgtaccaacagtctttagaagtcaatccgcccgccgcggcgtgaccgtcattccacgggatccacttcctggtct

SEQ ID NO: 17431 - RNA, 3801 nt, Homo sapiens
  source 1..3801: mol_type = other RNA
tcaggccaggcacagtggctcactcctgtaatctcagcactttgggaggtggagtcgggtggatcataaagtcagaagatagagaccattctggctaacacggtgaaacccagtctctactaaaaacacaaaaaattacccaggtgtggtggcacacaactgtagtgtcagctacttgggagactgaggcaggagaattgcttgaacctgggaggaggaggttgcagtgagctgagatcgtgccactgcactccaacctgggcgacagagcaagactccatctcaaaaaaaaaacaagaaaaagaaaataaaggctgggaaaagtagctcccatctgttggctaggctgttctcaaactcgtgagctccagtgacctacctgtctttgcctctcaaagtgctggaattacaggcatgagccatggcccccagtgcaatcctcttaacataaacagtttaatggcaattaatgcttgaaatcaatgttaaatcaacaaactcaggtcaaggctgatttgactctaatgtcaattaatgcttgatggtttgctatactcactgcatttgaaacaactgtctccaaaaggaattgtctgatggtctgcaaggagtgaccttggactgaagacccttccacactgatgacatttgtaagatttctgtccagcatggattctctgatgtctaatgaggtgtgaatgtgaagtaaacgctttgccacaatcatcacacttgtgaggtttctctcctgtatgaatcctcctatgttttgcataggatgaagcttgactgaagaccttgcctcaatcatgacatttataaggtttctctccagcatgagttcaccagtgaaatgcaaggcatgaacgatgtctgaaaaatttgccacatttattacacttgtaagatctcttcactgtggattctccaatgatgtgcaatggttgtagcattactgaaaactttgtgacaatcattacattagtcaagtttccctataccatggattgcttgatggtgaataagtggtgactgcccactaaagggtttgccacactcattgcacttgtaaggtttctctccagtgtgaattctagtatggggtgccacgtgtgaatcattcccgaaagccttgtcacaaaccttacatttctatggcttttctccagtgtgaattctcctatgtatttgaagctggatttgtgaatgaaaactttgtcacattgttcacgtttgtaagatttctatgcagtatgaagtctatgatgacttgcaaggtgtgattgttgattaaaaaccatgtcacattcattgtgcttgtaaggtttctctccactatgaattacaaggtgtgaattttgaccttttaattacaaggtgtgaattttgaccaacggtcttgccacactcattacacttataatgagtttctctccagtgtgaattctagtatgttttgccagatatgcattatatgcaaaaaccttgtcacaaaccttacctctgtatggtttctcttcaatgtgaattttcttatgtgttttaaggtttgatttacaactgaaaacttttgtcacattcctcccatttgtaaggtttctctccagtatgaagtctatggtgatgtgcaaaggttgctttttgattaaaaaccttgccacattcattatgcttgtaaggtttctctccagtatgaattgccttatgacttacagggttgaattgtgatggaaggtcttgccacactcattacactattaaggcttctctccactatgaagcctatgatggtatacaagggatgacatctgactgaaggtcttgccacactcattacacttgtaaggtttctctccagtatgaagcctacgatggattataagcgatgatgtctgaccgaaggtcttgccacactcattacacttgtaaggtttctctccagtatgaactctctgatgttgtgccaggtgtgaatccctctggaaagccttgtcacaaaccttacatttgtatggtttctctccagtatgaatcctcctgtgtctttccaggtttgatttgcgactgaaaactttgcaacattcttcacatttgtaaggtttctctccactatgaatcctcctatgtctttcaaggtgtgatttgcgactgaaaactttgtcacactcttcacatttgtaaggtttctctccagtatgaagtctatgatggcgtgcaagggttgatagtcgattaaaaactttgccacattcattacatgtgtaaggtttctctccagtgtgaagtatagtatgttttgccagatatgaattatatgcgaaagcctcatcacaaaccttacatttgtatggtttctctccagtatgaatcctcttatgtctttcaaggtgtgatttgcgactgaaaactttgtcacattcttcacattcataaggtttctctccagtatgaagcgctttgtgaatgaagagggatgaattatgaccaaaggtcttgccacactcattacacttgtaaggtttctcaccagtgtgacatctacgatggcaggcaaggtatcgcttctgattaaagaccttgccacatacatcacatttacattgtttctcttctaagtgaattatctgatgtttttttaagagtgagctgcaattaaaggatttgaagctctgtatacattcaaaagatttttctctcatgtgtacttcccatttttgtgtgagtaatgaagaatggagggaattatttccatacttattagaaatatgggttttgggcctacaacaaattctttgggatgttgaaactgaggaagcattgttgatagacttctcaacttgattaccaattttcccttcagactgaaatatgtgcggttcaggcagatgcaaatgaaagcttgatccaagctgatctttaatacgcttgtttccagcatgcctttgatcatgttggcctgtactaccagccaactctttgatttctgtcatgggtgctgcatggccatttgtttcatcttctttccactgaaactcgaagccatgaatgtctttctcaatttcatggaaacaaaattctccaatgtgatgacttgcttgtctgtgcaatgtccctgtgtggatcacttctgtattgccttgccctgttgacgacaacgtcttcaacatgcatttggaagagatatctgtagtcccaggtacttggaaggctgaggcaggagaattgcttgaacctgggaagtggaggttgcagtgagcggagatgacaccactgtactttagccgggatgacagaccaaaactccagggagacgaggttcctataattctccagcatcacgtccctgtataaagtcctctgagcagggtccaggcatttccactcctcctgagagaattctatggccacgtccctgaatgtcaatagacccacgtacttcgtgcatattaatacgtgactcccattggcagctgctccaatcctggtccacagtgagctgacagtgcatccagatgtggcccctgaacaatccctgctgcccaagagcactgacaccacaggaccctcaccccgtgtccatccatgtcggggtgtgagcccttcccaggacctgcccagtgcagcctcttcccaagttcatgacactgggtcacgagagacggaacctgaggaagagccatccctgactcctttgctttcctcttcctcttctgggtttctttctcacgtaccaacagtctttagaagtcaatccgcccgccgcggcgtgaccgtcattccacgggatccacttcctggtct

SEQ ID NO: 17432 - RNA, 3565 nt, Homo sapiens
  source 1..3565: mol_type = other RNA
tcaggccaggcacagtggctcactcctgtaatctcagcactttgggaggtggagtcgggtggatcataaagtcagaagatagagaccattctggctaacacggtgaaacccagtctctactaaaaacacaaaaaattacccaggtgtggtggcacacaactgtagtgtcagctacttgggagactgaggcaggagaattgcttgaacctgggaggaggaggttgcagtgagctgagatcgtgccactgcactccaacctgggcgacagagcaagactccatctcaaaaaaaaaacaagaaaaagaaaataaaggctgggaaaagtagctcccatctgttggctaggctgttctcaaactcgtgagctccagtgacctacctgtctttgcctctcaaagtgctggaattacaggcatgagccatggcccccagtgcaatcctcttaacataaacagtttaatggcaattaatgcttgaaatcaatgttaaatcaacaaactcaggtcaaggctgatttgactctaatgtcaattaatgcttgatggtttgctatactcactgcatttgaaacaactgtctccaaaaggaattgtctgatggtctgcaaggagtgaccttggactgaagacccttccacactgatgacatttgtaagatttctgtccagcatggattctctgatgtctaatgaggtgtgaatgtgaagtaaacgctttgccacaatcatcacacttgtgaggtttctctcctgtatgaatcctcctatgttttgcataggatgaagcttgactgaagaccttgcctcaatcatgacatttataaggtttctctccagcatgagttcaccagtgaaatgcaaggcatgaacgatgtctgaaaaatttgccacatttattacacttgtaagatctcttcactgtggattctccaatgatgtgcaatggttgtagcattactgaaaactttgtgacaatcattacattagtcaagtttccctataccatggattgcttgatggtgaataagtggtgactgcccactaaagggtttgccacactcattgcacttgtaaggtttctctccagtgtgaattctagtatggggtgccacgtgtgaatcattcccgaaagccttgtcacaaaccttacatttctatggcttttctccagtgtgaattctcctatgtatttgaagctggatttgtgaatgaaaactttgtcacattgttcacgtttgtaagatttctatgcagtatgaagtctatgatgacttgcaaggtgtgattgttgattaaaaaccatgtcacattcattgtgcttgtaaggtttctctccactatgaattacaaggtgtgaattttgaccttttaattacaaggtgtgaattttgaccaacggtcttgccacactcattacacttataatgagtttctctccagtgtgaattctagtatgttttgccagatatgcattatatgcaaaaaccttgtcacaaaccttacctctgtatggtttctcttcaatgtgaattttcttatgtgttttaaggtttgatttacaactgaaaacttttgtcacattcctcccatttgtaaggtttctctccagtatgaagtctatggtgatgtgcaaaggttgctttttgattaaaaaccttgccacattcattatgcttgtaaggtttctctccagtatgaattgccttatgacttacagggttgaattgtgatggaaggtcttgccacactcattacactattaaggcttctctccactatgaagcctatgatggtatacaagggatgacatctgactgaaggtcttgccacactcattacacttgtaaggtttctctccagtatgaagcctacgatggattataagcgatgatgtctgaccgaaggtcttgccacactcattacacttgtaaggtttctctccagtatgaactctctgatgttgtgccaggtgtgaatccctctggaaagccttgtcacaaaccttacatttgtatggtttctctccagtatgaatcctcctgtgtctttccaggtttgatttgcgactgaaaactttgcaacattcttcacatttgtaaggtttctctccactatgaatcctcctatgtctttcaaggtgtgatttgcgactgaaaactttgtcacactcttcacatttgtaaggtttctctccagtatgaagtctatgatggcgtgcaagggttgatagtcgattaaaaactttgccacattcattacatgtgtaaggtttctctccagtgtgaagtatagtatgttttgccagatatgaattatatgcgaaagcctcatcacaaaccttacatttgtatggtttctctccagtatgaatcctcttatgtctttcaaggtgtgatttgcgactgaaaactttgtcacattcttcacattcataaggtttctctccagtatgaagcgctttgtgaatgaagagggatgaattatgaccaaaggtcttgccacactcattacacttgtaaggtttctcaccagtgtgacatctacgatggcaggcaaggtatcgcttctgattaaagaccttgccacatacatcacatttacattgtttctcttctaagtgaattatctgatgtttttttaagagtgagctgcaattaaaggatttgaagctctgtatacattcaaaagatttttctctcatgtgtacttcccatttttgtgtgagtaatgaagaatggagggaattatttccatacttattagaaatatgggttttgggcctacaacaaattctttgggatgttgaaactgaggaagcattgttgatagacttctcaacttgattaccaattttcccttcagactgaaatatgtgcggttcaggcagatgcaaatgaaagcttgatccaagctgatctttaatacgcttgtttccagcatgcctttgatcatgttggcctgtactaccagccaactctttgatttctgtcatgggtgctgcatggccatttgtttcatcttctttccactgaaactcgaagccatgaatgtctttctcaatttcatggaaacaaaattctccaatgtgatgacttgcttgtctgtgcaatgtccctgtgtggatcacttctgtattgccttgccctgttgacgacaacgtcttcaacatgcatttggaagagatatctgtagtcccaggtacttggaaggctgaggcaggagaattgcttgaacctgggaagtggaggttgcagtgagcggagatgacaccactgtactttagccgggatgacagaccaaaactccagggagacgaggttcctataattctccagcatcacgtccctgtataaagtcctctgagcagggtccaggcatttccactcctcctgagagaattctatggccacgtccctgaatgtcaatagaccctgaggaagagccatccctgactcctttgctttcctcttcctcttctgggtttctttctcacgtaccaacagtctttagaagtcaatccgcccgccgcggcgtgaccgtcattccacgggatccacttcctggtct

SEQ ID NO: 17433 - RNA, 3810 nt, Homo sapiens
  source 1..3810: mol_type = other RNA
tcaggccaggcacagtggctcactcctgtaatctcagcactttgggaggtggagtcgggtggatcataaagtcagaagatagagaccattctggctaacacggtgaaacccagtctctactaaaaacacaaaaaattacccaggtgtggtggcacacaactgtagtgtcagctacttgggagactgaggcaggagaattgcttgaacctgggaggaggaggttgcagtgagctgagatcgtgccactgcactccaacctgggcgacagagcaagactccatctcaaaaaaaaaacaagaaaaagaaaataaaggctgggaaaagtagctcccatctgttggctaggctgttctcaaactcgtgagctccagtgacctacctgtctttgcctctcaaagtgctggaattacaggcatgagccatggcccccagtgcaatcctcttaacataaacagtttaatggcaattaatgcttgaaatcaatgttaaatcaacaaactcaggtcaaggctgatttgactctaatgtcaattaatgcttgatggtttgctatactcactgcatttgaaacaactgtctccaaaaggaattgtctgatggtctgcaaggagtgaccttggactgaagacccttccacactgatgacatttgtaagatttctgtccagcatggattctctgatgtctaatgaggtgtgaatgtgaagtaaacgctttgccacaatcatcacacttgtgaggtttctctcctgtatgaatcctcctatgttttgcataggatgaagcttgactgaagaccttgcctcaatcatgacatttataaggtttctctccagcatgagttcaccagtgaaatgcaaggcatgaacgatgtctgaaaaatttgccacatttattacacttgtaagatctcttcactgtggattctccaatgatgtgcaatggttgtagcattactgaaaactttgtgacaatcattacattagtcaagtttccctataccatggattgcttgatggtgaataagtggtgactgcccactaaagggtttgccacactcattgcacttgtaaggtttctctccagtgtgaattctagtatggggtgccacgtgtgaatcattcccgaaagccttgtcacaaaccttacatttctatggcttttctccagtgtgaattctcctatgtatttgaagctggatttgtgaatgaaaactttgtcacattgttcacgtttgtaagatttctatgcagtatgaagtctatgatgacttgcaaggtgtgattgttgattaaaaaccatgtcacattcattgtgcttgtaaggtttctctccactatgaattacaaggtgtgaattttgaccttttaattacaaggtgtgaattttgaccaacggtcttgccacactcattacacttataatgagtttctctccagtgtgaattctagtatgttttgccagatatgcattatatgcaaaaaccttgtcacaaaccttacctctgtatggtttctcttcaatgtgaattttcttatgtgttttaaggtttgatttacaactgaaaacttttgtcacattcctcccatttgtaaggtttctctccagtatgaagtctatggtgatgtgcaaaggttgctttttgattaaaaaccttgccacattcattatgcttgtaaggtttctctccagtatgaattgccttatgacttacagggttgaattgtgatggaaggtcttgccacactcattacactattaaggcttctctccactatgaagcctatgatggtatacaagggatgacatctgactgaaggtcttgccacactcattacacttgtaaggtttctctccagtatgaagcctacgatggattataagcgatgatgtctgaccgaaggtcttgccacactcattacacttgtaaggtttctctccagtatgaactctctgatgttgtgccaggtgtgaatccctctggaaagccttgtcacaaaccttacatttgtatggtttctctccagtatgaatcctcctgtgtctttccaggtttgatttgcgactgaaaactttgcaacattcttcacatttgtaaggtttctctccactatgaatcctcctatgtctttcaaggtgtgatttgcgactgaaaactttgtcacactcttcacatttgtaaggtttctctccagtatgaagtctatgatggcgtgcaagggttgatagtcgattaaaaactttgccacattcattacatgtgtaaggtttctctccagtgtgaagtatagtatgttttgccagatatgaattatatgcgaaagcctcatcacaaaccttacatttgtatggtttctctccagtatgaatcctcttatgtctttcaaggtgtgatttgcgactgaaaactttgtcacattcttcacattcataaggtttctctccagtatgaagcgctttgtgaatgaagagggatgaattatgaccaaaggtcttgccacactcattacacttgtaaggtttctcaccagtgtgacatctacgatggcaggcaaggtatcgcttctgattaaagaccttgccacatacatcacatttacattgtttctcttctaagtgaattatctgatgtttttttaagagtgagctgcaattaaaggatttgaagctctgtatacattcaaaagatttttctctcatgtgtacttcccatttttgtgtgagtaatgaagaatggagggaattatttccatacttattagaaatatgggttttgggcctacaacaaattctttgggatgttgaaactgaggaagcattgttgatagacttctcaacttgattaccaattttcccttcagactgaaatatgtgcggttcaggcagatgcaaatgaaagcttgatccaagctgatctttaatacgcttgtttccagcatgcctttgatcatgttggcctgtactaccagccaactctttgatttctgtcatgggtgctgcatggccatttgtttcatcttctttccactgaaactcgaagccatgaatgtctttctcaatttcatggaaacaaaattctccaatgtgatgacttgcttgtctgtgcaatgtccctgtgtggatcacttctgtattgccttgccctgttgacgacaacgtcttcaacatgcatttggaagagatatctgtagtcccaggtacttggaaggctgaggcaggagaattgcttgaacctgggaagtggaggttgcagtgagcggagatgacaccactgtactttagccgggatgacagaccaaaactccagggagacgaggttcctataattctccagcatcacgtccctgtataaagtcctctgagcagggtccaggcatttccactcctcctgagagaattctatggccacgtccctgaatgtcaatagaccttcgtgcatattaatacgtgactcccattggcagctgctccaatcctggtccacagtgagctgacagtgcatccagatgtggcccctgaacaatccctgctgcccaagagcactgacaccacaggaccctcaccccgtgtccatccatgtcggggtgtgagcccttcccaggacctgcccagtgcagcctcttcccaagttcatgacactgggtcacgagagacggaacctaagcgagatgagagggactgaggaagagccatccctgactcctttgctttcctcttcctcttctgggtttctttctcacgtaccaacagtctttagaagtcaatccgcccgccgcggcgtgaccgtcattccacgggatccacttcctgg

SEQ ID NO: 17434 - RNA, 1806 nt, Homo sapiens
  source 1..1806: mol_type = other RNA
tcaggccaggcacagtggctcacttatgtaatccctgcactttgggaggccaaggtgggcagatcgcctgaggtcaggagttcaagaccagcctggccaacatggtgaaaccccatctctactaaaaatacaaaaattagccaggcatggtagtgcacacctgtagtcccagctactcagcaggctaagacacaagaatcgcttgaacccaggaagcagaggttgctgtgagctgagatcgcaccactgcattccggcctgggtgacagagcaagactgtctcaaaaaataaaaataataataataataataataaagatgttggggaagccgggtgcagtggctcacgcctgcaatcccagcactttgggaggccgaggcaggcagaacacatgaggtcaggagttcaagaccagcctggttaacatggcaaaaccctgtctctactaaaaatacaaaaattagctgggcgtggtggtgggcgcctgtaatcccagctacacaggaggctgaggcaggagaatcacttgaaccctggaggcagaggttacagtgagccagactgcagactaggtgacaagagtgaaactctgtctcaaaaaaaaaaaaaaaaaaagttgggaaatagatcatgatcacaactggcaagatccctatcctcagggagcttcctttctagcagggagaaaacacctgacataaaccagtaaagcaagtgagctagataatttcagagaggatgacattcaagaaggaaagacaccatgtaaaataacagagaggttgggagtttgtgacatcatgtttttatcttctcaccacttctgccagcagcaactccattaatcagtgctggattatcgtattttggcttcatctcgtttctaaatactattcttgcaaagcctctttcaccagcatcccttacccacaagtaatctcttctttcacttgtccacaaaaaatagcacattgattttgactaggtttgtttaagaagaaatgcactgattagaccataagcctatttgctctcccctgcctagcctcaggaacctcatcctcagtcacttaccctgcaggtataagggacttacagttagggacagtcttcctctgtctctccaccccactgactcaccagcttctttcaatactcaggtgaaaacatctttgcaccctttgctattaagaaagagactggacacagtctgcaaaaacaatctttgctttgtatttctgaatgcccttcacggtatagccccacttacgagctagtttacaggcagtctctccagcctccactcctgtattcataggaagaactttgtggtagttgaaaagtttagtaatatactcctcatattcaccaagtacgttattatagaaagctctagatgttaaggtcaatttgtccacttgactcttcagagcattcacaatcttggggtgacaatgcccttggttgacagcactgtaagaactcaggaagtcaaaatattttctgccttctacatcccataagtaaataccttttcctctctccagggctacaggtaaaggatggtagttgtgtgcaccatacttatattccctttcaaaaatgtcatcagaggttggagggccttggactgtttttttagttgcaacagatgtagcagaagccactgaagaatgaactccgcgactaagtacagcaaacctctgcaaatgtgctagtttggaaaacattgtgtccttcaagtagaaaaaccacagatctgacagcgcctgaggacaaccgggtacacgcggcgtctatgaagc

SEQ ID NO: 17435 - RNA, 8871 nt, Homo sapiens
  source 1..8871: mol_type = other RNA
tcaggccaggcacagtggctcactttgggaggcccaggcaggtggatcacgaggtcaggagatcgagaccatcctggttaacatgatgaaaccctgtctctactaaaaatacaaaaaaattagctggtcgtggtggcacgcacctgtaatcccagctactcgggaggctgaggcaggagaattgcatgaacccaggaggcagagcttgcagtgagctgagatggcgccactgcactccagcctgggcgacagagtgagactccatctcaaaataataataataataattttaaaaaagaaaaaatcatttagtagcaaaaaaaagtgaagaaataaatcaattaccaccaatacattcatcagtcaattgtaaaattgaaaataagccaatttccattatccggtgagtaagtaacctgataaaaacaagtgccctggagttcagatggctttagtggagctcggcctaacatataactgaggagtaatacaggcactgagagaatttagctccataacaagaaaacttgtgtacaagttagggctcagctacacaaacagactgaaaacgggcatttagacatttctctttcaaacagcatgaatacctaatgtcagtgagccccatgacttatatacctttaagctcatataaattgaaatttgaaggattccagccttttcccaggagaaaacttgttgttttgcactatctgtaaatctatgtgaattttcagggcttgggaagggaagagacacataggctcagttaatctgccccgatgcaacctggtttgcacctgtacaatattgcaccaaagcaacaacagcaagtgagggtcccaggtgagaagaggctcactgattctagaaaatctttattctgtaaccgaacacatcctgttttcatctagaagtagtgccttagccatatgaaggagggaactgagaacttctacatgtatgtctcagctgctctgtagagaaagaggggtgtagattccatgagttgcttaattttgctataaaggacaatatctcaacgggaaccctttatttcctcccagctagaggaagctagcagaaaaggcagcccggctctttgctggctctggctgttcatgtcctgccggctcctcccatcactcccttaggagctgggctccatgtccttgataaacatgtgggaaccttgctccctcaagggtattgccaatttagaaaagcacatctgcacactggactcttgttgggccttgtgtagtttggaaagccgaccccggtttcacgtacatggagaaactcagaatgcctaggattttgagtattttaagttacaggaaaacaggactctttcttatgtccaattctgacattgtcaaaggaaaactggttggctaggtttgagacttatataatttatgtaatgaggcctttgaatttatatagaaagagcctgaacttttattaaactggctttgcagagctactaaaggagtgatggcttttaaaatctcttctgaaatggcttgatagaatttagggtagaattattcctctactcttggaataatgttcttttgtctctaatacccaggccttggagaattagaatatggcagttcagtaggctgtggtaggaggaccctttttctgggtgcccggcaatcactaacagtgatgtgtactcagaaacagtcattgggagagcaggctgacagtggacctgctaaacactagtttgatacaaaatgttaattgaaagttacaatatattttataatatatcaatatatttcatatttaaaataaactgttatgctttctcctatcattaaaaaatagcaagcagtacagaggcaagatgcaaattcatattaaagctcatctgattctgaatataaacacttcagtttctgagcttgccatgaaaatgtttcctccattaacatcctgtcattctcttgttgttctcgtggccagtgcagaatggagagtctgggaccaaaattgagttgttgcgccattaaaaaacgtatctgatgaaggtggatcagtcctggttgagattcaaaaactgagacaacatgacacagctagagaatgttgtttattccttgtccttcttgagtgaagctggacgttggctgcttcgatctgattcagatatatatatatatatatatatatatatatatatatatatatatatatgtactttttctttttggctataaatgtcaacatctctttgggatcctaactgcaggttggagttgaattttgtgcttttcctccaccagcttggttggtcacgatgtgtctcttttgcttgtttcaacacatagcccaggcccaagattacagcttccaggatacatttttcaggtgtgtaaacaactgtcacagggcacttggcacctagatttggaggtcatatgttgaagatttgacaatggttttgttcagagggaactccagttcacgtttgggtgtttccagtaatggcgtaagacaaaaagatcacagttatatttttttctatctgtatatatgtatataccattgcactgagtactttttaataagctgtggtctgtttcaataaaaatctacatattactcgtctaacaggagtttaacattaatttctattcatgcagcctggcacaagctttctactaccacaagcagacagttactattgcgatccctgtaaactcctttctcagtggtgttaatgatcccatttccctaatgtttattttggcggcagtagagaaggaaaggatactgtctggggcgtcatcaagcccaccgactgcaaggggagagaaggggttgttcgtgcctactgggaagtcaccagatagctgtctaaggtactgaaatcaaaccctgcagagtcaatagggatccttcatctgcttctagcaactcttaggggaagaagaatgaatgtagaaaactggggacatattttaggatttaaaaacagtaacttcaaaagagtagtaacctactggtagtgcaatgacttcacagtatctcagttgtggtactgtgatgggagcaacaccgtttgtcctgggatgaaacattgattcttaatttggagtgtactgtttgttgagttgcactctggaggaggaggaaggttctggaactacgtgctaatcccatatttctccctgctgattttaccactatttaatgtgcactaattactttttggtaactactgactgcattcaaacgtaacatcaaggtgtgatctagatacagtcagtctgggctgctgttgatgacaaaggtgatttcatttgttctctattgaaaacattgtacttaagaatattaattattctcttcattttaagtacagagaaattgatgtattaggtgcttatatgaattggccaaagatgtggatccagtcttaagatttttatttattctgattttgtatgactaggtttcttcttttccatgattgtttattcacaaggaaattataaaaatttaagggggaaatcccccactatattaaaatcattacttcttcaatgctcttccttcttggcttttaataataaaaatagcttgtacatgctcagcgcttggaatttacttttgcgtacattttctatgtctcctaattcacaagattgttgttctaccactggcccctgctgaggtcggtcagtggtgacttggggccttccccccttgttcttttggattgtattaagcacttctagagacatgatgtcatgaagttacgtattaggaagatggcaagagcagttcatagacactttatgacaatttattgatgatgatcatatatatgtggcctttgatccaaaggtgaagacttttatttggacttcaatctaaggaggagtgagcccctagtctggtgtaatttaccaactaatgctatgtcctgaaattccactgagattagtggtcttaaagtatcacagtacatccctgactttacagtacatgaagctttaatatggcttaagcaatggcaggggtgggggtggttctgtatttctaattcaagtgtctagatattttaggaatattagagtgattttacctgtcactgagttgtcagaaagattatagtaggggatctgccattgggtcagtcctctaggagtgggcagatcttgatcagtacagtattggagtgaggttacataattaatagtttttacatatagccgattttttttttttttttgagacggagtcttgctcggtcacccaagctggagtgcaatggcacgatcttggctcactgcaacctccacttccggggttcaagtgattctcctgccgcagcctcccaagtagctgggactacaggtgtccaccaccaaacccagctaatttttgtatttttagtagagatggggttttgccatgttggccaggctggtcttgaactcctgacctcaggtgatcctctcgccttgcccaaagtcctgggattacaggcatgagccaccgcacctggctatatataccagattcttgagcagataattaaacctcctccaccacaaaacttgaaaataaggtacaagaaggcatgacatgagaatccacctgccccttttcccatctgactgtgatgctgaggtgtggtggaattagccaaaagatgtaggaagaaaacttgggtgagctacacccagaataattaatacttaagtcatcaagggttgattgtacttgcaggagaacgggtaactttcccacataaagctgaaatgctagtacagagaaatagccttccatttgctattacaggatcaatgtgcaggtttgatcactttttttttgaagcattttcttttgccaagaataaaaatcatgtatagctattgcactaccaataggtcaattcatgctacaaatgtccatgtgtttctaggatgccagtggctactgctaccagaaataactccagtcactcccttgactagtgttgctagtttggtctttagggtttacctaagtgagagcatcaatgatgggttaaagtcacagaccacaatgaataaatcacagtctgtgcacacttttggccaggaagagtggcagtggaatcttgcatgtcatttggttgaaattaagactaaatctctatatgtgcacacacccacactcacacccacacgcacacatatcacagggttatagcagaatgaaaacggtgggtaggaatcaccagttgaaggctgtaggtttaaatgatcaggattggcacactcagatcagcccaccagtggtcttcactttgtgaaatggaactaatgccacaaggaaactgcatggttacttcatctgtttacacatctgcttatatgttcagctgaactgtcactgaaaacaggagcaccattcttgggacatgaaacaaggaggaggggaaacattcagataatcaacagttaatagaacaagtaaaaaaataagccaacagcaggtgcggcatctctggtatgcaaaacaactaatgaaagtgttcaaaggaattatcaaggcaggccattaagactataaaccatcaaaagagcagcagcaatagcaagagagaaagaagagggttagcaagagactagatcttcctgaaaaagtggccttggctctacaattgtctaccttgtgctgtccttagaagaacaggcccagtgctacagaataaaaatctccatgccaagccactgccttcagaatggtgatgatgtcttcttacaaaggtaaacccaagatgacaaccacaagcaaaaaaatcacccttttgttttaccatcaacagatgaaatagtccatacagtgccattcaatttcccacaggcagaaaccaaagacctcagaatgagaaagtcatggttttcacgtcacaaatgttacgtgtggtcagattatggagcaatgaaaacatttttctgcgccgctcattacactaaatcttgatgtttctgaagtctcttggagtttgagatgtattggaatagtttttcgcaccaagattaacatggcacagtaggaacaggctactgacaaatccatgtccacttaccttacccacaaggttccctaagggttcccttcattctcacaatatttcattttgagatgacttaaggtcaggtagaagggaccacataggccactcttcatcacttctcctcctagctcagaggctcacaattgaggcacttggcccttttgcactactaacatctggggctggaaacctgttgctggataaatacagctcagcaaatccccaaccatatttctattcactaaggtgttattggattgctcctgtttgtgcatgtctgcacacacatgcacaatttcttgtcctctccctccacacttacagacatacacctggtcatgtggaccatcgaaacacaacttgtttggatggaagaagaaaactctgcagatgctgttatttttagaagcctgcttatccctcctgaatgccaacaattttggcttggcatccatttcaaatcaagcaaggtgcatatccaggacaaagcaatgtgcattatgtctgaagggatccacatcttcagtgaaactcagaatgtggccagaactagctaactacctgaactgaaagcaccccatgttcagattcagaccaactcaaaacacatgtaaggggtgcctattgtatgcagggtaaggtgtcaagtccctttttatttggattaagctcaaataagaaaggacctgaagcgaacgtgggatgtgtatgtgtgtacatgtacacgtttgcaaacacacaggtttatgtgggtattaatatcgagtggaaaatctggctttttatttgtctgtgtctttttttttttttttcagtctgattcgagtatatctgttttggcaagttgtgggcagctctcttttacttttgtcacccagaggcttccgtagacaaaaggaaaggagagaggtgtgttcaaagacccccatggcgaagagcccatcccccaagcctgacacaaccctccctcccagcggacccctcttctggactggcttcgctgttggctacttcagtgcatctgacccccaccccccgcgtgaagacctgagattgagcgtggatttctgttctccaccaactctgcagcaagggccctgccagaggcgtcgcttcctgtcatctcctcttcccgctcccaagtagaggcacctaaacagagattagatttctggtttcaaggcatgtcggaccaagcacgctgaatgaacatgagttagttaattagctcggtctctcttctttccgttccctggtctgaatgtttcttgatggcaaagcgaccaggagagagttgatttgcatcttaagacctatgggtaatgcttctggagtggggagatttatttagcaactgcttgaacttgtgtacggggtcgggaaggaggtggagctgaccccaatggggctatcggagattggggtgtgggtggtgcccactgccacgctgacaccccgggcctcgatgatggcagacaggagctgctgctgctgctggcgcagggtgtcggcgatgagcagcggcagggagttgaagctggcggtgagatgctccagcttcgactccaggctgccaatctgcttctccaggtcttcgctccggtcattgagttctgtgattaagtcatacatgacattctgcatcttggaaaggtccaccagagtgttggcttggtcactcagcttcctctgttccatcttgacgctcctcaactggtggatagcttggaggaacttcctctggtgtttcctcactttggcatggtcaatcttctttagcagctttgtgtgtttatagattaaccatgtttcccgaaggacattggctgcagcattcttgatccgcttggtgagctgagtgtccatcatgaagttatgaacgtgcttctccgctttggtgagttccagctttcgggccaccacggccaccacaagggcagtgcagcctgcacccatgatgccagtgaggagacagacacctttcccacagtatgtgtggggcaccatgtccccataaccaatggaaaggaatgtgatggagatgagccacatggcacccagaaagttactagttacgtcctgctggtcatggtaccaagcaggaagtgatgagccagaaggctgggctggtgattcaggactttcacagacacggacggtccaggcagcaatgatccacagagagatgctgaacacgagcagcacagtgccagggcagatggtcatgagcgtcttcatgacaaagcgggtgttgaagttgatcttgttgagggccccgatgctgcgggacgaggcatcggtgaagagcttgctgtgcagcagcatgactcgggcgatcaggtacaggcgcaggaacatggggatagacaggatgatgtccacatcggcctccgcccgggagggtgtgtaggagaaggccaggcgtgccgtccagaagaacttgtactcgccaggaatggggtggatggcgcacaccagcatctccaggctgatgtacaggatgcgctcgtaggtcatggctatccgccagtcatccgcgccattgtcgatcacgaagagctggacttcacgtgtgtggtaggcgatgatcaagcccaaaaggatgatggtggacagactgataaggcatttcagggccaacgaaaacatggagtccttcctccatctccactccctctgggagggaaaccccctcctccgtcttggggctggactgagaggctggagcagtggggccagctccccgctaaagccagtgcctgctgttctccatccgg

SEQ ID NO: 17436 - RNA, 9999 nt, Homo sapiens
  source 1..9999: mol_type = other RNA
tcaggccaggcacagtggctcactttgggaggcccaggcaggtggatcacgaggtcaggagatcgagaccatcctggttaacatgatgaaaccctgtctctactaaaaatacaaaaaaattagctggtcgtggtggcacgcacctgtaatcccagctactcgggaggctgaggcaggagaattgcatgaacccaggaggcagagcttgcagtgagctgagatggcgccactgcactccagcctgggcgacagagtgagactccatctcaaaataataataataataattttaaaaaagaaaaaatcatttagtagcaaaaaaaagtgaagaaataaatcaattaccaccaatacattcatcagtcaattgtaaaattgaaaataagccaatttccattatccggtgagtaagtaacctgataaaaacaagtgccctggagttcagatggctttagtggagctcggcctaacatataactgaggagtaatacaggcactgagagaatttagctccataacaagaaaacttgtgtacaagttagggctcagctacacaaacagactgaaaacgggcatttagacatttctctttcaaacagcatgaatacctaatgtcagtgagccccatgacttatatacctttaagctcatataaattgaaatttgaaggattccagccttttcccaggagaaaacttgttgttttgcactatctgtaaatctatgtgaattttcagggcttgggaagggaagagacacataggctcagttaatctgccccgatgcaacctggtttgcacctgtacaatattgcaccaaagcaacaacagcaagtgagggtcccaggtgagaagaggctcactgattctagaaaatctttattctgtaaccgaacacatcctgttttcatctagaagtagtgccttagccatatgaaggagggaactgagaacttctacatgtatgtctcagctgctctgtagagaaagaggggtgtagattccatgagttgcttaattttgctataaaggacaatatctcaacgggaaccctttatttcctcccagctagaggaagctagcagaaaaggcagcccggctctttgctggctctggctgttcatgtcctgccggctcctcccatcactcccttaggagctgggctccatgtccttgataaacatgtgggaaccttgctccctcaagggtattgccaatttagaaaagcacatctgcacactggactcttgttgggccttgtgtagtttggaaagccgaccccggtttcacgtacatggagaaactcagaatgcctaggattttgagtattttaagttacaggaaaacaggactctttcttatgtccaattctgacattgtcaaaggaaaactggttggctaggtttgagacttatataatttatgtaatgaggcctttgaatttatatagaaagagcctgaacttttattaaactggctttgcagagctactaaaggagtgatggcttttaaaatctcttctgaaatggcttgatagaatttagggtagaattattcctctactcttggaataatgttcttttgtctctaatacccaggccttggagaattagaatatggcagttcagtaggctgtggtaggaggaccctttttctgggtgcccggcaatcactaacagtgatgtgtactcagaaacagtcattgggagagcaggctgacagtggacctgctaaacactagtttgatacaaaatgttaattgaaagttacaatatattttataatatatcaatatatttcatatttaaaataaactgttatgctttctcctatcattaaaaaatagcaagcagtacagaggcaagatgcaaattcatattaaagctcatctgattctgaatataaacacttcagtttctgagcttgccatgaaaatgtttcctccattaacatcctgtcattctcttgttgttctcgtggccagtgcagaatggagagtctgggaccaaaattgagttgttgcgccattaaaaaacgtatctgatgaaggtggatcagtcctggttgagattcaaaaactgagacaacatgacacagctagagaatgttgtttattccttgtccttcttgagtgaagctggacgttggctgcttcgatctgattcagatatatatatatatatatatatatatatatatatatatatatatatatgtactttttctttttggctataaatgtcaacatctctttgggatcctaactgcaggttggagttgaattttgtgcttttcctccaccagcttggttggtcacgatgtgtctcttttgcttgtttcaacacatagcccaggcccaagattacagcttccaggatacatttttcaggtgtgtaaacaactgtcacagggcacttggcacctagatttggaggtcatatgttgaagatttgacaatggttttgttcagagggaactccagttcacgtttgggtgtttccagtaatggcgtaagacaaaaagatcacagttatatttttttctatctgtatatatgtatataccattgcactgagtactttttaataagctgtggtctgtttcaataaaaatctacatattactcgtctaacaggagtttaacattaatttctattcatgcagcctggcacaagctttctactaccacaagcagacagttactattgcgatccctgtaaactcctttctcagtggtgttaatgatcccatttccctaatgtttattttggcggcagtagagaaggaaaggatactgtctggggcgtcatcaagcccaccgactgcaaggggagagaaggggttgttcgtgcctactgggaagtcaccagatagctgtctaaggtactgaaatcaaaccctgcagagtcaatagggatccttcatctgcttctagcaactcttaggggaagaagaatgaatgtagaaaactggggacatattttaggatttaaaaacagtaacttcaaaagagtagtaacctactggtagtgcaatgacttcacagtatctcagttgtggtactgtgatgggagcaacaccgtttgtcctgggatgaaacattgattcttaatttggagtgtactgtttgttgagttgcactctggaggaggaggaaggttctggaactacgtgctaatcccatatttctccctgctgattttaccactatttaatgtgcactaattactttttggtaactactgactgcattcaaacgtaacatcaaggtgtgatctagatacagtcagtctgggctgctgttgatgacaaaggtgatttcatttgttctctattgaaaacattgtacttaagaatattaattattctcttcattttaagtacagagaaattgatgtattaggtgcttatatgaattggccaaagatgtggatccagtcttaagatttttatttattctgattttgtatgactaggtttcttcttttccatgattgtttattcacaaggaaattataaaaatttaagggggaaatcccccactatattaaaatcattacttcttcaatgctcttccttcttggcttttaataataaaaatagcttgtacatgctcagcgcttggaatttacttttgcgtacattttctatgtctcctaattcacaagattgttgttctaccactggcccctgctgaggtcggtcagtggtgacttggggccttccccccttgttcttttggattgtattaagcacttctagagacatgatgtcatgaagttacgtattaggaagatggcaagagcagttcatagacactttatgacaatttattgatgatgatcatatatatgtggcctttgatccaaaggtgaagacttttatttggacttcaatctaaggaggagtgagcccctagtctggtgtaatttaccaactaatgctatgtcctgaaattccactgagattagtggtcttaaagtatcacagtacatccctgactttacagtacatgaagctttaatatggcttaagcaatggcaggggtgggggtggttctgtatttctaattcaagtgtctagatattttaggaatattagagtgattttacctgtcactgagttgtcagaaagattatagtaggggatctgccattgggtcagtcctctaggagtgggcagatcttgatcagtacagtattggagtgaggttacataattaatagtttttacatatagccgattttttttttttttttgagacggagtcttgctcggtcacccaagctggagtgcaatggcacgatcttggctcactgcaacctccacttccggggttcaagtgattctcctgccgcagcctcccaagtagctgggactacaggtgtccaccaccaaacccagctaatttttgtatttttagtagagatggggttttgccatgttggccaggctggtcttgaactcctgacctcaggtgatcctctcgccttgcccaaagtcctgggattacaggcatgagccaccgcacctggctatatataccagattcttgagcagataattaaacctcctccaccacaaaacttgaaaataaggtacaagaaggcatgacatgagaatccacctgccccttttcccatctgactgtgatgctgaggtgtggtggaattagccaaaagatgtaggaagaaaacttgggtgagctacacccagaataattaatacttaagtcatcaagggttgattgtacttgcaggagaacgggtaactttcccacataaagctgaaatgctagtacagagaaatagccttccatttgctattacaggatcaatgtgcaggtttgatcactttttttttgaagcattttcttttgccaagaataaaaatcatgtatagctattgcactaccaataggtcaattcatgctacaaatgtccatgtgtttctaggatgccagtggctactgctaccagaaataactccagtcactcccttgactagtgttgctagtttggtctttagggtttacctaagtgagagcatcaatgatgggttaaagtcacagaccacaatgaataaatcacagtctgtgcacacttttggccaggaagagtggcagtggaatcttgcatgtcatttggttgaaattaagactaaatctctatatgtgcacacacccacactcacacccacacgcacacatatcacagggttatagcagaatgaaaacggtgggtaggaatcaccagttgaaggctgtaggtttaaatgatcaggattggcacactcagatcagcccaccagtggtcttcactttgtgaaatggaactaatgccacaaggaaactgcatggttacttcatctgtttacacatctgcttatatgttcagctgaactgtcactgaaaacaggagcaccattcttgggacatgaaacaaggaggaggggaaacattcagataatcaacagttaatagaacaagtaaaaaaataagccaacagcaggtgcggcatctctggtatgcaaaacaactaatgaaagtgttcaaaggaattatcaaggcaggccattaagactataaaccatcaaaagagcagcagcaatagcaagagagaaagaagagggttagcaagagactagatcttcctgaaaaagtggccttggctctacaattgtctaccttgtgctgtccttagaagaacaggcccagtgctacagaataaaaatctccatgccaagccactgccttcagaatggtgatgatgtcttcttacaaaggtaaacccaagatgacaaccacaagcaaaaaaatcacccttttgttttaccatcaacagatgaaatagtccatacagtgccattcaatttcccacaggcagaaaccaaagacctcagaatgagaaagtcatggttttcacgtcacaaatgttacgtgtggtcagattatggagcaatgaaaacatttttctgcgccgctcattacactaaatcttgatgtttctgaagtctcttggagtttgagatgtattggaatagtttttcgcaccaagattaacatggcacagtaggaacaggctactgacaaatccatgtccacttaccttacccacaaggttccctaagggttcccttcattctcacaatatttcattttgagatgacttaaggtcaggtagaagggaccacataggccactcttcatcacttctcctcctagctcagaggctcacaattgaggcacttggcccttttgcactactaacatctggggctggaaacctgttgctggataaatacagctcagcaaatccccaaccatatttctattcactaaggtgttattggattgctcctgtttgtgcatgtctgcacacacatgcacaatttcttgtcctctccctccacacttacagacatacacctggtcatgtggaccatcgaaacacaacttgtttggatggaagaagaaaactctgcagatgctgttatttttagaagcctgcttatccctcctgaatgccaacaattttggcttggcatccatttcaaatcaagcaaggtgcatatccaggacaaagcaatgtgcattatgtctgaagggatccacatcttcagtgaaactcagaatgtggccagaactagctaactacctgaactgaaagcaccccatgttcagattcagaccaactcaaaacacatgtaaggggtgcctattgtatgcagggtaaggtgtcaagtccctttttatttggattaagctcaaataagaaaggacctgaagcgaacgtgggatgtgtatgtgtgtacatgtacacgtttgcaaacacacaggtttatgtgggtattaatatcgagtggaaaatctggctttttatttgtctgtgtctttttttttttttttcagtctgattcgagtatatctgttttggcaagttgtgggcagctctcttttacttttgtcacccagaggcttccgtagacaaaaggaaaggagagaggtgtgttcaaagacccccatggcgaagagcccatcccccaagcctgacacaaccctccctcccagcggacccctcttctggactggcttcgctgttggctacttcagtgcatctgacccccaccccccgcgtgaagacctgagattgagcgtggatttctgttctccaccaactctgcagcaagggccctgccagaggcgtcgcttcctgtcatctcctcttcccgctcccaagtagaggcacctaaacagagattagatttctggtttcaaggcatgtcggaccaagcacgctgaatgaacatgagttagttaattagctcggtctctcttctttccgttccctggtctgaatgtttcttgatggcaaagcgaccaggagagagttgatttgcatcttaagacctatgggtaatgcttctggagtggggagatttatttagcaactgcttgaacttgtgtacggggtcgggaaggaggtggagctgaccccaatggggctatcggagattggggtgtgggtggtgcccactgccacgctgacaccccgggcctcgatgatggcagacaggagctgctgctgctgctggcgcagggtgtcggcgatgagcagcggcagggagttgaagctggcggtgagatgctccagcttcgactccaggctgccaatctgcttctccaggtcttcgctccggtcattgagttctgtgattaagtcatacatgacattctgcatcttggaaaggtccaccagagtgttggcttggtcactcagcttcctctgttccatcttgacgctcctcaactggtggatagcttggaggaacttcctctggtgtttcctcactttggcatggtcaatcttctttagcagctttgtgtgtttatagattaaccatgtttcccgaaggacattggctgcagcattcttgatccgcttggtgagctgagtgtccatcatgaagttatgaacgtgcttctccgctttggtgagttccagctttcgggccaccacggccaccacaagggcagtgcagcctgcacccatgatgccagtgaggagacagacacctttcccacagtatgtgtggggcaccatgtccccataaccaatggaaaggaatgtgatggagatgagccacatggcacccagaaagttactagttacgtcctgctggtcatggtaccaagcaggaagtgatgagccagaaggctgggctggtgattcaggactttcacagacacggacggtccaggcagcaatgatccacagagagatgctgaacacgagcagcacagtgccagggcagatggtcatgagcgtcttcatgacaaagcgggtgttgaagttgatcttgttgagggccccgatgctgcgggacgaggcatcggtgaagagcttgctgtgcagcagcatgactcgggcgatcaggtacaggcgcaggaacatggggatagacaggatgatgtccacatcggcctccgcccgggagggtgtgtaggagaaggccaggcgtgccgtccagaagaacttgtactcgccaggaatggggtggatggcgcacaccagcatctccaggctgatgtacaggatgcgctcgtaggtcatggctatccgccagtcatccgcgccattgtcgatcacgaagagctggacttcacgtgtgtggtaggcgatgatcaagcccaaaaggatgatggtggacagactgataaggcatttcagggccaacgaaaacatggagtcctttgagtacaaaccccaagagagctcggtctctatcaccataacaacaattccaaacatcccaaaaatcagagcatagtcactcagtcgctttctcttttcaaacagggccctcctgtgtcccagcttatagccaatgttttggtttttccgcttgttggctttggggaaggtggtgctgctggcggtggtgccggcatgctggtggttgtgggtggcattagggtgatggagcagggtctggtgggcatggttgtcctcccgggaggagatgacgatctccggggggttgctagggctgaaaagctggaggggttggccctcagtctcggcctcgatgaggttcctccgggaggcgctgaggcggctgaggggcttcatgaccccaccgctatacttgcaggagctcatggcgatctccgtgaaggggttgctgtcccgccggtgcaccagggggctggcctgtcggtgccggctgcctccgccaggcccacttgtagctgtggaacttggagagtggccaagcaagtggtcattgagattgagctggctgccttgcctggaggaagggtggaggatggcggtggagttggacgaagggggggccctgaaagcggtgggagaggagtgcagcaggccagggtggacgggctggctctggagttgggcgagctgagacaggggatgcggtggctgctgctgctgctgctgctgctgctgctgctgctgctgctgaagctgcggaggctgaggctgcagcgagggtcccaggggctgctggggggctgctggtggcgctggcggtggtggctgctgctgctgttgctgctgctgctgctgctgctgctcatccccagaggatggacaggggcacttggggtcttcatccaagtcccccacccccgagtcatggaagtgcccagaagtgtccatcttggggcctggctgtattccctgcagcacaagcccccaccccaaagccaccctcgctccaaagatgtcctcaaagaaagccaggcatccaatctcccccaccagtatcttggctccagtcctctctttggcttgcttcggttctctggggctgcctggagtccagacgctgccactcaagaatgcattgtattgggcagggagggagagcaggaggggagcttggagaaagaagagggggtgaaagaactctctcaggaggtggtcctctaggagcgtgtgaggccaggctcagcttcactcctcgctggctcaat

SEQ ID NO: 17437 - RNA, 8826 nt, Homo sapiens
  source 1..8826: mol_type = other RNA
tcaggccaggcacagtggctcactttgggaggcccaggcaggtggatcacgaggtcaggagatcgagaccatcctggttaacatgatgaaaccctgtctctactaaaaatacaaaaaaattagctggtcgtggtggcacgcacctgtaatcccagctactcgggaggctgaggcaggagaattgcatgaacccaggaggcagagcttgcagtgagctgagatggcgccactgcactccagcctgggcgacagagtgagactccatctcaaaataataataataataattttaaaaaagaaaaaatcatttagtagcaaaaaaaagtgaagaaataaatcaattaccaccaatacattcatcagtcaattgtaaaattgaaaataagccaatttccattatccggtgagtaagtaacctgataaaaacaagtgccctggagttcagatggctttagtggagctcggcctaacatataactgaggagtaatacaggcactgagagaatttagctccataacaagaaaacttgtgtacaagttagggctcagctacacaaacagactgaaaacgggcatttagacatttctctttcaaacagcatgaatacctaatgtcagtgagccccatgacttatatacctttaagctcatataaattgaaatttgaaggattccagccttttcccaggagaaaacttgttgttttgcactatctgtaaatctatgtgaattttcagggcttgggaagggaagagacacataggctcagttaatctgccccgatgcaacctggtttgcacctgtacaatattgcaccaaagcaacaacagcaagtgagggtcccaggtgagaagaggctcactgattctagaaaatctttattctgtaaccgaacacatcctgttttcatctagaagtagtgccttagccatatgaaggagggaactgagaacttctacatgtatgtctcagctgctctgtagagaaagaggggtgtagattccatgagttgcttaattttgctataaaggacaatatctcaacgggaaccctttatttcctcccagctagaggaagctagcagaaaaggcagcccggctctttgctggctctggctgttcatgtcctgccggctcctcccatcactcccttaggagctgggctccatgtccttgataaacatgtgggaaccttgctccctcaagggtattgccaatttagaaaagcacatctgcacactggactcttgttgggccttgtgtagtttggaaagccgaccccggtttcacgtacatggagaaactcagaatgcctaggattttgagtattttaagttacaggaaaacaggactctttcttatgtccaattctgacattgtcaaaggaaaactggttggctaggtttgagacttatataatttatgtaatgaggcctttgaatttatatagaaagagcctgaacttttattaaactggctttgcagagctactaaaggagtgatggcttttaaaatctcttctgaaatggcttgatagaatttagggtagaattattcctctactcttggaataatgttcttttgtctctaatacccaggccttggagaattagaatatggcagttcagtaggctgtggtaggaggaccctttttctgggtgcccggcaatcactaacagtgatgtgtactcagaaacagtcattgggagagcaggctgacagtggacctgctaaacactagtttgatacaaaatgttaattgaaagttacaatatattttataatatatcaatatatttcatatttaaaataaactgttatgctttctcctatcattaaaaaatagcaagcagtacagaggcaagatgcaaattcatattaaagctcatctgattctgaatataaacacttcagtttctgagcttgccatgaaaatgtttcctccattaacatcctgtcattctcttgttgttctcgtggccagtgcagaatggagagtctgggaccaaaattgagttgttgcgccattaaaaaacgtatctgatgaaggtggatcagtcctggttgagattcaaaaactgagacaacatgacacagctagagaatgttgtttattccttgtccttcttgagtgaagctggacgttggctgcttcgatctgattcagatatatatatatatatatatatatatatatatatatatatatatatatgtactttttctttttggctataaatgtcaacatctctttgggatcctaactgcaggttggagttgaattttgtgcttttcctccaccagcttggttggtcacgatgtgtctcttttgcttgtttcaacacatagcccaggcccaagattacagcttccaggatacatttttcaggtgtgtaaacaactgtcacagggcacttggcacctagatttggaggtcatatgttgaagatttgacaatggttttgttcagagggaactccagttcacgtttgggtgtttccagtaatggcgtaagacaaaaagatcacagttatatttttttctatctgtatatatgtatataccattgcactgagtactttttaataagctgtggtctgtttcaataaaaatctacatattactcgtctaacaggagtttaacattaatttctattcatgcagcctggcacaagctttctactaccacaagcagacagttactattgcgatccctgtaaactcctttctcagtggtgttaatgatcccatttccctaatgtttattttggcggcagtagagaaggaaaggatactgtctggggcgtcatcaagcccaccgactgcaaggggagagaaggggttgttcgtgcctactgggaagtcaccagatagctgtctaaggtactgaaatcaaaccctgcagagtcaatagggatccttcatctgcttctagcaactcttaggggaagaagaatgaatgtagaaaactggggacatattttaggatttaaaaacagtaacttcaaaagagtagtaacctactggtagtgcaatgacttcacagtatctcagttgtggtactgtgatgggagcaacaccgtttgtcctgggatgaaacattgattcttaatttggagtgtactgtttgttgagttgcactctggaggaggaggaaggttctggaactacgtgctaatcccatatttctccctgctgattttaccactatttaatgtgcactaattactttttggtaactactgactgcattcaaacgtaacatcaaggtgtgatctagatacagtcagtctgggctgctgttgatgacaaaggtgatttcatttgttctctattgaaaacattgtacttaagaatattaattattctcttcattttaagtacagagaaattgatgtattaggtgcttatatgaattggccaaagatgtggatccagtcttaagatttttatttattctgattttgtatgactaggtttcttcttttccatgattgtttattcacaaggaaattataaaaatttaagggggaaatcccccactatattaaaatcattacttcttcaatgctcttccttcttggcttttaataataaaaatagcttgtacatgctcagcgcttggaatttacttttgcgtacattttctatgtctcctaattcacaagattgttgttctaccactggcccctgctgaggtcggtcagtggtgacttggggccttccccccttgttcttttggattgtattaagcacttctagagacatgatgtcatgaagttacgtattaggaagatggcaagagcagttcatagacactttatgacaatttattgatgatgatcatatatatgtggcctttgatccaaaggtgaagacttttatttggacttcaatctaaggaggagtgagcccctagtctggtgtaatttaccaactaatgctatgtcctgaaattccactgagattagtggtcttaaagtatcacagtacatccctgactttacagtacatgaagctttaatatggcttaagcaatggcaggggtgggggtggttctgtatttctaattcaagtgtctagatattttaggaatattagagtgattttacctgtcactgagttgtcagaaagattatagtaggggatctgccattgggtcagtcctctaggagtgggcagatcttgatcagtacagtattggagtgaggttacataattaatagtttttacatatagccgattttttttttttttttgagacggagtcttgctcggtcacccaagctggagtgcaatggcacgatcttggctcactgcaacctccacttccggggttcaagtgattctcctgccgcagcctcccaagtagctgggactacaggtgtccaccaccaaacccagctaatttttgtatttttagtagagatggggttttgccatgttggccaggctggtcttgaactcctgacctcaggtgatcctctcgccttgcccaaagtcctgggattacaggcatgagccaccgcacctggctatatataccagattcttgagcagataattaaacctcctccaccacaaaacttgaaaataaggtacaagaaggcatgacatgagaatccacctgccccttttcccatctgactgtgatgctgaggtgtggtggaattagccaaaagatgtaggaagaaaacttgggtgagctacacccagaataattaatacttaagtcatcaagggttgattgtacttgcaggagaacgggtaactttcccacataaagctgaaatgctagtacagagaaatagccttccatttgctattacaggatcaatgtgcaggtttgatcactttttttttgaagcattttcttttgccaagaataaaaatcatgtatagctattgcactaccaataggtcaattcatgctacaaatgtccatgtgtttctaggatgccagtggctactgctaccagaaataactccagtcactcccttgactagtgttgctagtttggtctttagggtttacctaagtgagagcatcaatgatgggttaaagtcacagaccacaatgaataaatcacagtctgtgcacacttttggccaggaagagtggcagtggaatcttgcatgtcatttggttgaaattaagactaaatctctatatgtgcacacacccacactcacacccacacgcacacatatcacagggttatagcagaatgaaaacggtgggtaggaatcaccagttgaaggctgtaggtttaaatgatcaggattggcacactcagatcagcccaccagtggtcttcactttgtgaaatggaactaatgccacaaggaaactgcatggttacttcatctgtttacacatctgcttatatgttcagctgaactgtcactgaaaacaggagcaccattcttgggacatgaaacaaggaggaggggaaacattcagataatcaacagttaatagaacaagtaaaaaaataagccaacagcaggtgcggcatctctggtatgcaaaacaactaatgaaagtgttcaaaggaattatcaaggcaggccattaagactataaaccatcaaaagagcagcagcaatagcaagagagaaagaagagggttagcaagagactagatcttcctgaaaaagtggccttggctctacaattgtctaccttgtgctgtccttagaagaacaggcccagtgctacagaataaaaatctccatgccaagccactgccttcagaatggtgatgatgtcttcttacaaaggtaaacccaagatgacaaccacaagcaaaaaaatcacccttttgttttaccatcaacagatgaaatagtccatacagtgccattcaatttcccacaggcagaaaccaaagacctcagaatgagaaagtcatggttttcacgtcacaaatgttacgtgtggtcagattatggagcaatgaaaacatttttctgcgccgctcattacactaaatcttgatgtttctgaagtctcttggagtttgagatgtattggaatagtttttcgcaccaagattaacatggcacagtaggaacaggctactgacaaatccatgtccacttaccttacccacaaggttccctaagggttcccttcattctcacaatatttcattttgagatgacttaaggtcaggtagaagggaccacataggccactcttcatcacttctcctcctagctcagaggctcacaattgaggcacttggcccttttgcactactaacatctggggctggaaacctgttgctggataaatacagctcagcaaatccccaaccatatttctattcactaaggtgttattggattgctcctgtttgtgcatgtctgcacacacatgcacaatttcttgtcctctccctccacacttacagacatacacctggtcatgtggaccatcgaaacacaacttgtttggatggaagaagaaaactctgcagatgctgttatttttagaagcctgcttatccctcctgaatgccaacaattttggcttggcatccatttcaaatcaagcaaggtgcatatccaggacaaagcaatgtgcattatgtctgaagggatccacatcttcagtgaaactcagaatgtggccagaactagctaactacctgaactgaaagcaccccatgttcagattcagaccaactcaaaacacatgtaaggggtgcctattgtatgcagggtaaggtgtcaagtccctttttatttggattaagctcaaataagaaaggacctgaagcgaacgtgggatgtgtatgtgtgtacatgtacacgtttgcaaacacacaggtttatgtgggtattaatatcgagtggaaaatctggctttttatttgtctgtgtctttttttttttttttcagtctgattcgagtatatctgttttggcaagttgtgggcagctctcttttacttttgtcacccagaggcttccgtagacaaaaggaaaggagagaggtgtgttcaaagacccccatggcgaagagcccatcccccaagcctgacacaaccctccctcccagcggacccctcttctggactggcttcgctgttggctacttcagtgcatctgacccccaccccccgcgtgaagacctgagattgagcgtggatttctgttctccaccaactctgcagcaagggccctgccagaggcgtcgcttcctgtcatctcctcttcccgctcccaagtagaggcacctaaacagagattagatttctggtttcaaggcatgtcggaccaagcacgctgaatgaacatgagttagttaattagctcggtctctcttctttccgttccctggtctgaatgtttcttgatggcaaagcgaccaggagagagttgatttgcatcttaagacctatgggtaatgcttctggagtggggagatttatttagcaactgcttgaacttgtgtacggggtcgggaaggaggtggagctgaccccaatggggctatcggagattggggtgtgggtggtgcccactgccacgctgacaccccgggcctcgatgatggcagacaggagctgctgctgctgctggcgcagggtgtcggcgatgagcagcggcagggagttgaagctggcggtgagatgctccagcttcgactccaggctgccaatctgcttctccaggtcttcgctccggtcattgagttctgtgattaagtcatacatgacattctgcatcttggaaaggtccaccagagtgttggcttggtcactcagcttcctctgttccatcttgacgctcctcaactggtggatagcttggaggaacttcctctggtgtttcctcactttggcatggtcaatcttctttagcagctttgtgtgtttatagattaaccatgtttcccgaaggacattggctgcagcattcttgatccgcttggtgagctgagtgtccatcatgaagttatgaacgtgcttctccgctttggtgagttccagctttcgggccaccacggccaccacaagggcagtgcagcctgcacccatgatgccagtgaggagacagacacctttcccacagtatgtgtggggcaccatgtccccataaccaatggaaaggaatgtgatggagatgagccacatggcacccagaaagttactagttacgtcctgctggtcatggtacctttcacagacacggacggtccaggcagcaatgatccacagagagatgctgaacacgagcagcacagtgccagggcagatggtcatgagcgtcttcatgacaaagcgggtgttgaagttgatcttgttgagggccccgatgctgcgggacgaggcatcggtgaagagcttgctgtgcagcagcatgactcgggcgatcaggtacaggcgcaggaacatggggatagacaggatgatgtccacatcggcctccgcccgggagggtgtgtaggagaaggccaggcgtgccgtccagaagaacttgtactcgccaggaatggggtggatggcgcacaccagcatctccaggctgatgtacaggatgcgctcgtaggtcatggctatccgccagtcatccgcgccattgtcgatcacgaagagctggacttcacgtgtgtggtaggcgatgatcaagcccaaaaggatgatggtggacagactgataaggcatttcagggccaacgaaaacatggagtccttcctccatctccactccctctgggagggaaaccccctcctccgtcttggggctggactgagaggctggagcagtggggccagctccccgctaaagccagtgcctgctgttctccatccgg

SEQ ID NO: 17438 - RNA, 8886 nt, Homo sapiens
  source 1..8886: mol_type = other RNA
tcaggccaggcacagtggctcactttgggaggcccaggcaggtggatcacgaggtcaggagatcgagaccatcctggttaacatgatgaaaccctgtctctactaaaaatacaaaaaaattagctggtcgtggtggcacgcacctgtaatcccagctactcgggaggctgaggcaggagaattgcatgaacccaggaggcagagcttgcagtgagctgagatggcgccactgcactccagcctgggcgacagagtgagactccatctcaaaataataataataataattttaaaaaagaaaaaatcatttagtagcaaaaaaaagtgaagaaataaatcaattaccaccaatacattcatcagtcaattgtaaaattgaaaataagccaatttccattatccggtgagtaagtaacctgataaaaacaagtgccctggagttcagatggctttagtggagctcggcctaacatataactgaggagtaatacaggcactgagagaatttagctccataacaagaaaacttgtgtacaagttagggctcagctacacaaacagactgaaaacgggcatttagacatttctctttcaaacagcatgaatacctaatgtcagtgagccccatgacttatatacctttaagctcatataaattgaaatttgaaggattccagccttttcccaggagaaaacttgttgttttgcactatctgtaaatctatgtgaattttcagggcttgggaagggaagagacacataggctcagttaatctgccccgatgcaacctggtttgcacctgtacaatattgcaccaaagcaacaacagcaagtgagggtcccaggtgagaagaggctcactgattctagaaaatctttattctgtaaccgaacacatcctgttttcatctagaagtagtgccttagccatatgaaggagggaactgagaacttctacatgtatgtctcagctgctctgtagagaaagaggggtgtagattccatgagttgcttaattttgctataaaggacaatatctcaacgggaaccctttatttcctcccagctagaggaagctagcagaaaaggcagcccggctctttgctggctctggctgttcatgtcctgccggctcctcccatcactcccttaggagctgggctccatgtccttgataaacatgtgggaaccttgctccctcaagggtattgccaatttagaaaagcacatctgcacactggactcttgttgggccttgtgtagtttggaaagccgaccccggtttcacgtacatggagaaactcagaatgcctaggattttgagtattttaagttacaggaaaacaggactctttcttatgtccaattctgacattgtcaaaggaaaactggttggctaggtttgagacttatataatttatgtaatgaggcctttgaatttatatagaaagagcctgaacttttattaaactggctttgcagagctactaaaggagtgatggcttttaaaatctcttctgaaatggcttgatagaatttagggtagaattattcctctactcttggaataatgttcttttgtctctaatacccaggccttggagaattagaatatggcagttcagtaggctgtggtaggaggaccctttttctgggtgcccggcaatcactaacagtgatgtgtactcagaaacagtcattgggagagcaggctgacagtggacctgctaaacactagtttgatacaaaatgttaattgaaagttacaatatattttataatatatcaatatatttcatatttaaaataaactgttatgctttctcctatcattaaaaaatagcaagcagtacagaggcaagatgcaaattcatattaaagctcatctgattctgaatataaacacttcagtttctgagcttgccatgaaaatgtttcctccattaacatcctgtcattctcttgttgttctcgtggccagtgcagaatggagagtctgggaccaaaattgagttgttgcgccattaaaaaacgtatctgatgaaggtggatcagtcctggttgagattcaaaaactgagacaacatgacacagctagagaatgttgtttattccttgtccttcttgagtgaagctggacgttggctgcttcgatctgattcagatatatatatatatatatatatatatatatatatatatatatatatatgtactttttctttttggctataaatgtcaacatctctttgggatcctaactgcaggttggagttgaattttgtgcttttcctccaccagcttggttggtcacgatgtgtctcttttgcttgtttcaacacatagcccaggcccaagattacagcttccaggatacatttttcaggtgtgtaaacaactgtcacagggcacttggcacctagatttggaggtcatatgttgaagatttgacaatggttttgttcagagggaactccagttcacgtttgggtgtttccagtaatggcgtaagacaaaaagatcacagttatatttttttctatctgtatatatgtatataccattgcactgagtactttttaataagctgtggtctgtttcaataaaaatctacatattactcgtctaacaggagtttaacattaatttctattcatgcagcctggcacaagctttctactaccacaagcagacagttactattgcgatccctgtaaactcctttctcagtggtgttaatgatcccatttccctaatgtttattttggcggcagtagagaaggaaaggatactgtctggggcgtcatcaagcccaccgactgcaaggggagagaaggggttgttcgtgcctactgggaagtcaccagatagctgtctaaggtactgaaatcaaaccctgcagagtcaatagggatccttcatctgcttctagcaactcttaggggaagaagaatgaatgtagaaaactggggacatattttaggatttaaaaacagtaacttcaaaagagtagtaacctactggtagtgcaatgacttcacagtatctcagttgtggtactgtgatgggagcaacaccgtttgtcctgggatgaaacattgattcttaatttggagtgtactgtttgttgagttgcactctggaggaggaggaaggttctggaactacgtgctaatcccatatttctccctgctgattttaccactatttaatgtgcactaattactttttggtaactactgactgcattcaaacgtaacatcaaggtgtgatctagatacagtcagtctgggctgctgttgatgacaaaggtgatttcatttgttctctattgaaaacattgtacttaagaatattaattattctcttcattttaagtacagagaaattgatgtattaggtgcttatatgaattggccaaagatgtggatccagtcttaagatttttatttattctgattttgtatgactaggtttcttcttttccatgattgtttattcacaaggaaattataaaaatttaagggggaaatcccccactatattaaaatcattacttcttcaatgctcttccttcttggcttttaataataaaaatagcttgtacatgctcagcgcttggaatttacttttgcgtacattttctatgtctcctaattcacaagattgttgttctaccactggcccctgctgaggtcggtcagtggtgacttggggccttccccccttgttcttttggattgtattaagcacttctagagacatgatgtcatgaagttacgtattaggaagatggcaagagcagttcatagacactttatgacaatttattgatgatgatcatatatatgtggcctttgatccaaaggtgaagacttttatttggacttcaatctaaggaggagtgagcccctagtctggtgtaatttaccaactaatgctatgtcctgaaattccactgagattagtggtcttaaagtatcacagtacatccctgactttacagtacatgaagctttaatatggcttaagcaatggcaggggtgggggtggttctgtatttctaattcaagtgtctagatattttaggaatattagagtgattttacctgtcactgagttgtcagaaagattatagtaggggatctgccattgggtcagtcctctaggagtgggcagatcttgatcagtacagtattggagtgaggttacataattaatagtttttacatatagccgattttttttttttttttgagacggagtcttgctcggtcacccaagctggagtgcaatggcacgatcttggctcactgcaacctccacttccggggttcaagtgattctcctgccgcagcctcccaagtagctgggactacaggtgtccaccaccaaacccagctaatttttgtatttttagtagagatggggttttgccatgttggccaggctggtcttgaactcctgacctcaggtgatcctctcgccttgcccaaagtcctgggattacaggcatgagccaccgcacctggctatatataccagattcttgagcagataattaaacctcctccaccacaaaacttgaaaataaggtacaagaaggcatgacatgagaatccacctgccccttttcccatctgactgtgatgctgaggtgtggtggaattagccaaaagatgtaggaagaaaacttgggtgagctacacccagaataattaatacttaagtcatcaagggttgattgtacttgcaggagaacgggtaactttcccacataaagctgaaatgctagtacagagaaatagccttccatttgctattacaggatcaatgtgcaggtttgatcactttttttttgaagcattttcttttgccaagaataaaaatcatgtatagctattgcactaccaataggtcaattcatgctacaaatgtccatgtgtttctaggatgccagtggctactgctaccagaaataactccagtcactcccttgactagtgttgctagtttggtctttagggtttacctaagtgagagcatcaatgatgggttaaagtcacagaccacaatgaataaatcacagtctgtgcacacttttggccaggaagagtggcagtggaatcttgcatgtcatttggttgaaattaagactaaatctctatatgtgcacacacccacactcacacccacacgcacacatatcacagggttatagcagaatgaaaacggtgggtaggaatcaccagttgaaggctgtaggtttaaatgatcaggattggcacactcagatcagcccaccagtggtcttcactttgtgaaatggaactaatgccacaaggaaactgcatggttacttcatctgtttacacatctgcttatatgttcagctgaactgtcactgaaaacaggagcaccattcttgggacatgaaacaaggaggaggggaaacattcagataatcaacagttaatagaacaagtaaaaaaataagccaacagcaggtgcggcatctctggtatgcaaaacaactaatgaaagtgttcaaaggaattatcaaggcaggccattaagactataaaccatcaaaagagcagcagcaatagcaagagagaaagaagagggttagcaagagactagatcttcctgaaaaagtggccttggctctacaattgtctaccttgtgctgtccttagaagaacaggcccagtgctacagaataaaaatctccatgccaagccactgccttcagaatggtgatgatgtcttcttacaaaggtaaacccaagatgacaaccacaagcaaaaaaatcacccttttgttttaccatcaacagatgaaatagtccatacagtgccattcaatttcccacaggcagaaaccaaagacctcagaatgagaaagtcatggttttcacgtcacaaatgttacgtgtggtcagattatggagcaatgaaaacatttttctgcgccgctcattacactaaatcttgatgtttctgaagtctcttggagtttgagatgtattggaatagtttttcgcaccaagattaacatggcacagtaggaacaggctactgacaaatccatgtccacttaccttacccacaaggttccctaagggttcccttcattctcacaatatttcattttgagatgacttaaggtcaggtagaagggaccacataggccactcttcatcacttctcctcctagctcagaggctcacaattgaggcacttggcccttttgcactactaacatctggggctggaaacctgttgctggataaatacagctcagcaaatccccaaccatatttctattcactaaggtgttattggattgctcctgtttgtgcatgtctgcacacacatgcacaatttcttgtcctctccctccacacttacagacatacacctggtcatgtggaccatcgaaacacaacttgtttggatggaagaagaaaactctgcagatgctgttatttttagaagcctgcttatccctcctgaatgccaacaattttggcttggcatccatttcaaatcaagcaaggtgcatatccaggacaaagcaatgtgcattatgtctgaagggatccacatcttcagtgaaactcagaatgtggccagaactagctaactacctgaactgaaagcaccccatgttcagattcagaccaactcaaaacacatgtaaggggtgcctattgtatgcagggtaaggtgtcaagtccctttttatttggattaagctcaaataagaaaggacctgaagcgaacgtgggatgtgtatgtgtgtacatgtacacgtttgcaaacacacaggtttatgtgggtattaatatcgagtggaaaatctggctttttatttgtctgtgtctttttttttttttttcagtctgattcgagtatatctgttttggcaagttgtgggcagctctcttttacttttgtcacccagaggcttccgtagacaaaaggaaaggagagaggtgtgttcaaagacccccatggcgaagagcccatcccccaagcctgacacaaccctccctcccagcggacccctcttctggactggcttcgctgttggctacttcagtgcatctgacccccaccccccgcgtgaagacctgagattgagcgtggatttctgttctccaccaactctgcagcaagggccctgccagaggcgtcgcttcctgtcatctcctcttcccgctcccaagtagaggcacctaaacagagattagatttctggtttcaaggcatgtcggaccaagcacgctgaatgaacatgagttagttaattagctcggtctctcttctttccgttccctggtctgaatgtttcttgatggcaaagcgaccaggagagagttgatttgcatcttaagacctatgggtaatgcttctggagtggggagatttatttagcaactgcttgaacttgtgtacggggtcgggaaggaggtggagctgaccccaatggggctatcggagattggggtgtgggtggtgcccactgccacgctgacaccccgggcctcgatgatggcagacaggagctgctgctgctgctggcgcagggtgtcggcgatgagcagcggcagggagttgaagctggcggtgagatgctccagcttcgactccaggctgccaatctgcttctccaggtcttcgctccggtcattgagttctgtgattaagtcatacatgacattctgcatcttggaaaggtccaccagagtgttggcttggtcactcagcttcctctgttccatcttgacgctcctcaactggtggatagcttggaggaacttcctctggtgtttcctcactttggcatggtcaatcttctttagcagctttgtgtgtttatagattaaccatgtttcccgaaggacattggctgcagcattcttgatccgcttggtgagctgagtgtccatcatgaagttatgaacgtgcttctccgctttggtgagttccagctttcgggccaccacggccaccacaagggcagtgcagcctgcacccatgatgccagtgaggagacagacacctttcccacagtatgtgtggggcaccatgtccccataaccaatggaaaggaatgtgatggagatgagccacatggcacccagaaagttactagttacgtcctgctggtcatggtacctttcacagacacggacggtccaggcagcaatgatccacagagagatgctgaacacgagcagcacagtgccagggcagatggtcatgagcgtcttcatgacaaagcgggtgttgaagttgatcttgttgagggccccgatgctgcgggacgaggcatcggtgaagagcttgctgtgcagcagcatgactcgggcgatcaggtacaggcgcaggaacatggggatagacaggatgatgtccacatcggcctccgcccgggagggtgtgtaggagaaggccaggcgtgccgtccagaagaacttgtactcgccaggaatggggtggatggcgcacaccagcatctccaggctgatgtacaggatgcgctcgtaggtcatggctatccgccagtcatccgcgccattgtcgatcacgaagagctggacttcacgtgtgtggtaggcgatgatcaagcccaaaaggatgatggtggacagactgataaggcatttcagggccaacgaaaacatggagtcctttataggtctctccatctataacctgaagcaaaacaccaaacaactgtccttgcagatgtcgcgtggcaggcctggtatcagcaagctctaaggagtaggtgccagctcagtccctgcaaggagtgtcctttaagctgactttcctgttaatttgacactgagcagcactcctgtccttt

SEQ ID NO: 17439 - RNA, 9954 nt, Homo sapiens
  source 1..9954: mol_type = other RNA
tcaggccaggcacagtggctcactttgggaggcccaggcaggtggatcacgaggtcaggagatcgagaccatcctggttaacatgatgaaaccctgtctctactaaaaatacaaaaaaattagctggtcgtggtggcacgcacctgtaatcccagctactcgggaggctgaggcaggagaattgcatgaacccaggaggcagagcttgcagtgagctgagatggcgccactgcactccagcctgggcgacagagtgagactccatctcaaaataataataataataattttaaaaaagaaaaaatcatttagtagcaaaaaaaagtgaagaaataaatcaattaccaccaatacattcatcagtcaattgtaaaattgaaaataagccaatttccattatccggtgagtaagtaacctgataaaaacaagtgccctggagttcagatggctttagtggagctcggcctaacatataactgaggagtaatacaggcactgagagaatttagctccataacaagaaaacttgtgtacaagttagggctcagctacacaaacagactgaaaacgggcatttagacatttctctttcaaacagcatgaatacctaatgtcagtgagccccatgacttatatacctttaagctcatataaattgaaatttgaaggattccagccttttcccaggagaaaacttgttgttttgcactatctgtaaatctatgtgaattttcagggcttgggaagggaagagacacataggctcagttaatctgccccgatgcaacctggtttgcacctgtacaatattgcaccaaagcaacaacagcaagtgagggtcccaggtgagaagaggctcactgattctagaaaatctttattctgtaaccgaacacatcctgttttcatctagaagtagtgccttagccatatgaaggagggaactgagaacttctacatgtatgtctcagctgctctgtagagaaagaggggtgtagattccatgagttgcttaattttgctataaaggacaatatctcaacgggaaccctttatttcctcccagctagaggaagctagcagaaaaggcagcccggctctttgctggctctggctgttcatgtcctgccggctcctcccatcactcccttaggagctgggctccatgtccttgataaacatgtgggaaccttgctccctcaagggtattgccaatttagaaaagcacatctgcacactggactcttgttgggccttgtgtagtttggaaagccgaccccggtttcacgtacatggagaaactcagaatgcctaggattttgagtattttaagttacaggaaaacaggactctttcttatgtccaattctgacattgtcaaaggaaaactggttggctaggtttgagacttatataatttatgtaatgaggcctttgaatttatatagaaagagcctgaacttttattaaactggctttgcagagctactaaaggagtgatggcttttaaaatctcttctgaaatggcttgatagaatttagggtagaattattcctctactcttggaataatgttcttttgtctctaatacccaggccttggagaattagaatatggcagttcagtaggctgtggtaggaggaccctttttctgggtgcccggcaatcactaacagtgatgtgtactcagaaacagtcattgggagagcaggctgacagtggacctgctaaacactagtttgatacaaaatgttaattgaaagttacaatatattttataatatatcaatatatttcatatttaaaataaactgttatgctttctcctatcattaaaaaatagcaagcagtacagaggcaagatgcaaattcatattaaagctcatctgattctgaatataaacacttcagtttctgagcttgccatgaaaatgtttcctccattaacatcctgtcattctcttgttgttctcgtggccagtgcagaatggagagtctgggaccaaaattgagttgttgcgccattaaaaaacgtatctgatgaaggtggatcagtcctggttgagattcaaaaactgagacaacatgacacagctagagaatgttgtttattccttgtccttcttgagtgaagctggacgttggctgcttcgatctgattcagatatatatatatatatatatatatatatatatatatatatatatatatgtactttttctttttggctataaatgtcaacatctctttgggatcctaactgcaggttggagttgaattttgtgcttttcctccaccagcttggttggtcacgatgtgtctcttttgcttgtttcaacacatagcccaggcccaagattacagcttccaggatacatttttcaggtgtgtaaacaactgtcacagggcacttggcacctagatttggaggtcatatgttgaagatttgacaatggttttgttcagagggaactccagttcacgtttgggtgtttccagtaatggcgtaagacaaaaagatcacagttatatttttttctatctgtatatatgtatataccattgcactgagtactttttaataagctgtggtctgtttcaataaaaatctacatattactcgtctaacaggagtttaacattaatttctattcatgcagcctggcacaagctttctactaccacaagcagacagttactattgcgatccctgtaaactcctttctcagtggtgttaatgatcccatttccctaatgtttattttggcggcagtagagaaggaaaggatactgtctggggcgtcatcaagcccaccgactgcaaggggagagaaggggttgttcgtgcctactgggaagtcaccagatagctgtctaaggtactgaaatcaaaccctgcagagtcaatagggatccttcatctgcttctagcaactcttaggggaagaagaatgaatgtagaaaactggggacatattttaggatttaaaaacagtaacttcaaaagagtagtaacctactggtagtgcaatgacttcacagtatctcagttgtggtactgtgatgggagcaacaccgtttgtcctgggatgaaacattgattcttaatttggagtgtactgtttgttgagttgcactctggaggaggaggaaggttctggaactacgtgctaatcccatatttctccctgctgattttaccactatttaatgtgcactaattactttttggtaactactgactgcattcaaacgtaacatcaaggtgtgatctagatacagtcagtctgggctgctgttgatgacaaaggtgatttcatttgttctctattgaaaacattgtacttaagaatattaattattctcttcattttaagtacagagaaattgatgtattaggtgcttatatgaattggccaaagatgtggatccagtcttaagatttttatttattctgattttgtatgactaggtttcttcttttccatgattgtttattcacaaggaaattataaaaatttaagggggaaatcccccactatattaaaatcattacttcttcaatgctcttccttcttggcttttaataataaaaatagcttgtacatgctcagcgcttggaatttacttttgcgtacattttctatgtctcctaattcacaagattgttgttctaccactggcccctgctgaggtcggtcagtggtgacttggggccttccccccttgttcttttggattgtattaagcacttctagagacatgatgtcatgaagttacgtattaggaagatggcaagagcagttcatagacactttatgacaatttattgatgatgatcatatatatgtggcctttgatccaaaggtgaagacttttatttggacttcaatctaaggaggagtgagcccctagtctggtgtaatttaccaactaatgctatgtcctgaaattccactgagattagtggtcttaaagtatcacagtacatccctgactttacagtacatgaagctttaatatggcttaagcaatggcaggggtgggggtggttctgtatttctaattcaagtgtctagatattttaggaatattagagtgattttacctgtcactgagttgtcagaaagattatagtaggggatctgccattgggtcagtcctctaggagtgggcagatcttgatcagtacagtattggagtgaggttacataattaatagtttttacatatagccgattttttttttttttttgagacggagtcttgctcggtcacccaagctggagtgcaatggcacgatcttggctcactgcaacctccacttccggggttcaagtgattctcctgccgcagcctcccaagtagctgggactacaggtgtccaccaccaaacccagctaatttttgtatttttagtagagatggggttttgccatgttggccaggctggtcttgaactcctgacctcaggtgatcctctcgccttgcccaaagtcctgggattacaggcatgagccaccgcacctggctatatataccagattcttgagcagataattaaacctcctccaccacaaaacttgaaaataaggtacaagaaggcatgacatgagaatccacctgccccttttcccatctgactgtgatgctgaggtgtggtggaattagccaaaagatgtaggaagaaaacttgggtgagctacacccagaataattaatacttaagtcatcaagggttgattgtacttgcaggagaacgggtaactttcccacataaagctgaaatgctagtacagagaaatagccttccatttgctattacaggatcaatgtgcaggtttgatcactttttttttgaagcattttcttttgccaagaataaaaatcatgtatagctattgcactaccaataggtcaattcatgctacaaatgtccatgtgtttctaggatgccagtggctactgctaccagaaataactccagtcactcccttgactagtgttgctagtttggtctttagggtttacctaagtgagagcatcaatgatgggttaaagtcacagaccacaatgaataaatcacagtctgtgcacacttttggccaggaagagtggcagtggaatcttgcatgtcatttggttgaaattaagactaaatctctatatgtgcacacacccacactcacacccacacgcacacatatcacagggttatagcagaatgaaaacggtgggtaggaatcaccagttgaaggctgtaggtttaaatgatcaggattggcacactcagatcagcccaccagtggtcttcactttgtgaaatggaactaatgccacaaggaaactgcatggttacttcatctgtttacacatctgcttatatgttcagctgaactgtcactgaaaacaggagcaccattcttgggacatgaaacaaggaggaggggaaacattcagataatcaacagttaatagaacaagtaaaaaaataagccaacagcaggtgcggcatctctggtatgcaaaacaactaatgaaagtgttcaaaggaattatcaaggcaggccattaagactataaaccatcaaaagagcagcagcaatagcaagagagaaagaagagggttagcaagagactagatcttcctgaaaaagtggccttggctctacaattgtctaccttgtgctgtccttagaagaacaggcccagtgctacagaataaaaatctccatgccaagccactgccttcagaatggtgatgatgtcttcttacaaaggtaaacccaagatgacaaccacaagcaaaaaaatcacccttttgttttaccatcaacagatgaaatagtccatacagtgccattcaatttcccacaggcagaaaccaaagacctcagaatgagaaagtcatggttttcacgtcacaaatgttacgtgtggtcagattatggagcaatgaaaacatttttctgcgccgctcattacactaaatcttgatgtttctgaagtctcttggagtttgagatgtattggaatagtttttcgcaccaagattaacatggcacagtaggaacaggctactgacaaatccatgtccacttaccttacccacaaggttccctaagggttcccttcattctcacaatatttcattttgagatgacttaaggtcaggtagaagggaccacataggccactcttcatcacttctcctcctagctcagaggctcacaattgaggcacttggcccttttgcactactaacatctggggctggaaacctgttgctggataaatacagctcagcaaatccccaaccatatttctattcactaaggtgttattggattgctcctgtttgtgcatgtctgcacacacatgcacaatttcttgtcctctccctccacacttacagacatacacctggtcatgtggaccatcgaaacacaacttgtttggatggaagaagaaaactctgcagatgctgttatttttagaagcctgcttatccctcctgaatgccaacaattttggcttggcatccatttcaaatcaagcaaggtgcatatccaggacaaagcaatgtgcattatgtctgaagggatccacatcttcagtgaaactcagaatgtggccagaactagctaactacctgaactgaaagcaccccatgttcagattcagaccaactcaaaacacatgtaaggggtgcctattgtatgcagggtaaggtgtcaagtccctttttatttggattaagctcaaataagaaaggacctgaagcgaacgtgggatgtgtatgtgtgtacatgtacacgtttgcaaacacacaggtttatgtgggtattaatatcgagtggaaaatctggctttttatttgtctgtgtctttttttttttttttcagtctgattcgagtatatctgttttggcaagttgtgggcagctctcttttacttttgtcacccagaggcttccgtagacaaaaggaaaggagagaggtgtgttcaaagacccccatggcgaagagcccatcccccaagcctgacacaaccctccctcccagcggacccctcttctggactggcttcgctgttggctacttcagtgcatctgacccccaccccccgcgtgaagacctgagattgagcgtggatttctgttctccaccaactctgcagcaagggccctgccagaggcgtcgcttcctgtcatctcctcttcccgctcccaagtagaggcacctaaacagagattagatttctggtttcaaggcatgtcggaccaagcacgctgaatgaacatgagttagttaattagctcggtctctcttctttccgttccctggtctgaatgtttcttgatggcaaagcgaccaggagagagttgatttgcatcttaagacctatgggtaatgcttctggagtggggagatttatttagcaactgcttgaacttgtgtacggggtcgggaaggaggtggagctgaccccaatggggctatcggagattggggtgtgggtggtgcccactgccacgctgacaccccgggcctcgatgatggcagacaggagctgctgctgctgctggcgcagggtgtcggcgatgagcagcggcagggagttgaagctggcggtgagatgctccagcttcgactccaggctgccaatctgcttctccaggtcttcgctccggtcattgagttctgtgattaagtcatacatgacattctgcatcttggaaaggtccaccagagtgttggcttggtcactcagcttcctctgttccatcttgacgctcctcaactggtggatagcttggaggaacttcctctggtgtttcctcactttggcatggtcaatcttctttagcagctttgtgtgtttatagattaaccatgtttcccgaaggacattggctgcagcattcttgatccgcttggtgagctgagtgtccatcatgaagttatgaacgtgcttctccgctttggtgagttccagctttcgggccaccacggccaccacaagggcagtgcagcctgcacccatgatgccagtgaggagacagacacctttcccacagtatgtgtggggcaccatgtccccataaccaatggaaaggaatgtgatggagatgagccacatggcacccagaaagttactagttacgtcctgctggtcatggtacctttcacagacacggacggtccaggcagcaatgatccacagagagatgctgaacacgagcagcacagtgccagggcagatggtcatgagcgtcttcatgacaaagcgggtgttgaagttgatcttgttgagggccccgatgctgcgggacgaggcatcggtgaagagcttgctgtgcagcagcatgactcgggcgatcaggtacaggcgcaggaacatggggatagacaggatgatgtccacatcggcctccgcccgggagggtgtgtaggagaaggccaggcgtgccgtccagaagaacttgtactcgccaggaatggggtggatggcgcacaccagcatctccaggctgatgtacaggatgcgctcgtaggtcatggctatccgccagtcatccgcgccattgtcgatcacgaagagctggacttcacgtgtgtggtaggcgatgatcaagcccaaaaggatgatggtggacagactgataaggcatttcagggccaacgaaaacatggagtcctttgagtacaaaccccaagagagctcggtctctatcaccataacaacaattccaaacatcccaaaaatcagagcatagtcactcagtcgctttctcttttcaaacagggccctcctgtgtcccagcttatagccaatgttttggtttttccgcttgttggctttggggaaggtggtgctgctggcggtggtgccggcatgctggtggttgtgggtggcattagggtgatggagcagggtctggtgggcatggttgtcctcccgggaggagatgacgatctccggggggttgctagggctgaaaagctggaggggttggccctcagtctcggcctcgatgaggttcctccgggaggcgctgaggcggctgaggggcttcatgaccccaccgctatacttgcaggagctcatggcgatctccgtgaaggggttgctgtcccgccggtgcaccagggggctggcctgtcggtgccggctgcctccgccaggcccacttgtagctgtggaacttggagagtggccaagcaagtggtcattgagattgagctggctgccttgcctggaggaagggtggaggatggcggtggagttggacgaagggggggccctgaaagcggtgggagaggagtgcagcaggccagggtggacgggctggctctggagttgggcgagctgagacaggggatgcggtggctgctgctgctgctgctgctgctgctgctgctgctgctgctgaagctgcggaggctgaggctgcagcgagggtcccaggggctgctggggggctgctggtggcgctggcggtggtggctgctgctgctgttgctgctgctgctgctgctgctgctcatccccagaggatggacaggggcacttggggtcttcatccaagtcccccacccccgagtcatggaagtgcccagaagtgtccatcttggggcctggctgtattccctgcagcacaagcccccaccccaaagccaccctcgctccaaagatgtcctcaaagaaagccaggcatccaatctcccccaccagtatcttggctccagtcctctctttggcttgcttcggttctctggggctgcctggagtccagacgctgccactcaagaatgcattgtattgggcagggagggagagcaggaggggagcttggagaaagaagagggggtgaaagaactctctcaggaggtggtcctctaggagcgtgtgaggccaggctcagcttcactcctcgctggctcaat

SEQ ID NO: 17440 - RNA, 1933 nt, Homo sapiens
  source 1..1933: mol_type = other RNA
tcaggccaggcacagtggctcactttgggaggctgaggtgggcagatcacctgaggtcaggagttcaagaccagcctggccaacatggcaaaaccccgtctctactaaaaatacaaaaattagcaggacatcgtgatgtgtgcctgtaatcccagctacttgggaggttgagacaggagaatcgattgaacctaggaagcggaggttgcagtgagttgagattgcgccactgcactccagcctaggcaacagagcaagactccatctcaaaaaaaaaaaaaacaaataaaaataaaaaagcaaatctgaattcaaaccaatacctttaaagagaaatgtaaaactcagtttaatttcaagtttgtatagagaatgtatgccacagtttgtattttataaacacaacctatcttattataaatacaaaataagaaaaagtgatacgttagctgttatgaagggtgaaaacattatataaacttcaaaaggctgctttctgcatctgcatctatgtaatttcatggttctctaccaatttcatttacagaaataatctctatagtcaaattattgttcactttcatgccccaacatgggaagtggtaggtgaatatctgtaggaatacaatttattgtctgctcctccactcagaagtagccctgtgtctgtccagtctacactcagaactttgtcttcatgagcagccagatcatagagaggagccttacaacttcttgtatcccacagcttaacaatgttatctaaagatcctgaaatcagctgctgttcatgggtaggagaccattttactgatgtcacccaaccagtatgtgacgttagggacagcgacaccaaagaaccatctttagttcggggatcccacagtctgatatgcctatctgtgcttccagatgctaaacgtttacaaagtggagaataggaaatacaattaaacactttatttcctgtcaaagttgacttaagactgccagactcaacatcccacactctaattgtatggtcccaagatgcactgcagatttcttcagcatctgaccacagaactgaggaaactgcctccatgtggccagagagggtcactatgggagtccttgttagtcccaactgttctgtcttctgtttctttcttggtcgatttgtggactcctccatttcatcttcttcatctgtagggactgtagaccagatctttagcatcttatcccaggagccactgcaaaatttagttcctgagccatcaacagctatagaatctacacttccagcatgacctctacagcagtgtagggctttcactttgtttctctctacattccactcccataagagaatagtctgatccatagaagcactcaataataagcaggacaaactatcattcctctgcccctttaattgaactgatccagtcatcatggaacatgcattgctctggctggggtgcagtatacttctccacgtattctatttccacaacttcttctgatgagatgttctccatttccatgtgtttgtccaagggcattcgcagaaactggcccttaataaggaaatcaaactccacatgtttgtggaactcatttttgtcctttagtagtttattgatgatgttactaaggtcggcaatttcagaggcagcagggattgagaagggaacatcatctacggcatatttcttgttatcagtgtagaagcgtgtttggagctgagccatggcgaggagtacacacgacttgcccacggaaacgtacgggttagcagacccacaacacgaagctcctgccttttaagactacaaagaggcagctcaaaattagactgcacaggtaagcgaggaactgcagtctaagcctggactctgccttctgccctccggtctcctctgcagaaagcacgaggttgcccttctac

SEQ ID NO: 17441 - RNA, 2049 nt, Homo sapiens
  source 1..2049: mol_type = other RNA
tcaggccaggcacagtggctcactttgggaggctgaggtgggcagatcacctgaggtcaggagttcaagaccagcctggccaacatggcaaaaccccgtctctactaaaaatacaaaaattagcaggacatcgtgatgtgtgcctgtaatcccagctacttgggaggttgagacaggagaatcgattgaacctaggaagcggaggttgcagtgagttgagattgcgccactgcactccagcctaggcaacagagcaagactccatctcaaaaaaaaaaaaaacaaataaaaataaaaaagcaaatctgaattcaaaccaatacctttaaagagaaatgtaaaactcagtttaatttcaagtttgtatagagaatgtatgccacagtttgtattttataaacacaacctatcttattataaatacaaaataagaaaaagtgatacgttagctgttatgaagggtgaaaacattatataaacttcaaaaggctgctttctgcatctgcatctatgtaatttcatggttctctaccaatttcatttacagaaataatctctatagtcaaattattgttcactttcatgccccaacatgggaagtggtaggtgaatatctgtaggaatacaatttattgtctgctcctccactcagaagtagccctgtgtctgtccagtctacactcagaactttgtcttcatgagcagccagatcatagagaggagccttacaacttcttgtatcccacagcttaacaatgttatctaaagatcctgaaatcagctgctgttcatgggtaggagaccattttactgatgtcacccaaccagtatgtgacgttagggacagcgacaccaaagaaccatctttagttcggggatcccacagtctgatatgcctatctgtgcttccagatgctaaacgtttacaaagtggagaataggaaatacaattaaacactttatttcctgtcaaagttgacttaagactgccagactcaacatcccacactctaattgtatggtcccaagatgcactgcagatttcttcagcatctgaccacagaactgaggaaactgcctccatgtggccagagagggtcactatgggagtccttgttagtcccaactgttctgtcttctgtttctttcttggtcgatttgtggactcctccatttcatcttcttcatctgtagggactgtagaccagatctttagcatcttatcccaggagccactgcaaaatttagttcctgagccatcaacagctatagaatctacacttccagcatgacctctacagcagtgtagggctttcactttgtttctctctacattccactcccataagagaatagtctgatccatagaagcactcaataataagcaggacaaactatcttttttcacccaggccacatcttttacaacatccgtatgtcccacaattgtcattattgactttccttccaaggaccagatccgagaagtcttatcataagaaccagtcaagatccattcctctgcccctttaattgaactgatccagtcatcatggaacatgcattgctctggctggggtgcagtatacttctccacgtattctatttccacaacttcttctgatgagatgttctccatttccatgtgtttgtccaagggcattcgcagaaactggcccttaataaggaaatcaaactccacatgtttgtggaactcatttttgtcctttagtagtttattgatgatgttactaaggtcggcaatttcagaggcagcagggattgagaagggaacatcatctacggcatatttcttgttatcagtgtagaagcgtgtttggagctgagccatggcgaggagtacacacgacttgcccacggaaacgtacgggttagcagacccacaacacgaagctcctgccttttaagactacaaagaggcagctcaaaattagactgcacaggtaagcgaggaactgcagtctaagcctggactctgccttctgccctccggtctcctctgcagaaagcacgaggttgcccttctac

SEQ ID NO: 17442 - RNA, 1133 nt, Homo sapiens
  source 1..1133: mol_type = other RNA
tcaggccaggcacagtggctcagcctgtaatcccggcactttgggaggcccaggtgggcggatcactagaggtcagaagttcaagatcagcctggccaacatggtgaaaccccatctctactaaaaatacaaaaattaccgggcatggtggtgtgcacatgtagtcccagcaactcaggaggctgaagtcccagcaactcaggaggctgaggcaggagaaccccttgaacctgggaggcagatgttgcagtgagctgagatcatgccactgcactccagcctgggtgacagagcaatgctctgtctcaaaataaagccttggatcatagaaacccagtgtggggaggggctcctgatctggatggattaagcaatacaatttttttttaacagtatctttttaatggccttttctactttttcctgtctaggcttcctgttaagacctcagttaccccagaacaccctgggttatttttctcctcacctccaatacttcagtgttgccagataaaacgcagagtgcccagttaaatttgaatttcaaataaacaacagggagtcctgtatttttacttgctaaatctggcaagttcatgggagggcttatgtgttctatttttctctctgggcttatctgcaaatttaggataataactcacccttttcttcctgttactcatacacaatgactatgcaccctgctaaaagtcacttgactgaagagatggttcacttcatgttagggtaagggcaggctatctagaaatggtcttgattgatcagtgttgaagttacccaggaaaaaaaaaaaacacccattcagacattggcatttaatataatttttgtcaaatgagtccgtcatacgaaacgagagcatcattttgagtagccagatgtcaacattgctctgatagagctaggtgatggggtagaagggaatcctaacaacaacaaaataactcagcagaacctgtgctgtaccatatttactctttatggtggtaatatatatatatataacatagaatttaccattgtaataattcttaagtggcattaaatatattcacattattgtacaaccattactgataacaatctccagaactttttttcatcttcccaga

SEQ ID NO: 17443 - RNA, 49 nt, Homo sapiens
  source 1..49: mol_type = other RNA
tcaggccaggcacagtggctcaggcctgtaatcccagcattttgggagg

SEQ ID NO: 17444 - RNA, 13861 nt, Homo sapiens
  source 1..13861: mol_type = other RNA
tcaggccaggcacagtggctcatacctggaatcccagcactttgggaggccgaggcaggcagatcacctgaggtcaaggtatttgagaccagcctggccaacatggtgaaaccccatctctactaaaaatacagaaattagctgggtgtggtggtgcacacctgtaatgctagctactcgggaggctgaggtaggagaatcgcttgaacctgggaggcagaggttgcaataagcctagatcatgccactgcactcaagcctgggagacagagcgagactacatcttaaaaaaaaaaaaaaaagtattatgagagaggataatgtattgtaatgtattgtagaggctaaataaaattatgctcatgtcagaaaaaaagagtatttctcaaaataaaattcactgaaactggatgtttattttgactgagatatagtatatcctcaaattgccatagaaagtttacaagaatattagaggtaaattataaatatcagggcctttttaaaaaaaaaagattctgcttataacttggtatttgtttataataaaaattatagtagccaataatgaacacttactctggcttggttatttacttaggtcaaaagaaggaggagcggttaaactgtgggatcaggaactgaggcggtgccgtgccttcaggcttgagacaggacaagccacagattgtgttcgttctgtgtgcagaggcaaagtaagatgttccatgagctgatacagtgcagcagaaaacagaaagtggttattactgtgattccctcaccctttgcagcctaatgaacaatacttaataatgcataacgatggatttgcttgccaacattactctgtctttgctgctttctttgccaaagttagcaccagtgtggtgcataagctaggaagctattctgtctaaatactgtatgtaaacctccaatattttctagaatctgccaatttaacaactctagtagacataattgaaagcccttggcagttgactcatattaggacagctgtctccattttttaaaaaaacacacattccctagataaaacgtgcagtaaacaaacaatgaaatactactcagccataaaaaataatgaaattctgtcattcttggtggcaacatggatgagactggaggacatgatgtgaagtgaaataagccaggcacagaaagataaatacatgttctcactcctgtgcagaaactaaaaaagttgatcccacagaggtggagagtagaatagtggttactggaggcggacaagggggagggggagggggatagggaaggactggttaaaggatacaagtttacacagccagataggaatagtatgttttagtattctgtagtactgtaggatgactatagttaagaatcacgtatttatgtattttcaggtatttacaagagaggattttgaaagtttccatcacaaagaaatgataaatgtctgaggtgatggttatgcgtattaccctatgccctatagatatgtataattatgtgtcaatttcaaaataaaaattcaaaactacaactcctatgaaaatttttgagcgtgtttgtacttattaagtgtatttataaatcatacggatattatcttcagcctgcatattaaattgtagttaagcttttactttttaactaaaaaataaattctattattttttcctatatcccactgcactgaccccagtttggaaatcctaagattatcaaataaaaactttgattattgaagaatccaggtgtactgccacagaaaagttctattctgtagcatggactctaatatgtaatctagcccattgtgcttacagatagatgtgtgcctgtagtcatagaaaaatttgcatgagctaatgactgccttgctactagattagctcaaagcaaaaagttctctgaaagcaggtcaatagggtcatttttatattatgaagaagaaaagcagctgttgtattacattcactgtattggtcctgcttgtgtttcagggcaagatccttgttgggacaaggaatgctgaaataatcgaagttggagagaaaaatgcagcttgtaatattttagttaacggtcatgtggatgggccaatctggggactagcaacacatccttccagggattttttcctttctgctgcagaagatgggacagtgagactttgggatattgctgataaagtaagtacagataatttttttaaaagaggttacaacttctaaaaagaaaagttggaagttctaaattgctagtacttaaagaactgccagaattctgttgagcattttgaggggaaactggtataatttagaagtacttcacttaatgtttcctatgactctttttttttttttttttaaatgcagaagatgttaaacaaagtgaatttgggacatgctgctcgtactgtgtgttacagccctgaaggggacatggtggctattggaatgaaaaatggagaatttatcattttactagtgagttctctaaaaatatggggaaagaagagagacaggagatgtgcaatccatgatatcaggttagtgaacaaatggaatagagtttctagtatatacttgatttaacttccatttgtaaaattttccatagccttgccttcaaaaagaggtccccagggcctgtagcatttcccgtattataaattgtatgctaaaatatggctgtttgtatactacttaattcttcttgctaaattataaacccactgggcaccaactataatagcaagtactagtaggtaatgtttgatgaattcatgttaacacttagccatgtccattaagttcatcccaccaagaggtatctcccactgtaatacaagagagctatctgcccttcaaaagttgtcaccctggaaaactaaagttgtgatttcaaacatatcttctcttagtaacctcagtttgggaatatgtagttcattaatttaatcaatacctattgattaaatgttccagaatccaaattaatttaaatgtttcttaaacctttgtttttcagtgcttaagcatttttcaacagtggctaccatttacggagtacttccgtgtgatcagtagataagattattgaatctaggtctgtcaaaagcttgtacacttttcatcagtaaaatccttttacaaatgaaaccttcctcagaacttcaatatataaaatagtaacagtggcttcccttagcttttacatgtctctatcgtacctcagtaagactcatgggccatttcaagagactgaattgtcccatatgactccaaagattgctaggcaaatagcatttcactttgtcttttaaataagttcttcaggccgggcgcggtggctcatgcctgtaatcccagcactttgggaggccgaggcaggcagatcacctgaagtcaggagtactcgaccagcctggccaacatagtgaaaccccatctcaactaaaaatacaaaaatcagccgggcgtggtggcaggcgcctgtaatcccagctactcagggggctgaaacaggagaatcgcttgaacccgggaggcggaggttgcgccatcgcactccagcctgggagacaagagcgagacttcgtctcaaaaaaaaaaaattcttcttccaagattcaagttgtgtcatttcaccttaataactggaggttagttaagctgggctgtgttctttgcttaatattaagacaacgttttttccagatggaagaaaactatcttaatgaattgttagcttattaattatgtaatgctaatggcttttaaaagctgagatgttctgactgggtgttgtggctcacacctgtaatcccagtaccttgggaggccaagggggaaggattgcttgaggccaggagtttgggaccatagtgagaccccgcctctatttaaaaaattaaattttgttttgttttgttttgagttggagttttgctcttgttgcccatgctgaagtgcaatggtgcaatctcagctcaccacaacctgtgcctcctgggttcaagcgattctcctgcttcagcctcccgagtagatgggattacaggcgtgcaccaccatgcctggctaattttgtatttttagtagagacagggtttctctatgttggtcaggctggtctcaaactctcgacctcaggtgatctgcccgcctccgcttcccaaagttctgggattataggtgtgagccactgggcctggcctaagaaagtttttttaagccattagacgtttttaaaggaattgggagatgacaattggggaaatatttaaaatttaagtaaaatataaagcttccttatttcatgtaacccagacaatctcagtatacatgatcagttgtgtctgacaggtaaatctatttgaggccttatcacacgttacttttaagaactagaaaggaaaagtcactgatcttaagtatttataatacttcatgtggtctaatactttttacgttttgttttgattcagatttagtccggattcccggtatctggcagtaggttctagtgagaactcagtggatttttatgacctaacgctgggccccactcttaacagaatcagctactgcaaagacattccaagctttgtcattcaaatggacttctctgcagatagcagttatctccaggtacagtaccaatactgtatacccaggtggcaagttcttctgcttttacatttcgtgttagtgaatgcatttaaagttcctgagctccagagctccagcttctcaactcctccctttgtaccttctgacctacagctcccctttcctcccccacttatcagagcttttctcctattaagtttttgtagtgatcttttgcatacttaataatgttagacatgtaaatcaagtagcaatatgctagtattctgtaaaccccctgtggattttgtctctcacctaatggaattcttgtcccattttaatctgatgaaaaaggtctctagtggctgctataaacggcatgtctatgaagtgccttcaggaaaacatcttatggatcatgccgctattgacagaattacttgggctacatggactaggtaaatacttatatattcacaaggcaagaactgactttgaaggccagttagaaaatcctatttctgaactgttagagccattccaataaggaatagtaattgagtttcaagtttttgttaccatattttgaaatggtatgttcatgttgggacccctttttattgaatatatttccatgttttatcagtttccatgatttatcaagttttttttttaaggaaatcaaagttttaactttaaagataccctgatatttttcttaatgctaaatttaatgactggcaaaaaggtattgggtgctgttaagcaactgttattaattctctatctaaaggaatgctatcttgaatctattagaagtcaaagcttccaaatttgttcaaatttcctggctgtatgacaggtaaccatgactatccatttttttggccaatgaaaaatgccatcaaattcctgtatcagccaggcatatagtggctcatgcctgtaatctctgatgtagcaggccgaggtgggaggatcacttgagcctagaagttttgataccagcctgggcaacatagcaagaccccatctctgaaatttttttaattcctatgtcataagtcatttttatttttgtagagatagggatctcacaatattgcccaggctggtctcaaactcttggcctcaagcagtcctcctgcctcagcctcccaaaatgttgggattactggtatgtgctgctggacccagccaagtagcacttttaatttgaaaaatagttctatcagttttcagtcaggcgcggtggctcagcctgtaatcccagcactttgggaggccgagcgggggtgatcacctgaggtcgggagttcgagactagcctgaccaacatggagaaaccctgtctctactaaaaatacaaaataagccgggcatgttagcgcatgcctgtgatcccagctactcgggaggctgaggcaggagaattgcttgaacccaggaggcagaggttgcggtgagccgagatcatgccattgcactccagcctgggtaacaagagcgaaaactccgtctcaaaaaaaaaaaaagaaaaaatagttctatcagttttcataaagtactactttaatcttaaaaagattaatctagaaacccttcaaattataaaatgtcatttttaaaaggcaggagttgatatcctgatgaaattcaggtctccaaacaacttaccataatttacttcctgtattttaagtaacatgatagggtacttagagattaattgccaagaaactttttgaatatagtcaacctgcccgcacttgccatgatgagttttcttttgttccttccctctagtattctaggagatgaggttttgggaatctggtccagacatgctgagaaagctgatgtcaactgtgcctgtgtatctcattcaggaatcagtcttgttacaggagatgactttggcatggttaagttatttgacttcccatgtccagaaaaatttgtaagtttgtgttttgtttactattatcagtttactcctaattttgatgtcttatcatcagcacttttccccatatatttaaaatgttttgtcctaatttctaaatttttccccaaactttctaaatctatttactttgaaataaaagctattagaaacaaatcctctccctcgagtaataccatctttggaaccatcctacaaaagctgtaattagcttttcaccaaacctataatcagttatcaaatttcaaatgcttttccttagagaaaaatggtcagagtacctggagacatctgactgcccacacagcctggttttgcagatccactactcatgctgaaaagcattctaatcactggctgcggtgctaactccctactctctccacagctcttgtcatagagattatagttcctaataagagcctttgacttctgtgtgcaccaaatgccctgagcttgtctgtcattgttttttaggcaaaacacaaaaggttcttgggtcattcgccccatgtgacaaatattcgatttaccagtggtgatcgacatgttgttagtgctggaggtgatgactgcaggttagtaactttctcagcccatgaagagcagactatgttactagttaagagacttaatacaacaactcctacagctttggtttatgaaatcagctagtcaacattagtagaaggtagtataaccagatggctcttcagaatctcatatttatgcaaatacagaataaaaggagttaaagaggaaaaatattacacatgtaacctgaaagcacaactgaaaaatattaaactgttatgaaaatctaaaaacataattaactccctgcaattttcttctctgattgcagcttatttgtctggaaatgtgtacatacacctcactgagagatgctgagatgactacagaaattaactttgagaccagaattacagagaagaaaaaccaaaacccaaccctgcatggtcaagtggtgctaacccaagactgtaacagggagaaatgcccagaatcatcaaaatagtgaaagactgatctgttcaaaatatttgctatatgcactgggtataatccgtaatccatacactgccagataatgccatttcaaggaaggatcgaatacttgatggtaaaggccaagtccccctgtattgggaagtgtgtgatttcggcagacctgctgggaaaatttagggtagagcactctttacagaagaactcaaaaacccaatttggataattttcattatctttttagcaaaatggtttcttaatgtttatattttattttcaaggttcattgtttaatgaaatattttattcttgcatttccataaggaaagggaaagtcatgatcatcctaaaggatcacagtttttaaaaggcaaacattttccctaaggaaacagacacaagctttcctagagaatatgatgttttttaggcattaataaggtccttttttataaaggacacttttctcctagtagttttgaattcaggaacagatccaaagttagcagtatatggctgctacatttccattttcattttcgagccatcagtttatgttcagatgccatctctgtaatcgcacatttaaaacataactgtagcctcactaatggaaaagtagtatgatgaacaatcattcccaatggtgtacaatgtaagggttttagggagcaacagtatttaactggaagaaagaattgcatatttaatgtagtctaatatatacacatttgtttaacatgtaaacaaaagtgttaaattcacatatacaacattatacaatttaatcactcttggaataaaatttttatagccttttttctattgggaaaatttgtttagatgtgtgccactccataggtttatttccaaaatgaatgagcccaactccatttgtaaaaacttgtcagttagaattcctttttttagtggattagggctgaattcttagatccttatttcttttcactttaaatgctgccaaagatcactactcatcattcaggaattcgctgtctagcctatctgtagtttcctgaagattgaaaattatgtagactgctatttaaaaatatatttttctaagtgtgaggtttaagatgctgtattgaccctatgagtttttaatgtgttaattatctttatagcataatagatcgctttaggttcctggaatcccatttggtctgacaggatatatgaagattcttaatacctattttctgtgtctaatacttggttaatactaaaaatagaaatgactaaattacatcacagaaagcataaccagtgattgaacctggtagttttaaagctctaaatagctgtggctgaaggactgattatggggctaagaagcttgaaacgtaagttggtacttgttcatcagtggattctcctaaattaagccaaattttgaaatacatgactattaagtttctactcatgtatttacagtcagtcaataaattaaaggaggaaaaaaatccctgaacaacctgcccataaaaagaaaaatactctacatttgagcctgctgcagttttaaattttccctctgggtcaagtttgccagcttttggctacagagaaattatatttccattacagtgcaggtagaaactctgtaaccttaagcatgtaaactacatagaataaaactgtttccactgcatttctgtccttcaaagtggccaacctgattaagtcagccttaatcactgctgctgtcagtttcacgactaaaggtcatattgactaagtagtcatcagctgaccacctcgctgtatcagccagcaacgaggggaaggtgaagaaacatgataggccatatagaatctgccctatgtttacttttttaacccagataattatttttgtgtgcagtatctaagctcctgattgtgtaacctgggacttctggcaccttttgttccattcattttatgtataaaatgcatgccaaagcacactgtgccctctggtacccttgcttccaatcgccaaccatgctcatttccttcctttttttgtggtccctttttgtggtgatcattttaaaccacgtcatccaacaaatgttttatggtcaaccttagcttgttcataagccatagcaactgaaagattaaactcttaaatatgtgtctgggcagtggctattaaatagcaaaaaacaatcagattttagtattttattatttccttgtaaaatggctgaactaaattaaacccttgtttcccatttgttctataatttatagtgaaactgagaacaaaactatctttataaatgatagctaaaagtatttccagatatttaaacaatttaaaataaatttcttctgcagagatgcaaagcatctcaacactggaatgaacaaatgccttaaattcaatggagtaaacctttagaatgaagaggaactgtcatttcacccaagccgaagacaacagccttatgcacttgtgtgctctgtctttgctgcttctcgtgtttcaagcctttcctgtgggatcagcacagcaaagtgcaacttaccaaatggtttaatgactggttaattctttcttctcccaatggaaaagcaatggcaacacaacagtagactgctggcttgacaatcttaaacgtgagcctttgcacatgtaggtttatcatcatttgagtatacgactaagcaagtcaatgaactttttttttttttttagcagtttaatttggtcctgagaatgttgcagtctttattaccccttttgcattaatccacttttctaaccaccttttaagctttaatttttaacactatacaccaagtctttgaaatcagtgatctgttatttaactctaaagcatttgacacttcttgccttaacagttttaaaaaccacacacaaaaaaactctgtaagtaatacagtaggccaaaagtttcatcctatctatcttgcagtttacctatctgatctgatctctgtaattatagttctgtcatttaaaatatactatttaaatctaatttttacatttcaaaaattatcttcagtagtaactaagtatattttctgtggattctgagaatgttatttttcagaatgtgagaatatatatgtacatttataatcttgtgactttaaagtctgttttcagatacagtatgtaaatacttgtaaaaaaatttgtataattttgtgataatgtagtttcccaaaaaaattatttagaaggcattatgttattagtaaatgagagcactgtatagaactgttcctattttctgcacttgccattccagctgcctccactgtccatacccacctcattcatcctgtcacagaaggcaggaaaactgggaactttaccaaagtagcactcagcctgagaggcctgtataatcatgcttttcaaactaaattcacttaaaaattaaaaagcagaattgaatattttaagcagcctcagtacctttggccaatgctgttttcatggtggattatgaacattatataatctttgggaaaagtgaaagtagtacaatttttagaataatgacaactgcctcactgcatctctccactcacacagcaaccgtgtagccccctaagctgcagtaccatgactaaccatgatgtcaatttcatatgctgatcctcacaacagcagtgcacaaacatgccccaaatattttaacagaatttagctcttccttaagctgtcttttcatagtaaaaacaaaacaaaaacacccaatgttaaaaccacataataaacttacaaacttgaaaaattagacacttcagatagataggcaataaaacttcatattatgaaagcaatatattccaagtttcaaagatttgacaagttctgtagagtatctttcatcagtacatgaaaacttccaaactgcatgatcttctgccaggcaggactgggtgctattcgctggtttgaggtcgaatccatttcaaggcatgtcgtggtgggacattaatggtgggatggtagaatgtgcagtccggtcttgtacattgagtgttaaacctacaatgttttggatgatagaagggacattccatcttcttacaagcagggaagtaacggcagagctgactactggaaggtggtgctggtggtgcaactgctggttttggagacagtactggaattcttctactcacatgagtgaagggacaatctggtttagtacactttgcatcatatttacaatttgggtgaacaaacaaacatttttcagcaaatttacaattggggaaggctttgcagggtgagatggggtgatggtaggcacactcatccccatttttacaagcaggccagtacttgcagcgctccaaaagtttttctggtttctgtgccacactcagttcactcatctcagcatttgggtcctcaagctgcctgctcagcaagtgcaactgctgtgggtggaggagacctctgagtcccttgtttgaggctgcagtttggtttacgggtttcattccttcaaagcacatgtcctcctcttgatctgacatgtatcctggggggctggggacaccatccagcgtcactataaacttgggacttgcaggtttatctggttgtacaagatctcgtgtctgcataaggtgtcctgaaagtacccgaagggaatctgcagtcttcatccccgactcttggtttggtgccactactacttcctcagacagctttggcttcttcagaataaatgatcttgtgtctgcatggaccatggattccatgtcatagtaatcttgactcatctgcagagtttctgccattactgggtcgatttgcagtcgggataataattgcctctgttgagttccttgatttttttctacagaatctccttttgtttcctcttctttaatggggggacttattctgggggtcctactttgtccctggaccacttctgctagcaattcttcttgagaagttcgagttctgggagcaactggaagtgtctgtttctgtggaactgtagagtagttagttgtttttgttacggattcttgagcttcagatatagccttcaaaatcagattcttgttagcttgtttagaaggtggaagagaaggtctcctttcaggctttgcaggcacagacacactgctggagatgcttcctgttcgagacccgtaatcatcatcttcttcctcctcttctccatcatgattgaatttttttactttaacaactgaacttaccacaggcaactttctcttccgaaagttttcatcctccatactcattttctccgagttgtttctaaagaacggactatacgtttcttctaagctgttaagcacctctggttcacacaaacgtcctgtttcatatacccaactactctgcatatcaagctgcttggcagcatgaatactattctgctgctgttgaaattgcaacctgtttaaatgaacaccactatctgcatttctacttgcaggtggtcgataaatttcaatagaagggcgagaagaaccatatgtaagtgtcactgtaggttttttctgagataagggattctcctgcacaaagttgaggtcttcgtcaatgagatcatctggttctggcttaatatcaatcacatcttcagagggtgctggctccctcaaaggtttcactgttgacattagtcgggttgcagctccatcatcgtaagtctgtctgacatttgtggtttttgactcctgcgaacttgtagaaactctggaatctcttttttcaggtctcgcgctaggaatggcaagtggtggcactgcagcttcatgcctcctctcatctccccgactgaaattgctcttgtttgaaggcacgttactatcaaagatgttggtatcagaagacttcagactagagggttcagttgtaacagagcgaagtttatctaatacaccatgaagccatacggtgaatcgaattgtgttgttccctagaaacagggacagatcctctgtcatttggtcctgacttttcttgttggccaccatcaccataatgtaatcaggaagttcttcatcaacataagctcctaattcttgtaatttccccttaatggcactccggatcttgcggctgatctcggtgccgatctccatggctctgcggcgtgcgggaactcagcactgcgcggcgcttggcttacccggaggctgccgcggactcctaccccgcagccgggacaccaccgcctcc

SEQ ID NO: 17445 - RNA, 13786 nt, Homo sapiens
  source 1..13786: mol_type = other RNA
tcaggccaggcacagtggctcatacctggaatcccagcactttgggaggccgaggcaggcagatcacctgaggtcaaggtatttgagaccagcctggccaacatggtgaaaccccatctctactaaaaatacagaaattagctgggtgtggtggtgcacacctgtaatgctagctactcgggaggctgaggtaggagaatcgcttgaacctgggaggcagaggttgcaataagcctagatcatgccactgcactcaagcctgggagacagagcgagactacatcttaaaaaaaaaaaaaaaagtattatgagagaggataatgtattgtaatgtattgtagaggctaaataaaattatgctcatgtcagaaaaaaagagtatttctcaaaataaaattcactgaaactggatgtttattttgactgagatatagtatatcctcaaattgccatagaaagtttacaagaatattagaggtaaattataaatatcagggcctttttaaaaaaaaaagattctgcttataacttggtatttgtttataataaaaattatagtagccaataatgaacacttactctggcttggttatttacttaggtcaaaagaaggaggagcggttaaactgtgggatcaggaactgaggcggtgccgtgccttcaggcttgagacaggacaagccacagattgtgttcgttctgtgtgcagaggcaaagtaagatgttccatgagctgatacagtgcagcagaaaacagaaagtggttattactgtgattccctcaccctttgcagcctaatgaacaatacttaataatgcataacgatggatttgcttgccaacattactctgtctttgctgctttctttgccaaagttagcaccagtgtggtgcataagctaggaagctattctgtctaaatactgtatgtaaacctccaatattttctagaatctgccaatttaacaactctagtagacataattgaaagcccttggcagttgactcatattaggacagctgtctccattttttaaaaaaacacacattccctagataaaacgtgcagtaaacaaacaatgaaatactactcagccataaaaaataatgaaattctgtcattcttggtggcaacatggatgagactggaggacatgatgtgaagtgaaataagccaggcacagaaagataaatacatgttctcactcctgtgcagaaactaaaaaagttgatcccacagaggtggagagtagaatagtggttactggaggcggacaagggggagggggagggggatagggaaggactggttaaaggatacaagtttacacagccagataggaatagtatgttttagtattctgtagtactgtaggatgactatagttaagaatcacgtatttatgtattttcaggtatttacaagagaggattttgaaagtttccatcacaaagaaatgataaatgtctgaggtgatggttatgcgtattaccctatgccctatagatatgtataattatgtgtcaatttcaaaataaaaattcaaaactacaactcctatgaaaatttttgagcgtgtttgtacttattaagtgtatttataaatcatacggatattatcttcagcctgcatattaaattgtagttaagcttttactttttaactaaaaaataaattctattattttttcctatatcccactgcactgaccccagtttggaaatcctaagattatcaaataaaaactttgattattgaagaatccaggtgtactgccacagaaaagttctattctgtagcatggactctaatatgtaatctagcccattgtgcttacagatagatgtgtgcctgtagtcatagaaaaatttgcatgagctaatgactgccttgctactagattagctcaaagcaaaaagttctctgaaagcaggtcaatagggtcatttttatattatgaagaagaaaagcagctgttgtattacattcactgtattggtcctgcttgtgtttcagggcaagatccttgttgggacaaggaatgctgaaataatcgaagttggagagaaaaatgcagcttgtaatattttagttaacggtcatgtggatgggccaatctggggactagcaacacatccttccagggattttttcctttctgctgcagaagatgggacagtgagactttgggatattgctgataaagtaagtacagataatttttttaaaagaggttacaacttctaaaaagaaaagttggaagttctaaattgctagtacttaaagaactgccagaattctgttgagcattttgaggggaaactggtataatttagaagtacttcacttaatgtttcctatgactctttttttttttttttttaaatgcagaagatgttaaacaaagtgaatttgggacatgctgctcgtactgtgtgttacagccctgaaggggacatggtggctattggaatgaaaaatggagaatttatcattttactagtgagttctctaaaaatatggggaaagaagagagacaggagatgtgcaatccatgatatcaggttagtgaacaaatggaatagagtttctagtatatacttgatttaacttccatttgtaaaattttccatagccttgccttcaaaaagaggtccccagggcctgtagcatttcccgtattataaattgtatgctaaaatatggctgtttgtatactacttaattcttcttgctaaattataaacccactgggcaccaactataatagcaagtactagtaggtaatgtttgatgaattcatgttaacacttagccatgtccattaagttcatcccaccaagaggtatctcccactgtaatacaagagagctatctgcccttcaaaagttgtcaccctggaaaactaaagttgtgatttcaaacatatcttctcttagtaacctcagtttgggaatatgtagttcattaatttaatcaatacctattgattaaatgttccagaatccaaattaatttaaatgtttcttaaacctttgtttttcagtgcttaagcatttttcaacagtggctaccatttacggagtacttccgtgtgatcagtagataagattattgaatctaggtctgtcaaaagcttgtacacttttcatcagtaaaatccttttacaaatgaaaccttcctcagaacttcaatatataaaatagtaacagtggcttcccttagcttttacatgtctctatcgtacctcagtaagactcatgggccatttcaagagactgaattgtcccatatgactccaaagattgctaggcaaatagcatttcactttgtcttttaaataagttcttcaggccgggcgcggtggctcatgcctgtaatcccagcactttgggaggccgaggcaggcagatcacctgaagtcaggagtactcgaccagcctggccaacatagtgaaaccccatctcaactaaaaatacaaaaatcagccgggcgtggtggcaggcgcctgtaatcccagctactcagggggctgaaacaggagaatcgcttgaacccgggaggcggaggttgcgccatcgcactccagcctgggagacaagagcgagacttcgtctcaaaaaaaaaaaattcttcttccaagattcaagttgtgtcatttcaccttaataactggaggttagttaagctgggctgtgttctttgcttaatattaagacaacgttttttccagatggaagaaaactatcttaatgaattgttagcttattaattatgtaatgctaatggcttttaaaagctgagatgttctgactgggtgttgtggctcacacctgtaatcccagtaccttgggaggccaagggggaaggattgcttgaggccaggagtttgggaccatagtgagaccccgcctctatttaaaaaattaaattttgttttgttttgttttgagttggagttttgctcttgttgcccatgctgaagtgcaatggtgcaatctcagctcaccacaacctgtgcctcctgggttcaagcgattctcctgcttcagcctcccgagtagatgggattacaggcgtgcaccaccatgcctggctaattttgtatttttagtagagacagggtttctctatgttggtcaggctggtctcaaactctcgacctcaggtgatctgcccgcctccgcttcccaaagttctgggattataggtgtgagccactgggcctggcctaagaaagtttttttaagccattagacgtttttaaaggaattgggagatgacaattggggaaatatttaaaatttaagtaaaatataaagcttccttatttcatgtaacccagacaatctcagtatacatgatcagttgtgtctgacaggtaaatctatttgaggccttatcacacgttacttttaagaactagaaaggaaaagtcactgatcttaagtatttataatacttcatgtggtctaatactttttacgttttgttttgattcagatttagtccggattcccggtatctggcagtaggttctagtgagaactcagtggatttttatgacctaacgctgggccccactcttaacagaatcagctactgcaaagacattccaagctttgtcattcaaatggacttctctgcagatagcagttatctccaggtacagtaccaatactgtatacccaggtggcaagttcttctgcttttacatttcgtgttagtgaatgcatttaaagttcctgagctccagagctccagcttctcaactcctccctttgtaccttctgacctacagctcccctttcctcccccacttatcagagcttttctcctattaagtttttgtagtgatcttttgcatacttaataatgttagacatgtaaatcaagtagcaatatgctagtattctgtaaaccccctgtggattttgtctctcacctaatggaattcttgtcccattttaatctgatgaaaaaggtctctagtggctgctataaacggcatgtctatgaagtgccttcaggaaaacatcttatggatcatgccgctattgacagaattacttgggctacatggactaggtaaatacttatatattcacaaggcaagaactgactttgaaggccagttagaaaatcctatttctgaactgttagagccattccaataaggaatagtaattgagtttcaagtttttgttaccatattttgaaatggtatgttcatgttgggacccctttttattgaatatatttccatgttttatcagtttccatgatttatcaagttttttttttaaggaaatcaaagttttaactttaaagataccctgatatttttcttaatgctaaatttaatgactggcaaaaaggtattgggtgctgttaagcaactgttattaattctctatctaaaggaatgctatcttgaatctattagaagtcaaagcttccaaatttgttcaaatttcctggctgtatgacaggtaaccatgactatccatttttttggccaatgaaaaatgccatcaaattcctgtatcagccaggcatatagtggctcatgcctgtaatctctgatgtagcaggccgaggtgggaggatcacttgagcctagaagttttgataccagcctgggcaacatagcaagaccccatctctgaaatttttttaattcctatgtcataagtcatttttatttttgtagagatagggatctcacaatattgcccaggctggtctcaaactcttggcctcaagcagtcctcctgcctcagcctcccaaaatgttgggattactggtatgtgctgctggacccagccaagtagcacttttaatttgaaaaatagttctatcagttttcagtcaggcgcggtggctcagcctgtaatcccagcactttgggaggccgagcgggggtgatcacctgaggtcgggagttcgagactagcctgaccaacatggagaaaccctgtctctactaaaaatacaaaataagccgggcatgttagcgcatgcctgtgatcccagctactcgggaggctgaggcaggagaattgcttgaacccaggaggcagaggttgcggtgagccgagatcatgccattgcactccagcctgggtaacaagagcgaaaactccgtctcaaaaaaaaaaaaagaaaaaatagttctatcagttttcataaagtactactttaatcttaaaaagattaatctagaaacccttcaaattataaaatgtcatttttaaaaggcaggagttgatatcctgatgaaattcaggtctccaaacaacttaccataatttacttcctgtattttaagtaacatgatagggtacttagagattaattgccaagaaactttttgaatatagtcaacctgcccgcacttgccatgatgagttttcttttgttccttccctctagtattctaggagatgaggttttgggaatctggtccagacatgctgagaaagctgatgtcaactgtgcctgtgtatctcattcaggaatcagtcttgttacaggagatgactttggcatggttaagttatttgacttcccatgtccagaaaaatttgtaagtttgtgttttgtttactattatcagtttactcctaattttgatgtcttatcatcagcacttttccccatatatttaaaatgttttgtcctaatttctaaatttttccccaaactttctaaatctatttactttgaaataaaagctattagaaacaaatcctctccctcgagtaataccatctttggaaccatcctacaaaagctgtaattagcttttcaccaaacctataatcagttatcaaatttcaaatgcttttccttagagaaaaatggtcagagtacctggagacatctgactgcccacacagcctggttttgcagatccactactcatgctgaaaagcattctaatcactggctgcggtgctaactccctactctctccacagctcttgtcatagagattatagttcctaataagagcctttgacttctgtgtgcaccaaatgccctgagcttgtctgtcattgttttttaggcaaaacacaaaaggttcttgggtcattcgccccatgtgacaaatattcgatttaccagtggtgatcgacatgttgttagtgctggaggtgatgactgcaggttagtaactttctcagcccatgaagagcagactatgttactagttaagagacttaatacaacaactcctacagctttggtttatgaaatcagctagtcaacattagtagaaggtagtataaccagatggctcttcagaatctcatatttatgcaaatacagaataaaaggagttaaagaggaaaaatattacacatgtaacctgaaagcacaactgaaaaatattaaactgttatgaaaatctaaaaacataattaactccctgcaattttcttctctgattgcagcttatttgtctggaaatgtgtacatacacctcactgagagatgctgagatgactacagaaattaactttgagaccagaattacagagaagaaaaaccaaaacccaaccctgcatggtcaagtggtgctaacccaagactgtaacagggagaaatgcccagaatcatcaaaatagtgaaagactgatctgttcaaaatatttgctatatgcactgggtataatccgtaatccatacactgccagataatgccatttcaaggaaggatcgaatacttgatggtaaaggccaagtccccctgtattgggaagtgtgtgatttcggcagacctgctgggaaaatttagggtagagcactctttacagaagaactcaaaaacccaatttggataattttcattatctttttagcaaaatggtttcttaatgtttatattttattttcaaggttcattgtttaatgaaatattttattcttgcatttccataaggaaagggaaagtcatgatcatcctaaaggatcacagtttttaaaaggcaaacattttccctaaggaaacagacacaagctttcctagagaatatgatgttttttaggcattaataaggtccttttttataaaggacacttttctcctagtagttttgaattcaggaacagatccaaagttagcagtatatggctgctacatttccattttcattttcgagccatcagtttatgttcagatgccatctctgtaatcgcacatttaaaacataactgtagcctcactaatggaaaagtagtatgatgaacaatcattcccaatggtgtacaatgtaagggttttagggagcaacagtatttaactggaagaaagaattgcatatttaatgtagtctaatatatacacatttgtttaacatgtaaacaaaagtgttaaattcacatatacaacattatacaatttaatcactcttggaataaaatttttatagccttttttctattgggaaaatttgtttagatgtgtgccactccataggtttatttccaaaatgaatgagcccaactccatttgtaaaaacttgtcagttagaattcctttttttagtggattagggctgaattcttagatccttatttcttttcactttaaatgctgccaaagatcactactcatcattcaggaattcgctgtctagcctatctgtagtttcctgaagattgaaaattatgtagactgctatttaaaaatatatttttctaagtgtgaggtttaagatgctgtattgaccctatgagtttttaatgtgttaattatctttatagcataatagatcgctttaggttcctggaatcccatttggtctgacaggatatatgaagattcttaatacctattttctgtgtctaatacttggttaatactaaaaatagaaatgactaaattacatcacagaaagcataaccagtgattgaacctggtagttttaaagctctaaatagctgtggctgaaggactgattatggggctaagaagcttgaaacgtaagttggtacttgttcatcagtggattctcctaaattaagccaaattttgaaatacatgactattaagtttctactcatgtatttacagtcagtcaataaattaaaggaggaaaaaaatccctgaacaacctgcccataaaaagaaaaatactctacatttgagcctgctgcagttttaaattttccctctgggtcaagtttgccagcttttggctacagagaaattatatttccattacagtgcaggtagaaactctgtaaccttaagcatgtaaactacatagaataaaactgtttccactgcatttctgtccttcaaagtggccaacctgattaagtcagccttaatcactgctgctgtcagtttcacgactaaaggtcatattgactaagtagtcatcagctgaccacctcgctgtatcagccagcaacgaggggaaggtgaagaaacatgataggccatatagaatctgccctatgtttacttttttaacccagataattatttttgtgtgcagtatctaagctcctgattgtgtaacctgggacttctggcaccttttgttccattcattttatgtataaaatgcatgccaaagcacactgtgccctctggtacccttgcttccaatcgccaaccatgctcatttccttcctttttttgtggtccctttttgtggtgatcattttaaaccacgtcatccaacaaatgttttatggtcaaccttagcttgttcataagccatagcaactgaaagattaaactcttaaatatgtgtctgggcagtggctattaaatagcaaaaaacaatcagattttagtattttattatttccttgtaaaatggctgaactaaattaaacccttgtttcccatttgttctataatttatagtgaaactgagaacaaaactatctttataaatgatagctaaaagtatttccagatatttaaacaatttaaaataaatttcttctgcagagatgcaaagcatctcaacactggaatgaacaaatgccttaaattcaatggagtaaacctttagaatgaagaggaactgtcatttcacccaagccgaagacaacagccttatgcacttgtgtgctctgtctttgctgcttctcgtgtttcaagcctttcctgtgggatcagcacagcaaagtgcaacttaccaaatggtttaatgactggttaattctttcttctcccaatggaaaagcaatggcaacacaacagtagactgctggcttgacaatcttaaacgtgagcctttgcacatgtaggtttatcatcatttgagtatacgactaagcaagtcaatgaactttttttttttttttagcagtttaatttggtcctgagaatgttgcagtctttattaccccttttgcattaatccacttttctaaccaccttttaagctttaatttttaacactatacaccaagtctttgaaatcagtgatctgttatttaactctaaagcatttgacacttcttgccttaacagttttaaaaaccacacacaaaaaaactctgtaagtaatacagtaggccaaaagtttcatcctatctatcttgcagtttacctatctgatctgatctctgtaattatagttctgtcatttaaaatatactatttaaatctaatttttacatttcaaaaattatcttcagtagtaactaagtatattttctgtggattctgagaatgttatttttcagaatgtgagaatatatatgtacatttataatcttgtgactttaaagtctgttttcagatacagtatgtaaatacttgtaaaaaaatttgtataattttgtgataatgtagtttcccaaaaaaattatttagaaggcattatgttattagtaaatgagagcactgtatagaactgttcctattttctgcacttgccattccagctgcctccactgtccatacccacctcattcatcctgtcacagaaggcaggaaaactgggaactttaccaaagtagcactcagcctgagaggcctgtataatcatgcttttcaaactaaattcacttaaaaattaaaaagcagaattgaatattttaagcagcctcagtacctttggccaatgctgttttcatggtggattatgaacattatataatctttgggaaaagtgaaagtagtacaatttttagaataatgacaactgcctcactgcatctctccactcacacagcaaccgtgtagccccctaagctgcagtaccatgactaaccatgatgtcaatttcatatgctgatcctcacaacagcagtgcacaaacatgccccaaatattttaacagaatttagctcttccttaagctgtcttttcatagtaaaaacaaaacaaaaacacccaatgttaaaaccacataataaacttacaaacttgaaaaattagacacttcagatagataggcaataaaacttcatattatgaaagcaatatattccaagtttcaaagatttgacaagttctgtagagtatctttcatcagtacatgaaaacttccaaactgcatgatcttctgccaggcaggactgggtgctattcgctggtttgaggtcgaatccatttcaaggcatgtcgtggtgggacattaatggtgggatggtagaatgtgcagtccggtcttgtacattgagtgttaaacctacaatgttttggatgatagaagggacattccatcttcttacaagcagggaagtaacggcagagctgactactggaaggtggtgctggtggtgcaactgctggttttggagacagtactggaattcttctactcacatgagtgaagggacaatctggtttagtacactttgcatcatatttacaatttgggtgaacaaacaaacatttttcagcaaatttacaattggggaaggctttgcagggtgagatggggtgatggtaggcacactcatccccatttttacaagcaggccagtacttgcagcgctccaaaagtttttctggtttctgtgccacactcagttcactcatctcagcatttgggtcctcaagctgcctgctcagcaagtgcaactgctgtgggtggaggagacctctgagtcccttgtttgaggctgcagtttggtttacgggtttcattccttcaaagcacatgtcctcctcttgatctgacatgtatcctggggggctggggacaccatccagcgtcactataaacttgggacttgcaggtttatctggttgtacaagatctcgtgtctgcataaggtgtcctgaaagtacccgaagggaatctgcagtcttcatccccgactcttggtttggtgccactactacttcctcagacagctttggcttcttcagaataaatgatcttgtgtctgcatggaccatggattccatgtcatagtaatcttgatttttttctacagaatctccttttgtttcctcttctttaatggggggacttattctgggggtcctactttgtccctggaccacttctgctagcaattcttcttgagaagttcgagttctgggagcaactggaagtgtctgtttctgtggaactgtagagtagttagttgtttttgttacggattcttgagcttcagatatagccttcaaaatcagattcttgttagcttgtttagaaggtggaagagaaggtctcctttcaggctttgcaggcacagacacactgctggagatgcttcctgttcgagacccgtaatcatcatcttcttcctcctcttctccatcatgattgaatttttttactttaacaactgaacttaccacaggcaactttctcttccgaaagttttcatcctccatactcattttctccgagttgtttctaaagaacggactatacgtttcttctaagctgttaagcacctctggttcacacaaacgtcctgtttcatatacccaactactctgcatatcaagctgcttggcagcatgaatactattctgctgctgttgaaattgcaacctgtttaaatgaacaccactatctgcatttctacttgcaggtggtcgataaatttcaatagaagggcgagaagaaccatatgtaagtgtcactgtaggttttttctgagataagggattctcctgcacaaagttgaggtcttcgtcaatgagatcatctggttctggcttaatatcaatcacatcttcagagggtgctggctccctcaaaggtttcactgttgacattagtcgggttgcagctccatcatcgtaagtctgtctgacatttgtggtttttgactcctgcgaacttgtagaaactctggaatctcttttttcaggtctcgcgctaggaatggcaagtggtggcactgcagcttcatgcctcctctcatctccccgactgaaattgctcttgtttgaaggcacgttactatcaaagatgttggtatcagaagacttcagactagagggttcagttgtaacagagcgaagtttatctaatacaccatgaagccatacggtgaatcgaattgtgttgttccctagaaacagggacagatcctctgtcatttggtcctgacttttcttgttggccaccatcaccataatgtaatcaggaagttcttcatcaacataagctcctaattcttgtaatttccccttaatggcactccggatcttgcggctgatctcggtgccgatctccatggctctgcggcgtgcgggaactcagcactgcgcggcgcttggcttacccggaggctgccgcggactcctaccccgcagccgggacaccaccgcctcc

SEQ ID NO: 17446 - RNA, 13761 nt, Homo sapiens
  source 1..13761: mol_type = other RNA
tcaggccaggcacagtggctcatacctggaatcccagcactttgggaggccgaggcaggcagatcacctgaggtcaaggtatttgagaccagcctggccaacatggtgaaaccccatctctactaaaaatacagaaattagctgggtgtggtggtgcacacctgtaatgctagctactcgggaggctgaggtaggagaatcgcttgaacctgggaggcagaggttgcaataagcctagatcatgccactgcactcaagcctgggagacagagcgagactacatcttaaaaaaaaaaaaaaaagtattatgagagaggataatgtattgtaatgtattgtagaggctaaataaaattatgctcatgtcagaaaaaaagagtatttctcaaaataaaattcactgaaactggatgtttattttgactgagatatagtatatcctcaaattgccatagaaagtttacaagaatattagaggtaaattataaatatcagggcctttttaaaaaaaaaagattctgcttataacttggtatttgtttataataaaaattatagtagccaataatgaacacttactctggcttggttatttacttaggtcaaaagaaggaggagcggttaaactgtgggatcaggaactgaggcggtgccgtgccttcaggcttgagacaggacaagccacagattgtgttcgttctgtgtgcagaggcaaagtaagatgttccatgagctgatacagtgcagcagaaaacagaaagtggttattactgtgattccctcaccctttgcagcctaatgaacaatacttaataatgcataacgatggatttgcttgccaacattactctgtctttgctgctttctttgccaaagttagcaccagtgtggtgcataagctaggaagctattctgtctaaatactgtatgtaaacctccaatattttctagaatctgccaatttaacaactctagtagacataattgaaagcccttggcagttgactcatattaggacagctgtctccattttttaaaaaaacacacattccctagataaaacgtgcagtaaacaaacaatgaaatactactcagccataaaaaataatgaaattctgtcattcttggtggcaacatggatgagactggaggacatgatgtgaagtgaaataagccaggcacagaaagataaatacatgttctcactcctgtgcagaaactaaaaaagttgatcccacagaggtggagagtagaatagtggttactggaggcggacaagggggagggggagggggatagggaaggactggttaaaggatacaagtttacacagccagataggaatagtatgttttagtattctgtagtactgtaggatgactatagttaagaatcacgtatttatgtattttcaggtatttacaagagaggattttgaaagtttccatcacaaagaaatgataaatgtctgaggtgatggttatgcgtattaccctatgccctatagatatgtataattatgtgtcaatttcaaaataaaaattcaaaactacaactcctatgaaaatttttgagcgtgtttgtacttattaagtgtatttataaatcatacggatattatcttcagcctgcatattaaattgtagttaagcttttactttttaactaaaaaataaattctattattttttcctatatcccactgcactgaccccagtttggaaatcctaagattatcaaataaaaactttgattattgaagaatccaggtgtactgccacagaaaagttctattctgtagcatggactctaatatgtaatctagcccattgtgcttacagatagatgtgtgcctgtagtcatagaaaaatttgcatgagctaatgactgccttgctactagattagctcaaagcaaaaagttctctgaaagcaggtcaatagggtcatttttatattatgaagaagaaaagcagctgttgtattacattcactgtattggtcctgcttgtgtttcagggcaagatccttgttgggacaaggaatgctgaaataatcgaagttggagagaaaaatgcagcttgtaatattttagttaacggtcatgtggatgggccaatctggggactagcaacacatccttccagggattttttcctttctgctgcagaagatgggacagtgagactttgggatattgctgataaagtaagtacagataatttttttaaaagaggttacaacttctaaaaagaaaagttggaagttctaaattgctagtacttaaagaactgccagaattctgttgagcattttgaggggaaactggtataatttagaagtacttcacttaatgtttcctatgactctttttttttttttttttaaatgcagaagatgttaaacaaagtgaatttgggacatgctgctcgtactgtgtgttacagccctgaaggggacatggtggctattggaatgaaaaatggagaatttatcattttactagtgagttctctaaaaatatggggaaagaagagagacaggagatgtgcaatccatgatatcaggttagtgaacaaatggaatagagtttctagtatatacttgatttaacttccatttgtaaaattttccatagccttgccttcaaaaagaggtccccagggcctgtagcatttcccgtattataaattgtatgctaaaatatggctgtttgtatactacttaattcttcttgctaaattataaacccactgggcaccaactataatagcaagtactagtaggtaatgtttgatgaattcatgttaacacttagccatgtccattaagttcatcccaccaagaggtatctcccactgtaatacaagagagctatctgcccttcaaaagttgtcaccctggaaaactaaagttgtgatttcaaacatatcttctcttagtaacctcagtttgggaatatgtagttcattaatttaatcaatacctattgattaaatgttccagaatccaaattaatttaaatgtttcttaaacctttgtttttcagtgcttaagcatttttcaacagtggctaccatttacggagtacttccgtgtgatcagtagataagattattgaatctaggtctgtcaaaagcttgtacacttttcatcagtaaaatccttttacaaatgaaaccttcctcagaacttcaatatataaaatagtaacagtggcttcccttagcttttacatgtctctatcgtacctcagtaagactcatgggccatttcaagagactgaattgtcccatatgactccaaagattgctaggcaaatagcatttcactttgtcttttaaataagttcttcaggccgggcgcggtggctcatgcctgtaatcccagcactttgggaggccgaggcaggcagatcacctgaagtcaggagtactcgaccagcctggccaacatagtgaaaccccatctcaactaaaaatacaaaaatcagccgggcgtggtggcaggcgcctgtaatcccagctactcagggggctgaaacaggagaatcgcttgaacccgggaggcggaggttgcgccatcgcactccagcctgggagacaagagcgagacttcgtctcaaaaaaaaaaaattcttcttccaagattcaagttgtgtcatttcaccttaataactggaggttagttaagctgggctgtgttctttgcttaatattaagacaacgttttttccagatggaagaaaactatcttaatgaattgttagcttattaattatgtaatgctaatggcttttaaaagctgagatgttctgactgggtgttgtggctcacacctgtaatcccagtaccttgggaggccaagggggaaggattgcttgaggccaggagtttgggaccatagtgagaccccgcctctatttaaaaaattaaattttgttttgttttgttttgagttggagttttgctcttgttgcccatgctgaagtgcaatggtgcaatctcagctcaccacaacctgtgcctcctgggttcaagcgattctcctgcttcagcctcccgagtagatgggattacaggcgtgcaccaccatgcctggctaattttgtatttttagtagagacagggtttctctatgttggtcaggctggtctcaaactctcgacctcaggtgatctgcccgcctccgcttcccaaagttctgggattataggtgtgagccactgggcctggcctaagaaagtttttttaagccattagacgtttttaaaggaattgggagatgacaattggggaaatatttaaaatttaagtaaaatataaagcttccttatttcatgtaacccagacaatctcagtatacatgatcagttgtgtctgacaggtaaatctatttgaggccttatcacacgttacttttaagaactagaaaggaaaagtcactgatcttaagtatttataatacttcatgtggtctaatactttttacgttttgttttgattcagatttagtccggattcccggtatctggcagtaggttctagtgagaactcagtggatttttatgacctaacgctgggccccactcttaacagaatcagctactgcaaagacattccaagctttgtcattcaaatggacttctctgcagatagcagttatctccaggtacagtaccaatactgtatacccaggtggcaagttcttctgcttttacatttcgtgttagtgaatgcatttaaagttcctgagctccagagctccagcttctcaactcctccctttgtaccttctgacctacagctcccctttcctcccccacttatcagagcttttctcctattaagtttttgtagtgatcttttgcatacttaataatgttagacatgtaaatcaagtagcaatatgctagtattctgtaaaccccctgtggattttgtctctcacctaatggaattcttgtcccattttaatctgatgaaaaaggtctctagtggctgctataaacggcatgtctatgaagtgccttcaggaaaacatcttatggatcatgccgctattgacagaattacttgggctacatggactaggtaaatacttatatattcacaaggcaagaactgactttgaaggccagttagaaaatcctatttctgaactgttagagccattccaataaggaatagtaattgagtttcaagtttttgttaccatattttgaaatggtatgttcatgttgggacccctttttattgaatatatttccatgttttatcagtttccatgatttatcaagttttttttttaaggaaatcaaagttttaactttaaagataccctgatatttttcttaatgctaaatttaatgactggcaaaaaggtattgggtgctgttaagcaactgttattaattctctatctaaaggaatgctatcttgaatctattagaagtcaaagcttccaaatttgttcaaatttcctggctgtatgacaggtaaccatgactatccatttttttggccaatgaaaaatgccatcaaattcctgtatcagccaggcatatagtggctcatgcctgtaatctctgatgtagcaggccgaggtgggaggatcacttgagcctagaagttttgataccagcctgggcaacatagcaagaccccatctctgaaatttttttaattcctatgtcataagtcatttttatttttgtagagatagggatctcacaatattgcccaggctggtctcaaactcttggcctcaagcagtcctcctgcctcagcctcccaaaatgttgggattactggtatgtgctgctggacccagccaagtagcacttttaatttgaaaaatagttctatcagttttcagtcaggcgcggtggctcagcctgtaatcccagcactttgggaggccgagcgggggtgatcacctgaggtcgggagttcgagactagcctgaccaacatggagaaaccctgtctctactaaaaatacaaaataagccgggcatgttagcgcatgcctgtgatcccagctactcgggaggctgaggcaggagaattgcttgaacccaggaggcagaggttgcggtgagccgagatcatgccattgcactccagcctgggtaacaagagcgaaaactccgtctcaaaaaaaaaaaaagaaaaaatagttctatcagttttcataaagtactactttaatcttaaaaagattaatctagaaacccttcaaattataaaatgtcatttttaaaaggcaggagttgatatcctgatgaaattcaggtctccaaacaacttaccataatttacttcctgtattttaagtaacatgatagggtacttagagattaattgccaagaaactttttgaatatagtcaacctgcccgcacttgccatgatgagttttcttttgttccttccctctagtattctaggagatgaggttttgggaatctggtccagacatgctgagaaagctgatgtcaactgtgcctgtgtatctcattcaggaatcagtcttgttacaggagatgactttggcatggttaagttatttgacttcccatgtccagaaaaatttgtaagtttgtgttttgtttactattatcagtttactcctaattttgatgtcttatcatcagcacttttccccatatatttaaaatgttttgtcctaatttctaaatttttccccaaactttctaaatctatttactttgaaataaaagctattagaaacaaatcctctccctcgagtaataccatctttggaaccatcctacaaaagctgtaattagcttttcaccaaacctataatcagttatcaaatttcaaatgcttttccttagagaaaaatggtcagagtacctggagacatctgactgcccacacagcctggttttgcagatccactactcatgctgaaaagcattctaatcactggctgcggtgctaactccctactctctccacagctcttgtcatagagattatagttcctaataagagcctttgacttctgtgtgcaccaaatgccctgagcttgtctgtcattgttttttaggcaaaacacaaaaggttcttgggtcattcgccccatgtgacaaatattcgatttaccagtggtgatcgacatgttgttagtgctggaggtgatgactgcaggttagtaactttctcagcccatgaagagcagactatgttactagttaagagacttaatacaacaactcctacagctttggtttatgaaatcagctagtcaacattagtagaaggtagtataaccagatggctcttcagaatctcatatttatgcaaatacagaataaaaggagttaaagaggaaaaatattacacatgtaacctgaaagcacaactgaaaaatattaaactgttatgaaaatctaaaaacataattaactccctgcaattttcttctctgattgcagcttatttgtctggaaatgtgtacatacacctcactgagagatgctgagatgactacagaaattaactttgagaccagaattacagagaagaaaaaccaaaacccaaccctgcatggtcaagtggtgctaacccaagactgtaacagggagaaatgcccagaatcatcaaaatagtgaaagactgatctgttcaaaatatttgctatatgcactgggtataatccgtaatccatacactgccagataatgccatttcaaggaaggatcgaatacttgatggtaaaggccaagtccccctgtattgggaagtgtgtgatttcggcagacctgctgggaaaatttagggtagagcactctttacagaagaactcaaaaacccaatttggataattttcattatctttttagcaaaatggtttcttaatgtttatattttattttcaaggttcattgtttaatgaaatattttattcttgcatttccataaggaaagggaaagtcatgatcatcctaaaggatcacagtttttaaaaggcaaacattttccctaaggaaacagacacaagctttcctagagaatatgatgttttttaggcattaataaggtccttttttataaaggacacttttctcctagtagttttgaattcaggaacagatccaaagttagcagtatatggctgctacatttccattttcattttcgagccatcagtttatgttcagatgccatctctgtaatcgcacatttaaaacataactgtagcctcactaatggaaaagtagtatgatgaacaatcattcccaatggtgtacaatgtaagggttttagggagcaacagtatttaactggaagaaagaattgcatatttaatgtagtctaatatatacacatttgtttaacatgtaaacaaaagtgttaaattcacatatacaacattatacaatttaatcactcttggaataaaatttttatagccttttttctattgggaaaatttgtttagatgtgtgccactccataggtttatttccaaaatgaatgagcccaactccatttgtaaaaacttgtcagttagaattcctttttttagtggattagggctgaattcttagatccttatttcttttcactttaaatgctgccaaagatcactactcatcattcaggaattcgctgtctagcctatctgtagtttcctgaagattgaaaattatgtagactgctatttaaaaatatatttttctaagtgtgaggtttaagatgctgtattgaccctatgagtttttaatgtgttaattatctttatagcataatagatcgctttaggttcctggaatcccatttggtctgacaggatatatgaagattcttaatacctattttctgtgtctaatacttggttaatactaaaaatagaaatgactaaattacatcacagaaagcataaccagtgattgaacctggtagttttaaagctctaaatagctgtggctgaaggactgattatggggctaagaagcttgaaacgtaagttggtacttgttcatcagtggattctcctaaattaagccaaattttgaaatacatgactattaagtttctactcatgtatttacagtcagtcaataaattaaaggaggaaaaaaatccctgaacaacctgcccataaaaagaaaaatactctacatttgagcctgctgcagttttaaattttccctctgggtcaagtttgccagcttttggctacagagaaattatatttccattacagtgcaggtagaaactctgtaaccttaagcatgtaaactacatagaataaaactgtttccactgcatttctgtccttcaaagtggccaacctgattaagtcagccttaatcactgctgctgtcagtttcacgactaaaggtcatattgactaagtagtcatcagctgaccacctcgctgtatcagccagcaacgaggggaaggtgaagaaacatgataggccatatagaatctgccctatgtttacttttttaacccagataattatttttgtgtgcagtatctaagctcctgattgtgtaacctgggacttctggcaccttttgttccattcattttatgtataaaatgcatgccaaagcacactgtgccctctggtacccttgcttccaatcgccaaccatgctcatttccttcctttttttgtggtccctttttgtggtgatcattttaaaccacgtcatccaacaaatgttttatggtcaaccttagcttgttcataagccatagcaactgaaagattaaactcttaaatatgtgtctgggcagtggctattaaatagcaaaaaacaatcagattttagtattttattatttccttgtaaaatggctgaactaaattaaacccttgtttcccatttgttctataatttatagtgaaactgagaacaaaactatctttataaatgatagctaaaagtatttccagatatttaaacaatttaaaataaatttcttctgcagagatgcaaagcatctcaacactggaatgaacaaatgccttaaattcaatggagtaaacctttagaatgaagaggaactgtcatttcacccaagccgaagacaacagccttatgcacttgtgtgctctgtctttgctgcttctcgtgtttcaagcctttcctgtgggatcagcacagcaaagtgcaacttaccaaatggtttaatgactggttaattctttcttctcccaatggaaaagcaatggcaacacaacagtagactgctggcttgacaatcttaaacgtgagcctttgcacatgtaggtttatcatcatttgagtatacgactaagcaagtcaatgaactttttttttttttttagcagtttaatttggtcctgagaatgttgcagtctttattaccccttttgcattaatccacttttctaaccaccttttaagctttaatttttaacactatacaccaagtctttgaaatcagtgatctgttatttaactctaaagcatttgacacttcttgccttaacagttttaaaaaccacacacaaaaaaactctgtaagtaatacagtaggccaaaagtttcatcctatctatcttgcagtttacctatctgatctgatctctgtaattatagttctgtcatttaaaatatactatttaaatctaatttttacatttcaaaaattatcttcagtagtaactaagtatattttctgtggattctgagaatgttatttttcagaatgtgagaatatatatgtacatttataatcttgtgactttaaagtctgttttcagatacagtatgtaaatacttgtaaaaaaatttgtataattttgtgataatgtagtttcccaaaaaaattatttagaaggcattatgttattagtaaatgagagcactgtatagaactgttcctattttctgcacttgccattccagctgcctccactgtccatacccacctcattcatcctgtcacagaaggcaggaaaactgggaactttaccaaagtagcactcagcctgagaggcctgtataatcatgcttttcaaactaaattcacttaaaaattaaaaagcagaattgaatattttaagcagcctcagtacctttggccaatgctgttttcatggtggattatgaacattatataatctttgggaaaagtgaaagtagtacaatttttagaataatgacaactgcctcactgcatctctccactcacacagcaaccgtgtagccccctaagctgcagtaccatgactaaccatgatgtcaatttcatatgctgatcctcacaacagcagtgcacaaacatgccccaaatattttaacagaatttagctcttccttaagctgtcttttcatagtaaaaacaaaacaaaaacacccaatgttaaaaccacataataaacttacaaacttgaaaaattagacacttcagatagataggcaataaaacttcatattatgaaagcaatatattccaagtttcaaagatttgacaagttctgtagagtatctttcatcagtacatgaaaacttccaaactgcatgatcttctgccaggcaggactgggtgctattcgctggtttgaggtcgaatccatttcaaggcatgtcgtggtgggacattaatggtgggatggtagaatgtgcagtccggtcttgtacattgagtgttaaacctacaatgttttggatgatagaagggacattccatcttcttacaagcagggaagtaacggcagagctgactactggaaggtggtgctggtggtgcaactgctggttttggagacagtactggaattcttctactcacatgagtgaagggacaatctggtttagtacactttgcatcatatttacaatttgggtgaacaaacaaacatttttcagcaaatttacaattggggaaggctttgcagggtgagatggggtgatggtaggcacactcatccccatttttacaagcaggccagtacttgcagcgctccaaaagtttttctggtttctgtgccacactcagttcactcatctcagcgttagaaaagctaccatttgggtcctcaagctgcctgctcagcaagtgcaactgctgtgggtggaggagacctctgagtcccttgtttgaggctgcagtttggtttacgggtttcattccttcaaagcacatgtcctcctcttgatctgacatgtatcctggggggctggggacaccatccagcgtcactataaacttgggacttgcaggtttatctggttgtacaagatctcgtgtctgcataaggtgtcctgaaagtacccgaagggaatctgcagtcttcatccccgactcttggtttggtgccactactacttcctcagacagctttggcttcttcagaataaatgatcttgtgtctgcatggaccatggattccatgtcatagtaatcttgactcatctgcagagtttctgccattactgggtcgatttgcagtcgggataataattgcctctgttgagttccttgatttttttctacagaatctccttttgtttcctcttctttaatggggggacttattctgggggtcctactttgtccctggaccacttctgctagcaattcttcttgagaagttcgagttctgggagcaactggaagtgtctgtttctgtggaactgtagagtagttagttgtttttgttacggattcttgagcttcagatatagccttcaaaatcagattcttgttagcttgtttagaaggtggaagagaaggtctcctttcaggctttgcaggcacagacacactgctggagatgcttcctgttcgagacccgtaatcatcatcttcttcctcctcttctccatcatgattgaatttttttactttaacaactgaacttaccacaggcaactttctcttccgaaagttttcatcctccatactcattttctccgagttgtttctaaagaacggactatacgtttcttctaagctgttaagcacctctggttcacacaaacgtcctgtttcatatacccaactactctgcatatcaagctgcttggcagcatgaatactattctgctgctgttgaaattgcaacctgtttaaatgaacaccactatctgcatttctacttgcaggtggtcgataaatttcaatagaagggcgagaagaaccatatgtaagtgtcactgtaggttttttctgagataagggattctcctgcacaaagttgaggtcttcgtcaatgagatcatctggttctggcttaatatcaatcacatcttcagagggtgctggctccctcaaaggtttcactgttgacattagtcgggttgcagctccatcatcgtaagtctgtctgacatttgtggtttttgactcctgcgaacttgtagaaactctggaatctcttttttcaggtctcgcgctaggaatggcaagtggtggcactgcagcttcatgcctcctctcatctccccgactgaaattgctcttgtttgaaggcacgttactatcaaagatgttggtatcagaagacttcagactagagggttcagttgtaacagagcgaagtttatctaatacaccatgaagccaacataagctcctaattcttgtaatttccccttaatggcactccggatcttgcggctgatctcggtgccgatctccatggctctgcggcgtgcgggaactcagcactgcgcggcgcttggcttacccggaggctgccgcggactcctaccccgcagccgggacaccaccgcctcc

SEQ ID NO: 17447 - RNA, 13876 nt, Homo sapiens
  source 1..13876: mol_type = other RNA
tcaggccaggcacagtggctcatacctggaatcccagcactttgggaggccgaggcaggcagatcacctgaggtcaaggtatttgagaccagcctggccaacatggtgaaaccccatctctactaaaaatacagaaattagctgggtgtggtggtgcacacctgtaatgctagctactcgggaggctgaggtaggagaatcgcttgaacctgggaggcagaggttgcaataagcctagatcatgccactgcactcaagcctgggagacagagcgagactacatcttaaaaaaaaaaaaaaaagtattatgagagaggataatgtattgtaatgtattgtagaggctaaataaaattatgctcatgtcagaaaaaaagagtatttctcaaaataaaattcactgaaactggatgtttattttgactgagatatagtatatcctcaaattgccatagaaagtttacaagaatattagaggtaaattataaatatcagggcctttttaaaaaaaaaagattctgcttataacttggtatttgtttataataaaaattatagtagccaataatgaacacttactctggcttggttatttacttaggtcaaaagaaggaggagcggttaaactgtgggatcaggaactgaggcggtgccgtgccttcaggcttgagacaggacaagccacagattgtgttcgttctgtgtgcagaggcaaagtaagatgttccatgagctgatacagtgcagcagaaaacagaaagtggttattactgtgattccctcaccctttgcagcctaatgaacaatacttaataatgcataacgatggatttgcttgccaacattactctgtctttgctgctttctttgccaaagttagcaccagtgtggtgcataagctaggaagctattctgtctaaatactgtatgtaaacctccaatattttctagaatctgccaatttaacaactctagtagacataattgaaagcccttggcagttgactcatattaggacagctgtctccattttttaaaaaaacacacattccctagataaaacgtgcagtaaacaaacaatgaaatactactcagccataaaaaataatgaaattctgtcattcttggtggcaacatggatgagactggaggacatgatgtgaagtgaaataagccaggcacagaaagataaatacatgttctcactcctgtgcagaaactaaaaaagttgatcccacagaggtggagagtagaatagtggttactggaggcggacaagggggagggggagggggatagggaaggactggttaaaggatacaagtttacacagccagataggaatagtatgttttagtattctgtagtactgtaggatgactatagttaagaatcacgtatttatgtattttcaggtatttacaagagaggattttgaaagtttccatcacaaagaaatgataaatgtctgaggtgatggttatgcgtattaccctatgccctatagatatgtataattatgtgtcaatttcaaaataaaaattcaaaactacaactcctatgaaaatttttgagcgtgtttgtacttattaagtgtatttataaatcatacggatattatcttcagcctgcatattaaattgtagttaagcttttactttttaactaaaaaataaattctattattttttcctatatcccactgcactgaccccagtttggaaatcctaagattatcaaataaaaactttgattattgaagaatccaggtgtactgccacagaaaagttctattctgtagcatggactctaatatgtaatctagcccattgtgcttacagatagatgtgtgcctgtagtcatagaaaaatttgcatgagctaatgactgccttgctactagattagctcaaagcaaaaagttctctgaaagcaggtcaatagggtcatttttatattatgaagaagaaaagcagctgttgtattacattcactgtattggtcctgcttgtgtttcagggcaagatccttgttgggacaaggaatgctgaaataatcgaagttggagagaaaaatgcagcttgtaatattttagttaacggtcatgtggatgggccaatctggggactagcaacacatccttccagggattttttcctttctgctgcagaagatgggacagtgagactttgggatattgctgataaagtaagtacagataatttttttaaaagaggttacaacttctaaaaagaaaagttggaagttctaaattgctagtacttaaagaactgccagaattctgttgagcattttgaggggaaactggtataatttagaagtacttcacttaatgtttcctatgactctttttttttttttttttaaatgcagaagatgttaaacaaagtgaatttgggacatgctgctcgtactgtgtgttacagccctgaaggggacatggtggctattggaatgaaaaatggagaatttatcattttactagtgagttctctaaaaatatggggaaagaagagagacaggagatgtgcaatccatgatatcaggttagtgaacaaatggaatagagtttctagtatatacttgatttaacttccatttgtaaaattttccatagccttgccttcaaaaagaggtccccagggcctgtagcatttcccgtattataaattgtatgctaaaatatggctgtttgtatactacttaattcttcttgctaaattataaacccactgggcaccaactataatagcaagtactagtaggtaatgtttgatgaattcatgttaacacttagccatgtccattaagttcatcccaccaagaggtatctcccactgtaatacaagagagctatctgcccttcaaaagttgtcaccctggaaaactaaagttgtgatttcaaacatatcttctcttagtaacctcagtttgggaatatgtagttcattaatttaatcaatacctattgattaaatgttccagaatccaaattaatttaaatgtttcttaaacctttgtttttcagtgcttaagcatttttcaacagtggctaccatttacggagtacttccgtgtgatcagtagataagattattgaatctaggtctgtcaaaagcttgtacacttttcatcagtaaaatccttttacaaatgaaaccttcctcagaacttcaatatataaaatagtaacagtggcttcccttagcttttacatgtctctatcgtacctcagtaagactcatgggccatttcaagagactgaattgtcccatatgactccaaagattgctaggcaaatagcatttcactttgtcttttaaataagttcttcaggccgggcgcggtggctcatgcctgtaatcccagcactttgggaggccgaggcaggcagatcacctgaagtcaggagtactcgaccagcctggccaacatagtgaaaccccatctcaactaaaaatacaaaaatcagccgggcgtggtggcaggcgcctgtaatcccagctactcagggggctgaaacaggagaatcgcttgaacccgggaggcggaggttgcgccatcgcactccagcctgggagacaagagcgagacttcgtctcaaaaaaaaaaaattcttcttccaagattcaagttgtgtcatttcaccttaataactggaggttagttaagctgggctgtgttctttgcttaatattaagacaacgttttttccagatggaagaaaactatcttaatgaattgttagcttattaattatgtaatgctaatggcttttaaaagctgagatgttctgactgggtgttgtggctcacacctgtaatcccagtaccttgggaggccaagggggaaggattgcttgaggccaggagtttgggaccatagtgagaccccgcctctatttaaaaaattaaattttgttttgttttgttttgagttggagttttgctcttgttgcccatgctgaagtgcaatggtgcaatctcagctcaccacaacctgtgcctcctgggttcaagcgattctcctgcttcagcctcccgagtagatgggattacaggcgtgcaccaccatgcctggctaattttgtatttttagtagagacagggtttctctatgttggtcaggctggtctcaaactctcgacctcaggtgatctgcccgcctccgcttcccaaagttctgggattataggtgtgagccactgggcctggcctaagaaagtttttttaagccattagacgtttttaaaggaattgggagatgacaattggggaaatatttaaaatttaagtaaaatataaagcttccttatttcatgtaacccagacaatctcagtatacatgatcagttgtgtctgacaggtaaatctatttgaggccttatcacacgttacttttaagaactagaaaggaaaagtcactgatcttaagtatttataatacttcatgtggtctaatactttttacgttttgttttgattcagatttagtccggattcccggtatctggcagtaggttctagtgagaactcagtggatttttatgacctaacgctgggccccactcttaacagaatcagctactgcaaagacattccaagctttgtcattcaaatggacttctctgcagatagcagttatctccaggtacagtaccaatactgtatacccaggtggcaagttcttctgcttttacatttcgtgttagtgaatgcatttaaagttcctgagctccagagctccagcttctcaactcctccctttgtaccttctgacctacagctcccctttcctcccccacttatcagagcttttctcctattaagtttttgtagtgatcttttgcatacttaataatgttagacatgtaaatcaagtagcaatatgctagtattctgtaaaccccctgtggattttgtctctcacctaatggaattcttgtcccattttaatctgatgaaaaaggtctctagtggctgctataaacggcatgtctatgaagtgccttcaggaaaacatcttatggatcatgccgctattgacagaattacttgggctacatggactaggtaaatacttatatattcacaaggcaagaactgactttgaaggccagttagaaaatcctatttctgaactgttagagccattccaataaggaatagtaattgagtttcaagtttttgttaccatattttgaaatggtatgttcatgttgggacccctttttattgaatatatttccatgttttatcagtttccatgatttatcaagttttttttttaaggaaatcaaagttttaactttaaagataccctgatatttttcttaatgctaaatttaatgactggcaaaaaggtattgggtgctgttaagcaactgttattaattctctatctaaaggaatgctatcttgaatctattagaagtcaaagcttccaaatttgttcaaatttcctggctgtatgacaggtaaccatgactatccatttttttggccaatgaaaaatgccatcaaattcctgtatcagccaggcatatagtggctcatgcctgtaatctctgatgtagcaggccgaggtgggaggatcacttgagcctagaagttttgataccagcctgggcaacatagcaagaccccatctctgaaatttttttaattcctatgtcataagtcatttttatttttgtagagatagggatctcacaatattgcccaggctggtctcaaactcttggcctcaagcagtcctcctgcctcagcctcccaaaatgttgggattactggtatgtgctgctggacccagccaagtagcacttttaatttgaaaaatagttctatcagttttcagtcaggcgcggtggctcagcctgtaatcccagcactttgggaggccgagcgggggtgatcacctgaggtcgggagttcgagactagcctgaccaacatggagaaaccctgtctctactaaaaatacaaaataagccgggcatgttagcgcatgcctgtgatcccagctactcgggaggctgaggcaggagaattgcttgaacccaggaggcagaggttgcggtgagccgagatcatgccattgcactccagcctgggtaacaagagcgaaaactccgtctcaaaaaaaaaaaaagaaaaaatagttctatcagttttcataaagtactactttaatcttaaaaagattaatctagaaacccttcaaattataaaatgtcatttttaaaaggcaggagttgatatcctgatgaaattcaggtctccaaacaacttaccataatttacttcctgtattttaagtaacatgatagggtacttagagattaattgccaagaaactttttgaatatagtcaacctgcccgcacttgccatgatgagttttcttttgttccttccctctagtattctaggagatgaggttttgggaatctggtccagacatgctgagaaagctgatgtcaactgtgcctgtgtatctcattcaggaatcagtcttgttacaggagatgactttggcatggttaagttatttgacttcccatgtccagaaaaatttgtaagtttgtgttttgtttactattatcagtttactcctaattttgatgtcttatcatcagcacttttccccatatatttaaaatgttttgtcctaatttctaaatttttccccaaactttctaaatctatttactttgaaataaaagctattagaaacaaatcctctccctcgagtaataccatctttggaaccatcctacaaaagctgtaattagcttttcaccaaacctataatcagttatcaaatttcaaatgcttttccttagagaaaaatggtcagagtacctggagacatctgactgcccacacagcctggttttgcagatccactactcatgctgaaaagcattctaatcactggctgcggtgctaactccctactctctccacagctcttgtcatagagattatagttcctaataagagcctttgacttctgtgtgcaccaaatgccctgagcttgtctgtcattgttttttaggcaaaacacaaaaggttcttgggtcattcgccccatgtgacaaatattcgatttaccagtggtgatcgacatgttgttagtgctggaggtgatgactgcaggttagtaactttctcagcccatgaagagcagactatgttactagttaagagacttaatacaacaactcctacagctttggtttatgaaatcagctagtcaacattagtagaaggtagtataaccagatggctcttcagaatctcatatttatgcaaatacagaataaaaggagttaaagaggaaaaatattacacatgtaacctgaaagcacaactgaaaaatattaaactgttatgaaaatctaaaaacataattaactccctgcaattttcttctctgattgcagcttatttgtctggaaatgtgtacatacacctcactgagagatgctgagatgactacagaaattaactttgagaccagaattacagagaagaaaaaccaaaacccaaccctgcatggtcaagtggtgctaacccaagactgtaacagggagaaatgcccagaatcatcaaaatagtgaaagactgatctgttcaaaatatttgctatatgcactgggtataatccgtaatccatacactgccagataatgccatttcaaggaaggatcgaatacttgatggtaaaggccaagtccccctgtattgggaagtgtgtgatttcggcagacctgctgggaaaatttagggtagagcactctttacagaagaactcaaaaacccaatttggataattttcattatctttttagcaaaatggtttcttaatgtttatattttattttcaaggttcattgtttaatgaaatattttattcttgcatttccataaggaaagggaaagtcatgatcatcctaaaggatcacagtttttaaaaggcaaacattttccctaaggaaacagacacaagctttcctagagaatatgatgttttttaggcattaataaggtccttttttataaaggacacttttctcctagtagttttgaattcaggaacagatccaaagttagcagtatatggctgctacatttccattttcattttcgagccatcagtttatgttcagatgccatctctgtaatcgcacatttaaaacataactgtagcctcactaatggaaaagtagtatgatgaacaatcattcccaatggtgtacaatgtaagggttttagggagcaacagtatttaactggaagaaagaattgcatatttaatgtagtctaatatatacacatttgtttaacatgtaaacaaaagtgttaaattcacatatacaacattatacaatttaatcactcttggaataaaatttttatagccttttttctattgggaaaatttgtttagatgtgtgccactccataggtttatttccaaaatgaatgagcccaactccatttgtaaaaacttgtcagttagaattcctttttttagtggattagggctgaattcttagatccttatttcttttcactttaaatgctgccaaagatcactactcatcattcaggaattcgctgtctagcctatctgtagtttcctgaagattgaaaattatgtagactgctatttaaaaatatatttttctaagtgtgaggtttaagatgctgtattgaccctatgagtttttaatgtgttaattatctttatagcataatagatcgctttaggttcctggaatcccatttggtctgacaggatatatgaagattcttaatacctattttctgtgtctaatacttggttaatactaaaaatagaaatgactaaattacatcacagaaagcataaccagtgattgaacctggtagttttaaagctctaaatagctgtggctgaaggactgattatggggctaagaagcttgaaacgtaagttggtacttgttcatcagtggattctcctaaattaagccaaattttgaaatacatgactattaagtttctactcatgtatttacagtcagtcaataaattaaaggaggaaaaaaatccctgaacaacctgcccataaaaagaaaaatactctacatttgagcctgctgcagttttaaattttccctctgggtcaagtttgccagcttttggctacagagaaattatatttccattacagtgcaggtagaaactctgtaaccttaagcatgtaaactacatagaataaaactgtttccactgcatttctgtccttcaaagtggccaacctgattaagtcagccttaatcactgctgctgtcagtttcacgactaaaggtcatattgactaagtagtcatcagctgaccacctcgctgtatcagccagcaacgaggggaaggtgaagaaacatgataggccatatagaatctgccctatgtttacttttttaacccagataattatttttgtgtgcagtatctaagctcctgattgtgtaacctgggacttctggcaccttttgttccattcattttatgtataaaatgcatgccaaagcacactgtgccctctggtacccttgcttccaatcgccaaccatgctcatttccttcctttttttgtggtccctttttgtggtgatcattttaaaccacgtcatccaacaaatgttttatggtcaaccttagcttgttcataagccatagcaactgaaagattaaactcttaaatatgtgtctgggcagtggctattaaatagcaaaaaacaatcagattttagtattttattatttccttgtaaaatggctgaactaaattaaacccttgtttcccatttgttctataatttatagtgaaactgagaacaaaactatctttataaatgatagctaaaagtatttccagatatttaaacaatttaaaataaatttcttctgcagagatgcaaagcatctcaacactggaatgaacaaatgccttaaattcaatggagtaaacctttagaatgaagaggaactgtcatttcacccaagccgaagacaacagccttatgcacttgtgtgctctgtctttgctgcttctcgtgtttcaagcctttcctgtgggatcagcacagcaaagtgcaacttaccaaatggtttaatgactggttaattctttcttctcccaatggaaaagcaatggcaacacaacagtagactgctggcttgacaatcttaaacgtgagcctttgcacatgtaggtttatcatcatttgagtatacgactaagcaagtcaatgaactttttttttttttttagcagtttaatttggtcctgagaatgttgcagtctttattaccccttttgcattaatccacttttctaaccaccttttaagctttaatttttaacactatacaccaagtctttgaaatcagtgatctgttatttaactctaaagcatttgacacttcttgccttaacagttttaaaaaccacacacaaaaaaactctgtaagtaatacagtaggccaaaagtttcatcctatctatcttgcagtttacctatctgatctgatctctgtaattatagttctgtcatttaaaatatactatttaaatctaatttttacatttcaaaaattatcttcagtagtaactaagtatattttctgtggattctgagaatgttatttttcagaatgtgagaatatatatgtacatttataatcttgtgactttaaagtctgttttcagatacagtatgtaaatacttgtaaaaaaatttgtataattttgtgataatgtagtttcccaaaaaaattatttagaaggcattatgttattagtaaatgagagcactgtatagaactgttcctattttctgcacttgccattccagctgcctccactgtccatacccacctcattcatcctgtcacagaaggcaggaaaactgggaactttaccaaagtagcactcagcctgagaggcctgtataatcatgcttttcaaactaaattcacttaaaaattaaaaagcagaattgaatattttaagcagcctcagtacctttggccaatgctgttttcatggtggattatgaacattatataatctttgggaaaagtgaaagtagtacaatttttagaataatgacaactgcctcactgcatctctccactcacacagcaaccgtgtagccccctaagctgcagtaccatgactaaccatgatgtcaatttcatatgctgatcctcacaacagcagtgcacaaacatgccccaaatattttaacagaatttagctcttccttaagctgtcttttcatagtaaaaacaaaacaaaaacacccaatgttaaaaccacataataaacttacaaacttgaaaaattagacacttcagatagataggcaataaaacttcatattatgaaagcaatatattccaagtttcaaagatttgacaagttctgtagagtatctttcatcagtacatgaaaacttccaaactgcatgatcttctgccaggcaggactgggtgctattcgctggtttgaggtcgaatccatttcaaggcatgtcgtggtgggacattaatggtgggatggtagaatgtgcagtccggtcttgtacattgagtgttaaacctacaatgttttggatgatagaagggacattccatcttcttacaagcagggaagtaacggcagagctgactactggaaggtggtgctggtggtgcaactgctggttttggagacagtactggaattcttctactcacatgagtgaagggacaatctggtttagtacactttgcatcatatttacaatttgggtgaacaaacaaacatttttcagcaaatttacaattggggaaggctttgcagggtgagatggggtgatggtaggcacactcatccccatttttacaagcaggccagtacttgcagcgctccaaaagtttttctggtttctgtgccacactcagttcactcatctcagcgttagaaaagctaccatttgggtcctcaagctgcctgctcagcaagtgcaactgctgtgggtggaggagacctctgagtcccttgtttgaggctgcagtttggtttacgggtttcattccttcaaagcacatgtcctcctcttgatctgacatgtatcctggggggctggggacaccatccagcgtcactataaacttgggacttgcaggtttatctggttgtacaagatctcgtgtctgcataaggtgtcctgaaagtacccgaagggaatctgcagtcttcatccccgactcttggtttggtgccactactacttcctcagacagctttggcttcttcagaataaatgatcttgtgtctgcatggaccatggattccatgtcatagtaatcttgactcatctgcagagtttctgccattactgggtcgatttgcagtcgggataataattgcctctgttgagttccttgatttttttctacagaatctccttttgtttcctcttctttaatggggggacttattctgggggtcctactttgtccctggaccacttctgctagcaattcttcttgagaagttcgagttctgggagcaactggaagtgtctgtttctgtggaactgtagagtagttagttgtttttgttacggattcttgagcttcagatatagccttcaaaatcagattcttgttagcttgtttagaaggtggaagagaaggtctcctttcaggctttgcaggcacagacacactgctggagatgcttcctgttcgagacccgtaatcatcatcttcttcctcctcttctccatcatgattgaatttttttactttaacaactgaacttaccacaggcaactttctcttccgaaagttttcatcctccatactcattttctccgagttgtttctaaagaacggactatacgtttcttctaagctgttaagcacctctggttcacacaaacgtcctgtttcatatacccaactactctgcatatcaagctgcttggcagcatgaatactattctgctgctgttgaaattgcaacctgtttaaatgaacaccactatctgcatttctacttgcaggtggtcgataaatttcaatagaagggcgagaagaaccatatgtaagtgtcactgtaggttttttctgagataagggattctcctgcacaaagttgaggtcttcgtcaatgagatcatctggttctggcttaatatcaatcacatcttcagagggtgctggctccctcaaaggtttcactgttgacattagtcgggttgcagctccatcatcgtaagtctgtctgacatttgtggtttttgactcctgcgaacttgtagaaactctggaatctcttttttcaggtctcgcgctaggaatggcaagtggtggcactgcagcttcatgcctcctctcatctccccgactgaaattgctcttgtttgaaggcacgttactatcaaagatgttggtatcagaagacttcagactagagggttcagttgtaacagagcgaagtttatctaatacaccatgaagccatacggtgaatcgaattgtgttgttccctagaaacagggacagatcctctgtcatttggtcctgacttttcttgttggccaccatcaccataatgtaatcaggaagttcttcatcaacataagctcctaattcttgtaatttccccttaatggcactccggatcttgcggctgatctcggtgccgatctccatggctctgcggcgtgcgggaactcagcactgcgcggcgcttggcttacccggaggctgccgcggactcctaccccgcagccgggacaccaccgcctcc

SEQ ID NO: 17448 - RNA, 14057 nt, Homo sapiens
  source 1..14057: mol_type = other RNA
tcaggccaggcacagtggctcatacctggaatcccagcactttgggaggccgaggcaggcagatcacctgaggtcaaggtatttgagaccagcctggccaacatggtgaaaccccatctctactaaaaatacagaaattagctgggtgtggtggtgcacacctgtaatgctagctactcgggaggctgaggtaggagaatcgcttgaacctgggaggcagaggttgcaataagcctagatcatgccactgcactcaagcctgggagacagagcgagactacatcttaaaaaaaaaaaaaaaagtattatgagagaggataatgtattgtaatgtattgtagaggctaaataaaattatgctcatgtcagaaaaaaagagtatttctcaaaataaaattcactgaaactggatgtttattttgactgagatatagtatatcctcaaattgccatagaaagtttacaagaatattagaggtaaattataaatatcagggcctttttaaaaaaaaaagattctgcttataacttggtatttgtttataataaaaattatagtagccaataatgaacacttactctggcttggttatttacttaggtcaaaagaaggaggagcggttaaactgtgggatcaggaactgaggcggtgccgtgccttcaggcttgagacaggacaagccacagattgtgttcgttctgtgtgcagaggcaaagtaagatgttccatgagctgatacagtgcagcagaaaacagaaagtggttattactgtgattccctcaccctttgcagcctaatgaacaatacttaataatgcataacgatggatttgcttgccaacattactctgtctttgctgctttctttgccaaagttagcaccagtgtggtgcataagctaggaagctattctgtctaaatactgtatgtaaacctccaatattttctagaatctgccaatttaacaactctagtagacataattgaaagcccttggcagttgactcatattaggacagctgtctccattttttaaaaaaacacacattccctagataaaacgtgcagtaaacaaacaatgaaatactactcagccataaaaaataatgaaattctgtcattcttggtggcaacatggatgagactggaggacatgatgtgaagtgaaataagccaggcacagaaagataaatacatgttctcactcctgtgcagaaactaaaaaagttgatcccacagaggtggagagtagaatagtggttactggaggcggacaagggggagggggagggggatagggaaggactggttaaaggatacaagtttacacagccagataggaatagtatgttttagtattctgtagtactgtaggatgactatagttaagaatcacgtatttatgtattttcaggtatttacaagagaggattttgaaagtttccatcacaaagaaatgataaatgtctgaggtgatggttatgcgtattaccctatgccctatagatatgtataattatgtgtcaatttcaaaataaaaattcaaaactacaactcctatgaaaatttttgagcgtgtttgtacttattaagtgtatttataaatcatacggatattatcttcagcctgcatattaaattgtagttaagcttttactttttaactaaaaaataaattctattattttttcctatatcccactgcactgaccccagtttggaaatcctaagattatcaaataaaaactttgattattgaagaatccaggtgtactgccacagaaaagttctattctgtagcatggactctaatatgtaatctagcccattgtgcttacagatagatgtgtgcctgtagtcatagaaaaatttgcatgagctaatgactgccttgctactagattagctcaaagcaaaaagttctctgaaagcaggtcaatagggtcatttttatattatgaagaagaaaagcagctgttgtattacattcactgtattggtcctgcttgtgtttcagggcaagatccttgttgggacaaggaatgctgaaataatcgaagttggagagaaaaatgcagcttgtaatattttagttaacggtcatgtggatgggccaatctggggactagcaacacatccttccagggattttttcctttctgctgcagaagatgggacagtgagactttgggatattgctgataaagtaagtacagataatttttttaaaagaggttacaacttctaaaaagaaaagttggaagttctaaattgctagtacttaaagaactgccagaattctgttgagcattttgaggggaaactggtataatttagaagtacttcacttaatgtttcctatgactctttttttttttttttttaaatgcagaagatgttaaacaaagtgaatttgggacatgctgctcgtactgtgtgttacagccctgaaggggacatggtggctattggaatgaaaaatggagaatttatcattttactagtgagttctctaaaaatatggggaaagaagagagacaggagatgtgcaatccatgatatcaggttagtgaacaaatggaatagagtttctagtatatacttgatttaacttccatttgtaaaattttccatagccttgccttcaaaaagaggtccccagggcctgtagcatttcccgtattataaattgtatgctaaaatatggctgtttgtatactacttaattcttcttgctaaattataaacccactgggcaccaactataatagcaagtactagtaggtaatgtttgatgaattcatgttaacacttagccatgtccattaagttcatcccaccaagaggtatctcccactgtaatacaagagagctatctgcccttcaaaagttgtcaccctggaaaactaaagttgtgatttcaaacatatcttctcttagtaacctcagtttgggaatatgtagttcattaatttaatcaatacctattgattaaatgttccagaatccaaattaatttaaatgtttcttaaacctttgtttttcagtgcttaagcatttttcaacagtggctaccatttacggagtacttccgtgtgatcagtagataagattattgaatctaggtctgtcaaaagcttgtacacttttcatcagtaaaatccttttacaaatgaaaccttcctcagaacttcaatatataaaatagtaacagtggcttcccttagcttttacatgtctctatcgtacctcagtaagactcatgggccatttcaagagactgaattgtcccatatgactccaaagattgctaggcaaatagcatttcactttgtcttttaaataagttcttcaggccgggcgcggtggctcatgcctgtaatcccagcactttgggaggccgaggcaggcagatcacctgaagtcaggagtactcgaccagcctggccaacatagtgaaaccccatctcaactaaaaatacaaaaatcagccgggcgtggtggcaggcgcctgtaatcccagctactcagggggctgaaacaggagaatcgcttgaacccgggaggcggaggttgcgccatcgcactccagcctgggagacaagagcgagacttcgtctcaaaaaaaaaaaattcttcttccaagattcaagttgtgtcatttcaccttaataactggaggttagttaagctgggctgtgttctttgcttaatattaagacaacgttttttccagatggaagaaaactatcttaatgaattgttagcttattaattatgtaatgctaatggcttttaaaagctgagatgttctgactgggtgttgtggctcacacctgtaatcccagtaccttgggaggccaagggggaaggattgcttgaggccaggagtttgggaccatagtgagaccccgcctctatttaaaaaattaaattttgttttgttttgttttgagttggagttttgctcttgttgcccatgctgaagtgcaatggtgcaatctcagctcaccacaacctgtgcctcctgggttcaagcgattctcctgcttcagcctcccgagtagatgggattacaggcgtgcaccaccatgcctggctaattttgtatttttagtagagacagggtttctctatgttggtcaggctggtctcaaactctcgacctcaggtgatctgcccgcctccgcttcccaaagttctgggattataggtgtgagccactgggcctggcctaagaaagtttttttaagccattagacgtttttaaaggaattgggagatgacaattggggaaatatttaaaatttaagtaaaatataaagcttccttatttcatgtaacccagacaatctcagtatacatgatcagttgtgtctgacaggtaaatctatttgaggccttatcacacgttacttttaagaactagaaaggaaaagtcactgatcttaagtatttataatacttcatgtggtctaatactttttacgttttgttttgattcagatttagtccggattcccggtatctggcagtaggttctagtgagaactcagtggatttttatgacctaacgctgggccccactcttaacagaatcagctactgcaaagacattccaagctttgtcattcaaatggacttctctgcagatagcagttatctccaggtacagtaccaatactgtatacccaggtggcaagttcttctgcttttacatttcgtgttagtgaatgcatttaaagttcctgagctccagagctccagcttctcaactcctccctttgtaccttctgacctacagctcccctttcctcccccacttatcagagcttttctcctattaagtttttgtagtgatcttttgcatacttaataatgttagacatgtaaatcaagtagcaatatgctagtattctgtaaaccccctgtggattttgtctctcacctaatggaattcttgtcccattttaatctgatgaaaaaggtctctagtggctgctataaacggcatgtctatgaagtgccttcaggaaaacatcttatggatcatgccgctattgacagaattacttgggctacatggactaggtaaatacttatatattcacaaggcaagaactgactttgaaggccagttagaaaatcctatttctgaactgttagagccattccaataaggaatagtaattgagtttcaagtttttgttaccatattttgaaatggtatgttcatgttgggacccctttttattgaatatatttccatgttttatcagtttccatgatttatcaagttttttttttaaggaaatcaaagttttaactttaaagataccctgatatttttcttaatgctaaatttaatgactggcaaaaaggtattgggtgctgttaagcaactgttattaattctctatctaaaggaatgctatcttgaatctattagaagtcaaagcttccaaatttgttcaaatttcctggctgtatgacaggtaaccatgactatccatttttttggccaatgaaaaatgccatcaaattcctgtatcagccaggcatatagtggctcatgcctgtaatctctgatgtagcaggccgaggtgggaggatcacttgagcctagaagttttgataccagcctgggcaacatagcaagaccccatctctgaaatttttttaattcctatgtcataagtcatttttatttttgtagagatagggatctcacaatattgcccaggctggtctcaaactcttggcctcaagcagtcctcctgcctcagcctcccaaaatgttgggattactggtatgtgctgctggacccagccaagtagcacttttaatttgaaaaatagttctatcagttttcagtcaggcgcggtggctcagcctgtaatcccagcactttgggaggccgagcgggggtgatcacctgaggtcgggagttcgagactagcctgaccaacatggagaaaccctgtctctactaaaaatacaaaataagccgggcatgttagcgcatgcctgtgatcccagctactcgggaggctgaggcaggagaattgcttgaacccaggaggcagaggttgcggtgagccgagatcatgccattgcactccagcctgggtaacaagagcgaaaactccgtctcaaaaaaaaaaaaagaaaaaatagttctatcagttttcataaagtactactttaatcttaaaaagattaatctagaaacccttcaaattataaaatgtcatttttaaaaggcaggagttgatatcctgatgaaattcaggtctccaaacaacttaccataatttacttcctgtattttaagtaacatgatagggtacttagagattaattgccaagaaactttttgaatatagtcaacctgcccgcacttgccatgatgagttttcttttgttccttccctctagtattctaggagatgaggttttgggaatctggtccagacatgctgagaaagctgatgtcaactgtgcctgtgtatctcattcaggaatcagtcttgttacaggagatgactttggcatggttaagttatttgacttcccatgtccagaaaaatttgtaagtttgtgttttgtttactattatcagtttactcctaattttgatgtcttatcatcagcacttttccccatatatttaaaatgttttgtcctaatttctaaatttttccccaaactttctaaatctatttactttgaaataaaagctattagaaacaaatcctctccctcgagtaataccatctttggaaccatcctacaaaagctgtaattagcttttcaccaaacctataatcagttatcaaatttcaaatgcttttccttagagaaaaatggtcagagtacctggagacatctgactgcccacacagcctggttttgcagatccactactcatgctgaaaagcattctaatcactggctgcggtgctaactccctactctctccacagctcttgtcatagagattatagttcctaataagagcctttgacttctgtgtgcaccaaatgccctgagcttgtctgtcattgttttttaggcaaaacacaaaaggttcttgggtcattcgccccatgtgacaaatattcgatttaccagtggtgatcgacatgttgttagtgctggaggtgatgactgcaggttagtaactttctcagcccatgaagagcagactatgttactagttaagagacttaatacaacaactcctacagctttggtttatgaaatcagctagtcaacattagtagaaggtagtataaccagatggctcttcagaatctcatatttatgcaaatacagaataaaaggagttaaagaggaaaaatattacacatgtaacctgaaagcacaactgaaaaatattaaactgttatgaaaatctaaaaacataattaactccctgcaattttcttctctgattgcagcttatttgtctggaaatgtgtacatacacctcactgagagatgctgagatgactacagaaattaactttgagaccagaattacagagaagaaaaaccaaaacccaaccctgcatggtcaagtggtgctaacccaagactgtaacagggagaaatgcccagaatcatcaaaatagtgaaagactgatctgttcaaaatatttgctatatgcactgggtataatccgtaatccatacactgccagataatgccatttcaaggaaggatcgaatacttgatggtaaaggccaagtccccctgtattgggaagtgtgtgatttcggcagacctgctgggaaaatttagggtagagcactctttacagaagaactcaaaaacccaatttggataattttcattatctttttagcaaaatggtttcttaatgtttatattttattttcaaggttcattgtttaatgaaatattttattcttgcatttccataaggaaagggaaagtcatgatcatcctaaaggatcacagtttttaaaaggcaaacattttccctaaggaaacagacacaagctttcctagagaatatgatgttttttaggcattaataaggtccttttttataaaggacacttttctcctagtagttttgaattcaggaacagatccaaagttagcagtatatggctgctacatttccattttcattttcgagccatcagtttatgttcagatgccatctctgtaatcgcacatttaaaacataactgtagcctcactaatggaaaagtagtatgatgaacaatcattcccaatggtgtacaatgtaagggttttagggagcaacagtatttaactggaagaaagaattgcatatttaatgtagtctaatatatacacatttgtttaacatgtaaacaaaagtgttaaattcacatatacaacattatacaatttaatcactcttggaataaaatttttatagccttttttctattgggaaaatttgtttagatgtgtgccactccataggtttatttccaaaatgaatgagcccaactccatttgtaaaaacttgtcagttagaattcctttttttagtggattagggctgaattcttagatccttatttcttttcactttaaatgctgccaaagatcactactcatcattcaggaattcgctgtctagcctatctgtagtttcctgaagattgaaaattatgtagactgctatttaaaaatatatttttctaagtgtgaggtttaagatgctgtattgaccctatgagtttttaatgtgttaattatctttatagcataatagatcgctttaggttcctggaatcccatttggtctgacaggatatatgaagattcttaatacctattttctgtgtctaatacttggttaatactaaaaatagaaatgactaaattacatcacagaaagcataaccagtgattgaacctggtagttttaaagctctaaatagctgtggctgaaggactgattatggggctaagaagcttgaaacgtaagttggtacttgttcatcagtggattctcctaaattaagccaaattttgaaatacatgactattaagtttctactcatgtatttacagtcagtcaataaattaaaggaggaaaaaaatccctgaacaacctgcccataaaaagaaaaatactctacatttgagcctgctgcagttttaaattttccctctgggtcaagtttgccagcttttggctacagagaaattatatttccattacagtgcaggtagaaactctgtaaccttaagcatgtaaactacatagaataaaactgtttccactgcatttctgtccttcaaagtggccaacctgattaagtcagccttaatcactgctgctgtcagtttcacgactaaaggtcatattgactaagtagtcatcagctgaccacctcgctgtatcagccagcaacgaggggaaggtgaagaaacatgataggccatatagaatctgccctatgtttacttttttaacccagataattatttttgtgtgcagtatctaagctcctgattgtgtaacctgggacttctggcaccttttgttccattcattttatgtataaaatgcatgccaaagcacactgtgccctctggtacccttgcttccaatcgccaaccatgctcatttccttcctttttttgtggtccctttttgtggtgatcattttaaaccacgtcatccaacaaatgttttatggtcaaccttagcttgttcataagccatagcaactgaaagattaaactcttaaatatgtgtctgggcagtggctattaaatagcaaaaaacaatcagattttagtattttattatttccttgtaaaatggctgaactaaattaaacccttgtttcccatttgttctataatttatagtgaaactgagaacaaaactatctttataaatgatagctaaaagtatttccagatatttaaacaatttaaaataaatttcttctgcagagatgcaaagcatctcaacactggaatgaacaaatgccttaaattcaatggagtaaacctttagaatgaagaggaactgtcatttcacccaagccgaagacaacagccttatgcacttgtgtgctctgtctttgctgcttctcgtgtttcaagcctttcctgtgggatcagcacagcaaagtgcaacttaccaaatggtttaatgactggttaattctttcttctcccaatggaaaagcaatggcaacacaacagtagactgctggcttgacaatcttaaacgtgagcctttgcacatgtaggtttatcatcatttgagtatacgactaagcaagtcaatgaactttttttttttttttagcagtttaatttggtcctgagaatgttgcagtctttattaccccttttgcattaatccacttttctaaccaccttttaagctttaatttttaacactatacaccaagtctttgaaatcagtgatctgttatttaactctaaagcatttgacacttcttgccttaacagttttaaaaaccacacacaaaaaaactctgtaagtaatacagtaggccaaaagtttcatcctatctatcttgcagtttacctatctgatctgatctctgtaattatagttctgtcatttaaaatatactatttaaatctaatttttacatttcaaaaattatcttcagtagtaactaagtatattttctgtggattctgagaatgttatttttcagaatgtgagaatatatatgtacatttataatcttgtgactttaaagtctgttttcagatacagtatgtaaatacttgtaaaaaaatttgtataattttgtgataatgtagtttcccaaaaaaattatttagaaggcattatgttattagtaaatgagagcactgtatagaactgttcctattttctgcacttgccattccagctgcctccactgtccatacccacctcattcatcctgtcacagaaggcaggaaaactgggaactttaccaaagtagcactcagcctgagaggcctgtataatcatgcttttcaaactaaattcacttaaaaattaaaaagcagaattgaatattttaagcagcctcagtacctttggccaatgctgttttcatggtggattatgaacattatataatctttgggaaaagtgaaagtagtacaatttttagaataatgacaactgcctcactgcatctctccactcacacagcaaccgtgtagccccctaagctgcagtaccatgactaaccatgatgtcaatttcatatgctgatcctcacaacagcagtgcacaaacatgccccaaatattttaacagaatttagctcttccttaagctgtcttttcatagtaaaaacaaaacaaaaacacccaatgttaaaaccacataataaacttacaaacttgaaaaattagacacttcagatagataggcaataaaacttcatattatgaaagcaatatattccaagtttcaaagatttgacaagttctgtagagtatctttcatcagtacatgaaaacttccaaactgcatgatcttctgccaggcaggactgggtgctattcgctggtttgaggtcgaatccatttcaaggcatgtcgtggtgggacattaatggtgggatggtagaatgtgcagtccggtcttgtacattgagtgttaaacctacaatgttttggatgatagaagggacattccatcttcttacaagcagggaagtaacggcagagctgactactggaaggtggtgctggtggtgcaactgctggttttggagacagtactggaattcttctactcacatgagtgaagggacaatctggtttagtacactttgcatcatatttacaatttgggtgaacaaacaaacatttttcagcaaatttacaattggggaaggctttgcagggtgagatggggtgatggtaggcacactcatccccatttttacaagcaggccagtacttgcagcgctccaaaagtttttctggtttctgtgccacactcagttcactcatctcagcgttagaaaagctaccatttgggtcctcaagctgcctgctcagcaagtgcaactgctgtgggtggaggagacctctgagtcccttgtttgaggctgcagtttggtttacgggtttcattccttcaaagcacatgtcctcctcttgatctgacatgtatcctggggggctggggacaccatccagcgtcactataaacttgggacttgcaggtttatctggttgtacaagatctcgtgtctgcataaggtgtcctgaaagtacccgaagggaatctgcagtcttcatccccgactcttggtttggtgccactactacttcctcagacagctttggcttcttcagaataaatgatcttgtgtctgcatggaccatggattccatgtcatagtaatcttgactcatctgcagagtttctgccattactgggtcgatttgcagtcgggataataattgcctctgttgagttccttgatttttttctacagaatctccttttgtttcctcttctttaatggggggacttattctgggggtcctactttgtccctggaccacttctgctagcaattcttcttgagaagttcgagttctgggagcaactggaagtgtctgtttctgtggaactgtagagtagttagttgtttttgttacggattcttgagcttcagatatagccttcaaaatcagattcttgttagcttgtttagaaggtggaagagaaggtctcctttcaggctttgcaggcacagacacactgctggagatgcttcctgttcgagacccgtaatcatcatcttcttcctcctcttctccatcatgattgaatttttttactttaacaactgaacttaccacaggcaactttctcttccgaaagttttcatcctccatactcattttctccgagttgtttctaaagaacggactatacgtttcttctaagctgttaagcacctctggttcacacaaacgtcctgtttcatatacccaactactctgcatatcaagctgcttggcagcatgaatactattctgctgctgttgaaattgcaacctgtttaaatgaacaccactatctgcatttctacttgcaggtggtcgataaatttcaatagaagggcgagaagaaccatatgtaagtgtcactgtaggttttttctgagataagggattctcctgcacaaagttgaggtcttcgtcaatgagatcatctggttctggcttaatatcaatcacatcttcagagggtgctggctccctcaaaggtttcactgttgacattagtcgggttgcagctccatcatcgtaagtctgtctgacatttgtggtttttgactcctgcgaacttgtagaaactctggaatctcttttttcaggtctcgcgctaggaatggcaagtggtggcactgcagcttcatgcctcctctcatctccccgactgaaattgctcttgtttgaaggcacgttactatcaaagatgttggtatcagaagacttcagactagagggttcagttgtaacagagcgaagtttatctaatacaccatgaagccatacggtgaatcgaattgtgttgttccctagaaacagggacagatcctctgtcatttggtcctgacttttcttgttggccaccatcaccataatgtaatcaggaagttcttcatctatttaaaaggaaaggtagatcaaaactttgtttcctcaaaactttcttcttaaagttgatgtgcttgaaaatatagatgtagctctaagctttagagtcgcagagctctactggaattacattggacaagatggcttagctttaatttttttctcttcattccacaggtatttcaaatacaacataagctcctaattcttgtaatttccccttaatggcactccggatcttgcggctgatctcggtgccgatctccatggctctgcggcgtgcgggaactcagcactgcgcggcgcttggcttacccggaggctgccgcggactcctaccccgcagccgggacaccaccgcctcc

SEQ ID NO: 17449 - RNA, 13686 nt, Homo sapiens
  source 1..13686: mol_type = other RNA
tcaggccaggcacagtggctcatacctggaatcccagcactttgggaggccgaggcaggcagatcacctgaggtcaaggtatttgagaccagcctggccaacatggtgaaaccccatctctactaaaaatacagaaattagctgggtgtggtggtgcacacctgtaatgctagctactcgggaggctgaggtaggagaatcgcttgaacctgggaggcagaggttgcaataagcctagatcatgccactgcactcaagcctgggagacagagcgagactacatcttaaaaaaaaaaaaaaaagtattatgagagaggataatgtattgtaatgtattgtagaggctaaataaaattatgctcatgtcagaaaaaaagagtatttctcaaaataaaattcactgaaactggatgtttattttgactgagatatagtatatcctcaaattgccatagaaagtttacaagaatattagaggtaaattataaatatcagggcctttttaaaaaaaaaagattctgcttataacttggtatttgtttataataaaaattatagtagccaataatgaacacttactctggcttggttatttacttaggtcaaaagaaggaggagcggttaaactgtgggatcaggaactgaggcggtgccgtgccttcaggcttgagacaggacaagccacagattgtgttcgttctgtgtgcagaggcaaagtaagatgttccatgagctgatacagtgcagcagaaaacagaaagtggttattactgtgattccctcaccctttgcagcctaatgaacaatacttaataatgcataacgatggatttgcttgccaacattactctgtctttgctgctttctttgccaaagttagcaccagtgtggtgcataagctaggaagctattctgtctaaatactgtatgtaaacctccaatattttctagaatctgccaatttaacaactctagtagacataattgaaagcccttggcagttgactcatattaggacagctgtctccattttttaaaaaaacacacattccctagataaaacgtgcagtaaacaaacaatgaaatactactcagccataaaaaataatgaaattctgtcattcttggtggcaacatggatgagactggaggacatgatgtgaagtgaaataagccaggcacagaaagataaatacatgttctcactcctgtgcagaaactaaaaaagttgatcccacagaggtggagagtagaatagtggttactggaggcggacaagggggagggggagggggatagggaaggactggttaaaggatacaagtttacacagccagataggaatagtatgttttagtattctgtagtactgtaggatgactatagttaagaatcacgtatttatgtattttcaggtatttacaagagaggattttgaaagtttccatcacaaagaaatgataaatgtctgaggtgatggttatgcgtattaccctatgccctatagatatgtataattatgtgtcaatttcaaaataaaaattcaaaactacaactcctatgaaaatttttgagcgtgtttgtacttattaagtgtatttataaatcatacggatattatcttcagcctgcatattaaattgtagttaagcttttactttttaactaaaaaataaattctattattttttcctatatcccactgcactgaccccagtttggaaatcctaagattatcaaataaaaactttgattattgaagaatccaggtgtactgccacagaaaagttctattctgtagcatggactctaatatgtaatctagcccattgtgcttacagatagatgtgtgcctgtagtcatagaaaaatttgcatgagctaatgactgccttgctactagattagctcaaagcaaaaagttctctgaaagcaggtcaatagggtcatttttatattatgaagaagaaaagcagctgttgtattacattcactgtattggtcctgcttgtgtttcagggcaagatccttgttgggacaaggaatgctgaaataatcgaagttggagagaaaaatgcagcttgtaatattttagttaacggtcatgtggatgggccaatctggggactagcaacacatccttccagggattttttcctttctgctgcagaagatgggacagtgagactttgggatattgctgataaagtaagtacagataatttttttaaaagaggttacaacttctaaaaagaaaagttggaagttctaaattgctagtacttaaagaactgccagaattctgttgagcattttgaggggaaactggtataatttagaagtacttcacttaatgtttcctatgactctttttttttttttttttaaatgcagaagatgttaaacaaagtgaatttgggacatgctgctcgtactgtgtgttacagccctgaaggggacatggtggctattggaatgaaaaatggagaatttatcattttactagtgagttctctaaaaatatggggaaagaagagagacaggagatgtgcaatccatgatatcaggttagtgaacaaatggaatagagtttctagtatatacttgatttaacttccatttgtaaaattttccatagccttgccttcaaaaagaggtccccagggcctgtagcatttcccgtattataaattgtatgctaaaatatggctgtttgtatactacttaattcttcttgctaaattataaacccactgggcaccaactataatagcaagtactagtaggtaatgtttgatgaattcatgttaacacttagccatgtccattaagttcatcccaccaagaggtatctcccactgtaatacaagagagctatctgcccttcaaaagttgtcaccctggaaaactaaagttgtgatttcaaacatatcttctcttagtaacctcagtttgggaatatgtagttcattaatttaatcaatacctattgattaaatgttccagaatccaaattaatttaaatgtttcttaaacctttgtttttcagtgcttaagcatttttcaacagtggctaccatttacggagtacttccgtgtgatcagtagataagattattgaatctaggtctgtcaaaagcttgtacacttttcatcagtaaaatccttttacaaatgaaaccttcctcagaacttcaatatataaaatagtaacagtggcttcccttagcttttacatgtctctatcgtacctcagtaagactcatgggccatttcaagagactgaattgtcccatatgactccaaagattgctaggcaaatagcatttcactttgtcttttaaataagttcttcaggccgggcgcggtggctcatgcctgtaatcccagcactttgggaggccgaggcaggcagatcacctgaagtcaggagtactcgaccagcctggccaacatagtgaaaccccatctcaactaaaaatacaaaaatcagccgggcgtggtggcaggcgcctgtaatcccagctactcagggggctgaaacaggagaatcgcttgaacccgggaggcggaggttgcgccatcgcactccagcctgggagacaagagcgagacttcgtctcaaaaaaaaaaaattcttcttccaagattcaagttgtgtcatttcaccttaataactggaggttagttaagctgggctgtgttctttgcttaatattaagacaacgttttttccagatggaagaaaactatcttaatgaattgttagcttattaattatgtaatgctaatggcttttaaaagctgagatgttctgactgggtgttgtggctcacacctgtaatcccagtaccttgggaggccaagggggaaggattgcttgaggccaggagtttgggaccatagtgagaccccgcctctatttaaaaaattaaattttgttttgttttgttttgagttggagttttgctcttgttgcccatgctgaagtgcaatggtgcaatctcagctcaccacaacctgtgcctcctgggttcaagcgattctcctgcttcagcctcccgagtagatgggattacaggcgtgcaccaccatgcctggctaattttgtatttttagtagagacagggtttctctatgttggtcaggctggtctcaaactctcgacctcaggtgatctgcccgcctccgcttcccaaagttctgggattataggtgtgagccactgggcctggcctaagaaagtttttttaagccattagacgtttttaaaggaattgggagatgacaattggggaaatatttaaaatttaagtaaaatataaagcttccttatttcatgtaacccagacaatctcagtatacatgatcagttgtgtctgacaggtaaatctatttgaggccttatcacacgttacttttaagaactagaaaggaaaagtcactgatcttaagtatttataatacttcatgtggtctaatactttttacgttttgttttgattcagatttagtccggattcccggtatctggcagtaggttctagtgagaactcagtggatttttatgacctaacgctgggccccactcttaacagaatcagctactgcaaagacattccaagctttgtcattcaaatggacttctctgcagatagcagttatctccaggtacagtaccaatactgtatacccaggtggcaagttcttctgcttttacatttcgtgttagtgaatgcatttaaagttcctgagctccagagctccagcttctcaactcctccctttgtaccttctgacctacagctcccctttcctcccccacttatcagagcttttctcctattaagtttttgtagtgatcttttgcatacttaataatgttagacatgtaaatcaagtagcaatatgctagtattctgtaaaccccctgtggattttgtctctcacctaatggaattcttgtcccattttaatctgatgaaaaaggtctctagtggctgctataaacggcatgtctatgaagtgccttcaggaaaacatcttatggatcatgccgctattgacagaattacttgggctacatggactaggtaaatacttatatattcacaaggcaagaactgactttgaaggccagttagaaaatcctatttctgaactgttagagccattccaataaggaatagtaattgagtttcaagtttttgttaccatattttgaaatggtatgttcatgttgggacccctttttattgaatatatttccatgttttatcagtttccatgatttatcaagttttttttttaaggaaatcaaagttttaactttaaagataccctgatatttttcttaatgctaaatttaatgactggcaaaaaggtattgggtgctgttaagcaactgttattaattctctatctaaaggaatgctatcttgaatctattagaagtcaaagcttccaaatttgttcaaatttcctggctgtatgacaggtaaccatgactatccatttttttggccaatgaaaaatgccatcaaattcctgtatcagccaggcatatagtggctcatgcctgtaatctctgatgtagcaggccgaggtgggaggatcacttgagcctagaagttttgataccagcctgggcaacatagcaagaccccatctctgaaatttttttaattcctatgtcataagtcatttttatttttgtagagatagggatctcacaatattgcccaggctggtctcaaactcttggcctcaagcagtcctcctgcctcagcctcccaaaatgttgggattactggtatgtgctgctggacccagccaagtagcacttttaatttgaaaaatagttctatcagttttcagtcaggcgcggtggctcagcctgtaatcccagcactttgggaggccgagcgggggtgatcacctgaggtcgggagttcgagactagcctgaccaacatggagaaaccctgtctctactaaaaatacaaaataagccgggcatgttagcgcatgcctgtgatcccagctactcgggaggctgaggcaggagaattgcttgaacccaggaggcagaggttgcggtgagccgagatcatgccattgcactccagcctgggtaacaagagcgaaaactccgtctcaaaaaaaaaaaaagaaaaaatagttctatcagttttcataaagtactactttaatcttaaaaagattaatctagaaacccttcaaattataaaatgtcatttttaaaaggcaggagttgatatcctgatgaaattcaggtctccaaacaacttaccataatttacttcctgtattttaagtaacatgatagggtacttagagattaattgccaagaaactttttgaatatagtcaacctgcccgcacttgccatgatgagttttcttttgttccttccctctagtattctaggagatgaggttttgggaatctggtccagacatgctgagaaagctgatgtcaactgtgcctgtgtatctcattcaggaatcagtcttgttacaggagatgactttggcatggttaagttatttgacttcccatgtccagaaaaatttgtaagtttgtgttttgtttactattatcagtttactcctaattttgatgtcttatcatcagcacttttccccatatatttaaaatgttttgtcctaatttctaaatttttccccaaactttctaaatctatttactttgaaataaaagctattagaaacaaatcctctccctcgagtaataccatctttggaaccatcctacaaaagctgtaattagcttttcaccaaacctataatcagttatcaaatttcaaatgcttttccttagagaaaaatggtcagagtacctggagacatctgactgcccacacagcctggttttgcagatccactactcatgctgaaaagcattctaatcactggctgcggtgctaactccctactctctccacagctcttgtcatagagattatagttcctaataagagcctttgacttctgtgtgcaccaaatgccctgagcttgtctgtcattgttttttaggcaaaacacaaaaggttcttgggtcattcgccccatgtgacaaatattcgatttaccagtggtgatcgacatgttgttagtgctggaggtgatgactgcaggttagtaactttctcagcccatgaagagcagactatgttactagttaagagacttaatacaacaactcctacagctttggtttatgaaatcagctagtcaacattagtagaaggtagtataaccagatggctcttcagaatctcatatttatgcaaatacagaataaaaggagttaaagaggaaaaatattacacatgtaacctgaaagcacaactgaaaaatattaaactgttatgaaaatctaaaaacataattaactccctgcaattttcttctctgattgcagcttatttgtctggaaatgtgtacatacacctcactgagagatgctgagatgactacagaaattaactttgagaccagaattacagagaagaaaaaccaaaacccaaccctgcatggtcaagtggtgctaacccaagactgtaacagggagaaatgcccagaatcatcaaaatagtgaaagactgatctgttcaaaatatttgctatatgcactgggtataatccgtaatccatacactgccagataatgccatttcaaggaaggatcgaatacttgatggtaaaggccaagtccccctgtattgggaagtgtgtgatttcggcagacctgctgggaaaatttagggtagagcactctttacagaagaactcaaaaacccaatttggataattttcattatctttttagcaaaatggtttcttaatgtttatattttattttcaaggttcattgtttaatgaaatattttattcttgcatttccataaggaaagggaaagtcatgatcatcctaaaggatcacagtttttaaaaggcaaacattttccctaaggaaacagacacaagctttcctagagaatatgatgttttttaggcattaataaggtccttttttataaaggacacttttctcctagtagttttgaattcaggaacagatccaaagttagcagtatatggctgctacatttccattttcattttcgagccatcagtttatgttcagatgccatctctgtaatcgcacatttaaaacataactgtagcctcactaatggaaaagtagtatgatgaacaatcattcccaatggtgtacaatgtaagggttttagggagcaacagtatttaactggaagaaagaattgcatatttaatgtagtctaatatatacacatttgtttaacatgtaaacaaaagtgttaaattcacatatacaacattatacaatttaatcactcttggaataaaatttttatagccttttttctattgggaaaatttgtttagatgtgtgccactccataggtttatttccaaaatgaatgagcccaactccatttgtaaaaacttgtcagttagaattcctttttttagtggattagggctgaattcttagatccttatttcttttcactttaaatgctgccaaagatcactactcatcattcaggaattcgctgtctagcctatctgtagtttcctgaagattgaaaattatgtagactgctatttaaaaatatatttttctaagtgtgaggtttaagatgctgtattgaccctatgagtttttaatgtgttaattatctttatagcataatagatcgctttaggttcctggaatcccatttggtctgacaggatatatgaagattcttaatacctattttctgtgtctaatacttggttaatactaaaaatagaaatgactaaattacatcacagaaagcataaccagtgattgaacctggtagttttaaagctctaaatagctgtggctgaaggactgattatggggctaagaagcttgaaacgtaagttggtacttgttcatcagtggattctcctaaattaagccaaattttgaaatacatgactattaagtttctactcatgtatttacagtcagtcaataaattaaaggaggaaaaaaatccctgaacaacctgcccataaaaagaaaaatactctacatttgagcctgctgcagttttaaattttccctctgggtcaagtttgccagcttttggctacagagaaattatatttccattacagtgcaggtagaaactctgtaaccttaagcatgtaaactacatagaataaaactgtttccactgcatttctgtccttcaaagtggccaacctgattaagtcagccttaatcactgctgctgtcagtttcacgactaaaggtcatattgactaagtagtcatcagctgaccacctcgctgtatcagccagcaacgaggggaaggtgaagaaacatgataggccatatagaatctgccctatgtttacttttttaacccagataattatttttgtgtgcagtatctaagctcctgattgtgtaacctgggacttctggcaccttttgttccattcattttatgtataaaatgcatgccaaagcacactgtgccctctggtacccttgcttccaatcgccaaccatgctcatttccttcctttttttgtggtccctttttgtggtgatcattttaaaccacgtcatccaacaaatgttttatggtcaaccttagcttgttcataagccatagcaactgaaagattaaactcttaaatatgtgtctgggcagtggctattaaatagcaaaaaacaatcagattttagtattttattatttccttgtaaaatggctgaactaaattaaacccttgtttcccatttgttctataatttatagtgaaactgagaacaaaactatctttataaatgatagctaaaagtatttccagatatttaaacaatttaaaataaatttcttctgcagagatgcaaagcatctcaacactggaatgaacaaatgccttaaattcaatggagtaaacctttagaatgaagaggaactgtcatttcacccaagccgaagacaacagccttatgcacttgtgtgctctgtctttgctgcttctcgtgtttcaagcctttcctgtgggatcagcacagcaaagtgcaacttaccaaatggtttaatgactggttaattctttcttctcccaatggaaaagcaatggcaacacaacagtagactgctggcttgacaatcttaaacgtgagcctttgcacatgtaggtttatcatcatttgagtatacgactaagcaagtcaatgaactttttttttttttttagcagtttaatttggtcctgagaatgttgcagtctttattaccccttttgcattaatccacttttctaaccaccttttaagctttaatttttaacactatacaccaagtctttgaaatcagtgatctgttatttaactctaaagcatttgacacttcttgccttaacagttttaaaaaccacacacaaaaaaactctgtaagtaatacagtaggccaaaagtttcatcctatctatcttgcagtttacctatctgatctgatctctgtaattatagttctgtcatttaaaatatactatttaaatctaatttttacatttcaaaaattatcttcagtagtaactaagtatattttctgtggattctgagaatgttatttttcagaatgtgagaatatatatgtacatttataatcttgtgactttaaagtctgttttcagatacagtatgtaaatacttgtaaaaaaatttgtataattttgtgataatgtagtttcccaaaaaaattatttagaaggcattatgttattagtaaatgagagcactgtatagaactgttcctattttctgcacttgccattccagctgcctccactgtccatacccacctcattcatcctgtcacagaaggcaggaaaactgggaactttaccaaagtagcactcagcctgagaggcctgtataatcatgcttttcaaactaaattcacttaaaaattaaaaagcagaattgaatattttaagcagcctcagtacctttggccaatgctgttttcatggtggattatgaacattatataatctttgggaaaagtgaaagtagtacaatttttagaataatgacaactgcctcactgcatctctccactcacacagcaaccgtgtagccccctaagctgcagtaccatgactaaccatgatgtcaatttcatatgctgatcctcacaacagcagtgcacaaacatgccccaaatattttaacagaatttagctcttccttaagctgtcttttcatagtaaaaacaaaacaaaaacacccaatgttaaaaccacataataaacttacaaacttgaaaaattagacacttcagatagataggcaataaaacttcatattatgaaagcaatatattccaagtttcaaagatttgacaagttctgtagagtatctttcatcagtacatgaaaacttccaaactgcatgatcttctgccaggcaggactgggtgctattcgctggtttgaggtcgaatccatttcaaggcatgtcgtggtgggacattaatggtgggatggtagaatgtgcagtccggtcttgtacattgagtgttaaacctacaatgttttggatgatagaagggacattccatcttcttacaagcagggaagtaacggcagagctgactactggaaggtggtgctggtggtgcaactgctggttttggagacagtactggaattcttctactcacatgagtgaagggacaatctggtttagtacactttgcatcatatttacaatttgggtgaacaaacaaacatttttcagcaaatttacaattggggaaggctttgcagggtgagatggggtgatggtaggcacactcatccccatttttacaagcaggccagtacttgcagcgctccaaaagtttttctggtttctgtgccacactcagttcactcatctcagcgttagaaaagctaccatttgggtcctcaagctgcctgctcagcaagtgcaactgctgtgggtggaggagacctctgagtcccttgtttgaggctgcagtttggtttacgggtttcattccttcaaagcacatgtcctcctcttgatctgacatgtatcctggggggctggggacaccatccagcgtcactataaacttgggacttgcaggtttatctggttgtacaagatctcgtgtctgcataaggtgtcctgaaagtacccgaagggaatctgcagtcttcatccccgactcttggtttggtgccactactacttcctcagacagctttggcttcttcagaataaatgatcttgtgtctgcatggaccatggattccatgtcatagtaatcttgatttttttctacagaatctccttttgtttcctcttctttaatggggggacttattctgggggtcctactttgtccctggaccacttctgctagcaattcttcttgagaagttcgagttctgggagcaactggaagtgtctgtttctgtggaactgtagagtagttagttgtttttgttacggattcttgagcttcagatatagccttcaaaatcagattcttgttagcttgtttagaaggtggaagagaaggtctcctttcaggctttgcaggcacagacacactgctggagatgcttcctgttcgagacccgtaatcatcatcttcttcctcctcttctccatcatgattgaatttttttactttaacaactgaacttaccacaggcaactttctcttccgaaagttttcatcctccatactcattttctccgagttgtttctaaagaacggactatacgtttcttctaagctgttaagcacctctggttcacacaaacgtcctgtttcatatacccaactactctgcatatcaagctgcttggcagcatgaatactattctgctgctgttgaaattgcaacctgtttaaatgaacaccactatctgcatttctacttgcaggtggtcgataaatttcaatagaagggcgagaagaaccatatgtaagtgtcactgtaggttttttctgagataagggattctcctgcacaaagttgaggtcttcgtcaatgagatcatctggttctggcttaatatcaatcacatcttcagagggtgctggctccctcaaaggtttcactgttgacattagtcgggttgcagctccatcatcgtaagtctgtctgacatttgtggtttttgactcctgcgaacttgtagaaactctggaatctcttttttcaggtctcgcgctaggaatggcaagtggtggcactgcagcttcatgcctcctctcatctccccgactgaaattgctcttgtttgaaggcacgttactatcaaagatgttggtatcagaagacttcagactagagggttcagttgtaacagagcgaagtttatctaatacaccatgaagccaacataagctcctaattcttgtaatttccccttaatggcactccggatcttgcggctgatctcggtgccgatctccatggctctgcggcgtgcgggaactcagcactgcgcggcgcttggcttacccggaggctgccgcggactcctaccccgcagccgggacaccaccgcctcc

SEQ ID NO: 17450 - RNA, 13801 nt, Homo sapiens
  source 1..13801: mol_type = other RNA
tcaggccaggcacagtggctcatacctggaatcccagcactttgggaggccgaggcaggcagatcacctgaggtcaaggtatttgagaccagcctggccaacatggtgaaaccccatctctactaaaaatacagaaattagctgggtgtggtggtgcacacctgtaatgctagctactcgggaggctgaggtaggagaatcgcttgaacctgggaggcagaggttgcaataagcctagatcatgccactgcactcaagcctgggagacagagcgagactacatcttaaaaaaaaaaaaaaaagtattatgagagaggataatgtattgtaatgtattgtagaggctaaataaaattatgctcatgtcagaaaaaaagagtatttctcaaaataaaattcactgaaactggatgtttattttgactgagatatagtatatcctcaaattgccatagaaagtttacaagaatattagaggtaaattataaatatcagggcctttttaaaaaaaaaagattctgcttataacttggtatttgtttataataaaaattatagtagccaataatgaacacttactctggcttggttatttacttaggtcaaaagaaggaggagcggttaaactgtgggatcaggaactgaggcggtgccgtgccttcaggcttgagacaggacaagccacagattgtgttcgttctgtgtgcagaggcaaagtaagatgttccatgagctgatacagtgcagcagaaaacagaaagtggttattactgtgattccctcaccctttgcagcctaatgaacaatacttaataatgcataacgatggatttgcttgccaacattactctgtctttgctgctttctttgccaaagttagcaccagtgtggtgcataagctaggaagctattctgtctaaatactgtatgtaaacctccaatattttctagaatctgccaatttaacaactctagtagacataattgaaagcccttggcagttgactcatattaggacagctgtctccattttttaaaaaaacacacattccctagataaaacgtgcagtaaacaaacaatgaaatactactcagccataaaaaataatgaaattctgtcattcttggtggcaacatggatgagactggaggacatgatgtgaagtgaaataagccaggcacagaaagataaatacatgttctcactcctgtgcagaaactaaaaaagttgatcccacagaggtggagagtagaatagtggttactggaggcggacaagggggagggggagggggatagggaaggactggttaaaggatacaagtttacacagccagataggaatagtatgttttagtattctgtagtactgtaggatgactatagttaagaatcacgtatttatgtattttcaggtatttacaagagaggattttgaaagtttccatcacaaagaaatgataaatgtctgaggtgatggttatgcgtattaccctatgccctatagatatgtataattatgtgtcaatttcaaaataaaaattcaaaactacaactcctatgaaaatttttgagcgtgtttgtacttattaagtgtatttataaatcatacggatattatcttcagcctgcatattaaattgtagttaagcttttactttttaactaaaaaataaattctattattttttcctatatcccactgcactgaccccagtttggaaatcctaagattatcaaataaaaactttgattattgaagaatccaggtgtactgccacagaaaagttctattctgtagcatggactctaatatgtaatctagcccattgtgcttacagatagatgtgtgcctgtagtcatagaaaaatttgcatgagctaatgactgccttgctactagattagctcaaagcaaaaagttctctgaaagcaggtcaatagggtcatttttatattatgaagaagaaaagcagctgttgtattacattcactgtattggtcctgcttgtgtttcagggcaagatccttgttgggacaaggaatgctgaaataatcgaagttggagagaaaaatgcagcttgtaatattttagttaacggtcatgtggatgggccaatctggggactagcaacacatccttccagggattttttcctttctgctgcagaagatgggacagtgagactttgggatattgctgataaagtaagtacagataatttttttaaaagaggttacaacttctaaaaagaaaagttggaagttctaaattgctagtacttaaagaactgccagaattctgttgagcattttgaggggaaactggtataatttagaagtacttcacttaatgtttcctatgactctttttttttttttttttaaatgcagaagatgttaaacaaagtgaatttgggacatgctgctcgtactgtgtgttacagccctgaaggggacatggtggctattggaatgaaaaatggagaatttatcattttactagtgagttctctaaaaatatggggaaagaagagagacaggagatgtgcaatccatgatatcaggttagtgaacaaatggaatagagtttctagtatatacttgatttaacttccatttgtaaaattttccatagccttgccttcaaaaagaggtccccagggcctgtagcatttcccgtattataaattgtatgctaaaatatggctgtttgtatactacttaattcttcttgctaaattataaacccactgggcaccaactataatagcaagtactagtaggtaatgtttgatgaattcatgttaacacttagccatgtccattaagttcatcccaccaagaggtatctcccactgtaatacaagagagctatctgcccttcaaaagttgtcaccctggaaaactaaagttgtgatttcaaacatatcttctcttagtaacctcagtttgggaatatgtagttcattaatttaatcaatacctattgattaaatgttccagaatccaaattaatttaaatgtttcttaaacctttgtttttcagtgcttaagcatttttcaacagtggctaccatttacggagtacttccgtgtgatcagtagataagattattgaatctaggtctgtcaaaagcttgtacacttttcatcagtaaaatccttttacaaatgaaaccttcctcagaacttcaatatataaaatagtaacagtggcttcccttagcttttacatgtctctatcgtacctcagtaagactcatgggccatttcaagagactgaattgtcccatatgactccaaagattgctaggcaaatagcatttcactttgtcttttaaataagttcttcaggccgggcgcggtggctcatgcctgtaatcccagcactttgggaggccgaggcaggcagatcacctgaagtcaggagtactcgaccagcctggccaacatagtgaaaccccatctcaactaaaaatacaaaaatcagccgggcgtggtggcaggcgcctgtaatcccagctactcagggggctgaaacaggagaatcgcttgaacccgggaggcggaggttgcgccatcgcactccagcctgggagacaagagcgagacttcgtctcaaaaaaaaaaaattcttcttccaagattcaagttgtgtcatttcaccttaataactggaggttagttaagctgggctgtgttctttgcttaatattaagacaacgttttttccagatggaagaaaactatcttaatgaattgttagcttattaattatgtaatgctaatggcttttaaaagctgagatgttctgactgggtgttgtggctcacacctgtaatcccagtaccttgggaggccaagggggaaggattgcttgaggccaggagtttgggaccatagtgagaccccgcctctatttaaaaaattaaattttgttttgttttgttttgagttggagttttgctcttgttgcccatgctgaagtgcaatggtgcaatctcagctcaccacaacctgtgcctcctgggttcaagcgattctcctgcttcagcctcccgagtagatgggattacaggcgtgcaccaccatgcctggctaattttgtatttttagtagagacagggtttctctatgttggtcaggctggtctcaaactctcgacctcaggtgatctgcccgcctccgcttcccaaagttctgggattataggtgtgagccactgggcctggcctaagaaagtttttttaagccattagacgtttttaaaggaattgggagatgacaattggggaaatatttaaaatttaagtaaaatataaagcttccttatttcatgtaacccagacaatctcagtatacatgatcagttgtgtctgacaggtaaatctatttgaggccttatcacacgttacttttaagaactagaaaggaaaagtcactgatcttaagtatttataatacttcatgtggtctaatactttttacgttttgttttgattcagatttagtccggattcccggtatctggcagtaggttctagtgagaactcagtggatttttatgacctaacgctgggccccactcttaacagaatcagctactgcaaagacattccaagctttgtcattcaaatggacttctctgcagatagcagttatctccaggtacagtaccaatactgtatacccaggtggcaagttcttctgcttttacatttcgtgttagtgaatgcatttaaagttcctgagctccagagctccagcttctcaactcctccctttgtaccttctgacctacagctcccctttcctcccccacttatcagagcttttctcctattaagtttttgtagtgatcttttgcatacttaataatgttagacatgtaaatcaagtagcaatatgctagtattctgtaaaccccctgtggattttgtctctcacctaatggaattcttgtcccattttaatctgatgaaaaaggtctctagtggctgctataaacggcatgtctatgaagtgccttcaggaaaacatcttatggatcatgccgctattgacagaattacttgggctacatggactaggtaaatacttatatattcacaaggcaagaactgactttgaaggccagttagaaaatcctatttctgaactgttagagccattccaataaggaatagtaattgagtttcaagtttttgttaccatattttgaaatggtatgttcatgttgggacccctttttattgaatatatttccatgttttatcagtttccatgatttatcaagttttttttttaaggaaatcaaagttttaactttaaagataccctgatatttttcttaatgctaaatttaatgactggcaaaaaggtattgggtgctgttaagcaactgttattaattctctatctaaaggaatgctatcttgaatctattagaagtcaaagcttccaaatttgttcaaatttcctggctgtatgacaggtaaccatgactatccatttttttggccaatgaaaaatgccatcaaattcctgtatcagccaggcatatagtggctcatgcctgtaatctctgatgtagcaggccgaggtgggaggatcacttgagcctagaagttttgataccagcctgggcaacatagcaagaccccatctctgaaatttttttaattcctatgtcataagtcatttttatttttgtagagatagggatctcacaatattgcccaggctggtctcaaactcttggcctcaagcagtcctcctgcctcagcctcccaaaatgttgggattactggtatgtgctgctggacccagccaagtagcacttttaatttgaaaaatagttctatcagttttcagtcaggcgcggtggctcagcctgtaatcccagcactttgggaggccgagcgggggtgatcacctgaggtcgggagttcgagactagcctgaccaacatggagaaaccctgtctctactaaaaatacaaaataagccgggcatgttagcgcatgcctgtgatcccagctactcgggaggctgaggcaggagaattgcttgaacccaggaggcagaggttgcggtgagccgagatcatgccattgcactccagcctgggtaacaagagcgaaaactccgtctcaaaaaaaaaaaaagaaaaaatagttctatcagttttcataaagtactactttaatcttaaaaagattaatctagaaacccttcaaattataaaatgtcatttttaaaaggcaggagttgatatcctgatgaaattcaggtctccaaacaacttaccataatttacttcctgtattttaagtaacatgatagggtacttagagattaattgccaagaaactttttgaatatagtcaacctgcccgcacttgccatgatgagttttcttttgttccttccctctagtattctaggagatgaggttttgggaatctggtccagacatgctgagaaagctgatgtcaactgtgcctgtgtatctcattcaggaatcagtcttgttacaggagatgactttggcatggttaagttatttgacttcccatgtccagaaaaatttgtaagtttgtgttttgtttactattatcagtttactcctaattttgatgtcttatcatcagcacttttccccatatatttaaaatgttttgtcctaatttctaaatttttccccaaactttctaaatctatttactttgaaataaaagctattagaaacaaatcctctccctcgagtaataccatctttggaaccatcctacaaaagctgtaattagcttttcaccaaacctataatcagttatcaaatttcaaatgcttttccttagagaaaaatggtcagagtacctggagacatctgactgcccacacagcctggttttgcagatccactactcatgctgaaaagcattctaatcactggctgcggtgctaactccctactctctccacagctcttgtcatagagattatagttcctaataagagcctttgacttctgtgtgcaccaaatgccctgagcttgtctgtcattgttttttaggcaaaacacaaaaggttcttgggtcattcgccccatgtgacaaatattcgatttaccagtggtgatcgacatgttgttagtgctggaggtgatgactgcaggttagtaactttctcagcccatgaagagcagactatgttactagttaagagacttaatacaacaactcctacagctttggtttatgaaatcagctagtcaacattagtagaaggtagtataaccagatggctcttcagaatctcatatttatgcaaatacagaataaaaggagttaaagaggaaaaatattacacatgtaacctgaaagcacaactgaaaaatattaaactgttatgaaaatctaaaaacataattaactccctgcaattttcttctctgattgcagcttatttgtctggaaatgtgtacatacacctcactgagagatgctgagatgactacagaaattaactttgagaccagaattacagagaagaaaaaccaaaacccaaccctgcatggtcaagtggtgctaacccaagactgtaacagggagaaatgcccagaatcatcaaaatagtgaaagactgatctgttcaaaatatttgctatatgcactgggtataatccgtaatccatacactgccagataatgccatttcaaggaaggatcgaatacttgatggtaaaggccaagtccccctgtattgggaagtgtgtgatttcggcagacctgctgggaaaatttagggtagagcactctttacagaagaactcaaaaacccaatttggataattttcattatctttttagcaaaatggtttcttaatgtttatattttattttcaaggttcattgtttaatgaaatattttattcttgcatttccataaggaaagggaaagtcatgatcatcctaaaggatcacagtttttaaaaggcaaacattttccctaaggaaacagacacaagctttcctagagaatatgatgttttttaggcattaataaggtccttttttataaaggacacttttctcctagtagttttgaattcaggaacagatccaaagttagcagtatatggctgctacatttccattttcattttcgagccatcagtttatgttcagatgccatctctgtaatcgcacatttaaaacataactgtagcctcactaatggaaaagtagtatgatgaacaatcattcccaatggtgtacaatgtaagggttttagggagcaacagtatttaactggaagaaagaattgcatatttaatgtagtctaatatatacacatttgtttaacatgtaaacaaaagtgttaaattcacatatacaacattatacaatttaatcactcttggaataaaatttttatagccttttttctattgggaaaatttgtttagatgtgtgccactccataggtttatttccaaaatgaatgagcccaactccatttgtaaaaacttgtcagttagaattcctttttttagtggattagggctgaattcttagatccttatttcttttcactttaaatgctgccaaagatcactactcatcattcaggaattcgctgtctagcctatctgtagtttcctgaagattgaaaattatgtagactgctatttaaaaatatatttttctaagtgtgaggtttaagatgctgtattgaccctatgagtttttaatgtgttaattatctttatagcataatagatcgctttaggttcctggaatcccatttggtctgacaggatatatgaagattcttaatacctattttctgtgtctaatacttggttaatactaaaaatagaaatgactaaattacatcacagaaagcataaccagtgattgaacctggtagttttaaagctctaaatagctgtggctgaaggactgattatggggctaagaagcttgaaacgtaagttggtacttgttcatcagtggattctcctaaattaagccaaattttgaaatacatgactattaagtttctactcatgtatttacagtcagtcaataaattaaaggaggaaaaaaatccctgaacaacctgcccataaaaagaaaaatactctacatttgagcctgctgcagttttaaattttccctctgggtcaagtttgccagcttttggctacagagaaattatatttccattacagtgcaggtagaaactctgtaaccttaagcatgtaaactacatagaataaaactgtttccactgcatttctgtccttcaaagtggccaacctgattaagtcagccttaatcactgctgctgtcagtttcacgactaaaggtcatattgactaagtagtcatcagctgaccacctcgctgtatcagccagcaacgaggggaaggtgaagaaacatgataggccatatagaatctgccctatgtttacttttttaacccagataattatttttgtgtgcagtatctaagctcctgattgtgtaacctgggacttctggcaccttttgttccattcattttatgtataaaatgcatgccaaagcacactgtgccctctggtacccttgcttccaatcgccaaccatgctcatttccttcctttttttgtggtccctttttgtggtgatcattttaaaccacgtcatccaacaaatgttttatggtcaaccttagcttgttcataagccatagcaactgaaagattaaactcttaaatatgtgtctgggcagtggctattaaatagcaaaaaacaatcagattttagtattttattatttccttgtaaaatggctgaactaaattaaacccttgtttcccatttgttctataatttatagtgaaactgagaacaaaactatctttataaatgatagctaaaagtatttccagatatttaaacaatttaaaataaatttcttctgcagagatgcaaagcatctcaacactggaatgaacaaatgccttaaattcaatggagtaaacctttagaatgaagaggaactgtcatttcacccaagccgaagacaacagccttatgcacttgtgtgctctgtctttgctgcttctcgtgtttcaagcctttcctgtgggatcagcacagcaaagtgcaacttaccaaatggtttaatgactggttaattctttcttctcccaatggaaaagcaatggcaacacaacagtagactgctggcttgacaatcttaaacgtgagcctttgcacatgtaggtttatcatcatttgagtatacgactaagcaagtcaatgaactttttttttttttttagcagtttaatttggtcctgagaatgttgcagtctttattaccccttttgcattaatccacttttctaaccaccttttaagctttaatttttaacactatacaccaagtctttgaaatcagtgatctgttatttaactctaaagcatttgacacttcttgccttaacagttttaaaaaccacacacaaaaaaactctgtaagtaatacagtaggccaaaagtttcatcctatctatcttgcagtttacctatctgatctgatctctgtaattatagttctgtcatttaaaatatactatttaaatctaatttttacatttcaaaaattatcttcagtagtaactaagtatattttctgtggattctgagaatgttatttttcagaatgtgagaatatatatgtacatttataatcttgtgactttaaagtctgttttcagatacagtatgtaaatacttgtaaaaaaatttgtataattttgtgataatgtagtttcccaaaaaaattatttagaaggcattatgttattagtaaatgagagcactgtatagaactgttcctattttctgcacttgccattccagctgcctccactgtccatacccacctcattcatcctgtcacagaaggcaggaaaactgggaactttaccaaagtagcactcagcctgagaggcctgtataatcatgcttttcaaactaaattcacttaaaaattaaaaagcagaattgaatattttaagcagcctcagtacctttggccaatgctgttttcatggtggattatgaacattatataatctttgggaaaagtgaaagtagtacaatttttagaataatgacaactgcctcactgcatctctccactcacacagcaaccgtgtagccccctaagctgcagtaccatgactaaccatgatgtcaatttcatatgctgatcctcacaacagcagtgcacaaacatgccccaaatattttaacagaatttagctcttccttaagctgtcttttcatagtaaaaacaaaacaaaaacacccaatgttaaaaccacataataaacttacaaacttgaaaaattagacacttcagatagataggcaataaaacttcatattatgaaagcaatatattccaagtttcaaagatttgacaagttctgtagagtatctttcatcagtacatgaaaacttccaaactgcatgatcttctgccaggcaggactgggtgctattcgctggtttgaggtcgaatccatttcaaggcatgtcgtggtgggacattaatggtgggatggtagaatgtgcagtccggtcttgtacattgagtgttaaacctacaatgttttggatgatagaagggacattccatcttcttacaagcagggaagtaacggcagagctgactactggaaggtggtgctggtggtgcaactgctggttttggagacagtactggaattcttctactcacatgagtgaagggacaatctggtttagtacactttgcatcatatttacaatttgggtgaacaaacaaacatttttcagcaaatttacaattggggaaggctttgcagggtgagatggggtgatggtaggcacactcatccccatttttacaagcaggccagtacttgcagcgctccaaaagtttttctggtttctgtgccacactcagttcactcatctcagcgttagaaaagctaccatttgggtcctcaagctgcctgctcagcaagtgcaactgctgtgggtggaggagacctctgagtcccttgtttgaggctgcagtttggtttacgggtttcattccttcaaagcacatgtcctcctcttgatctgacatgtatcctggggggctggggacaccatccagcgtcactataaacttgggacttgcaggtttatctggttgtacaagatctcgtgtctgcataaggtgtcctgaaagtacccgaagggaatctgcagtcttcatccccgactcttggtttggtgccactactacttcctcagacagctttggcttcttcagaataaatgatcttgtgtctgcatggaccatggattccatgtcatagtaatcttgatttttttctacagaatctccttttgtttcctcttctttaatggggggacttattctgggggtcctactttgtccctggaccacttctgctagcaattcttcttgagaagttcgagttctgggagcaactggaagtgtctgtttctgtggaactgtagagtagttagttgtttttgttacggattcttgagcttcagatatagccttcaaaatcagattcttgttagcttgtttagaaggtggaagagaaggtctcctttcaggctttgcaggcacagacacactgctggagatgcttcctgttcgagacccgtaatcatcatcttcttcctcctcttctccatcatgattgaatttttttactttaacaactgaacttaccacaggcaactttctcttccgaaagttttcatcctccatactcattttctccgagttgtttctaaagaacggactatacgtttcttctaagctgttaagcacctctggttcacacaaacgtcctgtttcatatacccaactactctgcatatcaagctgcttggcagcatgaatactattctgctgctgttgaaattgcaacctgtttaaatgaacaccactatctgcatttctacttgcaggtggtcgataaatttcaatagaagggcgagaagaaccatatgtaagtgtcactgtaggttttttctgagataagggattctcctgcacaaagttgaggtcttcgtcaatgagatcatctggttctggcttaatatcaatcacatcttcagagggtgctggctccctcaaaggtttcactgttgacattagtcgggttgcagctccatcatcgtaagtctgtctgacatttgtggtttttgactcctgcgaacttgtagaaactctggaatctcttttttcaggtctcgcgctaggaatggcaagtggtggcactgcagcttcatgcctcctctcatctccccgactgaaattgctcttgtttgaaggcacgttactatcaaagatgttggtatcagaagacttcagactagagggttcagttgtaacagagcgaagtttatctaatacaccatgaagccatacggtgaatcgaattgtgttgttccctagaaacagggacagatcctctgtcatttggtcctgacttttcttgttggccaccatcaccataatgtaatcaggaagttcttcatcaacataagctcctaattcttgtaatttccccttaatggcactccggatcttgcggctgatctcggtgccgatctccatggctctgcggcgtgcgggaactcagcactgcgcggcgcttggcttacccggaggctgccgcggactcctaccccgcagccgggacaccaccgcctcc

SEQ ID NO: 17451 - RNA, 13982 nt, Homo sapiens
  source 1..13982: mol_type = other RNA
tcaggccaggcacagtggctcatacctggaatcccagcactttgggaggccgaggcaggcagatcacctgaggtcaaggtatttgagaccagcctggccaacatggtgaaaccccatctctactaaaaatacagaaattagctgggtgtggtggtgcacacctgtaatgctagctactcgggaggctgaggtaggagaatcgcttgaacctgggaggcagaggttgcaataagcctagatcatgccactgcactcaagcctgggagacagagcgagactacatcttaaaaaaaaaaaaaaaagtattatgagagaggataatgtattgtaatgtattgtagaggctaaataaaattatgctcatgtcagaaaaaaagagtatttctcaaaataaaattcactgaaactggatgtttattttgactgagatatagtatatcctcaaattgccatagaaagtttacaagaatattagaggtaaattataaatatcagggcctttttaaaaaaaaaagattctgcttataacttggtatttgtttataataaaaattatagtagccaataatgaacacttactctggcttggttatttacttaggtcaaaagaaggaggagcggttaaactgtgggatcaggaactgaggcggtgccgtgccttcaggcttgagacaggacaagccacagattgtgttcgttctgtgtgcagaggcaaagtaagatgttccatgagctgatacagtgcagcagaaaacagaaagtggttattactgtgattccctcaccctttgcagcctaatgaacaatacttaataatgcataacgatggatttgcttgccaacattactctgtctttgctgctttctttgccaaagttagcaccagtgtggtgcataagctaggaagctattctgtctaaatactgtatgtaaacctccaatattttctagaatctgccaatttaacaactctagtagacataattgaaagcccttggcagttgactcatattaggacagctgtctccattttttaaaaaaacacacattccctagataaaacgtgcagtaaacaaacaatgaaatactactcagccataaaaaataatgaaattctgtcattcttggtggcaacatggatgagactggaggacatgatgtgaagtgaaataagccaggcacagaaagataaatacatgttctcactcctgtgcagaaactaaaaaagttgatcccacagaggtggagagtagaatagtggttactggaggcggacaagggggagggggagggggatagggaaggactggttaaaggatacaagtttacacagccagataggaatagtatgttttagtattctgtagtactgtaggatgactatagttaagaatcacgtatttatgtattttcaggtatttacaagagaggattttgaaagtttccatcacaaagaaatgataaatgtctgaggtgatggttatgcgtattaccctatgccctatagatatgtataattatgtgtcaatttcaaaataaaaattcaaaactacaactcctatgaaaatttttgagcgtgtttgtacttattaagtgtatttataaatcatacggatattatcttcagcctgcatattaaattgtagttaagcttttactttttaactaaaaaataaattctattattttttcctatatcccactgcactgaccccagtttggaaatcctaagattatcaaataaaaactttgattattgaagaatccaggtgtactgccacagaaaagttctattctgtagcatggactctaatatgtaatctagcccattgtgcttacagatagatgtgtgcctgtagtcatagaaaaatttgcatgagctaatgactgccttgctactagattagctcaaagcaaaaagttctctgaaagcaggtcaatagggtcatttttatattatgaagaagaaaagcagctgttgtattacattcactgtattggtcctgcttgtgtttcagggcaagatccttgttgggacaaggaatgctgaaataatcgaagttggagagaaaaatgcagcttgtaatattttagttaacggtcatgtggatgggccaatctggggactagcaacacatccttccagggattttttcctttctgctgcagaagatgggacagtgagactttgggatattgctgataaagtaagtacagataatttttttaaaagaggttacaacttctaaaaagaaaagttggaagttctaaattgctagtacttaaagaactgccagaattctgttgagcattttgaggggaaactggtataatttagaagtacttcacttaatgtttcctatgactctttttttttttttttttaaatgcagaagatgttaaacaaagtgaatttgggacatgctgctcgtactgtgtgttacagccctgaaggggacatggtggctattggaatgaaaaatggagaatttatcattttactagtgagttctctaaaaatatggggaaagaagagagacaggagatgtgcaatccatgatatcaggttagtgaacaaatggaatagagtttctagtatatacttgatttaacttccatttgtaaaattttccatagccttgccttcaaaaagaggtccccagggcctgtagcatttcccgtattataaattgtatgctaaaatatggctgtttgtatactacttaattcttcttgctaaattataaacccactgggcaccaactataatagcaagtactagtaggtaatgtttgatgaattcatgttaacacttagccatgtccattaagttcatcccaccaagaggtatctcccactgtaatacaagagagctatctgcccttcaaaagttgtcaccctggaaaactaaagttgtgatttcaaacatatcttctcttagtaacctcagtttgggaatatgtagttcattaatttaatcaatacctattgattaaatgttccagaatccaaattaatttaaatgtttcttaaacctttgtttttcagtgcttaagcatttttcaacagtggctaccatttacggagtacttccgtgtgatcagtagataagattattgaatctaggtctgtcaaaagcttgtacacttttcatcagtaaaatccttttacaaatgaaaccttcctcagaacttcaatatataaaatagtaacagtggcttcccttagcttttacatgtctctatcgtacctcagtaagactcatgggccatttcaagagactgaattgtcccatatgactccaaagattgctaggcaaatagcatttcactttgtcttttaaataagttcttcaggccgggcgcggtggctcatgcctgtaatcccagcactttgggaggccgaggcaggcagatcacctgaagtcaggagtactcgaccagcctggccaacatagtgaaaccccatctcaactaaaaatacaaaaatcagccgggcgtggtggcaggcgcctgtaatcccagctactcagggggctgaaacaggagaatcgcttgaacccgggaggcggaggttgcgccatcgcactccagcctgggagacaagagcgagacttcgtctcaaaaaaaaaaaattcttcttccaagattcaagttgtgtcatttcaccttaataactggaggttagttaagctgggctgtgttctttgcttaatattaagacaacgttttttccagatggaagaaaactatcttaatgaattgttagcttattaattatgtaatgctaatggcttttaaaagctgagatgttctgactgggtgttgtggctcacacctgtaatcccagtaccttgggaggccaagggggaaggattgcttgaggccaggagtttgggaccatagtgagaccccgcctctatttaaaaaattaaattttgttttgttttgttttgagttggagttttgctcttgttgcccatgctgaagtgcaatggtgcaatctcagctcaccacaacctgtgcctcctgggttcaagcgattctcctgcttcagcctcccgagtagatgggattacaggcgtgcaccaccatgcctggctaattttgtatttttagtagagacagggtttctctatgttggtcaggctggtctcaaactctcgacctcaggtgatctgcccgcctccgcttcccaaagttctgggattataggtgtgagccactgggcctggcctaagaaagtttttttaagccattagacgtttttaaaggaattgggagatgacaattggggaaatatttaaaatttaagtaaaatataaagcttccttatttcatgtaacccagacaatctcagtatacatgatcagttgtgtctgacaggtaaatctatttgaggccttatcacacgttacttttaagaactagaaaggaaaagtcactgatcttaagtatttataatacttcatgtggtctaatactttttacgttttgttttgattcagatttagtccggattcccggtatctggcagtaggttctagtgagaactcagtggatttttatgacctaacgctgggccccactcttaacagaatcagctactgcaaagacattccaagctttgtcattcaaatggacttctctgcagatagcagttatctccaggtacagtaccaatactgtatacccaggtggcaagttcttctgcttttacatttcgtgttagtgaatgcatttaaagttcctgagctccagagctccagcttctcaactcctccctttgtaccttctgacctacagctcccctttcctcccccacttatcagagcttttctcctattaagtttttgtagtgatcttttgcatacttaataatgttagacatgtaaatcaagtagcaatatgctagtattctgtaaaccccctgtggattttgtctctcacctaatggaattcttgtcccattttaatctgatgaaaaaggtctctagtggctgctataaacggcatgtctatgaagtgccttcaggaaaacatcttatggatcatgccgctattgacagaattacttgggctacatggactaggtaaatacttatatattcacaaggcaagaactgactttgaaggccagttagaaaatcctatttctgaactgttagagccattccaataaggaatagtaattgagtttcaagtttttgttaccatattttgaaatggtatgttcatgttgggacccctttttattgaatatatttccatgttttatcagtttccatgatttatcaagttttttttttaaggaaatcaaagttttaactttaaagataccctgatatttttcttaatgctaaatttaatgactggcaaaaaggtattgggtgctgttaagcaactgttattaattctctatctaaaggaatgctatcttgaatctattagaagtcaaagcttccaaatttgttcaaatttcctggctgtatgacaggtaaccatgactatccatttttttggccaatgaaaaatgccatcaaattcctgtatcagccaggcatatagtggctcatgcctgtaatctctgatgtagcaggccgaggtgggaggatcacttgagcctagaagttttgataccagcctgggcaacatagcaagaccccatctctgaaatttttttaattcctatgtcataagtcatttttatttttgtagagatagggatctcacaatattgcccaggctggtctcaaactcttggcctcaagcagtcctcctgcctcagcctcccaaaatgttgggattactggtatgtgctgctggacccagccaagtagcacttttaatttgaaaaatagttctatcagttttcagtcaggcgcggtggctcagcctgtaatcccagcactttgggaggccgagcgggggtgatcacctgaggtcgggagttcgagactagcctgaccaacatggagaaaccctgtctctactaaaaatacaaaataagccgggcatgttagcgcatgcctgtgatcccagctactcgggaggctgaggcaggagaattgcttgaacccaggaggcagaggttgcggtgagccgagatcatgccattgcactccagcctgggtaacaagagcgaaaactccgtctcaaaaaaaaaaaaagaaaaaatagttctatcagttttcataaagtactactttaatcttaaaaagattaatctagaaacccttcaaattataaaatgtcatttttaaaaggcaggagttgatatcctgatgaaattcaggtctccaaacaacttaccataatttacttcctgtattttaagtaacatgatagggtacttagagattaattgccaagaaactttttgaatatagtcaacctgcccgcacttgccatgatgagttttcttttgttccttccctctagtattctaggagatgaggttttgggaatctggtccagacatgctgagaaagctgatgtcaactgtgcctgtgtatctcattcaggaatcagtcttgttacaggagatgactttggcatggttaagttatttgacttcccatgtccagaaaaatttgtaagtttgtgttttgtttactattatcagtttactcctaattttgatgtcttatcatcagcacttttccccatatatttaaaatgttttgtcctaatttctaaatttttccccaaactttctaaatctatttactttgaaataaaagctattagaaacaaatcctctccctcgagtaataccatctttggaaccatcctacaaaagctgtaattagcttttcaccaaacctataatcagttatcaaatttcaaatgcttttccttagagaaaaatggtcagagtacctggagacatctgactgcccacacagcctggttttgcagatccactactcatgctgaaaagcattctaatcactggctgcggtgctaactccctactctctccacagctcttgtcatagagattatagttcctaataagagcctttgacttctgtgtgcaccaaatgccctgagcttgtctgtcattgttttttaggcaaaacacaaaaggttcttgggtcattcgccccatgtgacaaatattcgatttaccagtggtgatcgacatgttgttagtgctggaggtgatgactgcaggttagtaactttctcagcccatgaagagcagactatgttactagttaagagacttaatacaacaactcctacagctttggtttatgaaatcagctagtcaacattagtagaaggtagtataaccagatggctcttcagaatctcatatttatgcaaatacagaataaaaggagttaaagaggaaaaatattacacatgtaacctgaaagcacaactgaaaaatattaaactgttatgaaaatctaaaaacataattaactccctgcaattttcttctctgattgcagcttatttgtctggaaatgtgtacatacacctcactgagagatgctgagatgactacagaaattaactttgagaccagaattacagagaagaaaaaccaaaacccaaccctgcatggtcaagtggtgctaacccaagactgtaacagggagaaatgcccagaatcatcaaaatagtgaaagactgatctgttcaaaatatttgctatatgcactgggtataatccgtaatccatacactgccagataatgccatttcaaggaaggatcgaatacttgatggtaaaggccaagtccccctgtattgggaagtgtgtgatttcggcagacctgctgggaaaatttagggtagagcactctttacagaagaactcaaaaacccaatttggataattttcattatctttttagcaaaatggtttcttaatgtttatattttattttcaaggttcattgtttaatgaaatattttattcttgcatttccataaggaaagggaaagtcatgatcatcctaaaggatcacagtttttaaaaggcaaacattttccctaaggaaacagacacaagctttcctagagaatatgatgttttttaggcattaataaggtccttttttataaaggacacttttctcctagtagttttgaattcaggaacagatccaaagttagcagtatatggctgctacatttccattttcattttcgagccatcagtttatgttcagatgccatctctgtaatcgcacatttaaaacataactgtagcctcactaatggaaaagtagtatgatgaacaatcattcccaatggtgtacaatgtaagggttttagggagcaacagtatttaactggaagaaagaattgcatatttaatgtagtctaatatatacacatttgtttaacatgtaaacaaaagtgttaaattcacatatacaacattatacaatttaatcactcttggaataaaatttttatagccttttttctattgggaaaatttgtttagatgtgtgccactccataggtttatttccaaaatgaatgagcccaactccatttgtaaaaacttgtcagttagaattcctttttttagtggattagggctgaattcttagatccttatttcttttcactttaaatgctgccaaagatcactactcatcattcaggaattcgctgtctagcctatctgtagtttcctgaagattgaaaattatgtagactgctatttaaaaatatatttttctaagtgtgaggtttaagatgctgtattgaccctatgagtttttaatgtgttaattatctttatagcataatagatcgctttaggttcctggaatcccatttggtctgacaggatatatgaagattcttaatacctattttctgtgtctaatacttggttaatactaaaaatagaaatgactaaattacatcacagaaagcataaccagtgattgaacctggtagttttaaagctctaaatagctgtggctgaaggactgattatggggctaagaagcttgaaacgtaagttggtacttgttcatcagtggattctcctaaattaagccaaattttgaaatacatgactattaagtttctactcatgtatttacagtcagtcaataaattaaaggaggaaaaaaatccctgaacaacctgcccataaaaagaaaaatactctacatttgagcctgctgcagttttaaattttccctctgggtcaagtttgccagcttttggctacagagaaattatatttccattacagtgcaggtagaaactctgtaaccttaagcatgtaaactacatagaataaaactgtttccactgcatttctgtccttcaaagtggccaacctgattaagtcagccttaatcactgctgctgtcagtttcacgactaaaggtcatattgactaagtagtcatcagctgaccacctcgctgtatcagccagcaacgaggggaaggtgaagaaacatgataggccatatagaatctgccctatgtttacttttttaacccagataattatttttgtgtgcagtatctaagctcctgattgtgtaacctgggacttctggcaccttttgttccattcattttatgtataaaatgcatgccaaagcacactgtgccctctggtacccttgcttccaatcgccaaccatgctcatttccttcctttttttgtggtccctttttgtggtgatcattttaaaccacgtcatccaacaaatgttttatggtcaaccttagcttgttcataagccatagcaactgaaagattaaactcttaaatatgtgtctgggcagtggctattaaatagcaaaaaacaatcagattttagtattttattatttccttgtaaaatggctgaactaaattaaacccttgtttcccatttgttctataatttatagtgaaactgagaacaaaactatctttataaatgatagctaaaagtatttccagatatttaaacaatttaaaataaatttcttctgcagagatgcaaagcatctcaacactggaatgaacaaatgccttaaattcaatggagtaaacctttagaatgaagaggaactgtcatttcacccaagccgaagacaacagccttatgcacttgtgtgctctgtctttgctgcttctcgtgtttcaagcctttcctgtgggatcagcacagcaaagtgcaacttaccaaatggtttaatgactggttaattctttcttctcccaatggaaaagcaatggcaacacaacagtagactgctggcttgacaatcttaaacgtgagcctttgcacatgtaggtttatcatcatttgagtatacgactaagcaagtcaatgaactttttttttttttttagcagtttaatttggtcctgagaatgttgcagtctttattaccccttttgcattaatccacttttctaaccaccttttaagctttaatttttaacactatacaccaagtctttgaaatcagtgatctgttatttaactctaaagcatttgacacttcttgccttaacagttttaaaaaccacacacaaaaaaactctgtaagtaatacagtaggccaaaagtttcatcctatctatcttgcagtttacctatctgatctgatctctgtaattatagttctgtcatttaaaatatactatttaaatctaatttttacatttcaaaaattatcttcagtagtaactaagtatattttctgtggattctgagaatgttatttttcagaatgtgagaatatatatgtacatttataatcttgtgactttaaagtctgttttcagatacagtatgtaaatacttgtaaaaaaatttgtataattttgtgataatgtagtttcccaaaaaaattatttagaaggcattatgttattagtaaatgagagcactgtatagaactgttcctattttctgcacttgccattccagctgcctccactgtccatacccacctcattcatcctgtcacagaaggcaggaaaactgggaactttaccaaagtagcactcagcctgagaggcctgtataatcatgcttttcaaactaaattcacttaaaaattaaaaagcagaattgaatattttaagcagcctcagtacctttggccaatgctgttttcatggtggattatgaacattatataatctttgggaaaagtgaaagtagtacaatttttagaataatgacaactgcctcactgcatctctccactcacacagcaaccgtgtagccccctaagctgcagtaccatgactaaccatgatgtcaatttcatatgctgatcctcacaacagcagtgcacaaacatgccccaaatattttaacagaatttagctcttccttaagctgtcttttcatagtaaaaacaaaacaaaaacacccaatgttaaaaccacataataaacttacaaacttgaaaaattagacacttcagatagataggcaataaaacttcatattatgaaagcaatatattccaagtttcaaagatttgacaagttctgtagagtatctttcatcagtacatgaaaacttccaaactgcatgatcttctgccaggcaggactgggtgctattcgctggtttgaggtcgaatccatttcaaggcatgtcgtggtgggacattaatggtgggatggtagaatgtgcagtccggtcttgtacattgagtgttaaacctacaatgttttggatgatagaagggacattccatcttcttacaagcagggaagtaacggcagagctgactactggaaggtggtgctggtggtgcaactgctggttttggagacagtactggaattcttctactcacatgagtgaagggacaatctggtttagtacactttgcatcatatttacaatttgggtgaacaaacaaacatttttcagcaaatttacaattggggaaggctttgcagggtgagatggggtgatggtaggcacactcatccccatttttacaagcaggccagtacttgcagcgctccaaaagtttttctggtttctgtgccacactcagttcactcatctcagcgttagaaaagctaccatttgggtcctcaagctgcctgctcagcaagtgcaactgctgtgggtggaggagacctctgagtcccttgtttgaggctgcagtttggtttacgggtttcattccttcaaagcacatgtcctcctcttgatctgacatgtatcctggggggctggggacaccatccagcgtcactataaacttgggacttgcaggtttatctggttgtacaagatctcgtgtctgcataaggtgtcctgaaagtacccgaagggaatctgcagtcttcatccccgactcttggtttggtgccactactacttcctcagacagctttggcttcttcagaataaatgatcttgtgtctgcatggaccatggattccatgtcatagtaatcttgatttttttctacagaatctccttttgtttcctcttctttaatggggggacttattctgggggtcctactttgtccctggaccacttctgctagcaattcttcttgagaagttcgagttctgggagcaactggaagtgtctgtttctgtggaactgtagagtagttagttgtttttgttacggattcttgagcttcagatatagccttcaaaatcagattcttgttagcttgtttagaaggtggaagagaaggtctcctttcaggctttgcaggcacagacacactgctggagatgcttcctgttcgagacccgtaatcatcatcttcttcctcctcttctccatcatgattgaatttttttactttaacaactgaacttaccacaggcaactttctcttccgaaagttttcatcctccatactcattttctccgagttgtttctaaagaacggactatacgtttcttctaagctgttaagcacctctggttcacacaaacgtcctgtttcatatacccaactactctgcatatcaagctgcttggcagcatgaatactattctgctgctgttgaaattgcaacctgtttaaatgaacaccactatctgcatttctacttgcaggtggtcgataaatttcaatagaagggcgagaagaaccatatgtaagtgtcactgtaggttttttctgagataagggattctcctgcacaaagttgaggtcttcgtcaatgagatcatctggttctggcttaatatcaatcacatcttcagagggtgctggctccctcaaaggtttcactgttgacattagtcgggttgcagctccatcatcgtaagtctgtctgacatttgtggtttttgactcctgcgaacttgtagaaactctggaatctcttttttcaggtctcgcgctaggaatggcaagtggtggcactgcagcttcatgcctcctctcatctccccgactgaaattgctcttgtttgaaggcacgttactatcaaagatgttggtatcagaagacttcagactagagggttcagttgtaacagagcgaagtttatctaatacaccatgaagccatacggtgaatcgaattgtgttgttccctagaaacagggacagatcctctgtcatttggtcctgacttttcttgttggccaccatcaccataatgtaatcaggaagttcttcatctatttaaaaggaaaggtagatcaaaactttgtttcctcaaaactttcttcttaaagttgatgtgcttgaaaatatagatgtagctctaagctttagagtcgcagagctctactggaattacattggacaagatggcttagctttaatttttttctcttcattccacaggtatttcaaatacaacataagctcctaattcttgtaatttccccttaatggcactccggatcttgcggctgatctcggtgccgatctccatggctctgcggcgtgcgggaactcagcactgcgcggcgcttggcttacccggaggctgccgcggactcctaccccgcagccgggacaccaccgcctcc

SEQ ID NO: 17452 - RNA, 13716 nt, Homo sapiens
  source 1..13716: mol_type = other RNA
tcaggccaggcacagtggctcatacctggaatcccagcactttgggaggccgaggcaggcagatcacctgaggtcaaggtatttgagaccagcctggccaacatggtgaaaccccatctctactaaaaatacagaaattagctgggtgtggtggtgcacacctgtaatgctagctactcgggaggctgaggtaggagaatcgcttgaacctgggaggcagaggttgcaataagcctagatcatgccactgcactcaagcctgggagacagagcgagactacatcttaaaaaaaaaaaaaaaagtattatgagagaggataatgtattgtaatgtattgtagaggctaaataaaattatgctcatgtcagaaaaaaagagtatttctcaaaataaaattcactgaaactggatgtttattttgactgagatatagtatatcctcaaattgccatagaaagtttacaagaatattagaggtaaattataaatatcagggcctttttaaaaaaaaaagattctgcttataacttggtatttgtttataataaaaattatagtagccaataatgaacacttactctggcttggttatttacttaggtcaaaagaaggaggagcggttaaactgtgggatcaggaactgaggcggtgccgtgccttcaggcttgagacaggacaagccacagattgtgttcgttctgtgtgcagaggcaaagtaagatgttccatgagctgatacagtgcagcagaaaacagaaagtggttattactgtgattccctcaccctttgcagcctaatgaacaatacttaataatgcataacgatggatttgcttgccaacattactctgtctttgctgctttctttgccaaagttagcaccagtgtggtgcataagctaggaagctattctgtctaaatactgtatgtaaacctccaatattttctagaatctgccaatttaacaactctagtagacataattgaaagcccttggcagttgactcatattaggacagctgtctccattttttaaaaaaacacacattccctagataaaacgtgcagtaaacaaacaatgaaatactactcagccataaaaaataatgaaattctgtcattcttggtggcaacatggatgagactggaggacatgatgtgaagtgaaataagccaggcacagaaagataaatacatgttctcactcctgtgcagaaactaaaaaagttgatcccacagaggtggagagtagaatagtggttactggaggcggacaagggggagggggagggggatagggaaggactggttaaaggatacaagtttacacagccagataggaatagtatgttttagtattctgtagtactgtaggatgactatagttaagaatcacgtatttatgtattttcaggtatttacaagagaggattttgaaagtttccatcacaaagaaatgataaatgtctgaggtgatggttatgcgtattaccctatgccctatagatatgtataattatgtgtcaatttcaaaataaaaattcaaaactacaactcctatgaaaatttttgagcgtgtttgtacttattaagtgtatttataaatcatacggatattatcttcagcctgcatattaaattgtagttaagcttttactttttaactaaaaaataaattctattattttttcctatatcccactgcactgaccccagtttggaaatcctaagattatcaaataaaaactttgattattgaagaatccaggtgtactgccacagaaaagttctattctgtagcatggactctaatatgtaatctagcccattgtgcttacagatagatgtgtgcctgtagtcatagaaaaatttgcatgagctaatgactgccttgctactagattagctcaaagcaaaaagttctctgaaagcaggtcaatagggtcatttttatattatgaagaagaaaagcagctgttgtattacattcactgtattggtcctgcttgtgtttcagggcaagatccttgttgggacaaggaatgctgaaataatcgaagttggagagaaaaatgcagcttgtaatattttagttaacggtcatgtggatgggccaatctggggactagcaacacatccttccagggattttttcctttctgctgcagaagatgggacagtgagactttgggatattgctgataaagtaagtacagataatttttttaaaagaggttacaacttctaaaaagaaaagttggaagttctaaattgctagtacttaaagaactgccagaattctgttgagcattttgaggggaaactggtataatttagaagtacttcacttaatgtttcctatgactctttttttttttttttttaaatgcagaagatgttaaacaaagtgaatttgggacatgctgctcgtactgtgtgttacagccctgaaggggacatggtggctattggaatgaaaaatggagaatttatcattttactagtgagttctctaaaaatatggggaaagaagagagacaggagatgtgcaatccatgatatcaggttagtgaacaaatggaatagagtttctagtatatacttgatttaacttccatttgtaaaattttccatagccttgccttcaaaaagaggtccccagggcctgtagcatttcccgtattataaattgtatgctaaaatatggctgtttgtatactacttaattcttcttgctaaattataaacccactgggcaccaactataatagcaagtactagtaggtaatgtttgatgaattcatgttaacacttagccatgtccattaagttcatcccaccaagaggtatctcccactgtaatacaagagagctatctgcccttcaaaagttgtcaccctggaaaactaaagttgtgatttcaaacatatcttctcttagtaacctcagtttgggaatatgtagttcattaatttaatcaatacctattgattaaatgttccagaatccaaattaatttaaatgtttcttaaacctttgtttttcagtgcttaagcatttttcaacagtggctaccatttacggagtacttccgtgtgatcagtagataagattattgaatctaggtctgtcaaaagcttgtacacttttcatcagtaaaatccttttacaaatgaaaccttcctcagaacttcaatatataaaatagtaacagtggcttcccttagcttttacatgtctctatcgtacctcagtaagactcatgggccatttcaagagactgaattgtcccatatgactccaaagattgctaggcaaatagcatttcactttgtcttttaaataagttcttcaggccgggcgcggtggctcatgcctgtaatcccagcactttgggaggccgaggcaggcagatcacctgaagtcaggagtactcgaccagcctggccaacatagtgaaaccccatctcaactaaaaatacaaaaatcagccgggcgtggtggcaggcgcctgtaatcccagctactcagggggctgaaacaggagaatcgcttgaacccgggaggcggaggttgcgccatcgcactccagcctgggagacaagagcgagacttcgtctcaaaaaaaaaaaattcttcttccaagattcaagttgtgtcatttcaccttaataactggaggttagttaagctgggctgtgttctttgcttaatattaagacaacgttttttccagatggaagaaaactatcttaatgaattgttagcttattaattatgtaatgctaatggcttttaaaagctgagatgttctgactgggtgttgtggctcacacctgtaatcccagtaccttgggaggccaagggggaaggattgcttgaggccaggagtttgggaccatagtgagaccccgcctctatttaaaaaattaaattttgttttgttttgttttgagttggagttttgctcttgttgcccatgctgaagtgcaatggtgcaatctcagctcaccacaacctgtgcctcctgggttcaagcgattctcctgcttcagcctcccgagtagatgggattacaggcgtgcaccaccatgcctggctaattttgtatttttagtagagacagggtttctctatgttggtcaggctggtctcaaactctcgacctcaggtgatctgcccgcctccgcttcccaaagttctgggattataggtgtgagccactgggcctggcctaagaaagtttttttaagccattagacgtttttaaaggaattgggagatgacaattggggaaatatttaaaatttaagtaaaatataaagcttccttatttcatgtaacccagacaatctcagtatacatgatcagttgtgtctgacaggtaaatctatttgaggccttatcacacgttacttttaagaactagaaaggaaaagtcactgatcttaagtatttataatacttcatgtggtctaatactttttacgttttgttttgattcagatttagtccggattcccggtatctggcagtaggttctagtgagaactcagtggatttttatgacctaacgctgggccccactcttaacagaatcagctactgcaaagacattccaagctttgtcattcaaatggacttctctgcagatagcagttatctccaggtacagtaccaatactgtatacccaggtggcaagttcttctgcttttacatttcgtgttagtgaatgcatttaaagttcctgagctccagagctccagcttctcaactcctccctttgtaccttctgacctacagctcccctttcctcccccacttatcagagcttttctcctattaagtttttgtagtgatcttttgcatacttaataatgttagacatgtaaatcaagtagcaatatgctagtattctgtaaaccccctgtggattttgtctctcacctaatggaattcttgtcccattttaatctgatgaaaaaggtctctagtggctgctataaacggcatgtctatgaagtgccttcaggaaaacatcttatggatcatgccgctattgacagaattacttgggctacatggactaggtaaatacttatatattcacaaggcaagaactgactttgaaggccagttagaaaatcctatttctgaactgttagagccattccaataaggaatagtaattgagtttcaagtttttgttaccatattttgaaatggtatgttcatgttgggacccctttttattgaatatatttccatgttttatcagtttccatgatttatcaagttttttttttaaggaaatcaaagttttaactttaaagataccctgatatttttcttaatgctaaatttaatgactggcaaaaaggtattgggtgctgttaagcaactgttattaattctctatctaaaggaatgctatcttgaatctattagaagtcaaagcttccaaatttgttcaaatttcctggctgtatgacaggtaaccatgactatccatttttttggccaatgaaaaatgccatcaaattcctgtatcagccaggcatatagtggctcatgcctgtaatctctgatgtagcaggccgaggtgggaggatcacttgagcctagaagttttgataccagcctgggcaacatagcaagaccccatctctgaaatttttttaattcctatgtcataagtcatttttatttttgtagagatagggatctcacaatattgcccaggctggtctcaaactcttggcctcaagcagtcctcctgcctcagcctcccaaaatgttgggattactggtatgtgctgctggacccagccaagtagcacttttaatttgaaaaatagttctatcagttttcagtcaggcgcggtggctcagcctgtaatcccagcactttgggaggccgagcgggggtgatcacctgaggtcgggagttcgagactagcctgaccaacatggagaaaccctgtctctactaaaaatacaaaataagccgggcatgttagcgcatgcctgtgatcccagctactcgggaggctgaggcaggagaattgcttgaacccaggaggcagaggttgcggtgagccgagatcatgccattgcactccagcctgggtaacaagagcgaaaactccgtctcaaaaaaaaaaaaagaaaaaatagttctatcagttttcataaagtactactttaatcttaaaaagattaatctagaaacccttcaaattataaaatgtcatttttaaaaggcaggagttgatatcctgatgaaattcaggtctccaaacaacttaccataatttacttcctgtattttaagtaacatgatagggtacttagagattaattgccaagaaactttttgaatatagtcaacctgcccgcacttgccatgatgagttttcttttgttccttccctctagtattctaggagatgaggttttgggaatctggtccagacatgctgagaaagctgatgtcaactgtgcctgtgtatctcattcaggaatcagtcttgttacaggagatgactttggcatggttaagttatttgacttcccatgtccagaaaaatttgtaagtttgtgttttgtttactattatcagtttactcctaattttgatgtcttatcatcagcacttttccccatatatttaaaatgttttgtcctaatttctaaatttttccccaaactttctaaatctatttactttgaaataaaagctattagaaacaaatcctctccctcgagtaataccatctttggaaccatcctacaaaagctgtaattagcttttcaccaaacctataatcagttatcaaatttcaaatgcttttccttagagaaaaatggtcagagtacctggagacatctgactgcccacacagcctggttttgcagatccactactcatgctgaaaagcattctaatcactggctgcggtgctaactccctactctctccacagctcttgtcatagagattatagttcctaataagagcctttgacttctgtgtgcaccaaatgccctgagcttgtctgtcattgttttttaggcaaaacacaaaaggttcttgggtcattcgccccatgtgacaaatattcgatttaccagtggtgatcgacatgttgttagtgctggaggtgatgactgcaggttagtaactttctcagcccatgaagagcagactatgttactagttaagagacttaatacaacaactcctacagctttggtttatgaaatcagctagtcaacattagtagaaggtagtataaccagatggctcttcagaatctcatatttatgcaaatacagaataaaaggagttaaagaggaaaaatattacacatgtaacctgaaagcacaactgaaaaatattaaactgttatgaaaatctaaaaacataattaactccctgcaattttcttctctgattgcagcttatttgtctggaaatgtgtacatacacctcactgagagatgctgagatgactacagaaattaactttgagaccagaattacagagaagaaaaaccaaaacccaaccctgcatggtcaagtggtgctaacccaagactgtaacagggagaaatgcccagaatcatcaaaatagtgaaagactgatctgttcaaaatatttgctatatgcactgggtataatccgtaatccatacactgccagataatgccatttcaaggaaggatcgaatacttgatggtaaaggccaagtccccctgtattgggaagtgtgtgatttcggcagacctgctgggaaaatttagggtagagcactctttacagaagaactcaaaaacccaatttggataattttcattatctttttagcaaaatggtttcttaatgtttatattttattttcaaggttcattgtttaatgaaatattttattcttgcatttccataaggaaagggaaagtcatgatcatcctaaaggatcacagtttttaaaaggcaaacattttccctaaggaaacagacacaagctttcctagagaatatgatgttttttaggcattaataaggtccttttttataaaggacacttttctcctagtagttttgaattcaggaacagatccaaagttagcagtatatggctgctacatttccattttcattttcgagccatcagtttatgttcagatgccatctctgtaatcgcacatttaaaacataactgtagcctcactaatggaaaagtagtatgatgaacaatcattcccaatggtgtacaatgtaagggttttagggagcaacagtatttaactggaagaaagaattgcatatttaatgtagtctaatatatacacatttgtttaacatgtaaacaaaagtgttaaattcacatatacaacattatacaatttaatcactcttggaataaaatttttatagccttttttctattgggaaaatttgtttagatgtgtgccactccataggtttatttccaaaatgaatgagcccaactccatttgtaaaaacttgtcagttagaattcctttttttagtggattagggctgaattcttagatccttatttcttttcactttaaatgctgccaaagatcactactcatcattcaggaattcgctgtctagcctatctgtagtttcctgaagattgaaaattatgtagactgctatttaaaaatatatttttctaagtgtgaggtttaagatgctgtattgaccctatgagtttttaatgtgttaattatctttatagcataatagatcgctttaggttcctggaatcccatttggtctgacaggatatatgaagattcttaatacctattttctgtgtctaatacttggttaatactaaaaatagaaatgactaaattacatcacagaaagcataaccagtgattgaacctggtagttttaaagctctaaatagctgtggctgaaggactgattatggggctaagaagcttgaaacgtaagttggtacttgttcatcagtggattctcctaaattaagccaaattttgaaatacatgactattaagtttctactcatgtatttacagtcagtcaataaattaaaggaggaaaaaaatccctgaacaacctgcccataaaaagaaaaatactctacatttgagcctgctgcagttttaaattttccctctgggtcaagtttgccagcttttggctacagagaaattatatttccattacagtgcaggtagaaactctgtaaccttaagcatgtaaactacatagaataaaactgtttccactgcatttctgtccttcaaagtggccaacctgattaagtcagccttaatcactgctgctgtcagtttcacgactaaaggtcatattgactaagtagtcatcagctgaccacctcgctgtatcagccagcaacgaggggaaggtgaagaaacatgataggccatatagaatctgccctatgtttacttttttaacccagataattatttttgtgtgcagtatctaagctcctgattgtgtaacctgggacttctggcaccttttgttccattcattttatgtataaaatgcatgccaaagcacactgtgccctctggtacccttgcttccaatcgccaaccatgctcatttccttcctttttttgtggtccctttttgtggtgatcattttaaaccacgtcatccaacaaatgttttatggtcaaccttagcttgttcataagccatagcaactgaaagattaaactcttaaatatgtgtctgggcagtggctattaaatagcaaaaaacaatcagattttagtattttattatttccttgtaaaatggctgaactaaattaaacccttgtttcccatttgttctataatttatagtgaaactgagaacaaaactatctttataaatgatagctaaaagtatttccagatatttaaacaatttaaaataaatttcttctgcagagatgcaaagcatctcaacactggaatgaacaaatgccttaaattcaatggagtaaacctttagaatgaagaggaactgtcatttcacccaagccgaagacaacagccttatgcacttgtgtgctctgtctttgctgcttctcgtgtttcaagcctttcctgtgggatcagcacagcaaagtgcaacttaccaaatggtttaatgactggttaattctttcttctcccaatggaaaagcaatggcaacacaacagtagactgctggcttgacaatcttaaacgtgagcctttgcacatgtaggtttatcatcatttgagtatacgactaagcaagtcaatgaactttttttttttttttagcagtttaatttggtcctgagaatgttgcagtctttattaccccttttgcattaatccacttttctaaccaccttttaagctttaatttttaacactatacaccaagtctttgaaatcagtgatctgttatttaactctaaagcatttgacacttcttgccttaacagttttaaaaaccacacacaaaaaaactctgtaagtaatacagtaggccaaaagtttcatcctatctatcttgcagtttacctatctgatctgatctctgtaattatagttctgtcatttaaaatatactatttaaatctaatttttacatttcaaaaattatcttcagtagtaactaagtatattttctgtggattctgagaatgttatttttcagaatgtgagaatatatatgtacatttataatcttgtgactttaaagtctgttttcagatacagtatgtaaatacttgtaaaaaaatttgtataattttgtgataatgtagtttcccaaaaaaattatttagaaggcattatgttattagtaaatgagagcactgtatagaactgttcctattttctgcacttgccattccagctgcctccactgtccatacccacctcattcatcctgtcacagaaggcaggaaaactgggaactttaccaaagtagcactcagcctgagaggcctgtataatcatgcttttcaaactaaattcacttaaaaattaaaaagcagaattgaatattttaagcagcctcagtacctttggccaatgctgttttcatggtggattatgaacattatataatctttgggaaaagtgaaagtagtacaatttttagaataatgacaactgcctcactgcatctctccactcacacagcaaccgtgtagccccctaagctgcagtaccatgactaaccatgatgtcaatttcatatgctgatcctcacaacagcagtgcacaaacatgccccaaatattttaacagaatttagctcttccttaagctgtcttttcatagtaaaaacaaaacaaaaacacccaatgttaaaaccacataataaacttacaaacttgaaaaattagacacttcagatagataggcaataaaacttcatattatgaaagcaatatattccaagtttcaaagatttgacaagttctgtagagtatctttcatcagtacatgaaaacttccaaactgcatgatcttctgccaggcaggactgggtgctattcgctggtttgaggtcgaatccatttcaaggcatgtcgtggtgggacattaatggtgggatggtagaatgtgcagtccggtcttgtacattgagtgttaaacctacaatgttttggatgatagaagggacattccatcttcttacaagcagggaagtaacggcagagctgactactggaaggtggtgctggtggtgcaactgctggttttggagacagtactggaattcttctactcacatgagtgaagggacaatctggtttagtacactttgcatcatatttacaatttgggtgaacaaacaaacatttttcagcaaatttacaattggggaaggctttgcagggtgagatggggtgatggtaggcacactcatccccatttttacaagcaggccagtacttgcagcgctccaaaagtttttctggtttctgtgccacactcagttcactcatctcagcgttagaaaagctaccatttgggtcctcaagctgcctgctcagcaagtgcaactgctgtgggtggaggagacctctgagtcccttgtttgaggctgcagtttggtttacgggtttcattccttcaaagcacatgtcctcctcttgatctgacatgtatcctggggggctggggacaccatccagcgtcactataaacttgggacttgcaggtttatctggttgtacaagatctcttgactcatctgcagagtttctgccattactgggtcgatttgcagtcgggataataattgcctctgttgagttccttgatttttttctacagaatctccttttgtttcctcttctttaatggggggacttattctgggggtcctactttgtccctggaccacttctgctagcaattcttcttgagaagttcgagttctgggagcaactggaagtgtctgtttctgtggaactgtagagtagttagttgtttttgttacggattcttgagcttcagatatagccttcaaaatcagattcttgttagcttgtttagaaggtggaagagaaggtctcctttcaggctttgcaggcacagacacactgctggagatgcttcctgttcgagacccgtaatcatcatcttcttcctcctcttctccatcatgattgaatttttttactttaacaactgaacttaccacaggcaactttctcttccgaaagttttcatcctccatactcattttctccgagttgtttctaaagaacggactatacgtttcttctaagctgttaagcacctctggttcacacaaacgtcctgtttcatatacccaactactctgcatatcaagctgcttggcagcatgaatactattctgctgctgttgaaattgcaacctgtttaaatgaacaccactatctgcatttctacttgcaggtggtcgataaatttcaatagaagggcgagaagaaccatatgtaagtgtcactgtaggttttttctgagataagggattctcctgcacaaagttgaggtcttcgtcaatgagatcatctggttctggcttaatatcaatcacatcttcagagggtgctggctccctcaaaggtttcactgttgacattagtcgggttgcagctccatcatcgtaagtctgtctgacatttgtggtttttgactcctgcgaacttgtagaaactctggaatctcttttttcaggtctcgcgctaggaatggcaagtggtggcactgcagcttcatgcctcctctcatctccccgactgaaattgctcttgtttgaaggcacgttactatcaaagatgttggtatcagaagacttcagactagagggttcagttgtaacagagcgaagtttatctaatacaccatgaagccatacggtgaatcgaattgtgttgttccctagaaacagggacagatcctctgtcatttggtcctgacttttcttgttggccaccatcaccataatgtaatcaggaagttcttcatcaacataagctcctaattcttgtaatttccccttaatggcactccggatcttgcggctgatctcggtgccgatctccatggctctgcggcgtgcgggaactcagcactgcgcggcgcttggcttacccggaggctgccgcggactcctaccccgcagccgggacaccaccgcctcc

SEQ ID NO: 17453 - RNA, 13252 nt, Homo sapiens
  source 1..13252: mol_type = other RNA
tcaggccaggcacagtggctcatacctggaatcccagcactttgggaggccgaggcaggcagatcacctgaggtcaaggtatttgagaccagcctggccaacatggtgaaaccccatctctactaaaaatacagaaattagctgggtgtggtggtgcacacctgtaatgctagctactcgggaggctgaggtaggagaatcgcttgaacctgggaggcagaggttgcaataagcctagatcatgccactgcactcaagcctgggagacagagcgagactacatcttaaaaaaaaaaaaaaaagtattatgagagaggataatgtattgtaatgtattgtagaggctaaataaaattatgctcatgtcagaaaaaaagagtatttctcaaaataaaattcactgaaactggatgtttattttgactgagatatagtatatcctcaaattgccatagaaagtttacaagaatattagaggtaaattataaatatcagggcctttttaaaaaaaaaagattctgcttataacttggtatttgtttataataaaaattatagtagccaataatgaacacttactctggcttggttatttacttaggtcaaaagaaggaggagcggttaaactgtgggatcaggaactgaggcggtgccgtgccttcaggcttgagacaggacaagccacagattgtgttcgttctgtgtgcagaggcaaagtaagatgttccatgagctgatacagtgcagcagaaaacagaaagtggttattactgtgattccctcaccctttgcagcctaatgaacaatacttaataatgcataacgatggatttgcttgccaacattactctgtctttgctgctttctttgccaaagttagcaccagtgtggtgcataagctaggaagctattctgtctaaatactgtatgtaaacctccaatattttctagaatctgccaatttaacaactctagtagacataattgaaagcccttggcagttgactcatattaggacagctgtctccattttttaaaaaaacacacattccctagataaaacgtgcagtaaacaaacaatgaaatactactcagccataaaaaataatgaaattctgtcattcttggtggcaacatggatgagactggaggacatgatgtgaagtgaaataagccaggcacagaaagataaatacatgttctcactcctgtgcagaaactaaaaaagttgatcccacagaggtggagagtagaatagtggttactggaggcggacaagggggagggggagggggatagggaaggactggttaaaggatacaagtttacacagccagataggaatagtatgttttagtattctgtagtactgtaggatgactatagttaagaatcacgtatttatgtattttcaggtatttacaagagaggattttgaaagtttccatcacaaagaaatgataaatgtctgaggtgatggttatgcgtattaccctatgccctatagatatgtataattatgtgtcaatttcaaaataaaaattcaaaactacaactcctatgaaaatttttgagcgtgtttgtacttattaagtgtatttataaatcatacggatattatcttcagcctgcatattaaattgtagttaagcttttactttttaactaaaaaataaattctattattttttcctatatcccactgcactgaccccagtttggaaatcctaagattatcaaataaaaactttgattattgaagaatccaggtgtactgccacagaaaagttctattctgtagcatggactctaatatgtaatctagcccattgtgcttacagatagatgtgtgcctgtagtcatagaaaaatttgcatgagctaatgactgccttgctactagattagctcaaagcaaaaagttctctgaaagcaggtcaatagggtcatttttatattatgaagaagaaaagcagctgttgtattacattcactgtattggtcctgcttgtgtttcagggcaagatccttgttgggacaaggaatgctgaaataatcgaagttggagagaaaaatgcagcttgtaatattttagttaacggtcatgtggatgggccaatctggggactagcaacacatccttccagggattttttcctttctgctgcagaagatgggacagtgagactttgggatattgctgataaagtaagtacagataatttttttaaaagaggttacaacttctaaaaagaaaagttggaagttctaaattgctagtacttaaagaactgccagaattctgttgagcattttgaggggaaactggtataatttagaagtacttcacttaatgtttcctatgactctttttttttttttttttaaatgcagaagatgttaaacaaagtgaatttgggacatgctgctcgtactgtgtgttacagccctgaaggggacatggtggctattggaatgaaaaatggagaatttatcattttactagtgagttctctaaaaatatggggaaagaagagagacaggagatgtgcaatccatgatatcaggttagtgaacaaatggaatagagtttctagtatatacttgatttaacttccatttgtaaaattttccatagccttgccttcaaaaagaggtccccagggcctgtagcatttcccgtattataaattgtatgctaaaatatggctgtttgtatactacttaattcttcttgctaaattataaacccactgggcaccaactataatagcaagtactagtaggtaatgtttgatgaattcatgttaacacttagccatgtccattaagttcatcccaccaagaggtatctcccactgtaatacaagagagctatctgcccttcaaaagttgtcaccctggaaaactaaagttgtgatttcaaacatatcttctcttagtaacctcagtttgggaatatgtagttcattaatttaatcaatacctattgattaaatgttccagaatccaaattaatttaaatgtttcttaaacctttgtttttcagtgcttaagcatttttcaacagtggctaccatttacggagtacttccgtgtgatcagtagataagattattgaatctaggtctgtcaaaagcttgtacacttttcatcagtaaaatccttttacaaatgaaaccttcctcagaacttcaatatataaaatagtaacagtggcttcccttagcttttacatgtctctatcgtacctcagtaagactcatgggccatttcaagagactgaattgtcccatatgactccaaagattgctaggcaaatagcatttcactttgtcttttaaataagttcttcaggccgggcgcggtggctcatgcctgtaatcccagcactttgggaggccgaggcaggcagatcacctgaagtcaggagtactcgaccagcctggccaacatagtgaaaccccatctcaactaaaaatacaaaaatcagccgggcgtggtggcaggcgcctgtaatcccagctactcagggggctgaaacaggagaatcgcttgaacccgggaggcggaggttgcgccatcgcactccagcctgggagacaagagcgagacttcgtctcaaaaaaaaaaaattcttcttccaagattcaagttgtgtcatttcaccttaataactggaggttagttaagctgggctgtgttctttgcttaatattaagacaacgttttttccagatggaagaaaactatcttaatgaattgttagcttattaattatgtaatgctaatggcttttaaaagctgagatgttctgactgggtgttgtggctcacacctgtaatcccagtaccttgggaggccaagggggaaggattgcttgaggccaggagtttgggaccatagtgagaccccgcctctatttaaaaaattaaattttgttttgttttgttttgagttggagttttgctcttgttgcccatgctgaagtgcaatggtgcaatctcagctcaccacaacctgtgcctcctgggttcaagcgattctcctgcttcagcctcccgagtagatgggattacaggcgtgcaccaccatgcctggctaattttgtatttttagtagagacagggtttctctatgttggtcaggctggtctcaaactctcgacctcaggtgatctgcccgcctccgcttcccaaagttctgggattataggtgtgagccactgggcctggcctaagaaagtttttttaagccattagacgtttttaaaggaattgggagatgacaattggggaaatatttaaaatttaagtaaaatataaagcttccttatttcatgtaacccagacaatctcagtatacatgatcagttgtgtctgacaggtaaatctatttgaggccttatcacacgttacttttaagaactagaaaggaaaagtcactgatcttaagtatttataatacttcatgtggtctaatactttttacgttttgttttgattcagatttagtccggattcccggtatctggcagtaggttctagtgagaactcagtggatttttatgacctaacgctgggccccactcttaacagaatcagctactgcaaagacattccaagctttgtcattcaaatggacttctctgcagatagcagttatctccaggtacagtaccaatactgtatacccaggtggcaagttcttctgcttttacatttcgtgttagtgaatgcatttaaagttcctgagctccagagctccagcttctcaactcctccctttgtaccttctgacctacagctcccctttcctcccccacttatcagagcttttctcctattaagtttttgtagtgatcttttgcatacttaataatgttagacatgtaaatcaagtagcaatatgctagtattctgtaaaccccctgtggattttgtctctcacctaatggaattcttgtcccattttaatctgatgaaaaaggtctctagtggctgctataaacggcatgtctatgaagtgccttcaggaaaacatcttatggatcatgccgctattgacagaattacttgggctacatggactaggtaaatacttatatattcacaaggcaagaactgactttgaaggccagttagaaaatcctatttctgaactgttagagccattccaataaggaatagtaattgagtttcaagtttttgttaccatattttgaaatggtatgttcatgttgggacccctttttattgaatatatttccatgttttatcagtttccatgatttatcaagttttttttttaaggaaatcaaagttttaactttaaagataccctgatatttttcttaatgctaaatttaatgactggcaaaaaggtattgggtgctgttaagcaactgttattaattctctatctaaaggaatgctatcttgaatctattagaagtcaaagcttccaaatttgttcaaatttcctggctgtatgacaggtaaccatgactatccatttttttggccaatgaaaaatgccatcaaattcctgtatcagccaggcatatagtggctcatgcctgtaatctctgatgtagcaggccgaggtgggaggatcacttgagcctagaagttttgataccagcctgggcaacatagcaagaccccatctctgaaatttttttaattcctatgtcataagtcatttttatttttgtagagatagggatctcacaatattgcccaggctggtctcaaactcttggcctcaagcagtcctcctgcctcagcctcccaaaatgttgggattactggtatgtgctgctggacccagccaagtagcacttttaatttgaaaaatagttctatcagttttcagtcaggcgcggtggctcagcctgtaatcccagcactttgggaggccgagcgggggtgatcacctgaggtcgggagttcgagactagcctgaccaacatggagaaaccctgtctctactaaaaatacaaaataagccgggcatgttagcgcatgcctgtgatcccagctactcgggaggctgaggcaggagaattgcttgaacccaggaggcagaggttgcggtgagccgagatcatgccattgcactccagcctgggtaacaagagcgaaaactccgtctcaaaaaaaaaaaaagaaaaaatagttctatcagttttcataaagtactactttaatcttaaaaagattaatctagaaacccttcaaattataaaatgtcatttttaaaaggcaggagttgatatcctgatgaaattcaggtctccaaacaacttaccataatttacttcctgtattttaagtaacatgatagggtacttagagattaattgccaagaaactttttgaatatagtcaacctgcccgcacttgccatgatgagttttcttttgttccttccctctagtattctaggagatgaggttttgggaatctggtccagacatgctgagaaagctgatgtcaactgtgcctgtgtatctcattcaggaatcagtcttgttacaggagatgactttggcatggttaagttatttgacttcccatgtccagaaaaatttgtaagtttgtgttttgtttactattatcagtttactcctaattttgatgtcttatcatcagcacttttccccatatatttaaaatgttttgtcctaatttctaaatttttccccaaactttctaaatctatttactttgaaataaaagctattagaaacaaatcctctccctcgagtaataccatctttggaaccatcctacaaaagctgtaattagcttttcaccaaacctataatcagttatcaaatttcaaatgcttttccttagagaaaaatggtcagagtacctggagacatctgactgcccacacagcctggttttgcagatccactactcatgctgaaaagcattctaatcactggctgcggtgctaactccctactctctccacagctcttgtcatagagattatagttcctaataagagcctttgacttctgtgtgcaccaaatgccctgagcttgtctgtcattgttttttaggcaaaacacaaaaggttcttgggtcattcgccccatgtgacaaatattcgatttaccagtggtgatcgacatgttgttagtgctggaggtgatgactgcaggttagtaactttctcagcccatgaagagcagactatgttactagttaagagacttaatacaacaactcctacagctttggtttatgaaatcagctagtcaacattagtagaaggtagtataaccagatggctcttcagaatctcatatttatgcaaatacagaataaaaggagttaaagaggaaaaatattacacatgtaacctgaaagcacaactgaaaaatattaaactgttatgaaaatctaaaaacataattaactccctgcaattttcttctctgattgcagcttatttgtctggaaatgtgtacatacacctcactgagagatgctgagatgactacagaaattaactttgagaccagaattacagagaagaaaaaccaaaacccaaccctgcatggtcaagtggtgctaacccaagactgtaacagggagaaatgcccagaatcatcaaaatagtgaaagactgatctgttcaaaatatttgctatatgcactgggtataatccgtaatccatacactgccagataatgccatttcaaggaaggatcgaatacttgatggtaaaggccaagtccccctgtattgggaagtgtgtgatttcggcagacctgctgggaaaatttagggtagagcactctttacagaagaactcaaaaacccaatttggataattttcattatctttttagcaaaatggtttcttaatgtttatattttattttcaaggttcattgtttaatgaaatattttattcttgcatttccataaggaaagggaaagtcatgatcatcctaaaggatcacagtttttaaaaggcaaacattttccctaaggaaacagacacaagctttcctagagaatatgatgttttttaggcattaataaggtccttttttataaaggacacttttctcctagtagttttgaattcaggaacagatccaaagttagcagtatatggctgctacatttccattttcattttcgagccatcagtttatgttcagatgccatctctgtaatcgcacatttaaaacataactgtagcctcactaatggaaaagtagtatgatgaacaatcattcccaatggtgtacaatgtaagggttttagggagcaacagtatttaactggaagaaagaattgcatatttaatgtagtctaatatatacacatttgtttaacatgtaaacaaaagtgttaaattcacatatacaacattatacaatttaatcactcttggaataaaatttttatagccttttttctattgggaaaatttgtttagatgtgtgccactccataggtttatttccaaaatgaatgagcccaactccatttgtaaaaacttgtcagttagaattcctttttttagtggattagggctgaattcttagatccttatttcttttcactttaaatgctgccaaagatcactactcatcattcaggaattcgctgtctagcctatctgtagtttcctgaagattgaaaattatgtagactgctatttaaaaatatatttttctaagtgtgaggtttaagatgctgtattgaccctatgagtttttaatgtgttaattatctttatagcataatagatcgctttaggttcctggaatcccatttggtctgacaggatatatgaagattcttaatacctattttctgtgtctaatacttggttaatactaaaaatagaaatgactaaattacatcacagaaagcataaccagtgattgaacctggtagttttaaagctctaaatagctgtggctgaaggactgattatggggctaagaagcttgaaacgtaagttggtacttgttcatcagtggattctcctaaattaagccaaattttgaaatacatgactattaagtttctactcatgtatttacagtcagtcaataaattaaaggaggaaaaaaatccctgaacaacctgcccataaaaagaaaaatactctacatttgagcctgctgcagttttaaattttccctctgggtcaagtttgccagcttttggctacagagaaattatatttccattacagtgcaggtagaaactctgtaaccttaagcatgtaaactacatagaataaaactgtttccactgcatttctgtccttcaaagtggccaacctgattaagtcagccttaatcactgctgctgtcagtttcacgactaaaggtcatattgactaagtagtcatcagctgaccacctcgctgtatcagccagcaacgaggggaaggtgaagaaacatgataggccatatagaatctgccctatgtttacttttttaacccagataattatttttgtgtgcagtatctaagctcctgattgtgtaacctgggacttctggcaccttttgttccattcattttatgtataaaatgcatgccaaagcacactgtgccctctggtacccttgcttccaatcgccaaccatgctcatttccttcctttttttgtggtccctttttgtggtgatcattttaaaccacgtcatccaacaaatgttttatggtcaaccttagcttgttcataagccatagcaactgaaagattaaactcttaaatatgtgtctgggcagtggctattaaatagcaaaaaacaatcagattttagtattttattatttccttgtaaaatggctgaactaaattaaacccttgtttcccatttgttctataatttatagtgaaactgagaacaaaactatctttataaatgatagctaaaagtatttccagatatttaaacaatttaaaataaatttcttctgcagagatgcaaagcatctcaacactggaatgaacaaatgccttaaattcaatggagtaaacctttagaatgaagaggaactgtcatttcacccaagccgaagacaacagccttatgcacttgtgtgctctgtctttgctgcttctcgtgtttcaagcctttcctgtgggatcagcacagcaaagtgcaacttaccaaatggtttaatgactggttaattctttcttctcccaatggaaaagcaatggcaacacaacagtagactgctggcttgacaatcttaaacgtgagcctttgcacatgtaggtttatcatcatttgagtatacgactaagcaagtcaatgaactttttttttttttttagcagtttaatttggtcctgagaatgttgcagtctttattaccccttttgcattaatccacttttctaaccaccttttaagctttaatttttaacactatacaccaagtctttgaaatcagtgatctgttatttaactctaaagcatttgacacttcttgccttaacagttttaaaaaccacacacaaaaaaactctgtaagtaatacagtaggccaaaagtttcatcctatctatcttgcagtttacctatctgatctgatctctgtaattatagttctgtcatttaaaatatactatttaaatctaatttttacatttcaaaaattatcttcagtagtaactaagtatattttctgtggattctgagaatgttatttttcagaatgtgagaatatatatgtacatttataatcttgtgactttaaagtctgttttcagatacagtatgtaaatacttgtaaaaaaatttgtataattttgtgataatgtagtttcccaaaaaaattatttagaaggcattatgttattagtaaatgagagcactgtatagaactgttcctattttctgcacttgccattccagctgcctccactgtccatacccacctcattcatcctgtcacagaaggcaggaaaactgggaactttaccaaagtagcactcagcctgagaggcctgtataatcatgcttttcaaactaaattcacttaaaaattaaaaagcagaattgaatattttaagcagcctcagtacctttggccaatgctgttttcatggtggattatgaacattatataatctttgggaaaagtgaaagtagtacaatttttagaataatgacaactgcctcactgcatctctccactcacacagcaaccgtgtagccccctaagctgcagtaccatgactaaccatgatgtcaatttcatatgctgatcctcacaacagcagtgcacaaacatgccccaaatattttaacagaatttagctcttccttaagctgtcttttcatagtaaaaacaaaacaaaaacacccaatgttaaaaccacataataaacttacaaacttgaaaaattagacacttcagatagataggcaataaaacttcatattatgaaagcaatatattccaagtttcaaagatttgacaagttctgtagagtatctttcatcagtacatgaaaacttccaaactgcatgatcttctgccaggcaggactgggtgctattcgctggtttgaggtcgaatccatttcaaggcatgtcgtggtgggacattaatggtgggatggtagaatgtgcagtccggtcttgtacattgagtgttaaacctacaatgttttggatgatagaagggacattccatcttcttacaagcagggaagtaacggcagagctgactactggaaggtggtgctggtggtgcaactgctggttttggagacagtactggaattcttctactcacatgagtgaagggacaatctggtttagtacactttgcatcatatttacaatttgggtgaacaaacaaacatttttcagcaaatttacaattggggaaggctttgcagggtgagatggggtgatggtaggcacactcatccccatttttacaagcaggccagtacttgcagcgctccaaaagtttttctggtttctgtgccacactcagttcactcatctcagctgtagagtagttagttgtttttgttacggattcttgagcttcagatatagccttcaaaatcagattcttgttagcttgtttagaaggtggaagagaaggtctcctttcaggctttgcaggcacagacacactgctggagatgcttcctgttcgagacccgtaatcatcatcttcttcctcctcttctccatcatgattgaatttttttactttaacaactgaacttaccacaggcaactttctcttccgaaagttttcatcctccatactcattttctccgagttgtttctaaagaacggactatacgtttcttctaagctgttaagcacctctggttcacacaaacgtcctgtttcatatacccaactactctgcatatcaagctgcttggcagcatgaatactattctgctgctgttgaaattgcaacctgtttaaatgaacaccactatctgcatttctacttgcaggtggtcgataaatttcaatagaagggcgagaagaaccatatgtaagtgtcactgtaggttttttctgagataagggattctcctgcacaaagttgaggtcttcgtcaatgagatcatctggttctggcttaatatcaatcacatcttcagagggtgctggctccctcaaaggtttcactgttgacattagtcgggttgcagctccatcatcgtaagtctgtctgacatttgtggtttttgactcctgcgaacttgtagaaactctggaatctcttttttcaggtctcgcgctaggaatggcaagtggtggcactgcagcttcatgcctcctctcatctccccgactgaaattgctcttgtttgaaggcacgttactatcaaagatgttggtatcagaagacttcagactagagggttcagttgtaacagagcgaagtttatctaatacaccatgaagccatacggtgaatcgaattgtgttgttccctagaaacagggacagatcctctgtcatttggtcctgacttttcttgttggccaccatcaccataatgtaatcaggaagttcttcatcaacataagctcctaattcttgtaatttccccttaatggcactccggatcttgcggctgatctcggtgccgatctccatggctctgcggcgtgcgggaactcagcactgcgcggcgcttggcttacccggaggctgccgcggactcctaccccgcagccgggacaccaccgcctcc

SEQ ID NO: 17454 - RNA, 13368 nt, Homo sapiens
  source 1..13368: mol_type = other RNA
tcaggccaggcacagtggctcatacctggaatcccagcactttgggaggccgaggcaggcagatcacctgaggtcaaggtatttgagaccagcctggccaacatggtgaaaccccatctctactaaaaatacagaaattagctgggtgtggtggtgcacacctgtaatgctagctactcgggaggctgaggtaggagaatcgcttgaacctgggaggcagaggttgcaataagcctagatcatgccactgcactcaagcctgggagacagagcgagactacatcttaaaaaaaaaaaaaaaagtattatgagagaggataatgtattgtaatgtattgtagaggctaaataaaattatgctcatgtcagaaaaaaagagtatttctcaaaataaaattcactgaaactggatgtttattttgactgagatatagtatatcctcaaattgccatagaaagtttacaagaatattagaggtaaattataaatatcagggcctttttaaaaaaaaaagattctgcttataacttggtatttgtttataataaaaattatagtagccaataatgaacacttactctggcttggttatttacttaggtcaaaagaaggaggagcggttaaactgtgggatcaggaactgaggcggtgccgtgccttcaggcttgagacaggacaagccacagattgtgttcgttctgtgtgcagaggcaaagtaagatgttccatgagctgatacagtgcagcagaaaacagaaagtggttattactgtgattccctcaccctttgcagcctaatgaacaatacttaataatgcataacgatggatttgcttgccaacattactctgtctttgctgctttctttgccaaagttagcaccagtgtggtgcataagctaggaagctattctgtctaaatactgtatgtaaacctccaatattttctagaatctgccaatttaacaactctagtagacataattgaaagcccttggcagttgactcatattaggacagctgtctccattttttaaaaaaacacacattccctagataaaacgtgcagtaaacaaacaatgaaatactactcagccataaaaaataatgaaattctgtcattcttggtggcaacatggatgagactggaggacatgatgtgaagtgaaataagccaggcacagaaagataaatacatgttctcactcctgtgcagaaactaaaaaagttgatcccacagaggtggagagtagaatagtggttactggaggcggacaagggggagggggagggggatagggaaggactggttaaaggatacaagtttacacagccagataggaatagtatgttttagtattctgtagtactgtaggatgactatagttaagaatcacgtatttatgtattttcaggtatttacaagagaggattttgaaagtttccatcacaaagaaatgataaatgtctgaggtgatggttatgcgtattaccctatgccctatagatatgtataattatgtgtcaatttcaaaataaaaattcaaaactacaactcctatgaaaatttttgagcgtgtttgtacttattaagtgtatttataaatcatacggatattatcttcagcctgcatattaaattgtagttaagcttttactttttaactaaaaaataaattctattattttttcctatatcccactgcactgaccccagtttggaaatcctaagattatcaaataaaaactttgattattgaagaatccaggtgtactgccacagaaaagttctattctgtagcatggactctaatatgtaatctagcccattgtgcttacagatagatgtgtgcctgtagtcatagaaaaatttgcatgagctaatgactgccttgctactagattagctcaaagcaaaaagttctctgaaagcaggtcaatagggtcatttttatattatgaagaagaaaagcagctgttgtattacattcactgtattggtcctgcttgtgtttcagggcaagatccttgttgggacaaggaatgctgaaataatcgaagttggagagaaaaatgcagcttgtaatattttagttaacggtcatgtggatgggccaatctggggactagcaacacatccttccagggattttttcctttctgctgcagaagatgggacagtgagactttgggatattgctgataaagtaagtacagataatttttttaaaagaggttacaacttctaaaaagaaaagttggaagttctaaattgctagtacttaaagaactgccagaattctgttgagcattttgaggggaaactggtataatttagaagtacttcacttaatgtttcctatgactctttttttttttttttttaaatgcagaagatgttaaacaaagtgaatttgggacatgctgctcgtactgtgtgttacagccctgaaggggacatggtggctattggaatgaaaaatggagaatttatcattttactagtgagttctctaaaaatatggggaaagaagagagacaggagatgtgcaatccatgatatcaggttagtgaacaaatggaatagagtttctagtatatacttgatttaacttccatttgtaaaattttccatagccttgccttcaaaaagaggtccccagggcctgtagcatttcccgtattataaattgtatgctaaaatatggctgtttgtatactacttaattcttcttgctaaattataaacccactgggcaccaactataatagcaagtactagtaggtaatgtttgatgaattcatgttaacacttagccatgtccattaagttcatcccaccaagaggtatctcccactgtaatacaagagagctatctgcccttcaaaagttgtcaccctggaaaactaaagttgtgatttcaaacatatcttctcttagtaacctcagtttgggaatatgtagttcattaatttaatcaatacctattgattaaatgttccagaatccaaattaatttaaatgtttcttaaacctttgtttttcagtgcttaagcatttttcaacagtggctaccatttacggagtacttccgtgtgatcagtagataagattattgaatctaggtctgtcaaaagcttgtacacttttcatcagtaaaatccttttacaaatgaaaccttcctcagaacttcaatatataaaatagtaacagtggcttcccttagcttttacatgtctctatcgtacctcagtaagactcatgggccatttcaagagactgaattgtcccatatgactccaaagattgctaggcaaatagcatttcactttgtcttttaaataagttcttcaggccgggcgcggtggctcatgcctgtaatcccagcactttgggaggccgaggcaggcagatcacctgaagtcaggagtactcgaccagcctggccaacatagtgaaaccccatctcaactaaaaatacaaaaatcagccgggcgtggtggcaggcgcctgtaatcccagctactcagggggctgaaacaggagaatcgcttgaacccgggaggcggaggttgcgccatcgcactccagcctgggagacaagagcgagacttcgtctcaaaaaaaaaaaattcttcttccaagattcaagttgtgtcatttcaccttaataactggaggttagttaagctgggctgtgttctttgcttaatattaagacaacgttttttccagatggaagaaaactatcttaatgaattgttagcttattaattatgtaatgctaatggcttttaaaagctgagatgttctgactgggtgttgtggctcacacctgtaatcccagtaccttgggaggccaagggggaaggattgcttgaggccaggagtttgggaccatagtgagaccccgcctctatttaaaaaattaaattttgttttgttttgttttgagttggagttttgctcttgttgcccatgctgaagtgcaatggtgcaatctcagctcaccacaacctgtgcctcctgggttcaagcgattctcctgcttcagcctcccgagtagatgggattacaggcgtgcaccaccatgcctggctaattttgtatttttagtagagacagggtttctctatgttggtcaggctggtctcaaactctcgacctcaggtgatctgcccgcctccgcttcccaaagttctgggattataggtgtgagccactgggcctggcctaagaaagtttttttaagccattagacgtttttaaaggaattgggagatgacaattggggaaatatttaaaatttaagtaaaatataaagcttccttatttcatgtaacccagacaatctcagtatacatgatcagttgtgtctgacaggtaaatctatttgaggccttatcacacgttacttttaagaactagaaaggaaaagtcactgatcttaagtatttataatacttcatgtggtctaatactttttacgttttgttttgattcagatttagtccggattcccggtatctggcagtaggttctagtgagaactcagtggatttttatgacctaacgctgggccccactcttaacagaatcagctactgcaaagacattccaagctttgtcattcaaatggacttctctgcagatagcagttatctccaggtacagtaccaatactgtatacccaggtggcaagttcttctgcttttacatttcgtgttagtgaatgcatttaaagttcctgagctccagagctccagcttctcaactcctccctttgtaccttctgacctacagctcccctttcctcccccacttatcagagcttttctcctattaagtttttgtagtgatcttttgcatacttaataatgttagacatgtaaatcaagtagcaatatgctagtattctgtaaaccccctgtggattttgtctctcacctaatggaattcttgtcccattttaatctgatgaaaaaggtctctagtggctgctataaacggcatgtctatgaagtgccttcaggaaaacatcttatggatcatgccgctattgacagaattacttgggctacatggactaggtaaatacttatatattcacaaggcaagaactgactttgaaggccagttagaaaatcctatttctgaactgttagagccattccaataaggaatagtaattgagtttcaagtttttgttaccatattttgaaatggtatgttcatgttgggacccctttttattgaatatatttccatgttttatcagtttccatgatttatcaagttttttttttaaggaaatcaaagttttaactttaaagataccctgatatttttcttaatgctaaatttaatgactggcaaaaaggtattgggtgctgttaagcaactgttattaattctctatctaaaggaatgctatcttgaatctattagaagtcaaagcttccaaatttgttcaaatttcctggctgtatgacaggtaaccatgactatccatttttttggccaatgaaaaatgccatcaaattcctgtatcagccaggcatatagtggctcatgcctgtaatctctgatgtagcaggccgaggtgggaggatcacttgagcctagaagttttgataccagcctgggcaacatagcaagaccccatctctgaaatttttttaattcctatgtcataagtcatttttatttttgtagagatagggatctcacaatattgcccaggctggtctcaaactcttggcctcaagcagtcctcctgcctcagcctcccaaaatgttgggattactggtatgtgctgctggacccagccaagtagcacttttaatttgaaaaatagttctatcagttttcagtcaggcgcggtggctcagcctgtaatcccagcactttgggaggccgagcgggggtgatcacctgaggtcgggagttcgagactagcctgaccaacatggagaaaccctgtctctactaaaaatacaaaataagccgggcatgttagcgcatgcctgtgatcccagctactcgggaggctgaggcaggagaattgcttgaacccaggaggcagaggttgcggtgagccgagatcatgccattgcactccagcctgggtaacaagagcgaaaactccgtctcaaaaaaaaaaaaagaaaaaatagttctatcagttttcataaagtactactttaatcttaaaaagattaatctagaaacccttcaaattataaaatgtcatttttaaaaggcaggagttgatatcctgatgaaattcaggtctccaaacaacttaccataatttacttcctgtattttaagtaacatgatagggtacttagagattaattgccaagaaactttttgaatatagtcaacctgcccgcacttgccatgatgagttttcttttgttccttccctctagtattctaggagatgaggttttgggaatctggtccagacatgctgagaaagctgatgtcaactgtgcctgtgtatctcattcaggaatcagtcttgttacaggagatgactttggcatggttaagttatttgacttcccatgtccagaaaaatttgtaagtttgtgttttgtttactattatcagtttactcctaattttgatgtcttatcatcagcacttttccccatatatttaaaatgttttgtcctaatttctaaatttttccccaaactttctaaatctatttactttgaaataaaagctattagaaacaaatcctctccctcgagtaataccatctttggaaccatcctacaaaagctgtaattagcttttcaccaaacctataatcagttatcaaatttcaaatgcttttccttagagaaaaatggtcagagtacctggagacatctgactgcccacacagcctggttttgcagatccactactcatgctgaaaagcattctaatcactggctgcggtgctaactccctactctctccacagctcttgtcatagagattatagttcctaataagagcctttgacttctgtgtgcaccaaatgccctgagcttgtctgtcattgttttttaggcaaaacacaaaaggttcttgggtcattcgccccatgtgacaaatattcgatttaccagtggtgatcgacatgttgttagtgctggaggtgatgactgcaggttagtaactttctcagcccatgaagagcagactatgttactagttaagagacttaatacaacaactcctacagctttggtttatgaaatcagctagtcaacattagtagaaggtagtataaccagatggctcttcagaatctcatatttatgcaaatacagaataaaaggagttaaagaggaaaaatattacacatgtaacctgaaagcacaactgaaaaatattaaactgttatgaaaatctaaaaacataattaactccctgcaattttcttctctgattgcagcttatttgtctggaaatgtgtacatacacctcactgagagatgctgagatgactacagaaattaactttgagaccagaattacagagaagaaaaaccaaaacccaaccctgcatggtcaagtggtgctaacccaagactgtaacagggagaaatgcccagaatcatcaaaatagtgaaagactgatctgttcaaaatatttgctatatgcactgggtataatccgtaatccatacactgccagataatgccatttcaaggaaggatcgaatacttgatggtaaaggccaagtccccctgtattgggaagtgtgtgatttcggcagacctgctgggaaaatttagggtagagcactctttacagaagaactcaaaaacccaatttggataattttcattatctttttagcaaaatggtttcttaatgtttatattttattttcaaggttcattgtttaatgaaatattttattcttgcatttccataaggaaagggaaagtcatgatcatcctaaaggatcacagtttttaaaaggcaaacattttccctaaggaaacagacacaagctttcctagagaatatgatgttttttaggcattaataaggtccttttttataaaggacacttttctcctagtagttttgaattcaggaacagatccaaagttagcagtatatggctgctacatttccattttcattttcgagccatcagtttatgttcagatgccatctctgtaatcgcacatttaaaacataactgtagcctcactaatggaaaagtagtatgatgaacaatcattcccaatggtgtacaatgtaagggttttagggagcaacagtatttaactggaagaaagaattgcatatttaatgtagtctaatatatacacatttgtttaacatgtaaacaaaagtgttaaattcacatatacaacattatacaatttaatcactcttggaataaaatttttatagccttttttctattgggaaaatttgtttagatgtgtgccactccataggtttatttccaaaatgaatgagcccaactccatttgtaaaaacttgtcagttagaattcctttttttagtggattagggctgaattcttagatccttatttcttttcactttaaatgctgccaaagatcactactcatcattcaggaattcgctgtctagcctatctgtagtttcctgaagattgaaaattatgtagactgctatttaaaaatatatttttctaagtgtgaggtttaagatgctgtattgaccctatgagtttttaatgtgttaattatctttatagcataatagatcgctttaggttcctggaatcccatttggtctgacaggatatatgaagattcttaatacctattttctgtgtctaatacttggttaatactaaaaatagaaatgactaaattacatcacagaaagcataaccagtgattgaacctggtagttttaaagctctaaatagctgtggctgaaggactgattatggggctaagaagcttgaaacgtaagttggtacttgttcatcagtggattctcctaaattaagccaaattttgaaatacatgactattaagtttctactcatgtatttacagtcagtcaataaattaaaggaggaaaaaaatccctgaacaacctgcccataaaaagaaaaatactctacatttgagcctgctgcagttttaaattttccctctgggtcaagtttgccagcttttggctacagagaaattatatttccattacagtgcaggtagaaactctgtaaccttaagcatgtaaactacatagaataaaactgtttccactgcatttctgtccttcaaagtggccaacctgattaagtcagccttaatcactgctgctgtcagtttcacgactaaaggtcatattgactaagtagtcatcagctgaccacctcgctgtatcagccagcaacgaggggaaggtgaagaaacatgataggccatatagaatctgccctatgtttacttttttaacccagataattatttttgtgtgcagtatctaagctcctgattgtgtaacctgggacttctggcaccttttgttccattcattttatgtataaaatgcatgccaaagcacactgtgccctctggtacccttgcttccaatcgccaaccatgctcatttccttcctttttttgtggtccctttttgtggtgatcattttaaaccacgtcatccaacaaatgttttatggtcaaccttagcttgttcataagccatagcaactgaaagattaaactcttaaatatgtgtctgggcagtggctattaaatagcaaaaaacaatcagattttagtattttattatttccttgtaaaatggctgaactaaattaaacccttgtttcccatttgttctataatttatagtgaaactgagaacaaaactatctttataaatgatagctaaaagtatttccagatatttaaacaatttaaaataaatttcttctgcagagatgcaaagcatctcaacactggaatgaacaaatgccttaaattcaatggagtaaacctttagaatgaagaggaactgtcatttcacccaagccgaagacaacagccttatgcacttgtgtgctctgtctttgctgcttctcgtgtttcaagcctttcctgtgggatcagcacagcaaagtgcaacttaccaaatggtttaatgactggttaattctttcttctcccaatggaaaagcaatggcaacacaacagtagactgctggcttgacaatcttaaacgtgagcctttgcacatgtaggtttatcatcatttgagtatacgactaagcaagtcaatgaactttttttttttttttagcagtttaatttggtcctgagaatgttgcagtctttattaccccttttgcattaatccacttttctaaccaccttttaagctttaatttttaacactatacaccaagtctttgaaatcagtgatctgttatttaactctaaagcatttgacacttcttgccttaacagttttaaaaaccacacacaaaaaaactctgtaagtaatacagtaggccaaaagtttcatcctatctatcttgcagtttacctatctgatctgatctctgtaattatagttctgtcatttaaaatatactatttaaatctaatttttacatttcaaaaattatcttcagtagtaactaagtatattttctgtggattctgagaatgttatttttcagaatgtgagaatatatatgtacatttataatcttgtgactttaaagtctgttttcagatacagtatgtaaatacttgtaaaaaaatttgtataattttgtgataatgtagtttcccaaaaaaattatttagaaggcattatgttattagtaaatgagagcactgtatagaactgttcctattttctgcacttgccattccagctgcctccactgtccatacccacctcattcatcctgtcacagaaggcaggaaaactgggaactttaccaaagtagcactcagcctgagaggcctgtataatcatgcttttcaaactaaattcacttaaaaattaaaaagcagaattgaatattttaagcagcctcagtacctttggccaatgctgttttcatggtggattatgaacattatataatctttgggaaaagtgaaagtagtacaatttttagaataatgacaactgcctcactgcatctctccactcacacagcaaccgtgtagccccctaagctgcagtaccatgactaaccatgatgtcaatttcatatgctgatcctcacaacagcagtgcacaaacatgccccaaatattttaacagaatttagctcttccttaagctgtcttttcatagtaaaaacaaaacaaaaacacccaatgttaaaaccacataataaacttacaaacttgaaaaattagacacttcagatagataggcaataaaacttcatattatgaaagcaatatattccaagtttcaaagatttgacaagttctgtagagtatctttcatcagtacatgaaaacttccaaactgcatgatcttctgccaggcaggactgggtgctattcgctggtttgaggtcgaatccatttcaaggcatgtcgtggtgggacattaatggtgggatggtagaatgtgcagtccggtcttgtacattgagtgttaaacctacaatgttttggatgatagaagggacattccatcttcttacaagcagggaagtaacggcagagctgactactggaaggtggtgctggtggtgcaactgctggttttggagacagtactggaattcttctactcacatgagtgaagggacaatctggtttagtacactttgcatcatatttacaatttgggtgaacaaacaaacatttttcagcaaatttacaattggggaaggctttgcagggtgagatggggtgatggtaggcacactcatccccatttttacaagcaggccagtacttgcagcgctccaaaagtttttctggtttctgtgccacactcagttcactcatctcagcttgactcatctgcagagtttctgccattactgggtcgatttgcagtcgggataataattgcctctgttgagttccttgatttttttctacagaatctccttttgtttcctcttctttaatggggggacttattctgggggtcctactttgtccctggaccacttctgctagcaattcttcttgagaagttcgagttctgggagcaactggaagtgtctgtttctgtggaactgtagagtagttagttgtttttgttacggattcttgagcttcagatatagccttcaaaatcagattcttgttagcttgtttagaaggtggaagagaaggtctcctttcaggctttgcaggcacagacacactgctggagatgcttcctgttcgagacccgtaatcatcatcttcttcctcctcttctccatcatgattgaatttttttactttaacaactgaacttaccacaggcaactttctcttccgaaagttttcatcctccatactcattttctccgagttgtttctaaagaacggactatacgtttcttctaagctgttaagcacctctggttcacacaaacgtcctgtttcatatacccaactactctgcatatcaagctgcttggcagcatgaatactattctgctgctgttgaaattgcaacctgtttaaatgaacaccactatctgcatttctacttgcaggtggtcgataaatttcaatagaagggcgagaagaaccatatgtaagtgtcactgtaggttttttctgagataagggattctcctgcacaaagttgaggtcttcgtcaatgagatcatctggttctggcttaatatcaatcacatcttcagagggtgctggctccctcaaaggtttcactgttgacattagtcgggttgcagctccatcatcgtaagtctgtctgacatttgtggtttttgactcctgcgaacttgtagaaactctggaatctcttttttcaggtctcgcgctaggaatggcaagtggtggcactgcagcttcatgcctcctctcatctccccgactgaaattgctcttgtttgaaggcacgttactatcaaagatgttggtatcagaagacttcagactagagggttcagttgtaacagagcgaagtttatctaatacaccatgaagccaacataagctcctaattcttgtaatttccccttaatggcactccggatcttgcggctgatctcggtgccgatctccatggctctgcggcgtgcgggaactcagcactgcgcggcgcttggcttacccggaggctgccgcggactcctaccccgcagccgggacaccaccgcctcc

SEQ ID NO: 17455 - RNA, 13483 nt, Homo sapiens
  source 1..13483: mol_type = other RNA
tcaggccaggcacagtggctcatacctggaatcccagcactttgggaggccgaggcaggcagatcacctgaggtcaaggtatttgagaccagcctggccaacatggtgaaaccccatctctactaaaaatacagaaattagctgggtgtggtggtgcacacctgtaatgctagctactcgggaggctgaggtaggagaatcgcttgaacctgggaggcagaggttgcaataagcctagatcatgccactgcactcaagcctgggagacagagcgagactacatcttaaaaaaaaaaaaaaaagtattatgagagaggataatgtattgtaatgtattgtagaggctaaataaaattatgctcatgtcagaaaaaaagagtatttctcaaaataaaattcactgaaactggatgtttattttgactgagatatagtatatcctcaaattgccatagaaagtttacaagaatattagaggtaaattataaatatcagggcctttttaaaaaaaaaagattctgcttataacttggtatttgtttataataaaaattatagtagccaataatgaacacttactctggcttggttatttacttaggtcaaaagaaggaggagcggttaaactgtgggatcaggaactgaggcggtgccgtgccttcaggcttgagacaggacaagccacagattgtgttcgttctgtgtgcagaggcaaagtaagatgttccatgagctgatacagtgcagcagaaaacagaaagtggttattactgtgattccctcaccctttgcagcctaatgaacaatacttaataatgcataacgatggatttgcttgccaacattactctgtctttgctgctttctttgccaaagttagcaccagtgtggtgcataagctaggaagctattctgtctaaatactgtatgtaaacctccaatattttctagaatctgccaatttaacaactctagtagacataattgaaagcccttggcagttgactcatattaggacagctgtctccattttttaaaaaaacacacattccctagataaaacgtgcagtaaacaaacaatgaaatactactcagccataaaaaataatgaaattctgtcattcttggtggcaacatggatgagactggaggacatgatgtgaagtgaaataagccaggcacagaaagataaatacatgttctcactcctgtgcagaaactaaaaaagttgatcccacagaggtggagagtagaatagtggttactggaggcggacaagggggagggggagggggatagggaaggactggttaaaggatacaagtttacacagccagataggaatagtatgttttagtattctgtagtactgtaggatgactatagttaagaatcacgtatttatgtattttcaggtatttacaagagaggattttgaaagtttccatcacaaagaaatgataaatgtctgaggtgatggttatgcgtattaccctatgccctatagatatgtataattatgtgtcaatttcaaaataaaaattcaaaactacaactcctatgaaaatttttgagcgtgtttgtacttattaagtgtatttataaatcatacggatattatcttcagcctgcatattaaattgtagttaagcttttactttttaactaaaaaataaattctattattttttcctatatcccactgcactgaccccagtttggaaatcctaagattatcaaataaaaactttgattattgaagaatccaggtgtactgccacagaaaagttctattctgtagcatggactctaatatgtaatctagcccattgtgcttacagatagatgtgtgcctgtagtcatagaaaaatttgcatgagctaatgactgccttgctactagattagctcaaagcaaaaagttctctgaaagcaggtcaatagggtcatttttatattatgaagaagaaaagcagctgttgtattacattcactgtattggtcctgcttgtgtttcagggcaagatccttgttgggacaaggaatgctgaaataatcgaagttggagagaaaaatgcagcttgtaatattttagttaacggtcatgtggatgggccaatctggggactagcaacacatccttccagggattttttcctttctgctgcagaagatgggacagtgagactttgggatattgctgataaagtaagtacagataatttttttaaaagaggttacaacttctaaaaagaaaagttggaagttctaaattgctagtacttaaagaactgccagaattctgttgagcattttgaggggaaactggtataatttagaagtacttcacttaatgtttcctatgactctttttttttttttttttaaatgcagaagatgttaaacaaagtgaatttgggacatgctgctcgtactgtgtgttacagccctgaaggggacatggtggctattggaatgaaaaatggagaatttatcattttactagtgagttctctaaaaatatggggaaagaagagagacaggagatgtgcaatccatgatatcaggttagtgaacaaatggaatagagtttctagtatatacttgatttaacttccatttgtaaaattttccatagccttgccttcaaaaagaggtccccagggcctgtagcatttcccgtattataaattgtatgctaaaatatggctgtttgtatactacttaattcttcttgctaaattataaacccactgggcaccaactataatagcaagtactagtaggtaatgtttgatgaattcatgttaacacttagccatgtccattaagttcatcccaccaagaggtatctcccactgtaatacaagagagctatctgcccttcaaaagttgtcaccctggaaaactaaagttgtgatttcaaacatatcttctcttagtaacctcagtttgggaatatgtagttcattaatttaatcaatacctattgattaaatgttccagaatccaaattaatttaaatgtttcttaaacctttgtttttcagtgcttaagcatttttcaacagtggctaccatttacggagtacttccgtgtgatcagtagataagattattgaatctaggtctgtcaaaagcttgtacacttttcatcagtaaaatccttttacaaatgaaaccttcctcagaacttcaatatataaaatagtaacagtggcttcccttagcttttacatgtctctatcgtacctcagtaagactcatgggccatttcaagagactgaattgtcccatatgactccaaagattgctaggcaaatagcatttcactttgtcttttaaataagttcttcaggccgggcgcggtggctcatgcctgtaatcccagcactttgggaggccgaggcaggcagatcacctgaagtcaggagtactcgaccagcctggccaacatagtgaaaccccatctcaactaaaaatacaaaaatcagccgggcgtggtggcaggcgcctgtaatcccagctactcagggggctgaaacaggagaatcgcttgaacccgggaggcggaggttgcgccatcgcactccagcctgggagacaagagcgagacttcgtctcaaaaaaaaaaaattcttcttccaagattcaagttgtgtcatttcaccttaataactggaggttagttaagctgggctgtgttctttgcttaatattaagacaacgttttttccagatggaagaaaactatcttaatgaattgttagcttattaattatgtaatgctaatggcttttaaaagctgagatgttctgactgggtgttgtggctcacacctgtaatcccagtaccttgggaggccaagggggaaggattgcttgaggccaggagtttgggaccatagtgagaccccgcctctatttaaaaaattaaattttgttttgttttgttttgagttggagttttgctcttgttgcccatgctgaagtgcaatggtgcaatctcagctcaccacaacctgtgcctcctgggttcaagcgattctcctgcttcagcctcccgagtagatgggattacaggcgtgcaccaccatgcctggctaattttgtatttttagtagagacagggtttctctatgttggtcaggctggtctcaaactctcgacctcaggtgatctgcccgcctccgcttcccaaagttctgggattataggtgtgagccactgggcctggcctaagaaagtttttttaagccattagacgtttttaaaggaattgggagatgacaattggggaaatatttaaaatttaagtaaaatataaagcttccttatttcatgtaacccagacaatctcagtatacatgatcagttgtgtctgacaggtaaatctatttgaggccttatcacacgttacttttaagaactagaaaggaaaagtcactgatcttaagtatttataatacttcatgtggtctaatactttttacgttttgttttgattcagatttagtccggattcccggtatctggcagtaggttctagtgagaactcagtggatttttatgacctaacgctgggccccactcttaacagaatcagctactgcaaagacattccaagctttgtcattcaaatggacttctctgcagatagcagttatctccaggtacagtaccaatactgtatacccaggtggcaagttcttctgcttttacatttcgtgttagtgaatgcatttaaagttcctgagctccagagctccagcttctcaactcctccctttgtaccttctgacctacagctcccctttcctcccccacttatcagagcttttctcctattaagtttttgtagtgatcttttgcatacttaataatgttagacatgtaaatcaagtagcaatatgctagtattctgtaaaccccctgtggattttgtctctcacctaatggaattcttgtcccattttaatctgatgaaaaaggtctctagtggctgctataaacggcatgtctatgaagtgccttcaggaaaacatcttatggatcatgccgctattgacagaattacttgggctacatggactaggtaaatacttatatattcacaaggcaagaactgactttgaaggccagttagaaaatcctatttctgaactgttagagccattccaataaggaatagtaattgagtttcaagtttttgttaccatattttgaaatggtatgttcatgttgggacccctttttattgaatatatttccatgttttatcagtttccatgatttatcaagttttttttttaaggaaatcaaagttttaactttaaagataccctgatatttttcttaatgctaaatttaatgactggcaaaaaggtattgggtgctgttaagcaactgttattaattctctatctaaaggaatgctatcttgaatctattagaagtcaaagcttccaaatttgttcaaatttcctggctgtatgacaggtaaccatgactatccatttttttggccaatgaaaaatgccatcaaattcctgtatcagccaggcatatagtggctcatgcctgtaatctctgatgtagcaggccgaggtgggaggatcacttgagcctagaagttttgataccagcctgggcaacatagcaagaccccatctctgaaatttttttaattcctatgtcataagtcatttttatttttgtagagatagggatctcacaatattgcccaggctggtctcaaactcttggcctcaagcagtcctcctgcctcagcctcccaaaatgttgggattactggtatgtgctgctggacccagccaagtagcacttttaatttgaaaaatagttctatcagttttcagtcaggcgcggtggctcagcctgtaatcccagcactttgggaggccgagcgggggtgatcacctgaggtcgggagttcgagactagcctgaccaacatggagaaaccctgtctctactaaaaatacaaaataagccgggcatgttagcgcatgcctgtgatcccagctactcgggaggctgaggcaggagaattgcttgaacccaggaggcagaggttgcggtgagccgagatcatgccattgcactccagcctgggtaacaagagcgaaaactccgtctcaaaaaaaaaaaaagaaaaaatagttctatcagttttcataaagtactactttaatcttaaaaagattaatctagaaacccttcaaattataaaatgtcatttttaaaaggcaggagttgatatcctgatgaaattcaggtctccaaacaacttaccataatttacttcctgtattttaagtaacatgatagggtacttagagattaattgccaagaaactttttgaatatagtcaacctgcccgcacttgccatgatgagttttcttttgttccttccctctagtattctaggagatgaggttttgggaatctggtccagacatgctgagaaagctgatgtcaactgtgcctgtgtatctcattcaggaatcagtcttgttacaggagatgactttggcatggttaagttatttgacttcccatgtccagaaaaatttgtaagtttgtgttttgtttactattatcagtttactcctaattttgatgtcttatcatcagcacttttccccatatatttaaaatgttttgtcctaatttctaaatttttccccaaactttctaaatctatttactttgaaataaaagctattagaaacaaatcctctccctcgagtaataccatctttggaaccatcctacaaaagctgtaattagcttttcaccaaacctataatcagttatcaaatttcaaatgcttttccttagagaaaaatggtcagagtacctggagacatctgactgcccacacagcctggttttgcagatccactactcatgctgaaaagcattctaatcactggctgcggtgctaactccctactctctccacagctcttgtcatagagattatagttcctaataagagcctttgacttctgtgtgcaccaaatgccctgagcttgtctgtcattgttttttaggcaaaacacaaaaggttcttgggtcattcgccccatgtgacaaatattcgatttaccagtggtgatcgacatgttgttagtgctggaggtgatgactgcaggttagtaactttctcagcccatgaagagcagactatgttactagttaagagacttaatacaacaactcctacagctttggtttatgaaatcagctagtcaacattagtagaaggtagtataaccagatggctcttcagaatctcatatttatgcaaatacagaataaaaggagttaaagaggaaaaatattacacatgtaacctgaaagcacaactgaaaaatattaaactgttatgaaaatctaaaaacataattaactccctgcaattttcttctctgattgcagcttatttgtctggaaatgtgtacatacacctcactgagagatgctgagatgactacagaaattaactttgagaccagaattacagagaagaaaaaccaaaacccaaccctgcatggtcaagtggtgctaacccaagactgtaacagggagaaatgcccagaatcatcaaaatagtgaaagactgatctgttcaaaatatttgctatatgcactgggtataatccgtaatccatacactgccagataatgccatttcaaggaaggatcgaatacttgatggtaaaggccaagtccccctgtattgggaagtgtgtgatttcggcagacctgctgggaaaatttagggtagagcactctttacagaagaactcaaaaacccaatttggataattttcattatctttttagcaaaatggtttcttaatgtttatattttattttcaaggttcattgtttaatgaaatattttattcttgcatttccataaggaaagggaaagtcatgatcatcctaaaggatcacagtttttaaaaggcaaacattttccctaaggaaacagacacaagctttcctagagaatatgatgttttttaggcattaataaggtccttttttataaaggacacttttctcctagtagttttgaattcaggaacagatccaaagttagcagtatatggctgctacatttccattttcattttcgagccatcagtttatgttcagatgccatctctgtaatcgcacatttaaaacataactgtagcctcactaatggaaaagtagtatgatgaacaatcattcccaatggtgtacaatgtaagggttttagggagcaacagtatttaactggaagaaagaattgcatatttaatgtagtctaatatatacacatttgtttaacatgtaaacaaaagtgttaaattcacatatacaacattatacaatttaatcactcttggaataaaatttttatagccttttttctattgggaaaatttgtttagatgtgtgccactccataggtttatttccaaaatgaatgagcccaactccatttgtaaaaacttgtcagttagaattcctttttttagtggattagggctgaattcttagatccttatttcttttcactttaaatgctgccaaagatcactactcatcattcaggaattcgctgtctagcctatctgtagtttcctgaagattgaaaattatgtagactgctatttaaaaatatatttttctaagtgtgaggtttaagatgctgtattgaccctatgagtttttaatgtgttaattatctttatagcataatagatcgctttaggttcctggaatcccatttggtctgacaggatatatgaagattcttaatacctattttctgtgtctaatacttggttaatactaaaaatagaaatgactaaattacatcacagaaagcataaccagtgattgaacctggtagttttaaagctctaaatagctgtggctgaaggactgattatggggctaagaagcttgaaacgtaagttggtacttgttcatcagtggattctcctaaattaagccaaattttgaaatacatgactattaagtttctactcatgtatttacagtcagtcaataaattaaaggaggaaaaaaatccctgaacaacctgcccataaaaagaaaaatactctacatttgagcctgctgcagttttaaattttccctctgggtcaagtttgccagcttttggctacagagaaattatatttccattacagtgcaggtagaaactctgtaaccttaagcatgtaaactacatagaataaaactgtttccactgcatttctgtccttcaaagtggccaacctgattaagtcagccttaatcactgctgctgtcagtttcacgactaaaggtcatattgactaagtagtcatcagctgaccacctcgctgtatcagccagcaacgaggggaaggtgaagaaacatgataggccatatagaatctgccctatgtttacttttttaacccagataattatttttgtgtgcagtatctaagctcctgattgtgtaacctgggacttctggcaccttttgttccattcattttatgtataaaatgcatgccaaagcacactgtgccctctggtacccttgcttccaatcgccaaccatgctcatttccttcctttttttgtggtccctttttgtggtgatcattttaaaccacgtcatccaacaaatgttttatggtcaaccttagcttgttcataagccatagcaactgaaagattaaactcttaaatatgtgtctgggcagtggctattaaatagcaaaaaacaatcagattttagtattttattatttccttgtaaaatggctgaactaaattaaacccttgtttcccatttgttctataatttatagtgaaactgagaacaaaactatctttataaatgatagctaaaagtatttccagatatttaaacaatttaaaataaatttcttctgcagagatgcaaagcatctcaacactggaatgaacaaatgccttaaattcaatggagtaaacctttagaatgaagaggaactgtcatttcacccaagccgaagacaacagccttatgcacttgtgtgctctgtctttgctgcttctcgtgtttcaagcctttcctgtgggatcagcacagcaaagtgcaacttaccaaatggtttaatgactggttaattctttcttctcccaatggaaaagcaatggcaacacaacagtagactgctggcttgacaatcttaaacgtgagcctttgcacatgtaggtttatcatcatttgagtatacgactaagcaagtcaatgaactttttttttttttttagcagtttaatttggtcctgagaatgttgcagtctttattaccccttttgcattaatccacttttctaaccaccttttaagctttaatttttaacactatacaccaagtctttgaaatcagtgatctgttatttaactctaaagcatttgacacttcttgccttaacagttttaaaaaccacacacaaaaaaactctgtaagtaatacagtaggccaaaagtttcatcctatctatcttgcagtttacctatctgatctgatctctgtaattatagttctgtcatttaaaatatactatttaaatctaatttttacatttcaaaaattatcttcagtagtaactaagtatattttctgtggattctgagaatgttatttttcagaatgtgagaatatatatgtacatttataatcttgtgactttaaagtctgttttcagatacagtatgtaaatacttgtaaaaaaatttgtataattttgtgataatgtagtttcccaaaaaaattatttagaaggcattatgttattagtaaatgagagcactgtatagaactgttcctattttctgcacttgccattccagctgcctccactgtccatacccacctcattcatcctgtcacagaaggcaggaaaactgggaactttaccaaagtagcactcagcctgagaggcctgtataatcatgcttttcaaactaaattcacttaaaaattaaaaagcagaattgaatattttaagcagcctcagtacctttggccaatgctgttttcatggtggattatgaacattatataatctttgggaaaagtgaaagtagtacaatttttagaataatgacaactgcctcactgcatctctccactcacacagcaaccgtgtagccccctaagctgcagtaccatgactaaccatgatgtcaatttcatatgctgatcctcacaacagcagtgcacaaacatgccccaaatattttaacagaatttagctcttccttaagctgtcttttcatagtaaaaacaaaacaaaaacacccaatgttaaaaccacataataaacttacaaacttgaaaaattagacacttcagatagataggcaataaaacttcatattatgaaagcaatatattccaagtttcaaagatttgacaagttctgtagagtatctttcatcagtacatgaaaacttccaaactgcatgatcttctgccaggcaggactgggtgctattcgctggtttgaggtcgaatccatttcaaggcatgtcgtggtgggacattaatggtgggatggtagaatgtgcagtccggtcttgtacattgagtgttaaacctacaatgttttggatgatagaagggacattccatcttcttacaagcagggaagtaacggcagagctgactactggaaggtggtgctggtggtgcaactgctggttttggagacagtactggaattcttctactcacatgagtgaagggacaatctggtttagtacactttgcatcatatttacaatttgggtgaacaaacaaacatttttcagcaaatttacaattggggaaggctttgcagggtgagatggggtgatggtaggcacactcatccccatttttacaagcaggccagtacttgcagcgctccaaaagtttttctggtttctgtgccacactcagttcactcatctcagcttgactcatctgcagagtttctgccattactgggtcgatttgcagtcgggataataattgcctctgttgagttccttgatttttttctacagaatctccttttgtttcctcttctttaatggggggacttattctgggggtcctactttgtccctggaccacttctgctagcaattcttcttgagaagttcgagttctgggagcaactggaagtgtctgtttctgtggaactgtagagtagttagttgtttttgttacggattcttgagcttcagatatagccttcaaaatcagattcttgttagcttgtttagaaggtggaagagaaggtctcctttcaggctttgcaggcacagacacactgctggagatgcttcctgttcgagacccgtaatcatcatcttcttcctcctcttctccatcatgattgaatttttttactttaacaactgaacttaccacaggcaactttctcttccgaaagttttcatcctccatactcattttctccgagttgtttctaaagaacggactatacgtttcttctaagctgttaagcacctctggttcacacaaacgtcctgtttcatatacccaactactctgcatatcaagctgcttggcagcatgaatactattctgctgctgttgaaattgcaacctgtttaaatgaacaccactatctgcatttctacttgcaggtggtcgataaatttcaatagaagggcgagaagaaccatatgtaagtgtcactgtaggttttttctgagataagggattctcctgcacaaagttgaggtcttcgtcaatgagatcatctggttctggcttaatatcaatcacatcttcagagggtgctggctccctcaaaggtttcactgttgacattagtcgggttgcagctccatcatcgtaagtctgtctgacatttgtggtttttgactcctgcgaacttgtagaaactctggaatctcttttttcaggtctcgcgctaggaatggcaagtggtggcactgcagcttcatgcctcctctcatctccccgactgaaattgctcttgtttgaaggcacgttactatcaaagatgttggtatcagaagacttcagactagagggttcagttgtaacagagcgaagtttatctaatacaccatgaagccatacggtgaatcgaattgtgttgttccctagaaacagggacagatcctctgtcatttggtcctgacttttcttgttggccaccatcaccataatgtaatcaggaagttcttcatcaacataagctcctaattcttgtaatttccccttaatggcactccggatcttgcggctgatctcggtgccgatctccatggctctgcggcgtgcgggaactcagcactgcgcggcgcttggcttacccggaggctgccgcggactcctaccccgcagccgggacaccaccgcctcc

SEQ ID NO: 17456 - RNA, 13459 nt, Homo sapiens
  source 1..13459: mol_type = other RNA
tcaggccaggcacagtggctcatacctggaatcccagcactttgggaggccgaggcaggcagatcacctgaggtcaaggtatttgagaccagcctggccaacatggtgaaaccccatctctactaaaaatacagaaattagctgggtgtggtggtgcacacctgtaatgctagctactcgggaggctgaggtaggagaatcgcttgaacctgggaggcagaggttgcaataagcctagatcatgccactgcactcaagcctgggagacagagcgagactacatcttaaaaaaaaaaaaaaaagtattatgagagaggataatgtattgtaatgtattgtagaggctaaataaaattatgctcatgtcagaaaaaaagagtatttctcaaaataaaattcactgaaactggatgtttattttgactgagatatagtatatcctcaaattgccatagaaagtttacaagaatattagaggtaaattataaatatcagggcctttttaaaaaaaaaagattctgcttataacttggtatttgtttataataaaaattatagtagccaataatgaacacttactctggcttggttatttacttaggtcaaaagaaggaggagcggttaaactgtgggatcaggaactgaggcggtgccgtgccttcaggcttgagacaggacaagccacagattgtgttcgttctgtgtgcagaggcaaagtaagatgttccatgagctgatacagtgcagcagaaaacagaaagtggttattactgtgattccctcaccctttgcagcctaatgaacaatacttaataatgcataacgatggatttgcttgccaacattactctgtctttgctgctttctttgccaaagttagcaccagtgtggtgcataagctaggaagctattctgtctaaatactgtatgtaaacctccaatattttctagaatctgccaatttaacaactctagtagacataattgaaagcccttggcagttgactcatattaggacagctgtctccattttttaaaaaaacacacattccctagataaaacgtgcagtaaacaaacaatgaaatactactcagccataaaaaataatgaaattctgtcattcttggtggcaacatggatgagactggaggacatgatgtgaagtgaaataagccaggcacagaaagataaatacatgttctcactcctgtgcagaaactaaaaaagttgatcccacagaggtggagagtagaatagtggttactggaggcggacaagggggagggggagggggatagggaaggactggttaaaggatacaagtttacacagccagataggaatagtatgttttagtattctgtagtactgtaggatgactatagttaagaatcacgtatttatgtattttcaggtatttacaagagaggattttgaaagtttccatcacaaagaaatgataaatgtctgaggtgatggttatgcgtattaccctatgccctatagatatgtataattatgtgtcaatttcaaaataaaaattcaaaactacaactcctatgaaaatttttgagcgtgtttgtacttattaagtgtatttataaatcatacggatattatcttcagcctgcatattaaattgtagttaagcttttactttttaactaaaaaataaattctattattttttcctatatcccactgcactgaccccagtttggaaatcctaagattatcaaataaaaactttgattattgaagaatccaggtgtactgccacagaaaagttctattctgtagcatggactctaatatgtaatctagcccattgtgcttacagatagatgtgtgcctgtagtcatagaaaaatttgcatgagctaatgactgccttgctactagattagctcaaagcaaaaagttctctgaaagcaggtcaatagggtcatttttatattatgaagaagaaaagcagctgttgtattacattcactgtattggtcctgcttgtgtttcagggcaagatccttgttgggacaaggaatgctgaaataatcgaagttggagagaaaaatgcagcttgtaatattttagttaacggtcatgtggatgggccaatctggggactagcaacacatccttccagggattttttcctttctgctgcagaagatgggacagtgagactttgggatattgctgataaagtaagtacagataatttttttaaaagaggttacaacttctaaaaagaaaagttggaagttctaaattgctagtacttaaagaactgccagaattctgttgagcattttgaggggaaactggtataatttagaagtacttcacttaatgtttcctatgactctttttttttttttttttaaatgcagaagatgttaaacaaagtgaatttgggacatgctgctcgtactgtgtgttacagccctgaaggggacatggtggctattggaatgaaaaatggagaatttatcattttactagtgagttctctaaaaatatggggaaagaagagagacaggagatgtgcaatccatgatatcaggttagtgaacaaatggaatagagtttctagtatatacttgatttaacttccatttgtaaaattttccatagccttgccttcaaaaagaggtccccagggcctgtagcatttcccgtattataaattgtatgctaaaatatggctgtttgtatactacttaattcttcttgctaaattataaacccactgggcaccaactataatagcaagtactagtaggtaatgtttgatgaattcatgttaacacttagccatgtccattaagttcatcccaccaagaggtatctcccactgtaatacaagagagctatctgcccttcaaaagttgtcaccctggaaaactaaagttgtgatttcaaacatatcttctcttagtaacctcagtttgggaatatgtagttcattaatttaatcaatacctattgattaaatgttccagaatccaaattaatttaaatgtttcttaaacctttgtttttcagtgcttaagcatttttcaacagtggctaccatttacggagtacttccgtgtgatcagtagataagattattgaatctaggtctgtcaaaagcttgtacacttttcatcagtaaaatccttttacaaatgaaaccttcctcagaacttcaatatataaaatagtaacagtggcttcccttagcttttacatgtctctatcgtacctcagtaagactcatgggccatttcaagagactgaattgtcccatatgactccaaagattgctaggcaaatagcatttcactttgtcttttaaataagttcttcaggccgggcgcggtggctcatgcctgtaatcccagcactttgggaggccgaggcaggcagatcacctgaagtcaggagtactcgaccagcctggccaacatagtgaaaccccatctcaactaaaaatacaaaaatcagccgggcgtggtggcaggcgcctgtaatcccagctactcagggggctgaaacaggagaatcgcttgaacccgggaggcggaggttgcgccatcgcactccagcctgggagacaagagcgagacttcgtctcaaaaaaaaaaaattcttcttccaagattcaagttgtgtcatttcaccttaataactggaggttagttaagctgggctgtgttctttgcttaatattaagacaacgttttttccagatggaagaaaactatcttaatgaattgttagcttattaattatgtaatgctaatggcttttaaaagctgagatgttctgactgggtgttgtggctcacacctgtaatcccagtaccttgggaggccaagggggaaggattgcttgaggccaggagtttgggaccatagtgagaccccgcctctatttaaaaaattaaattttgttttgttttgttttgagttggagttttgctcttgttgcccatgctgaagtgcaatggtgcaatctcagctcaccacaacctgtgcctcctgggttcaagcgattctcctgcttcagcctcccgagtagatgggattacaggcgtgcaccaccatgcctggctaattttgtatttttagtagagacagggtttctctatgttggtcaggctggtctcaaactctcgacctcaggtgatctgcccgcctccgcttcccaaagttctgggattataggtgtgagccactgggcctggcctaagaaagtttttttaagccattagacgtttttaaaggaattgggagatgacaattggggaaatatttaaaatttaagtaaaatataaagcttccttatttcatgtaacccagacaatctcagtatacatgatcagttgtgtctgacaggtaaatctatttgaggccttatcacacgttacttttaagaactagaaaggaaaagtcactgatcttaagtatttataatacttcatgtggtctaatactttttacgttttgttttgattcagatttagtccggattcccggtatctggcagtaggttctagtgagaactcagtggatttttatgacctaacgctgggccccactcttaacagaatcagctactgcaaagacattccaagctttgtcattcaaatggacttctctgcagatagcagttatctccaggtacagtaccaatactgtatacccaggtggcaagttcttctgcttttacatttcgtgttagtgaatgcatttaaagttcctgagctccagagctccagcttctcaactcctccctttgtaccttctgacctacagctcccctttcctcccccacttatcagagcttttctcctattaagtttttgtagtgatcttttgcatacttaataatgttagacatgtaaatcaagtagcaatatgctagtattctgtaaaccccctgtggattttgtctctcacctaatggaattcttgtcccattttaatctgatgaaaaaggtctctagtggctgctataaacggcatgtctatgaagtgccttcaggaaaacatcttatggatcatgccgctattgacagaattacttgggctacatggactaggtaaatacttatatattcacaaggcaagaactgactttgaaggccagttagaaaatcctatttctgaactgttagagccattccaataaggaatagtaattgagtttcaagtttttgttaccatattttgaaatggtatgttcatgttgggacccctttttattgaatatatttccatgttttatcagtttccatgatttatcaagttttttttttaaggaaatcaaagttttaactttaaagataccctgatatttttcttaatgctaaatttaatgactggcaaaaaggtattgggtgctgttaagcaactgttattaattctctatctaaaggaatgctatcttgaatctattagaagtcaaagcttccaaatttgttcaaatttcctggctgtatgacaggtaaccatgactatccatttttttggccaatgaaaaatgccatcaaattcctgtatcagccaggcatatagtggctcatgcctgtaatctctgatgtagcaggccgaggtgggaggatcacttgagcctagaagttttgataccagcctgggcaacatagcaagaccccatctctgaaatttttttaattcctatgtcataagtcatttttatttttgtagagatagggatctcacaatattgcccaggctggtctcaaactcttggcctcaagcagtcctcctgcctcagcctcccaaaatgttgggattactggtatgtgctgctggacccagccaagtagcacttttaatttgaaaaatagttctatcagttttcagtcaggcgcggtggctcagcctgtaatcccagcactttgggaggccgagcgggggtgatcacctgaggtcgggagttcgagactagcctgaccaacatggagaaaccctgtctctactaaaaatacaaaataagccgggcatgttagcgcatgcctgtgatcccagctactcgggaggctgaggcaggagaattgcttgaacccaggaggcagaggttgcggtgagccgagatcatgccattgcactccagcctgggtaacaagagcgaaaactccgtctcaaaaaaaaaaaaagaaaaaatagttctatcagttttcataaagtactactttaatcttaaaaagattaatctagaaacccttcaaattataaaatgtcatttttaaaaggcaggagttgatatcctgatgaaattcaggtctccaaacaacttaccataatttacttcctgtattttaagtaacatgatagggtacttagagattaattgccaagaaactttttgaatatagtcaacctgcccgcacttgccatgatgagttttcttttgttccttccctctagtattctaggagatgaggttttgggaatctggtccagacatgctgagaaagctgatgtcaactgtgcctgtgtatctcattcaggaatcagtcttgttacaggagatgactttggcatggttaagttatttgacttcccatgtccagaaaaatttgtaagtttgtgttttgtttactattatcagtttactcctaattttgatgtcttatcatcagcacttttccccatatatttaaaatgttttgtcctaatttctaaatttttccccaaactttctaaatctatttactttgaaataaaagctattagaaacaaatcctctccctcgagtaataccatctttggaaccatcctacaaaagctgtaattagcttttcaccaaacctataatcagttatcaaatttcaaatgcttttccttagagaaaaatggtcagagtacctggagacatctgactgcccacacagcctggttttgcagatccactactcatgctgaaaagcattctaatcactggctgcggtgctaactccctactctctccacagctcttgtcatagagattatagttcctaataagagcctttgacttctgtgtgcaccaaatgccctgagcttgtctgtcattgttttttaggcaaaacacaaaaggttcttgggtcattcgccccatgtgacaaatattcgatttaccagtggtgatcgacatgttgttagtgctggaggtgatgactgcaggttagtaactttctcagcccatgaagagcagactatgttactagttaagagacttaatacaacaactcctacagctttggtttatgaaatcagctagtcaacattagtagaaggtagtataaccagatggctcttcagaatctcatatttatgcaaatacagaataaaaggagttaaagaggaaaaatattacacatgtaacctgaaagcacaactgaaaaatattaaactgttatgaaaatctaaaaacataattaactccctgcaattttcttctctgattgcagcttatttgtctggaaatgtgtacatacacctcactgagagatgctgagatgactacagaaattaactttgagaccagaattacagagaagaaaaaccaaaacccaaccctgcatggtcaagtggtgctaacccaagactgtaacagggagaaatgcccagaatcatcaaaatagtgaaagactgatctgttcaaaatatttgctatatgcactgggtataatccgtaatccatacactgccagataatgccatttcaaggaaggatcgaatacttgatggtaaaggccaagtccccctgtattgggaagtgtgtgatttcggcagacctgctgggaaaatttagggtagagcactctttacagaagaactcaaaaacccaatttggataattttcattatctttttagcaaaatggtttcttaatgtttatattttattttcaaggttcattgtttaatgaaatattttattcttgcatttccataaggaaagggaaagtcatgatcatcctaaaggatcacagtttttaaaaggcaaacattttccctaaggaaacagacacaagctttcctagagaatatgatgttttttaggcattaataaggtccttttttataaaggacacttttctcctagtagttttgaattcaggaacagatccaaagttagcagtatatggctgctacatttccattttcattttcgagccatcagtttatgttcagatgccatctctgtaatcgcacatttaaaacataactgtagcctcactaatggaaaagtagtatgatgaacaatcattcccaatggtgtacaatgtaagggttttagggagcaacagtatttaactggaagaaagaattgcatatttaatgtagtctaatatatacacatttgtttaacatgtaaacaaaagtgttaaattcacatatacaacattatacaatttaatcactcttggaataaaatttttatagccttttttctattgggaaaatttgtttagatgtgtgccactccataggtttatttccaaaatgaatgagcccaactccatttgtaaaaacttgtcagttagaattcctttttttagtggattagggctgaattcttagatccttatttcttttcactttaaatgctgccaaagatcactactcatcattcaggaattcgctgtctagcctatctgtagtttcctgaagattgaaaattatgtagactgctatttaaaaatatatttttctaagtgtgaggtttaagatgctgtattgaccctatgagtttttaatgtgttaattatctttatagcataatagatcgctttaggttcctggaatcccatttggtctgacaggatatatgaagattcttaatacctattttctgtgtctaatacttggttaatactaaaaatagaaatgactaaattacatcacagaaagcataaccagtgattgaacctggtagttttaaagctctaaatagctgtggctgaaggactgattatggggctaagaagcttgaaacgtaagttggtacttgttcatcagtggattctcctaaattaagccaaattttgaaatacatgactattaagtttctactcatgtatttacagtcagtcaataaattaaaggaggaaaaaaatccctgaacaacctgcccataaaaagaaaaatactctacatttgagcctgctgcagttttaaattttccctctgggtcaagtttgccagcttttggctacagagaaattatatttccattacagtgcaggtagaaactctgtaaccttaagcatgtaaactacatagaataaaactgtttccactgcatttctgtccttcaaagtggccaacctgattaagtcagccttaatcactgctgctgtcagtttcacgactaaaggtcatattgactaagtagtcatcagctgaccacctcgctgtatcagccagcaacgaggggaaggtgaagaaacatgataggccatatagaatctgccctatgtttacttttttaacccagataattatttttgtgtgcagtatctaagctcctgattgtgtaacctgggacttctggcaccttttgttccattcattttatgtataaaatgcatgccaaagcacactgtgccctctggtacccttgcttccaatcgccaaccatgctcatttccttcctttttttgtggtccctttttgtggtgatcattttaaaccacgtcatccaacaaatgttttatggtcaaccttagcttgttcataagccatagcaactgaaagattaaactcttaaatatgtgtctgggcagtggctattaaatagcaaaaaacaatcagattttagtattttattatttccttgtaaaatggctgaactaaattaaacccttgtttcccatttgttctataatttatagtgaaactgagaacaaaactatctttataaatgatagctaaaagtatttccagatatttaaacaatttaaaataaatttcttctgcagagatgcaaagcatctcaacactggaatgaacaaatgccttaaattcaatggagtaaacctttagaatgaagaggaactgtcatttcacccaagccgaagacaacagccttatgcacttgtgtgctctgtctttgctgcttctcgtgtttcaagcctttcctgtgggatcagcacagcaaagtgcaacttaccaaatggtttaatgactggttaattctttcttctcccaatggaaaagcaatggcaacacaacagtagactgctggcttgacaatcttaaacgtgagcctttgcacatgtaggtttatcatcatttgagtatacgactaagcaagtcaatgaactttttttttttttttagcagtttaatttggtcctgagaatgttgcagtctttattaccccttttgcattaatccacttttctaaccaccttttaagctttaatttttaacactatacaccaagtctttgaaatcagtgatctgttatttaactctaaagcatttgacacttcttgccttaacagttttaaaaaccacacacaaaaaaactctgtaagtaatacagtaggccaaaagtttcatcctatctatcttgcagtttacctatctgatctgatctctgtaattatagttctgtcatttaaaatatactatttaaatctaatttttacatttcaaaaattatcttcagtagtaactaagtatattttctgtggattctgagaatgttatttttcagaatgtgagaatatatatgtacatttataatcttgtgactttaaagtctgttttcagatacagtatgtaaatacttgtaaaaaaatttgtataattttgtgataatgtagtttcccaaaaaaattatttagaaggcattatgttattagtaaatgagagcactgtatagaactgttcctattttctgcacttgccattccagctgcctccactgtccatacccacctcattcatcctgtcacagaaggcaggaaaactgggaactttaccaaagtagcactcagcctgagaggcctgtataatcatgcttttcaaactaaattcacttaaaaattaaaaagcagaattgaatattttaagcagcctcagtacctttggccaatgctgttttcatggtggattatgaacattatataatctttgggaaaagtgaaagtagtacaatttttagaataatgacaactgcctcactgcatctctccactcacacagcaaccgtgtagccccctaagctgcagtaccatgactaaccatgatgtcaatttcatatgctgatcctcacaacagcagtgcacaaacatgccccaaatattttaacagaatttagctcttccttaagctgtcttttcatagtaaaaacaaaacaaaaacacccaatgttaaaaccacataataaacttacaaacttgaaaaattagacacttcagatagataggcaataaaacttcatattatgaaagcaatatattccaagtttcaaagatttgacaagttctgtagagtatctttcatcagtacatgaaaacttccaaactgcatgatcttctgccaggcaggactgggtgctattcgctggtttgaggtcgaatccatttcaaggcatgtcgtggtgggacattaatggtgggatggtagaatgtgcagtccggtcttgtacattgagtgttaaacctacaatgttttggatgatagaagggacattccatcttcttacaagcagggaagtaacggcagagctgactactggaaggtggtgctggtggtgcaactgctggttttggagacagtactggaattcttctactcacatgagtgaagggacaatctggtttagtacactttgcatcatatttacaatttgggtgaacaaacaaacatttttcagcaaatttacaattggggaaggctttgcagggtgagatggggtgatggtaggcacactcatccccatttttacaagcaggccagtacttgcagcgctccaaaagtttttctggtttctgtgccacactcagttcactcatctcagcttgactcatctgcagagtttctgccattactgggtcgatttgcagtcgggataataattgcctctgttgagttccttgatttttttctacagaatctccttttgtttcctcttctttaatggggggacttattctgggggtcctactttgtccctggaccacttctgctagcaattcttcttgagaagttcgagttctgggagcaactggaagtgtctgtttctgtggaactgtagagtagttagttgtttttgttacggattcttgagcttcagatatagccttcaaaatcagattcttgttagcttgtttagaaggtggaagagaaggtctcctttcaggctttgcaggcacagacacactgctggagatgcttcctgttcgagacccgtaatcatcatcttcttcctcctcttctccatcatgattgaatttttttactttaacaactgaacttaccacaggcaactttctcttccgaaagttttcatcctccatactcattttctccgagttgtttctaaagaacggactatacgtttcttctaagctgttaagcacctctggttcacacaaacgtcctgtttcatatacccaactactctgcatatcaagctgcttggcagcatgaatactattctgctgctgttgaaattgcaacctgtttaaatgaacaccactatctgcatttctacttgcaggtggtcgataaatttcaatagaagggcgagaagaaccatatgtaagtgtcactgtaggttttttctgagataagggattctcctgcacaaagttgaggtcttcgtcaatgagatcatctggttctggcttaatatcaatcacatcttcagagggtgctggctccctcaaaggtttcactgttgacattagtcgggttgcagctccatcatcgtaagtctgtctgacatttgtggtttttgactcctgcgaacttgtagaaactctggaatctcttttttcaggtctcgcgctaggaatggcaagtggtggcactgcagcttcatgcctcctctcatctccccgactgaaattgctcttgtttgaaggcacgttactatcaaagatgttggtatcagaagacttcagactagagggttcagttgtaacagagcgaagtttatctaatacaccatgaagccatacggtgaatcgaattgtgttgttccctagaaacagggacagatcctctgtcatttggtcctgacttttcttgttggccaccatcaccataatgtaatcaggaagttcttcatcaacataagctcctaattcttgtaatttccccttaatggcactctcccgcagcggatccaaagcggcgccgtgcgccgcggtggtggctccagccgggcctgcgcctgtccttccatttcccggcggctacttcagccgcagccacgctccg

SEQ ID NO: 17457 - RNA, 13293 nt, Homo sapiens
  source 1..13293: mol_type = other RNA
tcaggccaggcacagtggctcatacctggaatcccagcactttgggaggccgaggcaggcagatcacctgaggtcaaggtatttgagaccagcctggccaacatggtgaaaccccatctctactaaaaatacagaaattagctgggtgtggtggtgcacacctgtaatgctagctactcgggaggctgaggtaggagaatcgcttgaacctgggaggcagaggttgcaataagcctagatcatgccactgcactcaagcctgggagacagagcgagactacatcttaaaaaaaaaaaaaaaagtattatgagagaggataatgtattgtaatgtattgtagaggctaaataaaattatgctcatgtcagaaaaaaagagtatttctcaaaataaaattcactgaaactggatgtttattttgactgagatatagtatatcctcaaattgccatagaaagtttacaagaatattagaggtaaattataaatatcagggcctttttaaaaaaaaaagattctgcttataacttggtatttgtttataataaaaattatagtagccaataatgaacacttactctggcttggttatttacttaggtcaaaagaaggaggagcggttaaactgtgggatcaggaactgaggcggtgccgtgccttcaggcttgagacaggacaagccacagattgtgttcgttctgtgtgcagaggcaaagtaagatgttccatgagctgatacagtgcagcagaaaacagaaagtggttattactgtgattccctcaccctttgcagcctaatgaacaatacttaataatgcataacgatggatttgcttgccaacattactctgtctttgctgctttctttgccaaagttagcaccagtgtggtgcataagctaggaagctattctgtctaaatactgtatgtaaacctccaatattttctagaatctgccaatttaacaactctagtagacataattgaaagcccttggcagttgactcatattaggacagctgtctccattttttaaaaaaacacacattccctagataaaacgtgcagtaaacaaacaatgaaatactactcagccataaaaaataatgaaattctgtcattcttggtggcaacatggatgagactggaggacatgatgtgaagtgaaataagccaggcacagaaagataaatacatgttctcactcctgtgcagaaactaaaaaagttgatcccacagaggtggagagtagaatagtggttactggaggcggacaagggggagggggagggggatagggaaggactggttaaaggatacaagtttacacagccagataggaatagtatgttttagtattctgtagtactgtaggatgactatagttaagaatcacgtatttatgtattttcaggtatttacaagagaggattttgaaagtttccatcacaaagaaatgataaatgtctgaggtgatggttatgcgtattaccctatgccctatagatatgtataattatgtgtcaatttcaaaataaaaattcaaaactacaactcctatgaaaatttttgagcgtgtttgtacttattaagtgtatttataaatcatacggatattatcttcagcctgcatattaaattgtagttaagcttttactttttaactaaaaaataaattctattattttttcctatatcccactgcactgaccccagtttggaaatcctaagattatcaaataaaaactttgattattgaagaatccaggtgtactgccacagaaaagttctattctgtagcatggactctaatatgtaatctagcccattgtgcttacagatagatgtgtgcctgtagtcatagaaaaatttgcatgagctaatgactgccttgctactagattagctcaaagcaaaaagttctctgaaagcaggtcaatagggtcatttttatattatgaagaagaaaagcagctgttgtattacattcactgtattggtcctgcttgtgtttcagggcaagatccttgttgggacaaggaatgctgaaataatcgaagttggagagaaaaatgcagcttgtaatattttagttaacggtcatgtggatgggccaatctggggactagcaacacatccttccagggattttttcctttctgctgcagaagatgggacagtgagactttgggatattgctgataaagtaagtacagataatttttttaaaagaggttacaacttctaaaaagaaaagttggaagttctaaattgctagtacttaaagaactgccagaattctgttgagcattttgaggggaaactggtataatttagaagtacttcacttaatgtttcctatgactctttttttttttttttttaaatgcagaagatgttaaacaaagtgaatttgggacatgctgctcgtactgtgtgttacagccctgaaggggacatggtggctattggaatgaaaaatggagaatttatcattttactagtgagttctctaaaaatatggggaaagaagagagacaggagatgtgcaatccatgatatcaggttagtgaacaaatggaatagagtttctagtatatacttgatttaacttccatttgtaaaattttccatagccttgccttcaaaaagaggtccccagggcctgtagcatttcccgtattataaattgtatgctaaaatatggctgtttgtatactacttaattcttcttgctaaattataaacccactgggcaccaactataatagcaagtactagtaggtaatgtttgatgaattcatgttaacacttagccatgtccattaagttcatcccaccaagaggtatctcccactgtaatacaagagagctatctgcccttcaaaagttgtcaccctggaaaactaaagttgtgatttcaaacatatcttctcttagtaacctcagtttgggaatatgtagttcattaatttaatcaatacctattgattaaatgttccagaatccaaattaatttaaatgtttcttaaacctttgtttttcagtgcttaagcatttttcaacagtggctaccatttacggagtacttccgtgtgatcagtagataagattattgaatctaggtctgtcaaaagcttgtacacttttcatcagtaaaatccttttacaaatgaaaccttcctcagaacttcaatatataaaatagtaacagtggcttcccttagcttttacatgtctctatcgtacctcagtaagactcatgggccatttcaagagactgaattgtcccatatgactccaaagattgctaggcaaatagcatttcactttgtcttttaaataagttcttcaggccgggcgcggtggctcatgcctgtaatcccagcactttgggaggccgaggcaggcagatcacctgaagtcaggagtactcgaccagcctggccaacatagtgaaaccccatctcaactaaaaatacaaaaatcagccgggcgtggtggcaggcgcctgtaatcccagctactcagggggctgaaacaggagaatcgcttgaacccgggaggcggaggttgcgccatcgcactccagcctgggagacaagagcgagacttcgtctcaaaaaaaaaaaattcttcttccaagattcaagttgtgtcatttcaccttaataactggaggttagttaagctgggctgtgttctttgcttaatattaagacaacgttttttccagatggaagaaaactatcttaatgaattgttagcttattaattatgtaatgctaatggcttttaaaagctgagatgttctgactgggtgttgtggctcacacctgtaatcccagtaccttgggaggccaagggggaaggattgcttgaggccaggagtttgggaccatagtgagaccccgcctctatttaaaaaattaaattttgttttgttttgttttgagttggagttttgctcttgttgcccatgctgaagtgcaatggtgcaatctcagctcaccacaacctgtgcctcctgggttcaagcgattctcctgcttcagcctcccgagtagatgggattacaggcgtgcaccaccatgcctggctaattttgtatttttagtagagacagggtttctctatgttggtcaggctggtctcaaactctcgacctcaggtgatctgcccgcctccgcttcccaaagttctgggattataggtgtgagccactgggcctggcctaagaaagtttttttaagccattagacgtttttaaaggaattgggagatgacaattggggaaatatttaaaatttaagtaaaatataaagcttccttatttcatgtaacccagacaatctcagtatacatgatcagttgtgtctgacaggtaaatctatttgaggccttatcacacgttacttttaagaactagaaaggaaaagtcactgatcttaagtatttataatacttcatgtggtctaatactttttacgttttgttttgattcagatttagtccggattcccggtatctggcagtaggttctagtgagaactcagtggatttttatgacctaacgctgggccccactcttaacagaatcagctactgcaaagacattccaagctttgtcattcaaatggacttctctgcagatagcagttatctccaggtacagtaccaatactgtatacccaggtggcaagttcttctgcttttacatttcgtgttagtgaatgcatttaaagttcctgagctccagagctccagcttctcaactcctccctttgtaccttctgacctacagctcccctttcctcccccacttatcagagcttttctcctattaagtttttgtagtgatcttttgcatacttaataatgttagacatgtaaatcaagtagcaatatgctagtattctgtaaaccccctgtggattttgtctctcacctaatggaattcttgtcccattttaatctgatgaaaaaggtctctagtggctgctataaacggcatgtctatgaagtgccttcaggaaaacatcttatggatcatgccgctattgacagaattacttgggctacatggactaggtaaatacttatatattcacaaggcaagaactgactttgaaggccagttagaaaatcctatttctgaactgttagagccattccaataaggaatagtaattgagtttcaagtttttgttaccatattttgaaatggtatgttcatgttgggacccctttttattgaatatatttccatgttttatcagtttccatgatttatcaagttttttttttaaggaaatcaaagttttaactttaaagataccctgatatttttcttaatgctaaatttaatgactggcaaaaaggtattgggtgctgttaagcaactgttattaattctctatctaaaggaatgctatcttgaatctattagaagtcaaagcttccaaatttgttcaaatttcctggctgtatgacaggtaaccatgactatccatttttttggccaatgaaaaatgccatcaaattcctgtatcagccaggcatatagtggctcatgcctgtaatctctgatgtagcaggccgaggtgggaggatcacttgagcctagaagttttgataccagcctgggcaacatagcaagaccccatctctgaaatttttttaattcctatgtcataagtcatttttatttttgtagagatagggatctcacaatattgcccaggctggtctcaaactcttggcctcaagcagtcctcctgcctcagcctcccaaaatgttgggattactggtatgtgctgctggacccagccaagtagcacttttaatttgaaaaatagttctatcagttttcagtcaggcgcggtggctcagcctgtaatcccagcactttgggaggccgagcgggggtgatcacctgaggtcgggagttcgagactagcctgaccaacatggagaaaccctgtctctactaaaaatacaaaataagccgggcatgttagcgcatgcctgtgatcccagctactcgggaggctgaggcaggagaattgcttgaacccaggaggcagaggttgcggtgagccgagatcatgccattgcactccagcctgggtaacaagagcgaaaactccgtctcaaaaaaaaaaaaagaaaaaatagttctatcagttttcataaagtactactttaatcttaaaaagattaatctagaaacccttcaaattataaaatgtcatttttaaaaggcaggagttgatatcctgatgaaattcaggtctccaaacaacttaccataatttacttcctgtattttaagtaacatgatagggtacttagagattaattgccaagaaactttttgaatatagtcaacctgcccgcacttgccatgatgagttttcttttgttccttccctctagtattctaggagatgaggttttgggaatctggtccagacatgctgagaaagctgatgtcaactgtgcctgtgtatctcattcaggaatcagtcttgttacaggagatgactttggcatggttaagttatttgacttcccatgtccagaaaaatttgtaagtttgtgttttgtttactattatcagtttactcctaattttgatgtcttatcatcagcacttttccccatatatttaaaatgttttgtcctaatttctaaatttttccccaaactttctaaatctatttactttgaaataaaagctattagaaacaaatcctctccctcgagtaataccatctttggaaccatcctacaaaagctgtaattagcttttcaccaaacctataatcagttatcaaatttcaaatgcttttccttagagaaaaatggtcagagtacctggagacatctgactgcccacacagcctggttttgcagatccactactcatgctgaaaagcattctaatcactggctgcggtgctaactccctactctctccacagctcttgtcatagagattatagttcctaataagagcctttgacttctgtgtgcaccaaatgccctgagcttgtctgtcattgttttttaggcaaaacacaaaaggttcttgggtcattcgccccatgtgacaaatattcgatttaccagtggtgatcgacatgttgttagtgctggaggtgatgactgcaggttagtaactttctcagcccatgaagagcagactatgttactagttaagagacttaatacaacaactcctacagctttggtttatgaaatcagctagtcaacattagtagaaggtagtataaccagatggctcttcagaatctcatatttatgcaaatacagaataaaaggagttaaagaggaaaaatattacacatgtaacctgaaagcacaactgaaaaatattaaactgttatgaaaatctaaaaacataattaactccctgcaattttcttctctgattgcagcttatttgtctggaaatgtgtacatacacctcactgagagatgctgagatgactacagaaattaactttgagaccagaattacagagaagaaaaaccaaaacccaaccctgcatggtcaagtggtgctaacccaagactgtaacagggagaaatgcccagaatcatcaaaatagtgaaagactgatctgttcaaaatatttgctatatgcactgggtataatccgtaatccatacactgccagataatgccatttcaaggaaggatcgaatacttgatggtaaaggccaagtccccctgtattgggaagtgtgtgatttcggcagacctgctgggaaaatttagggtagagcactctttacagaagaactcaaaaacccaatttggataattttcattatctttttagcaaaatggtttcttaatgtttatattttattttcaaggttcattgtttaatgaaatattttattcttgcatttccataaggaaagggaaagtcatgatcatcctaaaggatcacagtttttaaaaggcaaacattttccctaaggaaacagacacaagctttcctagagaatatgatgttttttaggcattaataaggtccttttttataaaggacacttttctcctagtagttttgaattcaggaacagatccaaagttagcagtatatggctgctacatttccattttcattttcgagccatcagtttatgttcagatgccatctctgtaatcgcacatttaaaacataactgtagcctcactaatggaaaagtagtatgatgaacaatcattcccaatggtgtacaatgtaagggttttagggagcaacagtatttaactggaagaaagaattgcatatttaatgtagtctaatatatacacatttgtttaacatgtaaacaaaagtgttaaattcacatatacaacattatacaatttaatcactcttggaataaaatttttatagccttttttctattgggaaaatttgtttagatgtgtgccactccataggtttatttccaaaatgaatgagcccaactccatttgtaaaaacttgtcagttagaattcctttttttagtggattagggctgaattcttagatccttatttcttttcactttaaatgctgccaaagatcactactcatcattcaggaattcgctgtctagcctatctgtagtttcctgaagattgaaaattatgtagactgctatttaaaaatatatttttctaagtgtgaggtttaagatgctgtattgaccctatgagtttttaatgtgttaattatctttatagcataatagatcgctttaggttcctggaatcccatttggtctgacaggatatatgaagattcttaatacctattttctgtgtctaatacttggttaatactaaaaatagaaatgactaaattacatcacagaaagcataaccagtgattgaacctggtagttttaaagctctaaatagctgtggctgaaggactgattatggggctaagaagcttgaaacgtaagttggtacttgttcatcagtggattctcctaaattaagccaaattttgaaatacatgactattaagtttctactcatgtatttacagtcagtcaataaattaaaggaggaaaaaaatccctgaacaacctgcccataaaaagaaaaatactctacatttgagcctgctgcagttttaaattttccctctgggtcaagtttgccagcttttggctacagagaaattatatttccattacagtgcaggtagaaactctgtaaccttaagcatgtaaactacatagaataaaactgtttccactgcatttctgtccttcaaagtggccaacctgattaagtcagccttaatcactgctgctgtcagtttcacgactaaaggtcatattgactaagtagtcatcagctgaccacctcgctgtatcagccagcaacgaggggaaggtgaagaaacatgataggccatatagaatctgccctatgtttacttttttaacccagataattatttttgtgtgcagtatctaagctcctgattgtgtaacctgggacttctggcaccttttgttccattcattttatgtataaaatgcatgccaaagcacactgtgccctctggtacccttgcttccaatcgccaaccatgctcatttccttcctttttttgtggtccctttttgtggtgatcattttaaaccacgtcatccaacaaatgttttatggtcaaccttagcttgttcataagccatagcaactgaaagattaaactcttaaatatgtgtctgggcagtggctattaaatagcaaaaaacaatcagattttagtattttattatttccttgtaaaatggctgaactaaattaaacccttgtttcccatttgttctataatttatagtgaaactgagaacaaaactatctttataaatgatagctaaaagtatttccagatatttaaacaatttaaaataaatttcttctgcagagatgcaaagcatctcaacactggaatgaacaaatgccttaaattcaatggagtaaacctttagaatgaagaggaactgtcatttcacccaagccgaagacaacagccttatgcacttgtgtgctctgtctttgctgcttctcgtgtttcaagcctttcctgtgggatcagcacagcaaagtgcaacttaccaaatggtttaatgactggttaattctttcttctcccaatggaaaagcaatggcaacacaacagtagactgctggcttgacaatcttaaacgtgagcctttgcacatgtaggtttatcatcatttgagtatacgactaagcaagtcaatgaactttttttttttttttagcagtttaatttggtcctgagaatgttgcagtctttattaccccttttgcattaatccacttttctaaccaccttttaagctttaatttttaacactatacaccaagtctttgaaatcagtgatctgttatttaactctaaagcatttgacacttcttgccttaacagttttaaaaaccacacacaaaaaaactctgtaagtaatacagtaggccaaaagtttcatcctatctatcttgcagtttacctatctgatctgatctctgtaattatagttctgtcatttaaaatatactatttaaatctaatttttacatttcaaaaattatcttcagtagtaactaagtatattttctgtggattctgagaatgttatttttcagaatgtgagaatatatatgtacatttataatcttgtgactttaaagtctgttttcagatacagtatgtaaatacttgtaaaaaaatttgtataattttgtgataatgtagtttcccaaaaaaattatttagaaggcattatgttattagtaaatgagagcactgtatagaactgttcctattttctgcacttgccattccagctgcctccactgtccatacccacctcattcatcctgtcacagaaggcaggaaaactgggaactttaccaaagtagcactcagcctgagaggcctgtataatcatgcttttcaaactaaattcacttaaaaattaaaaagcagaattgaatattttaagcagcctcagtacctttggccaatgctgttttcatggtggattatgaacattatataatctttgggaaaagtgaaagtagtacaatttttagaataatgacaactgcctcactgcatctctccactcacacagcaaccgtgtagccccctaagctgcagtaccatgactaaccatgatgtcaatttcatatgctgatcctcacaacagcagtgcacaaacatgccccaaatattttaacagaatttagctcttccttaagctgtcttttcatagtaaaaacaaaacaaaaacacccaatgttaaaaccacataataaacttacaaacttgaaaaattagacacttcagatagataggcaataaaacttcatattatgaaagcaatatattccaagtttcaaagatttgacaagttctgtagagtatctttcatcagtacatgaaaacttccaaactgcatgatcttctgccaggcaggactgggtgctattcgctggtttgaggtcgaatccatttcaaggcatgtcgtggtgggacattaatggtgggatggtagaatgtgcagtccggtcttgtacattgagtgttaaacctacaatgttttggatgatagaagggacattccatcttcttacaagcagggaagtaacggcagagctgactactggaaggtggtgctggtggtgcaactgctggttttggagacagtactggaattcttctactcacatgagtgaagggacaatctggtttagtacactttgcatcatatttacaatttgggtgaacaaacaaacatttttcagcaaatttacaattggggaaggctttgcagggtgagatggggtgatggtaggcacactcatccccatttttacaagcaggccagtacttgcagcgctccaaaagtttttctggtttctgtgccacactcagttcactcatctcagcttgatttttttctacagaatctccttttgtttcctcttctttaatggggggacttattctgggggtcctactttgtccctggaccacttctgctagcaattcttcttgagaagttcgagttctgggagcaactggaagtgtctgtttctgtggaactgtagagtagttagttgtttttgttacggattcttgagcttcagatatagccttcaaaatcagattcttgttagcttgtttagaaggtggaagagaaggtctcctttcaggctttgcaggcacagacacactgctggagatgcttcctgttcgagacccgtaatcatcatcttcttcctcctcttctccatcatgattgaatttttttactttaacaactgaacttaccacaggcaactttctcttccgaaagttttcatcctccatactcattttctccgagttgtttctaaagaacggactatacgtttcttctaagctgttaagcacctctggttcacacaaacgtcctgtttcatatacccaactactctgcatatcaagctgcttggcagcatgaatactattctgctgctgttgaaattgcaacctgtttaaatgaacaccactatctgcatttctacttgcaggtggtcgataaatttcaatagaagggcgagaagaaccatatgtaagtgtcactgtaggttttttctgagataagggattctcctgcacaaagttgaggtcttcgtcaatgagatcatctggttctggcttaatatcaatcacatcttcagagggtgctggctccctcaaaggtttcactgttgacattagtcgggttgcagctccatcatcgtaagtctgtctgacatttgtggtttttgactcctgcgaacttgtagaaactctggaatctcttttttcaggtctcgcgctaggaatggcaagtggtggcactgcagcttcatgcctcctctcatctccccgactgaaattgctcttgtttgaaggcacgttactatcaaagatgttggtatcagaagacttcagactagagggttcagttgtaacagagcgaagtttatctaatacaccatgaagccaacataagctcctaattcttgtaatttccccttaatggcactccggatcttgcggctgatctcggtgccgatctccatggctctgcggcgtgcgggaactcagcactgcgcggcgcttggcttacccggaggctgccgcggactcctaccccgcagccgggacaccaccgcctcc

SEQ ID NO: 17458 - RNA, 13408 nt, Homo sapiens
  source 1..13408: mol_type = other RNA
tcaggccaggcacagtggctcatacctggaatcccagcactttgggaggccgaggcaggcagatcacctgaggtcaaggtatttgagaccagcctggccaacatggtgaaaccccatctctactaaaaatacagaaattagctgggtgtggtggtgcacacctgtaatgctagctactcgggaggctgaggtaggagaatcgcttgaacctgggaggcagaggttgcaataagcctagatcatgccactgcactcaagcctgggagacagagcgagactacatcttaaaaaaaaaaaaaaaagtattatgagagaggataatgtattgtaatgtattgtagaggctaaataaaattatgctcatgtcagaaaaaaagagtatttctcaaaataaaattcactgaaactggatgtttattttgactgagatatagtatatcctcaaattgccatagaaagtttacaagaatattagaggtaaattataaatatcagggcctttttaaaaaaaaaagattctgcttataacttggtatttgtttataataaaaattatagtagccaataatgaacacttactctggcttggttatttacttaggtcaaaagaaggaggagcggttaaactgtgggatcaggaactgaggcggtgccgtgccttcaggcttgagacaggacaagccacagattgtgttcgttctgtgtgcagaggcaaagtaagatgttccatgagctgatacagtgcagcagaaaacagaaagtggttattactgtgattccctcaccctttgcagcctaatgaacaatacttaataatgcataacgatggatttgcttgccaacattactctgtctttgctgctttctttgccaaagttagcaccagtgtggtgcataagctaggaagctattctgtctaaatactgtatgtaaacctccaatattttctagaatctgccaatttaacaactctagtagacataattgaaagcccttggcagttgactcatattaggacagctgtctccattttttaaaaaaacacacattccctagataaaacgtgcagtaaacaaacaatgaaatactactcagccataaaaaataatgaaattctgtcattcttggtggcaacatggatgagactggaggacatgatgtgaagtgaaataagccaggcacagaaagataaatacatgttctcactcctgtgcagaaactaaaaaagttgatcccacagaggtggagagtagaatagtggttactggaggcggacaagggggagggggagggggatagggaaggactggttaaaggatacaagtttacacagccagataggaatagtatgttttagtattctgtagtactgtaggatgactatagttaagaatcacgtatttatgtattttcaggtatttacaagagaggattttgaaagtttccatcacaaagaaatgataaatgtctgaggtgatggttatgcgtattaccctatgccctatagatatgtataattatgtgtcaatttcaaaataaaaattcaaaactacaactcctatgaaaatttttgagcgtgtttgtacttattaagtgtatttataaatcatacggatattatcttcagcctgcatattaaattgtagttaagcttttactttttaactaaaaaataaattctattattttttcctatatcccactgcactgaccccagtttggaaatcctaagattatcaaataaaaactttgattattgaagaatccaggtgtactgccacagaaaagttctattctgtagcatggactctaatatgtaatctagcccattgtgcttacagatagatgtgtgcctgtagtcatagaaaaatttgcatgagctaatgactgccttgctactagattagctcaaagcaaaaagttctctgaaagcaggtcaatagggtcatttttatattatgaagaagaaaagcagctgttgtattacattcactgtattggtcctgcttgtgtttcagggcaagatccttgttgggacaaggaatgctgaaataatcgaagttggagagaaaaatgcagcttgtaatattttagttaacggtcatgtggatgggccaatctggggactagcaacacatccttccagggattttttcctttctgctgcagaagatgggacagtgagactttgggatattgctgataaagtaagtacagataatttttttaaaagaggttacaacttctaaaaagaaaagttggaagttctaaattgctagtacttaaagaactgccagaattctgttgagcattttgaggggaaactggtataatttagaagtacttcacttaatgtttcctatgactctttttttttttttttttaaatgcagaagatgttaaacaaagtgaatttgggacatgctgctcgtactgtgtgttacagccctgaaggggacatggtggctattggaatgaaaaatggagaatttatcattttactagtgagttctctaaaaatatggggaaagaagagagacaggagatgtgcaatccatgatatcaggttagtgaacaaatggaatagagtttctagtatatacttgatttaacttccatttgtaaaattttccatagccttgccttcaaaaagaggtccccagggcctgtagcatttcccgtattataaattgtatgctaaaatatggctgtttgtatactacttaattcttcttgctaaattataaacccactgggcaccaactataatagcaagtactagtaggtaatgtttgatgaattcatgttaacacttagccatgtccattaagttcatcccaccaagaggtatctcccactgtaatacaagagagctatctgcccttcaaaagttgtcaccctggaaaactaaagttgtgatttcaaacatatcttctcttagtaacctcagtttgggaatatgtagttcattaatttaatcaatacctattgattaaatgttccagaatccaaattaatttaaatgtttcttaaacctttgtttttcagtgcttaagcatttttcaacagtggctaccatttacggagtacttccgtgtgatcagtagataagattattgaatctaggtctgtcaaaagcttgtacacttttcatcagtaaaatccttttacaaatgaaaccttcctcagaacttcaatatataaaatagtaacagtggcttcccttagcttttacatgtctctatcgtacctcagtaagactcatgggccatttcaagagactgaattgtcccatatgactccaaagattgctaggcaaatagcatttcactttgtcttttaaataagttcttcaggccgggcgcggtggctcatgcctgtaatcccagcactttgggaggccgaggcaggcagatcacctgaagtcaggagtactcgaccagcctggccaacatagtgaaaccccatctcaactaaaaatacaaaaatcagccgggcgtggtggcaggcgcctgtaatcccagctactcagggggctgaaacaggagaatcgcttgaacccgggaggcggaggttgcgccatcgcactccagcctgggagacaagagcgagacttcgtctcaaaaaaaaaaaattcttcttccaagattcaagttgtgtcatttcaccttaataactggaggttagttaagctgggctgtgttctttgcttaatattaagacaacgttttttccagatggaagaaaactatcttaatgaattgttagcttattaattatgtaatgctaatggcttttaaaagctgagatgttctgactgggtgttgtggctcacacctgtaatcccagtaccttgggaggccaagggggaaggattgcttgaggccaggagtttgggaccatagtgagaccccgcctctatttaaaaaattaaattttgttttgttttgttttgagttggagttttgctcttgttgcccatgctgaagtgcaatggtgcaatctcagctcaccacaacctgtgcctcctgggttcaagcgattctcctgcttcagcctcccgagtagatgggattacaggcgtgcaccaccatgcctggctaattttgtatttttagtagagacagggtttctctatgttggtcaggctggtctcaaactctcgacctcaggtgatctgcccgcctccgcttcccaaagttctgggattataggtgtgagccactgggcctggcctaagaaagtttttttaagccattagacgtttttaaaggaattgggagatgacaattggggaaatatttaaaatttaagtaaaatataaagcttccttatttcatgtaacccagacaatctcagtatacatgatcagttgtgtctgacaggtaaatctatttgaggccttatcacacgttacttttaagaactagaaaggaaaagtcactgatcttaagtatttataatacttcatgtggtctaatactttttacgttttgttttgattcagatttagtccggattcccggtatctggcagtaggttctagtgagaactcagtggatttttatgacctaacgctgggccccactcttaacagaatcagctactgcaaagacattccaagctttgtcattcaaatggacttctctgcagatagcagttatctccaggtacagtaccaatactgtatacccaggtggcaagttcttctgcttttacatttcgtgttagtgaatgcatttaaagttcctgagctccagagctccagcttctcaactcctccctttgtaccttctgacctacagctcccctttcctcccccacttatcagagcttttctcctattaagtttttgtagtgatcttttgcatacttaataatgttagacatgtaaatcaagtagcaatatgctagtattctgtaaaccccctgtggattttgtctctcacctaatggaattcttgtcccattttaatctgatgaaaaaggtctctagtggctgctataaacggcatgtctatgaagtgccttcaggaaaacatcttatggatcatgccgctattgacagaattacttgggctacatggactaggtaaatacttatatattcacaaggcaagaactgactttgaaggccagttagaaaatcctatttctgaactgttagagccattccaataaggaatagtaattgagtttcaagtttttgttaccatattttgaaatggtatgttcatgttgggacccctttttattgaatatatttccatgttttatcagtttccatgatttatcaagttttttttttaaggaaatcaaagttttaactttaaagataccctgatatttttcttaatgctaaatttaatgactggcaaaaaggtattgggtgctgttaagcaactgttattaattctctatctaaaggaatgctatcttgaatctattagaagtcaaagcttccaaatttgttcaaatttcctggctgtatgacaggtaaccatgactatccatttttttggccaatgaaaaatgccatcaaattcctgtatcagccaggcatatagtggctcatgcctgtaatctctgatgtagcaggccgaggtgggaggatcacttgagcctagaagttttgataccagcctgggcaacatagcaagaccccatctctgaaatttttttaattcctatgtcataagtcatttttatttttgtagagatagggatctcacaatattgcccaggctggtctcaaactcttggcctcaagcagtcctcctgcctcagcctcccaaaatgttgggattactggtatgtgctgctggacccagccaagtagcacttttaatttgaaaaatagttctatcagttttcagtcaggcgcggtggctcagcctgtaatcccagcactttgggaggccgagcgggggtgatcacctgaggtcgggagttcgagactagcctgaccaacatggagaaaccctgtctctactaaaaatacaaaataagccgggcatgttagcgcatgcctgtgatcccagctactcgggaggctgaggcaggagaattgcttgaacccaggaggcagaggttgcggtgagccgagatcatgccattgcactccagcctgggtaacaagagcgaaaactccgtctcaaaaaaaaaaaaagaaaaaatagttctatcagttttcataaagtactactttaatcttaaaaagattaatctagaaacccttcaaattataaaatgtcatttttaaaaggcaggagttgatatcctgatgaaattcaggtctccaaacaacttaccataatttacttcctgtattttaagtaacatgatagggtacttagagattaattgccaagaaactttttgaatatagtcaacctgcccgcacttgccatgatgagttttcttttgttccttccctctagtattctaggagatgaggttttgggaatctggtccagacatgctgagaaagctgatgtcaactgtgcctgtgtatctcattcaggaatcagtcttgttacaggagatgactttggcatggttaagttatttgacttcccatgtccagaaaaatttgtaagtttgtgttttgtttactattatcagtttactcctaattttgatgtcttatcatcagcacttttccccatatatttaaaatgttttgtcctaatttctaaatttttccccaaactttctaaatctatttactttgaaataaaagctattagaaacaaatcctctccctcgagtaataccatctttggaaccatcctacaaaagctgtaattagcttttcaccaaacctataatcagttatcaaatttcaaatgcttttccttagagaaaaatggtcagagtacctggagacatctgactgcccacacagcctggttttgcagatccactactcatgctgaaaagcattctaatcactggctgcggtgctaactccctactctctccacagctcttgtcatagagattatagttcctaataagagcctttgacttctgtgtgcaccaaatgccctgagcttgtctgtcattgttttttaggcaaaacacaaaaggttcttgggtcattcgccccatgtgacaaatattcgatttaccagtggtgatcgacatgttgttagtgctggaggtgatgactgcaggttagtaactttctcagcccatgaagagcagactatgttactagttaagagacttaatacaacaactcctacagctttggtttatgaaatcagctagtcaacattagtagaaggtagtataaccagatggctcttcagaatctcatatttatgcaaatacagaataaaaggagttaaagaggaaaaatattacacatgtaacctgaaagcacaactgaaaaatattaaactgttatgaaaatctaaaaacataattaactccctgcaattttcttctctgattgcagcttatttgtctggaaatgtgtacatacacctcactgagagatgctgagatgactacagaaattaactttgagaccagaattacagagaagaaaaaccaaaacccaaccctgcatggtcaagtggtgctaacccaagactgtaacagggagaaatgcccagaatcatcaaaatagtgaaagactgatctgttcaaaatatttgctatatgcactgggtataatccgtaatccatacactgccagataatgccatttcaaggaaggatcgaatacttgatggtaaaggccaagtccccctgtattgggaagtgtgtgatttcggcagacctgctgggaaaatttagggtagagcactctttacagaagaactcaaaaacccaatttggataattttcattatctttttagcaaaatggtttcttaatgtttatattttattttcaaggttcattgtttaatgaaatattttattcttgcatttccataaggaaagggaaagtcatgatcatcctaaaggatcacagtttttaaaaggcaaacattttccctaaggaaacagacacaagctttcctagagaatatgatgttttttaggcattaataaggtccttttttataaaggacacttttctcctagtagttttgaattcaggaacagatccaaagttagcagtatatggctgctacatttccattttcattttcgagccatcagtttatgttcagatgccatctctgtaatcgcacatttaaaacataactgtagcctcactaatggaaaagtagtatgatgaacaatcattcccaatggtgtacaatgtaagggttttagggagcaacagtatttaactggaagaaagaattgcatatttaatgtagtctaatatatacacatttgtttaacatgtaaacaaaagtgttaaattcacatatacaacattatacaatttaatcactcttggaataaaatttttatagccttttttctattgggaaaatttgtttagatgtgtgccactccataggtttatttccaaaatgaatgagcccaactccatttgtaaaaacttgtcagttagaattcctttttttagtggattagggctgaattcttagatccttatttcttttcactttaaatgctgccaaagatcactactcatcattcaggaattcgctgtctagcctatctgtagtttcctgaagattgaaaattatgtagactgctatttaaaaatatatttttctaagtgtgaggtttaagatgctgtattgaccctatgagtttttaatgtgttaattatctttatagcataatagatcgctttaggttcctggaatcccatttggtctgacaggatatatgaagattcttaatacctattttctgtgtctaatacttggttaatactaaaaatagaaatgactaaattacatcacagaaagcataaccagtgattgaacctggtagttttaaagctctaaatagctgtggctgaaggactgattatggggctaagaagcttgaaacgtaagttggtacttgttcatcagtggattctcctaaattaagccaaattttgaaatacatgactattaagtttctactcatgtatttacagtcagtcaataaattaaaggaggaaaaaaatccctgaacaacctgcccataaaaagaaaaatactctacatttgagcctgctgcagttttaaattttccctctgggtcaagtttgccagcttttggctacagagaaattatatttccattacagtgcaggtagaaactctgtaaccttaagcatgtaaactacatagaataaaactgtttccactgcatttctgtccttcaaagtggccaacctgattaagtcagccttaatcactgctgctgtcagtttcacgactaaaggtcatattgactaagtagtcatcagctgaccacctcgctgtatcagccagcaacgaggggaaggtgaagaaacatgataggccatatagaatctgccctatgtttacttttttaacccagataattatttttgtgtgcagtatctaagctcctgattgtgtaacctgggacttctggcaccttttgttccattcattttatgtataaaatgcatgccaaagcacactgtgccctctggtacccttgcttccaatcgccaaccatgctcatttccttcctttttttgtggtccctttttgtggtgatcattttaaaccacgtcatccaacaaatgttttatggtcaaccttagcttgttcataagccatagcaactgaaagattaaactcttaaatatgtgtctgggcagtggctattaaatagcaaaaaacaatcagattttagtattttattatttccttgtaaaatggctgaactaaattaaacccttgtttcccatttgttctataatttatagtgaaactgagaacaaaactatctttataaatgatagctaaaagtatttccagatatttaaacaatttaaaataaatttcttctgcagagatgcaaagcatctcaacactggaatgaacaaatgccttaaattcaatggagtaaacctttagaatgaagaggaactgtcatttcacccaagccgaagacaacagccttatgcacttgtgtgctctgtctttgctgcttctcgtgtttcaagcctttcctgtgggatcagcacagcaaagtgcaacttaccaaatggtttaatgactggttaattctttcttctcccaatggaaaagcaatggcaacacaacagtagactgctggcttgacaatcttaaacgtgagcctttgcacatgtaggtttatcatcatttgagtatacgactaagcaagtcaatgaactttttttttttttttagcagtttaatttggtcctgagaatgttgcagtctttattaccccttttgcattaatccacttttctaaccaccttttaagctttaatttttaacactatacaccaagtctttgaaatcagtgatctgttatttaactctaaagcatttgacacttcttgccttaacagttttaaaaaccacacacaaaaaaactctgtaagtaatacagtaggccaaaagtttcatcctatctatcttgcagtttacctatctgatctgatctctgtaattatagttctgtcatttaaaatatactatttaaatctaatttttacatttcaaaaattatcttcagtagtaactaagtatattttctgtggattctgagaatgttatttttcagaatgtgagaatatatatgtacatttataatcttgtgactttaaagtctgttttcagatacagtatgtaaatacttgtaaaaaaatttgtataattttgtgataatgtagtttcccaaaaaaattatttagaaggcattatgttattagtaaatgagagcactgtatagaactgttcctattttctgcacttgccattccagctgcctccactgtccatacccacctcattcatcctgtcacagaaggcaggaaaactgggaactttaccaaagtagcactcagcctgagaggcctgtataatcatgcttttcaaactaaattcacttaaaaattaaaaagcagaattgaatattttaagcagcctcagtacctttggccaatgctgttttcatggtggattatgaacattatataatctttgggaaaagtgaaagtagtacaatttttagaataatgacaactgcctcactgcatctctccactcacacagcaaccgtgtagccccctaagctgcagtaccatgactaaccatgatgtcaatttcatatgctgatcctcacaacagcagtgcacaaacatgccccaaatattttaacagaatttagctcttccttaagctgtcttttcatagtaaaaacaaaacaaaaacacccaatgttaaaaccacataataaacttacaaacttgaaaaattagacacttcagatagataggcaataaaacttcatattatgaaagcaatatattccaagtttcaaagatttgacaagttctgtagagtatctttcatcagtacatgaaaacttccaaactgcatgatcttctgccaggcaggactgggtgctattcgctggtttgaggtcgaatccatttcaaggcatgtcgtggtgggacattaatggtgggatggtagaatgtgcagtccggtcttgtacattgagtgttaaacctacaatgttttggatgatagaagggacattccatcttcttacaagcagggaagtaacggcagagctgactactggaaggtggtgctggtggtgcaactgctggttttggagacagtactggaattcttctactcacatgagtgaagggacaatctggtttagtacactttgcatcatatttacaatttgggtgaacaaacaaacatttttcagcaaatttacaattggggaaggctttgcagggtgagatggggtgatggtaggcacactcatccccatttttacaagcaggccagtacttgcagcgctccaaaagtttttctggtttctgtgccacactcagttcactcatctcagcttgatttttttctacagaatctccttttgtttcctcttctttaatggggggacttattctgggggtcctactttgtccctggaccacttctgctagcaattcttcttgagaagttcgagttctgggagcaactggaagtgtctgtttctgtggaactgtagagtagttagttgtttttgttacggattcttgagcttcagatatagccttcaaaatcagattcttgttagcttgtttagaaggtggaagagaaggtctcctttcaggctttgcaggcacagacacactgctggagatgcttcctgttcgagacccgtaatcatcatcttcttcctcctcttctccatcatgattgaatttttttactttaacaactgaacttaccacaggcaactttctcttccgaaagttttcatcctccatactcattttctccgagttgtttctaaagaacggactatacgtttcttctaagctgttaagcacctctggttcacacaaacgtcctgtttcatatacccaactactctgcatatcaagctgcttggcagcatgaatactattctgctgctgttgaaattgcaacctgtttaaatgaacaccactatctgcatttctacttgcaggtggtcgataaatttcaatagaagggcgagaagaaccatatgtaagtgtcactgtaggttttttctgagataagggattctcctgcacaaagttgaggtcttcgtcaatgagatcatctggttctggcttaatatcaatcacatcttcagagggtgctggctccctcaaaggtttcactgttgacattagtcgggttgcagctccatcatcgtaagtctgtctgacatttgtggtttttgactcctgcgaacttgtagaaactctggaatctcttttttcaggtctcgcgctaggaatggcaagtggtggcactgcagcttcatgcctcctctcatctccccgactgaaattgctcttgtttgaaggcacgttactatcaaagatgttggtatcagaagacttcagactagagggttcagttgtaacagagcgaagtttatctaatacaccatgaagccatacggtgaatcgaattgtgttgttccctagaaacagggacagatcctctgtcatttggtcctgacttttcttgttggccaccatcaccataatgtaatcaggaagttcttcatcaacataagctcctaattcttgtaatttccccttaatggcactccggatcttgcggctgatctcggtgccgatctccatggctctgcggcgtgcgggaactcagcactgcgcggcgcttggcttacccggaggctgccgcggactcctaccccgcagccgggacaccaccgcctcc

SEQ ID NO: 17459 - RNA, 13858 nt, Homo sapiens
  source 1..13858: mol_type = other RNA
tcaggccaggcacagtggctcatacctggaatcccagcactttgggaggccgaggcaggcagatcacctgaggtcaaggtatttgagaccagcctggccaacatggtgaaaccccatctctactaaaaatacagaaattagctgggtgtggtggtgcacacctgtaatgctagctactcgggaggctgaggtaggagaatcgcttgaacctgggaggcagaggttgcaataagcctagatcatgccactgcactcaagcctgggagacagagcgagactacatcttaaaaaaaaaaaaaaaagtattatgagagaggataatgtattgtaatgtattgtagaggctaaataaaattatgctcatgtcagaaaaaaagagtatttctcaaaataaaattcactgaaactggatgtttattttgactgagatatagtatatcctcaaattgccatagaaagtttacaagaatattagaggtaaattataaatatcagggcctttttaaaaaaaaaagattctgcttataacttggtatttgtttataataaaaattatagtagccaataatgaacacttactctggcttggttatttacttaggtcaaaagaaggaggagcggttaaactgtgggatcaggaactgaggcggtgccgtgccttcaggcttgagacaggacaagccacagattgtgttcgttctgtgtgcagaggcaaagtaagatgttccatgagctgatacagtgcagcagaaaacagaaagtggttattactgtgattccctcaccctttgcagcctaatgaacaatacttaataatgcataacgatggatttgcttgccaacattactctgtctttgctgctttctttgccaaagttagcaccagtgtggtgcataagctaggaagctattctgtctaaatactgtatgtaaacctccaatattttctagaatctgccaatttaacaactctagtagacataattgaaagcccttggcagttgactcatattaggacagctgtctccattttttaaaaaaacacacattccctagataaaacgtgcagtaaacaaacaatgaaatactactcagccataaaaaataatgaaattctgtcattcttggtggcaacatggatgagactggaggacatgatgtgaagtgaaataagccaggcacagaaagataaatacatgttctcactcctgtgcagaaactaaaaaagttgatcccacagaggtggagagtagaatagtggttactggaggcggacaagggggagggggagggggatagggaaggactggttaaaggatacaagtttacacagccagataggaatagtatgttttagtattctgtagtactgtaggatgactatagttaagaatcacgtatttatgtattttcaggtatttacaagagaggattttgaaagtttccatcacaaagaaatgataaatgtctgaggtgatggttatgcgtattaccctatgccctatagatatgtataattatgtgtcaatttcaaaataaaaattcaaaactacaactcctatgaaaatttttgagcgtgtttgtacttattaagtgtatttataaatcatacggatattatcttcagcctgcatattaaattgtagttaagcttttactttttaactaaaaaataaattctattattttttcctatatcccactgcactgaccccagtttggaaatcctaagattatcaaataaaaactttgattattgaagaatccaggtgtactgccacagaaaagttctattctgtagcatggactctaatatgtaatctagcccattgtgcttacagatagatgtgtgcctgtagtcatagaaaaatttgcatgagctaatgactgccttgctactagattagctcaaagcaaaaagttctctgaaagcaggtcaatagggtcatttttatattatgaagaagaaaagcagctgttgtattacattcactgtattggtcctgcttgtgtttcagggcaagatccttgttgggacaaggaatgctgaaataatcgaagttggagagaaaaatgcagcttgtaatattttagttaacggtcatgtggatgggccaatctggggactagcaacacatccttccagggattttttcctttctgctgcagaagatgggacagtgagactttgggatattgctgataaagtaagtacagataatttttttaaaagaggttacaacttctaaaaagaaaagttggaagttctaaattgctagtacttaaagaactgccagaattctgttgagcattttgaggggaaactggtataatttagaagtacttcacttaatgtttcctatgactctttttttttttttttttaaatgcagaagatgttaaacaaagtgaatttgggacatgctgctcgtactgtgtgttacagccctgaaggggacatggtggctattggaatgaaaaatggagaatttatcattttactagtgagttctctaaaaatatggggaaagaagagagacaggagatgtgcaatccatgatatcaggttagtgaacaaatggaatagagtttctagtatatacttgatttaacttccatttgtaaaattttccatagccttgccttcaaaaagaggtccccagggcctgtagcatttcccgtattataaattgtatgctaaaatatggctgtttgtatactacttaattcttcttgctaaattataaacccactgggcaccaactataatagcaagtactagtaggtaatgtttgatgaattcatgttaacacttagccatgtccattaagttcatcccaccaagaggtatctcccactgtaatacaagagagctatctgcccttcaaaagttgtcaccctggaaaactaaagttgtgatttcaaacatatcttctcttagtaacctcagtttgggaatatgtagttcattaatttaatcaatacctattgattaaatgttccagaatccaaattaatttaaatgtttcttaaacctttgtttttcagtgcttaagcatttttcaacagtggctaccatttacggagtacttccgtgtgatcagtagataagattattgaatctaggtctgtcaaaagcttgtacacttttcatcagtaaaatccttttacaaatgaaaccttcctcagaacttcaatatataaaatagtaacagtggcttcccttagcttttacatgtctctatcgtacctcagtaagactcatgggccatttcaagagactgaattgtcccatatgactccaaagattgctaggcaaatagcatttcactttgtcttttaaataagttcttcaggccgggcgcggtggctcatgcctgtaatcccagcactttgggaggccgaggcaggcagatcacctgaagtcaggagtactcgaccagcctggccaacatagtgaaaccccatctcaactaaaaatacaaaaatcagccgggcgtggtggcaggcgcctgtaatcccagctactcagggggctgaaacaggagaatcgcttgaacccgggaggcggaggttgcgccatcgcactccagcctgggagacaagagcgagacttcgtctcaaaaaaaaaaaattcttcttccaagattcaagttgtgtcatttcaccttaataactggaggttagttaagctgggctgtgttctttgcttaatattaagacaacgttttttccagatggaagaaaactatcttaatgaattgttagcttattaattatgtaatgctaatggcttttaaaagctgagatgttctgactgggtgttgtggctcacacctgtaatcccagtaccttgggaggccaagggggaaggattgcttgaggccaggagtttgggaccatagtgagaccccgcctctatttaaaaaattaaattttgttttgttttgttttgagttggagttttgctcttgttgcccatgctgaagtgcaatggtgcaatctcagctcaccacaacctgtgcctcctgggttcaagcgattctcctgcttcagcctcccgagtagatgggattacaggcgtgcaccaccatgcctggctaattttgtatttttagtagagacagggtttctctatgttggtcaggctggtctcaaactctcgacctcaggtgatctgcccgcctccgcttcccaaagttctgggattataggtgtgagccactgggcctggcctaagaaagtttttttaagccattagacgtttttaaaggaattgggagatgacaattggggaaatatttaaaatttaagtaaaatataaagcttccttatttcatgtaacccagacaatctcagtatacatgatcagttgtgtctgacaggtaaatctatttgaggccttatcacacgttacttttaagaactagaaaggaaaagtcactgatcttaagtatttataatacttcatgtggtctaatactttttacgttttgttttgattcagatttagtccggattcccggtatctggcagtaggttctagtgagaactcagtggatttttatgacctaacgctgggccccactcttaacagaatcagctactgcaaagacattccaagctttgtcattcaaatggacttctctgcagatagcagttatctccaggtacagtaccaatactgtatacccaggtggcaagttcttctgcttttacatttcgtgttagtgaatgcatttaaagttcctgagctccagagctccagcttctcaactcctccctttgtaccttctgacctacagctcccctttcctcccccacttatcagagcttttctcctattaagtttttgtagtgatcttttgcatacttaataatgttagacatgtaaatcaagtagcaatatgctagtattctgtaaaccccctgtggattttgtctctcacctaatggaattcttgtcccattttaatctgatgaaaaaggtctctagtggctgctataaacggcatgtctatgaagtgccttcaggaaaacatcttatggatcatgccgctattgacagaattacttgggctacatggactaggtaaatacttatatattcacaaggcaagaactgactttgaaggccagttagaaaatcctatttctgaactgttagagccattccaataaggaatagtaattgagtttcaagtttttgttaccatattttgaaatggtatgttcatgttgggacccctttttattgaatatatttccatgttttatcagtttccatgatttatcaagttttttttttaaggaaatcaaagttttaactttaaagataccctgatatttttcttaatgctaaatttaatgactggcaaaaaggtattgggtgctgttaagcaactgttattaattctctatctaaaggaatgctatcttgaatctattagaagtcaaagcttccaaatttgttcaaatttcctggctgtatgacaggtaaccatgactatccatttttttggccaatgaaaaatgccatcaaattcctgtatcagccaggcatatagtggctcatgcctgtaatctctgatgtagcaggccgaggtgggaggatcacttgagcctagaagttttgataccagcctgggcaacatagcaagaccccatctctgaaatttttttaattcctatgtcataagtcatttttatttttgtagagatagggatctcacaatattgcccaggctggtctcaaactcttggcctcaagcagtcctcctgcctcagcctcccaaaatgttgggattactggtatgtgctgctggacccagccaagtagcacttttaatttgaaaaatagttctatcagttttcagtcaggcgcggtggctcagcctgtaatcccagcactttgggaggccgagcgggggtgatcacctgaggtcgggagttcgagactagcctgaccaacatggagaaaccctgtctctactaaaaatacaaaataagccgggcatgttagcgcatgcctgtgatcccagctactcgggaggctgaggcaggagaattgcttgaacccaggaggcagaggttgcggtgagccgagatcatgccattgcactccagcctgggtaacaagagcgaaaactccgtctcaaaaaaaaaaaaagaaaaaatagttctatcagttttcataaagtactactttaatcttaaaaagattaatctagaaacccttcaaattataaaatgtcatttttaaaaggcaggagttgatatcctgatgaaattcaggtctccaaacaacttaccataatttacttcctgtattttaagtaacatgatagggtacttagagattaattgccaagaaactttttgaatatagtcaacctgcccgcacttgccatgatgagttttcttttgttccttccctctagtattctaggagatgaggttttgggaatctggtccagacatgctgagaaagctgatgtcaactgtgcctgtgtatctcattcaggaatcagtcttgttacaggagatgactttggcatggttaagttatttgacttcccatgtccagaaaaatttgtaagtttgtgttttgtttactattatcagtttactcctaattttgatgtcttatcatcagcacttttccccatatatttaaaatgttttgtcctaatttctaaatttttccccaaactttctaaatctatttactttgaaataaaagctattagaaacaaatcctctccctcgagtaataccatctttggaaccatcctacaaaagctgtaattagcttttcaccaaacctataatcagttatcaaatttcaaatgcttttccttagagaaaaatggtcagagtacctggagacatctgactgcccacacagcctggttttgcagatccactactcatgctgaaaagcattctaatcactggctgcggtgctaactccctactctctccacagctcttgtcatagagattatagttcctaataagagcctttgacttctgtgtgcaccaaatgccctgagcttgtctgtcattgttttttaggcaaaacacaaaaggttcttgggtcattcgccccatgtgacaaatattcgatttaccagtggtgatcgacatgttgttagtgctggaggtgatgactgcaggttagtaactttctcagcccatgaagagcagactatgttactagttaagagacttaatacaacaactcctacagctttggtttatgaaatcagctagtcaacattagtagaaggtagtataaccagatggctcttcagaatctcatatttatgcaaatacagaataaaaggagttaaagaggaaaaatattacacatgtaacctgaaagcacaactgaaaaatattaaactgttatgaaaatctaaaaacataattaactccctgcaattttcttctctgattgcagcttatttgtctggaaatgtgtacatacacctcactgagagatgctgagatgactacagaaattaactttgagaccagaattacagagaagaaaaaccaaaacccaaccctgcatggtcaagtggtgctaacccaagactgtaacagggagaaatgcccagaatcatcaaaatagtgaaagactgatctgttcaaaatatttgctatatgcactgggtataatccgtaatccatacactgccagataatgccatttcaaggaaggatcgaatacttgatggtaaaggccaagtccccctgtattgggaagtgtgtgatttcggcagacctgctgggaaaatttagggtagagcactctttacagaagaactcaaaaacccaatttggataattttcattatctttttagcaaaatggtttcttaatgtttatattttattttcaaggttcattgtttaatgaaatattttattcttgcatttccataaggaaagggaaagtcatgatcatcctaaaggatcacagtttttaaaaggcaaacattttccctaaggaaacagacacaagctttcctagagaatatgatgttttttaggcattaataaggtccttttttataaaggacacttttctcctagtagttttgaattcaggaacagatccaaagttagcagtatatggctgctacatttccattttcattttcgagccatcagtttatgttcagatgccatctctgtaatcgcacatttaaaacataactgtagcctcactaatggaaaagtagtatgatgaacaatcattcccaatggtgtacaatgtaagggttttagggagcaacagtatttaactggaagaaagaattgcatatttaatgtagtctaatatatacacatttgtttaacatgtaaacaaaagtgttaaattcacatatacaacattatacaatttaatcactcttggaataaaatttttatagccttttttctattgggaaaatttgtttagatgtgtgccactccataggtttatttccaaaatgaatgagcccaactccatttgtaaaaacttgtcagttagaattcctttttttagtggattagggctgaattcttagatccttatttcttttcactttaaatgctgccaaagatcactactcatcattcaggaattcgctgtctagcctatctgtagtttcctgaagattgaaaattatgtagactgctatttaaaaatatatttttctaagtgtgaggtttaagatgctgtattgaccctatgagtttttaatgtgttaattatctttatagcataatagatcgctttaggttcctggaatcccatttggtctgacaggatatatgaagattcttaatacctattttctgtgtctaatacttggttaatactaaaaatagaaatgactaaattacatcacagaaagcataaccagtgattgaacctggtagttttaaagctctaaatagctgtggctgaaggactgattatggggctaagaagcttgaaacgtaagttggtacttgttcatcagtggattctcctaaattaagccaaattttgaaatacatgactattaagtttctactcatgtatttacagtcagtcaataaattaaaggaggaaaaaaatccctgaacaacctgcccataaaaagaaaaatactctacatttgagcctgctgcagttttaaattttccctctgggtcaagtttgccagcttttggctacagagaaattatatttccattacagtgcaggtagaaactctgtaaccttaagcatgtaaactacatagaataaaactgtttccactgcatttctgtccttcaaagtggccaacctgattaagtcagccttaatcactgctgctgtcagtttcacgactaaaggtcatattgactaagtagtcatcagctgaccacctcgctgtatcagccagcaacgaggggaaggtgaagaaacatgataggccatatagaatctgccctatgtttacttttttaacccagataattatttttgtgtgcagtatctaagctcctgattgtgtaacctgggacttctggcaccttttgttccattcattttatgtataaaatgcatgccaaagcacactgtgccctctggtacccttgcttccaatcgccaaccatgctcatttccttcctttttttgtggtccctttttgtggtgatcattttaaaccacgtcatccaacaaatgttttatggtcaaccttagcttgttcataagccatagcaactgaaagattaaactcttaaatatgtgtctgggcagtggctattaaatagcaaaaaacaatcagattttagtattttattatttccttgtaaaatggctgaactaaattaaacccttgtttcccatttgttctataatttatagtgaaactgagaacaaaactatctttataaatgatagctaaaagtatttccagatatttaaacaatttaaaataaatttcttctgcagagatgcaaagcatctcaacactggaatgaacaaatgccttaaattcaatggagtaaacctttagaatgaagaggaactgtcatttcacccaagccgaagacaacagccttatgcacttgtgtgctctgtctttgctgcttctcgtgtttcaagcctttcctgtgggatcagcacagcaaagtgcaacttaccaaatggtttaatgactggttaattctttcttctcccaatggaaaagcaatggcaacacaacagtagactgctggcttgacaatcttaaacgtgagcctttgcacatgtaggtttatcatcatttgagtatacgactaagcaagtcaatgaactttttttttttttttagcagtttaatttggtcctgagaatgttgcagtctttattaccccttttgcattaatccacttttctaaccaccttttaagctttaatttttaacactatacaccaagtctttgaaatcagtgatctgttatttaactctaaagcatttgacacttcttgccttaacagttttaaaaaccacacacaaaaaaactctgtaagtaatacagtaggccaaaagtttcatcctatctatcttgcagtttacctatctgatctgatctctgtaattatagttctgtcatttaaaatatactatttaaatctaatttttacatttcaaaaattatcttcagtagtaactaagtatattttctgtggattctgagaatgttatttttcagaatgtgagaatatatatgtacatttataatcttgtgactttaaagtctgttttcagatacagtatgtaaatacttgtaaaaaaatttgtataattttgtgataatgtagtttcccaaaaaaattatttagaaggcattatgttattagtaaatgagagcactgtatagaactgttcctattttctgcacttgccattccagctgcctccactgtccatacccacctcattcatcctgtcacagaaggcaggaaaactgggaactttaccaaagtagcactcagcctgagaggcctgtataatcatgcttttcaaactaaattcacttaaaaattaaaaagcagaattgaatattttaagcagcctcagtacctttggccaatgctgttttcatggtggattatgaacattatataatctttgggaaaagtgaaagtagtacaatttttagaataatgacaactgcctcactgcatctctccactcacacagcaaccgtgtagccccctaagctgcagtaccatgactaaccatgatgtcaatttcatatgctgatcctcacaacagcagtgcacaaacatgccccaaatattttaacagaatttagctcttccttaagctgtcttttcatagtaaaaacaaaacaaaaacacccaatgttaaaaccacataataaacttacaaacttgaaaaattagacacttcagatagataggcaataaaacttcatattatgaaagcaatatattccaagtttcaaagatttgacaagttctgtagagtatctttcatcagtacatgaaaacttccaaactgcatgatcttctgccaggcaggactgggtgctattcgctggtttgaggtcgaatccatttcaaggcatgtcgtggtgggacattaatggtgggatggtagaatgtgcagtccggtcttgtacattgagtgttaaacctacaatgttttggatgatagaagggacattccatcttcttacaagcagggaagtaacggcagagctgactactggaaggtggtgctggtggtgcaactggttttggagacagtactggaattcttctactcacatgagtgaagggacaatctggtttagtacactttgcatcatatttacaatttgggtgaacaaacaaacatttttcagcaaatttacaattggggaaggctttgcagggtgagatggggtgatggtaggcacactcatccccatttttacaagcaggccagtacttgcagcgctccaaaagtttttctggtttctgtgccacactcagttcactcatctcagcatttgggtcctcaagctgcctgctcagcaagtgcaactgctgtgggtggaggagacctctgagtcccttgtttgaggctgcagtttggtttacgggtttcattccttcaaagcacatgtcctcctcttgatctgacatgtatcctggggggctggggacaccatccagcgtcactataaacttgggacttgcaggtttatctggttgtacaagatctcgtgtctgcataaggtgtcctgaaagtacccgaagggaatctgcagtcttcatccccgactcttggtttggtgccactactacttcctcagacagctttggcttcttcagaataaatgatcttgtgtctgcatggaccatggattccatgtcatagtaatcttgactcatctgcagagtttctgccattactgggtcgatttgcagtcgggataataattgcctctgttgagttccttgatttttttctacagaatctccttttgtttcctcttctttaatggggggacttattctgggggtcctactttgtccctggaccacttctgctagcaattcttcttgagaagttcgagttctgggagcaactggaagtgtctgtttctgtggaactgtagagtagttagttgtttttgttacggattcttgagcttcagatatagccttcaaaatcagattcttgttagcttgtttagaaggtggaagagaaggtctcctttcaggctttgcaggcacagacacactgctggagatgcttcctgttcgagacccgtaatcatcatcttcttcctcctcttctccatcatgattgaatttttttactttaacaactgaacttaccacaggcaactttctcttccgaaagttttcatcctccatactcattttctccgagttgtttctaaagaacggactatacgtttcttctaagctgttaagcacctctggttcacacaaacgtcctgtttcatatacccaactactctgcatatcaagctgcttggcagcatgaatactattctgctgctgttgaaattgcaacctgtttaaatgaacaccactatctgcatttctacttgcaggtggtcgataaatttcaatagaagggcgagaagaaccatatgtaagtgtcactgtaggttttttctgagataagggattctcctgcacaaagttgaggtcttcgtcaatgagatcatctggttctggcttaatatcaatcacatcttcagagggtgctggctccctcaaaggtttcactgttgacattagtcgggttgcagctccatcatcgtaagtctgtctgacatttgtggtttttgactcctgcgaacttgtagaaactctggaatctcttttttcaggtctcgcgctaggaatggcaagtggtggcactgcagcttcatgcctcctctcatctccccgactgaaattgctcttgtttgaaggcacgttactatcaaagatgttggtatcagaagacttcagactagagggttcagttgtaacagagcgaagtttatctaatacaccatgaagccatacggtgaatcgaattgtgttgttccctagaaacagggacagatcctctgtcatttggtcctgacttttcttgttggccaccatcaccataatgtaatcaggaagttcttcatcaacataagctcctaattcttgtaatttccccttaatggcactccggatcttgcggctgatctcggtgccgatctccatggctctgcggcgtgcgggaactcagcactgcgcggcgcttggcttacccggaggctgccgcggactcctaccccgcagccgggacaccaccgcctcc

SEQ ID NO: 17460 - RNA, 13783 nt, Homo sapiens
  source 1..13783: mol_type = other RNA
tcaggccaggcacagtggctcatacctggaatcccagcactttgggaggccgaggcaggcagatcacctgaggtcaaggtatttgagaccagcctggccaacatggtgaaaccccatctctactaaaaatacagaaattagctgggtgtggtggtgcacacctgtaatgctagctactcgggaggctgaggtaggagaatcgcttgaacctgggaggcagaggttgcaataagcctagatcatgccactgcactcaagcctgggagacagagcgagactacatcttaaaaaaaaaaaaaaaagtattatgagagaggataatgtattgtaatgtattgtagaggctaaataaaattatgctcatgtcagaaaaaaagagtatttctcaaaataaaattcactgaaactggatgtttattttgactgagatatagtatatcctcaaattgccatagaaagtttacaagaatattagaggtaaattataaatatcagggcctttttaaaaaaaaaagattctgcttataacttggtatttgtttataataaaaattatagtagccaataatgaacacttactctggcttggttatttacttaggtcaaaagaaggaggagcggttaaactgtgggatcaggaactgaggcggtgccgtgccttcaggcttgagacaggacaagccacagattgtgttcgttctgtgtgcagaggcaaagtaagatgttccatgagctgatacagtgcagcagaaaacagaaagtggttattactgtgattccctcaccctttgcagcctaatgaacaatacttaataatgcataacgatggatttgcttgccaacattactctgtctttgctgctttctttgccaaagttagcaccagtgtggtgcataagctaggaagctattctgtctaaatactgtatgtaaacctccaatattttctagaatctgccaatttaacaactctagtagacataattgaaagcccttggcagttgactcatattaggacagctgtctccattttttaaaaaaacacacattccctagataaaacgtgcagtaaacaaacaatgaaatactactcagccataaaaaataatgaaattctgtcattcttggtggcaacatggatgagactggaggacatgatgtgaagtgaaataagccaggcacagaaagataaatacatgttctcactcctgtgcagaaactaaaaaagttgatcccacagaggtggagagtagaatagtggttactggaggcggacaagggggagggggagggggatagggaaggactggttaaaggatacaagtttacacagccagataggaatagtatgttttagtattctgtagtactgtaggatgactatagttaagaatcacgtatttatgtattttcaggtatttacaagagaggattttgaaagtttccatcacaaagaaatgataaatgtctgaggtgatggttatgcgtattaccctatgccctatagatatgtataattatgtgtcaatttcaaaataaaaattcaaaactacaactcctatgaaaatttttgagcgtgtttgtacttattaagtgtatttataaatcatacggatattatcttcagcctgcatattaaattgtagttaagcttttactttttaactaaaaaataaattctattattttttcctatatcccactgcactgaccccagtttggaaatcctaagattatcaaataaaaactttgattattgaagaatccaggtgtactgccacagaaaagttctattctgtagcatggactctaatatgtaatctagcccattgtgcttacagatagatgtgtgcctgtagtcatagaaaaatttgcatgagctaatgactgccttgctactagattagctcaaagcaaaaagttctctgaaagcaggtcaatagggtcatttttatattatgaagaagaaaagcagctgttgtattacattcactgtattggtcctgcttgtgtttcagggcaagatccttgttgggacaaggaatgctgaaataatcgaagttggagagaaaaatgcagcttgtaatattttagttaacggtcatgtggatgggccaatctggggactagcaacacatccttccagggattttttcctttctgctgcagaagatgggacagtgagactttgggatattgctgataaagtaagtacagataatttttttaaaagaggttacaacttctaaaaagaaaagttggaagttctaaattgctagtacttaaagaactgccagaattctgttgagcattttgaggggaaactggtataatttagaagtacttcacttaatgtttcctatgactctttttttttttttttttaaatgcagaagatgttaaacaaagtgaatttgggacatgctgctcgtactgtgtgttacagccctgaaggggacatggtggctattggaatgaaaaatggagaatttatcattttactagtgagttctctaaaaatatggggaaagaagagagacaggagatgtgcaatccatgatatcaggttagtgaacaaatggaatagagtttctagtatatacttgatttaacttccatttgtaaaattttccatagccttgccttcaaaaagaggtccccagggcctgtagcatttcccgtattataaattgtatgctaaaatatggctgtttgtatactacttaattcttcttgctaaattataaacccactgggcaccaactataatagcaagtactagtaggtaatgtttgatgaattcatgttaacacttagccatgtccattaagttcatcccaccaagaggtatctcccactgtaatacaagagagctatctgcccttcaaaagttgtcaccctggaaaactaaagttgtgatttcaaacatatcttctcttagtaacctcagtttgggaatatgtagttcattaatttaatcaatacctattgattaaatgttccagaatccaaattaatttaaatgtttcttaaacctttgtttttcagtgcttaagcatttttcaacagtggctaccatttacggagtacttccgtgtgatcagtagataagattattgaatctaggtctgtcaaaagcttgtacacttttcatcagtaaaatccttttacaaatgaaaccttcctcagaacttcaatatataaaatagtaacagtggcttcccttagcttttacatgtctctatcgtacctcagtaagactcatgggccatttcaagagactgaattgtcccatatgactccaaagattgctaggcaaatagcatttcactttgtcttttaaataagttcttcaggccgggcgcggtggctcatgcctgtaatcccagcactttgggaggccgaggcaggcagatcacctgaagtcaggagtactcgaccagcctggccaacatagtgaaaccccatctcaactaaaaatacaaaaatcagccgggcgtggtggcaggcgcctgtaatcccagctactcagggggctgaaacaggagaatcgcttgaacccgggaggcggaggttgcgccatcgcactccagcctgggagacaagagcgagacttcgtctcaaaaaaaaaaaattcttcttccaagattcaagttgtgtcatttcaccttaataactggaggttagttaagctgggctgtgttctttgcttaatattaagacaacgttttttccagatggaagaaaactatcttaatgaattgttagcttattaattatgtaatgctaatggcttttaaaagctgagatgttctgactgggtgttgtggctcacacctgtaatcccagtaccttgggaggccaagggggaaggattgcttgaggccaggagtttgggaccatagtgagaccccgcctctatttaaaaaattaaattttgttttgttttgttttgagttggagttttgctcttgttgcccatgctgaagtgcaatggtgcaatctcagctcaccacaacctgtgcctcctgggttcaagcgattctcctgcttcagcctcccgagtagatgggattacaggcgtgcaccaccatgcctggctaattttgtatttttagtagagacagggtttctctatgttggtcaggctggtctcaaactctcgacctcaggtgatctgcccgcctccgcttcccaaagttctgggattataggtgtgagccactgggcctggcctaagaaagtttttttaagccattagacgtttttaaaggaattgggagatgacaattggggaaatatttaaaatttaagtaaaatataaagcttccttatttcatgtaacccagacaatctcagtatacatgatcagttgtgtctgacaggtaaatctatttgaggccttatcacacgttacttttaagaactagaaaggaaaagtcactgatcttaagtatttataatacttcatgtggtctaatactttttacgttttgttttgattcagatttagtccggattcccggtatctggcagtaggttctagtgagaactcagtggatttttatgacctaacgctgggccccactcttaacagaatcagctactgcaaagacattccaagctttgtcattcaaatggacttctctgcagatagcagttatctccaggtacagtaccaatactgtatacccaggtggcaagttcttctgcttttacatttcgtgttagtgaatgcatttaaagttcctgagctccagagctccagcttctcaactcctccctttgtaccttctgacctacagctcccctttcctcccccacttatcagagcttttctcctattaagtttttgtagtgatcttttgcatacttaataatgttagacatgtaaatcaagtagcaatatgctagtattctgtaaaccccctgtggattttgtctctcacctaatggaattcttgtcccattttaatctgatgaaaaaggtctctagtggctgctataaacggcatgtctatgaagtgccttcaggaaaacatcttatggatcatgccgctattgacagaattacttgggctacatggactaggtaaatacttatatattcacaaggcaagaactgactttgaaggccagttagaaaatcctatttctgaactgttagagccattccaataaggaatagtaattgagtttcaagtttttgttaccatattttgaaatggtatgttcatgttgggacccctttttattgaatatatttccatgttttatcagtttccatgatttatcaagttttttttttaaggaaatcaaagttttaactttaaagataccctgatatttttcttaatgctaaatttaatgactggcaaaaaggtattgggtgctgttaagcaactgttattaattctctatctaaaggaatgctatcttgaatctattagaagtcaaagcttccaaatttgttcaaatttcctggctgtatgacaggtaaccatgactatccatttttttggccaatgaaaaatgccatcaaattcctgtatcagccaggcatatagtggctcatgcctgtaatctctgatgtagcaggccgaggtgggaggatcacttgagcctagaagttttgataccagcctgggcaacatagcaagaccccatctctgaaatttttttaattcctatgtcataagtcatttttatttttgtagagatagggatctcacaatattgcccaggctggtctcaaactcttggcctcaagcagtcctcctgcctcagcctcccaaaatgttgggattactggtatgtgctgctggacccagccaagtagcacttttaatttgaaaaatagttctatcagttttcagtcaggcgcggtggctcagcctgtaatcccagcactttgggaggccgagcgggggtgatcacctgaggtcgggagttcgagactagcctgaccaacatggagaaaccctgtctctactaaaaatacaaaataagccgggcatgttagcgcatgcctgtgatcccagctactcgggaggctgaggcaggagaattgcttgaacccaggaggcagaggttgcggtgagccgagatcatgccattgcactccagcctgggtaacaagagcgaaaactccgtctcaaaaaaaaaaaaagaaaaaatagttctatcagttttcataaagtactactttaatcttaaaaagattaatctagaaacccttcaaattataaaatgtcatttttaaaaggcaggagttgatatcctgatgaaattcaggtctccaaacaacttaccataatttacttcctgtattttaagtaacatgatagggtacttagagattaattgccaagaaactttttgaatatagtcaacctgcccgcacttgccatgatgagttttcttttgttccttccctctagtattctaggagatgaggttttgggaatctggtccagacatgctgagaaagctgatgtcaactgtgcctgtgtatctcattcaggaatcagtcttgttacaggagatgactttggcatggttaagttatttgacttcccatgtccagaaaaatttgtaagtttgtgttttgtttactattatcagtttactcctaattttgatgtcttatcatcagcacttttccccatatatttaaaatgttttgtcctaatttctaaatttttccccaaactttctaaatctatttactttgaaataaaagctattagaaacaaatcctctccctcgagtaataccatctttggaaccatcctacaaaagctgtaattagcttttcaccaaacctataatcagttatcaaatttcaaatgcttttccttagagaaaaatggtcagagtacctggagacatctgactgcccacacagcctggttttgcagatccactactcatgctgaaaagcattctaatcactggctgcggtgctaactccctactctctccacagctcttgtcatagagattatagttcctaataagagcctttgacttctgtgtgcaccaaatgccctgagcttgtctgtcattgttttttaggcaaaacacaaaaggttcttgggtcattcgccccatgtgacaaatattcgatttaccagtggtgatcgacatgttgttagtgctggaggtgatgactgcaggttagtaactttctcagcccatgaagagcagactatgttactagttaagagacttaatacaacaactcctacagctttggtttatgaaatcagctagtcaacattagtagaaggtagtataaccagatggctcttcagaatctcatatttatgcaaatacagaataaaaggagttaaagaggaaaaatattacacatgtaacctgaaagcacaactgaaaaatattaaactgttatgaaaatctaaaaacataattaactccctgcaattttcttctctgattgcagcttatttgtctggaaatgtgtacatacacctcactgagagatgctgagatgactacagaaattaactttgagaccagaattacagagaagaaaaaccaaaacccaaccctgcatggtcaagtggtgctaacccaagactgtaacagggagaaatgcccagaatcatcaaaatagtgaaagactgatctgttcaaaatatttgctatatgcactgggtataatccgtaatccatacactgccagataatgccatttcaaggaaggatcgaatacttgatggtaaaggccaagtccccctgtattgggaagtgtgtgatttcggcagacctgctgggaaaatttagggtagagcactctttacagaagaactcaaaaacccaatttggataattttcattatctttttagcaaaatggtttcttaatgtttatattttattttcaaggttcattgtttaatgaaatattttattcttgcatttccataaggaaagggaaagtcatgatcatcctaaaggatcacagtttttaaaaggcaaacattttccctaaggaaacagacacaagctttcctagagaatatgatgttttttaggcattaataaggtccttttttataaaggacacttttctcctagtagttttgaattcaggaacagatccaaagttagcagtatatggctgctacatttccattttcattttcgagccatcagtttatgttcagatgccatctctgtaatcgcacatttaaaacataactgtagcctcactaatggaaaagtagtatgatgaacaatcattcccaatggtgtacaatgtaagggttttagggagcaacagtatttaactggaagaaagaattgcatatttaatgtagtctaatatatacacatttgtttaacatgtaaacaaaagtgttaaattcacatatacaacattatacaatttaatcactcttggaataaaatttttatagccttttttctattgggaaaatttgtttagatgtgtgccactccataggtttatttccaaaatgaatgagcccaactccatttgtaaaaacttgtcagttagaattcctttttttagtggattagggctgaattcttagatccttatttcttttcactttaaatgctgccaaagatcactactcatcattcaggaattcgctgtctagcctatctgtagtttcctgaagattgaaaattatgtagactgctatttaaaaatatatttttctaagtgtgaggtttaagatgctgtattgaccctatgagtttttaatgtgttaattatctttatagcataatagatcgctttaggttcctggaatcccatttggtctgacaggatatatgaagattcttaatacctattttctgtgtctaatacttggttaatactaaaaatagaaatgactaaattacatcacagaaagcataaccagtgattgaacctggtagttttaaagctctaaatagctgtggctgaaggactgattatggggctaagaagcttgaaacgtaagttggtacttgttcatcagtggattctcctaaattaagccaaattttgaaatacatgactattaagtttctactcatgtatttacagtcagtcaataaattaaaggaggaaaaaaatccctgaacaacctgcccataaaaagaaaaatactctacatttgagcctgctgcagttttaaattttccctctgggtcaagtttgccagcttttggctacagagaaattatatttccattacagtgcaggtagaaactctgtaaccttaagcatgtaaactacatagaataaaactgtttccactgcatttctgtccttcaaagtggccaacctgattaagtcagccttaatcactgctgctgtcagtttcacgactaaaggtcatattgactaagtagtcatcagctgaccacctcgctgtatcagccagcaacgaggggaaggtgaagaaacatgataggccatatagaatctgccctatgtttacttttttaacccagataattatttttgtgtgcagtatctaagctcctgattgtgtaacctgggacttctggcaccttttgttccattcattttatgtataaaatgcatgccaaagcacactgtgccctctggtacccttgcttccaatcgccaaccatgctcatttccttcctttttttgtggtccctttttgtggtgatcattttaaaccacgtcatccaacaaatgttttatggtcaaccttagcttgttcataagccatagcaactgaaagattaaactcttaaatatgtgtctgggcagtggctattaaatagcaaaaaacaatcagattttagtattttattatttccttgtaaaatggctgaactaaattaaacccttgtttcccatttgttctataatttatagtgaaactgagaacaaaactatctttataaatgatagctaaaagtatttccagatatttaaacaatttaaaataaatttcttctgcagagatgcaaagcatctcaacactggaatgaacaaatgccttaaattcaatggagtaaacctttagaatgaagaggaactgtcatttcacccaagccgaagacaacagccttatgcacttgtgtgctctgtctttgctgcttctcgtgtttcaagcctttcctgtgggatcagcacagcaaagtgcaacttaccaaatggtttaatgactggttaattctttcttctcccaatggaaaagcaatggcaacacaacagtagactgctggcttgacaatcttaaacgtgagcctttgcacatgtaggtttatcatcatttgagtatacgactaagcaagtcaatgaactttttttttttttttagcagtttaatttggtcctgagaatgttgcagtctttattaccccttttgcattaatccacttttctaaccaccttttaagctttaatttttaacactatacaccaagtctttgaaatcagtgatctgttatttaactctaaagcatttgacacttcttgccttaacagttttaaaaaccacacacaaaaaaactctgtaagtaatacagtaggccaaaagtttcatcctatctatcttgcagtttacctatctgatctgatctctgtaattatagttctgtcatttaaaatatactatttaaatctaatttttacatttcaaaaattatcttcagtagtaactaagtatattttctgtggattctgagaatgttatttttcagaatgtgagaatatatatgtacatttataatcttgtgactttaaagtctgttttcagatacagtatgtaaatacttgtaaaaaaatttgtataattttgtgataatgtagtttcccaaaaaaattatttagaaggcattatgttattagtaaatgagagcactgtatagaactgttcctattttctgcacttgccattccagctgcctccactgtccatacccacctcattcatcctgtcacagaaggcaggaaaactgggaactttaccaaagtagcactcagcctgagaggcctgtataatcatgcttttcaaactaaattcacttaaaaattaaaaagcagaattgaatattttaagcagcctcagtacctttggccaatgctgttttcatggtggattatgaacattatataatctttgggaaaagtgaaagtagtacaatttttagaataatgacaactgcctcactgcatctctccactcacacagcaaccgtgtagccccctaagctgcagtaccatgactaaccatgatgtcaatttcatatgctgatcctcacaacagcagtgcacaaacatgccccaaatattttaacagaatttagctcttccttaagctgtcttttcatagtaaaaacaaaacaaaaacacccaatgttaaaaccacataataaacttacaaacttgaaaaattagacacttcagatagataggcaataaaacttcatattatgaaagcaatatattccaagtttcaaagatttgacaagttctgtagagtatctttcatcagtacatgaaaacttccaaactgcatgatcttctgccaggcaggactgggtgctattcgctggtttgaggtcgaatccatttcaaggcatgtcgtggtgggacattaatggtgggatggtagaatgtgcagtccggtcttgtacattgagtgttaaacctacaatgttttggatgatagaagggacattccatcttcttacaagcagggaagtaacggcagagctgactactggaaggtggtgctggtggtgcaactggttttggagacagtactggaattcttctactcacatgagtgaagggacaatctggtttagtacactttgcatcatatttacaatttgggtgaacaaacaaacatttttcagcaaatttacaattggggaaggctttgcagggtgagatggggtgatggtaggcacactcatccccatttttacaagcaggccagtacttgcagcgctccaaaagtttttctggtttctgtgccacactcagttcactcatctcagcatttgggtcctcaagctgcctgctcagcaagtgcaactgctgtgggtggaggagacctctgagtcccttgtttgaggctgcagtttggtttacgggtttcattccttcaaagcacatgtcctcctcttgatctgacatgtatcctggggggctggggacaccatccagcgtcactataaacttgggacttgcaggtttatctggttgtacaagatctcgtgtctgcataaggtgtcctgaaagtacccgaagggaatctgcagtcttcatccccgactcttggtttggtgccactactacttcctcagacagctttggcttcttcagaataaatgatcttgtgtctgcatggaccatggattccatgtcatagtaatcttgatttttttctacagaatctccttttgtttcctcttctttaatggggggacttattctgggggtcctactttgtccctggaccacttctgctagcaattcttcttgagaagttcgagttctgggagcaactggaagtgtctgtttctgtggaactgtagagtagttagttgtttttgttacggattcttgagcttcagatatagccttcaaaatcagattcttgttagcttgtttagaaggtggaagagaaggtctcctttcaggctttgcaggcacagacacactgctggagatgcttcctgttcgagacccgtaatcatcatcttcttcctcctcttctccatcatgattgaatttttttactttaacaactgaacttaccacaggcaactttctcttccgaaagttttcatcctccatactcattttctccgagttgtttctaaagaacggactatacgtttcttctaagctgttaagcacctctggttcacacaaacgtcctgtttcatatacccaactactctgcatatcaagctgcttggcagcatgaatactattctgctgctgttgaaattgcaacctgtttaaatgaacaccactatctgcatttctacttgcaggtggtcgataaatttcaatagaagggcgagaagaaccatatgtaagtgtcactgtaggttttttctgagataagggattctcctgcacaaagttgaggtcttcgtcaatgagatcatctggttctggcttaatatcaatcacatcttcagagggtgctggctccctcaaaggtttcactgttgacattagtcgggttgcagctccatcatcgtaagtctgtctgacatttgtggtttttgactcctgcgaacttgtagaaactctggaatctcttttttcaggtctcgcgctaggaatggcaagtggtggcactgcagcttcatgcctcctctcatctccccgactgaaattgctcttgtttgaaggcacgttactatcaaagatgttggtatcagaagacttcagactagagggttcagttgtaacagagcgaagtttatctaatacaccatgaagccatacggtgaatcgaattgtgttgttccctagaaacagggacagatcctctgtcatttggtcctgacttttcttgttggccaccatcaccataatgtaatcaggaagttcttcatcaacataagctcctaattcttgtaatttccccttaatggcactccggatcttgcggctgatctcggtgccgatctccatggctctgcggcgtgcgggaactcagcactgcgcggcgcttggcttacccggaggctgccgcggactcctaccccgcagccgggacaccaccgcctcc

SEQ ID NO: 17461 - RNA, 13758 nt, Homo sapiens
  source 1..13758: mol_type = other RNA
tcaggccaggcacagtggctcatacctggaatcccagcactttgggaggccgaggcaggcagatcacctgaggtcaaggtatttgagaccagcctggccaacatggtgaaaccccatctctactaaaaatacagaaattagctgggtgtggtggtgcacacctgtaatgctagctactcgggaggctgaggtaggagaatcgcttgaacctgggaggcagaggttgcaataagcctagatcatgccactgcactcaagcctgggagacagagcgagactacatcttaaaaaaaaaaaaaaaagtattatgagagaggataatgtattgtaatgtattgtagaggctaaataaaattatgctcatgtcagaaaaaaagagtatttctcaaaataaaattcactgaaactggatgtttattttgactgagatatagtatatcctcaaattgccatagaaagtttacaagaatattagaggtaaattataaatatcagggcctttttaaaaaaaaaagattctgcttataacttggtatttgtttataataaaaattatagtagccaataatgaacacttactctggcttggttatttacttaggtcaaaagaaggaggagcggttaaactgtgggatcaggaactgaggcggtgccgtgccttcaggcttgagacaggacaagccacagattgtgttcgttctgtgtgcagaggcaaagtaagatgttccatgagctgatacagtgcagcagaaaacagaaagtggttattactgtgattccctcaccctttgcagcctaatgaacaatacttaataatgcataacgatggatttgcttgccaacattactctgtctttgctgctttctttgccaaagttagcaccagtgtggtgcataagctaggaagctattctgtctaaatactgtatgtaaacctccaatattttctagaatctgccaatttaacaactctagtagacataattgaaagcccttggcagttgactcatattaggacagctgtctccattttttaaaaaaacacacattccctagataaaacgtgcagtaaacaaacaatgaaatactactcagccataaaaaataatgaaattctgtcattcttggtggcaacatggatgagactggaggacatgatgtgaagtgaaataagccaggcacagaaagataaatacatgttctcactcctgtgcagaaactaaaaaagttgatcccacagaggtggagagtagaatagtggttactggaggcggacaagggggagggggagggggatagggaaggactggttaaaggatacaagtttacacagccagataggaatagtatgttttagtattctgtagtactgtaggatgactatagttaagaatcacgtatttatgtattttcaggtatttacaagagaggattttgaaagtttccatcacaaagaaatgataaatgtctgaggtgatggttatgcgtattaccctatgccctatagatatgtataattatgtgtcaatttcaaaataaaaattcaaaactacaactcctatgaaaatttttgagcgtgtttgtacttattaagtgtatttataaatcatacggatattatcttcagcctgcatattaaattgtagttaagcttttactttttaactaaaaaataaattctattattttttcctatatcccactgcactgaccccagtttggaaatcctaagattatcaaataaaaactttgattattgaagaatccaggtgtactgccacagaaaagttctattctgtagcatggactctaatatgtaatctagcccattgtgcttacagatagatgtgtgcctgtagtcatagaaaaatttgcatgagctaatgactgccttgctactagattagctcaaagcaaaaagttctctgaaagcaggtcaatagggtcatttttatattatgaagaagaaaagcagctgttgtattacattcactgtattggtcctgcttgtgtttcagggcaagatccttgttgggacaaggaatgctgaaataatcgaagttggagagaaaaatgcagcttgtaatattttagttaacggtcatgtggatgggccaatctggggactagcaacacatccttccagggattttttcctttctgctgcagaagatgggacagtgagactttgggatattgctgataaagtaagtacagataatttttttaaaagaggttacaacttctaaaaagaaaagttggaagttctaaattgctagtacttaaagaactgccagaattctgttgagcattttgaggggaaactggtataatttagaagtacttcacttaatgtttcctatgactctttttttttttttttttaaatgcagaagatgttaaacaaagtgaatttgggacatgctgctcgtactgtgtgttacagccctgaaggggacatggtggctattggaatgaaaaatggagaatttatcattttactagtgagttctctaaaaatatggggaaagaagagagacaggagatgtgcaatccatgatatcaggttagtgaacaaatggaatagagtttctagtatatacttgatttaacttccatttgtaaaattttccatagccttgccttcaaaaagaggtccccagggcctgtagcatttcccgtattataaattgtatgctaaaatatggctgtttgtatactacttaattcttcttgctaaattataaacccactgggcaccaactataatagcaagtactagtaggtaatgtttgatgaattcatgttaacacttagccatgtccattaagttcatcccaccaagaggtatctcccactgtaatacaagagagctatctgcccttcaaaagttgtcaccctggaaaactaaagttgtgatttcaaacatatcttctcttagtaacctcagtttgggaatatgtagttcattaatttaatcaatacctattgattaaatgttccagaatccaaattaatttaaatgtttcttaaacctttgtttttcagtgcttaagcatttttcaacagtggctaccatttacggagtacttccgtgtgatcagtagataagattattgaatctaggtctgtcaaaagcttgtacacttttcatcagtaaaatccttttacaaatgaaaccttcctcagaacttcaatatataaaatagtaacagtggcttcccttagcttttacatgtctctatcgtacctcagtaagactcatgggccatttcaagagactgaattgtcccatatgactccaaagattgctaggcaaatagcatttcactttgtcttttaaataagttcttcaggccgggcgcggtggctcatgcctgtaatcccagcactttgggaggccgaggcaggcagatcacctgaagtcaggagtactcgaccagcctggccaacatagtgaaaccccatctcaactaaaaatacaaaaatcagccgggcgtggtggcaggcgcctgtaatcccagctactcagggggctgaaacaggagaatcgcttgaacccgggaggcggaggttgcgccatcgcactccagcctgggagacaagagcgagacttcgtctcaaaaaaaaaaaattcttcttccaagattcaagttgtgtcatttcaccttaataactggaggttagttaagctgggctgtgttctttgcttaatattaagacaacgttttttccagatggaagaaaactatcttaatgaattgttagcttattaattatgtaatgctaatggcttttaaaagctgagatgttctgactgggtgttgtggctcacacctgtaatcccagtaccttgggaggccaagggggaaggattgcttgaggccaggagtttgggaccatagtgagaccccgcctctatttaaaaaattaaattttgttttgttttgttttgagttggagttttgctcttgttgcccatgctgaagtgcaatggtgcaatctcagctcaccacaacctgtgcctcctgggttcaagcgattctcctgcttcagcctcccgagtagatgggattacaggcgtgcaccaccatgcctggctaattttgtatttttagtagagacagggtttctctatgttggtcaggctggtctcaaactctcgacctcaggtgatctgcccgcctccgcttcccaaagttctgggattataggtgtgagccactgggcctggcctaagaaagtttttttaagccattagacgtttttaaaggaattgggagatgacaattggggaaatatttaaaatttaagtaaaatataaagcttccttatttcatgtaacccagacaatctcagtatacatgatcagttgtgtctgacaggtaaatctatttgaggccttatcacacgttacttttaagaactagaaaggaaaagtcactgatcttaagtatttataatacttcatgtggtctaatactttttacgttttgttttgattcagatttagtccggattcccggtatctggcagtaggttctagtgagaactcagtggatttttatgacctaacgctgggccccactcttaacagaatcagctactgcaaagacattccaagctttgtcattcaaatggacttctctgcagatagcagttatctccaggtacagtaccaatactgtatacccaggtggcaagttcttctgcttttacatttcgtgttagtgaatgcatttaaagttcctgagctccagagctccagcttctcaactcctccctttgtaccttctgacctacagctcccctttcctcccccacttatcagagcttttctcctattaagtttttgtagtgatcttttgcatacttaataatgttagacatgtaaatcaagtagcaatatgctagtattctgtaaaccccctgtggattttgtctctcacctaatggaattcttgtcccattttaatctgatgaaaaaggtctctagtggctgctataaacggcatgtctatgaagtgccttcaggaaaacatcttatggatcatgccgctattgacagaattacttgggctacatggactaggtaaatacttatatattcacaaggcaagaactgactttgaaggccagttagaaaatcctatttctgaactgttagagccattccaataaggaatagtaattgagtttcaagtttttgttaccatattttgaaatggtatgttcatgttgggacccctttttattgaatatatttccatgttttatcagtttccatgatttatcaagttttttttttaaggaaatcaaagttttaactttaaagataccctgatatttttcttaatgctaaatttaatgactggcaaaaaggtattgggtgctgttaagcaactgttattaattctctatctaaaggaatgctatcttgaatctattagaagtcaaagcttccaaatttgttcaaatttcctggctgtatgacaggtaaccatgactatccatttttttggccaatgaaaaatgccatcaaattcctgtatcagccaggcatatagtggctcatgcctgtaatctctgatgtagcaggccgaggtgggaggatcacttgagcctagaagttttgataccagcctgggcaacatagcaagaccccatctctgaaatttttttaattcctatgtcataagtcatttttatttttgtagagatagggatctcacaatattgcccaggctggtctcaaactcttggcctcaagcagtcctcctgcctcagcctcccaaaatgttgggattactggtatgtgctgctggacccagccaagtagcacttttaatttgaaaaatagttctatcagttttcagtcaggcgcggtggctcagcctgtaatcccagcactttgggaggccgagcgggggtgatcacctgaggtcgggagttcgagactagcctgaccaacatggagaaaccctgtctctactaaaaatacaaaataagccgggcatgttagcgcatgcctgtgatcccagctactcgggaggctgaggcaggagaattgcttgaacccaggaggcagaggttgcggtgagccgagatcatgccattgcactccagcctgggtaacaagagcgaaaactccgtctcaaaaaaaaaaaaagaaaaaatagttctatcagttttcataaagtactactttaatcttaaaaagattaatctagaaacccttcaaattataaaatgtcatttttaaaaggcaggagttgatatcctgatgaaattcaggtctccaaacaacttaccataatttacttcctgtattttaagtaacatgatagggtacttagagattaattgccaagaaactttttgaatatagtcaacctgcccgcacttgccatgatgagttttcttttgttccttccctctagtattctaggagatgaggttttgggaatctggtccagacatgctgagaaagctgatgtcaactgtgcctgtgtatctcattcaggaatcagtcttgttacaggagatgactttggcatggttaagttatttgacttcccatgtccagaaaaatttgtaagtttgtgttttgtttactattatcagtttactcctaattttgatgtcttatcatcagcacttttccccatatatttaaaatgttttgtcctaatttctaaatttttccccaaactttctaaatctatttactttgaaataaaagctattagaaacaaatcctctccctcgagtaataccatctttggaaccatcctacaaaagctgtaattagcttttcaccaaacctataatcagttatcaaatttcaaatgcttttccttagagaaaaatggtcagagtacctggagacatctgactgcccacacagcctggttttgcagatccactactcatgctgaaaagcattctaatcactggctgcggtgctaactccctactctctccacagctcttgtcatagagattatagttcctaataagagcctttgacttctgtgtgcaccaaatgccctgagcttgtctgtcattgttttttaggcaaaacacaaaaggttcttgggtcattcgccccatgtgacaaatattcgatttaccagtggtgatcgacatgttgttagtgctggaggtgatgactgcaggttagtaactttctcagcccatgaagagcagactatgttactagttaagagacttaatacaacaactcctacagctttggtttatgaaatcagctagtcaacattagtagaaggtagtataaccagatggctcttcagaatctcatatttatgcaaatacagaataaaaggagttaaagaggaaaaatattacacatgtaacctgaaagcacaactgaaaaatattaaactgttatgaaaatctaaaaacataattaactccctgcaattttcttctctgattgcagcttatttgtctggaaatgtgtacatacacctcactgagagatgctgagatgactacagaaattaactttgagaccagaattacagagaagaaaaaccaaaacccaaccctgcatggtcaagtggtgctaacccaagactgtaacagggagaaatgcccagaatcatcaaaatagtgaaagactgatctgttcaaaatatttgctatatgcactgggtataatccgtaatccatacactgccagataatgccatttcaaggaaggatcgaatacttgatggtaaaggccaagtccccctgtattgggaagtgtgtgatttcggcagacctgctgggaaaatttagggtagagcactctttacagaagaactcaaaaacccaatttggataattttcattatctttttagcaaaatggtttcttaatgtttatattttattttcaaggttcattgtttaatgaaatattttattcttgcatttccataaggaaagggaaagtcatgatcatcctaaaggatcacagtttttaaaaggcaaacattttccctaaggaaacagacacaagctttcctagagaatatgatgttttttaggcattaataaggtccttttttataaaggacacttttctcctagtagttttgaattcaggaacagatccaaagttagcagtatatggctgctacatttccattttcattttcgagccatcagtttatgttcagatgccatctctgtaatcgcacatttaaaacataactgtagcctcactaatggaaaagtagtatgatgaacaatcattcccaatggtgtacaatgtaagggttttagggagcaacagtatttaactggaagaaagaattgcatatttaatgtagtctaatatatacacatttgtttaacatgtaaacaaaagtgttaaattcacatatacaacattatacaatttaatcactcttggaataaaatttttatagccttttttctattgggaaaatttgtttagatgtgtgccactccataggtttatttccaaaatgaatgagcccaactccatttgtaaaaacttgtcagttagaattcctttttttagtggattagggctgaattcttagatccttatttcttttcactttaaatgctgccaaagatcactactcatcattcaggaattcgctgtctagcctatctgtagtttcctgaagattgaaaattatgtagactgctatttaaaaatatatttttctaagtgtgaggtttaagatgctgtattgaccctatgagtttttaatgtgttaattatctttatagcataatagatcgctttaggttcctggaatcccatttggtctgacaggatatatgaagattcttaatacctattttctgtgtctaatacttggttaatactaaaaatagaaatgactaaattacatcacagaaagcataaccagtgattgaacctggtagttttaaagctctaaatagctgtggctgaaggactgattatggggctaagaagcttgaaacgtaagttggtacttgttcatcagtggattctcctaaattaagccaaattttgaaatacatgactattaagtttctactcatgtatttacagtcagtcaataaattaaaggaggaaaaaaatccctgaacaacctgcccataaaaagaaaaatactctacatttgagcctgctgcagttttaaattttccctctgggtcaagtttgccagcttttggctacagagaaattatatttccattacagtgcaggtagaaactctgtaaccttaagcatgtaaactacatagaataaaactgtttccactgcatttctgtccttcaaagtggccaacctgattaagtcagccttaatcactgctgctgtcagtttcacgactaaaggtcatattgactaagtagtcatcagctgaccacctcgctgtatcagccagcaacgaggggaaggtgaagaaacatgataggccatatagaatctgccctatgtttacttttttaacccagataattatttttgtgtgcagtatctaagctcctgattgtgtaacctgggacttctggcaccttttgttccattcattttatgtataaaatgcatgccaaagcacactgtgccctctggtacccttgcttccaatcgccaaccatgctcatttccttcctttttttgtggtccctttttgtggtgatcattttaaaccacgtcatccaacaaatgttttatggtcaaccttagcttgttcataagccatagcaactgaaagattaaactcttaaatatgtgtctgggcagtggctattaaatagcaaaaaacaatcagattttagtattttattatttccttgtaaaatggctgaactaaattaaacccttgtttcccatttgttctataatttatagtgaaactgagaacaaaactatctttataaatgatagctaaaagtatttccagatatttaaacaatttaaaataaatttcttctgcagagatgcaaagcatctcaacactggaatgaacaaatgccttaaattcaatggagtaaacctttagaatgaagaggaactgtcatttcacccaagccgaagacaacagccttatgcacttgtgtgctctgtctttgctgcttctcgtgtttcaagcctttcctgtgggatcagcacagcaaagtgcaacttaccaaatggtttaatgactggttaattctttcttctcccaatggaaaagcaatggcaacacaacagtagactgctggcttgacaatcttaaacgtgagcctttgcacatgtaggtttatcatcatttgagtatacgactaagcaagtcaatgaactttttttttttttttagcagtttaatttggtcctgagaatgttgcagtctttattaccccttttgcattaatccacttttctaaccaccttttaagctttaatttttaacactatacaccaagtctttgaaatcagtgatctgttatttaactctaaagcatttgacacttcttgccttaacagttttaaaaaccacacacaaaaaaactctgtaagtaatacagtaggccaaaagtttcatcctatctatcttgcagtttacctatctgatctgatctctgtaattatagttctgtcatttaaaatatactatttaaatctaatttttacatttcaaaaattatcttcagtagtaactaagtatattttctgtggattctgagaatgttatttttcagaatgtgagaatatatatgtacatttataatcttgtgactttaaagtctgttttcagatacagtatgtaaatacttgtaaaaaaatttgtataattttgtgataatgtagtttcccaaaaaaattatttagaaggcattatgttattagtaaatgagagcactgtatagaactgttcctattttctgcacttgccattccagctgcctccactgtccatacccacctcattcatcctgtcacagaaggcaggaaaactgggaactttaccaaagtagcactcagcctgagaggcctgtataatcatgcttttcaaactaaattcacttaaaaattaaaaagcagaattgaatattttaagcagcctcagtacctttggccaatgctgttttcatggtggattatgaacattatataatctttgggaaaagtgaaagtagtacaatttttagaataatgacaactgcctcactgcatctctccactcacacagcaaccgtgtagccccctaagctgcagtaccatgactaaccatgatgtcaatttcatatgctgatcctcacaacagcagtgcacaaacatgccccaaatattttaacagaatttagctcttccttaagctgtcttttcatagtaaaaacaaaacaaaaacacccaatgttaaaaccacataataaacttacaaacttgaaaaattagacacttcagatagataggcaataaaacttcatattatgaaagcaatatattccaagtttcaaagatttgacaagttctgtagagtatctttcatcagtacatgaaaacttccaaactgcatgatcttctgccaggcaggactgggtgctattcgctggtttgaggtcgaatccatttcaaggcatgtcgtggtgggacattaatggtgggatggtagaatgtgcagtccggtcttgtacattgagtgttaaacctacaatgttttggatgatagaagggacattccatcttcttacaagcagggaagtaacggcagagctgactactggaaggtggtgctggtggtgcaactggttttggagacagtactggaattcttctactcacatgagtgaagggacaatctggtttagtacactttgcatcatatttacaatttgggtgaacaaacaaacatttttcagcaaatttacaattggggaaggctttgcagggtgagatggggtgatggtaggcacactcatccccatttttacaagcaggccagtacttgcagcgctccaaaagtttttctggtttctgtgccacactcagttcactcatctcagcgttagaaaagctaccatttgggtcctcaagctgcctgctcagcaagtgcaactgctgtgggtggaggagacctctgagtcccttgtttgaggctgcagtttggtttacgggtttcattccttcaaagcacatgtcctcctcttgatctgacatgtatcctggggggctggggacaccatccagcgtcactataaacttgggacttgcaggtttatctggttgtacaagatctcgtgtctgcataaggtgtcctgaaagtacccgaagggaatctgcagtcttcatccccgactcttggtttggtgccactactacttcctcagacagctttggcttcttcagaataaatgatcttgtgtctgcatggaccatggattccatgtcatagtaatcttgactcatctgcagagtttctgccattactgggtcgatttgcagtcgggataataattgcctctgttgagttccttgatttttttctacagaatctccttttgtttcctcttctttaatggggggacttattctgggggtcctactttgtccctggaccacttctgctagcaattcttcttgagaagttcgagttctgggagcaactggaagtgtctgtttctgtggaactgtagagtagttagttgtttttgttacggattcttgagcttcagatatagccttcaaaatcagattcttgttagcttgtttagaaggtggaagagaaggtctcctttcaggctttgcaggcacagacacactgctggagatgcttcctgttcgagacccgtaatcatcatcttcttcctcctcttctccatcatgattgaatttttttactttaacaactgaacttaccacaggcaactttctcttccgaaagttttcatcctccatactcattttctccgagttgtttctaaagaacggactatacgtttcttctaagctgttaagcacctctggttcacacaaacgtcctgtttcatatacccaactactctgcatatcaagctgcttggcagcatgaatactattctgctgctgttgaaattgcaacctgtttaaatgaacaccactatctgcatttctacttgcaggtggtcgataaatttcaatagaagggcgagaagaaccatatgtaagtgtcactgtaggttttttctgagataagggattctcctgcacaaagttgaggtcttcgtcaatgagatcatctggttctggcttaatatcaatcacatcttcagagggtgctggctccctcaaaggtttcactgttgacattagtcgggttgcagctccatcatcgtaagtctgtctgacatttgtggtttttgactcctgcgaacttgtagaaactctggaatctcttttttcaggtctcgcgctaggaatggcaagtggtggcactgcagcttcatgcctcctctcatctccccgactgaaattgctcttgtttgaaggcacgttactatcaaagatgttggtatcagaagacttcagactagagggttcagttgtaacagagcgaagtttatctaatacaccatgaagccaacataagctcctaattcttgtaatttccccttaatggcactccggatcttgcggctgatctcggtgccgatctccatggctctgcggcgtgcgggaactcagcactgcgcggcgcttggcttacccggaggctgccgcggactcctaccccgcagccgggacaccaccgcctcc

SEQ ID NO: 17462 - RNA, 13873 nt, Homo sapiens
  source 1..13873: mol_type = other RNA
tcaggccaggcacagtggctcatacctggaatcccagcactttgggaggccgaggcaggcagatcacctgaggtcaaggtatttgagaccagcctggccaacatggtgaaaccccatctctactaaaaatacagaaattagctgggtgtggtggtgcacacctgtaatgctagctactcgggaggctgaggtaggagaatcgcttgaacctgggaggcagaggttgcaataagcctagatcatgccactgcactcaagcctgggagacagagcgagactacatcttaaaaaaaaaaaaaaaagtattatgagagaggataatgtattgtaatgtattgtagaggctaaataaaattatgctcatgtcagaaaaaaagagtatttctcaaaataaaattcactgaaactggatgtttattttgactgagatatagtatatcctcaaattgccatagaaagtttacaagaatattagaggtaaattataaatatcagggcctttttaaaaaaaaaagattctgcttataacttggtatttgtttataataaaaattatagtagccaataatgaacacttactctggcttggttatttacttaggtcaaaagaaggaggagcggttaaactgtgggatcaggaactgaggcggtgccgtgccttcaggcttgagacaggacaagccacagattgtgttcgttctgtgtgcagaggcaaagtaagatgttccatgagctgatacagtgcagcagaaaacagaaagtggttattactgtgattccctcaccctttgcagcctaatgaacaatacttaataatgcataacgatggatttgcttgccaacattactctgtctttgctgctttctttgccaaagttagcaccagtgtggtgcataagctaggaagctattctgtctaaatactgtatgtaaacctccaatattttctagaatctgccaatttaacaactctagtagacataattgaaagcccttggcagttgactcatattaggacagctgtctccattttttaaaaaaacacacattccctagataaaacgtgcagtaaacaaacaatgaaatactactcagccataaaaaataatgaaattctgtcattcttggtggcaacatggatgagactggaggacatgatgtgaagtgaaataagccaggcacagaaagataaatacatgttctcactcctgtgcagaaactaaaaaagttgatcccacagaggtggagagtagaatagtggttactggaggcggacaagggggagggggagggggatagggaaggactggttaaaggatacaagtttacacagccagataggaatagtatgttttagtattctgtagtactgtaggatgactatagttaagaatcacgtatttatgtattttcaggtatttacaagagaggattttgaaagtttccatcacaaagaaatgataaatgtctgaggtgatggttatgcgtattaccctatgccctatagatatgtataattatgtgtcaatttcaaaataaaaattcaaaactacaactcctatgaaaatttttgagcgtgtttgtacttattaagtgtatttataaatcatacggatattatcttcagcctgcatattaaattgtagttaagcttttactttttaactaaaaaataaattctattattttttcctatatcccactgcactgaccccagtttggaaatcctaagattatcaaataaaaactttgattattgaagaatccaggtgtactgccacagaaaagttctattctgtagcatggactctaatatgtaatctagcccattgtgcttacagatagatgtgtgcctgtagtcatagaaaaatttgcatgagctaatgactgccttgctactagattagctcaaagcaaaaagttctctgaaagcaggtcaatagggtcatttttatattatgaagaagaaaagcagctgttgtattacattcactgtattggtcctgcttgtgtttcagggcaagatccttgttgggacaaggaatgctgaaataatcgaagttggagagaaaaatgcagcttgtaatattttagttaacggtcatgtggatgggccaatctggggactagcaacacatccttccagggattttttcctttctgctgcagaagatgggacagtgagactttgggatattgctgataaagtaagtacagataatttttttaaaagaggttacaacttctaaaaagaaaagttggaagttctaaattgctagtacttaaagaactgccagaattctgttgagcattttgaggggaaactggtataatttagaagtacttcacttaatgtttcctatgactctttttttttttttttttaaatgcagaagatgttaaacaaagtgaatttgggacatgctgctcgtactgtgtgttacagccctgaaggggacatggtggctattggaatgaaaaatggagaatttatcattttactagtgagttctctaaaaatatggggaaagaagagagacaggagatgtgcaatccatgatatcaggttagtgaacaaatggaatagagtttctagtatatacttgatttaacttccatttgtaaaattttccatagccttgccttcaaaaagaggtccccagggcctgtagcatttcccgtattataaattgtatgctaaaatatggctgtttgtatactacttaattcttcttgctaaattataaacccactgggcaccaactataatagcaagtactagtaggtaatgtttgatgaattcatgttaacacttagccatgtccattaagttcatcccaccaagaggtatctcccactgtaatacaagagagctatctgcccttcaaaagttgtcaccctggaaaactaaagttgtgatttcaaacatatcttctcttagtaacctcagtttgggaatatgtagttcattaatttaatcaatacctattgattaaatgttccagaatccaaattaatttaaatgtttcttaaacctttgtttttcagtgcttaagcatttttcaacagtggctaccatttacggagtacttccgtgtgatcagtagataagattattgaatctaggtctgtcaaaagcttgtacacttttcatcagtaaaatccttttacaaatgaaaccttcctcagaacttcaatatataaaatagtaacagtggcttcccttagcttttacatgtctctatcgtacctcagtaagactcatgggccatttcaagagactgaattgtcccatatgactccaaagattgctaggcaaatagcatttcactttgtcttttaaataagttcttcaggccgggcgcggtggctcatgcctgtaatcccagcactttgggaggccgaggcaggcagatcacctgaagtcaggagtactcgaccagcctggccaacatagtgaaaccccatctcaactaaaaatacaaaaatcagccgggcgtggtggcaggcgcctgtaatcccagctactcagggggctgaaacaggagaatcgcttgaacccgggaggcggaggttgcgccatcgcactccagcctgggagacaagagcgagacttcgtctcaaaaaaaaaaaattcttcttccaagattcaagttgtgtcatttcaccttaataactggaggttagttaagctgggctgtgttctttgcttaatattaagacaacgttttttccagatggaagaaaactatcttaatgaattgttagcttattaattatgtaatgctaatggcttttaaaagctgagatgttctgactgggtgttgtggctcacacctgtaatcccagtaccttgggaggccaagggggaaggattgcttgaggccaggagtttgggaccatagtgagaccccgcctctatttaaaaaattaaattttgttttgttttgttttgagttggagttttgctcttgttgcccatgctgaagtgcaatggtgcaatctcagctcaccacaacctgtgcctcctgggttcaagcgattctcctgcttcagcctcccgagtagatgggattacaggcgtgcaccaccatgcctggctaattttgtatttttagtagagacagggtttctctatgttggtcaggctggtctcaaactctcgacctcaggtgatctgcccgcctccgcttcccaaagttctgggattataggtgtgagccactgggcctggcctaagaaagtttttttaagccattagacgtttttaaaggaattgggagatgacaattggggaaatatttaaaatttaagtaaaatataaagcttccttatttcatgtaacccagacaatctcagtatacatgatcagttgtgtctgacaggtaaatctatttgaggccttatcacacgttacttttaagaactagaaaggaaaagtcactgatcttaagtatttataatacttcatgtggtctaatactttttacgttttgttttgattcagatttagtccggattcccggtatctggcagtaggttctagtgagaactcagtggatttttatgacctaacgctgggccccactcttaacagaatcagctactgcaaagacattccaagctttgtcattcaaatggacttctctgcagatagcagttatctccaggtacagtaccaatactgtatacccaggtggcaagttcttctgcttttacatttcgtgttagtgaatgcatttaaagttcctgagctccagagctccagcttctcaactcctccctttgtaccttctgacctacagctcccctttcctcccccacttatcagagcttttctcctattaagtttttgtagtgatcttttgcatacttaataatgttagacatgtaaatcaagtagcaatatgctagtattctgtaaaccccctgtggattttgtctctcacctaatggaattcttgtcccattttaatctgatgaaaaaggtctctagtggctgctataaacggcatgtctatgaagtgccttcaggaaaacatcttatggatcatgccgctattgacagaattacttgggctacatggactaggtaaatacttatatattcacaaggcaagaactgactttgaaggccagttagaaaatcctatttctgaactgttagagccattccaataaggaatagtaattgagtttcaagtttttgttaccatattttgaaatggtatgttcatgttgggacccctttttattgaatatatttccatgttttatcagtttccatgatttatcaagttttttttttaaggaaatcaaagttttaactttaaagataccctgatatttttcttaatgctaaatttaatgactggcaaaaaggtattgggtgctgttaagcaactgttattaattctctatctaaaggaatgctatcttgaatctattagaagtcaaagcttccaaatttgttcaaatttcctggctgtatgacaggtaaccatgactatccatttttttggccaatgaaaaatgccatcaaattcctgtatcagccaggcatatagtggctcatgcctgtaatctctgatgtagcaggccgaggtgggaggatcacttgagcctagaagttttgataccagcctgggcaacatagcaagaccccatctctgaaatttttttaattcctatgtcataagtcatttttatttttgtagagatagggatctcacaatattgcccaggctggtctcaaactcttggcctcaagcagtcctcctgcctcagcctcccaaaatgttgggattactggtatgtgctgctggacccagccaagtagcacttttaatttgaaaaatagttctatcagttttcagtcaggcgcggtggctcagcctgtaatcccagcactttgggaggccgagcgggggtgatcacctgaggtcgggagttcgagactagcctgaccaacatggagaaaccctgtctctactaaaaatacaaaataagccgggcatgttagcgcatgcctgtgatcccagctactcgggaggctgaggcaggagaattgcttgaacccaggaggcagaggttgcggtgagccgagatcatgccattgcactccagcctgggtaacaagagcgaaaactccgtctcaaaaaaaaaaaaagaaaaaatagttctatcagttttcataaagtactactttaatcttaaaaagattaatctagaaacccttcaaattataaaatgtcatttttaaaaggcaggagttgatatcctgatgaaattcaggtctccaaacaacttaccataatttacttcctgtattttaagtaacatgatagggtacttagagattaattgccaagaaactttttgaatatagtcaacctgcccgcacttgccatgatgagttttcttttgttccttccctctagtattctaggagatgaggttttgggaatctggtccagacatgctgagaaagctgatgtcaactgtgcctgtgtatctcattcaggaatcagtcttgttacaggagatgactttggcatggttaagttatttgacttcccatgtccagaaaaatttgtaagtttgtgttttgtttactattatcagtttactcctaattttgatgtcttatcatcagcacttttccccatatatttaaaatgttttgtcctaatttctaaatttttccccaaactttctaaatctatttactttgaaataaaagctattagaaacaaatcctctccctcgagtaataccatctttggaaccatcctacaaaagctgtaattagcttttcaccaaacctataatcagttatcaaatttcaaatgcttttccttagagaaaaatggtcagagtacctggagacatctgactgcccacacagcctggttttgcagatccactactcatgctgaaaagcattctaatcactggctgcggtgctaactccctactctctccacagctcttgtcatagagattatagttcctaataagagcctttgacttctgtgtgcaccaaatgccctgagcttgtctgtcattgttttttaggcaaaacacaaaaggttcttgggtcattcgccccatgtgacaaatattcgatttaccagtggtgatcgacatgttgttagtgctggaggtgatgactgcaggttagtaactttctcagcccatgaagagcagactatgttactagttaagagacttaatacaacaactcctacagctttggtttatgaaatcagctagtcaacattagtagaaggtagtataaccagatggctcttcagaatctcatatttatgcaaatacagaataaaaggagttaaagaggaaaaatattacacatgtaacctgaaagcacaactgaaaaatattaaactgttatgaaaatctaaaaacataattaactccctgcaattttcttctctgattgcagcttatttgtctggaaatgtgtacatacacctcactgagagatgctgagatgactacagaaattaactttgagaccagaattacagagaagaaaaaccaaaacccaaccctgcatggtcaagtggtgctaacccaagactgtaacagggagaaatgcccagaatcatcaaaatagtgaaagactgatctgttcaaaatatttgctatatgcactgggtataatccgtaatccatacactgccagataatgccatttcaaggaaggatcgaatacttgatggtaaaggccaagtccccctgtattgggaagtgtgtgatttcggcagacctgctgggaaaatttagggtagagcactctttacagaagaactcaaaaacccaatttggataattttcattatctttttagcaaaatggtttcttaatgtttatattttattttcaaggttcattgtttaatgaaatattttattcttgcatttccataaggaaagggaaagtcatgatcatcctaaaggatcacagtttttaaaaggcaaacattttccctaaggaaacagacacaagctttcctagagaatatgatgttttttaggcattaataaggtccttttttataaaggacacttttctcctagtagttttgaattcaggaacagatccaaagttagcagtatatggctgctacatttccattttcattttcgagccatcagtttatgttcagatgccatctctgtaatcgcacatttaaaacataactgtagcctcactaatggaaaagtagtatgatgaacaatcattcccaatggtgtacaatgtaagggttttagggagcaacagtatttaactggaagaaagaattgcatatttaatgtagtctaatatatacacatttgtttaacatgtaaacaaaagtgttaaattcacatatacaacattatacaatttaatcactcttggaataaaatttttatagccttttttctattgggaaaatttgtttagatgtgtgccactccataggtttatttccaaaatgaatgagcccaactccatttgtaaaaacttgtcagttagaattcctttttttagtggattagggctgaattcttagatccttatttcttttcactttaaatgctgccaaagatcactactcatcattcaggaattcgctgtctagcctatctgtagtttcctgaagattgaaaattatgtagactgctatttaaaaatatatttttctaagtgtgaggtttaagatgctgtattgaccctatgagtttttaatgtgttaattatctttatagcataatagatcgctttaggttcctggaatcccatttggtctgacaggatatatgaagattcttaatacctattttctgtgtctaatacttggttaatactaaaaatagaaatgactaaattacatcacagaaagcataaccagtgattgaacctggtagttttaaagctctaaatagctgtggctgaaggactgattatggggctaagaagcttgaaacgtaagttggtacttgttcatcagtggattctcctaaattaagccaaattttgaaatacatgactattaagtttctactcatgtatttacagtcagtcaataaattaaaggaggaaaaaaatccctgaacaacctgcccataaaaagaaaaatactctacatttgagcctgctgcagttttaaattttccctctgggtcaagtttgccagcttttggctacagagaaattatatttccattacagtgcaggtagaaactctgtaaccttaagcatgtaaactacatagaataaaactgtttccactgcatttctgtccttcaaagtggccaacctgattaagtcagccttaatcactgctgctgtcagtttcacgactaaaggtcatattgactaagtagtcatcagctgaccacctcgctgtatcagccagcaacgaggggaaggtgaagaaacatgataggccatatagaatctgccctatgtttacttttttaacccagataattatttttgtgtgcagtatctaagctcctgattgtgtaacctgggacttctggcaccttttgttccattcattttatgtataaaatgcatgccaaagcacactgtgccctctggtacccttgcttccaatcgccaaccatgctcatttccttcctttttttgtggtccctttttgtggtgatcattttaaaccacgtcatccaacaaatgttttatggtcaaccttagcttgttcataagccatagcaactgaaagattaaactcttaaatatgtgtctgggcagtggctattaaatagcaaaaaacaatcagattttagtattttattatttccttgtaaaatggctgaactaaattaaacccttgtttcccatttgttctataatttatagtgaaactgagaacaaaactatctttataaatgatagctaaaagtatttccagatatttaaacaatttaaaataaatttcttctgcagagatgcaaagcatctcaacactggaatgaacaaatgccttaaattcaatggagtaaacctttagaatgaagaggaactgtcatttcacccaagccgaagacaacagccttatgcacttgtgtgctctgtctttgctgcttctcgtgtttcaagcctttcctgtgggatcagcacagcaaagtgcaacttaccaaatggtttaatgactggttaattctttcttctcccaatggaaaagcaatggcaacacaacagtagactgctggcttgacaatcttaaacgtgagcctttgcacatgtaggtttatcatcatttgagtatacgactaagcaagtcaatgaactttttttttttttttagcagtttaatttggtcctgagaatgttgcagtctttattaccccttttgcattaatccacttttctaaccaccttttaagctttaatttttaacactatacaccaagtctttgaaatcagtgatctgttatttaactctaaagcatttgacacttcttgccttaacagttttaaaaaccacacacaaaaaaactctgtaagtaatacagtaggccaaaagtttcatcctatctatcttgcagtttacctatctgatctgatctctgtaattatagttctgtcatttaaaatatactatttaaatctaatttttacatttcaaaaattatcttcagtagtaactaagtatattttctgtggattctgagaatgttatttttcagaatgtgagaatatatatgtacatttataatcttgtgactttaaagtctgttttcagatacagtatgtaaatacttgtaaaaaaatttgtataattttgtgataatgtagtttcccaaaaaaattatttagaaggcattatgttattagtaaatgagagcactgtatagaactgttcctattttctgcacttgccattccagctgcctccactgtccatacccacctcattcatcctgtcacagaaggcaggaaaactgggaactttaccaaagtagcactcagcctgagaggcctgtataatcatgcttttcaaactaaattcacttaaaaattaaaaagcagaattgaatattttaagcagcctcagtacctttggccaatgctgttttcatggtggattatgaacattatataatctttgggaaaagtgaaagtagtacaatttttagaataatgacaactgcctcactgcatctctccactcacacagcaaccgtgtagccccctaagctgcagtaccatgactaaccatgatgtcaatttcatatgctgatcctcacaacagcagtgcacaaacatgccccaaatattttaacagaatttagctcttccttaagctgtcttttcatagtaaaaacaaaacaaaaacacccaatgttaaaaccacataataaacttacaaacttgaaaaattagacacttcagatagataggcaataaaacttcatattatgaaagcaatatattccaagtttcaaagatttgacaagttctgtagagtatctttcatcagtacatgaaaacttccaaactgcatgatcttctgccaggcaggactgggtgctattcgctggtttgaggtcgaatccatttcaaggcatgtcgtggtgggacattaatggtgggatggtagaatgtgcagtccggtcttgtacattgagtgttaaacctacaatgttttggatgatagaagggacattccatcttcttacaagcagggaagtaacggcagagctgactactggaaggtggtgctggtggtgcaactggttttggagacagtactggaattcttctactcacatgagtgaagggacaatctggtttagtacactttgcatcatatttacaatttgggtgaacaaacaaacatttttcagcaaatttacaattggggaaggctttgcagggtgagatggggtgatggtaggcacactcatccccatttttacaagcaggccagtacttgcagcgctccaaaagtttttctggtttctgtgccacactcagttcactcatctcagcgttagaaaagctaccatttgggtcctcaagctgcctgctcagcaagtgcaactgctgtgggtggaggagacctctgagtcccttgtttgaggctgcagtttggtttacgggtttcattccttcaaagcacatgtcctcctcttgatctgacatgtatcctggggggctggggacaccatccagcgtcactataaacttgggacttgcaggtttatctggttgtacaagatctcgtgtctgcataaggtgtcctgaaagtacccgaagggaatctgcagtcttcatccccgactcttggtttggtgccactactacttcctcagacagctttggcttcttcagaataaatgatcttgtgtctgcatggaccatggattccatgtcatagtaatcttgactcatctgcagagtttctgccattactgggtcgatttgcagtcgggataataattgcctctgttgagttccttgatttttttctacagaatctccttttgtttcctcttctttaatggggggacttattctgggggtcctactttgtccctggaccacttctgctagcaattcttcttgagaagttcgagttctgggagcaactggaagtgtctgtttctgtggaactgtagagtagttagttgtttttgttacggattcttgagcttcagatatagccttcaaaatcagattcttgttagcttgtttagaaggtggaagagaaggtctcctttcaggctttgcaggcacagacacactgctggagatgcttcctgttcgagacccgtaatcatcatcttcttcctcctcttctccatcatgattgaatttttttactttaacaactgaacttaccacaggcaactttctcttccgaaagttttcatcctccatactcattttctccgagttgtttctaaagaacggactatacgtttcttctaagctgttaagcacctctggttcacacaaacgtcctgtttcatatacccaactactctgcatatcaagctgcttggcagcatgaatactattctgctgctgttgaaattgcaacctgtttaaatgaacaccactatctgcatttctacttgcaggtggtcgataaatttcaatagaagggcgagaagaaccatatgtaagtgtcactgtaggttttttctgagataagggattctcctgcacaaagttgaggtcttcgtcaatgagatcatctggttctggcttaatatcaatcacatcttcagagggtgctggctccctcaaaggtttcactgttgacattagtcgggttgcagctccatcatcgtaagtctgtctgacatttgtggtttttgactcctgcgaacttgtagaaactctggaatctcttttttcaggtctcgcgctaggaatggcaagtggtggcactgcagcttcatgcctcctctcatctccccgactgaaattgctcttgtttgaaggcacgttactatcaaagatgttggtatcagaagacttcagactagagggttcagttgtaacagagcgaagtttatctaatacaccatgaagccatacggtgaatcgaattgtgttgttccctagaaacagggacagatcctctgtcatttggtcctgacttttcttgttggccaccatcaccataatgtaatcaggaagttcttcatcaacataagctcctaattcttgtaatttccccttaatggcactccggatcttgcggctgatctcggtgccgatctccatggctctgcggcgtgcgggaactcagcactgcgcggcgcttggcttacccggaggctgccgcggactcctaccccgcagccgggacaccaccgcctcc

SEQ ID NO: 17463 - RNA, 13849 nt, Homo sapiens
  source 1..13849: mol_type = other RNA
tcaggccaggcacagtggctcatacctggaatcccagcactttgggaggccgaggcaggcagatcacctgaggtcaaggtatttgagaccagcctggccaacatggtgaaaccccatctctactaaaaatacagaaattagctgggtgtggtggtgcacacctgtaatgctagctactcgggaggctgaggtaggagaatcgcttgaacctgggaggcagaggttgcaataagcctagatcatgccactgcactcaagcctgggagacagagcgagactacatcttaaaaaaaaaaaaaaaagtattatgagagaggataatgtattgtaatgtattgtagaggctaaataaaattatgctcatgtcagaaaaaaagagtatttctcaaaataaaattcactgaaactggatgtttattttgactgagatatagtatatcctcaaattgccatagaaagtttacaagaatattagaggtaaattataaatatcagggcctttttaaaaaaaaaagattctgcttataacttggtatttgtttataataaaaattatagtagccaataatgaacacttactctggcttggttatttacttaggtcaaaagaaggaggagcggttaaactgtgggatcaggaactgaggcggtgccgtgccttcaggcttgagacaggacaagccacagattgtgttcgttctgtgtgcagaggcaaagtaagatgttccatgagctgatacagtgcagcagaaaacagaaagtggttattactgtgattccctcaccctttgcagcctaatgaacaatacttaataatgcataacgatggatttgcttgccaacattactctgtctttgctgctttctttgccaaagttagcaccagtgtggtgcataagctaggaagctattctgtctaaatactgtatgtaaacctccaatattttctagaatctgccaatttaacaactctagtagacataattgaaagcccttggcagttgactcatattaggacagctgtctccattttttaaaaaaacacacattccctagataaaacgtgcagtaaacaaacaatgaaatactactcagccataaaaaataatgaaattctgtcattcttggtggcaacatggatgagactggaggacatgatgtgaagtgaaataagccaggcacagaaagataaatacatgttctcactcctgtgcagaaactaaaaaagttgatcccacagaggtggagagtagaatagtggttactggaggcggacaagggggagggggagggggatagggaaggactggttaaaggatacaagtttacacagccagataggaatagtatgttttagtattctgtagtactgtaggatgactatagttaagaatcacgtatttatgtattttcaggtatttacaagagaggattttgaaagtttccatcacaaagaaatgataaatgtctgaggtgatggttatgcgtattaccctatgccctatagatatgtataattatgtgtcaatttcaaaataaaaattcaaaactacaactcctatgaaaatttttgagcgtgtttgtacttattaagtgtatttataaatcatacggatattatcttcagcctgcatattaaattgtagttaagcttttactttttaactaaaaaataaattctattattttttcctatatcccactgcactgaccccagtttggaaatcctaagattatcaaataaaaactttgattattgaagaatccaggtgtactgccacagaaaagttctattctgtagcatggactctaatatgtaatctagcccattgtgcttacagatagatgtgtgcctgtagtcatagaaaaatttgcatgagctaatgactgccttgctactagattagctcaaagcaaaaagttctctgaaagcaggtcaatagggtcatttttatattatgaagaagaaaagcagctgttgtattacattcactgtattggtcctgcttgtgtttcagggcaagatccttgttgggacaaggaatgctgaaataatcgaagttggagagaaaaatgcagcttgtaatattttagttaacggtcatgtggatgggccaatctggggactagcaacacatccttccagggattttttcctttctgctgcagaagatgggacagtgagactttgggatattgctgataaagtaagtacagataatttttttaaaagaggttacaacttctaaaaagaaaagttggaagttctaaattgctagtacttaaagaactgccagaattctgttgagcattttgaggggaaactggtataatttagaagtacttcacttaatgtttcctatgactctttttttttttttttttaaatgcagaagatgttaaacaaagtgaatttgggacatgctgctcgtactgtgtgttacagccctgaaggggacatggtggctattggaatgaaaaatggagaatttatcattttactagtgagttctctaaaaatatggggaaagaagagagacaggagatgtgcaatccatgatatcaggttagtgaacaaatggaatagagtttctagtatatacttgatttaacttccatttgtaaaattttccatagccttgccttcaaaaagaggtccccagggcctgtagcatttcccgtattataaattgtatgctaaaatatggctgtttgtatactacttaattcttcttgctaaattataaacccactgggcaccaactataatagcaagtactagtaggtaatgtttgatgaattcatgttaacacttagccatgtccattaagttcatcccaccaagaggtatctcccactgtaatacaagagagctatctgcccttcaaaagttgtcaccctggaaaactaaagttgtgatttcaaacatatcttctcttagtaacctcagtttgggaatatgtagttcattaatttaatcaatacctattgattaaatgttccagaatccaaattaatttaaatgtttcttaaacctttgtttttcagtgcttaagcatttttcaacagtggctaccatttacggagtacttccgtgtgatcagtagataagattattgaatctaggtctgtcaaaagcttgtacacttttcatcagtaaaatccttttacaaatgaaaccttcctcagaacttcaatatataaaatagtaacagtggcttcccttagcttttacatgtctctatcgtacctcagtaagactcatgggccatttcaagagactgaattgtcccatatgactccaaagattgctaggcaaatagcatttcactttgtcttttaaataagttcttcaggccgggcgcggtggctcatgcctgtaatcccagcactttgggaggccgaggcaggcagatcacctgaagtcaggagtactcgaccagcctggccaacatagtgaaaccccatctcaactaaaaatacaaaaatcagccgggcgtggtggcaggcgcctgtaatcccagctactcagggggctgaaacaggagaatcgcttgaacccgggaggcggaggttgcgccatcgcactccagcctgggagacaagagcgagacttcgtctcaaaaaaaaaaaattcttcttccaagattcaagttgtgtcatttcaccttaataactggaggttagttaagctgggctgtgttctttgcttaatattaagacaacgttttttccagatggaagaaaactatcttaatgaattgttagcttattaattatgtaatgctaatggcttttaaaagctgagatgttctgactgggtgttgtggctcacacctgtaatcccagtaccttgggaggccaagggggaaggattgcttgaggccaggagtttgggaccatagtgagaccccgcctctatttaaaaaattaaattttgttttgttttgttttgagttggagttttgctcttgttgcccatgctgaagtgcaatggtgcaatctcagctcaccacaacctgtgcctcctgggttcaagcgattctcctgcttcagcctcccgagtagatgggattacaggcgtgcaccaccatgcctggctaattttgtatttttagtagagacagggtttctctatgttggtcaggctggtctcaaactctcgacctcaggtgatctgcccgcctccgcttcccaaagttctgggattataggtgtgagccactgggcctggcctaagaaagtttttttaagccattagacgtttttaaaggaattgggagatgacaattggggaaatatttaaaatttaagtaaaatataaagcttccttatttcatgtaacccagacaatctcagtatacatgatcagttgtgtctgacaggtaaatctatttgaggccttatcacacgttacttttaagaactagaaaggaaaagtcactgatcttaagtatttataatacttcatgtggtctaatactttttacgttttgttttgattcagatttagtccggattcccggtatctggcagtaggttctagtgagaactcagtggatttttatgacctaacgctgggccccactcttaacagaatcagctactgcaaagacattccaagctttgtcattcaaatggacttctctgcagatagcagttatctccaggtacagtaccaatactgtatacccaggtggcaagttcttctgcttttacatttcgtgttagtgaatgcatttaaagttcctgagctccagagctccagcttctcaactcctccctttgtaccttctgacctacagctcccctttcctcccccacttatcagagcttttctcctattaagtttttgtagtgatcttttgcatacttaataatgttagacatgtaaatcaagtagcaatatgctagtattctgtaaaccccctgtggattttgtctctcacctaatggaattcttgtcccattttaatctgatgaaaaaggtctctagtggctgctataaacggcatgtctatgaagtgccttcaggaaaacatcttatggatcatgccgctattgacagaattacttgggctacatggactaggtaaatacttatatattcacaaggcaagaactgactttgaaggccagttagaaaatcctatttctgaactgttagagccattccaataaggaatagtaattgagtttcaagtttttgttaccatattttgaaatggtatgttcatgttgggacccctttttattgaatatatttccatgttttatcagtttccatgatttatcaagttttttttttaaggaaatcaaagttttaactttaaagataccctgatatttttcttaatgctaaatttaatgactggcaaaaaggtattgggtgctgttaagcaactgttattaattctctatctaaaggaatgctatcttgaatctattagaagtcaaagcttccaaatttgttcaaatttcctggctgtatgacaggtaaccatgactatccatttttttggccaatgaaaaatgccatcaaattcctgtatcagccaggcatatagtggctcatgcctgtaatctctgatgtagcaggccgaggtgggaggatcacttgagcctagaagttttgataccagcctgggcaacatagcaagaccccatctctgaaatttttttaattcctatgtcataagtcatttttatttttgtagagatagggatctcacaatattgcccaggctggtctcaaactcttggcctcaagcagtcctcctgcctcagcctcccaaaatgttgggattactggtatgtgctgctggacccagccaagtagcacttttaatttgaaaaatagttctatcagttttcagtcaggcgcggtggctcagcctgtaatcccagcactttgggaggccgagcgggggtgatcacctgaggtcgggagttcgagactagcctgaccaacatggagaaaccctgtctctactaaaaatacaaaataagccgggcatgttagcgcatgcctgtgatcccagctactcgggaggctgaggcaggagaattgcttgaacccaggaggcagaggttgcggtgagccgagatcatgccattgcactccagcctgggtaacaagagcgaaaactccgtctcaaaaaaaaaaaaagaaaaaatagttctatcagttttcataaagtactactttaatcttaaaaagattaatctagaaacccttcaaattataaaatgtcatttttaaaaggcaggagttgatatcctgatgaaattcaggtctccaaacaacttaccataatttacttcctgtattttaagtaacatgatagggtacttagagattaattgccaagaaactttttgaatatagtcaacctgcccgcacttgccatgatgagttttcttttgttccttccctctagtattctaggagatgaggttttgggaatctggtccagacatgctgagaaagctgatgtcaactgtgcctgtgtatctcattcaggaatcagtcttgttacaggagatgactttggcatggttaagttatttgacttcccatgtccagaaaaatttgtaagtttgtgttttgtttactattatcagtttactcctaattttgatgtcttatcatcagcacttttccccatatatttaaaatgttttgtcctaatttctaaatttttccccaaactttctaaatctatttactttgaaataaaagctattagaaacaaatcctctccctcgagtaataccatctttggaaccatcctacaaaagctgtaattagcttttcaccaaacctataatcagttatcaaatttcaaatgcttttccttagagaaaaatggtcagagtacctggagacatctgactgcccacacagcctggttttgcagatccactactcatgctgaaaagcattctaatcactggctgcggtgctaactccctactctctccacagctcttgtcatagagattatagttcctaataagagcctttgacttctgtgtgcaccaaatgccctgagcttgtctgtcattgttttttaggcaaaacacaaaaggttcttgggtcattcgccccatgtgacaaatattcgatttaccagtggtgatcgacatgttgttagtgctggaggtgatgactgcaggttagtaactttctcagcccatgaagagcagactatgttactagttaagagacttaatacaacaactcctacagctttggtttatgaaatcagctagtcaacattagtagaaggtagtataaccagatggctcttcagaatctcatatttatgcaaatacagaataaaaggagttaaagaggaaaaatattacacatgtaacctgaaagcacaactgaaaaatattaaactgttatgaaaatctaaaaacataattaactccctgcaattttcttctctgattgcagcttatttgtctggaaatgtgtacatacacctcactgagagatgctgagatgactacagaaattaactttgagaccagaattacagagaagaaaaaccaaaacccaaccctgcatggtcaagtggtgctaacccaagactgtaacagggagaaatgcccagaatcatcaaaatagtgaaagactgatctgttcaaaatatttgctatatgcactgggtataatccgtaatccatacactgccagataatgccatttcaaggaaggatcgaatacttgatggtaaaggccaagtccccctgtattgggaagtgtgtgatttcggcagacctgctgggaaaatttagggtagagcactctttacagaagaactcaaaaacccaatttggataattttcattatctttttagcaaaatggtttcttaatgtttatattttattttcaaggttcattgtttaatgaaatattttattcttgcatttccataaggaaagggaaagtcatgatcatcctaaaggatcacagtttttaaaaggcaaacattttccctaaggaaacagacacaagctttcctagagaatatgatgttttttaggcattaataaggtccttttttataaaggacacttttctcctagtagttttgaattcaggaacagatccaaagttagcagtatatggctgctacatttccattttcattttcgagccatcagtttatgttcagatgccatctctgtaatcgcacatttaaaacataactgtagcctcactaatggaaaagtagtatgatgaacaatcattcccaatggtgtacaatgtaagggttttagggagcaacagtatttaactggaagaaagaattgcatatttaatgtagtctaatatatacacatttgtttaacatgtaaacaaaagtgttaaattcacatatacaacattatacaatttaatcactcttggaataaaatttttatagccttttttctattgggaaaatttgtttagatgtgtgccactccataggtttatttccaaaatgaatgagcccaactccatttgtaaaaacttgtcagttagaattcctttttttagtggattagggctgaattcttagatccttatttcttttcactttaaatgctgccaaagatcactactcatcattcaggaattcgctgtctagcctatctgtagtttcctgaagattgaaaattatgtagactgctatttaaaaatatatttttctaagtgtgaggtttaagatgctgtattgaccctatgagtttttaatgtgttaattatctttatagcataatagatcgctttaggttcctggaatcccatttggtctgacaggatatatgaagattcttaatacctattttctgtgtctaatacttggttaatactaaaaatagaaatgactaaattacatcacagaaagcataaccagtgattgaacctggtagttttaaagctctaaatagctgtggctgaaggactgattatggggctaagaagcttgaaacgtaagttggtacttgttcatcagtggattctcctaaattaagccaaattttgaaatacatgactattaagtttctactcatgtatttacagtcagtcaataaattaaaggaggaaaaaaatccctgaacaacctgcccataaaaagaaaaatactctacatttgagcctgctgcagttttaaattttccctctgggtcaagtttgccagcttttggctacagagaaattatatttccattacagtgcaggtagaaactctgtaaccttaagcatgtaaactacatagaataaaactgtttccactgcatttctgtccttcaaagtggccaacctgattaagtcagccttaatcactgctgctgtcagtttcacgactaaaggtcatattgactaagtagtcatcagctgaccacctcgctgtatcagccagcaacgaggggaaggtgaagaaacatgataggccatatagaatctgccctatgtttacttttttaacccagataattatttttgtgtgcagtatctaagctcctgattgtgtaacctgggacttctggcaccttttgttccattcattttatgtataaaatgcatgccaaagcacactgtgccctctggtacccttgcttccaatcgccaaccatgctcatttccttcctttttttgtggtccctttttgtggtgatcattttaaaccacgtcatccaacaaatgttttatggtcaaccttagcttgttcataagccatagcaactgaaagattaaactcttaaatatgtgtctgggcagtggctattaaatagcaaaaaacaatcagattttagtattttattatttccttgtaaaatggctgaactaaattaaacccttgtttcccatttgttctataatttatagtgaaactgagaacaaaactatctttataaatgatagctaaaagtatttccagatatttaaacaatttaaaataaatttcttctgcagagatgcaaagcatctcaacactggaatgaacaaatgccttaaattcaatggagtaaacctttagaatgaagaggaactgtcatttcacccaagccgaagacaacagccttatgcacttgtgtgctctgtctttgctgcttctcgtgtttcaagcctttcctgtgggatcagcacagcaaagtgcaacttaccaaatggtttaatgactggttaattctttcttctcccaatggaaaagcaatggcaacacaacagtagactgctggcttgacaatcttaaacgtgagcctttgcacatgtaggtttatcatcatttgagtatacgactaagcaagtcaatgaactttttttttttttttagcagtttaatttggtcctgagaatgttgcagtctttattaccccttttgcattaatccacttttctaaccaccttttaagctttaatttttaacactatacaccaagtctttgaaatcagtgatctgttatttaactctaaagcatttgacacttcttgccttaacagttttaaaaaccacacacaaaaaaactctgtaagtaatacagtaggccaaaagtttcatcctatctatcttgcagtttacctatctgatctgatctctgtaattatagttctgtcatttaaaatatactatttaaatctaatttttacatttcaaaaattatcttcagtagtaactaagtatattttctgtggattctgagaatgttatttttcagaatgtgagaatatatatgtacatttataatcttgtgactttaaagtctgttttcagatacagtatgtaaatacttgtaaaaaaatttgtataattttgtgataatgtagtttcccaaaaaaattatttagaaggcattatgttattagtaaatgagagcactgtatagaactgttcctattttctgcacttgccattccagctgcctccactgtccatacccacctcattcatcctgtcacagaaggcaggaaaactgggaactttaccaaagtagcactcagcctgagaggcctgtataatcatgcttttcaaactaaattcacttaaaaattaaaaagcagaattgaatattttaagcagcctcagtacctttggccaatgctgttttcatggtggattatgaacattatataatctttgggaaaagtgaaagtagtacaatttttagaataatgacaactgcctcactgcatctctccactcacacagcaaccgtgtagccccctaagctgcagtaccatgactaaccatgatgtcaatttcatatgctgatcctcacaacagcagtgcacaaacatgccccaaatattttaacagaatttagctcttccttaagctgtcttttcatagtaaaaacaaaacaaaaacacccaatgttaaaaccacataataaacttacaaacttgaaaaattagacacttcagatagataggcaataaaacttcatattatgaaagcaatatattccaagtttcaaagatttgacaagttctgtagagtatctttcatcagtacatgaaaacttccaaactgcatgatcttctgccaggcaggactgggtgctattcgctggtttgaggtcgaatccatttcaaggcatgtcgtggtgggacattaatggtgggatggtagaatgtgcagtccggtcttgtacattgagtgttaaacctacaatgttttggatgatagaagggacattccatcttcttacaagcagggaagtaacggcagagctgactactggaaggtggtgctggtggtgcaactggttttggagacagtactggaattcttctactcacatgagtgaagggacaatctggtttagtacactttgcatcatatttacaatttgggtgaacaaacaaacatttttcagcaaatttacaattggggaaggctttgcagggtgagatggggtgatggtaggcacactcatccccatttttacaagcaggccagtacttgcagcgctccaaaagtttttctggtttctgtgccacactcagttcactcatctcagcgttagaaaagctaccatttgggtcctcaagctgcctgctcagcaagtgcaactgctgtgggtggaggagacctctgagtcccttgtttgaggctgcagtttggtttacgggtttcattccttcaaagcacatgtcctcctcttgatctgacatgtatcctggggggctggggacaccatccagcgtcactataaacttgggacttgcaggtttatctggttgtacaagatctcgtgtctgcataaggtgtcctgaaagtacccgaagggaatctgcagtcttcatccccgactcttggtttggtgccactactacttcctcagacagctttggcttcttcagaataaatgatcttgtgtctgcatggaccatggattccatgtcatagtaatcttgactcatctgcagagtttctgccattactgggtcgatttgcagtcgggataataattgcctctgttgagttccttgatttttttctacagaatctccttttgtttcctcttctttaatggggggacttattctgggggtcctactttgtccctggaccacttctgctagcaattcttcttgagaagttcgagttctgggagcaactggaagtgtctgtttctgtggaactgtagagtagttagttgtttttgttacggattcttgagcttcagatatagccttcaaaatcagattcttgttagcttgtttagaaggtggaagagaaggtctcctttcaggctttgcaggcacagacacactgctggagatgcttcctgttcgagacccgtaatcatcatcttcttcctcctcttctccatcatgattgaatttttttactttaacaactgaacttaccacaggcaactttctcttccgaaagttttcatcctccatactcattttctccgagttgtttctaaagaacggactatacgtttcttctaagctgttaagcacctctggttcacacaaacgtcctgtttcatatacccaactactctgcatatcaagctgcttggcagcatgaatactattctgctgctgttgaaattgcaacctgtttaaatgaacaccactatctgcatttctacttgcaggtggtcgataaatttcaatagaagggcgagaagaaccatatgtaagtgtcactgtaggttttttctgagataagggattctcctgcacaaagttgaggtcttcgtcaatgagatcatctggttctggcttaatatcaatcacatcttcagagggtgctggctccctcaaaggtttcactgttgacattagtcgggttgcagctccatcatcgtaagtctgtctgacatttgtggtttttgactcctgcgaacttgtagaaactctggaatctcttttttcaggtctcgcgctaggaatggcaagtggtggcactgcagcttcatgcctcctctcatctccccgactgaaattgctcttgtttgaaggcacgttactatcaaagatgttggtatcagaagacttcagactagagggttcagttgtaacagagcgaagtttatctaatacaccatgaagccatacggtgaatcgaattgtgttgttccctagaaacagggacagatcctctgtcatttggtcctgacttttcttgttggccaccatcaccataatgtaatcaggaagttcttcatcaacataagctcctaattcttgtaatttccccttaatggcactctcccgcagcggatccaaagcggcgccgtgcgccgcggtggtggctccagccgggcctgcgcctgtccttccatttcccggcggctacttcagccgcagccacgctccg

SEQ ID NO: 17464 - RNA, 14054 nt, Homo sapiens
  source 1..14054: mol_type = other RNA
tcaggccaggcacagtggctcatacctggaatcccagcactttgggaggccgaggcaggcagatcacctgaggtcaaggtatttgagaccagcctggccaacatggtgaaaccccatctctactaaaaatacagaaattagctgggtgtggtggtgcacacctgtaatgctagctactcgggaggctgaggtaggagaatcgcttgaacctgggaggcagaggttgcaataagcctagatcatgccactgcactcaagcctgggagacagagcgagactacatcttaaaaaaaaaaaaaaaagtattatgagagaggataatgtattgtaatgtattgtagaggctaaataaaattatgctcatgtcagaaaaaaagagtatttctcaaaataaaattcactgaaactggatgtttattttgactgagatatagtatatcctcaaattgccatagaaagtttacaagaatattagaggtaaattataaatatcagggcctttttaaaaaaaaaagattctgcttataacttggtatttgtttataataaaaattatagtagccaataatgaacacttactctggcttggttatttacttaggtcaaaagaaggaggagcggttaaactgtgggatcaggaactgaggcggtgccgtgccttcaggcttgagacaggacaagccacagattgtgttcgttctgtgtgcagaggcaaagtaagatgttccatgagctgatacagtgcagcagaaaacagaaagtggttattactgtgattccctcaccctttgcagcctaatgaacaatacttaataatgcataacgatggatttgcttgccaacattactctgtctttgctgctttctttgccaaagttagcaccagtgtggtgcataagctaggaagctattctgtctaaatactgtatgtaaacctccaatattttctagaatctgccaatttaacaactctagtagacataattgaaagcccttggcagttgactcatattaggacagctgtctccattttttaaaaaaacacacattccctagataaaacgtgcagtaaacaaacaatgaaatactactcagccataaaaaataatgaaattctgtcattcttggtggcaacatggatgagactggaggacatgatgtgaagtgaaataagccaggcacagaaagataaatacatgttctcactcctgtgcagaaactaaaaaagttgatcccacagaggtggagagtagaatagtggttactggaggcggacaagggggagggggagggggatagggaaggactggttaaaggatacaagtttacacagccagataggaatagtatgttttagtattctgtagtactgtaggatgactatagttaagaatcacgtatttatgtattttcaggtatttacaagagaggattttgaaagtttccatcacaaagaaatgataaatgtctgaggtgatggttatgcgtattaccctatgccctatagatatgtataattatgtgtcaatttcaaaataaaaattcaaaactacaactcctatgaaaatttttgagcgtgtttgtacttattaagtgtatttataaatcatacggatattatcttcagcctgcatattaaattgtagttaagcttttactttttaactaaaaaataaattctattattttttcctatatcccactgcactgaccccagtttggaaatcctaagattatcaaataaaaactttgattattgaagaatccaggtgtactgccacagaaaagttctattctgtagcatggactctaatatgtaatctagcccattgtgcttacagatagatgtgtgcctgtagtcatagaaaaatttgcatgagctaatgactgccttgctactagattagctcaaagcaaaaagttctctgaaagcaggtcaatagggtcatttttatattatgaagaagaaaagcagctgttgtattacattcactgtattggtcctgcttgtgtttcagggcaagatccttgttgggacaaggaatgctgaaataatcgaagttggagagaaaaatgcagcttgtaatattttagttaacggtcatgtggatgggccaatctggggactagcaacacatccttccagggattttttcctttctgctgcagaagatgggacagtgagactttgggatattgctgataaagtaagtacagataatttttttaaaagaggttacaacttctaaaaagaaaagttggaagttctaaattgctagtacttaaagaactgccagaattctgttgagcattttgaggggaaactggtataatttagaagtacttcacttaatgtttcctatgactctttttttttttttttttaaatgcagaagatgttaaacaaagtgaatttgggacatgctgctcgtactgtgtgttacagccctgaaggggacatggtggctattggaatgaaaaatggagaatttatcattttactagtgagttctctaaaaatatggggaaagaagagagacaggagatgtgcaatccatgatatcaggttagtgaacaaatggaatagagtttctagtatatacttgatttaacttccatttgtaaaattttccatagccttgccttcaaaaagaggtccccagggcctgtagcatttcccgtattataaattgtatgctaaaatatggctgtttgtatactacttaattcttcttgctaaattataaacccactgggcaccaactataatagcaagtactagtaggtaatgtttgatgaattcatgttaacacttagccatgtccattaagttcatcccaccaagaggtatctcccactgtaatacaagagagctatctgcccttcaaaagttgtcaccctggaaaactaaagttgtgatttcaaacatatcttctcttagtaacctcagtttgggaatatgtagttcattaatttaatcaatacctattgattaaatgttccagaatccaaattaatttaaatgtttcttaaacctttgtttttcagtgcttaagcatttttcaacagtggctaccatttacggagtacttccgtgtgatcagtagataagattattgaatctaggtctgtcaaaagcttgtacacttttcatcagtaaaatccttttacaaatgaaaccttcctcagaacttcaatatataaaatagtaacagtggcttcccttagcttttacatgtctctatcgtacctcagtaagactcatgggccatttcaagagactgaattgtcccatatgactccaaagattgctaggcaaatagcatttcactttgtcttttaaataagttcttcaggccgggcgcggtggctcatgcctgtaatcccagcactttgggaggccgaggcaggcagatcacctgaagtcaggagtactcgaccagcctggccaacatagtgaaaccccatctcaactaaaaatacaaaaatcagccgggcgtggtggcaggcgcctgtaatcccagctactcagggggctgaaacaggagaatcgcttgaacccgggaggcggaggttgcgccatcgcactccagcctgggagacaagagcgagacttcgtctcaaaaaaaaaaaattcttcttccaagattcaagttgtgtcatttcaccttaataactggaggttagttaagctgggctgtgttctttgcttaatattaagacaacgttttttccagatggaagaaaactatcttaatgaattgttagcttattaattatgtaatgctaatggcttttaaaagctgagatgttctgactgggtgttgtggctcacacctgtaatcccagtaccttgggaggccaagggggaaggattgcttgaggccaggagtttgggaccatagtgagaccccgcctctatttaaaaaattaaattttgttttgttttgttttgagttggagttttgctcttgttgcccatgctgaagtgcaatggtgcaatctcagctcaccacaacctgtgcctcctgggttcaagcgattctcctgcttcagcctcccgagtagatgggattacaggcgtgcaccaccatgcctggctaattttgtatttttagtagagacagggtttctctatgttggtcaggctggtctcaaactctcgacctcaggtgatctgcccgcctccgcttcccaaagttctgggattataggtgtgagccactgggcctggcctaagaaagtttttttaagccattagacgtttttaaaggaattgggagatgacaattggggaaatatttaaaatttaagtaaaatataaagcttccttatttcatgtaacccagacaatctcagtatacatgatcagttgtgtctgacaggtaaatctatttgaggccttatcacacgttacttttaagaactagaaaggaaaagtcactgatcttaagtatttataatacttcatgtggtctaatactttttacgttttgttttgattcagatttagtccggattcccggtatctggcagtaggttctagtgagaactcagtggatttttatgacctaacgctgggccccactcttaacagaatcagctactgcaaagacattccaagctttgtcattcaaatggacttctctgcagatagcagttatctccaggtacagtaccaatactgtatacccaggtggcaagttcttctgcttttacatttcgtgttagtgaatgcatttaaagttcctgagctccagagctccagcttctcaactcctccctttgtaccttctgacctacagctcccctttcctcccccacttatcagagcttttctcctattaagtttttgtagtgatcttttgcatacttaataatgttagacatgtaaatcaagtagcaatatgctagtattctgtaaaccccctgtggattttgtctctcacctaatggaattcttgtcccattttaatctgatgaaaaaggtctctagtggctgctataaacggcatgtctatgaagtgccttcaggaaaacatcttatggatcatgccgctattgacagaattacttgggctacatggactaggtaaatacttatatattcacaaggcaagaactgactttgaaggccagttagaaaatcctatttctgaactgttagagccattccaataaggaatagtaattgagtttcaagtttttgttaccatattttgaaatggtatgttcatgttgggacccctttttattgaatatatttccatgttttatcagtttccatgatttatcaagttttttttttaaggaaatcaaagttttaactttaaagataccctgatatttttcttaatgctaaatttaatgactggcaaaaaggtattgggtgctgttaagcaactgttattaattctctatctaaaggaatgctatcttgaatctattagaagtcaaagcttccaaatttgttcaaatttcctggctgtatgacaggtaaccatgactatccatttttttggccaatgaaaaatgccatcaaattcctgtatcagccaggcatatagtggctcatgcctgtaatctctgatgtagcaggccgaggtgggaggatcacttgagcctagaagttttgataccagcctgggcaacatagcaagaccccatctctgaaatttttttaattcctatgtcataagtcatttttatttttgtagagatagggatctcacaatattgcccaggctggtctcaaactcttggcctcaagcagtcctcctgcctcagcctcccaaaatgttgggattactggtatgtgctgctggacccagccaagtagcacttttaatttgaaaaatagttctatcagttttcagtcaggcgcggtggctcagcctgtaatcccagcactttgggaggccgagcgggggtgatcacctgaggtcgggagttcgagactagcctgaccaacatggagaaaccctgtctctactaaaaatacaaaataagccgggcatgttagcgcatgcctgtgatcccagctactcgggaggctgaggcaggagaattgcttgaacccaggaggcagaggttgcggtgagccgagatcatgccattgcactccagcctgggtaacaagagcgaaaactccgtctcaaaaaaaaaaaaagaaaaaatagttctatcagttttcataaagtactactttaatcttaaaaagattaatctagaaacccttcaaattataaaatgtcatttttaaaaggcaggagttgatatcctgatgaaattcaggtctccaaacaacttaccataatttacttcctgtattttaagtaacatgatagggtacttagagattaattgccaagaaactttttgaatatagtcaacctgcccgcacttgccatgatgagttttcttttgttccttccctctagtattctaggagatgaggttttgggaatctggtccagacatgctgagaaagctgatgtcaactgtgcctgtgtatctcattcaggaatcagtcttgttacaggagatgactttggcatggttaagttatttgacttcccatgtccagaaaaatttgtaagtttgtgttttgtttactattatcagtttactcctaattttgatgtcttatcatcagcacttttccccatatatttaaaatgttttgtcctaatttctaaatttttccccaaactttctaaatctatttactttgaaataaaagctattagaaacaaatcctctccctcgagtaataccatctttggaaccatcctacaaaagctgtaattagcttttcaccaaacctataatcagttatcaaatttcaaatgcttttccttagagaaaaatggtcagagtacctggagacatctgactgcccacacagcctggttttgcagatccactactcatgctgaaaagcattctaatcactggctgcggtgctaactccctactctctccacagctcttgtcatagagattatagttcctaataagagcctttgacttctgtgtgcaccaaatgccctgagcttgtctgtcattgttttttaggcaaaacacaaaaggttcttgggtcattcgccccatgtgacaaatattcgatttaccagtggtgatcgacatgttgttagtgctggaggtgatgactgcaggttagtaactttctcagcccatgaagagcagactatgttactagttaagagacttaatacaacaactcctacagctttggtttatgaaatcagctagtcaacattagtagaaggtagtataaccagatggctcttcagaatctcatatttatgcaaatacagaataaaaggagttaaagaggaaaaatattacacatgtaacctgaaagcacaactgaaaaatattaaactgttatgaaaatctaaaaacataattaactccctgcaattttcttctctgattgcagcttatttgtctggaaatgtgtacatacacctcactgagagatgctgagatgactacagaaattaactttgagaccagaattacagagaagaaaaaccaaaacccaaccctgcatggtcaagtggtgctaacccaagactgtaacagggagaaatgcccagaatcatcaaaatagtgaaagactgatctgttcaaaatatttgctatatgcactgggtataatccgtaatccatacactgccagataatgccatttcaaggaaggatcgaatacttgatggtaaaggccaagtccccctgtattgggaagtgtgtgatttcggcagacctgctgggaaaatttagggtagagcactctttacagaagaactcaaaaacccaatttggataattttcattatctttttagcaaaatggtttcttaatgtttatattttattttcaaggttcattgtttaatgaaatattttattcttgcatttccataaggaaagggaaagtcatgatcatcctaaaggatcacagtttttaaaaggcaaacattttccctaaggaaacagacacaagctttcctagagaatatgatgttttttaggcattaataaggtccttttttataaaggacacttttctcctagtagttttgaattcaggaacagatccaaagttagcagtatatggctgctacatttccattttcattttcgagccatcagtttatgttcagatgccatctctgtaatcgcacatttaaaacataactgtagcctcactaatggaaaagtagtatgatgaacaatcattcccaatggtgtacaatgtaagggttttagggagcaacagtatttaactggaagaaagaattgcatatttaatgtagtctaatatatacacatttgtttaacatgtaaacaaaagtgttaaattcacatatacaacattatacaatttaatcactcttggaataaaatttttatagccttttttctattgggaaaatttgtttagatgtgtgccactccataggtttatttccaaaatgaatgagcccaactccatttgtaaaaacttgtcagttagaattcctttttttagtggattagggctgaattcttagatccttatttcttttcactttaaatgctgccaaagatcactactcatcattcaggaattcgctgtctagcctatctgtagtttcctgaagattgaaaattatgtagactgctatttaaaaatatatttttctaagtgtgaggtttaagatgctgtattgaccctatgagtttttaatgtgttaattatctttatagcataatagatcgctttaggttcctggaatcccatttggtctgacaggatatatgaagattcttaatacctattttctgtgtctaatacttggttaatactaaaaatagaaatgactaaattacatcacagaaagcataaccagtgattgaacctggtagttttaaagctctaaatagctgtggctgaaggactgattatggggctaagaagcttgaaacgtaagttggtacttgttcatcagtggattctcctaaattaagccaaattttgaaatacatgactattaagtttctactcatgtatttacagtcagtcaataaattaaaggaggaaaaaaatccctgaacaacctgcccataaaaagaaaaatactctacatttgagcctgctgcagttttaaattttccctctgggtcaagtttgccagcttttggctacagagaaattatatttccattacagtgcaggtagaaactctgtaaccttaagcatgtaaactacatagaataaaactgtttccactgcatttctgtccttcaaagtggccaacctgattaagtcagccttaatcactgctgctgtcagtttcacgactaaaggtcatattgactaagtagtcatcagctgaccacctcgctgtatcagccagcaacgaggggaaggtgaagaaacatgataggccatatagaatctgccctatgtttacttttttaacccagataattatttttgtgtgcagtatctaagctcctgattgtgtaacctgggacttctggcaccttttgttccattcattttatgtataaaatgcatgccaaagcacactgtgccctctggtacccttgcttccaatcgccaaccatgctcatttccttcctttttttgtggtccctttttgtggtgatcattttaaaccacgtcatccaacaaatgttttatggtcaaccttagcttgttcataagccatagcaactgaaagattaaactcttaaatatgtgtctgggcagtggctattaaatagcaaaaaacaatcagattttagtattttattatttccttgtaaaatggctgaactaaattaaacccttgtttcccatttgttctataatttatagtgaaactgagaacaaaactatctttataaatgatagctaaaagtatttccagatatttaaacaatttaaaataaatttcttctgcagagatgcaaagcatctcaacactggaatgaacaaatgccttaaattcaatggagtaaacctttagaatgaagaggaactgtcatttcacccaagccgaagacaacagccttatgcacttgtgtgctctgtctttgctgcttctcgtgtttcaagcctttcctgtgggatcagcacagcaaagtgcaacttaccaaatggtttaatgactggttaattctttcttctcccaatggaaaagcaatggcaacacaacagtagactgctggcttgacaatcttaaacgtgagcctttgcacatgtaggtttatcatcatttgagtatacgactaagcaagtcaatgaactttttttttttttttagcagtttaatttggtcctgagaatgttgcagtctttattaccccttttgcattaatccacttttctaaccaccttttaagctttaatttttaacactatacaccaagtctttgaaatcagtgatctgttatttaactctaaagcatttgacacttcttgccttaacagttttaaaaaccacacacaaaaaaactctgtaagtaatacagtaggccaaaagtttcatcctatctatcttgcagtttacctatctgatctgatctctgtaattatagttctgtcatttaaaatatactatttaaatctaatttttacatttcaaaaattatcttcagtagtaactaagtatattttctgtggattctgagaatgttatttttcagaatgtgagaatatatatgtacatttataatcttgtgactttaaagtctgttttcagatacagtatgtaaatacttgtaaaaaaatttgtataattttgtgataatgtagtttcccaaaaaaattatttagaaggcattatgttattagtaaatgagagcactgtatagaactgttcctattttctgcacttgccattccagctgcctccactgtccatacccacctcattcatcctgtcacagaaggcaggaaaactgggaactttaccaaagtagcactcagcctgagaggcctgtataatcatgcttttcaaactaaattcacttaaaaattaaaaagcagaattgaatattttaagcagcctcagtacctttggccaatgctgttttcatggtggattatgaacattatataatctttgggaaaagtgaaagtagtacaatttttagaataatgacaactgcctcactgcatctctccactcacacagcaaccgtgtagccccctaagctgcagtaccatgactaaccatgatgtcaatttcatatgctgatcctcacaacagcagtgcacaaacatgccccaaatattttaacagaatttagctcttccttaagctgtcttttcatagtaaaaacaaaacaaaaacacccaatgttaaaaccacataataaacttacaaacttgaaaaattagacacttcagatagataggcaataaaacttcatattatgaaagcaatatattccaagtttcaaagatttgacaagttctgtagagtatctttcatcagtacatgaaaacttccaaactgcatgatcttctgccaggcaggactgggtgctattcgctggtttgaggtcgaatccatttcaaggcatgtcgtggtgggacattaatggtgggatggtagaatgtgcagtccggtcttgtacattgagtgttaaacctacaatgttttggatgatagaagggacattccatcttcttacaagcagggaagtaacggcagagctgactactggaaggtggtgctggtggtgcaactggttttggagacagtactggaattcttctactcacatgagtgaagggacaatctggtttagtacactttgcatcatatttacaatttgggtgaacaaacaaacatttttcagcaaatttacaattggggaaggctttgcagggtgagatggggtgatggtaggcacactcatccccatttttacaagcaggccagtacttgcagcgctccaaaagtttttctggtttctgtgccacactcagttcactcatctcagcgttagaaaagctaccatttgggtcctcaagctgcctgctcagcaagtgcaactgctgtgggtggaggagacctctgagtcccttgtttgaggctgcagtttggtttacgggtttcattccttcaaagcacatgtcctcctcttgatctgacatgtatcctggggggctggggacaccatccagcgtcactataaacttgggacttgcaggtttatctggttgtacaagatctcgtgtctgcataaggtgtcctgaaagtacccgaagggaatctgcagtcttcatccccgactcttggtttggtgccactactacttcctcagacagctttggcttcttcagaataaatgatcttgtgtctgcatggaccatggattccatgtcatagtaatcttgactcatctgcagagtttctgccattactgggtcgatttgcagtcgggataataattgcctctgttgagttccttgatttttttctacagaatctccttttgtttcctcttctttaatggggggacttattctgggggtcctactttgtccctggaccacttctgctagcaattcttcttgagaagttcgagttctgggagcaactggaagtgtctgtttctgtggaactgtagagtagttagttgtttttgttacggattcttgagcttcagatatagccttcaaaatcagattcttgttagcttgtttagaaggtggaagagaaggtctcctttcaggctttgcaggcacagacacactgctggagatgcttcctgttcgagacccgtaatcatcatcttcttcctcctcttctccatcatgattgaatttttttactttaacaactgaacttaccacaggcaactttctcttccgaaagttttcatcctccatactcattttctccgagttgtttctaaagaacggactatacgtttcttctaagctgttaagcacctctggttcacacaaacgtcctgtttcatatacccaactactctgcatatcaagctgcttggcagcatgaatactattctgctgctgttgaaattgcaacctgtttaaatgaacaccactatctgcatttctacttgcaggtggtcgataaatttcaatagaagggcgagaagaaccatatgtaagtgtcactgtaggttttttctgagataagggattctcctgcacaaagttgaggtcttcgtcaatgagatcatctggttctggcttaatatcaatcacatcttcagagggtgctggctccctcaaaggtttcactgttgacattagtcgggttgcagctccatcatcgtaagtctgtctgacatttgtggtttttgactcctgcgaacttgtagaaactctggaatctcttttttcaggtctcgcgctaggaatggcaagtggtggcactgcagcttcatgcctcctctcatctccccgactgaaattgctcttgtttgaaggcacgttactatcaaagatgttggtatcagaagacttcagactagagggttcagttgtaacagagcgaagtttatctaatacaccatgaagccatacggtgaatcgaattgtgttgttccctagaaacagggacagatcctctgtcatttggtcctgacttttcttgttggccaccatcaccataatgtaatcaggaagttcttcatctatttaaaaggaaaggtagatcaaaactttgtttcctcaaaactttcttcttaaagttgatgtgcttgaaaatatagatgtagctctaagctttagagtcgcagagctctactggaattacattggacaagatggcttagctttaatttttttctcttcattccacaggtatttcaaatacaacataagctcctaattcttgtaatttccccttaatggcactccggatcttgcggctgatctcggtgccgatctccatggctctgcggcgtgcgggaactcagcactgcgcggcgcttggcttacccggaggctgccgcggactcctaccccgcagccgggacaccaccgcctcc

SEQ ID NO: 17465 - RNA, 13683 nt, Homo sapiens
  source 1..13683: mol_type = other RNA
tcaggccaggcacagtggctcatacctggaatcccagcactttgggaggccgaggcaggcagatcacctgaggtcaaggtatttgagaccagcctggccaacatggtgaaaccccatctctactaaaaatacagaaattagctgggtgtggtggtgcacacctgtaatgctagctactcgggaggctgaggtaggagaatcgcttgaacctgggaggcagaggttgcaataagcctagatcatgccactgcactcaagcctgggagacagagcgagactacatcttaaaaaaaaaaaaaaaagtattatgagagaggataatgtattgtaatgtattgtagaggctaaataaaattatgctcatgtcagaaaaaaagagtatttctcaaaataaaattcactgaaactggatgtttattttgactgagatatagtatatcctcaaattgccatagaaagtttacaagaatattagaggtaaattataaatatcagggcctttttaaaaaaaaaagattctgcttataacttggtatttgtttataataaaaattatagtagccaataatgaacacttactctggcttggttatttacttaggtcaaaagaaggaggagcggttaaactgtgggatcaggaactgaggcggtgccgtgccttcaggcttgagacaggacaagccacagattgtgttcgttctgtgtgcagaggcaaagtaagatgttccatgagctgatacagtgcagcagaaaacagaaagtggttattactgtgattccctcaccctttgcagcctaatgaacaatacttaataatgcataacgatggatttgcttgccaacattactctgtctttgctgctttctttgccaaagttagcaccagtgtggtgcataagctaggaagctattctgtctaaatactgtatgtaaacctccaatattttctagaatctgccaatttaacaactctagtagacataattgaaagcccttggcagttgactcatattaggacagctgtctccattttttaaaaaaacacacattccctagataaaacgtgcagtaaacaaacaatgaaatactactcagccataaaaaataatgaaattctgtcattcttggtggcaacatggatgagactggaggacatgatgtgaagtgaaataagccaggcacagaaagataaatacatgttctcactcctgtgcagaaactaaaaaagttgatcccacagaggtggagagtagaatagtggttactggaggcggacaagggggagggggagggggatagggaaggactggttaaaggatacaagtttacacagccagataggaatagtatgttttagtattctgtagtactgtaggatgactatagttaagaatcacgtatttatgtattttcaggtatttacaagagaggattttgaaagtttccatcacaaagaaatgataaatgtctgaggtgatggttatgcgtattaccctatgccctatagatatgtataattatgtgtcaatttcaaaataaaaattcaaaactacaactcctatgaaaatttttgagcgtgtttgtacttattaagtgtatttataaatcatacggatattatcttcagcctgcatattaaattgtagttaagcttttactttttaactaaaaaataaattctattattttttcctatatcccactgcactgaccccagtttggaaatcctaagattatcaaataaaaactttgattattgaagaatccaggtgtactgccacagaaaagttctattctgtagcatggactctaatatgtaatctagcccattgtgcttacagatagatgtgtgcctgtagtcatagaaaaatttgcatgagctaatgactgccttgctactagattagctcaaagcaaaaagttctctgaaagcaggtcaatagggtcatttttatattatgaagaagaaaagcagctgttgtattacattcactgtattggtcctgcttgtgtttcagggcaagatccttgttgggacaaggaatgctgaaataatcgaagttggagagaaaaatgcagcttgtaatattttagttaacggtcatgtggatgggccaatctggggactagcaacacatccttccagggattttttcctttctgctgcagaagatgggacagtgagactttgggatattgctgataaagtaagtacagataatttttttaaaagaggttacaacttctaaaaagaaaagttggaagttctaaattgctagtacttaaagaactgccagaattctgttgagcattttgaggggaaactggtataatttagaagtacttcacttaatgtttcctatgactctttttttttttttttttaaatgcagaagatgttaaacaaagtgaatttgggacatgctgctcgtactgtgtgttacagccctgaaggggacatggtggctattggaatgaaaaatggagaatttatcattttactagtgagttctctaaaaatatggggaaagaagagagacaggagatgtgcaatccatgatatcaggttagtgaacaaatggaatagagtttctagtatatacttgatttaacttccatttgtaaaattttccatagccttgccttcaaaaagaggtccccagggcctgtagcatttcccgtattataaattgtatgctaaaatatggctgtttgtatactacttaattcttcttgctaaattataaacccactgggcaccaactataatagcaagtactagtaggtaatgtttgatgaattcatgttaacacttagccatgtccattaagttcatcccaccaagaggtatctcccactgtaatacaagagagctatctgcccttcaaaagttgtcaccctggaaaactaaagttgtgatttcaaacatatcttctcttagtaacctcagtttgggaatatgtagttcattaatttaatcaatacctattgattaaatgttccagaatccaaattaatttaaatgtttcttaaacctttgtttttcagtgcttaagcatttttcaacagtggctaccatttacggagtacttccgtgtgatcagtagataagattattgaatctaggtctgtcaaaagcttgtacacttttcatcagtaaaatccttttacaaatgaaaccttcctcagaacttcaatatataaaatagtaacagtggcttcccttagcttttacatgtctctatcgtacctcagtaagactcatgggccatttcaagagactgaattgtcccatatgactccaaagattgctaggcaaatagcatttcactttgtcttttaaataagttcttcaggccgggcgcggtggctcatgcctgtaatcccagcactttgggaggccgaggcaggcagatcacctgaagtcaggagtactcgaccagcctggccaacatagtgaaaccccatctcaactaaaaatacaaaaatcagccgggcgtggtggcaggcgcctgtaatcccagctactcagggggctgaaacaggagaatcgcttgaacccgggaggcggaggttgcgccatcgcactccagcctgggagacaagagcgagacttcgtctcaaaaaaaaaaaattcttcttccaagattcaagttgtgtcatttcaccttaataactggaggttagttaagctgggctgtgttctttgcttaatattaagacaacgttttttccagatggaagaaaactatcttaatgaattgttagcttattaattatgtaatgctaatggcttttaaaagctgagatgttctgactgggtgttgtggctcacacctgtaatcccagtaccttgggaggccaagggggaaggattgcttgaggccaggagtttgggaccatagtgagaccccgcctctatttaaaaaattaaattttgttttgttttgttttgagttggagttttgctcttgttgcccatgctgaagtgcaatggtgcaatctcagctcaccacaacctgtgcctcctgggttcaagcgattctcctgcttcagcctcccgagtagatgggattacaggcgtgcaccaccatgcctggctaattttgtatttttagtagagacagggtttctctatgttggtcaggctggtctcaaactctcgacctcaggtgatctgcccgcctccgcttcccaaagttctgggattataggtgtgagccactgggcctggcctaagaaagtttttttaagccattagacgtttttaaaggaattgggagatgacaattggggaaatatttaaaatttaagtaaaatataaagcttccttatttcatgtaacccagacaatctcagtatacatgatcagttgtgtctgacaggtaaatctatttgaggccttatcacacgttacttttaagaactagaaaggaaaagtcactgatcttaagtatttataatacttcatgtggtctaatactttttacgttttgttttgattcagatttagtccggattcccggtatctggcagtaggttctagtgagaactcagtggatttttatgacctaacgctgggccccactcttaacagaatcagctactgcaaagacattccaagctttgtcattcaaatggacttctctgcagatagcagttatctccaggtacagtaccaatactgtatacccaggtggcaagttcttctgcttttacatttcgtgttagtgaatgcatttaaagttcctgagctccagagctccagcttctcaactcctccctttgtaccttctgacctacagctcccctttcctcccccacttatcagagcttttctcctattaagtttttgtagtgatcttttgcatacttaataatgttagacatgtaaatcaagtagcaatatgctagtattctgtaaaccccctgtggattttgtctctcacctaatggaattcttgtcccattttaatctgatgaaaaaggtctctagtggctgctataaacggcatgtctatgaagtgccttcaggaaaacatcttatggatcatgccgctattgacagaattacttgggctacatggactaggtaaatacttatatattcacaaggcaagaactgactttgaaggccagttagaaaatcctatttctgaactgttagagccattccaataaggaatagtaattgagtttcaagtttttgttaccatattttgaaatggtatgttcatgttgggacccctttttattgaatatatttccatgttttatcagtttccatgatttatcaagttttttttttaaggaaatcaaagttttaactttaaagataccctgatatttttcttaatgctaaatttaatgactggcaaaaaggtattgggtgctgttaagcaactgttattaattctctatctaaaggaatgctatcttgaatctattagaagtcaaagcttccaaatttgttcaaatttcctggctgtatgacaggtaaccatgactatccatttttttggccaatgaaaaatgccatcaaattcctgtatcagccaggcatatagtggctcatgcctgtaatctctgatgtagcaggccgaggtgggaggatcacttgagcctagaagttttgataccagcctgggcaacatagcaagaccccatctctgaaatttttttaattcctatgtcataagtcatttttatttttgtagagatagggatctcacaatattgcccaggctggtctcaaactcttggcctcaagcagtcctcctgcctcagcctcccaaaatgttgggattactggtatgtgctgctggacccagccaagtagcacttttaatttgaaaaatagttctatcagttttcagtcaggcgcggtggctcagcctgtaatcccagcactttgggaggccgagcgggggtgatcacctgaggtcgggagttcgagactagcctgaccaacatggagaaaccctgtctctactaaaaatacaaaataagccgggcatgttagcgcatgcctgtgatcccagctactcgggaggctgaggcaggagaattgcttgaacccaggaggcagaggttgcggtgagccgagatcatgccattgcactccagcctgggtaacaagagcgaaaactccgtctcaaaaaaaaaaaaagaaaaaatagttctatcagttttcataaagtactactttaatcttaaaaagattaatctagaaacccttcaaattataaaatgtcatttttaaaaggcaggagttgatatcctgatgaaattcaggtctccaaacaacttaccataatttacttcctgtattttaagtaacatgatagggtacttagagattaattgccaagaaactttttgaatatagtcaacctgcccgcacttgccatgatgagttttcttttgttccttccctctagtattctaggagatgaggttttgggaatctggtccagacatgctgagaaagctgatgtcaactgtgcctgtgtatctcattcaggaatcagtcttgttacaggagatgactttggcatggttaagttatttgacttcccatgtccagaaaaatttgtaagtttgtgttttgtttactattatcagtttactcctaattttgatgtcttatcatcagcacttttccccatatatttaaaatgttttgtcctaatttctaaatttttccccaaactttctaaatctatttactttgaaataaaagctattagaaacaaatcctctccctcgagtaataccatctttggaaccatcctacaaaagctgtaattagcttttcaccaaacctataatcagttatcaaatttcaaatgcttttccttagagaaaaatggtcagagtacctggagacatctgactgcccacacagcctggttttgcagatccactactcatgctgaaaagcattctaatcactggctgcggtgctaactccctactctctccacagctcttgtcatagagattatagttcctaataagagcctttgacttctgtgtgcaccaaatgccctgagcttgtctgtcattgttttttaggcaaaacacaaaaggttcttgggtcattcgccccatgtgacaaatattcgatttaccagtggtgatcgacatgttgttagtgctggaggtgatgactgcaggttagtaactttctcagcccatgaagagcagactatgttactagttaagagacttaatacaacaactcctacagctttggtttatgaaatcagctagtcaacattagtagaaggtagtataaccagatggctcttcagaatctcatatttatgcaaatacagaataaaaggagttaaagaggaaaaatattacacatgtaacctgaaagcacaactgaaaaatattaaactgttatgaaaatctaaaaacataattaactccctgcaattttcttctctgattgcagcttatttgtctggaaatgtgtacatacacctcactgagagatgctgagatgactacagaaattaactttgagaccagaattacagagaagaaaaaccaaaacccaaccctgcatggtcaagtggtgctaacccaagactgtaacagggagaaatgcccagaatcatcaaaatagtgaaagactgatctgttcaaaatatttgctatatgcactgggtataatccgtaatccatacactgccagataatgccatttcaaggaaggatcgaatacttgatggtaaaggccaagtccccctgtattgggaagtgtgtgatttcggcagacctgctgggaaaatttagggtagagcactctttacagaagaactcaaaaacccaatttggataattttcattatctttttagcaaaatggtttcttaatgtttatattttattttcaaggttcattgtttaatgaaatattttattcttgcatttccataaggaaagggaaagtcatgatcatcctaaaggatcacagtttttaaaaggcaaacattttccctaaggaaacagacacaagctttcctagagaatatgatgttttttaggcattaataaggtccttttttataaaggacacttttctcctagtagttttgaattcaggaacagatccaaagttagcagtatatggctgctacatttccattttcattttcgagccatcagtttatgttcagatgccatctctgtaatcgcacatttaaaacataactgtagcctcactaatggaaaagtagtatgatgaacaatcattcccaatggtgtacaatgtaagggttttagggagcaacagtatttaactggaagaaagaattgcatatttaatgtagtctaatatatacacatttgtttaacatgtaaacaaaagtgttaaattcacatatacaacattatacaatttaatcactcttggaataaaatttttatagccttttttctattgggaaaatttgtttagatgtgtgccactccataggtttatttccaaaatgaatgagcccaactccatttgtaaaaacttgtcagttagaattcctttttttagtggattagggctgaattcttagatccttatttcttttcactttaaatgctgccaaagatcactactcatcattcaggaattcgctgtctagcctatctgtagtttcctgaagattgaaaattatgtagactgctatttaaaaatatatttttctaagtgtgaggtttaagatgctgtattgaccctatgagtttttaatgtgttaattatctttatagcataatagatcgctttaggttcctggaatcccatttggtctgacaggatatatgaagattcttaatacctattttctgtgtctaatacttggttaatactaaaaatagaaatgactaaattacatcacagaaagcataaccagtgattgaacctggtagttttaaagctctaaatagctgtggctgaaggactgattatggggctaagaagcttgaaacgtaagttggtacttgttcatcagtggattctcctaaattaagccaaattttgaaatacatgactattaagtttctactcatgtatttacagtcagtcaataaattaaaggaggaaaaaaatccctgaacaacctgcccataaaaagaaaaatactctacatttgagcctgctgcagttttaaattttccctctgggtcaagtttgccagcttttggctacagagaaattatatttccattacagtgcaggtagaaactctgtaaccttaagcatgtaaactacatagaataaaactgtttccactgcatttctgtccttcaaagtggccaacctgattaagtcagccttaatcactgctgctgtcagtttcacgactaaaggtcatattgactaagtagtcatcagctgaccacctcgctgtatcagccagcaacgaggggaaggtgaagaaacatgataggccatatagaatctgccctatgtttacttttttaacccagataattatttttgtgtgcagtatctaagctcctgattgtgtaacctgggacttctggcaccttttgttccattcattttatgtataaaatgcatgccaaagcacactgtgccctctggtacccttgcttccaatcgccaaccatgctcatttccttcctttttttgtggtccctttttgtggtgatcattttaaaccacgtcatccaacaaatgttttatggtcaaccttagcttgttcataagccatagcaactgaaagattaaactcttaaatatgtgtctgggcagtggctattaaatagcaaaaaacaatcagattttagtattttattatttccttgtaaaatggctgaactaaattaaacccttgtttcccatttgttctataatttatagtgaaactgagaacaaaactatctttataaatgatagctaaaagtatttccagatatttaaacaatttaaaataaatttcttctgcagagatgcaaagcatctcaacactggaatgaacaaatgccttaaattcaatggagtaaacctttagaatgaagaggaactgtcatttcacccaagccgaagacaacagccttatgcacttgtgtgctctgtctttgctgcttctcgtgtttcaagcctttcctgtgggatcagcacagcaaagtgcaacttaccaaatggtttaatgactggttaattctttcttctcccaatggaaaagcaatggcaacacaacagtagactgctggcttgacaatcttaaacgtgagcctttgcacatgtaggtttatcatcatttgagtatacgactaagcaagtcaatgaactttttttttttttttagcagtttaatttggtcctgagaatgttgcagtctttattaccccttttgcattaatccacttttctaaccaccttttaagctttaatttttaacactatacaccaagtctttgaaatcagtgatctgttatttaactctaaagcatttgacacttcttgccttaacagttttaaaaaccacacacaaaaaaactctgtaagtaatacagtaggccaaaagtttcatcctatctatcttgcagtttacctatctgatctgatctctgtaattatagttctgtcatttaaaatatactatttaaatctaatttttacatttcaaaaattatcttcagtagtaactaagtatattttctgtggattctgagaatgttatttttcagaatgtgagaatatatatgtacatttataatcttgtgactttaaagtctgttttcagatacagtatgtaaatacttgtaaaaaaatttgtataattttgtgataatgtagtttcccaaaaaaattatttagaaggcattatgttattagtaaatgagagcactgtatagaactgttcctattttctgcacttgccattccagctgcctccactgtccatacccacctcattcatcctgtcacagaaggcaggaaaactgggaactttaccaaagtagcactcagcctgagaggcctgtataatcatgcttttcaaactaaattcacttaaaaattaaaaagcagaattgaatattttaagcagcctcagtacctttggccaatgctgttttcatggtggattatgaacattatataatctttgggaaaagtgaaagtagtacaatttttagaataatgacaactgcctcactgcatctctccactcacacagcaaccgtgtagccccctaagctgcagtaccatgactaaccatgatgtcaatttcatatgctgatcctcacaacagcagtgcacaaacatgccccaaatattttaacagaatttagctcttccttaagctgtcttttcatagtaaaaacaaaacaaaaacacccaatgttaaaaccacataataaacttacaaacttgaaaaattagacacttcagatagataggcaataaaacttcatattatgaaagcaatatattccaagtttcaaagatttgacaagttctgtagagtatctttcatcagtacatgaaaacttccaaactgcatgatcttctgccaggcaggactgggtgctattcgctggtttgaggtcgaatccatttcaaggcatgtcgtggtgggacattaatggtgggatggtagaatgtgcagtccggtcttgtacattgagtgttaaacctacaatgttttggatgatagaagggacattccatcttcttacaagcagggaagtaacggcagagctgactactggaaggtggtgctggtggtgcaactggttttggagacagtactggaattcttctactcacatgagtgaagggacaatctggtttagtacactttgcatcatatttacaatttgggtgaacaaacaaacatttttcagcaaatttacaattggggaaggctttgcagggtgagatggggtgatggtaggcacactcatccccatttttacaagcaggccagtacttgcagcgctccaaaagtttttctggtttctgtgccacactcagttcactcatctcagcgttagaaaagctaccatttgggtcctcaagctgcctgctcagcaagtgcaactgctgtgggtggaggagacctctgagtcccttgtttgaggctgcagtttggtttacgggtttcattccttcaaagcacatgtcctcctcttgatctgacatgtatcctggggggctggggacaccatccagcgtcactataaacttgggacttgcaggtttatctggttgtacaagatctcgtgtctgcataaggtgtcctgaaagtacccgaagggaatctgcagtcttcatccccgactcttggtttggtgccactactacttcctcagacagctttggcttcttcagaataaatgatcttgtgtctgcatggaccatggattccatgtcatagtaatcttgatttttttctacagaatctccttttgtttcctcttctttaatggggggacttattctgggggtcctactttgtccctggaccacttctgctagcaattcttcttgagaagttcgagttctgggagcaactggaagtgtctgtttctgtggaactgtagagtagttagttgtttttgttacggattcttgagcttcagatatagccttcaaaatcagattcttgttagcttgtttagaaggtggaagagaaggtctcctttcaggctttgcaggcacagacacactgctggagatgcttcctgttcgagacccgtaatcatcatcttcttcctcctcttctccatcatgattgaatttttttactttaacaactgaacttaccacaggcaactttctcttccgaaagttttcatcctccatactcattttctccgagttgtttctaaagaacggactatacgtttcttctaagctgttaagcacctctggttcacacaaacgtcctgtttcatatacccaactactctgcatatcaagctgcttggcagcatgaatactattctgctgctgttgaaattgcaacctgtttaaatgaacaccactatctgcatttctacttgcaggtggtcgataaatttcaatagaagggcgagaagaaccatatgtaagtgtcactgtaggttttttctgagataagggattctcctgcacaaagttgaggtcttcgtcaatgagatcatctggttctggcttaatatcaatcacatcttcagagggtgctggctccctcaaaggtttcactgttgacattagtcgggttgcagctccatcatcgtaagtctgtctgacatttgtggtttttgactcctgcgaacttgtagaaactctggaatctcttttttcaggtctcgcgctaggaatggcaagtggtggcactgcagcttcatgcctcctctcatctccccgactgaaattgctcttgtttgaaggcacgttactatcaaagatgttggtatcagaagacttcagactagagggttcagttgtaacagagcgaagtttatctaatacaccatgaagccaacataagctcctaattcttgtaatttccccttaatggcactccggatcttgcggctgatctcggtgccgatctccatggctctgcggcgtgcgggaactcagcactgcgcggcgcttggcttacccggaggctgccgcggactcctaccccgcagccgggacaccaccgcctcc

SEQ ID NO: 17466 - RNA, 13798 nt, Homo sapiens
  source 1..13798: mol_type = other RNA
tcaggccaggcacagtggctcatacctggaatcccagcactttgggaggccgaggcaggcagatcacctgaggtcaaggtatttgagaccagcctggccaacatggtgaaaccccatctctactaaaaatacagaaattagctgggtgtggtggtgcacacctgtaatgctagctactcgggaggctgaggtaggagaatcgcttgaacctgggaggcagaggttgcaataagcctagatcatgccactgcactcaagcctgggagacagagcgagactacatcttaaaaaaaaaaaaaaaagtattatgagagaggataatgtattgtaatgtattgtagaggctaaataaaattatgctcatgtcagaaaaaaagagtatttctcaaaataaaattcactgaaactggatgtttattttgactgagatatagtatatcctcaaattgccatagaaagtttacaagaatattagaggtaaattataaatatcagggcctttttaaaaaaaaaagattctgcttataacttggtatttgtttataataaaaattatagtagccaataatgaacacttactctggcttggttatttacttaggtcaaaagaaggaggagcggttaaactgtgggatcaggaactgaggcggtgccgtgccttcaggcttgagacaggacaagccacagattgtgttcgttctgtgtgcagaggcaaagtaagatgttccatgagctgatacagtgcagcagaaaacagaaagtggttattactgtgattccctcaccctttgcagcctaatgaacaatacttaataatgcataacgatggatttgcttgccaacattactctgtctttgctgctttctttgccaaagttagcaccagtgtggtgcataagctaggaagctattctgtctaaatactgtatgtaaacctccaatattttctagaatctgccaatttaacaactctagtagacataattgaaagcccttggcagttgactcatattaggacagctgtctccattttttaaaaaaacacacattccctagataaaacgtgcagtaaacaaacaatgaaatactactcagccataaaaaataatgaaattctgtcattcttggtggcaacatggatgagactggaggacatgatgtgaagtgaaataagccaggcacagaaagataaatacatgttctcactcctgtgcagaaactaaaaaagttgatcccacagaggtggagagtagaatagtggttactggaggcggacaagggggagggggagggggatagggaaggactggttaaaggatacaagtttacacagccagataggaatagtatgttttagtattctgtagtactgtaggatgactatagttaagaatcacgtatttatgtattttcaggtatttacaagagaggattttgaaagtttccatcacaaagaaatgataaatgtctgaggtgatggttatgcgtattaccctatgccctatagatatgtataattatgtgtcaatttcaaaataaaaattcaaaactacaactcctatgaaaatttttgagcgtgtttgtacttattaagtgtatttataaatcatacggatattatcttcagcctgcatattaaattgtagttaagcttttactttttaactaaaaaataaattctattattttttcctatatcccactgcactgaccccagtttggaaatcctaagattatcaaataaaaactttgattattgaagaatccaggtgtactgccacagaaaagttctattctgtagcatggactctaatatgtaatctagcccattgtgcttacagatagatgtgtgcctgtagtcatagaaaaatttgcatgagctaatgactgccttgctactagattagctcaaagcaaaaagttctctgaaagcaggtcaatagggtcatttttatattatgaagaagaaaagcagctgttgtattacattcactgtattggtcctgcttgtgtttcagggcaagatccttgttgggacaaggaatgctgaaataatcgaagttggagagaaaaatgcagcttgtaatattttagttaacggtcatgtggatgggccaatctggggactagcaacacatccttccagggattttttcctttctgctgcagaagatgggacagtgagactttgggatattgctgataaagtaagtacagataatttttttaaaagaggttacaacttctaaaaagaaaagttggaagttctaaattgctagtacttaaagaactgccagaattctgttgagcattttgaggggaaactggtataatttagaagtacttcacttaatgtttcctatgactctttttttttttttttttaaatgcagaagatgttaaacaaagtgaatttgggacatgctgctcgtactgtgtgttacagccctgaaggggacatggtggctattggaatgaaaaatggagaatttatcattttactagtgagttctctaaaaatatggggaaagaagagagacaggagatgtgcaatccatgatatcaggttagtgaacaaatggaatagagtttctagtatatacttgatttaacttccatttgtaaaattttccatagccttgccttcaaaaagaggtccccagggcctgtagcatttcccgtattataaattgtatgctaaaatatggctgtttgtatactacttaattcttcttgctaaattataaacccactgggcaccaactataatagcaagtactagtaggtaatgtttgatgaattcatgttaacacttagccatgtccattaagttcatcccaccaagaggtatctcccactgtaatacaagagagctatctgcccttcaaaagttgtcaccctggaaaactaaagttgtgatttcaaacatatcttctcttagtaacctcagtttgggaatatgtagttcattaatttaatcaatacctattgattaaatgttccagaatccaaattaatttaaatgtttcttaaacctttgtttttcagtgcttaagcatttttcaacagtggctaccatttacggagtacttccgtgtgatcagtagataagattattgaatctaggtctgtcaaaagcttgtacacttttcatcagtaaaatccttttacaaatgaaaccttcctcagaacttcaatatataaaatagtaacagtggcttcccttagcttttacatgtctctatcgtacctcagtaagactcatgggccatttcaagagactgaattgtcccatatgactccaaagattgctaggcaaatagcatttcactttgtcttttaaataagttcttcaggccgggcgcggtggctcatgcctgtaatcccagcactttgggaggccgaggcaggcagatcacctgaagtcaggagtactcgaccagcctggccaacatagtgaaaccccatctcaactaaaaatacaaaaatcagccgggcgtggtggcaggcgcctgtaatcccagctactcagggggctgaaacaggagaatcgcttgaacccgggaggcggaggttgcgccatcgcactccagcctgggagacaagagcgagacttcgtctcaaaaaaaaaaaattcttcttccaagattcaagttgtgtcatttcaccttaataactggaggttagttaagctgggctgtgttctttgcttaatattaagacaacgttttttccagatggaagaaaactatcttaatgaattgttagcttattaattatgtaatgctaatggcttttaaaagctgagatgttctgactgggtgttgtggctcacacctgtaatcccagtaccttgggaggccaagggggaaggattgcttgaggccaggagtttgggaccatagtgagaccccgcctctatttaaaaaattaaattttgttttgttttgttttgagttggagttttgctcttgttgcccatgctgaagtgcaatggtgcaatctcagctcaccacaacctgtgcctcctgggttcaagcgattctcctgcttcagcctcccgagtagatgggattacaggcgtgcaccaccatgcctggctaattttgtatttttagtagagacagggtttctctatgttggtcaggctggtctcaaactctcgacctcaggtgatctgcccgcctccgcttcccaaagttctgggattataggtgtgagccactgggcctggcctaagaaagtttttttaagccattagacgtttttaaaggaattgggagatgacaattggggaaatatttaaaatttaagtaaaatataaagcttccttatttcatgtaacccagacaatctcagtatacatgatcagttgtgtctgacaggtaaatctatttgaggccttatcacacgttacttttaagaactagaaaggaaaagtcactgatcttaagtatttataatacttcatgtggtctaatactttttacgttttgttttgattcagatttagtccggattcccggtatctggcagtaggttctagtgagaactcagtggatttttatgacctaacgctgggccccactcttaacagaatcagctactgcaaagacattccaagctttgtcattcaaatggacttctctgcagatagcagttatctccaggtacagtaccaatactgtatacccaggtggcaagttcttctgcttttacatttcgtgttagtgaatgcatttaaagttcctgagctccagagctccagcttctcaactcctccctttgtaccttctgacctacagctcccctttcctcccccacttatcagagcttttctcctattaagtttttgtagtgatcttttgcatacttaataatgttagacatgtaaatcaagtagcaatatgctagtattctgtaaaccccctgtggattttgtctctcacctaatggaattcttgtcccattttaatctgatgaaaaaggtctctagtggctgctataaacggcatgtctatgaagtgccttcaggaaaacatcttatggatcatgccgctattgacagaattacttgggctacatggactaggtaaatacttatatattcacaaggcaagaactgactttgaaggccagttagaaaatcctatttctgaactgttagagccattccaataaggaatagtaattgagtttcaagtttttgttaccatattttgaaatggtatgttcatgttgggacccctttttattgaatatatttccatgttttatcagtttccatgatttatcaagttttttttttaaggaaatcaaagttttaactttaaagataccctgatatttttcttaatgctaaatttaatgactggcaaaaaggtattgggtgctgttaagcaactgttattaattctctatctaaaggaatgctatcttgaatctattagaagtcaaagcttccaaatttgttcaaatttcctggctgtatgacaggtaaccatgactatccatttttttggccaatgaaaaatgccatcaaattcctgtatcagccaggcatatagtggctcatgcctgtaatctctgatgtagcaggccgaggtgggaggatcacttgagcctagaagttttgataccagcctgggcaacatagcaagaccccatctctgaaatttttttaattcctatgtcataagtcatttttatttttgtagagatagggatctcacaatattgcccaggctggtctcaaactcttggcctcaagcagtcctcctgcctcagcctcccaaaatgttgggattactggtatgtgctgctggacccagccaagtagcacttttaatttgaaaaatagttctatcagttttcagtcaggcgcggtggctcagcctgtaatcccagcactttgggaggccgagcgggggtgatcacctgaggtcgggagttcgagactagcctgaccaacatggagaaaccctgtctctactaaaaatacaaaataagccgggcatgttagcgcatgcctgtgatcccagctactcgggaggctgaggcaggagaattgcttgaacccaggaggcagaggttgcggtgagccgagatcatgccattgcactccagcctgggtaacaagagcgaaaactccgtctcaaaaaaaaaaaaagaaaaaatagttctatcagttttcataaagtactactttaatcttaaaaagattaatctagaaacccttcaaattataaaatgtcatttttaaaaggcaggagttgatatcctgatgaaattcaggtctccaaacaacttaccataatttacttcctgtattttaagtaacatgatagggtacttagagattaattgccaagaaactttttgaatatagtcaacctgcccgcacttgccatgatgagttttcttttgttccttccctctagtattctaggagatgaggttttgggaatctggtccagacatgctgagaaagctgatgtcaactgtgcctgtgtatctcattcaggaatcagtcttgttacaggagatgactttggcatggttaagttatttgacttcccatgtccagaaaaatttgtaagtttgtgttttgtttactattatcagtttactcctaattttgatgtcttatcatcagcacttttccccatatatttaaaatgttttgtcctaatttctaaatttttccccaaactttctaaatctatttactttgaaataaaagctattagaaacaaatcctctccctcgagtaataccatctttggaaccatcctacaaaagctgtaattagcttttcaccaaacctataatcagttatcaaatttcaaatgcttttccttagagaaaaatggtcagagtacctggagacatctgactgcccacacagcctggttttgcagatccactactcatgctgaaaagcattctaatcactggctgcggtgctaactccctactctctccacagctcttgtcatagagattatagttcctaataagagcctttgacttctgtgtgcaccaaatgccctgagcttgtctgtcattgttttttaggcaaaacacaaaaggttcttgggtcattcgccccatgtgacaaatattcgatttaccagtggtgatcgacatgttgttagtgctggaggtgatgactgcaggttagtaactttctcagcccatgaagagcagactatgttactagttaagagacttaatacaacaactcctacagctttggtttatgaaatcagctagtcaacattagtagaaggtagtataaccagatggctcttcagaatctcatatttatgcaaatacagaataaaaggagttaaagaggaaaaatattacacatgtaacctgaaagcacaactgaaaaatattaaactgttatgaaaatctaaaaacataattaactccctgcaattttcttctctgattgcagcttatttgtctggaaatgtgtacatacacctcactgagagatgctgagatgactacagaaattaactttgagaccagaattacagagaagaaaaaccaaaacccaaccctgcatggtcaagtggtgctaacccaagactgtaacagggagaaatgcccagaatcatcaaaatagtgaaagactgatctgttcaaaatatttgctatatgcactgggtataatccgtaatccatacactgccagataatgccatttcaaggaaggatcgaatacttgatggtaaaggccaagtccccctgtattgggaagtgtgtgatttcggcagacctgctgggaaaatttagggtagagcactctttacagaagaactcaaaaacccaatttggataattttcattatctttttagcaaaatggtttcttaatgtttatattttattttcaaggttcattgtttaatgaaatattttattcttgcatttccataaggaaagggaaagtcatgatcatcctaaaggatcacagtttttaaaaggcaaacattttccctaaggaaacagacacaagctttcctagagaatatgatgttttttaggcattaataaggtccttttttataaaggacacttttctcctagtagttttgaattcaggaacagatccaaagttagcagtatatggctgctacatttccattttcattttcgagccatcagtttatgttcagatgccatctctgtaatcgcacatttaaaacataactgtagcctcactaatggaaaagtagtatgatgaacaatcattcccaatggtgtacaatgtaagggttttagggagcaacagtatttaactggaagaaagaattgcatatttaatgtagtctaatatatacacatttgtttaacatgtaaacaaaagtgttaaattcacatatacaacattatacaatttaatcactcttggaataaaatttttatagccttttttctattgggaaaatttgtttagatgtgtgccactccataggtttatttccaaaatgaatgagcccaactccatttgtaaaaacttgtcagttagaattcctttttttagtggattagggctgaattcttagatccttatttcttttcactttaaatgctgccaaagatcactactcatcattcaggaattcgctgtctagcctatctgtagtttcctgaagattgaaaattatgtagactgctatttaaaaatatatttttctaagtgtgaggtttaagatgctgtattgaccctatgagtttttaatgtgttaattatctttatagcataatagatcgctttaggttcctggaatcccatttggtctgacaggatatatgaagattcttaatacctattttctgtgtctaatacttggttaatactaaaaatagaaatgactaaattacatcacagaaagcataaccagtgattgaacctggtagttttaaagctctaaatagctgtggctgaaggactgattatggggctaagaagcttgaaacgtaagttggtacttgttcatcagtggattctcctaaattaagccaaattttgaaatacatgactattaagtttctactcatgtatttacagtcagtcaataaattaaaggaggaaaaaaatccctgaacaacctgcccataaaaagaaaaatactctacatttgagcctgctgcagttttaaattttccctctgggtcaagtttgccagcttttggctacagagaaattatatttccattacagtgcaggtagaaactctgtaaccttaagcatgtaaactacatagaataaaactgtttccactgcatttctgtccttcaaagtggccaacctgattaagtcagccttaatcactgctgctgtcagtttcacgactaaaggtcatattgactaagtagtcatcagctgaccacctcgctgtatcagccagcaacgaggggaaggtgaagaaacatgataggccatatagaatctgccctatgtttacttttttaacccagataattatttttgtgtgcagtatctaagctcctgattgtgtaacctgggacttctggcaccttttgttccattcattttatgtataaaatgcatgccaaagcacactgtgccctctggtacccttgcttccaatcgccaaccatgctcatttccttcctttttttgtggtccctttttgtggtgatcattttaaaccacgtcatccaacaaatgttttatggtcaaccttagcttgttcataagccatagcaactgaaagattaaactcttaaatatgtgtctgggcagtggctattaaatagcaaaaaacaatcagattttagtattttattatttccttgtaaaatggctgaactaaattaaacccttgtttcccatttgttctataatttatagtgaaactgagaacaaaactatctttataaatgatagctaaaagtatttccagatatttaaacaatttaaaataaatttcttctgcagagatgcaaagcatctcaacactggaatgaacaaatgccttaaattcaatggagtaaacctttagaatgaagaggaactgtcatttcacccaagccgaagacaacagccttatgcacttgtgtgctctgtctttgctgcttctcgtgtttcaagcctttcctgtgggatcagcacagcaaagtgcaacttaccaaatggtttaatgactggttaattctttcttctcccaatggaaaagcaatggcaacacaacagtagactgctggcttgacaatcttaaacgtgagcctttgcacatgtaggtttatcatcatttgagtatacgactaagcaagtcaatgaactttttttttttttttagcagtttaatttggtcctgagaatgttgcagtctttattaccccttttgcattaatccacttttctaaccaccttttaagctttaatttttaacactatacaccaagtctttgaaatcagtgatctgttatttaactctaaagcatttgacacttcttgccttaacagttttaaaaaccacacacaaaaaaactctgtaagtaatacagtaggccaaaagtttcatcctatctatcttgcagtttacctatctgatctgatctctgtaattatagttctgtcatttaaaatatactatttaaatctaatttttacatttcaaaaattatcttcagtagtaactaagtatattttctgtggattctgagaatgttatttttcagaatgtgagaatatatatgtacatttataatcttgtgactttaaagtctgttttcagatacagtatgtaaatacttgtaaaaaaatttgtataattttgtgataatgtagtttcccaaaaaaattatttagaaggcattatgttattagtaaatgagagcactgtatagaactgttcctattttctgcacttgccattccagctgcctccactgtccatacccacctcattcatcctgtcacagaaggcaggaaaactgggaactttaccaaagtagcactcagcctgagaggcctgtataatcatgcttttcaaactaaattcacttaaaaattaaaaagcagaattgaatattttaagcagcctcagtacctttggccaatgctgttttcatggtggattatgaacattatataatctttgggaaaagtgaaagtagtacaatttttagaataatgacaactgcctcactgcatctctccactcacacagcaaccgtgtagccccctaagctgcagtaccatgactaaccatgatgtcaatttcatatgctgatcctcacaacagcagtgcacaaacatgccccaaatattttaacagaatttagctcttccttaagctgtcttttcatagtaaaaacaaaacaaaaacacccaatgttaaaaccacataataaacttacaaacttgaaaaattagacacttcagatagataggcaataaaacttcatattatgaaagcaatatattccaagtttcaaagatttgacaagttctgtagagtatctttcatcagtacatgaaaacttccaaactgcatgatcttctgccaggcaggactgggtgctattcgctggtttgaggtcgaatccatttcaaggcatgtcgtggtgggacattaatggtgggatggtagaatgtgcagtccggtcttgtacattgagtgttaaacctacaatgttttggatgatagaagggacattccatcttcttacaagcagggaagtaacggcagagctgactactggaaggtggtgctggtggtgcaactggttttggagacagtactggaattcttctactcacatgagtgaagggacaatctggtttagtacactttgcatcatatttacaatttgggtgaacaaacaaacatttttcagcaaatttacaattggggaaggctttgcagggtgagatggggtgatggtaggcacactcatccccatttttacaagcaggccagtacttgcagcgctccaaaagtttttctggtttctgtgccacactcagttcactcatctcagcgttagaaaagctaccatttgggtcctcaagctgcctgctcagcaagtgcaactgctgtgggtggaggagacctctgagtcccttgtttgaggctgcagtttggtttacgggtttcattccttcaaagcacatgtcctcctcttgatctgacatgtatcctggggggctggggacaccatccagcgtcactataaacttgggacttgcaggtttatctggttgtacaagatctcgtgtctgcataaggtgtcctgaaagtacccgaagggaatctgcagtcttcatccccgactcttggtttggtgccactactacttcctcagacagctttggcttcttcagaataaatgatcttgtgtctgcatggaccatggattccatgtcatagtaatcttgatttttttctacagaatctccttttgtttcctcttctttaatggggggacttattctgggggtcctactttgtccctggaccacttctgctagcaattcttcttgagaagttcgagttctgggagcaactggaagtgtctgtttctgtggaactgtagagtagttagttgtttttgttacggattcttgagcttcagatatagccttcaaaatcagattcttgttagcttgtttagaaggtggaagagaaggtctcctttcaggctttgcaggcacagacacactgctggagatgcttcctgttcgagacccgtaatcatcatcttcttcctcctcttctccatcatgattgaatttttttactttaacaactgaacttaccacaggcaactttctcttccgaaagttttcatcctccatactcattttctccgagttgtttctaaagaacggactatacgtttcttctaagctgttaagcacctctggttcacacaaacgtcctgtttcatatacccaactactctgcatatcaagctgcttggcagcatgaatactattctgctgctgttgaaattgcaacctgtttaaatgaacaccactatctgcatttctacttgcaggtggtcgataaatttcaatagaagggcgagaagaaccatatgtaagtgtcactgtaggttttttctgagataagggattctcctgcacaaagttgaggtcttcgtcaatgagatcatctggttctggcttaatatcaatcacatcttcagagggtgctggctccctcaaaggtttcactgttgacattagtcgggttgcagctccatcatcgtaagtctgtctgacatttgtggtttttgactcctgcgaacttgtagaaactctggaatctcttttttcaggtctcgcgctaggaatggcaagtggtggcactgcagcttcatgcctcctctcatctccccgactgaaattgctcttgtttgaaggcacgttactatcaaagatgttggtatcagaagacttcagactagagggttcagttgtaacagagcgaagtttatctaatacaccatgaagccatacggtgaatcgaattgtgttgttccctagaaacagggacagatcctctgtcatttggtcctgacttttcttgttggccaccatcaccataatgtaatcaggaagttcttcatcaacataagctcctaattcttgtaatttccccttaatggcactccggatcttgcggctgatctcggtgccgatctccatggctctgcggcgtgcgggaactcagcactgcgcggcgcttggcttacccggaggctgccgcggactcctaccccgcagccgggacaccaccgcctcc

SEQ ID NO: 17467 - RNA, 13249 nt, Homo sapiens
  source 1..13249: mol_type = other RNA
tcaggccaggcacagtggctcatacctggaatcccagcactttgggaggccgaggcaggcagatcacctgaggtcaaggtatttgagaccagcctggccaacatggtgaaaccccatctctactaaaaatacagaaattagctgggtgtggtggtgcacacctgtaatgctagctactcgggaggctgaggtaggagaatcgcttgaacctgggaggcagaggttgcaataagcctagatcatgccactgcactcaagcctgggagacagagcgagactacatcttaaaaaaaaaaaaaaaagtattatgagagaggataatgtattgtaatgtattgtagaggctaaataaaattatgctcatgtcagaaaaaaagagtatttctcaaaataaaattcactgaaactggatgtttattttgactgagatatagtatatcctcaaattgccatagaaagtttacaagaatattagaggtaaattataaatatcagggcctttttaaaaaaaaaagattctgcttataacttggtatttgtttataataaaaattatagtagccaataatgaacacttactctggcttggttatttacttaggtcaaaagaaggaggagcggttaaactgtgggatcaggaactgaggcggtgccgtgccttcaggcttgagacaggacaagccacagattgtgttcgttctgtgtgcagaggcaaagtaagatgttccatgagctgatacagtgcagcagaaaacagaaagtggttattactgtgattccctcaccctttgcagcctaatgaacaatacttaataatgcataacgatggatttgcttgccaacattactctgtctttgctgctttctttgccaaagttagcaccagtgtggtgcataagctaggaagctattctgtctaaatactgtatgtaaacctccaatattttctagaatctgccaatttaacaactctagtagacataattgaaagcccttggcagttgactcatattaggacagctgtctccattttttaaaaaaacacacattccctagataaaacgtgcagtaaacaaacaatgaaatactactcagccataaaaaataatgaaattctgtcattcttggtggcaacatggatgagactggaggacatgatgtgaagtgaaataagccaggcacagaaagataaatacatgttctcactcctgtgcagaaactaaaaaagttgatcccacagaggtggagagtagaatagtggttactggaggcggacaagggggagggggagggggatagggaaggactggttaaaggatacaagtttacacagccagataggaatagtatgttttagtattctgtagtactgtaggatgactatagttaagaatcacgtatttatgtattttcaggtatttacaagagaggattttgaaagtttccatcacaaagaaatgataaatgtctgaggtgatggttatgcgtattaccctatgccctatagatatgtataattatgtgtcaatttcaaaataaaaattcaaaactacaactcctatgaaaatttttgagcgtgtttgtacttattaagtgtatttataaatcatacggatattatcttcagcctgcatattaaattgtagttaagcttttactttttaactaaaaaataaattctattattttttcctatatcccactgcactgaccccagtttggaaatcctaagattatcaaataaaaactttgattattgaagaatccaggtgtactgccacagaaaagttctattctgtagcatggactctaatatgtaatctagcccattgtgcttacagatagatgtgtgcctgtagtcatagaaaaatttgcatgagctaatgactgccttgctactagattagctcaaagcaaaaagttctctgaaagcaggtcaatagggtcatttttatattatgaagaagaaaagcagctgttgtattacattcactgtattggtcctgcttgtgtttcagggcaagatccttgttgggacaaggaatgctgaaataatcgaagttggagagaaaaatgcagcttgtaatattttagttaacggtcatgtggatgggccaatctggggactagcaacacatccttccagggattttttcctttctgctgcagaagatgggacagtgagactttgggatattgctgataaagtaagtacagataatttttttaaaagaggttacaacttctaaaaagaaaagttggaagttctaaattgctagtacttaaagaactgccagaattctgttgagcattttgaggggaaactggtataatttagaagtacttcacttaatgtttcctatgactctttttttttttttttttaaatgcagaagatgttaaacaaagtgaatttgggacatgctgctcgtactgtgtgttacagccctgaaggggacatggtggctattggaatgaaaaatggagaatttatcattttactagtgagttctctaaaaatatggggaaagaagagagacaggagatgtgcaatccatgatatcaggttagtgaacaaatggaatagagtttctagtatatacttgatttaacttccatttgtaaaattttccatagccttgccttcaaaaagaggtccccagggcctgtagcatttcccgtattataaattgtatgctaaaatatggctgtttgtatactacttaattcttcttgctaaattataaacccactgggcaccaactataatagcaagtactagtaggtaatgtttgatgaattcatgttaacacttagccatgtccattaagttcatcccaccaagaggtatctcccactgtaatacaagagagctatctgcccttcaaaagttgtcaccctggaaaactaaagttgtgatttcaaacatatcttctcttagtaacctcagtttgggaatatgtagttcattaatttaatcaatacctattgattaaatgttccagaatccaaattaatttaaatgtttcttaaacctttgtttttcagtgcttaagcatttttcaacagtggctaccatttacggagtacttccgtgtgatcagtagataagattattgaatctaggtctgtcaaaagcttgtacacttttcatcagtaaaatccttttacaaatgaaaccttcctcagaacttcaatatataaaatagtaacagtggcttcccttagcttttacatgtctctatcgtacctcagtaagactcatgggccatttcaagagactgaattgtcccatatgactccaaagattgctaggcaaatagcatttcactttgtcttttaaataagttcttcaggccgggcgcggtggctcatgcctgtaatcccagcactttgggaggccgaggcaggcagatcacctgaagtcaggagtactcgaccagcctggccaacatagtgaaaccccatctcaactaaaaatacaaaaatcagccgggcgtggtggcaggcgcctgtaatcccagctactcagggggctgaaacaggagaatcgcttgaacccgggaggcggaggttgcgccatcgcactccagcctgggagacaagagcgagacttcgtctcaaaaaaaaaaaattcttcttccaagattcaagttgtgtcatttcaccttaataactggaggttagttaagctgggctgtgttctttgcttaatattaagacaacgttttttccagatggaagaaaactatcttaatgaattgttagcttattaattatgtaatgctaatggcttttaaaagctgagatgttctgactgggtgttgtggctcacacctgtaatcccagtaccttgggaggccaagggggaaggattgcttgaggccaggagtttgggaccatagtgagaccccgcctctatttaaaaaattaaattttgttttgttttgttttgagttggagttttgctcttgttgcccatgctgaagtgcaatggtgcaatctcagctcaccacaacctgtgcctcctgggttcaagcgattctcctgcttcagcctcccgagtagatgggattacaggcgtgcaccaccatgcctggctaattttgtatttttagtagagacagggtttctctatgttggtcaggctggtctcaaactctcgacctcaggtgatctgcccgcctccgcttcccaaagttctgggattataggtgtgagccactgggcctggcctaagaaagtttttttaagccattagacgtttttaaaggaattgggagatgacaattggggaaatatttaaaatttaagtaaaatataaagcttccttatttcatgtaacccagacaatctcagtatacatgatcagttgtgtctgacaggtaaatctatttgaggccttatcacacgttacttttaagaactagaaaggaaaagtcactgatcttaagtatttataatacttcatgtggtctaatactttttacgttttgttttgattcagatttagtccggattcccggtatctggcagtaggttctagtgagaactcagtggatttttatgacctaacgctgggccccactcttaacagaatcagctactgcaaagacattccaagctttgtcattcaaatggacttctctgcagatagcagttatctccaggtacagtaccaatactgtatacccaggtggcaagttcttctgcttttacatttcgtgttagtgaatgcatttaaagttcctgagctccagagctccagcttctcaactcctccctttgtaccttctgacctacagctcccctttcctcccccacttatcagagcttttctcctattaagtttttgtagtgatcttttgcatacttaataatgttagacatgtaaatcaagtagcaatatgctagtattctgtaaaccccctgtggattttgtctctcacctaatggaattcttgtcccattttaatctgatgaaaaaggtctctagtggctgctataaacggcatgtctatgaagtgccttcaggaaaacatcttatggatcatgccgctattgacagaattacttgggctacatggactaggtaaatacttatatattcacaaggcaagaactgactttgaaggccagttagaaaatcctatttctgaactgttagagccattccaataaggaatagtaattgagtttcaagtttttgttaccatattttgaaatggtatgttcatgttgggacccctttttattgaatatatttccatgttttatcagtttccatgatttatcaagttttttttttaaggaaatcaaagttttaactttaaagataccctgatatttttcttaatgctaaatttaatgactggcaaaaaggtattgggtgctgttaagcaactgttattaattctctatctaaaggaatgctatcttgaatctattagaagtcaaagcttccaaatttgttcaaatttcctggctgtatgacaggtaaccatgactatccatttttttggccaatgaaaaatgccatcaaattcctgtatcagccaggcatatagtggctcatgcctgtaatctctgatgtagcaggccgaggtgggaggatcacttgagcctagaagttttgataccagcctgggcaacatagcaagaccccatctctgaaatttttttaattcctatgtcataagtcatttttatttttgtagagatagggatctcacaatattgcccaggctggtctcaaactcttggcctcaagcagtcctcctgcctcagcctcccaaaatgttgggattactggtatgtgctgctggacccagccaagtagcacttttaatttgaaaaatagttctatcagttttcagtcaggcgcggtggctcagcctgtaatcccagcactttgggaggccgagcgggggtgatcacctgaggtcgggagttcgagactagcctgaccaacatggagaaaccctgtctctactaaaaatacaaaataagccgggcatgttagcgcatgcctgtgatcccagctactcgggaggctgaggcaggagaattgcttgaacccaggaggcagaggttgcggtgagccgagatcatgccattgcactccagcctgggtaacaagagcgaaaactccgtctcaaaaaaaaaaaaagaaaaaatagttctatcagttttcataaagtactactttaatcttaaaaagattaatctagaaacccttcaaattataaaatgtcatttttaaaaggcaggagttgatatcctgatgaaattcaggtctccaaacaacttaccataatttacttcctgtattttaagtaacatgatagggtacttagagattaattgccaagaaactttttgaatatagtcaacctgcccgcacttgccatgatgagttttcttttgttccttccctctagtattctaggagatgaggttttgggaatctggtccagacatgctgagaaagctgatgtcaactgtgcctgtgtatctcattcaggaatcagtcttgttacaggagatgactttggcatggttaagttatttgacttcccatgtccagaaaaatttgtaagtttgtgttttgtttactattatcagtttactcctaattttgatgtcttatcatcagcacttttccccatatatttaaaatgttttgtcctaatttctaaatttttccccaaactttctaaatctatttactttgaaataaaagctattagaaacaaatcctctccctcgagtaataccatctttggaaccatcctacaaaagctgtaattagcttttcaccaaacctataatcagttatcaaatttcaaatgcttttccttagagaaaaatggtcagagtacctggagacatctgactgcccacacagcctggttttgcagatccactactcatgctgaaaagcattctaatcactggctgcggtgctaactccctactctctccacagctcttgtcatagagattatagttcctaataagagcctttgacttctgtgtgcaccaaatgccctgagcttgtctgtcattgttttttaggcaaaacacaaaaggttcttgggtcattcgccccatgtgacaaatattcgatttaccagtggtgatcgacatgttgttagtgctggaggtgatgactgcaggttagtaactttctcagcccatgaagagcagactatgttactagttaagagacttaatacaacaactcctacagctttggtttatgaaatcagctagtcaacattagtagaaggtagtataaccagatggctcttcagaatctcatatttatgcaaatacagaataaaaggagttaaagaggaaaaatattacacatgtaacctgaaagcacaactgaaaaatattaaactgttatgaaaatctaaaaacataattaactccctgcaattttcttctctgattgcagcttatttgtctggaaatgtgtacatacacctcactgagagatgctgagatgactacagaaattaactttgagaccagaattacagagaagaaaaaccaaaacccaaccctgcatggtcaagtggtgctaacccaagactgtaacagggagaaatgcccagaatcatcaaaatagtgaaagactgatctgttcaaaatatttgctatatgcactgggtataatccgtaatccatacactgccagataatgccatttcaaggaaggatcgaatacttgatggtaaaggccaagtccccctgtattgggaagtgtgtgatttcggcagacctgctgggaaaatttagggtagagcactctttacagaagaactcaaaaacccaatttggataattttcattatctttttagcaaaatggtttcttaatgtttatattttattttcaaggttcattgtttaatgaaatattttattcttgcatttccataaggaaagggaaagtcatgatcatcctaaaggatcacagtttttaaaaggcaaacattttccctaaggaaacagacacaagctttcctagagaatatgatgttttttaggcattaataaggtccttttttataaaggacacttttctcctagtagttttgaattcaggaacagatccaaagttagcagtatatggctgctacatttccattttcattttcgagccatcagtttatgttcagatgccatctctgtaatcgcacatttaaaacataactgtagcctcactaatggaaaagtagtatgatgaacaatcattcccaatggtgtacaatgtaagggttttagggagcaacagtatttaactggaagaaagaattgcatatttaatgtagtctaatatatacacatttgtttaacatgtaaacaaaagtgttaaattcacatatacaacattatacaatttaatcactcttggaataaaatttttatagccttttttctattgggaaaatttgtttagatgtgtgccactccataggtttatttccaaaatgaatgagcccaactccatttgtaaaaacttgtcagttagaattcctttttttagtggattagggctgaattcttagatccttatttcttttcactttaaatgctgccaaagatcactactcatcattcaggaattcgctgtctagcctatctgtagtttcctgaagattgaaaattatgtagactgctatttaaaaatatatttttctaagtgtgaggtttaagatgctgtattgaccctatgagtttttaatgtgttaattatctttatagcataatagatcgctttaggttcctggaatcccatttggtctgacaggatatatgaagattcttaatacctattttctgtgtctaatacttggttaatactaaaaatagaaatgactaaattacatcacagaaagcataaccagtgattgaacctggtagttttaaagctctaaatagctgtggctgaaggactgattatggggctaagaagcttgaaacgtaagttggtacttgttcatcagtggattctcctaaattaagccaaattttgaaatacatgactattaagtttctactcatgtatttacagtcagtcaataaattaaaggaggaaaaaaatccctgaacaacctgcccataaaaagaaaaatactctacatttgagcctgctgcagttttaaattttccctctgggtcaagtttgccagcttttggctacagagaaattatatttccattacagtgcaggtagaaactctgtaaccttaagcatgtaaactacatagaataaaactgtttccactgcatttctgtccttcaaagtggccaacctgattaagtcagccttaatcactgctgctgtcagtttcacgactaaaggtcatattgactaagtagtcatcagctgaccacctcgctgtatcagccagcaacgaggggaaggtgaagaaacatgataggccatatagaatctgccctatgtttacttttttaacccagataattatttttgtgtgcagtatctaagctcctgattgtgtaacctgggacttctggcaccttttgttccattcattttatgtataaaatgcatgccaaagcacactgtgccctctggtacccttgcttccaatcgccaaccatgctcatttccttcctttttttgtggtccctttttgtggtgatcattttaaaccacgtcatccaacaaatgttttatggtcaaccttagcttgttcataagccatagcaactgaaagattaaactcttaaatatgtgtctgggcagtggctattaaatagcaaaaaacaatcagattttagtattttattatttccttgtaaaatggctgaactaaattaaacccttgtttcccatttgttctataatttatagtgaaactgagaacaaaactatctttataaatgatagctaaaagtatttccagatatttaaacaatttaaaataaatttcttctgcagagatgcaaagcatctcaacactggaatgaacaaatgccttaaattcaatggagtaaacctttagaatgaagaggaactgtcatttcacccaagccgaagacaacagccttatgcacttgtgtgctctgtctttgctgcttctcgtgtttcaagcctttcctgtgggatcagcacagcaaagtgcaacttaccaaatggtttaatgactggttaattctttcttctcccaatggaaaagcaatggcaacacaacagtagactgctggcttgacaatcttaaacgtgagcctttgcacatgtaggtttatcatcatttgagtatacgactaagcaagtcaatgaactttttttttttttttagcagtttaatttggtcctgagaatgttgcagtctttattaccccttttgcattaatccacttttctaaccaccttttaagctttaatttttaacactatacaccaagtctttgaaatcagtgatctgttatttaactctaaagcatttgacacttcttgccttaacagttttaaaaaccacacacaaaaaaactctgtaagtaatacagtaggccaaaagtttcatcctatctatcttgcagtttacctatctgatctgatctctgtaattatagttctgtcatttaaaatatactatttaaatctaatttttacatttcaaaaattatcttcagtagtaactaagtatattttctgtggattctgagaatgttatttttcagaatgtgagaatatatatgtacatttataatcttgtgactttaaagtctgttttcagatacagtatgtaaatacttgtaaaaaaatttgtataattttgtgataatgtagtttcccaaaaaaattatttagaaggcattatgttattagtaaatgagagcactgtatagaactgttcctattttctgcacttgccattccagctgcctccactgtccatacccacctcattcatcctgtcacagaaggcaggaaaactgggaactttaccaaagtagcactcagcctgagaggcctgtataatcatgcttttcaaactaaattcacttaaaaattaaaaagcagaattgaatattttaagcagcctcagtacctttggccaatgctgttttcatggtggattatgaacattatataatctttgggaaaagtgaaagtagtacaatttttagaataatgacaactgcctcactgcatctctccactcacacagcaaccgtgtagccccctaagctgcagtaccatgactaaccatgatgtcaatttcatatgctgatcctcacaacagcagtgcacaaacatgccccaaatattttaacagaatttagctcttccttaagctgtcttttcatagtaaaaacaaaacaaaaacacccaatgttaaaaccacataataaacttacaaacttgaaaaattagacacttcagatagataggcaataaaacttcatattatgaaagcaatatattccaagtttcaaagatttgacaagttctgtagagtatctttcatcagtacatgaaaacttccaaactgcatgatcttctgccaggcaggactgggtgctattcgctggtttgaggtcgaatccatttcaaggcatgtcgtggtgggacattaatggtgggatggtagaatgtgcagtccggtcttgtacattgagtgttaaacctacaatgttttggatgatagaagggacattccatcttcttacaagcagggaagtaacggcagagctgactactggaaggtggtgctggtggtgcaactggttttggagacagtactggaattcttctactcacatgagtgaagggacaatctggtttagtacactttgcatcatatttacaatttgggtgaacaaacaaacatttttcagcaaatttacaattggggaaggctttgcagggtgagatggggtgatggtaggcacactcatccccatttttacaagcaggccagtacttgcagcgctccaaaagtttttctggtttctgtgccacactcagttcactcatctcagctgtagagtagttagttgtttttgttacggattcttgagcttcagatatagccttcaaaatcagattcttgttagcttgtttagaaggtggaagagaaggtctcctttcaggctttgcaggcacagacacactgctggagatgcttcctgttcgagacccgtaatcatcatcttcttcctcctcttctccatcatgattgaatttttttactttaacaactgaacttaccacaggcaactttctcttccgaaagttttcatcctccatactcattttctccgagttgtttctaaagaacggactatacgtttcttctaagctgttaagcacctctggttcacacaaacgtcctgtttcatatacccaactactctgcatatcaagctgcttggcagcatgaatactattctgctgctgttgaaattgcaacctgtttaaatgaacaccactatctgcatttctacttgcaggtggtcgataaatttcaatagaagggcgagaagaaccatatgtaagtgtcactgtaggttttttctgagataagggattctcctgcacaaagttgaggtcttcgtcaatgagatcatctggttctggcttaatatcaatcacatcttcagagggtgctggctccctcaaaggtttcactgttgacattagtcgggttgcagctccatcatcgtaagtctgtctgacatttgtggtttttgactcctgcgaacttgtagaaactctggaatctcttttttcaggtctcgcgctaggaatggcaagtggtggcactgcagcttcatgcctcctctcatctccccgactgaaattgctcttgtttgaaggcacgttactatcaaagatgttggtatcagaagacttcagactagagggttcagttgtaacagagcgaagtttatctaatacaccatgaagccatacggtgaatcgaattgtgttgttccctagaaacagggacagatcctctgtcatttggtcctgacttttcttgttggccaccatcaccataatgtaatcaggaagttcttcatcaacataagctcctaattcttgtaatttccccttaatggcactccggatcttgcggctgatctcggtgccgatctccatggctctgcggcgtgcgggaactcagcactgcgcggcgcttggcttacccggaggctgccgcggactcctaccccgcagccgggacaccaccgcctcc

SEQ ID NO: 17468 - RNA, 13365 nt, Homo sapiens
  source 1..13365: mol_type = other RNA
tcaggccaggcacagtggctcatacctggaatcccagcactttgggaggccgaggcaggcagatcacctgaggtcaaggtatttgagaccagcctggccaacatggtgaaaccccatctctactaaaaatacagaaattagctgggtgtggtggtgcacacctgtaatgctagctactcgggaggctgaggtaggagaatcgcttgaacctgggaggcagaggttgcaataagcctagatcatgccactgcactcaagcctgggagacagagcgagactacatcttaaaaaaaaaaaaaaaagtattatgagagaggataatgtattgtaatgtattgtagaggctaaataaaattatgctcatgtcagaaaaaaagagtatttctcaaaataaaattcactgaaactggatgtttattttgactgagatatagtatatcctcaaattgccatagaaagtttacaagaatattagaggtaaattataaatatcagggcctttttaaaaaaaaaagattctgcttataacttggtatttgtttataataaaaattatagtagccaataatgaacacttactctggcttggttatttacttaggtcaaaagaaggaggagcggttaaactgtgggatcaggaactgaggcggtgccgtgccttcaggcttgagacaggacaagccacagattgtgttcgttctgtgtgcagaggcaaagtaagatgttccatgagctgatacagtgcagcagaaaacagaaagtggttattactgtgattccctcaccctttgcagcctaatgaacaatacttaataatgcataacgatggatttgcttgccaacattactctgtctttgctgctttctttgccaaagttagcaccagtgtggtgcataagctaggaagctattctgtctaaatactgtatgtaaacctccaatattttctagaatctgccaatttaacaactctagtagacataattgaaagcccttggcagttgactcatattaggacagctgtctccattttttaaaaaaacacacattccctagataaaacgtgcagtaaacaaacaatgaaatactactcagccataaaaaataatgaaattctgtcattcttggtggcaacatggatgagactggaggacatgatgtgaagtgaaataagccaggcacagaaagataaatacatgttctcactcctgtgcagaaactaaaaaagttgatcccacagaggtggagagtagaatagtggttactggaggcggacaagggggagggggagggggatagggaaggactggttaaaggatacaagtttacacagccagataggaatagtatgttttagtattctgtagtactgtaggatgactatagttaagaatcacgtatttatgtattttcaggtatttacaagagaggattttgaaagtttccatcacaaagaaatgataaatgtctgaggtgatggttatgcgtattaccctatgccctatagatatgtataattatgtgtcaatttcaaaataaaaattcaaaactacaactcctatgaaaatttttgagcgtgtttgtacttattaagtgtatttataaatcatacggatattatcttcagcctgcatattaaattgtagttaagcttttactttttaactaaaaaataaattctattattttttcctatatcccactgcactgaccccagtttggaaatcctaagattatcaaataaaaactttgattattgaagaatccaggtgtactgccacagaaaagttctattctgtagcatggactctaatatgtaatctagcccattgtgcttacagatagatgtgtgcctgtagtcatagaaaaatttgcatgagctaatgactgccttgctactagattagctcaaagcaaaaagttctctgaaagcaggtcaatagggtcatttttatattatgaagaagaaaagcagctgttgtattacattcactgtattggtcctgcttgtgtttcagggcaagatccttgttgggacaaggaatgctgaaataatcgaagttggagagaaaaatgcagcttgtaatattttagttaacggtcatgtggatgggccaatctggggactagcaacacatccttccagggattttttcctttctgctgcagaagatgggacagtgagactttgggatattgctgataaagtaagtacagataatttttttaaaagaggttacaacttctaaaaagaaaagttggaagttctaaattgctagtacttaaagaactgccagaattctgttgagcattttgaggggaaactggtataatttagaagtacttcacttaatgtttcctatgactctttttttttttttttttaaatgcagaagatgttaaacaaagtgaatttgggacatgctgctcgtactgtgtgttacagccctgaaggggacatggtggctattggaatgaaaaatggagaatttatcattttactagtgagttctctaaaaatatggggaaagaagagagacaggagatgtgcaatccatgatatcaggttagtgaacaaatggaatagagtttctagtatatacttgatttaacttccatttgtaaaattttccatagccttgccttcaaaaagaggtccccagggcctgtagcatttcccgtattataaattgtatgctaaaatatggctgtttgtatactacttaattcttcttgctaaattataaacccactgggcaccaactataatagcaagtactagtaggtaatgtttgatgaattcatgttaacacttagccatgtccattaagttcatcccaccaagaggtatctcccactgtaatacaagagagctatctgcccttcaaaagttgtcaccctggaaaactaaagttgtgatttcaaacatatcttctcttagtaacctcagtttgggaatatgtagttcattaatttaatcaatacctattgattaaatgttccagaatccaaattaatttaaatgtttcttaaacctttgtttttcagtgcttaagcatttttcaacagtggctaccatttacggagtacttccgtgtgatcagtagataagattattgaatctaggtctgtcaaaagcttgtacacttttcatcagtaaaatccttttacaaatgaaaccttcctcagaacttcaatatataaaatagtaacagtggcttcccttagcttttacatgtctctatcgtacctcagtaagactcatgggccatttcaagagactgaattgtcccatatgactccaaagattgctaggcaaatagcatttcactttgtcttttaaataagttcttcaggccgggcgcggtggctcatgcctgtaatcccagcactttgggaggccgaggcaggcagatcacctgaagtcaggagtactcgaccagcctggccaacatagtgaaaccccatctcaactaaaaatacaaaaatcagccgggcgtggtggcaggcgcctgtaatcccagctactcagggggctgaaacaggagaatcgcttgaacccgggaggcggaggttgcgccatcgcactccagcctgggagacaagagcgagacttcgtctcaaaaaaaaaaaattcttcttccaagattcaagttgtgtcatttcaccttaataactggaggttagttaagctgggctgtgttctttgcttaatattaagacaacgttttttccagatggaagaaaactatcttaatgaattgttagcttattaattatgtaatgctaatggcttttaaaagctgagatgttctgactgggtgttgtggctcacacctgtaatcccagtaccttgggaggccaagggggaaggattgcttgaggccaggagtttgggaccatagtgagaccccgcctctatttaaaaaattaaattttgttttgttttgttttgagttggagttttgctcttgttgcccatgctgaagtgcaatggtgcaatctcagctcaccacaacctgtgcctcctgggttcaagcgattctcctgcttcagcctcccgagtagatgggattacaggcgtgcaccaccatgcctggctaattttgtatttttagtagagacagggtttctctatgttggtcaggctggtctcaaactctcgacctcaggtgatctgcccgcctccgcttcccaaagttctgggattataggtgtgagccactgggcctggcctaagaaagtttttttaagccattagacgtttttaaaggaattgggagatgacaattggggaaatatttaaaatttaagtaaaatataaagcttccttatttcatgtaacccagacaatctcagtatacatgatcagttgtgtctgacaggtaaatctatttgaggccttatcacacgttacttttaagaactagaaaggaaaagtcactgatcttaagtatttataatacttcatgtggtctaatactttttacgttttgttttgattcagatttagtccggattcccggtatctggcagtaggttctagtgagaactcagtggatttttatgacctaacgctgggccccactcttaacagaatcagctactgcaaagacattccaagctttgtcattcaaatggacttctctgcagatagcagttatctccaggtacagtaccaatactgtatacccaggtggcaagttcttctgcttttacatttcgtgttagtgaatgcatttaaagttcctgagctccagagctccagcttctcaactcctccctttgtaccttctgacctacagctcccctttcctcccccacttatcagagcttttctcctattaagtttttgtagtgatcttttgcatacttaataatgttagacatgtaaatcaagtagcaatatgctagtattctgtaaaccccctgtggattttgtctctcacctaatggaattcttgtcccattttaatctgatgaaaaaggtctctagtggctgctataaacggcatgtctatgaagtgccttcaggaaaacatcttatggatcatgccgctattgacagaattacttgggctacatggactaggtaaatacttatatattcacaaggcaagaactgactttgaaggccagttagaaaatcctatttctgaactgttagagccattccaataaggaatagtaattgagtttcaagtttttgttaccatattttgaaatggtatgttcatgttgggacccctttttattgaatatatttccatgttttatcagtttccatgatttatcaagttttttttttaaggaaatcaaagttttaactttaaagataccctgatatttttcttaatgctaaatttaatgactggcaaaaaggtattgggtgctgttaagcaactgttattaattctctatctaaaggaatgctatcttgaatctattagaagtcaaagcttccaaatttgttcaaatttcctggctgtatgacaggtaaccatgactatccatttttttggccaatgaaaaatgccatcaaattcctgtatcagccaggcatatagtggctcatgcctgtaatctctgatgtagcaggccgaggtgggaggatcacttgagcctagaagttttgataccagcctgggcaacatagcaagaccccatctctgaaatttttttaattcctatgtcataagtcatttttatttttgtagagatagggatctcacaatattgcccaggctggtctcaaactcttggcctcaagcagtcctcctgcctcagcctcccaaaatgttgggattactggtatgtgctgctggacccagccaagtagcacttttaatttgaaaaatagttctatcagttttcagtcaggcgcggtggctcagcctgtaatcccagcactttgggaggccgagcgggggtgatcacctgaggtcgggagttcgagactagcctgaccaacatggagaaaccctgtctctactaaaaatacaaaataagccgggcatgttagcgcatgcctgtgatcccagctactcgggaggctgaggcaggagaattgcttgaacccaggaggcagaggttgcggtgagccgagatcatgccattgcactccagcctgggtaacaagagcgaaaactccgtctcaaaaaaaaaaaaagaaaaaatagttctatcagttttcataaagtactactttaatcttaaaaagattaatctagaaacccttcaaattataaaatgtcatttttaaaaggcaggagttgatatcctgatgaaattcaggtctccaaacaacttaccataatttacttcctgtattttaagtaacatgatagggtacttagagattaattgccaagaaactttttgaatatagtcaacctgcccgcacttgccatgatgagttttcttttgttccttccctctagtattctaggagatgaggttttgggaatctggtccagacatgctgagaaagctgatgtcaactgtgcctgtgtatctcattcaggaatcagtcttgttacaggagatgactttggcatggttaagttatttgacttcccatgtccagaaaaatttgtaagtttgtgttttgtttactattatcagtttactcctaattttgatgtcttatcatcagcacttttccccatatatttaaaatgttttgtcctaatttctaaatttttccccaaactttctaaatctatttactttgaaataaaagctattagaaacaaatcctctccctcgagtaataccatctttggaaccatcctacaaaagctgtaattagcttttcaccaaacctataatcagttatcaaatttcaaatgcttttccttagagaaaaatggtcagagtacctggagacatctgactgcccacacagcctggttttgcagatccactactcatgctgaaaagcattctaatcactggctgcggtgctaactccctactctctccacagctcttgtcatagagattatagttcctaataagagcctttgacttctgtgtgcaccaaatgccctgagcttgtctgtcattgttttttaggcaaaacacaaaaggttcttgggtcattcgccccatgtgacaaatattcgatttaccagtggtgatcgacatgttgttagtgctggaggtgatgactgcaggttagtaactttctcagcccatgaagagcagactatgttactagttaagagacttaatacaacaactcctacagctttggtttatgaaatcagctagtcaacattagtagaaggtagtataaccagatggctcttcagaatctcatatttatgcaaatacagaataaaaggagttaaagaggaaaaatattacacatgtaacctgaaagcacaactgaaaaatattaaactgttatgaaaatctaaaaacataattaactccctgcaattttcttctctgattgcagcttatttgtctggaaatgtgtacatacacctcactgagagatgctgagatgactacagaaattaactttgagaccagaattacagagaagaaaaaccaaaacccaaccctgcatggtcaagtggtgctaacccaagactgtaacagggagaaatgcccagaatcatcaaaatagtgaaagactgatctgttcaaaatatttgctatatgcactgggtataatccgtaatccatacactgccagataatgccatttcaaggaaggatcgaatacttgatggtaaaggccaagtccccctgtattgggaagtgtgtgatttcggcagacctgctgggaaaatttagggtagagcactctttacagaagaactcaaaaacccaatttggataattttcattatctttttagcaaaatggtttcttaatgtttatattttattttcaaggttcattgtttaatgaaatattttattcttgcatttccataaggaaagggaaagtcatgatcatcctaaaggatcacagtttttaaaaggcaaacattttccctaaggaaacagacacaagctttcctagagaatatgatgttttttaggcattaataaggtccttttttataaaggacacttttctcctagtagttttgaattcaggaacagatccaaagttagcagtatatggctgctacatttccattttcattttcgagccatcagtttatgttcagatgccatctctgtaatcgcacatttaaaacataactgtagcctcactaatggaaaagtagtatgatgaacaatcattcccaatggtgtacaatgtaagggttttagggagcaacagtatttaactggaagaaagaattgcatatttaatgtagtctaatatatacacatttgtttaacatgtaaacaaaagtgttaaattcacatatacaacattatacaatttaatcactcttggaataaaatttttatagccttttttctattgggaaaatttgtttagatgtgtgccactccataggtttatttccaaaatgaatgagcccaactccatttgtaaaaacttgtcagttagaattcctttttttagtggattagggctgaattcttagatccttatttcttttcactttaaatgctgccaaagatcactactcatcattcaggaattcgctgtctagcctatctgtagtttcctgaagattgaaaattatgtagactgctatttaaaaatatatttttctaagtgtgaggtttaagatgctgtattgaccctatgagtttttaatgtgttaattatctttatagcataatagatcgctttaggttcctggaatcccatttggtctgacaggatatatgaagattcttaatacctattttctgtgtctaatacttggttaatactaaaaatagaaatgactaaattacatcacagaaagcataaccagtgattgaacctggtagttttaaagctctaaatagctgtggctgaaggactgattatggggctaagaagcttgaaacgtaagttggtacttgttcatcagtggattctcctaaattaagccaaattttgaaatacatgactattaagtttctactcatgtatttacagtcagtcaataaattaaaggaggaaaaaaatccctgaacaacctgcccataaaaagaaaaatactctacatttgagcctgctgcagttttaaattttccctctgggtcaagtttgccagcttttggctacagagaaattatatttccattacagtgcaggtagaaactctgtaaccttaagcatgtaaactacatagaataaaactgtttccactgcatttctgtccttcaaagtggccaacctgattaagtcagccttaatcactgctgctgtcagtttcacgactaaaggtcatattgactaagtagtcatcagctgaccacctcgctgtatcagccagcaacgaggggaaggtgaagaaacatgataggccatatagaatctgccctatgtttacttttttaacccagataattatttttgtgtgcagtatctaagctcctgattgtgtaacctgggacttctggcaccttttgttccattcattttatgtataaaatgcatgccaaagcacactgtgccctctggtacccttgcttccaatcgccaaccatgctcatttccttcctttttttgtggtccctttttgtggtgatcattttaaaccacgtcatccaacaaatgttttatggtcaaccttagcttgttcataagccatagcaactgaaagattaaactcttaaatatgtgtctgggcagtggctattaaatagcaaaaaacaatcagattttagtattttattatttccttgtaaaatggctgaactaaattaaacccttgtttcccatttgttctataatttatagtgaaactgagaacaaaactatctttataaatgatagctaaaagtatttccagatatttaaacaatttaaaataaatttcttctgcagagatgcaaagcatctcaacactggaatgaacaaatgccttaaattcaatggagtaaacctttagaatgaagaggaactgtcatttcacccaagccgaagacaacagccttatgcacttgtgtgctctgtctttgctgcttctcgtgtttcaagcctttcctgtgggatcagcacagcaaagtgcaacttaccaaatggtttaatgactggttaattctttcttctcccaatggaaaagcaatggcaacacaacagtagactgctggcttgacaatcttaaacgtgagcctttgcacatgtaggtttatcatcatttgagtatacgactaagcaagtcaatgaactttttttttttttttagcagtttaatttggtcctgagaatgttgcagtctttattaccccttttgcattaatccacttttctaaccaccttttaagctttaatttttaacactatacaccaagtctttgaaatcagtgatctgttatttaactctaaagcatttgacacttcttgccttaacagttttaaaaaccacacacaaaaaaactctgtaagtaatacagtaggccaaaagtttcatcctatctatcttgcagtttacctatctgatctgatctctgtaattatagttctgtcatttaaaatatactatttaaatctaatttttacatttcaaaaattatcttcagtagtaactaagtatattttctgtggattctgagaatgttatttttcagaatgtgagaatatatatgtacatttataatcttgtgactttaaagtctgttttcagatacagtatgtaaatacttgtaaaaaaatttgtataattttgtgataatgtagtttcccaaaaaaattatttagaaggcattatgttattagtaaatgagagcactgtatagaactgttcctattttctgcacttgccattccagctgcctccactgtccatacccacctcattcatcctgtcacagaaggcaggaaaactgggaactttaccaaagtagcactcagcctgagaggcctgtataatcatgcttttcaaactaaattcacttaaaaattaaaaagcagaattgaatattttaagcagcctcagtacctttggccaatgctgttttcatggtggattatgaacattatataatctttgggaaaagtgaaagtagtacaatttttagaataatgacaactgcctcactgcatctctccactcacacagcaaccgtgtagccccctaagctgcagtaccatgactaaccatgatgtcaatttcatatgctgatcctcacaacagcagtgcacaaacatgccccaaatattttaacagaatttagctcttccttaagctgtcttttcatagtaaaaacaaaacaaaaacacccaatgttaaaaccacataataaacttacaaacttgaaaaattagacacttcagatagataggcaataaaacttcatattatgaaagcaatatattccaagtttcaaagatttgacaagttctgtagagtatctttcatcagtacatgaaaacttccaaactgcatgatcttctgccaggcaggactgggtgctattcgctggtttgaggtcgaatccatttcaaggcatgtcgtggtgggacattaatggtgggatggtagaatgtgcagtccggtcttgtacattgagtgttaaacctacaatgttttggatgatagaagggacattccatcttcttacaagcagggaagtaacggcagagctgactactggaaggtggtgctggtggtgcaactggttttggagacagtactggaattcttctactcacatgagtgaagggacaatctggtttagtacactttgcatcatatttacaatttgggtgaacaaacaaacatttttcagcaaatttacaattggggaaggctttgcagggtgagatggggtgatggtaggcacactcatccccatttttacaagcaggccagtacttgcagcgctccaaaagtttttctggtttctgtgccacactcagttcactcatctcagcttgactcatctgcagagtttctgccattactgggtcgatttgcagtcgggataataattgcctctgttgagttccttgatttttttctacagaatctccttttgtttcctcttctttaatggggggacttattctgggggtcctactttgtccctggaccacttctgctagcaattcttcttgagaagttcgagttctgggagcaactggaagtgtctgtttctgtggaactgtagagtagttagttgtttttgttacggattcttgagcttcagatatagccttcaaaatcagattcttgttagcttgtttagaaggtggaagagaaggtctcctttcaggctttgcaggcacagacacactgctggagatgcttcctgttcgagacccgtaatcatcatcttcttcctcctcttctccatcatgattgaatttttttactttaacaactgaacttaccacaggcaactttctcttccgaaagttttcatcctccatactcattttctccgagttgtttctaaagaacggactatacgtttcttctaagctgttaagcacctctggttcacacaaacgtcctgtttcatatacccaactactctgcatatcaagctgcttggcagcatgaatactattctgctgctgttgaaattgcaacctgtttaaatgaacaccactatctgcatttctacttgcaggtggtcgataaatttcaatagaagggcgagaagaaccatatgtaagtgtcactgtaggttttttctgagataagggattctcctgcacaaagttgaggtcttcgtcaatgagatcatctggttctggcttaatatcaatcacatcttcagagggtgctggctccctcaaaggtttcactgttgacattagtcgggttgcagctccatcatcgtaagtctgtctgacatttgtggtttttgactcctgcgaacttgtagaaactctggaatctcttttttcaggtctcgcgctaggaatggcaagtggtggcactgcagcttcatgcctcctctcatctccccgactgaaattgctcttgtttgaaggcacgttactatcaaagatgttggtatcagaagacttcagactagagggttcagttgtaacagagcgaagtttatctaatacaccatgaagccaacataagctcctaattcttgtaatttccccttaatggcactccggatcttgcggctgatctcggtgccgatctccatggctctgcggcgtgcgggaactcagcactgcgcggcgcttggcttacccggaggctgccgcggactcctaccccgcagccgggacaccaccgcctcc

SEQ ID NO: 17469 - RNA, 12796 nt, Homo sapiens
  source 1..12796: mol_type = other RNA
tcaggccaggcacagtggctcatacctggaatcccagcactttgggaggccgaggcaggcagatcacctgaggtcaaggtatttgagaccagcctggccaacatggtgaaaccccatctctactaaaaatacagaaattagctgggtgtggtggtgcacacctgtaatgctagctactcgggaggctgaggtaggagaatcgcttgaacctgggaggcagaggttgcaataagcctagatcatgccactgcactcaagcctgggagacagagcgagactacatcttaaaaaaaaaaaaaaaagtattatgagagaggataatgtattgtaatgtattgtagaggctaaataaaattatgctcatgtcagaaaaaaagagtatttctcaaaataaaattcactgaaactggatgtttattttgactgagatatagtatatcctcaaattgccatagaaagtttacaagaatattagaggtaaattataaatatcagggcctttttaaaaaaaaaagattctgcttataacttggtatttgtttataataaaaattatagtagccaataatgaacacttactctggcttggttatttacttaggtcaaaagaaggaggagcggttaaactgtgggatcaggaactgaggcggtgccgtgccttcaggcttgagacaggacaagccacagattgtgttcgttctgtgtgcagaggcaaagtaagatgttccatgagctgatacagtgcagcagaaaacagaaagtggttattactgtgattccctcaccctttgcagcctaatgaacaatacttaataatgcataacgatggatttgcttgccaacattactctgtctttgctgctttctttgccaaagttagcaccagtgtggtgcataagctaggaagctattctgtctaaatactgtatgtaaacctccaatattttctagaatctgccaatttaacaactctagtagacataattgaaagcccttggcagttgactcatattaggacagctgtctccattttttaaaaaaacacacattccctagataaaacgtgcagtaaacaaacaatgaaatactactcagccataaaaaataatgaaattctgtcattcttggtggcaacatggatgagactggaggacatgatgtgaagtgaaataagccaggcacagaaagataaatacatgttctcactcctgtgcagaaactaaaaaagttgatcccacagaggtggagagtagaatagtggttactggaggcggacaagggggagggggagggggatagggaaggactggttaaaggatacaagtttacacagccagataggaatagtatgttttagtattctgtagtactgtaggatgactatagttaagaatcacgtatttatgtattttcaggtatttacaagagaggattttgaaagtttccatcacaaagaaatgataaatgtctgaggtgatggttatgcgtattaccctatgccctatagatatgtataattatgtgtcaatttcaaaataaaaattcaaaactacaactcctatgaaaatttttgagcgtgtttgtacttattaagtgtatttataaatcatacggatattatcttcagcctgcatattaaattgtagttaagcttttactttttaactaaaaaataaattctattattttttcctatatcccactgcactgaccccagtttggaaatcctaagattatcaaataaaaactttgattattgaagaatccaggtgtactgccacagaaaagttctattctgtagcatggactctaatatgtaatctagcccattgtgcttacagatagatgtgtgcctgtagtcatagaaaaatttgcatgagctaatgactgccttgctactagattagctcaaagcaaaaagttctctgaaagcaggtcaatagggtcatttttatattatgaagaagaaaagcagctgttgtattacattcactgtattggtcctgcttgtgtttcagggcaagatccttgttgggacaaggaatgctgaaataatcgaagttggagagaaaaatgcagcttgtaatattttagttaacggtcatgtggatgggccaatctggggactagcaacacatccttccagggattttttcctttctgctgcagaagatgggacagtgagactttgggatattgctgataaagtaagtacagataatttttttaaaagaggttacaacttctaaaaagaaaagttggaagttctaaattgctagtacttaaagaactgccagaattctgttgagcattttgaggggaaactggtataatttagaagtacttcacttaatgtttcctatgactctttttttttttttttttaaatgcagaagatgttaaacaaagtgaatttgggacatgctgctcgtactgtgtgttacagccctgaaggggacatggtggctattggaatgaaaaatggagaatttatcattttactagtgagttctctaaaaatatggggaaagaagagagacaggagatgtgcaatccatgatatcaggttagtgaacaaatggaatagagtttctagtatatacttgatttaacttccatttgtaaaattttccatagccttgccttcaaaaagaggtccccagggcctgtagcatttcccgtattataaattgtatgctaaaatatggctgtttgtatactacttaattcttcttgctaaattataaacccactgggcaccaactataatagcaagtactagtaggtaatgtttgatgaattcatgttaacacttagccatgtccattaagttcatcccaccaagaggtatctcccactgtaatacaagagagctatctgcccttcaaaagttgtcaccctggaaaactaaagttgtgatttcaaacatatcttctcttagtaacctcagtttgggaatatgtagttcattaatttaatcaatacctattgattaaatgttccagaatccaaattaatttaaatgtttcttaaacctttgtttttcagtgcttaagcatttttcaacagtggctaccatttacggagtacttccgtgtgatcagtagataagattattgaatctaggtctgtcaaaagcttgtacacttttcatcagtaaaatccttttacaaatgaaaccttcctcagaacttcaatatataaaatagtaacagtggcttcccttagcttttacatgtctctatcgtacctcagtaagactcatgggccatttcaagagactgaattgtcccatatgactccaaagattgctaggcaaatagcatttcactttgtcttttaaataagttcttcaggccgggcgcggtggctcatgcctgtaatcccagcactttgggaggccgaggcaggcagatcacctgaagtcaggagtactcgaccagcctggccaacatagtgaaaccccatctcaactaaaaatacaaaaatcagccgggcgtggtggcaggcgcctgtaatcccagctactcagggggctgaaacaggagaatcgcttgaacccgggaggcggaggttgcgccatcgcactccagcctgggagacaagagcgagacttcgtctcaaaaaaaaaaaattcttcttccaagattcaagttgtgtcatttcaccttaataactggaggttagttaagctgggctgtgttctttgcttaatattaagacaacgttttttccagatggaagaaaactatcttaatgaattgttagcttattaattatgtaatgctaatggcttttaaaagctgagatgttctgactgggtgttgtggctcacacctgtaatcccagtaccttgggaggccaagggggaaggattgcttgaggccaggagtttgggaccatagtgagaccccgcctctatttaaaaaattaaattttgttttgttttgttttgagttggagttttgctcttgttgcccatgctgaagtgcaatggtgcaatctcagctcaccacaacctgtgcctcctgggttcaagcgattctcctgcttcagcctcccgagtagatgggattacaggcgtgcaccaccatgcctggctaattttgtatttttagtagagacagggtttctctatgttggtcaggctggtctcaaactctcgacctcaggtgatctgcccgcctccgcttcccaaagttctgggattataggtgtgagccactgggcctggcctaagaaagtttttttaagccattagacgtttttaaaggaattgggagatgacaattggggaaatatttaaaatttaagtaaaatataaagcttccttatttcatgtaacccagacaatctcagtatacatgatcagttgtgtctgacaggtaaatctatttgaggccttatcacacgttacttttaagaactagaaaggaaaagtcactgatcttaagtatttataatacttcatgtggtctaatactttttacgttttgttttgattcagatttagtccggattcccggtatctggcagtaggttctagtgagaactcagtggatttttatgacctaacgctgggccccactcttaacagaatcagctactgcaaagacattccaagctttgtcattcaaatggacttctctgcagatagcagttatctccaggtacagtaccaatactgtatacccaggtggcaagttcttctgcttttacatttcgtgttagtgaatgcatttaaagttcctgagctccagagctccagcttctcaactcctccctttgtaccttctgacctacagctcccctttcctcccccacttatcagagcttttctcctattaagtttttgtagtgatcttttgcatacttaataatgttagacatgtaaatcaagtagcaatatgctagtattctgtaaaccccctgtggattttgtctctcacctaatggaattcttgtcccattttaatctgatgaaaaaggtctctagtggctgctataaacggcatgtctatgaagtgccttcaggaaaacatcttatggatcatgccgctattgacagaattacttgggctacatggactaggtaaatacttatatattcacaaggcaagaactgactttgaaggccagttagaaaatcctatttctgaactgttagagccattccaataaggaatagtaattgagtttcaagtttttgttaccatattttgaaatggtatgttcatgttgggacccctttttattgaatatatttccatgttttatcagtttccatgatttatcaagttttttttttaaggaaatcaaagttttaactttaaagataccctgatatttttcttaatgctaaatttaatgactggcaaaaaggtattgggtgctgttaagcaactgttattaattctctatctaaaggaatgctatcttgaatctattagaagtcaaagcttccaaatttgttcaaatttcctggctgtatgacaggtaaccatgactatccatttttttggccaatgaaaaatgccatcaaattcctgtatcagccaggcatatagtggctcatgcctgtaatctctgatgtagcaggccgaggtgggaggatcacttgagcctagaagttttgataccagcctgggcaacatagcaagaccccatctctgaaatttttttaattcctatgtcataagtcatttttatttttgtagagatagggatctcacaatattgcccaggctggtctcaaactcttggcctcaagcagtcctcctgcctcagcctcccaaaatgttgggattactggtatgtgctgctggacccagccaagtagcacttttaatttgaaaaatagttctatcagttttcagtcaggcgcggtggctcagcctgtaatcccagcactttgggaggccgagcgggggtgatcacctgaggtcgggagttcgagactagcctgaccaacatggagaaaccctgtctctactaaaaatacaaaataagccgggcatgttagcgcatgcctgtgatcccagctactcgggaggctgaggcaggagaattgcttgaacccaggaggcagaggttgcggtgagccgagatcatgccattgcactccagcctgggtaacaagagcgaaaactccgtctcaaaaaaaaaaaaagaaaaaatagttctatcagttttcataaagtactactttaatcttaaaaagattaatctagaaacccttcaaattataaaatgtcatttttaaaaggcaggagttgatatcctgatgaaattcaggtctccaaacaacttaccataatttacttcctgtattttaagtaacatgatagggtacttagagattaattgccaagaaactttttgaatatagtcaacctgcccgcacttgccatgatgagttttcttttgttccttccctctagtattctaggagatgaggttttgggaatctggtccagacatgctgagaaagctgatgtcaactgtgcctgtgtatctcattcaggaatcagtcttgttacaggagatgactttggcatggttaagttatttgacttcccatgtccagaaaaatttgtaagtttgtgttttgtttactattatcagtttactcctaattttgatgtcttatcatcagcacttttccccatatatttaaaatgttttgtcctaatttctaaatttttccccaaactttctaaatctatttactttgaaataaaagctattagaaacaaatcctctccctcgagtaataccatctttggaaccatcctacaaaagctgtaattagcttttcaccaaacctataatcagttatcaaatttcaaatgcttttccttagagaaaaatggtcagagtacctggagacatctgactgcccacacagcctggttttgcagatccactactcatgctgaaaagcattctaatcactggctgcggtgctaactccctactctctccacagctcttgtcatagagattatagttcctaataagagcctttgacttctgtgtgcaccaaatgccctgagcttgtctgtcattgttttttaggcaaaacacaaaaggttcttgggtcattcgccccatgtgacaaatattcgatttaccagtggtgatcgacatgttgttagtgctggaggtgatgactgcaggttagtaactttctcagcccatgaagagcagactatgttactagttaagagacttaatacaacaactcctacagctttggtttatgaaatcagctagtcaacattagtagaaggtagtataaccagatggctcttcagaatctcatatttatgcaaatacagaataaaaggagttaaagaggaaaaatattacacatgtaacctgaaagcacaactgaaaaatattaaactgttatgaaaatctaaaaacataattaactccctgcaattttcttctctgattgcagcttatttgtctggaaatgtgtacatacacctcactgagagatgctgagatgactacagaaattaactttgagaccagaattacagagaagaaaaaccaaaacccaaccctgcatggtcaagtggtgctaacccaagactgtaacagggagaaatgcccagaatcatcaaaatagtgaaagactgatctgttcaaaatatttgctatatgcactgggtataatccgtaatccatacactgccagataatgccatttcaaggaaggatcgaatacttgatggtaaaggccaagtccccctgtattgggaagtgtgtgatttcggcagacctgctgggaaaatttagggtagagcactctttacagaagaactcaaaaacccaatttggataattttcattatctttttagcaaaatggtttcttaatgtttatattttattttcaaggttcattgtttaatgaaatattttattcttgcatttccataaggaaagggaaagtcatgatcatcctaaaggatcacagtttttaaaaggcaaacattttccctaaggaaacagacacaagctttcctagagaatatgatgttttttaggcattaataaggtccttttttataaaggacacttttctcctagtagttttgaattcaggaacagatccaaagttagcagtatatggctgctacatttccattttcattttcgagccatcagtttatgttcagatgccatctctgtaatcgcacatttaaaacataactgtagcctcactaatggaaaagtagtatgatgaacaatcattcccaatggtgtacaatgtaagggttttagggagcaacagtatttaactggaagaaagaattgcatatttaatgtagtctaatatatacacatttgtttaacatgtaaacaaaagtgttaaattcacatatacaacattatacaatttaatcactcttggaataaaatttttatagccttttttctattgggaaaatttgtttagatgtgtgccactccataggtttatttccaaaatgaatgagcccaactccatttgtaaaaacttgtcagttagaattcctttttttagtggattagggctgaattcttagatccttatttcttttcactttaaatgctgccaaagatcactactcatcattcaggaattcgctgtctagcctatctgtagtttcctgaagattgaaaattatgtagactgctatttaaaaatatatttttctaagtgtgaggtttaagatgctgtattgaccctatgagtttttaatgtgttaattatctttatagcataatagatcgctttaggttcctggaatcccatttggtctgacaggatatatgaagattcttaatacctattttctgtgtctaatacttggttaatactaaaaatagaaatgactaaattacatcacagaaagcataaccagtgattgaacctggtagttttaaagctctaaatagctgtggctgaaggactgattatggggctaagaagcttgaaacgtaagttggtacttgttcatcagtggattctcctaaattaagccaaattttgaaatacatgactattaagtttctactcatgtatttacagtcagtcaataaattaaaggaggaaaaaaatccctgaacaacctgcccataaaaagaaaaatactctacatttgagcctgctgcagttttaaattttccctctgggtcaagtttgccagcttttggctacagagaaattatatttccattacagtgcaggtagaaactctgtaaccttaagcatgtaaactacatagaataaaactgtttccactgcatttctgtccttcaaagtggccaacctgattaagtcagccttaatcactgctgctgtcagtttcacgactaaaggtcatattgactaagtagtcatcagctgaccacctcgctgtatcagccagcaacgaggggaaggtgaagaaacatgataggccatatagaatctgccctatgtttacttttttaacccagataattatttttgtgtgcagtatctaagctcctgattgtgtaacctgggacttctggcaccttttgttccattcattttatgtataaaatgcatgccaaagcacactgtgccctctggtacccttgcttccaatcgccaaccatgctcatttccttcctttttttgtggtccctttttgtggtgatcattttaaaccacgtcatccaacaaatgttttatggtcaaccttagcttgttcataagccatagcaactgaaagattaaactcttaaatatgtgtctgggcagtggctattaaatagcaaaaaacaatcagattttagtattttattatttccttgtaaaatggctgaactaaattaaacccttgtttcccatttgttctataatttatagtgaaactgagaacaaaactatctttataaatgatagctaaaagtatttccagatatttaaacaatttaaaataaatttcttctgcagagatgcaaagcatctcaacactggaatgaacaaatgccttaaattcaatggagtaaacctttagaatgaagaggaactgtcatttcacccaagccgaagacaacagccttatgcacttgtgtgctctgtctttgctgcttctcgtgtttcaagcctttcctgtgggatcagcacagcaaagtgcaacttaccaaatggtttaatgactggttaattctttcttctcccaatggaaaagcaatggcaacacaacagtagactgctggcttgacaatcttaaacgtgagcctttgcacatgtaggtttatcatcatttgagtatacgactaagcaagtcaatgaactttttttttttttttagcagtttaatttggtcctgagaatgttgcagtctttattaccccttttgcattaatccacttttctaaccaccttttaagctttaatttttaacactatacaccaagtctttgaaatcagtgatctgttatttaactctaaagcatttgacacttcttgccttaacagttttaaaaaccacacacaaaaaaactctgtaagtaatacagtaggccaaaagtttcatcctatctatcttgcagtttacctatctgatctgatctctgtaattatagttctgtcatttaaaatatactatttaaatctaatttttacatttcaaaaattatcttcagtagtaactaagtatattttctgtggattctgagaatgttatttttcagaatgtgagaatatatatgtacatttataatcttgtgactttaaagtctgttttcagatacagtatgtaaatacttgtaaaaaaatttgtataattttgtgataatgtagtttcccaaaaaaattatttagaaggcattatgttattagtaaatgagagcactgtatagaactgttcctattttctgcacttgccattccagctgcctccactgtccatacccacctcattcatcctgtcacagaaggcaggaaaactgggaactttaccaaagtagcactcagcctgagaggcctgtataatcatgcttttcaaactaaattcacttaaaaattaaaaagcagaattgaatattttaagcagcctcagtacctttggccaatgctgttttcatggtggattatgaacattatataatctttgggaaaagtgaaagtagtacaatttttagaataatgacaactgcctcactgcatctctccactcacacagcaaccgtgtagccccctaagctgcagtaccatgactaaccatgatgtcaatttcatatgctgatcctcacaacagcagtgcacaaacatgccccaaatattttaacagaatttagctcttccttaagctgtcttttcatagtaaaaacaaaacaaaaacacccaatgttaaaaccacataataaacttacaaacttgaaaaattagacacttcagatagataggcaataaaacttcatattatgaaagcaatatattccaagtttcaaagatttgacaagttctgtagagtatctttcatcagtacatgaaaacttccaaactgcatgatcttctgccaggcaggactgggtgctattcgctggtttgaggtcgaatccatttcaaggcatgtcgtggtgggacattaatggtgggatggtagaatgtgcagtccggtcttgtacattgagtgttaaacctacaatgttttggatgatagaagggacattccatcttcttacaagcagggaagtaacggcagagctgactactggaaggtggtgctggtggtgcaactggttttggagacagtactggaattcttctactcacatgagtgaagggacaatctggtttagtacactttgcatcatatttacaatttgggtgaacaaacaaacatttttcagcaaatttacaattggggaaggctttgcagggtgagatggggtgatggtaggcacactcatccccatttttacaagcaggccagtacttgcagcgctccaaaagtttttctggtttctgtgccacactcagttcactcatctcagcttgactcatctgcagagtttctgccattactgggtcgatttgcagtcgggataataattgcctctgttgagttcctttctcaacgtttctaaggaagccgattatttttacatcagtagttcttgactgtgattcagtatcttcttcttgatcttcaaactgtctgttgcattcatatgttgttgaatattcattcattttaacctccaaagatgaaatttttgcttcattcttggacactctaacatttagatcaaaaagatttgcttccactgtcaaaatagctgctttcattcctttaatttcattgatatcagctgatattttccttaaaaggtgggaaatattgtctagctcattcagtgaacaagaggagcttgttatggaacctaagtccactggctccggtggaagaaaaattggtagaggtggtgatggaaactttgaagacattctcataaaggtgacaggaacctcaaagacattttcataaaattctctcccttaaaatctgataattttttcttcacagctcattaagttatttcatcgaaagtaaaagcagtgatcaaggctgttaccttaagacgtattaagagcaaataacatcttaaaacctgtaattcaaaagatggggttgtacatttctagagtcagaattcaaaactaaatgtgaaaaagctaaacgtaccagaccaattgctcttcgctacaactaagaagccctaatacgtagggccctacatcctctaagtaccatctgtat

SEQ ID NO: 17470 - RNA, 13290 nt, Homo sapiens
  source 1..13290: mol_type = other RNA
tcaggccaggcacagtggctcatacctggaatcccagcactttgggaggccgaggcaggcagatcacctgaggtcaaggtatttgagaccagcctggccaacatggtgaaaccccatctctactaaaaatacagaaattagctgggtgtggtggtgcacacctgtaatgctagctactcgggaggctgaggtaggagaatcgcttgaacctgggaggcagaggttgcaataagcctagatcatgccactgcactcaagcctgggagacagagcgagactacatcttaaaaaaaaaaaaaaaagtattatgagagaggataatgtattgtaatgtattgtagaggctaaataaaattatgctcatgtcagaaaaaaagagtatttctcaaaataaaattcactgaaactggatgtttattttgactgagatatagtatatcctcaaattgccatagaaagtttacaagaatattagaggtaaattataaatatcagggcctttttaaaaaaaaaagattctgcttataacttggtatttgtttataataaaaattatagtagccaataatgaacacttactctggcttggttatttacttaggtcaaaagaaggaggagcggttaaactgtgggatcaggaactgaggcggtgccgtgccttcaggcttgagacaggacaagccacagattgtgttcgttctgtgtgcagaggcaaagtaagatgttccatgagctgatacagtgcagcagaaaacagaaagtggttattactgtgattccctcaccctttgcagcctaatgaacaatacttaataatgcataacgatggatttgcttgccaacattactctgtctttgctgctttctttgccaaagttagcaccagtgtggtgcataagctaggaagctattctgtctaaatactgtatgtaaacctccaatattttctagaatctgccaatttaacaactctagtagacataattgaaagcccttggcagttgactcatattaggacagctgtctccattttttaaaaaaacacacattccctagataaaacgtgcagtaaacaaacaatgaaatactactcagccataaaaaataatgaaattctgtcattcttggtggcaacatggatgagactggaggacatgatgtgaagtgaaataagccaggcacagaaagataaatacatgttctcactcctgtgcagaaactaaaaaagttgatcccacagaggtggagagtagaatagtggttactggaggcggacaagggggagggggagggggatagggaaggactggttaaaggatacaagtttacacagccagataggaatagtatgttttagtattctgtagtactgtaggatgactatagttaagaatcacgtatttatgtattttcaggtatttacaagagaggattttgaaagtttccatcacaaagaaatgataaatgtctgaggtgatggttatgcgtattaccctatgccctatagatatgtataattatgtgtcaatttcaaaataaaaattcaaaactacaactcctatgaaaatttttgagcgtgtttgtacttattaagtgtatttataaatcatacggatattatcttcagcctgcatattaaattgtagttaagcttttactttttaactaaaaaataaattctattattttttcctatatcccactgcactgaccccagtttggaaatcctaagattatcaaataaaaactttgattattgaagaatccaggtgtactgccacagaaaagttctattctgtagcatggactctaatatgtaatctagcccattgtgcttacagatagatgtgtgcctgtagtcatagaaaaatttgcatgagctaatgactgccttgctactagattagctcaaagcaaaaagttctctgaaagcaggtcaatagggtcatttttatattatgaagaagaaaagcagctgttgtattacattcactgtattggtcctgcttgtgtttcagggcaagatccttgttgggacaaggaatgctgaaataatcgaagttggagagaaaaatgcagcttgtaatattttagttaacggtcatgtggatgggccaatctggggactagcaacacatccttccagggattttttcctttctgctgcagaagatgggacagtgagactttgggatattgctgataaagtaagtacagataatttttttaaaagaggttacaacttctaaaaagaaaagttggaagttctaaattgctagtacttaaagaactgccagaattctgttgagcattttgaggggaaactggtataatttagaagtacttcacttaatgtttcctatgactctttttttttttttttttaaatgcagaagatgttaaacaaagtgaatttgggacatgctgctcgtactgtgtgttacagccctgaaggggacatggtggctattggaatgaaaaatggagaatttatcattttactagtgagttctctaaaaatatggggaaagaagagagacaggagatgtgcaatccatgatatcaggttagtgaacaaatggaatagagtttctagtatatacttgatttaacttccatttgtaaaattttccatagccttgccttcaaaaagaggtccccagggcctgtagcatttcccgtattataaattgtatgctaaaatatggctgtttgtatactacttaattcttcttgctaaattataaacccactgggcaccaactataatagcaagtactagtaggtaatgtttgatgaattcatgttaacacttagccatgtccattaagttcatcccaccaagaggtatctcccactgtaatacaagagagctatctgcccttcaaaagttgtcaccctggaaaactaaagttgtgatttcaaacatatcttctcttagtaacctcagtttgggaatatgtagttcattaatttaatcaatacctattgattaaatgttccagaatccaaattaatttaaatgtttcttaaacctttgtttttcagtgcttaagcatttttcaacagtggctaccatttacggagtacttccgtgtgatcagtagataagattattgaatctaggtctgtcaaaagcttgtacacttttcatcagtaaaatccttttacaaatgaaaccttcctcagaacttcaatatataaaatagtaacagtggcttcccttagcttttacatgtctctatcgtacctcagtaagactcatgggccatttcaagagactgaattgtcccatatgactccaaagattgctaggcaaatagcatttcactttgtcttttaaataagttcttcaggccgggcgcggtggctcatgcctgtaatcccagcactttgggaggccgaggcaggcagatcacctgaagtcaggagtactcgaccagcctggccaacatagtgaaaccccatctcaactaaaaatacaaaaatcagccgggcgtggtggcaggcgcctgtaatcccagctactcagggggctgaaacaggagaatcgcttgaacccgggaggcggaggttgcgccatcgcactccagcctgggagacaagagcgagacttcgtctcaaaaaaaaaaaattcttcttccaagattcaagttgtgtcatttcaccttaataactggaggttagttaagctgggctgtgttctttgcttaatattaagacaacgttttttccagatggaagaaaactatcttaatgaattgttagcttattaattatgtaatgctaatggcttttaaaagctgagatgttctgactgggtgttgtggctcacacctgtaatcccagtaccttgggaggccaagggggaaggattgcttgaggccaggagtttgggaccatagtgagaccccgcctctatttaaaaaattaaattttgttttgttttgttttgagttggagttttgctcttgttgcccatgctgaagtgcaatggtgcaatctcagctcaccacaacctgtgcctcctgggttcaagcgattctcctgcttcagcctcccgagtagatgggattacaggcgtgcaccaccatgcctggctaattttgtatttttagtagagacagggtttctctatgttggtcaggctggtctcaaactctcgacctcaggtgatctgcccgcctccgcttcccaaagttctgggattataggtgtgagccactgggcctggcctaagaaagtttttttaagccattagacgtttttaaaggaattgggagatgacaattggggaaatatttaaaatttaagtaaaatataaagcttccttatttcatgtaacccagacaatctcagtatacatgatcagttgtgtctgacaggtaaatctatttgaggccttatcacacgttacttttaagaactagaaaggaaaagtcactgatcttaagtatttataatacttcatgtggtctaatactttttacgttttgttttgattcagatttagtccggattcccggtatctggcagtaggttctagtgagaactcagtggatttttatgacctaacgctgggccccactcttaacagaatcagctactgcaaagacattccaagctttgtcattcaaatggacttctctgcagatagcagttatctccaggtacagtaccaatactgtatacccaggtggcaagttcttctgcttttacatttcgtgttagtgaatgcatttaaagttcctgagctccagagctccagcttctcaactcctccctttgtaccttctgacctacagctcccctttcctcccccacttatcagagcttttctcctattaagtttttgtagtgatcttttgcatacttaataatgttagacatgtaaatcaagtagcaatatgctagtattctgtaaaccccctgtggattttgtctctcacctaatggaattcttgtcccattttaatctgatgaaaaaggtctctagtggctgctataaacggcatgtctatgaagtgccttcaggaaaacatcttatggatcatgccgctattgacagaattacttgggctacatggactaggtaaatacttatatattcacaaggcaagaactgactttgaaggccagttagaaaatcctatttctgaactgttagagccattccaataaggaatagtaattgagtttcaagtttttgttaccatattttgaaatggtatgttcatgttgggacccctttttattgaatatatttccatgttttatcagtttccatgatttatcaagttttttttttaaggaaatcaaagttttaactttaaagataccctgatatttttcttaatgctaaatttaatgactggcaaaaaggtattgggtgctgttaagcaactgttattaattctctatctaaaggaatgctatcttgaatctattagaagtcaaagcttccaaatttgttcaaatttcctggctgtatgacaggtaaccatgactatccatttttttggccaatgaaaaatgccatcaaattcctgtatcagccaggcatatagtggctcatgcctgtaatctctgatgtagcaggccgaggtgggaggatcacttgagcctagaagttttgataccagcctgggcaacatagcaagaccccatctctgaaatttttttaattcctatgtcataagtcatttttatttttgtagagatagggatctcacaatattgcccaggctggtctcaaactcttggcctcaagcagtcctcctgcctcagcctcccaaaatgttgggattactggtatgtgctgctggacccagccaagtagcacttttaatttgaaaaatagttctatcagttttcagtcaggcgcggtggctcagcctgtaatcccagcactttgggaggccgagcgggggtgatcacctgaggtcgggagttcgagactagcctgaccaacatggagaaaccctgtctctactaaaaatacaaaataagccgggcatgttagcgcatgcctgtgatcccagctactcgggaggctgaggcaggagaattgcttgaacccaggaggcagaggttgcggtgagccgagatcatgccattgcactccagcctgggtaacaagagcgaaaactccgtctcaaaaaaaaaaaaagaaaaaatagttctatcagttttcataaagtactactttaatcttaaaaagattaatctagaaacccttcaaattataaaatgtcatttttaaaaggcaggagttgatatcctgatgaaattcaggtctccaaacaacttaccataatttacttcctgtattttaagtaacatgatagggtacttagagattaattgccaagaaactttttgaatatagtcaacctgcccgcacttgccatgatgagttttcttttgttccttccctctagtattctaggagatgaggttttgggaatctggtccagacatgctgagaaagctgatgtcaactgtgcctgtgtatctcattcaggaatcagtcttgttacaggagatgactttggcatggttaagttatttgacttcccatgtccagaaaaatttgtaagtttgtgttttgtttactattatcagtttactcctaattttgatgtcttatcatcagcacttttccccatatatttaaaatgttttgtcctaatttctaaatttttccccaaactttctaaatctatttactttgaaataaaagctattagaaacaaatcctctccctcgagtaataccatctttggaaccatcctacaaaagctgtaattagcttttcaccaaacctataatcagttatcaaatttcaaatgcttttccttagagaaaaatggtcagagtacctggagacatctgactgcccacacagcctggttttgcagatccactactcatgctgaaaagcattctaatcactggctgcggtgctaactccctactctctccacagctcttgtcatagagattatagttcctaataagagcctttgacttctgtgtgcaccaaatgccctgagcttgtctgtcattgttttttaggcaaaacacaaaaggttcttgggtcattcgccccatgtgacaaatattcgatttaccagtggtgatcgacatgttgttagtgctggaggtgatgactgcaggttagtaactttctcagcccatgaagagcagactatgttactagttaagagacttaatacaacaactcctacagctttggtttatgaaatcagctagtcaacattagtagaaggtagtataaccagatggctcttcagaatctcatatttatgcaaatacagaataaaaggagttaaagaggaaaaatattacacatgtaacctgaaagcacaactgaaaaatattaaactgttatgaaaatctaaaaacataattaactccctgcaattttcttctctgattgcagcttatttgtctggaaatgtgtacatacacctcactgagagatgctgagatgactacagaaattaactttgagaccagaattacagagaagaaaaaccaaaacccaaccctgcatggtcaagtggtgctaacccaagactgtaacagggagaaatgcccagaatcatcaaaatagtgaaagactgatctgttcaaaatatttgctatatgcactgggtataatccgtaatccatacactgccagataatgccatttcaaggaaggatcgaatacttgatggtaaaggccaagtccccctgtattgggaagtgtgtgatttcggcagacctgctgggaaaatttagggtagagcactctttacagaagaactcaaaaacccaatttggataattttcattatctttttagcaaaatggtttcttaatgtttatattttattttcaaggttcattgtttaatgaaatattttattcttgcatttccataaggaaagggaaagtcatgatcatcctaaaggatcacagtttttaaaaggcaaacattttccctaaggaaacagacacaagctttcctagagaatatgatgttttttaggcattaataaggtccttttttataaaggacacttttctcctagtagttttgaattcaggaacagatccaaagttagcagtatatggctgctacatttccattttcattttcgagccatcagtttatgttcagatgccatctctgtaatcgcacatttaaaacataactgtagcctcactaatggaaaagtagtatgatgaacaatcattcccaatggtgtacaatgtaagggttttagggagcaacagtatttaactggaagaaagaattgcatatttaatgtagtctaatatatacacatttgtttaacatgtaaacaaaagtgttaaattcacatatacaacattatacaatttaatcactcttggaataaaatttttatagccttttttctattgggaaaatttgtttagatgtgtgccactccataggtttatttccaaaatgaatgagcccaactccatttgtaaaaacttgtcagttagaattcctttttttagtggattagggctgaattcttagatccttatttcttttcactttaaatgctgccaaagatcactactcatcattcaggaattcgctgtctagcctatctgtagtttcctgaagattgaaaattatgtagactgctatttaaaaatatatttttctaagtgtgaggtttaagatgctgtattgaccctatgagtttttaatgtgttaattatctttatagcataatagatcgctttaggttcctggaatcccatttggtctgacaggatatatgaagattcttaatacctattttctgtgtctaatacttggttaatactaaaaatagaaatgactaaattacatcacagaaagcataaccagtgattgaacctggtagttttaaagctctaaatagctgtggctgaaggactgattatggggctaagaagcttgaaacgtaagttggtacttgttcatcagtggattctcctaaattaagccaaattttgaaatacatgactattaagtttctactcatgtatttacagtcagtcaataaattaaaggaggaaaaaaatccctgaacaacctgcccataaaaagaaaaatactctacatttgagcctgctgcagttttaaattttccctctgggtcaagtttgccagcttttggctacagagaaattatatttccattacagtgcaggtagaaactctgtaaccttaagcatgtaaactacatagaataaaactgtttccactgcatttctgtccttcaaagtggccaacctgattaagtcagccttaatcactgctgctgtcagtttcacgactaaaggtcatattgactaagtagtcatcagctgaccacctcgctgtatcagccagcaacgaggggaaggtgaagaaacatgataggccatatagaatctgccctatgtttacttttttaacccagataattatttttgtgtgcagtatctaagctcctgattgtgtaacctgggacttctggcaccttttgttccattcattttatgtataaaatgcatgccaaagcacactgtgccctctggtacccttgcttccaatcgccaaccatgctcatttccttcctttttttgtggtccctttttgtggtgatcattttaaaccacgtcatccaacaaatgttttatggtcaaccttagcttgttcataagccatagcaactgaaagattaaactcttaaatatgtgtctgggcagtggctattaaatagcaaaaaacaatcagattttagtattttattatttccttgtaaaatggctgaactaaattaaacccttgtttcccatttgttctataatttatagtgaaactgagaacaaaactatctttataaatgatagctaaaagtatttccagatatttaaacaatttaaaataaatttcttctgcagagatgcaaagcatctcaacactggaatgaacaaatgccttaaattcaatggagtaaacctttagaatgaagaggaactgtcatttcacccaagccgaagacaacagccttatgcacttgtgtgctctgtctttgctgcttctcgtgtttcaagcctttcctgtgggatcagcacagcaaagtgcaacttaccaaatggtttaatgactggttaattctttcttctcccaatggaaaagcaatggcaacacaacagtagactgctggcttgacaatcttaaacgtgagcctttgcacatgtaggtttatcatcatttgagtatacgactaagcaagtcaatgaactttttttttttttttagcagtttaatttggtcctgagaatgttgcagtctttattaccccttttgcattaatccacttttctaaccaccttttaagctttaatttttaacactatacaccaagtctttgaaatcagtgatctgttatttaactctaaagcatttgacacttcttgccttaacagttttaaaaaccacacacaaaaaaactctgtaagtaatacagtaggccaaaagtttcatcctatctatcttgcagtttacctatctgatctgatctctgtaattatagttctgtcatttaaaatatactatttaaatctaatttttacatttcaaaaattatcttcagtagtaactaagtatattttctgtggattctgagaatgttatttttcagaatgtgagaatatatatgtacatttataatcttgtgactttaaagtctgttttcagatacagtatgtaaatacttgtaaaaaaatttgtataattttgtgataatgtagtttcccaaaaaaattatttagaaggcattatgttattagtaaatgagagcactgtatagaactgttcctattttctgcacttgccattccagctgcctccactgtccatacccacctcattcatcctgtcacagaaggcaggaaaactgggaactttaccaaagtagcactcagcctgagaggcctgtataatcatgcttttcaaactaaattcacttaaaaattaaaaagcagaattgaatattttaagcagcctcagtacctttggccaatgctgttttcatggtggattatgaacattatataatctttgggaaaagtgaaagtagtacaatttttagaataatgacaactgcctcactgcatctctccactcacacagcaaccgtgtagccccctaagctgcagtaccatgactaaccatgatgtcaatttcatatgctgatcctcacaacagcagtgcacaaacatgccccaaatattttaacagaatttagctcttccttaagctgtcttttcatagtaaaaacaaaacaaaaacacccaatgttaaaaccacataataaacttacaaacttgaaaaattagacacttcagatagataggcaataaaacttcatattatgaaagcaatatattccaagtttcaaagatttgacaagttctgtagagtatctttcatcagtacatgaaaacttccaaactgcatgatcttctgccaggcaggactgggtgctattcgctggtttgaggtcgaatccatttcaaggcatgtcgtggtgggacattaatggtgggatggtagaatgtgcagtccggtcttgtacattgagtgttaaacctacaatgttttggatgatagaagggacattccatcttcttacaagcagggaagtaacggcagagctgactactggaaggtggtgctggtggtgcaactggttttggagacagtactggaattcttctactcacatgagtgaagggacaatctggtttagtacactttgcatcatatttacaatttgggtgaacaaacaaacatttttcagcaaatttacaattggggaaggctttgcagggtgagatggggtgatggtaggcacactcatccccatttttacaagcaggccagtacttgcagcgctccaaaagtttttctggtttctgtgccacactcagttcactcatctcagcttgatttttttctacagaatctccttttgtttcctcttctttaatggggggacttattctgggggtcctactttgtccctggaccacttctgctagcaattcttcttgagaagttcgagttctgggagcaactggaagtgtctgtttctgtggaactgtagagtagttagttgtttttgttacggattcttgagcttcagatatagccttcaaaatcagattcttgttagcttgtttagaaggtggaagagaaggtctcctttcaggctttgcaggcacagacacactgctggagatgcttcctgttcgagacccgtaatcatcatcttcttcctcctcttctccatcatgattgaatttttttactttaacaactgaacttaccacaggcaactttctcttccgaaagttttcatcctccatactcattttctccgagttgtttctaaagaacggactatacgtttcttctaagctgttaagcacctctggttcacacaaacgtcctgtttcatatacccaactactctgcatatcaagctgcttggcagcatgaatactattctgctgctgttgaaattgcaacctgtttaaatgaacaccactatctgcatttctacttgcaggtggtcgataaatttcaatagaagggcgagaagaaccatatgtaagtgtcactgtaggttttttctgagataagggattctcctgcacaaagttgaggtcttcgtcaatgagatcatctggttctggcttaatatcaatcacatcttcagagggtgctggctccctcaaaggtttcactgttgacattagtcgggttgcagctccatcatcgtaagtctgtctgacatttgtggtttttgactcctgcgaacttgtagaaactctggaatctcttttttcaggtctcgcgctaggaatggcaagtggtggcactgcagcttcatgcctcctctcatctccccgactgaaattgctcttgtttgaaggcacgttactatcaaagatgttggtatcagaagacttcagactagagggttcagttgtaacagagcgaagtttatctaatacaccatgaagccaacataagctcctaattcttgtaatttccccttaatggcactccggatcttgcggctgatctcggtgccgatctccatggctctgcggcgtgcgggaactcagcactgcgcggcgcttggcttacccggaggctgccgcggactcctaccccgcagccgggacaccaccgcctcc

SEQ ID NO: 17471 - RNA, 13405 nt, Homo sapiens
  source 1..13405: mol_type = other RNA
tcaggccaggcacagtggctcatacctggaatcccagcactttgggaggccgaggcaggcagatcacctgaggtcaaggtatttgagaccagcctggccaacatggtgaaaccccatctctactaaaaatacagaaattagctgggtgtggtggtgcacacctgtaatgctagctactcgggaggctgaggtaggagaatcgcttgaacctgggaggcagaggttgcaataagcctagatcatgccactgcactcaagcctgggagacagagcgagactacatcttaaaaaaaaaaaaaaaagtattatgagagaggataatgtattgtaatgtattgtagaggctaaataaaattatgctcatgtcagaaaaaaagagtatttctcaaaataaaattcactgaaactggatgtttattttgactgagatatagtatatcctcaaattgccatagaaagtttacaagaatattagaggtaaattataaatatcagggcctttttaaaaaaaaaagattctgcttataacttggtatttgtttataataaaaattatagtagccaataatgaacacttactctggcttggttatttacttaggtcaaaagaaggaggagcggttaaactgtgggatcaggaactgaggcggtgccgtgccttcaggcttgagacaggacaagccacagattgtgttcgttctgtgtgcagaggcaaagtaagatgttccatgagctgatacagtgcagcagaaaacagaaagtggttattactgtgattccctcaccctttgcagcctaatgaacaatacttaataatgcataacgatggatttgcttgccaacattactctgtctttgctgctttctttgccaaagttagcaccagtgtggtgcataagctaggaagctattctgtctaaatactgtatgtaaacctccaatattttctagaatctgccaatttaacaactctagtagacataattgaaagcccttggcagttgactcatattaggacagctgtctccattttttaaaaaaacacacattccctagataaaacgtgcagtaaacaaacaatgaaatactactcagccataaaaaataatgaaattctgtcattcttggtggcaacatggatgagactggaggacatgatgtgaagtgaaataagccaggcacagaaagataaatacatgttctcactcctgtgcagaaactaaaaaagttgatcccacagaggtggagagtagaatagtggttactggaggcggacaagggggagggggagggggatagggaaggactggttaaaggatacaagtttacacagccagataggaatagtatgttttagtattctgtagtactgtaggatgactatagttaagaatcacgtatttatgtattttcaggtatttacaagagaggattttgaaagtttccatcacaaagaaatgataaatgtctgaggtgatggttatgcgtattaccctatgccctatagatatgtataattatgtgtcaatttcaaaataaaaattcaaaactacaactcctatgaaaatttttgagcgtgtttgtacttattaagtgtatttataaatcatacggatattatcttcagcctgcatattaaattgtagttaagcttttactttttaactaaaaaataaattctattattttttcctatatcccactgcactgaccccagtttggaaatcctaagattatcaaataaaaactttgattattgaagaatccaggtgtactgccacagaaaagttctattctgtagcatggactctaatatgtaatctagcccattgtgcttacagatagatgtgtgcctgtagtcatagaaaaatttgcatgagctaatgactgccttgctactagattagctcaaagcaaaaagttctctgaaagcaggtcaatagggtcatttttatattatgaagaagaaaagcagctgttgtattacattcactgtattggtcctgcttgtgtttcagggcaagatccttgttgggacaaggaatgctgaaataatcgaagttggagagaaaaatgcagcttgtaatattttagttaacggtcatgtggatgggccaatctggggactagcaacacatccttccagggattttttcctttctgctgcagaagatgggacagtgagactttgggatattgctgataaagtaagtacagataatttttttaaaagaggttacaacttctaaaaagaaaagttggaagttctaaattgctagtacttaaagaactgccagaattctgttgagcattttgaggggaaactggtataatttagaagtacttcacttaatgtttcctatgactctttttttttttttttttaaatgcagaagatgttaaacaaagtgaatttgggacatgctgctcgtactgtgtgttacagccctgaaggggacatggtggctattggaatgaaaaatggagaatttatcattttactagtgagttctctaaaaatatggggaaagaagagagacaggagatgtgcaatccatgatatcaggttagtgaacaaatggaatagagtttctagtatatacttgatttaacttccatttgtaaaattttccatagccttgccttcaaaaagaggtccccagggcctgtagcatttcccgtattataaattgtatgctaaaatatggctgtttgtatactacttaattcttcttgctaaattataaacccactgggcaccaactataatagcaagtactagtaggtaatgtttgatgaattcatgttaacacttagccatgtccattaagttcatcccaccaagaggtatctcccactgtaatacaagagagctatctgcccttcaaaagttgtcaccctggaaaactaaagttgtgatttcaaacatatcttctcttagtaacctcagtttgggaatatgtagttcattaatttaatcaatacctattgattaaatgttccagaatccaaattaatttaaatgtttcttaaacctttgtttttcagtgcttaagcatttttcaacagtggctaccatttacggagtacttccgtgtgatcagtagataagattattgaatctaggtctgtcaaaagcttgtacacttttcatcagtaaaatccttttacaaatgaaaccttcctcagaacttcaatatataaaatagtaacagtggcttcccttagcttttacatgtctctatcgtacctcagtaagactcatgggccatttcaagagactgaattgtcccatatgactccaaagattgctaggcaaatagcatttcactttgtcttttaaataagttcttcaggccgggcgcggtggctcatgcctgtaatcccagcactttgggaggccgaggcaggcagatcacctgaagtcaggagtactcgaccagcctggccaacatagtgaaaccccatctcaactaaaaatacaaaaatcagccgggcgtggtggcaggcgcctgtaatcccagctactcagggggctgaaacaggagaatcgcttgaacccgggaggcggaggttgcgccatcgcactccagcctgggagacaagagcgagacttcgtctcaaaaaaaaaaaattcttcttccaagattcaagttgtgtcatttcaccttaataactggaggttagttaagctgggctgtgttctttgcttaatattaagacaacgttttttccagatggaagaaaactatcttaatgaattgttagcttattaattatgtaatgctaatggcttttaaaagctgagatgttctgactgggtgttgtggctcacacctgtaatcccagtaccttgggaggccaagggggaaggattgcttgaggccaggagtttgggaccatagtgagaccccgcctctatttaaaaaattaaattttgttttgttttgttttgagttggagttttgctcttgttgcccatgctgaagtgcaatggtgcaatctcagctcaccacaacctgtgcctcctgggttcaagcgattctcctgcttcagcctcccgagtagatgggattacaggcgtgcaccaccatgcctggctaattttgtatttttagtagagacagggtttctctatgttggtcaggctggtctcaaactctcgacctcaggtgatctgcccgcctccgcttcccaaagttctgggattataggtgtgagccactgggcctggcctaagaaagtttttttaagccattagacgtttttaaaggaattgggagatgacaattggggaaatatttaaaatttaagtaaaatataaagcttccttatttcatgtaacccagacaatctcagtatacatgatcagttgtgtctgacaggtaaatctatttgaggccttatcacacgttacttttaagaactagaaaggaaaagtcactgatcttaagtatttataatacttcatgtggtctaatactttttacgttttgttttgattcagatttagtccggattcccggtatctggcagtaggttctagtgagaactcagtggatttttatgacctaacgctgggccccactcttaacagaatcagctactgcaaagacattccaagctttgtcattcaaatggacttctctgcagatagcagttatctccaggtacagtaccaatactgtatacccaggtggcaagttcttctgcttttacatttcgtgttagtgaatgcatttaaagttcctgagctccagagctccagcttctcaactcctccctttgtaccttctgacctacagctcccctttcctcccccacttatcagagcttttctcctattaagtttttgtagtgatcttttgcatacttaataatgttagacatgtaaatcaagtagcaatatgctagtattctgtaaaccccctgtggattttgtctctcacctaatggaattcttgtcccattttaatctgatgaaaaaggtctctagtggctgctataaacggcatgtctatgaagtgccttcaggaaaacatcttatggatcatgccgctattgacagaattacttgggctacatggactaggtaaatacttatatattcacaaggcaagaactgactttgaaggccagttagaaaatcctatttctgaactgttagagccattccaataaggaatagtaattgagtttcaagtttttgttaccatattttgaaatggtatgttcatgttgggacccctttttattgaatatatttccatgttttatcagtttccatgatttatcaagttttttttttaaggaaatcaaagttttaactttaaagataccctgatatttttcttaatgctaaatttaatgactggcaaaaaggtattgggtgctgttaagcaactgttattaattctctatctaaaggaatgctatcttgaatctattagaagtcaaagcttccaaatttgttcaaatttcctggctgtatgacaggtaaccatgactatccatttttttggccaatgaaaaatgccatcaaattcctgtatcagccaggcatatagtggctcatgcctgtaatctctgatgtagcaggccgaggtgggaggatcacttgagcctagaagttttgataccagcctgggcaacatagcaagaccccatctctgaaatttttttaattcctatgtcataagtcatttttatttttgtagagatagggatctcacaatattgcccaggctggtctcaaactcttggcctcaagcagtcctcctgcctcagcctcccaaaatgttgggattactggtatgtgctgctggacccagccaagtagcacttttaatttgaaaaatagttctatcagttttcagtcaggcgcggtggctcagcctgtaatcccagcactttgggaggccgagcgggggtgatcacctgaggtcgggagttcgagactagcctgaccaacatggagaaaccctgtctctactaaaaatacaaaataagccgggcatgttagcgcatgcctgtgatcccagctactcgggaggctgaggcaggagaattgcttgaacccaggaggcagaggttgcggtgagccgagatcatgccattgcactccagcctgggtaacaagagcgaaaactccgtctcaaaaaaaaaaaaagaaaaaatagttctatcagttttcataaagtactactttaatcttaaaaagattaatctagaaacccttcaaattataaaatgtcatttttaaaaggcaggagttgatatcctgatgaaattcaggtctccaaacaacttaccataatttacttcctgtattttaagtaacatgatagggtacttagagattaattgccaagaaactttttgaatatagtcaacctgcccgcacttgccatgatgagttttcttttgttccttccctctagtattctaggagatgaggttttgggaatctggtccagacatgctgagaaagctgatgtcaactgtgcctgtgtatctcattcaggaatcagtcttgttacaggagatgactttggcatggttaagttatttgacttcccatgtccagaaaaatttgtaagtttgtgttttgtttactattatcagtttactcctaattttgatgtcttatcatcagcacttttccccatatatttaaaatgttttgtcctaatttctaaatttttccccaaactttctaaatctatttactttgaaataaaagctattagaaacaaatcctctccctcgagtaataccatctttggaaccatcctacaaaagctgtaattagcttttcaccaaacctataatcagttatcaaatttcaaatgcttttccttagagaaaaatggtcagagtacctggagacatctgactgcccacacagcctggttttgcagatccactactcatgctgaaaagcattctaatcactggctgcggtgctaactccctactctctccacagctcttgtcatagagattatagttcctaataagagcctttgacttctgtgtgcaccaaatgccctgagcttgtctgtcattgttttttaggcaaaacacaaaaggttcttgggtcattcgccccatgtgacaaatattcgatttaccagtggtgatcgacatgttgttagtgctggaggtgatgactgcaggttagtaactttctcagcccatgaagagcagactatgttactagttaagagacttaatacaacaactcctacagctttggtttatgaaatcagctagtcaacattagtagaaggtagtataaccagatggctcttcagaatctcatatttatgcaaatacagaataaaaggagttaaagaggaaaaatattacacatgtaacctgaaagcacaactgaaaaatattaaactgttatgaaaatctaaaaacataattaactccctgcaattttcttctctgattgcagcttatttgtctggaaatgtgtacatacacctcactgagagatgctgagatgactacagaaattaactttgagaccagaattacagagaagaaaaaccaaaacccaaccctgcatggtcaagtggtgctaacccaagactgtaacagggagaaatgcccagaatcatcaaaatagtgaaagactgatctgttcaaaatatttgctatatgcactgggtataatccgtaatccatacactgccagataatgccatttcaaggaaggatcgaatacttgatggtaaaggccaagtccccctgtattgggaagtgtgtgatttcggcagacctgctgggaaaatttagggtagagcactctttacagaagaactcaaaaacccaatttggataattttcattatctttttagcaaaatggtttcttaatgtttatattttattttcaaggttcattgtttaatgaaatattttattcttgcatttccataaggaaagggaaagtcatgatcatcctaaaggatcacagtttttaaaaggcaaacattttccctaaggaaacagacacaagctttcctagagaatatgatgttttttaggcattaataaggtccttttttataaaggacacttttctcctagtagttttgaattcaggaacagatccaaagttagcagtatatggctgctacatttccattttcattttcgagccatcagtttatgttcagatgccatctctgtaatcgcacatttaaaacataactgtagcctcactaatggaaaagtagtatgatgaacaatcattcccaatggtgtacaatgtaagggttttagggagcaacagtatttaactggaagaaagaattgcatatttaatgtagtctaatatatacacatttgtttaacatgtaaacaaaagtgttaaattcacatatacaacattatacaatttaatcactcttggaataaaatttttatagccttttttctattgggaaaatttgtttagatgtgtgccactccataggtttatttccaaaatgaatgagcccaactccatttgtaaaaacttgtcagttagaattcctttttttagtggattagggctgaattcttagatccttatttcttttcactttaaatgctgccaaagatcactactcatcattcaggaattcgctgtctagcctatctgtagtttcctgaagattgaaaattatgtagactgctatttaaaaatatatttttctaagtgtgaggtttaagatgctgtattgaccctatgagtttttaatgtgttaattatctttatagcataatagatcgctttaggttcctggaatcccatttggtctgacaggatatatgaagattcttaatacctattttctgtgtctaatacttggttaatactaaaaatagaaatgactaaattacatcacagaaagcataaccagtgattgaacctggtagttttaaagctctaaatagctgtggctgaaggactgattatggggctaagaagcttgaaacgtaagttggtacttgttcatcagtggattctcctaaattaagccaaattttgaaatacatgactattaagtttctactcatgtatttacagtcagtcaataaattaaaggaggaaaaaaatccctgaacaacctgcccataaaaagaaaaatactctacatttgagcctgctgcagttttaaattttccctctgggtcaagtttgccagcttttggctacagagaaattatatttccattacagtgcaggtagaaactctgtaaccttaagcatgtaaactacatagaataaaactgtttccactgcatttctgtccttcaaagtggccaacctgattaagtcagccttaatcactgctgctgtcagtttcacgactaaaggtcatattgactaagtagtcatcagctgaccacctcgctgtatcagccagcaacgaggggaaggtgaagaaacatgataggccatatagaatctgccctatgtttacttttttaacccagataattatttttgtgtgcagtatctaagctcctgattgtgtaacctgggacttctggcaccttttgttccattcattttatgtataaaatgcatgccaaagcacactgtgccctctggtacccttgcttccaatcgccaaccatgctcatttccttcctttttttgtggtccctttttgtggtgatcattttaaaccacgtcatccaacaaatgttttatggtcaaccttagcttgttcataagccatagcaactgaaagattaaactcttaaatatgtgtctgggcagtggctattaaatagcaaaaaacaatcagattttagtattttattatttccttgtaaaatggctgaactaaattaaacccttgtttcccatttgttctataatttatagtgaaactgagaacaaaactatctttataaatgatagctaaaagtatttccagatatttaaacaatttaaaataaatttcttctgcagagatgcaaagcatctcaacactggaatgaacaaatgccttaaattcaatggagtaaacctttagaatgaagaggaactgtcatttcacccaagccgaagacaacagccttatgcacttgtgtgctctgtctttgctgcttctcgtgtttcaagcctttcctgtgggatcagcacagcaaagtgcaacttaccaaatggtttaatgactggttaattctttcttctcccaatggaaaagcaatggcaacacaacagtagactgctggcttgacaatcttaaacgtgagcctttgcacatgtaggtttatcatcatttgagtatacgactaagcaagtcaatgaactttttttttttttttagcagtttaatttggtcctgagaatgttgcagtctttattaccccttttgcattaatccacttttctaaccaccttttaagctttaatttttaacactatacaccaagtctttgaaatcagtgatctgttatttaactctaaagcatttgacacttcttgccttaacagttttaaaaaccacacacaaaaaaactctgtaagtaatacagtaggccaaaagtttcatcctatctatcttgcagtttacctatctgatctgatctctgtaattatagttctgtcatttaaaatatactatttaaatctaatttttacatttcaaaaattatcttcagtagtaactaagtatattttctgtggattctgagaatgttatttttcagaatgtgagaatatatatgtacatttataatcttgtgactttaaagtctgttttcagatacagtatgtaaatacttgtaaaaaaatttgtataattttgtgataatgtagtttcccaaaaaaattatttagaaggcattatgttattagtaaatgagagcactgtatagaactgttcctattttctgcacttgccattccagctgcctccactgtccatacccacctcattcatcctgtcacagaaggcaggaaaactgggaactttaccaaagtagcactcagcctgagaggcctgtataatcatgcttttcaaactaaattcacttaaaaattaaaaagcagaattgaatattttaagcagcctcagtacctttggccaatgctgttttcatggtggattatgaacattatataatctttgggaaaagtgaaagtagtacaatttttagaataatgacaactgcctcactgcatctctccactcacacagcaaccgtgtagccccctaagctgcagtaccatgactaaccatgatgtcaatttcatatgctgatcctcacaacagcagtgcacaaacatgccccaaatattttaacagaatttagctcttccttaagctgtcttttcatagtaaaaacaaaacaaaaacacccaatgttaaaaccacataataaacttacaaacttgaaaaattagacacttcagatagataggcaataaaacttcatattatgaaagcaatatattccaagtttcaaagatttgacaagttctgtagagtatctttcatcagtacatgaaaacttccaaactgcatgatcttctgccaggcaggactgggtgctattcgctggtttgaggtcgaatccatttcaaggcatgtcgtggtgggacattaatggtgggatggtagaatgtgcagtccggtcttgtacattgagtgttaaacctacaatgttttggatgatagaagggacattccatcttcttacaagcagggaagtaacggcagagctgactactggaaggtggtgctggtggtgcaactggttttggagacagtactggaattcttctactcacatgagtgaagggacaatctggtttagtacactttgcatcatatttacaatttgggtgaacaaacaaacatttttcagcaaatttacaattggggaaggctttgcagggtgagatggggtgatggtaggcacactcatccccatttttacaagcaggccagtacttgcagcgctccaaaagtttttctggtttctgtgccacactcagttcactcatctcagcttgatttttttctacagaatctccttttgtttcctcttctttaatggggggacttattctgggggtcctactttgtccctggaccacttctgctagcaattcttcttgagaagttcgagttctgggagcaactggaagtgtctgtttctgtggaactgtagagtagttagttgtttttgttacggattcttgagcttcagatatagccttcaaaatcagattcttgttagcttgtttagaaggtggaagagaaggtctcctttcaggctttgcaggcacagacacactgctggagatgcttcctgttcgagacccgtaatcatcatcttcttcctcctcttctccatcatgattgaatttttttactttaacaactgaacttaccacaggcaactttctcttccgaaagttttcatcctccatactcattttctccgagttgtttctaaagaacggactatacgtttcttctaagctgttaagcacctctggttcacacaaacgtcctgtttcatatacccaactactctgcatatcaagctgcttggcagcatgaatactattctgctgctgttgaaattgcaacctgtttaaatgaacaccactatctgcatttctacttgcaggtggtcgataaatttcaatagaagggcgagaagaaccatatgtaagtgtcactgtaggttttttctgagataagggattctcctgcacaaagttgaggtcttcgtcaatgagatcatctggttctggcttaatatcaatcacatcttcagagggtgctggctccctcaaaggtttcactgttgacattagtcgggttgcagctccatcatcgtaagtctgtctgacatttgtggtttttgactcctgcgaacttgtagaaactctggaatctcttttttcaggtctcgcgctaggaatggcaagtggtggcactgcagcttcatgcctcctctcatctccccgactgaaattgctcttgtttgaaggcacgttactatcaaagatgttggtatcagaagacttcagactagagggttcagttgtaacagagcgaagtttatctaatacaccatgaagccatacggtgaatcgaattgtgttgttccctagaaacagggacagatcctctgtcatttggtcctgacttttcttgttggccaccatcaccataatgtaatcaggaagttcttcatcaacataagctcctaattcttgtaatttccccttaatggcactccggatcttgcggctgatctcggtgccgatctccatggctctgcggcgtgcgggaactcagcactgcgcggcgcttggcttacccggaggctgccgcggactcctaccccgcagccgggacaccaccgcctcc

SEQ ID NO: 17472 - RNA, 13586 nt, Homo sapiens
  source 1..13586: mol_type = other RNA
tcaggccaggcacagtggctcatacctggaatcccagcactttgggaggccgaggcaggcagatcacctgaggtcaaggtatttgagaccagcctggccaacatggtgaaaccccatctctactaaaaatacagaaattagctgggtgtggtggtgcacacctgtaatgctagctactcgggaggctgaggtaggagaatcgcttgaacctgggaggcagaggttgcaataagcctagatcatgccactgcactcaagcctgggagacagagcgagactacatcttaaaaaaaaaaaaaaaagtattatgagagaggataatgtattgtaatgtattgtagaggctaaataaaattatgctcatgtcagaaaaaaagagtatttctcaaaataaaattcactgaaactggatgtttattttgactgagatatagtatatcctcaaattgccatagaaagtttacaagaatattagaggtaaattataaatatcagggcctttttaaaaaaaaaagattctgcttataacttggtatttgtttataataaaaattatagtagccaataatgaacacttactctggcttggttatttacttaggtcaaaagaaggaggagcggttaaactgtgggatcaggaactgaggcggtgccgtgccttcaggcttgagacaggacaagccacagattgtgttcgttctgtgtgcagaggcaaagtaagatgttccatgagctgatacagtgcagcagaaaacagaaagtggttattactgtgattccctcaccctttgcagcctaatgaacaatacttaataatgcataacgatggatttgcttgccaacattactctgtctttgctgctttctttgccaaagttagcaccagtgtggtgcataagctaggaagctattctgtctaaatactgtatgtaaacctccaatattttctagaatctgccaatttaacaactctagtagacataattgaaagcccttggcagttgactcatattaggacagctgtctccattttttaaaaaaacacacattccctagataaaacgtgcagtaaacaaacaatgaaatactactcagccataaaaaataatgaaattctgtcattcttggtggcaacatggatgagactggaggacatgatgtgaagtgaaataagccaggcacagaaagataaatacatgttctcactcctgtgcagaaactaaaaaagttgatcccacagaggtggagagtagaatagtggttactggaggcggacaagggggagggggagggggatagggaaggactggttaaaggatacaagtttacacagccagataggaatagtatgttttagtattctgtagtactgtaggatgactatagttaagaatcacgtatttatgtattttcaggtatttacaagagaggattttgaaagtttccatcacaaagaaatgataaatgtctgaggtgatggttatgcgtattaccctatgccctatagatatgtataattatgtgtcaatttcaaaataaaaattcaaaactacaactcctatgaaaatttttgagcgtgtttgtacttattaagtgtatttataaatcatacggatattatcttcagcctgcatattaaattgtagttaagcttttactttttaactaaaaaataaattctattattttttcctatatcccactgcactgaccccagtttggaaatcctaagattatcaaataaaaactttgattattgaagaatccaggtgtactgccacagaaaagttctattctgtagcatggactctaatatgtaatctagcccattgtgcttacagatagatgtgtgcctgtagtcatagaaaaatttgcatgagctaatgactgccttgctactagattagctcaaagcaaaaagttctctgaaagcaggtcaatagggtcatttttatattatgaagaagaaaagcagctgttgtattacattcactgtattggtcctgcttgtgtttcagggcaagatccttgttgggacaaggaatgctgaaataatcgaagttggagagaaaaatgcagcttgtaatattttagttaacggtcatgtggatgggccaatctggggactagcaacacatccttccagggattttttcctttctgctgcagaagatgggacagtgagactttgggatattgctgataaagtaagtacagataatttttttaaaagaggttacaacttctaaaaagaaaagttggaagttctaaattgctagtacttaaagaactgccagaattctgttgagcattttgaggggaaactggtataatttagaagtacttcacttaatgtttcctatgactctttttttttttttttttaaatgcagaagatgttaaacaaagtgaatttgggacatgctgctcgtactgtgtgttacagccctgaaggggacatggtggctattggaatgaaaaatggagaatttatcattttactagtgagttctctaaaaatatggggaaagaagagagacaggagatgtgcaatccatgatatcaggttagtgaacaaatggaatagagtttctagtatatacttgatttaacttccatttgtaaaattttccatagccttgccttcaaaaagaggtccccagggcctgtagcatttcccgtattataaattgtatgctaaaatatggctgtttgtatactacttaattcttcttgctaaattataaacccactgggcaccaactataatagcaagtactagtaggtaatgtttgatgaattcatgttaacacttagccatgtccattaagttcatcccaccaagaggtatctcccactgtaatacaagagagctatctgcccttcaaaagttgtcaccctggaaaactaaagttgtgatttcaaacatatcttctcttagtaacctcagtttgggaatatgtagttcattaatttaatcaatacctattgattaaatgttccagaatccaaattaatttaaatgtttcttaaacctttgtttttcagtgcttaagcatttttcaacagtggctaccatttacggagtacttccgtgtgatcagtagataagattattgaatctaggtctgtcaaaagcttgtacacttttcatcagtaaaatccttttacaaatgaaaccttcctcagaacttcaatatataaaatagtaacagtggcttcccttagcttttacatgtctctatcgtacctcagtaagactcatgggccatttcaagagactgaattgtcccatatgactccaaagattgctaggcaaatagcatttcactttgtcttttaaataagttcttcaggccgggcgcggtggctcatgcctgtaatcccagcactttgggaggccgaggcaggcagatcacctgaagtcaggagtactcgaccagcctggccaacatagtgaaaccccatctcaactaaaaatacaaaaatcagccgggcgtggtggcaggcgcctgtaatcccagctactcagggggctgaaacaggagaatcgcttgaacccgggaggcggaggttgcgccatcgcactccagcctgggagacaagagcgagacttcgtctcaaaaaaaaaaaattcttcttccaagattcaagttgtgtcatttcaccttaataactggaggttagttaagctgggctgtgttctttgcttaatattaagacaacgttttttccagatggaagaaaactatcttaatgaattgttagcttattaattatgtaatgctaatggcttttaaaagctgagatgttctgactgggtgttgtggctcacacctgtaatcccagtaccttgggaggccaagggggaaggattgcttgaggccaggagtttgggaccatagtgagaccccgcctctatttaaaaaattaaattttgttttgttttgttttgagttggagttttgctcttgttgcccatgctgaagtgcaatggtgcaatctcagctcaccacaacctgtgcctcctgggttcaagcgattctcctgcttcagcctcccgagtagatgggattacaggcgtgcaccaccatgcctggctaattttgtatttttagtagagacagggtttctctatgttggtcaggctggtctcaaactctcgacctcaggtgatctgcccgcctccgcttcccaaagttctgggattataggtgtgagccactgggcctggcctaagaaagtttttttaagccattagacgtttttaaaggaattgggagatgacaattggggaaatatttaaaatttaagtaaaatataaagcttccttatttcatgtaacccagacaatctcagtatacatgatcagttgtgtctgacaggtaaatctatttgaggccttatcacacgttacttttaagaactagaaaggaaaagtcactgatcttaagtatttataatacttcatgtggtctaatactttttacgttttgttttgattcagatttagtccggattcccggtatctggcagtaggttctagtgagaactcagtggatttttatgacctaacgctgggccccactcttaacagaatcagctactgcaaagacattccaagctttgtcattcaaatggacttctctgcagatagcagttatctccaggtacagtaccaatactgtatacccaggtggcaagttcttctgcttttacatttcgtgttagtgaatgcatttaaagttcctgagctccagagctccagcttctcaactcctccctttgtaccttctgacctacagctcccctttcctcccccacttatcagagcttttctcctattaagtttttgtagtgatcttttgcatacttaataatgttagacatgtaaatcaagtagcaatatgctagtattctgtaaaccccctgtggattttgtctctcacctaatggaattcttgtcccattttaatctgatgaaaaaggtctctagtggctgctataaacggcatgtctatgaagtgccttcaggaaaacatcttatggatcatgccgctattgacagaattacttgggctacatggactaggtaaatacttatatattcacaaggcaagaactgactttgaaggccagttagaaaatcctatttctgaactgttagagccattccaataaggaatagtaattgagtttcaagtttttgttaccatattttgaaatggtatgttcatgttgggacccctttttattgaatatatttccatgttttatcagtttccatgatttatcaagttttttttttaaggaaatcaaagttttaactttaaagataccctgatatttttcttaatgctaaatttaatgactggcaaaaaggtattgggtgctgttaagcaactgttattaattctctatctaaaggaatgctatcttgaatctattagaagtcaaagcttccaaatttgttcaaatttcctggctgtatgacaggtaaccatgactatccatttttttggccaatgaaaaatgccatcaaattcctgtatcagccaggcatatagtggctcatgcctgtaatctctgatgtagcaggccgaggtgggaggatcacttgagcctagaagttttgataccagcctgggcaacatagcaagaccccatctctgaaatttttttaattcctatgtcataagtcatttttatttttgtagagatagggatctcacaatattgcccaggctggtctcaaactcttggcctcaagcagtcctcctgcctcagcctcccaaaatgttgggattactggtatgtgctgctggacccagccaagtagcacttttaatttgaaaaatagttctatcagttttcagtcaggcgcggtggctcagcctgtaatcccagcactttgggaggccgagcgggggtgatcacctgaggtcgggagttcgagactagcctgaccaacatggagaaaccctgtctctactaaaaatacaaaataagccgggcatgttagcgcatgcctgtgatcccagctactcgggaggctgaggcaggagaattgcttgaacccaggaggcagaggttgcggtgagccgagatcatgccattgcactccagcctgggtaacaagagcgaaaactccgtctcaaaaaaaaaaaaagaaaaaatagttctatcagttttcataaagtactactttaatcttaaaaagattaatctagaaacccttcaaattataaaatgtcatttttaaaaggcaggagttgatatcctgatgaaattcaggtctccaaacaacttaccataatttacttcctgtattttaagtaacatgatagggtacttagagattaattgccaagaaactttttgaatatagtcaacctgcccgcacttgccatgatgagttttcttttgttccttccctctagtattctaggagatgaggttttgggaatctggtccagacatgctgagaaagctgatgtcaactgtgcctgtgtatctcattcaggaatcagtcttgttacaggagatgactttggcatggttaagttatttgacttcccatgtccagaaaaatttgtaagtttgtgttttgtttactattatcagtttactcctaattttgatgtcttatcatcagcacttttccccatatatttaaaatgttttgtcctaatttctaaatttttccccaaactttctaaatctatttactttgaaataaaagctattagaaacaaatcctctccctcgagtaataccatctttggaaccatcctacaaaagctgtaattagcttttcaccaaacctataatcagttatcaaatttcaaatgcttttccttagagaaaaatggtcagagtacctggagacatctgactgcccacacagcctggttttgcagatccactactcatgctgaaaagcattctaatcactggctgcggtgctaactccctactctctccacagctcttgtcatagagattatagttcctaataagagcctttgacttctgtgtgcaccaaatgccctgagcttgtctgtcattgttttttaggcaaaacacaaaaggttcttgggtcattcgccccatgtgacaaatattcgatttaccagtggtgatcgacatgttgttagtgctggaggtgatgactgcaggttagtaactttctcagcccatgaagagcagactatgttactagttaagagacttaatacaacaactcctacagctttggtttatgaaatcagctagtcaacattagtagaaggtagtataaccagatggctcttcagaatctcatatttatgcaaatacagaataaaaggagttaaagaggaaaaatattacacatgtaacctgaaagcacaactgaaaaatattaaactgttatgaaaatctaaaaacataattaactccctgcaattttcttctctgattgcagcttatttgtctggaaatgtgtacatacacctcactgagagatgctgagatgactacagaaattaactttgagaccagaattacagagaagaaaaaccaaaacccaaccctgcatggtcaagtggtgctaacccaagactgtaacagggagaaatgcccagaatcatcaaaatagtgaaagactgatctgttcaaaatatttgctatatgcactgggtataatccgtaatccatacactgccagataatgccatttcaaggaaggatcgaatacttgatggtaaaggccaagtccccctgtattgggaagtgtgtgatttcggcagacctgctgggaaaatttagggtagagcactctttacagaagaactcaaaaacccaatttggataattttcattatctttttagcaaaatggtttcttaatgtttatattttattttcaaggttcattgtttaatgaaatattttattcttgcatttccataaggaaagggaaagtcatgatcatcctaaaggatcacagtttttaaaaggcaaacattttccctaaggaaacagacacaagctttcctagagaatatgatgttttttaggcattaataaggtccttttttataaaggacacttttctcctagtagttttgaattcaggaacagatccaaagttagcagtatatggctgctacatttccattttcattttcgagccatcagtttatgttcagatgccatctctgtaatcgcacatttaaaacataactgtagcctcactaatggaaaagtagtatgatgaacaatcattcccaatggtgtacaatgtaagggttttagggagcaacagtatttaactggaagaaagaattgcatatttaatgtagtctaatatatacacatttgtttaacatgtaaacaaaagtgttaaattcacatatacaacattatacaatttaatcactcttggaataaaatttttatagccttttttctattgggaaaatttgtttagatgtgtgccactccataggtttatttccaaaatgaatgagcccaactccatttgtaaaaacttgtcagttagaattcctttttttagtggattagggctgaattcttagatccttatttcttttcactttaaatgctgccaaagatcactactcatcattcaggaattcgctgtctagcctatctgtagtttcctgaagattgaaaattatgtagactgctatttaaaaatatatttttctaagtgtgaggtttaagatgctgtattgaccctatgagtttttaatgtgttaattatctttatagcataatagatcgctttaggttcctggaatcccatttggtctgacaggatatatgaagattcttaatacctattttctgtgtctaatacttggttaatactaaaaatagaaatgactaaattacatcacagaaagcataaccagtgattgaacctggtagttttaaagctctaaatagctgtggctgaaggactgattatggggctaagaagcttgaaacgtaagttggtacttgttcatcagtggattctcctaaattaagccaaattttgaaatacatgactattaagtttctactcatgtatttacagtcagtcaataaattaaaggaggaaaaaaatccctgaacaacctgcccataaaaagaaaaatactctacatttgagcctgctgcagttttaaattttccctctgggtcaagtttgccagcttttggctacagagaaattatatttccattacagtgcaggtagaaactctgtaaccttaagcatgtaaactacatagaataaaactgtttccactgcatttctgtccttcaaagtggccaacctgattaagtcagccttaatcactgctgctgtcagtttcacgactaaaggtcatattgactaagtagtcatcagctgaccacctcgctgtatcagccagcaacgaggggaaggtgaagaaacatgataggccatatagaatctgccctatgtttacttttttaacccagataattatttttgtgtgcagtatctaagctcctgattgtgtaacctgggacttctggcaccttttgttccattcattttatgtataaaatgcatgccaaagcacactgtgccctctggtacccttgcttccaatcgccaaccatgctcatttccttcctttttttgtggtccctttttgtggtgatcattttaaaccacgtcatccaacaaatgttttatggtcaaccttagcttgttcataagccatagcaactgaaagattaaactcttaaatatgtgtctgggcagtggctattaaatagcaaaaaacaatcagattttagtattttattatttccttgtaaaatggctgaactaaattaaacccttgtttcccatttgttctataatttatagtgaaactgagaacaaaactatctttataaatgatagctaaaagtatttccagatatttaaacaatttaaaataaatttcttctgcagagatgcaaagcatctcaacactggaatgaacaaatgccttaaattcaatggagtaaacctttagaatgaagaggaactgtcatttcacccaagccgaagacaacagccttatgcacttgtgtgctctgtctttgctgcttctcgtgtttcaagcctttcctgtgggatcagcacagcaaagtgcaacttaccaaatggtttaatgactggttaattctttcttctcccaatggaaaagcaatggcaacacaacagtagactgctggcttgacaatcttaaacgtgagcctttgcacatgtaggtttatcatcatttgagtatacgactaagcaagtcaatgaactttttttttttttttagcagtttaatttggtcctgagaatgttgcagtctttattaccccttttgcattaatccacttttctaaccaccttttaagctttaatttttaacactatacaccaagtctttgaaatcagtgatctgttatttaactctaaagcatttgacacttcttgccttaacagttttaaaaaccacacacaaaaaaactctgtaagtaatacagtaggccaaaagtttcatcctatctatcttgcagtttacctatctgatctgatctctgtaattatagttctgtcatttaaaatatactatttaaatctaatttttacatttcaaaaattatcttcagtagtaactaagtatattttctgtggattctgagaatgttatttttcagaatgtgagaatatatatgtacatttataatcttgtgactttaaagtctgttttcagatacagtatgtaaatacttgtaaaaaaatttgtataattttgtgataatgtagtttcccaaaaaaattatttagaaggcattatgttattagtaaatgagagcactgtatagaactgttcctattttctgcacttgccattccagctgcctccactgtccatacccacctcattcatcctgtcacagaaggcaggaaaactgggaactttaccaaagtagcactcagcctgagaggcctgtataatcatgcttttcaaactaaattcacttaaaaattaaaaagcagaattgaatattttaagcagcctcagtacctttggccaatgctgttttcatggtggattatgaacattatataatctttgggaaaagtgaaagtagtacaatttttagaataatgacaactgcctcactgcatctctccactcacacagcaaccgtgtagccccctaagctgcagtaccatgactaaccatgatgtcaatttcatatgctgatcctcacaacagcagtgcacaaacatgccccaaatattttaacagaatttagctcttccttaagctgtcttttcatagtaaaaacaaaacaaaaacacccaatgttaaaaccacataataaacttacaaacttgaaaaattagacacttcagatagataggcaataaaacttcatattatgaaagcaatatattccaagtttcaaagatttgacaagttctgtagagtatctttcatcagtacatgaaaacttccaaactgcatgatcttctgccaggcaggactgggtgctattcgctggtttgaggtcgaatccatttcaaggcatgtcgtggtgggacattaatggtgggatggtagaatgtgcagtccggtcttgtacattgagtgttaaacctacaatgttttggatgatagaagggacattccatcttcttacaagcagggaagtaacggcagagctgactactggaaggtggtgctggtggtgcaactggttttggagacagtactggaattcttctactcacatgagtgaagggacaatctggtttagtacactttgcatcatatttacaatttgggtgaacaaacaaacatttttcagcaaatttacaattggggaaggctttgcagggtgagatggggtgatggtaggcacactcatccccatttttacaagcaggccagtacttgcagcgctccaaaagtttttctggtttctgtgccacactcagttcactcatctcagcttgatttttttctacagaatctccttttgtttcctcttctttaatggggggacttattctgggggtcctactttgtccctggaccacttctgctagcaattcttcttgagaagttcgagttctgggagcaactggaagtgtctgtttctgtggaactgtagagtagttagttgtttttgttacggattcttgagcttcagatatagccttcaaaatcagattcttgttagcttgtttagaaggtggaagagaaggtctcctttcaggctttgcaggcacagacacactgctggagatgcttcctgttcgagacccgtaatcatcatcttcttcctcctcttctccatcatgattgaatttttttactttaacaactgaacttaccacaggcaactttctcttccgaaagttttcatcctccatactcattttctccgagttgtttctaaagaacggactatacgtttcttctaagctgttaagcacctctggttcacacaaacgtcctgtttcatatacccaactactctgcatatcaagctgcttggcagcatgaatactattctgctgctgttgaaattgcaacctgtttaaatgaacaccactatctgcatttctacttgcaggtggtcgataaatttcaatagaagggcgagaagaaccatatgtaagtgtcactgtaggttttttctgagataagggattctcctgcacaaagttgaggtcttcgtcaatgagatcatctggttctggcttaatatcaatcacatcttcagagggtgctggctccctcaaaggtttcactgttgacattagtcgggttgcagctccatcatcgtaagtctgtctgacatttgtggtttttgactcctgcgaacttgtagaaactctggaatctcttttttcaggtctcgcgctaggaatggcaagtggtggcactgcagcttcatgcctcctctcatctccccgactgaaattgctcttgtttgaaggcacgttactatcaaagatgttggtatcagaagacttcagactagagggttcagttgtaacagagcgaagtttatctaatacaccatgaagccatacggtgaatcgaattgtgttgttccctagaaacagggacagatcctctgtcatttggtcctgacttttcttgttggccaccatcaccataatgtaatcaggaagttcttcatctatttaaaaggaaaggtagatcaaaactttgtttcctcaaaactttcttcttaaagttgatgtgcttgaaaatatagatgtagctctaagctttagagtcgcagagctctactggaattacattggacaagatggcttagctttaatttttttctcttcattccacaggtatttcaaatacaacataagctcctaattcttgtaatttccccttaatggcactccggatcttgcggctgatctcggtgccgatctccatggctctgcggcgtgcgggaactcagcactgcgcggcgcttggcttacccggaggctgccgcggactcctaccccgcagccgggacaccaccgcctcc

SEQ ID NO: 17473 - RNA, 14424 nt, Homo sapiens
  source 1..14424: mol_type = other RNA
tcaggccaggcacagtggctcatacctgtaatgccagcactttgggaggccaaggcaggtggatcacttgaagtcaggagtttgagaccagtctggccatcatggcagaaccctgtctctactacaaacacaaaaattagctgggtgtggtggtgagtgcttgtaatcccagctactcagaaggctgaggcatgaaaattgcttgaacctgggaggtggaggctgcagtgagccgagattgcatcactgcactccaacctgggtgacagagagactgcctcaaaaaaaaaaaagatggaaattttagaatttccctagatagaggggattttgaagcaacagaagtagatgaaattaccaagaaaaaatatacaagtagaggagatatttacacaagtagaagtagcaggcacggggatggagaagtcagaaaaacaatgcagttattcattttatatatatatatatatatatgagatagggtcttgctctgtcacttaggctggagtgcagtagtgagatcccagcatactgcaaccttgacctcctgggctcaagtgatcctcccctctcagcctcctgagtagctgatactacaggtgcatgccaccacactcagctaatttttaaattttttgtagagatagggtcttactatattgcccaggctgtgtcaacttcctgggctcaagcaatcctcctgcctcagcctcccaaactactgggattataggcatgagccactgcacctagcctgaaattattcattagtgtggaaatccagggtagacatatttatgagggaggcatggtcagtagcgcaaaacattactaagaggtcatggaggctgagtaccaagaatggaccattatacatagaaattaggtcttcgtttggtgactttttttttttttgagatggagtctcgctctgtcaccaggctggagtgcagtggcatgatctcaactcactgcaacctctgcctcccaggttcaagcagttctcctgcctcagccccccgagtagctgggactacaggcgcccgccaccacacccagctaatttttgtatttttagtagagacggggtttcaccatgttggccaggatggtctcgatctcttgacctcatgatctgcccacctcagcctcccaaagtgctgggattacaggcgtgagccaccgcgcccagccgttttgtgactttcaagagtgaagttgtactagaatgctcaagatagaagcctggttgcaaatggtcaaaagagatgtaagcaggtaggaaatcgaagacatgtgctttgcaaaaatacaaccatccaggaatggtgagagaaggacatagtttgtgaggttaacaggattatgtaacattttgggaattttgtttgattttgtttgtaagttatggtaagaccagagaatgtttctttggagtctgagcggagaacagatgaaagttgtaaaataaatgggggataagtgatggacaagaccaagtaagaggttagagagattgggattgaaaatttagttaatttctcccaacctcagcagggagaaaatgacagtcagctcagaattcaatgaaaagcccatctctgtttcagagtgggggaagaaattatggatgattctaatttttctttcagcttagctgtattttccaatttttctagaatgtaaaaattatttgaacattaaattttatttttctgaaagagcacatgagatagctgtctcatttgtccagtagtgctgactgggtgtgacagagttttttacctccctcacagcttcctctggggtcaacccccctgcccctatgcgccatcttcgtcacacctctctgggctgctcagtcctgatctgatagtcatgaaggagagcaagcaacgtttacctttgtagaagttagaaaagtgagacatctttctgctatgtttgaacacagtacagtgttctgtgagtacaatgtacaatgaggaaggcgaggtagatcatgtaaatgctgaaagctccatatgtgcttgatgactgggaagaaagaacaataaaatttaagaggaaaatacttgcctgtgtactgctttaaaagctgtggcctaagtatagcaaagaagtctcttcatatttgctaatactcattaattgcttattaagtatactcacttaagaattcacttttattaagtaccttcagtcttctcatcagttttgcactaagacgcgtacgctactgttcagtatagtgtttatatggatgctaaattggtacagatttctcctttaaaaagcatgaaatagataattaacttccatttttatgaatatttatcacagtagattaacttgaaacatgtagctttttcagtgtgcggcaataaaacggtatagtgattttgtgttttagtttgtaaatgtattacctgtacctagtgttatttgacaagtatctttacaaaattagatattagtcccatgctccttgaatttgtcacctgctcatcaagcaggccaagaatatatttgggtgagaagagatagactatcctaggctaatccttatggtaacaatggtacctggaaaaatgtcggaaaacaatttcccttggttttgtgtttgttgcacaatcaaaatgcagctgatgggatctgttgagttagtgctgactggtggtagcttcttctgggatccttctgccagctcctggactgagcactgtcccatctttcagttgctggaatgtcaccagcacagttagaaccctggtggtgcagggcacagcagcaaggcccacggggaaggaatgcccagcttgggcagagccaagcaagggtgactgtagcaaccttgttaccccaagcttaactgttcctctgtgacccttactggtatcactttgggccacttatctgcctggcacatgtcaaaactacctattaatgtccaagggccagacttgctgcagaatccaaagtttatattgataaggctgccacaaaataaattcagttcttctgtatcagccatgttacattctggctctgattatcaaaggtagaccttaaattgccttccgttccatgccactcttgtcctagctttccaactacaccctcccacactctgtatccagcctccccaccctgccagaaggtagtggtgtttctcattttatgactgtattaatgatagagctaagctggctgtcagtcatgatgcttcactccacatggattagtagtaacataactatgacagaacttagaatttgttgtaattcagtggtattttataaacacagccctggcctaggactgactaaacactaaatactatatctgcatttttctattaagattgcaatggccaggcacagtggcttaaacgtctgtaatcccagcactttgggaggctgaggtgggtggatcacgaagtcaggagatcaaggccatcctgactaacacggtgaaaccccgtctctactaaaaatagaaaaaattagctgggcgtggtggcacatgcctgtagtcccagctacttgggaggctgaggcaggagaatcgcttgaactcgggaggcggaggttgcaatgagccaagatcgcgccactgcactccagcctggtgacagagcaagactccatctcaaaaaaaaaaaaaaaaagattgcactaagtacattttcttctaggctgatttctaaaacattattccaggaagatatatgatttttgttaactttaggaacttttataaaactataatgacttttttggactaaattatatgtcagttttgatcatttgtgttattaatgtttcattatttgctttcaataaaattgtcttactattcattctcccttcaaccataggtatggaacaggatgtttcttactatgtaatacaggccataaggttggttttttaaattaaaaaattgatttaaaagtctaagttcatctaaataatgcttgaacataatttactattaaacaacttttagtctttagcttttacttaatctttatcagggtttaatttagagctcaatacaaaatttgaatcgttctaataagaaccattttagactctttgaattttatatgtgtgtttttaattgtgctggtgggaaatctagactgagacctcatcaaattcttaatgcaaatctaatttgaaacaaggaataaactttttatacagcttaaatgtgttcttaattctgatcgttttgactgtaaggatttattttaaaaattggtttattgattgcattattttgtacctatgttattttaactttaaaaaaaagttctcatgttatcttttcattttccactactgaaatcttttttttttctttcttacagtgtgtattttctgatcatggccttctcaccacagtggcttacaaacttggcagagacaaaccagtatattatgctttggaagtaagttctttttaatcaatatggataatatgacaaacattcaaagctaataaaaattacagtgttttctaacacttttctggtaaatcttaatacagaggactcaaaaagttctgctttcttggcatttgattgagttgaaggaacctgaaactgatctgggtgtcaggactcacaggagaccttgattagattggttcctcagttcttatgccaattaatcatgtcaccttaggcatattacttgagagctctacaatgtaaggttttttttttttttatctctaaagtttaatcggattaacgtgctctctaacatttctttcatcttgaaaattctttgattttataaataaaatgctccagtgttccaaagagaaccctgggcacaaataggcagaacaactctcttcacttgtctcctcataaaaataaattttgtgtaacattttgatatagaaaagaaagtgaggagatttatgccacttatcactggaaacatttgtttcaaacatttttgtatgttatagtaggaatatgccagcctaagcctataggatatggtaagttagtgttagaaatatttatttataaagtcaaagaaataatattctttttgtaaaattagatacatttcttataagcatttctatataattaattttgaaatggctaccttataatgcacaagtatacacttgatctgcagactcattgaggctcattttttggagtgcctgataataatttggtcacaagttaaagacttctagttagagttaaaacattttattagtcattatgcctagcacatgaggaatattagtttatttctatttttctcccttccccaccccataaacactataatatttctccccagctccttttctatggatggaagcatttgtgaaaacttagtctgtatattaaatgtatcttaacacttctcagaacttaaaatcctacaagccctctccctctctactttccctctgtggagagtgcatagcacaacactaggcacatagaatatgcacttgataagtgttacctataatataataagaatatgattctgctttttttcttcttgcatgggaaacaatcagtgctttagaatacaggtgccttagacctgggacaggcctcagggacaggggtcactcggtcttaactcccctcccaatgtgaaaaaccttctcctgtctcctttaccagtagccatccaacttctatctgaagacagcacccaaagttgcttcttaataacacctctagcattggacctgcattggttgtcaaaagtgttccaacattagaggctgcggtcagtttctctgggtcttcctcctccagggtaaactgacccaatgccttgatctcacatggtttctggatgctttatagttctgagctcccttcattgggtgcattgcaattcatgtcgtccagaatggaatataacattctacatctaatctgacctgtactcaatcaataggatgatttgtgcctctcctaccataagcactacttttgctcctctagcctgagagttcattaatttagactaatatttattaaattaatatttattaattaaaataattaatattaatttagacttcatattattggccctgggagcatatgctaaaaaacctagctcgttttcaaatgaatcattgtcaaaccaagtctgctctgttctgtatttgtgtagtttttttgttaaatctaaattcaggtctttgtttcttcctgtttaatttcataatagtgattttagcctattcctatatagtctgaattcgttttcactctttactgttactctttcagttttgtctcatctagagatttaacaagtatatgctttatgattttgtttcaatttatgtaatgcttttagatgcttagaattgtaaaagctcagagagacgctagatcatatgacaatataccctcctatccccttgttttacacgtgaggaaaccgagattagaaaagtgaaattggagtcccttggccaagtaacttttgacaacagtaagtagcagatccagatgcttggacatcaaagccttgatgcctaggccaccctgctgtaccatttccttccttgtaagtctgaaagttctgggctccagtctcccaagtccagtgttgttgtcactgcatctagcttatgtcccttccttcatctgctaacctagcggtctcagcaacaacaacaacacacatacgcatactaatatgttaacggtgtagttagaatttttttctttgttttcttaatttttttttacaattaacaaacatttaaaaaaaattaaattaaaccaaaccaaaaaacaagggtggggaataatgctagactggtaaaactttttatcagtaaacacatgctaatttcacttggtcatactaattcctttttttgtaaatgcttacaaagtatatatttaataatattgtctttcatttgatcaattgttgttaggcttagaagttggagataggaaaattttagtctttatgctctttaaaacctaaaactatagctacccatcttcagtcttttagtctttttccattcttcctctgctgatttgggaacaataagatacatttctatgtttttattttggtgattttttttcttttgcgtataccctcagatttttaagatattgtttaaccatatatttttctaagagtgtatgtcattttttggtatttttaatctcccgaccatgataaggaactctaatattttattctaccgcctccatcaccaattgtgttattttgtttaaagctttcatttcccccattttgttcaacatgtaataattactgttgttttctttgcagtccacagtaaatcatatttattgacttatttttcttagtttgtgtccagtatcatttctttggtctcacaccttttttattcccacctacttttttcctttttttcttcttctttttttttttgctgaggggcatccttctatagttcttttagttttagtgtgggatagtaagcctattctttttaggtttgtctttgttttgccctcactctgaggatgagtataaaagcctatattaacaattgtttttcccacatcccttctggccattttcgatgttgatgagacctctgctgtcaatatgtggttcatttgtagataatctggtttattgtctgggagtttctaacattatctctttatcattgatgttctgtagttttactatgatatgcctgtgtttggatttatttttatttatcctgttaggtacttggatccaagtctgtcttcagatctggaaagttctcagcaattatctcttcaaatattgctcctctaccattacctccatcctcttctggaattgctattggatgaatattggaacctttcaacccatcatccatgtctcttaactgcccttttatatttttttaatctctttgtttctctgtgctgcgtccctggtgagtttctcagtatctaccttccatttccaaatcctctctttaaaacaaacaagacaaatcataaaagccttttttgtattgtgaaatataagacacatagagaaaaatgcattaaatatcaatgtacaacttgaaaaattattataaaggctcatgtaacttgttcatagaacgccgccaatcccaagaacctctatttgccccacgatcacaacttcctccctctccctgagataaacatcagcctgacttttatcataatcacttccttacttttctttgtagttctaacacttaaatgtgcagccctgaacaccagagtttagttttgcatgtgtttaatatttgatatattaaaaatataaaagaaaagagagagagagcatgtgcatgcatatctgagtcacttagtatgtatttttttgtattttttgatctggcttctttcactcaacattatgtttgtgagattcatccacagtattatacatagctgtttttttcattgcttcttattgctatatgaaattattgaagtttagtatttattcagctgttgatgacattcgagttgttttcagtatttggctattatgaaaaatgctgctatgaacatttttgtatatgcctcctgatgtaaatgtattcacctttctgtaggagtagaatttctaggccatagattatgtgtatcttcactttgagtagatagtgcaaaccatttttcacagtagatgtgtcaagttacactcctaccagcaatatgggggaatgctagtttactcatcctctctatctagtctagagtttaccccatctagtacatttttcatcttatttaatattttcatttctatagtttttatttggttatttttcacatccacctgattttgtttcagttctcttttttttttattcttagtttcatgtttgtttgtttttaaaatggaagtcatttcctaatttatctccgaatacttaaaacatatgtattttaaaatctgtgttaggccggaatgaactctagtccagctattaagtttgttggatttcttttttcttttctttttttttttttttttttttttttgagatggagtctcgctctgtcgcccaggctggaattcagtggcctgatctcggctcactgcaagctctgtctcccaggttcacgccattctcctgcctcagcctcccgagtagctgggactacagatgcccaccaccatgcccggctaattttttgtatttttagtaaagactggaaataacgaagtttcaccgtgttagccaggatggtctcgatctcctgacctggtgatccgcccgcctcggcctcccaaagtgctggaattacaggcgtgagccaccgcgcccggccttgttggatttcttaatacaagatttcttcgtatagtttagaattgtcacttccagccttgtcttccattaagccatatagcctcagtcagcaaatacacagttgcttgtttttctagcatccctacacaagtaagagagcgccacctagctcctggcttcaagcattgagcctgattctattccctgtcttgcgcaaaacattttggacccctttcttctggaggaaccagttcccagccaccactcctactccctgacacatatagaaaaataaatcagaagccatcatgcttgtggcttcagtcctgtttggttatgtgtttccgtgtctgtccacatagatgttattctgtatttgagtcagcatgttgtttcagttttctcttttatatcgtgtctgttatcctctgtggttagaacaaaggggatttttgaagtacaaactcattatttctgctcatgtaagcatctgcatcttctttttcatcaccaagagaactctttttctctccctgaagcccctggcaggtgatagtaaggcctgacattttaatacctctaaattctcattttcattatttgtaaaaagaaataggtgttcatgatccttaagttgttctgtgacattaaactcatattaaactggttaaatttgtcccaccctttctagttggaaaatatttctcagtagtggaagagactggagcaaaatagagccattgagtggttctgccttccctctggcatccttgttcctcttctttttccaaatactgtttcacaaaacaaaaatccttttgggaacttttaatatgagtatgaacctgagcttacttatgacttgagacttccatgttccgtgttttgtcactagaatatagatttcctgaggccagggtacttgtctatcttgtttaccactctgtcccagcaggctggcagataatacatacccattaaatattgttcaaataccgaatcctatgttaggccatttttttctttttaaatatgagcttcaaagagggttccctatattgcctccctggtttctttaaatatctcttcccctatcttttctttgttatggtttaacgattatagcgttaagatttcctttttagagtttttcatccttcttgagctaaatccctattttaggtataaacctatgtaatagattatctattgctgtgtaacaagattaccacaaacttaagtggcttaaaacaacacatttattgtttctcagttcccatgggttcagaatccaggcacagcttagctgggtaccctgctcagagtctcacagggctgcagtcaagatgttgactgaggctctgctgtcatctgaggtttaatctgcttccaggttcattcaggttattggcaaaattcagttccttgtggttgtggaactgaggacttcagtttcttgctacctgtcagatggaggccaccctcagctcctagggctacctgcagttccctgctatctgagggacccccagtggttctctgcttccttaaagtcaggaagggagggaatatctccagcaagacaggcacagtaaatcatgtaatggaagcacgtacacatcaccacacatatcccatcacttttgacatgtactgttgggtagaagaaagtcacagatatcaccacgctcaagaggcgaggattatgcaagggtatgcacatcaggaggcagggatcatgggagccaccttaattaaaagtctatctgccacaagcatataaacattgtttatgaacttttataatgttctttcttgaaaagtatactttctgagcaataaatgcttttaattttagttccccaacttgttactgaagtattaatgaaatctgttacatttcaaaaataatgttgctccaattcaactcttccctttctctatgcaattaaaaatgctatagagttagacactgcatttgtaatctaatatatacaaattaactacattataaatcatatacgtacagatacatagcactgtagtatacacaaaactgtgtttgctatgcctgatgaatgattgtaagcaatttagggtaatctttactttacctgatttttctccatactcaccaattttcaccctaattgccttgtaagctacaattctactgcatcctgaaatatcctgctttatttttatactgtttgtggcagtggcattcatgtcaaggagcttttgaagaaaaatgtatttgcctgctatgacattacatcagatctacttgattatttttaattcaatcttcctatagcctgtttattagcctttcactttccaggctacatgtctagttttaaaataatttattcctcttgccctgttataatttaatttattattctttacaccctctcactttcattgcatctcccttagtgtacaactattaagcttgcatgcatcttttccagggaatcataacctagaacaagggctgattcaaatttgtagatgatatactaaagtattggatctttatacttagggtgtaatttatggtaacttaactgataacaagtagacagtcaccttcttttatcattttaggttttggctgctatactcttttcctgtccagctttgaaacattattaccatcttccattttatttcctgcctctgaattcagaagaccacatgtcttttgtgaattagagatgtctctcatttttatttctttaaaagctaaatcataccatgtattatatcctgacagcaaaattatttacttttttcagataagtgtttttatctaccttttattgtgttatattgaatctagtttttcaatcacaacaaaacacttctgtgtattcctgatgacagaatttaaaacagttatctcctggagccttaacagtgactatgtattttttttcttttgttttaatctaaataatactctgattctcaactaattacctctaatcaaaaccttgattttccttttgctaaaatcatattgctttctcttaaaaatatggtgtaagcatgtaacatcctatctttttcaatggaaatgaggtatatcagcacgtggtttcctagagtataaagtcccaccagctgtgccacaaaatcactttactagactcctagcacagtggcttctaaaaattcgcagtttaactgtacttgcctaaaacaattatgtatgcatttcttggttagatgctatttaaggacagtgtctttgagagtataaggaggagggacacctgtttttgtttttctttttcaattaggtctagaattatactgcccatggcagccatggccacatgcagctattgagcactggaaatgtggctagtctgaattgagatgtgctgtaagtgtaaagtatataccagatttcaaagatagtacaaaaaaaaatctcaataatttaatattgatttcatgttgaaattttttttaatacattgggttaaataaaatattaattttaccttccttttacctttttaatgtggcaaaaatataaattacatatgtgactcactttatatttctgttggacagcactggtctagaaactcttacatatttactagtatttggcagctgctatctctgaattgtctgtttccaaaggaaatttgaatcttaaatctctttaaaccaaaattttacttagttctcttgaatgatcccactaagtacctaaatatgtaaatgtgtcaaacttaatacaacaacttattttaggcagggaatgagctgtgttagagtcccttgtaaggtatttcttgaattgtttttgtcccatttttaaagccttgtcatatttgcacagctatgccagatctgttcctcaaatacttcctgtggttaaaaagccattttatatatgtaatgatacagagtactgtatgtatgtctacatatataaaaatgtataaacagaacaattgtggcattctgtagctttgcagtaacatagtaacttctcatagaagctatgaatgatggaatataccagcatattcattctctagtttacttacattttgacaactgacaacaagaaggcatgaccatttgtaattcagttaatagaactgaggacaggtccctacatttaatattacctgacgtttggtttggagtgactctgtggaagtaatttacattaataatctatatgaatgaactatcagagctaaaaaaaatttcttggtattcctaatggttcgtgctgatacttctttttttttttgccttcaggatctttttataatagctttattgagatatagttcatattccacacaatttacccttttcaaatatacagttcaatggtttatagtaatactatatttacagatttttacaaccatcaccacaatctaactttagaacattgtcaccaccccaaaaagaaaccccataaccaccccctatcccccagcccaggcaaccactaatctactttctgtctctatggatttgtctgttctggacatttcatatgaatgggatcgtacaatatatcgtcttctgtgcctggcttctttcactttgcataatgttttcaatgctcatccatgttgtagcatgtattaagacatcattccttttcatagtccaataatactccattgtgtagacatactgcgttttatctattcatcagtcagtgatatttggctgatacttttttaacattaaagaaattaatgaagtcaatatttacatttagtaagaaccttcacatatattctcatattgagcctcacagtaatttgtttaggtaagtgttgtcatagtcatcattttataggtgaagaaatggaggctcagaaagcctaagtaacttaggcaagttacttagatgaacttgctaagattaacttactaagttacttagattagttactaagattacacagcaattaagtactagaactgggactcaaagccagtttatccaactctgaaatatgtttttattgttattgccacagctctaggtgattttgttttaaagaaaaattacttactagctagctt

SEQ ID NO: 17474 - RNA, 115 nt, Homo sapiens
  source 1..115: mol_type = other RNA
tcaggccaggcacagtggctcatacttgtaatcccagcactttgggaggccaaggcaggcagatcacctgaggtcaggagttcgagaccagcctggccaacatatagtgaaactc

SEQ ID NO: 17475 - RNA, 7356 nt, Homo sapiens
  source 1..7356: mol_type = other RNA
tcaggccaggcacagtggctcatccctacaatcccagcactttgggaggccaaggttggaggatcacttgagcccaggagtttgagaccagcctgggaaagattacaagaccccatctctacaaaaagtacaaaaattatctgggcatggtgatatgcctgtagtcccagctattcaggaggctggggtgggagaatctcttgcatccaggaggttcagggtacagtgagccaagcttctgccactgcactgcagcctgggggacacagcgagaccctgtctctttaaaacacacacacacacacacacacacccctccatactctcaaagttaatctcttaacaattcccacagtttttccctatgtactttttatatatctaaaaccaggatctaacaagtttagatcctggtttttctcctaattaacataagcatcttcttatgttttctacacttagagagcatttgtaggttttgtttgtttgtttgagacagagtcttactctgccacccaggctggagtgcagtgcaatcccagctcactgcaacctctgcctccagtgttcaagcgattctcatgtgtcggcctcccaaatagatgggattacaggtgcctgccaccaagcccggctaatttttgtatttttttgtagagatggggtttcaccatgttggccaggctggtctcgaactcctggcctcaggtgatccgcccacctcagcctcccaaagtgcttggattacaggcatgagccactgtgctcagctggcatttgttatataacagaccattccttgaaaatgccaacaaaacaaaacttttcaccaccctaaccagaaaaatgaacttttttttctaaattgccctatttctgtcagtgattccaatctcctaccaaagaaacatttactctgaaataattaagtccttaaaactctgtgttgaattgattactcttccccgctttcagtcttctaaggcctgtctgttcctatcacatgtttctccaatccacccttactactctactgtgatgtcaacacaaatttctgaattattaaagaaacttccaaggaagtctcttttactccaatctctttaccctccccagtcaaagctgcagtaaaacctgtactttaagaagaaggctttcaggtcatttctcccttgtgagattatacaaagtttggatgcaaaataaaaatctaaaccaagaaggttgtgataagttcctcctttatgcagcctcatcacatctcctccttgacagtattaatatgctgtgcttatcttctcctccaacaccaggcccatccctacatttttccctcatggaatttattctcctcacctgctctattcttctttctcttctctgtgtccaattaagccaatgttcaagggtcatttcagagtgtacttcaagaccaagtgccctggtagttctagtcctttctctgcactccgtatcggtaagaatcacagaatgaactatggtcttctaattgtttttatacacacttccctgtactccaactagatacaaacaccgtgccttacactaccagccacgtggctggaccaggcaaggtaaagttggtggccaagggagaaggtctacaaacgcaccccaaacaaggatcccacccatggctttgctgcatcagcaaaaactctgatgaactaaagtcctcctccaaaaagacctagaggaaatatccaaatgaacagatcacttaacaatatgtagattatttaacagtaaaacaggcgattgccagagtaaatattttccatacgctacacaagccttaaaacattgaagttaaagctgaaaacattgacattaaagttggtttctatggatgtcaactacaactctgacagcaccattaataattcacatttcttagtttcttttggaatccagtcaactcctttctctagtttcaagaacccctaactccaagcacaactgtctgtgcttcaggtttcaactgcaaatagctagtttgtcagtacatgtcacattcattttttaattttctgtttagttacttaccaggctacacacaatatctgtctcaacattaacattattcataaccattttacctccccctcctcttgtgaacatgagaattattttaacacaccaaagagttaaaacagagacccagtcaattttaggtgtttggtaacaccctgccattttgtacaagaagtggctgtgaaccagagtctatttcagtggccaaattccatagtagaagtgagcttaaaaatactcaaggtcctaatgtgcttccagtctagaaggaccacatttgtaaggcattcctttggatcttgagtgatcataagcccctggaaagcaggtactactctctctctgcttcttgtttgttcaaaacaaactttttgggcacctaccatggtctatgtgctgtgctggacactgggaatgtaaagaggaacaaactacagttccttccctccaagaacttggtctacaagaacctagcaatgttgggtgcacagtagatatttaatacgtattaaatgggtatttccataaagagtccccataggttctctgggcccacgatgagaactcaaccattcatttcacaaatgataagtttgcagttgggccaaaaacctttaatttcaatgaaaccataacctgcaatggcttatgtcagagaacaacataaatatttgctttaagagctggtgccaagaatctcatgcaaactttaggcaaaatgttttagctgaggggtacttggctaaaaccagagggcttggaaggaggaaaatgtaatgcagagtctgctgaactttgacccatggcatcagtgaagtccaacaacttttcaagtcttggtcttctcatttgtaaaatggggacaatgcaaggctatgatttattcctcacaggaaaaaaagtcctctggaaatgtaaaagccgcattagagtaatgtttaataattcaagatgaggtctggaagaacatcaacagtctctcaccctctgtgcccaggcattttgaaagggcactgtgccaaagtccattagtgctgggaatacacatcagcaggaagccttttgcatcttgactccctttccattgagcccctgaaatcagatgcctaacaggaagataggaagctgaagtgttatgggaccccagctatcagtcaaacggttttcctaatgtctcctttttagttgttttgttttaaagaaagaattagctttcacaatcaaggttgctgtgattctaaaaatcccacaaaaatgcccgcttggaatgcctagcttttcaaggcttcaggtaacctgaaagtcctctgattcagatactggcagaacctgaacatgctgacagcttggattaatttgggggaaaggatgcaaggggcaataaaatattctaacttcagattcaaagaggcagcaatatggtgaagaaaagcacaaagttccaaaaccagactgacgttctctcccccaactgacttgtacattcagtgaattaactcagctgtgtatttccccaatatatcagcctggtgagagatgccataaacagacctgcaggcaaccctacagacatcccttatccctcccctcctccaggggtataaaggaaagctaacattaagtgaaagacataagtctagagctgcaatgtccatagtggtagtcaccaggaatgtgtgaatagccagcatccaatagatagctagtccaaattgagacgtgctatgtggataaaatatccaccagatcaaaaagactagtatggaggaatgtaaaatatttcaatattttatactgaatacatgctgaaataatattttgggtatattaggcttaaaatatataattaaaaataatttcatctgtttttttatttcttcatgtagctactagaaaattttacagtataggcaaggctctcaattgtagcccaaactgtatttttcttggacagtgctggctcagagcatcccagtttcacctggatcctttgaaaggacaaattgaacatatggaaatgcagtcaggctcacaaaacaaataacctcattttccatgaggtgaccttgacaccattgaaagaatgaagccgattacatggctgtcctctcacagttgatctccaagtacaagactgtttcttgtcaggctaaatgctctcttgcaatgatctgttttagataataccaagaaaagctctacagggtatgggtcaaagcacaggtactggagtcaggccgacctgggtttgaatcccatctctgccactttctagctgggtaatctcaggaatattatttaatatattaaggtgcctattctctgtaacaggacaatcagatttcttcacagagaaggggagggaagggttaacacagcaagggagatgaagaatcttgggcaccatgcctaacagacagcacttgagaatggtagccatctagtaaaattctagcaatcttatctgagcaccttccagaataatgatgaggtaggggagacggggatggggtgcaaaggagatgggaccacttgtccacagaccttggagtcagtgaattaaagccgaatcctcaggaacggtatttattccacacagtgcaacactgccctctagtgacaaagaggtggaaaagctttcagagcatgaggcaagcaaggaagaaaaatacatttttccaggctctaagacagtaagttctccaaatcagagagatcatatcaaagaataattttttctcatgagtcacctttaaagcagtgacatggagtatgaagagcaatattatcaagatttactaccaacccagaggttgtcactttgttaattatataatatctcaaataggaaaaacagtaattctctctagacatattaaatgtgacacctaaaaagaagaaagtctgagtgttccaggttactcgacattattctggtaggacagcacggaggtttaagattcatgtataacagtttgtaaaccagatttgatcacagatttggttaatgcaactaacaaggtcaaaacttaaggctgaactggtatacaaacttggaaggaatacttaccatttttaacctcttttctccttgcagagcacctaagtgaggctaacagtaccctgggttgttgtggggagtaaataagaaagaacaccgaaatgcccagcagagtgtctaacacacaagcagtaagtgttagctgctgctatttttgttgtttctgttgttccaactgccacaggcccaaatggaggaaaagccataagataaaataactccttttacttttttgggttaaaaccaaggcttacctagtttcatttcctgatgcatctaccaatcaaatgtatcattttataacaagaacatcttagcacaactttgatgtccctgagattataatgctaactgaagtttggtaatagtttagaattcagatactgatctttaataaggcagaaagatgatgctgtaatcaaaaccgtctgcagagacaagacgtgtcaccatttctatcgtaaacctactatggtcgttttaggcagtctctgcccatcttcattcttctcaattaacttggatgaaaaacataatactttaaattggaaattttttataataattttcctcacttaattttcatttttaatatagtgatctcacgtccaaacatttcccatttgatgatcaccgggtaaccatgtgaccccttaagccagtcccagacaactataatacatgctttctagtattgtacagttcttgtttcaatatcctgtagtcacttctatatccttgtcatggtatggtcctaagacaatccagccacagaatgtgtaacccagataaatcataccagcacaagcacaaaaccgaagaacttttggcagtgaggcctgcattgttaaaatcagcacattatatgcctggaaataacccaggtatctgatgactccaacccaaaccaagagcgtagaggttccaagaaaaatgctgcagagatcatagtttgtgagattcagccgttgatgaactcccactggtcggtgtcacacacaggccgcttgtacttctccaggaagaaatttagaaatctcttccgtaaccttagagcaagaacaatggatcttgtacacagaataagagatgccaagcaaatcacaatgacaaatgcatcaaacaccaggacatactgagcatttttctgagtagatccaaatatgttcaagtctttacattcttcaattttggcatcactgtcaaaatagattttgattttgccactgtgagctttattgtcaaagataatcgtattctgaaagacataacagtctggtaactcacgggaatgaattgtctgtaggtcaatgcctttaagatgaaaggagatttcaacctgtaagagccgataaaattccagtctgaagaatgatgagttcttccagtccggaggcttcttggagaggtcctgaaggtctaattgaacacaatcgagctcaacgtcgttgtcaatattcagtgtctcattagaaggaaacatggtccctttcttgtaatgctgcttacagacttttaagccaattctattgtcttcattttctccataaccaagggtccccagggtaatgtcctttagctgatgatactgattaatagcaaaaaagatgctctcataggcatcctcttgagtatatacactgcagctgtagtcatcttcatctgtaccagaatatcctttcaaaaacaagtgcttaaaagcaacagtgttatcttctttgaaagcaaccaccagctggttacttaaaccaaaacgaacaagctgtgtggtgaccatgactatcttcaaaatctgcaaacccagtttccacggaatctggcgtctggctcggtatttttcacaagggctcatgaagtaaaacttcaggtcttcccttagacattcttctttcatctcagaatcacgatgtgccattgcatttctgacggttaacctgaaaacacctgatcctctctccggaatccttgcctggggaaaacgataaggctgccgggccatgcctcctccttcaaaactttccagggctctcgggattcggaacaggaaacaccgttcacggccgactcatttcgccctcgccgtaacgcgtccgccgaagttggagccctgcaaagcggggttcccttctcttaccctttctgccggccgcgtggtgcgcgcagaccccggcccgagagcaggcgccgcagtcgtggagtgcggcgggcagttctcgggcggctgaaaggcggctctgtgt

SEQ ID NO: 17476 - RNA, 7429 nt, Homo sapiens
  source 1..7429: mol_type = other RNA
tcaggccaggcacagtggctcatccctacaatcccagcactttgggaggccaaggttggaggatcacttgagcccaggagtttgagaccagcctgggaaagattacaagaccccatctctacaaaaagtacaaaaattatctgggcatggtgatatgcctgtagtcccagctattcaggaggctggggtgggagaatctcttgcatccaggaggttcagggtacagtgagccaagcttctgccactgcactgcagcctgggggacacagcgagaccctgtctctttaaaacacacacacacacacacacacacccctccatactctcaaagttaatctcttaacaattcccacagtttttccctatgtactttttatatatctaaaaccaggatctaacaagtttagatcctggtttttctcctaattaacataagcatcttcttatgttttctacacttagagagcatttgtaggttttgtttgtttgtttgagacagagtcttactctgccacccaggctggagtgcagtgcaatcccagctcactgcaacctctgcctccagtgttcaagcgattctcatgtgtcggcctcccaaatagatgggattacaggtgcctgccaccaagcccggctaatttttgtatttttttgtagagatggggtttcaccatgttggccaggctggtctcgaactcctggcctcaggtgatccgcccacctcagcctcccaaagtgcttggattacaggcatgagccactgtgctcagctggcatttgttatataacagaccattccttgaaaatgccaacaaaacaaaacttttcaccaccctaaccagaaaaatgaacttttttttctaaattgccctatttctgtcagtgattccaatctcctaccaaagaaacatttactctgaaataattaagtccttaaaactctgtgttgaattgattactcttccccgctttcagtcttctaaggcctgtctgttcctatcacatgtttctccaatccacccttactactctactgtgatgtcaacacaaatttctgaattattaaagaaacttccaaggaagtctcttttactccaatctctttaccctccccagtcaaagctgcagtaaaacctgtactttaagaagaaggctttcaggtcatttctcccttgtgagattatacaaagtttggatgcaaaataaaaatctaaaccaagaaggttgtgataagttcctcctttatgcagcctcatcacatctcctccttgacagtattaatatgctgtgcttatcttctcctccaacaccaggcccatccctacatttttccctcatggaatttattctcctcacctgctctattcttctttctcttctctgtgtccaattaagccaatgttcaagggtcatttcagagtgtacttcaagaccaagtgccctggtagttctagtcctttctctgcactccgtatcggtaagaatcacagaatgaactatggtcttctaattgtttttatacacacttccctgtactccaactagatacaaacaccgtgccttacactaccagccacgtggctggaccaggcaaggtaaagttggtggccaagggagaaggtctacaaacgcaccccaaacaaggatcccacccatggctttgctgcatcagcaaaaactctgatgaactaaagtcctcctccaaaaagacctagaggaaatatccaaatgaacagatcacttaacaatatgtagattatttaacagtaaaacaggcgattgccagagtaaatattttccatacgctacacaagccttaaaacattgaagttaaagctgaaaacattgacattaaagttggtttctatggatgtcaactacaactctgacagcaccattaataattcacatttcttagtttcttttggaatccagtcaactcctttctctagtttcaagaacccctaactccaagcacaactgtctgtgcttcaggtttcaactgcaaatagctagtttgtcagtacatgtcacattcattttttaattttctgtttagttacttaccaggctacacacaatatctgtctcaacattaacattattcataaccattttacctccccctcctcttgtgaacatgagaattattttaacacaccaaagagttaaaacagagacccagtcaattttaggtgtttggtaacaccctgccattttgtacaagaagtggctgtgaaccagagtctatttcagtggccaaattccatagtagaagtgagcttaaaaatactcaaggtcctaatgtgcttccagtctagaaggaccacatttgtaaggcattcctttggatcttgagtgatcataagcccctggaaagcaggtactactctctctctgcttcttgtttgttcaaaacaaactttttgggcacctaccatggtctatgtgctgtgctggacactgggaatgtaaagaggaacaaactacagttccttccctccaagaacttggtctacaagaacctagcaatgttgggtgcacagtagatatttaatacgtattaaatgggtatttccataaagagtccccataggttctctgggcccacgatgagaactcaaccattcatttcacaaatgataagtttgcagttgggccaaaaacctttaatttcaatgaaaccataacctgcaatggcttatgtcagagaacaacataaatatttgctttaagagctggtgccaagaatctcatgcaaactttaggcaaaatgttttagctgaggggtacttggctaaaaccagagggcttggaaggaggaaaatgtaatgcagagtctgctgaactttgacccatggcatcagtgaagtccaacaacttttcaagtcttggtcttctcatttgtaaaatggggacaatgcaaggctatgatttattcctcacaggaaaaaaagtcctctggaaatgtaaaagccgcattagagtaatgtttaataattcaagatgaggtctggaagaacatcaacagtctctcaccctctgtgcccaggcattttgaaagggcactgtgccaaagtccattagtgctgggaatacacatcagcaggaagccttttgcatcttgactccctttccattgagcccctgaaatcagatgcctaacaggaagataggaagctgaagtgttatgggaccccagctatcagtcaaacggttttcctaatgtctcctttttagttgttttgttttaaagaaagaattagctttcacaatcaaggttgctgtgattctaaaaatcccacaaaaatgcccgcttggaatgcctagcttttcaaggcttcaggtaacctgaaagtcctctgattcagatactggcagaacctgaacatgctgacagcttggattaatttgggggaaaggatgcaaggggcaataaaatattctaacttcagattcaaagaggcagcaatatggtgaagaaaagcacaaagttccaaaaccagactgacgttctctcccccaactgacttgtacattcagtgaattaactcagctgtgtatttccccaatatatcagcctggtgagagatgccataaacagacctgcaggcaaccctacagacatcccttatccctcccctcctccaggggtataaaggaaagctaacattaagtgaaagacataagtctagagctgcaatgtccatagtggtagtcaccaggaatgtgtgaatagccagcatccaatagatagctagtccaaattgagacgtgctatgtggataaaatatccaccagatcaaaaagactagtatggaggaatgtaaaatatttcaatattttatactgaatacatgctgaaataatattttgggtatattaggcttaaaatatataattaaaaataatttcatctgtttttttatttcttcatgtagctactagaaaattttacagtataggcaaggctctcaattgtagcccaaactgtatttttcttggacagtgctggctcagagcatcccagtttcacctggatcctttgaaaggacaaattgaacatatggaaatgcagtcaggctcacaaaacaaataacctcattttccatgaggtgaccttgacaccattgaaagaatgaagccgattacatggctgtcctctcacagttgatctccaagtacaagactgtttcttgtcaggctaaatgctctcttgcaatgatctgttttagataataccaagaaaagctctacagggtatgggtcaaagcacaggtactggagtcaggccgacctgggtttgaatcccatctctgccactttctagctgggtaatctcaggaatattatttaatatattaaggtgcctattctctgtaacaggacaatcagatttcttcacagagaaggggagggaagggttaacacagcaagggagatgaagaatcttgggcaccatgcctaacagacagcacttgagaatggtagccatctagtaaaattctagcaatcttatctgagcaccttccagaataatgatgaggtaggggagacggggatggggtgcaaaggagatgggaccacttgtccacagaccttggagtcagtgaattaaagccgaatcctcaggaacggtatttattccacacagtgcaacactgccctctagtgacaaagaggtggaaaagctttcagagcatgaggcaagcaaggaagaaaaatacatttttccaggctctaagacagtaagttctccaaatcagagagatcatatcaaagaataattttttctcatgagtcacctttaaagcagtgacatggagtatgaagagcaatattatcaagatttactaccaacccagaggttgtcactttgttaattatataatatctcaaataggaaaaacagtaattctctctagacatattaaatgtgacacctaaaaagaagaaagtctgagtgttccaggttactcgacattattctggtaggacagcacggaggtttaagattcatgtataacagtttgtaaaccagatttgatcacagatttggttaatgcaactaacaaggtcaaaacttaaggctgaactggtatacaaacttggaaggaatacttaccatttttaacctcttttctccttgcagagcacctaagtgaggctaacagtaccctgggttgttgtggggagtaaataagaaagaacaccgaaatgcccagcagagtgtctaacacacaagcagtaagtgttagctgctgctatttttgttgtttctgttgttccaactgccacaggcccaaatggaggaaaagccataagataaaataactccttttacttttttgggttaaaaccaaggcttacctagtttcatttcctgatgcatctaccaatcaaatgtatcattttataacaagaacatcttagcacaactttgatgtccctgagattataatgctaactgaagtttggtaatagtttagaattcagatactgatctttaataaggcagaaagatgatgctgtaatcaaaaccgtctgcagagacaagacgtgtcaccatttctatcgtaaacctactatggtcgttttaggcagtctctgcccatcttcattcttctcaattaacttggatgaaaaacataatactttaaattggaaattttttataataattttcctcacttaattttcatttttaatatagtgatctcacgtccaaacatttcccatttgatgatcaccgggtaaccatgtgaccccttaagccagtcccagacaactataatacatgctttctagtattgtacagttcttgtttcaatatcctgtagtcacttctatatccttgtcatggtatggtcctaagacaatccagccacagaatgtgtaacccagataaatcataccagcacaagcacaaaaccgaagaacttttggcagtgaggcctgcattgttaaaatcagcacattatatgcctggaaataacccaggtatctgatgactccaacccaaaccaagagcgtagaggttccaagaaaaatgctgcagagatcatagtttgtgagattctttgctttgatttccatttttaatatggagccaatgattgtcattaggtcgctgataatcaccaggacataccagccgttgatgaactcccactggtcggtgtcacacacaggccgcttgtacttctccaggaagaaatttagaaatctcttccgtaaccttagagcaagaacaatggatcttgtacacagaataagagatgccaagcaaatcacaatgacaaatgcatcaaacaccaggacatactgagcatttttctgagtagatccaaatatgttcaagtctttacattcttcaattttggcatcactgtcaaaatagattttgattttgccactgtgagctttattgtcaaagataatcgtattctgaaagacataacagtctggtaactcacgggaatgaattgtctgtaggtcaatgcctttaagatgaaaggagatttcaacctgtaagagccgataaaattccagtctgaagaatgatgagttcttccagtccggaggcttcttggagaggtcctgaaggtctaattgaacacaatcgagctcaacgtcgttgtcaatattcagtgtctcattagaaggaaacatggtccctttcttgtaatgctgcttacagacttttaagccaattctattgtcttcattttctccataaccaagggtccccagggtaatgtcctttagctgatgatactgattaatagcaaaaaagatgctctcataggcatcctcttgagtatatacactgcagctgtagtcatcttcatctgtaccagaatatcctttcaaaaacaagtgcttaaaagcaacagtgttatcttctttgaaagcaaccaccagctggttacttaaaccaaaacgaacaagctgtgtggtgaccatgactatcttcaaaatctgcaaacccagtttccacggaatctggcgtctggctcggtatttttcacaagggctcatgaagtaaaacttcaggtcttcccttagacattcttctttcatctcagaatcacgatgtgccattgcatttctgacggttaacctgaaaacacctgatcctctctccggaatccttgcctggggaaaacgataaggctgccgggccatgcctcctccttcaaaactttccagggctctcgggattcggaacaggaaacaccgttcacggccgactcatttcgccctcgccgtaacgcgtccgccgaagttggagccctgcaaagcggggttcccttctcttaccctttctgccggccgcgtggtgcgcgcagaccccggcccgagagcaggcgccgcagtcgtggagtgcggcgggcagttctcgggcggctgaaaggcggctctgtgt

SEQ ID NO: 17477 - RNA, 694 nt, Homo sapiens
  source 1..694: mol_type = other RNA
tcaggccaggcacagtggctcatctcatgcctgtaatcccagcactttgggaggccgaggtgggtggatcaccagaggtcaggagcctgagaccagcctggccaacacagtgaaaccctgtttctaataaagaggctgaggcacgagaatctcttgaacccagggttgcagtgagccaagaccgcaccactgcactccagactgggagacagagcaagaccccgtcatgattgctgttccaccaaatccaatgtccacagttaaaacttgatgcttctgaagacctaggggaaggctatagataaaggtatgacgcaggttctcctagaaacaatgcaagctgggcagaagcttcaaagagtagatggagcctggtttttgcttggaatcagattcctcgctactccaatatggctttaaccacctcttggtgtctcagctaagaatgcctgcctcagttcagcctggaaatccaccacaggtacttgctgctgctgagaacgcctcgggtacaactgacactcttggttgctcagtgaggcagtccttctgcgtttgacttggacttccacctctggtacgtgctgttctgtagttcgtctcaggtgtaagcgatcccttgcccgctccatcgcgtcactgaccgctcctcagacagatgcgtcaggcatctccggcggccgctccactctgc

SEQ ID NO: 17478 - RNA, 818 nt, Homo sapiens
  source 1..818: mol_type = other RNA
tcaggccaggcacagtggctcatctcatgcctgtaatcccagcactttgggaggccgaggtgggtggatcaccagaggtcaggagcctgagaccagcctggccaacacagtgaaaccctgtttctaataaagaggctgaggcacgagaatctcttgaacccagggttgcagtgagccaagaccgcaccactgcactccagactgggagacagagcaagaccccgtcatgattgctgttccaccaaatccaatgtccacagttaaaacttgatgcttctgaagacctaggggaaggctatagataaaggtatgacgcaggttctcctagaaacaatgcaagctgggcagaagcttcaaagagtagatggagcctggtttttgcttggaatcagattcctcgctactccaatatggctttaaccacctcttggtgtctcagctaagaatgcctgcctcagttcagcctggaaatccaccacaggtacttgctgctgctgagaacgcctcgggtacaactgacactttcaaattatcctgtgtgaacaatcctttctccccaggggtgaggggagggagatgctgctaaagcatttgcagggagatgtttaggccgtccttcatattgatcctcctgacaagtcactactcttggttgctcagtgaggcagtccttctgcgtttgacttggacttccacctctggtacgtgctgttctgtagttcgtctcaggtgtaagcgatcccttgcccgctccatcgcgtcactgaccgctcctcagacagatgcgtcaggcatctccggcggccgctccactctgc

SEQ ID NO: 17479 - RNA, 543 nt, Homo sapiens
  source 1..543: mol_type = other RNA
tcaggccaggcacagtggctcatctcatgcctgtaatcccagcactttgggaggccgaggtgggtggatcaccagaggtcaggagcctgagaccagcctggccaacacagtgaaaccctgtttctaataaagaggctgaggcacgagaatctcttgaacccagggttgcagtgagccaagaccgcaccactgcactccagactgggagacagagcaagaccccgtcatgattgctgttccaccaaatccaatgtccacagttaaaacttgatgcttctgaagacctaggggaaggctatagataaaggtatgacgcaggttctcctagaaacaatgcaagctgggcagaagcttcaaagagtagatggagctcttggttgctcagtgaggcagtccttctgcgtttgacttggacttccacctctggtacgtgctgttctgtagttcgtctcaggtgtaagcgatcccttgcccgctccatcgcgtcactgaccgctcctcagacagatgcgtcaggcatctccggcggccgctccactctgc

SEQ ID NO: 17480 - RNA, 1030 nt, Homo sapiens
  source 1..1030: mol_type = other RNA
tcaggccaggcacagtggctcatctcatgcctgtaatcccagcactttgggaggccgaggtgggtggatcaccagaggtcaggagcctgagaccagcctggccaacacagtgaaaccctgtttctaataaagaggctgaggcacgagaatctcttgaacccagggttgcagtgagccaagaccgcaccactgcactccagactgggagacagagcaagaccccgtctggtttttgcttggaatcagattcctcgctactccaatatggctttaaccacctcttggtgtctcagctaagaatgcctgcctcagttcagcctggaaatccaccacaggtacttgctgctgctgagaacgcctcgggtacaactgacactcttggttgctcagtgaggcagtccttctgcgtttgacttggacttccacctctggtacgtgctgttctgtagttcgtctcaggtgtaagcgatccctctctcaacgtgtgttcctcagaccagtcctggcacttgttcgaaatgcagattcttctgccgcaaaccaaaccataagagaaagtagattcagccactggtaaaaggggcagcaaaaatctgtagaggagattctggtggaagagtatgttcagggaatgttgccttctgagttccacttacatatgctggagaagtgccccacgtggctgctagctgtgtggagacttgatgggagtcccaattaccttcgtcaaagtatctcatttgcagtttgctgttaggatgctctcaccctgtggtgtatctttcatcaggtggtggtgagctggccactgtgaattttcagatccacagatcccacttacatcaggaaggtgtcattgatcagcgaccacagttactgtagagaaaagcctttcttatgcaaaaaggccgcattcctcaaatagccccagagagagggcagggggcagctgaccttgcccccgcaaaccacacagaaggctctgagctcagctacagtggctgcggccagcccttggtgggcgtggtct

SEQ ID NO: 17481 - RNA, 548 nt, Homo sapiens
  source 1..548: mol_type = other RNA
tcaggccaggcacagtggctcatctcatgcctgtaatcccagcactttgggaggccgaggtgggtggatcaccagaggtcaggagcctgagaccagcctggccaacacagtgaaaccctgtttctaataaagaggctgaggcacgagaatctcttgaacccagggttgcagtgagccaagaccgcaccactgcactccagactgggagacagagcaagaccccgtctggtttttgcttggaatcagattcctcgctactccaatatggctttaaccacctcttggtgtctcagctaagaatgcctgcctcagttcagcctggaaatccaccacaggtacttgctgctgctgagaacgcctcgggtacaactgacactcttggttgctcagtgaggcagtccttctgcgtttgacttggacttccacctctggtacgtgctgttctgtagttcgtctcaggtgtaagcgatcccttgcccgctccatcgcgtcactgaccgctcctcagacagatgcgtcaggcatctccggcggccgctccactctgc

SEQ ID NO: 17482 - RNA, 3845 nt, Homo sapiens
  source 1..3845: mol_type = other RNA
tcaggccaggcacagtggctcatgcagtgggagggtagcttgaattcaggagtttgagaccagcgtggacaacttagtaagactgtctctataagaaaatcgaaatatcagccgagtgtggtggcgtgcacttgtgatcccagctacttgtgaggctgaggcaggacgactgcttgagcccaggaggtcaaggctgcagtgagctgtgattatgccactacactccagcatgggggacatctttcttctaagactacacacacatgaaatgtgatccttctgtgagctgcggctgagtggatggaactggcgatgccgaggactcaggagatggggacagacttttcactgccattgtttgatttcctctagaaacctcaggagttgattcgtaagaaataacagtttcttcctgttcgtcaacactgttctttgtattttcttcaggatgctcttctggtttatgatttgcggtctgtgtttcatcttgagggctgaatgtaacatcctcaggcattttgtctttgtttctttctttatccatcatttccacagaatttactccatttggctcaggttcaaaaagcatttcatatgaaatgttttcagttttttttaactctttgctgaagtccacattttggggttcggtttcttttagttgaacaatttctgttgcaggagtttcatggtctggctttacatcattttctctaatggcagtgtccagttccttatcatccctccttcgagtctgagtagtcctaaatggattatcccttaaatttgaagggctttgtaagggtgactggtctgaagcaccgataacatttaacccttttttcttctccctcaggcacgcttgttgatgtcttcttattctttccatttgctcttccacagtcatccttggtcgagtactttcagccaaacagagctgttccactgcacttcttggtctttccgttcttagatccatcatcttcttagttttcctcaaggttacataggaagctattgtcgaagattcgggtgttggtgattttgctcttggagggactactccaacaggaaagtgggaacctttaacaactgaagtttctatctctgaaacaggttctgatttttcttctccattagattcatcaacttctgccactgttgttaactctggttcactcttgtagagtctataatctggaccctcatttttgtacttaactgttgagaaaggctttgatcctatcatacctatttctgtagtacctctttgctgcttatgtttactcagcccttccatgacatcctgaattcgccaaagttctttctgaatctgtgcacgctgaattcctgctgattccgtctgaacttcaccaaggtgatccagctgctcttgcatctggttcctggtaacagttacatcgtattctaacttatcatattctctccatgctcgttccaattcggcagtggctcgagaaagttctcgacacgtactaagcagtccattttgtaaatcatccctttgtaacaccactgtctgaatggctgctgggttatctgcatgcatttctatctcttggctggctgatagcaaagcttgctcaagcgtgtatttctccttgtggagttgctgaagtttctcttccagagcatgcaccactttatcttgttcacataatcggcttaacttggcatcaatatctacttcttcaggtctgtatttgtataatgtgcctctaccttcatcttgtgacagctgatgatccaaatatatggtgttcctttggagatgatgtgaaagaatttcattctttgggctgtgggcctcaagctttagctgcatgagctgtgctaacgtatgctcccggatactactcagttcggcttgctgccgtctcagctttattagcagcagcgtaagctcctctggcgttttcccttggaggctctggggactaacagactgtaaagtcaggccagctggcactgaccttctgtcaggcacatagacatgcttagggtgatgggccctgtgtctgcggtctattgtcacatctcctctctgaattggtgaagacacttccgatctgtaagttcgttgaggggagtatccctgataagcagctattgacccgtgggaaggtgatgtgggaatagagtgcattgtctggtcagaaatatttaccatggttttgggactactcaaagtactgtgtcgagggagggtgctctgtttgttataaaactgacgctgctgccattcgtagagctgccacattgtgtcatctctcatggacctccgtttctcctccgctccgggtcctaatgtcttgtcatgagtggaaggggttacactgcagatactttcaggccttgtcttgctgtttcttgggagtgttctataaccttcagggtagcgggccataatctgggctctgtgacttggcatatttcttggtaatgtttggtaagaaattactcccctggtttcttcttcatgacccctccccttctggattttaatccactgttccaactgctgcattgaatttgttctctgtatgactcgatcggcctctgtgtataagggccctgtattggggcgatttccacctctaagatctgccaggctaacattgactattttgttctctgaactgctcaagttgattggtctgtagtgcacagtctgagcagggcatgctgacccactctcatattcagatggcagagaattcagctttacactattaatttttgttaagggtctatcttgaccatccttctgaaatccatatttttcagcttctaatgcctttttttcttcaattttgctcatttccttgtttttttgattgttttggatctctggtttaattagcactctatggttgggaatgttattggtttctttagttggtgcattttcagatgtaatcttgtccactcttttcacaggttctgtctgtactagggcagcatctaacatggctttcatccacaactccatttcctttcctgtatcagtgcagaaataataggtccgcatgtttggatgggctgccttaaaagcatatttgcgattaatgtgatcttcagaggtaagcaaagctatctgaaaactaggtaacagtatgcttcccaggataccctcttctttctcatctctataataaaagaggcaaaggtcagaaagcacaaaccagcgtttcttccacaatttcatgccagtactgtcctgtttataaagccaacctcgtctgacaaccggtgcattaggattccttttaattgaatttgacctctttccaaaattatgaactttttttgaagctcgtgaagttctgcctacagggctcattggatgcactgcataatctgaagtcacgttatagttagaagcttcatttatcatacttattggccgttccttcttttcttcagatgtcatggttgcaacagtctgttcattcactacaaaaatacaattgtcctgtgatggttgtcctgtgactggatgtttgcaggtcactttcctttcattatggtttatatagtatcttgcaccttcaaaagtatatgcttcttcccagccagtaggcaaatctgtgctctgccgccggtgtccggtgaccaccgcctcgccggtgacggggtgcagccaggtggtgctcttggcctcctcgttgatgaagaagactcggccgcccctggtgatcccgtaagtccaggaccggggcagggagatccactccaggttcagatccgccgccatgtctgatccctagccgccgccgccgccttctcctgctgccgccgcggctgccgagggaggagggaac

SEQ ID NO: 17483 - RNA, 311 nt, Homo sapiens
  source 1..311: mol_type = other RNA
tcaggccaggcacagtggctcatgcccgtaatcccagcagtttgggaggccaaggcgggtggatcacctgaggtcaggagtttgagattagccagaccaacatggagaaaccccgcctctactaaaactacaaaaaattagctgggcatggtggctcatgcctgtaatcccagatactcaggaagctgaggcaggagaattgcttgaacccaggaggtggaggttgcagtgagccaagatcacgccattgcactccagcctgggcaacaagagcaaaactccatctcaaaaaaaaaaaaaaaaaaaaaaaa

SEQ ID NO: 17484 - RNA, 1973 nt, Homo sapiens
  source 1..1973: mol_type = other RNA
tcaggccaggcacagtggctcatgcctaaaatcccagcaccttgggaggccgaggtgggggaattgcttgagtccagaaattcaagcccagcctgggtgacatggtgaaaccctgtctcttttggatcattgtgagtcaacagctgtatgtcaaattgtttagcaaatgcagtcaaatctggtggcatcacacagcaggaggcaagattaacttggttactatttggttttacctgtgcccactgatacagctgttccaactgtgttttgtctagatcagaggtacctatggcaacaatctttttgctctgaactaagttttctaattcctcccagtaaggctgtaaatgctccaaggaaagattaactccatcttcaataggaggtgaagcaatgatcacagaatccagctgtgcaactccaaggactgaacaggccatgtcaactgcacttctagttgatgatgaagagtttgattctacaatgaacagttttgcagaaactttcatttcttctctttcatcaggatttatcttttctactgcatgagatacagtgcattccaagacatctggaaactccctgaccaaatctgggttgatttgggaactccattcattcaaggttttttggatacaatcatgaagctcctcgctgtgcgtggacgggcacttcttccgcaggcggccccagttcagcaggttccccgtctgcaggtgcagggtgcgggcccgcgccaggagcgccttggccgcgcggctgtcggtgcccatggcagcggccgcccaggggccgcgcagcgaaggggctgcgggcgggcgggcaggcaggcggccgccccacaggacgcggtgcccgaggcccgagagagacccgagagggagcgcgaggctgccggcgccgcgcggctggagcctggtctgcgctcgggcccgagggaggccggacggcggctgggcggcggcgggaaaggaaggcaccggtggctgcggctccggctccggctactgcggccgcagcgggagagctgattccaaactgagggagctgtttcctggaagacaatgactaagcagaaatcgtagccgagaaagtgcttcgtaaccgttactcatcccgcggcggggcaggggcggggcgcgaatgggctgcgggacgccggcccgcaagtgactggcccttggcctgcggcgggcgtggcgacgggtggtgcgcggcgggcgcgcgggtcgagagagcgtggcggcgcggcccggagcgcagcgcgcggcagggctccccctggcggtcagaggacagcgcgaggcagacaccgcctccgcctggtgaggtagacaccgcctccgcctggtgaggtctcccggcgttcaggtcgcggctccgcccacggccgccccagggtgggcttcctacacgtctctttaaagggcagcctgagcggccaccgggactcggaaatgctacgtagttttcgttctcagaagcagctgtttatgcgcaagcgcccccttcttcttttcgctttgctaccttcaaggaccttctcccaaactgctaatttttcttcatccgttaaaggtctattgattcacattatttgctggcagtgtgtgaagtcaacgaacaagactgagtctttgcccttgagacgcgtacactctacccagagacaagttctaagcacaggaaacaagtaattttataagaacatcatagggcagttattctccagatgaattcagattaaagaggacacttgagccggtgagatcacagaaagcttttatcacccacccctttagaggtggtcgagattatttacccctattaaatttcacgtgtggtggtggactcggtataaacatcaaattgaacatgtattgagctttcctcaacaatctttcacattcgttgaggtgaatcagattattaaaggcaaaatgagattctcattataagcggggacaatatag

SEQ ID NO: 17485 - RNA, 1914 nt, Homo sapiens
  source 1..1914: mol_type = other RNA
tcaggccaggcacagtggctcatgcctaaaatcccagcaccttgggaggccgaggtgggggaattgcttgagtccagaaattcaagcccagcctgggtgacatggtgaaaccctgtctcttttggatcattgtgagtcaacagctgtatgtcaaattgtttagcaaatgcagtcaaatctggtggcatcacacagcaggaggcaagattaacttggttactatttggttttacctgtgcccactgatacagctgttccaactgtgttttgtctagatcagaggtacctatggcaacaatctttttgctctgaactaagttttctaattcctcccagtaaggctgtaaatgctccaaggaaagattaactccatcttcaataggaggtgaagcaatgatcacagaatccagctgtgcaactccaaggactgaacaggccatgtcaactgcacttctagttgatgatgaagagtttgattctacaatgaacagttttgcagaaactttcatttcttctctttcatcaggatttatcttttctactgcatgagatacagtgcattccaagacatctggaaactcctcctcgctgtgcgtggacgggcacttcttccgcaggcggccccagttcagcaggttccccgtctgcaggtgcagggtgcgggcccgcgccaggagcgccttggccgcgcggctgtcggtgcccatggcagcggccgcccaggggccgcgcagcgaaggggctgcgggcgggcgggcaggcaggcggccgccccacaggacgcggtgcccgaggcccgagagagacccgagagggagcgcgaggctgccggcgccgcgcggctggagcctggtctgcgctcgggcccgagggaggccggacggcggctgggcggcggcgggaaaggaaggcaccggtggctgcggctccggctccggctactgcggccgcagcgggagagctgattccaaactgagggagctgtttcctggaagacaatgactaagcagaaatcgtagccgagaaagtgcttcgtaaccgttactcatcccgcggcggggcaggggcggggcgcgaatgggctgcgggacgccggcccgcaagtgactggcccttggcctgcggcgggcgtggcgacgggtggtgcgcggcgggcgcgcgggtcgagagagcgtggcggcgcggcccggagcgcagcgcgcggcagggctccccctggcggtcagaggacagcgcgaggcagacaccgcctccgcctggtgaggtagacaccgcctccgcctggtgaggtctcccggcgttcaggtcgcggctccgcccacggccgccccagggtgggcttcctacacgtctctttaaagggcagcctgagcggccaccgggactcggaaatgctacgtagttttcgttctcagaagcagctgtttatgcgcaagcgcccccttcttcttttcgctttgctaccttcaaggaccttctcccaaactgctaatttttcttcatccgttaaaggtctattgattcacattatttgctggcagtgtgtgaagtcaacgaacaagactgagtctttgcccttgagacgcgtacactctacccagagacaagttctaagcacaggaaacaagtaattttataagaacatcatagggcagttattctccagatgaattcagattaaagaggacacttgagccggtgagatcacagaaagcttttatcacccacccctttagaggtggtcgagattatttacccctattaaatttcacgtgtggtggtggactcggtataaacatcaaattgaacatgtattgagctttcctcaacaatctttcacattcgttgaggtgaatcagattattaaaggcaaaatgagattctcattataagcggggacaatatagctattga

SEQ ID NO: 17486 - RNA, 559 nt, Homo sapiens
  source 1..559: mol_type = other RNA
tcaggccaggcacagtggctcatgcctataatcccagcactggcttggtgacatgtagctcaggtatcgcattgcagggcacctggccgtcactgagggcaccgactatcagcaccgcgtcgaaggtcccttccgggctgggcagaggctcctggcccagggtgcagaggctgaggcgctgatagaggccgggggcctgggcctgttccagcatccctgggctcccatccaccccatgcagctggaggaagcctggagcccgcagctcggcagccactaggcctgtgccacaggccacgtccaggatcagggcactgtggggcgggcctggaagggcttgtgtgaggcagtccactgcgaggcggggcgcacggtacagcagggtggccacatcctggtcgtagtccggagcccagcggtcatagaaatggagcttttgggccaggtcggggatgccatgcgcggccctgacccgcgcccgcacctcgggcaggctcccaccctcctcctgggccatgctccgccaatccagcgcgcctcgggcgtgtgggcaacagga

SEQ ID NO: 17487 - RNA, 1167 nt, Homo sapiens
  source 1..1167: mol_type = other RNA
tcaggccaggcacagtggctcatgcctataatcccagcactttgggaagccaaggtgggtggatcacctgaggtcaggagttcgagaccagcctggccaacatggtgaaaacccatctctactaaaaacacaaaaattagctgggtgtggtggtgcacgcctgtagtcccagctactcaggaggctgaggcaagagaatcgcttgaacctgggaggcagaggttgcagtgagccaagattgtgccactgcactccagcttgggtgacagagtgggactctgtctgaaaaaacaaacaaacaaaattatcctaagcaaatacggtgtctgaagactaagctgaccctgtttccaaagtcaaatgtccataggctttggaaatatcatgagtggcatgtcgcaaatcggttatccagtcactctttgcctatctgaagagaatacaaattacacaactttttatcaccaaagataattccacagattgtgtaagtgcatggtcatgaaatagttgaaattggtctttctttgaaagatagcataactaggccaggcgcagtggctcatgcctgtaatcccagcactttgggaggccgaggtgggtggatcaccaggtcaggagatcgagaccatcctgctaacatgatgaaaccccgtctctattaaaaatacaaaaaaattagccaggcgtggtggtgggcacctgtagtcccagctactcgggaggctgaggcagaagaatggtgtgaacccgggaggcggagcttgcagtgagccgagatcgtgccactgcactccagcctgggcgacagagtgaaactccattgagaatcttggcagtgaaatcagagaatccaaatgggtcatcagaggggtgccgcaggttcaggtagattgggtgtagtttccatggcaaagaagagatatggatgttttaaaagaaaatatcctttgcagaactgcaataatgttgatccctatagtgaattgtctttttctttccacttcatcacctctagcaagtttctcttcaacgtgcctaaacacctagaattcctgttctgtcttctaaaatgctgtcatcacctccattgcccaaatctagttcaaaagtgaggagagaaaaaaaattgaaatttgcaagctgtttatgcctaacaacaacatt

SEQ ID NO: 17488 - RNA, 3961 nt, Homo sapiens
  source 1..3961: mol_type = other RNA
tcaggccaggcacagtggctcatgcctataatcccagcactttgggaggccaaggcaggaggatcacttgagcccaggaattcaagaccaggctgggcaacattgtgagagttggctctaaaaaaacttaaaaattagcagggtgtggtggcccatgcctatactcccagctacttgtggggctgaggtgagaggatcacttgagcccaggaggtcaaggctgcagtaagccatgatcacaccactgtaccccagcctgcgcaatgaagcaagaccccgcctcaaaaaataaaaataaagtttatattttaaagcacataattactattctcattcatctttaatttaaatacttggtattaattcccatttacagttgtgtttttctcagtctcaacctcagcttcaagtaacttggtatcttagattgcatttgcagtgacttagagctctgcttcctttctttatgtatgataaagcagaaagagacagacacaggatgtagtgataggagggcacaggaaacataaaacccctcaggtatttttcggtcacctgggctctcttctctttctcattcaagagtgtttttgctgcaactgtacagcaaaaacacaaaactactcatctctgaatagctgatacctttataacttcccacccactccttgttatggtgatttcagttacaaatggacttaattaaatggaatgtaccacttacaaagatcaaaaggctttcaaaaatttttcttaagatttttgaacaaagatttaactgtttctattaaaatgcaataagatggaaactctgtttcctctgatgtgattattatgcattgtatacctatatcaaaatatctcaagcaccccataaatatataaacctactatgtacccacaaaaattaaaaattaaaaacttttttttaatgcaataagaattaaacctgttttgcagagaaataagacagtggaaaaaatcaagttatacatatacatatatattacatacatatacatatataacatgcatatacatatataaaatatacatgtattattatatataataatatacatatatattaaacctattaaggtattaatgacatataagatcttgtaaagacagtgaatgtaaataaaactaaagatgttattccagtcagaaagttaccacctttatgccctctgagctcatcaagcttcataggatttgaatgaaataataaagtatatctgtatttgataaagacattatgagaaggcagaactgacattgtgtctgctgcataaacctgtctattttggtctctgttccaaagttattgtttccccaaatttttgtttattaccctgtcatgtaaagatagaagaatgatgaaacttgcaaatcaaagtatataataattatgagagaatggttttcttagcctgggcaacatggcaaaccccatctctacaaaaaatacaaaaattagctgagcagggtagcaaatgcctgtagtcccagctgcttgggaggctgaggtgggaggatcacttgagctgggggtcgaggccacagtgagccgtgatcacaccattgcactccagcctgggtgacagcgagaccgtgtctcaaaaacaaaaaaaaaaaggagttttcttgaggcttcatcactagaccattattctgtaacatcttcagagagttacctttactccctgtctccactcttcacctccctctcactcatcacctcattgttacggctttcagccccatctctccaaataaactgctctaggtaagctgttataggtaagtttagcaatggcctccatattattgaatctagccattgttttttaatctttattttttccctttagcagtattcagcattgttaaccaccctatccttaactctatcgtttccctgtggtttctatgacatgacactctcctgattgtgtccctctgtctttactgcttcctctctgttccctttggaggtcattcttccttacctggctgttaaattgctgaagctccctagggcttgtttgatctcaggtccttcatcatataaagctacacactgtccttagattatttcagccatactctagctttaattatgtaagatgactcacaaactcatcttcctagttctggctacactctgaactccagactcttctttgactttttcaccttgatatttcaaagcacttcaacaacatgctcaaaacaaactcatcatctcccttcccagtcgtggctctcttttagtgttcccgatcctagtgcaccacctatccaattgtgcaaaccagaaatctagtcatcagtcatgacatctccctctttctcactccccatttccagtctatccccatttcctgttggttttcatttccatgtatttctagaattcattcattgctgtctcttcccctgccttcccaccaaaactaccatcctcacttgcctgcactgcagcaatagtccactcattaatctcctagcacttacccttgttcctttgtaaatcattctctatcctgtaatcttttcaaaacacaaatctgacctcttacgataaagacaagaagacttaccctgtcctgcaagcccagcatagtctggcccctgtgtcccactccaccctccttgcatggcacattcgttcttgccctctctactttagctatgctggtctctgtttgggccctcatactggccatgtgtatcagtcaagatcaagtcaggagataagaaccatactggttatttgaataggagaaatgtaatgtaaagcattgttaattaaaacagtaggaggttactaactactagaaggggtaaaagaggaccataaggtgtccacatttagcatgagagcagttactatatctgtactgaagaaaatgagacaataaaggaactaaggcctaggggaggcccccaagccaagactgagattctgacctgatcgaagaaggtgtgtggctaccagaggaacgtgcagccttgtggtggtgaagaaacttgtcaaagggcacagactgagctcttctgttaagaggctgccattgccagagggtgtagatggattggagctgctcaaagccactgacagtggcgggaggtggggaatggcacgaggatgtaggttggagctcctctgaatggctgctgggttctcaagatcagatgatgtgctttgctgcaattacctccatacgttatgtcagtcacacacttggcactggcagtcagctccgctggcactgcagccttctttgcagaataaaggcccacaataagagcttgaggagttcagaaatctttcccttgtaaaggagcttaatccattgcgtccttactgctcatccatttacgttcctggtcagtgatgtgttgaaggaatgattttttaatagaggcttcaaattttctttgcttataactgtggcttagagatttggttttcctgatgtctactggtgtcatcagtggcttgctggcatctgatacttatctcttttcttttttggtagaatggatcttctaaccaaagacggagatttaatccacagtatcataacaacaggctaaatgggcctgccaagtcgcagggcagtgggaatgaagccgagccactgggaaagggcaacagccgccacgaacacagaagacagccgcacaacggcttccggcccaaaaacaaaggcggtgccaaaaatcaagaggcttccttggggatgaagacccccgaggccccggcccattctgaaaagccccggcgaaggcagcacgctgcagacacctcggaggccaggcccttccggggtagtgtcggtagggtttcacagtgcaatctctgccccacgagaatagaagtttccacagatgcagcagttctctcagtcccggctgtgacgttggtggcctgagctaggaggaaaaa

SEQ ID NO: 17489 - RNA, 4488 nt, Homo sapiens
  source 1..4488: mol_type = other RNA
tcaggccaggcacagtggctcatgcctataatcccagcactttgggaggccgaggcgggcagatcacgaggtcaggagatcaagaccatcctggctaacacggtgaaaccccgtctctactaaaaatacaaaaatttagccgggcatggtggcaggtgcctgtagtcccagctactcgggaggctgaggcaggagaatggcgtgaacccaggaggcagagcttgcagtgagccaagatcgtgccactgcactccagcctgggcaacagagcgagactccatctcaaaaaaaaaaaaaaagcaagatgtgctaacatctaacacctttatgttcaacaacttgaagttatctctgaagaaattattttctcactttttttgcttttcagagactagagagcaactttactcactacataaatttatttgcattgttacatcttgtgttcagagtcttgataaaactatagccacggcttacaacattattaaacaagcttcttacagaaaccaaaaatatttacttttaaagaagacatgataatatagtgcaaacaacagtcatgtgtcagagtgtaacaactgattcaaaacctttagaactaagtttcaacaggacagaattttgctcaatagaatttacatattttctttcctttaaaatggttttcatagcctgtataatcaatttgacatggtatttataacttattttccttgtaatgaaaagtatcaacaataattagttgtttatccatttgtgtgataaatgtcatatatattatttagtgaaacttaagttcttcagatttaaagcaattttgtggtgaaattaaccctgttagatagtagaaaagaaccatcagtgcttctgttgacacttctgtaccttactaccaataaaaaggccacgaggtaaaaaggcacatagaattctataaaaaacatatttaaatgaatcagagttgctaaataaagaacaaggatgtgaaaaaaagtaccaaaattccaatattgggagttagatttcctgtttcagtgttattaatattgaccttaatagattcctggtaaaaatcattatttttaaaatcctacaaaaagtaaaactttgttggaaacgactatgttcacttcctgttcaaacaataaaaataaattaaacagtaagaaaacatatttttcagttcatagcgcctgaagagaaacatatacattaaaaataaaattcactgtaattactcaaatcctgcttatagaactgatatatttacatttatactgaagtttcagagtttttagtggagttccgcactttctcagccacactgagctattagaaatcacatttggaaatgtgttgagacaaatgtgtttgagacccaagactttctcaaaaaatgctgaaaaagaggtgtgtgtgcatatatatatgcatgctacttaactttaaaaatatgtaccatttatgtttcttaaccttttcaatgcccatggagtaaaagtaaacaaaaacaattgtattatttctaatggtctgcagctatctttaattttctatgttaggtgtatacattttttaatttaaaaaactatcaagttccattttgaccttagaattatagagtcaactaaatgattcactttgacttgatacatttcaccttgtcctttgtctccatctatttaaaagagaaatttataagtgaacaaaaaggctgcaataatgcagttctactcctgtatacttaactgtgatcttcatgcagatcaatctaaagtctcttgtatgcatatacttgcaaaactagagtgttttcctttaaatgggaaaatgttttgtgtccttggggcttcatgaaaagatttgccgctgatgccaaaaagaggtgaggaggaaataaagttcataagtcttgcatatcttcatccagctggacagtctggagcttggcaagctcttttttgtctgtttccaggtcttcacagacagtatcaaccatgccatctaagacatacttggatttagagtccagcatcattaagctacttgttgctttgctctcagaatttgataagaaattctctttcatgttagctaccgattgcagaaccaaacgatgttcttggacaaaatcctgatgtactgctggggaggggtgacctacctgatcttcagctgtaggaactatttccccaagggcagcctgagtcatagggactgacaataggtcttgaccagtaataagggagcagttctgaagagttgcatagttagtgttgctgacagatgtcacagtagatttgcttgccaccggtgcagacattggttggctatcggcaatgtcgcggtttagctcagtgggatttagtagtgtagagggactgagagaaaaattgtgagttggagatacattaactaatgaggaggccagtggatgcaggccactccccgagatgttttcagaagacaggtttgcatttacttgtgcattctgattgacaggcatcaactgagaaaataccaggctcctttccaagccttcctgtttcacagatcctatagtctggcctgtattaggaaccgtgtataccactgcactgggagcaagagagctcaagaaaacctttccttgctggactgtggtagactcacttgtaaatgtgcttccatctgaagtgcttgagcttactgagatattaccttgtgaagctgccactgacacagggggcagctgcagtggagagaatccaatgctcccattaaggaactggctgtttgctccggaattggggatctggacaatgccatactggttaatttgcactggtgtagtaaaagtcactacagaccctccatcttgggaagccactgtttgaatgccttctcttttcacctcagtgctgggtatcaggcctgggaatgagacagggacactggggctgtaggacgtggtggttgctgagttagcagaactctggaggactttgaattccttcacgtcctgggaagtagaccccagtatgtcagtcatggatataccattgctcacaatgtttgatgacatttttggtgggttcaatgccactgcctgtgtatttcccacatttaatccattaaggataactccactgggtccctgaataaaagaatttccattaaggaagacaggtgaagtacttgcaggtaccaagcttccattcaacagaactccagaagagcttaatgatatcttagcatttccaatttgttgcatatatactggctccatatgactggaaaggctgaggttggtgatgccatcagatgaactggagagtgggtgaggagataaatcctcatgtcccttgctggattcatcttcagtgctggggttgccatctgactcactgctcccaaacttctactccaccagactgacaactctctcattcaacaaagtggctgtccttgttgtaggaaaaggcactttcaacccaagaacagttatgtgcagtcgcctttgaatccaaaggaagccaaaggggcctatttaacaaacaccatccagtgcccttttggactgggtctcggaggggttcctgtcgcgctgccggcggttcttgaaccagttgctgacctgggtgagggagaggccggtgatcttggccaggtgccgcttctcggcgggcgaagggtagcgattctgcttgtagagctccttgagcgcgttgcgcgacttctccttgaaacaatacaccgtctcctcgccgtcccagatggtgcggggcagggggaatttcctgcgcagccggtacttgtctacggctcccagcggccggccgcgggctcgctcggcctcggtgtagcgcgccttgtaccagagctgctgcagcagcgggtggttggccgactcgaagctgtggctctcgaggatgctgtagagctcggggtagatgccctggtggaaggccacgagcgcccgcgccttcagcaggctctcgttgccacgtagcaggtcgctctggggcagggaccacaggaaccgggccaggcggtccaggttgcccccctgctgcagtgcctcgcacacgcaggcgacgtggtcgggcgagaaggccagcggggtctgcgcggcggcggcggcggcgtggtggtgcctgcccagaagttccgagtggagttgtacctgatccgccgccgctccggccgccgccgccgccactgccccttcctctccgctcaccctggcggcagcggtcgcggcgtcccccggctccaggggaaaaggggctggagccggggggctcagccctaccgccgcgccccccgccacttctcggtgcgcctcctgcccttccgaggcgctttccatcccattctcttgcttgatgtccgccgcacttgcgatctgcccggtgggggaggaagaggacattttttgttgtttattttcctccctccctcactccctcgcactcttttcctctttctttcctcctctcttac

SEQ ID NO: 17490 - RNA, 4529 nt, Homo sapiens
  source 1..4529: mol_type = other RNA
tcaggccaggcacagtggctcatgcctataatcccagcactttgggaggccgaggcgggcagatcacgaggtcaggagatcaagaccatcctggctaacacggtgaaaccccgtctctactaaaaatacaaaaatttagccgggcatggtggcaggtgcctgtagtcccagctactcgggaggctgaggcaggagaatggcgtgaacccaggaggcagagcttgcagtgagccaagatcgtgccactgcactccagcctgggcaacagagcgagactccatctcaaaaaaaaaaaaaaagcaagatgtgctaacatctaacacctttatgttcaacaacttgaagttatctctgaagaaattattttctcactttttttgcttttcagagactagagagcaactttactcactacataaatttatttgcattgttacatcttgtgttcagagtcttgataaaactatagccacggcttacaacattattaaacaagcttcttacagaaaccaaaaatatttacttttaaagaagacatgataatatagtgcaaacaacagtcatgtgtcagagtgtaacaactgattcaaaacctttagaactaagtttcaacaggacagaattttgctcaatagaatttacatattttctttcctttaaaatggttttcatagcctgtataatcaatttgacatggtatttataacttattttccttgtaatgaaaagtatcaacaataattagttgtttatccatttgtgtgataaatgtcatatatattatttagtgaaacttaagttcttcagatttaaagcaattttgtggtgaaattaaccctgttagatagtagaaaagaaccatcagtgcttctgttgacacttctgtaccttactaccaataaaaaggccacgaggtaaaaaggcacatagaattctataaaaaacatatttaaatgaatcagagttgctaaataaagaacaaggatgtgaaaaaaagtaccaaaattccaatattgggagttagatttcctgtttcagtgttattaatattgaccttaatagattcctggtaaaaatcattatttttaaaatcctacaaaaagtaaaactttgttggaaacgactatgttcacttcctgttcaaacaataaaaataaattaaacagtaagaaaacatatttttcagttcatagcgcctgaagagaaacatatacattaaaaataaaattcactgtaattactcaaatcctgcttatagaactgatatatttacatttatactgaagtttcagagtttttagtggagttccgcactttctcagccacactgagctattagaaatcacatttggaaatgtgttgagacaaatgtgtttgagacccaagactttctcaaaaaatgctgaaaaagaggtgtgtgtgcatatatatatgcatgctacttaactttaaaaatatgtaccatttatgtttcttaaccttttcaatgcccatggagtaaaagtaaacaaaaacaattgtattatttctaatggtctgcagctatctttaattttctatgttaggtgtatacattttttaatttaaaaaactatcaagttccattttgaccttagaattatagagtcaactaaatgattcactttgacttgatacatttcaccttgtcctttgtctccatctatttaaaagagaaatttataagtgaacaaaaaggctgcaataatgcagttctactcctgtatacttaactgtgatcttcatgcagatcaatctaaagtctcttgtatgcatatacttgcaaaactagagtgttttcctttaaatgggaaaatgttttgtgtccttggggcttcatgaaaagatttgccgctgatgccaaaaagaggtgaggaggaaataaagttcataagtcttgcatatcttcatccagctggacagtctggagcttggcaagctcttttttgtctgtttccaggtcttcacagacagtatcaaccatgccatctaagacatacttggatttagagtccagcatcattaagctacttgttgctttgctctcagaatttgataagaaattctctttcatgttagctaccgattgcagaaccaaacgatgttcttggacaaaatcctgatgtactgctggggaggggtgacctacctgatcttcagctgtaggaactatttccccaagggcagcctgagtcatagggactgacaataggtcttgaccagtaataagggagcagttctgaagagttgcatagttagtgttgctgacagatgtcacagtagatttgcttgccaccggtgcagacattggttggctatcggcaatgtcgcggtttagctcagtgggatttagtagtgtagagggactgagagaaaaattgtgagttggagatacattaactaatgaggaggccagtggatgcaggccactccccgagatgttttcagaagacaggtttgcatttacttgtgcattctgattgacaggcatcaactgagaaaataccaggctcctttccaagccttcctgtttcacagatcctatagtctggcctgtattaggaaccgtgtataccactgcactgggagcaagagagctcaagaaaacctttccttgctggactgtggtagactcacttgtaaatgtgcttccatctgaagtgcttgagcttactgagatattaccttgtgaagctgccactgacacagggggcagctgcagtggagagaatccaatgctcccattaaggaactggctgtttgctccggaattggggatctggacaatgccatactggttaatttgcactggtgtagtaaaagtcactacagaccctccatcttgggaagccactgtttgaatgccttctcttttcacctcagtgctgggtatcaggcctgggaatgagacagggacactggggctgtaggacgtggtggttgctgagttagcagaactctggaggactttgaattccttcacgtcctgggaagtagaccccagtatgtcagtcatggatataccattgctcacaatgtttgatgacatttttggtgggttcaatgccactgcctgtgtatttcccacatttaatccattaaggataactccactgggtccctgaataaaagaatttccattaaggaagacaggtgaagtacttgcaggtaccaagcttccattcaacagaactccagaagagcttaatgatatcttagcatttccaatttgttgcatatatactggctccatatgactggaaaggctgaggttggtgatgccatcagatgaactggagagtgggtgaggagataaatcctcatgtcccttgctggattcatcttcagtgctggggttgccatctgactcacttttggactgggtctcggaggggttcctgtcgcgctgccggcggttcttgaaccagttgctgacctgggtgagggagaggccggtgatcttggccaggtgccgcttctcggcgggcgaagggtagcgattctgcttgtagagctccttgagcgcgttgcgcgacttctccttgaaacaatacaccgtctcctcgccgtcccagatggtgcggggcagggggaatttcctgcgcagccggtacttgtctacggctcccagcggccggccgcgggctcgctcggcctcggtgtagcgcgccttgtaccagagctgctgcagcagcgggtggttggccgactcgaagctgtggctctcgaggatgctgtagagctcggggtagatgccctggtggaaggccacgagcgcccgcgccttcagcaggctctcgttgccacgtagcaggtcgctctggggcagggaccacaggaaccgggccaggcggtccaggttgcccccctgctgcagtgcctcgcacacgcaggcgacgtggtcgggcgagaaggccagcggggtctgcgcggcggcggcggcggcgtggtggtgcctgcccagaagttccgagtggagttgtacctgatccgccgccgctccggccgccgccgccgccactgccccttcctctccgctcaccctggcggcagcggtcgcggcgtcccccggctccaggggaaaaggggctggagccggggggctcagccctaccgccgcgccccccgccacttctcggtgcgcctcctgcccttccgaggcgctttccatcccattctcttgcttgatgtccgccgcacttgcgatctgcccggtgggggaggaagaggacattttttgttgtttattttcctccctccctcactccctcgcactcttttcctctttctttcctcctctcttactcctcctccttcgtctccctccctcctctccccctccggaaagcccactccctccctcctggtttcggctgtatctggccgatcaggtttccccccggccacgcagtcaccattaagatagctgttagagcaaagtagtgtaaacggatagctgctttctgccgttcccccaacgtgactcctccggttgctgcatactatatggc

SEQ ID NO: 17491 - RNA, 2209 nt, Homo sapiens
  source 1..2209: mol_type = other RNA
tcaggccaggcacagtggctcatgcctataatcccagcagtttttgaagctgaggcaggaggatcccttgaggccaggagttcaagaccagcctgggcaatatagtgggacccagactgtataaaaattttgtttaaattagccaggggtggtggtgttcgcgtgtagtcccagatacttgggaggctgaggcaagaggatcacttgattctctgtttggaggatgttgaggccactgtcgcaccgctgttccagcctgggcgacagagtgagactctgtctctccacttgtctcaatactatagagctgaaacctttctcaccacttgatttagcttcaaattgatgtagtgtaattccttctccagctccacagcatataaaaaaagttctcgaaattcttcttgagtgacaggctggtagtcatcttgaatttccatagaataatactttttctcaagcctctctttccattttttcatctgctctgcgttttgaatctcattttcgtcaaagccttctcttctggcttgttcagccaaatctccgctgcctttggttttcttgtcttcatctttttgagctttcttcagtctgaatttctcgagaacatttttgtaactctgtttaatcattttgccaagttcaaaatctagccttctgcctattgaatagtcagctttcacttcagaataggtatcattaataattgccaagaacatattcagcaggacaaagaacacaaaaaagatgaaagtgatgaagtaaatgggtcccaagataggattggcttgctgaataccagcaaaattaaaatctccaagaacaattcgaaattgtgcaaatatggaattctgaaaagtggaaaagtcatcaacttgtgatccaaaaacaagaaatcctaactgggcataagcaaagaatattataaaaaacatgatggcaaatcctactatgtctttaacacaacgggacaaggttgatgacagctgagacattgtcttgttaaagcttatgaatttgaatatctttatccatgcaaaaaagatggtaatagcaattatattattgtaataaatgtgccagcatgcaagaaaatagaaatctgaatatttttcagtacttttcaacagctgtccaagtaagagaaaaatttgtacattatagtatgtgttgaaggaaacagccacaaaacacaacagcaaaagtagcaattctagccagttccaaatacttttgaaataggcagacttaaattcttttatttttttgacttcttgtgttgtgaagacaaaaagaaaaatacagaatgtgatttcacaggaagcaataaaatagtcatagtagctaacatatctgaggagcttcacagagtaaaactgccatgaagtaagtattcctccagttgcagggaattctgccaccaatctgataatacaaaatagatttacattagcattatataaggaaaaatcaataaaaataactctagtccctcttgtgatccagctgttcagtcgaaggtcaatgaacttgtttttggtttcagatttcgattttgataaagtgaaaatgtatcccccatttcggtaaacaccaagaaatccccagtgccaaggggagttggtattagaagtagaatatctccattcagtattaatttgaaggccaaaattagagaggtcttcatttgcagaagtatatttgccataacattcactcatcaaagactgaaaagatgaatagactttgcatgtgttgttgcggacttttagttgacgaactctgggaactcctagaagtatattttcatagtagatgcgactgctgttctttaaattatacagctgctggttattgtaccatgaatcccagtacagaccttccaaaaggggtccttccataaacttccaaaaatcagttatgctgcgaatggacttaaagttggttctttcttcaccaggcacagaagtgtccaaaaatagagatgacataaccttgtttaagtaatacatatgtgggtttaccatcccaaaagtcaatatacataggtttattaaaaaaataaagtagagtaacaattcctgaagtgtggttgtaatttctacttcctttctgtaatgcaacttatgtttcgaagccccgcctcggtgccaccgtgacgcctcagccatggcggacctgcactacaccgcccgttcgttcgcct

SEQ ID NO: 17492 - RNA, 1668 nt, Homo sapiens
  source 1..1668: mol_type = other RNA
tcaggccaggcacagtggctcatgcctataatcccggcactctgggaggccaaggcaggaggatcacttgagcccaggacttccagaccagcctgggcaacacagcgagacccccatctctacaaaaaatatttaaaaactagctgggcgtggtggcacatgtctgtagtctcagctactcaggaggctgaggactgcttgagcccgagaggtccaggctgcagtgagccatgatcgcaccactgcactccagcctggtgacagagcaagatcctgtctcaaaaaaagtaaataaataaaataaataaataaatcagctaattaaatcagggagatgccctccacctttccataagggtgggtaggtgattagagccttagcatccacatttcttcatctacaaaacagggcaaataccatcaacccaaggtgggggtggggggaggggcagtgaagactgagatgatacatttgacaaaaatgctatacaaatgttaattaattaattaaatgcaaagttcctcctggcccccaagggtagtataccattgctctcaggaaaaacattgtgaacctccctcctctcctggggctacagagccaggccctgcagacagcactggagaaccaaccctggttcctaactcaacactcccgactagtctggaagcagcaggaggaaggctggcttggtcatcctccctgctgccctgacagggaaagaagcaggcccagagaagcccagttaagtcaaagtcagggacagggggaccccagcctctggagcagaggcacccacggctccaacacatctcctgggctccaagcctcctcctcatgctgcacggctctgcttcagaaggttttcttctgaagcacttctcccctctgcctccttgcctgctctgagaggaatgggctgtgaaataaaccttccgaaattacatacttgaagttagccaaagagcatggaagtagccttccaaaagcttatccaactacgaatcacttctgctcaaaaaattaacaaatcaatgagaaaatctttagtgaaaagtttgagcagctgtaaggggagggggcattacactgggaacccgaatgtgtggtggctcttgcctgcgccctgcctctaaacaaccacataaccttaaacaagtcatttagcctggctgggcctcagtttcctcatcgaggaaatgggagggtgagataaaggatctgtgtgatcttttagtgtccctaagtcctgttttccgaggaaaggtgatccgcaccctattatccgggaactgccctccacttttctataaggcaaatgagtgcttcgagccttgacctctgcagccaggcagggaaacagagaactaaaatatgaagccaagagctgagaactgtgcgtcattcagcagttaagacaaaaactcttgaagctatgacttacgtgtgtggaggatgcaatttcatttacaattcttatttaagatacttgccagaaatacactcactacgaaacaaaatgctgtgggggcatcctgtagggaggtggaaaaggccttcttctgatggctcatcttagagccagggcggactgcaggcacgtgaacccagtcctgggcacccttcactgtctccaactctaatcctgagaggctcctacgagtcat

SEQ ID NO: 17493 - RNA, 8861 nt, Homo sapiens
  source 1..8861: mol_type = other RNA
tcaggccaggcacagtggctcatgcctataatcctagcactttgggaggcgaggcaggcagatcacttgaggtcagaagttcgagaccagcctgctcaacatggcgaaaccccgtctctattaaaaatacaaaaattagccaggcgtggtggtacacgtctgttaagtcccagctactcggagggtttaggcaggagaatcgcttgaacctcgggaggtagaggttgcagtgagttgagatcatgccactgcattccagcttgggcgacatagcaagactctgtctccaaaagacaagtaacttcccttttactattgtttctatcctcttctctgttctatcgtggggcaatggagggggcagtctctgttcgagacagatccacttcacactctgtcccattcattttgggggagacttttctcccttcttcccttttggactctttctggatggctgacattatcagagcctcggcacttgggctgtttgctattttttcccacccatctgtccaaactactttattcattcagggattataactggccacactacagaatgagaaggtagaaggtagaagaggaggaggggtgtcatttgtttcttgcctttctgcatgagctgcctcttagctgtcaatgaaggaacaaagcatggagtagggcatgaagacagggaccgagcagggcagagacagcactcccaacctattcacattgccctgtgggcccgagctagttctgccaagttttgatcaaaaagtcacctttgaaatggctaaaattaagcttttaaaaaatgttctaatgagaagggcttgaatccaaaaagaaagagaatgaaagaaagaaagagagagagagagggagagagggagggacggaaggaggaagagaagagaagagaagagaatctctgtaattggtgagatttaacaatcagagggacctcaacattcccttgtggaggctagggaggatgaggcttggagtctctgccacccttgctaacctgaatcacagtccctaggctcttcacataaaaggtggggcttgtgtcttccttggccaatcccctcattccactacctctgcctgccccaaaatgagctgcctaggctctttaagtggcactggtctgacactttggggagcaggccagagaccagggtgatgccctcacggtccccatcagaatcctgcctctgcccaccacccccaggaccaatccagactttgcctgagcctgaaggaacaggcaggaaaactggcgcagccaggaggaaaagggcctttatttccatacatcgggtaaacaggggagagcacagcccagtgagtacaaaccaattgcaggagagaaggggggcggcagatgggagcagcaccaggcactgcacttgggctcccaagtctggtggagttctcagggataacctttttagggtgggggctgggacctccagaccacatggtgttgtgtctgggataagtgtgtgggggcagggaggttggaagaatgacacgggctcaggacacagagtgaggactcatgtctaatgagcaccggccaaaacttccatcttcagtttttctgatcacaagtcctcaaccccaagccttccctctcaagttgagtttatggtccagaccacctggacagagcaggagggaggcagtgcttggatcagccctgaactgctgtagttggaatgggtttaccttaaataggtcattgcacataacacgctgagacaaagagggtggggtgggggctggaggtgcggatggtccacacacacacttgtctgcgtaggcttgctcaacccagcccagcagcaccggagagcccctccgcacctcattcttaagaacctggacccggctctcctcaccagcgtctccagctgcacagagaaaggactgctctctgaagggtgaagatggagatgacattcccgagtcgttcttgggagccccagctaccactacagccccctcccactctcagggatgcagctgtgatggagaggttgggtatttaaattaaaaagtagaaagacagcaggcaccaagaagagagagcccccaccccacacgagagggaaggcactgcttctcctcccccaatcctccccatggacccagcaacctagagtgtcccagtaggcaacctgtccaccgtccctgagcagggagctgagagggaggtcaacgtgctggctccatgcagtgccaggccacctgccactgcccacggtgacacagggtagaagccaagagtctggcattttgagacagaggagcaaaaagttctcttcagaaactcctctttcccccacctcttccacgtggagacatcagacacccatagcctggaaagtgcccctgacagaagaaggtcagggtgtttcccatgcagatcagcagtcgggtgggggagaccggtgccccaccacttcctgggagaggtgcccaggcagccacaggccctggggtgagagggctgccaaccactcccctgggctatgcgttagtctccgtcagcttggcctctgtgtcgctgtcactcagataactgtgggagtatcgcggtctggaggtgttgtcgagagggtcgtgctcatcatctgaccgatcaggggcaagggacttccagtagctggtggggctggaactctttaagctgccatcatcagaagctgccttggaaggtcccttgttttttgacaaccaggacttgaccccgtcaacacggtcctccagctccgagtccacatcagagtctccctcaagtttattctttcttttctgatactttgtcaccatgtcctgcaaactgttgatgaggtcctcattctcatcactctccatctcatcctcaatggcagcctgcaggtccccgatgcgcttgaatgccaactttaggtcagcctgcaggctctggttagcagcctccaggctttctagatccatctccagttcgtgcttcttgcggctcgcctcggcctccttcctggcaagctcgcccatctcctccttggtgtcccggagctgcctctgtagccgcttgttctgttccttctcccggttctcggctgcaatgcgctgatcccgctcctcagtcagcttctccatgttttccttgagacggctagccaggctctccagccgtttcacttgcgtcctttcaaactccaggcgtgtctccagctcccgtatcttagcttcctgcctgctcaccagggacttgtccaccatggactgctccaggaactccacctggctctggagggcttgtagcttctcctgcagctcctgcttctctttgttggcttcttctagctgagcttggagatcatttatctgagccaggtcccgggaagcctgagccacggcagccttgtgcttcttcatcaattcgttcatgtcttcctgatcttcctccagccggttctggatctcattcttctcacgctgaaggcggctcagctgctcctccagcgctgtcttggctttggcgatgtcatcaatctgcaggtgcaggtcttcgatctccacctccattgctttccgtgctttcacggctgccgcacaggtgaactctgactcctccagctggttcttgagctgggcaatctctcgcttgctgggagcactgttcttcaggtggtccagcatgagctgggcatctgccagcagggccttggtgcgcttcaggtccttccgcagccgcttctctgactcaaagtcccgccggttcacctggtcgctgagggtggcgagcttgccctccagctcccgcttctctcgcagaaccttctgcttgtcctcatactcttcctctagctgcacctccatctgttttaacttcttctgacacgactgccgggcctcctccacctcctcatcccgactctccatctccttagaatgggtctgtctcatccgctccatctccatctccagacgcagcttggcctgttccagcatctggatggtccctgcctgctcatccagctcttcttcctgatccttgactttggcctccaggtcccggagctgtttcttgaccttggccagagaagcctcatccttggactcttgggaagaaatgtcctggagctctgcctctagagacacaaccttctgggtgaaccctgcaatgtccatgtctttttcctctagttgctgcttcaggctgaaagcctcagcgaggagcatgtccttctcccgctgcagcttctcccgctgcagcttctcccgctgggcctcctcatgcgcctgcgagagctcactgtcaaacctcctctgcttcttctccagttcgtggttgcggacctgctggccctccaggtgcagcttggtgtcttgcagctcagccgtcagtcgctggcacttcttcttgagctgctgcagagcccgctgactctcctcactatctgcctgcaggtccccgagccgccgttccagctgcctcttgttctgctgctccacctccagcttgtcctcaaactcctgctggagccgtttcttggtgaagtccacctcccgcacagcccgctcatacttcagccgccactcgccacctgcatcatcatcatccacttccccgttgatctccgctgcccggatgagacgggcctccatcacctccatttccataacctccatctgcttcttcagtgcatcgtactgggtctgcagttccttcatctccttctcagcccggagcctctctgctgtctccgcgtccagcagctgggaggcggactctcctgtgttacgctcatctgtcagctccgatgtcagctctgagatccggctctccagccggtcactgttgagccgcagctcgttcctctccttctccgccttctcgagcttgctccgcagctgctggatctcctcgtctttgttccggatctgctcctctgacagctgtacttcgatgaggggcctcactgtggtaaaaagcttccaccagggccagtccttcacccctttgttcttcttgatgttcttctgtacacagcgaatggccaggtcctggatctttctcttcttgaagtgctggcgggccaggtagcccctgcaggctgcttggaacagggttaggttcctgctggtttgttcatcccgctgctcctccagccgtgccaaggtgcccgcccggaagaacacccggctcaggcccatgcagcagctgctcttctccagatccaagcactccagcagctcctccactgcccgcctttcatccaccacgatgtagttacgcccgtgtttcttggtcaggtgcggggccaggacatcaaagcggcggcggaactcggaaaacaccatgtggtcagggtaaccttggcggtacatgcgcatggcatcgagcaggcgggagccgcggagctgggtgcggagcaggggcacgtcgagctgcaggagcccagcctcgcagtggtctcccgagggcaggtccagctcactgctgctgctgactcggcgggaggaggcggaacggggctccccagcccagccctcagctacaggcaggaagcagtgcacaaaatgcagctttgacttcttgatggtgtcgatgagggcgtccacctgtagcttcatctggatgcacagtgacttctttttgacagccgccatgcctgtggtaaaggttttccgcatgctggtggcccggcgcagtgccagctgcgagccgccctccaggcccgcgatggagccagagagcaccgtggcactgcctgcgcggcccagaaacaggttgctgatgatttttttctgggagtcctgcaggagccggggggcattctgggtggctgggttctgcttggtgtagttcagccagccagtcacattgtactctacccagttggtgccatggctgtggcccaggagaaagtggtgtggtttgctgctgtgcagaagggggctttggccttttttgtcaccttcctgggggccataataggagaaaaggcgctccaggagggtgtcctcactggcccctggcaccagagcctcctcttccaatagccagagcaggcccctcgcctcgtctgtgcgggccagcgagcggaccagggactgatgggaggcctggtccacagcagccacagagtcatccgtcgggggttccaagtcgtcaaacgccagctcgatgttctcctccttgtatctttccaactcctgcacgaaggtgcgctcgtggaagagcctctgcagccggtcttgggtgtagttgtggcacagctcctcaaaggaggctccgcgggctgacccaccctgctcagggttctggaagcccggggtgtcgacaatcatcatggagcagagtgagtgctggctggacttgagagccctattcaccagggagacgagaagggtgaagagctcgctgtagaggccggccgccatgccctcaaggcactccagtgcactcagtttcgggcctgtcccatctcccaggccactctcctcggggccctggcggaaggaggtggagcgctgcagggtgccacccttgtgctggtgcttgaagatggctgaggacagctcctccaggctgcagcccagtaggtacgcagccttctgggcccactcatggcgggcaaactgcttgcgcccagcttcagcagcttctttggtggctcccgcagcccccaggtggtagatggcagccagaatgaaccagcaggccttctgttcatcgggggagatgcccagcaccttcatggccgcctgcagcttactaaactgctgagctgccttctgcttttcctcaggcttggccagtggcacaatcccaaacacattgttctctgccaagtggttgaggtggagctctgtcctgagggtgccatccccacaggccagcaggtagtagaagacgttgaatgtggcttcactggctgggcgccgagccacacgcagcttctccagaagcattgtctgaatggaggctgaggccacctggccagcttggtcaaagtccagggagaggatctgggagaagcgggtggcattgccattaatgatggtggggctgttcccaaaggcttccaggagggtgtacagagcctgccacttctccacagaaaacaccttgttcccgctgatgcccgcgatggtggccaggtactgcaccagatgctggcagctggtggtcttgccactgccactactgcccaggaggatgattgactgatcctgacggctcatcagcatcgccctgtatgcggtctgggccactgcatagatgtggggtgccatgtcctcccgccgacaacccttgaacatgtgcatcaccttctcagagtacacagcaggggccccacgggggccaagaaccagcaggctggggccagcatacgtgtgcagcaggctagcgccatagcgctggcgcaaggtgtgcaggacgctggactcattgaggtacaccagtgaggccagatcctccagacggtcgcaggagggagcattagccttctcaacgtcatcctcatccacatccaggatggccccatcgtggtccagcttcacacgcaccttcccctcaggcaagttgagctcctcagatttgagttgactggccagtgagaagccgtccctatggaccagccacaccttctccgtctcattccaggcctcttctgctgcaatctgttcttctgttttcgcatcggatggctccctgcgaggtccctcgccgctccgcagccagctcctgctgagctcgctgagctctggaatgggctgcaccttgagccgcacgctgtcccctgactgccggatcatctccacaatctcatccctggacttgctctccacattgtgcccattaatctccaccagtcgatctcctggcaccagccccagggccaggtccttggtgcctgcaccaggctcagcaaagtggaccacacgccgacaggcctggccctcggggccccgatccagcatggttgtgcgccgcagggagaagccaaagtctccagtgggccgtcgttgcagctccagctcccggagggtaggtgggggcaggggcaccacggggggcaggcgcaggtcgactgggaactttttagtcactagctcaggggctcgggatcggtgccctggtcgagggatgcctgggccaggatgctgcaccagctgtccctctagagtcctcacctccacctgtggcgagggggcggcagagtgctctgagggcgtcgaggtttctgaggcgctctcatcccggctacgctgggagaaggaaaagcgcttgacaatcatctgtgagttctgcttggccagtgagccgaacttggctgcccgctgcagcaccgagccacggaagctaccctcctcacccttgaggtcatcgctggagctggctgtacttaggtggcccgagtccaggatgacgctgccccggttactatcggagtcaatgtcagtcaggtgcaggtcagagccgctggccaccttgatggggatggggttggagatttccaggcgcgtcttggattcacgcttggaggagcggttcaggttgaagaagccacgtcgcaggctcatctcctccaggctccgaagctctgccgctgacatccgctcctttttctcctttttctccttcttctccttccgcccgccatctttgtccttgtctttcttcattaggttaaacatggtgggggtgctgtttgtaggggtagcacccccagaggattatgagtgcttagcacagggccttggtgccccactttgctgcggccaccggagcccgcccggcaggcagcagaagcggagacgcggcatccagcagcctcggcccggtcagggatggagcagagcgc

SEQ ID NO: 17494 - RNA, 8821 nt, Homo sapiens
  source 1..8821: mol_type = other RNA
tcaggccaggcacagtggctcatgcctataatcctagcactttgggaggcgaggcaggcagatcacttgaggtcagaagttcgagaccagcctgctcaacatggcgaaaccccgtctctattaaaaatacaaaaattagccaggcgtggtggtacacgtctgttaagtcccagctactcggagggtttaggcaggagaatcgcttgaacctcgggaggtagaggttgcagtgagttgagatcatgccactgcattccagcttgggcgacatagcaagactctgtctccaaaagacaagtaacttcccttttactattgtttctatcctcttctctgttctatcgtggggcaatggagggggcagtctctgttcgagacagatccacttcacactctgtcccattcattttgggggagacttttctcccttcttcccttttggactctttctggatggctgacattatcagagcctcggcacttgggctgtttgctattttttcccacccatctgtccaaactactttattcattcagggattataactggccacactacagaatgagaaggtagaaggtagaagaggaggaggggtgtcatttgtttcttgcctttctgcatgagctgcctcttagctgtcaatgaaggaacaaagcatggagtagggcatgaagacagggaccgagcagggcagagacagcactcccaacctattcacattgccctgtgggcccgagctagttctgccaagttttgatcaaaaagtcacctttgaaatggctaaaattaagcttttaaaaaatgttctaatgagaagggcttgaatccaaaaagaaagagaatgaaagaaagaaagagagagagagagggagagagggagggacggaaggaggaagagaagagaagagaagagaatctctgtaattggtgagatttaacaatcagagggacctcaacattcccttgtggaggctagggaggatgaggcttggagtctctgccacccttgctaacctgaatcacagtccctaggctcttcacataaaaggtggggcttgtgtcttccttggccaatcccctcattccactacctctgcctgccccaaaatgagctgcctaggctctttaagtggcactggtctgacactttggggagcaggccagagaccagggtgatgccctcacggtccccatcagaatcctgcctctgcccaccacccccaggaccaatccagactttgcctgagcctgaaggaacaggcaggaaaactggcgcagccaggaggaaaagggcctttatttccatacatcgggtaaacaggggagagcacagcccagtgagtacaaaccaattgcaggagagaaggggggcggcagatgggagcagcaccaggcactgcacttgggctcccaagtctggtggagttctcagggataacctttttagggtgggggctgggacctccagaccacatggtgttgtgtctgggataagtgtgtgggggcagggaggttggaagaatgacacgggctcaggacacagagtgaggactcatgtctaatgagcaccggccaaaacttccatcttcagtttttctgatcacaagtcctcaaccccaagccttccctctcaagttgagtttatggtccagaccacctggacagagcaggagggaggcagtgcttggatcagccctgaactgctgtagttggaatgggtttaccttaaataggtcattgcacataacacgctgagacaaagagggtggggtgggggctggaggtgcggatggtccacacacacacttgtctgcgtaggcttgctcaacccagcccagcagcaccggagagcccctccgcacctcattcttaagaacctggacccggctctcctcaccagcgtctccagctgcacagagaaaggactgctctctgaagggtgaagatggagatgacattcccgagtcgttcttgggagccccagctaccactacagccccctcccactctcagggatgcagctgtgatggagaggttgggtatttaaattaaaaagtagaaagacagcaggcaccaagaagagagagcccccaccccacacgagagggaaggcactgcttctcctcccccaatcctccccatggacccagcaacctagagtgtcccagtaggcaacctgtccaccgtccctgagcagggagctgagagggaggtcaacgtgctggctccatgcagtgccaggccacctgccactgcccacggtgacacagggtagaagccaagagtctggcattttgagacagaggagcaaaaagttctcttcagaaactcctctttcccccacctcttccacgtggagacatcagacacccatagcctggaaagtgcccctgacagaagaaggtcagggtgtttcccatgcagatcagcagtcgggtgggggagaccggtgccccaccacttcctgggagaggtgcccaggcagccacaggccctggggtgagagggctgccaaccactcccctgggctatgcgttagtctccgtcagcttggcctctgtgtcgctgtcactcagataactgtgggagtatcgcggtctggaggtgttgtcgagagggtcgtgctcatcatctgaccgatcaggggcaagggacttccagtagctggtggggctggaactctttaagctgccatcatcagaagctgccttggaaggtcccttgttttttgacaaccaggacttgaccccgtcaacacggtcctccagctccgagtccacatcagagtctccctcactgttgatgaggtcctcattctcatcactctccatctcatcctcaatggcagcctgcaggtccccgatgcgcttgaatgccaactttaggtcagcctgcaggctctggttagcagcctccaggctttctagatccatctccagttcgtgcttcttgcggctcgcctcggcctccttcctggcaagctcgcccatctcctccttggtgtcccggagctgcctctgtagccgcttgttctgttccttctcccggttctcggctgcaatgcgctgatcccgctcctcagtcagcttctccatgttttccttgagacggctagccaggctctccagccgtttcacttgcgtcctttcaaactccaggcgtgtctccagctcccgtatcttagcttcctgcctgctcaccagggacttgtccaccatggactgctccaggaactccacctggctctggagggcttgtagcttctcctgcagctcctgcttctctttgttggcttcttctagctgagcttggagatcatttatctgagccaggtcccgggaagcctgagccacggcagccttgtgcttcttcatcaattcgttcatgtcttcctgatcttcctccagccggttctggatctcattcttctcacgctgaaggcggctcagctgctcctccagcgctgtcttggctttggcgatgtcatcaatctgcaggtgcaggtcttcgatctccacctccattgctttccgtgctttcacggctgccgcacaggtgaactctgactcctccagctggttcttgagctgggcaatctctcgcttgctgggagcactgttcttcaggtggtccagcatgagctgggcatctgccagcagggccttggtgcgcttcaggtccttccgcagccgcttctctgactcaaagtcccgccggttcacctggtcgctgagggtggcgagcttgccctccagctcccgcttctctcgcagaaccttctgcttgtcctcatactcttcctctagctgcacctccatctgttttaactgttccagcatctggatggtccctgcctgctcatccagctcttcttcctgatccttgactttggcctccaggtcccggagctgtttcttgaccttggccagagaagcctcatccttggactcttgggaagaaatgtcctggagctctgcctctagagacacaaccttctgggtgaaccctgcaatgtccatgtctttttcctctagttgctgcttcaggctgaaagcctcagcgaggagcatgtccttctcccgctgcagcttctcccgctgcagcttctcccgctgggcctcctcatgcgcctgcgagagctcactgtcaaacctcctctgcttcttctccagttcgtggttgcggacctgctggccctccaggtgcagcttggtgtcttgcagctcagccgtcagtcgctggcacttcttcttgagctgctgcagagcccgctgactctcctcactatctgcctgcaggtccccgagccgccgttccagctgcctcttgttctgctgctccacctccagcttgtcctcaaactcctgctggagccgtttcttggtgaagtccacctcccgcacagcccgctcatacttcagccgccactcgccacctgcatcatcatcatccacttccccgttgatctccgctgcccggatgagacgggcctccatcacctccatttccataacctccatctgcttcttcagtgcatcgtactgggtctgcagttccttcatctccttctcagcccggagcctctctgctgtctccgcgtccagcagctgggaggcggactctcctgtgttacgctcatctgtcagctccgatgtcagctctgagatccggctctccagccggtcactgttgagccgcagctcgttcctctccttctccgccttctcgagcttgctccgcagctgctggatctcctcgtctttgttccggatctgctcctctgacagctgtacttcgatgaggggcctcactgtggtaaaaagcttccaccagggccagtccttcacccctttgttcttcttgatgttcttctgtacacagcgaatggccaggtcctggatctttctcttcttgaagtgctggcgggccaggtagcccctgcaggctgcttggaacagggttaggttcctgctggtttgttcatcccgctgctcctccagccgtgccaaggtgcccgcccggaagaacacccggctcaggcccatgcagcagctgctcttctccagatccaagcactccagcagctcctccactgcccgcctttcatccaccacgatgtagttacgcccgtgtttcttggtcaggtgcggggccaggacatcaaagcggcggcggaactcggaaaacaccatgtggtcagggtaaccttggcggtacatgcgcatggcatcgagcaggcgggagccgcggagctgggtgcggagcaggggcacgtcgagctgcaggagcccagcctcgcagtggtctcccgagggcaggtccagctcactgctgctgctgactcggcgggaggaggcggaacggggctccccagcccagccctcagctacaggcaggaagcagtgcacaaaatgcagctttgacttcttgatggtgtcgatgagggcgtccacctgtagcttcatctggatgcacagtgacttctttttgacagccgccatgcctgtggtaaaggttttccgcatgctggtggcccggcgcagtgccagctgcgagccgccctccaggcccgcgatggagccagagagcaccgtggcactgcctgcgcggcccagaaacaggttgctgatgatttttttctgggagtcctgcaggagccggggggcattctgggtggctgggttctgcttggtgtagttcagccagccagtcacattgtactctacccagttggtgccatggctgtggcccaggagaaagtggtgtggtttgctgctgtgcagaagggggctttggccttttttgtcaccttcctgggggccataataggagaaaaggcgctccaggagggtgtcctcactggcccctggcaccagagcctcctcttccaatagccagagcaggcccctcgcctcgtctgtgcgggccagcgagcggaccagggactgatgggaggcctggtccacagcagccacagagtcatccgtcgggggttccaagtcgtcaaacgccagctcgatgttctcctccttgtatctttccaactcctgcacgaaggtgcgctcgtggaagagcctctgcagccggtcttgggtgtagttgtggcacagctcctcaaaggaggctccgcgggctgacccaccctgctcagggttctggaagcccggggtgtcgacaatcatcatggagcagagtgagtgctggctggacttgagagccctattcaccagggagacgagaagggtgaagagctcgctgtagaggccggccgccatgccctcaaggcactccagtgcactcagtttcgggcctgtcccatctcccaggccactctcctcggggccctggcggaaggaggtggagcgctgcagggtgccacccttgtgctggtgcttgaagatggctgaggacagctcctccaggctgcagcccagtaggtacgcagccttctgggcccactcatggcgggcaaactgcttgcgcccagcttcagcagcttctttggtggctcccgcagcccccaggtggtagatggcagccagaatgaaccagcaggccttctgttcatcgggggagatgcccagcaccttcatggccgcctgcagcttactaaactgctgagctgccttctgcttttcctcaggcttggccagtggcacaatcccaaacacattgttctctgccaagtggttgaggtggagctctgtcctgagggtgccatccccacaggccagcaggtagtagaagacgttgaatgtggcttcactggctgggcgccgagccacacgcagcttctccagaagcattgtctgaatggaggctgaggccacctggccagcttggtcaaagtccagggagaggatctgggagaagcgggtggcattgccattaatgatggtggggctgttcccaaaggcttccaggagggtgtacagagcctgccacttctccacagaaaacaccttgttcccgctgatgcccgcgatggtggccaggtactgcaccagatgctggcagctggtggtcttgccactgccactactgcccaggaggatgattgactgatcctgacggctcatcagcatcgccctgtatgcggtctgggccactgcatagatgtggggtgccatgtcctcccgccgacaacccttgaacatgtgcatcaccttctcagagtacacagcaggggccccacgggggccaagaaccagcaggctggggccagcatacgtgtgcagcaggctagcgccatagcgctggcgcaaggtgtgcaggacgctggactcattgaggtacaccagtgaggccagatcctccagacggtcgcaggagggagcattagccttctcaacgtcatcctcatccacatccaggatggccccatcgtggtccagcttcacacgcaccttcccctcaggcaagttgagctcctcagatttgagttgactggccagtgagaagccgtccctatggaccagccacaccttctccgtctcattccaggcctcttctgctgcaatctgttcttctgttttcgcatcggatggctccctgcgaggtccctcgccgctccgcagccagctcctgctgagctcgctgagctctggaatgggctgcaccttgagccgcacgctgtcccctgactgccggatcatctccacaatctcatccctggacttgctctccacattgtgcccattaatctccaccagtcgatctcctggcaccagccccagggccaggtccttggtgcctgcaccaggctcagcaaagtggaccacacgccgacaggcctggccctcggggccccgatccagcatggttgtgcgccgcagggagaagccaaagtctccagtgggccgtcgttgcagctccagctcccggagggtaggtgggggcaggggcaccacggggggcaggcgcaggtcgactgggaactttttagtcactagctcaggggctcgggatcggtgccctggtcgagggatgcctgggccaggatgctgcaccagctgtccctctagagtcctcacctccacctgtggcgagggggcggcagagtgctctgagggcgtcgaggtttctgaggcgctctcatcccggctacgctgggagaaggaaaagcgcttgacaatcatctgtgagttctgcttggccagtgagccgaacttggctgcccgctgcagcaccgagccacggaagctaccctcctcacccttgaggtcatcgctggagctggctgtacttaggtggcccgagtccaggatgacgctgccccggttactatcggagtcaatgtcagtcaggtgcaggtcagagccgctggccaccttgatggggatggggttggagatttccaggcgcgtcttggattcacgcttggaggagcggttcaggttgaagaagccacgtcgcaggctcatctcctccaggctccgaagctctgccgctgacatccgctcctttttctcctttttctccttcttctccttccgcccgccatctttgtccttgtctttcttcattaggttaaacatggtgggggtgctgtttgtaggggtagcacccccagaggattatgagtgcttagcacagggccttggtgccccactttgctgctccctgagcggccgtttcctccagccccgggaccccggctctctccccgcgctctgcccctcgccaagggttgtagcagcggccggaggggtagccagcacctggcctggccccgtgctccagggggagcctcctcccggccggctgtgctgagctccgcagcgccgggtgactccctgccaggtcacacggagcttatct

SEQ ID NO: 17495 - RNA, 8873 nt, Homo sapiens
  source 1..8873: mol_type = other RNA
tcaggccaggcacagtggctcatgcctataatcctagcactttgggaggcgaggcaggcagatcacttgaggtcagaagttcgagaccagcctgctcaacatggcgaaaccccgtctctattaaaaatacaaaaattagccaggcgtggtggtacacgtctgttaagtcccagctactcggagggtttaggcaggagaatcgcttgaacctcgggaggtagaggttgcagtgagttgagatcatgccactgcattccagcttgggcgacatagcaagactctgtctccaaaagacaagtaacttcccttttactattgtttctatcctcttctctgttctatcgtggggcaatggagggggcagtctctgttcgagacagatccacttcacactctgtcccattcattttgggggagacttttctcccttcttcccttttggactctttctggatggctgacattatcagagcctcggcacttgggctgtttgctattttttcccacccatctgtccaaactactttattcattcagggattataactggccacactacagaatgagaaggtagaaggtagaagaggaggaggggtgtcatttgtttcttgcctttctgcatgagctgcctcttagctgtcaatgaaggaacaaagcatggagtagggcatgaagacagggaccgagcagggcagagacagcactcccaacctattcacattgccctgtgggcccgagctagttctgccaagttttgatcaaaaagtcacctttgaaatggctaaaattaagcttttaaaaaatgttctaatgagaagggcttgaatccaaaaagaaagagaatgaaagaaagaaagagagagagagagggagagagggagggacggaaggaggaagagaagagaagagaagagaatctctgtaattggtgagatttaacaatcagagggacctcaacattcccttgtggaggctagggaggatgaggcttggagtctctgccacccttgctaacctgaatcacagtccctaggctcttcacataaaaggtggggcttgtgtcttccttggccaatcccctcattccactacctctgcctgccccaaaatgagctgcctaggctctttaagtggcactggtctgacactttggggagcaggccagagaccagggtgatgccctcacggtccccatcagaatcctgcctctgcccaccacccccaggaccaatccagactttgcctgagcctgaaggaacaggcaggaaaactggcgcagccaggaggaaaagggcctttatttccatacatcgggtaaacaggggagagcacagcccagtgagtacaaaccaattgcaggagagaaggggggcggcagatgggagcagcaccaggcactgcacttgggctcccaagtctggtggagttctcagggataacctttttagggtgggggctgggacctccagaccacatggtgttgtgtctgggataagtgtgtgggggcagggaggttggaagaatgacacgggctcaggacacagagtgaggactcatgtctaatgagcaccggccaaaacttccatcttcagtttttctgatcacaagtcctcaaccccaagccttccctctcaagttgagtttatggtccagaccacctggacagagcaggagggaggcagtgcttggatcagccctgaactgctgtagttggaatgggtttaccttaaataggtcattgcacataacacgctgagacaaagagggtggggtgggggctggaggtgcggatggtccacacacacacttgtctgcgtaggcttgctcaacccagcccagcagcaccggagagcccctccgcacctcattcttaagaacctggacccggctctcctcaccagcgtctccagctgcacagagaaaggactgctctctgaagggtgaagatggagatgacattcccgagtcgttcttgggagccccagctaccactacagccccctcccactctcagggatgcagctgtgatggagaggttgggtatttaaattaaaaagtagaaagacagcaggcaccaagaagagagagcccccaccccacacgagagggaaggcactgcttctcctcccccaatcctccccatggacccagcaacctagagtgtcccagtaggcaacctgtccaccgtccctgagcagggagctgagagggaggtcaacgtgctggctccatgcagtgccaggccacctgccactgcccacggtgacacagggtagaagccaagagtctggcattttgagacagaggagcaaaaagttctcttcagaaactcctctttcccccacctcttccacgtggagacatcagacacccatagcctggaaagtgcccctgacagaagaaggtcagggtgtttcccatgcagatcagcagtcgggtgggggagaccggtgccccaccacttcctgggagaggtgcccaggcagccacaggccctggggtgagagggctgccaaccactcccctgggctatgcgttagtctccgtcagcttggcctctgtgtcgctgtcactcagataactgtgggagtatcgcggtctggaggtgttgtcgagagggtcgtgctcatcatctgaccgatcaggggcaagggacttccagtagctggtggggctggaactctttaagctgccatcatcagaagctgccttggaaggtcccttgttttttgacaaccaggacttgaccccgtcaacacggtcctccagctccgagtccacatcagagtctccctcactgttgatgaggtcctcattctcatcactctccatctcatcctcaatggcagcctgcaggtccccgatgcgcttgaatgccaactttaggtcagcctgcaggctctggttagcagcctccaggctttctagatccatctccagttcgtgcttcttgcggctcgcctcggcctccttcctggcaagctcgcccatctcctccttggtgtcccggagctgcctctgtagccgcttgttctgttccttctcccggttctcggctgcaatgcgctgatcccgctcctcagtcagcttctccatgttttccttgagacggctagccaggctctccagccgtttcacttgcgtcctttcaaactccaggcgtgtctccagctcccgtatcttagcttcctgcctgctcaccagggacttgtccaccatggactgctccaggaactccacctggctctggagggcttgtagcttctcctgcagctcctgcttctctttgttggcttcttctagctgagcttggagatcatttatctgagccaggtcccgggaagcctgagccacggcagccttgtgcttcttcatcaattcgttcatgtcttcctgatcttcctccagccggttctggatctcattcttctcacgctgaaggcggctcagctgctcctccagcgctgtcttggctttggcgatgtcatcaatctgcaggtgcaggtcttcgatctccacctccattgctttccgtgctttcacggctgccgcacaggtgaactctgactcctccagctggttcttgagctgggcaatctctcgcttgctgggagcactgttcttcaggtggtccagcatgagctgggcatctgccagcagggccttggtgcgcttcaggtccttccgcagccgcttctctgactcaaagtcccgccggttcacctggtcgctgagggtggcgagcttgccctccagctcccgcttctctcgcagaaccttctgcttgtcctcatactcttcctctagctgcacctccatctgttttaacttcttctgacacgactgccgggcctcctccacctcctcatcccgactctccatctccttagaatgggtctgtctcatccgctccatctccatctccagacgcagcttggcctgttccagcatctggatggtccctgcctgctcatccagctcttcttcctgatccttgactttggcctccaggtcccggagctgtttcttgaccttggccagagaagcctcatccttggactcttgggaagaaatgtcctggagctctgcctctagagacacaaccttctgggtgaaccctgcaatgtccatgtctttttcctctagttgctgcttcaggctgaaagcctcagcgaggagcatgtccttctcccgctgcagcttctcccgctgcagcttctcccgctgggcctcctcatgcgcctgcgagagctcactgtcaaacctcctctgcttcttctccagttcgtggttgcggacctgctggccctccaggtgcagcttggtgtcttgcagctcagccgtcagtcgctggcacttcttcttgagctgctgcagagcccgctgactctcctcactatctgcctgcaggtccccgagccgccgttccagctgcctcttgttctgctgctccacctccagcttgtcctcaaactcctgctggagccgtttcttggtgaagtccacctcccgcacagcccgctcatacttcagccgccactcgccacctgcatcatcatcatccacttccccgttgatctccgctgcccggatgagacgggcctccatcacctccatttccataacctccatctgcttcttcagtgcatcgtactgggtctgcagttccttcatctccttctcagcccggagcctctctgctgtctccgcgtccagcagctgggaggcggactctcctgtgttacgctcatctgtcagctccgatgtcagctctgagatccggctctccagccggtcactgttgagccgcagctcgttcctctccttctccgccttctcgagcttgctccgcagctgctggatctcctcgtctttgttccggatctgctcctctgacagctgtacttcgatgaggggcctcactgtggtaaaaagcttccaccagggccagtccttcacccctttgttcttcttgatgttcttctgtacacagcgaatggccaggtcctggatctttctcttcttgaagtgctggcgggccaggtagcccctgcaggctgcttggaacagggttaggttcctgctggtttgttcatcccgctgctcctccagccgtgccaaggtgcccgcccggaagaacacccggctcaggcccatgcagcagctgctcttctccagatccaagcactccagcagctcctccactgcccgcctttcatccaccacgatgtagttacgcccgtgtttcttggtcaggtgcggggccaggacatcaaagcggcggcggaactcggaaaacaccatgtggtcagggtaaccttggcggtacatgcgcatggcatcgagcaggcgggagccgcggagctgggtgcggagcaggggcacgtcgagctgcaggagcccagcctcgcagtggtctcccgagggcaggtccagctcactgctgctgctgactcggcgggaggaggcggaacggggctccccagcccagccctcagctacaggcaggaagcagtgcacaaaatgcagctttgacttcttgatggtgtcgatgagggcgtccacctgtagcttcatctggatgcacagtgacttctttttgacagccgccatgcctgtggtaaaggttttccgcatgctggtggcccggcgcagtgccagctgcgagccgccctccaggcccgcgatggagccagagagcaccgtggcactgcctgcgcggcccagaaacaggttgctgatgatttttttctgggagtcctgcaggagccggggggcattctgggtggctgggttctgcttggtgtagttcagccagccagtcacattgtactctacccagttggtgccatggctgtggcccaggagaaagtggtgtggtttgctgctgtgcagaagggggctttggccttttttgtcaccttcctgggggccataataggagaaaaggcgctccaggagggtgtcctcactggcccctggcaccagagcctcctcttccaatagccagagcaggcccctcgcctcgtctgtgcgggccagcgagcggaccagggactgatgggaggcctggtccacagcagccacagagtcatccgtcgggggttccaagtcgtcaaacgccagctcgatgttctcctccttgtatctttccaactcctgcacgaaggtgcgctcgtggaagagcctctgcagccggtcttgggtgtagttgtggcacagctcctcaaaggaggctccgcgggctgacccaccctgctcagggttctggaagcccggggtgtcgacaatcatcatggagcagagtgagtgctggctggacttgagagccctattcaccagggagacgagaagggtgaagagctcgctgtagaggccggccgccatgccctcaaggcactccagtgcactcagtttcgggcctgtcccatctcccaggccactctcctcggggccctggcggaaggaggtggagcgctgcagggtgccacccttgtgctggtgcttgaagatggctgaggacagctcctccaggctgcagcccagtaggtacgcagccttctgggcccactcatggcgggcaaactgcttgcgcccagcttcagcagcttccgcttgctcctcgggggcctctttggtggctcccgcagcccccaggtggtagatggcagccagaatgaaccagcaggccttctgttcatcgggggagatgcccagcaccttcatggccgcctgcagcttactaaactgctgagctgccttctgcttttcctcaggcttggccagtggcacaatcccaaacacattgttctctgccaagtggttgaggtggagctctgtcctgagggtgccatccccacaggccagcaggtagtagaagacgttgaatgtggcttcactggctgggcgccgagccacacgcagcttctccagaagcattgtctgaatggaggctgaggccacctggccagcttggtcaaagtccagggagaggatctgggagaagcgggtggcattgccattaatgatggtggggctgttcccaaaggcttccaggagggtgtacagagcctgccacttctccacagaaaacaccttgttcccgctgatgcccgcgatggtggccaggtactgcaccagatgctggcagctggtggtcttgccactgccactactgcccaggaggatgattgactgatcctgacggctcatcagcatcgccctgtatgcggtctgggccactgcatagatgtggggtgccatgtcctcccgccgacaacccttgaacatgtgcatcaccttctcagagtacacagcaggggccccacgggggccaagaaccagcaggctggggccagcatacgtgtgcagcaggctagcgccatagcgctggcgcaaggtgtgcaggacgctggactcattgaggtacaccagtgaggccagatcctccagacggtcgcaggagggagcattagccttctcaacgtcatcctcatccacatccaggatggccccatcgtggtccagcttcacacgcaccttcccctcaggcaagttgagctcctcagatttgagttgactggccagtgagaagccgtccctatggaccagccacaccttctccgtctcattccaggcctcttctgctgcaatctgttcttctgttttcgcctggctgtgggcatgagaggcggcctcagagtccagatcggatggctccctgcgaggtccctcgccgctccgcagccagctcctgctgagctcgctgagctctggaatgggctgcaccttgagccgcacgctgtcccctgactgccggatcatctccacaatctcatccctggacttgctctccacattgtgcccattaatctccaccagtcgatctcctggcaccagccccagggccaggtccttggtgcctgcaccaggctcagcaaagtggaccacacgccgacaggcctggccctcggggccccgatccagcatggttgtgcgccgcagggagaagccaaagtctccagtgggccgtcgttgcagctccagctcccggagggtaggtgggggcaggggcaccacggggggcaggcgcaggtcgactgggaactttttagtcactagctcaggggctcgggatcggtgccctggtcgagggatgcctgggccaggatgctgcaccagctgtccctctagagtcctcacctccacctgtggcgagggggcggcagagtgctctgagggcgtcgaggtttctgaggcgctctcatcccggctacgctgggagaaggaaaagcgcttgacaatcatctgtgagttctgcttggccagtgagccgaacttggctgcccgctgcagcaccgagccacggaagctaccctcctcacccttgaggtcatcgctggagctggctgtacttaggtggcccgagtccaggatgacgctgccccggttactatcggagtcaatgtcagtcaggtgcaggtcagagccgctggccaccttgatggggatggggttggagatttccaggcgcgtcttggattcacgcttggaggagcggttcaggttgaagaagccacgtcgcaggctcatctcctccaggctccgaagctctgccgctgacatccgctcctttttctcctttttctccttcttctccttccgcccgccatctttgtccttgtctttcttcattaggttaaacatggtgggggtgctgtttgtaggggtagcacccccagaggattatgagtgcttagcacagggccttggtgccccactttgctgcggccaccggagcccgcccggcaggcagcagaagcggagacgcggcatccagcagcctcggcccggtcagggatggagcagagcgc

SEQ ID NO: 17496 - RNA, 8816 nt, Homo sapiens
  source 1..8816: mol_type = other RNA
tcaggccaggcacagtggctcatgcctataatcctagcactttgggaggcgaggcaggcagatcacttgaggtcagaagttcgagaccagcctgctcaacatggcgaaaccccgtctctattaaaaatacaaaaattagccaggcgtggtggtacacgtctgttaagtcccagctactcggagggtttaggcaggagaatcgcttgaacctcgggaggtagaggttgcagtgagttgagatcatgccactgcattccagcttgggcgacatagcaagactctgtctccaaaagacaagtaacttcccttttactattgtttctatcctcttctctgttctatcgtggggcaatggagggggcagtctctgttcgagacagatccacttcacactctgtcccattcattttgggggagacttttctcccttcttcccttttggactctttctggatggctgacattatcagagcctcggcacttgggctgtttgctattttttcccacccatctgtccaaactactttattcattcagggattataactggccacactacagaatgagaaggtagaaggtagaagaggaggaggggtgtcatttgtttcttgcctttctgcatgagctgcctcttagctgtcaatgaaggaacaaagcatggagtagggcatgaagacagggaccgagcagggcagagacagcactcccaacctattcacattgccctgtgggcccgagctagttctgccaagttttgatcaaaaagtcacctttgaaatggctaaaattaagcttttaaaaaatgttctaatgagaagggcttgaatccaaaaagaaagagaatgaaagaaagaaagagagagagagagggagagagggagggacggaaggaggaagagaagagaagagaagagaatctctgtaattggtgagatttaacaatcagagggacctcaacattcccttgtggaggctagggaggatgaggcttggagtctctgccacccttgctaacctgaatcacagtccctaggctcttcacataaaaggtggggcttgtgtcttccttggccaatcccctcattccactacctctgcctgccccaaaatgagctgcctaggctctttaagtggcactggtctgacactttggggagcaggccagagaccagggtgatgccctcacggtccccatcagaatcctgcctctgcccaccacccccaggaccaatccagactttgcctgagcctgaaggaacaggcaggaaaactggcgcagccaggaggaaaagggcctttatttccatacatcgggtaaacaggggagagcacagcccagtgagtacaaaccaattgcaggagagaaggggggcggcagatgggagcagcaccaggcactgcacttgggctcccaagtctggtggagttctcagggataacctttttagggtgggggctgggacctccagaccacatggtgttgtgtctgggataagtgtgtgggggcagggaggttggaagaatgacacgggctcaggacacagagtgaggactcatgtctaatgagcaccggccaaaacttccatcttcagtttttctgatcacaagtcctcaaccccaagccttccctctcaagttgagtttatggtccagaccacctggacagagcaggagggaggcagtgcttggatcagccctgaactgctgtagttggaatgggtttaccttaaataggtcattgcacataacacgctgagacaaagagggtggggtgggggctggaggtgcggatggtccacacacacacttgtctgcgtaggcttgctcaacccagcccagcagcaccggagagcccctccgcacctcattcttaagaacctggacccggctctcctcaccagcgtctccagctgcacagagaaaggactgctctctgaagggtgaagatggagatgacattcccgagtcgttcttgggagccccagctaccactacagccccctcccactctcagggatgcagctgtgatggagaggttgggtatttaaattaaaaagtagaaagacagcaggcaccaagaagagagagcccccaccccacacgagagggaaggcactgcttctcctcccccaatcctccccatggacccagcaacctagagtgtcccagtaggcaacctgtccaccgtccctgagcagggagctgagagggaggtcaacgtgctggctccatgcagtgccaggccacctgccactgcccacggtgacacagggtagaagccaagagtctggcattttgagacagaggagcaaaaagttctcttcagaaactcctctttcccccacctcttccacgtggagacatcagacacccatagcctggaaagtgcccctgacagaagaaggtcagggtgtttcccatgcagatcagcagtcgggtgggggagaccggtgccccaccacttcctgggagaggtgcccaggcagccacaggccctggggtgagagggctgccaaccactcccctgggctatgcgttagtctccgtcagcttggcctctgtgtcgctgtcactcagataactgtgggagtatcgcggtctggaggtgttgtcgagagggtcgtgctcatcatctgaccgatcaggggcaagggacttccagtagctggtggggctggaactctttaagctgccatcatcagaagctgccttggaaggtcccttgttttttgacaaccaggacttgaccccgtcaacacggtcctccagctccgagtccacatcagagtctccctcactgttgatgaggtcctcattctcatcactctccatctcatcctcaatggcagcctgcaggtccccgatgcgcttgaatgccaactttaggtcagcctgcaggctctggttagcagcctccaggctttctagatccatctccagttcgtgcttcttgcggctcgcctcggcctccttcctggcaagctcgcccatctcctccttggtgtcccggagctgcctctgtagccgcttgttctgttccttctcccggttctcggctgcaatgcgctgatcccgctcctcagtcagcttctccatgttttccttgagacggctagccaggctctccagccgtttcacttgcgtcctttcaaactccaggcgtgtctccagctcccgtatcttagcttcctgcctgctcaccagggacttgtccaccatggactgctccaggaactccacctggctctggagggcttgtagcttctcctgcagctcctgcttctctttgttggcttcttctagctgagcttggagatcatttatctgagccaggtcccgggaagcctgagccacggcagccttgtgcttcttcatcaattcgttcatgtcttcctgatcttcctccagccggttctggatctcattcttctcacgctgaaggcggctcagctgctcctccagcgctgtcttggctttggcgatgtcatcaatctgcaggtgcaggtcttcgatctccacctccattgctttccgtgctttcacggctgccgcacaggtgaactctgactcctccagctggttcttgagctgggcaatctctcgcttgctgggagcactgttcttcaggtggtccagcatgagctgggcatctgccagcagggccttggtgcgcttcaggtccttccgcagccgcttctctgactcaaagtcccgccggttcacctggtcgctgagggtggcgagcttgccctccagctcccgcttctctcgcagaaccttctgcttgtcctcatactcttcctctagctgcacctccatctgttttaacttcttctgacacgactgccgggcctcctccacctcctcatcccgactctccatctccttagaatgggtctgtctcatccgctccatctccatctccagacgcagcttggcctgttccagcatctggatggtccctgcctgctcatccagctcttcttcctgatccttgactttggcctccaggtcccggagctgtttcttgaccttggccagagaagcctcatccttggactcttgggaagaaatgtcctggagctctgcctctagagacacaaccttctgggtgaaccctgcaatgtccatgtctttttcctctagttgctgcttcaggctgaaagcctcagcgaggagcatgtccttctcccgctgcagcttctcccgctgcagcttctcccgctgggcctcctcatgcgcctgcgagagctcactgtcaaacctcctctgcttcttctccagttcgtggttgcggacctgctggccctccaggtgcagcttggtgtcttgcagctcagccgtcagtcgctggcacttcttcttgagctgctgcagagcccgctgactctcctcactatctgcctgcaggtccccgagccgccgttccagctgcctcttgttctgctgctccacctccagcttgtcctcaaactcctgctggagccgtttcttggtgaagtccacctcccgcacagcccgctcatacttcagccgccactcgccacctgcatcatcatcatccacttccccgttgatctccgctgcccggatgagacgggcctccatcacctccatttccataacctccatctgcttcttcagtgcatcgtactgggtctgcagttccttcatctccttctcagcccggagcctctctgctgtctccgcgtccagcagctgggaggcggactctcctgtgttacgctcatctgtcagctccgatgtcagctctgagatccggctctccagccggtcactgttgagccgcagctcgttcctctccttctccgccttctcgagcttgctccgcagctgctggatctcctcgtctttgttccggatctgctcctctgacagctgtacttcgatgaggggcctcactgtggtaaaaagcttccaccagggccagtccttcacccctttgttcttcttgatgttcttctgtacacagcgaatggccaggtcctggatctttctcttcttgaagtgctggcgggccaggtagcccctgcaggctgcttggaacagggttaggttcctgctggtttgttcatcccgctgctcctccagccgtgccaaggtgcccgcccggaagaacacccggctcaggcccatgcagcagctgctcttctccagatccaagcactccagcagctcctccactgcccgcctttcatccaccacgatgtagttacgcccgtgtttcttggtcaggtgcggggccaggacatcaaagcggcggcggaactcggaaaacaccatgtggtcagggtaaccttggcggtacatgcgcatggcatcgagcaggcgggagccgcggagctgggtgcggagcaggggcacgtcgagctgcaggagcccagcctcgcagtggtctcccgagggcaggtccagctcactgctgctgctgactcggcgggaggaggcggaacggggctccccagcccagccctcagctacaggcaggaagcagtgcacaaaatgcagctttgacttcttgatggtgtcgatgagggcgtccacctgtagcttcatctggatgcacagtgacttctttttgacagccgccatgcctgtggtaaaggttttccgcatgctggtggcccggcgcagtgccagctgcgagccgccctccaggcccgcgatggagccagagagcaccgtggcactgcctgcgcggcccagaaacaggttgctgatgatttttttctgggagtcctgcaggagccggggggcattctgggtggctgggttctgcttggtgtagttcagccagccagtcacattgtactctacccagttggtgccatggctgtggcccaggagaaagtggtgtggtttgctgctgtgcagaagggggctttggccttttttgtcaccttcctgggggccataataggagaaaaggcgctccaggagggtgtcctcactggcccctggcaccagagcctcctcttccaatagccagagcaggcccctcgcctcgtctgtgcgggccagcgagcggaccagggactgatgggaggcctggtccacagcagccacagagtcatccgtcgggggttccaagtcgtcaaacgccagctcgatgttctcctccttgtatctttccaactcctgcacgaaggtgcgctcgtggaagagcctctgcagccggtcttgggtgtagttgtggcacagctcctcaaaggaggctccgcgggctgacccaccctgctcagggttctggaagcccggggtgtcgacaatcatcatggagcagagtgagtgctggctggacttgagagccctattcaccagggagacgagaagggtgaagagctcgctgtagaggccggccgccatgccctcaaggcactccagtgcactcagtttcgggcctgtcccatctcccaggccactctcctcggggccctggcggaaggaggtggagcgctgcagggtgccacccttgtgctggtgcttgaagatggctgaggacagctcctccaggctgcagcccagtaggtacgcagccttctgggcccactcatggcgggcaaactgcttgcgcccagcttcagcagcttctttggtggctcccgcagcccccaggtggtagatggcagccagaatgaaccagcaggccttctgttcatcgggggagatgcccagcaccttcatggccgcctgcagcttactaaactgctgagctgccttctgcttttcctcaggcttggccagtggcacaatcccaaacacattgttctctgccaagtggttgaggtggagctctgtcctgagggtgccatccccacaggccagcaggtagtagaagacgttgaatgtggcttcactggctgggcgccgagccacacgcagcttctccagaagcattgtctgaatggaggctgaggccacctggccagcttggtcaaagtccagggagaggatctgggagaagcgggtggcattgccattaatgatggtggggctgttcccaaaggcttccaggagggtgtacagagcctgccacttctccacagaaaacaccttgttcccgctgatgcccgcgatggtggccaggtactgcaccagatgctggcagctggtggtcttgccactgccactactgcccaggaggatgattgactgatcctgacggctcatcagcatcgccctgtatgcggtctgggccactgcatagatgtggggtgccatgtcctcccgccgacaacccttgaacatgtgcatcaccttctcagagtacacagcaggggccccacgggggccaagaaccagcaggctggggccagcatacgtgtgcagcaggctagcgccatagcgctggcgcaaggtgtgcaggacgctggactcattgaggtacaccagtgaggccagatcctccagacggtcgcaggagggagcattagccttctcaacgtcatcctcatccacatccaggatggccccatcgtggtccagcttcacacgcaccttcccctcaggcaagttgagctcctcagatttgagttgactggccagtgagaagccgtccctatggaccagccacaccttctccgtctcattccaggcctcttctgctgcaatctgttcttctgttttcgcatcggatggctccctgcgaggtccctcgccgctccgcagccagctcctgctgagctcgctgagctctggaatgggctgcaccttgagccgcacgctgtcccctgactgccggatcatctccacaatctcatccctggacttgctctccacattgtgcccattaatctccaccagtcgatctcctggcaccagccccagggccaggtccttggtgcctgcaccaggctcagcaaagtggaccacacgccgacaggcctggccctcggggccccgatccagcatggttgtgcgccgcagggagaagccaaagtctccagtgggccgtcgttgcagctccagctcccggagggtaggtgggggcaggggcaccacggggggcaggcgcaggtcgactgggaactttttagtcactagctcaggggctcgggatcggtgccctggtcgagggatgcctgggccaggatgctgcaccagctgtccctctagagtcctcacctccacctgtggcgagggggcggcagagtgctctgagggcgtcgaggtttctgaggcgctctcatcccggctacgctgggagaaggaaaagcgcttgacaatcatctgtgagttctgcttggccagtgagccgaacttggctgcccgctgcagcaccgagccacggaagctaccctcctcacccttgaggtcatcgctggagctggctgtacttaggtggcccgagtccaggatgacgctgccccggttactatcggagtcaatgtcagtcaggtgcaggtcagagccgctggccaccttgatggggatggggttggagatttccaggcgcgtcttggattcacgcttggaggagcggttcaggttgaagaagccacgtcgcaggctcatctcctccaggctccgaagctctgccgctgacatccgctcctttttctcctttttctccttcttctccttccgcccgccatctttgtccttgtctttcttcattaggttaaacatggtgggggtgctgtttgtaggggtagcacccccagaggattatgagtgcttagcacagggccttggtgccccactttgctgcggccaccggagcccgcccggcaggcagcagaagcggagacgcggcatccagcagcctcggcccggtcagggatggagcagagcgc

SEQ ID NO: 17497 - RNA, 8852 nt, Homo sapiens
  source 1..8852: mol_type = other RNA
tcaggccaggcacagtggctcatgcctataatcctagcactttgggaggcgaggcaggcagatcacttgaggtcagaagttcgagaccagcctgctcaacatggcgaaaccccgtctctattaaaaatacaaaaattagccaggcgtggtggtacacgtctgttaagtcccagctactcggagggtttaggcaggagaatcgcttgaacctcgggaggtagaggttgcagtgagttgagatcatgccactgcattccagcttgggcgacatagcaagactctgtctccaaaagacaagtaacttcccttttactattgtttctatcctcttctctgttctatcgtggggcaatggagggggcagtctctgttcgagacagatccacttcacactctgtcccattcattttgggggagacttttctcccttcttcccttttggactctttctggatggctgacattatcagagcctcggcacttgggctgtttgctattttttcccacccatctgtccaaactactttattcattcagggattataactggccacactacagaatgagaaggtagaaggtagaagaggaggaggggtgtcatttgtttcttgcctttctgcatgagctgcctcttagctgtcaatgaaggaacaaagcatggagtagggcatgaagacagggaccgagcagggcagagacagcactcccaacctattcacattgccctgtgggcccgagctagttctgccaagttttgatcaaaaagtcacctttgaaatggctaaaattaagcttttaaaaaatgttctaatgagaagggcttgaatccaaaaagaaagagaatgaaagaaagaaagagagagagagagggagagagggagggacggaaggaggaagagaagagaagagaagagaatctctgtaattggtgagatttaacaatcagagggacctcaacattcccttgtggaggctagggaggatgaggcttggagtctctgccacccttgctaacctgaatcacagtccctaggctcttcacataaaaggtggggcttgtgtcttccttggccaatcccctcattccactacctctgcctgccccaaaatgagctgcctaggctctttaagtggcactggtctgacactttggggagcaggccagagaccagggtgatgccctcacggtccccatcagaatcctgcctctgcccaccacccccaggaccaatccagactttgcctgagcctgaaggaacaggcaggaaaactggcgcagccaggaggaaaagggcctttatttccatacatcgggtaaacaggggagagcacagcccagtgagtacaaaccaattgcaggagagaaggggggcggcagatgggagcagcaccaggcactgcacttgggctcccaagtctggtggagttctcagggataacctttttagggtgggggctgggacctccagaccacatggtgttgtgtctgggataagtgtgtgggggcagggaggttggaagaatgacacgggctcaggacacagagtgaggactcatgtctaatgagcaccggccaaaacttccatcttcagtttttctgatcacaagtcctcaaccccaagccttccctctcaagttgagtttatggtccagaccacctggacagagcaggagggaggcagtgcttggatcagccctgaactgctgtagttggaatgggtttaccttaaataggtcattgcacataacacgctgagacaaagagggtggggtgggggctggaggtgcggatggtccacacacacacttgtctgcgtaggcttgctcaacccagcccagcagcaccggagagcccctccgcacctcattcttaagaacctggacccggctctcctcaccagcgtctccagctgcacagagaaaggactgctctctgaagggtgaagatggagatgacattcccgagtcgttcttgggagccccagctaccactacagccccctcccactctcagggatgcagctgtgatggagaggttgggtatttaaattaaaaagtagaaagacagcaggcaccaagaagagagagcccccaccccacacgagagggaaggcactgcttctcctcccccaatcctccccatggacccagcaacctagagtgtcccagtaggcaacctgtccaccgtccctgagcagggagctgagagggaggtcaacgtgctggctccatgcagtgccaggccacctgccactgcccacggtgacacagggtagaagccaagagtctggcattttgagacagaggagcaaaaagttctcttcagaaactcctctttcccccacctcttccacgtggagacatcagacacccatagcctggaaagtgcccctgacagaagaaggtcagggtgtttcccatgcagatcagcagtcgggtgggggagaccggtgccccaccacttcctgggagaggtgcccaggcagccacaggccctggggtgagagggctgccaaccactcccctgggctatgcgttagtctccgtcagcttggcctctgtgtcgctgtcactcagataactgtgggagtatcgcggtctggaggtgttgtcgagagggtcgtgctcatcatctgaccgatcaggggcaagggacttccagtagctggtggggctggaactctttaagctgccatcatcagaagctgccttggaaggtcccttgttttttgacaaccaggacttgaccccgtcaacacggtcctccagctccgagtccacatcagagtctccctcactgttgatgaggtcctcattctcatcactctccatctcatcctcaatggcagcctgcaggtccccgatgcgcttgaatgccaactttaggtcagcctgcaggctctggttagcagcctccaggctttctagatccatctccagttcgtgcttcttgcggctcgcctcggcctccttcctggcaagctcgcccatctcctccttggtgtcccggagctgcctctgtagccgcttgttctgttccttctcccggttctcggctgcaatgcgctgatcccgctcctcagtcagcttctccatgttttccttgagacggctagccaggctctccagccgtttcacttgcgtcctttcaaactccaggcgtgtctccagctcccgtatcttagcttcctgcctgctcaccagggacttgtccaccatggactgctccaggaactccacctggctctggagggcttgtagcttctcctgcagctcctgcttctctttgttggcttcttctagctgagcttggagatcatttatctgagccaggtcccgggaagcctgagccacggcagccttgtgcttcttcatcaattcgttcatgtcttcctgatcttcctccagccggttctggatctcattcttctcacgctgaaggcggctcagctgctcctccagcgctgtcttggctttggcgatgtcatcaatctgcaggtgcaggtcttcgatctccacctccattgctttccgtgctttcacggctgccgcacaggtgaactctgactcctccagctggttcttgagctgggcaatctctcgcttgctgggagcactgttcttcaggtggtccagcatgagctgggcatctgccagcagggccttggtgcgcttcaggtccttccgcagccgcttctctgactcaaagtcccgccggttcacctggtcgctgagggtggcgagcttgccctccagctcccgcttctctcgcagaaccttctgcttgtcctcatactcttcctctagctgcacctccatctgttttaacttcttctgacacgactgccgggcctcctccacctcctcatcccgactctccatctccttagaatgggtctgtctcatccgctccatctccatctccagacgcagcttggcctgttccagcatctggatggtccctgcctgctcatccagctcttcttcctgatccttgactttggcctccaggtcccggagctgtttcttgaccttggccagagaagcctcatccttggactcttgggaagaaatgtcctggagctctgcctctagagacacaaccttctgggtgaaccctgcaatgtccatgtctttttcctctagttgctgcttcaggctgaaagcctcagcgaggagcatgtccttctcccgctgcagcttctcccgctgcagcttctcccgctgggcctcctcatgcgcctgcgagagctcactgtcaaacctcctctgcttcttctccagttcgtggttgcggacctgctggccctccaggtgcagcttggtgtcttgcagctcagccgtcagtcgctggcacttcttcttgagctgctgcagagcccgctgactctcctcactatctgcctgcaggtccccgagccgccgttccagctgcctcttgttctgctgctccacctccagcttgtcctcaaactcctgctggagccgtttcttggtgaagtccacctcccgcacagcccgctcatacttcagccgccactcgccacctgcatcatcatcatccacttccccgttgatctccgctgcccggatgagacgggcctccatcacctccatttccataacctccatctgcttcttcagtgcatcgtactgggtctgcagttccttcatctccttctcagcccggagcctctctgctgtctccgcgtccagcagctgggaggcggactctcctgtgttacgctcatctgtcagctccgatgtcagctctgagatccggctctccagccggtcactgttgagccgcagctcgttcctctccttctccgccttctcgagcttgctccgcagctgctggatctcctcgtctttgttccggatctgctcctctgacagctgtacttcgatgaggggcctcactgtggtaaaaagcttccaccagggccagtccttcacccctttgttcttcttgatgttcttctgtacacagcgaatggccaggtcctggatctttctcttcttgaagtgctggcgggccaggtagcccctgcaggctgcttggaacagggttaggttcctgctggtttgttcatcccgctgctcctccagccgtgccaaggtgcccgcccggaagaacacccggctcaggcccatgcagcagctgctcttctccagatccaagcactccagcagctcctccactgcccgcctttcatccaccacgatgtagttacgcccgtgtttcttggtcaggtgcggggccaggacatcaaagcggcggcggaactcggaaaacaccatgtggtcagggtaaccttggcggtacatgcgcatggcatcgagcaggcgggagccgcggagctgggtgcggagcaggggcacgtcgagctgcaggagcccagcctcgcagtggtctcccgagggcaggtccagctcactgctgctgctgactcggcgggaggaggcggaacggggctccccagcccagccctcagctacaggcaggaagcagtgcacaaaatgcagctttgacttcttgatggtgtcgatgagggcgtccacctgtagcttcatctggatgcacagtgacttctttttgacagccgccatgcctgtggtaaaggttttccgcatgctggtggcccggcgcagtgccagctgcgagccgccctccaggcccgcgatggagccagagagcaccgtggcactgcctgcgcggcccagaaacaggttgctgatgatttttttctgggagtcctgcaggagccggggggcattctgggtggctgggttctgcttggtgtagttcagccagccagtcacattgtactctacccagttggtgccatggctgtggcccaggagaaagtggtgtggtttgctgctgtgcagaagggggctttggccttttttgtcaccttcctgggggccataataggagaaaaggcgctccaggagggtgtcctcactggcccctggcaccagagcctcctcttccaatagccagagcaggcccctcgcctcgtctgtgcgggccagcgagcggaccagggactgatgggaggcctggtccacagcagccacagagtcatccgtcgggggttccaagtcgtcaaacgccagctcgatgttctcctccttgtatctttccaactcctgcacgaaggtgcgctcgtggaagagcctctgcagccggtcttgggtgtagttgtggcacagctcctcaaaggaggctccgcgggctgacccaccctgctcagggttctggaagcccggggtgtcgacaatcatcatggagcagagtgagtgctggctggacttgagagccctattcaccagggagacgagaagggtgaagagctcgctgtagaggccggccgccatgccctcaaggcactccagtgcactcagtttcgggcctgtcccatctcccaggccactctcctcggggccctggcggaaggaggtggagcgctgcagggtgccacccttgtgctggtgcttgaagatggctgaggacagctcctccaggctgcagcccagtaggtacgcagccttctgggcccactcatggcgggcaaactgcttgcgcccagcttcagcagcttctttggtggctcccgcagcccccaggtggtagatggcagccagaatgaaccagcaggccttctgttcatcgggggagatgcccagcaccttcatggccgcctgcagcttactaaactgctgagctgccttctgcttttcctcaggcttggccagtggcacaatcccaaacacattgttctctgccaagtggttgaggtggagctctgtcctgagggtgccatccccacaggccagcaggtagtagaagacgttgaatgtggcttcactggctgggcgccgagccacacgcagcttctccagaagcattgtctgaatggaggctgaggccacctggccagcttggtcaaagtccagggagaggatctgggagaagcgggtggcattgccattaatgatggtggggctgttcccaaaggcttccaggagggtgtacagagcctgccacttctccacagaaaacaccttgttcccgctgatgcccgcgatggtggccaggtactgcaccagatgctggcagctggtggtcttgccactgccactactgcccaggaggatgattgactgatcctgacggctcatcagcatcgccctgtatgcggtctgggccactgcatagatgtggggtgccatgtcctcccgccgacaacccttgaacatgtgcatcaccttctcagagtacacagcaggggccccacgggggccaagaaccagcaggctggggccagcatacgtgtgcagcaggctagcgccatagcgctggcgcaaggtgtgcaggacgctggactcattgaggtacaccagtgaggccagatcctccagacggtcgcaggagggagcattagccttctcaacgtcatcctcatccacatccaggatggccccatcgtggtccagcttcacacgcaccttcccctcaggcaagttgagctcctcagatttgagttgactggccagtgagaagccgtccctatggaccagccacaccttctccgtctcattccaggcctcttctgctgcaatctgttcttctgttttcgcctggctgtgggcatgagaggcggcctcagagtccagatcggatggctccctgcgaggtccctcgccgctccgcagccagctcctgctgagctcgctgagctctggaatgggctgcaccttgagccgcacgctgtcccctgactgccggatcatctccacaatctcatccctggacttgctctccacattgtgcccattaatctccaccagtcgatctcctggcaccagccccagggccaggtccttggtgcctgcaccaggctcagcaaagtggaccacacgccgacaggcctggccctcggggccccgatccagcatggttgtgcgccgcagggagaagccaaagtctccagtgggccgtcgttgcagctccagctcccggagggtaggtgggggcaggggcaccacggggggcaggcgcaggtcgactgggaactttttagtcactagctcaggggctcgggatcggtgccctggtcgagggatgcctgggccaggatgctgcaccagctgtccctctagagtcctcacctccacctgtggcgagggggcggcagagtgctctgagggcgtcgaggtttctgaggcgctctcatcccggctacgctgggagaaggaaaagcgcttgacaatcatctgtgagttctgcttggccagtgagccgaacttggctgcccgctgcagcaccgagccacggaagctaccctcctcacccttgaggtcatcgctggagctggctgtacttaggtggcccgagtccaggatgacgctgccccggttactatcggagtcaatgtcagtcaggtgcaggtcagagccgctggccaccttgatggggatggggttggagatttccaggcgcgtcttggattcacgcttggaggagcggttcaggttgaagaagccacgtcgcaggctcatctcctccaggctccgaagctctgccgctgacatccgctcctttttctcctttttctccttcttctccttccgcccgccatctttgtccttgtctttcttcattaggttaaacatggtgggggtgctgtttgtaggggtagcacccccagaggattatgagtgcttagcacagggccttggtgccccactttgctgcggccaccggagcccgcccggcaggcagcagaagcggagacgcggcatccagcagcctcggcccggtcagggatggagcagagcgc

SEQ ID NO: 17498 - RNA, 7769 nt, Homo sapiens
  source 1..7769: mol_type = other RNA
tcaggccaggcacagtggctcatgcctataatcctagcactttgggaggcgaggcaggcagatcacttgaggtcagaagttcgagaccagcctgctcaacatggcgaaaccccgtctctattaaaaatacaaaaattagccaggcgtggtggtacacgtctgttaagtcccagctactcggagggtttaggcaggagaatcgcttgaacctcgggaggtagaggttgcagtgagttgagatcatgccactgcattccagcttgggcgacatagcaagactctgtctccaaaagacaagtaacttcccttttactattgtttctatcctcttctctgttctatcgtggggcaatggagggggcagtctctgttcgagacagatccacttcacactctgtcccattcattttgggggagacttttctcccttcttcccttttggactctttctggatggctgacattatcagagcctcggcacttgggctgtttgctattttttcccacccatctgtccaaactactttattcattcagggattataactggccacactacagaatgagaaggtagaaggtagaagaggaggaggggtgtcatttgtttcttgcctttctgcatgagctgcctcttagctgtcaatgaaggaacaaagcatggagtagggcatgaagacagggaccgagcagggcagagacagcactcccaacctattcacattgccctgtgggcccgagctagttctgccaagttttgatcaaaaagtcacctttgaaatggctaaaattaagcttttaaaaaatgttctaatgagaagggcttgaatccaaaaagaaagagaatgaaagaaagaaagagagagagagagggagagagggagggacggaaggaggaagagaagagaagagaagagaatctctgtaattggtgagatttaacaatcagagggacctcaacattcccttgtggaggctagggaggatgaggcttggagtctctgccacccttgctaacctgaatcacagtccctaggctcttcacataaaaggtggggcttgtgtcttccttggccaatcccctcattccactacctctgcctgccccaaaatgagctgcctaggctctttaagtggcactggtctgacactttggggagcaggccagagaccagggtgatgccctcacggtccccatcagaatcctgcctctgcccaccacccccaggaccaatccagactttgcctgagcctgaaggaacaggcaggaaaactggcgcagccaggaggaaaagggcctttatttccatacatcgggtaaacaggggagagcacagcccagtgagtacaaaccaattgcaggagagaaggggggcggcagatgggagcagcaccaggcactgcacttgggctcccaagtctggtggagttctcagggataacctttttagggtgggggctgggacctccagaccacatggtgttgtgtctgggataagtgtgtgggggcagggaggttggaagaatgacacgggctcaggacacagagtgaggactcatgtctaatgagcaccggccaaaacttccatcttcagtttttctgatcacaagtcctcaaccccaagccttccctctcaagttgagtttatggtccagaccacctggacagagcaggagggaggcagtgcttggatcagccctgaactgctgtagttggaatgggtttaccttaaataggtcattgcacataacacgctgagacaaagagggtggggtgggggctggaggtgcggatggtccacacacacacttgtctgcgtaggcttgctcaacccagcccagcagcaccggagagcccctccgcacctcattcttaagaacctggacccggctctcctcaccagcgtctccagctgcacagagaaaggactgctctctgaagggtgaagatggagatgacattcccgagtcgttcttgggagccccagctaccactacagccccctcccactctcagggatgcagctgtgatggagaggttgggtatttaaattaaaaagtagaaagacagcaggcaccaagaagagagagcccccaccccacacgagagggaaggcactgcttctcctcccccaatcctccccatggacccagcaacctagagtgtcccagtaggcaacctgtccaccgtccctgagcagggagctgagagggaggtcaacgtgctggctccatgcagtgccaggccacctgccactgcccacggtgacacagggtagaagccaagagtctggcattttgagacagaggagcaaaaagttctcttcagaaactcctctttcccccacctcttccacgtggagacatcagacacccatagcctggaaagtgcccctgacagaagaaggtcagggtgtttcccatgcagatcagcagtcgggtgggggagaccggtgccccaccacttcctgggagaggtgcccaggcagccacaggccctggggtgagagggctgccaaccactcccctgggctatgcgttagtctccgtcagcttggcctctgtgtcgctgtcactcagataactgtgggagtatcgcggtctggaggtgttgtcgagagggtcgtgctcatcatctgaccgatcaggggcaagggacttccagtagctggtggggctggaactctttaagctgccatcatcagaagctgccttggaaggtcccttgttttttgacaaccaggacttgaccccgtcaacacggtcctccagctccgagtccacatcagagtctccctcactgttgatgaggtcctcattctcatcactctccatctcatcctcaatggcagcctgcaggtccccgatgcgcttgaatgccaactttaggtcagcctgcaggctctggttagcagcctccaggctttctagatccatctccagttcgtgcttcttgcggctcgcctcggcctccttcctggcaagctcgcccatctcctccttggtgtcccggagctgcctctgtagccgcttgttctgttccttctcccggttctcggctgcaatgcgctgatcccgctcctcagtcagcttctccatgttttccttgagacggctagccaggctctccagccgtttcacttgcgtcctttcaaactccaggcgtgtctccagctcccgtatcttagcttcctgcctgctcaccagggacttgtccaccatggactgctccaggaactccacctggctctggagggcttgtagcttctcctgcagctcctgcttctctttgttggcttcttctagctgagcttggagatcatttatctgagccaggtcccgggaagcctgagccacggcagccttgtgcttcttcatcaattcgttcatgtcttcctgatcttcctccagccggttctggatctcattcttctcacgctgaaggcggctcagctgctcctccagcgctgtcttggctttggcgatgtcatcaatctgcaggtgcaggtcttcgatctccacctccattgctttccgtgctttcacggctgccgcacaggtgaactctgactcctccagctggttcttgagctgggcaatctctcgcttgctgggagcactgttcttcaggtggtccagcatgagctgggcatctgccagcagggccttggtgcgcttcaggtccttccgcagccgcttctctgactcaaagtcccgccggttcacctggtcgctgagggtggcgagcttgccctccagctcccgcttctctcgcagaaccttctgcttgtcctcatactcttcctctagctgcacctccatctgttttaacttcttctgacacgactgccgggcctcctccacctcctcatcccgactctccatctccttagaatgggtctgtctcatccgctccatctccatctccagacgcagcttggcctgttccagcatctggatggtccctgcctgctcatccagctcttcttcctgatccttgactttggcctccaggtcccggagctgtttcttgaccttggccagagaagcctcatccttggactcttgggaagaaatgtcctggagctctgcctctagagacacaaccttctgggtgaaccctgcaatgtccatgtctttttcctctagttgctgcttcaggctgaaagcctcagcgaggagcatgtccttctcccgctgcagcttctcccgctgcagcttctcccgctgggcctcctcatgcgcctgcgagagctcactgtcaaacctcctctgcttcttctccagttcgtggttgcggacctgctggccctccaggtgcagcttggtgtcttgcagctcagccgtcagtcgctggcacttcttcttgagctgctgcagagcccgctgactctcctcactatctgcctgcaggtccccgagccgccgttccagctgcctcttgttctgctgctccacctccagcttgtcctcaaactcctgctggagccgtttcttggtgaagtccacctcccgcacagcccgctcatacttcagccgccactcgccacctgcatcatcatcatccacttccccgttgatctccgctgcccggatgagacgggcctccatcacctccatttccataacctccatctgcttcttcagtgcatcgtactgggtctgcagttccttcatctccttctcagcccggagcctctctgctgtctccgcgtccagcagctgggaggcggactctcctgtgttacgctcatctgtcagctccgatgtcagctctgagatccggctctccagccggtcactgttgagccgcagctcgttcctctccttctccgccttctcgagcttgctccgcagctgctggatctcctcgtctttgttccggatctgctcctctgacagctgtacttcgatgaggggcctcactgtggtaaaaagcttccaccagggccagtccttcacccctttgttcttcttgatgttcttctgtacacagcgaatggccaggtcctggatctttctcttcttgaagtgctggcgggccaggtagcccctgcaggctgcttggaacagggttaggttcctgctggtttgttcatcccgctgctcctccagccgtgccaaggtgcccgcccggaagaacacccggctcaggcccatgcagcagctgctcttctccagatccaagcactccagcagctcctccactgcccgcctttcatccaccacgatgtagttacgcccgtgtttcttggtcaggtgcggggccaggacatcaaagcggcggcggaactcggaaaacaccatgtggtcagggtaaccttggcggtacatgcgcatggcatcgagcaggcgggagccgcggagctgggtgcggagcaggggcacgtcgagctgcaggagcccagcctcgcagtggtctcccgagggcaggtccagctcactgctgctgctgactcggcgggaggaggcggaacggggctccccagcccagccctcagctacaggcaggaagcagtgcacaaaatgcagctttgacttcttgatggtgtcgatgagggcgtccacctgtagcttcatctggatgcacagtgacttctttttgacagccgccatgcctgtggtaaaggttttccgcatgctggtggcccggcgcagtgccagctgcgagccgccctccaggcccgcgatggagccagagagcaccgtggcactgcctgcgcggcccagaaacaggttgctgatgatttttttctgggagtcctgcaggagccggggggcattctgggtggctgggttctgcttggtgtagttcagccagccagtcacattgtactctacccagttggtgccatggctgtggcccaggagaaagtggtgtggtttgctgctgtgcagaagggggctttggccttttttgtcaccttcctgggggccataataggagaaaaggcgctccaggagggtgtcctcactggcccctggcaccagagcctcctcttccaatagccagagcaggcccctcgcctcgtctgtgcgggccagcgagcggaccagggactgatgggaggcctggtccacagcagccacagagtcatccgtcgggggttccaagtcgtcaaacgccagctcgatgttctcctccttgtatctttccaactcctgcacgaaggtgcgctcgtggaagagcctctgcagccggtcttgggtgtagttgtggcacagctcctcaaaggaggctccgcgggctgacccaccctgctcagggttctggaagcccggggtgtcgacaatcatcatggagcagagtgagtgctggctggacttgagagccctattcaccagggagacgagaagggtgaagagctcgctgtagaggccggccgccatgccctcaaggcactccagtgcactcagtttcgggcctgtcccatctcccaggccactctcctcggggccctggcggaaggaggtggagcgctgcagggtgccacccttgtgctggtgcttgaagatggctgaggacagctcctccaggctgcagcccagtaggtacgcagccttctgggcccactcatggcgggcaaactgcttgcgcccagcttcagcagcttctttggtggctcccgcagcccccaggtggtagatggcagccagaatgaaccagcaggccttctgttcatcgggggagatgcccagcaccttcatggccgcctgcagcttactaaactgctgagctgccttctgcttttcctcaggcttggccagtggcacaatcccaaacacattgttctctgccaagtggttgaggtggagctctgtcctgagggtgccatccccacaggccagcaggtagtagaagacgttgaatgtggcttcactggctgggcgccgagccacacgcagcttctccagaagcattgtctgaatggaggctgaggccacctggccagcttggtcaaagtccagggagaggatctgggagaagcgggtggcattgccattaatgatggtggggctgttcccaaaggcttccaggagggtgtacagagcctgccacttctccacagaaaacaccttgttcccgctgatgcccgcgatggtggccaggtactgcaccagatgctggcagctggtggtcttgccactgccactactgcccaggaggatgattgactgatcctgacggctcatcagcatcgccctgtatgcggtctgggccactgcatagatgtggggtgccatgtcctcccgccgacaacccttgaacatgtgcatcaccttctcagagtacacagcaggggccccacgggggccaagaaccagcaggctggggccagcatacgtgtgcagcaggctagcgccatagcgctggcgcaaggtgtgcaggacgctggactcattgaggtacaccagtgaggccagatcctccagacggtcgcaggagggagcattagccttctcaacgtcatcctcatccacatccaggatggccccatcgtggtccagcttcacacgcaccttcccctcaggcaagttgagctcctcagatttgagttgactggccagtgagaagccgtccctatggaccagccacaccttctccgtctcattccaggcctcttctgctgcaatctgttcttctgttttcgctatgagccaggcacaggggaaggcacttcatacaggtctcctcattgaatcctcataacaacacactttccgcatggcctggcctggagcagcccagagcaaggagactccgctctgat

SEQ ID NO: 17499 - RNA, 2035 nt, Homo sapiens
  source 1..2035: mol_type = other RNA
tcaggccaggcacagtggctcatgcctataatcctaggactttaggaggctgaggtgggaggatcacttgaatccaggaattcgagaccagcctgggcaacatggcaaaatcccatctctacaaaaacacacattagctgggcgtggtagtgtgtacttgtagtcacacacacccttgggaggctgaggtgggaggatcacttgagctcaggaggcagaggttgcagtgagccgagatggtgccatggcactccaacctgggcgacagagatcccatttcaaaaaaaaaaaggaacagattgggggctgcattgttaggctacactgaggaaatgttcctcttatggatccacagaagaaaaatgacttttagtgccacgtgccttgcaattatctctagcaaaacagcctagctccctcaaccccactgtgtgtctgggaaaagacagtaaaaacatttccttgagaggtgaagactaaaaggaagctaccggctcactgtgcacaggtgagaaaatgtcacggtaaaggagcaccatgtgttgattttaacagctttttctaactggaggaatctgtcacatgccatagaaaaattgctccctgccctctgaaaaaaaaaaaaatgtcatacagaaaaatcaggttcataaaagaaagtatacatccaaagtaggcaaaaactatggtttatgttttcaaaatatgcaaaataatttcactatataataccttgatttgcatgtgacttagtacttatttcatattaaccagattcacttgctttcataaatctgtgttttagaaaatctattttttaaaaatatctatttttaagccagaagataaaccttacatttgtgcatccatgtgtaaagcaatcctgcttggcattatgcagccaagatactaaaagattaataacataattttaaaaagctccagatacagactaacaaataatatatttccttaaattttctgggctatactactgacctgaattcatgcaatctgaattttcagatataagtaccactcaatggttggttgttacaacttagaagcaatagggttgggaagaccttcaaaatattggccattaaatcataagtaaaattattcttagagctggattatcataagtggagtgccctaacttttcttatttcatactcagcaaattgattctaacattcataatcatgcccttttatgtgctttaagtggacatactgactttgcagtctatactttgtaagagagcaggtaactctagcacagaagaaaccatgtaatgcggaactggggaggacttcagtggcactattccatttttattgatccagactgttgctttcaatcctgcattgaggcctccttggatgtcggtttctaatgtgtcaccgaccatcacacagtccccaggttgtactccgagaagattgcagcagtaataaaatatggacggtgctggtttctcctctctctgctctccacctacaacaacagcgtcaaaataggactgacaggcacaagcctcaatcttctccctctgggtctgtctgtccccattcgttaatagaagtaggcggacctcctttcgaagttcagtaagcatggctttgacgtcttctgctagtgtcatatgctgtaaacgtgtagatttccaaaggaaataacattcttcagccaattttctattggctgcaccaccttttgtttcctggattgcttcttcccaatgtgaagtccttaaatcagtaatgcatgtattgtaaggatgaaaacattccttgctgagtttaacttgaactttatcacagatgatttcagcctcttctttataatggtattttgattgtaagagttttatcacctccaacatgcctctcctgctcgccccggccgtgtcgatgagagtgttgtccaagtcaaagaaaaccgcccgcacgcggctcagccccatagcgccggccgctggcgcgaaccgtagccttgccaccgccgcctgcgcatgcgcaaggcggactgc

SEQ ID NO: 17500 - RNA, 28 nt, Homo sapiens
  source 1..28: mol_type = other RNA
tcaggccaggcacagtggctcatgcctg

SEQ ID NO: 17501 - RNA, 3377 nt, Homo sapiens
  source 1..3377: mol_type = other RNA
tcaggccaggcacagtggctcatgcctgcaatcgaagcattttgggaggctgaggtgggtggatcacctgaggtcaggagttcgagaccagcctggccaacatggtgaaaacccgtctctactgaaaatacaaaaaattagccgagcatggtggcgcatgcctgtaatcccagcagcttgggattgggaagcaggagaatcgcttgaacctgggaggcggtggttgcagtgagtcaaaattgcaccactgcactccagcctgggcaatagagtgagactccatctcaaaaaaaaaaaaaaaaaaaaagaaagcgacaaaaagaaatccattttcacaggaaaccaaaaatgagcattttggactcagtctgctaaatgattattcctttcctgatacagattttggttttgagagtcaaacagggatcggcagcacagcgtgacttcggttttgattcagaaccattttactaggctcagaaaatcatgctttgtcgagttctgatggattccaagggaaatcacctatcaggtaaagctgtactttctctcaccaagaccctggaggtagcatttccacttccattctttgccgatggctcctgtgactgaacacagaagctgttttctgaaataagacgaaagcgtttgtggaagacccacagaataaaaatagagatacaggtgcttactttcaattcttttcttttaaatgtaaataatcgctccatgctccatgccgccacttacctcagctgaatacaaaacagctgaatccttttgaatcctttgtttttttctttttttgagacagggtcctgctgttgcccaggctggagtggcagtggtgccatcccagttcaatgaagcctcaaatccctgggctcaagggatcctcccgtctcagcctcctgagtagtagggactacaggcacgcaccaccacatcagctccgggcgacagaatgaggctccttttttaaaaaaaaaaaaaaaaaaaaactgactctgaagcttaaaaccttcacctttaggaagaaatcgtatttgtttgtttgagaccgagtttcactcttgttgcccaggctggagtgcaatggtgtggtcttggctcaccgcaacctccgcctcccaggttcaagagattctcctgcctcagcctcccaaagacctgggattacagacgtgcatcaccatgcctggctaatttttgtatttttagtagagacagggtttcaccatgttggccaggctggtcttgaactcctgacctcaggtgatctgcctgccttggcctcccaaagtgctagggttacaggtgtgagccactgtgcccggcctgaggaatcgtatttggattactcatctctccggccactttacttacaaaaaactaaactaagaagtaaataagccagaacccctccctactcatcccctttggtctccccaagaagaggaggattctaagaaaggagctggagagacagtggggtcttcgggggttccctgagacgcctcttcctgcccttgttccagctttggaattggaaggagggaacctgtgtctgaagtgattgacaggtggggacaggagtgtggattctggcctgtgcttgacactcaaacccaagctacggcaagggttagcagcccatggagggagaggccaggaggcccggggagactgctgtccctgagcagctgcgccgggctgtgcttgcccctggtggtcaccatgcaacctcaggggaaccttcaacctggtgaatggcaactggttcctctgttgagcaaagtctccaaggaaagccgggttctccagagaatcttaacaccctgaccagccgggaatctgctccatgatgtgtggatggggacacatctctgagggcccctgacagcttatttaatcacacagaggataggtgcacagatgtgggtccctcagattgtaaacagtgctgtgtggtcctcaggacatcaaggtccactgggtgggggcactgtggccacagctgtgggccaccggcttcccgaatctcactgctacccttatgcagatgaacgcccacccgtgggccaggacgctggtaccggtggaacttgctgcctgaggatctaggaggtagaagaagctgagttggcagctgctctcccaatggagccgagagcatcaatagcgggggcttctggtgcagcagacatgcacttctgcccctgcagcagggactcacagaagtgcctacccccaggaaggcagcacctatgcacagaactagaaaggacaaaagctcaggtgcttggaagttcccctggggtcccttgggattcctgagattctcctggcttggaaggcgcgggagccttgggagtgccagccgggctcttggtgggaggctgagaagagcagcagcagcaacagagagagaagagccgagttcggacggcgcgggtgcagaggacgaacatgatgcagttggcacctccctgaaacgtgttcccgataccatgcagaaccaccagcaccggcgtctgcacggccggggagccacagagggtcagcacgaaccgcacggtgctccagaccctgaggccgatgaagatgagcgggatgagcaccagcttcttgtccgccatggaggagtggcgcagcaggcggtgctcctgggagaggatgggccggtactcagagagtgccgtgtgcgctctgttgatgtgcttccggaccaggaggtacagcagaggcagcagcacatatgccagcatctcccacagcttccccgtcagcagcatccacaggacatggtccttggcctccaggtcgatccagcaccagcccacagacacgtccgaggcgtcatagccaatcttcttcagggcgacggctgccacagtgatgaccaacgggaccccccagctgacgacatggaaggcccaaagcaggcgatctgtgcgaggcccgcgcgcggcgcggacgatgctgaggtacaagtagagcgcaatggccacggtccagaagaaggagctggtgttggcgaaggtggacagcgcgccctgcagcacgcagtcccacgacgggcccgcgaagttctgcagcactccgtagaagtaggaggcggccgagagcaggtcggccagcgacaggaagagcagcaggcgccgtgcccggctgcgcaggtcgggccacagggcgtgcgtggccaccagcaggcccgagccgagcgcggagagtgcgcacgacagcagcaccacggcgcgctccgacggcaccagctcggtgggcggcggggacggctgcatggcgtggggggccaggagccggagcgccgcgaggacagaagccgggccgcgcgtgcggccacgccgccgccgtct

SEQ ID NO: 17502 - RNA, 1812 nt, Homo sapiens
  source 1..1812: mol_type = other RNA
tcaggccaggcacagtggctcatgcctgtaaccccaacactttgggaggccaaagcaggcagaccacctgaggttaggagattgagaccagcctgaccaacatggagaaaccccatctctactaaaaatacaaaattagccaggtgtggtggtgcagccctgtaatcctagctactaaggagagttacttgaacccagaaggtggaggttgtggtgagccaaaattatgccattgcactccagcctgggaaacaacagcagaattacctctcaaaaaaataataataataaaataatcctttgtcacgttcttggtttctgtccaatatgaattctcttatgtttattaaggtctgaggaccagttaaaagctttgccacattctttacatttgtaaggtttctctccagtatgagttgtcttatgttcagttagatttgaggatgtagtatacgctttgccacattcttcacatttgtagggtttctctccagtatgagttctcctatgtttatggaggcctgcagaccatgtaaaggctttgccacattcttcacatttgtatggtttctctccagtatgaattatcttatgcatagtaaggtgtgaggagcgggtgaaggctttgccacattcttcacatttgtagggtttctctcccgtatgaatcttctcatgtttactaaggatcgaggatgaaataaaggctttgccacatttatcacacgtgtacggtttctctccagtatgaattttcttatgtgaagaaagagttgcaggatggttaaaagctttgtcacattctttacatttgtagggttgctctccagtatggattatcttatgtgtagtaagggtataggggtacataaaggctttgccacattcttcacaaatgtagggtttctctccactatgaattttcttatgtgtagtaaagctagagaagtacttaaagactttgccacattcttcacatttgtagggtttctctctagtatgagttatcttatgtgtagtaaggtgtgaggaccggttgaaggctttgccacattcttcacatttgtatggtttctctccagtatcaatttttttatgtgtagtatgggttgaggactggttaaaagctttgtcaccttctatatatttcaaaggttttttttcagtatgtcttcttttatgtctctttgaatttgaaaattgatgaaagactttcacatatttaccacattgaaatattttgctctgggtagttgtcaaacattggttaagtccattataacctcttttgtgtaacttacactcatccacactttcacagccttttttaaagtgtaaattgccatgtccacatttttcaaattttctcagtatcactttttggtaagaatcttttatgctctgctctggccaaaggtcttgggcaaaatgagaacacacaactgggggtttggcaatcatctcatgtctcttcatagtcagaggttttattccttgctccagacaggtgatcaggtctggcttagagacaataataccaaggaagaccaggtgtctgtagttctctaacatcacatccctatataaattctgctgtgcagtgtccaggcaatgccactcctccagagagaattctacagccacatctctaaattgcaatgattccatttctaggcttctaaggggtcccggcatcttggctgtggatctcccaatacctacaggacacagggccacagagggtgggcctctaggagcagaggacacagagtagcgaagaggcgacctagagctccagatgcagcgagagac

SEQ ID NO: 17503 - RNA, 4110 nt, Homo sapiens
  source 1..4110: mol_type = other RNA
tcaggccaggcacagtggctcatgcctgtaaccctagcactttgggaggccgaggtgggtggttcacttgaggtcaggagttcgagaccagcccggccaatatggtgaaaccccatctctactgaaaatacaaaattaggcatggtggcagtgtgtctgtaatcccagctgcttgggaggctgaggcaggagaatcacttgaacccgggaggcagaggttgcagtgagctgagatcacgccactgcactccagcctgggggacagtgagattccttctcaaaaaaataaaaataaaaataataaatttactattattctgtattctggcaaacacggattcatatactttgcaggaaactcttaatacatacaaggagacaagagcaagttctgagcagtgatcacagccatcagcatattctagtggagggtaaatcagtaaaatttcatggtgaataaaaatgattttcccattcaccatgttcagctgactggaaaggctgccaccagccgcctacacacggtcctgaaccagcctgtgcgcctgccttgtggagcctttgtccttttgctgatgtggtttatcctgaacttgcatttgcatcccaagcttccctttccgtcgttttttgctatcatatgggaaaaactcttaccaggcagaatccaacacgtgcgctctgcacaaaaatcagttcatctgaagaacaagtgaccacagggcaggctctataataccttttccaaaccacaggacaggtctgaaatggtggcttactccttatttaataaactggcatttcctccacagcgcaggtctgaaatggtgacttactcattaataaactggcatttcatccacagggcaggtctgaaacagtgacttacttgttaataaactggcattttcctccacagggcaggtctgaaacggtggcttactcgttaataaactggcatttcctccacagggcaggtatgaaacggtgacttactcgttatttaataaactggcatttcctccacagggcaggcttgaaacggtgacttactcattatttaataaactggcacttcctccacagggcaggtttgaaacggtggcttactcgttaataaactggcatttcctccacaggacaggcttaaaacggtgacttactcgttactaaactggcatttcctccacagggcaggtttgaaacggtgacttactcgttaataaactggcatttcctccacagggcaggtttgaaatggtggcttactcgttatttaataaactggcatttcctccacagggcaggcttgaaacggtggcttactcgttatttaataaactggcatttcctccacagggcaggcttgaaatggtggcttactccttatttaataaacgggcatttcctccacagggcaggcttgaaacggtggcttactcgttatttaataaacgggcatttcctccacagggcaggcttgaaacggtggcttactccttatttaataaactggcatttccttcacagggcaggtttgaaacggtggcttattcgttaataaactggcatttcctccacaggacaggtttgaaacagtgacttactcgttaataaactggcatttcctccacagggcaggtttgaaacagtggcttactcgttatttaataaactggcatttccaccacagggcaggtctgaaacggtggcttactcgttatttaataaactggcatttcctccacagggcaggcttgaaacggtggcttactcgttatttaataaactggcatttcctccacagggcaggtttgaaacggtggcttactcgttatttaataaactggcatttcctccacagggcaggtttgaaacggtggcttactcgttatttaataaactggcatttcctccacagggcaggcttgaaatgatggcttactcgttatttaataaactggcatttatttcctggtcttgccactctagctgcacttctaaccttggccttctaacagcaaagcacattggcttggagatgccactgctggcatcagtggatgccgacccaaagcaaggaaaaggtcacagtgatccagaagatggcgagaacccagggatcaaagttaccaggggggaaaaaggcattttttggatttacttttggggcaacgaaagaaaatgcagagaaaatgcaggggtggggctgagtcccaccaggtggcaggaaaaggcaggtgcaggtgggcgtggtgagaaggcccaccttgtagtcttccctggcatgcgcgccccgtgactccttccgtgcctctgctccgtagatggtctgcagcgcacacagcatcaggttctgcagctccagggtctccaccaggtccgtgttccagaccattccccggtcgaacgtcttcaggtgctttaggtctccatagagcttgctgattttcccacaaccttcttgcaacacgcttcccacacggaacacggcagcatgattttgcattgacttctgcatgctgagtcgcagttccgatgttcttatgcttccatcagcaaatctcaatttgtcaagattcatgacagattcttccccagcgtttggtttaattggagggactttatctccaggcctgcatgactcttcgatgctcagggcacatgcccgaccaaagacaaccaggtccaagagcgagtttgccccgaggcggttggcaccatgtaccgaggcacaggcggcctccccacaggcgtacaggccgggcacaatctgatcctggccattcacgtgcctcaggacctgccccttgtagttggtgggaatgccgcccatgttataatgcacggtggggaggacagggatcggctccttcgtgacgtccacgccagcgaagatcatggctgtctctgaaatgccaggcaggcgcgtggccagctgctctggaggtaggtggtgcagctgcaggtagacgtgatctttctcagggccacagcctcttccttctcggatctccagagtcatggaccgagacaccacatctctagacgccaggtccttcgcgacaggggcgtatcgctccataaacctttcgccttgactgttaatgagaatgcctccctctccacgacatccttccgtaatgagacaaccagcaccatatatgcctgtagggtggaactgaacaaactctaggtcctggcaaggaaggcctgccctggtgatcatggccgtgccgtcgccagtgctggtgtgggcagacgtgcagctgaagtaggtgcgcccgtagcctcctgtggcaacaacagtgttctttgctcttatgcgatggatggacccgtcctctatgcacagtgcgatgacaccacggcactccccattctccatcaggagatccaaggcaaaatactccacaaaatagctggtatcatatcgcagagaccttccatataaggtgtgcaatagcgagtggccagtccgatcagccacacagcagcaccgatgggcctgcccgccctttccaaacttgaggctctgtccaccaaatgcacgctgataaatcttcccatcttcagttctgctaaacggcatgccataattttctagctcgaccacggcggcgggggcctgctccgtcatgtagtggatggcatcctggtcccccagccagtcggagcccttcacggtgtcgtagaaatgccacctccagttgtcctcctccatgttccccagagcagcattgattcctccctgtgctgcaacagtgtgtgacctggtaggaaacagcttggtaacacatgctgtattaaaccctgcctcagaaaggccaaatgcagctcgcaagcctgcccctccagcgcctaccaccactgcatcaaattcatgatccactactggatactgagcagaaatggaatctgaaactttagcagatgccctcttgttcccatcaacagtgaagtgaaaacctcgggttcctgtttgcaacactgttggccacgccttggccagcgccaggcgccgagcgctcagcagccgcgacaggccccggacccccgacatgtctgctgttgccgccgcgcagtcccgccagtccctgcgcagactgc

SEQ ID NO: 17504 - RNA, 55 nt, Homo sapiens
  source 1..55: mol_type = other RNA
tcaggccaggcacagtggctcatgcctgtaacttcagcactttgggaggctaagg

SEQ ID NO: 17505 - RNA, 32 nt, Homo sapiens
  source 1..32: mol_type = other RNA
tcaggccaggcacagtggctcatgcctgtaat

SEQ ID NO: 17506 - RNA, 933 nt, Homo sapiens
  source 1..933: mol_type = other RNA
tcaggccaggcacagtggctcatgcctgtaatcacagcactttcagaggcccgaggtgggaggatcacttgagcccaggagtttaaggctgcagtaagtcatgatcgtgccacactgcactccagtctggccaacagagcgagaccctgtctcaaaaacagaaacaaaagcagaaacccagtgatgtcatcagggacccaggtttgtttcctttcatatgtccactccgccatctctggtatatcagactcgtgctttgtgttgatgataaccgctgcagttctacatagaatttataatcatgggaaagtccagtagtagaagaggggatattcccccctttataggtttatttttatcagtggtatacattacttcaggatcctgcagcaaagttctcctcaggtctcatttgccatgcctgggtccccagcacttcctaaacaattcaatgacaggaggagggaataactgtgataggtgtagactgatagagacccttgcccttcctagcatcacagaccccctcagaggaagatgaaacccgaaacaatatcagagcactccccagcaaagagggagatggatgtggggaggcagaccacaatatttgctaccgttttttgtttttatttgttcgtttttgtttcacttaaagactcttcttcctggccaggcatggtggctcatgcctgtaatcccagcactttgggaggcagagtgggcggattgtgaggtcaagagatcaagaccattagaccattctggcaaacatggtgaaaccccgtctctactaaaaatacagaagttagctgggcgtggtggcacacgcctgtagtcccagctactagggaggctaaggcaggagaatcacttgaacccgggaggcggaggttgcagttagccagagatcatgccactgcactccagctt

SEQ ID NO: 17507 - RNA, 44 nt, Homo sapiens
  source 1..44: mol_type = other RNA
tcaggccaggcacagtggctcatgcctgtaatcccaacactttg

SEQ ID NO: 17508 - RNA, 169 nt, Homo sapiens
  source 1..169: mol_type = other RNA
tcaggccaggcacagtggctcatgcctgtaatcccaacactttgggaggctctggaggaggattgcttgaggccaagagttcaagaccaacctgggcaacacagcaagaccccatctctacaaaaaataaaaatgaaaaaattagccaggcgtagtggcacatgcctgt

SEQ ID NO: 17509 - RNA, 119 nt, Homo sapiens
  source 1..119: mol_type = other RNA
tcaggccaggcacagtggctcatgcctgtaatcccacacttggggaggctcaggcggcagatcacctgaggtcaggaggtaaagaccagcctggccaacatggtgaaaccccgtctata

SEQ ID NO: 17510 - RNA, 1514 nt, Homo sapiens
  source 1..1514: mol_type = other RNA
tcaggccaggcacagtggctcatgcctgtaatcccagcaatttaggaggccaatgcaggtgaatcgcttgagcctaggagtttgagactggcctaggcaacatagtaaaacccttcctccattttctaaaaaaaaaacataacctaatatacactgagagggatggagggcattaaatgattgccaccatctggggttactcacaaatattccttgctccccggccacccaccatggcctgtttcttttactctgagtaggtttcttaatttgtgggggctgctaccagagcttttgacttcttcctagttcaggagtctccctattgtgttccagggcttttaacatcagtcccaaggccctattcaccacttcctccaggaaacctccagatcttcatagcaagagtttctgttggtttgcctacttagtccagaatttctgaaatgtaaatgcagattagaatacacaatttgtaagacacaatcctgtccttcagggatttcagccctagataaatgtgtgaggtgatggctagcccaattactctgatttgttcatcacacattgtatgtaggtatcaaaatattacaggtaccatccaaattggtacaactattattaatcaatttaaaaagaaaaataaaaaggaattttaacccttaaaaagtttaacagtaaagcaatagacatcaccagcagggtgggattcattgtcagaatcattgtaaaggcagccagggttttgacagcttagaggaaggagggtgactctgggctggggtaaccatgttggtctctgggataaggaagaaaagctgcttcagggcctctcttcagtggcttctacttcaggctggtcccatagaaattcctcagtaagtattttctgcaggcaccaaatgtctccagtggaaatgtgctccttggaaaattcagtaggtcagtagttgtatgttttagaacttgcattcatctgccagtaacagtggcttgtacagcctggtgaggtgggcagtcaagggtgaagtcatcagagatccaggctcctgccaaccctcttctgcacagtcctttgtacatggtgttccttctcaaagttatctcatggtctgggatgactgctagggatctagacatcatgtcttacagcatctgtttatatctcattggccacctctagctgcaagggaggcaggaaatgtagtgtagctaggcacattgccatctgaagaggagatggggccacaaaacagggcttgaaggtatcagataagctcacgtaggttttaatgggccgcgggagtcgggtaggagaaggccctggcttcagctgtaacttggtttccaactttctttcggttccctccgaaatccctcccatttgtgggaggcgttttctgccagtcacccacgtccatttggtttgcatcccaattcggccttgccaccggctcccagaagctctgcgtgctgcgggtggccccggcgtctacctcgcgctcgggtggaaa

SEQ ID NO: 17511 - RNA, 40 nt, Homo sapiens
  source 1..40: mol_type = other RNA
tcaggccaggcacagtggctcatgcctgtaatcccagcac

SEQ ID NO: 17512 - RNA, 80 nt, Homo sapiens
  source 1..80: mol_type = other RNA
tcaggccaggcacagtggctcatgcctgtaatcccagcactctgggaggctgaggtgggaggaacacttgagcccaggag

SEQ ID NO: 17513 - RNA, 1628 nt, Homo sapiens
  source 1..1628: mol_type = other RNA
tcaggccaggcacagtggctcatgcctgtaatcccagcactttgcgaggccaaggcaggcagatcaccagaggccaggagtttgagaccagcctgtccaaaatggtgaaaccctgtttctactaaaaatacaaaaaattagccgggagtggtggcaggtgcctgtaatctcagctactcaggaggctgaggcaggagaatcgcttaaacccaggaagtggaagctgcagtgagctgagatcgcaccattgcactccagcctgggcaacaagaacgaaactctatctcaaaaaaaaaaaaaaaaaaagagaaaaaagtatttcctcgcatctcacctagtcaaaacccagggcccacataccctacctatcccatgcatgtgagacgctcacactatcaacataaaaagtcccttagtatcacctcattaccaatagcagcacaacaacaagtcaagttagaggtgaagctcagctcaccaatcaggttattctgatttggatcagttagaaggaaaggtaggagaggctcaatatcttgaaaacaatgctcatttgcatacatggataaatacttaatggcccagcatgagttccatcaatacagaggcagtgtgtattcactcctgtgttccgtgaatagatcttctcttggtgccctaaattacatttcctataatcatgttaacaaaaaggacagatgtgtagaacaatctatcagaggcagtcataaaagtatttaaagtctctgttgccagaaaaaggggtccctacccagaccctaagggagggttcctggatcttgtgcaggaaggaattcaaggcaagtcacagagtgcagtaagaagagatcactggccaggcgcagtggctcatacctgtcatttcccagcactttgggaggccaaggcaggtggatcacgaggtcaggagttcaagaccagtctgtccgagatggtgaaactctgtctctcctaaaaatacaaaaattagctgggcgtggtggcgggcacctgtaataccagctgcttgggaggctgaggcaggagaatcacttgaacccgggaggcagaggttgcagtgagccaagattgcgccgctgcactccaacctggttgacagagcaagactgtaatcccagctactcaggaggccaaggcaggagaactgcttgaatccaggggggcagaggttgcattgagctgacatggctccagcctgcgtgacagagcaagactgtgtctcaaaaataataataaggcaggacgtggtggctcacacctgtaatcccagcactttgggaggctgaggtgtgtggatcacttgaggtcaggagttcgagaccagcctggccaacatggtgaaagcccatctctactaaaactacaaaaattagccaggcattgtggtgggcacctataatcccagctacttgggaggctgaggcacgagagttgcttgaactgggaggcaggggttacagtgagccaagatcgtgacaatgcactccagcctgggtgacagagtgagattttgtctcaagagttccctaagttttaaatgttctccaagattccttctgtgtctacatcttatgattctgaatctattgcatttccatattttcttt

SEQ ID NO: 17514 - RNA, 1272 nt, Homo sapiens
  source 1..1272: mol_type = other RNA
tcaggccaggcacagtggctcatgcctgtaatcccagcactttggcaggccgaggtagacagatcacaaggtcaggagatcgagaccatcctggctaacatggtgaaaccccatctctactaaaaatacacacacaaaaaaaattagccgggcgtggtggtgggtgcctgtagtcccagctactcgggaggctgaggcaggagaatggcatgaacccggaaggcagagcttgcagtgagctgagatcgcgccactgcgctccagcctgggtggcagagtaagactccatctcaaaaaaaaaaaaaaaaaagaggatgtcaataactatgaaatgcatagaaaagaatacaactgaatgcacatcaaattgttgatggcagtttctctaagcaagggcatgggatgaggtgcaggctgtggtgaagatgaacttttctttttttacttttggtttggtttaagtatacattcctgtatttattgtgtaattaataaatggaaagatccatagatgaataactgccttgtaacgtcagacattctttaatggaatgaacatgtggcacatggatctttgggagtttgggttggattttggggatgttaaggtctcctatcaatcttagttaacatgtcacagcttctggtccctgacttagatcacctctgtgtaccctcagcctactgaggaaaaaggcaggaatcacctctgtgtcattgaagcggtgaggctccaggcatgggttccacctgaccacctggggagacggcatgaagtccaaaaatggataaatggatgttcttgtaaagttgaatccatgaatgccatcttctggaaacactataatctgtacatccttttgggctgcagtcatcacttgctgttcatagatgtcaaggttctggttcatgagctccaaggcctcttggcggctgatgagagccagagggttcagactcaggatggatggatgctcatacacggcagccacataatattcagcctcgtgatggtcagccacgctctcctccccggtgtgggctcccagggcaaccacgtaacagccgcagaggaaaagagcaagcttacttctggctccagacataatgcagaccacaaatctgctcttagcgcgccttccgccctgaatatgcgcatgcgccattctccctttacagccccgaaaacgctccagctggccgactcggagacaatggcgagaggcctcagagttcggcttcttacctgctttgcataggcagcaatctcct

SEQ ID NO: 17515 - RNA, 1333 nt, Homo sapiens
  source 1..1333: mol_type = other RNA
tcaggccaggcacagtggctcatgcctgtaatcccagcactttgggaagccaaggcaggaggatcaccgaagcccaagacttccagcctaggcaacatggcgagatcccgtctcttcaaaaaatacgaaaattagccgggtgtgggtggcatgcacctgtagttccagcaacttgggaggctgaggtgggaggattgtttgagccagggaagtcaaggctgcagtgacccgaggttgtgccgctgtgctccagcctgggtgacaaagtgagagacccttatccaaaaccacatcactcttcctgagttctaggaccttggaaagataccgacagagctcagcattagcctctccctctgatggaggtgctgcaatagctacatttacagcctctgctgtcaaatctgttacagcattttgtttggagccaggttttgcatggatggctatggtgacgcatcctttaggatcaactgccacaggacctaagggaggaagtggtctctctggttccttgctctggcttttacccttggtcgtcgcaccagccttcttaggcatctcggcgcaaagaagccgagcggagccccgagtattgggtgttgcccgaaggtgcctcagcccgctgcggagccgcagcatccccgcctgggaaggcgccggaagagccctctgcgcttgcgcaggtagccggcaggagcggccccaccgcccggcgcatccgctctggccagagggcgacaccttaaggccggcgggagcgagtctcgtggccgcagaacatgcgcgagtctcttttgttctggaacgggccgagccccaggaagtggagctgcggagctgaggcctcaccgtgtcttggcccaccctgctcagctgataggaaggtgtgtcacctctttcctaatcggggaaagaaaggtattgtcacttctcagaattggagagcgcggcaaggagtgcacagggccaggtgtcttctcgctcccacagccaagcagcagatgcagagtcccacgcgctgcctgtggccatcaagtcgatatagagcctcgtggcggcttggcccttgtgaatcttccacgtatcgatggcgcacctaccttgtgccaggcgcagcggatcccacaatgtaaaagaagaggaaatacactgcgacatgtgatatggagagacatgaaacaaatcagcagaggcaagatcatggagtcactgaaggctttcaagcaagggattattagcagcccaatttgctgggttttagaaagacaccggctgcactgtggccgacagaggaaaagccagagacagggagatccgccccctaaatggg

SEQ ID NO: 17516 - RNA, 2559 nt, Homo sapiens
  source 1..2559: mol_type = other RNA
tcaggccaggcacagtggctcatgcctgtaatcccagcactttgggaggcagaggcagtcaggtcccttgaggtcaggagttcgagaccagcctggccaacatggtgaaaccctgtctccaccaaaagtacaaaaatttgtcgggggtggtggtgcatgactgtagtcccagctacttgggaggctgaggcaggagaatcgcttgaacccgagaggcagaggttgcagtgagccgagatcgtgccacttcaccccagcctgggcaacaaactgagactgtgcctcaaaaataaataaataaataaaataaaaataaataaataagtgtttagtaagttttctttaaatgaatgaaggtagaaattacagcttttctgagactgttttcaagtctttggctatgtgcataagagcagttaccacattacaaaggctctccagagagttgggtgggataatgggtatcagaggtctttgtaaatttaacatttgtagccaaattttgcaaggacacaaatttggcctgagaaaggaggaagaggctccggcatactggagtccttgcccatgccaggtgtcttttctgcatggcagggtcccaggacctggggcagcagtctgattccagctccccatctgaactctatctcagcccagcccagactccttgcaatgtcttacttccagttgttgctaaaaatctgatacattttattttatgacagcaccaaactcattggtcttccctatcttgataaatagcaactcaatttttcccatcactcaggccaaaacttggagtcattcccaacatctctctctatatcactcctcacatccaattgatcagtaaatccttctaactatatccagcatccagcttatcacacttctatcactaccatgctatccaagcagtccccccaccccacccccaaccaaacatgtcacctggtacaccaacatgatttctctctaaagagaaatctcttttcaacaagccatttgcctggatctaacatcaaagtctgaatacaatttctgaccctgccaccagtatcattttgcaacattttccacagactatataatctaatattatatgatgagtaggcgtgatgcaggcctggtggcaccacactgcagccatgtcataacgacaagtctatgagcatatttgtctcctgcgtcacaagacccaggcctgactagggtctaccatgacaagcaacacttggaactactaacctgtatgtgacaggaagggggaacaccatcaaacgctgaagtttataaaacagaaaaagtgagtatacatgatcctctatgatatcacaccattgaattaacctatcctgaaactgccagacttcttgtgtcagataattaaactcttattgcttaaaccacttattagtttttctgttgcagccaaaaacatccttcatccttatcaacacatctgctattggtaagtgttcattaaatgaacagctaaaactagaaaggattatggcaatttttaaaaaatcaaatacagttagtcagttaaaatacaataataaaactattccagaaacacaatagagaaataggatacatgatgctactaaaaatctcagattagatagtcattaatattaaatctaaagttcctgactccagagggaaaaaagaagaataccaacattttaggagagaaaaacgttttcctgatactaatcctatgtgaaatctaccatgagaagataagggatatagaataacattatagaggcaatgtttctatggcaaagattgttcatgctcgccaaatatccaagtgttccatatcccagaccccatgaatcccagtgggatcatgtcactaattcttaacaatggaatgtgagctaaagtgatgtatcatttgtgatccaggaaggatgcacttctccacaccttctggatctcctgtccatacagctggaaacaaaatgctctcaagatgacagtttccaaataaaagcaacttggatccctgagctgtcacttgatggaaagccaagcaggagaccaacccaatctacatcagattgtgatactaaaaagaaataaatcttgttgtgttaagccactgagattttcgggtttatctgttccactgaatagctcagcttagcctggctactacagtatccaacaataactttacactctacttaagatttttagaatcaagaatgccatttggaagagacagatggttgaggtttaattcttctaagttgaacacatccttccttttcataacaatcctagttcctcttccaaacacaacgcagaaatgcacaccatgatttggtatcttcttgagtccagtaattatcctatctctctaagagctgtcctttctcagggaactcttgttcacatccgttctgtttcatcctttcaatgcagcatttaagaagcaggtacctccggatccacgccaccgcccccacgggttccgcccctcgagggtggtgccccccgagcccgcccctaaggacgcggcgctgcgaggtggtccggaac

SEQ ID NO: 17517 - RNA, 2651 nt, Homo sapiens
  source 1..2651: mol_type = other RNA
tcaggccaggcacagtggctcatgcctgtaatcccagcactttgggaggcagaggcagtcaggtcccttgaggtcaggagttcgagaccagcctggccaacatggtgaaaccctgtctccaccaaaagtacaaaaatttgtcgggggtggtggtgcatgactgtagtcccagctacttgggaggctgaggcaggagaatcgcttgaacccgagaggcagaggttgcagtgagccgagatcgtgccacttcaccccagcctgggcaacaaactgagactgtgcctcaaaaataaataaataaataaaataaaaataaataaataagtgtttagtaagttttctttaaatgaatgaaggtagaaattacagcttttctgagactgttttcaagtctttggctatgtgcataagagcagttaccacattacaaaggctctccagagagttgggtgggataatgggtatcagaggtctttgtaaatttaacatttgtagccaaattttgcaaggacacaaatttggcctgagaaaggaggaagaggctccggcatactggagtccttgcccatgccaggtgtcttttctgcatggcagggtcccaggacctggggcagcagtctgattccagctccccatctgaactctatctcagcccagcccagactccttgcaatgtcttacttccagttgttgctaaaaatctgatacattttattttatgacagcaccaaactcattggtcttccctatcttgataaatagcaactcaatttttcccatcactcaggccaaaacttggagtcattcccaacatctctctctatatcactcctcacatccaattgatcagtaaatccttctaactatatccagcatccagcttatcacacttctatcactaccatgctatccaagcagtccccccaccccacccccaaccaaacatgtcacctggtacaccaacatgatttctctctaaagagaaatctcttttcaacaagccatttgcctggatctaacatcaaagtctgaatacaatttctgaccctgccaccagtatcattttgcaacattttccacagactatataatctaatattatatgatgagtaggcgtgatgcaggcctggtggcaccacactgcagccatgtcataacgacaagtctatgagcatatttgtctcctgcgtcacaagacccaggcctgactagggtctaccatgacaagcaacacttggaactactaacctgtatgtgacaggaagggggaacaccatcaaacgctgaagtttataaaacagaaaaagtgagtatacatgatcctctatgatatcacaccattgaattaacctatcctgaaactgccagacttcttgtgtcagataattaaactcttattgcttaaaccacttattagtttttctgttgcagccaaaaacatccttcatccttatcaacacatctgctattggtaagtgttcattaaatgaacagctaaaactagaaaggattatggcaatttttaaaaaatcaaatacagttagtcagttaaaatacaataataaaactattccagaaacacaatagagaaataggatacatgatgctactaaaaatctcagattagatagtcattaatattaaatctaaagttcctgactccagagggaaaaaagaagaataccaacattttaggagagaaaaacgttttcctgatactaatcctatgtgaaatctaccatgagaagataagggatatagaataacattatagaggcaatgtttctatggcaaagattgttcatgctcgccaaatatccaagtgttccatatcccagaccccatgaatcccagtgggatcatgtcactaattcttaacaatggaatgtgagctaaagtgatgtatcatttgtgatccaggaaggatgcacttctccacaccttctggatctcctgtccatacagctggaaacaaaatgctctcaagatgacagtttccaaataaaagcaacttggatccctgagctgtcacttgatggaaagccaagcaggagaccaacccaatctacatcagattgtgatactaaaaagaaataaatcttgttgtgttaagccactgagattttcgggtttatctgttccactgaatagctcagcttagcctggctactacagtatccaacaataactttacactctacttaagatttttagaatcaagaatgccatttggaagagacagatggttgaggtttaattcttctaagttgaacacatccttccttttcataacaatcctagttcctcttccaaacacaacgcagaaatgcacaccatgatttggtatcttcttgagtccagtaattatcctatctctctaagagctgtcctttctcagggaactcttgttcacatccgttctgtttcatcctttcaatgcagcatttaagaagccaactggaaggctagctgatcctgctgctttcacaatatttttgcattggccttagattgaatctttcatgcaagcatcttgctcagaaaccaggtacctccggatccacgccaccgcccccacgggttccgcccctcgagggtggtgccccccgagcccgcccctaaggacgcggcgctgcgaggtggtccggaac

SEQ ID NO: 17518 - RNA, 2725 nt, Homo sapiens
  source 1..2725: mol_type = other RNA
tcaggccaggcacagtggctcatgcctgtaatcccagcactttgggaggcagaggcagtcaggtcccttgaggtcaggagttcgagaccagcctggccaacatggtgaaaccctgtctccaccaaaagtacaaaaatttgtcgggggtggtggtgcatgactgtagtcccagctacttgggaggctgaggcaggagaatcgcttgaacccgagaggcagaggttgcagtgagccgagatcgtgccacttcaccccagcctgggcaacaaactgagactgtgcctcaaaaataaataaataaataaaataaaaataaataaataagtgtttagtaagttttctttaaatgaatgaaggtagaaattacagcttttctgagactgttttcaagtctttggctatgtgcataagagcagttaccacattacaaaggctctccagagagttgggtgggataatgggtatcagaggtctttgtaaatttaacatttgtagccaaattttgcaaggacacaaatttggcctgagaaaggaggaagaggctccggcatactggagtccttgcccatgccaggtgtcttttctgcatggcagggtcccaggacctggggcagcagtctgattccagctccccatctgaactctatctcagcccagcccagactccttgcaatgtcttacttccagttgttgctaaaaatctgatacattttattttatgacagcaccaaactcattggtcttccctatcttgataaatagcaactcaatttttcccatcactcaggccaaaacttggagtcattcccaacatctctctctatatcactcctcacatccaattgatcagtaaatccttctaactatatccagcatccagcttatcacacttctatcactaccatgctatccaagcagtccccccaccccacccccaaccaaacatgtcacctggtacaccaacatgatttctctctaaagagaaatctcttttcaacaagccatttgcctggatctaacatcaaagtctgaatacaatttctgaccctgccaccagtatcattttgcaacattttccacagactatataatctaatattatatgatgagtaggcgtgatgcaggcctggtggcaccacactgcagccatgtcataacgacaagtctatgagcatatttgtctcctgcgtcacaagacccaggcctgactagggtctaccatgacaagcaacacttggaactactaacctgtatgtgacaggaagggggaacaccatcaaacgctgaagtttataaaacagaaaaagtgagtatacatgatcctctatgatatcacaccattgaattaacctatcctgaaactgccagacttcttgtgtcagataattaaactcttattgcttaaaccacttattagtttttctgttgcagccaaaaacatccttcatccttatcaacacatctgctattggtaagtgttcattaaatgaacagctaaaactagaaaggattatggcaatttttaaaaaatcaaatacagttagtcagttaaaatacaataataaaactattccagaaacacaatagagaaataggatacatgatgctactaaaaatctcagattagatagtcattaatattaaatctaaagttcctgactccagagggaaaaaagaagaataccaacattttaggagagaaaaacgttttcctgatactaatcctatgtgaaatctaccatgagaagataagggatatagaataacattatagaggcaatgtttctatggcaaagattgttcatgctcgccaaatatccaagtgttccatatcccagaccccatgaatcccagtgggatcatgtcactaattcttaacaatggaatgtgagctaaagtgatgtatcatttgtgatccaggaaggatgcacttctccacaccttctggatctcctgtccatacagctggaaacaaaatgctctcaagatgacagtttccaaataaaagcaacttggatccctgagctgtcacttgatggaaagccaagcaggagaccaacccaatctacatcagattgtgatactaaaaagaaataaatcttgttgtgttaagccactgagattttcgggtttatctgttccactgaatagctcagcttagcctggctactacagtatccaacaataactttacactctacttaagatttttagaatcaagaatgccatttggaagagacagatggttgaggtttaattcttctaagttgaacacatccttccttttcataacaatcctagttcctcttccaaacacaacgcagaaatgcacaccatgatttggtatcttcttgagtccagtaattatcctatctctctaagagctgtcctttctcagggaactcttgttcacatccgttctgtttcatcctttcaatgcagcatttaagaagccaactggaaggctagctgatcctgctgctttcacaatatttttgcattggccttagattgaatctttcatgcaagcatcttgctcagaaacctgaaaggagagagaatgaggacttcactgtgcttatatgaactggctatataattgtttttgtgcttgcggaacaatagatccttgtacctgaggcaaaatttgattcaaagcttgcttttatcaaaaaatagctctaggtagcaaggttgtagcaaaggagatacagcttccacccac
